European Patent Application EP 4 520 821 A1 - sequence listing, part 13

SEQ ID NO: 17519 - RNA, 5308 nt, Homo sapiens
  source 1..5308: mol_type = other RNA
tcaggccaggcacagtggctcatgcctgtaatcccagcactttgggaggccaaggcaggcagatcacctgaggttgggagttcgggaccagcctgaccaacacggagaaaccccgcctcttctaaaaatacaaaattggctgggcgtggtggtgcatgcctgtaatcccagctactcgggaggctgagacatgagaatagcttgaacccaggaggcagaggttgtggtgagccgagattgtgccattgcactcctgcttgggcaacaaaagcaaaactcttgtctaaaaaaaaaaaaaaagacaccactacacacctatcagaatagttcaaaatactgccaacatgaagtggtggcaaagatacagagcaatgggaacccatacaatgctggtgagaatgcaaaatgtacaggcactttggaaatcattttggcagtttcttataaaattaggtgcacacttaaccatgtgatccagcaatccctctggataaaatatcaggcaaaaacctgttatgttaatgttttaacaactttatacacaatcgctaaaaagtggaaacaaaccaattatctctcaaatagtgaatggataaactgtagtctatccatatgagagaacactacttagcaataaagaggaatgaactagagggatgaatataaagggacagtgggagatcttgtgggtgatgaaaccgttctgtatctagattatggaatagtgtttcactacatgataattttaaagaactttatagtattaaagagctaaacactattaaataatcaaatgtatgcagccttcaggtatttctattttaactaacattggatttcagagaacagactgaaaacactattgttcatcctttccctgctgagtagtgcagtgttcattttacaatttcatttaaattgaggttaagttacatacagaacagaattgccagatttagcagacagaggaacctggttaagtttaatttcaaataaaaatttggtaggttccctactaccacccttggtagcttttttcttttatccttggttttcatcagttttacctgttacgttagttatgattttctttatttattccacttggggttcactcagtttattggatctgtgagttgatagctttaccaaatttgaggtaattctggcctgtaagttacttatattttcttctgccctattttccttctattcttctggaaatccagttacatatgttaaatagcttgatatttccccaaatggcattgaggctttctgttgtcttccttctaatcttttcttctcttttcctcagattggacaatttctttcatgtgtcatctctatgctacggttaaacccaaccattttcttttaatgttaccacattttgggtgagaatatatatctatattcattcattacaaccaccctacctttttgtccatgaacatagttctaaaaactgctttaaaaatccttgtctgccaattccaccatcatctagtttatgttcggatttttttttctgttgtctgctcttttttttttttttaaaccataagctataaactgtatttccttatttctctggataccctatagcattttattgtattccagtcattgtttatatgttatacagattcattttatcatactctgaagagtgctaagctttgatctcatttaaagtattggctaatcaccttgattttatattatgttaaaggtttcatccttagttttagcataaatctttagtcttgtgcacagcctttactaatacatggccattctggggtttgggaagctcaaggttctatcaagcccttctaacttgtcagaattcaaacttgaaactgtgtcttctattgcaatagaaaacagccgtctctgttcagcttcttgagccttccaactgtggctttccaccaaggtccttggagtcttcccggggcatgcacggtttgagagttagctaaggatttaaggagagatcatatgcagacaggaagcctcctccatttctgacaccttcatttctaggatctgctgctttaattttcagttcttctagcggcctttaattccatcctaacacctcaagccagtaagattgcaactttctcttgagttctagccacgccttaccacacagtctgggaaagaccgaaggggaaaaaccatatatagttcacagctggtttcagtgactccctagagtttttagaccattgtttattatattttgtccacagtttataattgggagggtttgtacattacaagctattacaccattaccaaaaccagaagtccttcattatatagttcttaaatgtttagtttaacatatgagaagaaaataatatacaactggtatttaaatgtacttggctctctccccttctgtgtctaacagattgaaaatgaggccaggcatagtggctcatgcctgtaatcccagcactttgggaggccaaggtgggtggatcacttgaggtcaggagttcaagaccagcctggccaacatggcgaaaccccatctctacacacacacacacaaaatagccaggtgtggtgccgccacatgactgtaatcccagctactcgggaggctgaggcaggataatcgcttgaacctgggaggcagaggttgcagtgagccaagattgcaccactacactctagcctgggctacagagtgagactgtgtctcaaaaataaataaataaataaataaaaaataataaagaaaaaagagatgtttcatatatatataaatatttcttatctcaaatgaagtaaaataagtcaaataatctttagctaattgatgatcccagggaatagggaaatctgttcaaatttcaatgaatttactaagtaaagagctcagaaaaattggttaggccatggaaatacttagagttgaaccaactgaactaggatataagaaagctatttctattcagaactgaaactctttgaaatgaaatataataaatggagtgttatttaatactagtaagaagagtgtgactactcgcacatatacaatggcatattaactgaattaagttatatggcatatcttgactaatccattgttgccttaaaacttacatttttaaaaattttattttgtagtcagcaagttttccatttgtctgcttggatgtgaaagatgctatttaaaaccaaacagcaactgtacaaggctggctgaacatttataattaaacaatcttataacctccaaaatacagcagagtatgagccacgtaattaggatgtcagctaaccaagacagtgaattcagaagaatgtcattttgtggcatgtgctcagctgagctttaagtcagactgctggatggaaatgtaatctttctacctttgtttatatacactaataccagctgctgtcaggacaactcctcatgcagtagggacagctaacttttttaaaaagaagaaaattataaacatattttgtgaacatttactaatcttttatttgcttttcttggcactcataacattttttaccctttaaaacagattcaagtgattcaaattccagttacctctaagttatattctgttaacaaccaccttgtataaattggtttcataaataaaaactgctcttaaatgattctgtcagtggatgtctatccacaagctttccagcctggtctgctttatgtgtacatcctgaaaatttgccaaaatagcagcaacaactgatgatatcatagggaaaaaactcactgccacaagaaaccaagcattgttgagtcaacttctttttggtcacttgttttatacttactagataagccaaaagacctgtttgttacacaaacatgcatgcatccaggtattaatccattctcacactgctatgaagaaatacccgagactgggtaattataaaagaggtttaattttcgactcacagttccacatggctgggaaggcctcaggaaacttaacaatcacggtggaaggcacctcttcacagggcggcaagagtgagaatgagagccagtaggggaaatgccaggcacttataaaaccatcagatctcatgaaagctcactatcatgagaatagcatgagggaaactgcccccatgattcaattacctaccacaacacctgggaattatgaggattaaaattcaagatgagacttgggtggggatacatccaaaccatatcaatccatatatggctgaaatttacatcagacaatggtaaatatctatgttcaaagtccattgatgctttgagattctgagctattttctggtatggaaaacagacttagcatctccatctccattggatgtatgctgcctcctgtgatgatcaaggaatgcaatggttctcccaagtccacagtgcacatttgccttaaagtgcctgctgcaattttctggtcgtcggctccaaccctggctaagccaacacaaagtgtctcctcggtaactgctggttcttctcctcgtattctttgattttgaacaatctccagaagctgctgggctgcttggtttacactcatataccgtggaggttcatagatcttccttcccttgattagattttccaaagactgctcctttactttgatgtctagtaaacataatgtgtgcatgccattttgtctgttcttcttcactttgtcaaagaagctttctggtctccaagtgtctgtccaaaaaacaatagaaactgtctctccaaacttatataactgtaaaccacagcagcctacagcattcattatggaggcattgtgaataactctataaggaattcccagctttgttgctcttagaacaagatcactgtgtgttgtggccccaaatggatcaccaaccacaaggaatgcaacatcactgatatcagcatcctttaaaatattatctgcttcttgttccacttcttctctatcagcaacaaccaattttcttccataaaactcttccaaggcttccttccctacagttaggactgaggtgtaggcttccagatacactcgactgcagcgtctaacaacttccaggcccttgactgtgatgtccttggcatctcccaggcccaacccgatgagataaagcatttcaaacttgaggagaagagagacagttttgcctcttgttacacaaacctaggagcagccaattacccgctgagagaatcgtaggtagttctctggcctttacaaattcttaactaccacctttccgcagaagcaactgcaaaagcgccggctccgtgcagagaaaa

SEQ ID NO: 17520 - RNA, 5088 nt, Homo sapiens
  source 1..5088: mol_type = other RNA
tcaggccaggcacagtggctcatgcctgtaatcccagcactttgggaggccaaggcaggcagatcacctgaggttgggagttcgggaccagcctgaccaacacggagaaaccccgcctcttctaaaaatacaaaattggctgggcgtggtggtgcatgcctgtaatcccagctactcgggaggctgagacatgagaatagcttgaacccaggaggcagaggttgtggtgagccgagattgtgccattgcactcctgcttgggcaacaaaagcaaaactcttgtctaaaaaaaaaaaaaaagacaccactacacacctatcagaatagttcaaaatactgccaacatgaagtggtggcaaagatacagagcaatgggaacccatacaatgctggtgagaatgcaaaatgtacaggcactttggaaatcattttggcagtttcttataaaattaggtgcacacttaaccatgtgatccagcaatccctctggataaaatatcaggcaaaaacctgttatgttaatgttttaacaactttatacacaatcgctaaaaagtggaaacaaaccaattatctctcaaatagtgaatggataaactgtagtctatccatatgagagaacactacttagcaataaagaggaatgaactagagggatgaatataaagggacagtgggagatcttgtgggtgatgaaaccgttctgtatctagattatggaatagtgtttcactacatgataattttaaagaactttatagtattaaagagctaaacactattaaataatcaaatgtatgcagccttcaggtatttctattttaactaacattggatttcagagaacagactgaaaacactattgttcatcctttccctgctgagtagtgcagtgttcattttacaatttcatttaaattgaggttaagttacatacagaacagaattgccagatttagcagacagaggaacctggttaagtttaatttcaaataaaaatttggtaggttccctactaccacccttggtagcttttttcttttatccttggttttcatcagttttacctgttacgttagttatgattttctttatttattccacttggggttcactcagtttattggatctgtgagttgatagctttaccaaatttgaggtaattctggcctgtaagttacttatattttcttctgccctattttccttctattcttctggaaatccagttacatatgttaaatagcttgatatttccccaaatggcattgaggctttctgttgtcttccttctaatcttttcttctcttttcctcagattggacaatttctttcatgtgtcatctctatgctacggttaaacccaaccattttcttttaatgttaccacattttgggtgagaatatatatctatattcattcattacaaccaccctacctttttgtccatgaacatagttctaaaaactgctttaaaaatccttgtctgccaattccaccatcatctagtttatgttcggatttttttttctgttgtctgctcttttttttttttttaaaccataagctataaactgtatttccttatttctctggataccctatagcattttattgtattccagtcattgtttatatgttatacagattcattttatcatactctgaagagtgctaagctttgatctcatttaaagtattggctaatcaccttgattttatattatgttaaaggtttcatccttagttttagcataaatctttagtcttgtgcacagcctttactaatacatggccattctggggtttgggaagctcaaggttctatcaagcccttctaacttgtcagaattcaaacttgaaactgtgtcttctattgcaatagaaaacagccgtctctgttcagcttcttgagccttccaactgtggctttccaccaaggtccttggagtcttcccggggcatgcacggtttgagagttagctaaggatttaaggagagatcatatgcagacaggaagcctcctccatttctgacaccttcatttctaggatctgctgctttaattttcagttcttctagcggcctttaattccatcctaacacctcaagccagtaagattgcaactttctcttgagttctagccacgccttaccacacagtctgggaaagaccgaaggggaaaaaccatatatagttcacagctggtttcagtgactccctagagtttttagaccattgtttattatattttgtccacagtttataattgggagggtttgtacattacaagctattacaccattaccaaaaccagaagtccttcattatatagttcttaaatgtttagtttaacatatgagaagaaaataatatacaactggtatttaaatgtacttggctctctccccttctgtgtctaacagattgaaaatgaggccaggcatagtggctcatgcctgtaatcccagcactttgggaggccaaggtgggtggatcacttgaggtcaggagttcaagaccagcctggccaacatggcgaaaccccatctctacacacacacacacaaaatagccaggtgtggtgccgccacatgactgtaatcccagctactcgggaggctgaggcaggataatcgcttgaacctgggaggcagaggttgcagtgagccaagattgcaccactacactctagcctgggctacagagtgagactgtgtctcaaaaataaataaataaataaataaaaaataataaagaaaaaagagatgtttcatatatatataaatatttcttatctcaaatgaagtaaaataagtcaaataatctttagctaattgatgatcccagggaatagggaaatctgttcaaatttcaatgaatttactaagtaaagagctcagaaaaattggttaggccatggaaatacttagagttgaaccaactgaactaggatataagaaagctatttctattcagaactgaaactctttgaaatgaaatataataaatggagtgttatttaatactagtaagaagagtgtgactactcgcacatatacaatggcatattaactgaattaagttatatggcatatcttgactaatccattgttgccttaaaacttacatttttaaaaattttattttgtagtcagcaagttttccatttgtctgcttggatgtgaaagatgctatttaaaaccaaacagcaactgtacaaggctggctgaacatttataattaaacaatcttataacctccaaaatacagcagagtatgagccacgtaattaggatgtcagctaaccaagacagtgaattcagaagaatgtcattttgtggcatgtgctcagctgagctttaagtcagactgctggatggaaatgtaatctttctacctttgtttatatacactaataccagctgctgtcaggacaactcctcatgcagtagggacagctaacttttttaaaaagaagaaaattataaacatattttgtgaacatttactaatcttttatttgcttttcttggcactcataacattttttaccctttaaaacagattcaagtgattcaaattccagttacctctaagttatattctgttaacaaccaccttgtataaattggtttcataaataaaaactgctcttaaatgattctgtcagtggatgtctatccacaagctttccagcctggtctgctttatgtgtacatcctgaaaatttgccaaaatagcagcaacaactgatgatatcatagggaaaaaactcactgccacaagaaaccaagcattgttgagtcaacttctttttggtcacttgttttatacttactagataagccaaaagacctgtttgttacacaaacatgcatgcatccaggtattaatccattctcacactgctatgaagaaatacccgagactgggtaattataaaagaggtttaattttcgactcacagttccacatggctgggaaggcctcaggaaacttaacaatcacggtggaaggcacctcttcacagggcggcaagagtgagaatgagagccagtaggggaaatgccaggcacttataaaaccatcagatctcatgaaagctcactatcatgagaatagcatgagggaaactgcccccatgattcaattacctaccacaacacctgggaattatgaggattaaaattcaagatgagacttgggtggggatacatccaaaccatatcaatccatatatggctgaaatttacatcagacaatggtaaatatctatgttcaaagtccattgatgctttgagattctgagctattttctggtatggaaaacagacttagcatctccatctccattggatgtatgctgcctcctgtgatgatcaaggaatgcaatggttctcccaagtccacagtgcacatttgccttaaagtgcctgctgcaattttctggtcgtcggctccaaccctggctaagccaacacaaagtgtctcctcggtaactgctggttcttctcctcgtattctttgattttgaacaatctccagaagctgctgggctgcttggtttacactcatataccgtggaggttcatagatcttccttcccttgattagattttccaaagactgctcctttactttgatgtctagtaaacataatgtgtgcatgccattttgtctgttcttcttcactttgtcaaagaagctttctggtctccaagtgtctgtccaaaaaacaatagaaactgtctctccaaacttatataactgtaaaccacagcagcctacagcattcattatggaggcattgtgaataactctataaggaattcccagctttgttgctcttagaacaagatcactgtgtgttgtggccccaaatggatcaccaaccacaaggaatgcaacatcactgatatcagcatcctttaaaatattatctgcttcttgttccacttcttctctatcagcaacaaccaattttcttccataaaactcttccagttttgcctcttgttacacaaacctaggagcagccaattacccgctgagagaatcgtaggtagttctctggcctttacaa

SEQ ID NO: 17521 - RNA, 5115 nt, Homo sapiens
  source 1..5115: mol_type = other RNA
tcaggccaggcacagtggctcatgcctgtaatcccagcactttgggaggccaaggcaggcagatcacctgaggttgggagttcgggaccagcctgaccaacacggagaaaccccgcctcttctaaaaatacaaaattggctgggcgtggtggtgcatgcctgtaatcccagctactcgggaggctgagacatgagaatagcttgaacccaggaggcagaggttgtggtgagccgagattgtgccattgcactcctgcttgggcaacaaaagcaaaactcttgtctaaaaaaaaaaaaaaagacaccactacacacctatcagaatagttcaaaatactgccaacatgaagtggtggcaaagatacagagcaatgggaacccatacaatgctggtgagaatgcaaaatgtacaggcactttggaaatcattttggcagtttcttataaaattaggtgcacacttaaccatgtgatccagcaatccctctggataaaatatcaggcaaaaacctgttatgttaatgttttaacaactttatacacaatcgctaaaaagtggaaacaaaccaattatctctcaaatagtgaatggataaactgtagtctatccatatgagagaacactacttagcaataaagaggaatgaactagagggatgaatataaagggacagtgggagatcttgtgggtgatgaaaccgttctgtatctagattatggaatagtgtttcactacatgataattttaaagaactttatagtattaaagagctaaacactattaaataatcaaatgtatgcagccttcaggtatttctattttaactaacattggatttcagagaacagactgaaaacactattgttcatcctttccctgctgagtagtgcagtgttcattttacaatttcatttaaattgaggttaagttacatacagaacagaattgccagatttagcagacagaggaacctggttaagtttaatttcaaataaaaatttggtaggttccctactaccacccttggtagcttttttcttttatccttggttttcatcagttttacctgttacgttagttatgattttctttatttattccacttggggttcactcagtttattggatctgtgagttgatagctttaccaaatttgaggtaattctggcctgtaagttacttatattttcttctgccctattttccttctattcttctggaaatccagttacatatgttaaatagcttgatatttccccaaatggcattgaggctttctgttgtcttccttctaatcttttcttctcttttcctcagattggacaatttctttcatgtgtcatctctatgctacggttaaacccaaccattttcttttaatgttaccacattttgggtgagaatatatatctatattcattcattacaaccaccctacctttttgtccatgaacatagttctaaaaactgctttaaaaatccttgtctgccaattccaccatcatctagtttatgttcggatttttttttctgttgtctgctcttttttttttttttaaaccataagctataaactgtatttccttatttctctggataccctatagcattttattgtattccagtcattgtttatatgttatacagattcattttatcatactctgaagagtgctaagctttgatctcatttaaagtattggctaatcaccttgattttatattatgttaaaggtttcatccttagttttagcataaatctttagtcttgtgcacagcctttactaatacatggccattctggggtttgggaagctcaaggttctatcaagcccttctaacttgtcagaattcaaacttgaaactgtgtcttctattgcaatagaaaacagccgtctctgttcagcttcttgagccttccaactgtggctttccaccaaggtccttggagtcttcccggggcatgcacggtttgagagttagctaaggatttaaggagagatcatatgcagacaggaagcctcctccatttctgacaccttcatttctaggatctgctgctttaattttcagttcttctagcggcctttaattccatcctaacacctcaagccagtaagattgcaactttctcttgagttctagccacgccttaccacacagtctgggaaagaccgaaggggaaaaaccatatatagttcacagctggtttcagtgactccctagagtttttagaccattgtttattatattttgtccacagtttataattgggagggtttgtacattacaagctattacaccattaccaaaaccagaagtccttcattatatagttcttaaatgtttagtttaacatatgagaagaaaataatatacaactggtatttaaatgtacttggctctctccccttctgtgtctaacagattgaaaatgaggccaggcatagtggctcatgcctgtaatcccagcactttgggaggccaaggtgggtggatcacttgaggtcaggagttcaagaccagcctggccaacatggcgaaaccccatctctacacacacacacacaaaatagccaggtgtggtgccgccacatgactgtaatcccagctactcgggaggctgaggcaggataatcgcttgaacctgggaggcagaggttgcagtgagccaagattgcaccactacactctagcctgggctacagagtgagactgtgtctcaaaaataaataaataaataaataaaaaataataaagaaaaaagagatgtttcatatatatataaatatttcttatctcaaatgaagtaaaataagtcaaataatctttagctaattgatgatcccagggaatagggaaatctgttcaaatttcaatgaatttactaagtaaagagctcagaaaaattggttaggccatggaaatacttagagttgaaccaactgaactaggatataagaaagctatttctattcagaactgaaactctttgaaatgaaatataataaatggagtgttatttaatactagtaagaagagtgtgactactcgcacatatacaatggcatattaactgaattaagttatatggcatatcttgactaatccattgttgccttaaaacttacatttttaaaaattttattttgtagtcagcaagttttccatttgtctgcttggatgtgaaagatgctatttaaaaccaaacagcaactgtacaaggctggctgaacatttataattaaacaatcttataacctccaaaatacagcagagtatgagccacgtaattaggatgtcagctaaccaagacagtgaattcagaagaatgtcattttgtggcatgtgctcagctgagctttaagtcagactgctggatggaaatgtaatctttctacctttgtttatatacactaataccagctgctgtcaggacaactcctcatgcagtagggacagctaacttttttaaaaagaagaaaattataaacatattttgtgaacatttactaatcttttatttgcttttcttggcactcataacattttttaccctttaaaacagattcaagtgattcaaattccagttacctctaagttatattctgttaacaaccaccttgtataaattggtttcataaataaaaactgctcttaaatgattctgtcagtggatgtctatccacaagctttccagcctggtctgctttatgtgtacatcctgaaaatttgccaaaatagcagcaacaactgatgatatcatagggaaaaaactcactgccacaagaaaccaagcattgttgagtcaacttctttttggtcacttgttttatacttactagataagccaaaagacctgtttgttacacaaacatgcatgcatccaggtattaatccattctcacactgctatgaagaaatacccgagactgggtaattataaaagaggtttaattttcgactcacagttccacatggctgggaaggcctcaggaaacttaacaatcacggtggaaggcacctcttcacagggcggcaagagtgagaatgagagccagtaggggaaatgccaggcacttataaaaccatcagatctcatgaaagctcactatcatgagaatagcatgagggaaactgcccccatgattcaattacctaccacaacacctgggaattatgaggattaaaattcaagatgagacttgggtggggatacatccaaaccatatcaatccatatatggctgaaatttacatcagacaatggtaaatatctatgttcaaagtccattgatgctttgagattctgagctattttctggtatggaaaacagacttagcatctccatctccattggatgtatgctgcctcctgtgatgatcaaggaatgcaatggttctcccaagtccacagtgcacatttgccttaaagtgcctgctgcaattttctggtcgtcggctccaaccctggctaagccaacacaaagtgtctcctcggtaactgctggttcttctcctcgtattctttgattttgaacaatctccagaagctgctgggctgcttggtttacactcatataccgtggaggttcatagatcttccttcccttgattagattttccaaagactgctcctttactttgatgtctagtaaacataatgtgtgcatgccattttgtctgttcttcttcactttgtcaaagaagctttctggtctccaagtgtctgtccaaaaaacaatagaaactgtctctccaaacttatataactgtaaaccacagcagcctacagcattcattatggaggcattgtgaataactctataaggaattcccagctttgttgctcttagaacaagatcactgtgtgttgtggccccaaatggatcaccaaccacaaggaatgcaacatcactgatatcagcatcctttaaaatattatctgcttcttgttccacttcttctctatcagcaacaaccaattttcttccataaaactcttcccgctgagagaatcgtaggtagttctctggcctttacaaattcttaactaccacctttccgcagaagcaactgcaaaagcgccggctccgtgcagagaaaaggcccacg

SEQ ID NO: 17522 - RNA, 5095 nt, Homo sapiens
  source 1..5095: mol_type = other RNA
tcaggccaggcacagtggctcatgcctgtaatcccagcactttgggaggccaaggcaggcagatcacctgaggttgggagttcgggaccagcctgaccaacacggagaaaccccgcctcttctaaaaatacaaaattggctgggcgtggtggtgcatgcctgtaatcccagctactcgggaggctgagacatgagaatagcttgaacccaggaggcagaggttgtggtgagccgagattgtgccattgcactcctgcttgggcaacaaaagcaaaactcttgtctaaaaaaaaaaaaaaagacaccactacacacctatcagaatagttcaaaatactgccaacatgaagtggtggcaaagatacagagcaatgggaacccatacaatgctggtgagaatgcaaaatgtacaggcactttggaaatcattttggcagtttcttataaaattaggtgcacacttaaccatgtgatccagcaatccctctggataaaatatcaggcaaaaacctgttatgttaatgttttaacaactttatacacaatcgctaaaaagtggaaacaaaccaattatctctcaaatagtgaatggataaactgtagtctatccatatgagagaacactacttagcaataaagaggaatgaactagagggatgaatataaagggacagtgggagatcttgtgggtgatgaaaccgttctgtatctagattatggaatagtgtttcactacatgataattttaaagaactttatagtattaaagagctaaacactattaaataatcaaatgtatgcagccttcaggtatttctattttaactaacattggatttcagagaacagactgaaaacactattgttcatcctttccctgctgagtagtgcagtgttcattttacaatttcatttaaattgaggttaagttacatacagaacagaattgccagatttagcagacagaggaacctggttaagtttaatttcaaataaaaatttggtaggttccctactaccacccttggtagcttttttcttttatccttggttttcatcagttttacctgttacgttagttatgattttctttatttattccacttggggttcactcagtttattggatctgtgagttgatagctttaccaaatttgaggtaattctggcctgtaagttacttatattttcttctgccctattttccttctattcttctggaaatccagttacatatgttaaatagcttgatatttccccaaatggcattgaggctttctgttgtcttccttctaatcttttcttctcttttcctcagattggacaatttctttcatgtgtcatctctatgctacggttaaacccaaccattttcttttaatgttaccacattttgggtgagaatatatatctatattcattcattacaaccaccctacctttttgtccatgaacatagttctaaaaactgctttaaaaatccttgtctgccaattccaccatcatctagtttatgttcggatttttttttctgttgtctgctcttttttttttttttaaaccataagctataaactgtatttccttatttctctggataccctatagcattttattgtattccagtcattgtttatatgttatacagattcattttatcatactctgaagagtgctaagctttgatctcatttaaagtattggctaatcaccttgattttatattatgttaaaggtttcatccttagttttagcataaatctttagtcttgtgcacagcctttactaatacatggccattctggggtttgggaagctcaaggttctatcaagcccttctaacttgtcagaattcaaacttgaaactgtgtcttctattgcaatagaaaacagccgtctctgttcagcttcttgagccttccaactgtggctttccaccaaggtccttggagtcttcccggggcatgcacggtttgagagttagctaaggatttaaggagagatcatatgcagacaggaagcctcctccatttctgacaccttcatttctaggatctgctgctttaattttcagttcttctagcggcctttaattccatcctaacacctcaagccagtaagattgcaactttctcttgagttctagccacgccttaccacacagtctgggaaagaccgaaggggaaaaaccatatatagttcacagctggtttcagtgactccctagagtttttagaccattgtttattatattttgtccacagtttataattgggagggtttgtacattacaagctattacaccattaccaaaaccagaagtccttcattatatagttcttaaatgtttagtttaacatatgagaagaaaataatatacaactggtatttaaatgtacttggctctctccccttctgtgtctaacagattgaaaatgaggccaggcatagtggctcatgcctgtaatcccagcactttgggaggccaaggtgggtggatcacttgaggtcaggagttcaagaccagcctggccaacatggcgaaaccccatctctacacacacacacacaaaatagccaggtgtggtgccgccacatgactgtaatcccagctactcgggaggctgaggcaggataatcgcttgaacctgggaggcagaggttgcagtgagccaagattgcaccactacactctagcctgggctacagagtgagactgtgtctcaaaaataaataaataaataaataaaaaataataaagaaaaaagagatgtttcatatatatataaatatttcttatctcaaatgaagtaaaataagtcaaataatctttagctaattgatgatcccagggaatagggaaatctgttcaaatttcaatgaatttactaagtaaagagctcagaaaaattggttaggccatggaaatacttagagttgaaccaactgaactaggatataagaaagctatttctattcagaactgaaactctttgaaatgaaatataataaatggagtgttatttaatactagtaagaagagtgtgactactcgcacatatacaatggcatattaactgaattaagttatatggcatatcttgactaatccattgttgccttaaaacttacatttttaaaaattttattttgtagtcagcaagttttccatttgtctgcttggatgtgaaagatgctatttaaaaccaaacagcaactgtacaaggctggctgaacatttataattaaacaatcttataacctccaaaatacagcagagtatgagccacgtaattaggatgtcagctaaccaagacagtgaattcagaagaatgtcattttgtggcatgtgctcagctgagctttaagtcagactgctggatggaaatgtaatctttctacctttgtttatatacactaataccagctgctgtcaggacaactcctcatgcagtagggacagctaacttttttaaaaagaagaaaattataaacatattttgtgaacatttactaatcttttatttgcttttcttggcactcataacattttttaccctttaaaacagattcaagtgattcaaattccagttacctctaagttatattctgttaacaaccaccttgtataaattggtttcataaataaaaactgctcttaaatgattctgtcagtggatgtctatccacaagctttccagcctggtctgctttatgtgtacatcctgaaaatttgccaaaatagcagcaacaactgatgatatcatagggaaaaaactcactgccacaagaaaccaagcattgttgagtcaacttctttttggtcacttgttttatacttactagataagccaaaagacctgtttgttacacaaacatgcatgcatccaggtattaatccattctcacactgctatgaagaaatacccgagactgggtaattataaaagaggtttaattttcgactcacagttccacatggctgggaaggcctcaggaaacttaacaatcacggtggaaggcacctcttcacagggcggcaagagtgagaatgagagccagtaggggaaatgccaggcacttataaaaccatcagatctcatgaaagctcactatcatgagaatagcatgagggaaactgcccccatgattcaattacctaccacaacacctgggaattatgaggattaaaattcaagatgagacttgggtggggatacatccaaaccatatcaatccatatatggctgaaatttacatcagacaatggtaaatatctatgttcaaagtccattgatgctttgagattctgagctattttctggtatggaaaacagacttagcatctccatctccattggatgtatgctgcctcctgtgatgatcaaggaatgcaatggttctcccaagtccacagtgcacatttgccttaaagtgcctgctgcaattttctggtcgtcggctccaaccctggctaagccaacacaaagtgtctcctcggtaactgctggttcttctcctcgtattctttgattttgaacaatctccagaagctgctgggctgcttggtttacactcatataccgtggaggttcatagatcttccttcccttgattagattttccaaagactgctcctttactttgatgtctagtaaacataatgtgtgcatgccattttgtctgttcttcttcactttgtcaaagaagctttctggtctccaagtgtctgtccaaaaaacaatagaaactgtctctccaaacttatataactgtaaaccacagcagcctacagcattcattatggaggcattgtgaataactctataaggaattcccagctttgttgctcttagaacaagatcactgtgtgttgtggccccaaatggatcaccaaccacaaggaatgcaacatcactgatatcagcatcctttaaaatattatctgcttcttgttccacttcttctctatcagcaacaaccaattttcttccataaaactcttcctaggagcagccaattacccgctgagagaatcgtaggtagttctctggcctttacaaattcttaactaccacctttccgcagaagcaac

SEQ ID NO: 17523 - RNA, 5204 nt, Homo sapiens
  source 1..5204: mol_type = other RNA
tcaggccaggcacagtggctcatgcctgtaatcccagcactttgggaggccaaggcaggcagatcacctgaggttgggagttcgggaccagcctgaccaacacggagaaaccccgcctcttctaaaaatacaaaattggctgggcgtggtggtgcatgcctgtaatcccagctactcgggaggctgagacatgagaatagcttgaacccaggaggcagaggttgtggtgagccgagattgtgccattgcactcctgcttgggcaacaaaagcaaaactcttgtctaaaaaaaaaaaaaaagacaccactacacacctatcagaatagttcaaaatactgccaacatgaagtggtggcaaagatacagagcaatgggaacccatacaatgctggtgagaatgcaaaatgtacaggcactttggaaatcattttggcagtttcttataaaattaggtgcacacttaaccatgtgatccagcaatccctctggataaaatatcaggcaaaaacctgttatgttaatgttttaacaactttatacacaatcgctaaaaagtggaaacaaaccaattatctctcaaatagtgaatggataaactgtagtctatccatatgagagaacactacttagcaataaagaggaatgaactagagggatgaatataaagggacagtgggagatcttgtgggtgatgaaaccgttctgtatctagattatggaatagtgtttcactacatgataattttaaagaactttatagtattaaagagctaaacactattaaataatcaaatgtatgcagccttcaggtatttctattttaactaacattggatttcagagaacagactgaaaacactattgttcatcctttccctgctgagtagtgcagtgttcattttacaatttcatttaaattgaggttaagttacatacagaacagaattgccagatttagcagacagaggaacctggttaagtttaatttcaaataaaaatttggtaggttccctactaccacccttggtagcttttttcttttatccttggttttcatcagttttacctgttacgttagttatgattttctttatttattccacttggggttcactcagtttattggatctgtgagttgatagctttaccaaatttgaggtaattctggcctgtaagttacttatattttcttctgccctattttccttctattcttctggaaatccagttacatatgttaaatagcttgatatttccccaaatggcattgaggctttctgttgtcttccttctaatcttttcttctcttttcctcagattggacaatttctttcatgtgtcatctctatgctacggttaaacccaaccattttcttttaatgttaccacattttgggtgagaatatatatctatattcattcattacaaccaccctacctttttgtccatgaacatagttctaaaaactgctttaaaaatccttgtctgccaattccaccatcatctagtttatgttcggatttttttttctgttgtctgctcttttttttttttttaaaccataagctataaactgtatttccttatttctctggataccctatagcattttattgtattccagtcattgtttatatgttatacagattcattttatcatactctgaagagtgctaagctttgatctcatttaaagtattggctaatcaccttgattttatattatgttaaaggtttcatccttagttttagcataaatctttagtcttgtgcacagcctttactaatacatggccattctggggtttgggaagctcaaggttctatcaagcccttctaacttgtcagaattcaaacttgaaactgtgtcttctattgcaatagaaaacagccgtctctgttcagcttcttgagccttccaactgtggctttccaccaaggtccttggagtcttcccggggcatgcacggtttgagagttagctaaggatttaaggagagatcatatgcagacaggaagcctcctccatttctgacaccttcatttctaggatctgctgctttaattttcagttcttctagcggcctttaattccatcctaacacctcaagccagtaagattgcaactttctcttgagttctagccacgccttaccacacagtctgggaaagaccgaaggggaaaaaccatatatagttcacagctggtttcagtgactccctagagtttttagaccattgtttattatattttgtccacagtttataattgggagggtttgtacattacaagctattacaccattaccaaaaccagaagtccttcattatatagttcttaaatgtttagtttaacatatgagaagaaaataatatacaactggtatttaaatgtacttggctctctccccttctgtgtctaacagattgaaaatgaggccaggcatagtggctcatgcctgtaatcccagcactttgggaggccaaggtgggtggatcacttgaggtcaggagttcaagaccagcctggccaacatggcgaaaccccatctctacacacacacacacaaaatagccaggtgtggtgccgccacatgactgtaatcccagctactcgggaggctgaggcaggataatcgcttgaacctgggaggcagaggttgcagtgagccaagattgcaccactacactctagcctgggctacagagtgagactgtgtctcaaaaataaataaataaataaataaaaaataataaagaaaaaagagatgtttcatatatatataaatatttcttatctcaaatgaagtaaaataagtcaaataatctttagctaattgatgatcccagggaatagggaaatctgttcaaatttcaatgaatttactaagtaaagagctcagaaaaattggttaggccatggaaatacttagagttgaaccaactgaactaggatataagaaagctatttctattcagaactgaaactctttgaaatgaaatataataaatggagtgttatttaatactagtaagaagagtgtgactactcgcacatatacaatggcatattaactgaattaagttatatggcatatcttgactaatccattgttgccttaaaacttacatttttaaaaattttattttgtagtcagcaagttttccatttgtctgcttggatgtgaaagatgctatttaaaaccaaacagcaactgtacaaggctggctgaacatttataattaaacaatcttataacctccaaaatacagcagagtatgagccacgtaattaggatgtcagctaaccaagacagtgaattcagaagaatgtcattttgtggcatgtgctcagctgagctttaagtcagactgctggatggaaatgtaatctttctacctttgtttatatacactaataccagctgctgtcaggacaactcctcatgcagtagggacagctaacttttttaaaaagaagaaaattataaacatattttgtgaacatttactaatcttttatttgcttttcttggcactcataacattttttaccctttaaaacagattcaagtgattcaaattccagttacctctaagttatattctgttaacaaccaccttgtataaattggtttcataaataaaaactgctcttaaatgattctgtcagtggatgtctatccacaagctttccagcctggtctgctttatgtgtacatcctgaaaatttgccaaaatagcagcaacaactgatgatatcatagggaaaaaactcactgccacaagaaaccaagcattgttgagtcaacttctttttggtcacttgttttatacttactagataagccaaaagacctgtttgttacacaaacatgcatgcatccaggtattaatccattctcacactgctatgaagaaatacccgagactgggtaattataaaagaggtttaattttcgactcacagttccacatggctgggaaggcctcaggaaacttaacaatcacggtggaaggcacctcttcacagggcggcaagagtgagaatgagagccagtaggggaaatgccaggcacttataaaaccatcagatctcatgaaagctcactatcatgagaatagcatgagggaaactgcccccatgattcaattacctaccacaacacctgggaattatgaggattaaaattcaagatgagacttgggtggggatacatccaaaccatatcaatccatatatggctgaaatttacatcagacaatggtaaatatctatgttcaaagtccattgatgctttgagattctgagctattttctggtatggaaaacagacttagcatctccatctccattggatgtatgctgcctcctgtgatgatcaaggaatgcaatggttctcccaagtccacagtgcacatttgccttaaagtgcctgctgcaattttctggtcgtcggctccaaccctggctaagccaacacaaagtgtctcctcggtaactgttgattagattttccaaagactgctcctttactttgatgtctagtaaacataatgtgtgcatgccattttgtctgttcttcttcactttgtcaaagaagctttctggtctccaagtgtctgtccaaaaaacaatagaaactgtctctccaaacttatataactgtaaaccacagcagcctacagcattcattatggaggcattgtgaataactctataaggaattcccagctttgttgctcttagaacaagatcactgtgtgttgtggccccaaatggatcaccaaccacaaggaatgcaacatcactgatatcagcatcctttaaaatattatctgcttcttgttccacttcttctctatcagcaacaaccaattttcttccataaaactcttccaaggcttccttccctacagttaggactgaggtgtaggcttccagatacactcgactgcagcgtctaacaacttccaggcccttgactgtgatgtccttggcatctcccaggcccaacccgatgagataaagcatttcaaacttgaggagaagagagacagttttgcctcttgttacacaaacctaggagcagccaattacccgctgagagaatcgtaggtagttctctggcctttacaaattcttaactaccacctttccgcagaagcaactgcaaaagcgccggctccgtgcagagaaaa

SEQ ID NO: 17524 - RNA, 5184 nt, Homo sapiens
  source 1..5184: mol_type = other RNA
tcaggccaggcacagtggctcatgcctgtaatcccagcactttgggaggccaaggcaggcagatcacctgaggttgggagttcgggaccagcctgaccaacacggagaaaccccgcctcttctaaaaatacaaaattggctgggcgtggtggtgcatgcctgtaatcccagctactcgggaggctgagacatgagaatagcttgaacccaggaggcagaggttgtggtgagccgagattgtgccattgcactcctgcttgggcaacaaaagcaaaactcttgtctaaaaaaaaaaaaaaagacaccactacacacctatcagaatagttcaaaatactgccaacatgaagtggtggcaaagatacagagcaatgggaacccatacaatgctggtgagaatgcaaaatgtacaggcactttggaaatcattttggcagtttcttataaaattaggtgcacacttaaccatgtgatccagcaatccctctggataaaatatcaggcaaaaacctgttatgttaatgttttaacaactttatacacaatcgctaaaaagtggaaacaaaccaattatctctcaaatagtgaatggataaactgtagtctatccatatgagagaacactacttagcaataaagaggaatgaactagagggatgaatataaagggacagtgggagatcttgtgggtgatgaaaccgttctgtatctagattatggaatagtgtttcactacatgataattttaaagaactttatagtattaaagagctaaacactattaaataatcaaatgtatgcagccttcaggtatttctattttaactaacattggatttcagagaacagactgaaaacactattgttcatcctttccctgctgagtagtgcagtgttcattttacaatttcatttaaattgaggttaagttacatacagaacagaattgccagatttagcagacagaggaacctggttaagtttaatttcaaataaaaatttggtaggttccctactaccacccttggtagcttttttcttttatccttggttttcatcagttttacctgttacgttagttatgattttctttatttattccacttggggttcactcagtttattggatctgtgagttgatagctttaccaaatttgaggtaattctggcctgtaagttacttatattttcttctgccctattttccttctattcttctggaaatccagttacatatgttaaatagcttgatatttccccaaatggcattgaggctttctgttgtcttccttctaatcttttcttctcttttcctcagattggacaatttctttcatgtgtcatctctatgctacggttaaacccaaccattttcttttaatgttaccacattttgggtgagaatatatatctatattcattcattacaaccaccctacctttttgtccatgaacatagttctaaaaactgctttaaaaatccttgtctgccaattccaccatcatctagtttatgttcggatttttttttctgttgtctgctcttttttttttttttaaaccataagctataaactgtatttccttatttctctggataccctatagcattttattgtattccagtcattgtttatatgttatacagattcattttatcatactctgaagagtgctaagctttgatctcatttaaagtattggctaatcaccttgattttatattatgttaaaggtttcatccttagttttagcataaatctttagtcttgtgcacagcctttactaatacatggccattctggggtttgggaagctcaaggttctatcaagcccttctaacttgtcagaattcaaacttgaaactgtgtcttctattgcaatagaaaacagccgtctctgttcagcttcttgagccttccaactgtggctttccaccaaggtccttggagtcttcccggggcatgcacggtttgagagttagctaaggatttaaggagagatcatatgcagacaggaagcctcctccatttctgacaccttcatttctaggatctgctgctttaattttcagttcttctagcggcctttaattccatcctaacacctcaagccagtaagattgcaactttctcttgagttctagccacgccttaccacacagtctgggaaagaccgaaggggaaaaaccatatatagttcacagctggtttcagtgactccctagagtttttagaccattgtttattatattttgtccacagtttataattgggagggtttgtacattacaagctattacaccattaccaaaaccagaagtccttcattatatagttcttaaatgtttagtttaacatatgagaagaaaataatatacaactggtatttaaatgtacttggctctctccccttctgtgtctaacagattgaaaatgaggccaggcatagtggctcatgcctgtaatcccagcactttgggaggccaaggtgggtggatcacttgaggtcaggagttcaagaccagcctggccaacatggcgaaaccccatctctacacacacacacacaaaatagccaggtgtggtgccgccacatgactgtaatcccagctactcgggaggctgaggcaggataatcgcttgaacctgggaggcagaggttgcagtgagccaagattgcaccactacactctagcctgggctacagagtgagactgtgtctcaaaaataaataaataaataaataaaaaataataaagaaaaaagagatgtttcatatatatataaatatttcttatctcaaatgaagtaaaataagtcaaataatctttagctaattgatgatcccagggaatagggaaatctgttcaaatttcaatgaatttactaagtaaagagctcagaaaaattggttaggccatggaaatacttagagttgaaccaactgaactaggatataagaaagctatttctattcagaactgaaactctttgaaatgaaatataataaatggagtgttatttaatactagtaagaagagtgtgactactcgcacatatacaatggcatattaactgaattaagttatatggcatatcttgactaatccattgttgccttaaaacttacatttttaaaaattttattttgtagtcagcaagttttccatttgtctgcttggatgtgaaagatgctatttaaaaccaaacagcaactgtacaaggctggctgaacatttataattaaacaatcttataacctccaaaatacagcagagtatgagccacgtaattaggatgtcagctaaccaagacagtgaattcagaagaatgtcattttgtggcatgtgctcagctgagctttaagtcagactgctggatggaaatgtaatctttctacctttgtttatatacactaataccagctgctgtcaggacaactcctcatgcagtagggacagctaacttttttaaaaagaagaaaattataaacatattttgtgaacatttactaatcttttatttgcttttcttggcactcataacattttttaccctttaaaacagattcaagtgattcaaattccagttacctctaagttatattctgttaacaaccaccttgtataaattggtttcataaataaaaactgctcttaaatgattctgtcagtggatgtctatccacaagctttccagcctggtctgctttatgtgtacatcctgaaaatttgccaaaatagcagcaacaactgatgatatcatagggaaaaaactcactgccacaagaaaccaagcattgttgagtcaacttctttttggtcacttgttttatacttactagataagccaaaagacctgtttgttacacaaacatgcatgcatccaggtattaatccattctcacactgctatgaagaaatacccgagactgggtaattataaaagaggtttaattttcgactcacagttccacatggctgggaaggcctcaggaaacttaacaatcacggtggaaggcacctcttcacagggcggcaagagtgagaatgagagccagtaggggaaatgccaggcacttataaaaccatcagatctcatgaaagctcactatcatgagaatagcatgagggaaactgcccccatgattcaattacctaccacaacacctgggaattatgaggattaaaattcaagatgagacttgggtggggatacatccaaaccatatcaatccatatatggctgaaatttacatcagacaatggtaaatatctatgttcaaagtccattgatgctttgagattctgagctattttctggtatggaaaacagacttagcatctccatctccattggatgtatgctgcctcctgtgatgatcaaggaatgcaatggttctcccaagtccacagtgcacatttgccttaaagtgcctgctgcaattttctggtcgtcggctccaaccctggctaagccaacacaaagtgtctcctcggtaactgttgattagattttccaaagactgctcctttactttgatgtctagtaaacataatgtgtgcatgccattttgtctgttcttcttcactttgtcaaagaagctttctggtctccaagtgtctgtccaaaaaacaatagaaactgtctctccaaacttatataactgtaaaccacagcagcctacagcattcattatggaggcattgtgaataactctataaggaattcccagctttgttgctcttagaacaagatcactgtgtgttgtggccccaaatggatcaccaaccacaaggaatgcaacatcactgatatcagcatcctttaaaatattatctgcttcttgttccacttcttctctatcagcaacaaccaattttcttccataaaactcttccaaggcttccttccctacagttaggactgaggtgtaggcttccagatacactcgactgcagcgtctaacaacttccaggcccttgactgtgatgtccttggcatctcccaggcccaacccgatgagataaagcatttcaaacttgaggagaagagagaccgctgagagaatcgtaggtagttctctggcctttacaaattcttaactaccacctttccgcagaagcaactgcaaaagcgccggctccgtgcagagaaaaggcccacgccgccggcctcacct

SEQ ID NO: 17525 - RNA, 5180 nt, Homo sapiens
  source 1..5180: mol_type = other RNA
tcaggccaggcacagtggctcatgcctgtaatcccagcactttgggaggccaaggcaggcagatcacctgaggttgggagttcgggaccagcctgaccaacacggagaaaccccgcctcttctaaaaatacaaaattggctgggcgtggtggtgcatgcctgtaatcccagctactcgggaggctgagacatgagaatagcttgaacccaggaggcagaggttgtggtgagccgagattgtgccattgcactcctgcttgggcaacaaaagcaaaactcttgtctaaaaaaaaaaaaaaagacaccactacacacctatcagaatagttcaaaatactgccaacatgaagtggtggcaaagatacagagcaatgggaacccatacaatgctggtgagaatgcaaaatgtacaggcactttggaaatcattttggcagtttcttataaaattaggtgcacacttaaccatgtgatccagcaatccctctggataaaatatcaggcaaaaacctgttatgttaatgttttaacaactttatacacaatcgctaaaaagtggaaacaaaccaattatctctcaaatagtgaatggataaactgtagtctatccatatgagagaacactacttagcaataaagaggaatgaactagagggatgaatataaagggacagtgggagatcttgtgggtgatgaaaccgttctgtatctagattatggaatagtgtttcactacatgataattttaaagaactttatagtattaaagagctaaacactattaaataatcaaatgtatgcagccttcaggtatttctattttaactaacattggatttcagagaacagactgaaaacactattgttcatcctttccctgctgagtagtgcagtgttcattttacaatttcatttaaattgaggttaagttacatacagaacagaattgccagatttagcagacagaggaacctggttaagtttaatttcaaataaaaatttggtaggttccctactaccacccttggtagcttttttcttttatccttggttttcatcagttttacctgttacgttagttatgattttctttatttattccacttggggttcactcagtttattggatctgtgagttgatagctttaccaaatttgaggtaattctggcctgtaagttacttatattttcttctgccctattttccttctattcttctggaaatccagttacatatgttaaatagcttgatatttccccaaatggcattgaggctttctgttgtcttccttctaatcttttcttctcttttcctcagattggacaatttctttcatgtgtcatctctatgctacggttaaacccaaccattttcttttaatgttaccacattttgggtgagaatatatatctatattcattcattacaaccaccctacctttttgtccatgaacatagttctaaaaactgctttaaaaatccttgtctgccaattccaccatcatctagtttatgttcggatttttttttctgttgtctgctcttttttttttttttaaaccataagctataaactgtatttccttatttctctggataccctatagcattttattgtattccagtcattgtttatatgttatacagattcattttatcatactctgaagagtgctaagctttgatctcatttaaagtattggctaatcaccttgattttatattatgttaaaggtttcatccttagttttagcataaatctttagtcttgtgcacagcctttactaatacatggccattctggggtttgggaagctcaaggttctatcaagcccttctaacttgtcagaattcaaacttgaaactgtgtcttctattgcaatagaaaacagccgtctctgttcagcttcttgagccttccaactgtggctttccaccaaggtccttggagtcttcccggggcatgcacggtttgagagttagctaaggatttaaggagagatcatatgcagacaggaagcctcctccatttctgacaccttcatttctaggatctgctgctttaattttcagttcttctagcggcctttaattccatcctaacacctcaagccagtaagattgcaactttctcttgagttctagccacgccttaccacacagtctgggaaagaccgaaggggaaaaaccatatatagttcacagctggtttcagtgactccctagagtttttagaccattgtttattatattttgtccacagtttataattgggagggtttgtacattacaagctattacaccattaccaaaaccagaagtccttcattatatagttcttaaatgtttagtttaacatatgagaagaaaataatatacaactggtatttaaatgtacttggctctctccccttctgtgtctaacagattgaaaatgaggccaggcatagtggctcatgcctgtaatcccagcactttgggaggccaaggtgggtggatcacttgaggtcaggagttcaagaccagcctggccaacatggcgaaaccccatctctacacacacacacacaaaatagccaggtgtggtgccgccacatgactgtaatcccagctactcgggaggctgaggcaggataatcgcttgaacctgggaggcagaggttgcagtgagccaagattgcaccactacactctagcctgggctacagagtgagactgtgtctcaaaaataaataaataaataaataaaaaataataaagaaaaaagagatgtttcatatatatataaatatttcttatctcaaatgaagtaaaataagtcaaataatctttagctaattgatgatcccagggaatagggaaatctgttcaaatttcaatgaatttactaagtaaagagctcagaaaaattggttaggccatggaaatacttagagttgaaccaactgaactaggatataagaaagctatttctattcagaactgaaactctttgaaatgaaatataataaatggagtgttatttaatactagtaagaagagtgtgactactcgcacatatacaatggcatattaactgaattaagttatatggcatatcttgactaatccattgttgccttaaaacttacatttttaaaaattttattttgtagtcagcaagttttccatttgtctgcttggatgtgaaagatgctatttaaaaccaaacagcaactgtacaaggctggctgaacatttataattaaacaatcttataacctccaaaatacagcagagtatgagccacgtaattaggatgtcagctaaccaagacagtgaattcagaagaatgtcattttgtggcatgtgctcagctgagctttaagtcagactgctggatggaaatgtaatctttctacctttgtttatatacactaataccagctgctgtcaggacaactcctcatgcagtagggacagctaacttttttaaaaagaagaaaattataaacatattttgtgaacatttactaatcttttatttgcttttcttggcactcataacattttttaccctttaaaacagattcaagtgattcaaattccagttacctctaagttatattctgttaacaaccaccttgtataaattggtttcataaataaaaactgctcttaaatgattctgtcagtggatgtctatccacaagctttccagcctggtctgctttatgtgtacatcctgaaaatttgccaaaatagcagcaacaactgatgatatcatagggaaaaaactcactgccacaagaaaccaagcattgttgagtcaacttctttttggtcacttgttttatacttactagataagccaaaagacctgtttgttacacaaacatgcatgcatccaggtattaatccattctcacactgctatgaagaaatacccgagactgggtaattataaaagaggtttaattttcgactcacagttccacatggctgggaaggcctcaggaaacttaacaatcacggtggaaggcacctcttcacagggcggcaagagtgagaatgagagccagtaggggaaatgccaggcacttataaaaccatcagatctcatgaaagctcactatcatgagaatagcatgagggaaactgcccccatgattcaattacctaccacaacacctgggaattatgaggattaaaattcaagatgagacttgggtggggatacatccaaaccatatcaatccatatatggctgaaatttacatcagacaatggtaaatatctatgttcaaagtccattgatgctttgagattctgagctattttctggtatggaaaacagacttagcatctccatctccattggatgtatgctgcctcctgtgatgatcaaggaatgcaatggttctcccaagtccacagtgcacatttgccttaaagtgcctgctgcaattttctggtcgtcggctccaaccctggctaagccaacacaaagtgtctcctcggtaactgttgattagattttccaaagactgctcctttactttgatgtctagtaaacataatgtgtgcatgccattttgtctgttcttcttcactttgtcaaagaagctttctggtctccaagtgtctgtccaaaaaacaatagaaactgtctctccaaacttatataactgtaaaccacagcagcctacagcattcattatggaggcattgtgaataactctataaggaattcccagctttgttgctcttagaacaagatcactgtgtgttgtggccccaaatggatcaccaaccacaaggaatgcaacatcactgatatcagcatcctttaaaatattatctgcttcttgttccacttcttctctatcagcaacaaccaattttcttccataaaactcttccaaggcttccttccctacagttaggactgaggtgtaggcttccagatacactcgactgcagcgtctaacaacttccaggcccttgactgtgatgtccttggcatctcccaggcccaacccgatgagataaagcatttcaaacttgaggagaagagagactaggagcagccaattacccgctgagagaatcgtaggtagttctctggcctttacaaattcttaactaccacctttccgcagaagcaactgcaaaagcgccggctccgtgcagagaaaag

SEQ ID NO: 17526 - RNA, 304 nt, Homo sapiens
  source 1..304: mol_type = other RNA
tcaggccaggcacagtggctcatgcctgtaatcccagcactttgggaggccaaggcgtgggggttcacttgaggttaggcgttggagatcagcctggccaacatggtgaaaccttttctctactaaaaatacaaaaaaaaaaaaaaatcagccggtcatggtggtgggcacctgtaatcccagctactcaggaggctgaggtgggagaattgcttgaaaccaggaagtggaggttgcagtgagccaagatcacaccactgcactctagcctgtaggacagagcaaaattcggtctcaaaaaaaa

SEQ ID NO: 17527 - RNA, 3838 nt, Homo sapiens
  source 1..3838: mol_type = other RNA
tcaggccaggcacagtggctcatgcctgtaatcccagcactttgggaggccaaggtgggcagatcacctgaggtcaggagttcgagaccagcctggccaacatgataaaatcccgtctctactaaaaatacaaaaaattagccaggcgtggtggcgggcgcctggaatcccagctactcgggaggctgaggcaggaaaatcgcttgaactagagaggcggaggtggcagtgagcggagatcacggcattgcactccagcctgggcgacagggtgagactacatctcaaaaacaaaaaactaaaataataaaattttacaggaagagaaactatggccacagtggggagtggcatgactccctaagcaagttcaggtcagacagggcaaagaattctgactgcagggaggaggaatggctggttttccagagatagatcagaacaacagaagctccctgtgctccagcctcggctgtggtgcactgacctctcaccccaggcaggctgaagaggaaacccctgcagaggtggccttggacacctggttcctggaagcagctggctgccgtcatctgcagggcctgcagttccaccgcaccctatggccccctggggtcacagcctcccacatccgctaaccagcctcatcacttgtttccgccagcaaaccacaggtccccagaacacacccaggggaagggggctgcaggaccttctcccccagtcagtcactgtcagtgggcccaagtgctgacctcagtttaggtttccctgacataaggtgctaagaaaaatcacaaggattctagggtccctgccagcccctacctccctgagtctgtttcattaaaaatccagcctggaaggtgtgccagggagagtgacctgctggaactccatggcagaaagtaaggggatggattggggctgggcctgagccaggtattgcctggaagacttgggcatctgggtaccaccgtccctacgcacccttggcctgcttagggtccactgttcccatcccatcgtagctgttacttcctccaaaaaatcttccgggagcccccagtccctgcacacccagctgccctggacactgtgccgtaagcacctcatacccagctgtccccagactgggctgtgaactcagccaggccagaggcccctgtctggaatgggaccaggcatgcaggaggtacccaataactgctcgctaatgcagggaatgaagcagctgtagctgcagggccttctagctctgtagcccgctcagtgtatgcaagttctggaacggggacagccactcaggaggtacccagtaaccaggcactaatgcagggaatgaagcagctgtagctgcagggccttctagctctgcagcagcactgccctggcctgacctgaggcagcagaactggtgagtggggtgtgggctcccagcccagactgcccaagtttgggtcctgatctgttactcgctgtgcaccctggggaagtcactcagtgacctgcaccctggaagacaagacaaccaactgttggggttcccgggtactgctgcggtcaccacttagacatcagcatgggcacccagtaagctggtaatcccctccttcccaatcaagccccagccaccaaggcaaagctcactgctgctttattggaggcaacagcccctactggagcctgtgtcttagcgttcctgggggtcccagggccagccccggcccccacccagctgccctggccctgcctggctcccagcccacttaggggtgagtgtgatggggggaccagtgttcctgtccttggagcccaggcacagcttggtcctgggtttctgggattgggacagggcaagttagtgtggggcaacagagtcccttcgtcctctggagcctggcgcctggttcagccctagaacccaacctgctggatgagactggctgggtcctacgagatgtccatcacagaggccctaggcaagcacagccttgctcctgctcaccctcccatgtgggcccatgtccgtctgtgtggcctggggtcagggcccctgtgactgccttggcctggcagccacatggactgccatcacctaggcccagtgtagccgtaggggtgccgcagcagcaggctctggtggctgggcagcacgtgggtgtggtagtgctccaccatgctgcccacactcacaaacaggacctcgccctccaggtagaacttagagtccttctcaaaaatgcgatagttcctcactttgttagaggtttcgtcccacacaaccaggaccttccccgacttggtagaggagttccggatgcagtagagtccatcctggggctctccccgggggcttgtagccttgaacaacctttccacttcgcaggactccgtggtgttgacgaagaccgagttgggcagtggcaccttctcatagtcctcgtccgagtcgtccccgccagtgtcagcctgtgagggttgccggggcttttcaaaggagaagctcctgaaactctgcccatcggggggtgatcgctggaggtgcgggagctgcggcttctctggcctgggcaggactgcgggccgcgccatggcctcaggcactggcagcttcagcgcaggaggccggggagccacggggggcacaaagagtccgggcatggctgcctcccttggggggtcctcttcagctatcttcaggaacttgggcttgttggctggcacaggtgggggctcagatgtgggtggtcctcggggggacaggtggaaggacttgagtttgtcacagtttctggaggtggcagtggccatgatggcagcactggaagtggagcaggccccgtggccaggggtccagggctccgggctggggctggcactctcccggaagcaagggggtttccggaggccgggtgcggtgggcatggtgctcagagggggatcgctcatccttcggggggtagcaggtaccctggggcaaggctcagcccgcctcgggcacagtgggtccctcttggagtcctcagcagccaggccaacatctgggaggccgtgcttagggggcgggggtggcagtaggggaccggggcccttggaggtaaaggagtgggcccggggcatgtcagagaaggctggcttcctgggcgtgggcactgggggtggtgggtaagccggtgggtgcatcagggcatcctcaagccttccgggctccggggagtcaggctccaggtaggagtcatcctcatcgtcgtgctcatagtcttcattgtccgtggggtacggggaaaggctgatatccacaggccgctcaactgcgccgtagaagctgtctgtgtccgagctggagtcgctggtgtccaagggcaggtctttcttttcgtggaagtggccaatctccctgcgcagcaaggccatccagctcttgcgctcctcctcggaggaggccgagaagaaccacgtgcggtgcttcttgctgatatggatgatcttgaaggggaaaacgttgttggacgtggtctcctcagccgcccgcatcacccggttatagccactcagggagaaggcgccctgcggggaggcagaggtgctactcttgaagtagtagacgcagcgtttgtggatgatgacaaagcgcaggggccatttcagcagctgcagctgggtaccgcccttcttgtgcaggtagccagccttggccacgcccccaggcatggttagcaggttctgggcaccaatggccttcatagggacaggccaatgcatctcttcagccgccatgaagccgccgagcgctctcctggcccgcgggccctgggtcgaggcggcggcttgactc

SEQ ID NO: 17528 - RNA, 4041 nt, Homo sapiens
  source 1..4041: mol_type = other RNA
tcaggccaggcacagtggctcatgcctgtaatcccagcactttgggaggccaaggtgggcagatcacctgaggtcaggagttcgagaccagcctggccaacatgataaaatcccgtctctactaaaaatacaaaaaattagccaggcgtggtggcgggcgcctggaatcccagctactcgggaggctgaggcaggaaaatcgcttgaactagagaggcggaggtggcagtgagcggagatcacggcattgcactccagcctgggcgacagggtgagactacatctcaaaaacaaaaaactaaaataataaaattttacaggaagagaaactatggccacagtggggagtggcatgactccctaagcaagttcaggtcagacagggcaaagaattctgactgcagggaggaggaatggctggttttccagagatagatcagaacaacagaagctccctgtgctccagcctcggctgtggtgcactgacctctcaccccaggcaggctgaagaggaaacccctgcagaggtggccttggacacctggttcctggaagcagctggctgccgtcatctgcagggcctgcagttccaccgcaccctatggccccctggggtcacagcctcccacatccgctaaccagcctcatcacttgtttccgccagcaaaccacaggtccccagaacacacccaggggaagggggctgcaggaccttctcccccagtcagtcactgtcagtgggcccaagtgctgacctcagtttaggtttccctgacataaggtgctaagaaaaatcacaaggattctagggtccctgccagcccctacctccctgagtctgtttcattaaaaatccagcctggaaggtgtgccagggagagtgacctgctggaactccatggcagaaagtaaggggatggattggggctgggcctgagccaggtattgcctggaagacttgggcatctgggtaccaccgtccctacgcacccttggcctgcttagggtccactgttcccatcccatcgtagctgttacttcctccaaaaaatcttccgggagcccccagtccctgcacacccagctgccctggacactgtgccgtaagcacctcatacccagctgtccccagactgggctgtgaactcagccaggccagaggcccctgtctggaatgggaccaggcatgcaggaggtacccaataactgctcgctaatgcagggaatgaagcagctgtagctgcagggccttctagctctgtagcccgctcagtgtatgcaagttctggaacggggacagccactcaggaggtacccagtaaccaggcactaatgcagggaatgaagcagctgtagctgcagggccttctagctctgcagcagcactgccctggcctgacctgaggcagcagaactggtgagtggggtgtgggctcccagcccagactgcccaagtttgggtcctgatctgttactcgctgtgcaccctggggaagtcactcagtgacctgcaccctggaagacaagacaaccaactgttggggttcccgggtactgctgcggtcaccacttagacatcagcatgggcacccagtaagctggtaatcccctccttcccaatcaagccccagccaccaaggcaaagctcactgctgctttattggaggcaacagcccctactggagcctgtgtcttagcgttcctgggggtcccagggccagccccggcccccacccagctgccctggccctgcctggctcccagcccacttaggggtgagtgtgatggggggaccagtgttcctgtccttggagcccaggcacagcttggtcctgggtttctgggattgggacagggcaagttagtgtggggcaacagagtcccttcgtcctctggagcctggcgcctggttcagccctagaacccaacctgctggatgagactggctgggtcctacgagatgtccatcacagaggccctaggcaagcacagccttgctcctgctcaccctcccatgtgggcccatgtccgtctgtgtggcctggggtcagggcccctgtgactgccttggcctggcagccacatggactgccatcacctaggcccagtgtagccgtaggggtgccgcagcagcaggctctggtggctgggcagcacgtgggtgtggtagtgctccaccatgctgcccacactcacaaacaggacctcgccctccaggtagaacttagagtccttctcaaaaatgcgatagttcctcactttgttagaggtttcgtcccacacaaccaggaccttccccgacttggtagaggagttccggatgcagtagagtccatcctggggctctccccgggggcttgtagccttgaacaacctttccacttcgcaggactccgtggtgttgacgaagaccgagttgggcagtggcaccttctcatagtcctcgtccgagtcgtccccgccagtgtcagcctgtgagggttgccggggcttttcaaaggagaagctcctgaaactctgcccatcggggggtgatcgctggaggtgcgggagctgcggcttctctggcctgggcaggactgcgggccgcgccatggcctcaggcactggcagcttcagcgcaggaggccggggagccacggggggcacaaagagtccgggcatggctgcctcccttggggggtcctcttcagctatcttcaggaacttgggcttgttggctggcacaggtgggggctcagatgtgggtggtcctcggggggacaggtggaaggacttgagtttgtcacagtttctggaggtggcagtggccatgatggcagcactggaagtggagcaggccccgtggccaggggtccagggctccgggctggggctggcactctcccggaagcaagggggtttccggaggccgggtgcggtgggcatggtgctcagagggggatcgctcatccttcggggggtagcaggtaccctggggcaaggctcagcccgcctcgggcacagtgggtccctcttggagtcctcagcagccaggccaacatctgggaggccgtgcttagggggcgggggtggcagtaggggaccggggcccttggaggtaaaggagtgggcccggggcatgtcagagaaggctggcttcctgggcgtgggcactgggggtggtgggtaagccggtgggtgcatcagggcatcctcaagccttccgggctccggggagtcaggctccaggtaggagtcatcctcatcgtcgtgctcatagtcttcattgtccgtggggtacggggaaaggctgatatccacaggccgctcaactgcgccgtagaagctgtctgtgtccgagctggagtcgctggtgtccaagggcaggtctttcttttcgtggaagtggccaatctccctgcgcagcaaggccatccagctcttgcgctcctcctcggaggaggccgagaagaaccacgtgcggtgcttcttgctgatatggatgatcttgaaggggaaaacgttgttggacgtggtctcctcagccgcccgcatcacccggttatagccactcagggagaaggcgccctgcggggaggcagaggtgctactcttgaagtagtagacgcagcgtttgtggatgatgacaaagcgcaggggccatttcagcagctgcagctgggtaccgcccttcttgtgcaggtagccagccttggccacgcccccaggcatggttagcaggttctgggcaccaatggccttcatagggacaggccaatgcatctcttcagccgccatgaagctatagtacccggaggaggcttatccaggaggatcgattgagccaggagttccaggaggcagtaagctatgattggccactgctctccagtctgggcaactgagctggagctaaaattaaaaaattaaaaacaaaataaataaaaagaaaaatactctctgcttttagcaaaccagcaccctccaacaaaagtgcaagaggaagtcttcaaggcatcaggctgtcttctgccggcctcggcctgggtcacccggctg

SEQ ID NO: 17529 - RNA, 3971 nt, Homo sapiens
  source 1..3971: mol_type = other RNA
tcaggccaggcacagtggctcatgcctgtaatcccagcactttgggaggccaaggtgggcagatcacctgaggtcaggagttcgagaccagcctggccaacatgataaaatcccgtctctactaaaaatacaaaaaattagccaggcgtggtggcgggcgcctggaatcccagctactcgggaggctgaggcaggaaaatcgcttgaactagagaggcggaggtggcagtgagcggagatcacggcattgcactccagcctgggcgacagggtgagactacatctcaaaaacaaaaaactaaaataataaaattttacaggaagagaaactatggccacagtggggagtggcatgactccctaagcaagttcaggtcagacagggcaaagaattctgactgcagggaggaggaatggctggttttccagagatagatcagaacaacagaagctccctgtgctccagcctcggctgtggtgcactgacctctcaccccaggcaggctgaagaggaaacccctgcagaggtggccttggacacctggttcctggaagcagctggctgccgtcatctgcagggcctgcagttccaccgcaccctatggccccctggggtcacagcctcccacatccgctaaccagcctcatcacttgtttccgccagcaaaccacaggtccccagaacacacccaggggaagggggctgcaggaccttctcccccagtcagtcactgtcagtgggcccaagtgctgacctcagtttaggtttccctgacataaggtgctaagaaaaatcacaaggattctagggtccctgccagcccctacctccctgagtctgtttcattaaaaatccagcctggaaggtgtgccagggagagtgacctgctggaactccatggcagaaagtaaggggatggattggggctgggcctgagccaggtattgcctggaagacttgggcatctgggtaccaccgtccctacgcacccttggcctgcttagggtccactgttcccatcccatcgtagctgttacttcctccaaaaaatcttccgggagcccccagtccctgcacacccagctgccctggacactgtgccgtaagcacctcatacccagctgtccccagactgggctgtgaactcagccaggccagaggcccctgtctggaatgggaccaggcatgcaggaggtacccaataactgctcgctaatgcagggaatgaagcagctgtagctgcagggccttctagctctgtagcccgctcagtgtatgcaagttctggaacggggacagccactcaggaggtacccagtaaccaggcactaatgcagggaatgaagcagctgtagctgcagggccttctagctctgcagcagcactgccctggcctgacctgaggcagcagaactggtgagtggggtgtgggctcccagcccagactgcccaagtttgggtcctgatctgttactcgctgtgcaccctggggaagtcactcagtgacctgcaccctggaagacaagacaaccaactgttggggttcccgggtactgctgcggtcaccacttagacatcagcatgggcacccagtaagctggtaatcccctccttcccaatcaagccccagccaccaaggcaaagctcactgctgctttattggaggcaacagcccctactggagcctgtgtcttagcgttcctgggggtcccagggccagccccggcccccacccagctgccctggccctgcctggctcccagcccacttaggggtgagtgtgatggggggaccagtgttcctgtccttggagcccaggcacagcttggtcctgggtttctgggattgggacagggcaagttagtgtggggcaacagagtcccttcgtcctctggagcctggcgcctggttcagccctagaacccaacctgctggatgagactggctgggtcctacgagatgtccatcacagaggccctaggcaagcacagccttgctcctgctcaccctcccatgtgggcccatgtccgtctgtgtggcctggggtcagggcccctgtgactgccttggcctggcagccacatggactgccatcacctaggcccagtgtagccgtaggggtgccgcagcagcaggctctggtggctgggcagcacgtgggtgtggtagtgctccaccatgctgcccacactcacaaacaggacctcgccctccaggtagaacttagagtccttctcaaaaatgcgatagttcctcactttgttagaggtttcgtcccacacaaccaggaccttccccgacttggtagaggagttccggatgcagtagagtccatcctggggctctccccgggggcttgtagccttgaacaacctttccacttcgcaggactccgtggtgttgacgaagaccgagttgggcagtggcaccttctcatagtcctcgtccgagtcgtccccgccagtgtcagcctgtgagggttgccggggcttttcaaaggagaagctcctgaaactctgcccatcggggggtgatcgctggaggtgcgggagctgcggcttctctggcctgggcaggactgcgggccgcgccatggcctcaggcactggcagcttcagcgcaggaggccggggagccacggggggcacaaagagtccgggcatggctgcctcccttggggggtcctcttcagctatcttcaggaacttgggcttgttggctggcacaggtgggggctcagatgtgggtggtcctcggggggacaggtggaaggacttgagtttgtcacagtttctggaggtggcagtggccatgatggcagcactggaagtggagcaggccccgtggccaggggtccagggctccgggctggggctggcactctcccggaagcaagggggtttccggaggccgggtgcggtgggcatggtgctcagagggggatcgctcatccttcggggggtagcaggtaccctggggcaaggctcagcccgcctcgggcacagtgggtccctcttggagtcctcagcagccaggccaacatctgggaggccgtgcttagggggcgggggtggcagtaggggaccggggcccttggaggtaaaggagtgggcccggggcatgtcagagaaggctggcttcctgggcgtgggcactgggggtggtgggtaagccggtgggtgcatcagggcatcctcaagccttccgggctccggggagtcaggctccaggtaggagtcatcctcatcgtcgtgctcatagtcttcattgtccgtggggtacggggaaaggctgatatccacaggccgctcaactgcgccgtagaagctgtctgtgtccgagctggagtcgctggtgtccaagggcaggtctttcttttcgtggaagtggccaatctccctgcgcagcaaggccatccagctcttgcgctcctcctcggaggaggccgagaagaaccacgtgcggtgcttcttgctgatatggatgatcttgaaggggaaaacgttgttggacgtggtctcctcagccgcccgcatcacccggttatagccactcagggagaaggcgccctgcggggaggcagaggtgctactcttgaagtagtagacgcagcgtttgtggatgatgacaaagcgcaggggccatttcagcagctgcagctgggtaccgcccttcttgtgcaggtagccagccttggccacgcccccaggcatggttagcaggttctgggcaccaatggccttcatagggacaggccaatgcatctcttcagccgccatgaagctgatggtgctgacccaacacatggccctccgtcctcgtgacctgctcggggccggtgtcctggggcccagggaggccatgcggctcaggggccaccagcccaggcagcctacatctcccagacatgtgaggcctgacgcgcctggctgccccacagctgtgcccacagctcactcctgctgcttct

SEQ ID NO: 17530 - RNA, 4005 nt, Homo sapiens
  source 1..4005: mol_type = other RNA
tcaggccaggcacagtggctcatgcctgtaatcccagcactttgggaggccaaggtgggcagatcacctgaggtcaggagttcgagaccagcctggccaacatgataaaatcccgtctctactaaaaatacaaaaaattagccaggcgtggtggcgggcgcctggaatcccagctactcgggaggctgaggcaggaaaatcgcttgaactagagaggcggaggtggcagtgagcggagatcacggcattgcactccagcctgggcgacagggtgagactacatctcaaaaacaaaaaactaaaataataaaattttacaggaagagaaactatggccacagtggggagtggcatgactccctaagcaagttcaggtcagacagggcaaagaattctgactgcagggaggaggaatggctggttttccagagatagatcagaacaacagaagctccctgtgctccagcctcggctgtggtgcactgacctctcaccccaggcaggctgaagaggaaacccctgcagaggtggccttggacacctggttcctggaagcagctggctgccgtcatctgcagggcctgcagttccaccgcaccctatggccccctggggtcacagcctcccacatccgctaaccagcctcatcacttgtttccgccagcaaaccacaggtccccagaacacacccaggggaagggggctgcaggaccttctcccccagtcagtcactgtcagtgggcccaagtgctgacctcagtttaggtttccctgacataaggtgctaagaaaaatcacaaggattctagggtccctgccagcccctacctccctgagtctgtttcattaaaaatccagcctggaaggtgtgccagggagagtgacctgctggaactccatggcagaaagtaaggggatggattggggctgggcctgagccaggtattgcctggaagacttgggcatctgggtaccaccgtccctacgcacccttggcctgcttagggtccactgttcccatcccatcgtagctgttacttcctccaaaaaatcttccgggagcccccagtccctgcacacccagctgccctggacactgtgccgtaagcacctcatacccagctgtccccagactgggctgtgaactcagccaggccagaggcccctgtctggaatgggaccaggcatgcaggaggtacccaataactgctcgctaatgcagggaatgaagcagctgtagctgcagggccttctagctctgtagcccgctcagtgtatgcaagttctggaacggggacagccactcaggaggtacccagtaaccaggcactaatgcagggaatgaagcagctgtagctgcagggccttctagctctgcagcagcactgccctggcctgacctgaggcagcagaactggtgagtggggtgtgggctcccagcccagactgcccaagtttgggtcctgatctgttactcgctgtgcaccctggggaagtcactcagtgacctgcaccctggaagacaagacaaccaactgttggggttcccgggtactgctgcggtcaccacttagacatcagcatgggcacccagtaagctggtaatcccctccttcccaatcaagccccagccaccaaggcaaagctcactgctgctttattggaggcaacagcccctactggagcctgtgtcttagcgttcctgggggtcccagggccagccccggcccccacccagctgccctggccctgcctggctcccagcccacttaggggtgagtgtgatggggggaccagtgttcctgtccttggagcccaggcacagcttggtcctgggtttctgggattgggacagggcaagttagtgtggggcaacagagtcccttcgtcctctggagcctggcgcctggttcagccctagaacccaacctgctggatgagactggctgggtcctacgagatgtccatcacagaggccctaggcaagcacagccttgctcctgctcaccctcccatgtgggcccatgtccgtctgtgtggcctggggtcagggcccctgtgactgccttggcctggcagccacatggactgccatcacctaggcccagtgtagccgtaggggtgccgcagcagcaggctctggtggctgggcagcacgtgggtgtggtagtgctccaccatgctgcccacactcacaaacaggacctcgccctccaggtagaacttagagtccttctcaaaaatgcgatagttcctcactttgttagaggtttcgtcccacacaaccaggaccttccccgacttggtagaggagttccggatgcagtagagtccatcctggggctctccccgggggcttgtagccttgaacaacctttccacttcgcaggactccgtggtgttgacgaagaccgagttgggcagtggcaccttctcatagtcctcgtccgagtcgtccccgccagtgtcagcctgtgagggttgccggggcttttcaaaggagaagctcctgaaactctgcccatcggggggtgatcgctggaggtgcgggagctgcggcttctctggcctgggcaggactgcgggccgcgccatggcctcaggcactggcagcttcagcgcaggaggccggggagccacggggggcacaaagagtccgggcatggctgcctcccttggggggtcctcttcagctatcttcaggaacttgggcttgttggctggcacaggtgggggctcagatgtgggtggtcctcggggggacaggtggaaggacttgagtttgtcacagtttctggaggtggcagtggccatgatggcagcactggaagtggagcaggccccgtggccaggggtccagggctccgggctggggctggcactctcccggaagcaagggggtttccggaggccgggtgcggtgggcatggtgctcagagggggatcgctcatccttcggggggtagcaggtaccctggggcaaggctcagcccgcctcgggcacagtgggtccctcttggagtcctcagcagccaggccaacatctgggaggccgtgcttagggggcgggggtggcagtaggggaccggggcccttggaggtaaaggagtgggcccggggcatgtcagagaaggctggcttcctgggcgtgggcactgggggtggtgggtaagccggtgggtgcatcagggcatcctcaagccttccgggctccggggagtcaggctccaggtaggagtcatcctcatcgtcgtgctcatagtcttcattgtccgtggggtacggggaaaggctgatatccacaggccgctcaactgcgccgtagaagctgtctgtgtccgagctggagtcgctggtgtccaagggcaggtctttcttttcgtggaagtggccaatctccctgcgcagcaaggccatccagctcttgcgctcctcctcggaggaggccgagaagaaccacgtgcggtgcttcttgctgatatggatgatcttgaaggggaaaacgttgttggacgtggtctcctcagccgcccgcatcacccggttatagccactcagggagaaggcgccctgcggggaggcagaggtgctactcttgaagtagtagacgcagcgtttgtggatgatgacaaagcgcaggggccatttcagcagctgcagctgggtaccgcccttcttgtgcaggtagccagccttggccacgcccccaggcatggttagcaggttctgggcaccaatggccttcatagggacaggccaatgcatctcttcagccgccatgaagggcgtccacgcggcgggcatggccggcttccccggggcgatccacgcccgcctcccctgcgagcaccggcacggccccgggccgcgtcccccggccgccgccgcctcgtcccgggcgcccgcctcccgccggccccagctccgcggccgcggcccggagcccgccatgcccgccggccctggcctggcagccgccggctcctcccctctcggcgggggact

SEQ ID NO: 17531 - RNA, 2956 nt, Homo sapiens
  source 1..2956: mol_type = other RNA
tcaggccaggcacagtggctcatgcctgtaatcccagcactttgggaggccgaggcgggcggaccacctgaggttgggagtttgagatttagcctgaccaacatggagaaaccttgtctctattaaaaaatacaaaaaattagacaggcatggtggcgcatgcctgtaatcccagctacttgggaggctgaggcaggagaatcgcttgaacccaggaggcggaggttgcggtgagccgagattgtgccattgcactccagcctggacaacaagagcaaaactccgtctcaaaacaaaaaaaaaagatgagaaaactctcaaagatttatagaagcaggagtagaaagtttccctatgaaaaagcataggctgttttggtaccctgtggccaagaatccaattaaaatcactgtcacccacaaaaaccttcatctgatattttacttttgaacaccaaaaaaaaaaaaaaaaaaaatcaacatagatgtaatcattacaatcacgtatgggatttagatacaaagaaaaaaatctctattgggctggagaccattatcaaagcaaatctgttgtttattgtctttttaaaaatttttcataggtgctgtagaatggataaagttcaagaaaggcaaaagcttcaaaatataagaaaataattttaataacagcatcatctcttttttagagtttcagaatgagaaaatcaacatgaagaaaaacagtgttgagaagaattttagaggttgtctagtacattcctagctttattttagcaaaagtgctttaaagaaattcacatgttaaaaatacattctattttgaacacagccagataaggagatttctgtacctcttttagtatcccatttcaatgactgtcactctgaagtgactctgaggttttccttaaatacctcctaaatctggtcacattgtttttttgttttattctttaaaaagatggaaggttagtagtattcattctctacataatgacaattcctcttataacttcaaaactttcaaaaaccatttatgagacattttcacatacattatctatttaacccttgaaataatcccattactatttgtcacagatggagaaattcaaggcttagagagttaaaacaattgaagctggcgggggtgggggtggtgtggaaatgggataatcccaagcttattatattcaatccttagagtcaaattcagctagctacttcgtatataactaagtcactaacccctttacttctttccactccagaataagaaattttattttaacaaagacttagcaaacagtaaaatcagagggcttgcttctatggagaatccatgtgtcactttatttttcacgctgtgtatttttgcagtgaagatgtgtaatttgtaacaccatcattccccttcttccaccaactgtacccagatttccctcaggggctgtcaatcatattgttgagccttcccctgtctaaagacttagcacagaatccaggctgctccaaatcggcactttttcccagaaatctgaatcttaggtgggtgacagaagattggaaatggccagagttcatccatttcacagatgagttctctgagcctgccctagtttctaagaggccatccttcagcttctactcccttctcccagtgagtccattttcagataaattcattttctgcttaagttagccagtgttggtttctgttgcttgcaagcagagaaccttgactgatagagctcttcagaggggtagataagaatatgtatttattaattctgcctctattatgtatttattatctaggtgggaaatactaaaatgaaatcagccttttggcattttgtaaactaagaaaattcactcatgttgcacaaagtagtaatgttttattccttgatcaagggcaacaataagttggcaagttttccagaatcctggctacatttttcaggaaaatgaaaaatggcttctgggaccttggattattcaggaagtacagaaaattcagaaagtgtcaaatgtgtttaacgaggtactttcctgtgacaagttctttctcagaattgcttagagaggacaaaaggcactgtagcaatacatcctctcataacccctccatgctaggcgaaagggaaacacaggtgtcaggcctcaaaacgcctggctagtttgtcagagacagctgcagccaaggtgctaaataagccctggttatcaggactttcaagtctaaaaggaaaaactggtttacaaaaaaaaaaaggtgcaactgtccactcaacattggcccaaggtgaggcggagttctcttagacaactgtcttaaaattcactacatgaagaagcattgtatcagattcttttctcttcccaggactggcaaagagagcaatggcctatcaatactttgaaattgccacaataccacccttatttcacagttcatagagattataagccaactatcaaaggatactatgatccgctatctggagtaattcactcaataaacaaaagcttctacaacatgtctggcatgttacggaggagataaagaattataaaggaagaagcttgcttactgtaagataattttcaatctgagaaaataaggcaaacaaatatgaaataactagtaacaggcaacgcaggaagaaccccaactgccaagttcagacagtaaaaaatcaaggattccaaaccctgagatccactccctcagctgtaactcaaagacagttccttggccacataaacacaggcactttatatcctttcctttttaattaagagctgatttcaacaccaaagcaaagatccatcagaaaagcacatcggtataaagagggcggaaggagggtgggggggaagaaggtaagaaaaaataactactgggtactaggcttagtacctgagtgacaaaataatctgtacaccaa

SEQ ID NO: 17532 - RNA, 2637 nt, Homo sapiens
  source 1..2637: mol_type = other RNA
tcaggccaggcacagtggctcatgcctgtaatcccagcactttgggaggccgaggtgggtggatcacttgaagccaggagttcgagaccagcctggccaacatagcaaaaccttgtctctattacaaatatgcccatgtgctaggtgtggtgggacacacctgtaatcccagctacccaggagaatcgcttaaacccgggaggcggaagttgcagtgagctgagatcataacaccgcactccaccctgagtgacagggcaagactcaaaaaataaaaaaggaacattaactagggttagaaactaacttcattctttttagaattcaacagttttcctaggtcaccaattccaccttttgttcttattaaggcgcaaagtcacaggacccccttcctgggagtcactgtcattaaatctattgccgtcagctcagcccagggtaggcaaggttcaagaatgggaagtgcttttgtctggggaaacacgcaggtaatgtgatgctaggaaggaggatgtgcaggtgggtgagagcccaggagggagcagctggtgcctgacagggtgagccatcagggctgggcctgggtacagccccaggagaaggagcctgtgcagaagtagcagttcagtggattccacctcctatgtcacaatccagcaggtggccaggactcagcctgggttttaagtgagtaatgccttccctgtctcagagattagctctaacagtgtcactagaggaagccctggcgagggtgggggggcgtagtgtggggacaaggaggccagatagaaagtgctggaatgttctggaacagatctgtttctggaggagaggctgagtatggagagtcaacagaatgtgaccaccttcagagggaggagctgggccgtctccaataaatccagggacaaatgccttcagtcctcagactgttccaatagaggggacgccacgtatcccagggttccctttccaactcatgtcaacacctgcagtccctttgaggagactaaatgtatttcatgctggaaagaacagattttctctcattaaaaatagccccactaaaggagaccaacatgctagaagtgcggcaccagggcctcaagactacacttcggaacatgaagagggctggggaccgctcggcccaagtctggatcttgtaaccaacagatgccgagcttgccgttcaactaggcacagaaagcagactcggtctgggattccagttggtctgattcagttcaagagggtcacagtcagaagaaagctttttccattaggagcttcagcagagtgaagagttcaacacagcaaacaggcaggcagctcctttgtatatgtgacggggtggccctgactgtaaacacagccctaccagtcactgcagctcatggcctgagaagacattccagtggcagcctcgggtgtccactcagttcacatattctggtttcacctgcccaagctgtcttcaggcatgaggtcttgtcagaattgggatgtggatgtctcctatgttaccatttattgtgtgggggcagccatcatcctatttgtctggtccatcaagcctagagcagtgagaagggcagccccttggatggtcctcctcagcagtctgtaccttcccagtttcccgctgcacaaggtcccgcatctcttctgtccagcccagaagctccactaggctttccacgccgtgaaccacgtcccccagctgggccacgtccctgctgcgaggatgccaagccaagggccccaccaagtcccggttgatgagcagtcggggaactgagctccgcacggcctcggtcaagctggcaaaaggctccacctccagggaggtcccaaggatgagcagcagatctgccatggggaaatcaaccacatgcagcaagaacctctggggcagcggctccccaaagaacacaatgtcgggcttcacaacgccggtgcagaccgggcagcggggaaccctgtctgccatcacgtcagcccgaatgtcctcccctgggaagggtctttggcagactgtgcaggtggcagaggcaaaggttccatgagcttcaaccagctttgaggcagggatgcccgacactctctcaagcccatcgatgttctgcgtgtagagccgcagaagcagccccttgtcatgaagcagccggagaaagtagtgagtgacgttgggcttgtagtttccagggtacagctccttggccaaagtgaaaaagggcttggggttgtgaaagaagaatgggagttcaaaaatggcctcggggtacgggagatcgtactgctggaggttgctgtacaggccactccccggcgatctcgaaaagaagaaactgggagctgctgccctcggctgcctccggaatgccctgggcacctcgggtctgggaggcctctgcaaggggcgcgccgggtccaagggctcaccgcgggccccatggctgcctctcagccccgcactcacatcgtccctgccgccaagcaccagccgacagccgcaggcctgaaacggccccacgcctcccccggcctcgacccgttcaactacccggccccacagccggagggctgccgcggcgcgccaaccccagaacgccatgttccgcgcagtcc

SEQ ID NO: 17533 - RNA, 2683 nt, Homo sapiens
  source 1..2683: mol_type = other RNA
tcaggccaggcacagtggctcatgcctgtaatcccagcactttgggaggccgaggtgggtggatcacttgaagccaggagttcgagaccagcctggccaacatagcaaaaccttgtctctattacaaatatgcccatgtgctaggtgtggtgggacacacctgtaatcccagctacccaggagaatcgcttaaacccgggaggcggaagttgcagtgagctgagatcataacaccgcactccaccctgagtgacagggcaagactcaaaaaataaaaaaggaacattaactagggttagaaactaacttcattctttttagaattcaacagttttcctaggtcaccaattccaccttttgttcttattaaggcgcaaagtcacaggacccccttcctgggagtcactgtcattaaatctattgccgtcagctcagcccagggtaggcaaggttcaagaatgggaagtgcttttgtctggggaaacacgcaggtaatgtgatgctaggaaggaggatgtgcaggtgggtgagagcccaggagggagcagctggtgcctgacagggtgagccatcagggctgggcctgggtacagccccaggagaaggagcctgtgcagaagtagcagttcagtggattccacctcctatgtcacaatccagcaggtggccaggactcagcctgggttttaagtgagtaatgccttccctgtctcagagattagctctaacagtgtcactagaggaagccctggcgagggtgggggggcgtagtgtggggacaaggaggccagatagaaagtgctggaatgttctggaacagatctgtttctggaggagaggctgagtatggagagtcaacagaatgtgaccaccttcagagggaggagctgggccgtctccaataaatccagggacaaatgccttcagtcctcagactgttccaatagaggggacgccacgtatcccagggttccctttccaactcatgtcaacacctgcagtccctttgaggagactaaatgtatttcatgctggaaagaacagattttctctcattaaaaatagccccactaaaggagaccaacatgctagaagtgcggcaccagggcctcaagactacacttcggaacatgaagagggctggggaccgctcggcccaagtctggatcttgtaaccaacagatgccgagcttgccgttcaactaggcacagaaagcagactcggtctgggattccagttggtctgattcagttcaagagggtcacagtcagaagaaagctttttccattaggagcttcagcagagtgaagagttcaacacagcaaacaggcaggcagctcctttgtatatgtgacggggtggccctgactgtaaacacagccctaccagtcactgcagctcatggcctgagaagacattccagtggcagcctcgggtgtccactcagttcacatattctggtttcacctgcccaagctgtcttcaggcatgaggtcttgtcagaattgggatgtggatgtctcctatgttaccatttattgtgtgggggcagccatcatcctatttgtctggtccatcaagcctagagcagtgagaagggcagccccttggatggtcctcctcagcagtctgtaccttcccagtttcccgctgcacaaggtcccgcatctcttctgtccagcccagaagctccactaggctttccacgccgtgaaccacgtcccccagctgggccacgtccctgctgcgaggatgccaagccaagggccccaccaagtcccggttgatgagcagtcggggaactgagctccgcacggcctcggtcaagctggcaaaaggctccacctccagggaggtcccaaggatgagcagcagatctgccatggggaaatcaaccacatgcagcaagaacctctggggcagcggctccccaaagaacacaatgtcgggcttcacaacgccggtgcagaccgggcagcggggaaccctgtctgccatcacgtcagcccgaatgtcctcccctgggaagggtctttggcagactgtgcaggtggcagaggcaaaggttccatgagcttcaaccagctttgaggcagggatgcccgacactctctcaagcccatcgatgttctgcgtgtagagccgcagaagcagccccttgtcatgaagcagccggagaaagtagtgagtgacgttgggcttgtagtttccagggtacagctccttggccaaagtgaaaaagggcttggggttgtgaaagaagaatgggagttcaaaaatggcctcggggtacgggagatcgtactgctggaggttgctgtacaggccactccccggcgatctgaagtctggaatgccactgggtgtgctgatgccggcccccaccatgaccaccaccctctggcaggctctggcccgaatcagctcagctacatcctgcagggaaagcttccccttgtcactgctgcctccacttccaacaacacttgaagcacccacagaaaaagatatggaccttcttccacctttaataatcgtccctgccgccaagcaccagccgacagccgcaggcctgaaacggccccacgcctcccccggcctcgacccgttcaactacccggccccacagccggagggctgccgcggcgcgccaaccccagaacgccatgttccgcgcagtcc

SEQ ID NO: 17534 - RNA, 2829 nt, Homo sapiens
  source 1..2829: mol_type = other RNA
tcaggccaggcacagtggctcatgcctgtaatcccagcactttgggaggccgaggtgggtggatcacttgaagccaggagttcgagaccagcctggccaacatagcaaaaccttgtctctattacaaatatgcccatgtgctaggtgtggtgggacacacctgtaatcccagctacccaggagaatcgcttaaacccgggaggcggaagttgcagtgagctgagatcataacaccgcactccaccctgagtgacagggcaagactcaaaaaataaaaaaggaacattaactagggttagaaactaacttcattctttttagaattcaacagttttcctaggtcaccaattccaccttttgttcttattaaggcgcaaagtcacaggacccccttcctgggagtcactgtcattaaatctattgccgtcagctcagcccagggtaggcaaggttcaagaatgggaagtgcttttgtctggggaaacacgcaggtaatgtgatgctaggaaggaggatgtgcaggtgggtgagagcccaggagggagcagctggtgcctgacagggtgagccatcagggctgggcctgggtacagccccaggagaaggagcctgtgcagaagtagcagttcagtggattccacctcctatgtcacaatccagcaggtggccaggactcagcctgggttttaagtgagtaatgccttccctgtctcagagattagctctaacagtgtcactagaggaagccctggcgagggtgggggggcgtagtgtggggacaaggaggccagatagaaagtgctggaatgttctggaacagatctgtttctggaggagaggctgagtatggagagtcaacagaatgtgaccaccttcagagggaggagctgggccgtctccaataaatccagggacaaatgccttcagtcctcagactgttccaatagaggggacgccacgtatcccagggttccctttccaactcatgtcaacacctgcagtccctttgaggagactaaatgtatttcatgctggaaagaacagattttctctcattaaaaatagccccactaaaggagaccaacatgctagaagtgcggcaccagggcctcaagactacacttcggaacatgaagagggctggggaccgctcggcccaagtctggatcttgtaaccaacagatgccgagcttgccgttcaactaggcacagaaagcagactcggtctgggattccagttggtctgattcagttcaagagggtcacagtcagaagaaagctttttccattaggagcttcagcagagtgaagagttcaacacagcaaacaggcaggcagctcctttgtatatgtgacggggtggccctgactgtaaacacagccctaccagtcactgcagctcatggcctgagaagacattccagtggcagcctcgggtgtccactcagttcacatattctggtttcacctgcccaagctgtcttcaggcatgaggtcttgtcagaattgggatgtggatgtctcctatgttaccatttattgtgtgggggcagccatcatcctatttgtctggtccatcaagcctagagcagtgagaagggcagccccttggatggtcctcctcagcagtctgtaccttcccagtttcccgctgcacaaggtcccgcatctcttctgtccagcccagaagctccactaggctttccacgccgtgaaccacgtcccccagctgggccacgtccctgctgcgaggatgccaagccaagggccccaccaagtcccggttgatgagcagtcggggaactgagctccgcacggcctcggtcaagctggcaaaaggctccacctccagggaggtcccaaggatgagcagcagatctgccatggggaaatcaaccacatgcagcaagaacctctggggcagcggctccccaaagaacacaatgtcgggcttcacaacgccggtgcagaccgggcagcggggaaccctgtctgccatcacgtcagcccgaatgtcctcccctgggaagggtctttggcagactgtgcaggtggcagaggcaaaggttccatgagcttcaaccagctttgaggcagggatgcccgacactctctcaagcccatcgatgttctgcgtgtagagccgcagaagcagccccttgtcatgaagcagccggagaaagtagtgagtgacgttgggcttgtagtttccagggtacagctccttggccaaagtgaaaaagggcttggggttgtgaaagaagaatgggagttcaaaaatggcctcggggtacgggagatcgtactgctggaggttgctgtacaggccactccccggcgatctgaagtctggaatgccactgggtgtgctgatgccggcccccaccatgaccaccaccctctggcaggctctggcccgaatcagctcagctacatcctgcagggaaagcttccccttgtcactgctgcctccacttccaacaacacttgaagcacccacagaaaaagatatggaccttcttccacctttaatactcgaaaagaagaaactgggagctgctgccctcggctgcctccggaatgccctgggcacctcgggtctgggaggcctctgcaaggggcgcgccgggtccaagggctcaccgcgggccccatggctgcctctcagccccgcactcacatcgtccctgccgccaagcaccagccgacagccgcaggcctgaaacggccccacgcctcccccggcctcgacccgttcaactacccggccccacagccggagggctgccgcggcgcgccaaccccagaacgccatgttccgcgcagtcc

SEQ ID NO: 17535 - RNA, 2850 nt, Homo sapiens
  source 1..2850: mol_type = other RNA
tcaggccaggcacagtggctcatgcctgtaatcccagcactttgggaggccgaggtgggtggatcacttgaagccaggagttcgagaccagcctggccaacatagcaaaaccttgtctctattacaaatatgcccatgtgctaggtgtggtgggacacacctgtaatcccagctacccaggagaatcgcttaaacccgggaggcggaagttgcagtgagctgagatcataacaccgcactccaccctgagtgacagggcaagactcaaaaaataaaaaaggaacattaactagggttagaaactaacttcattctttttagaattcaacagttttcctaggtcaccaattccaccttttgttcttattaaggcgcaaagtcacaggacccccttcctgggagtcactgtcattaaatctattgccgtcagctcagcccagggtaggcaaggttcaagaatgggaagtgcttttgtctggggaaacacgcaggtaatgtgatgctaggaaggaggatgtgcaggtgggtgagagcccaggagggagcagctggtgcctgacagggtgagccatcagggctgggcctgggtacagccccaggagaaggagcctgtgcagaagtagcagttcagtggattccacctcctatgtcacaatccagcaggtggccaggactcagcctgggttttaagtgagtaatgccttccctgtctcagagattagctctaacagtgtcactagaggaagccctggcgagggtgggggggcgtagtgtggggacaaggaggccagatagaaagtgctggaatgttctggaacagatctgtttctggaggagaggctgagtatggagagtcaacagaatgtgaccaccttcagagggaggagctgggccgtctccaataaatccagggacaaatgccttcagtcctcagactgttccaatagaggggacgccacgtatcccagggttccctttccaactcatgtcaacacctgcagtccctttgaggagactaaatgtatttcatgctggaaagaacagattttctctcattaaaaatagccccactaaaggagaccaacatgctagaagtgcggcaccagggcctcaagactacacttcggaacatgaagagggctggggaccgctcggcccaagtctggatcttgtaaccaacagatgccgagcttgccgttcaactaggcacagaaagcagactcggtctgggattccagttggtctgattcagttcaagagggtcacagtcagaagaaagctttttccattaggagcttcagcagagtgaagagttcaacacagcaaacaggcaggcagctcctttgtatatgtgacggggtggccctgactgtaaacacagccctaccagtcactgcagctcatggcctgagaagacattccagtggcagcctcgggtgtccactcagttcacatattctggtttcacctgcccaagctgtcttcaggcatgaggtcttgtcagaattgggatgtggatgtctcctatgttaccatttattgtgtgggggcagccatcatcctatttgtctggtccatcaagcctagagcagtgagaagggcagccccttggatggtcctcctcagcagtctgtaccttcccagtttcccgctgcacaaggtcccgcatctcttctgtccagcccagaagctccactaggctttccacgccgtgaaccacgtcccccagctgggccacgtccctgctgcgaggatgccaagccaagggccccaccaagtcccggttgatgagcagtcggggaactgagctccgcacggcctcggtcaagctggcaaaaggctccacctccagggaggtcccaaggatgagcagcagatctgccatggggaaatcaaccacatgcagcaagaacctctggggcagcggctccccaaagaacacaatgtcgggcttcacaacgccggtgcagaccgggcagcggggaaccctgtctgccatcacgtcagcccgaatgtcctcccctgggaagggtctttggcagactgtgcaggtggcagaggcaaaggttccatgagcttcaaccagctttgaggcagggatgcccgacactctctcaagcccatcgatgttctgcgtgtagagccgcagaagcagccccttgtcatgaagcagccggagaaagtagtgagtgacgttgggcttgtagtttccagggtacagctccttggccaaagtgaaaaagggcttggggttgtgaaagaagaatgggagttcaaaaatggcctcggggtacgggagatcgtactgctggaggttgctgtacaggccactccccggcgatctgaagtctggaatgccactgggtgtgctgatgccggcccccaccatgaccaccaccctctggcaggctctggcccgaatcagctcagctacatcctgcagggaaagcttccccttgtcactgctgcctccacttccaacaacacttgaagcacccacagaaaaagatatggaccttcttccacctttaatactttttcaacccggatggcggtgatagttaatactttctgagcgcttttactatggtcaggcattatatttacacctaatcctcgcaaaacactactgggaagatcctcatttgacaggagcaattccgggtcacaaaggctgacaccacaaagctagtccgtagcgggttcgaccacaggcgcccacactctttgacgcctcaatggcacagccaagtgcgcgggaagtgggctgcaaacgccggagagttttgtccggagcgcagagacgcgctgtaaccgagcaaccagcggggcccgcccccggcctgctac

SEQ ID NO: 17536 - RNA, 2753 nt, Homo sapiens
  source 1..2753: mol_type = other RNA
tcaggccaggcacagtggctcatgcctgtaatcccagcactttgggaggccgaggtgggtggatcacttgaagccaggagttcgagaccagcctggccaacatagcaaaaccttgtctctattacaaatatgcccatgtgctaggtgtggtgggacacacctgtaatcccagctacccaggagaatcgcttaaacccgggaggcggaagttgcagtgagctgagatcataacaccgcactccaccctgagtgacagggcaagactcaaaaaataaaaaaggaacattaactagggttagaaactaacttcattctttttagaattcaacagttttcctaggtcaccaattccaccttttgttcttattaaggcgcaaagtcacaggacccccttcctgggagtcactgtcattaaatctattgccgtcagctcagcccagggtaggcaaggttcaagaatgggaagtgcttttgtctggggaaacacgcaggtaatgtgatgctaggaaggaggatgtgcaggtgggtgagagcccaggagggagcagctggtgcctgacagggtgagccatcagggctgggcctgggtacagccccaggagaaggagcctgtgcagaagtagcagttcagtggattccacctcctatgtcacaatccagcaggtggccaggactcagcctgggttttaagtgagtaatgccttccctgtctcagagattagctctaacagtgtcactagaggaagccctggcgagggtgggggggcgtagtgtggggacaaggaggccagatagaaagtgctggaatgttctggaacagatctgtttctggaggagaggctgagtatggagagtcaacagaatgtgaccaccttcagagggaggagctgggccgtctccaataaatccagggacaaatgccttcagtcctcagactgttccaatagaggggacgccacgtatcccagggttccctttccaactcatgtcaacacctgcagtccctttgaggagactaaatgtatttcatgctggaaagaacagattttctctcattaaaaatagccccactaaaggagaccaacatgctagaagtgcggcaccagggcctcaagactacacttcggaacatgaagagggctggggaccgctcggcccaagtctggatcttgtaaccaacagatgccgagcttgccgttcaactaggcacagaaagcagactcggtctgggattccagttggtctgattcagttcaagagggtcacagtcagaagaaagctttttccattaggagcttcagcagagtgaagagttcaacacagcaaacaggcaggcagctcctttgtatatgtgacggggtggccctgactgtaaacacagccctaccagtcactgcagctcatggcctgagaagacattccagtggcagcctcgggtgtccactcagttcacatattctggtttcacctgcccaagctgtcttcaggcatgaggtcttgtcagaattgggatgtggatgtctcctatgttaccatttattgtgtgggggcagccatcatcctatttgtctggtccatcaagcctagagcagtgagaagggcagccccttggatggtcctcctcagcagtctgtaccttcccagtttcccgctgcacaaggtcccgcatctcttctgtccagcccagaagctccactaggctttccacgccgtgaaccacgtcccccagctgggccacgtccctgctgcgaggatgccaagccaagggccccaccaagtcccggttgatgagcagtcggggaactgagctccgcacggcctcggtcaagctggcaaaaggctccacctccagggaggtcccaaggatgagcagcagatctgccatggggaaatcaaccacatgcagcaagaacctctggggcagcggctccccaaagaacacaatgtcgggcttcacaacgccggtgcagaccgggcagcggggaaccctgtctgccatcacgtcagcccgaatgtcctcccctgggaagggtctttggcagactgtgcaggtggcagaggcaaaggttccatgagcttcaaccagctttgaggcagggatgcccgacactctctcaagcccatcgatgttctgcgtgtagagccgcagaagcagccccttgtcatgaagcagccggagaaagtagtgagtgacgttgggcttgtagtttccagggtacagctccttggccaaagtgaaaaagggcttggggttgtgaaagaagaatgggagttcaaaaatggcctcggggtacgggagatcgtactgctggaggttgctgtacaggccactccccggcgatctgaagtctggaatgccactgggtgtgctgatgccggcccccaccatgaccaccaccctctggcaggctctggcccgaatcagctcagctacatcctttttcaacccggatggcggtgatagttaatactttctgagcgcttttactatggtcaggcattatatttacacctaatcctcgcaaaacactactgggaagatcctcatttgacaggagcaattccgggtcacaaaggctgacaccacaaagctagtccgtagcgggttcgaccacaggcgcccacactctttgacgcctcaatggcacagccaagtgcgcgggaagtgggctgcaaacgccggagagttttgtccggagcgcagagacgcgctgtaaccgagcaaccagcggggcccgcccccggcctgctac

SEQ ID NO: 17537 - RNA, 2939 nt, Homo sapiens
  source 1..2939: mol_type = other RNA
tcaggccaggcacagtggctcatgcctgtaatcccagcactttgggaggccgaggtgggtggatcacttgaagccaggagttcgagaccagcctggccaacatagcaaaaccttgtctctattacaaatatgcccatgtgctaggtgtggtgggacacacctgtaatcccagctacccaggagaatcgcttaaacccgggaggcggaagttgcagtgagctgagatcataacaccgcactccaccctgagtgacagggcaagactcaaaaaataaaaaaggaacattaactagggttagaaactaacttcattctttttagaattcaacagttttcctaggtcaccaattccaccttttgttcttattaaggcgcaaagtcacaggacccccttcctgggagtcactgtcattaaatctattgccgtcagctcagcccagggtaggcaaggttcaagaatgggaagtgcttttgtctggggaaacacgcaggtaatgtgatgctaggaaggaggatgtgcaggtgggtgagagcccaggagggagcagctggtgcctgacagggtgagccatcagggctgggcctgggtacagccccaggagaaggagcctgtgcagaagtagcagttcagtggattccacctcctatgtcacaatccagcaggtggccaggactcagcctgggttttaagtgagtaatgccttccctgtctcagagattagctctaacagtgtcactagaggaagccctggcgagggtgggggggcgtagtgtggggacaaggaggccagatagaaagtgctggaatgttctggaacagatctgtttctggaggagaggctgagtatggagagtcaacagaatgtgaccaccttcagagggaggagctgggccgtctccaataaatccagggacaaatgccttcagtcctcagactgttccaatagaggggacgccacgtatcccagggttccctttccaactcatgtcaacacctgcagtccctttgaggagactaaatgtatttcatgctggaaagaacagattttctctcattaaaaatagccccactaaaggagaccaacatgctagaagtgcggcaccagggcctcaagactacacttcggaacatgaagagggctggggaccgctcggcccaagtctggatcttgtaaccaacagatgccgagcttgccgttcaactaggcacagaaagcagactcggtctgggattccagttggtctgattcagttcaagagggtcacagtcagaagaaagctttttccattaggagcttcagcagagtgaagagttcaacacagcaaacaggcaggcagctcctttgtatatgtgacggggtggccctgactgtaaacacagccctaccagtcactgcagctcatggcctgagaagacattccagtggcagcctcgggtgtccactcagttcacatattctggtttcacctgcccaagctgtcttcaggcatgaggtcttgtcagaattgggatgtggatgtctcctatgttaccatttattgtgtgggggcagccatcatcctatttgtctggtccatcaagcctagagcagtgagaagggcagccccttggatggtcctcctcagcagtctgtaccttcccagtttcccgctgcacaaggtcccgcatctcttctgtccagcccagaagctccactaggctttccacgccgtgaaccacgtcccccagctgggccacgtccctgctgcgaggatgccaagccaagggccccaccaagtcccggttgatgagcagtcggggaactgagctccgcacggcctcggtcaagctggcaaaaggctccacctccagggaggtcccaaggatgagcagcagatctgccatggggaaatcaaccacatgcagcaagaacctctggggcagcggctccccaaagaacacaatgtcgggcttcacaacgccggtgcagaccgggcagcggggaaccctgtctgccatcacgtcagcccgaatgtcctcccctgggaagggtctttggcagactgtgcaggtggcagaggcaaaggttccatgagcttcaaccagctttgaggcagggatgcccgacactgaaattcaagccaaagcgaagtgttgctgccgcctccgagatgagcacgcaaggccaagagcacaacttctgggcttggcaggactcctctctcaagcccatcgatgttctgcgtgtagagccgcagaagcagccccttgtcatgaagcagccggagaaagtagtgagtgacgttgggcttgtagtttccagggtacagctccttggccaaagtgaaaaagggcttggggttgtgaaagaagaatgggagttcaaaaatggcctcggggtacgggagatcgtactgctggaggttgctgtacaggccactccccggcgatctgaagtctggaatgccactgggtgtgctgatgccggcccccaccatgaccaccaccctctggcaggctctggcccgaatcagctcagctacatcctgcagggaaagcttccccttgtcactgctgcctccacttccaacaacacttgaagcacccacagaaaaagatatggaccttcttccacctttaatactttttcaacccggatggcggtgatagttaatactttctgagcgcttttactatggtcaggcattatatttacacctaatcctcgcaaaacactactgggaagatcctcatttgacaggagcaattccgggtcacaaaggctgacaccacaaagctagtccgtagcgggttcgaccacaggcgcccacactctttgacgcctcaatggcacagccaagtgcgcgggaagtgggctgcaaacgccggagagttttgtccggagcgcagagacgcgctgtaaccgagcaaccagcggggcccgcccccggcctgctac

SEQ ID NO: 17538 - RNA, 2837 nt, Homo sapiens
  source 1..2837: mol_type = other RNA
tcaggccaggcacagtggctcatgcctgtaatcccagcactttgggaggccgaggtgggtggatcacttgaagccaggagttcgagaccagcctggccaacatagcaaaaccttgtctctattacaaatatgcccatgtgctaggtgtggtgggacacacctgtaatcccagctacccaggagaatcgcttaaacccgggaggcggaagttgcagtgagctgagatcataacaccgcactccaccctgagtgacagggcaagactcaaaaaataaaaaaggaacattaactagggttagaaactaacttcattctttttagaattcaacagttttcctaggtcaccaattccaccttttgttcttattaaggcgcaaagtcacaggacccccttcctgggagtcactgtcattaaatctattgccgtcagctcagcccagggtaggcaaggttcaagaatgggaagtgcttttgtctggggaaacacgcaggtaatgtgatgctaggaaggaggatgtgcaggtgggtgagagcccaggagggagcagctggtgcctgacagggtgagccatcagggctgggcctgggtacagccccaggagaaggagcctgtgcagaagtagcagttcagtggattccacctcctatgtcacaatccagcaggtggccaggactcagcctgggttttaagtgagtaatgccttccctgtctcagagattagctctaacagtgtcactagaggaagccctggcgagggtgggggggcgtagtgtggggacaaggaggccagatagaaagtgctggaatgttctggaacagatctgtttctggaggagaggctgagtatggagagtcaacagaatgtgaccaccttcagagggaggagctgggccgtctccaataaatccagggacaaatgccttcagtcctcagactgttccaatagaggggacgccacgtatcccagggttccctttccaactcatgtcaacacctgcagtccctttgaggagactaaatgtatttcatgctggaaagaacagattttctctcattaaaaatagccccactaaaggagaccaacatgctagaagtgcggcaccagggcctcaagactacacttcggaacatgaagagggctggggaccgctcggcccaagtctggatcttgtaaccaacagatgccgagcttgccgttcaactaggcacagaaagcagactcggtctgggattccagttggtctgattcagttcaagagggtcacagtcagaagaaagctttttccattaggagcttcagcagagtgaagagttcaacacagcaaacaggcaggcagctcctttgtatatgtgacggggtggccctgactgtaaacacagccctaccagtcactgcagctcatggcctgagaagacattccagtggcagcctcgggtgtccactcagttcacatattctggtttcacctgcccaagctgtcttcaggcatgaggtcttgtcagaattgggatgtggatgtctcctatgttaccatttattgtgtgggggcagccatcatcctatttgtctggtccatcaagcctagagcagtgagaagggcagccccttggatggtcctcctcagcagtctgtaccttcccagtttcccgctgcacaaggtcccgcatctcttctgtccagcccagaagctccactaggctttccacgccgtgaaccacgtcccccagctgggccacgtccctgctgcgaggatgccaagccaagggccccaccaagtcccggttgatgagcagtcggggaactgagctccgcacggcctcggtcaagctggcaaaaggctccacctccagggaggtcccaaggatgagcagcagatctgccatggggaaatcaaccacatgcagcaagaacctctggggcagcggctccccaaagaacacaatgtcgggcttcacaacgccggtgcagaccgggcagcggggaaccctgtctgccatcacgtcagcccgaatgtcctcccctgggaagggtctttggcagactgtgcaggtggcagaggcaaaggttccatgagcttcaaccagctttgaggcagggatgcccgacactgaaattcaagccaaagcgaagtgttgctgccgcctccgagatgagcacgcaaggccaagagcacaacttctgggcttggcaggactcctggaaggaggcacagccccttggggttgtgatgtcctcaagcctggttttcatgcccgtatcacctctctcaagcccatcgatgttctgcgtgtagagccgcagaagcagccccttgtcatgaagcagccggagaaagtagtgagtgacgttgggcttgtagtttccagggtacagctccttggccaaagtgaaaaagggcttggggttgtgaaagaagaatgggagttcaaaaatggcctcggggtacgggagatcgtactgctggaggttgctgtacaggccactccccggcgatctgaagtctggaatgccactgggtgtgctgatgccggcccccaccatgaccaccaccctctggcaggctctggcccgaatcagctcagctacatcctgcagggaaagcttccccttgtcactgctgcctccacttccaacaacacttgaagcacccacagaaaaagatatggaccttcttccacctttaataatcgtccctgccgccaagcaccagccgacagccgcaggcctgaaacggccccacgcctcccccggcctcgacccgttcaactacccggccccacagccggagggctgccgcggcgcgccaaccccagaacgccatgttccgcgcagtcc

SEQ ID NO: 17539 - RNA, 3388 nt, Homo sapiens
  source 1..3388: mol_type = other RNA
tcaggccaggcacagtggctcatgcctgtaatcccagcactttgggaggccgaggtgggtggatcacttgaagccaggagttcgagaccagcctggccaacatagcaaaaccttgtctctattacaaatatgcccatgtgctaggtgtggtgggacacacctgtaatcccagctacccaggagaatcgcttaaacccgggaggcggaagttgcagtgagctgagatcataacaccgcactccaccctgagtgacagggcaagactcaaaaaataaaaaaggaacattaactagggttagaaactaacttcattctttttagaattcaacagttttcctaggtcaccaattccaccttttgttcttattaaggcgcaaagtcacaggacccccttcctgggagtcactgtcattaaatctattgccgtcagctcagcccagggtaggcaaggttcaagaatgggaagtgcttttgtctggggaaacacgcaggtaatgtgatgctaggaaggaggatgtgcaggtgggtgagagcccaggagggagcagctggtgcctgacagggtgagccatcagggctgggcctgggtacagccccaggagaaggagcctgtgcagaagtagcagttcagtggattccacctcctatgtcacaatccagcaggtggccaggactcagcctgggttttaagtgagtaatgccttccctgtctcagagattagctctaacagtgtcactagaggaagccctggcgagggtgggggggcgtagtgtggggacaaggaggccagatagaaagtgctggaatgttctggaacagatctgtttctggaggagaggctgagtatggagagtcaacagaatgtgaccaccttcagagggaggagctgggccgtctccaataaatccagggacaaatgccttcagtcctcagactgttccaatagaggggacgccacgtatcccagggttccctttccaactcatgtcaacacctgcagtccctttgaggagactaaatgtatttcatgctggaaagaacagattttctctcattaaaaatagccccactaaaggagaccaacatgctagaagtgcggcaccagggcctcaagactacacttcggaacatgaagagggctggggaccgctcggcccaagtctggatcttgtaaccaacagatgccgagcttgccgttcaactaggcacagaaagcagactcggtctgggattccagttggtctgattcagttcaagagggtcacagtcagaagaaagctttttccattaggagcttcagcagagtgaagagttcaacacagcaaacaggcaggcagctcctttgtatatgtgacggggtggccctgactgtaaacacagccctaccagtcactgcagctcatggcctgagaagacattccagtggcagcctcgggtgtccactcagttcacatattctggtttcacctgcccaagctgtcttcaggcatgaggtcttgtcagaattgggatgtggatgtctcctatgttaccatttattgtgtgggggcagccatcatcctatttgtctggtccatcaagcctagagcagtgagaagggcagccccttggatggtcctcctcagcagtctgtaccttcccagtttcccgctgcacaaggtcccgcatctcttctgtccagcccagaagctccactaggctttccacgccgtgaaccacgtcccccagctgggccacgtccctgctgcgaggatgccaagccaagggccccaccaagtcccggttgatgagcagtcggggaactgagctccgcacggcctcggtcaagctggcaaaaggctccacctgaaaaatgggccaaacgtgaggggcacagtgtccactttacaagctcctcaggatgtttcatgccacagccaccgaggccttggaggagcagcagattggcagtcagagcctgcgatatagggaaaacccaccaccaatctcatttcttcagctgagctcctgccgcttggcctccgtgacggttttctcccctccgcctctctctctctctcccacttcttgctgtttccacacatccttgcttttccccacctccgttccaaggctcatcagggatccaaccttcctgcctcctctttgtgagcacgttctgttctccctgtcctccccacctcgctgtctcccagcatgacgcagagggacaacagcacagactcgtccatctcctctggctagccctgcttgctctgacagccaccaccagcatcgggcacccagacgagctggtgcccccgagcaggagttactgttacgtctctccatggtcttccccacccagcctctagagaggcctagctcggtgccatcaggcttcttcatacagctctcaaagcttctccagggaggtcccaaggatgagcagcagatctgccatggggaaatcaaccacatgcagcaagaacctctggggcagcggctccccaaagaacacaatgtcgggcttcacaacgccggtgcagaccgggcagcggggaaccctgtctgccatcacgtcagcccgaatgtcctcccctgggaagggtctttggcagactgtgcaggtggcagaggcaaaggttccatgagcttcaaccagctttgaggcagggatgcccgacactctctcaagcccatcgatgttctgcgtgtagagccgcagaagcagccccttgtcatgaagcagccggagaaagtagtgagtgacgttgggcttgtagtttccagggtacagctccttggccaaagtgaaaaagggcttggggttgtgaaagaagaatgggagttcaaaaatggcctcggggtacgggagatcgtactgctggaggttgctgtacaggccactccccggcgatctgaagtctggaatgccactgggtgtgctgatgccggcccccaccatgaccaccaccctctggcaggctctggcccgaatcagctcagctacatcctgcagggaaagcttccccttgtcactgctgcctccacttccaacaacacttgaagcacccacagaaaaagatatggaccttcttccacctttaatactcgaaaagaagaaactgggagctgctgccctcggctgcctccggaatgccctgggcacctcgggtctgggaggcctctgcaaggggcgcgccgggtccaagggctcaccgcgggccccatggctgcctctcagccccgcactcacatcgtccctgccgccaagcaccagccgacagccgcaggcctgaaacggccccacgcctcccccggcctcgacccgttcaactacccggccccacagccggagggctgccgcggcgcgccaaccccagaacgccatgttccgcgcagtcc

SEQ ID NO: 17540 - RNA, 3146 nt, Homo sapiens
  source 1..3146: mol_type = other RNA
tcaggccaggcacagtggctcatgcctgtaatcccagcactttgggaggccgaggtgggtggatcacttgaagccaggagttcgagaccagcctggccaacatagcaaaaccttgtctctattacaaatatgcccatgtgctaggtgtggtgggacacacctgtaatcccagctacccaggagaatcgcttaaacccgggaggcggaagttgcagtgagctgagatcataacaccgcactccaccctgagtgacagggcaagactcaaaaaataaaaaaggaacattaactagggttagaaactaacttcattctttttagaattcaacagttttcctaggtcaccaattccaccttttgttcttattaaggcgcaaagtcacaggacccccttcctgggagtcactgtcattaaatctattgccgtcagctcagcccagggtaggcaaggttcaagaatgggaagtgcttttgtctggggaaacacgcaggtaatgtgatgctaggaaggaggatgtgcaggtgggtgagagcccaggagggagcagctggtgcctgacagggtgagccatcagggctgggcctgggtacagccccaggagaaggagcctgtgcagaagtagcagttcagtggattccacctcctatgtcacaatccagcaggtggccaggactcagcctgggttttaagtgagtaatgccttccctgtctcagagattagctctaacagtgtcactagaggaagccctggcgagggtgggggggcgtagtgtggggacaaggaggccagatagaaagtgctggaatgttctggaacagatctgtttctggaggagaggctgagtatggagagtcaacagaatgtgaccaccttcagagggaggagctgggccgtctccaataaatccagggacaaatgccttcagtcctcagactgttccaatagaggggacgccacgtatcccagggttccctttccaactcatgtcaacacctgcagtccctttgaggagactaaatgtatttcatgctggaaagaacagattttctctcattaaaaatagccccactaaaggagaccaacatgctagaagtgcggcaccagggcctcaagactacacttcggaacatgaagagggctggggaccgctcggcccaagtctggatcttgtaaccaacagatgccgagcttgccgttcaactaggcacagaaagcagactcggtctgggattccagttggtctgattcagttcaagagggtcacagtcagaagaaagctttttccattaggagcttcagcagagtgaagagttcaacacagcaaacaggcaggcagctcctttgtatatgtgacggggtggccctgactgtaaacacagccctaccagtcactgcagctcatggcctgagaagacattccagtggcagcctcgggtgtccactcagttcacatattctggtttcacctgcccaagctgtcttcaggcatgaggtcttgtcagaattgggatgtggatgtctcctatgttaccatttattgtgtgggggcagccatcatcctatttgtctggtccatcaagcctagagcagtgagaagggcagccccttggatggtcctcctcagcagtctgtaccttcccagtttcccgctgcacaaggtcccgcatctcttctgtccagcccagaagctccactaggctttccacgccgtgaaccacgtcccccagctgggccacgtccctgctgcgaggatgccaagccaagggccccaccaagtcccggttgatgagcagtcggggaactgagctccgcacggcctcggtcaagctggcaaaaggctccacctgaaaaatgggccaaacgtgaggggcacagtgtccactttacaagctcctcaggatgtttcatgccacagccaccgaggccttggaggagcagcagattggcagtcagagcctgcgatatagggaaaacccaccaccaatctcatttcttcagctgagctcctgccgcttggcctccgtgacggttttctcccctccgcctctctctctctctcccacttcttgctgtttccacacatccttgcttttccccacctccgttccaaggctcatcagggatccaaccttcctgcctcctctttgtgagcacgttctgttctccctgtcctccccacctcgctgtctcccagcatgacgcagagggacaacagcacagactcgtccatctcctctggctagccctgcttgctctgacagccaccaccagcatcgggcacccagacgagctggtgcccccgagcaggagttactgttacgtctctccatggtcttccccacccagcctctagagaggcctagctcggtgccatcaggcttcttcatacagctctcaaagcttctctctcaagcccatcgatgttctgcgtgtagagccgcagaagcagccccttgtcatgaagcagccggagaaagtagtgagtgacgttgggcttgtagtttccagggtacagctccttggccaaagtgaaaaagggcttggggttgtgaaagaagaatgggagttcaaaaatggcctcggggtacgggagatcgtactgctggaggttgctgtacaggccactccccggcgatctgaagtctggaatgccactgggtgtgctgatgccggcccccaccatgaccaccaccctctggcaggctctggcccgaatcagctcagctacatcctgcagggaaagcttccccttgtcactgctgcctccacttccaacaacacttgaagcacccacagaaaaagatatggaccttcttccacctttaatactttttcaacccggatggcggtgatagttaatactttctgagcgcttttactatggtcaggcattatatttacacctaatcctcgcaaaacactactgggaagatcctcatttgacaggagcaattccgggtcacaaaggctgacaccacaaagctagtccgtagcgggttcgaccacaggcgcccacactctttgacgcctcaatggcacagccaagtgcgcgggaagtgggctgcaaacgccggagagttttgtccggagcgcagagacgcgctgtaaccgagcaaccagcggggcccgcccccggcctgctac

SEQ ID NO: 17541 - RNA, 2419 nt, Homo sapiens
  source 1..2419: mol_type = other RNA
tcaggccaggcacagtggctcatgcctgtaatcccagcactttgggaggccgaggtgggtggatcacttgaagccaggagttcgagaccagcctggccaacatagcaaaaccttgtctctattacaaatatgcccatgtgctaggtgtggtgggacacacctgtaatcccagctacccaggagaatcgcttaaacccgggaggcggaagttgcagtgagctgagatcataacaccgcactccaccctgagtgacagggcaagactcaaaaaataaaaaaggaacattaactagggttagaaactaacttcattctttttagaattcaacagttttcctaggtcaccaattccaccttttgttcttattaaggcgcaaagtcacaggacccccttcctgggagtcactgtcattaaatctattgccgtcagctcagcccagggtaggcaaggttcaagaatgggaagtgcttttgtctggggaaacacgcaggtaatgtgatgctaggaaggaggatgtgcaggtgggtgagagcccaggagggagcagctggtgcctgacagggtgagccatcagggctgggcctgggtacagccccaggagaaggagcctgtgcagaagtagcagttcagtggattccacctcctatgtcacaatccagcaggtggccaggactcagcctgggttttaagtgagtaatgccttccctgtctcagagattagctctaacagtgtcactagaggaagccctggcgagggtgggggggcgtagtgtggggacaaggaggccagatagaaagtgctggaatgttctggaacagatctgtttctggaggagaggctgagtatggagagtcaacagaatgtgaccaccttcagagggaggagctgggccgtctccaataaatccagggacaaatgccttcagtcctcagactgttccaatagaggggacgccacgtatcccagggttccctttccaactcatgtcaacacctgcagtccctttgaggagactaaatgtatttcatgctggaaagaacagattttctctcattaaaaatagccccactaaaggagaccaacatgctagaagtgcggcaccagggcctcaagactacacttcggaacatgaagagggctggggaccgctcggcccaagtctggatcttgtaaccaacagatgccgagcttgccgttcaactaggcacagaaagcagactcggtctgggattccagttggtctgattcagttcaagagggtcacagtcagaagaaagctttttccattaggagcttcagcagagtgaagagttcaacacagcaaacaggcaggcagctcctttgtatatgtgacggggtggccctgactgtaaacacagccctaccagtcactgcagctcatggcctgagaagacattccagtggcagcctcgggtgtccactcagttcacatattctggtttcacctgcccaagctgtcttcaggcatgaggtcttgtcagaattgggatgtggatgtctcctatgttaccatttattgtgtgggggcagccatcatcctatttgtctggtccatcaagctccagggaggtcccaaggatgagcagcagatctgccatggggaaatcaaccacatgcagcaagaacctctggggcagcggctccccaaagaacacaatgtcgggcttcacaacgccggtgcagaccgggcagcggggaaccctgtctgccatcacgtcagcccgaatgtcctcccctgggaagggtctttggcagactgtgcaggtggcagaggcaaaggttccatgagcttcaaccagctttgaggcagggatgcccgacactctctcaagcccatcgatgttctgcgtgtagagccgcagaagcagccccttgtcatgaagcagccggagaaagtagtgagtgacgttgggcttgtagtttccagggtacagctccttggccaaagtgaaaaagggcttggggttgtgaaagaagaatgggagttcaaaaatggcctcggggtacgggagatcgtactgctggaggttgctgtacaggccactccccggcgatctgaagtctggaatgccactgggtgtgctgatgccggcccccaccatgaccaccaccctctggcaggctctggcccgaatcagctcagctacatcctgcagggaaagcttccccttgtcactgctgcctccacttccaacaacacttgaagcacccacagaaaaagatatggaccttcttccacctttaataatcgtccctgccgccaagcaccagccgacagccgcaggcctgaaacggccccacgcctcccccggcctcgacccgttcaactacccggccccacagccggagggctgccgcggcgcgccaaccccagaacgccatgttccgcgcagtcc

SEQ ID NO: 17542 - RNA, 2511 nt, Homo sapiens
  source 1..2511: mol_type = other RNA
tcaggccaggcacagtggctcatgcctgtaatcccagcactttgggaggccgaggtgggtggatcacttgaagccaggagttcgagaccagcctggccaacatagcaaaaccttgtctctattacaaatatgcccatgtgctaggtgtggtgggacacacctgtaatcccagctacccaggagaatcgcttaaacccgggaggcggaagttgcagtgagctgagatcataacaccgcactccaccctgagtgacagggcaagactcaaaaaataaaaaaggaacattaactagggttagaaactaacttcattctttttagaattcaacagttttcctaggtcaccaattccaccttttgttcttattaaggcgcaaagtcacaggacccccttcctgggagtcactgtcattaaatctattgccgtcagctcagcccagggtaggcaaggttcaagaatgggaagtgcttttgtctggggaaacacgcaggtaatgtgatgctaggaaggaggatgtgcaggtgggtgagagcccaggagggagcagctggtgcctgacagggtgagccatcagggctgggcctgggtacagccccaggagaaggagcctgtgcagaagtagcagttcagtggattccacctcctatgtcacaatccagcaggtggccaggactcagcctgggttttaagtgagtaatgccttccctgtctcagagattagctctaacagtgtcactagaggaagccctggcgagggtgggggggcgtagtgtggggacaaggaggccagatagaaagtgctggaatgttctggaacagatctgtttctggaggagaggctgagtatggagagtcaacagaatgtgaccaccttcagagggaggagctgggccgtctccaataaatccagggacaaatgccttcagtcctcagactgttccaatagaggggacgccacgtatcccagggttccctttccaactcatgtcaacacctgcagtccctttgaggagactaaatgtatttcatgctggaaagaacagattttctctcattaaaaatagccccactaaaggagaccaacatgctagaagtgcggcaccagggcctcaagactacacttcggaacatgaagagggctggggaccgctcggcccaagtctggatcttgtaaccaacagatgccgagcttgccgttcaactaggcacagaaagcagactcggtctgggattccagttggtctgattcagttcaagagggtcacagtcagaagaaagctttttccattaggagcttcagcagagtgaagagttcaacacagcaaacaggcaggcagctcctttgtatatgtgacggggtggccctgactgtaaacacagccctaccagtcactgcagctcatggcctgagaagacattccagtggcagcctcgggtgtccactcagttcacatattctggtttcacctgcccaagctgtcttcaggcatgaggtcttgtcagaattgggatgtggatgtctcctatgttaccatttattgtgtgggggcagccatcatcctatttgtctggtccatcaagctccagggaggtcccaaggatgagcagcagatctgccatggggaaatcaaccacatgcagcaagaacctctggggcagcggctccccaaagaacacaatgtcgggcttcacaacgccggtgcagaccgggcagcggggaaccctgtctgccatcacgtcagcccgaatgtcctcccctgggaagggtctttggcagactgtgcaggtggcagaggcaaaggttccatgagcttcaaccagctttgaggcagggatgcccgacactctctcaagcccatcgatgttctgcgtgtagagccgcagaagcagccccttgtcatgaagcagccggagaaagtagtgagtgacgttgggcttgtagtttccagggtacagctccttggccaaagtgaaaaagggcttggggttgtgaaagaagaatgggagttcaaaaatggcctcggggtacgggagatcgtactgctggaggttgctgtacaggccactccccggcgatctgaagtctggaatgccactgggtgtgctgatgccggcccccaccatgaccaccaccctctggcaggctctggcccgaatcagctcagctacatcctgcagggaaagcttccccttgtcactgctgcctccacttccaacaacacttgaagcacccacagaaaaagatatggaccttcttccacctttaatactaatcctcgcaaaacactactgggaagatcctcatttgacaggagcaattccgggtcacaaaggctgacaccacaaagctagtccgtagcgggttcgaccacaggcgcccacactctttgacgcctcaatggcacagccaagtgcgcgggaagtgggctgcaaacgccggagagttttgtccggagcgcagagacgcgctgtaaccgagcaaccagcggggcccgcccccggcctgctac

SEQ ID NO: 17543 - RNA, 2613 nt, Homo sapiens
  source 1..2613: mol_type = other RNA
tcaggccaggcacagtggctcatgcctgtaatcccagcactttgggaggccgaggtgggtggatcacttgaagccaggagttcgagaccagcctggccaacatagcaaaaccttgtctctattacaaatatgcccatgtgctaggtgtggtgggacacacctgtaatcccagctacccaggagaatcgcttaaacccgggaggcggaagttgcagtgagctgagatcataacaccgcactccaccctgagtgacagggcaagactcaaaaaataaaaaaggaacattaactagggttagaaactaacttcattctttttagaattcaacagttttcctaggtcaccaattccaccttttgttcttattaaggcgcaaagtcacaggacccccttcctgggagtcactgtcattaaatctattgccgtcagctcagcccagggtaggcaaggttcaagaatgggaagtgcttttgtctggggaaacacgcaggtaatgtgatgctaggaaggaggatgtgcaggtgggtgagagcccaggagggagcagctggtgcctgacagggtgagccatcagggctgggcctgggtacagccccaggagaaggagcctgtgcagaagtagcagttcagtggattccacctcctatgtcacaatccagcaggtggccaggactcagcctgggttttaagtgagtaatgccttccctgtctcagagattagctctaacagtgtcactagaggaagccctggcgagggtgggggggcgtagtgtggggacaaggaggccagatagaaagtgctggaatgttctggaacagatctgtttctggaggagaggctgagtatggagagtcaacagaatgtgaccaccttcagagggaggagctgggccgtctccaataaatccagggacaaatgccttcagtcctcagactgttccaatagaggggacgccacgtatcccagggttccctttccaactcatgtcaacacctgcagtccctttgaggagactaaatgtatttcatgctggaaagaacagattttctctcattaaaaatagccccactaaaggagaccaacatgctagaagtgcggcaccagggcctcaagactacacttcggaacatgaagagggctggggaccgctcggcccaagtctggatcttgtaaccaacagatgccgagcttgccgttcaactaggcacagaaagcagactcggtctgggattccagttggtctgattcagttcaagagggtcacagtcagaagaaagctttttccattaggagcttcagcagagtgaagagttcaacacagcaaacaggcaggcagctcctttgtatatgtgacggggtggccctgactgtaaacacagccctaccagtcactgcagctcatggcctgagaagacattccagtggcagcctcgggtgtccactcagttcacatattctggtttcacctgcccaagctgtcttcaggcatgaggtcttgtcagaattgggatgtggatgtctcctatgttaccatttattgtgtgggggcagccatcatcctatttgtctggtccatcaagcttcccagtttcccgctgcacaaggtcccgcatctcttctgtccagcccagaagctccactaggctttccacgccgtgaaccacgtcccccagctgggccacgtccctgctgcgaggatgccaagccaagggccccaccaagtcccggttgatgagcagtcggggaactgagctccgcacggcctcggtcaagctggcaaaaggctccacccgaatgtcctcccctgggaagggtctttggcagactgtgcaggtggcagaggcaaaggttccatgagcttcaaccagctttgaggcagggatgcccgacactctctcaagcccatcgatgttctgcgtgtagagccgcagaagcagccccttgtcatgaagcagccggagaaagtagtgagtgacgttgggcttgtagtttccagggtacagctccttggccaaagtgaaaaagggcttggggttgtgaaagaagaatgggagttcaaaaatggcctcggggtacgggagatcgtactgctggaggttgctgtacaggccactccccggcgatctgaagtctggaatgccactgggtgtgctgatgccggcccccaccatgaccaccaccctctggcaggctctggcccgaatcagctcagctacatcctgcagggaaagcttccccttgtcactgctgcctccacttccaacaacacttgaagcacccacagaaaaagatatggaccttcttccacctttaatactcgaaaagaagaaactgggagctgctgccctcggctgcctccggaatgccctgggcacctcgggtctgggaggcctctgcaaggggcgcgccgggtccaagggctcaccgcgggccccatggctgcctctcagccccgcactcacatcgtccctgccgccaagcaccagccgacagccgcaggcctgaaacggccccacgcctcccccggcctcgacccgttcaactacccggccccacagccggagggctgccgcggcgcgccaaccccagaacgccatgttccgcgcagtcc

SEQ ID NO: 17544 - RNA, 2103 nt, Homo sapiens
  source 1..2103: mol_type = other RNA
tcaggccaggcacagtggctcatgcctgtaatcccagcactttgggaggccgaggtgggtggatcacttgaagccaggagttcgagaccagcctggccaacatagcaaaaccttgtctctattacaaatatgcccatgtgctaggtgtggtgggacacacctgtaatcccagctacccaggagaatcgcttaaacccgggaggcggaagttgcagtgagctgagatcataacaccgcactccaccctgagtgacagggcaagactcaaaaaataaaaaaggaacattaactagggttagaaactaacttcattctttttagaattcaacagttttcctaggtcaccaattccaccttttgttcttattaaggcgcaaagtcacaggacccccttcctgggagtcactgtcattaaatctattgccgtcagctcagcccagggtaggcaaggttcaagaatgggaagtgcttttgtctggggaaacacgcaggtaatgtgatgctaggaaggaggatgtgcaggtgggtgagagcccaggagggagcagctggtgcctgacagggtgagccatcagggctgggcctgggtacagccccaggagaaggagcctgtgcagaagtagcagttcagtggattccacctcctatgtcacaatccagcaggtggccaggactcagcctgggttttaagtgagtaatgccttccctgtctcagagattagctctaacagtgtcactagaggaagccctggcgagggtgggggggcgtagtgtggggacaaggaggccagatagaaagtgctggaatgttctggaacagatctgtttctggaggagaggctgagtatggagagtcaacagaatgtgaccaccttcagagggaggagctgggccgtctccaataaatccagggacaaatgccttcagtcctcagactgttccaatagaggggacgccacgtatcccagggttccctttccaactcatgtcaacacctgcagtccctttgaggagactaaatgtatttcatgctggaaagaacagattttctctcattaaaaatagccccactaaaggagaccaacatgctagaagtgcggcaccagggcctcaagactacacttcggaacatgaagagggctggggaccgctcggcccaagtctggatcttgtaaccaacagatgccgagcttgccgttcaactaggcacagaaagcagactcggtctgggattccagttggtctgattcagttcaagagggtcacagtcagaagaaagctttttccattaggagcttcagcagagtgaagagttcaacacagcaaacaggcaggcagctcctttgtatatgtgacggggtggccctgactgtaaacacagccctaccagtcactgcagctcatggcctgagaagacattccagtggcagcctcgggtgtccactcagttcacatattctggtttcacctgcccaagctgtcttcaggcatgaggtcttgtcagaattgggatgtggatgtctcctatgttaccatttattgtgtgggggcagccatcatcctatttgtctggtccatcaagcttcccagtttcccgctgcacaaggtcccgcatctcttctgtccagcccagaagctccactaggctttccacgccgtgaaccacgtcccccagctgggccacgtccctgctgcgaggatgccaagccaagggccccaccaagtcccggttgatgagcagtcggggaactgagctccgcacggcctcggtcaagctggcaaaaggctccacctccagggaggtcccaaggatgagcagcagatctgccatggggaaatcaaccacatgcagcaagaacctctggggcagcggctccccaaagaacacaatgtcgggcttcacaacgccggtgcagaccgggcagcggggaaccctgtctgccatcacgtcagcatcgtccctgccgccaagcaccagccgacagccgcaggcctgaaacggccccacgcctcccccggcctcgacccgttcaactacccggccccacagccggagggctgccgcggcgcgccaaccccagaacgccatgttccgcgcagtcc

SEQ ID NO: 17545 - RNA, 3038 nt, Homo sapiens
  source 1..3038: mol_type = other RNA
tcaggccaggcacagtggctcatgcctgtaatcccagcactttgggaggccgaggtgggtggatcacttgaagccaggagttcgagaccagcctggccaacatagcaaaaccttgtctctattacaaatatgcccatgtgctaggtgtggtgggacacacctgtaatcccagctacccaggagaatcgcttaaacccgggaggcggaagttgcagtgagctgagatcataacaccgcactccaccctgagtgacagggcaagactcaaaaaataaaaaaggaacattaactagggttagaaactaacttcattctttttagaattcaacagttttcctaggtcaccaattccaccttttgttcttattaaggcgcaaagtcacaggacccccttcctgggagtcactgtcattaaatctattgccgtcagctcagcccagggtaggcaaggttcaagaatgggaagtgcttttgtctggggaaacacgcaggtaatgtgatgctaggaaggaggatgtgcaggtgggtgagagcccaggagggagcagctggtgcctgacagggtgagccatcagggctgggcctgggtacagccccaggagaaggagcctgtgcagaagtagcagttcagtggattccacctcctatgtcacaatccagcaggtggccaggactcagcctgggttttaagtgagtaatgccttccctgtctcagagattagctctaacagtgtcactagaggaagccctggcgagggtgggggggcgtagtgtggggacaaggaggccagatagaaagtgctggaatgttctggaacagatctgtttctggaggagaggctgagtatggagagtcaacagaatgtgaccaccttcagagggaggagctgggccgtctccaataaatccagggacaaatgccttcagtcctcagactgttccaatagaggggacgccacgtatcccagggttccctttccaactcatgtcaacacctgcagtccctttgaggagactaaatgtatttcatgctggaaagaacagattttctctcattaaaaatagccccactaaaggagaccaacatgctagaagtgcggcaccagggcctcaagactacacttcggaacatgaagagggctggggaccgctcggcccaagtctggatcttgtaaccaacagatgccgagcttgccgttcaactaggcacagaaagcagactcggtctgggattccagttggtctgattcagttcaagagggtcacagtcagaagaaagctttttccattaggagcttcagcagagtgaagagttcaacacagcaaacaggcaggcagctcctttgtatatgtgacggggtggccctgactgtaaacacagccctaccagtcactgcagctcatggcctgagaagacattccagtggcagcctcgggtgtccactcagttcacatattctggtttcacctgcccaagctgtcttcaggcatgaggtcttgtcagaattgggatgtggatgtctcctatgttaccatttattgtgtgggggcagccatcatcctatttgtctggtccatcaagcttcccagtttcccgctgcacaaggtcccgcatctcttctgtccagcccagaagctccactaggctttccacgccgtgaaccacgtcccccagctgggccacgtccctgctgcgaggatgccaagccaagggccccaccaagtcccggttgatgagcagtcggggaactgagctccgcacggcctcggtcaagctggcaaaaggctccacctccagggaggtcccaaggatgagcagcagatctgccatggggaaatcaaccacatgcagcaagaacctctggggcagcggctccccaaagaacacaatgtcgggcttcacaacgccggtgcagaccgggcagcggggaaccctgtctgccatcacgtcagcccagaatgcagcacaagaagcagcaattacaggacagaagagtgatcaggaacagcaggagagagaaggtctaatgtatgttcaatcagaggtccctaaagagaggggccagatagtgggctaggggcaactcatatccgaagagataacggcagagtatgatccagcaaccatgaaagacgccaacccgcagattcaggatctcaagcaagtgagggctactgagccagcctgagggtgcccacaggaaaaacatgagtcacggcacatctgtgcttgtttctgtcccaagaggttctcaggaggtttagtaattacatgtggtccttcaaagagggagggtggctgtgaggtgagtggttacgtacttgtgagacttcagtaagtgcccagtaaatgtacattttacccgaatgtcctcccctgggaagggtctttggcagactgtgcaggtggcagaggcaaaggttccatgagcttcaaccagctttgaggcagggatgcccgacactctctcaagcccatcgatgttctgcgtgtagagccgcagaagcagccccttgtcatgaagcagccggagaaagtagtgagtgacgttgggcttgtagtttccagggtacagctccttggccaaagtgaaaaagggcttggggttgtgaaagaagaatgggagttcaaaaatggcctcggggtacgggagatcgtactgctggaggttgctgtacaggccactccccggcgatctgaagtctggaatgccactgggtgtgctgatgccggcccccaccatgaccaccaccctctggcaggctctggcccgaatcagctcagctacatcctgcagggaaagcttccccttgtcactgctgcctccacttccaacaacacttgaagcacccacagaaaaagatatggaccttcttccacctttaataatcgtccctgccgccaagcaccagccgacagccgcaggcctgaaacggccccacgcctcccccggcctcgacccgttcaactacccggccccacagccggagggctgccgcggcgcgccaaccccagaacgccatgttccgcgcagtcc

SEQ ID NO: 17546 - RNA, 3184 nt, Homo sapiens
  source 1..3184: mol_type = other RNA
tcaggccaggcacagtggctcatgcctgtaatcccagcactttgggaggccgaggtgggtggatcacttgaagccaggagttcgagaccagcctggccaacatagcaaaaccttgtctctattacaaatatgcccatgtgctaggtgtggtgggacacacctgtaatcccagctacccaggagaatcgcttaaacccgggaggcggaagttgcagtgagctgagatcataacaccgcactccaccctgagtgacagggcaagactcaaaaaataaaaaaggaacattaactagggttagaaactaacttcattctttttagaattcaacagttttcctaggtcaccaattccaccttttgttcttattaaggcgcaaagtcacaggacccccttcctgggagtcactgtcattaaatctattgccgtcagctcagcccagggtaggcaaggttcaagaatgggaagtgcttttgtctggggaaacacgcaggtaatgtgatgctaggaaggaggatgtgcaggtgggtgagagcccaggagggagcagctggtgcctgacagggtgagccatcagggctgggcctgggtacagccccaggagaaggagcctgtgcagaagtagcagttcagtggattccacctcctatgtcacaatccagcaggtggccaggactcagcctgggttttaagtgagtaatgccttccctgtctcagagattagctctaacagtgtcactagaggaagccctggcgagggtgggggggcgtagtgtggggacaaggaggccagatagaaagtgctggaatgttctggaacagatctgtttctggaggagaggctgagtatggagagtcaacagaatgtgaccaccttcagagggaggagctgggccgtctccaataaatccagggacaaatgccttcagtcctcagactgttccaatagaggggacgccacgtatcccagggttccctttccaactcatgtcaacacctgcagtccctttgaggagactaaatgtatttcatgctggaaagaacagattttctctcattaaaaatagccccactaaaggagaccaacatgctagaagtgcggcaccagggcctcaagactacacttcggaacatgaagagggctggggaccgctcggcccaagtctggatcttgtaaccaacagatgccgagcttgccgttcaactaggcacagaaagcagactcggtctgggattccagttggtctgattcagttcaagagggtcacagtcagaagaaagctttttccattaggagcttcagcagagtgaagagttcaacacagcaaacaggcaggcagctcctttgtatatgtgacggggtggccctgactgtaaacacagccctaccagtcactgcagctcatggcctgagaagacattccagtggcagcctcgggtgtccactcagttcacatattctggtttcacctgcccaagctgtcttcaggcatgaggtcttgtcagaattgggatgtggatgtctcctatgttaccatttattgtgtgggggcagccatcatcctatttgtctggtccatcaagcttcccagtttcccgctgcacaaggtcccgcatctcttctgtccagcccagaagctccactaggctttccacgccgtgaaccacgtcccccagctgggccacgtccctgctgcgaggatgccaagccaagggccccaccaagtcccggttgatgagcagtcggggaactgagctccgcacggcctcggtcaagctggcaaaaggctccacctccagggaggtcccaaggatgagcagcagatctgccatggggaaatcaaccacatgcagcaagaacctctggggcagcggctccccaaagaacacaatgtcgggcttcacaacgccggtgcagaccgggcagcggggaaccctgtctgccatcacgtcagcccagaatgcagcacaagaagcagcaattacaggacagaagagtgatcaggaacagcaggagagagaaggtctaatgtatgttcaatcagaggtccctaaagagaggggccagatagtgggctaggggcaactcatatccgaagagataacggcagagtatgatccagcaaccatgaaagacgccaacccgcagattcaggatctcaagcaagtgagggctactgagccagcctgagggtgcccacaggaaaaacatgagtcacggcacatctgtgcttgtttctgtcccaagaggttctcaggaggtttagtaattacatgtggtccttcaaagagggagggtggctgtgaggtgagtggttacgtacttgtgagacttcagtaagtgcccagtaaatgtacattttacccgaatgtcctcccctgggaagggtctttggcagactgtgcaggtggcagaggcaaaggttccatgagcttcaaccagctttgaggcagggatgcccgacactctctcaagcccatcgatgttctgcgtgtagagccgcagaagcagccccttgtcatgaagcagccggagaaagtagtgagtgacgttgggcttgtagtttccagggtacagctccttggccaaagtgaaaaagggcttggggttgtgaaagaagaatgggagttcaaaaatggcctcggggtacgggagatcgtactgctggaggttgctgtacaggccactccccggcgatctgaagtctggaatgccactgggtgtgctgatgccggcccccaccatgaccaccaccctctggcaggctctggcccgaatcagctcagctacatcctgcagggaaagcttccccttgtcactgctgcctccacttccaacaacacttgaagcacccacagaaaaagatatggaccttcttccacctttaatactcgaaaagaagaaactgggagctgctgccctcggctgcctccggaatgccctgggcacctcgggtctgggaggcctctgcaaggggcgcgccgggtccaagggctcaccgcgggccccatggctgcctctcagccccgcactcacatcgtccctgccgccaagcaccagccgacagccgcaggcctgaaacggccccacgcctcccccggcctcgacccgttcaactacccggccccacagccggagggctgccgcggcgcgccaaccccagaacgccatgttccgcgcagtcc

SEQ ID NO: 17547 - RNA, 3205 nt, Homo sapiens
  source 1..3205: mol_type = other RNA
tcaggccaggcacagtggctcatgcctgtaatcccagcactttgggaggccgaggtgggtggatcacttgaagccaggagttcgagaccagcctggccaacatagcaaaaccttgtctctattacaaatatgcccatgtgctaggtgtggtgggacacacctgtaatcccagctacccaggagaatcgcttaaacccgggaggcggaagttgcagtgagctgagatcataacaccgcactccaccctgagtgacagggcaagactcaaaaaataaaaaaggaacattaactagggttagaaactaacttcattctttttagaattcaacagttttcctaggtcaccaattccaccttttgttcttattaaggcgcaaagtcacaggacccccttcctgggagtcactgtcattaaatctattgccgtcagctcagcccagggtaggcaaggttcaagaatgggaagtgcttttgtctggggaaacacgcaggtaatgtgatgctaggaaggaggatgtgcaggtgggtgagagcccaggagggagcagctggtgcctgacagggtgagccatcagggctgggcctgggtacagccccaggagaaggagcctgtgcagaagtagcagttcagtggattccacctcctatgtcacaatccagcaggtggccaggactcagcctgggttttaagtgagtaatgccttccctgtctcagagattagctctaacagtgtcactagaggaagccctggcgagggtgggggggcgtagtgtggggacaaggaggccagatagaaagtgctggaatgttctggaacagatctgtttctggaggagaggctgagtatggagagtcaacagaatgtgaccaccttcagagggaggagctgggccgtctccaataaatccagggacaaatgccttcagtcctcagactgttccaatagaggggacgccacgtatcccagggttccctttccaactcatgtcaacacctgcagtccctttgaggagactaaatgtatttcatgctggaaagaacagattttctctcattaaaaatagccccactaaaggagaccaacatgctagaagtgcggcaccagggcctcaagactacacttcggaacatgaagagggctggggaccgctcggcccaagtctggatcttgtaaccaacagatgccgagcttgccgttcaactaggcacagaaagcagactcggtctgggattccagttggtctgattcagttcaagagggtcacagtcagaagaaagctttttccattaggagcttcagcagagtgaagagttcaacacagcaaacaggcaggcagctcctttgtatatgtgacggggtggccctgactgtaaacacagccctaccagtcactgcagctcatggcctgagaagacattccagtggcagcctcgggtgtccactcagttcacatattctggtttcacctgcccaagctgtcttcaggcatgaggtcttgtcagaattgggatgtggatgtctcctatgttaccatttattgtgtgggggcagccatcatcctatttgtctggtccatcaagcttcccagtttcccgctgcacaaggtcccgcatctcttctgtccagcccagaagctccactaggctttccacgccgtgaaccacgtcccccagctgggccacgtccctgctgcgaggatgccaagccaagggccccaccaagtcccggttgatgagcagtcggggaactgagctccgcacggcctcggtcaagctggcaaaaggctccacctccagggaggtcccaaggatgagcagcagatctgccatggggaaatcaaccacatgcagcaagaacctctggggcagcggctccccaaagaacacaatgtcgggcttcacaacgccggtgcagaccgggcagcggggaaccctgtctgccatcacgtcagcccagaatgcagcacaagaagcagcaattacaggacagaagagtgatcaggaacagcaggagagagaaggtctaatgtatgttcaatcagaggtccctaaagagaggggccagatagtgggctaggggcaactcatatccgaagagataacggcagagtatgatccagcaaccatgaaagacgccaacccgcagattcaggatctcaagcaagtgagggctactgagccagcctgagggtgcccacaggaaaaacatgagtcacggcacatctgtgcttgtttctgtcccaagaggttctcaggaggtttagtaattacatgtggtccttcaaagagggagggtggctgtgaggtgagtggttacgtacttgtgagacttcagtaagtgcccagtaaatgtacattttacccgaatgtcctcccctgggaagggtctttggcagactgtgcaggtggcagaggcaaaggttccatgagcttcaaccagctttgaggcagggatgcccgacactctctcaagcccatcgatgttctgcgtgtagagccgcagaagcagccccttgtcatgaagcagccggagaaagtagtgagtgacgttgggcttgtagtttccagggtacagctccttggccaaagtgaaaaagggcttggggttgtgaaagaagaatgggagttcaaaaatggcctcggggtacgggagatcgtactgctggaggttgctgtacaggccactccccggcgatctgaagtctggaatgccactgggtgtgctgatgccggcccccaccatgaccaccaccctctggcaggctctggcccgaatcagctcagctacatcctgcagggaaagcttccccttgtcactgctgcctccacttccaacaacacttgaagcacccacagaaaaagatatggaccttcttccacctttaatactttttcaacccggatggcggtgatagttaatactttctgagcgcttttactatggtcaggcattatatttacacctaatcctcgcaaaacactactgggaagatcctcatttgacaggagcaattccgggtcacaaaggctgacaccacaaagctagtccgtagcgggttcgaccacaggcgcccacactctttgacgcctcaatggcacagccaagtgcgcgggaagtgggctgcaaacgccggagagttttgtccggagcgcagagacgcgctgtaaccgagcaaccagcggggcccgcccccggcctgctac

SEQ ID NO: 17548 - RNA, 3273 nt, Homo sapiens
  source 1..3273: mol_type = other RNA
tcaggccaggcacagtggctcatgcctgtaatcccagcactttgggaggccgaggtgggtggatcacttgaagccaggagttcgagaccagcctggccaacatagcaaaaccttgtctctattacaaatatgcccatgtgctaggtgtggtgggacacacctgtaatcccagctacccaggagaatcgcttaaacccgggaggcggaagttgcagtgagctgagatcataacaccgcactccaccctgagtgacagggcaagactcaaaaaataaaaaaggaacattaactagggttagaaactaacttcattctttttagaattcaacagttttcctaggtcaccaattccaccttttgttcttattaaggcgcaaagtcacaggacccccttcctgggagtcactgtcattaaatctattgccgtcagctcagcccagggtaggcaaggttcaagaatgggaagtgcttttgtctggggaaacacgcaggtaatgtgatgctaggaaggaggatgtgcaggtgggtgagagcccaggagggagcagctggtgcctgacagggtgagccatcagggctgggcctgggtacagccccaggagaaggagcctgtgcagaagtagcagttcagtggattccacctcctatgtcacaatccagcaggtggccaggactcagcctgggttttaagtgagtaatgccttccctgtctcagagattagctctaacagtgtcactagaggaagccctggcgagggtgggggggcgtagtgtggggacaaggaggccagatagaaagtgctggaatgttctggaacagatctgtttctggaggagaggctgagtatggagagtcaacagaatgtgaccaccttcagagggaggagctgggccgtctccaataaatccagggacaaatgccttcagtcctcagactgttccaatagaggggacgccacgtatcccagggttccctttccaactcatgtcaacacctgcagtccctttgaggagactaaatgtatttcatgctggaaagaacagattttctctcattaaaaatagccccactaaaggagaccaacatgctagaagtgcggcaccagggcctcaagactacacttcggaacatgaagagggctggggaccgctcggcccaagtctggatcttgtaaccaacagatgccgagcttgccgttcaactaggcacagaaagcagactcggtctgggattccagttggtctgattcagttcaagagggtcacagtcagaagaaagctttttccattaggagcttcagcagagtgaagagttcaacacagcaaacaggcaggcagctcctttgtatatgtgacggggtggccctgactgtaaacacagccctaccagtcactgcagctcatggcctgagaagacattccagtggcagcctcgggtgtccactcagttcacatattctggtttcacctgcccaagctgtcttcaggcatgaggtcttgtcagaattgggatgtggatgtctcctatgttaccatttattgtgtgggggcagccatcatcctatttgtctggtccatcaagcttcccagtttcccgctgcacaaggtcccgcatctcttctgtccagcccagaagctccactaggctttccacgccgtgaaccacgtcccccagctgggccacgtccctgctgcgaggatgccaagccaagggccccaccaagtcccggttgatgagcagtcggggaactgagctccgcacggcctcggtcaagctggcaaaaggctccacctccagggaggtcccaaggatgagcagcagatctgccatggggaaatcaaccacatgcagcaagaacctctggggcagcggctccccaaagaacacaatgtcgggcttcacaacgccggtgcagaccgggcagcggggaaccctgtctgccatcacgtcagcccagaatgcagcacaagaagcagcaattacaggacagaagagtgatcaggaacagcaggagagagaaggtctaatgtatgttcaatcagaggtccctaaagagaggggccagatagtgggctaggggcaactcatatccgaagagataacggcagagtatgatccagcaaccatgaaagacgccaacccgcagattcaggatctcaagcaagtgagggctactgagccagcctgagggtgcccacaggaaaaacatgagtcacggcacatctgtgcttgtttctgtcccaagaggttctcaggaggtttagtaattacatgtggtccttcaaagagggagggtggctgtgaggtgagtggttacgtacttgtgagacttcagtaagtgcccagtaaatgtacattttacccgaatgtcctcccctgggaagggtctttggcagactgtgcaggtggcagaggcaaaggttccatgagcttcaaccagctttgaggcagggatgcccgacactgaaattcaagccaaagcgaagtgttgctgccgcctccgagatgagcacgcaaggccaagagcacaacttctgggcttggcaggactcctctctcaagcccatcgatgttctgcgtgtagagccgcagaagcagccccttgtcatgaagcagccggagaaagtagtgagtgacgttgggcttgtagtttccagggtacagctccttggccaaagtgaaaaagggcttggggttgtgaaagaagaatgggagttcaaaaatggcctcggggtacgggagatcgtactgctggaggttgctgtacaggccactccccggcgatctgaagtctggaatgccactgggtgtgctgatgccggcccccaccatgaccaccaccctctggcaggctctggcccgaatcagctcagctacatcctgcagggaaagcttccccttgtcactgctgcctccacttccaacaacacttgaagcacccacagaaaaagatatggaccttcttccacctttaatactcgaaaagaagaaactgggagctgctgccctcggctgcctccggaatgccctgggcacctcgggtctgggaggcctctgcaaggggcgcgccgggtccaagggctcaccgcgggccccatggctgcctctcagccccgcactcacatcgtccctgccgccaagcaccagccgacagccgcaggcctgaaacggccccacgcctcccccggcctcgacccgttcaactacccggccccacagccggagggctgccgcggcgcgccaaccccagaacgccatgttccgcgcagtcc

SEQ ID NO: 17549 - RNA, 3294 nt, Homo sapiens
  source 1..3294: mol_type = other RNA
tcaggccaggcacagtggctcatgcctgtaatcccagcactttgggaggccgaggtgggtggatcacttgaagccaggagttcgagaccagcctggccaacatagcaaaaccttgtctctattacaaatatgcccatgtgctaggtgtggtgggacacacctgtaatcccagctacccaggagaatcgcttaaacccgggaggcggaagttgcagtgagctgagatcataacaccgcactccaccctgagtgacagggcaagactcaaaaaataaaaaaggaacattaactagggttagaaactaacttcattctttttagaattcaacagttttcctaggtcaccaattccaccttttgttcttattaaggcgcaaagtcacaggacccccttcctgggagtcactgtcattaaatctattgccgtcagctcagcccagggtaggcaaggttcaagaatgggaagtgcttttgtctggggaaacacgcaggtaatgtgatgctaggaaggaggatgtgcaggtgggtgagagcccaggagggagcagctggtgcctgacagggtgagccatcagggctgggcctgggtacagccccaggagaaggagcctgtgcagaagtagcagttcagtggattccacctcctatgtcacaatccagcaggtggccaggactcagcctgggttttaagtgagtaatgccttccctgtctcagagattagctctaacagtgtcactagaggaagccctggcgagggtgggggggcgtagtgtggggacaaggaggccagatagaaagtgctggaatgttctggaacagatctgtttctggaggagaggctgagtatggagagtcaacagaatgtgaccaccttcagagggaggagctgggccgtctccaataaatccagggacaaatgccttcagtcctcagactgttccaatagaggggacgccacgtatcccagggttccctttccaactcatgtcaacacctgcagtccctttgaggagactaaatgtatttcatgctggaaagaacagattttctctcattaaaaatagccccactaaaggagaccaacatgctagaagtgcggcaccagggcctcaagactacacttcggaacatgaagagggctggggaccgctcggcccaagtctggatcttgtaaccaacagatgccgagcttgccgttcaactaggcacagaaagcagactcggtctgggattccagttggtctgattcagttcaagagggtcacagtcagaagaaagctttttccattaggagcttcagcagagtgaagagttcaacacagcaaacaggcaggcagctcctttgtatatgtgacggggtggccctgactgtaaacacagccctaccagtcactgcagctcatggcctgagaagacattccagtggcagcctcgggtgtccactcagttcacatattctggtttcacctgcccaagctgtcttcaggcatgaggtcttgtcagaattgggatgtggatgtctcctatgttaccatttattgtgtgggggcagccatcatcctatttgtctggtccatcaagcttcccagtttcccgctgcacaaggtcccgcatctcttctgtccagcccagaagctccactaggctttccacgccgtgaaccacgtcccccagctgggccacgtccctgctgcgaggatgccaagccaagggccccaccaagtcccggttgatgagcagtcggggaactgagctccgcacggcctcggtcaagctggcaaaaggctccacctccagggaggtcccaaggatgagcagcagatctgccatggggaaatcaaccacatgcagcaagaacctctggggcagcggctccccaaagaacacaatgtcgggcttcacaacgccggtgcagaccgggcagcggggaaccctgtctgccatcacgtcagcccagaatgcagcacaagaagcagcaattacaggacagaagagtgatcaggaacagcaggagagagaaggtctaatgtatgttcaatcagaggtccctaaagagaggggccagatagtgggctaggggcaactcatatccgaagagataacggcagagtatgatccagcaaccatgaaagacgccaacccgcagattcaggatctcaagcaagtgagggctactgagccagcctgagggtgcccacaggaaaaacatgagtcacggcacatctgtgcttgtttctgtcccaagaggttctcaggaggtttagtaattacatgtggtccttcaaagagggagggtggctgtgaggtgagtggttacgtacttgtgagacttcagtaagtgcccagtaaatgtacattttacccgaatgtcctcccctgggaagggtctttggcagactgtgcaggtggcagaggcaaaggttccatgagcttcaaccagctttgaggcagggatgcccgacactgaaattcaagccaaagcgaagtgttgctgccgcctccgagatgagcacgcaaggccaagagcacaacttctgggcttggcaggactcctctctcaagcccatcgatgttctgcgtgtagagccgcagaagcagccccttgtcatgaagcagccggagaaagtagtgagtgacgttgggcttgtagtttccagggtacagctccttggccaaagtgaaaaagggcttggggttgtgaaagaagaatgggagttcaaaaatggcctcggggtacgggagatcgtactgctggaggttgctgtacaggccactccccggcgatctgaagtctggaatgccactgggtgtgctgatgccggcccccaccatgaccaccaccctctggcaggctctggcccgaatcagctcagctacatcctgcagggaaagcttccccttgtcactgctgcctccacttccaacaacacttgaagcacccacagaaaaagatatggaccttcttccacctttaatactttttcaacccggatggcggtgatagttaatactttctgagcgcttttactatggtcaggcattatatttacacctaatcctcgcaaaacactactgggaagatcctcatttgacaggagcaattccgggtcacaaaggctgacaccacaaagctagtccgtagcgggttcgaccacaggcgcccacactctttgacgcctcaatggcacagccaagtgcgcgggaagtgggctgcaaacgccggagagttttgtccggagcgcagagacgcgctgtaaccgagcaaccagcggggcccgcccccggcctgctac

SEQ ID NO: 17550 - RNA, 3359 nt, Homo sapiens
  source 1..3359: mol_type = other RNA
tcaggccaggcacagtggctcatgcctgtaatcccagcactttgggaggccgaggtgggtggatcacttgaagccaggagttcgagaccagcctggccaacatagcaaaaccttgtctctattacaaatatgcccatgtgctaggtgtggtgggacacacctgtaatcccagctacccaggagaatcgcttaaacccgggaggcggaagttgcagtgagctgagatcataacaccgcactccaccctgagtgacagggcaagactcaaaaaataaaaaaggaacattaactagggttagaaactaacttcattctttttagaattcaacagttttcctaggtcaccaattccaccttttgttcttattaaggcgcaaagtcacaggacccccttcctgggagtcactgtcattaaatctattgccgtcagctcagcccagggtaggcaaggttcaagaatgggaagtgcttttgtctggggaaacacgcaggtaatgtgatgctaggaaggaggatgtgcaggtgggtgagagcccaggagggagcagctggtgcctgacagggtgagccatcagggctgggcctgggtacagccccaggagaaggagcctgtgcagaagtagcagttcagtggattccacctcctatgtcacaatccagcaggtggccaggactcagcctgggttttaagtgagtaatgccttccctgtctcagagattagctctaacagtgtcactagaggaagccctggcgagggtgggggggcgtagtgtggggacaaggaggccagatagaaagtgctggaatgttctggaacagatctgtttctggaggagaggctgagtatggagagtcaacagaatgtgaccaccttcagagggaggagctgggccgtctccaataaatccagggacaaatgccttcagtcctcagactgttccaatagaggggacgccacgtatcccagggttccctttccaactcatgtcaacacctgcagtccctttgaggagactaaatgtatttcatgctggaaagaacagattttctctcattaaaaatagccccactaaaggagaccaacatgctagaagtgcggcaccagggcctcaagactacacttcggaacatgaagagggctggggaccgctcggcccaagtctggatcttgtaaccaacagatgccgagcttgccgttcaactaggcacagaaagcagactcggtctgggattccagttggtctgattcagttcaagagggtcacagtcagaagaaagctttttccattaggagcttcagcagagtgaagagttcaacacagcaaacaggcaggcagctcctttgtatatgtgacggggtggccctgactgtaaacacagccctaccagtcactgcagctcatggcctgagaagacattccagtggcagcctcgggtgtccactcagttcacatattctggtttcacctgcccaagctgtcttcaggcatgaggtcttgtcagaattgggatgtggatgtctcctatgttaccatttattgtgtgggggcagccatcatcctatttgtctggtccatcaagcttcccagtttcccgctgcacaaggtcccgcatctcttctgtccagcccagaagctccactaggctttccacgccgtgaaccacgtcccccagctgggccacgtccctgctgcgaggatgccaagccaagggccccaccaagtcccggttgatgagcagtcggggaactgagctccgcacggcctcggtcaagctggcaaaaggctccacctccagggaggtcccaaggatgagcagcagatctgccatggggaaatcaaccacatgcagcaagaacctctggggcagcggctccccaaagaacacaatgtcgggcttcacaacgccggtgcagaccgggcagcggggaaccctgtctgccatcacgtcagcccagaatgcagcacaagaagcagcaattacaggacagaagagtgatcaggaacagcaggagagagaaggtctaatgtatgttcaatcagaggtccctaaagagaggggccagatagtgggctaggggcaactcatatccgaagagataacggcagagtatgatccagcaaccatgaaagacgccaacccgcagattcaggatctcaagcaagtgagggctactgagccagcctgagggtgcccacaggaaaaacatgagtcacggcacatctgtgcttgtttctgtcccaagaggttctcaggaggtttagtaattacatgtggtccttcaaagagggagggtggctgtgaggtgagtggttacgtacttgtgagacttcagtaagtgcccagtaaatgtacattttacccgaatgtcctcccctgggaagggtctttggcagactgtgcaggtggcagaggcaaaggttccatgagcttcaaccagctttgaggcagggatgcccgacactgaaattcaagccaaagcgaagtgttgctgccgcctccgagatgagcacgcaaggccaagagcacaacttctgggcttggcaggactcctggaaggaggcacagccccttggggttgtgatgtcctcaagcctggttttcatgcccgtatcacctctctcaagcccatcgatgttctgcgtgtagagccgcagaagcagccccttgtcatgaagcagccggagaaagtagtgagtgacgttgggcttgtagtttccagggtacagctccttggccaaagtgaaaaagggcttggggttgtgaaagaagaatgggagttcaaaaatggcctcggggtacgggagatcgtactgctggaggttgctgtacaggccactccccggcgatctgaagtctggaatgccactgggtgtgctgatgccggcccccaccatgaccaccaccctctggcaggctctggcccgaatcagctcagctacatcctgcagggaaagcttccccttgtcactgctgcctccacttccaacaacacttgaagcacccacagaaaaagatatggaccttcttccacctttaatactttttcaacccggatggcggtgatagttaatactttctgagcgcttttactatggtcaggcattatatttacacctaatcctcgcaaaacactactgggaagatcctcatttgacaggagcaattccgggtcacaaaggctgacaccacaaagctagtccgtagcgggttcgaccacaggcgcccacactctttgacgcctcaatggcacagccaagtgcgcgggaagtgggctgcaaacgccggagagttttgtccggagcgcagagacgcgctgtaaccgagcaaccagcggggcccgcccccggcctgctac

SEQ ID NO: 17551 - RNA, 2532 nt, Homo sapiens
  source 1..2532: mol_type = other RNA
tcaggccaggcacagtggctcatgcctgtaatcccagcactttgggaggccgaggtgggtggatcacttgaagccaggagttcgagaccagcctggccaacatagcaaaaccttgtctctattacaaatatgcccatgtgctaggtgtggtgggacacacctgtaatcccagctacccaggagaatcgcttaaacccgggaggcggaagttgcagtgagctgagatcataacaccgcactccaccctgagtgacagggcaagactcaaaaaataaaaaaggaacattaactagggttagaaactaacttcattctttttagaattcaacagttttcctaggtcaccaattccaccttttgttcttattaaggcgcaaagtcacaggacccccttcctgggagtcactgtcattaaatctattgccgtcagctcagcccagggtaggcaaggttcaagaatgggaagtgcttttgtctggggaaacacgcaggtaatgtgatgctaggaaggaggatgtgcaggtgggtgagagcccaggagggagcagctggtgcctgacagggtgagccatcagggctgggcctgggtacagccccaggagaaggagcctgtgcagaagtagcagttcagtggattccacctcctatgtcacaatccagcaggtggccaggactcagcctgggttttaagtgagtaatgccttccctgtctcagagattagctctaacagtgtcactagaggaagccctggcgagggtgggggggcgtagtgtggggacaaggaggccagatagaaagtgctggaatgttctggaacagatctgtttctggaggagaggctgagtatggagagtcaacagaatgtgaccaccttcagagggaggagctgggccgtctccaataaatccagggacaaatgccttcagtcctcagactgttccaatagaggggacgccacgtatcccagggttccctttccaactcatgtcaacacctgcagtccctttgaggagactaaatgtatttcatgctggaaagaacagattttctctcattaaaaatagccccactaaaggagaccaacatgctagaagtgcggcaccagggcctcaagactacacttcggaacatgaagagggctggggaccgctcggcccaagtctggatcttgtaaccaacagatgccgagcttgccgttcaactaggcacagaaagcagactcggtctgggattccagttggtctgattcagttcaagagggtcacagtcagaagaaagctttttccattaggagcttcagcagagtgaagagttcaacacagcaaacaggcaggcagctcctttgtatatgtgacggggtggccctgactgtaaacacagccctaccagtcactgcagctcatggcctgagaagacattccagtggcagcctcgggtgtccactcagttcacatattctggtttcacctgcccaagctgtcttcaggcatgaggtcttgtcagaattgggatgtggatgtctcctatgttaccatttattgtgtgggggcagccatcatcctatttgtctggtccatcaagcttcccagtttcccgctgcacaaggtcccgcatctcttctgtccagcccagaagctccactaggctttccacgccgtgaaccacgtcccccagctgggccacgtccctgctgcgaggatgccaagccaagggccccaccaagtcccggttgatgagcagtcggggaactgagctccgcacggcctcggtcaagctggcaaaaggctccacctccagggaggtcccaaggatgagcagcagatctgccatggggaaatcaaccacatgcagcaagaacctctggggcagcggctccccaaagaacacaatgtcgggcttcacaacgccggtgcagaccgggcagcggggaaccctgtctgccatcacgtcagcccgaatgtcctcccctgggaagggtctttggcagactgtgcaggtggcagaggcaaaggttccatgagcttcaaccagctttgaggcagggatgcccgacactctctcaagcccatcgatgttctgcgtgtagagccgcagaagcagccccttgtcatgaagcagccggagaaagtagtgagtgacgttgggcttgtagtttccagggtacagctccttggccaaagtgaaaaagggcttggggttgtgaaagaagaatgggagttcaaaaatggcctcggggtacgggagatcgtactgctggaggttgctgtacaggccactccccggcgatctgaagtctggaatgccactgggtgtgctgatgccggcccccaccatgaccaccaccctctggcaggctctggcccgaatcagctcagctacatcatcgtccctgccgccaagcaccagccgacagccgcaggcctgaaacggccccacgcctcccccggcctcgacccgttcaactacccggccccacagccggagggctgccgcggcgcgccaaccccagaacgccatgttccgcgcagtcc

SEQ ID NO: 17552 - RNA, 2723 nt, Homo sapiens
  source 1..2723: mol_type = other RNA
tcaggccaggcacagtggctcatgcctgtaatcccagcactttgggaggccgaggtgggtggatcacttgaagccaggagttcgagaccagcctggccaacatagcaaaaccttgtctctattacaaatatgcccatgtgctaggtgtggtgggacacacctgtaatcccagctacccaggagaatcgcttaaacccgggaggcggaagttgcagtgagctgagatcataacaccgcactccaccctgagtgacagggcaagactcaaaaaataaaaaaggaacattaactagggttagaaactaacttcattctttttagaattcaacagttttcctaggtcaccaattccaccttttgttcttattaaggcgcaaagtcacaggacccccttcctgggagtcactgtcattaaatctattgccgtcagctcagcccagggtaggcaaggttcaagaatgggaagtgcttttgtctggggaaacacgcaggtaatgtgatgctaggaaggaggatgtgcaggtgggtgagagcccaggagggagcagctggtgcctgacagggtgagccatcagggctgggcctgggtacagccccaggagaaggagcctgtgcagaagtagcagttcagtggattccacctcctatgtcacaatccagcaggtggccaggactcagcctgggttttaagtgagtaatgccttccctgtctcagagattagctctaacagtgtcactagaggaagccctggcgagggtgggggggcgtagtgtggggacaaggaggccagatagaaagtgctggaatgttctggaacagatctgtttctggaggagaggctgagtatggagagtcaacagaatgtgaccaccttcagagggaggagctgggccgtctccaataaatccagggacaaatgccttcagtcctcagactgttccaatagaggggacgccacgtatcccagggttccctttccaactcatgtcaacacctgcagtccctttgaggagactaaatgtatttcatgctggaaagaacagattttctctcattaaaaatagccccactaaaggagaccaacatgctagaagtgcggcaccagggcctcaagactacacttcggaacatgaagagggctggggaccgctcggcccaagtctggatcttgtaaccaacagatgccgagcttgccgttcaactaggcacagaaagcagactcggtctgggattccagttggtctgattcagttcaagagggtcacagtcagaagaaagctttttccattaggagcttcagcagagtgaagagttcaacacagcaaacaggcaggcagctcctttgtatatgtgacggggtggccctgactgtaaacacagccctaccagtcactgcagctcatggcctgagaagacattccagtggcagcctcgggtgtccactcagttcacatattctggtttcacctgcccaagctgtcttcaggcatgaggtcttgtcagaattgggatgtggatgtctcctatgttaccatttattgtgtgggggcagccatcatcctatttgtctggtccatcaagcttcccagtttcccgctgcacaaggtcccgcatctcttctgtccagcccagaagctccactaggctttccacgccgtgaaccacgtcccccagctgggccacgtccctgctgcgaggatgccaagccaagggccccaccaagtcccggttgatgagcagtcggggaactgagctccgcacggcctcggtcaagctggcaaaaggctccacctccagggaggtcccaaggatgagcagcagatctgccatggggaaatcaaccacatgcagcaagaacctctggggcagcggctccccaaagaacacaatgtcgggcttcacaacgccggtgcagaccgggcagcggggaaccctgtctgccatcacgtcagcccgaatgtcctcccctgggaagggtctttggcagactgtgcaggtggcagaggcaaaggttccatgagcttcaaccagctttgaggcagggatgcccgacactctctcaagcccatcgatgttctgcgtgtagagccgcagaagcagccccttgtcatgaagcagccggagaaagtagtgagtgacgttgggcttgtagtttccagggtacagctccttggccaaagtgaaaaagggcttggggttgtgaaagaagaatgggagttcaaaaatggcctcggggtacgggagatcgtactgctggaggttgctgtacaggccactccccggcgatctgaagtctggaatgccactgggtgtgctgatgccggcccccaccatgaccaccaccctctggcaggctctggcccgaatcagctcagctacatcctgcagggaaagcttccccttgtcactgctgcctccacttccaacaacacttgaagcacccacagaaaaagatatggaccttcttccacctttaataacctaatcctcgcaaaacactactgggaagatcctcatttgacaggagcaattccgggtcacaaaggctgacaccacaaagctagtccgtagcgggttcgaccacaggcgcccacactctttgacgcctcaatggcacagccaagtgcgcgggaagtgggctgcaaacgccggagagttttgtccggagcgcagagacgcgctgtaaccgagcaaccagcggggcccgcccccggcctgctac

SEQ ID NO: 17553 - RNA, 2629 nt, Homo sapiens
  source 1..2629: mol_type = other RNA
tcaggccaggcacagtggctcatgcctgtaatcccagcactttgggaggccgaggtgggtggatcacttgaagccaggagttcgagaccagcctggccaacatagcaaaaccttgtctctattacaaatatgcccatgtgctaggtgtggtgggacacacctgtaatcccagctacccaggagaatcgcttaaacccgggaggcggaagttgcagtgagctgagatcataacaccgcactccaccctgagtgacagggcaagactcaaaaaataaaaaaggaacattaactagggttagaaactaacttcattctttttagaattcaacagttttcctaggtcaccaattccaccttttgttcttattaaggcgcaaagtcacaggacccccttcctgggagtcactgtcattaaatctattgccgtcagctcagcccagggtaggcaaggttcaagaatgggaagtgcttttgtctggggaaacacgcaggtaatgtgatgctaggaaggaggatgtgcaggtgggtgagagcccaggagggagcagctggtgcctgacagggtgagccatcagggctgggcctgggtacagccccaggagaaggagcctgtgcagaagtagcagttcagtggattccacctcctatgtcacaatccagcaggtggccaggactcagcctgggttttaagtgagtaatgccttccctgtctcagagattagctctaacagtgtcactagaggaagccctggcgagggtgggggggcgtagtgtggggacaaggaggccagatagaaagtgctggaatgttctggaacagatctgtttctggaggagaggctgagtatggagagtcaacagaatgtgaccaccttcagagggaggagctgggccgtctccaataaatccagggacaaatgccttcagtcctcagactgttccaatagaggggacgccacgtatcccagggttccctttccaactcatgtcaacacctgcagtccctttgaggagactaaatgtatttcatgctggaaagaacagattttctctcattaaaaatagccccactaaaggagaccaacatgctagaagtgcggcaccagggcctcaagactacacttcggaacatgaagagggctggggaccgctcggcccaagtctggatcttgtaaccaacagatgccgagcttgccgttcaactaggcacagaaagcagactcggtctgggattccagttggtctgattcagttcaagagggtcacagtcagaagaaagctttttccattaggagcttcagcagagtgaagagttcaacacagcaaacaggcaggcagctcctttgtatatgtgacggggtggccctgactgtaaacacagccctaccagtcactgcagctcatggcctgagaagacattccagtggcagcctcgggtgtccactcagttcacatattctggtttcacctgcccaagctgtcttcaggcatgaggtcttgtcagaattgggatgtggatgtctcctatgttaccatttattgtgtgggggcagccatcatcctatttgtctggtccatcaagcttcccagtttcccgctgcacaaggtcccgcatctcttctgtccagcccagaagctccactaggctttccacgccgtgaaccacgtcccccagctgggccacgtccctgctgcgaggatgccaagccaagggccccaccaagtcccggttgatgagcagtcggggaactgagctccgcacggcctcggtcaagctggcaaaaggctccacctccagggaggtcccaaggatgagcagcagatctgccatggggaaatcaaccacatgcagcaagaacctctggggcagcggctccccaaagaacacaatgtcgggcttcacaacgccggtgcagaccgggcagcggggaaccctgtctgccatcacgtcagcccgaatgtcctcccctgggaagggtctttggcagactgtgcaggtggcagaggcaaaggttccatgagcttcaaccagctttgaggcagggatgcccgacactctctcaagcccatcgatgttctgcgtgtagagccgcagaagcagccccttgtcatgaagcagccggagaaagtagtgagtgacgttgggcttgtagtttccagggtacagctccttggccaaagtgaaaaagggcttggggttgtgaaagaagaatgggagttcaaaaatggcctcggggtacgggagatcgtactgctggaggttgctgtacaggccactccccggcgatctgaagtctggaatgccactgggtgtgctgatgccggcccccaccatgaccaccaccctctggcaggctctggcccgaatcagctcagctacatcctgcagggaaagcttccccttgtcactgctgcctccacttccaacaacacttgaagcacccacagaaaaagatatggaccttcttccacctttaataatcgtccctgccgccaagcaccagccgacagccgcaggcctgaaacggccccacgcctcccccggcctcgacccgttcaactacccggccccacagccggagggctgccgcggcgcgccaaccccagaacgccatgttccgcgcagtcc

SEQ ID NO: 17554 - RNA, 2721 nt, Homo sapiens
  source 1..2721: mol_type = other RNA
tcaggccaggcacagtggctcatgcctgtaatcccagcactttgggaggccgaggtgggtggatcacttgaagccaggagttcgagaccagcctggccaacatagcaaaaccttgtctctattacaaatatgcccatgtgctaggtgtggtgggacacacctgtaatcccagctacccaggagaatcgcttaaacccgggaggcggaagttgcagtgagctgagatcataacaccgcactccaccctgagtgacagggcaagactcaaaaaataaaaaaggaacattaactagggttagaaactaacttcattctttttagaattcaacagttttcctaggtcaccaattccaccttttgttcttattaaggcgcaaagtcacaggacccccttcctgggagtcactgtcattaaatctattgccgtcagctcagcccagggtaggcaaggttcaagaatgggaagtgcttttgtctggggaaacacgcaggtaatgtgatgctaggaaggaggatgtgcaggtgggtgagagcccaggagggagcagctggtgcctgacagggtgagccatcagggctgggcctgggtacagccccaggagaaggagcctgtgcagaagtagcagttcagtggattccacctcctatgtcacaatccagcaggtggccaggactcagcctgggttttaagtgagtaatgccttccctgtctcagagattagctctaacagtgtcactagaggaagccctggcgagggtgggggggcgtagtgtggggacaaggaggccagatagaaagtgctggaatgttctggaacagatctgtttctggaggagaggctgagtatggagagtcaacagaatgtgaccaccttcagagggaggagctgggccgtctccaataaatccagggacaaatgccttcagtcctcagactgttccaatagaggggacgccacgtatcccagggttccctttccaactcatgtcaacacctgcagtccctttgaggagactaaatgtatttcatgctggaaagaacagattttctctcattaaaaatagccccactaaaggagaccaacatgctagaagtgcggcaccagggcctcaagactacacttcggaacatgaagagggctggggaccgctcggcccaagtctggatcttgtaaccaacagatgccgagcttgccgttcaactaggcacagaaagcagactcggtctgggattccagttggtctgattcagttcaagagggtcacagtcagaagaaagctttttccattaggagcttcagcagagtgaagagttcaacacagcaaacaggcaggcagctcctttgtatatgtgacggggtggccctgactgtaaacacagccctaccagtcactgcagctcatggcctgagaagacattccagtggcagcctcgggtgtccactcagttcacatattctggtttcacctgcccaagctgtcttcaggcatgaggtcttgtcagaattgggatgtggatgtctcctatgttaccatttattgtgtgggggcagccatcatcctatttgtctggtccatcaagcttcccagtttcccgctgcacaaggtcccgcatctcttctgtccagcccagaagctccactaggctttccacgccgtgaaccacgtcccccagctgggccacgtccctgctgcgaggatgccaagccaagggccccaccaagtcccggttgatgagcagtcggggaactgagctccgcacggcctcggtcaagctggcaaaaggctccacctccagggaggtcccaaggatgagcagcagatctgccatggggaaatcaaccacatgcagcaagaacctctggggcagcggctccccaaagaacacaatgtcgggcttcacaacgccggtgcagaccgggcagcggggaaccctgtctgccatcacgtcagcccgaatgtcctcccctgggaagggtctttggcagactgtgcaggtggcagaggcaaaggttccatgagcttcaaccagctttgaggcagggatgcccgacactctctcaagcccatcgatgttctgcgtgtagagccgcagaagcagccccttgtcatgaagcagccggagaaagtagtgagtgacgttgggcttgtagtttccagggtacagctccttggccaaagtgaaaaagggcttggggttgtgaaagaagaatgggagttcaaaaatggcctcggggtacgggagatcgtactgctggaggttgctgtacaggccactccccggcgatctgaagtctggaatgccactgggtgtgctgatgccggcccccaccatgaccaccaccctctggcaggctctggcccgaatcagctcagctacatcctgcagggaaagcttccccttgtcactgctgcctccacttccaacaacacttgaagcacccacagaaaaagatatggaccttcttccacctttaatactaatcctcgcaaaacactactgggaagatcctcatttgacaggagcaattccgggtcacaaaggctgacaccacaaagctagtccgtagcgggttcgaccacaggcgcccacactctttgacgcctcaatggcacagccaagtgcgcgggaagtgggctgcaaacgccggagagttttgtccggagcgcagagacgcgctgtaaccgagcaaccagcggggcccgcccccggcctgctac

SEQ ID NO: 17555 - RNA, 2775 nt, Homo sapiens
  source 1..2775: mol_type = other RNA
tcaggccaggcacagtggctcatgcctgtaatcccagcactttgggaggccgaggtgggtggatcacttgaagccaggagttcgagaccagcctggccaacatagcaaaaccttgtctctattacaaatatgcccatgtgctaggtgtggtgggacacacctgtaatcccagctacccaggagaatcgcttaaacccgggaggcggaagttgcagtgagctgagatcataacaccgcactccaccctgagtgacagggcaagactcaaaaaataaaaaaggaacattaactagggttagaaactaacttcattctttttagaattcaacagttttcctaggtcaccaattccaccttttgttcttattaaggcgcaaagtcacaggacccccttcctgggagtcactgtcattaaatctattgccgtcagctcagcccagggtaggcaaggttcaagaatgggaagtgcttttgtctggggaaacacgcaggtaatgtgatgctaggaaggaggatgtgcaggtgggtgagagcccaggagggagcagctggtgcctgacagggtgagccatcagggctgggcctgggtacagccccaggagaaggagcctgtgcagaagtagcagttcagtggattccacctcctatgtcacaatccagcaggtggccaggactcagcctgggttttaagtgagtaatgccttccctgtctcagagattagctctaacagtgtcactagaggaagccctggcgagggtgggggggcgtagtgtggggacaaggaggccagatagaaagtgctggaatgttctggaacagatctgtttctggaggagaggctgagtatggagagtcaacagaatgtgaccaccttcagagggaggagctgggccgtctccaataaatccagggacaaatgccttcagtcctcagactgttccaatagaggggacgccacgtatcccagggttccctttccaactcatgtcaacacctgcagtccctttgaggagactaaatgtatttcatgctggaaagaacagattttctctcattaaaaatagccccactaaaggagaccaacatgctagaagtgcggcaccagggcctcaagactacacttcggaacatgaagagggctggggaccgctcggcccaagtctggatcttgtaaccaacagatgccgagcttgccgttcaactaggcacagaaagcagactcggtctgggattccagttggtctgattcagttcaagagggtcacagtcagaagaaagctttttccattaggagcttcagcagagtgaagagttcaacacagcaaacaggcaggcagctcctttgtatatgtgacggggtggccctgactgtaaacacagccctaccagtcactgcagctcatggcctgagaagacattccagtggcagcctcgggtgtccactcagttcacatattctggtttcacctgcccaagctgtcttcaggcatgaggtcttgtcagaattgggatgtggatgtctcctatgttaccatttattgtgtgggggcagccatcatcctatttgtctggtccatcaagcttcccagtttcccgctgcacaaggtcccgcatctcttctgtccagcccagaagctccactaggctttccacgccgtgaaccacgtcccccagctgggccacgtccctgctgcgaggatgccaagccaagggccccaccaagtcccggttgatgagcagtcggggaactgagctccgcacggcctcggtcaagctggcaaaaggctccacctccagggaggtcccaaggatgagcagcagatctgccatggggaaatcaaccacatgcagcaagaacctctggggcagcggctccccaaagaacacaatgtcgggcttcacaacgccggtgcagaccgggcagcggggaaccctgtctgccatcacgtcagcccgaatgtcctcccctgggaagggtctttggcagactgtgcaggtggcagaggcaaaggttccatgagcttcaaccagctttgaggcagggatgcccgacactctctcaagcccatcgatgttctgcgtgtagagccgcagaagcagccccttgtcatgaagcagccggagaaagtagtgagtgacgttgggcttgtagtttccagggtacagctccttggccaaagtgaaaaagggcttggggttgtgaaagaagaatgggagttcaaaaatggcctcggggtacgggagatcgtactgctggaggttgctgtacaggccactccccggcgatctgaagtctggaatgccactgggtgtgctgatgccggcccccaccatgaccaccaccctctggcaggctctggcccgaatcagctcagctacatcctgcagggaaagcttccccttgtcactgctgcctccacttccaacaacacttgaagcacccacagaaaaagatatggaccttcttccacctttaatactcgaaaagaagaaactgggagctgctgccctcggctgcctccggaatgccctgggcacctcgggtctgggaggcctctgcaaggggcgcgccgggtccaagggctcaccgcgggccccatggctgcctctcagccccgcactcacatcgtccctgccgccaagcaccagccgacagccgcaggcctgaaacggccccacgcctcccccggcctcgacccgttcaactacccggccccacagccggagggctgccgcggcgcgccaaccccagaacgccatgttccgcgcagtcc

SEQ ID NO: 17556 - RNA, 2796 nt, Homo sapiens
  source 1..2796: mol_type = other RNA
tcaggccaggcacagtggctcatgcctgtaatcccagcactttgggaggccgaggtgggtggatcacttgaagccaggagttcgagaccagcctggccaacatagcaaaaccttgtctctattacaaatatgcccatgtgctaggtgtggtgggacacacctgtaatcccagctacccaggagaatcgcttaaacccgggaggcggaagttgcagtgagctgagatcataacaccgcactccaccctgagtgacagggcaagactcaaaaaataaaaaaggaacattaactagggttagaaactaacttcattctttttagaattcaacagttttcctaggtcaccaattccaccttttgttcttattaaggcgcaaagtcacaggacccccttcctgggagtcactgtcattaaatctattgccgtcagctcagcccagggtaggcaaggttcaagaatgggaagtgcttttgtctggggaaacacgcaggtaatgtgatgctaggaaggaggatgtgcaggtgggtgagagcccaggagggagcagctggtgcctgacagggtgagccatcagggctgggcctgggtacagccccaggagaaggagcctgtgcagaagtagcagttcagtggattccacctcctatgtcacaatccagcaggtggccaggactcagcctgggttttaagtgagtaatgccttccctgtctcagagattagctctaacagtgtcactagaggaagccctggcgagggtgggggggcgtagtgtggggacaaggaggccagatagaaagtgctggaatgttctggaacagatctgtttctggaggagaggctgagtatggagagtcaacagaatgtgaccaccttcagagggaggagctgggccgtctccaataaatccagggacaaatgccttcagtcctcagactgttccaatagaggggacgccacgtatcccagggttccctttccaactcatgtcaacacctgcagtccctttgaggagactaaatgtatttcatgctggaaagaacagattttctctcattaaaaatagccccactaaaggagaccaacatgctagaagtgcggcaccagggcctcaagactacacttcggaacatgaagagggctggggaccgctcggcccaagtctggatcttgtaaccaacagatgccgagcttgccgttcaactaggcacagaaagcagactcggtctgggattccagttggtctgattcagttcaagagggtcacagtcagaagaaagctttttccattaggagcttcagcagagtgaagagttcaacacagcaaacaggcaggcagctcctttgtatatgtgacggggtggccctgactgtaaacacagccctaccagtcactgcagctcatggcctgagaagacattccagtggcagcctcgggtgtccactcagttcacatattctggtttcacctgcccaagctgtcttcaggcatgaggtcttgtcagaattgggatgtggatgtctcctatgttaccatttattgtgtgggggcagccatcatcctatttgtctggtccatcaagcttcccagtttcccgctgcacaaggtcccgcatctcttctgtccagcccagaagctccactaggctttccacgccgtgaaccacgtcccccagctgggccacgtccctgctgcgaggatgccaagccaagggccccaccaagtcccggttgatgagcagtcggggaactgagctccgcacggcctcggtcaagctggcaaaaggctccacctccagggaggtcccaaggatgagcagcagatctgccatggggaaatcaaccacatgcagcaagaacctctggggcagcggctccccaaagaacacaatgtcgggcttcacaacgccggtgcagaccgggcagcggggaaccctgtctgccatcacgtcagcccgaatgtcctcccctgggaagggtctttggcagactgtgcaggtggcagaggcaaaggttccatgagcttcaaccagctttgaggcagggatgcccgacactctctcaagcccatcgatgttctgcgtgtagagccgcagaagcagccccttgtcatgaagcagccggagaaagtagtgagtgacgttgggcttgtagtttccagggtacagctccttggccaaagtgaaaaagggcttggggttgtgaaagaagaatgggagttcaaaaatggcctcggggtacgggagatcgtactgctggaggttgctgtacaggccactccccggcgatctgaagtctggaatgccactgggtgtgctgatgccggcccccaccatgaccaccaccctctggcaggctctggcccgaatcagctcagctacatcctgcagggaaagcttccccttgtcactgctgcctccacttccaacaacacttgaagcacccacagaaaaagatatggaccttcttccacctttaatactttttcaacccggatggcggtgatagttaatactttctgagcgcttttactatggtcaggcattatatttacacctaatcctcgcaaaacactactgggaagatcctcatttgacaggagcaattccgggtcacaaaggctgacaccacaaagctagtccgtagcgggttcgaccacaggcgcccacactctttgacgcctcaatggcacagccaagtgcgcgggaagtgggctgcaaacgccggagagttttgtccggagcgcagagacgcgctgtaaccgagcaaccagcggggcccgcccccggcctgctac

SEQ ID NO: 17557 - RNA, 2718 nt, Homo sapiens
  source 1..2718: mol_type = other RNA
tcaggccaggcacagtggctcatgcctgtaatcccagcactttgggaggccgaggtgggtggatcacttgaagccaggagttcgagaccagcctggccaacatagcaaaaccttgtctctattacaaatatgcccatgtgctaggtgtggtgggacacacctgtaatcccagctacccaggagaatcgcttaaacccgggaggcggaagttgcagtgagctgagatcataacaccgcactccaccctgagtgacagggcaagactcaaaaaataaaaaaggaacattaactagggttagaaactaacttcattctttttagaattcaacagttttcctaggtcaccaattccaccttttgttcttattaaggcgcaaagtcacaggacccccttcctgggagtcactgtcattaaatctattgccgtcagctcagcccagggtaggcaaggttcaagaatgggaagtgcttttgtctggggaaacacgcaggtaatgtgatgctaggaaggaggatgtgcaggtgggtgagagcccaggagggagcagctggtgcctgacagggtgagccatcagggctgggcctgggtacagccccaggagaaggagcctgtgcagaagtagcagttcagtggattccacctcctatgtcacaatccagcaggtggccaggactcagcctgggttttaagtgagtaatgccttccctgtctcagagattagctctaacagtgtcactagaggaagccctggcgagggtgggggggcgtagtgtggggacaaggaggccagatagaaagtgctggaatgttctggaacagatctgtttctggaggagaggctgagtatggagagtcaacagaatgtgaccaccttcagagggaggagctgggccgtctccaataaatccagggacaaatgccttcagtcctcagactgttccaatagaggggacgccacgtatcccagggttccctttccaactcatgtcaacacctgcagtccctttgaggagactaaatgtatttcatgctggaaagaacagattttctctcattaaaaatagccccactaaaggagaccaacatgctagaagtgcggcaccagggcctcaagactacacttcggaacatgaagagggctggggaccgctcggcccaagtctggatcttgtaaccaacagatgccgagcttgccgttcaactaggcacagaaagcagactcggtctgggattccagttggtctgattcagttcaagagggtcacagtcagaagaaagctttttccattaggagcttcagcagagtgaagagttcaacacagcaaacaggcaggcagctcctttgtatatgtgacggggtggccctgactgtaaacacagccctaccagtcactgcagctcatggcctgagaagacattccagtggcagcctcgggtgtccactcagttcacatattctggtttcacctgcccaagctgtcttcaggcatgaggtcttgtcagaattgggatgtggatgtctcctatgttaccatttattgtgtgggggcagccatcatcctatttgtctggtccatcaagcttcccagtttcccgctgcacaaggtcccgcatctcttctgtccagcccagaagctccactaggctttccacgccgtgaaccacgtcccccagctgggccacgtccctgctgcgaggatgccaagccaagggccccaccaagtcccggttgatgagcagtcggggaactgagctccgcacggcctcggtcaagctggcaaaaggctccacctccagggaggtcccaaggatgagcagcagatctgccatggggaaatcaaccacatgcagcaagaacctctggggcagcggctccccaaagaacacaatgtcgggcttcacaacgccggtgcagaccgggcagcggggaaccctgtctgccatcacgtcagcccgaatgtcctcccctgggaagggtctttggcagactgtgcaggtggcagaggcaaaggttccatgagcttcaaccagctttgaggcagggatgcccgacactgaaattcaagccaaagcgaagtgttgctgccgcctccgagatgagcacgcaaggccaagagcacaacttctgggcttggcaggactcctctctcaagcccatcgatgttctgcgtgtagagccgcagaagcagccccttgtcatgaagcagccggagaaagtagtgagtgacgttgggcttgtagtttccagggtacagctccttggccaaagtgaaaaagggcttggggttgtgaaagaagaatgggagttcaaaaatggcctcggggtacgggagatcgtactgctggaggttgctgtacaggccactccccggcgatctgaagtctggaatgccactgggtgtgctgatgccggcccccaccatgaccaccaccctctggcaggctctggcccgaatcagctcagctacatcctgcagggaaagcttccccttgtcactgctgcctccacttccaacaacacttgaagcacccacagaaaaagatatggaccttcttccacctttaataatcgtccctgccgccaagcaccagccgacagccgcaggcctgaaacggccccacgcctcccccggcctcgacccgttcaactacccggccccacagccggagggctgccgcggcgcgccaaccccagaacgccatgttccgcgcagtcc

SEQ ID NO: 17558 - RNA, 2864 nt, Homo sapiens
  source 1..2864: mol_type = other RNA
tcaggccaggcacagtggctcatgcctgtaatcccagcactttgggaggccgaggtgggtggatcacttgaagccaggagttcgagaccagcctggccaacatagcaaaaccttgtctctattacaaatatgcccatgtgctaggtgtggtgggacacacctgtaatcccagctacccaggagaatcgcttaaacccgggaggcggaagttgcagtgagctgagatcataacaccgcactccaccctgagtgacagggcaagactcaaaaaataaaaaaggaacattaactagggttagaaactaacttcattctttttagaattcaacagttttcctaggtcaccaattccaccttttgttcttattaaggcgcaaagtcacaggacccccttcctgggagtcactgtcattaaatctattgccgtcagctcagcccagggtaggcaaggttcaagaatgggaagtgcttttgtctggggaaacacgcaggtaatgtgatgctaggaaggaggatgtgcaggtgggtgagagcccaggagggagcagctggtgcctgacagggtgagccatcagggctgggcctgggtacagccccaggagaaggagcctgtgcagaagtagcagttcagtggattccacctcctatgtcacaatccagcaggtggccaggactcagcctgggttttaagtgagtaatgccttccctgtctcagagattagctctaacagtgtcactagaggaagccctggcgagggtgggggggcgtagtgtggggacaaggaggccagatagaaagtgctggaatgttctggaacagatctgtttctggaggagaggctgagtatggagagtcaacagaatgtgaccaccttcagagggaggagctgggccgtctccaataaatccagggacaaatgccttcagtcctcagactgttccaatagaggggacgccacgtatcccagggttccctttccaactcatgtcaacacctgcagtccctttgaggagactaaatgtatttcatgctggaaagaacagattttctctcattaaaaatagccccactaaaggagaccaacatgctagaagtgcggcaccagggcctcaagactacacttcggaacatgaagagggctggggaccgctcggcccaagtctggatcttgtaaccaacagatgccgagcttgccgttcaactaggcacagaaagcagactcggtctgggattccagttggtctgattcagttcaagagggtcacagtcagaagaaagctttttccattaggagcttcagcagagtgaagagttcaacacagcaaacaggcaggcagctcctttgtatatgtgacggggtggccctgactgtaaacacagccctaccagtcactgcagctcatggcctgagaagacattccagtggcagcctcgggtgtccactcagttcacatattctggtttcacctgcccaagctgtcttcaggcatgaggtcttgtcagaattgggatgtggatgtctcctatgttaccatttattgtgtgggggcagccatcatcctatttgtctggtccatcaagcttcccagtttcccgctgcacaaggtcccgcatctcttctgtccagcccagaagctccactaggctttccacgccgtgaaccacgtcccccagctgggccacgtccctgctgcgaggatgccaagccaagggccccaccaagtcccggttgatgagcagtcggggaactgagctccgcacggcctcggtcaagctggcaaaaggctccacctccagggaggtcccaaggatgagcagcagatctgccatggggaaatcaaccacatgcagcaagaacctctggggcagcggctccccaaagaacacaatgtcgggcttcacaacgccggtgcagaccgggcagcggggaaccctgtctgccatcacgtcagcccgaatgtcctcccctgggaagggtctttggcagactgtgcaggtggcagaggcaaaggttccatgagcttcaaccagctttgaggcagggatgcccgacactgaaattcaagccaaagcgaagtgttgctgccgcctccgagatgagcacgcaaggccaagagcacaacttctgggcttggcaggactcctctctcaagcccatcgatgttctgcgtgtagagccgcagaagcagccccttgtcatgaagcagccggagaaagtagtgagtgacgttgggcttgtagtttccagggtacagctccttggccaaagtgaaaaagggcttggggttgtgaaagaagaatgggagttcaaaaatggcctcggggtacgggagatcgtactgctggaggttgctgtacaggccactccccggcgatctgaagtctggaatgccactgggtgtgctgatgccggcccccaccatgaccaccaccctctggcaggctctggcccgaatcagctcagctacatcctgcagggaaagcttccccttgtcactgctgcctccacttccaacaacacttgaagcacccacagaaaaagatatggaccttcttccacctttaatactcgaaaagaagaaactgggagctgctgccctcggctgcctccggaatgccctgggcacctcgggtctgggaggcctctgcaaggggcgcgccgggtccaagggctcaccgcgggccccatggctgcctctcagccccgcactcacatcgtccctgccgccaagcaccagccgacagccgcaggcctgaaacggccccacgcctcccccggcctcgacccgttcaactacccggccccacagccggagggctgccgcggcgcgccaaccccagaacgccatgttccgcgcagtcc

SEQ ID NO: 17559 - RNA, 2885 nt, Homo sapiens
  source 1..2885: mol_type = other RNA
tcaggccaggcacagtggctcatgcctgtaatcccagcactttgggaggccgaggtgggtggatcacttgaagccaggagttcgagaccagcctggccaacatagcaaaaccttgtctctattacaaatatgcccatgtgctaggtgtggtgggacacacctgtaatcccagctacccaggagaatcgcttaaacccgggaggcggaagttgcagtgagctgagatcataacaccgcactccaccctgagtgacagggcaagactcaaaaaataaaaaaggaacattaactagggttagaaactaacttcattctttttagaattcaacagttttcctaggtcaccaattccaccttttgttcttattaaggcgcaaagtcacaggacccccttcctgggagtcactgtcattaaatctattgccgtcagctcagcccagggtaggcaaggttcaagaatgggaagtgcttttgtctggggaaacacgcaggtaatgtgatgctaggaaggaggatgtgcaggtgggtgagagcccaggagggagcagctggtgcctgacagggtgagccatcagggctgggcctgggtacagccccaggagaaggagcctgtgcagaagtagcagttcagtggattccacctcctatgtcacaatccagcaggtggccaggactcagcctgggttttaagtgagtaatgccttccctgtctcagagattagctctaacagtgtcactagaggaagccctggcgagggtgggggggcgtagtgtggggacaaggaggccagatagaaagtgctggaatgttctggaacagatctgtttctggaggagaggctgagtatggagagtcaacagaatgtgaccaccttcagagggaggagctgggccgtctccaataaatccagggacaaatgccttcagtcctcagactgttccaatagaggggacgccacgtatcccagggttccctttccaactcatgtcaacacctgcagtccctttgaggagactaaatgtatttcatgctggaaagaacagattttctctcattaaaaatagccccactaaaggagaccaacatgctagaagtgcggcaccagggcctcaagactacacttcggaacatgaagagggctggggaccgctcggcccaagtctggatcttgtaaccaacagatgccgagcttgccgttcaactaggcacagaaagcagactcggtctgggattccagttggtctgattcagttcaagagggtcacagtcagaagaaagctttttccattaggagcttcagcagagtgaagagttcaacacagcaaacaggcaggcagctcctttgtatatgtgacggggtggccctgactgtaaacacagccctaccagtcactgcagctcatggcctgagaagacattccagtggcagcctcgggtgtccactcagttcacatattctggtttcacctgcccaagctgtcttcaggcatgaggtcttgtcagaattgggatgtggatgtctcctatgttaccatttattgtgtgggggcagccatcatcctatttgtctggtccatcaagcttcccagtttcccgctgcacaaggtcccgcatctcttctgtccagcccagaagctccactaggctttccacgccgtgaaccacgtcccccagctgggccacgtccctgctgcgaggatgccaagccaagggccccaccaagtcccggttgatgagcagtcggggaactgagctccgcacggcctcggtcaagctggcaaaaggctccacctccagggaggtcccaaggatgagcagcagatctgccatggggaaatcaaccacatgcagcaagaacctctggggcagcggctccccaaagaacacaatgtcgggcttcacaacgccggtgcagaccgggcagcggggaaccctgtctgccatcacgtcagcccgaatgtcctcccctgggaagggtctttggcagactgtgcaggtggcagaggcaaaggttccatgagcttcaaccagctttgaggcagggatgcccgacactgaaattcaagccaaagcgaagtgttgctgccgcctccgagatgagcacgcaaggccaagagcacaacttctgggcttggcaggactcctctctcaagcccatcgatgttctgcgtgtagagccgcagaagcagccccttgtcatgaagcagccggagaaagtagtgagtgacgttgggcttgtagtttccagggtacagctccttggccaaagtgaaaaagggcttggggttgtgaaagaagaatgggagttcaaaaatggcctcggggtacgggagatcgtactgctggaggttgctgtacaggccactccccggcgatctgaagtctggaatgccactgggtgtgctgatgccggcccccaccatgaccaccaccctctggcaggctctggcccgaatcagctcagctacatcctgcagggaaagcttccccttgtcactgctgcctccacttccaacaacacttgaagcacccacagaaaaagatatggaccttcttccacctttaatactttttcaacccggatggcggtgatagttaatactttctgagcgcttttactatggtcaggcattatatttacacctaatcctcgcaaaacactactgggaagatcctcatttgacaggagcaattccgggtcacaaaggctgacaccacaaagctagtccgtagcgggttcgaccacaggcgcccacactctttgacgcctcaatggcacagccaagtgcgcgggaagtgggctgcaaacgccggagagttttgtccggagcgcagagacgcgctgtaaccgagcaaccagcggggcccgcccccggcctgctac

SEQ ID NO: 17560 - RNA, 2783 nt, Homo sapiens
  source 1..2783: mol_type = other RNA
tcaggccaggcacagtggctcatgcctgtaatcccagcactttgggaggccgaggtgggtggatcacttgaagccaggagttcgagaccagcctggccaacatagcaaaaccttgtctctattacaaatatgcccatgtgctaggtgtggtgggacacacctgtaatcccagctacccaggagaatcgcttaaacccgggaggcggaagttgcagtgagctgagatcataacaccgcactccaccctgagtgacagggcaagactcaaaaaataaaaaaggaacattaactagggttagaaactaacttcattctttttagaattcaacagttttcctaggtcaccaattccaccttttgttcttattaaggcgcaaagtcacaggacccccttcctgggagtcactgtcattaaatctattgccgtcagctcagcccagggtaggcaaggttcaagaatgggaagtgcttttgtctggggaaacacgcaggtaatgtgatgctaggaaggaggatgtgcaggtgggtgagagcccaggagggagcagctggtgcctgacagggtgagccatcagggctgggcctgggtacagccccaggagaaggagcctgtgcagaagtagcagttcagtggattccacctcctatgtcacaatccagcaggtggccaggactcagcctgggttttaagtgagtaatgccttccctgtctcagagattagctctaacagtgtcactagaggaagccctggcgagggtgggggggcgtagtgtggggacaaggaggccagatagaaagtgctggaatgttctggaacagatctgtttctggaggagaggctgagtatggagagtcaacagaatgtgaccaccttcagagggaggagctgggccgtctccaataaatccagggacaaatgccttcagtcctcagactgttccaatagaggggacgccacgtatcccagggttccctttccaactcatgtcaacacctgcagtccctttgaggagactaaatgtatttcatgctggaaagaacagattttctctcattaaaaatagccccactaaaggagaccaacatgctagaagtgcggcaccagggcctcaagactacacttcggaacatgaagagggctggggaccgctcggcccaagtctggatcttgtaaccaacagatgccgagcttgccgttcaactaggcacagaaagcagactcggtctgggattccagttggtctgattcagttcaagagggtcacagtcagaagaaagctttttccattaggagcttcagcagagtgaagagttcaacacagcaaacaggcaggcagctcctttgtatatgtgacggggtggccctgactgtaaacacagccctaccagtcactgcagctcatggcctgagaagacattccagtggcagcctcgggtgtccactcagttcacatattctggtttcacctgcccaagctgtcttcaggcatgaggtcttgtcagaattgggatgtggatgtctcctatgttaccatttattgtgtgggggcagccatcatcctatttgtctggtccatcaagcttcccagtttcccgctgcacaaggtcccgcatctcttctgtccagcccagaagctccactaggctttccacgccgtgaaccacgtcccccagctgggccacgtccctgctgcgaggatgccaagccaagggccccaccaagtcccggttgatgagcagtcggggaactgagctccgcacggcctcggtcaagctggcaaaaggctccacctccagggaggtcccaaggatgagcagcagatctgccatggggaaatcaaccacatgcagcaagaacctctggggcagcggctccccaaagaacacaatgtcgggcttcacaacgccggtgcagaccgggcagcggggaaccctgtctgccatcacgtcagcccgaatgtcctcccctgggaagggtctttggcagactgtgcaggtggcagaggcaaaggttccatgagcttcaaccagctttgaggcagggatgcccgacactgaaattcaagccaaagcgaagtgttgctgccgcctccgagatgagcacgcaaggccaagagcacaacttctgggcttggcaggactcctggaaggaggcacagccccttggggttgtgatgtcctcaagcctggttttcatgcccgtatcacctctctcaagcccatcgatgttctgcgtgtagagccgcagaagcagccccttgtcatgaagcagccggagaaagtagtgagtgacgttgggcttgtagtttccagggtacagctccttggccaaagtgaaaaagggcttggggttgtgaaagaagaatgggagttcaaaaatggcctcggggtacgggagatcgtactgctggaggttgctgtacaggccactccccggcgatctgaagtctggaatgccactgggtgtgctgatgccggcccccaccatgaccaccaccctctggcaggctctggcccgaatcagctcagctacatcctgcagggaaagcttccccttgtcactgctgcctccacttccaacaacacttgaagcacccacagaaaaagatatggaccttcttccacctttaataatcgtccctgccgccaagcaccagccgacagccgcaggcctgaaacggccccacgcctcccccggcctcgacccgttcaactacccggccccacagccggagggctgccgcggcgcgccaaccccagaacgccatgttccgcgcagtcc

SEQ ID NO: 17561 - RNA, 2950 nt, Homo sapiens
  source 1..2950: mol_type = other RNA
tcaggccaggcacagtggctcatgcctgtaatcccagcactttgggaggccgaggtgggtggatcacttgaagccaggagttcgagaccagcctggccaacatagcaaaaccttgtctctattacaaatatgcccatgtgctaggtgtggtgggacacacctgtaatcccagctacccaggagaatcgcttaaacccgggaggcggaagttgcagtgagctgagatcataacaccgcactccaccctgagtgacagggcaagactcaaaaaataaaaaaggaacattaactagggttagaaactaacttcattctttttagaattcaacagttttcctaggtcaccaattccaccttttgttcttattaaggcgcaaagtcacaggacccccttcctgggagtcactgtcattaaatctattgccgtcagctcagcccagggtaggcaaggttcaagaatgggaagtgcttttgtctggggaaacacgcaggtaatgtgatgctaggaaggaggatgtgcaggtgggtgagagcccaggagggagcagctggtgcctgacagggtgagccatcagggctgggcctgggtacagccccaggagaaggagcctgtgcagaagtagcagttcagtggattccacctcctatgtcacaatccagcaggtggccaggactcagcctgggttttaagtgagtaatgccttccctgtctcagagattagctctaacagtgtcactagaggaagccctggcgagggtgggggggcgtagtgtggggacaaggaggccagatagaaagtgctggaatgttctggaacagatctgtttctggaggagaggctgagtatggagagtcaacagaatgtgaccaccttcagagggaggagctgggccgtctccaataaatccagggacaaatgccttcagtcctcagactgttccaatagaggggacgccacgtatcccagggttccctttccaactcatgtcaacacctgcagtccctttgaggagactaaatgtatttcatgctggaaagaacagattttctctcattaaaaatagccccactaaaggagaccaacatgctagaagtgcggcaccagggcctcaagactacacttcggaacatgaagagggctggggaccgctcggcccaagtctggatcttgtaaccaacagatgccgagcttgccgttcaactaggcacagaaagcagactcggtctgggattccagttggtctgattcagttcaagagggtcacagtcagaagaaagctttttccattaggagcttcagcagagtgaagagttcaacacagcaaacaggcaggcagctcctttgtatatgtgacggggtggccctgactgtaaacacagccctaccagtcactgcagctcatggcctgagaagacattccagtggcagcctcgggtgtccactcagttcacatattctggtttcacctgcccaagctgtcttcaggcatgaggtcttgtcagaattgggatgtggatgtctcctatgttaccatttattgtgtgggggcagccatcatcctatttgtctggtccatcaagcttcccagtttcccgctgcacaaggtcccgcatctcttctgtccagcccagaagctccactaggctttccacgccgtgaaccacgtcccccagctgggccacgtccctgctgcgaggatgccaagccaagggccccaccaagtcccggttgatgagcagtcggggaactgagctccgcacggcctcggtcaagctggcaaaaggctccacctccagggaggtcccaaggatgagcagcagatctgccatggggaaatcaaccacatgcagcaagaacctctggggcagcggctccccaaagaacacaatgtcgggcttcacaacgccggtgcagaccgggcagcggggaaccctgtctgccatcacgtcagcccgaatgtcctcccctgggaagggtctttggcagactgtgcaggtggcagaggcaaaggttccatgagcttcaaccagctttgaggcagggatgcccgacactgaaattcaagccaaagcgaagtgttgctgccgcctccgagatgagcacgcaaggccaagagcacaacttctgggcttggcaggactcctggaaggaggcacagccccttggggttgtgatgtcctcaagcctggttttcatgcccgtatcacctctctcaagcccatcgatgttctgcgtgtagagccgcagaagcagccccttgtcatgaagcagccggagaaagtagtgagtgacgttgggcttgtagtttccagggtacagctccttggccaaagtgaaaaagggcttggggttgtgaaagaagaatgggagttcaaaaatggcctcggggtacgggagatcgtactgctggaggttgctgtacaggccactccccggcgatctgaagtctggaatgccactgggtgtgctgatgccggcccccaccatgaccaccaccctctggcaggctctggcccgaatcagctcagctacatcctgcagggaaagcttccccttgtcactgctgcctccacttccaacaacacttgaagcacccacagaaaaagatatggaccttcttccacctttaatactttttcaacccggatggcggtgatagttaatactttctgagcgcttttactatggtcaggcattatatttacacctaatcctcgcaaaacactactgggaagatcctcatttgacaggagcaattccgggtcacaaaggctgacaccacaaagctagtccgtagcgggttcgaccacaggcgcccacactctttgacgcctcaatggcacagccaagtgcgcgggaagtgggctgcaaacgccggagagttttgtccggagcgcagagacgcgctgtaaccgagcaaccagcggggcccgcccccggcctgctac

SEQ ID NO: 17562 - RNA, 2270 nt, Homo sapiens
  source 1..2270: mol_type = other RNA
tcaggccaggcacagtggctcatgcctgtaatcccagcactttgggaggccgaggtgggtggatcacttgaagccaggagttcgagaccagcctggccaacatagcaaaaccttgtctctattacaaatatgcccatgtgctaggtgtggtgggacacacctgtaatcccagctacccaggagaatcgcttaaacccgggaggcggaagttgcagtgagctgagatcataacaccgcactccaccctgagtgacagggcaagactcaaaaaataaaaaaggaacattaactagggttagaaactaacttcattctttttagaattcaacagttttcctaggtcaccaattccaccttttgttcttattaaggcgcaaagtcacaggacccccttcctgggagtcactgtcattaaatctattgccgtcagctcagcccagggtaggcaaggttcaagaatgggaagtgcttttgtctggggaaacacgcaggtaatgtgatgctaggaaggaggatgtgcaggtgggtgagagcccaggagggagcagctggtgcctgacagggtgagccatcagggctgggcctgggtacagccccaggagaaggagcctgtgcagaagtagcagttcagtggattccacctcctatgtcacaatccagcaggtggccaggactcagcctgggttttaagtgagtaatgccttccctgtctcagagattagctctaacagtgtcactagaggaagccctggcgagggtgggggggcgtagtgtggggacaaggaggccagatagaaagtgctggaatgttctggaacagatctgtttctggaggagaggctgagtatggagagtcaacagaatgtgaccaccttcagagggaggagctgggccgtctccaataaatccagggacaaatgccttcagtcctcagactgttccaatagaggggacgccacgtatcccagggttccctttccaactcatgtcaacacctgcagtccctttgaggagactaaatgtatttcatgctggaaagaacagattttctctcattaaaaatagccccactaaaggagaccaacatgctagaagtgcggcaccagggcctcaagactacacttcggaacatgaagagggctggggaccgctcggcccaagtctggatcttgtaaccaacagatgccgagcttgccgttcaactaggcacagaaagcagactcggtctgggattccagttggtctgattcagttcaagagggtcacagtcagaagaaagctttttccattaggagcttcagcagagtgaagagttcaacacagcaaacaggcaggcagctcctttgtatatgtgacggggtggccctgactgtaaacacagccctaccagtcactgcagctcatggcctgagaagacattccagtggcagcctcgggtgtccactcagttcacatattctggtttcacctgcccaagctgtcttcaggcatgaggtcttgtcagaattgggatgtggatgtctcctatgttaccatttattgtgtgggggcagccatcatcctatttgtctggtccatcaagcttcccagtttcccgctgcacaaggtcccgcatctcttctgtccagcccagaagctccactaggctttccacgccgtgaaccacgtcccccagctgggccacgtccctgctgcgaggatgccaagccaagggccccaccaagtcccggttgatgagcagtcggggaactgagctccgcacggcctcggtcaagctggcaaaaggctccacctccagggaggtcccaaggatgagcagcagatctgccatggggaaatcaaccacatgcagcaagaacctctggggcagcggctccccaaagaacacaatgtcgggcttcacaacgccggtgcagaccgggcagcggggaaccctgtctgccatcacgtcagcctttttcaacccggatggcggtgatagttaatactttctgagcgcttttactatggtcaggcattatatttacacctaatcctcgcaaaacactactgggaagatcctcatttgacaggagcaattccgggtcacaaaggctgacaccacaaagctagtccgtagcgggttcgaccacaggcgcccacactctttgacgcctcaatggcacagccaagtgcgcgggaagtgggctgcaaacgccggagagttttgtccggagcgcagagacgcgctgtaaccgagcaaccagcggggcccgcccccggcctgctac

SEQ ID NO: 17563 - RNA, 2670 nt, Homo sapiens
  source 1..2670: mol_type = other RNA
tcaggccaggcacagtggctcatgcctgtaatcccagcactttgggaggccgaggtgggtggatcacttgaagccaggagttcgagaccagcctggccaacatagcaaaaccttgtctctattacaaatatgcccatgtgctaggtgtggtgggacacacctgtaatcccagctacccaggagaatcgcttaaacccgggaggcggaagttgcagtgagctgagatcataacaccgcactccaccctgagtgacagggcaagactcaaaaaataaaaaaggaacattaactagggttagaaactaacttcattctttttagaattcaacagttttcctaggtcaccaattccaccttttgttcttattaaggcgcaaagtcacaggacccccttcctgggagtcactgtcattaaatctattgccgtcagctcagcccagggtaggcaaggttcaagaatgggaagtgcttttgtctggggaaacacgcaggtaatgtgatgctaggaaggaggatgtgcaggtgggtgagagcccaggagggagcagctggtgcctgacagggtgagccatcagggctgggcctgggtacagccccaggagaaggagcctgtgcagaagtagcagttcagtggattccacctcctatgtcacaatccagcaggtggccaggactcagcctgggttttaagtgagtaatgccttccctgtctcagagattagctctaacagtgtcactagaggaagccctggcgagggtgggggggcgtagtgtggggacaaggaggccagatagaaagtgctggaatgttctggaacagatctgtttctggaggagaggctgagtatggagagtcaacagaatgtgaccaccttcagagggaggagctgggccgtctccaataaatccagggacaaatgccttcagtcctcagactgttccaatagaggggacgccacgtatcccagggttccctttccaactcatgtcaacacctgcagtccctttgaggagactaaatgtatttcatgctggaaagaacagattttctctcattaaaaatagccccactaaaggagaccaacatgctagaagtgcggcaccagggcctcaagactacacttcggaacatgaagagggctggggaccgctcggcccaagtctggatcttgtaaccaacagatgccgagcttgccgttcaactaggcacagaaagcagactcggtctgggattccagttggtctgattcagttcaagagggtcacagtcagaagaaagctttttccattaggagcttcagcagagtgaagagttcaacacagcaaacaggcaggcagctcctttgtatatgtgacggggtggccctgactgtaaacacagccctaccagtcactgcagctcatggcctgagaagacattccagtggcagcctcgggtgtccactcagttcacatattctggtttcacctgcccaagctgtcttcaggcatgaggtcttgtcagaattgggatgtggatgtctcctatgttaccatttattgtgtgggggcagccatcatcctatttgtctggtccatcaagcttcccagtttcccgctgcacaaggtcccgcatctcttctgtccagcccagaagctccactaggctttccacgccgtgaaccacgtcccccagctgggccacgtccctgctgcgaggatgccaagccaagggccccaccaagtcccggttgatgagcagtcggggaactgagctccgcacggcctcggtcaagctggcaaaaggctccacctccagggaggtcccaaggatgagcagcagatctgccatggggaaatcaaccacatgcagcaagaacctctggggcagcggctccccaaagaacacaatgtcgggcttcacaacgccggtgcagaccgggcagcggggaaccctgtctgccatcacgtcagcttgtgagacttcagtaagtgcccagtaaatgtacattttacccgaatgtcctcccctgggaagggtctttggcagactgtgcaggtggcagaggcaaaggttccatgagcttcaaccagctttgaggcagggatgcccgacactctctcaagcccatcgatgttctgcgtgtagagccgcagaagcagccccttgtcatgaagcagccggagaaagtagtgagtgacgttgggcttgtagtttccagggtacagctccttggccaaagtgaaaaagggcttggggttgtgaaagaagaatgggagttcaaaaatggcctcggggtacgggagatcgtactgctggaggttgctgtacaggccactccccggcgatctgaagtctggaatgccactgggtgtgctgatgccggcccccaccatgaccaccaccctctggcaggctctggcccgaatcagctcagctacatcctgcagggaaagcttccccttgtcactgctgcctccacttccaacaacacttgaagcacccacagaaaaagatatggaccttcttccacctttaataatcgtccctgccgccaagcaccagccgacagccgcaggcctgaaacggccccacgcctcccccggcctcgacccgttcaactacccggccccacagccggagggctgccgcggcgcgccaaccccagaacgccatgttccgcgcagtcc

SEQ ID NO: 17564 - RNA, 2837 nt, Homo sapiens
  source 1..2837: mol_type = other RNA
tcaggccaggcacagtggctcatgcctgtaatcccagcactttgggaggccgaggtgggtggatcacttgaagccaggagttcgagaccagcctggccaacatagcaaaaccttgtctctattacaaatatgcccatgtgctaggtgtggtgggacacacctgtaatcccagctacccaggagaatcgcttaaacccgggaggcggaagttgcagtgagctgagatcataacaccgcactccaccctgagtgacagggcaagactcaaaaaataaaaaaggaacattaactagggttagaaactaacttcattctttttagaattcaacagttttcctaggtcaccaattccaccttttgttcttattaaggcgcaaagtcacaggacccccttcctgggagtcactgtcattaaatctattgccgtcagctcagcccagggtaggcaaggttcaagaatgggaagtgcttttgtctggggaaacacgcaggtaatgtgatgctaggaaggaggatgtgcaggtgggtgagagcccaggagggagcagctggtgcctgacagggtgagccatcagggctgggcctgggtacagccccaggagaaggagcctgtgcagaagtagcagttcagtggattccacctcctatgtcacaatccagcaggtggccaggactcagcctgggttttaagtgagtaatgccttccctgtctcagagattagctctaacagtgtcactagaggaagccctggcgagggtgggggggcgtagtgtggggacaaggaggccagatagaaagtgctggaatgttctggaacagatctgtttctggaggagaggctgagtatggagagtcaacagaatgtgaccaccttcagagggaggagctgggccgtctccaataaatccagggacaaatgccttcagtcctcagactgttccaatagaggggacgccacgtatcccagggttccctttccaactcatgtcaacacctgcagtccctttgaggagactaaatgtatttcatgctggaaagaacagattttctctcattaaaaatagccccactaaaggagaccaacatgctagaagtgcggcaccagggcctcaagactacacttcggaacatgaagagggctggggaccgctcggcccaagtctggatcttgtaaccaacagatgccgagcttgccgttcaactaggcacagaaagcagactcggtctgggattccagttggtctgattcagttcaagagggtcacagtcagaagaaagctttttccattaggagcttcagcagagtgaagagttcaacacagcaaacaggcaggcagctcctttgtatatgtgacggggtggccctgactgtaaacacagccctaccagtcactgcagctcatggcctgagaagacattccagtggcagcctcgggtgtccactcagttcacatattctggtttcacctgcccaagctgtcttcaggcatgaggtcttgtcagaattgggatgtggatgtctcctatgttaccatttattgtgtgggggcagccatcatcctatttgtctggtccatcaagcttcccagtttcccgctgcacaaggtcccgcatctcttctgtccagcccagaagctccactaggctttccacgccgtgaaccacgtcccccagctgggccacgtccctgctgcgaggatgccaagccaagggccccaccaagtcccggttgatgagcagtcggggaactgagctccgcacggcctcggtcaagctggcaaaaggctccacctccagggaggtcccaaggatgagcagcagatctgccatggggaaatcaaccacatgcagcaagaacctctggggcagcggctccccaaagaacacaatgtcgggcttcacaacgccggtgcagaccgggcagcggggaaccctgtctgccatcacgtcagcttgtgagacttcagtaagtgcccagtaaatgtacattttacccgaatgtcctcccctgggaagggtctttggcagactgtgcaggtggcagaggcaaaggttccatgagcttcaaccagctttgaggcagggatgcccgacactctctcaagcccatcgatgttctgcgtgtagagccgcagaagcagccccttgtcatgaagcagccggagaaagtagtgagtgacgttgggcttgtagtttccagggtacagctccttggccaaagtgaaaaagggcttggggttgtgaaagaagaatgggagttcaaaaatggcctcggggtacgggagatcgtactgctggaggttgctgtacaggccactccccggcgatctgaagtctggaatgccactgggtgtgctgatgccggcccccaccatgaccaccaccctctggcaggctctggcccgaatcagctcagctacatcctgcagggaaagcttccccttgtcactgctgcctccacttccaacaacacttgaagcacccacagaaaaagatatggaccttcttccacctttaatactttttcaacccggatggcggtgatagttaatactttctgagcgcttttactatggtcaggcattatatttacacctaatcctcgcaaaacactactgggaagatcctcatttgacaggagcaattccgggtcacaaaggctgacaccacaaagctagtccgtagcgggttcgaccacaggcgcccacactctttgacgcctcaatggcacagccaagtgcgcgggaagtgggctgcaaacgccggagagttttgtccggagcgcagagacgcgctgtaaccgagcaaccagcggggcccgcccccggcctgctac

SEQ ID NO: 17565 - RNA, 551 nt, Homo sapiens
  source 1..551: mol_type = other RNA
tcaggccaggcacagtggctcatgcctgtaatcccagcactttgggaggctgagatggatgaatcacgtgaggtcaggagttagagaccagcctggccaatgtggtgaaaccccatctttactaaaaatacaaaaattagctgggcgtggtggtgggcacttgtaatcccagctacttgagaggctgaggcaggagaatcgcttgaacccggggggcagaggttgcagtgagccatgatcgctctattgcactccagcctgggtgacaagagtgaaactccatttttctcatattccttccaataatttgttaggaggtggacctcagccagccccccagctcagtggtccagaggctcgggtcccgcgctgacgcccagcgcctccctcctccacagccgtcactgaccgctcgctcgcctctagcctggaccccgctgtccagcagtcccggctggcccgcgccgcgctcctcccgctctggcagtcctggcactggtaggacgcccgcagccttccaccctagagggcgccgggcgggcacgcgctgg

SEQ ID NO: 17566 - RNA, 2532 nt, Homo sapiens
  source 1..2532: mol_type = other RNA
tcaggccaggcacagtggctcatgcctgtaatcccagcactttgggaggctgaggcaggtggatcacctgaggttgggagttcgaggttggccaacatggtgaaaccccttctctactaaaaatacaaaaattagcctggcgtggtggtgaacacctgtaatcccagctactagggagactgaggcaggagaatcacttgaacctgggaggtggaggttgcagtgagagccaagatcatgccattgcactccagcctggacgacagagcaagactccatctcagaaaaaaaagaaaagaaaagaaaagaaaatatagtttactaattactacttaatattgtttaagggtctgtaatcccagcacttagcactttgggaggccagggcaggtggatcacctgaggtcaggagttccagaccagactgaccaacacggtgaaaccctgtctctactaaaaatacaaaaattagccgggcgtggtggcgggtgcctgtaatcccagctacttgagaggctgaggcggaagaatcgcttgaacctgggagactgaggttgcagtgagccaagatcgcaccactgcactctagcctgggtgacagggcaagaccctgtctcaaaaaaaaaaaatttaaaaaaagaatatgaaaagaaagtctttaaacaaatctgtacttcgccttcaaaaattgaagacttttttgttcaatatttatatatgactctttattcaaaatatacattaaattctatctagttaaatcctagtcattgaatcttgtagtgtcagtgaccatttaagaaccttacctttttaagcagatctctggcttcttgtgtgaggtagggaggcaaattgagtttacatttgaggattttgtcaattgttttctttctattctccccagtgaatgggggctaagagtagaagacaagtgaaaaatattagcagggagagaaaaatattagcatataagaaacaaattttgaataatattatccatttcctaaattagttatacatggagatcagaaatgtatgctgtgaaatgggctaactgctaaagacctttattttgttttacagacagggtctcaactatgttgtcaaggctagattctattaataatccttagctcaaatgatcctcccacctcagcctcctgagtagcttaggctacaggcatgcaccactgtggccggcagacgtgcagtttttaagcaacaggacagaggaagtagcagtgtcctggaaggaagcctgtgtttccaccattaactttctgtgtgataagtgagctatgtgattttatgcttcaatttctccatttataaaataagggcattatctattcaacatctatttcacaggcctgccatgacatagatcatttaaaagaaaatgtttcggaaagtatgggatcccatataatcatacagcattattagtgttaaactgctaataacaaatctttgggctttgaaaactccactggtaacatgttcagaaagcacaggacaggtctcttgctatagtgactcagcacagaccaataatacatgcagcttttaactgtgcacctactgctccagtcagcatgtcatacattaatgctcccaaactccaccaatccacagcacgattgtggccacttctcatcaagatttcaggggccatgtattctattgttccacaaaatgtgtgtgtgactgttccatcatgaatagattctttgcatagtccaaagtctgttagtttcacatgactatagaattgtttacggtatgtctccaccttggtgattaagcatgatattctccggcttcaggtctctgtagatgatccccttttgatgtaaatgccccaaagccatggagatttctgccaagtaaaagcaggcagtgtcttccataaatattccctctctttctaactgcataaatagttctcctccactgagatactcaaggatgaggtagagttttccaccagtctgaaaggcataaattaaatccacgatgaagggatgctttacttcctccagaatattccgttctgcttttgtatgagctgtatctttagcatttcttactatcattgcctttttaagcaccttcatggcaaatattttcccagtatttgctcctgttacttttcgtacttgaaaaacctttccatagccccctttaccaagtacccgaagtagctcaaaacattctggtctgattttttctggccctctgttcacactagtttctgagatttcaaatttctcacaatgttccatgccaagttcatatggtccaactcccccatggtccatgctttcatttaactgacccccctcctccagctcatcctcagagcccgcgtcctctggctggtccaggtctatgtcaaacactcctgccatgtcctcagcttccctgtctcggaagtccggggctgggtaaaagccgtcccgcctccttcgtcgcctcatgggcccggacccgccgcagccaccacagccgctgccgccatcaccggct

SEQ ID NO: 17567 - RNA, 2657 nt, Homo sapiens
  source 1..2657: mol_type = other RNA
tcaggccaggcacagtggctcatgcctgtaatcccagcactttgggatgctgaggcgggcggatcacgaggtcaagagatcgagaccaccctggccaacatgatgaaaccccgtctttattaaaaatacaaaaattagctgggcctggtgacacacgtttgtagtcccagctactctggaggctgaggcagaatctcttgaacccgggatgcggaggttgcagtgagctgagattgtgccactacactccagcctggcgagagggcaagactccgtctcaaaaaaaaaaaaaaagaaagaaaatattatgctaagtagtgaaatcttcagtcctgccccccgccccccaccacccacagctctttcagaagttaagaaaacaacaggaaaaagaacaattctgttgattgaaccaagactcaagataccatgaattaatccaagtctcagaaaataattaaaaaaaaaaaagacaatcccgatgaggttacaggacacaaaagataacaagagtcatcaccgaataagactaggaggccttccggaaagggacaattttctgaaaagcttgccgaaactcttcattaaacacagtgtagattattggattgatgagggagtttaaatagcctagccaggtgaagaagtcaaagagcgccgggtggatccagcaggagtcccggcagatggggaggaccagagacaccacgaagaagggcagccagcagatgataaaggcccccagaatgatgcccaggattttagtggctttcctttctcgagcagcagaaatcctcttgcgttccagggcactgtcagcaagcttgattttcacgtggttgaaaaagagaggggagccagccgagtgcgagtgcccctcatggaggctggagttgagcgagcagagcgaggacccggcagagcctgtgatgaggtgggccgtggtgaagcgcttcccatagagtgagggtggattcaggatgcggttccgggcagcccggtagatccggccatataggatgatgagcaacaccgagggaatgtagaaggccccacaggtggagtagatggtgtaggagatctgagaggtgttcaccagacagtccgacatctcctcctgggccttggcctgccgccagaagagcggggggatggagatgcagatggagatggcccagacaatggcgatcatggtggccgcgtggccagccgtcctgcgtttactgtattccagggcatctgtgattgcccagtacctgtccagagcaatgacacagagatgcaggatggaggctgtgcagcacgtgatgtcagaggacagccagatgtcacacaagatttggccaaagttccaggtgtgggtgatggtataggcgatgctgatgggcattaccaagatggaaaccaagaggtcggtggtggccagggagccaatcaggtagttggcaggggtgtggagcttcctggtgagtaagatggtggtgagtacaaaggcattggagaggactgtggccagtgtgatgacggaaaggaccacggcaagggagatcttgagcgcctggagggtcctgggatcccaagcctctgaggtttctgtggcattcagggatctgttggaggcctcctggggaaggccttctgctgactggttcagtggggacatgctaggtggctctctcttcccacagacctccacacatttggctccttccttcaaggttgtcctgacaacagagcaaagtcatccttctgcttcacactggtgggagccgtacaccagaacagaccacagtgaaaaggtctcaagaccagactattctctaagtacagttgcaataaaataaaattaaataacaataataataataatattaaacaagaccggactatttgaagaatgctgagacaactaccagctggtagttaaaggtctttcctaaaccacaggaatcccaagatgtctcagggtcctggaacttttcccagcagatggtcatgcccaggggacacatgctgaatttgttagacaattatcaggggatcacacccaggtgggcaatgccctgggattcttgcctttggcatctggctcttttcaaagcttgagacattcgtgtgtttaatgagaacttcagaattcccctcacagtaattgaaacgattctggatttagggttgcttctgaggagcttttaaaactagacacaaaaagaagttccagccgattcagagaagcagtccagtcagcacagcagctcgcggttttcccaggttcatcttgacgcatcctgagctacttaacttcggttcctatcccactgatcgttttagagcctgaacagacaaaacatcctggttaccaagactcgaagaatgcataagctgggaccaggcaaaacaaacagatcactgtgggctcacagagcagggacacattcagaagatccgctgcccggcgggcaggtgcgcacacccggcgtacccgcccgatccacttcctcgcgcggcgtctccccgtcgcggccgccttgtctccgccgcgacccccgccgaactcgggggccgcccgccccgccgccccggggccctttccggctcgcgccctcgcgatcccgcacctgcctccgcctctcccagagccctgcggctccttctcc

SEQ ID NO: 17568 - RNA, 1460 nt, Homo sapiens
  source 1..1460: mol_type = other RNA
tcaggccaggcacagtggctcatgcctgtaatcccagcactttgggtggccaaagtgggcaaatcacctgagaccaggagttcgagaccagcctggccaacatgacaaaaacccatctctactaaaaatacaaaaattagctgggcatggtggcacaggcctgtaatccctgctacttgggaggctgaggcaggagaatcgcttgaacccgggaggcagaggttgcactgagccaagatagtaccactgcactccagcctgggtgacagagactgtctcaaaaaaaaaaaagtatttgttgaatacctgttgtgtggtaggtactagggatacagcagtcaacataagagccagaaatctaaaaggtgaggaaatacacattctaagaatgtaaggaaaatttatgtcaatggtaatgatatggagaaaaatcaagcaatatggactccctatgaagtcatgcagaaattaaggtacaggggatgaagatatcctagagataaaaggcatggtgatattagtactgatattcctgaaagagaaagctgagtgttgtaggaaggatggggttttaattctggggccctctcttctggcaatatagagacggagaagggaagtcttaacatctgtatgttcccagaaaaatgtatctccctaattcttgtatgtaattttgaaggttcatggacacttctgaagccatttcatacgtattttaaattgcacccaagaagaaatatctgagatgtttgcattcccatatgtattaggataggctgagttgtgctgcagtacaaccccaaatcccaactcttaagggaccggggccaaaagtcccatcaaggtaaagttttatcctccaagaccaggctctctggaagtgctatatcagatttggatgtttgctcctactgttctggagacccaggaaccaaaaggatatcttctgttttccacatacttaatgtacagtggtggaactgtatctgcaacaaacattcttcacaaactcacgttttcctcaagcggcaccctcggcagcgctcaagtgagagtattccatccttggaatactccgagaaggttcgagccagaagttggattgcctgaaatgccgcttccagcgcactaagtaacttgaactgcgctaagcaactggccagaattggtttggtttggtttgaccctggggttcctccgtagtctgtaagtggagttgcgaactcaaccccttctccaaggcgggagtgtttctaggagggaacatacttccccttaaaggaagatcacgttgctaaagtaaaaaatttgaaggcgccctatgtgtagaacacttacgttcttggctttctggccactataaagatgggtcgggaatggcgccagctacgttaaaaagtaacgtgcaggaatggttcagttgcccggtgttgaccagagtagagatggttttgccc

SEQ ID NO: 17569 - RNA, 2549 nt, Homo sapiens
  source 1..2549: mol_type = other RNA
tcaggccaggcacagtggctcatgcctgtaatcccagcaggaagatcgcgaaaagcatttttcaaatgcacaaatgcttaaagattcaggagtaagtgggctattacacctgttaagcctattaccatgtagtttcattcctagtgaccaagtagacaaactgctaattatcaaagcataaaaggtattagactctgcaggagaaaagcaatgtagattagtctaattttatagctacttcaaattgccatctttttctattagaaccttgttcctattctgaatagcactcaatagaacttgtgaaaccatcaaactggcataaagcttactccactgacttcaaaatggacccttccactcatagggtgtacactagccactacacttatttcttatgtcatggcaaatagtcaactttcactgcccagtcattttaacccacgtttcaacatgcacatcccagtaatttggaaacattttgtttccaaagattcacttaacattggtttagcaacatgaagctttctatgcaacacaaggactcagtttttggcctgttttagtgacaggcaatcagcaacatgctgcatttctctccagtgttgtaatcaaagcaaccctcccatagctttaaatgatattccttccccttccaattatgtggggggaaaacaaccctattctccacccagaagtgttaactcaagaattacattttcaagaagtttccagattcgtaaaaccagaattagatgtctttcacctaaatgtctcggtgttgaccaaaggaacacacaggtttctcatttaacttttttaatgggtctcaaaattctgtgacaaatttttggtcaagttgtttccattaaaaagtactgattttaaaaactaataacttaaaactgccacacgcaaaaaagaaaaccaaagtggtccacaaaacattctcctttccttctgaaggttttacgatgcattgttatcattaaccagtcttttactactaaacttaaatggccaattgaaacaaacagttctgagaccgttcttccaccactgattaagagtggggtggcaggtattagggataatattcatttagccttctgagctttctgggcagacttggtgaccttgccagctccagcagccttcttgtccactgctttgatgacacccaccgcaactgtctgtctcatatcacgaacagcaaagcgacccaaaggtggatagtctgagaagctctcaacacacatgggcttgccaggaaccatatcaacaatggcagcatcaccagacttcaagaatttagggccatcttccagctttttaccagaacggcgatcaatcttttccttcagctcagcaaacttgcatgcaatgtgagccgtgtggcaatccaatacaggggcatagccggcgcttatttggcctggatggttcaggataatcacctgagcagtgaagccagctgcttccattggtgggtcatttttgctgtcaccagcaacgttgccacgacgaacatccttgacagacacattcttgacattgaagcccacattgtccccaggaagagcttcactcaaagcttcatggtgcatttcgacagattttacttccgttgtaacgttgactggagcaaaggtgaccaccataccgggtttgagaacaccagtctccactcggccaacaggaacagtaccaataccaccaattttgtagacatcctggagaggcaggcgcaagggcttgtcagttggacgagttggtggtaggatgcagtccagagcctcaagcagcgtggttccactggcattgccatccttacgggtgactttccatcccttgaaccaaggcatgttagcacttggctccagcatgttgtcaccattccaaccagaaattggcacaaatgctactgtgtcggggttgtagccaattttcttaatgtaagtgctgacttccttaacaatttcctcatatctcttctggctgtagggtggctcagtggaatccattttgttaacaccgacaattagttgtttcacacccagtgtgtaagccagaagggcatgctctcgggtctgcccattcttggagataccagcttcaaattcaccaacaccagcagcaacaatcaggacagcacagtcagcctgagatgtccctgtaatcatgtttttgataaagtctctgtgtcctggggcatcaatgatagtcacatagtacttgctggtctcaaatttccacaaggagatatcaatggtgataccacgttcacgctcagctttcagtttatccaagacccaggcatacttgaaggagccctttcccatctcagcagcctccttctcaaatttttcaatggttcttttgtcgatgccaccgcatttatagatcagatggccagtagtggtggacttgcccgaatctacgtgtccaatgacgacaatgttgatatgagtcttttcctttcccattttggcttttaggggtagttttcacgacacctgtgttctggcggcaaacccgttgcgaaaaag

SEQ ID NO: 17570 - RNA, 1999 nt, Homo sapiens
  source 1..1999: mol_type = other RNA
tcaggccaggcacagtggctcatgcctgtaatcccagcattttgagaggccaaggtgggtggatcacgaggtcaggagattgagaccattctggccaacatggtgaaaccctgtctctactaaaatacaataaaaaaaatagttgggtgtggtggcacactcctgtagtcccagctacacaggacactgaggcaggggaatcacttgaacctgggaggcggaggttgcattgagccgagatcacaccactgcactccagcctggtgacagagcaagacttcatctcttgtgatccactcacctcggcctcccaaagtgctgggattacacgcgtgagccactgtgcccggcctgtggtctattagttttcaatgcaactgtggaactctgagaattttttctttaaaaaactccaacacactcagttttcctgcaagtattaggattcgttgctgtttcttccactcatgcctggtaaagtggatggcttctctatgggctcatgcttttctatgggccaagagtttggtagcatcttgactgggagttcaggctcaacatgtctcagttagttgcagtcaagtcatcagccttagctgaagtactctgagagcttgattatgtcctcagggtgcacttcccagttggcttgctcacatggctgccatgttggtgctggttattagttgaaggctttttctctacgtaggcattctaatgggctctttgaggatcctcatgacatggcagttggcttcctccagaacaagttatccaagagagagcaaggaagagatacagtgtctttcatgactcagctttgaatacaactctgcaacatcctatgggctataaaagtcggtcctttctcatgggggaagagactaccaagtgtgtgaacacagtgtgagaggataattgcaggccatttcagaggtcataatcattatcttattttgcagatcagggaactaaaatcagagagacgaagtcatttgacaaagaacatagaacattgggaaaggtcacttaaacccagacactctgatttagagaaagcaagttttgaaactattctatatttatctccaatagatgatttctttattactgtcacatggatattaacataatagtcagataaatctttctgtaatgaaagtgctttccaaactcacgagtttgtcttttctttttctttccttttttctccctcccttctttttcttcctccttcttttcttcctttctttttctttcttcctttttctttcatttacatagaatattaacagcttggagaacatgttttgggaaatatcactgaggatggaggaatacggaggagtgacagggcacaggaaacttctggggtaagcgagatgttcattatcttgattgtggtgccggcttcatggatgtatacatatgtcaaaatttatcacactgtgcacattaaatgtgtgccattattgtatgcaaattatactacaataaagcagagatgaagtgagaaactcctggtgatggttgggtccatgatgccagatacctttaacaacagcactctttttccttctggggttgttcacgctgaagccctgggctgcaggaacctcacctgtctctattcgttaaagtctcagctcaaacaccactgtcccagataggcctcgtgaccgcaggactagaccacggttctctgcggagggcgtcagctccgtgagccacccttccagcacccactgccatggcgaatatttgcttgtttggccatccagggactgtttgagccccaagaccgcagggctcggggtctgtctttgctcaggacgataacctggggactggacagtaggccctcaggccttgggaccgctcaaagtgaaccggggccgggtgggggacccagggctctgcagccttaagaacgcctgtgcccccgggacgcaggggtcaggcccggcccggcccagaccgcctctgcctcctcctcctt

SEQ ID NO: 17571 - RNA, 1845 nt, Homo sapiens
  source 1..1845: mol_type = other RNA
tcaggccaggcacagtggctcatgcctgtaatcccagcattttgggaggccaaggcaggaggatcacttgagcccaggagttccaagaccagcttggtcaacatagtgaaacccctggtctctaccaaaaaaaaatcacaaaaattagtcaagcatggtggcagatgcctgttaagtctcagctaccaggcaggctgaggtggatcacttgagcccaggaagtcaaggatgcagtgagccatgatcaacccactgtactccagcctgggtgacagagtgagaccttgtctcaaaaaatataaatttttttggccaggtgtggtggctcgtgcctgtaatcccagcactttgggaagcagaggcaggtggatcatttgagtccaggagttgaagaccagcctgggcaaaacagacccgtttctaccaaaaaaaaaaaacaaaaattggcctggtgtggtagtgcacacctgtagtcccagctgctccagaggctaaggtggaaggacaatctgagcctggggacattgaggctgcagtgagccaagatcaagccagcgcactccagcctggacgatggcaaaaccctgtcttttcaaaaaataattcatatcctctctggggatgcagcccaataagcaagactcttgcctggtgaggacccgtctcaagattcaattcattccttcagtcactgtcatccccagtctcctccttttcttcctgagccatggagtcttctccctcttccctcagtcctgcgaagaagtcatcggtgctccaagtcttgctgctcagagcccgcagtggtcctcccttttttttgcgccgacggtagtcatccaccaccacagctcgcagctgggccatgtcccaaaacttgaggcgctggtcatggccactactggccaggaagcggccacagtgggagagggccagctcctccacaggctccccagtgtgctggcccacactgcccaccactcggttcggtaggatgttcacagccctgatgactccatcagtggagccagtacacagcagactctcggtgactggaaccatgcagtcgatagattcagctctcagggcaaagcggtcacttgtggccccaaagccattccaattgaagaggtagatggtaccttcactggagccacaggctaccttcttcccccatttcatgagagtgacagaggtcaggtccccagactgaggttctgagagcagctcaaaccgacgcctcttaatgttgaagatgccaaggcagccatccccgctggctgtcagcagcagctttttggctggatccagagccatgtctgcgatgtactcttcatgttgcctcatatccattaaggggccctccttccgctggtcccagagacagataccacctgtgtcatccccagtggccagaacattctcatccaccagcagaagactattgatgggggcaccatgagccttggaaacacgtctttccagttggccctgctccacatctagaacatggatggctttgtccttggagacagtaatgagcttctgcccatcttcagagaaggccacagctcggcaggccttgagatggtgacctgatgaccagagctccttggtttctccctcttggcaagagtaggaaaagacgaacacgtccccgtccacgtcccctgcagccagtaggtcacgggccggatggaacgccagcccactagccggagcttccagcacgatgtcttccggagtgtcccggatccgggttggggcttccatggagtctgggtcctcctcgtcgctcccatcctcagcgggcctctcctcacaagtgcggtccatgctgagaag

SEQ ID NO: 17572 - RNA, 149 nt, Homo sapiens
  source 1..149: mol_type = other RNA
tcaggccaggcacagtggctcatgcctgtaatcctagaactttgggaggccagggcaagagaatcacttgagcccaggagatagagactagcctgggcaacacagtgagaccccatctctacaaaaaactttaaaaactagctgggctc

SEQ ID NO: 17573 - RNA, 3036 nt, Homo sapiens
  source 1..3036: mol_type = other RNA
tcaggccaggcacagtggctcatgcctgtaatctcaacactttgggaggtaaggcaggaggatcatttgaagccacaagtacaaggtcagcctgggcaacaaagtgagacccccatctctacaaaaaataaaaaaaaattagccaggaaaggtggtgcacacctgtagtcctagctgcttgggaggctgaagcaggacgatcgcttgaccccaggagttggaggctgcagtgagctatgatcttgccactgcactccagtctcagtggacagaaaaaaaatttaatttttccagagaaaagggaagggaaaaagtgttccataatctaggatatgttcaagagcctttgctcttatagtcaaatatataaaaacaattttccttaaagaaataccagtctatgagccaaggcaagctttggctaaatgattggttagcttttatttggctctagaggtttccatggaaacagcctgagagacagaaaaggcagcattatcatctttatccatgatgccatctgataaaactgcacattgattcattcatgctattcagagcagatgtattacttctgataagcctggacaaagggaggcatgagttttatcccgtcacgctttgaatttcctgtcttcccctgtttgaaaccttaaattaaaatcctgataaaacctcctctgaacatttccctcaggagcctctagctgaagtaatgcttcaataatcagaagtcatatgaagaaacgtgaagccccaaatggagctccactgccaagttcttaaaattatatggcaccacgcttcctgtagctgaagaaattgttctgaagagtatttacaattccattatatcagatctcagccaggcaagaaatgtcatcataagtgtttattatatacagttgaagcaggtggcatcatccatcatttttcttcctcttgatgtctagatcagttgtgtgtgtattttaatatagtaacacaccctcacaattatctaatcttatttcaggttagtgcttcttggaaaggctacaaaagcagccatagctcagaattatgtatctgaagtaaacaaaaataaaaacctcaacaacaaaatattaaccaaacaaacaagataaagacgcatgcaacctatagcaccatacctaagaccacaaagggcaggagggttgacagaggtcttaagaggaatccagttttgggttttctcctaggatgagatcccaaatatagaacctatttgtagagtccaatacttttaaaaagggaaagcctgagaaattctgttaacagaaatatgaaaatccatgattttccagaagacagatgatttgacactgttcttattctaaaagcatcaaagacgttataccttagaaataaactgctcactttggaagatcagttaggcaatccctgccaacctcaatgaactaaaatgatatctcagtaagttaaaaatatgatacacccccaccaaggaccaatttactcatggaaagtagtttacagagcagttagctctctgacatctgtataaccctacagacatgtgctacattgaaaagattcaatcttgcacatatcattatatgctccacatggcaaaacatctgaaaaacactcagatgtttttcaaaaacctctgtgcattatgacattggtgtggaaatttagatctcagcttaatcctttccaaaagaagcgagtaaaagtcccgggaaaggtttacttagagatgagtgaagattctggtaatttaaaggtgatgggttaagaagctatagagctagaaacaacttcagatctcacctaatccctcatcttattgacggaaaaactgaagtcccaagataagtatcagatccaaccaatggaagaactgtgaccagaagagaaaccatgggactcttagttcagtgcttttccccatcatgtttatctggggctcctttaaatcttagcatgcataatttaataaagctctaaggaaaatgactgaaaagtatcagagaggaaaaatgctgccttctaatgaagactttggcaattcacgttctgatgtgcttaatattaacaaacggaaaaccccagtcatcttttggcaaaaatgttacttcttctaagaaacaggttccttttctgagagcgagctgattttgtaggtactgggttacagcattgtaggttacagctgacagttttcatatgccccatctttgtagttacagttagattctgcagatcctatatcatcaggtggactgaaatgactgctgccttgagactctgtatcaatacttttggtttctgactgaaggtggacagaaacctgaactgctatttcctggccttgttcattcagagagccatcatctgaatctcctcctggtgaattactccgtcccatctctgggttaatgacatagatgccaccttgagcattcaaggcaggtctctctttaattctttcacccaggtcatcagggtcgtccactcgcacagcctcaaacatctcctcaacaaaggctcgacagtttagaataagaggtggaagagggacacttcttgccagttcttcaatataacgagcaaactccatggtcttaaattgtgtgactttggcgagctccagagttttggctgaggtaatgatggggatacgttttgcaatctcaaaggccttctgaagtttctcagccccttcagttctaaagaactcattgatagccttctcagtcttgcgaagatggctgctcatcatgcacagccgtgtgacattcaagatgagtgtgattgtaaaggcaatcaggcaaacaatcatgtaatagacactcatgtctcccgaggtgaagataacacgtagggtgacagagtaggaggcacgaattggagaggtgacgaaacaggtatagagcccacggtcatcaaaagctacattggtgatgtttaggaagttatcagaaaccaaccactttccacccgaccgccgtctagctccttccggcctcagcggcggcttaactc

SEQ ID NO: 17574 - RNA, 3497 nt, Homo sapiens
  source 1..3497: mol_type = other RNA
tcaggccaggcacagtggctcatgcctgtaatctcaacactttgggaggtaaggcaggaggatcatttgaagccacaagtacaaggtcagcctgggcaacaaagtgagacccccatctctacaaaaaataaaaaaaaattagccaggaaaggtggtgcacacctgtagtcctagctgcttgggaggctgaagcaggacgatcgcttgaccccaggagttggaggctgcagtgagctatgatcttgccactgcactccagtctcagtggacagaaaaaaaatttaatttttccagagaaaagggaagggaaaaagtgttccataatctaggatatgttcaagagcctttgctcttatagtcaaatatataaaaacaattttccttaaagaaataccagtctatgagccaaggcaagctttggctaaatgattggttagcttttatttggctctagaggtttccatggaaacagcctgagagacagaaaaggcagcattatcatctttatccatgatgccatctgataaaactgcacattgattcattcatgctattcagagcagatgtattacttctgataagcctggacaaagggaggcatgagttttatcccgtcacgctttgaatttcctgtcttcccctgtttgaaaccttaaattaaaatcctgataaaacctcctctgaacatttccctcaggagcctctagctgaagtaatgcttcaataatcagaagtcatatgaagaaacgtgaagccccaaatggagctccactgccaagttcttaaaattatatggcaccacgcttcctgtagctgaagaaattgttctgaagagtatttacaattccattatatcagatctcagccaggcaagaaatgtcatcataagtgtttattatatacagttgaagcaggtggcatcatccatcatttttcttcctcttgatgtctagatcagttgtgtgtgtattttaatatagtaacacaccctcacaattatctaatcttatttcaggttagtgcttcttggaaaggctacaaaagcagccatagctcagaattatgtatctgaagtaaacaaaaataaaaacctcaacaacaaaatattaaccaaacaaacaagataaagacgcatgcaacctatagcaccatacctaagaccacaaagggcaggagggttgacagaggtcttaagaggaatccagttttgggttttctcctaggatgagatcccaaatatagaacctatttgtagagtccaatacttttaaaaagggaaagcctgagaaattctgttaacagaaatatgaaaatccatgattttccagaagacagatgatttgacactgttcttattctaaaagcatcaaagacgttataccttagaaataaactgctcactttggaagatcagttaggcaatccctgccaacctcaatgaactaaaatgatatctcagtaagttaaaaatatgatacacccccaccaaggaccaatttactcatggaaagtagtttacagagcagttagctctctgacatctgtataaccctacagacatgtgctacattgaaaagattcaatcttgcacatatcattatatgctccacatggcaaaacatctgaaaaacactcagatgtttttcaaaaacctctgtgcattatgacattggtgtggaaatttagatctcagcttaatcctttccaaaagaagcgagtaaaagtcccgggaaaggtttacttagagatgagtgaagattctggtaatttaaaggtgatgggttaagaagctatagagctagaaacaacttcagatctcacctaatccctcatcttattgacggaaaaactgaagtcccaagataagtatcagatccaaccaatggaagaactgtgaccagaagagaaaccatgggactcttagttcagtgcttttccccatcatgtttatctggggctcctttaaatcttagcatgcataatttaataaagctctaaggaaaatgactgaaaagtatcagagaggaaaaatgctgccttctaatgaagactttggcaattcacgttctgatgtgcttaatattaacaaacggaaaaccccagtcatcttttggcaaaaatgttacttcttctaagaaacaggttccttttctgagagcgagctgattttgtaggtactgggttacagcattgtaggttacagctgacagttttcatatgccccatctttgtagttacagttagattctgcagatcctatatcatcaggtggactgaaatgactgctgccttgagactctgtatcaatacttttggtttctgactgaaggtggacagaaacctgaactgctatttcctggccttgttcattcagagagccatcatctgaatctcctcctggtgaattactccgtcccatctctgggttaatgacatagatgccaccttgagcattcaaggcaggtctctctttaattctttcacccaggtcatcagggtcgtccactcgcacagcctcaaacatctcctcaacaaaggctcgacagtttagaataagaggtggaagagggacacttcttgccagttcttcaatataacgagcaaactccatggtcttaaattgtgtgactttggcgagctccagagttttggctgaggtaatgatggggatacgttttgcaatctcaaaggccttctgaagtttctcagccccttcagttctaaagaactcattgatagccttctcagtcttgcgaagatggctgctcatcatgcacagccgtgtgacattcaagatgagtgtgattgtaaaggcaatcaggcaaacaatcatgtaatagacactcatgtctcccgaggtgaagataacacgtagggtgacagagtaggaggcacgaattggagaggtgacgaaacaggtatagagcccacggtcatcaaaagctacattggtgatgtttaggaagttatcagaaaccaaccactttccacctctgcttctgccatccagttgctgtccttttgaattgtgccaatggacatcttcatagtgactggctgtgagaagacactcaattgaaacgctagttccctctttggctatgatgacatcatcatccgagtgggaacttgctgagagttcaaagcttgagggaaaggatgcattgtaagaactacgatttgcttccagtgaaaccatttggtcgaagtccacatcttccaaaacaaaagcagctggcacaataatacttgccactaaagtgaataagcaacaatgtagcttcatgggaaaatgggacaaaatcttgtttagatttggagaactcaaaaacttctacactacaacaaaagcacagcgggtaatttattgcttggtagagaaattttccaaacaagtggtagatccagttatattttctagtcttcaagattaaaagatgtgagtagagaacccgaccgccgtctagctccttccggcctcagcggcggcttaactc

SEQ ID NO: 17575 - RNA, 3794 nt, Homo sapiens
  source 1..3794: mol_type = other RNA
tcaggccaggcacagtggctcatgcctgtaatctcaacactttgggaggtaaggcaggaggatcatttgaagccacaagtacaaggtcagcctgggcaacaaagtgagacccccatctctacaaaaaataaaaaaaaattagccaggaaaggtggtgcacacctgtagtcctagctgcttgggaggctgaagcaggacgatcgcttgaccccaggagttggaggctgcagtgagctatgatcttgccactgcactccagtctcagtggacagaaaaaaaatttaatttttccagagaaaagggaagggaaaaagtgttccataatctaggatatgttcaagagcctttgctcttatagtcaaatatataaaaacaattttccttaaagaaataccagtctatgagccaaggcaagctttggctaaatgattggttagcttttatttggctctagaggtttccatggaaacagcctgagagacagaaaaggcagcattatcatctttatccatgatgccatctgataaaactgcacattgattcattcatgctattcagagcagatgtattacttctgataagcctggacaaagggaggcatgagttttatcccgtcacgctttgaatttcctgtcttcccctgtttgaaaccttaaattaaaatcctgataaaacctcctctgaacatttccctcaggagcctctagctgaagtaatgcttcaataatcagaagtcatatgaagaaacgtgaagccccaaatggagctccactgccaagttcttaaaattatatggcaccacgcttcctgtagctgaagaaattgttctgaagagtatttacaattccattatatcagatctcagccaggcaagaaatgtcatcataagtgtttattatatacagttgaagcaggtggcatcatccatcatttttcttcctcttgatgtctagatcagttgtgtgtgtattttaatatagtaacacaccctcacaattatctaatcttatttcaggttagtgcttcttggaaaggctacaaaagcagccatagctcagaattatgtatctgaagtaaacaaaaataaaaacctcaacaacaaaatattaaccaaacaaacaagataaagacgcatgcaacctatagcaccatacctaagaccacaaagggcaggagggttgacagaggtcttaagaggaatccagttttgggttttctcctaggatgagatcccaaatatagaacctatttgtagagtccaatacttttaaaaagggaaagcctgagaaattctgttaacagaaatatgaaaatccatgattttccagaagacagatgatttgacactgttcttattctaaaagcatcaaagacgttataccttagaaataaactgctcactttggaagatcagttaggcaatccctgccaacctcaatgaactaaaatgatatctcagtaagttaaaaatatgatacacccccaccaaggaccaatttactcatggaaagtagtttacagagcagttagctctctgacatctgtataaccctacagacatgtgctacattgaaaagattcaatcttgcacatatcattatatgctccacatggcaaaacatctgaaaaacactcagatgtttttcaaaaacctctgtgcattatgacattggtgtggaaatttagatctcagcttaatcctttccaaaagaagcgagtaaaagtcccgggaaaggtttacttagagatgagtgaagattctggtaatttaaaggtgatgggttaagaagctatagagctagaaacaacttcagatctcacctaatccctcatcttattgacggaaaaactgaagtcccaagataagtatcagatccaaccaatggaagaactgtgaccagaagagaaaccatgggactcttagttcagtgcttttccccatcatgtttatctggggctcctttaaatcttagcatgcataatttaataaagctctaaggaaaatgactgaaaagtatcagagaggaaaaatgctgccttctaatgaagactttggcaattcacgttctgatgtgcttaatattaacaaacggaaaaccccagtcatcttttggcaaaaatgttacttcttctaagaaacaggttccttttctgagagcgagctgattttgtaggtactgggttacagcattgtaggttacagctgacagttttcatatgccccatctttgtagttacagttagattctgcagatcctatatcatcaggtggactgaaatgactgctgccttgagactctgtatcaatacttttggtttctgactgaaggtggacagaaacctgaactgctatttcctggccttgttcattcagagagccatcatctgaatctcctcctggtgaattactccgtcccatctctgggttaatgacatagatgccaccttgagcattcaaggcaggtctctctttaattctttcacccaggtcatcagggtcgtccactcgcacagcctcaaacatctcctcaacaaaggctcgacagtttagaataagaggtggaagagggacacttcttgccagttcttcaatataacgagcaaactccatggtcttaaattgtgtgactttggcgagctccagagttttggctgaggtaatgatggggatacgttttgcaatctcaaaggccttctgaagtttctcagccccttcagttctaaagaactcattgatagccttctcagtcttgcgaagatggctgctcatcatgcacagccgtgtgacattcaagatgagtgtgattgtaaaggcaatcaggcaaacaatcatgtaatagacactcatgtctcccgaggtgaagataacacgtagggtgacagagtaggaggcacgaattggagaggtgacgaaacaggtatagagcccacggtcatcaaaagctacattggtgatgtttaggaagttatcagaaaccaaccactttccacctctgcttctgccatccagttgctgtccttttgaattgtgccaatggacatcttcatagtgactggctgtgagaagacactcaattgaaacgctagttccctctttggctatgatgacatcatcatccgagtgggaacttgctgagagttcaaagcttgagggaaaggatgcattgtaagaactacgatttgcttccagtgaaaccatttggtcgaagtccacatcttccaaaacaaaagcagctggcacaataatacttgccactaaagtgaataagcaacaatgtagcttcatgggaaaatgggacaaaatcttgtttagatttggagaactcaaaaacttctacactacaacaaaagcacagcgggtaatttattgcttggtagagaaattttccaaacaagtggtagatccagttatattttctagtcttcaagattaaaagatgtgagtagagaactaccaccttagataatcccgtttgttgacttgtttataatctgcttttcgcactgcttgagagcagggcccttccgttcgttgactgatgtgtccctggagcccagggcagtgcctggcaggtatctggctctcagtaagtgttcgatgaccgaactcccacacccaggccagactttcaaaagaatggcaaacattttcgcctcctgcactcccgaccccaagccacaggctacgactcacgcctcggcgctcctagtagtcccctcgcagcgaccccaaccaagccgtcacctacccgaccgccgtctagctccttccggcctcagcggcggcttaactc

SEQ ID NO: 17576 - RNA, 64 nt, Homo sapiens
  source 1..64: mol_type = other RNA
tcaggccaggcacagtggctcatgcctgtaatctcagcactttgggaggccgaggcaggtggat

SEQ ID NO: 17577 - RNA, 750 nt, Homo sapiens
  source 1..750: mol_type = other RNA
tcaggccaggcacagtggctcatgcctgtaatctcagggctttgggtggccaaggcaggtggatcacctgaggttagggattcgagaccaacctgaccaacatggtgaaacccgatctctactaaaaatacaaaattagccagtcatgggggtgcatgcttgtaatccctgctattcaggaggctgaggcaggagaattgcttgagcccgggagatggagtttgcagtgagccaaggttgcaacattgcactccagcctgggcaacaagaacgaaactgtctcaaacaaaaaaaaaaaagaaagaaagaaaagaaaaaatgctgagctacaacatagtaggttgaagagtgtcctccaaagcatccgcacccactcagaaactaagagtgcgatcttatttagaaacagagtcttcgcatatgtaatttgttaaaaatcttgtaatttgttaaaacctggattttgactgggccttaaattcagtggctgatgtctctatgagaaaagaataggacacacagattcagagaagatggtgacgtgaagatggagacagagattgaaatcatgcatctacaagtcaaacaatgccaaggattgctggcaaccaccaaaagaaaccagaacgtcatgggatggtttttccttcagagcctccagaaggaaccaaccctgctgacacctcggtttcaggctgtagacttctagactcctgaaccatgagagacaatatatgctttttttttttt

SEQ ID NO: 17578 - RNA, 112 nt, Homo sapiens
  source 1..112: mol_type = other RNA
tcaggccaggcacagtggctcatgcctgtaatctgagcactttgggaggccgagtcaggaggatctcttgaggccaggagttcaagaccagcctgggcaacatagggagacc

SEQ ID NO: 17579 - RNA, 85 nt, Homo sapiens
  source 1..85: mol_type = other RNA
tcaggccaggcacagtggctcatgcctgtaattccagcatgttgggaggctgaggtgggaggattacttaaggccaggagctcga

SEQ ID NO: 17580 - RNA, 68 nt, Homo sapiens
  source 1..68: mol_type = other RNA
tcaggccaggcacagtggctcatgcctgtaattccagtgtgctaggaggctgagaaggaaggattgct

SEQ ID NO: 17581 - RNA, 918 nt, Homo sapiens
  source 1..918: mol_type = other RNA
tcaggccaggcacagtggctcatgcctgtagtcccagcactttgggaggccaaggcgggcagatcacgaggtcaggagatcgagaccatcctggccaacatggtgaaaccctgattctactaaaaatacaaaaattagctgggcatggtggcatgcacctgtagtcccagctactcggaaggctgaggcaggagaatcacttgaacccaggaggcggaggttgcagtgagctgagattacaccactgcactccagcctggtgacagagtgagactctgtctcaaaaaaaagagagagagagagaggatagtcttggtcaatacgatttttgaacgtgacaaactatccccattttctttgctctaccagagttcttgacaaagagcataaaggaatcctggaggtggtgagattaattgaaggacagacttgagtcagataacactacctgctccttcacagcgtcaaatggattaaatgtgataatgcaaacagcctaacacacataataggttgatatatgatgacttgctttttcctgaactccagaaatcaatttcaataatcaggtggggaaaccagcagggaatccaatgtccagaaatcctagaagcttcctcccagtaatctccttggaagaagctgaccaggctcaggggaaataaagtagtagagaagtccatattggcctcttcctgtggtttcagctctgtgatcttgtggaaattactccaactctagatgcttcagtctccttatctgaaaaaacagccaggggttttcacagggcaggccaattacgtaaagcacatctccactgtgtgttgtcttaagataatgaggctcctcaccatcagcaagagctggcttgccaccttgggtcactgacttccccactctgtgccatctgtgaaatgt

SEQ ID NO: 17582 - RNA, 10920 nt, Homo sapiens
  source 1..10920: mol_type = other RNA
tcaggccaggcacagtggctcatgcctgtagtcccagcactttgggaggccgaggtgggcagatccacgaggtcaggagatcaagaccatcctaacatggtaaaaccccatctctactaacaatacaaaaaattagtcaggtgtggtggcacgtgcctgtagtcccagctactcaggaggctgaggcaggagaatcgcttgaacctgggaggcggaggttgcagtgagccgagattgtgccactgcaccctagcctaggcaacagagcaagactctgtctcaaaaaaaataaaaaaaaaaaaaagagagaaagagagagagagatgaggagttgctgcactgctgggtgtggagagccgaggaggattcaaagatggtcctgaagtcccagctggaagaagtaggcggcagcaatgtttttaatactgtaaattcatcacgtagcacaggtttggggtggagaaagaaaaattgcattggcttcagggcatgcccagatctttcctcatcttaggcgtttgctaatacatgcattttctaagctgatgtcttgcgtttaatcactgctccattcaaaagagagaaggaggttgtttcaaacctagttgatatcatttgacttccatgctattcacagggctattttatttgaaacaggtataccacagccttaaattgcaagttaatccaggatgttcctaggttggcagttaggaacatgtaattctttggaagggctaaaagtcagctctttaaattatctccatatgaaccttctctccaccttagggtggatccacttatttagtccactgccagtaccacactagaacccgggtggtcactggactccagaaacaacagtagccctctctctgttctgtctctttttgactatctctattctgttcctgaccctgatttctcctgccaagctcaattttgacagctgacaacggcaagccatggcttcccaaaacattattttcaggtcaacttataaatttcaagaacacatttggctccgcttcctgtggtactaagcctacttcttgacagcatttgcctttgttgtaaatagcaaagttcttctagttggatttttgctaagaagtgtgtggatgtggcatgtgacgacatctttagcttggattctagaaaggcactaccattgtgcatttggctaaaggaaacacattttacccgtgaatgccttctatttacaaatgctcagctagcacacaaagctaagtacaagcaataagtactatcctacaatgttactcatttctgaaagcacaaaatgatgactggtatagctttggagatgttttctggaaacccaataaaggaacagatctttgttattccacacctacaaagtcagaagatgcacagtcttttattcatgtttgaacaagcttccttcttgaacaatcaactataaagtgatgtgattctctactagaccaggaactccttgaggacagaatgagggtctaatccatattctaaatccacaccacctggcacaatacatgttgcatggttagggtcaactaagagttggttgaattaatcaataacacacagcaagagaattcacaaagagaggggagtaatcccccagcctcaatcactcggcaagtggaatcgctgggcactgattccagctctgtctcagtgcttgagacagagctgaatgtaatgtgaacatttcaaatgaacaggaaaactagactcacggataagcagtgtagtcatcaagacaacactgtcttggaggtttttctgaagttaaaaccatgctacataagcaataaattatgaaggctgagcatgtgaataaaatttaatgttgtcataaattttataacaaagttaatctgacacatttaatgacatgcataatcattagtatgcagcactgtaatcagacattgataataagcagttcacaccagtgactgtaagagtctttacttgtgttcagccaagccaactgcttggtatatttttctcccttcttagtcgttagttttccatacctacaataactatcagtggtgatgggcttctctgaccatgtgaataatttaatcctcaatgcacagatacagaaacccttgctgaagacagtgtggagcagagaaggctgtctccactccttccacctgaaacacctctgcagatggatatgggagctctgcctacagcccttggacctaaccacttcagtgtgttccagtgagtgtctggacctcggcctgaaagatttttccgaaactaaagaaaatttctctgacctaaagaccttaacctccaccccagaagctctcaccaaggactacagggaactggtggggaaaatccttatcccttactcctcaaggcacagggcagtaatgctgaggcttgtgcgccacacttgctcccagaggtccccagcgggctacctgcggtggtgaatgacctcctaacacgccccttgacggccttcctttccttgcctcacttctccactctcctaccagcattgcagggttcacatcccaaatataccactggcacttgaatcctggtctccaggtctgtttctggaaaaacccaagtaagacattgccccagtaatggggctagatgtctgaggcttcctcaagtatctacctcgaaagctcttactgctgtacacacatgcacatacacacacgtgcgtacaaccagtcacatctaagcaccccgaataccagcctgttgaaggtagcagagagctgcactataagccaaggctgctcccaagagccgctccatcactgaattggcgccccagcaagatgaaggaatgtaatcattggaaggatggagaatgttctctgaatcactgacaaattggaaggggtggagggcaagagtccacctggtggagagatggaaagagcgagagagcctggaatgataatgccattgcttagaaaaggctgctccagatgccatatctacagaaattgtacagcccaaacatctctgagcaataggtctctggtagtcttgatgtctagaccaacaattcccagttcattcttctcagggaaggagccaggatagtccagagactctcattctgctgttagattgaaagggttaggcacaacagccttggcaaagtcacaagggcaaattcacactaaagtgtaaatgacccacaactcctcttctatttttaggttggggaggtgctttagaacataaggaggaactaaagaatattcctgttacatacaaggcagagaaaagggaaactagtggtgacaagacaaatcatccctttgacatttggctggctctacctattacagctctgggggtgaggtgggaacaaaaagatgctgtgtaaagaagtatcttatgccatccctactgtagtgaggtgcagtttagaggggacactgatcaagcagagacccagagtgtttcgttccaagccagaaacagaaatgtataaaacacagcctttccagcatcagaaatgagtagtggtagtggagaactacccaaaacaggaaagaggaccacgtgaggtagagtgtcaaggccctacattccagtgcctctgctcatgactgtaattttgggtaggtcacttaaagtctctggacctcagttttgccatctgtgaaatagggataatactatccagcataaaattggttatgaggctcatgtagggcctgcctgggatgatgtgttgctaatggttaagaacacaacttctggggtctgactggacaggctgaaatccctgcttaacacgttccagcagagccctgggcgatctatttaacttttgttttctcacctgtaagctgagacgaaagtacccactttataagattattccaataattagttgaaataatgcatgcagagaattaagcatggtacttgttatttgttaaactagctattaaaatgtgtaaaatataaagtattgtatggattttaggacaatgcaaagactctttgcttgctgcaatagttcggggccctttcagatggctaaaggcagaatttgtatgtgtaaatatggtgtgcttgtctctgctctggatactgagggcttaccctgttattaaacttatttagtaaatattgaactgtcatgaggcctaacatttagttccagttattagataaaacatttgctttgaatggtatttgaattgccaggttctagattattctggttgacaaactcttcgtattttataaagaggctaaaattggtaagctatcacagaacagatgtgccattttcaaggtatattaaaccatgattcactgtaacattgttcctactggcaacaaattcagagcaggctggactttatttggtgaagaaacattgagtggaagagaaatgacattattttatgtatttacattttcaaattactgtggcttaaacctgttcagccaacattacccaccttcagtctgctaaataaatgattcagtacatttctaatttacagaattttttaacaaaagaaaatgtaatttgatagccaaatcaacgttaaacattatacatttaaaaaaccacaggcaaagacacaaacatgatgacactaacttttgttaaagtatgcttacctatggtttcctctgaggcacgttctttcatgctaagcttccaacataatatgaaaatgaaggagatgcattttgcaaagcaaaacagaccttaagcaaaatattatacttctcaaattaacactgttacaaagttttagaatttaataagttcattaatttaaaagtttggatgtctgagtccttctatcccaaaacaagatcttggagggtcttccacagccatgtaataccatggtcacatgaccctttccaaaattattaatctgaatttactatatgaggataaatctatctttttgaaaatatttaggaaaatgagcttggtatttataaaatgaagctctctttgggtggtatcctaagacacgtcaagccaatcagcctgtaactgtgaaaaaaacattggtaggtacaaaagtggggtgggagaggagtgacttaactttgttaagtgatgggaaagaaacactaatagcattatctcaataaaatgtgatttaaaaaaatttaaaatactaaatcattgaactgacaaagaaatataaatcattcagaaataaactcattaggtcatcaaatcctgttaaatctgcaattaggaagagcaaggtgtacaatccatacatttaaactcacaggctcactttgcacaacgtcaatttactccttaatatgttattaatacgcattttccaaaaggatgtattagtaaatggtacacatctacttcttggcaacatcatataacctggtacaacataagcattcttcttatagttaagaaatgtggatggtatcaaaattagaaaaataaatgccctattatgttgtggtcaggtttaaggcatgtgaattttatcttcatacaaaagattaaaatctagatattaaaaagtagtgcagtatcagtgatgctgcctcagttcccaaaatgtcacatcacaaaaatatcccataattgcctgtagtttattccttggctttcctcttttctctctgcatctttgtaacaattttttaaaagtggaaatataattgttggcaatgctaacagctgtagaaatgattacaagatgtggaaaagcataacaggaatgtcaagaatctgtttctggcagtaatatatatggaacattgttcaggacaaaagaggagaaggaagaaaaaaaggagaggggtttatcatctctaagaattttcaaactaaacctcattgcttaataggaaaaaaagattccatatttaaagttaagtcacctctaactactagctaaagcatgacatcaccagcactggagtcagcggaagtgtgtttttgaaggacagtgttgcaggagaatctggacaggttttagagccaggagagagaaaataattctacctctgacagttgaaggaccttaggcaaatcagtttacctctgctagactacactccaaaatttggacattcaaaaatttgatattaataaccacatgaaagtctcgtgttgaggtgaatatgtatttgttggtgaaagatatgttggtttttaaacagacagcactctgcaattgtaggctattgttttgttttgccagttgtcaaattctatccagctatacacacttgtgtggcctcctaatggtgtttttccagtggctaaaggtttatgaataagacacttttcctaatggaattaacccgatgcttttcttaaacatgtaaccttgagttcaccgcaaaaaacaatgcttcgattagagcaatgcatataataaaggttaccctcgtttcttagacactagacatcattcacaaaaagagaactgcttttgaaagggatgtatttgcactggaaagaatagttttctacttctaattataaatgatttattggtgaaagcaaaacaacagcctgtctgagaggcacttctatgagcatcctcacgtgtgatttgcaaggttgaagaagagggaaaaatgcctcaattgtaccaatggtgagaaaacacccaaagtacaaagcaggtttcaaaaaaaccatactcataaccaaggacaataataaagcaatgtgttgacatatactctataagtcttcctccataaatagtttatagaaattttgtaatttctgtaaatgcatcctataataattttgcatcttgctttttttttacatttaatatcaagtagatttctaaagggcaattatttgaaaattatcccaaatacatggggaaatatacatcaagtgaaaaaatgcagtgggtgatagagatatcaggaagcgcctcaaatatttctcatctcgttggagaaaaacaaacatgttctcatttagaatgagtgggagttacctaattgatttaggcctctatatttaacttctagtcaaaaaaggtagttctatctagcaacaatattatggggaacaaaagaaaaaattaactctctaaatttgcagtagggtcttttcttcagaagtaccaaatcccatctattaccagctccatgcttcaggcctaaaatggatctccctgaagcaatgacagaatttttgccaagtgactaggatataaacaccactttggttgcacagtgagacatatgctccaaagaaaactggttcaaaaacaggcaagtgggtttctacagaataaatgagagccctgtcaatggcttcatcttcagggctttgtgtctgtgcttgcgtggtggctcttgtttcatctatggataatggtggcacacagttttcataattccttacattaatgaactgctataaatttgtttttggtattctagagagtcctaacttcagcttctgggcaatgctgaggaggcaccctatattctagacttaccttttgcaaggtgtactctcagcattgtgggcgatttccatgggagaatattctatttaaagaactactgtcccagcataaaacaaaaaatcatttatgaagatgcaggagactcggaaagctctcaattattgtttgcacaagcacaatgtcacagcctcctttccccattccacaagggggtcaggaagagagtactcagctgtgagaaaagacatacagaagaattcatgtggtcatgagagcgaggacatggccgatcccccaaggaggatgtgtcatacacttcatgagcccaagagtgtgctgtagggtctgaagggcaagatgctggttcactgatgtaaaggagagggaaaaaagcttcaaccaactagaaaaacagtctctatgcatgctatttttgattttaaacacaggtatcaattccttctctcagagagtccattttaaaataggatacatttttaaaggaatatttaaaggacacattcattaaaatttattttaaaaacttttcaaaagaaacaaaaggtatgaattttatttaatccttgaggaaatggttcttttctcacacacataaatcactcattttgtttttctttatctcctttattaatctacattagaaaaataaacttttcatacactaagaacaaggaaaccactctcaattgacaaaatgttccaatccaacacaatgattactttcacctttaatttacaggcagccagattcaaaatccttaaagttgcttaaacttaaaaatgacaatgacaacctaaaaggtataatgttgattggaacagacatttaattggaaaattgatgattttccatttccaattaaatctctagatagaaatgaaaaaaattaaaaatcgtatttaagaaaagccaaatcttgggttgtgaggtatctttttaaggatgtttcagcagaaaaaaacaaaggctctcacaattgtgtagctgcctagattaagtgggtatcctgatcaaggagatgggggatgatttggctttagtattccaatgataaagtttataatgagaataacatgttgctacaaaatccagtctcttcctcagatgccttccacagagggcaggaagctttgtcagttttgtttgctgatgatgcctggttccgtcaacaaataacacctgataggcctggatcaagcatgcagctgtggagaacacccctgggactctaactctggcactctgcaagctgggtacttgggcaggacagcagcagcactcatgaactgggcagcacctgttggtgagggctgatcacatggattctctcatcccagccttacaatcagtccttcaggtacatactttttctgactttgctgatgaggaaactatgcacagaggttacacagcttaacaaagggttctcacctaatgaacaatgaaatgggattttagcctttctttgcatctggtcttagagccaatacccaagaagcactgtactgtatgcattgtctcagagaaacttactcttcctgggcctcagtctttaaaaggtgggcagttgacttaataagaattaaagatcaatgattaaggttcaaggcactccaaaattctggtctttattgaaaaggctacagaagtctcaccttaataataccctatagacttgatattcttggttaattaaatattggaaaccaatttcatagtaattgaggtcagaaaaaagtactcatgacattttagaatatgatgacaaagccatagataaatttcaatgcacctgtaattacttaaaactgttatagcatgcaatgtgttaccacaacagccagagaaatactaatttactcagcctattcttctagaccagtaaacactaggattaaatagatattttcattgaatttgttctacccttcattgccatttatagatagcttacttgtcatagattactttctaattgttttatgtttcctaactagcctgcaatactttggcaaggacctcaaacaatagtagacagtaggtgtaaaatagatggctacattgaacagatgactaaaaggatgcctcctaagtacctatatcttgaaatatatattattgtgccttgctttcaatttgtgattttaaaatctagaaatcacctgttttatgtaataacaataaaatccttctttgttgaaaacatgcacaaataaagtttacaagctcaaaaaattaaacagcagtaacggtcaagctttccaacaataaaatacattttggtaaggttttcattttacaaaaactcaaaatagctttatgagttcacaaaataatatgatatttttcaagatattaacatattcttataccggaagagcatagaataaaatttacttggagattgagcatttgcttctttaagaaatacttcttttagtatttttactttaatattatgaaagctacataattacattcagattcattaactactccagtagttaatttttaaaacttatgatgaatagttttgtttaaaatatataacattggtaatatgcaaatctgaatctgtaataaagaaggatttgcattcctgatttttttttctgatacaaccaatgacaaaataactaatggttccacagaggataaaatgtctcaaatctgttggttctgaaggtgaagcgagatttttgtactgataccgtgtatcactgagataccaggaggaaatggaattaaactcagatagttcaaatggagagattttaatgaagggacgacctacagaggtgtcggcagggttggggggaatcagcgagatatgcttagaacccaccgactggcaaacctccccctgaagatggagaaggaggaaggagtgttactggaatgagagcttgagtccaggggaggaggatgggctgctgaggaggcgacaccatcctgaaagaagaatcctctgccagaggcttttcagggtcatttcttcacactctctgcagggaagcacggagacagcaggaagaaatatcctaacctcactctcttccctctacaggtgcttccattggccaaatccacccagaggccagttggtggcgatcagctctcttcaagtggtatttaaatttcttctttcattttccttctggtaacaaagaagtctgtggctcaaaagatgtttctctaagaccccatcctattaggtctctgagctgagggccgacgagtgggggcgggcaggagggccgagggaggcggaacaggatcgaggcgcgaggcgggagtcgagaaagcgagcggccgaggcgactctcagtgcgcggacgcgggcgcgcgcccgcgctcccttcgtcgactcacggcgagagcccaaccctgctgccgcgcgccacccgcctcgccgcgcct

SEQ ID NO: 17583 - RNA, 15601 nt, Homo sapiens
  source 1..15601: mol_type = other RNA
tcaggccaggcacagtggctcatgcctgtagtcccagcactttgggaggccgaggtgggcagatccacgaggtcaggagatcaagaccatcctaacatggtaaaaccccatctctactaacaatacaaaaaattagtcaggtgtggtggcacgtgcctgtagtcccagctactcaggaggctgaggcaggagaatcgcttgaacctgggaggcggaggttgcagtgagccgagattgtgccactgcaccctagcctaggcaacagagcaagactctgtctcaaaaaaaataaaaaaaaaaaaaagagagaaagagagagagagatgaggagttgctgcactgctgggtgtggagagccgaggaggattcaaagatggtcctgaagtcccagctggaagaagtaggcggcagcaatgtttttaatactgtaaattcatcacgtagcacaggtttggggtggagaaagaaaaattgcattggcttcagggcatgcccagatctttcctcatcttaggcgtttgctaatacatgcattttctaagctgatgtcttgcgtttaatcactgctccattcaaaagagagaaggaggttgtttcaaacctagttgatatcatttgacttccatgctattcacagggctattttatttgaaacaggtataccacagccttaaattgcaagttaatccaggatgttcctaggttggcagttaggaacatgtaattctttggaagggctaaaagtcagctctttaaattatctccatatgaaccttctctccaccttagggtggatccacttatttagtccactgccagtaccacactagaacccgggtggtcactggactccagaaacaacagtagccctctctctgttctgtctctttttgactatctctattctgttcctgaccctgatttctcctgccaagctcaattttgacagctgacaacggcaagccatggcttcccaaaacattattttcaggtcaacttataaatttcaagaacacatttggctccgcttcctgtggtactaagcctacttcttgacagcatttgcctttgttgtaaatagcaaagttcttctagttggatttttgctaagaagtgtgtggatgtggcatgtgacgacatctttagcttggattctagaaaggcactaccattgtgcatttggctaaaggaaacacattttacccgtgaatgccttctatttacaaatgctcagctagcacacaaagctaagtacaagcaataagtactatcctacaatgttactcatttctgaaagcacaaaatgatgactggtatagctttggagatgttttctggaaacccaataaaggaacagatctttgttattccacacctacaaagtcagaagatgcacagtcttttattcatgtttgaacaagcttccttcttgaacaatcaactataaagtgatgtgattctctactagaccaggaactccttgaggacagaatgagggtctaatccatattctaaatccacaccacctggcacaatacatgttgcatggttagggtcaactaagagttggttgaattaatcaataacacacagcaagagaattcacaaagagaggggagtaatcccccagcctcaatcactcggcaagtggaatcgctgggcactgattccagctctgtctcagtgcttgagacagagctgaatgtaatgtgaacatttcaaatgaacaggaaaactagactcacggataagcagtgtagtcatcaagacaacactgtcttggaggtttttctgaagttaaaaccatgctacataagcaataaattatgaaggctgagcatgtgaataaaatttaatgttgtcataaattttataacaaagttaatctgacacatttaatgacatgcataatcattagtatgcagcactgtaatcagacattgataataagcagttcacaccagtgactgtaagagtctttacttgtgttcagccaagccaactgcttggtatatttttctcccttcttagtcgttagttttccatacctacaataactatcagtggtgatgggcttctctgaccatgtgaataatttaatcctcaatgcacagatacagaaacccttgctgaagacagtgtggagcagagaaggctgtctccactccttccacctgaaacacctctgcagatggatatgggagctctgcctacagcccttggacctaaccacttcagtgtgttccagtgagtgtctggacctcggcctgaaagatttttccgaaactaaagaaaatttctctgacctaaagaccttaacctccaccccagaagctctcaccaaggactacagggaactggtggggaaaatccttatcccttactcctcaaggcacagggcagtaatgctgaggcttgtgcgccacacttgctcccagaggtccccagcgggctacctgcggtggtgaatgacctcctaacacgccccttgacggccttcctttccttgcctcacttctccactctcctaccagcattgcagggttcacatcccaaatataccactggcacttgaatcctggtctccaggtctgtttctggaaaaacccaagtaagacattgccccagtaatggggctagatgtctgaggcttcctcaagtatctacctcgaaagctcttactgctgtacacacatgcacatacacacacgtgcgtacaaccagtcacatctaagcaccccgaataccagcctgttgaaggtagcagagagctgcactataagccaaggctgctcccaagagccgctccatcactgaattggcgccccagcaagatgaaggaatgtaatcattggaaggatggagaatgttctctgaatcactgacaaattggaaggggtggagggcaagagtccacctggtggagagatggaaagagcgagagagcctggaatgataatgccattgcttagaaaaggctgctccagatgccatatctacagaaattgtacagcccaaacatctctgagcaataggtctctggtagtcttgatgtctagaccaacaattcccagttcattcttctcagggaaggagccaggatagtccagagactctcattctgctgttagattgaaagggttaggcacaacagccttggcaaagtcacaagggcaaattcacactaaagtgtaaatgacccacaactcctcttctatttttaggttggggaggtgctttagaacataaggaggaactaaagaatattcctgttacatacaaggcagagaaaagggaaactagtggtgacaagacaaatcatccctttgacatttggctggctctacctattacagctctgggggtgaggtgggaacaaaaagatgctgtgtaaagaagtatcttatgccatccctactgtagtgaggtgcagtttagaggggacactgatcaagcagagacccagagtgtttcgttccaagccagaaacagaaatgtataaaacacagcctttccagcatcagaaatgagtagtggtagtggagaactacccaaaacaggaaagaggaccacgtgaggtagagtgtcaaggccctacattccagtgcctctgctcatgactgtaattttgggtaggtcacttaaagtctctggacctcagttttgccatctgtgaaatagggataatactatccagcataaaattggttatgaggctcatgtagggcctgcctgggatgatgtgttgctaatggttaagaacacaacttctggggtctgactggacaggctgaaatccctgcttaacacgttccagcagagccctgggcgatctatttaacttttgttttctcacctgtaagctgagacgaaagtacccactttataagattattccaataattagttgaaataatgcatgcagagaattaagcatggtacttgttatttgttaaactagctattaaaatgtgtaaaatataaagtattgtatggattttaggacaatgcaaagactctttgcttgctgcaatagttcggggccctttcagatggctaaaggcagaatttgtatgtgtaaatatggtgtgcttgtctctgctctggatactgagggcttaccctgttattaaacttatttagtaaatattgaactgtcatgaggcctaacatttagttccagttattagataaaacatttgctttgaatggtatttgaattgccaggttctagattattctggttgacaaactcttcgtattttataaagaggctaaaattggtaagctatcacagaacagatgtgccattttcaaggtatattaaaccatgattcactgtaacattgttcctactggcaacaaattcagagcaggctggactttatttggtgaagaaacattgagtggaagagaaatgacattattttatgtatttacattttcaaattactgtggcttaaacctgttcagccaacattacccaccttcagtctgctaaataaatgattcagtacatttctaatttacagaattttttaacaaaagaaaatgtaatttgatagccaaatcaacgttaaacattatacatttaaaaaaccacaggcaaagacacaaacatgatgacactaacttttgttaaagtatgcttacctatggtttcctctgaggcacgttctttcatgctaagcttccaacataatatgaaaatgaaggagatgcattttgcaaagcaaaacagaccttaagcaaaatattatacttctcaaattaacactgttacaaagttttagaatttaataagttcattaatttaaaagtttggatgtctgagtccttctatcccaaaacaagatcttggagggtcttccacagccatgtaataccatggtcacatgaccctttccaaaattattaatctgaatttactatatgaggataaatctatctttttgaaaatatttaggaaaatgagcttggtatttataaaatgaagctctctttgggtggtatcctaagacacgtcaagccaatcagcctgtaactgtgaaaaaaacattggtaggtacaaaagtggggtgggagaggagtgacttaactttgttaagtgatgggaaagaaacactaatagcattatctcaataaaatgtgatttaaaaaaatttaaaatactaaatcattgaactgacaaagaaatataaatcattcagaaataaactcattaggtcatcaaatcctgttaaatctgcaattaggaagagcaaggtgtacaatccatacatttaaactcacaggctcactttgcacaacgtcaatttactccttaatatgttattaatacgcattttccaaaaggatgtattagtaaatggtacacatctacttcttggcaacatcatataacctggtacaacataagcattcttcttatagttaagaaatgtggatggtatcaaaattagaaaaataaatgccctattatgttgtggtcaggtttaaggcatgtgaattttatcttcatacaaaagattaaaatctagatattaaaaagtagtgcagtatcagtgatgctgcctcagttcccaaaatgtcacatcacaaaaatatcccataattgcctgtagtttattccttggctttcctcttttctctctgcatctttgtaacaattttttaaaagtggaaatataattgttggcaatgctaacagctgtagaaatgattacaagatgtggaaaagcataacaggaatgtcaagaatctgtttctggcagtaatatatatggaacattgttcaggacaaaagaggagaaggaagaaaaaaaggagaggggtttatcatctctaagaattttcaaactaaacctcattgcttaataggaaaaaaagattccatatttaaagttaagtcacctctaactactagctaaagcatgacatcaccagcactggagtcagcggaagtgtgtttttgaaggacagtgttgcaggagaatctggacaggttttagagccaggagagagaaaataattctacctctgacagttgaaggaccttaggcaaatcagtttacctctgctagactacactccaaaatttggacattcaaaaatttgatattaataaccacatgaaagtctcgtgttgaggtgaatatgtatttgttggtgaaagatatgttggtttttaaacagacagcactctgcaattgtaggctattgttttgttttgccagttgtcaaattctatccagctatacacacttgtgtggcctcctaatggtgtttttccagtggctaaaggtttatgaataagacacttttcctaatggaattaacccgatgcttttcttaaacatgtaaccttgagttcaccgcaaaaaacaatgcttcgattagagcaatgcatataataaaggttaccctcgtttcttagacactagacatcattcacaaaaagagaactgcttttgaaagggatgtatttgcactggaaagaatagttttctacttctaattataaatgatttattggtgaaagcaaaacaacagcctgtctgagaggcacttctatgagcatcctcacgtgtgatttgcaaggttgaagaagagggaaaaatgcctcaattgtaccaatggtgagaaaacacccaaagtacaaagcaggtttcaaaaaaaccatactcataaccaaggacaataataaagcaatgtgttgacatatactctataagtcttcctccataaatagtttatagaaattttgtaatttctgtaaatgcatcctataataattttgcatcttgctttttttttacatttaatatcaagtagatttctaaagggcaattatttgaaaattatcccaaatacatggggaaatatacatcaagtgaaaaaatgcagtgggtgatagagatatcaggaagcgcctcaaatatttctcatctcgttggagaaaaacaaacatgttctcatttagaatgagtgggagttacctaattgatttaggcctctatatttaacttctagtcaaaaaaggtagttctatctagcaacaatattatggggaacaaaagaaaaaattaactctctaaatttgcagtagggtcttttcttcagaagtaccaaatcccatctattaccagctccatgcttcaggcctaaaatggatctccctgaagcaatgacagaatttttgccaagtgactaggatataaacaccactttggttgcacagtgagacatatgctccaaagaaaactggttcaaaaacaggcaagtgggtttctacagaataaatgagagccctgtcaatggcttcatcttcagggctttgtgtctgtgcttgcgtggtggctcttgtttcatctatggataatggtggcacacagttttcataattccttacattaatgaactgctataaatttgtttttggtattctagagagtcctaacttcagcttctgggcaatgctgaggaggcaccctatattctagacttaccttttgcaaggtgtactctcagcattgtgggcgatttccatgggagaatattctatttaaagaactactgtcccagcataaaacaaaaaatcatttatgaagatgcaggagactcggaaagctctcaattattgtttgcacaagcacaatgtcacagcctcctttccccattccacaagggggtcaggaagagagtactcagctgtgagaaaagacatacagaagaattcatgtggtcatgagagcgaggacatggccgatcccccaaggaggatgtgtcatacacttcatgagcccaagagtgtgctgtagggtctgaagggcaagatgctggttcactgatgtaaaggagagggaaaaaagcttcaaccaactagaaaaacagtctctatgcatgctatttttgattttaaacacaggtatcaattccttctctcagagagtccattttaaaataggatacatttttaaaggaatatttaaaggacacattcattaaaatttattttaaaaacttttcaaaagaaacaaaaggtatgaattttatttaatccttgaggaaatggttcttttctcacacacataaatcactcattttgtttttctttatctcctttattaatctacattagaaaaataaacttttcatacactaagaacaaggaaaccactctcaattgacaaaatgttccaatccaacacaatgattactttcacctttaatttacaggcagccagattcaaaatccttaaagttgcttaaacttaaaaatgacaatgacaacctaaaaggtataatgttgattggaacagacatttaattggaaaattgatgattttccatttccaattaaatctctagatagaaatgaaaaaaattaaaaatcgtatttaagaaaagccaaatcttgggttgtgaggtatctttttaaggatgtttcagcagaaaaaaacaaaggctctcacaattgtgtagctgcctagattaagtgggtatcctgatcaaggagatgggggatgatttggctttagtattccaatgataaagtttataatgagaataacatgttgctacaaaatccagtctcttcctcagatgccttccacagagggcaggaagctttgtcagttttgtttgctgatgatgcctggttccgtcaacaaataacacctgataggcctggatcaagcatgcagctgtggagaacacccctgggactctaactctggcactctgcaagctgggtacttgggcaggacagcagcagcactcatgaactgggcagcacctgttggtgagggctgatcacatggattctctcatcccagccttacaatcagtccttcaggtacatactttttctgactttgctgatgaggaaactatgcacagaggttacacagcttaacaaagggttctcacctaatgaacaatgaaatgggattttagcctttctttgcatctggtcttagagccaatacccaagaagcactgtactgtatgcattgtctcagagaaacttactcttcctgggcctcagtctttaaaaggtgggcagttgacttaataagaattaaagatcaatgattaaggttcaaggcactccaaaattctggtctttattgaaaaggctacagaagtctcaccttaataataccctatagacttgatattcttggttaattaaatattggaaaccaatttcatagtaattgaggtcagaaaaaagtactcatgacattttagaatatgatgacaaagccatagataaatttcaatgcacctgtaattacttaaaactgttatagcatgcaatgtgttaccacaacagccagagaaatactaatttactcagcctattcttctagaccagtaaacactaggattaaatagatattttcattgaatttgttctacccttcattgccatttatagatagcttacttgtcatagattactttctaattgttttatgtttcctaactagcctgcaatactttggcaaggacctcaaacaatagtagacagtaggtgtaaaatagatggctacattgaacagatgactaaaaggatgcctcctaagtacctatatcttgaaatatatattattgtgccttgctttcaatttgtgattttaaaatctagaaatcacctgttttatgtaataacaataaaatccttctttgttgaaaacatgcacaaataaagtttacaagctcaaaaaattaaacagcagtaacggtcaagctttccaacaataaaatacattttggtaaggttttcattttacaaaaactcaaaatagctttatgagttcacaaaataatatgatatttttcaagatattaacatattcttataccggaagagcatagaataaaatttacttggagattgagcatttgcttctttaagaaatacttcttttagtatttttactttaatattatgaaagctacataattacattcagattcattaactactccagtagttaatttttaaaacttatgatgaatagttttgtttaaaatatataacattggtaatatgcaaatctgaatctgtaataaagaaggatttgcattcctgatttttttttctgatacaaccaatgacaaaataactaatggttccacagaggataaaatgtctcaaatctgttggttctgaaggtgaagcgagatttttgtactgataccgtgtatcactgagataccaggaggaaatggaattaaactcagatagttcaaatggagagattttaatgaagggacgacctacagaggtgtcggcagggttggggggaatcagcgagatatgcttagaacccaccgactggcaaacctccccctgaagatggagaaggaggaaggagtgttactggaatgagagcttgagtccaggggaggaggatgggctgctgaggaggcgacaccatcctgaaagaagaatcctctgccagaggcttttcagggtcatttcttcacactctctgcagggaagcacggagacagcaggaagaaatatcctaacctcactctcttccctctacaggtgcttccattggccaaatccacccagaggccagttggtggcgatcagctctcttcaagtggtatttaaatttcttctttcattttccttctggtaacaaagaagtctgtggctcaaaagatgtttctctaagaccccatcctattaggtctctgagctgtgggaagtatttatacaattgcttgtgaatataagatccaggaatttccctaagatccctaacaaaattggtgataagtagtcccacatgttaatccagccacccacggatgacagcacttaccatttctttgataaatgtcaaatgcatttgaagtacctacctgaaatatttgtttaaatgctatctaatctattaattttatatatgtgtgagtctgttttgtataccttctgattataggataaatgtaaataaatccaaagagtaatcaaagctaccactttcaagaagccttctttgtagaaccggaagagtcttaaataggcttttcaggtatgcatctcttattatcgctgaactccaagtcctgcaaggcaggcatcatgtgtgggtcacctttacagtaggcacaggccttaaaacagtgacatgcacattgcaggcactccataaatgtttgctgaattggctaaaccttggtttgttcccataatcaaccaccacaaacagcacacagataattacttcttggaaagattccaactagtgtttgatgttacctacgtggtttttctctcaagatcttaagagcagctctgtaggattacattattttctgttttttttttcctttgaccttaatgtcatctacttcaataacagcttcatacaaaattcctaccagcacataccacagcagattcaaggccttgttttaaaaatggtgccagcttctcttaatttggaagatatattgtctctcctgaacatgggctaagaaaatgtataatttggtattaacataagagctgaagacactttaaatgcattgtttcatttttataagataaaaaaaattttaagaatcaaaatgttatcaacagacttgtccttcattaaaaagtaaaactgcatttgcctacattttatgaaagtgtccaattatgaacaattttgaaatgtaacttttaaaaatgtaaacagcaaaaatgttgtatttaaaataaatctggaaaggcagaaaaacaaaaaatacccagaagacagagtttttggtgaaagttaagatatttcatctttgaacaacttagaatctttcctgcattttatagtctagttccaggcattaatttgaaataaccttggaatcctaaatctaacacccttcggaacaaagtagcttttctcttctgctttatgagcaaatggactaaatactagggaatggtactgtctgggcctttgaaccaagattgaaagagatgaaatcctatatgatatgtataaacattagagaatccattttgatttaataaaaggttgaatttgttctatatcctgtgagaaaatggttcccttttcctgaaaatgttacctcattccaacaatagaaagttggtttttttccagggtgtggtgttggcgggggacagagttgccatgaatatggcatctatgaagactgctgttatattcatttctcaaaatgcactgtggtaggaaattcagaacgcagtgagagaaaataaatgtttgacttcaaaatataaggccgcatttaaagcagaaggtaaagtatagaacagttgacagtataaattctttatctgcaatcttgcagttccctaaatctctgtaacacatcacttttaaaagcctcagataagtggttctataataatttaccaataattcaacccctcaaaagtcttagcaagttaaaccttataatcttacattttagaaatgacccaacttgatccttttattcttcagaatatctctctcaaattttcatttgtttttcattaattgatgaataatgagacattttaggtacctgtccacaaagaaatgaaattttcactttccaggaacctaacaaatgaaaagatagaaatcaattccaacagaatattaccaaagaaatcttttagaatggactgttaaaattatttatttgtatttatctggctctactatttgtggtacatttccacttcaaagctaaacctcaaataacatcatagtgagtggttgacttcatgtttaactgagatcttgaagactgaaaaagaccacgacaaacacacatctattttcttggctactgcatccgtgttcatcaccattctgatagtctgcaatgtattgcagctcaccctttgggaaggactaaagtagacatctgtttgttctgcttactcagcattcctaccctaattttcctttggagaacccctttattctagaccacgtgaagctaatgccaaaccccattccaggggatgcacctgaatccaacctccatcatctaaacagtgccttctccacgttcagagaagagcaagtgactcaaactgccctcataagaacagacctgggacttctgctgcaaatattgaagagtaagtactcttttttcttgctaggactaagctggtagtaccttctatgaggctatcatatggaaacaacttgtctgaaaatgaagccacaactagaaaacagatcctggtaacccggattgatggatccagccctaccttaaatggcaagacctaacccgaggctttttgcatcaaccaataaagtccttaagccagtttgagttggttttgtcacttgcagctaaaagaattctgactctaacaatgtgacaatagcaaaaataaacataactgcttttgaggtttctaatggattttcctccctatatacatgatttcatttaatcctcacaattcaggaaagcacatatctattaacattaaattaatattcattattttgaacacatgctatgtggataagggatgaggaaagccaaggaagtaatcaacgtgaaatctcacttatatgggagggaagtggaggttacatatctcagggcacttaacagatatcatcaaatgaaagaataaacagtgtgtgggagaggcagtaggtgattcttcatcaattcctggatgaaaaattaggagataatgaactccgaacaggcagcctaatgagaatggctcaagcaacaggacatagagagggagttaggttagacatggggttcttgggaattttcacctcgtgggggggcgggggggtcgtgcagctgttgtcagtgggaaagggaaaaaggaaaaggctgagtttggaaggcagggagggaggagacaatgtgagtcagtgaaaaagggcccttagaatgacaagtctggaccagagagaggctaagactgaaaatacaagttgggtaaccactggcatacagatggcagttcaggcttgggcactgcccaccagagcctcagcatgaagagaagagggggaggctggccaccacctccctctaggtaatcgtcatcctgatgctgagctcctgaaaacaggctctttcactcgccccatctcttgctcttgattgcaacccggcattcaggaggcaccctgtaatatctgtggagtgaccgacaacacagcgccagggcactgagaagatcccagggcgccagggactggttctacaagggtgcccctcccggtcccctccagcgcgccgccagagctgccagtcttggctgctacacgggaggcagcctcattatgcagctctcacctcttaaattagttcatgctctcacattaggtgtaatcacagcttgcaacgctttctggggatgtctcagaaagatctgagttgaaaaaatatttttgtgtcattttaatttaaagtaaaattgctgcttcttccccgcccctttctttcctcctggcccacccagcgaccctggccggccgtgctcaacgggggcgggggtcggaggtgagatttcctccacataattccttaaacagctatcaactaagtctcaaagaaaaaaaaaagagatctagaagcagagacgtggctgctggcgatcccaaagctggtgttcgctcttgggggagagcgtaccctgggggaggccgggaggccgggccagaggctagcccagaggcagagggcaggagcgctcagccggcgccccgcgtctctccagctcccgacgctgcgctggctccgctgagcacgccaggatcaaggtcgcctggtggggaccggagcgccaggagcctgtgggaagcgttccagccggcctctgactgggatccggcgccgcgtttctgctttggacttgactgacaggtccccccgccctcccgccgccctactaccagcctgggttcatccttcagggctacgtctaccgcacccgggctggaaagcctggagcgcgcccttcctctcctcatcttctcagctctcctttctccctgccacttggcaaagctgcattttgactttcacgttttggactacgtgtgtgtagttccaagtccatgcgtggcacgaaaatccacttagggtaaaaattattctcgaaaaatcgcccatctcaggatctggtgtctacactcaaggctaggaggtgcaggtacgggtgcgtaaagcatgccgtaagggtgcacagtaaataaaaagtacggatgcaaaatgtaaattttaagtgcaaaacagaaaagcagtactcgttgccgccccgcacgctgggttttaaggggcacgaaggtgggcctcggctgcttttgctcagccccgcgtcctcagcgcccggcccagtacccggtactccgtaggggttcaatgatctcccctgaataagtgaacgaattaacaaatgaatgaatgaccgctcgatccgacctccgcggccggcagagcagtcgctggagaggcgggagagagcgagaggccaagctccaccatcgcggccgccggctggggcagagggacacggagacactcggcgccccggctccgcaccgagtccccg

SEQ ID NO: 17584 - RNA, 12172 nt, Homo sapiens
  source 1..12172: mol_type = other RNA
tcaggccaggcacagtggctcatgcctgtagtcccagcactttgggaggccgaggtgggcagatccacgaggtcaggagatcaagaccatcctaacatggtaaaaccccatctctactaacaatacaaaaaattagtcaggtgtggtggcacgtgcctgtagtcccagctactcaggaggctgaggcaggagaatcgcttgaacctgggaggcggaggttgcagtgagccgagattgtgccactgcaccctagcctaggcaacagagcaagactctgtctcaaaaaaaataaaaaaaaaaaaaagagagaaagagagagagagatgaggagttgctgcactgctgggtgtggagagccgaggaggattcaaagatggtcctgaagtcccagctggaagaagtaggcggcagcaatgtttttaatactgtaaattcatcacgtagcacaggtttggggtggagaaagaaaaattgcattggcttcagggcatgcccagatctttcctcatcttaggcgtttgctaatacatgcattttctaagctgatgtcttgcgtttaatcactgctccattcaaaagagagaaggaggttgtttcaaacctagttgatatcatttgacttccatgctattcacagggctattttatttgaaacaggtataccacagccttaaattgcaagttaatccaggatgttcctaggttggcagttaggaacatgtaattctttggaagggctaaaagtcagctctttaaattatctccatatgaaccttctctccaccttagggtggatccacttatttagtccactgccagtaccacactagaacccgggtggtcactggactccagaaacaacagtagccctctctctgttctgtctctttttgactatctctattctgttcctgaccctgatttctcctgccaagctcaattttgacagctgacaacggcaagccatggcttcccaaaacattattttcaggtcaacttataaatttcaagaacacatttggctccgcttcctgtggtactaagcctacttcttgacagcatttgcctttgttgtaaatagcaaagttcttctagttggatttttgctaagaagtgtgtggatgtggcatgtgacgacatctttagcttggattctagaaaggcactaccattgtgcatttggctaaaggaaacacattttacccgtgaatgccttctatttacaaatgctcagctagcacacaaagctaagtacaagcaataagtactatcctacaatgttactcatttctgaaagcacaaaatgatgactggtatagctttggagatgttttctggaaacccaataaaggaacagatctttgttattccacacctacaaagtcagaagatgcacagtcttttattcatgtttgaacaagcttccttcttgaacaatcaactataaagtgatgtgattctctactagaccaggaactccttgaggacagaatgagggtctaatccatattctaaatccacaccacctggcacaatacatgttgcatggttagggtcaactaagagttggttgaattaatcaataacacacagcaagagaattcacaaagagaggggagtaatcccccagcctcaatcactcggcaagtggaatcgctgggcactgattccagctctgtctcagtgcttgagacagagctgaatgtaatgtgaacatttcaaatgaacaggaaaactagactcacggataagcagtgtagtcatcaagacaacactgtcttggaggtttttctgaagttaaaaccatgctacataagcaataaattatgaaggctgagcatgtgaataaaatttaatgttgtcataaattttataacaaagttaatctgacacatttaatgacatgcataatcattagtatgcagcactgtaatcagacattgataataagcagttcacaccagtgactgtaagagtctttacttgtgttcagccaagccaactgcttggtatatttttctcccttcttagtcgttagttttccatacctacaataactatcagtggtgatgggcttctctgaccatgtgaataatttaatcctcaatgcacagatacagaaacccttgctgaagacagtgtggagcagagaaggctgtctccactccttccacctgaaacacctctgcagatggatatgggagctctgcctacagcccttggacctaaccacttcagtgtgttccagtgagtgtctggacctcggcctgaaagatttttccgaaactaaagaaaatttctctgacctaaagaccttaacctccaccccagaagctctcaccaaggactacagggaactggtggggaaaatccttatcccttactcctcaaggcacagggcagtaatgctgaggcttgtgcgccacacttgctcccagaggtccccagcgggctacctgcggtggtgaatgacctcctaacacgccccttgacggccttcctttccttgcctcacttctccactctcctaccagcattgcagggttcacatcccaaatataccactggcacttgaatcctggtctccaggtctgtttctggaaaaacccaagtaagacattgccccagtaatggggctagatgtctgaggcttcctcaagtatctacctcgaaagctcttactgctgtacacacatgcacatacacacacgtgcgtacaaccagtcacatctaagcaccccgaataccagcctgttgaaggtagcagagagctgcactataagccaaggctgctcccaagagccgctccatcactgaattggcgccccagcaagatgaaggaatgtaatcattggaaggatggagaatgttctctgaatcactgacaaattggaaggggtggagggcaagagtccacctggtggagagatggaaagagcgagagagcctggaatgataatgccattgcttagaaaaggctgctccagatgccatatctacagaaattgtacagcccaaacatctctgagcaataggtctctggtagtcttgatgtctagaccaacaattcccagttcattcttctcagggaaggagccaggatagtccagagactctcattctgctgttagattgaaagggttaggcacaacagccttggcaaagtcacaagggcaaattcacactaaagtgtaaatgacccacaactcctcttctatttttaggttggggaggtgctttagaacataaggaggaactaaagaatattcctgttacatacaaggcagagaaaagggaaactagtggtgacaagacaaatcatccctttgacatttggctggctctacctattacagctctgggggtgaggtgggaacaaaaagatgctgtgtaaagaagtatcttatgccatccctactgtagtgaggtgcagtttagaggggacactgatcaagcagagacccagagtgtttcgttccaagccagaaacagaaatgtataaaacacagcctttccagcatcagaaatgagtagtggtagtggagaactacccaaaacaggaaagaggaccacgtgaggtagagtgtcaaggccctacattccagtgcctctgctcatgactgtaattttgggtaggtcacttaaagtctctggacctcagttttgccatctgtgaaatagggataatactatccagcataaaattggttatgaggctcatgtagggcctgcctgggatgatgtgttgctaatggttaagaacacaacttctggggtctgactggacaggctgaaatccctgcttaacacgttccagcagagccctgggcgatctatttaacttttgttttctcacctgtaagctgagacgaaagtacccactttataagattattccaataattagttgaaataatgcatgcagagaattaagcatggtacttgttatttgttaaactagctattaaaatgtgtaaaatataaagtattgtatggattttaggacaatgcaaagactctttgcttgctgcaatagttcggggccctttcagatggctaaaggcagaatttgtatgtgtaaatatggtgtgcttgtctctgctctggatactgagggcttaccctgttattaaacttatttagtaaatattgaactgtcatgaggcctaacatttagttccagttattagataaaacatttgctttgaatggtatttgaattgccaggttctagattattctggttgacaaactcttcgtattttataaagaggctaaaattggtaagctatcacagaacagatgtgccattttcaaggtatattaaaccatgattcactgtaacattgttcctactggcaacaaattcagagcaggctggactttatttggtgaagaaacattgagtggaagagaaatgacattattttatgtatttacattttcaaattactgtggcttaaacctgttcagccaacattacccaccttcagtctgctaaataaatgattcagtacatttctaatttacagaattttttaacaaaagaaaatgtaatttgatagccaaatcaacgttaaacattatacatttaaaaaaccacaggcaaagacacaaacatgatgacactaacttttgttaaagtatgcttacctatggtttcctctgaggcacgttctttcatgctaagcttccaacataatatgaaaatgaaggagatgcattttgcaaagcaaaacagaccttaagcaaaatattatacttctcaaattaacactgttacaaagttttagaatttaataagttcattaatttaaaagtttggatgtctgagtccttctatcccaaaacaagatcttggagggtcttccacagccatgtaataccatggtcacatgaccctttccaaaattattaatctgaatttactatatgaggataaatctatctttttgaaaatatttaggaaaatgagcttggtatttataaaatgaagctctctttgggtggtatcctaagacacgtcaagccaatcagcctgtaactgtgaaaaaaacattggtaggtacaaaagtggggtgggagaggagtgacttaactttgttaagtgatgggaaagaaacactaatagcattatctcaataaaatgtgatttaaaaaaatttaaaatactaaatcattgaactgacaaagaaatataaatcattcagaaataaactcattaggtcatcaaatcctgttaaatctgcaattaggaagagcaaggtgtacaatccatacatttaaactcacaggctcactttgcacaacgtcaatttactccttaatatgttattaatacgcattttccaaaaggatgtattagtaaatggtacacatctacttcttggcaacatcatataacctggtacaacataagcattcttcttatagttaagaaatgtggatggtatcaaaattagaaaaataaatgccctattatgttgtggtcaggtttaaggcatgtgaattttatcttcatacaaaagattaaaatctagatattaaaaagtagtgcagtatcagtgatgctgcctcagttcccaaaatgtcacatcacaaaaatatcccataattgcctgtagtttattccttggctttcctcttttctctctgcatctttgtaacaattttttaaaagtggaaatataattgttggcaatgctaacagctgtagaaatgattacaagatgtggaaaagcataacaggaatgtcaagaatctgtttctggcagtaatatatatggaacattgttcaggacaaaagaggagaaggaagaaaaaaaggagaggggtttatcatctctaagaattttcaaactaaacctcattgcttaataggaaaaaaagattccatatttaaagttaagtcacctctaactactagctaaagcatgacatcaccagcactggagtcagcggaagtgtgtttttgaaggacagtgttgcaggagaatctggacaggttttagagccaggagagagaaaataattctacctctgacagttgaaggaccttaggcaaatcagtttacctctgctagactacactccaaaatttggacattcaaaaatttgatattaataaccacatgaaagtctcgtgttgaggtgaatatgtatttgttggtgaaagatatgttggtttttaaacagacagcactctgcaattgtaggctattgttttgttttgccagttgtcaaattctatccagctatacacacttgtgtggcctcctaatggtgtttttccagtggctaaaggtttatgaataagacacttttcctaatggaattaacccgatgcttttcttaaacatgtaaccttgagttcaccgcaaaaaacaatgcttcgattagagcaatgcatataataaaggttaccctcgtttcttagacactagacatcattcacaaaaagagaactgcttttgaaagggatgtatttgcactggaaagaatagttttctacttctaattataaatgatttattggtgaaagcaaaacaacagcctgtctgagaggcacttctatgagcatcctcacgtgtgatttgcaaggttgaagaagagggaaaaatgcctcaattgtaccaatggtgagaaaacacccaaagtacaaagcaggtttcaaaaaaaccatactcataaccaaggacaataataaagcaatgtgttgacatatactctataagtcttcctccataaatagtttatagaaattttgtaatttctgtaaatgcatcctataataattttgcatcttgctttttttttacatttaatatcaagtagatttctaaagggcaattatttgaaaattatcccaaatacatggggaaatatacatcaagtgaaaaaatgcagtgggtgatagagatatcaggaagcgcctcaaatatttctcatctcgttggagaaaaacaaacatgttctcatttagaatgagtgggagttacctaattgatttaggcctctatatttaacttctagtcaaaaaaggtagttctatctagcaacaatattatggggaacaaaagaaaaaattaactctctaaatttgcagtagggtcttttcttcagaagtaccaaatcccatctattaccagctccatgcttcaggcctaaaatggatctccctgaagcaatgacagaatttttgccaagtgactaggatataaacaccactttggttgcacagtgagacatatgctccaaagaaaactggttcaaaaacaggcaagtgggtttctacagaataaatgagagccctgtcaatggcttcatcttcagggctttgtgtctgtgcttgcgtggtggctcttgtttcatctatggataatggtggcacacagttttcataattccttacattaatgaactgctataaatttgtttttggtattctagagagtcctaacttcagcttctgggcaatgctgaggaggcaccctatattctagacttaccttttgcaaggtgtactctcagcattgtgggcgatttccatgggagaatattctatttaaagaactactgtcccagcataaaacaaaaaatcatttatgaagatgcaggagactcggaaagctctcaattattgtttgcacaagcacaatgtcacagcctcctttccccattccacaagggggtcaggaagagagtactcagctgtgagaaaagacatacagaagaattcatgtggtcatgagagcgaggacatggccgatcccccaaggaggatgtgtcatacacttcatgagcccaagagtgtgctgtagggtctgaagggcaagatgctggttcactgatgtaaaggagagggaaaaaagcttcaaccaactagaaaaacagtctctatgcatgctatttttgattttaaacacaggtatcaattccttctctcagagagtccattttaaaataggatacatttttaaaggaatatttaaaggacacattcattaaaatttattttaaaaacttttcaaaagaaacaaaaggtatgaattttatttaatccttgaggaaatggttcttttctcacacacataaatcactcattttgtttttctttatctcctttattaatctacattagaaaaataaacttttcatacactaagaacaaggaaaccactctcaattgacaaaatgttccaatccaacacaatgattactttcacctttaatttacaggcagccagattcaaaatccttaaagttgcttaaacttaaaaatgacaatgacaacctaaaaggtataatgttgattggaacagacatttaattggaaaattgatgattttccatttccaattaaatctctagatagaaatgaaaaaaattaaaaatcgtatttaagaaaagccaaatcttgggttgtgaggtatctttttaaggatgtttcagcagaaaaaaacaaaggctctcacaattgtgtagctgcctagattaagtgggtatcctgatcaaggagatgggggatgatttggctttagtattccaatgataaagtttataatgagaataacatgttgctacaaaatccagtctcttcctcagatgccttccacagagggcaggaagctttgtcagttttgtttgctgatgatgcctggttccgtcaacaaataacacctgataggcctggatcaagcatgcagctgtggagaacacccctgggactctaactctggcactctgcaagctgggtacttgggcaggacagcagcagcactcatgaactgggcagcacctgttggtgagggctgatcacatggattctctcatcccagccttacaatcagtccttcaggtacatactttttctgactttgctgatgaggaaactatgcacagaggttacacagcttaacaaagggttctcacctctcttcaagtggtatttaaatttcttctttcattttccttctggtaacaaagaagtctgtggctcaaaagatgtttctctaagaccccatcctattaggtctctgagattttagaaatgacccaacttgatccttttattcttcagaatatctctctcaaattttcatttgtttttcattaattgatgaataatgagacattttaggtacctgtccacaaagaaatgaaattttcactttccaggaacctaacaaatgaaaagatagaaatcaattccaacagaatattaccaaagaaatcttttagaatggactgttaaaattatttatttgtatttatctggctctactatttgtggtacatttccacttcaaagctaaacctcaaataacatcatagtgagtggttgacttcatgtttaactgagatcttgaagactgaaaaagaccacgacaaacacacatctattttcttggctactgcatccgtgttcatcaccattctgatagtctgcaatgtattgcagctcaccctttgggaaggactaaagtagacatctgtttgttctgcttactcagcattcctaccctaattttcctttggagaacccctttattctagaccacgtgaagctaatgccaaaccccattccaggggatgcacctgaatccaacctccatcatctaaacagtgccttctccacgttcagagaagagcaagtgactcaaactgccctcataagaacagacctgggacttctgctgcaaatattgaagagtaagtactcttttttcttgctaggactaagctggtagtaccttctatgaggctatcatatggaaacaacttgtctgaaaatgaagccacaactagaaaacagatcctggtaacccggattgatggatccagccctaccttaaatggcaagacctaacccgaggctttttgcatcaaccaataaagtccttaagccagtttgagttggttttgtcacttgcagctaaaagaattctgactctaacaatgtgacaatagcaaaaataaacataactgcttttgaggtttctaatggattttcctccctatatacatgatttcatttaatcctcacaattcaggaaagcacatatctattaacattaaattaatattcattattttgaacacatgctatgtggataagggatgaggaaagccaaggaagtaatcaacgtgaaatctcacttatatgggagggaagtggaggttacatatctcagggcacttaacagatatcatcaaatgaaagaataaacagtgtgtgggagaggcagtaggtgattcttcatcaattcctggatgaaaaattaggagataatgaactccgaacaggcagcctaatgagaatggctcaagcaacaggacatagagagggagttaggttagacatggggttcttgggaattttcacctcgtgggggggcgggggggtcgtgcagctgttgtcagtgggaaagggaaaaaggaaaaggctgagtttggaaggcagggagggaggagacaatgtgagtcagtgaaaaagggcccttagaatgacaagtctggaccagagagaggctaagactgaaaatacaagttgggtaaccactggcatacagatggcagttcaggcttgggcactgcccaccagagcctcagcatgaagagaagagggggaggctggccaccacctccctctaggtaatcgtcatcctgatgctgagctcctgaaaacaggctctttcactcgccccatctcttgctcttgattgcaacccggcattcaggaggcaccctgtaatatctgtggagtgaccgacaacacagcgccagggcactgagaagatcccagggcgccagggactggttctacaagggtgcccctcccggtcccctccagcgcgccgccagagctgccagtcttggctgctacacgggaggcagcctcattatgcagctctcacctcttaaattagttcatgctctcacattaggtgtaatcacagcttgcaacgctttctggggatgtctcagaaagatctgagttgaaaaaatatttttgtgtcattttaatttaaagtaaaattgctgcttcttccccgcccctttctttcctcctggcccacccagcgaccctggccggccgtgctcaacgggggcgggggtcggaggtgagatttcctccacataattccttaaacagctatcaactaagtctcaaagaaaaaaaaaagagatctagaagcagagacgtggctgctggcgatcccaaagctggtgttcgctcttgggggagagcgtaccctgggggaggccgggaggccgggccagaggctagcccagaggcagagggcaggagcgctcagccggcgccccgcgtctctccagctcccgacgctgcgctggctccgctgagcacgccaggatcaaggtcgcctggtggggaccggagcgccaggagcctgtgggaagcgttccagccggcctctgactgggatccggcgccgcgtttctgctttggacttgactgacaggtccccccgccctcccgccgccctactaccagcctgggttcatccttcagggctacgtctaccgcacccgggctggaaagcctggagcgcgcccttcctctcctcatcttctcagctctcctttctccctgccacttggcaaagctgcattttgactttcacgttttggactacgtgtgtgtagttccaagtccatgcgtggcacgaaaatccacttagggtaaaaattattctcgaaaaatcgcccatctcaggatctggtgtctacactcaaggctaggaggtgcaggtacgggtgcgtaaagcatgccgtaagggtgcacagtaaataaaaagtacggatgcaaaatgtaaattttaagtgcaaaacagaaaagcagtactcgttgccgccccgcacgctgggttttaaggggcacgaaggtgggcctcggctgcttttgctcagccccgcgtcctcagcgcccggcccagtacccggtactccgtaggggttcaatgatctcccctgaataagtgaacgaattaacaaatgaatgaatgaccgctcgatccgacctccgcggccggcagagcagtcgctggagaggcgggagagagcgagaggccaagctccaccatcgcggccgccggctggggcagagggacacggagacactcggcgccccggctccgcaccgagtccc

SEQ ID NO: 17585 - RNA, 13913 nt, Homo sapiens
  source 1..13913: mol_type = other RNA
tcaggccaggcacagtggctcatgcctgtagtcccagcactttgggaggccgaggtgggcagatccacgaggtcaggagatcaagaccatcctaacatggtaaaaccccatctctactaacaatacaaaaaattagtcaggtgtggtggcacgtgcctgtagtcccagctactcaggaggctgaggcaggagaatcgcttgaacctgggaggcggaggttgcagtgagccgagattgtgccactgcaccctagcctaggcaacagagcaagactctgtctcaaaaaaaataaaaaaaaaaaaaagagagaaagagagagagagatgaggagttgctgcactgctgggtgtggagagccgaggaggattcaaagatggtcctgaagtcccagctggaagaagtaggcggcagcaatgtttttaatactgtaaattcatcacgtagcacaggtttggggtggagaaagaaaaattgcattggcttcagggcatgcccagatctttcctcatcttaggcgtttgctaatacatgcattttctaagctgatgtcttgcgtttaatcactgctccattcaaaagagagaaggaggttgtttcaaacctagttgatatcatttgacttccatgctattcacagggctattttatttgaaacaggtataccacagccttaaattgcaagttaatccaggatgttcctaggttggcagttaggaacatgtaattctttggaagggctaaaagtcagctctttaaattatctccatatgaaccttctctccaccttagggtggatccacttatttagtccactgccagtaccacactagaacccgggtggtcactggactccagaaacaacagtagccctctctctgttctgtctctttttgactatctctattctgttcctgaccctgatttctcctgccaagctcaattttgacagctgacaacggcaagccatggcttcccaaaacattattttcaggtcaacttataaatttcaagaacacatttggctccgcttcctgtggtactaagcctacttcttgacagcatttgcctttgttgtaaatagcaaagttcttctagttggatttttgctaagaagtgtgtggatgtggcatgtgacgacatctttagcttggattctagaaaggcactaccattgtgcatttggctaaaggaaacacattttacccgtgaatgccttctatttacaaatgctcagctagcacacaaagctaagtacaagcaataagtactatcctacaatgttactcatttctgaaagcacaaaatgatgactggtatagctttggagatgttttctggaaacccaataaaggaacagatctttgttattccacacctacaaagtcagaagatgcacagtcttttattcatgtttgaacaagcttccttcttgaacaatcaactataaagtgatgtgattctctactagaccaggaactccttgaggacagaatgagggtctaatccatattctaaatccacaccacctggcacaatacatgttgcatggttagggtcaactaagagttggttgaattaatcaataacacacagcaagagaattcacaaagagaggggagtaatcccccagcctcaatcactcggcaagtggaatcgctgggcactgattccagctctgtctcagtgcttgagacagagctgaatgtaatgtgaacatttcaaatgaacaggaaaactagactcacggataagcagtgtagtcatcaagacaacactgtcttggaggtttttctgaagttaaaaccatgctacataagcaataaattatgaaggctgagcatgtgaataaaatttaatgttgtcataaattttataacaaagttaatctgacacatttaatgacatgcataatcattagtatgcagcactgtaatcagacattgataataagcagttcacaccagtgactgtaagagtctttacttgtgttcagccaagccaactgcttggtatatttttctcccttcttagtcgttagttttccatacctacaataactatcagtggtgatgggcttctctgaccatgtgaataatttaatcctcaatgcacagatacagaaacccttgctgaagacagtgtggagcagagaaggctgtctccactccttccacctgaaacacctctgcagatggatatgggagctctgcctacagcccttggacctaaccacttcagtgtgttccagtgagtgtctggacctcggcctgaaagatttttccgaaactaaagaaaatttctctgacctaaagaccttaacctccaccccagaagctctcaccaaggactacagggaactggtggggaaaatccttatcccttactcctcaaggcacagggcagtaatgctgaggcttgtgcgccacacttgctcccagaggtccccagcgggctacctgcggtggtgaatgacctcctaacacgccccttgacggccttcctttccttgcctcacttctccactctcctaccagcattgcagggttcacatcccaaatataccactggcacttgaatcctggtctccaggtctgtttctggaaaaacccaagtaagacattgccccagtaatggggctagatgtctgaggcttcctcaagtatctacctcgaaagctcttactgctgtacacacatgcacatacacacacgtgcgtacaaccagtcacatctaagcaccccgaataccagcctgttgaaggtagcagagagctgcactataagccaaggctgctcccaagagccgctccatcactgaattggcgccccagcaagatgaaggaatgtaatcattggaaggatggagaatgttctctgaatcactgacaaattggaaggggtggagggcaagagtccacctggtggagagatggaaagagcgagagagcctggaatgataatgccattgcttagaaaaggctgctccagatgccatatctacagaaattgtacagcccaaacatctctgagcaataggtctctggtagtcttgatgtctagaccaacaattcccagttcattcttctcagggaaggagccaggatagtccagagactctcattctgctgttagattgaaagggttaggcacaacagccttggcaaagtcacaagggcaaattcacactaaagtgtaaatgacccacaactcctcttctatttttaggttggggaggtgctttagaacataaggaggaactaaagaatattcctgttacatacaaggcagagaaaagggaaactagtggtgacaagacaaatcatccctttgacatttggctggctctacctattacagctctgggggtgaggtgggaacaaaaagatgctgtgtaaagaagtatcttatgccatccctactgtagtgaggtgcagtttagaggggacactgatcaagcagagacccagagtgtttcgttccaagccagaaacagaaatgtataaaacacagcctttccagcatcagaaatgagtagtggtagtggagaactacccaaaacaggaaagaggaccacgtgaggtagagtgtcaaggccctacattccagtgcctctgctcatgactgtaattttgggtaggtcacttaaagtctctggacctcagttttgccatctgtgaaatagggataatactatccagcataaaattggttatgaggctcatgtagggcctgcctgggatgatgtgttgctaatggttaagaacacaacttctggggtctgactggacaggctgaaatccctgcttaacacgttccagcagagccctgggcgatctatttaacttttgttttctcacctgtaagctgagacgaaagtacccactttataagattattccaataattagttgaaataatgcatgcagagaattaagcatggtacttgttatttgttaaactagctattaaaatgtgtaaaatataaagtattgtatggattttaggacaatgcaaagactctttgcttgctgcaatagttcggggccctttcagatggctaaaggcagaatttgtatgtgtaaatatggtgtgcttgtctctgctctggatactgagggcttaccctgttattaaacttatttagtaaatattgaactgtcatgaggcctaacatttagttccagttattagataaaacatttgctttgaatggtatttgaattgccaggttctagattattctggttgacaaactcttcgtattttataaagaggctaaaattggtaagctatcacagaacagatgtgccattttcaaggtatattaaaccatgattcactgtaacattgttcctactggcaacaaattcagagcaggctggactttatttggtgaagaaacattgagtggaagagaaatgacattattttatgtatttacattttcaaattactgtggcttaaacctgttcagccaacattacccaccttcagtctgctaaataaatgattcagtacatttctaatttacagaattttttaacaaaagaaaatgtaatttgatagccaaatcaacgttaaacattatacatttaaaaaaccacaggcaaagacacaaacatgatgacactaacttttgttaaagtatgcttacctatggtttcctctgaggcacgttctttcatgctaagcttccaacataatatgaaaatgaaggagatgcattttgcaaagcaaaacagaccttaagcaaaatattatacttctcaaattaacactgttacaaagttttagaatttaataagttcattaatttaaaagtttggatgtctgagtccttctatcccaaaacaagatcttggagggtcttccacagccatgtaataccatggtcacatgaccctttccaaaattattaatctgaatttactatatgaggataaatctatctttttgaaaatatttaggaaaatgagcttggtatttataaaatgaagctctctttgggtggtatcctaagacacgtcaagccaatcagcctgtaactgtgaaaaaaacattggtaggtacaaaagtggggtgggagaggagtgacttaactttgttaagtgatgggaaagaaacactaatagcattatctcaataaaatgtgatttaaaaaaatttaaaatactaaatcattgaactgacaaagaaatataaatcattcagaaataaactcattaggtcatcaaatcctgttaaatctgcaattaggaagagcaaggtgtacaatccatacatttaaactcacaggctcactttgcacaacgtcaatttactccttaatatgttattaatacgcattttccaaaaggatgtattagtaaatggtacacatctacttcttggcaacatcatataacctggtacaacataagcattcttcttatagttaagaaatgtggatggtatcaaaattagaaaaataaatgccctattatgttgtggtcaggtttaaggcatgtgaattttatcttcatacaaaagattaaaatctagatattaaaaagtagtgcagtatcagtgatgctgcctcagttcccaaaatgtcacatcacaaaaatatcccataattgcctgtagtttattccttggctttcctcttttctctctgcatctttgtaacaattttttaaaagtggaaatataattgttggcaatgctaacagctgtagaaatgattacaagatgtggaaaagcataacaggaatgtcaagaatctgtttctggcagtaatatatatggaacattgttcaggacaaaagaggagaaggaagaaaaaaaggagaggggtttatcatctctaagaattttcaaactaaacctcattgcttaataggaaaaaaagattccatatttaaagttaagtcacctctaactactagctaaagcatgacatcaccagcactggagtcagcggaagtgtgtttttgaaggacagtgttgcaggagaatctggacaggttttagagccaggagagagaaaataattctacctctgacagttgaaggaccttaggcaaatcagtttacctctgctagactacactccaaaatttggacattcaaaaatttgatattaataaccacatgaaagtctcgtgttgaggtgaatatgtatttgttggtgaaagatatgttggtttttaaacagacagcactctgcaattgtaggctattgttttgttttgccagttgtcaaattctatccagctatacacacttgtgtggcctcctaatggtgtttttccagtggctaaaggtttatgaataagacacttttcctaatggaattaacccgatgcttttcttaaacatgtaaccttgagttcaccgcaaaaaacaatgcttcgattagagcaatgcatataataaaggttaccctcgtttcttagacactagacatcattcacaaaaagagaactgcttttgaaagggatgtatttgcactggaaagaatagttttctacttctaattataaatgatttattggtgaaagcaaaacaacagcctgtctgagaggcacttctatgagcatcctcacgtgtgatttgcaaggttgaagaagagggaaaaatgcctcaattgtaccaatggtgagaaaacacccaaagtacaaagcaggtttcaaaaaaaccatactcataaccaaggacaataataaagcaatgtgttgacatatactctataagtcttcctccataaatagtttatagaaattttgtaatttctgtaaatgcatcctataataattttgcatcttgctttttttttacatttaatatcaagtagatttctaaagggcaattatttgaaaattatcccaaatacatggggaaatatacatcaagtgaaaaaatgcagtgggtgatagagatatcaggaagcgcctcaaatatttctcatctcgttggagaaaaacaaacatgttctcatttagaatgagtgggagttacctaattgatttaggcctctatatttaacttctagtcaaaaaaggtagttctatctagcaacaatattatggggaacaaaagaaaaaattaactctctaaatttgcagtagggtcttttcttcagaagtaccaaatcccatctattaccagctccatgcttcaggcctaaaatggatctccctgaagcaatgacagaatttttgccaagtgactaggatataaacaccactttggttgcacagtgagacatatgctccaaagaaaactggttcaaaaacaggcaagtgggtttctacagaataaatgagagccctgtcaatggcttcatcttcagggctttgtgtctgtgcttgcgtggtggctcttgtttcatctatggataatggtggcacacagttttcataattccttacattaatgaactgctataaatttgtttttggtattctagagagtcctaacttcagcttctgggcaatgctgaggaggcaccctatattctagacttaccttttgcaaggtgtactctcagcattgtgggcgatttccatgggagaatattctatttaaagaactactgtcccagcataaaacaaaaaatcatttatgaagatgcaggagactcggaaagctctcaattattgtttgcacaagcacaatgtcacagcctcctttccccattccacaagggggtcaggaagagagtactcagctgtgagaaaagacatacagaagaattcatgtggtcatgagagcgaggacatggccgatcccccaaggaggatgtgtcatacacttcatgagcccaagagtgtgctgtagggtctgaagggcaagatgctggttcactgatgtaaaggagagggaaaaaagcttcaaccaactagaaaaacagtctctatgcatgctatttttgattttaaacacaggtatcaattccttctctcagagagtccattttaaaataggatacatttttaaaggaatatttaaaggacacattcattaaaatttattttaaaaacttttcaaaagaaacaaaaggtatgaattttatttaatccttgaggaaatggttcttttctcacacacataaatcactcattttgtttttctttatctcctttattaatctacattagaaaaataaacttttcatacactaagaacaaggaaaccactctcaattgacaaaatgttccaatccaacacaatgattactttcacctttaatttacaggcagccagattcaaaatccttaaagttgcttaaacttaaaaatgacaatgacaacctaaaaggtataatgttgattggaacagacatttaattggaaaattgatgattttccatttccaattaaatctctagatagaaatgaaaaaaattaaaaatcgtatttaagaaaagccaaatcttgggttgtgaggtatctttttaaggatgtttcagcagaaaaaaacaaaggctctcacaattgtgtagctgcctagattaagtgggtatcctgatcaaggagatgggggatgatttggctttagtattccaatgataaagtttataatgagaataacatgttgctacaaaatccagtctcttcctcagatgccttccacagagggcaggaagctttgtcagttttgtttgctgatgatgcctggttccgtcaacaaataacacctgataggcctggatcaagcatgcagctgtggagaacacccctgggactctaactctggcactctgcaagctgggtacttgggcaggacagcagcagcactcatgaactgggcagcacctgttggtgagggctgatcacatggattctctcatcccagccttacaatcagtccttcaggtacatactttttctgactttgctgatgaggaaactatgcacagaggttacacagcttaacaaagggttctcacctctcttcaagtggtatttaaatttcttctttcattttccttctggtaacaaagaagtctgtggctcaaaagatgtttctctaagaccccatcctattaggtctctgagctgtgggaagtatttatacaattgcttgtgaatataagatccaggaatttccctaagatccctaacaaaattggtgataagtagtcccacatgttaatccagccacccacggatgacagcacttaccatttctttgataaatgtcaaatgcatttgaagtacctacctgaaatatttgtttaaatgctatctaatctattaattttatatatgtgtgagtctgttttgtataccttctgattataggataaatgtaaataaatccaaagagtaatcaaagctaccactttcaagaagccttctttgtagaaccggaagagtcttaaataggcttttcaggtatgcatctcttattatcgctgaactccaagtcctgcaaggcaggcatcatgtgtgggtcacctttacagtaggcacaggccttaaaacagtgacatgcacattgcaggcactccataaatgtttgctgaattggctaaaccttggtttgttcccataatcaaccaccacaaacagcacacagataattacttcttggaaagattccaactagtgtttgatgttacctacgtggtttttctctcaagatcttaagagcagctctgtaggattacattattttctgttttttttttcctttgaccttaatgtcatctacttcaataacagcttcatacaaaattcctaccagcacataccacagcagattcaaggccttgttttaaaaatggtgccagcttctcttaatttggaagatatattgtctctcctgaacatgggctaagaaaatgtataatttggtattaacataagagctgaagacactttaaatgcattgtttcatttttataagataaaaaaaattttaagaatcaaaatgttatcaacagacttgtccttcattaaaaagtaaaactgcatttgcctacattttatgaaagtgtccaattatgaacaattttgaaatgtaacttttaaaaatgtaaacagcaaaaatgttgtatttaaaataaatctggaaaggcagaaaaacaaaaaatacccagaagacagagtttttggtgaaagttaagatatttcatctttgaacaacttagaatctttcctgcattttatagtctagttccaggcattaatttgaaataaccttggaatcctaaatctaacacccttcggaacaaagtagcttttctcttctgctttatgagcaaatggactaaatactagggaatggtactgtctgggcctttgaaccaagattgaaagagatgaaatcctatatgatatgtataaacattagagaatccattttgatttaataaaaggttgaatttgttctatatcctgtgagaaaatggttcccttttcctgaaaatgttacctcattccaacaatagaaagttggtttttttccagggtgtggtgttggcgggggacagagttgccatgaatatggcatctatgaagactgctgttatattcatttctcaaaatgcactgtggtaggaaattcagaacgcagtgagagaaaataaatgtttgacttcaaaatataaggccgcatttaaagcagaaggtaaagtatagaacagttgacagtataaattctttatctgcaatcttgcagttccctaaatctctgtaacacatcacttttaaaagcctcagataagtggttctataataatttaccaataattcaacccctcaaaagtcttagcaagttaaaccttataatcttacattttagaaatgacccaacttgatccttttattcttcagaatatctctctcaaattttcatttgtttttcattaattgatgaataatgagacattttaggtacctgtccacaaagaaatgaaattttcactttccaggaacctaacaaatgaaaagatagaaatcaattccaacagaatattaccaaagaaatcttttagaatggactgttaaaattatttatttgtatttatctggctctactatttgtggtacatttccacttcaaagctaaacctcaaataacatcatagtgagtggttgacttcatgtttaactgagatcttgaagactgaaaaagaccacgacaaacacacatctattttcttggctactgcatccgtgttcatcaccattctgatagtctgcaatgtattgcagctcaccctttgggaaggactaaagtagacatctgtttgttctgcttactcagcattcctaccctaattttcctttggagaacccctttattctagaccacgtgaagctaatgccaaaccccattccaggggatgcacctgaatccaacctccatcatctaaacagtgccttctccacgttcagagaagagcaagtgactcaaactgccctcataagaacagacctgggacttctgctgcaaatattgaagagtaagtactcttttttcttgctaggactaagctggtagtaccttctatgaggctatcatatggaaacaacttgtctgaaaatgaagccacaactagaaaacagatcctggtaacccggattgatggatccagccctaccttaaatggcaagacctaacccgaggctttttgcatcaaccaataaagtccttaagccagtttgagttggttttgtcacttgcagctaaaagaattctgactctaacaatgtgacaatagcaaaaataaacataactgcttttgaggtttctaatggattttcctccctatatacatgatttcatttaatcctcacaattcaggaaagcacatatctattaacattaaattaatattcattattttgaacacatgctatgtggataagggatgaggaaagccaaggaagtaatcaacgtgaaatctcacttatatgggagggaagtggaggttacatatctcagggcacttaacagatatcatcaaatgaaagaataaacagtgtgtgggagaggcagtaggtgattcttcatcaattcctggatgaaaaattaggagataatgaactccgaacaggcagcctaatgagaatggctcaagcaacaggacatagagagggagttaggttagacatggggttcttgggaattttcacctcgtgggggggcgggggggtcgtgcagctgttgtcagtgggaaagggaaaaaggaaaaggctgagtttggaaggcagggagggaggagacaatgtgagtcagtgaaaaagggcccttagaatgacaagtctggaccagagagaggctaagactgaaaatacaagttgggtaaccactggcatacagatggcagttcaggcttgggcactgcccaccagagcctcagcatgaagagaagagggggaggctggccaccacctccctctaggtaatcgtcatcctgatgctgagctcctgaaaacaggctctttcactcgccccatctcttgctcttgattgcaacccggcattcaggaggcaccctgtaatatctgtggagtgaccgacaacacagcgccagggcactgagaagatcccagggcgccagggactggttctacaagggtgcccctcccggtcccctccagcgcgccgccagagctgccagtcttggctgctacacgggaggcagcctcattatgcagctctcacctcttaaattagttcatgctctcacattaggtgtaatcacagcttgcaacgctttctggggatgtctcagaaagatctgagttgaaaaaatatttttgtgtcattttaatttaaagtaaaattgctgcttcttccccgcccctttctttcctcctggcccacccagcgaccctggccggccgtgctcaacgggggcgggggtcggaggtgagatttcctccacataattccttaaacagctatcaactaagtctcaaagaaaaaaaaaagagatctagaagcagagacgtggctgctggcgatcccaaagctggtgttcgctcttgggggagagcgtaccctgggggaggccgggaggccgggccagaggctagcccagaggcagagggcaggagcgctcagccggcgccccgcgtctctccagctcccgacgctgcgctggctccgctgagcacgccaggatcaaggtcgcctggtggggaccggagcgccaggagcctgtgggaagcgttccagccggcctctgactgggatccggcgccgcgtttctgctttggacttgactgacaggtccccccgccctcccgccgccctactaccagcctgggttcatccttcagggctacgtctaccgcacccgggctggaaagcctggagcgcgcccttcctctcctcatcttctcagctctcctttctccctgccacttggcaaagctgcattttgactttcacgttttggactacgtgtgtgtagttccaagtccatgcgtggcacgaaaatccacttagggtaaaaattattctcgaaaaatcgcccatctcaggatctggtgtctacactcaaggctaggaggtgcaggtacgggtgcgtaaagcatgccgtaagggtgcacagtaaataaaaagtacggatgcaaaatgtaaattttaagtgcaaaacagaaaagcagtactcgttgccgccccgcacgctgggttttaaggggcacgaaggtgggcctcggctgcttttgctcagccccgcgtcctcagcgcccggcccagtacccggtactccgtaggggttcaatgatctcccctgaataagtgaacgaattaacaaatgaatgaatgaccgctcgatccgacctccgcggccggcagagcagtcgctggagaggcgggagagagcgagaggccaagctccaccatcgcggccgccggctggggcagagggacacggagacactcggcgccccggctccgcaccgagtc

SEQ ID NO: 17586 - RNA, 14293 nt, Homo sapiens
  source 1..14293: mol_type = other RNA
tcaggccaggcacagtggctcatgcctgtagtcccagcactttgggaggccgaggtgggcagatccacgaggtcaggagatcaagaccatcctaacatggtaaaaccccatctctactaacaatacaaaaaattagtcaggtgtggtggcacgtgcctgtagtcccagctactcaggaggctgaggcaggagaatcgcttgaacctgggaggcggaggttgcagtgagccgagattgtgccactgcaccctagcctaggcaacagagcaagactctgtctcaaaaaaaataaaaaaaaaaaaaagagagaaagagagagagagatgaggagttgctgcactgctgggtgtggagagccgaggaggattcaaagatggtcctgaagtcccagctggaagaagtaggcggcagcaatgtttttaatactgtaaattcatcacgtagcacaggtttggggtggagaaagaaaaattgcattggcttcagggcatgcccagatctttcctcatcttaggcgtttgctaatacatgcattttctaagctgatgtcttgcgtttaatcactgctccattcaaaagagagaaggaggttgtttcaaacctagttgatatcatttgacttccatgctattcacagggctattttatttgaaacaggtataccacagccttaaattgcaagttaatccaggatgttcctaggttggcagttaggaacatgtaattctttggaagggctaaaagtcagctctttaaattatctccatatgaaccttctctccaccttagggtggatccacttatttagtccactgccagtaccacactagaacccgggtggtcactggactccagaaacaacagtagccctctctctgttctgtctctttttgactatctctattctgttcctgaccctgatttctcctgccaagctcaattttgacagctgacaacggcaagccatggcttcccaaaacattattttcaggtcaacttataaatttcaagaacacatttggctccgcttcctgtggtactaagcctacttcttgacagcatttgcctttgttgtaaatagcaaagttcttctagttggatttttgctaagaagtgtgtggatgtggcatgtgacgacatctttagcttggattctagaaaggcactaccattgtgcatttggctaaaggaaacacattttacccgtgaatgccttctatttacaaatgctcagctagcacacaaagctaagtacaagcaataagtactatcctacaatgttactcatttctgaaagcacaaaatgatgactggtatagctttggagatgttttctggaaacccaataaaggaacagatctttgttattccacacctacaaagtcagaagatgcacagtcttttattcatgtttgaacaagcttccttcttgaacaatcaactataaagtgatgtgattctctactagaccaggaactccttgaggacagaatgagggtctaatccatattctaaatccacaccacctggcacaatacatgttgcatggttagggtcaactaagagttggttgaattaatcaataacacacagcaagagaattcacaaagagaggggagtaatcccccagcctcaatcactcggcaagtggaatcgctgggcactgattccagctctgtctcagtgcttgagacagagctgaatgtaatgtgaacatttcaaatgaacaggaaaactagactcacggataagcagtgtagtcatcaagacaacactgtcttggaggtttttctgaagttaaaaccatgctacataagcaataaattatgaaggctgagcatgtgaataaaatttaatgttgtcataaattttataacaaagttaatctgacacatttaatgacatgcataatcattagtatgcagcactgtaatcagacattgataataagcagttcacaccagtgactgtaagagtctttacttgtgttcagccaagccaactgcttggtatatttttctcccttcttagtcgttagttttccatacctacaataactatcagtggtgatgggcttctctgaccatgtgaataatttaatcctcaatgcacagatacagaaacccttgctgaagacagtgtggagcagagaaggctgtctccactccttccacctgaaacacctctgcagatggatatgggagctctgcctacagcccttggacctaaccacttcagtgtgttccagtgagtgtctggacctcggcctgaaagatttttccgaaactaaagaaaatttctctgacctaaagaccttaacctccaccccagaagctctcaccaaggactacagggaactggtggggaaaatccttatcccttactcctcaaggcacagggcagtaatgctgaggcttgtgcgccacacttgctcccagaggtccccagcgggctacctgcggtggtgaatgacctcctaacacgccccttgacggccttcctttccttgcctcacttctccactctcctaccagcattgcagggttcacatcccaaatataccactggcacttgaatcctggtctccaggtctgtttctggaaaaacccaagtaagacattgccccagtaatggggctagatgtctgaggcttcctcaagtatctacctcgaaagctcttactgctgtacacacatgcacatacacacacgtgcgtacaaccagtcacatctaagcaccccgaataccagcctgttgaaggtagcagagagctgcactataagccaaggctgctcccaagagccgctccatcactgaattggcgccccagcaagatgaaggaatgtaatcattggaaggatggagaatgttctctgaatcactgacaaattggaaggggtggagggcaagagtccacctggtggagagatggaaagagcgagagagcctggaatgataatgccattgcttagaaaaggctgctccagatgccatatctacagaaattgtacagcccaaacatctctgagcaataggtctctggtagtcttgatgtctagaccaacaattcccagttcattcttctcagggaaggagccaggatagtccagagactctcattctgctgttagattgaaagggttaggcacaacagccttggcaaagtcacaagggcaaattcacactaaagtgtaaatgacccacaactcctcttctatttttaggttggggaggtgctttagaacataaggaggaactaaagaatattcctgttacatacaaggcagagaaaagggaaactagtggtgacaagacaaatcatccctttgacatttggctggctctacctattacagctctgggggtgaggtgggaacaaaaagatgctgtgtaaagaagtatcttatgccatccctactgtagtgaggtgcagtttagaggggacactgatcaagcagagacccagagtgtttcgttccaagccagaaacagaaatgtataaaacacagcctttccagcatcagaaatgagtagtggtagtggagaactacccaaaacaggaaagaggaccacgtgaggtagagtgtcaaggccctacattccagtgcctctgctcatgactgtaattttgggtaggtcacttaaagtctctggacctcagttttgccatctgtgaaatagggataatactatccagcataaaattggttatgaggctcatgtagggcctgcctgggatgatgtgttgctaatggttaagaacacaacttctggggtctgactggacaggctgaaatccctgcttaacacgttccagcagagccctgggcgatctatttaacttttgttttctcacctgtaagctgagacgaaagtacccactttataagattattccaataattagttgaaataatgcatgcagagaattaagcatggtacttgttatttgttaaactagctattaaaatgtgtaaaatataaagtattgtatggattttaggacaatgcaaagactctttgcttgctgcaatagttcggggccctttcagatggctaaaggcagaatttgtatgtgtaaatatggtgtgcttgtctctgctctggatactgagggcttaccctgttattaaacttatttagtaaatattgaactgtcatgaggcctaacatttagttccagttattagataaaacatttgctttgaatggtatttgaattgccaggttctagattattctggttgacaaactcttcgtattttataaagaggctaaaattggtaagctatcacagaacagatgtgccattttcaaggtatattaaaccatgattcactgtaacattgttcctactggcaacaaattcagagcaggctggactttatttggtgaagaaacattgagtggaagagaaatgacattattttatgtatttacattttcaaattactgtggcttaaacctgttcagccaacattacccaccttcagtctgctaaataaatgattcagtacatttctaatttacagaattttttaacaaaagaaaatgtaatttgatagccaaatcaacgttaaacattatacatttaaaaaaccacaggcaaagacacaaacatgatgacactaacttttgttaaagtatgcttacctatggtttcctctgaggcacgttctttcatgctaagcttccaacataatatgaaaatgaaggagatgcattttgcaaagcaaaacagaccttaagcaaaatattatacttctcaaattaacactgttacaaagttttagaatttaataagttcattaatttaaaagtttggatgtctgagtccttctatcccaaaacaagatcttggagggtcttccacagccatgtaataccatggtcacatgaccctttccaaaattattaatctgaatttactatatgaggataaatctatctttttgaaaatatttaggaaaatgagcttggtatttataaaatgaagctctctttgggtggtatcctaagacacgtcaagccaatcagcctgtaactgtgaaaaaaacattggtaggtacaaaagtggggtgggagaggagtgacttaactttgttaagtgatgggaaagaaacactaatagcattatctcaataaaatgtgatttaaaaaaatttaaaatactaaatcattgaactgacaaagaaatataaatcattcagaaataaactcattaggtcatcaaatcctgttaaatctgcaattaggaagagcaaggtgtacaatccatacatttaaactcacaggctcactttgcacaacgtcaatttactccttaatatgttattaatacgcattttccaaaaggatgtattagtaaatggtacacatctacttcttggcaacatcatataacctggtacaacataagcattcttcttatagttaagaaatgtggatggtatcaaaattagaaaaataaatgccctattatgttgtggtcaggtttaaggcatgtgaattttatcttcatacaaaagattaaaatctagatattaaaaagtagtgcagtatcagtgatgctgcctcagttcccaaaatgtcacatcacaaaaatatcccataattgcctgtagtttattccttggctttcctcttttctctctgcatctttgtaacaattttttaaaagtggaaatataattgttggcaatgctaacagctgtagaaatgattacaagatgtggaaaagcataacaggaatgtcaagaatctgtttctggcagtaatatatatggaacattgttcaggacaaaagaggagaaggaagaaaaaaaggagaggggtttatcatctctaagaattttcaaactaaacctcattgcttaataggaaaaaaagattccatatttaaagttaagtcacctctaactactagctaaagcatgacatcaccagcactggagtcagcggaagtgtgtttttgaaggacagtgttgcaggagaatctggacaggttttagagccaggagagagaaaataattctacctctgacagttgaaggaccttaggcaaatcagtttacctctgctagactacactccaaaatttggacattcaaaaatttgatattaataaccacatgaaagtctcgtgttgaggtgaatatgtatttgttggtgaaagatatgttggtttttaaacagacagcactctgcaattgtaggctattgttttgttttgccagttgtcaaattctatccagctatacacacttgtgtggcctcctaatggtgtttttccagtggctaaaggtttatgaataagacacttttcctaatggaattaacccgatgcttttcttaaacatgtaaccttgagttcaccgcaaaaaacaatgcttcgattagagcaatgcatataataaaggttaccctcgtttcttagacactagacatcattcacaaaaagagaactgcttttgaaagggatgtatttgcactggaaagaatagttttctacttctaattataaatgatttattggtgaaagcaaaacaacagcctgtctgagaggcacttctatgagcatcctcacgtgtgatttgcaaggttgaagaagagggaaaaatgcctcaattgtaccaatggtgagaaaacacccaaagtacaaagcaggtttcaaaaaaaccatactcataaccaaggacaataataaagcaatgtgttgacatatactctataagtcttcctccataaatagtttatagaaattttgtaatttctgtaaatgcatcctataataattttgcatcttgctttttttttacatttaatatcaagtagatttctaaagggcaattatttgaaaattatcccaaatacatggggaaatatacatcaagtgaaaaaatgcagtgggtgatagagatatcaggaagcgcctcaaatatttctcatctcgttggagaaaaacaaacatgttctcatttagaatgagtgggagttacctaattgatttaggcctctatatttaacttctagtcaaaaaaggtagttctatctagcaacaatattatggggaacaaaagaaaaaattaactctctaaatttgcagtagggtcttttcttcagaagtaccaaatcccatctattaccagctccatgcttcaggcctaaaatggatctccctgaagcaatgacagaatttttgccaagtgactaggatataaacaccactttggttgcacagtgagacatatgctccaaagaaaactggttcaaaaacaggcaagtgggtttctacagaataaatgagagccctgtcaatggcttcatcttcagggctttgtgtctgtgcttgcgtggtggctcttgtttcatctatggataatggtggcacacagttttcataattccttacattaatgaactgctataaatttgtttttggtattctagagagtcctaacttcagcttctgggcaatgctgaggaggcaccctatattctagacttaccttttgcaaggtgtactctcagcattgtgggcgatttccatgggagaatattctatttaaagaactactgtcccagcataaaacaaaaaatcatttatgaagatgcaggagactcggaaagctctcaattattgtttgcacaagcacaatgtcacagcctcctttccccattccacaagggggtcaggaagagagtactcagctgtgagaaaagacatacagaagaattcatgtggtcatgagagcgaggacatggccgatcccccaaggaggatgtgtcatacacttcatgagcccaagagtgtgctgtagggtctgaagggcaagatgctggttcactgatgtaaaggagagggaaaaaagcttcaaccaactagaaaaacagtctctatgcatgctatttttgattttaaacacaggtatcaattccttctctcagagagtccattttaaaataggatacatttttaaaggaatatttaaaggacacattcattaaaatttattttaaaaacttttcaaaagaaacaaaaggtatgaattttatttaatccttgaggaaatggttcttttctcacacacataaatcactcattttgtttttctttatctcctttattaatctacattagaaaaataaacttttcatacactaagaacaaggaaaccactctcaattgacaaaatgttccaatccaacacaatgattactttcacctttaatttacaggcagccagattcaaaatccttaaagttgcttaaacttaaaaatgacaatgacaacctaaaaggtataatgttgattggaacagacatttaattggaaaattgatgattttccatttccaattaaatctctagatagaaatgaaaaaaattaaaaatcgtatttaagaaaagccaaatcttgggttgtgaggtatctttttaaggatgtttcagcagaaaaaaacaaaggctctcacaattgtgtagctgcctagattaagtgggtatcctgatcaaggagatgggggatgatttggctttagtattccaatgataaagtttataatgagaataacatgttgctacaaaatccagtctcttcctcagatgccttccacagagggcaggaagctttgtcagttttgtttgctgatgatgcctggttccgtcaacaaataacacctgtcacacggtgggtagtcaatatacatttgttgaataaatatgaaaaaaagaaatgtacaatatgtttgtgaagccaactgtgtgtgcattgctattgaggtacacaaaaagtctttgttttaaatttgagaatgaggactttcaatggaatatatctataaaaatgaaaaaaagacattactgtctggacttttgtacagcaagagaagaaaaaccactagccaagagccaactcacctgataggcctggatcaagcatgcagctgtggagaacacccctgggactctaactctggcactctgcaagctgggtacttgggcaggacagcagcagcactcatgaactgggcagcaccgactggcaaacctccccctgaagatggagaaggaggaaggagtgttactggaatgagagcttgagtccaggggaggaggatgggctgctgaggaggcgacaccatcctgaaagaagaatcctctgccagaggcttttcagggtcatttcttcacactctctgcagggaagcacggagacagcaggaagaaatatcctaacctcactctcttccctctacaggtgcttccattggccaaatccacccagaggccagttggtggcgatcagctctcttcaagtggtatttaaatttcttctttcattttccttctggtaacaaagaagtctgtggctcaaaagatgtttctctaagaccccatcctattaggtctctgagctgtgggaagtatttatacaattgcttgtgaatataagatccaggaatttccctaagatccctaacaaaattggtgataagtagtcccacatgttaatccagccacccacggatgacagcacttaccatttctttgataaatgtcaaatgcatttgaagtacctacctgaaatatttgtttaaatgctatctaatctattaattttatatatgtgtgagtctgttttgtataccttctgattataggataaatgtaaataaatccaaagagtaatcaaagctaccactttcaagaagccttctttgtagaaccggaagagtcttaaataggcttttcaggtatgcatctcttattatcgctgaactccaagtcctgcaaggcaggcatcatgtgtgggtcacctttacagtaggcacaggccttaaaacagtgacatgcacattgcaggcactccataaatgtttgctgaattggctaaaccttggtttgttcccataatcaaccaccacaaacagcacacagataattacttcttggaaagattccaactagtgtttgatgttacctacgtggtttttctctcaagatcttaagagcagctctgtaggattacattattttctgttttttttttcctttgaccttaatgtcatctacttcaataacagcttcatacaaaattcctaccagcacataccacagcagattcaaggccttgttttaaaaatggtgccagcttctcttaatttggaagatatattgtctctcctgaacatgggctaagaaaatgtataatttggtattaacataagagctgaagacactttaaatgcattgtttcatttttataagataaaaaaaattttaagaatcaaaatgttatcaacagacttgtccttcattaaaaagtaaaactgcatttgcctacattttatgaaagtgtccaattatgaacaattttgaaatgtaacttttaaaaatgtaaacagcaaaaatgttgtatttaaaataaatctggaaaggcagaaaaacaaaaaatacccagaagacagagtttttggtgaaagttaagatatttcatctttgaacaacttagaatctttcctgcattttatagtctagttccaggcattaatttgaaataaccttggaatcctaaatctaacacccttcggaacaaagtagcttttctcttctgctttatgagcaaatggactaaatactagggaatggtactgtctgggcctttgaaccaagattgaaagagatgaaatcctatatgatatgtataaacattagagaatccattttgatttaataaaaggttgaatttgttctatatcctgtgagaaaatggttcccttttcctgaaaatgttacctcattccaacaatagaaagttggtttttttccagggtgtggtgttggcgggggacagagttgccatgaatatggcatctatgaagactgctgttatattcatttctcaaaatgcactgtggtaggaaattcagaacgcagtgagagaaaataaatgtttgacttcaaaatataaggccgcatttaaagcagaaggtaaagtatagaacagttgacagtataaattctttatctgcaatcttgcagttccctaaatctctgtaacacatcacttttaaaagcctcagataagtggttctataataatttaccaataattcaacccctcaaaagtcttagcaagttaaaccttataatcttacattttagaaatgacccaacttgatccttttattcttcagaatatctctctcaaattttcatttgtttttcattaattgatgaataatgagacattttaggtacctgtccacaaagaaatgaaattttcactttccaggaacctaacaaatgaaaagatagaaatcaattccaacagaatattaccaaagaaatcttttagaatggactgttaaaattatttatttgtatttatctggctctactatttgtggtacatttccacttcaaagctaaacctcaaataacatcatagtgagtggttgacttcatgtttaactgagatcttgaagactgaaaaagaccacgacaaacacacatctattttcttggctactgcatccgtgttcatcaccattctgatagtctgcaatgtattgcagctcaccctttgggaaggactaaagtagacatctgtttgttctgcttactcagcattcctaccctaattttcctttggagaacccctttattctagaccacgtgaagctaatgccaaaccccattccaggggatgcacctgaatccaacctccatcatctaaacagtgccttctccacgttcagagaagagcaagtgactcaaactgccctcataagaacagacctgggacttctgctgcaaatattgaagagtaagtactcttttttcttgctaggactaagctggtagtaccttctatgaggctatcatatggaaacaacttgtctgaaaatgaagccacaactagaaaacagatcctggtaacccggattgatggatccagccctaccttaaatggcaagacctaacccgaggctttttgcatcaaccaataaagtccttaagccagtttgagttggttttgtcacttgcagctaaaagaattctgactctaacaatgtgacaatagcaaaaataaacataactgcttttgaggtttctaatggattttcctccctatatacatgatttcatttaatcctcacaattcaggaaagcacatatctattaacattaaattaatattcattattttgaacacatgctatgtggataagggatgaggaaagccaaggaagtaatcaacgtgaaatctcacttatatgggagggaagtggaggttacatatctcagggcacttaacagatatcatcaaatgaaagaataaacagtgtgtgggagaggcagtaggtgattcttcatcaattcctggatgaaaaattaggagataatgaactccgaacaggcagcctaatgagaatggctcaagcaacaggacatagagagggagttaggttagacatggggttcttgggaattttcacctcgtgggggggcgggggggtcgtgcagctgttgtcagtgggaaagggaaaaaggaaaaggctgagtttggaaggcagggagggaggagacaatgtgagtcagtgaaaaagggcccttagaatgacaagtctggaccagagagaggctaagactgaaaatacaagttgggtaaccactggcatacagatggcagttcaggcttgggcactgcccaccagagcctcagcatgaagagaagagggggaggctggccaccacctccctctaggtaatcgtcatcctgatgctgagctcctgaaaacaggctctttcactcgccccatctcttgctcttgattgcaacccggcattcaggaggcaccctgtaatatctgtggagtgaccgacaacacagcgccagggcactgagaagatcccagggcgccagggactggttctacaagggtgcccctcccggtcccctccagcgcgccgccagagctgccagtcttggctgctacacgggaggcagcctcattatgcagctctcacctcttaaattagttcatgctctcacattaggtgtaatcacagcttgcaacgctttctggggatgtctcagaaagatctgagttgaaaaaatatttttgtgtcattttaatttaaagtaaaattgctgcttcttccccgcccctttctttcctcctggcccacccagcgaccctggccggccgtgctcaacgggggcgggggtcggaggtgagatttcctccacataattccttaaacagctatcaactaagtctcaaagaaaaaaaaaagagatctagaagcagagacgtggctgctggcgatcccaaagctggtgttcgctcttgggggagagcgtaccctgggggaggccgggaggccgggccagaggctagcccagaggcagagggcaggagcgctcagccggcgccccgcgtctctccagctcccgacgctgcgctggctccgctgagcacgccaggatcaaggtcgcctggtggggaccggagcgccaggagcctgtgggaagcgttccagccggcctctgactgggatccggcgccgcgtttctgctttggacttgactgacaggtccccccgccctcccgccgccctactaccagcctgggttcatccttcagggctacgtctaccgcacccgggctggaaagcctggagcgcgcccttcctctcctcatcttctcagctctcctttctccctgccacttggcaaagctgcattttgactttcacgttttggactacgtgtgtgtagttccaagtccatgcgtggcacgaaaatccacttagggtaaaaattattctcgaaaaatcgcccatctcaggatctggtgtctacactcaaggctaggaggtgcaggtacgggtgcgtaaagcatgccgtaagggtgcacagtaaataaaaagtacggatgcaaaatgtaaattttaagtgcaaaacagaaaagcagtactcgttgccgccccgcacgctgggttttaaggggcacgaaggtgggcctcggctgcttttgctcagccccgcgtcctcagcgcccggcccagtacccggtactccgtaggggttcaatgatctcccctgaataagtgaacgaattaacaaatgaatgaatgaccgctcgatccgacctccgcggccggcagagcagtcgctggagaggcgggagagagcgagaggccaagctccaccatcgcggccgccggctggggcagagggacacggagacactcggcgccccggctccgcaccgagtccccg

SEQ ID NO: 17587 - RNA, 12280 nt, Homo sapiens
  source 1..12280: mol_type = other RNA
tcaggccaggcacagtggctcatgcctgtagtcccagcactttgggaggccgaggtgggcagatccacgaggtcaggagatcaagaccatcctaacatggtaaaaccccatctctactaacaatacaaaaaattagtcaggtgtggtggcacgtgcctgtagtcccagctactcaggaggctgaggcaggagaatcgcttgaacctgggaggcggaggttgcagtgagccgagattgtgccactgcaccctagcctaggcaacagagcaagactctgtctcaaaaaaaataaaaaaaaaaaaaagagagaaagagagagagagatgaggagttgctgcactgctgggtgtggagagccgaggaggattcaaagatggtcctgaagtcccagctggaagaagtaggcggcagcaatgtttttaatactgtaaattcatcacgtagcacaggtttggggtggagaaagaaaaattgcattggcttcagggcatgcccagatctttcctcatcttaggcgtttgctaatacatgcattttctaagctgatgtcttgcgtttaatcactgctccattcaaaagagagaaggaggttgtttcaaacctagttgatatcatttgacttccatgctattcacagggctattttatttgaaacaggtataccacagccttaaattgcaagttaatccaggatgttcctaggttggcagttaggaacatgtaattctttggaagggctaaaagtcagctctttaaattatctccatatgaaccttctctccaccttagggtggatccacttatttagtccactgccagtaccacactagaacccgggtggtcactggactccagaaacaacagtagccctctctctgttctgtctctttttgactatctctattctgttcctgaccctgatttctcctgccaagctcaattttgacagctgacaacggcaagccatggcttcccaaaacattattttcaggtcaacttataaatttcaagaacacatttggctccgcttcctgtggtactaagcctacttcttgacagcatttgcctttgttgtaaatagcaaagttcttctagttggatttttgctaagaagtgtgtggatgtggcatgtgacgacatctttagcttggattctagaaaggcactaccattgtgcatttggctaaaggaaacacattttacccgtgaatgccttctatttacaaatgctcagctagcacacaaagctaagtacaagcaataagtactatcctacaatgttactcatttctgaaagcacaaaatgatgactggtatagctttggagatgttttctggaaacccaataaaggaacagatctttgttattccacacctacaaagtcagaagatgcacagtcttttattcatgtttgaacaagcttccttcttgaacaatcaactataaagtgatgtgattctctactagaccaggaactccttgaggacagaatgagggtctaatccatattctaaatccacaccacctggcacaatacatgttgcatggttagggtcaactaagagttggttgaattaatcaataacacacagcaagagaattcacaaagagaggggagtaatcccccagcctcaatcactcggcaagtggaatcgctgggcactgattccagctctgtctcagtgcttgagacagagctgaatgtaatgtgaacatttcaaatgaacaggaaaactagactcacggataagcagtgtagtcatcaagacaacactgtcttggaggtttttctgaagttaaaaccatgctacataagcaataaattatgaaggctgagcatgtgaataaaatttaatgttgtcataaattttataacaaagttaatctgacacatttaatgacatgcataatcattagtatgcagcactgtaatcagacattgataataagcagttcacaccagtgactgtaagagtctttacttgtgttcagccaagccaactgcttggtatatttttctcccttcttagtcgttagttttccatacctacaataactatcagtggtgatgggcttctctgaccatgtgaataatttaatcctcaatgcacagatacagaaacccttgctgaagacagtgtggagcagagaaggctgtctccactccttccacctgaaacacctctgcagatggatatgggagctctgcctacagcccttggacctaaccacttcagtgtgttccagtgagtgtctggacctcggcctgaaagatttttccgaaactaaagaaaatttctctgacctaaagaccttaacctccaccccagaagctctcaccaaggactacagggaactggtggggaaaatccttatcccttactcctcaaggcacagggcagtaatgctgaggcttgtgcgccacacttgctcccagaggtccccagcgggctacctgcggtggtgaatgacctcctaacacgccccttgacggccttcctttccttgcctcacttctccactctcctaccagcattgcagggttcacatcccaaatataccactggcacttgaatcctggtctccaggtctgtttctggaaaaacccaagtaagacattgccccagtaatggggctagatgtctgaggcttcctcaagtatctacctcgaaagctcttactgctgtacacacatgcacatacacacacgtgcgtacaaccagtcacatctaagcaccccgaataccagcctgttgaaggtagcagagagctgcactataagccaaggctgctcccaagagccgctccatcactgaattggcgccccagcaagatgaaggaatgtaatcattggaaggatggagaatgttctctgaatcactgacaaattggaaggggtggagggcaagagtccacctggtggagagatggaaagagcgagagagcctggaatgataatgccattgcttagaaaaggctgctccagatgccatatctacagaaattgtacagcccaaacatctctgagcaataggtctctggtagtcttgatgtctagaccaacaattcccagttcattcttctcagggaaggagccaggatagtccagagactctcattctgctgttagattgaaagggttaggcacaacagccttggcaaagtcacaagggcaaattcacactaaagtgtaaatgacccacaactcctcttctatttttaggttggggaggtgctttagaacataaggaggaactaaagaatattcctgttacatacaaggcagagaaaagggaaactagtggtgacaagacaaatcatccctttgacatttggctggctctacctattacagctctgggggtgaggtgggaacaaaaagatgctgtgtaaagaagtatcttatgccatccctactgtagtgaggtgcagtttagaggggacactgatcaagcagagacccagagtgtttcgttccaagccagaaacagaaatgtataaaacacagcctttccagcatcagaaatgagtagtggtagtggagaactacccaaaacaggaaagaggaccacgtgaggtagagtgtcaaggccctacattccagtgcctctgctcatgactgtaattttgggtaggtcacttaaagtctctggacctcagttttgccatctgtgaaatagggataatactatccagcataaaattggttatgaggctcatgtagggcctgcctgggatgatgtgttgctaatggttaagaacacaacttctggggtctgactggacaggctgaaatccctgcttaacacgttccagcagagccctgggcgatctatttaacttttgttttctcacctgtaagctgagacgaaagtacccactttataagattattccaataattagttgaaataatgcatgcagagaattaagcatggtacttgttatttgttaaactagctattaaaatgtgtaaaatataaagtattgtatggattttaggacaatgcaaagactctttgcttgctgcaatagttcggggccctttcagatggctaaaggcagaatttgtatgtgtaaatatggtgtgcttgtctctgctctggatactgagggcttaccctgttattaaacttatttagtaaatattgaactgtcatgaggcctaacatttagttccagttattagataaaacatttgctttgaatggtatttgaattgccaggttctagattattctggttgacaaactcttcgtattttataaagaggctaaaattggtaagctatcacagaacagatgtgccattttcaaggtatattaaaccatgattcactgtaacattgttcctactggcaacaaattcagagcaggctggactttatttggtgaagaaacattgagtggaagagaaatgacattattttatgtatttacattttcaaattactgtggcttaaacctgttcagccaacattacccaccttcagtctgctaaataaatgattcagtacatttctaatttacagaattttttaacaaaagaaaatgtaatttgatagccaaatcaacgttaaacattatacatttaaaaaaccacaggcaaagacacaaacatgatgacactaacttttgttaaagtatgcttacctatggtttcctctgaggcacgttctttcatgctaagcttccaacataatatgaaaatgaaggagatgcattttgcaaagcaaaacagaccttaagcaaaatattatacttctcaaattaacactgttacaaagttttagaatttaataagttcattaatttaaaagtttggatgtctgagtccttctatcccaaaacaagatcttggagggtcttccacagccatgtaataccatggtcacatgaccctttccaaaattattaatctgaatttactatatgaggataaatctatctttttgaaaatatttaggaaaatgagcttggtatttataaaatgaagctctctttgggtggtatcctaagacacgtcaagccaatcagcctgtaactgtgaaaaaaacattggtaggtacaaaagtggggtgggagaggagtgacttaactttgttaagtgatgggaaagaaacactaatagcattatctcaataaaatgtgatttaaaaaaatttaaaatactaaatcattgaactgacaaagaaatataaatcattcagaaataaactcattaggtcatcaaatcctgttaaatctgcaattaggaagagcaaggtgtacaatccatacatttaaactcacaggctcactttgcacaacgtcaatttactccttaatatgttattaatacgcattttccaaaaggatgtattagtaaatggtacacatctacttcttggcaacatcatataacctggtacaacataagcattcttcttatagttaagaaatgtggatggtatcaaaattagaaaaataaatgccctattatgttgtggtcaggtttaaggcatgtgaattttatcttcatacaaaagattaaaatctagatattaaaaagtagtgcagtatcagtgatgctgcctcagttcccaaaatgtcacatcacaaaaatatcccataattgcctgtagtttattccttggctttcctcttttctctctgcatctttgtaacaattttttaaaagtggaaatataattgttggcaatgctaacagctgtagaaatgattacaagatgtggaaaagcataacaggaatgtcaagaatctgtttctggcagtaatatatatggaacattgttcaggacaaaagaggagaaggaagaaaaaaaggagaggggtttatcatctctaagaattttcaaactaaacctcattgcttaataggaaaaaaagattccatatttaaagttaagtcacctctaactactagctaaagcatgacatcaccagcactggagtcagcggaagtgtgtttttgaaggacagtgttgcaggagaatctggacaggttttagagccaggagagagaaaataattctacctctgacagttgaaggaccttaggcaaatcagtttacctctgctagactacactccaaaatttggacattcaaaaatttgatattaataaccacatgaaagtctcgtgttgaggtgaatatgtatttgttggtgaaagatatgttggtttttaaacagacagcactctgcaattgtaggctattgttttgttttgccagttgtcaaattctatccagctatacacacttgtgtggcctcctaatggtgtttttccagtggctaaaggtttatgaataagacacttttcctaatggaattaacccgatgcttttcttaaacatgtaaccttgagttcaccgcaaaaaacaatgcttcgattagagcaatgcatataataaaggttaccctcgtttcttagacactagacatcattcacaaaaagagaactgcttttgaaagggatgtatttgcactggaaagaatagttttctacttctaattataaatgatttattggtgaaagcaaaacaacagcctgtctgagaggcacttctatgagcatcctcacgtgtgatttgcaaggttgaagaagagggaaaaatgcctcaattgtaccaatggtgagaaaacacccaaagtacaaagcaggtttcaaaaaaaccatactcataaccaaggacaataataaagcaatgtgttgacatatactctataagtcttcctccataaatagtttatagaaattttgtaatttctgtaaatgcatcctataataattttgcatcttgctttttttttacatttaatatcaagtagatttctaaagggcaattatttgaaaattatcccaaatacatggggaaatatacatcaagtgaaaaaatgcagtgggtgatagagatatcaggaagcgcctcaaatatttctcatctcgttggagaaaaacaaacatgttctcatttagaatgagtgggagttacctaattgatttaggcctctatatttaacttctagtcaaaaaaggtagttctatctagcaacaatattatggggaacaaaagaaaaaattaactctctaaatttgcagtagggtcttttcttcagaagtaccaaatcccatctattaccagctccatgcttcaggcctaaaatggatctccctgaagcaatgacagaatttttgccaagtgactaggatataaacaccactttggttgcacagtgagacatatgctccaaagaaaactggttcaaaaacaggcaagtgggtttctacagaataaatgagagccctgtcaatggcttcatcttcagggctttgtgtctgtgcttgcgtggtggctcttgtttcatctatggataatggtggcacacagttttcataattccttacattaatgaactgctataaatttgtttttggtattctagagagtcctaacttcagcttctgggcaatgctgaggaggcaccctatattctagacttaccttttgcaaggtgtactctcagcattgtgggcgatttccatgggagaatattctatttaaagaactactgtcccagcataaaacaaaaaatcatttatgaagatgcaggagactcggaaagctctcaattattgtttgcacaagcacaatgtcacagcctcctttccccattccacaagggggtcaggaagagagtactcagctgtgagaaaagacatacagaagaattcatgtggtcatgagagcgaggacatggccgatcccccaaggaggatgtgtcatacacttcatgagcccaagagtgtgctgtagggtctgaagggcaagatgctggttcactgatgtaaaggagagggaaaaaagcttcaaccaactagaaaaacagtctctatgcatgctatttttgattttaaacacaggtatcaattccttctctcagagagtccattttaaaataggatacatttttaaaggaatatttaaaggacacattcattaaaatttattttaaaaacttttcaaaagaaacaaaaggtatgaattttatttaatccttgaggaaatggttcttttctcacacacataaatcactcattttgtttttctttatctcctttattaatctacattagaaaaataaacttttcatacactaagaacaaggaaaccactctcaattgacaaaatgttccaatccaacacaatgattactttcacctttaatttacaggcagccagattcaaaatccttaaagttgcttaaacttaaaaatgacaatgacaacctaaaaggtataatgttgattggaacagacatttaattggaaaattgatgattttccatttccaattaaatctctagatagaaatgaaaaaaattaaaaatcgtatttaagaaaagccaaatcttgggttgtgaggtatctttttaaggatgtttcagcagaaaaaaacaaaggctctcacaattgtgtagctgcctagattaagtgggtatcctgatcaaggagatgggggatgatttggctttagtattccaatgataaagtttataatgagaataacatgttgctacaaaatccagtctcttcctcagatgccttccacagagggcaggaagctttgtcagttttgtttgctgatgatgcctggttccgtcaacaaataacacctgtcacacggtgggtagtcaatatacatttgttgaataaatatgaaaaaaagaaatgtacaatatgtttgtgaagccaactgtgtgtgcattgctattgaggtacacaaaaagtctttgttttaaatttgagaatgaggactttcaatggaatatatctataaaaatgaaaaaaagacattactgtctggacttttgtacagcaagagaagaaaaaccactagccaagagccaactcacctgataggcctggatcaagcatgcagctgtggagaacacccctgggactctaactctggcactctgcaagctgggtacttgggcaggacagcagcagcactcatgaactgggcagcacctctcttcaagtggtatttaaatttcttctttcattttccttctggtaacaaagaagtctgtggctcaaaagatgtttctctaagaccccatcctattaggtctctgagattttagaaatgacccaacttgatccttttattcttcagaatatctctctcaaattttcatttgtttttcattaattgatgaataatgagacattttaggtacctgtccacaaagaaatgaaattttcactttccaggaacctaacaaatgaaaagatagaaatcaattccaacagaatattaccaaagaaatcttttagaatggactgttaaaattatttatttgtatttatctggctctactatttgtggtacatttccacttcaaagctaaacctcaaataacatcatagtgagtggttgacttcatgtttaactgagatcttgaagactgaaaaagaccacgacaaacacacatctattttcttggctactgcatccgtgttcatcaccattctgatagtctgcaatgtattgcagctcaccctttgggaaggactaaagtagacatctgtttgttctgcttactcagcattcctaccctaattttcctttggagaacccctttattctagaccacgtgaagctaatgccaaaccccattccaggggatgcacctgaatccaacctccatcatctaaacagtgccttctccacgttcagagaagagcaagtgactcaaactgccctcataagaacagacctgggacttctgctgcaaatattgaagagtaagtactcttttttcttgctaggactaagctggtagtaccttctatgaggctatcatatggaaacaacttgtctgaaaatgaagccacaactagaaaacagatcctggtaacccggattgatggatccagccctaccttaaatggcaagacctaacccgaggctttttgcatcaaccaataaagtccttaagccagtttgagttggttttgtcacttgcagctaaaagaattctgactctaacaatgtgacaatagcaaaaataaacataactgcttttgaggtttctaatggattttcctccctatatacatgatttcatttaatcctcacaattcaggaaagcacatatctattaacattaaattaatattcattattttgaacacatgctatgtggataagggatgaggaaagccaaggaagtaatcaacgtgaaatctcacttatatgggagggaagtggaggttacatatctcagggcacttaacagatatcatcaaatgaaagaataaacagtgtgtgggagaggcagtaggtgattcttcatcaattcctggatgaaaaattaggagataatgaactccgaacaggcagcctaatgagaatggctcaagcaacaggacatagagagggagttaggttagacatggggttcttgggaattttcacctcgtgggggggcgggggggtcgtgcagctgttgtcagtgggaaagggaaaaaggaaaaggctgagtttggaaggcagggagggaggagacaatgtgagtcagtgaaaaagggcccttagaatgacaagtctggaccagagagaggctaagactgaaaatacaagttgggtaaccactggcatacagatggcagttcaggcttgggcactgcccaccagagcctcagcatgaagagaagagggggaggctggccaccacctccctctaggtaatcgtcatcctgatgctgagctcctgaaaacaggctctttcactcgccccatctcttgctcttgattgcaacccggcattcaggaggcaccctgtaatatctgtggagtgaccgacaacacagcgccagggcactgagaagatcccagggcgccagggactggttctacaagggtgcccctcccggtcccctccagcgcgccgccagagctgccagtcttggctgctacacgggaggcagcctcattatgcagctctcacctcttaaattagttcatgctctcacattaggtgtaatcacagcttgcaacgctttctggggatgtctcagaaagatctgagttgaaaaaatatttttgtgtcattttaatttaaagtaaaattgctgcttcttccccgcccctttctttcctcctggcccacccagcgaccctggccggccgtgctcaacgggggcgggggtcggaggtgagatttcctccacataattccttaaacagctatcaactaagtctcaaagaaaaaaaaaagagatctagaagcagagacgtggctgctggcgatcccaaagctggtgttcgctcttgggggagagcgtaccctgggggaggccgggaggccgggccagaggctagcccagaggcagagggcaggagcgctcagccggcgccccgcgtctctccagctcccgacgctgcgctggctccgctgagcacgccaggatcaaggtcgcctggtggggaccggagcgccaggagcctgtgggaagcgttccagccggcctctgactgggatccggcgccgcgtttctgctttggacttgactgacaggtccccccgccctcccgccgccctactaccagcctgggttcatccttcagggctacgtctaccgcacccgggctggaaagcctggagcgcgcccttcctctcctcatcttctcagctctcctttctccctgccacttggcaaagctgcattttgactttcacgttttggactacgtgtgtgtagttccaagtccatgcgtggcacgaaaatccacttagggtaaaaattattctcgaaaaatcgcccatctcaggatctggtgtctacactcaaggctaggaggtgcaggtacgggtgcgtaaagcatgccgtaagggtgcacagtaaataaaaagtacggatgcaaaatgtaaattttaagtgcaaaacagaaaagcagtactcgttgccgccccgcacgctgggttttaaggggcacgaaggtgggcctcggctgcttttgctcagccccgcgtcctcagcgcccggcccagtacccggtactccgtaggggttcaatgatctcccctgaataagtgaacgaattaacaaatgaatgaatgaccgctcgatccgacctccgcggccggcagagcagtcgctggagaggcgggagagagcgagaggccaagctccaccatcgcggccgccggctggggcagagggacacggagacactcggcgccccggctccgcaccgagtccccg

SEQ ID NO: 17588 - RNA, 14023 nt, Homo sapiens
  source 1..14023: mol_type = other RNA
tcaggccaggcacagtggctcatgcctgtagtcccagcactttgggaggccgaggtgggcagatccacgaggtcaggagatcaagaccatcctaacatggtaaaaccccatctctactaacaatacaaaaaattagtcaggtgtggtggcacgtgcctgtagtcccagctactcaggaggctgaggcaggagaatcgcttgaacctgggaggcggaggttgcagtgagccgagattgtgccactgcaccctagcctaggcaacagagcaagactctgtctcaaaaaaaataaaaaaaaaaaaaagagagaaagagagagagagatgaggagttgctgcactgctgggtgtggagagccgaggaggattcaaagatggtcctgaagtcccagctggaagaagtaggcggcagcaatgtttttaatactgtaaattcatcacgtagcacaggtttggggtggagaaagaaaaattgcattggcttcagggcatgcccagatctttcctcatcttaggcgtttgctaatacatgcattttctaagctgatgtcttgcgtttaatcactgctccattcaaaagagagaaggaggttgtttcaaacctagttgatatcatttgacttccatgctattcacagggctattttatttgaaacaggtataccacagccttaaattgcaagttaatccaggatgttcctaggttggcagttaggaacatgtaattctttggaagggctaaaagtcagctctttaaattatctccatatgaaccttctctccaccttagggtggatccacttatttagtccactgccagtaccacactagaacccgggtggtcactggactccagaaacaacagtagccctctctctgttctgtctctttttgactatctctattctgttcctgaccctgatttctcctgccaagctcaattttgacagctgacaacggcaagccatggcttcccaaaacattattttcaggtcaacttataaatttcaagaacacatttggctccgcttcctgtggtactaagcctacttcttgacagcatttgcctttgttgtaaatagcaaagttcttctagttggatttttgctaagaagtgtgtggatgtggcatgtgacgacatctttagcttggattctagaaaggcactaccattgtgcatttggctaaaggaaacacattttacccgtgaatgccttctatttacaaatgctcagctagcacacaaagctaagtacaagcaataagtactatcctacaatgttactcatttctgaaagcacaaaatgatgactggtatagctttggagatgttttctggaaacccaataaaggaacagatctttgttattccacacctacaaagtcagaagatgcacagtcttttattcatgtttgaacaagcttccttcttgaacaatcaactataaagtgatgtgattctctactagaccaggaactccttgaggacagaatgagggtctaatccatattctaaatccacaccacctggcacaatacatgttgcatggttagggtcaactaagagttggttgaattaatcaataacacacagcaagagaattcacaaagagaggggagtaatcccccagcctcaatcactcggcaagtggaatcgctgggcactgattccagctctgtctcagtgcttgagacagagctgaatgtaatgtgaacatttcaaatgaacaggaaaactagactcacggataagcagtgtagtcatcaagacaacactgtcttggaggtttttctgaagttaaaaccatgctacataagcaataaattatgaaggctgagcatgtgaataaaatttaatgttgtcataaattttataacaaagttaatctgacacatttaatgacatgcataatcattagtatgcagcactgtaatcagacattgataataagcagttcacaccagtgactgtaagagtctttacttgtgttcagccaagccaactgcttggtatatttttctcccttcttagtcgttagttttccatacctacaataactatcagtggtgatgggcttctctgaccatgtgaataatttaatcctcaatgcacagatacagaaacccttgctgaagacagtgtggagcagagaaggctgtctccactccttccacctgaaacacctctgcagatggatatgggagctctgcctacagcccttggacctaaccacttcagtgtgttccagtgagtgtctggacctcggcctgaaagatttttccgaaactaaagaaaatttctctgacctaaagaccttaacctccaccccagaagctctcaccaaggactacagggaactggtggggaaaatccttatcccttactcctcaaggcacagggcagtaatgctgaggcttgtgcgccacacttgctcccagaggtccccagcgggctacctgcggtggtgaatgacctcctaacacgccccttgacggccttcctttccttgcctcacttctccactctcctaccagcattgcagggttcacatcccaaatataccactggcacttgaatcctggtctccaggtctgtttctggaaaaacccaagtaagacattgccccagtaatggggctagatgtctgaggcttcctcaagtatctacctcgaaagctcttactgctgtacacacatgcacatacacacacgtgcgtacaaccagtcacatctaagcaccccgaataccagcctgttgaaggtagcagagagctgcactataagccaaggctgctcccaagagccgctccatcactgaattggcgccccagcaagatgaaggaatgtaatcattggaaggatggagaatgttctctgaatcactgacaaattggaaggggtggagggcaagagtccacctggtggagagatggaaagagcgagagagcctggaatgataatgccattgcttagaaaaggctgctccagatgccatatctacagaaattgtacagcccaaacatctctgagcaataggtctctggtagtcttgatgtctagaccaacaattcccagttcattcttctcagggaaggagccaggatagtccagagactctcattctgctgttagattgaaagggttaggcacaacagccttggcaaagtcacaagggcaaattcacactaaagtgtaaatgacccacaactcctcttctatttttaggttggggaggtgctttagaacataaggaggaactaaagaatattcctgttacatacaaggcagagaaaagggaaactagtggtgacaagacaaatcatccctttgacatttggctggctctacctattacagctctgggggtgaggtgggaacaaaaagatgctgtgtaaagaagtatcttatgccatccctactgtagtgaggtgcagtttagaggggacactgatcaagcagagacccagagtgtttcgttccaagccagaaacagaaatgtataaaacacagcctttccagcatcagaaatgagtagtggtagtggagaactacccaaaacaggaaagaggaccacgtgaggtagagtgtcaaggccctacattccagtgcctctgctcatgactgtaattttgggtaggtcacttaaagtctctggacctcagttttgccatctgtgaaatagggataatactatccagcataaaattggttatgaggctcatgtagggcctgcctgggatgatgtgttgctaatggttaagaacacaacttctggggtctgactggacaggctgaaatccctgcttaacacgttccagcagagccctgggcgatctatttaacttttgttttctcacctgtaagctgagacgaaagtacccactttataagattattccaataattagttgaaataatgcatgcagagaattaagcatggtacttgttatttgttaaactagctattaaaatgtgtaaaatataaagtattgtatggattttaggacaatgcaaagactctttgcttgctgcaatagttcggggccctttcagatggctaaaggcagaatttgtatgtgtaaatatggtgtgcttgtctctgctctggatactgagggcttaccctgttattaaacttatttagtaaatattgaactgtcatgaggcctaacatttagttccagttattagataaaacatttgctttgaatggtatttgaattgccaggttctagattattctggttgacaaactcttcgtattttataaagaggctaaaattggtaagctatcacagaacagatgtgccattttcaaggtatattaaaccatgattcactgtaacattgttcctactggcaacaaattcagagcaggctggactttatttggtgaagaaacattgagtggaagagaaatgacattattttatgtatttacattttcaaattactgtggcttaaacctgttcagccaacattacccaccttcagtctgctaaataaatgattcagtacatttctaatttacagaattttttaacaaaagaaaatgtaatttgatagccaaatcaacgttaaacattatacatttaaaaaaccacaggcaaagacacaaacatgatgacactaacttttgttaaagtatgcttacctatggtttcctctgaggcacgttctttcatgctaagcttccaacataatatgaaaatgaaggagatgcattttgcaaagcaaaacagaccttaagcaaaatattatacttctcaaattaacactgttacaaagttttagaatttaataagttcattaatttaaaagtttggatgtctgagtccttctatcccaaaacaagatcttggagggtcttccacagccatgtaataccatggtcacatgaccctttccaaaattattaatctgaatttactatatgaggataaatctatctttttgaaaatatttaggaaaatgagcttggtatttataaaatgaagctctctttgggtggtatcctaagacacgtcaagccaatcagcctgtaactgtgaaaaaaacattggtaggtacaaaagtggggtgggagaggagtgacttaactttgttaagtgatgggaaagaaacactaatagcattatctcaataaaatgtgatttaaaaaaatttaaaatactaaatcattgaactgacaaagaaatataaatcattcagaaataaactcattaggtcatcaaatcctgttaaatctgcaattaggaagagcaaggtgtacaatccatacatttaaactcacaggctcactttgcacaacgtcaatttactccttaatatgttattaatacgcattttccaaaaggatgtattagtaaatggtacacatctacttcttggcaacatcatataacctggtacaacataagcattcttcttatagttaagaaatgtggatggtatcaaaattagaaaaataaatgccctattatgttgtggtcaggtttaaggcatgtgaattttatcttcatacaaaagattaaaatctagatattaaaaagtagtgcagtatcagtgatgctgcctcagttcccaaaatgtcacatcacaaaaatatcccataattgcctgtagtttattccttggctttcctcttttctctctgcatctttgtaacaattttttaaaagtggaaatataattgttggcaatgctaacagctgtagaaatgattacaagatgtggaaaagcataacaggaatgtcaagaatctgtttctggcagtaatatatatggaacattgttcaggacaaaagaggagaaggaagaaaaaaaggagaggggtttatcatctctaagaattttcaaactaaacctcattgcttaataggaaaaaaagattccatatttaaagttaagtcacctctaactactagctaaagcatgacatcaccagcactggagtcagcggaagtgtgtttttgaaggacagtgttgcaggagaatctggacaggttttagagccaggagagagaaaataattctacctctgacagttgaaggaccttaggcaaatcagtttacctctgctagactacactccaaaatttggacattcaaaaatttgatattaataaccacatgaaagtctcgtgttgaggtgaatatgtatttgttggtgaaagatatgttggtttttaaacagacagcactctgcaattgtaggctattgttttgttttgccagttgtcaaattctatccagctatacacacttgtgtggcctcctaatggtgtttttccagtggctaaaggtttatgaataagacacttttcctaatggaattaacccgatgcttttcttaaacatgtaaccttgagttcaccgcaaaaaacaatgcttcgattagagcaatgcatataataaaggttaccctcgtttcttagacactagacatcattcacaaaaagagaactgcttttgaaagggatgtatttgcactggaaagaatagttttctacttctaattataaatgatttattggtgaaagcaaaacaacagcctgtctgagaggcacttctatgagcatcctcacgtgtgatttgcaaggttgaagaagagggaaaaatgcctcaattgtaccaatggtgagaaaacacccaaagtacaaagcaggtttcaaaaaaaccatactcataaccaaggacaataataaagcaatgtgttgacatatactctataagtcttcctccataaatagtttatagaaattttgtaatttctgtaaatgcatcctataataattttgcatcttgctttttttttacatttaatatcaagtagatttctaaagggcaattatttgaaaattatcccaaatacatggggaaatatacatcaagtgaaaaaatgcagtgggtgatagagatatcaggaagcgcctcaaatatttctcatctcgttggagaaaaacaaacatgttctcatttagaatgagtgggagttacctaattgatttaggcctctatatttaacttctagtcaaaaaaggtagttctatctagcaacaatattatggggaacaaaagaaaaaattaactctctaaatttgcagtagggtcttttcttcagaagtaccaaatcccatctattaccagctccatgcttcaggcctaaaatggatctccctgaagcaatgacagaatttttgccaagtgactaggatataaacaccactttggttgcacagtgagacatatgctccaaagaaaactggttcaaaaacaggcaagtgggtttctacagaataaatgagagccctgtcaatggcttcatcttcagggctttgtgtctgtgcttgcgtggtggctcttgtttcatctatggataatggtggcacacagttttcataattccttacattaatgaactgctataaatttgtttttggtattctagagagtcctaacttcagcttctgggcaatgctgaggaggcaccctatattctagacttaccttttgcaaggtgtactctcagcattgtgggcgatttccatgggagaatattctatttaaagaactactgtcccagcataaaacaaaaaatcatttatgaagatgcaggagactcggaaagctctcaattattgtttgcacaagcacaatgtcacagcctcctttccccattccacaagggggtcaggaagagagtactcagctgtgagaaaagacatacagaagaattcatgtggtcatgagagcgaggacatggccgatcccccaaggaggatgtgtcatacacttcatgagcccaagagtgtgctgtagggtctgaagggcaagatgctggttcactgatgtaaaggagagggaaaaaagcttcaaccaactagaaaaacagtctctatgcatgctatttttgattttaaacacaggtatcaattccttctctcagagagtccattttaaaataggatacatttttaaaggaatatttaaaggacacattcattaaaatttattttaaaaacttttcaaaagaaacaaaaggtatgaattttatttaatccttgaggaaatggttcttttctcacacacataaatcactcattttgtttttctttatctcctttattaatctacattagaaaaataaacttttcatacactaagaacaaggaaaccactctcaattgacaaaatgttccaatccaacacaatgattactttcacctttaatttacaggcagccagattcaaaatccttaaagttgcttaaacttaaaaatgacaatgacaacctaaaaggtataatgttgattggaacagacatttaattggaaaattgatgattttccatttccaattaaatctctagatagaaatgaaaaaaattaaaaatcgtatttaagaaaagccaaatcttgggttgtgaggtatctttttaaggatgtttcagcagaaaaaaacaaaggctctcacaattgtgtagctgcctagattaagtgggtatcctgatcaaggagatgggggatgatttggctttagtattccaatgataaagtttataatgagaataacatgttgctacaaaatccagtctcttcctcagatgccttccacagagggcaggaagctttgtcagttttgtttgctgatgatgcctggttccgtcaacaaataacacctgtcacacggtgggtagtcaatatacatttgttgaataaatatgaaaaaaagaaatgtacaatatgtttgtgaagccaactgtgtgtgcattgctattgaggtacacaaaaagtctttgttttaaatttgagaatgaggactttcaatggaatatatctataaaaatgaaaaaaagacattactgtctggacttttgtacagcaagagaagaaaaaccactagccaagagccaactcacctgataggcctggatcaagcatgcagctgtggagaacacccctgggactctaactctggcactctgcaagctgggtacttgggcaggacagcagcagcactcatgaactgggcagcacctctcttcaagtggtatttaaatttcttctttcattttccttctggtaacaaagaagtctgtggctcaaaagatgtttctctaagaccccatcctattaggtctctgagctgtgggaagtatttatacaattgcttgtgaatataagatccaggaatttccctaagatccctaacaaaattggtgataagtagtcccacatgttaatccagccacccacggatgacagcacttaccatttctttgataaatgtcaaatgcatttgaagtacctacctgaaatatttgtttaaatgctatctaatctattaattttatatatgtgtgagtctgttttgtataccttctgattataggataaatgtaaataaatccaaagagtaatcaaagctaccactttcaagaagccttctttgtagaaccggaagagtcttaaataggcttttcaggtatgcatctcttattatcgctgaactccaagtcctgcaaggcaggcatcatgtgtgggtcacctttacagtaggcacaggccttaaaacagtgacatgcacattgcaggcactccataaatgtttgctgaattggctaaaccttggtttgttcccataatcaaccaccacaaacagcacacagataattacttcttggaaagattccaactagtgtttgatgttacctacgtggtttttctctcaagatcttaagagcagctctgtaggattacattattttctgttttttttttcctttgaccttaatgtcatctacttcaataacagcttcatacaaaattcctaccagcacataccacagcagattcaaggccttgttttaaaaatggtgccagcttctcttaatttggaagatatattgtctctcctgaacatgggctaagaaaatgtataatttggtattaacataagagctgaagacactttaaatgcattgtttcatttttataagataaaaaaaattttaagaatcaaaatgttatcaacagacttgtccttcattaaaaagtaaaactgcatttgcctacattttatgaaagtgtccaattatgaacaattttgaaatgtaacttttaaaaatgtaaacagcaaaaatgttgtatttaaaataaatctggaaaggcagaaaaacaaaaaatacccagaagacagagtttttggtgaaagttaagatatttcatctttgaacaacttagaatctttcctgcattttatagtctagttccaggcattaatttgaaataaccttggaatcctaaatctaacacccttcggaacaaagtagcttttctcttctgctttatgagcaaatggactaaatactagggaatggtactgtctgggcctttgaaccaagattgaaagagatgaaatcctatatgatatgtataaacattagagaatccattttgatttaataaaaggttgaatttgttctatatcctgtgagaaaatggttcccttttcctgaaaatgttacctcattccaacaatagaaagttggtttttttccagggtgtggtgttggcgggggacagagttgccatgaatatggcatctatgaagactgctgttatattcatttctcaaaatgcactgtggtaggaaattcagaacgcagtgagagaaaataaatgtttgacttcaaaatataaggccgcatttaaagcagaaggtaaagtatagaacagttgacagtataaattctttatctgcaatcttgcagttccctaaatctctgtaacacatcacttttaaaagcctcagataagtggttctataataatttaccaataattcaacccctcaaaagtcttagcaagttaaaccttataatcttacattttagaaatgacccaacttgatccttttattcttcagaatatctctctcaaattttcatttgtttttcattaattgatgaataatgagacattttaggtacctgtccacaaagaaatgaaattttcactttccaggaacctaacaaatgaaaagatagaaatcaattccaacagaatattaccaaagaaatcttttagaatggactgttaaaattatttatttgtatttatctggctctactatttgtggtacatttccacttcaaagctaaacctcaaataacatcatagtgagtggttgacttcatgtttaactgagatcttgaagactgaaaaagaccacgacaaacacacatctattttcttggctactgcatccgtgttcatcaccattctgatagtctgcaatgtattgcagctcaccctttgggaaggactaaagtagacatctgtttgttctgcttactcagcattcctaccctaattttcctttggagaacccctttattctagaccacgtgaagctaatgccaaaccccattccaggggatgcacctgaatccaacctccatcatctaaacagtgccttctccacgttcagagaagagcaagtgactcaaactgccctcataagaacagacctgggacttctgctgcaaatattgaagagtaagtactcttttttcttgctaggactaagctggtagtaccttctatgaggctatcatatggaaacaacttgtctgaaaatgaagccacaactagaaaacagatcctggtaacccggattgatggatccagccctaccttaaatggcaagacctaacccgaggctttttgcatcaaccaataaagtccttaagccagtttgagttggttttgtcacttgcagctaaaagaattctgactctaacaatgtgacaatagcaaaaataaacataactgcttttgaggtttctaatggattttcctccctatatacatgatttcatttaatcctcacaattcaggaaagcacatatctattaacattaaattaatattcattattttgaacacatgctatgtggataagggatgaggaaagccaaggaagtaatcaacgtgaaatctcacttatatgggagggaagtggaggttacatatctcagggcacttaacagatatcatcaaatgaaagaataaacagtgtgtgggagaggcagtaggtgattcttcatcaattcctggatgaaaaattaggagataatgaactccgaacaggcagcctaatgagaatggctcaagcaacaggacatagagagggagttaggttagacatggggttcttgggaattttcacctcgtgggggggcgggggggtcgtgcagctgttgtcagtgggaaagggaaaaaggaaaaggctgagtttggaaggcagggagggaggagacaatgtgagtcagtgaaaaagggcccttagaatgacaagtctggaccagagagaggctaagactgaaaatacaagttgggtaaccactggcatacagatggcagttcaggcttgggcactgcccaccagagcctcagcatgaagagaagagggggaggctggccaccacctccctctaggtaatcgtcatcctgatgctgagctcctgaaaacaggctctttcactcgccccatctcttgctcttgattgcaacccggcattcaggaggcaccctgtaatatctgtggagtgaccgacaacacagcgccagggcactgagaagatcccagggcgccagggactggttctacaagggtgcccctcccggtcccctccagcgcgccgccagagctgccagtcttggctgctacacgggaggcagcctcattatgcagctctcacctcttaaattagttcatgctctcacattaggtgtaatcacagcttgcaacgctttctggggatgtctcagaaagatctgagttgaaaaaatatttttgtgtcattttaatttaaagtaaaattgctgcttcttccccgcccctttctttcctcctggcccacccagcgaccctggccggccgtgctcaacgggggcgggggtcggaggtgagatttcctccacataattccttaaacagctatcaactaagtctcaaagaaaaaaaaaagagatctagaagcagagacgtggctgctggcgatcccaaagctggtgttcgctcttgggggagagcgtaccctgggggaggccgggaggccgggccagaggctagcccagaggcagagggcaggagcgctcagccggcgccccgcgtctctccagctcccgacgctgcgctggctccgctgagcacgccaggatcaaggtcgcctggtggggaccggagcgccaggagcctgtgggaagcgttccagccggcctctgactgggatccggcgccgcgtttctgctttggacttgactgacaggtccccccgccctcccgccgccctactaccagcctgggttcatccttcagggctacgtctaccgcacccgggctggaaagcctggagcgcgcccttcctctcctcatcttctcagctctcctttctccctgccacttggcaaagctgcattttgactttcacgttttggactacgtgtgtgtagttccaagtccatgcgtggcacgaaaatccacttagggtaaaaattattctcgaaaaatcgcccatctcaggatctggtgtctacactcaaggctaggaggtgcaggtacgggtgcgtaaagcatgccgtaagggtgcacagtaaataaaaagtacggatgcaaaatgtaaattttaagtgcaaaacagaaaagcagtactcgttgccgccccgcacgctgggttttaaggggcacgaaggtgggcctcggctgcttttgctcagccccgcgtcctcagcgcccggcccagtacccggtactccgtaggggttcaatgatctcccctgaataagtgaacgaattaacaaatgaatgaatgaccgctcgatccgacctccgcggccggcagagcagtcgctggagaggcgggagagagcgagaggccaagctccaccatcgcggccgccggctggggcagagggacacggagacactcggcgccccggctccgcaccgagtccccg

SEQ ID NO: 17589 - RNA, 11139 nt, Homo sapiens
  source 1..11139: mol_type = other RNA
tcaggccaggcacagtggctcatgcctgtagtcccagcactttgggaggccgaggtgggcagatccacgaggtcaggagatcaagaccatcctaacatggtaaaaccccatctctactaacaatacaaaaaattagtcaggtgtggtggcacgtgcctgtagtcccagctactcaggaggctgaggcaggagaatcgcttgaacctgggaggcggaggttgcagtgagccgagattgtgccactgcaccctagcctaggcaacagagcaagactctgtctcaaaaaaaataaaaaaaaaaaaaagagagaaagagagagagagatgaggagttgctgcactgctgggtgtggagagccgaggaggattcaaagatggtcctgaagtcccagctggaagaagtaggcggcagcaatgtttttaatactgtaaattcatcacgtagcacaggtttggggtggagaaagaaaaattgcattggcttcagggcatgcccagatctttcctcatcttaggcgtttgctaatacatgcattttctaagctgatgtcttgcgtttaatcactgctccattcaaaagagagaaggaggttgtttcaaacctagttgatatcatttgacttccatgctattcacagggctattttatttgaaacaggtataccacagccttaaattgcaagttaatccaggatgttcctaggttggcagttaggaacatgtaattctttggaagggctaaaagtcagctctttaaattatctccatatgaaccttctctccaccttagggtggatccacttatttagtccactgccagtaccacactagaacccgggtggtcactggactccagaaacaacagtagccctctctctgttctgtctctttttgactatctctattctgttcctgaccctgatttctcctgccaagctcaattttgacagctgacaacggcaagccatggcttcccaaaacattattttcaggtcaacttataaatttcaagaacacatttggctccgcttcctgtggtactaagcctacttcttgacagcatttgcctttgttgtaaatagcaaagttcttctagttggatttttgctaagaagtgtgtggatgtggcatgtgacgacatctttagcttggattctagaaaggcactaccattgtgcatttggctaaaggaaacacattttacccgtgaatgccttctatttacaaatgctcagctagcacacaaagctaagtacaagcaataagtactatcctacaatgttactcatttctgaaagcacaaaatgatgactggtatagctttggagatgttttctggaaacccaataaaggaacagatctttgttattccacacctacaaagtcagaagatgcacagtcttttattcatgtttgaacaagcttccttcttgaacaatcaactataaagtgatgtgattctctactagaccaggaactccttgaggacagaatgagggtctaatccatattctaaatccacaccacctggcacaatacatgttgcatggttagggtcaactaagagttggttgaattaatcaataacacacagcaagagaattcacaaagagaggggagtaatcccccagcctcaatcactcggcaagtggaatcgctgggcactgattccagctctgtctcagtgcttgagacagagctgaatgtaatgtgaacatttcaaatgaacaggaaaactagactcacggataagcagtgtagtcatcaagacaacactgtcttggaggtttttctgaagttaaaaccatgctacataagcaataaattatgaaggctgagcatgtgaataaaatttaatgttgtcataaattttataacaaagttaatctgacacatttaatgacatgcataatcattagtatgcagcactgtaatcagacattgataataagcagttcacaccagtgactgtaagagtctttacttgtgttcagccaagccaactgcttggtatatttttctcccttcttagtcgttagttttccatacctacaataactatcagtggtgatgggcttctctgaccatgtgaataatttaatcctcaatgcacagatacagaaacccttgctgaagacagtgtggagcagagaaggctgtctccactccttccacctgaaacacctctgcagatggatatgggagctctgcctacagcccttggacctaaccacttcagtgtgttccagtgagtgtctggacctcggcctgaaagatttttccgaaactaaagaaaatttctctgacctaaagaccttaacctccaccccagaagctctcaccaaggactacagggaactggtggggaaaatccttatcccttactcctcaaggcacagggcagtaatgctgaggcttgtgcgccacacttgctcccagaggtccccagcgggctacctgcggtggtgaatgacctcctaacacgccccttgacggccttcctttccttgcctcacttctccactctcctaccagcattgcagggttcacatcccaaatataccactggcacttgaatcctggtctccaggtctgtttctggaaaaacccaagtaagacattgccccagtaatggggctagatgtctgaggcttcctcaagtatctacctcgaaagctcttactgctgtacacacatgcacatacacacacgtgcgtacaaccagtcacatctaagcaccccgaataccagcctgttgaaggtagcagagagctgcactataagccaaggctgctcccaagagccgctccatcactgaattggcgccccagcaagatgaaggaatgtaatcattggaaggatggagaatgttctctgaatcactgacaaattggaaggggtggagggcaagagtccacctggtggagagatggaaagagcgagagagcctggaatgataatgccattgcttagaaaaggctgctccagatgccatatctacagaaattgtacagcccaaacatctctgagcaataggtctctggtagtcttgatgtctagaccaacaattcccagttcattcttctcagggaaggagccaggatagtccagagactctcattctgctgttagattgaaagggttaggcacaacagccttggcaaagtcacaagggcaaattcacactaaagtgtaaatgacccacaactcctcttctatttttaggttggggaggtgctttagaacataaggaggaactaaagaatattcctgttacatacaaggcagagaaaagggaaactagtggtgacaagacaaatcatccctttgacatttggctggctctacctattacagctctgggggtgaggtgggaacaaaaagatgctgtgtaaagaagtatcttatgccatccctactgtagtgaggtgcagtttagaggggacactgatcaagcagagacccagagtgtttcgttccaagccagaaacagaaatgtataaaacacagcctttccagcatcagaaatgagtagtggtagtggagaactacccaaaacaggaaagaggaccacgtgaggtagagtgtcaaggccctacattccagtgcctctgctcatgactgtaattttgggtaggtcacttaaagtctctggacctcagttttgccatctgtgaaatagggataatactatccagcataaaattggttatgaggctcatgtagggcctgcctgggatgatgtgttgctaatggttaagaacacaacttctggggtctgactggacaggctgaaatccctgcttaacacgttccagcagagccctgggcgatctatttaacttttgttttctcacctgtaagctgagacgaaagtacccactttataagattattccaataattagttgaaataatgcatgcagagaattaagcatggtacttgttatttgttaaactagctattaaaatgtgtaaaatataaagtattgtatggattttaggacaatgcaaagactctttgcttgctgcaatagttcggggccctttcagatggctaaaggcagaatttgtatgtgtaaatatggtgtgcttgtctctgctctggatactgagggcttaccctgttattaaacttatttagtaaatattgaactgtcatgaggcctaacatttagttccagttattagataaaacatttgctttgaatggtatttgaattgccaggttctagattattctggttgacaaactcttcgtattttataaagaggctaaaattggtaagctatcacagaacagatgtgccattttcaaggtatattaaaccatgattcactgtaacattgttcctactggcaacaaattcagagcaggctggactttatttggtgaagaaacattgagtggaagagaaatgacattattttatgtatttacattttcaaattactgtggcttaaacctgttcagccaacattacccaccttcagtctgctaaataaatgattcagtacatttctaatttacagaattttttaacaaaagaaaatgtaatttgatagccaaatcaacgttaaacattatacatttaaaaaaccacaggcaaagacacaaacatgatgacactaacttttgttaaagtatgcttacctatggtttcctctgaggcacgttctttcatgctaagcttccaacataatatgaaaatgaaggagatgcattttgcaaagcaaaacagaccttaagcaaaatattatacttctcaaattaacactgttacaaagttttagaatttaataagttcattaatttaaaagtttggatgtctgagtccttctatcccaaaacaagatcttggagggtcttccacagccatgtaataccatggtcacatgaccctttccaaaattattaatctgaatttactatatgaggataaatctatctttttgaaaatatttaggaaaatgagcttggtatttataaaatgaagctctctttgggtggtatcctaagacacgtcaagccaatcagcctgtaactgtgaaaaaaacattggtaggtacaaaagtggggtgggagaggagtgacttaactttgttaagtgatgggaaagaaacactaatagcattatctcaataaaatgtgatttaaaaaaatttaaaatactaaatcattgaactgacaaagaaatataaatcattcagaaataaactcattaggtcatcaaatcctgttaaatctgcaattaggaagagcaaggtgtacaatccatacatttaaactcacaggctcactttgcacaacgtcaatttactccttaatatgttattaatacgcattttccaaaaggatgtattagtaaatggtacacatctacttcttggcaacatcatataacctggtacaacataagcattcttcttatagttaagaaatgtggatggtatcaaaattagaaaaataaatgccctattatgttgtggtcaggtttaaggcatgtgaattttatcttcatacaaaagattaaaatctagatattaaaaagtagtgcagtatcagtgatgctgcctcagttcccaaaatgtcacatcacaaaaatatcccataattgcctgtagtttattccttggctttcctcttttctctctgcatctttgtaacaattttttaaaagtggaaatataattgttggcaatgctaacagctgtagaaatgattacaagatgtggaaaagcataacaggaatgtcaagaatctgtttctggcagtaatatatatggaacattgttcaggacaaaagaggagaaggaagaaaaaaaggagaggggtttatcatctctaagaattttcaaactaaacctcattgcttaataggaaaaaaagattccatatttaaagttaagtcacctctaactactagctaaagcatgacatcaccagcactggagtcagcggaagtgtgtttttgaaggacagtgttgcaggagaatctggacaggttttagagccaggagagagaaaataattctacctctgacagttgaaggaccttaggcaaatcagtttacctctgctagactacactccaaaatttggacattcaaaaatttgatattaataaccacatgaaagtctcgtgttgaggtgaatatgtatttgttggtgaaagatatgttggtttttaaacagacagcactctgcaattgtaggctattgttttgttttgccagttgtcaaattctatccagctatacacacttgtgtggcctcctaatggtgtttttccagtggctaaaggtttatgaataagacacttttcctaatggaattaacccgatgcttttcttaaacatgtaaccttgagttcaccgcaaaaaacaatgcttcgattagagcaatgcatataataaaggttaccctcgtttcttagacactagacatcattcacaaaaagagaactgcttttgaaagggatgtatttgcactggaaagaatagttttctacttctaattataaatgatttattggtgaaagcaaaacaacagcctgtctgagaggcacttctatgagcatcctcacgtgtgatttgcaaggttgaagaagagggaaaaatgcctcaattgtaccaatggtgagaaaacacccaaagtacaaagcaggtttcaaaaaaaccatactcataaccaaggacaataataaagcaatgtgttgacatatactctataagtcttcctccataaatagtttatagaaattttgtaatttctgtaaatgcatcctataataattttgcatcttgctttttttttacatttaatatcaagtagatttctaaagggcaattatttgaaaattatcccaaatacatggggaaatatacatcaagtgaaaaaatgcagtgggtgatagagatatcaggaagcgcctcaaatatttctcatctcgttggagaaaaacaaacatgttctcatttagaatgagtgggagttacctaattgatttaggcctctatatttaacttctagtcaaaaaaggtagttctatctagcaacaatattatggggaacaaaagaaaaaattaactctctaaatttgcagtagggtcttttcttcagaagtaccaaatcccatctattaccagctccatgcttcaggcctaaaatggatctccctgaagcaatgacagaatttttgccaagtgactaggatataaacaccactttggttgcacagtgagacatatgctccaaagaaaactggttcaaaaacaggcaagtgggtttctacagaataaatgagagccctgtcaatggcttcatcttcagggctttgtgtctgtgcttgcgtggtggctcttgtttcatctatggataatggtggcacacagttttcataattccttacattaatgaactgctataaatttgtttttggtattctagagagtcctaacttcagcttctgggcaatgctgaggaggcaccctatattctagacttaccttttgcaaggtgtactctcagcattgtgggcgatttccatgggagaatattctatttaaagaactactgtcccagcataaaacaaaaaatcatttatgaagatgcaggagactcggaaagctctcaattattgtttgcacaagcacaatgtcacagcctcctttccccattccacaagggggtcaggaagagagtactcagctgtgagaaaagacatacagaagaattcatgtggtcatgagagcgaggacatggccgatcccccaaggaggatgtgtcatacacttcatgagcccaagagtgtgctgtagggtctgaagggcaagatgctggttcactgatgtaaaggagagggaaaaaagcttcaaccaactagaaaaacagtctctatgcatgctatttttgattttaaacacaggtatcaattccttctctcagagagtccattttaaaataggatacatttttaaaggaatatttaaaggacacattcattaaaatttattttaaaaacttttcaaaagaaacaaaaggtatgaattttatttaatccttgaggaaatggttcttttctcacacacataaatcactcattttgtttttctttatctcctttattaatctacattagaaaaataaacttttcatacactaagaacaaggaaaccactctcaattgacaaaatgttccaatccaacacaatgattactttcacctttaatttacaggcagccagattcaaaatccttaaagttgcttaaacttaaaaatgacaatgacaacctaaaaggtataatgttgattggaacagacatttaattggaaaattgatgattttccatttccaattaaatctctagatagaaatgaaaaaaattaaaaatcgtatttaagaaaagccaaatcttgggttgtgaggtatctttttaaggatgtttcagcagaaaaaaacaaaggctctcacaattgtgtagctgcctagattaagtgggtatcctgatcaaggagatgggggatgatttggctttagtattccaatgataaagtttataatgagaataacatgttgctacaaaatccagtctcttcctcagatgccttccacagagggcaggaagctttgtcagttttgtttgctgatgatgcctggttccgtcaacaaataacacctgtcacacggtgggtagtcaatatacatttgttgaataaatatgaaaaaaagaaatgtacaatatgtttgtgaagccaactgtgtgtgcattgctattgaggtacacaaaaagtctttgttttaaatttgagaatgaggactttcaatggaatatatctataaaaatgaaaaaaagacattactgtctggacttttgtacagcaagagaagaaaaaccactagccaagagccaactcacctgataggcctggatcaagcatgcagctgtggagaacacccctgggactctaactctggcactctgcaagctgggtacttgggcaggacagcagcagcactcatgaactgggcagcacctgttggtgagggctgatcacatggattctctcatcccagccttacaatcagtccttcaggtacatactttttctgactttgctgatgaggaaactatgcacagaggttacacagcttaacaaagggttctcacctaatgaacaatgaaatgggattttagcctttctttgcatctggtcttagagccaatacccaagaagcactgtactgtatgcattgtctcagagaaacttactcttcctgggcctcagtctttaaaaggtgggcagttgacttaataagaattaaagatcaatgattaaggttcaaggcactccaaaattctggtctttattgaaaaggctacagaagtctcaccttaataataccctatagacttgatattcttggttaattaaatattggaaaccaatttcatagtaattgaggtcagaaaaaagtactcatgacattttagaatatgatgacaaagccatagataaatttcaatgcacctgtaattacttaaaactgttatagcatgcaatgtgttaccacaacagccagagaaatactaatttactcagcctattcttctagaccagtaaacactaggattaaatagatattttcattgaatttgttctacccttcattgccatttatagatagcttacttgtcatagattactttctaattgttttatgtttcctaactagcctgcaatactttggcaaggacctcaaacaatagtagacagtaggtgtaaaatagatggctacattgaacagatgactaaaaggatgcctcctaagtacctatatcttgaaatatatattattgtgccttgctttcaatttgtgattttaaaatctagaaatcacctgttttatgtaataacaataaaatccttctttgttgaaaacatgcacaaataaagtttacaagctcaaaaaattaaacagcagtaacggtcaagctttccaacaataaaatacattttggtaaggttttcattttacaaaaactcaaaatagctttatgagttcacaaaataatatgatatttttcaagatattaacatattcttataccggaagagcatagaataaaatttacttggagattgagcatttgcttctttaagaaatacttcttttagtatttttactttaatattatgaaagctacataattacattcagattcattaactactccagtagttaatttttaaaacttatgatgaatagttttgtttaaaatatataacattggtaatatgcaaatctgaatctgtaataaagaaggatttgcattcctgatttttttttctgatacaaccaatgacaaaataactaatggttccacagaggataaaatgtctcaaatctgttggttctgaaggtgaagcgagatttttgtactgataccgtgtatcactgagataccaggaggaaatggaattaaactcagatagttcaaatggagagattttaatgaagggacgacctacagaggtgtcggcagggttggggggaatcagcgagatatgcttagaacccaccgactggcaaacctccccctgaagatggagaaggaggaaggagtgttactggaatgagagcttgagtccaggggaggaggatgggctgctgaggaggcgacaccatcctgaaagaagaatcctctgccagaggcttttcagggtcatttcttcacactctctctcttcaagtggtatttaaatttcttctttcattttccttctggtaacaaagaagtctgtggctcaaaagatgtttctctaagaccccatcctattaggtctctgagattttagaaatgacccaacttgatccttttattcttcagaatatctctctcaaattttcatttgtttttcattaattgatgaataatgagacattttaggtacctgagggccgacgagtgggggcgggcaggagggccgagggaggcggaacaggatcgaggcgcgaggcgggagtcgagaaagcgagcggccgaggcgactctcagtgcgcggacgcgggcgcgcgcccgcgctcccttcgtcgactcacggcgagagcccaaccctgctgccgcgcgccaccc

SEQ ID NO: 17590 - RNA, 13988 nt, Homo sapiens
  source 1..13988: mol_type = other RNA
tcaggccaggcacagtggctcatgcctgtagtcccagcactttgggaggccgaggtgggcagatccacgaggtcaggagatcaagaccatcctaacatggtaaaaccccatctctactaacaatacaaaaaattagtcaggtgtggtggcacgtgcctgtagtcccagctactcaggaggctgaggcaggagaatcgcttgaacctgggaggcggaggttgcagtgagccgagattgtgccactgcaccctagcctaggcaacagagcaagactctgtctcaaaaaaaataaaaaaaaaaaaaagagagaaagagagagagagatgaggagttgctgcactgctgggtgtggagagccgaggaggattcaaagatggtcctgaagtcccagctggaagaagtaggcggcagcaatgtttttaatactgtaaattcatcacgtagcacaggtttggggtggagaaagaaaaattgcattggcttcagggcatgcccagatctttcctcatcttaggcgtttgctaatacatgcattttctaagctgatgtcttgcgtttaatcactgctccattcaaaagagagaaggaggttgtttcaaacctagttgatatcatttgacttccatgctattcacagggctattttatttgaaacaggtataccacagccttaaattgcaagttaatccaggatgttcctaggttggcagttaggaacatgtaattctttggaagggctaaaagtcagctctttaaattatctccatatgaaccttctctccaccttagggtggatccacttatttagtccactgccagtaccacactagaacccgggtggtcactggactccagaaacaacagtagccctctctctgttctgtctctttttgactatctctattctgttcctgaccctgatttctcctgccaagctcaattttgacagctgacaacggcaagccatggcttcccaaaacattattttcaggtcaacttataaatttcaagaacacatttggctccgcttcctgtggtactaagcctacttcttgacagcatttgcctttgttgtaaatagcaaagttcttctagttggatttttgctaagaagtgtgtggatgtggcatgtgacgacatctttagcttggattctagaaaggcactaccattgtgcatttggctaaaggaaacacattttacccgtgaatgccttctatttacaaatgctcagctagcacacaaagctaagtacaagcaataagtactatcctacaatgttactcatttctgaaagcacaaaatgatgactggtatagctttggagatgttttctggaaacccaataaaggaacagatctttgttattccacacctacaaagtcagaagatgcacagtcttttattcatgtttgaacaagcttccttcttgaacaatcaactataaagtgatgtgattctctactagaccaggaactccttgaggacagaatgagggtctaatccatattctaaatccacaccacctggcacaatacatgttgcatggttagggtcaactaagagttggttgaattaatcaataacacacagcaagagaattcacaaagagaggggagtaatcccccagcctcaatcactcggcaagtggaatcgctgggcactgattccagctctgtctcagtgcttgagacagagctgaatgtaatgtgaacatttcaaatgaacaggaaaactagactcacggataagcagtgtagtcatcaagacaacactgtcttggaggtttttctgaagttaaaaccatgctacataagcaataaattatgaaggctgagcatgtgaataaaatttaatgttgtcataaattttataacaaagttaatctgacacatttaatgacatgcataatcattagtatgcagcactgtaatcagacattgataataagcagttcacaccagtgactgtaagagtctttacttgtgttcagccaagccaactgcttggtatatttttctcccttcttagtcgttagttttccatacctacaataactatcagtggtgatgggcttctctgaccatgtgaataatttaatcctcaatgcacagatacagaaacccttgctgaagacagtgtggagcagagaaggctgtctccactccttccacctgaaacacctctgcagatggatatgggagctctgcctacagcccttggacctaaccacttcagtgtgttccagtgagtgtctggacctcggcctgaaagatttttccgaaactaaagaaaatttctctgacctaaagaccttaacctccaccccagaagctctcaccaaggactacagggaactggtggggaaaatccttatcccttactcctcaaggcacagggcagtaatgctgaggcttgtgcgccacacttgctcccagaggtccccagcgggctacctgcggtggtgaatgacctcctaacacgccccttgacggccttcctttccttgcctcacttctccactctcctaccagcattgcagggttcacatcccaaatataccactggcacttgaatcctggtctccaggtctgtttctggaaaaacccaagtaagacattgccccagtaatggggctagatgtctgaggcttcctcaagtatctacctcgaaagctcttactgctgtacacacatgcacatacacacacgtgcgtacaaccagtcacatctaagcaccccgaataccagcctgttgaaggtagcagagagctgcactataagccaaggctgctcccaagagccgctccatcactgaattggcgccccagcaagatgaaggaatgtaatcattggaaggatggagaatgttctctgaatcactgacaaattggaaggggtggagggcaagagtccacctggtggagagatggaaagagcgagagagcctggaatgataatgccattgcttagaaaaggctgctccagatgccatatctacagaaattgtacagcccaaacatctctgagcaataggtctctggtagtcttgatgtctagaccaacaattcccagttcattcttctcagggaaggagccaggatagtccagagactctcattctgctgttagattgaaagggttaggcacaacagccttggcaaagtcacaagggcaaattcacactaaagtgtaaatgacccacaactcctcttctatttttaggttggggaggtgctttagaacataaggaggaactaaagaatattcctgttacatacaaggcagagaaaagggaaactagtggtgacaagacaaatcatccctttgacatttggctggctctacctattacagctctgggggtgaggtgggaacaaaaagatgctgtgtaaagaagtatcttatgccatccctactgtagtgaggtgcagtttagaggggacactgatcaagcagagacccagagtgtttcgttccaagccagaaacagaaatgtataaaacacagcctttccagcatcagaaatgagtagtggtagtggagaactacccaaaacaggaaagaggaccacgtgaggtagagtgtcaaggccctacattccagtgcctctgctcatgactgtaattttgggtaggtcacttaaagtctctggacctcagttttgccatctgtgaaatagggataatactatccagcataaaattggttatgaggctcatgtagggcctgcctgggatgatgtgttgctaatggttaagaacacaacttctggggtctgactggacaggctgaaatccctgcttaacacgttccagcagagccctgggcgatctatttaacttttgttttctcacctgtaagctgagacgaaagtacccactttataagattattccaataattagttgaaataatgcatgcagagaattaagcatggtacttgttatttgttaaactagctattaaaatgtgtaaaatataaagtattgtatggattttaggacaatgcaaagactctttgcttgctgcaatagttcggggccctttcagatggctaaaggcagaatttgtatgtgtaaatatggtgtgcttgtctctgctctggatactgagggcttaccctgttattaaacttatttagtaaatattgaactgtcatgaggcctaacatttagttccagttattagataaaacatttgctttgaatggtatttgaattgccaggttctagattattctggttgacaaactcttcgtattttataaagaggctaaaattggtaagctatcacagaacagatgtgccattttcaaggtatattaaaccatgattcactgtaacattgttcctactggcaacaaattcagagcaggctggactttatttggtgaagaaacattgagtggaagagaaatgacattattttatgtatttacattttcaaattactgtggcttaaacctgttcagccaacattacccaccttcagtctgctaaataaatgattcagtacatttctaatttacagaattttttaacaaaagaaaatgtaatttgatagccaaatcaacgttaaacattatacatttaaaaaaccacaggcaaagacacaaacatgatgacactaacttttgttaaagtatgcttacctatggtttcctctgaggcacgttctttcatgctaagcttccaacataatatgaaaatgaaggagatgcattttgcaaagcaaaacagaccttaagcaaaatattatacttctcaaattaacactgttacaaagttttagaatttaataagttcattaatttaaaagtttggatgtctgagtccttctatcccaaaacaagatcttggagggtcttccacagccatgtaataccatggtcacatgaccctttccaaaattattaatctgaatttactatatgaggataaatctatctttttgaaaatatttaggaaaatgagcttggtatttataaaatgaagctctctttgggtggtatcctaagacacgtcaagccaatcagcctgtaactgtgaaaaaaacattggtaggtacaaaagtggggtgggagaggagtgacttaactttgttaagtgatgggaaagaaacactaatagcattatctcaataaaatgtgatttaaaaaaatttaaaatactaaatcattgaactgacaaagaaatataaatcattcagaaataaactcattaggtcatcaaatcctgttaaatctgcaattaggaagagcaaggtgtacaatccatacatttaaactcacaggctcactttgcacaacgtcaatttactccttaatatgttattaatacgcattttccaaaaggatgtattagtaaatggtacacatctacttcttggcaacatcatataacctggtacaacataagcattcttcttatagttaagaaatgtggatggtatcaaaattagaaaaataaatgccctattatgttgtggtcaggtttaaggcatgtgaattttatcttcatacaaaagattaaaatctagatattaaaaagtagtgcagtatcagtgatgctgcctcagttcccaaaatgtcacatcacaaaaatatcccataattgcctgtagtttattccttggctttcctcttttctctctgcatctttgtaacaattttttaaaagtggaaatataattgttggcaatgctaacagctgtagaaatgattacaagatgtggaaaagcataacaggaatgtcaagaatctgtttctggcagtaatatatatggaacattgttcaggacaaaagaggagaaggaagaaaaaaaggagaggggtttatcatctctaagaattttcaaactaaacctcattgcttaataggaaaaaaagattccatatttaaagttaagtcacctctaactactagctaaagcatgacatcaccagcactggagtcagcggaagtgtgtttttgaaggacagtgttgcaggagaatctggacaggttttagagccaggagagagaaaataattctacctctgacagttgaaggaccttaggcaaatcagtttacctctgctagactacactccaaaatttggacattcaaaaatttgatattaataaccacatgaaagtctcgtgttgaggtgaatatgtatttgttggtgaaagatatgttggtttttaaacagacagcactctgcaattgtaggctattgttttgttttgccagttgtcaaattctatccagctatacacacttgtgtggcctcctaatggtgtttttccagtggctaaaggtttatgaataagacacttttcctaatggaattaacccgatgcttttcttaaacatgtaaccttgagttcaccgcaaaaaacaatgcttcgattagagcaatgcatataataaaggttaccctcgtttcttagacactagacatcattcacaaaaagagaactgcttttgaaagggatgtatttgcactggaaagaatagttttctacttctaattataaatgatttattggtgaaagcaaaacaacagcctgtctgagaggcacttctatgagcatcctcacgtgtgatttgcaaggttgaagaagagggaaaaatgcctcaattgtaccaatggtgagaaaacacccaaagtacaaagcaggtttcaaaaaaaccatactcataaccaaggacaataataaagcaatgtgttgacatatactctataagtcttcctccataaatagtttatagaaattttgtaatttctgtaaatgcatcctataataattttgcatcttgctttttttttacatttaatatcaagtagatttctaaagggcaattatttgaaaattatcccaaatacatggggaaatatacatcaagtgaaaaaatgcagtgggtgatagagatatcaggaagcgcctcaaatatttctcatctcgttggagaaaaacaaacatgttctcatttagaatgagtgggagttacctaattgatttaggcctctatatttaacttctagtcaaaaaaggtagttctatctagcaacaatattatggggaacaaaagaaaaaattaactctctaaatttgcagtagggtcttttcttcagaagtaccaaatcccatctattaccagctccatgcttcaggcctaaaatggatctccctgaagcaatgacagaatttttgccaagtgactaggatataaacaccactttggttgcacagtgagacatatgctccaaagaaaactggttcaaaaacaggcaagtgggtttctacagaataaatgagagccctgtcaatggcttcatcttcagggctttgtgtctgtgcttgcgtggtggctcttgtttcatctatggataatggtggcacacagttttcataattccttacattaatgaactgctataaatttgtttttggtattctagagagtcctaacttcagcttctgggcaatgctgaggaggcaccctatattctagacttaccttttgcaaggtgtactctcagcattgtgggcgatttccatgggagaatattctatttaaagaactactgtcccagcataaaacaaaaaatcatttatgaagatgcaggagactcggaaagctctcaattattgtttgcacaagcacaatgtcacagcctcctttccccattccacaagggggtcaggaagagagtactcagctgtgagaaaagacatacagaagaattcatgtggtcatgagagcgaggacatggccgatcccccaaggaggatgtgtcatacacttcatgagcccaagagtgtgctgtagggtctgaagggcaagatgctggttcactgatgtaaaggagagggaaaaaagcttcaaccaactagaaaaacagtctctatgcatgctatttttgattttaaacacaggtatcaattccttctctcagagagtccattttaaaataggatacatttttaaaggaatatttaaaggacacattcattaaaatttattttaaaaacttttcaaaagaaacaaaaggtatgaattttatttaatccttgaggaaatggttcttttctcacacacataaatcactcattttgtttttctttatctcctttattaatctacattagaaaaataaacttttcatacactaagaacaaggaaaccactctcaattgacaaaatgttccaatccaacacaatgattactttcacctttaatttacaggcagccagattcaaaatccttaaagttgcttaaacttaaaaatgacaatgacaacctaaaaggtataatgttgattggaacagacatttaattggaaaattgatgattttccatttccaattaaatctctagatagaaatgaaaaaaattaaaaatcgtatttaagaaaagccaaatcttgggttgtgaggtatctttttaaggatgtttcagcagaaaaaaacaaaggctctcacaattgtgtagctgcctagattaagtgggtatcctgatcaaggagatgggggatgatttggctttagtattccaatgataaagtttataatgagaataacatgttgctacaaaatccagtctcttcctcagatgccttccacagagggcaggaagctttgtcagttttgtttgctgatgatgcctggttccgtcaacaaataacacctgtcacacggtgggtagtcaatatacatttgttgaataaatatgaaaaaaagaaatgtacaatatgtttgtgaagccaactgtgtgtgcattgctattgaggtacacaaaaagtctttgttttaaatttgagaatgaggactttcaatggaatatatctataaaaatgaaaaaaagacattactgtctggacttttgtacagcaagagaagaaaaaccactagccaagagccaactcacctgataggcctggatcaagcatgcagctgtggagaacacccctgggactctaactctggcactctgcaagctgggtacttgggcaggacagcagcagcactcatgaactgggcagcacctgttggtgagggctgatcacatggattctctcatcccagccttacaatcagtccttcaggtacatactttttctgactttgctgatgaggaaactatgcacagaggttacacagcttaacaaagggttctcacctaatgaacaatgaaatgggattttagcctttctttgcatctggtcttagagccaatacccaagaagcactgtactgtatgcattgtctcagagaaacttactcttcctgggcctcagtctttaaaaggtgggcagttgacttaataagaattaaagatcaatgattaaggttcaaggcactccaaaattctggtctttattgaaaaggctacagaagtctcaccttaataataccctatagacttgatattcttggttaattaaatattggaaaccaatttcatagtaattgaggtcagaaaaaagtactcatgacattttagaatatgatgacaaagccatagataaatttcaatgcacctgtaattacttaaaactgttatagcatgcaatgtgttaccacaacagccagagaaatactaatttactcagcctattcttctagaccagtaaacactaggattaaatagatattttcattgaatttgttctacccttcattgccatttatagatagcttacttgtcatagattactttctaattgttttatgtttcctaactagcctgcaatactttggcaaggacctcaaacaatagtagacagtaggtgtaaaatagatggctacattgaacagatgactaaaaggatgcctcctaagtacctatatcttgaaatatatattattgtgccttgctttcaatttgtgattttaaaatctagaaatcacctgttttatgtaataacaataaaatccttctttgttgaaaacatgcacaaataaagtttacaagctcaaaaaattaaacagcagtaacggtcaagctttccaacaataaaatacattttggtaaggttttcattttacaaaaactcaaaatagctttatgagttcacaaaataatatgatatttttcaagatattaacatattcttataccggaagagcatagaataaaatttacttggagattgagcatttgcttctttaagaaatacttcttttagtatttttactttaatattatgaaagctacataattacattcagattcattaactactccagtagttaatttttaaaacttatgatgaatagttttgtttaaaatatataacattggtaatatgcaaatctgaatctgtaataaagaaggatttgcattcctgatttttttttctgatacaaccaatgacaaaataactaatggttccacagaggataaaatgtctcaaatctgttggttctgaaggtgaagcgagatttttgtactgataccgtgtatcactgagataccaggaggaaatggaattaaactcagatagttcaaatggagagattttaatgaagggacgacctacagaggtgtcggcagggttggggggaatcagcgagatatgcttagaacccaccgactggcaaacctccccctgaagatggagaaggaggaaggagtgttactggaatgagagcttgagtccaggggaggaggatgggctgctgaggaggcgacaccatcctgaaagaagaatcctctgccagaggcttttcagggtcatttcttcacactctctctcttcaagtggtatttaaatttcttctttcattttccttctggtaacaaagaagtctgtggctcaaaagatgtttctctaagaccccatcctattaggtctctgagattttagaaatgacccaacttgatccttttattcttcagaatatctctctcaaattttcatttgtttttcattaattgatgaataatgagacattttaggtacctgtccacaaagaaatgaaattttcactttccaggaacctaacaaatgaaaagatagaaatcaattccaacagaatattaccaaagaaatcttttagaatggactgttaaaattatttatttgtatttatctggctctactatttgtggtacatttccacttcaaagctaaacctcaaataacatcatagtgagtggttgacttcatgtttaactgagatcttgaagactgaaaaagaccacgacaaacacacatctattttcttggctactgcatccgtgttcatcaccattctgatagtctgcaatgtattgcagctcaccctttgggaaggactaaagtagacatctgtttgttctgcttactcagcattcctaccctaattttcctttggagaacccctttattctagaccacgtgaagctaatgccaaaccccattccaggggatgcacctgaatccaacctccatcatctaaacagtgccttctccacgttcagagaagagcaagtgactcaaactgccctcataagaacagacctgggacttctgctgcaaatattgaagagtaagtactcttttttcttgctaggactaagctggtagtaccttctatgaggctatcatatggaaacaacttgtctgaaaatgaagccacaactagaaaacagatcctggtaacccggattgatggatccagccctaccttaaatggcaagacctaacccgaggctttttgcatcaaccaataaagtccttaagccagtttgagttggttttgtcacttgcagctaaaagaattctgactctaacaatgtgacaatagcaaaaataaacataactgcttttgaggtttctaatggattttcctccctatatacatgatttcatttaatcctcacaattcaggaaagcacatatctattaacattaaattaatattcattattttgaacacatgctatgtggataagggatgaggaaagccaaggaagtaatcaacgtgaaatctcacttatatgggagggaagtggaggttacatatctcagggcacttaacagatatcatcaaatgaaagaataaacagtgtgtgggagaggcagtaggtgattcttcatcaattcctggatgaaaaattaggagataatgaactccgaacaggcagcctaatgagaatggctcaagcaacaggacatagagagggagttaggttagacatggggttcttgggaattttcacctcgtgggggggcgggggggtcgtgcagctgttgtcagtgggaaagggaaaaaggaaaaggctgagtttggaaggcagggagggaggagacaatgtgagtcagtgaaaaagggcccttagaatgacaagtctggaccagagagaggctaagactgaaaatacaagttgggtaaccactggcatacagatggcagttcaggcttgggcactgcccaccagagcctcagcatgaagagaagagggggaggctggccaccacctccctctaggtaatcgtcatcctgatgctgagctcctgaaaacaggctctttcactcgccccatctcttgctcttgattgcaacccggcattcaggaggcaccctgtaatatctgtggagtgaccgacaacacagcgccagggcactgagaagatcccagggcgccagggactggttctacaagggtgcccctcccggtcccctccagcgcgccgccagagctgccagtcttggctgctacacgggaggcagcctcattatgcagctctcacctcttaaattagttcatgctctcacattaggtgtaatcacagcttgcaacgctttctggggatgtctcagaaagatctgagttgaaaaaatatttttgtgtcattttaatttaaagtaaaattgctgcttcttccccgcccctttctttcctcctggcccacccagcgaccctggccggccgtgctcaacgggggcgggggtcggaggtgagatttcctccacataattccttaaacagctatcaactaagtctcaaagaaaaaaaaaagagatctagaagcagagacgtggctgctggcgatcccaaagctggtgttcgctcttgggggagagcgtaccctgggggaggccgggaggccgggccagaggctagcccagaggcagagggcaggagcgctcagccggcgccccgcgtctctccagctcccgacgctgcgctggctccgctgagcacgccaggatcaaggtcgcctggtggggaccggagcgccaggagcctgtgggaagcgttccagccggcctctgactgggatccggcgccgcgtttctgctttggacttgactgacaggtccccccgccctcccgccgccctactaccagcctgggttcatccttcagggctacgtctaccgcacccgggctggaaagcctggagcgcgcccttcctctcctcatcttctcagctctcctttctccctgccacttggcaaagctgcattttgactttcacgttttggactacgtgtgtgtagttccaagtccatgcgtggcacgaaaatccacttagggtaaaaattattctcgaaaaatcgcccatctcaggatctggtgtctacactcaaggctaggaggtgcaggtacgggtgcgtaaagcatgccgtaagggtgcacagtaaataaaaagtacggatgcaaaatgtaaattttaagtgcaaaacagaaaagcagtactcgttgccgccccgcacgctgggttttaaggggcacgaaggtgggcctcggctgcttttgctcagccccgcgtcctcagcgcccggcccagtacccggtactccgtaggggttcaatgatctcccctgaataagtgaacgaattaacaaatgaatgaatgaccgctcgatccgacctccgcggccggcagagcagtcgctggagaggcgggagagagcgagaggccaagctccaccatcgcggccgccggctggggcagagggacacggagacactcggcgccccggctccgcaccgagtccccg

SEQ ID NO: 17591 - RNA, 11189 nt, Homo sapiens
  source 1..11189: mol_type = other RNA
tcaggccaggcacagtggctcatgcctgtagtcccagcactttgggaggccgaggtgggcagatccacgaggtcaggagatcaagaccatcctaacatggtaaaaccccatctctactaacaatacaaaaaattagtcaggtgtggtggcacgtgcctgtagtcccagctactcaggaggctgaggcaggagaatcgcttgaacctgggaggcggaggttgcagtgagccgagattgtgccactgcaccctagcctaggcaacagagcaagactctgtctcaaaaaaaataaaaaaaaaaaaaagagagaaagagagagagagatgaggagttgctgcactgctgggtgtggagagccgaggaggattcaaagatggtcctgaagtcccagctggaagaagtaggcggcagcaatgtttttaatactgtaaattcatcacgtagcacaggtttggggtggagaaagaaaaattgcattggcttcagggcatgcccagatctttcctcatcttaggcgtttgctaatacatgcattttctaagctgatgtcttgcgtttaatcactgctccattcaaaagagagaaggaggttgtttcaaacctagttgatatcatttgacttccatgctattcacagggctattttatttgaaacaggtataccacagccttaaattgcaagttaatccaggatgttcctaggttggcagttaggaacatgtaattctttggaagggctaaaagtcagctctttaaattatctccatatgaaccttctctccaccttagggtggatccacttatttagtccactgccagtaccacactagaacccgggtggtcactggactccagaaacaacagtagccctctctctgttctgtctctttttgactatctctattctgttcctgaccctgatttctcctgccaagctcaattttgacagctgacaacggcaagccatggcttcccaaaacattattttcaggtcaacttataaatttcaagaacacatttggctccgcttcctgtggtactaagcctacttcttgacagcatttgcctttgttgtaaatagcaaagttcttctagttggatttttgctaagaagtgtgtggatgtggcatgtgacgacatctttagcttggattctagaaaggcactaccattgtgcatttggctaaaggaaacacattttacccgtgaatgccttctatttacaaatgctcagctagcacacaaagctaagtacaagcaataagtactatcctacaatgttactcatttctgaaagcacaaaatgatgactggtatagctttggagatgttttctggaaacccaataaaggaacagatctttgttattccacacctacaaagtcagaagatgcacagtcttttattcatgtttgaacaagcttccttcttgaacaatcaactataaagtgatgtgattctctactagaccaggaactccttgaggacagaatgagggtctaatccatattctaaatccacaccacctggcacaatacatgttgcatggttagggtcaactaagagttggttgaattaatcaataacacacagcaagagaattcacaaagagaggggagtaatcccccagcctcaatcactcggcaagtggaatcgctgggcactgattccagctctgtctcagtgcttgagacagagctgaatgtaatgtgaacatttcaaatgaacaggaaaactagactcacggataagcagtgtagtcatcaagacaacactgtcttggaggtttttctgaagttaaaaccatgctacataagcaataaattatgaaggctgagcatgtgaataaaatttaatgttgtcataaattttataacaaagttaatctgacacatttaatgacatgcataatcattagtatgcagcactgtaatcagacattgataataagcagttcacaccagtgactgtaagagtctttacttgtgttcagccaagccaactgcttggtatatttttctcccttcttagtcgttagttttccatacctacaataactatcagtggtgatgggcttctctgaccatgtgaataatttaatcctcaatgcacagatacagaaacccttgctgaagacagtgtggagcagagaaggctgtctccactccttccacctgaaacacctctgcagatggatatgggagctctgcctacagcccttggacctaaccacttcagtgtgttccagtgagtgtctggacctcggcctgaaagatttttccgaaactaaagaaaatttctctgacctaaagaccttaacctccaccccagaagctctcaccaaggactacagggaactggtggggaaaatccttatcccttactcctcaaggcacagggcagtaatgctgaggcttgtgcgccacacttgctcccagaggtccccagcgggctacctgcggtggtgaatgacctcctaacacgccccttgacggccttcctttccttgcctcacttctccactctcctaccagcattgcagggttcacatcccaaatataccactggcacttgaatcctggtctccaggtctgtttctggaaaaacccaagtaagacattgccccagtaatggggctagatgtctgaggcttcctcaagtatctacctcgaaagctcttactgctgtacacacatgcacatacacacacgtgcgtacaaccagtcacatctaagcaccccgaataccagcctgttgaaggtagcagagagctgcactataagccaaggctgctcccaagagccgctccatcactgaattggcgccccagcaagatgaaggaatgtaatcattggaaggatggagaatgttctctgaatcactgacaaattggaaggggtggagggcaagagtccacctggtggagagatggaaagagcgagagagcctggaatgataatgccattgcttagaaaaggctgctccagatgccatatctacagaaattgtacagcccaaacatctctgagcaataggtctctggtagtcttgatgtctagaccaacaattcccagttcattcttctcagggaaggagccaggatagtccagagactctcattctgctgttagattgaaagggttaggcacaacagccttggcaaagtcacaagggcaaattcacactaaagtgtaaatgacccacaactcctcttctatttttaggttggggaggtgctttagaacataaggaggaactaaagaatattcctgttacatacaaggcagagaaaagggaaactagtggtgacaagacaaatcatccctttgacatttggctggctctacctattacagctctgggggtgaggtgggaacaaaaagatgctgtgtaaagaagtatcttatgccatccctactgtagtgaggtgcagtttagaggggacactgatcaagcagagacccagagtgtttcgttccaagccagaaacagaaatgtataaaacacagcctttccagcatcagaaatgagtagtggtagtggagaactacccaaaacaggaaagaggaccacgtgaggtagagtgtcaaggccctacattccagtgcctctgctcatgactgtaattttgggtaggtcacttaaagtctctggacctcagttttgccatctgtgaaatagggataatactatccagcataaaattggttatgaggctcatgtagggcctgcctgggatgatgtgttgctaatggttaagaacacaacttctggggtctgactggacaggctgaaatccctgcttaacacgttccagcagagccctgggcgatctatttaacttttgttttctcacctgtaagctgagacgaaagtacccactttataagattattccaataattagttgaaataatgcatgcagagaattaagcatggtacttgttatttgttaaactagctattaaaatgtgtaaaatataaagtattgtatggattttaggacaatgcaaagactctttgcttgctgcaatagttcggggccctttcagatggctaaaggcagaatttgtatgtgtaaatatggtgtgcttgtctctgctctggatactgagggcttaccctgttattaaacttatttagtaaatattgaactgtcatgaggcctaacatttagttccagttattagataaaacatttgctttgaatggtatttgaattgccaggttctagattattctggttgacaaactcttcgtattttataaagaggctaaaattggtaagctatcacagaacagatgtgccattttcaaggtatattaaaccatgattcactgtaacattgttcctactggcaacaaattcagagcaggctggactttatttggtgaagaaacattgagtggaagagaaatgacattattttatgtatttacattttcaaattactgtggcttaaacctgttcagccaacattacccaccttcagtctgctaaataaatgattcagtacatttctaatttacagaattttttaacaaaagaaaatgtaatttgatagccaaatcaacgttaaacattatacatttaaaaaaccacaggcaaagacacaaacatgatgacactaacttttgttaaagtatgcttacctatggtttcctctgaggcacgttctttcatgctaagcttccaacataatatgaaaatgaaggagatgcattttgcaaagcaaaacagaccttaagcaaaatattatacttctcaaattaacactgttacaaagttttagaatttaataagttcattaatttaaaagtttggatgtctgagtccttctatcccaaaacaagatcttggagggtcttccacagccatgtaataccatggtcacatgaccctttccaaaattattaatctgaatttactatatgaggataaatctatctttttgaaaatatttaggaaaatgagcttggtatttataaaatgaagctctctttgggtggtatcctaagacacgtcaagccaatcagcctgtaactgtgaaaaaaacattggtaggtacaaaagtggggtgggagaggagtgacttaactttgttaagtgatgggaaagaaacactaatagcattatctcaataaaatgtgatttaaaaaaatttaaaatactaaatcattgaactgacaaagaaatataaatcattcagaaataaactcattaggtcatcaaatcctgttaaatctgcaattaggaagagcaaggtgtacaatccatacatttaaactcacaggctcactttgcacaacgtcaatttactccttaatatgttattaatacgcattttccaaaaggatgtattagtaaatggtacacatctacttcttggcaacatcatataacctggtacaacataagcattcttcttatagttaagaaatgtggatggtatcaaaattagaaaaataaatgccctattatgttgtggtcaggtttaaggcatgtgaattttatcttcatacaaaagattaaaatctagatattaaaaagtagtgcagtatcagtgatgctgcctcagttcccaaaatgtcacatcacaaaaatatcccataattgcctgtagtttattccttggctttcctcttttctctctgcatctttgtaacaattttttaaaagtggaaatataattgttggcaatgctaacagctgtagaaatgattacaagatgtggaaaagcataacaggaatgtcaagaatctgtttctggcagtaatatatatggaacattgttcaggacaaaagaggagaaggaagaaaaaaaggagaggggtttatcatctctaagaattttcaaactaaacctcattgcttaataggaaaaaaagattccatatttaaagttaagtcacctctaactactagctaaagcatgacatcaccagcactggagtcagcggaagtgtgtttttgaaggacagtgttgcaggagaatctggacaggttttagagccaggagagagaaaataattctacctctgacagttgaaggaccttaggcaaatcagtttacctctgctagactacactccaaaatttggacattcaaaaatttgatattaataaccacatgaaagtctcgtgttgaggtgaatatgtatttgttggtgaaagatatgttggtttttaaacagacagcactctgcaattgtaggctattgttttgttttgccagttgtcaaattctatccagctatacacacttgtgtggcctcctaatggtgtttttccagtggctaaaggtttatgaataagacacttttcctaatggaattaacccgatgcttttcttaaacatgtaaccttgagttcaccgcaaaaaacaatgcttcgattagagcaatgcatataataaaggttaccctcgtttcttagacactagacatcattcacaaaaagagaactgcttttgaaagggatgtatttgcactggaaagaatagttttctacttctaattataaatgatttattggtgaaagcaaaacaacagcctgtctgagaggcacttctatgagcatcctcacgtgtgatttgcaaggttgaagaagagggaaaaatgcctcaattgtaccaatggtgagaaaacacccaaagtacaaagcaggtttcaaaaaaaccatactcataaccaaggacaataataaagcaatgtgttgacatatactctataagtcttcctccataaatagtttatagaaattttgtaatttctgtaaatgcatcctataataattttgcatcttgctttttttttacatttaatatcaagtagatttctaaagggcaattatttgaaaattatcccaaatacatggggaaatatacatcaagtgaaaaaatgcagtgggtgatagagatatcaggaagcgcctcaaatatttctcatctcgttggagaaaaacaaacatgttctcatttagaatgagtgggagttacctaattgatttaggcctctatatttaacttctagtcaaaaaaggtagttctatctagcaacaatattatggggaacaaaagaaaaaattaactctctaaatttgcagtagggtcttttcttcagaagtaccaaatcccatctattaccagctccatgcttcaggcctaaaatggatctccctgaagcaatgacagaatttttgccaagtgactaggatataaacaccactttggttgcacagtgagacatatgctccaaagaaaactggttcaaaaacaggcaagtgggtttctacagaataaatgagagccctgtcaatggcttcatcttcagggctttgtgtctgtgcttgcgtggtggctcttgtttcatctatggataatggtggcacacagttttcataattccttacattaatgaactgctataaatttgtttttggtattctagagagtcctaacttcagcttctgggcaatgctgaggaggcaccctatattctagacttaccttttgcaaggtgtactctcagcattgtgggcgatttccatgggagaatattctatttaaagaactactgtcccagcataaaacaaaaaatcatttatgaagatgcaggagactcggaaagctctcaattattgtttgcacaagcacaatgtcacagcctcctttccccattccacaagggggtcaggaagagagtactcagctgtgagaaaagacatacagaagaattcatgtggtcatgagagcgaggacatggccgatcccccaaggaggatgtgtcatacacttcatgagcccaagagtgtgctgtagggtctgaagggcaagatgctggttcactgatgtaaaggagagggaaaaaagcttcaaccaactagaaaaacagtctctatgcatgctatttttgattttaaacacaggtatcaattccttctctcagagagtccattttaaaataggatacatttttaaaggaatatttaaaggacacattcattaaaatttattttaaaaacttttcaaaagaaacaaaaggtatgaattttatttaatccttgaggaaatggttcttttctcacacacataaatcactcattttgtttttctttatctcctttattaatctacattagaaaaataaacttttcatacactaagaacaaggaaaccactctcaattgacaaaatgttccaatccaacacaatgattactttcacctttaatttacaggcagccagattcaaaatccttaaagttgcttaaacttaaaaatgacaatgacaacctaaaaggtataatgttgattggaacagacatttaattggaaaattgatgattttccatttccaattaaatctctagatagaaatgaaaaaaattaaaaatcgtatttaagaaaagccaaatcttgggttgtgaggtatctttttaaggatgtttcagcagaaaaaaacaaaggctctcacaattgtgtagctgcctagattaagtgggtatcctgatcaaggagatgggggatgatttggctttagtattccaatgataaagtttataatgagaataacatgttgctacaaaatccagtctcttcctcagatgccttccacagagggcaggaagctttgtcagttttgtttgctgatgatgcctggttccgtcaacaaataacacctgtcacacggtgggtagtcaatatacatttgttgaataaatatgaaaaaaagaaatgtacaatatgtttgtgaagccaactgtgtgtgcattgctattgaggtacacaaaaagtctttgttttaaatttgagaatgaggactttcaatggaatatatctataaaaatgaaaaaaagacattactgtctggacttttgtacagcaagagaagaaaaaccactagccaagagccaactcacctgataggcctggatcaagcatgcagctgtggagaacacccctgggactctaactctggcactctgcaagctgggtacttgggcaggacagcagcagcactcatgaactgggcagcacctgttggtgagggctgatcacatggattctctcatcccagccttacaatcagtccttcaggtacatactttttctgactttgctgatgaggaaactatgcacagaggttacacagcttaacaaagggttctcacctaatgaacaatgaaatgggattttagcctttctttgcatctggtcttagagccaatacccaagaagcactgtactgtatgcattgtctcagagaaacttactcttcctgggcctcagtctttaaaaggtgggcagttgacttaataagaattaaagatcaatgattaaggttcaaggcactccaaaattctggtctttattgaaaaggctacagaagtctcaccttaataataccctatagacttgatattcttggttaattaaatattggaaaccaatttcatagtaattgaggtcagaaaaaagtactcatgacattttagaatatgatgacaaagccatagataaatttcaatgcacctgtaattacttaaaactgttatagcatgcaatgtgttaccacaacagccagagaaatactaatttactcagcctattcttctagaccagtaaacactaggattaaatagatattttcattgaatttgttctacccttcattgccatttatagatagcttacttgtcatagattactttctaattgttttatgtttcctaactagcctgcaatactttggcaaggacctcaaacaatagtagacagtaggtgtaaaatagatggctacattgaacagatgactaaaaggatgcctcctaagtacctatatcttgaaatatatattattgtgccttgctttcaatttgtgattttaaaatctagaaatcacctgttttatgtaataacaataaaatccttctttgttgaaaacatgcacaaataaagtttacaagctcaaaaaattaaacagcagtaacggtcaagctttccaacaataaaatacattttggtaaggttttcattttacaaaaactcaaaatagctttatgagttcacaaaataatatgatatttttcaagatattaacatattcttataccggaagagcatagaataaaatttacttggagattgagcatttgcttctttaagaaatacttcttttagtatttttactttaatattatgaaagctacataattacattcagattcattaactactccagtagttaatttttaaaacttatgatgaatagttttgtttaaaatatataacattggtaatatgcaaatctgaatctgtaataaagaaggatttgcattcctgatttttttttctgatacaaccaatgacaaaataactaatggttccacagaggataaaatgtctcaaatctgttggttctgaaggtgaagcgagatttttgtactgataccgtgtatcactgagataccaggaggaaatggaattaaactcagatagttcaaatggagagattttaatgaagggacgacctacagaggtgtcggcagggttggggggaatcagcgagatatgcttagaacccaccgactggcaaacctccccctgaagatggagaaggaggaaggagtgttactggaatgagagcttgagtccaggggaggaggatgggctgctgaggaggcgacaccatcctgaaagaagaatcctctgccagaggcttttcagggtcatttcttcacactctctctcttcaagtggtatttaaatttcttctttcattttccttctggtaacaaagaagtctgtggctcaaaagatgtttctctaagaccccatcctattaggtctctgagattttagaaatgacccaacttgatccttttattcttcagaatatctctctcaaattttcatttgtttttcattaattgatgaataatgagacattttaggtacctgtccacaaagaaatgaaattttcactttccaggaacctgagggccgacgagtgggggcgggcaggagggccgagggaggcggaacaggatcgaggcgcgaggcgggagtcgagaaagcgagcggccgaggcgactctcagtgcgcggacgcgggcgcgcgcccgcgctcccttcgtcgactcacggcgagagcccaaccctgctgccgcgcgccacccgcctcgccgcgc

SEQ ID NO: 17592 - RNA, 11050 nt, Homo sapiens
  source 1..11050: mol_type = other RNA
tcaggccaggcacagtggctcatgcctgtagtcccagcactttgggaggccgaggtgggcagatccacgaggtcaggagatcaagaccatcctaacatggtaaaaccccatctctactaacaatacaaaaaattagtcaggtgtggtggcacgtgcctgtagtcccagctactcaggaggctgaggcaggagaatcgcttgaacctgggaggcggaggttgcagtgagccgagattgtgccactgcaccctagcctaggcaacagagcaagactctgtctcaaaaaaaataaaaaaaaaaaaaagagagaaagagagagagagatgaggagttgctgcactgctgggtgtggagagccgaggaggattcaaagatggtcctgaagtcccagctggaagaagtaggcggcagcaatgtttttaatactgtaaattcatcacgtagcacaggtttggggtggagaaagaaaaattgcattggcttcagggcatgcccagatctttcctcatcttaggcgtttgctaatacatgcattttctaagctgatgtcttgcgtttaatcactgctccattcaaaagagagaaggaggttgtttcaaacctagttgatatcatttgacttccatgctattcacagggctattttatttgaaacaggtataccacagccttaaattgcaagttaatccaggatgttcctaggttggcagttaggaacatgtaattctttggaagggctaaaagtcagctctttaaattatctccatatgaaccttctctccaccttagggtggatccacttatttagtccactgccagtaccacactagaacccgggtggtcactggactccagaaacaacagtagccctctctctgttctgtctctttttgactatctctattctgttcctgaccctgatttctcctgccaagctcaattttgacagctgacaacggcaagccatggcttcccaaaacattattttcaggtcaacttataaatttcaagaacacatttggctccgcttcctgtggtactaagcctacttcttgacagcatttgcctttgttgtaaatagcaaagttcttctagttggatttttgctaagaagtgtgtggatgtggcatgtgacgacatctttagcttggattctagaaaggcactaccattgtgcatttggctaaaggaaacacattttacccgtgaatgccttctatttacaaatgctcagctagcacacaaagctaagtacaagcaataagtactatcctacaatgttactcatttctgaaagcacaaaatgatgactggtatagctttggagatgttttctggaaacccaataaaggaacagatctttgttattccacacctacaaagtcagaagatgcacagtcttttattcatgtttgaacaagcttccttcttgaacaatcaactataaagtgatgtgattctctactagaccaggaactccttgaggacagaatgagggtctaatccatattctaaatccacaccacctggcacaatacatgttgcatggttagggtcaactaagagttggttgaattaatcaataacacacagcaagagaattcacaaagagaggggagtaatcccccagcctcaatcactcggcaagtggaatcgctgggcactgattccagctctgtctcagtgcttgagacagagctgaatgtaatgtgaacatttcaaatgaacaggaaaactagactcacggataagcagtgtagtcatcaagacaacactgtcttggaggtttttctgaagttaaaaccatgctacataagcaataaattatgaaggctgagcatgtgaataaaatttaatgttgtcataaattttataacaaagttaatctgacacatttaatgacatgcataatcattagtatgcagcactgtaatcagacattgataataagcagttcacaccagtgactgtaagagtctttacttgtgttcagccaagccaactgcttggtatatttttctcccttcttagtcgttagttttccatacctacaataactatcagtggtgatgggcttctctgaccatgtgaataatttaatcctcaatgcacagatacagaaacccttgctgaagacagtgtggagcagagaaggctgtctccactccttccacctgaaacacctctgcagatggatatgggagctctgcctacagcccttggacctaaccacttcagtgtgttccagtgagtgtctggacctcggcctgaaagatttttccgaaactaaagaaaatttctctgacctaaagaccttaacctccaccccagaagctctcaccaaggactacagggaactggtggggaaaatccttatcccttactcctcaaggcacagggcagtaatgctgaggcttgtgcgccacacttgctcccagaggtccccagcgggctacctgcggtggtgaatgacctcctaacacgccccttgacggccttcctttccttgcctcacttctccactctcctaccagcattgcagggttcacatcccaaatataccactggcacttgaatcctggtctccaggtctgtttctggaaaaacccaagtaagacattgccccagtaatggggctagatgtctgaggcttcctcaagtatctacctcgaaagctcttactgctgtacacacatgcacatacacacacgtgcgtacaaccagtcacatctaagcaccccgaataccagcctgttgaaggtagcagagagctgcactataagccaaggctgctcccaagagccgctccatcactgaattggcgccccagcaagatgaaggaatgtaatcattggaaggatggagaatgttctctgaatcactgacaaattggaaggggtggagggcaagagtccacctggtggagagatggaaagagcgagagagcctggaatgataatgccattgcttagaaaaggctgctccagatgccatatctacagaaattgtacagcccaaacatctctgagcaataggtctctggtagtcttgatgtctagaccaacaattcccagttcattcttctcagggaaggagccaggatagtccagagactctcattctgctgttagattgaaagggttaggcacaacagccttggcaaagtcacaagggcaaattcacactaaagtgtaaatgacccacaactcctcttctatttttaggttggggaggtgctttagaacataaggaggaactaaagaatattcctgttacatacaaggcagagaaaagggaaactagtggtgacaagacaaatcatccctttgacatttggctggctctacctattacagctctgggggtgaggtgggaacaaaaagatgctgtgtaaagaagtatcttatgccatccctactgtagtgaggtgcagtttagaggggacactgatcaagcagagacccagagtgtttcgttccaagccagaaacagaaatgtataaaacacagcctttccagcatcagaaatgagtagtggtagtggagaactacccaaaacaggaaagaggaccacgtgaggtagagtgtcaaggccctacattccagtgcctctgctcatgactgtaattttgggtaggtcacttaaagtctctggacctcagttttgccatctgtgaaatagggataatactatccagcataaaattggttatgaggctcatgtagggcctgcctgggatgatgtgttgctaatggttaagaacacaacttctggggtctgactggacaggctgaaatccctgcttaacacgttccagcagagccctgggcgatctatttaacttttgttttctcacctgtaagctgagacgaaagtacccactttataagattattccaataattagttgaaataatgcatgcagagaattaagcatggtacttgttatttgttaaactagctattaaaatgtgtaaaatataaagtattgtatggattttaggacaatgcaaagactctttgcttgctgcaatagttcggggccctttcagatggctaaaggcagaatttgtatgtgtaaatatggtgtgcttgtctctgctctggatactgagggcttaccctgttattaaacttatttagtaaatattgaactgtcatgaggcctaacatttagttccagttattagataaaacatttgctttgaatggtatttgaattgccaggttctagattattctggttgacaaactcttcgtattttataaagaggctaaaattggtaagctatcacagaacagatgtgccattttcaaggtatattaaaccatgattcactgtaacattgttcctactggcaacaaattcagagcaggctggactttatttggtgaagaaacattgagtggaagagaaatgacattattttatgtatttacattttcaaattactgtggcttaaacctgttcagccaacattacccaccttcagtctgctaaataaatgattcagtacatttctaatttacagaattttttaacaaaagaaaatgtaatttgatagccaaatcaacgttaaacattatacatttaaaaaaccacaggcaaagacacaaacatgatgacactaacttttgttaaagtatgcttacctatggtttcctctgaggcacgttctttcatgctaagcttccaacataatatgaaaatgaaggagatgcattttgcaaagcaaaacagaccttaagcaaaatattatacttctcaaattaacactgttacaaagttttagaatttaataagttcattaatttaaaagtttggatgtctgagtccttctatcccaaaacaagatcttggagggtcttccacagccatgtaataccatggtcacatgaccctttccaaaattattaatctgaatttactatatgaggataaatctatctttttgaaaatatttaggaaaatgagcttggtatttataaaatgaagctctctttgggtggtatcctaagacacgtcaagccaatcagcctgtaactgtgaaaaaaacattggtaggtacaaaagtggggtgggagaggagtgacttaactttgttaagtgatgggaaagaaacactaatagcattatctcaataaaatgtgatttaaaaaaatttaaaatactaaatcattgaactgacaaagaaatataaatcattcagaaataaactcattaggtcatcaaatcctgttaaatctgcaattaggaagagcaaggtgtacaatccatacatttaaactcacaggctcactttgcacaacgtcaatttactccttaatatgttattaatacgcattttccaaaaggatgtattagtaaatggtacacatctacttcttggcaacatcatataacctggtacaacataagcattcttcttatagttaagaaatgtggatggtatcaaaattagaaaaataaatgccctattatgttgtggtcaggtttaaggcatgtgaattttatcttcatacaaaagattaaaatctagatattaaaaagtagtgcagtatcagtgatgctgcctcagttcccaaaatgtcacatcacaaaaatatcccataattgcctgtagtttattccttggctttcctcttttctctctgcatctttgtaacaattttttaaaagtggaaatataattgttggcaatgctaacagctgtagaaatgattacaagatgtggaaaagcataacaggaatgtcaagaatctgtttctggcagtaatatatatggaacattgttcaggacaaaagaggagaaggaagaaaaaaaggagaggggtttatcatctctaagaattttcaaactaaacctcattgcttaataggaaaaaaagattccatatttaaagttaagtcacctctaactactagctaaagcatgacatcaccagcactggagtcagcggaagtgtgtttttgaaggacagtgttgcaggagaatctggacaggttttagagccaggagagagaaaataattctacctctgacagttgaaggaccttaggcaaatcagtttacctctgctagactacactccaaaatttggacattcaaaaatttgatattaataaccacatgaaagtctcgtgttgaggtgaatatgtatttgttggtgaaagatatgttggtttttaaacagacagcactctgcaattgtaggctattgttttgttttgccagttgtcaaattctatccagctatacacacttgtgtggcctcctaatggtgtttttccagtggctaaaggtttatgaataagacacttttcctaatggaattaacccgatgcttttcttaaacatgtaaccttgagttcaccgcaaaaaacaatgcttcgattagagcaatgcatataataaaggttaccctcgtttcttagacactagacatcattcacaaaaagagaactgcttttgaaagggatgtatttgcactggaaagaatagttttctacttctaattataaatgatttattggtgaaagcaaaacaacagcctgtctgagaggcacttctatgagcatcctcacgtgtgatttgcaaggttgaagaagagggaaaaatgcctcaattgtaccaatggtgagaaaacacccaaagtacaaagcaggtttcaaaaaaaccatactcataaccaaggacaataataaagcaatgtgttgacatatactctataagtcttcctccataaatagtttatagaaattttgtaatttctgtaaatgcatcctataataattttgcatcttgctttttttttacatttaatatcaagtagatttctaaagggcaattatttgaaaattatcccaaatacatggggaaatatacatcaagtgaaaaaatgcagtgggtgatagagatatcaggaagcgcctcaaatatttctcatctcgttggagaaaaacaaacatgttctcatttagaatgagtgggagttacctaattgatttaggcctctatatttaacttctagtcaaaaaaggtagttctatctagcaacaatattatggggaacaaaagaaaaaattaactctctaaatttgcagtagggtcttttcttcagaagtaccaaatcccatctattaccagctccatgcttcaggcctaaaatggatctccctgaagcaatgacagaatttttgccaagtgactaggatataaacaccactttggttgcacagtgagacatatgctccaaagaaaactggttcaaaaacaggcaagtgggtttctacagaataaatgagagccctgtcaatggcttcatcttcagggctttgtgtctgtgcttgcgtggtggctcttgtttcatctatggataatggtggcacacagttttcataattccttacattaatgaactgctataaatttgtttttggtattctagagagtcctaacttcagcttctgggcaatgctgaggaggcaccctatattctagacttaccttttgcaaggtgtactctcagcattgtgggcgatttccatgggagaatattctatttaaagaactactgtcccagcataaaacaaaaaatcatttatgaagatgcaggagactcggaaagctctcaattattgtttgcacaagcacaatgtcacagcctcctttccccattccacaagggggtcaggaagagagtactcagctgtgagaaaagacatacagaagaattcatgtggtcatgagagcgaggacatggccgatcccccaaggaggatgtgtcatacacttcatgagcccaagagtgtgctgtagggtctgaagggcaagatgctggttcactgatgtaaaggagagggaaaaaagcttcaaccaactagaaaaacagtctctatgcatgctatttttgattttaaacacaggtatcaattccttctctcagagagtccattttaaaataggatacatttttaaaggaatatttaaaggacacattcattaaaatttattttaaaaacttttcaaaagaaacaaaaggtatgaattttatttaatccttgaggaaatggttcttttctcacacacataaatcactcattttgtttttctttatctcctttattaatctacattagaaaaataaacttttcatacactaagaacaaggaaaccactctcaattgacaaaatgttccaatccaacacaatgattactttcacctttaatttacaggcagccagattcaaaatccttaaagttgcttaaacttaaaaatgacaatgacaacctaaaaggtataatgttgattggaacagacatttaattggaaaattgatgattttccatttccaattaaatctctagatagaaatgaaaaaaattaaaaatcgtatttaagaaaagccaaatcttgggttgtgaggtatctttttaaggatgtttcagcagaaaaaaacaaaggctctcacaattgtgtagctgcctagattaagtgggtatcctgatcaaggagatgggggatgatttggctttagtattccaatgataaagtttataatgagaataacatgttgctacaaaatccagtctcttcctcagatgccttccacagagggcaggaagctttgtcagttttgtttgctgatgatgcctggttccgtcaacaaataacacctgtcacacggtgggtagtcaatatacatttgttgaataaatatgaaaaaaagaaatgtacaatatgtttgtgaagccaactgtgtgtgcattgctattgaggtacacaaaaagtctttgttttaaatttgagaatgaggactttcaatggaatatatctataaaaatgaaaaaaagacattactgtctggacttttgtacagcaagagaagaaaaaccactagccaagagccaactcacctgataggcctggatcaagcatgcagctgtggagaacacccctgggactctaactctggcactctgcaagctgggtacttgggcaggacagcagcagcactcatgaactgggcagcacctgttggtgagggctgatcacatggattctctcatcccagccttacaatcagtccttcaggtacatactttttctgactttgctgatgaggaaactatgcacagaggttacacagcttaacaaagggttctcacctaatgaacaatgaaatgggattttagcctttctttgcatctggtcttagagccaatacccaagaagcactgtactgtatgcattgtctcagagaaacttactcttcctgggcctcagtctttaaaaggtgggcagttgacttaataagaattaaagatcaatgattaaggttcaaggcactccaaaattctggtctttattgaaaaggctacagaagtctcaccttaataataccctatagacttgatattcttggttaattaaatattggaaaccaatttcatagtaattgaggtcagaaaaaagtactcatgacattttagaatatgatgacaaagccatagataaatttcaatgcacctgtaattacttaaaactgttatagcatgcaatgtgttaccacaacagccagagaaatactaatttactcagcctattcttctagaccagtaaacactaggattaaatagatattttcattgaatttgttctacccttcattgccatttatagatagcttacttgtcatagattactttctaattgttttatgtttcctaactagcctgcaatactttggcaaggacctcaaacaatagtagacagtaggtgtaaaatagatggctacattgaacagatgactaaaaggatgcctcctaagtacctatatcttgaaatatatattattgtgccttgctttcaatttgtgattttaaaatctagaaatcacctgttttatgtaataacaataaaatccttctttgttgaaaacatgcacaaataaagtttacaagctcaaaaaattaaacagcagtaacggtcaagctttccaacaataaaatacattttggtaaggttttcattttacaaaaactcaaaatagctttatgagttcacaaaataatatgatatttttcaagatattaacatattcttataccggaagagcatagaataaaatttacttggagattgagcatttgcttctttaagaaatacttcttttagtatttttactttaatattatgaaagctacataattacattcagattcattaactactccagtagttaatttttaaaacttatgatgaatagttttgtttaaaatatataacattggtaatatgcaaatctgaatctgtaataaagaaggatttgcattcctgatttttttttctgatacaaccaatgacaaaataactaatggttccacagaggataaaatgtctcaaatctgttggttctgaaggtgaagcgagatttttgtactgataccgtgtatcactgagataccaggaggaaatggaattaaactcagatagttcaaatggagagattttaatgaagggacgacctacagaggtgtcggcagggttggggggaatcagcgagatatgcttagaacccaccgactggcaaacctccccctgaagatggagaaggaggaaggagtgttactggaatgagagcttgagtccaggggaggaggatgggctgctgaggaggcgacaccatcctgaaagaagaatcctctgccagaggcttttcagggtcatttcttcacactctctctcttcaagtggtatttaaatttcttctttcattttccttctggtaacaaagaagtctgtggctcaaaagatgtttctctaagaccccatcctattaggtctctgagctgagggccgacgagtgggggcgggcaggagggccgagggaggcggaacaggatcgaggcgcgaggcgggagtcgagaaagcgagcggccgaggcgactctcagtgcgcggacgcgggcgcgcgcccgcgctcccttcgtcgactcacggcgagagcccaaccctgctgccgcgcgccacccgcctcgccgcgcct

SEQ ID NO: 17593 - RNA, 11074 nt, Homo sapiens
  source 1..11074: mol_type = other RNA
tcaggccaggcacagtggctcatgcctgtagtcccagcactttgggaggccgaggtgggcagatccacgaggtcaggagatcaagaccatcctaacatggtaaaaccccatctctactaacaatacaaaaaattagtcaggtgtggtggcacgtgcctgtagtcccagctactcaggaggctgaggcaggagaatcgcttgaacctgggaggcggaggttgcagtgagccgagattgtgccactgcaccctagcctaggcaacagagcaagactctgtctcaaaaaaaataaaaaaaaaaaaaagagagaaagagagagagagatgaggagttgctgcactgctgggtgtggagagccgaggaggattcaaagatggtcctgaagtcccagctggaagaagtaggcggcagcaatgtttttaatactgtaaattcatcacgtagcacaggtttggggtggagaaagaaaaattgcattggcttcagggcatgcccagatctttcctcatcttaggcgtttgctaatacatgcattttctaagctgatgtcttgcgtttaatcactgctccattcaaaagagagaaggaggttgtttcaaacctagttgatatcatttgacttccatgctattcacagggctattttatttgaaacaggtataccacagccttaaattgcaagttaatccaggatgttcctaggttggcagttaggaacatgtaattctttggaagggctaaaagtcagctctttaaattatctccatatgaaccttctctccaccttagggtggatccacttatttagtccactgccagtaccacactagaacccgggtggtcactggactccagaaacaacagtagccctctctctgttctgtctctttttgactatctctattctgttcctgaccctgatttctcctgccaagctcaattttgacagctgacaacggcaagccatggcttcccaaaacattattttcaggtcaacttataaatttcaagaacacatttggctccgcttcctgtggtactaagcctacttcttgacagcatttgcctttgttgtaaatagcaaagttcttctagttggatttttgctaagaagtgtgtggatgtggcatgtgacgacatctttagcttggattctagaaaggcactaccattgtgcatttggctaaaggaaacacattttacccgtgaatgccttctatttacaaatgctcagctagcacacaaagctaagtacaagcaataagtactatcctacaatgttactcatttctgaaagcacaaaatgatgactggtatagctttggagatgttttctggaaacccaataaaggaacagatctttgttattccacacctacaaagtcagaagatgcacagtcttttattcatgtttgaacaagcttccttcttgaacaatcaactataaagtgatgtgattctctactagaccaggaactccttgaggacagaatgagggtctaatccatattctaaatccacaccacctggcacaatacatgttgcatggttagggtcaactaagagttggttgaattaatcaataacacacagcaagagaattcacaaagagaggggagtaatcccccagcctcaatcactcggcaagtggaatcgctgggcactgattccagctctgtctcagtgcttgagacagagctgaatgtaatgtgaacatttcaaatgaacaggaaaactagactcacggataagcagtgtagtcatcaagacaacactgtcttggaggtttttctgaagttaaaaccatgctacataagcaataaattatgaaggctgagcatgtgaataaaatttaatgttgtcataaattttataacaaagttaatctgacacatttaatgacatgcataatcattagtatgcagcactgtaatcagacattgataataagcagttcacaccagtgactgtaagagtctttacttgtgttcagccaagccaactgcttggtatatttttctcccttcttagtcgttagttttccatacctacaataactatcagtggtgatgggcttctctgaccatgtgaataatttaatcctcaatgcacagatacagaaacccttgctgaagacagtgtggagcagagaaggctgtctccactccttccacctgaaacacctctgcagatggatatgggagctctgcctacagcccttggacctaaccacttcagtgtgttccagtgagtgtctggacctcggcctgaaagatttttccgaaactaaagaaaatttctctgacctaaagaccttaacctccaccccagaagctctcaccaaggactacagggaactggtggggaaaatccttatcccttactcctcaaggcacagggcagtaatgctgaggcttgtgcgccacacttgctcccagaggtccccagcgggctacctgcggtggtgaatgacctcctaacacgccccttgacggccttcctttccttgcctcacttctccactctcctaccagcattgcagggttcacatcccaaatataccactggcacttgaatcctggtctccaggtctgtttctggaaaaacccaagtaagacattgccccagtaatggggctagatgtctgaggcttcctcaagtatctacctcgaaagctcttactgctgtacacacatgcacatacacacacgtgcgtacaaccagtcacatctaagcaccccgaataccagcctgttgaaggtagcagagagctgcactataagccaaggctgctcccaagagccgctccatcactgaattggcgccccagcaagatgaaggaatgtaatcattggaaggatggagaatgttctctgaatcactgacaaattggaaggggtggagggcaagagtccacctggtggagagatggaaagagcgagagagcctggaatgataatgccattgcttagaaaaggctgctccagatgccatatctacagaaattgtacagcccaaacatctctgagcaataggtctctggtagtcttgatgtctagaccaacaattcccagttcattcttctcagggaaggagccaggatagtccagagactctcattctgctgttagattgaaagggttaggcacaacagccttggcaaagtcacaagggcaaattcacactaaagtgtaaatgacccacaactcctcttctatttttaggttggggaggtgctttagaacataaggaggaactaaagaatattcctgttacatacaaggcagagaaaagggaaactagtggtgacaagacaaatcatccctttgacatttggctggctctacctattacagctctgggggtgaggtgggaacaaaaagatgctgtgtaaagaagtatcttatgccatccctactgtagtgaggtgcagtttagaggggacactgatcaagcagagacccagagtgtttcgttccaagccagaaacagaaatgtataaaacacagcctttccagcatcagaaatgagtagtggtagtggagaactacccaaaacaggaaagaggaccacgtgaggtagagtgtcaaggccctacattccagtgcctctgctcatgactgtaattttgggtaggtcacttaaagtctctggacctcagttttgccatctgtgaaatagggataatactatccagcataaaattggttatgaggctcatgtagggcctgcctgggatgatgtgttgctaatggttaagaacacaacttctggggtctgactggacaggctgaaatccctgcttaacacgttccagcagagccctgggcgatctatttaacttttgttttctcacctgtaagctgagacgaaagtacccactttataagattattccaataattagttgaaataatgcatgcagagaattaagcatggtacttgttatttgttaaactagctattaaaatgtgtaaaatataaagtattgtatggattttaggacaatgcaaagactctttgcttgctgcaatagttcggggccctttcagatggctaaaggcagaatttgtatgtgtaaatatggtgtgcttgtctctgctctggatactgagggcttaccctgttattaaacttatttagtaaatattgaactgtcatgaggcctaacatttagttccagttattagataaaacatttgctttgaatggtatttgaattgccaggttctagattattctggttgacaaactcttcgtattttataaagaggctaaaattggtaagctatcacagaacagatgtgccattttcaaggtatattaaaccatgattcactgtaacattgttcctactggcaacaaattcagagcaggctggactttatttggtgaagaaacattgagtggaagagaaatgacattattttatgtatttacattttcaaattactgtggcttaaacctgttcagccaacattacccaccttcagtctgctaaataaatgattcagtacatttctaatttacagaattttttaacaaaagaaaatgtaatttgatagccaaatcaacgttaaacattatacatttaaaaaaccacaggcaaagacacaaacatgatgacactaacttttgttaaagtatgcttacctatggtttcctctgaggcacgttctttcatgctaagcttccaacataatatgaaaatgaaggagatgcattttgcaaagcaaaacagaccttaagcaaaatattatacttctcaaattaacactgttacaaagttttagaatttaataagttcattaatttaaaagtttggatgtctgagtccttctatcccaaaacaagatcttggagggtcttccacagccatgtaataccatggtcacatgaccctttccaaaattattaatctgaatttactatatgaggataaatctatctttttgaaaatatttaggaaaatgagcttggtatttataaaatgaagctctctttgggtggtatcctaagacacgtcaagccaatcagcctgtaactgtgaaaaaaacattggtaggtacaaaagtggggtgggagaggagtgacttaactttgttaagtgatgggaaagaaacactaatagcattatctcaataaaatgtgatttaaaaaaatttaaaatactaaatcattgaactgacaaagaaatataaatcattcagaaataaactcattaggtcatcaaatcctgttaaatctgcaattaggaagagcaaggtgtacaatccatacatttaaactcacaggctcactttgcacaacgtcaatttactccttaatatgttattaatacgcattttccaaaaggatgtattagtaaatggtacacatctacttcttggcaacatcatataacctggtacaacataagcattcttcttatagttaagaaatgtggatggtatcaaaattagaaaaataaatgccctattatgttgtggtcaggtttaaggcatgtgaattttatcttcatacaaaagattaaaatctagatattaaaaagtagtgcagtatcagtgatgctgcctcagttcccaaaatgtcacatcacaaaaatatcccataattgcctgtagtttattccttggctttcctcttttctctctgcatctttgtaacaattttttaaaagtggaaatataattgttggcaatgctaacagctgtagaaatgattacaagatgtggaaaagcataacaggaatgtcaagaatctgtttctggcagtaatatatatggaacattgttcaggacaaaagaggagaaggaagaaaaaaaggagaggggtttatcatctctaagaattttcaaactaaacctcattgcttaataggaaaaaaagattccatatttaaagttaagtcacctctaactactagctaaagcatgacatcaccagcactggagtcagcggaagtgtgtttttgaaggacagtgttgcaggagaatctggacaggttttagagccaggagagagaaaataattctacctctgacagttgaaggaccttaggcaaatcagtttacctctgctagactacactccaaaatttggacattcaaaaatttgatattaataaccacatgaaagtctcgtgttgaggtgaatatgtatttgttggtgaaagatatgttggtttttaaacagacagcactctgcaattgtaggctattgttttgttttgccagttgtcaaattctatccagctatacacacttgtgtggcctcctaatggtgtttttccagtggctaaaggtttatgaataagacacttttcctaatggaattaacccgatgcttttcttaaacatgtaaccttgagttcaccgcaaaaaacaatgcttcgattagagcaatgcatataataaaggttaccctcgtttcttagacactagacatcattcacaaaaagagaactgcttttgaaagggatgtatttgcactggaaagaatagttttctacttctaattataaatgatttattggtgaaagcaaaacaacagcctgtctgagaggcacttctatgagcatcctcacgtgtgatttgcaaggttgaagaagagggaaaaatgcctcaattgtaccaatggtgagaaaacacccaaagtacaaagcaggtttcaaaaaaaccatactcataaccaaggacaataataaagcaatgtgttgacatatactctataagtcttcctccataaatagtttatagaaattttgtaatttctgtaaatgcatcctataataattttgcatcttgctttttttttacatttaatatcaagtagatttctaaagggcaattatttgaaaattatcccaaatacatggggaaatatacatcaagtgaaaaaatgcagtgggtgatagagatatcaggaagcgcctcaaatatttctcatctcgttggagaaaaacaaacatgttctcatttagaatgagtgggagttacctaattgatttaggcctctatatttaacttctagtcaaaaaaggtagttctatctagcaacaatattatggggaacaaaagaaaaaattaactctctaaatttgcagtagggtcttttcttcagaagtaccaaatcccatctattaccagctccatgcttcaggcctaaaatggatctccctgaagcaatgacagaatttttgccaagtgactaggatataaacaccactttggttgcacagtgagacatatgctccaaagaaaactggttcaaaaacaggcaagtgggtttctacagaataaatgagagccctgtcaatggcttcatcttcagggctttgtgtctgtgcttgcgtggtggctcttgtttcatctatggataatggtggcacacagttttcataattccttacattaatgaactgctataaatttgtttttggtattctagagagtcctaacttcagcttctgggcaatgctgaggaggcaccctatattctagacttaccttttgcaaggtgtactctcagcattgtgggcgatttccatgggagaatattctatttaaagaactactgtcccagcataaaacaaaaaatcatttatgaagatgcaggagactcggaaagctctcaattattgtttgcacaagcacaatgtcacagcctcctttccccattccacaagggggtcaggaagagagtactcagctgtgagaaaagacatacagaagaattcatgtggtcatgagagcgaggacatggccgatcccccaaggaggatgtgtcatacacttcatgagcccaagagtgtgctgtagggtctgaagggcaagatgctggttcactgatgtaaaggagagggaaaaaagcttcaaccaactagaaaaacagtctctatgcatgctatttttgattttaaacacaggtatcaattccttctctcagagagtccattttaaaataggatacatttttaaaggaatatttaaaggacacattcattaaaatttattttaaaaacttttcaaaagaaacaaaaggtatgaattttatttaatccttgaggaaatggttcttttctcacacacataaatcactcattttgtttttctttatctcctttattaatctacattagaaaaataaacttttcatacactaagaacaaggaaaccactctcaattgacaaaatgttccaatccaacacaatgattactttcacctttaatttacaggcagccagattcaaaatccttaaagttgcttaaacttaaaaatgacaatgacaacctaaaaggtataatgttgattggaacagacatttaattggaaaattgatgattttccatttccaattaaatctctagatagaaatgaaaaaaattaaaaatcgtatttaagaaaagccaaatcttgggttgtgaggtatctttttaaggatgtttcagcagaaaaaaacaaaggctctcacaattgtgtagctgcctagattaagtgggtatcctgatcaaggagatgggggatgatttggctttagtattccaatgataaagtttataatgagaataacatgttgctacaaaatccagtctcttcctcagatgccttccacagagggcaggaagctttgtcagttttgtttgctgatgatgcctggttccgtcaacaaataacacctgtcacacggtgggtagtcaatatacatttgttgaataaatatgaaaaaaagaaatgtacaatatgtttgtgaagccaactgtgtgtgcattgctattgaggtacacaaaaagtctttgttttaaatttgagaatgaggactttcaatggaatatatctataaaaatgaaaaaaagacattactgtctggacttttgtacagcaagagaagaaaaaccactagccaagagccaactcacctgataggcctggatcaagcatgcagctgtggagaacacccctgggactctaactctggcactctgcaagctgggtacttgggcaggacagcagcagcactcatgaactgggcagcacctgttggtgagggctgatcacatggattctctcatcccagccttacaatcagtccttcaggtacatactttttctgactttgctgatgaggaaactatgcacagaggttacacagcttaacaaagggttctcacctaatgaacaatgaaatgggattttagcctttctttgcatctggtcttagagccaatacccaagaagcactgtactgtatgcattgtctcagagaaacttactcttcctgggcctcagtctttaaaaggtgggcagttgacttaataagaattaaagatcaatgattaaggttcaaggcactccaaaattctggtctttattgaaaaggctacagaagtctcaccttaataataccctatagacttgatattcttggttaattaaatattggaaaccaatttcatagtaattgaggtcagaaaaaagtactcatgacattttagaatatgatgacaaagccatagataaatttcaatgcacctgtaattacttaaaactgttatagcatgcaatgtgttaccacaacagccagagaaatactaatttactcagcctattcttctagaccagtaaacactaggattaaatagatattttcattgaatttgttctacccttcattgccatttatagatagcttacttgtcatagattactttctaattgttttatgtttcctaactagcctgcaatactttggcaaggacctcaaacaatagtagacagtaggtgtaaaatagatggctacattgaacagatgactaaaaggatgcctcctaagtacctatatcttgaaatatatattattgtgccttgctttcaatttgtgattttaaaatctagaaatcacctgttttatgtaataacaataaaatccttctttgttgaaaacatgcacaaataaagtttacaagctcaaaaaattaaacagcagtaacggtcaagctttccaacaataaaatacattttggtaaggttttcattttacaaaaactcaaaatagctttatgagttcacaaaataatatgatatttttcaagatattaacatattcttataccggaagagcatagaataaaatttacttggagattgagcatttgcttctttaagaaatacttcttttagtatttttactttaatattatgaaagctacataattacattcagattcattaactactccagtagttaatttttaaaacttatgatgaatagttttgtttaaaatatataacattggtaatatgcaaatctgaatctgtaataaagaaggatttgcattcctgatttttttttctgatacaaccaatgacaaaataactaatggttccacagaggataaaatgtctcaaatctgttggttctgaaggtgaagcgagatttttgtactgataccgtgtatcactgagataccaggaggaaatggaattaaactcagatagttcaaatggagagattttaatgaagggacgacctacagaggtgtcggcagggttggggggaatcagcgagatatgcttagaacccaccgactggcaaacctccccctgaagatggagaaggaggaaggagtgttactggaatgagagcttgagtccaggggaggaggatgggctgctgaggaggcgacaccatcctgaaagaagaatcctctgccagaggcttttcagggtcatttcttcacactctctctcttcaagtggtatttaaatttcttctttcattttccttctggtaacaaagaagtctgtggctcaaaagatgtttctctaagaccccatcctattaggtctctgagctgtccacaaagaaatgaaattttcactttccaggaacctgagggccgacgagtgggggcgggcaggagggccgagggaggcggaacaggatcgaggcgcgaggcgggagtcgagaaagcgagcggccgaggcgactctcagtgcgcggacgcgggcgcgcgcccgcgctcccttcgtcgactcacggcgagagcccaaccctgctgccgcgcgccaccc

SEQ ID NO: 17594 - RNA, 15731 nt, Homo sapiens
  source 1..15731: mol_type = other RNA
tcaggccaggcacagtggctcatgcctgtagtcccagcactttgggaggccgaggtgggcagatccacgaggtcaggagatcaagaccatcctaacatggtaaaaccccatctctactaacaatacaaaaaattagtcaggtgtggtggcacgtgcctgtagtcccagctactcaggaggctgaggcaggagaatcgcttgaacctgggaggcggaggttgcagtgagccgagattgtgccactgcaccctagcctaggcaacagagcaagactctgtctcaaaaaaaataaaaaaaaaaaaaagagagaaagagagagagagatgaggagttgctgcactgctgggtgtggagagccgaggaggattcaaagatggtcctgaagtcccagctggaagaagtaggcggcagcaatgtttttaatactgtaaattcatcacgtagcacaggtttggggtggagaaagaaaaattgcattggcttcagggcatgcccagatctttcctcatcttaggcgtttgctaatacatgcattttctaagctgatgtcttgcgtttaatcactgctccattcaaaagagagaaggaggttgtttcaaacctagttgatatcatttgacttccatgctattcacagggctattttatttgaaacaggtataccacagccttaaattgcaagttaatccaggatgttcctaggttggcagttaggaacatgtaattctttggaagggctaaaagtcagctctttaaattatctccatatgaaccttctctccaccttagggtggatccacttatttagtccactgccagtaccacactagaacccgggtggtcactggactccagaaacaacagtagccctctctctgttctgtctctttttgactatctctattctgttcctgaccctgatttctcctgccaagctcaattttgacagctgacaacggcaagccatggcttcccaaaacattattttcaggtcaacttataaatttcaagaacacatttggctccgcttcctgtggtactaagcctacttcttgacagcatttgcctttgttgtaaatagcaaagttcttctagttggatttttgctaagaagtgtgtggatgtggcatgtgacgacatctttagcttggattctagaaaggcactaccattgtgcatttggctaaaggaaacacattttacccgtgaatgccttctatttacaaatgctcagctagcacacaaagctaagtacaagcaataagtactatcctacaatgttactcatttctgaaagcacaaaatgatgactggtatagctttggagatgttttctggaaacccaataaaggaacagatctttgttattccacacctacaaagtcagaagatgcacagtcttttattcatgtttgaacaagcttccttcttgaacaatcaactataaagtgatgtgattctctactagaccaggaactccttgaggacagaatgagggtctaatccatattctaaatccacaccacctggcacaatacatgttgcatggttagggtcaactaagagttggttgaattaatcaataacacacagcaagagaattcacaaagagaggggagtaatcccccagcctcaatcactcggcaagtggaatcgctgggcactgattccagctctgtctcagtgcttgagacagagctgaatgtaatgtgaacatttcaaatgaacaggaaaactagactcacggataagcagtgtagtcatcaagacaacactgtcttggaggtttttctgaagttaaaaccatgctacataagcaataaattatgaaggctgagcatgtgaataaaatttaatgttgtcataaattttataacaaagttaatctgacacatttaatgacatgcataatcattagtatgcagcactgtaatcagacattgataataagcagttcacaccagtgactgtaagagtctttacttgtgttcagccaagccaactgcttggtatatttttctcccttcttagtcgttagttttccatacctacaataactatcagtggtgatgggcttctctgaccatgtgaataatttaatcctcaatgcacagatacagaaacccttgctgaagacagtgtggagcagagaaggctgtctccactccttccacctgaaacacctctgcagatggatatgggagctctgcctacagcccttggacctaaccacttcagtgtgttccagtgagtgtctggacctcggcctgaaagatttttccgaaactaaagaaaatttctctgacctaaagaccttaacctccaccccagaagctctcaccaaggactacagggaactggtggggaaaatccttatcccttactcctcaaggcacagggcagtaatgctgaggcttgtgcgccacacttgctcccagaggtccccagcgggctacctgcggtggtgaatgacctcctaacacgccccttgacggccttcctttccttgcctcacttctccactctcctaccagcattgcagggttcacatcccaaatataccactggcacttgaatcctggtctccaggtctgtttctggaaaaacccaagtaagacattgccccagtaatggggctagatgtctgaggcttcctcaagtatctacctcgaaagctcttactgctgtacacacatgcacatacacacacgtgcgtacaaccagtcacatctaagcaccccgaataccagcctgttgaaggtagcagagagctgcactataagccaaggctgctcccaagagccgctccatcactgaattggcgccccagcaagatgaaggaatgtaatcattggaaggatggagaatgttctctgaatcactgacaaattggaaggggtggagggcaagagtccacctggtggagagatggaaagagcgagagagcctggaatgataatgccattgcttagaaaaggctgctccagatgccatatctacagaaattgtacagcccaaacatctctgagcaataggtctctggtagtcttgatgtctagaccaacaattcccagttcattcttctcagggaaggagccaggatagtccagagactctcattctgctgttagattgaaagggttaggcacaacagccttggcaaagtcacaagggcaaattcacactaaagtgtaaatgacccacaactcctcttctatttttaggttggggaggtgctttagaacataaggaggaactaaagaatattcctgttacatacaaggcagagaaaagggaaactagtggtgacaagacaaatcatccctttgacatttggctggctctacctattacagctctgggggtgaggtgggaacaaaaagatgctgtgtaaagaagtatcttatgccatccctactgtagtgaggtgcagtttagaggggacactgatcaagcagagacccagagtgtttcgttccaagccagaaacagaaatgtataaaacacagcctttccagcatcagaaatgagtagtggtagtggagaactacccaaaacaggaaagaggaccacgtgaggtagagtgtcaaggccctacattccagtgcctctgctcatgactgtaattttgggtaggtcacttaaagtctctggacctcagttttgccatctgtgaaatagggataatactatccagcataaaattggttatgaggctcatgtagggcctgcctgggatgatgtgttgctaatggttaagaacacaacttctggggtctgactggacaggctgaaatccctgcttaacacgttccagcagagccctgggcgatctatttaacttttgttttctcacctgtaagctgagacgaaagtacccactttataagattattccaataattagttgaaataatgcatgcagagaattaagcatggtacttgttatttgttaaactagctattaaaatgtgtaaaatataaagtattgtatggattttaggacaatgcaaagactctttgcttgctgcaatagttcggggccctttcagatggctaaaggcagaatttgtatgtgtaaatatggtgtgcttgtctctgctctggatactgagggcttaccctgttattaaacttatttagtaaatattgaactgtcatgaggcctaacatttagttccagttattagataaaacatttgctttgaatggtatttgaattgccaggttctagattattctggttgacaaactcttcgtattttataaagaggctaaaattggtaagctatcacagaacagatgtgccattttcaaggtatattaaaccatgattcactgtaacattgttcctactggcaacaaattcagagcaggctggactttatttggtgaagaaacattgagtggaagagaaatgacattattttatgtatttacattttcaaattactgtggcttaaacctgttcagccaacattacccaccttcagtctgctaaataaatgattcagtacatttctaatttacagaattttttaacaaaagaaaatgtaatttgatagccaaatcaacgttaaacattatacatttaaaaaaccacaggcaaagacacaaacatgatgacactaacttttgttaaagtatgcttacctatggtttcctctgaggcacgttctttcatgctaagcttccaacataatatgaaaatgaaggagatgcattttgcaaagcaaaacagaccttaagcaaaatattatacttctcaaattaacactgttacaaagttttagaatttaataagttcattaatttaaaagtttggatgtctgagtccttctatcccaaaacaagatcttggagggtcttccacagccatgtaataccatggtcacatgaccctttccaaaattattaatctgaatttactatatgaggataaatctatctttttgaaaatatttaggaaaatgagcttggtatttataaaatgaagctctctttgggtggtatcctaagacacgtcaagccaatcagcctgtaactgtgaaaaaaacattggtaggtacaaaagtggggtgggagaggagtgacttaactttgttaagtgatgggaaagaaacactaatagcattatctcaataaaatgtgatttaaaaaaatttaaaatactaaatcattgaactgacaaagaaatataaatcattcagaaataaactcattaggtcatcaaatcctgttaaatctgcaattaggaagagcaaggtgtacaatccatacatttaaactcacaggctcactttgcacaacgtcaatttactccttaatatgttattaatacgcattttccaaaaggatgtattagtaaatggtacacatctacttcttggcaacatcatataacctggtacaacataagcattcttcttatagttaagaaatgtggatggtatcaaaattagaaaaataaatgccctattatgttgtggtcaggtttaaggcatgtgaattttatcttcatacaaaagattaaaatctagatattaaaaagtagtgcagtatcagtgatgctgcctcagttcccaaaatgtcacatcacaaaaatatcccataattgcctgtagtttattccttggctttcctcttttctctctgcatctttgtaacaattttttaaaagtggaaatataattgttggcaatgctaacagctgtagaaatgattacaagatgtggaaaagcataacaggaatgtcaagaatctgtttctggcagtaatatatatggaacattgttcaggacaaaagaggagaaggaagaaaaaaaggagaggggtttatcatctctaagaattttcaaactaaacctcattgcttaataggaaaaaaagattccatatttaaagttaagtcacctctaactactagctaaagcatgacatcaccagcactggagtcagcggaagtgtgtttttgaaggacagtgttgcaggagaatctggacaggttttagagccaggagagagaaaataattctacctctgacagttgaaggaccttaggcaaatcagtttacctctgctagactacactccaaaatttggacattcaaaaatttgatattaataaccacatgaaagtctcgtgttgaggtgaatatgtatttgttggtgaaagatatgttggtttttaaacagacagcactctgcaattgtaggctattgttttgttttgccagttgtcaaattctatccagctatacacacttgtgtggcctcctaatggtgtttttccagtggctaaaggtttatgaataagacacttttcctaatggaattaacccgatgcttttcttaaacatgtaaccttgagttcaccgcaaaaaacaatgcttcgattagagcaatgcatataataaaggttaccctcgtttcttagacactagacatcattcacaaaaagagaactgcttttgaaagggatgtatttgcactggaaagaatagttttctacttctaattataaatgatttattggtgaaagcaaaacaacagcctgtctgagaggcacttctatgagcatcctcacgtgtgatttgcaaggttgaagaagagggaaaaatgcctcaattgtaccaatggtgagaaaacacccaaagtacaaagcaggtttcaaaaaaaccatactcataaccaaggacaataataaagcaatgtgttgacatatactctataagtcttcctccataaatagtttatagaaattttgtaatttctgtaaatgcatcctataataattttgcatcttgctttttttttacatttaatatcaagtagatttctaaagggcaattatttgaaaattatcccaaatacatggggaaatatacatcaagtgaaaaaatgcagtgggtgatagagatatcaggaagcgcctcaaatatttctcatctcgttggagaaaaacaaacatgttctcatttagaatgagtgggagttacctaattgatttaggcctctatatttaacttctagtcaaaaaaggtagttctatctagcaacaatattatggggaacaaaagaaaaaattaactctctaaatttgcagtagggtcttttcttcagaagtaccaaatcccatctattaccagctccatgcttcaggcctaaaatggatctccctgaagcaatgacagaatttttgccaagtgactaggatataaacaccactttggttgcacagtgagacatatgctccaaagaaaactggttcaaaaacaggcaagtgggtttctacagaataaatgagagccctgtcaatggcttcatcttcagggctttgtgtctgtgcttgcgtggtggctcttgtttcatctatggataatggtggcacacagttttcataattccttacattaatgaactgctataaatttgtttttggtattctagagagtcctaacttcagcttctgggcaatgctgaggaggcaccctatattctagacttaccttttgcaaggtgtactctcagcattgtgggcgatttccatgggagaatattctatttaaagaactactgtcccagcataaaacaaaaaatcatttatgaagatgcaggagactcggaaagctctcaattattgtttgcacaagcacaatgtcacagcctcctttccccattccacaagggggtcaggaagagagtactcagctgtgagaaaagacatacagaagaattcatgtggtcatgagagcgaggacatggccgatcccccaaggaggatgtgtcatacacttcatgagcccaagagtgtgctgtagggtctgaagggcaagatgctggttcactgatgtaaaggagagggaaaaaagcttcaaccaactagaaaaacagtctctatgcatgctatttttgattttaaacacaggtatcaattccttctctcagagagtccattttaaaataggatacatttttaaaggaatatttaaaggacacattcattaaaatttattttaaaaacttttcaaaagaaacaaaaggtatgaattttatttaatccttgaggaaatggttcttttctcacacacataaatcactcattttgtttttctttatctcctttattaatctacattagaaaaataaacttttcatacactaagaacaaggaaaccactctcaattgacaaaatgttccaatccaacacaatgattactttcacctttaatttacaggcagccagattcaaaatccttaaagttgcttaaacttaaaaatgacaatgacaacctaaaaggtataatgttgattggaacagacatttaattggaaaattgatgattttccatttccaattaaatctctagatagaaatgaaaaaaattaaaaatcgtatttaagaaaagccaaatcttgggttgtgaggtatctttttaaggatgtttcagcagaaaaaaacaaaggctctcacaattgtgtagctgcctagattaagtgggtatcctgatcaaggagatgggggatgatttggctttagtattccaatgataaagtttataatgagaataacatgttgctacaaaatccagtctcttcctcagatgccttccacagagggcaggaagctttgtcagttttgtttgctgatgatgcctggttccgtcaacaaataacacctgtcacacggtgggtagtcaatatacatttgttgaataaatatgaaaaaaagaaatgtacaatatgtttgtgaagccaactgtgtgtgcattgctattgaggtacacaaaaagtctttgttttaaatttgagaatgaggactttcaatggaatatatctataaaaatgaaaaaaagacattactgtctggacttttgtacagcaagagaagaaaaaccactagccaagagccaactcacctgataggcctggatcaagcatgcagctgtggagaacacccctgggactctaactctggcactctgcaagctgggtacttgggcaggacagcagcagcactcatgaactgggcagcacctgttggtgagggctgatcacatggattctctcatcccagccttacaatcagtccttcaggtacatactttttctgactttgctgatgaggaaactatgcacagaggttacacagcttaacaaagggttctcacctaatgaacaatgaaatgggattttagcctttctttgcatctggtcttagagccaatacccaagaagcactgtactgtatgcattgtctcagagaaacttactcttcctgggcctcagtctttaaaaggtgggcagttgacttaataagaattaaagatcaatgattaaggttcaaggcactccaaaattctggtctttattgaaaaggctacagaagtctcaccttaataataccctatagacttgatattcttggttaattaaatattggaaaccaatttcatagtaattgaggtcagaaaaaagtactcatgacattttagaatatgatgacaaagccatagataaatttcaatgcacctgtaattacttaaaactgttatagcatgcaatgtgttaccacaacagccagagaaatactaatttactcagcctattcttctagaccagtaaacactaggattaaatagatattttcattgaatttgttctacccttcattgccatttatagatagcttacttgtcatagattactttctaattgttttatgtttcctaactagcctgcaatactttggcaaggacctcaaacaatagtagacagtaggtgtaaaatagatggctacattgaacagatgactaaaaggatgcctcctaagtacctatatcttgaaatatatattattgtgccttgctttcaatttgtgattttaaaatctagaaatcacctgttttatgtaataacaataaaatccttctttgttgaaaacatgcacaaataaagtttacaagctcaaaaaattaaacagcagtaacggtcaagctttccaacaataaaatacattttggtaaggttttcattttacaaaaactcaaaatagctttatgagttcacaaaataatatgatatttttcaagatattaacatattcttataccggaagagcatagaataaaatttacttggagattgagcatttgcttctttaagaaatacttcttttagtatttttactttaatattatgaaagctacataattacattcagattcattaactactccagtagttaatttttaaaacttatgatgaatagttttgtttaaaatatataacattggtaatatgcaaatctgaatctgtaataaagaaggatttgcattcctgatttttttttctgatacaaccaatgacaaaataactaatggttccacagaggataaaatgtctcaaatctgttggttctgaaggtgaagcgagatttttgtactgataccgtgtatcactgagataccaggaggaaatggaattaaactcagatagttcaaatggagagattttaatgaagggacgacctacagaggtgtcggcagggttggggggaatcagcgagatatgcttagaacccaccgactggcaaacctccccctgaagatggagaaggaggaaggagtgttactggaatgagagcttgagtccaggggaggaggatgggctgctgaggaggcgacaccatcctgaaagaagaatcctctgccagaggcttttcagggtcatttcttcacactctctctcttcaagtggtatttaaatttcttctttcattttccttctggtaacaaagaagtctgtggctcaaaagatgtttctctaagaccccatcctattaggtctctgagctgtgggaagtatttatacaattgcttgtgaatataagatccaggaatttccctaagatccctaacaaaattggtgataagtagtcccacatgttaatccagccacccacggatgacagcacttaccatttctttgataaatgtcaaatgcatttgaagtacctacctgaaatatttgtttaaatgctatctaatctattaattttatatatgtgtgagtctgttttgtataccttctgattataggataaatgtaaataaatccaaagagtaatcaaagctaccactttcaagaagccttctttgtagaaccggaagagtcttaaataggcttttcaggtatgcatctcttattatcgctgaactccaagtcctgcaaggcaggcatcatgtgtgggtcacctttacagtaggcacaggccttaaaacagtgacatgcacattgcaggcactccataaatgtttgctgaattggctaaaccttggtttgttcccataatcaaccaccacaaacagcacacagataattacttcttggaaagattccaactagtgtttgatgttacctacgtggtttttctctcaagatcttaagagcagctctgtaggattacattattttctgttttttttttcctttgaccttaatgtcatctacttcaataacagcttcatacaaaattcctaccagcacataccacagcagattcaaggccttgttttaaaaatggtgccagcttctcttaatttggaagatatattgtctctcctgaacatgggctaagaaaatgtataatttggtattaacataagagctgaagacactttaaatgcattgtttcatttttataagataaaaaaaattttaagaatcaaaatgttatcaacagacttgtccttcattaaaaagtaaaactgcatttgcctacattttatgaaagtgtccaattatgaacaattttgaaatgtaacttttaaaaatgtaaacagcaaaaatgttgtatttaaaataaatctggaaaggcagaaaaacaaaaaatacccagaagacagagtttttggtgaaagttaagatatttcatctttgaacaacttagaatctttcctgcattttatagtctagttccaggcattaatttgaaataaccttggaatcctaaatctaacacccttcggaacaaagtagcttttctcttctgctttatgagcaaatggactaaatactagggaatggtactgtctgggcctttgaaccaagattgaaagagatgaaatcctatatgatatgtataaacattagagaatccattttgatttaataaaaggttgaatttgttctatatcctgtgagaaaatggttcccttttcctgaaaatgttacctcattccaacaatagaaagttggtttttttccagggtgtggtgttggcgggggacagagttgccatgaatatggcatctatgaagactgctgttatattcatttctcaaaatgcactgtggtaggaaattcagaacgcagtgagagaaaataaatgtttgacttcaaaatataaggccgcatttaaagcagaaggtaaagtatagaacagttgacagtataaattctttatctgcaatcttgcagttccctaaatctctgtaacacatcacttttaaaagcctcagataagtggttctataataatttaccaataattcaacccctcaaaagtcttagcaagttaaaccttataatcttacattttagaaatgacccaacttgatccttttattcttcagaatatctctctcaaattttcatttgtttttcattaattgatgaataatgagacattttaggtacctgtccacaaagaaatgaaattttcactttccaggaacctaacaaatgaaaagatagaaatcaattccaacagaatattaccaaagaaatcttttagaatggactgttaaaattatttatttgtatttatctggctctactatttgtggtacatttccacttcaaagctaaacctcaaataacatcatagtgagtggttgacttcatgtttaactgagatcttgaagactgaaaaagaccacgacaaacacacatctattttcttggctactgcatccgtgttcatcaccattctgatagtctgcaatgtattgcagctcaccctttgggaaggactaaagtagacatctgtttgttctgcttactcagcattcctaccctaattttcctttggagaacccctttattctagaccacgtgaagctaatgccaaaccccattccaggggatgcacctgaatccaacctccatcatctaaacagtgccttctccacgttcagagaagagcaagtgactcaaactgccctcataagaacagacctgggacttctgctgcaaatattgaagagtaagtactcttttttcttgctaggactaagctggtagtaccttctatgaggctatcatatggaaacaacttgtctgaaaatgaagccacaactagaaaacagatcctggtaacccggattgatggatccagccctaccttaaatggcaagacctaacccgaggctttttgcatcaaccaataaagtccttaagccagtttgagttggttttgtcacttgcagctaaaagaattctgactctaacaatgtgacaatagcaaaaataaacataactgcttttgaggtttctaatggattttcctccctatatacatgatttcatttaatcctcacaattcaggaaagcacatatctattaacattaaattaatattcattattttgaacacatgctatgtggataagggatgaggaaagccaaggaagtaatcaacgtgaaatctcacttatatgggagggaagtggaggttacatatctcagggcacttaacagatatcatcaaatgaaagaataaacagtgtgtgggagaggcagtaggtgattcttcatcaattcctggatgaaaaattaggagataatgaactccgaacaggcagcctaatgagaatggctcaagcaacaggacatagagagggagttaggttagacatggggttcttgggaattttcacctcgtgggggggcgggggggtcgtgcagctgttgtcagtgggaaagggaaaaaggaaaaggctgagtttggaaggcagggagggaggagacaatgtgagtcagtgaaaaagggcccttagaatgacaagtctggaccagagagaggctaagactgaaaatacaagttgggtaaccactggcatacagatggcagttcaggcttgggcactgcccaccagagcctcagcatgaagagaagagggggaggctggccaccacctccctctaggtaatcgtcatcctgatgctgagctcctgaaaacaggctctttcactcgccccatctcttgctcttgattgcaacccggcattcaggaggcaccctgtaatatctgtggagtgaccgacaacacagcgccagggcactgagaagatcccagggcgccagggactggttctacaagggtgcccctcccggtcccctccagcgcgccgccagagctgccagtcttggctgctacacgggaggcagcctcattatgcagctctcacctcttaaattagttcatgctctcacattaggtgtaatcacagcttgcaacgctttctggggatgtctcagaaagatctgagttgaaaaaatatttttgtgtcattttaatttaaagtaaaattgctgcttcttccccgcccctttctttcctcctggcccacccagcgaccctggccggccgtgctcaacgggggcgggggtcggaggtgagatttcctccacataattccttaaacagctatcaactaagtctcaaagaaaaaaaaaagagatctagaagcagagacgtggctgctggcgatcccaaagctggtgttcgctcttgggggagagcgtaccctgggggaggccgggaggccgggccagaggctagcccagaggcagagggcaggagcgctcagccggcgccccgcgtctctccagctcccgacgctgcgctggctccgctgagcacgccaggatcaaggtcgcctggtggggaccggagcgccaggagcctgtgggaagcgttccagccggcctctgactgggatccggcgccgcgtttctgctttggacttgactgacaggtccccccgccctcccgccgccctactaccagcctgggttcatccttcagggctacgtctaccgcacccgggctggaaagcctggagcgcgcccttcctctcctcatcttctcagctctcctttctccctgccacttggcaaagctgcattttgactttcacgttttggactacgtgtgtgtagttccaagtccatgcgtggcacgaaaatccacttagggtaaaaattattctcgaaaaatcgcccatctcaggatctggtgtctacactcaaggctaggaggtgcaggtacgggtgcgtaaagcatgccgtaagggtgcacagtaaataaaaagtacggatgcaaaatgtaaattttaagtgcaaaacagaaaagcagtactcgttgccgccccgcacgctgggttttaaggggcacgaaggtgggcctcggctgcttttgctcagccccgcgtcctcagcgcccggcccagtacccggtactccgtaggggttcaatgatctcccctgaataagtgaacgaattaacaaatgaatgaatgaccgctcgatccgacctccgcggccggcagagcagtcgctggagaggcgggagagagcgagaggccaagctccaccatcgcggccgccggctggggcagagggacacggagacactcggcgccccggctccgcaccgagtccccg

SEQ ID NO: 17595 - RNA, 11249 nt, Homo sapiens
  source 1..11249: mol_type = other RNA
tcaggccaggcacagtggctcatgcctgtagtcccagcactttgggaggccgaggtgggcagatccacgaggtcaggagatcaagaccatcctaacatggtaaaaccccatctctactaacaatacaaaaaattagtcaggtgtggtggcacgtgcctgtagtcccagctactcaggaggctgaggcaggagaatcgcttgaacctgggaggcggaggttgcagtgagccgagattgtgccactgcaccctagcctaggcaacagagcaagactctgtctcaaaaaaaataaaaaaaaaaaaaagagagaaagagagagagagatgaggagttgctgcactgctgggtgtggagagccgaggaggattcaaagatggtcctgaagtcccagctggaagaagtaggcggcagcaatgtttttaatactgtaaattcatcacgtagcacaggtttggggtggagaaagaaaaattgcattggcttcagggcatgcccagatctttcctcatcttaggcgtttgctaatacatgcattttctaagctgatgtcttgcgtttaatcactgctccattcaaaagagagaaggaggttgtttcaaacctagttgatatcatttgacttccatgctattcacagggctattttatttgaaacaggtataccacagccttaaattgcaagttaatccaggatgttcctaggttggcagttaggaacatgtaattctttggaagggctaaaagtcagctctttaaattatctccatatgaaccttctctccaccttagggtggatccacttatttagtccactgccagtaccacactagaacccgggtggtcactggactccagaaacaacagtagccctctctctgttctgtctctttttgactatctctattctgttcctgaccctgatttctcctgccaagctcaattttgacagctgacaacggcaagccatggcttcccaaaacattattttcaggtcaacttataaatttcaagaacacatttggctccgcttcctgtggtactaagcctacttcttgacagcatttgcctttgttgtaaatagcaaagttcttctagttggatttttgctaagaagtgtgtggatgtggcatgtgacgacatctttagcttggattctagaaaggcactaccattgtgcatttggctaaaggaaacacattttacccgtgaatgccttctatttacaaatgctcagctagcacacaaagctaagtacaagcaataagtactatcctacaatgttactcatttctgaaagcacaaaatgatgactggtatagctttggagatgttttctggaaacccaataaaggaacagatctttgttattccacacctacaaagtcagaagatgcacagtcttttattcatgtttgaacaagcttccttcttgaacaatcaactataaagtgatgtgattctctactagaccaggaactccttgaggacagaatgagggtctaatccatattctaaatccacaccacctggcacaatacatgttgcatggttagggtcaactaagagttggttgaattaatcaataacacacagcaagagaattcacaaagagaggggagtaatcccccagcctcaatcactcggcaagtggaatcgctgggcactgattccagctctgtctcagtgcttgagacagagctgaatgtaatgtgaacatttcaaatgaacaggaaaactagactcacggataagcagtgtagtcatcaagacaacactgtcttggaggtttttctgaagttaaaaccatgctacataagcaataaattatgaaggctgagcatgtgaataaaatttaatgttgtcataaattttataacaaagttaatctgacacatttaatgacatgcataatcattagtatgcagcactgtaatcagacattgataataagcagttcacaccagtgactgtaagagtctttacttgtgttcagccaagccaactgcttggtatatttttctcccttcttagtcgttagttttccatacctacaataactatcagtggtgatgggcttctctgaccatgtgaataatttaatcctcaatgcacagatacagaaacccttgctgaagacagtgtggagcagagaaggctgtctccactccttccacctgaaacacctctgcagatggatatgggagctctgcctacagcccttggacctaaccacttcagtgtgttccagtgagtgtctggacctcggcctgaaagatttttccgaaactaaagaaaatttctctgacctaaagaccttaacctccaccccagaagctctcaccaaggactacagggaactggtggggaaaatccttatcccttactcctcaaggcacagggcagtaatgctgaggcttgtgcgccacacttgctcccagaggtccccagcgggctacctgcggtggtgaatgacctcctaacacgccccttgacggccttcctttccttgcctcacttctccactctcctaccagcattgcagggttcacatcccaaatataccactggcacttgaatcctggtctccaggtctgtttctggaaaaacccaagtaagacattgccccagtaatggggctagatgtctgaggcttcctcaagtatctacctcgaaagctcttactgctgtacacacatgcacatacacacacgtgcgtacaaccagtcacatctaagcaccccgaataccagcctgttgaaggtagcagagagctgcactataagccaaggctgctcccaagagccgctccatcactgaattggcgccccagcaagatgaaggaatgtaatcattggaaggatggagaatgttctctgaatcactgacaaattggaaggggtggagggcaagagtccacctggtggagagatggaaagagcgagagagcctggaatgataatgccattgcttagaaaaggctgctccagatgccatatctacagaaattgtacagcccaaacatctctgagcaataggtctctggtagtcttgatgtctagaccaacaattcccagttcattcttctcagggaaggagccaggatagtccagagactctcattctgctgttagattgaaagggttaggcacaacagccttggcaaagtcacaagggcaaattcacactaaagtgtaaatgacccacaactcctcttctatttttaggttggggaggtgctttagaacataaggaggaactaaagaatattcctgttacatacaaggcagagaaaagggaaactagtggtgacaagacaaatcatccctttgacatttggctggctctacctattacagctctgggggtgaggtgggaacaaaaagatgctgtgtaaagaagtatcttatgccatccctactgtagtgaggtgcagtttagaggggacactgatcaagcagagacccagagtgtttcgttccaagccagaaacagaaatgtataaaacacagcctttccagcatcagaaatgagtagtggtagtggagaactacccaaaacaggaaagaggaccacgtgaggtagagtgtcaaggccctacattccagtgcctctgctcatgactgtaattttgggtaggtcacttaaagtctctggacctcagttttgccatctgtgaaatagggataatactatccagcataaaattggttatgaggctcatgtagggcctgcctgggatgatgtgttgctaatggttaagaacacaacttctggggtctgactggacaggctgaaatccctgcttaacacgttccagcagagccctgggcgatctatttaacttttgttttctcacctgtaagctgagacgaaagtacccactttataagattattccaataattagttgaaataatgcatgcagagaattaagcatggtacttgttatttgttaaactagctattaaaatgtgtaaaatataaagtattgtatggattttaggacaatgcaaagactctttgcttgctgcaatagttcggggccctttcagatggctaaaggcagaatttgtatgtgtaaatatggtgtgcttgtctctgctctggatactgagggcttaccctgttattaaacttatttagtaaatattgaactgtcatgaggcctaacatttagttccagttattagataaaacatttgctttgaatggtatttgaattgccaggttctagattattctggttgacaaactcttcgtattttataaagaggctaaaattggtaagctatcacagaacagatgtgccattttcaaggtatattaaaccatgattcactgtaacattgttcctactggcaacaaattcagagcaggctggactttatttggtgaagaaacattgagtggaagagaaatgacattattttatgtatttacattttcaaattactgtggcttaaacctgttcagccaacattacccaccttcagtctgctaaataaatgattcagtacatttctaatttacagaattttttaacaaaagaaaatgtaatttgatagccaaatcaacgttaaacattatacatttaaaaaaccacaggcaaagacacaaacatgatgacactaacttttgttaaagtatgcttacctatggtttcctctgaggcacgttctttcatgctaagcttccaacataatatgaaaatgaaggagatgcattttgcaaagcaaaacagaccttaagcaaaatattatacttctcaaattaacactgttacaaagttttagaatttaataagttcattaatttaaaagtttggatgtctgagtccttctatcccaaaacaagatcttggagggtcttccacagccatgtaataccatggtcacatgaccctttccaaaattattaatctgaatttactatatgaggataaatctatctttttgaaaatatttaggaaaatgagcttggtatttataaaatgaagctctctttgggtggtatcctaagacacgtcaagccaatcagcctgtaactgtgaaaaaaacattggtaggtacaaaagtggggtgggagaggagtgacttaactttgttaagtgatgggaaagaaacactaatagcattatctcaataaaatgtgatttaaaaaaatttaaaatactaaatcattgaactgacaaagaaatataaatcattcagaaataaactcattaggtcatcaaatcctgttaaatctgcaattaggaagagcaaggtgtacaatccatacatttaaactcacaggctcactttgcacaacgtcaatttactccttaatatgttattaatacgcattttccaaaaggatgtattagtaaatggtacacatctacttcttggcaacatcatataacctggtacaacataagcattcttcttatagttaagaaatgtggatggtatcaaaattagaaaaataaatgccctattatgttgtggtcaggtttaaggcatgtgaattttatcttcatacaaaagattaaaatctagatattaaaaagtagtgcagtatcagtgatgctgcctcagttcccaaaatgtcacatcacaaaaatatcccataattgcctgtagtttattccttggctttcctcttttctctctgcatctttgtaacaattttttaaaagtggaaatataattgttggcaatgctaacagctgtagaaatgattacaagatgtggaaaagcataacaggaatgtcaagaatctgtttctggcagtaatatatatggaacattgttcaggacaaaagaggagaaggaagaaaaaaaggagaggggtttatcatctctaagaattttcaaactaaacctcattgcttaataggaaaaaaagattccatatttaaagttaagtcacctctaactactagctaaagcatgacatcaccagcactggagtcagcggaagtgtgtttttgaaggacagtgttgcaggagaatctggacaggttttagagccaggagagagaaaataattctacctctgacagttgaaggaccttaggcaaatcagtttacctctgctagactacactccaaaatttggacattcaaaaatttgatattaataaccacatgaaagtctcgtgttgaggtgaatatgtatttgttggtgaaagatatgttggtttttaaacagacagcactctgcaattgtaggctattgttttgttttgccagttgtcaaattctatccagctatacacacttgtgtggcctcctaatggtgtttttccagtggctaaaggtttatgaataagacacttttcctaatggaattaacccgatgcttttcttaaacatgtaaccttgagttcaccgcaaaaaacaatgcttcgattagagcaatgcatataataaaggttaccctcgtttcttagacactagacatcattcacaaaaagagaactgcttttgaaagggatgtatttgcactggaaagaatagttttctacttctaattataaatgatttattggtgaaagcaaaacaacagcctgtctgagaggcacttctatgagcatcctcacgtgtgatttgcaaggttgaagaagagggaaaaatgcctcaattgtaccaatggtgagaaaacacccaaagtacaaagcaggtttcaaaaaaaccatactcataaccaaggacaataataaagcaatgtgttgacatatactctataagtcttcctccataaatagtttatagaaattttgtaatttctgtaaatgcatcctataataattttgcatcttgctttttttttacatttaatatcaagtagatttctaaagggcaattatttgaaaattatcccaaatacatggggaaatatacatcaagtgaaaaaatgcagtgggtgatagagatatcaggaagcgcctcaaatatttctcatctcgttggagaaaaacaaacatgttctcatttagaatgagtgggagttacctaattgatttaggcctctatatttaacttctagtcaaaaaaggtagttctatctagcaacaatattatggggaacaaaagaaaaaattaactctctaaatttgcagtagggtcttttcttcagaagtaccaaatcccatctattaccagctccatgcttcaggcctaaaatggatctccctgaagcaatgacagaatttttgccaagtgactaggatataaacaccactttggttgcacagtgagacatatgctccaaagaaaactggttcaaaaacaggcaagtgggtttctacagaataaatgagagccctgtcaatggcttcatcttcagggctttgtgtctgtgcttgcgtggtggctcttgtttcatctatggataatggtggcacacagttttcataattccttacattaatgaactgctataaatttgtttttggtattctagagagtcctaacttcagcttctgggcaatgctgaggaggcaccctatattctagacttaccttttgcaaggtgtactctcagcattgtgggcgatttccatgggagaatattctatttaaagaactactgtcccagcataaaacaaaaaatcatttatgaagatgcaggagactcggaaagctctcaattattgtttgcacaagcacaatgtcacagcctcctttccccattccacaagggggtcaggaagagagtactcagctgtgagaaaagacatacagaagaattcatgtggtcatgagagcgaggacatggccgatcccccaaggaggatgtgtcatacacttcatgagcccaagagtgtgctgtagggtctgaagggcaagatgctggttcactgatgtaaaggagagggaaaaaagcttcaaccaactagaaaaacagtctctatgcatgctatttttgattttaaacacaggtatcaattccttctctcagagagtccattttaaaataggatacatttttaaaggaatatttaaaggacacattcattaaaatttattttaaaaacttttcaaaagaaacaaaaggtatgaattttatttaatccttgaggaaatggttcttttctcacacacataaatcactcattttgtttttctttatctcctttattaatctacattagaaaaataaacttttcatacactaagaacaaggaaaccactctcaattgacaaaatgttccaatccaacacaatgattactttcacctttaatttacaggcagccagattcaaaatccttaaagttgcttaaacttaaaaatgacaatgacaacctaaaaggtataatgttgattggaacagacatttaattggaaaattgatgattttccatttccaattaaatctctagatagaaatgaaaaaaattaaaaatcgtatttaagaaaagccaaatcttgggttgtgaggtatctttttaaggatgtttcagcagaaaaaaacaaaggctctcacaattgtgtagctgcctagattaagtgggtatcctgatcaaggagatgggggatgatttggctttagtattccaatgataaagtttataatgagaataacatgttgctacaaaatccagtctcttcctcagatgccttccacagagggcaggaagctttgtcagttttgtttgctgatgatgcctggttccgtcaacaaataacacctgtcacacggtgggtagtcaatatacatttgttgaataaatatgaaaaaaagaaatgtacaatatgtttgtgaagccaactgtgtgtgcattgctattgaggtacacaaaaagtctttgttttaaatttgagaatgaggactttcaatggaatatatctataaaaatgaaaaaaagacattactgtctggacttttgtacagcaagagaagaaaaaccactagccaagagccaactcacctgataggcctggatcaagcatgcagctgtggagaacacccctgggactctaactctggcactctgcaagctgggtacttgggcaggacagcagcagcactcatgaactgggcagcacctgttggtgagggctgatcacatggattctctcatcccagccttacaatcagtccttcaggtacatactttttctgactttgctgatgaggaaactatgcacagaggttacacagcttaacaaagggttctcacctaatgaacaatgaaatgggattttagcctttctttgcatctggtcttagagccaatacccaagaagcactgtactgtatgcattgtctcagagaaacttactcttcctgggcctcagtctttaaaaggtgggcagttgacttaataagaattaaagatcaatgattaaggttcaaggcactccaaaattctggtctttattgaaaaggctacagaagtctcaccttaataataccctatagacttgatattcttggttaattaaatattggaaaccaatttcatagtaattgaggtcagaaaaaagtactcatgacattttagaatatgatgacaaagccatagataaatttcaatgcacctgtaattacttaaaactgttatagcatgcaatgtgttaccacaacagccagagaaatactaatttactcagcctattcttctagaccagtaaacactaggattaaatagatattttcattgaatttgttctacccttcattgccatttatagatagcttacttgtcatagattactttctaattgttttatgtttcctaactagcctgcaatactttggcaaggacctcaaacaatagtagacagtaggtgtaaaatagatggctacattgaacagatgactaaaaggatgcctcctaagtacctatatcttgaaatatatattattgtgccttgctttcaatttgtgattttaaaatctagaaatcacctgttttatgtaataacaataaaatccttctttgttgaaaacatgcacaaataaagtttacaagctcaaaaaattaaacagcagtaacggtcaagctttccaacaataaaatacattttggtaaggttttcattttacaaaaactcaaaatagctttatgagttcacaaaataatatgatatttttcaagatattaacatattcttataccggaagagcatagaataaaatttacttggagattgagcatttgcttctttaagaaatacttcttttagtatttttactttaatattatgaaagctacataattacattcagattcattaactactccagtagttaatttttaaaacttatgatgaatagttttgtttaaaatatataacattggtaatatgcaaatctgaatctgtaataaagaaggatttgcattcctgatttttttttctgatacaaccaatgacaaaataactaatggttccacagaggataaaatgtctcaaatctgttggttctgaaggtgaagcgagatttttgtactgataccgtgtatcactgagataccaggaggaaatggaattaaactcagatagttcaaatggagagattttaatgaagggacgacctacagaggtgtcggcagggttggggggaatcagcgagatatgcttagaacccaccgactggcaaacctccccctgaagatggagaaggaggaaggagtgttactggaatgagagcttgagtccaggggaggaggatgggctgctgaggaggcgacaccatcctgaaagaagaatcctctgccagaggcttttcagggtcatttcttcacactctctgcagggaagcacggagacagcaggaagaaatatcctaacctcactctcttccctctacaggtgcttccattggccaaatccacccagaggccagttggtggcgatcagctctcttcaagtggtatttaaatttcttctttcattttccttctggtaacaaagaagtctgtggctcaaaagatgtttctctaagaccccatcctattaggtctctgagattttagaaatgacccaacttgatccttttattcttcagaatatctctctcaaattttcatttgtttttcattaattgatgaataatgagacattttaggtacctgagggccgacgagtgggggcgggcaggagggccgagggaggcggaacaggatcgaggcgcgaggcgggagtcgagaaagcgagcggccgaggcgactctcagtgcgcggacgcgggcgcgcgcccgcgctcccttcgtcgactcacggcgagagcccaaccctgctgccgcgcgccaccc

SEQ ID NO: 17596 - RNA, 14098 nt, Homo sapiens
  source 1..14098: mol_type = other RNA
tcaggccaggcacagtggctcatgcctgtagtcccagcactttgggaggccgaggtgggcagatccacgaggtcaggagatcaagaccatcctaacatggtaaaaccccatctctactaacaatacaaaaaattagtcaggtgtggtggcacgtgcctgtagtcccagctactcaggaggctgaggcaggagaatcgcttgaacctgggaggcggaggttgcagtgagccgagattgtgccactgcaccctagcctaggcaacagagcaagactctgtctcaaaaaaaataaaaaaaaaaaaaagagagaaagagagagagagatgaggagttgctgcactgctgggtgtggagagccgaggaggattcaaagatggtcctgaagtcccagctggaagaagtaggcggcagcaatgtttttaatactgtaaattcatcacgtagcacaggtttggggtggagaaagaaaaattgcattggcttcagggcatgcccagatctttcctcatcttaggcgtttgctaatacatgcattttctaagctgatgtcttgcgtttaatcactgctccattcaaaagagagaaggaggttgtttcaaacctagttgatatcatttgacttccatgctattcacagggctattttatttgaaacaggtataccacagccttaaattgcaagttaatccaggatgttcctaggttggcagttaggaacatgtaattctttggaagggctaaaagtcagctctttaaattatctccatatgaaccttctctccaccttagggtggatccacttatttagtccactgccagtaccacactagaacccgggtggtcactggactccagaaacaacagtagccctctctctgttctgtctctttttgactatctctattctgttcctgaccctgatttctcctgccaagctcaattttgacagctgacaacggcaagccatggcttcccaaaacattattttcaggtcaacttataaatttcaagaacacatttggctccgcttcctgtggtactaagcctacttcttgacagcatttgcctttgttgtaaatagcaaagttcttctagttggatttttgctaagaagtgtgtggatgtggcatgtgacgacatctttagcttggattctagaaaggcactaccattgtgcatttggctaaaggaaacacattttacccgtgaatgccttctatttacaaatgctcagctagcacacaaagctaagtacaagcaataagtactatcctacaatgttactcatttctgaaagcacaaaatgatgactggtatagctttggagatgttttctggaaacccaataaaggaacagatctttgttattccacacctacaaagtcagaagatgcacagtcttttattcatgtttgaacaagcttccttcttgaacaatcaactataaagtgatgtgattctctactagaccaggaactccttgaggacagaatgagggtctaatccatattctaaatccacaccacctggcacaatacatgttgcatggttagggtcaactaagagttggttgaattaatcaataacacacagcaagagaattcacaaagagaggggagtaatcccccagcctcaatcactcggcaagtggaatcgctgggcactgattccagctctgtctcagtgcttgagacagagctgaatgtaatgtgaacatttcaaatgaacaggaaaactagactcacggataagcagtgtagtcatcaagacaacactgtcttggaggtttttctgaagttaaaaccatgctacataagcaataaattatgaaggctgagcatgtgaataaaatttaatgttgtcataaattttataacaaagttaatctgacacatttaatgacatgcataatcattagtatgcagcactgtaatcagacattgataataagcagttcacaccagtgactgtaagagtctttacttgtgttcagccaagccaactgcttggtatatttttctcccttcttagtcgttagttttccatacctacaataactatcagtggtgatgggcttctctgaccatgtgaataatttaatcctcaatgcacagatacagaaacccttgctgaagacagtgtggagcagagaaggctgtctccactccttccacctgaaacacctctgcagatggatatgggagctctgcctacagcccttggacctaaccacttcagtgtgttccagtgagtgtctggacctcggcctgaaagatttttccgaaactaaagaaaatttctctgacctaaagaccttaacctccaccccagaagctctcaccaaggactacagggaactggtggggaaaatccttatcccttactcctcaaggcacagggcagtaatgctgaggcttgtgcgccacacttgctcccagaggtccccagcgggctacctgcggtggtgaatgacctcctaacacgccccttgacggccttcctttccttgcctcacttctccactctcctaccagcattgcagggttcacatcccaaatataccactggcacttgaatcctggtctccaggtctgtttctggaaaaacccaagtaagacattgccccagtaatggggctagatgtctgaggcttcctcaagtatctacctcgaaagctcttactgctgtacacacatgcacatacacacacgtgcgtacaaccagtcacatctaagcaccccgaataccagcctgttgaaggtagcagagagctgcactataagccaaggctgctcccaagagccgctccatcactgaattggcgccccagcaagatgaaggaatgtaatcattggaaggatggagaatgttctctgaatcactgacaaattggaaggggtggagggcaagagtccacctggtggagagatggaaagagcgagagagcctggaatgataatgccattgcttagaaaaggctgctccagatgccatatctacagaaattgtacagcccaaacatctctgagcaataggtctctggtagtcttgatgtctagaccaacaattcccagttcattcttctcagggaaggagccaggatagtccagagactctcattctgctgttagattgaaagggttaggcacaacagccttggcaaagtcacaagggcaaattcacactaaagtgtaaatgacccacaactcctcttctatttttaggttggggaggtgctttagaacataaggaggaactaaagaatattcctgttacatacaaggcagagaaaagggaaactagtggtgacaagacaaatcatccctttgacatttggctggctctacctattacagctctgggggtgaggtgggaacaaaaagatgctgtgtaaagaagtatcttatgccatccctactgtagtgaggtgcagtttagaggggacactgatcaagcagagacccagagtgtttcgttccaagccagaaacagaaatgtataaaacacagcctttccagcatcagaaatgagtagtggtagtggagaactacccaaaacaggaaagaggaccacgtgaggtagagtgtcaaggccctacattccagtgcctctgctcatgactgtaattttgggtaggtcacttaaagtctctggacctcagttttgccatctgtgaaatagggataatactatccagcataaaattggttatgaggctcatgtagggcctgcctgggatgatgtgttgctaatggttaagaacacaacttctggggtctgactggacaggctgaaatccctgcttaacacgttccagcagagccctgggcgatctatttaacttttgttttctcacctgtaagctgagacgaaagtacccactttataagattattccaataattagttgaaataatgcatgcagagaattaagcatggtacttgttatttgttaaactagctattaaaatgtgtaaaatataaagtattgtatggattttaggacaatgcaaagactctttgcttgctgcaatagttcggggccctttcagatggctaaaggcagaatttgtatgtgtaaatatggtgtgcttgtctctgctctggatactgagggcttaccctgttattaaacttatttagtaaatattgaactgtcatgaggcctaacatttagttccagttattagataaaacatttgctttgaatggtatttgaattgccaggttctagattattctggttgacaaactcttcgtattttataaagaggctaaaattggtaagctatcacagaacagatgtgccattttcaaggtatattaaaccatgattcactgtaacattgttcctactggcaacaaattcagagcaggctggactttatttggtgaagaaacattgagtggaagagaaatgacattattttatgtatttacattttcaaattactgtggcttaaacctgttcagccaacattacccaccttcagtctgctaaataaatgattcagtacatttctaatttacagaattttttaacaaaagaaaatgtaatttgatagccaaatcaacgttaaacattatacatttaaaaaaccacaggcaaagacacaaacatgatgacactaacttttgttaaagtatgcttacctatggtttcctctgaggcacgttctttcatgctaagcttccaacataatatgaaaatgaaggagatgcattttgcaaagcaaaacagaccttaagcaaaatattatacttctcaaattaacactgttacaaagttttagaatttaataagttcattaatttaaaagtttggatgtctgagtccttctatcccaaaacaagatcttggagggtcttccacagccatgtaataccatggtcacatgaccctttccaaaattattaatctgaatttactatatgaggataaatctatctttttgaaaatatttaggaaaatgagcttggtatttataaaatgaagctctctttgggtggtatcctaagacacgtcaagccaatcagcctgtaactgtgaaaaaaacattggtaggtacaaaagtggggtgggagaggagtgacttaactttgttaagtgatgggaaagaaacactaatagcattatctcaataaaatgtgatttaaaaaaatttaaaatactaaatcattgaactgacaaagaaatataaatcattcagaaataaactcattaggtcatcaaatcctgttaaatctgcaattaggaagagcaaggtgtacaatccatacatttaaactcacaggctcactttgcacaacgtcaatttactccttaatatgttattaatacgcattttccaaaaggatgtattagtaaatggtacacatctacttcttggcaacatcatataacctggtacaacataagcattcttcttatagttaagaaatgtggatggtatcaaaattagaaaaataaatgccctattatgttgtggtcaggtttaaggcatgtgaattttatcttcatacaaaagattaaaatctagatattaaaaagtagtgcagtatcagtgatgctgcctcagttcccaaaatgtcacatcacaaaaatatcccataattgcctgtagtttattccttggctttcctcttttctctctgcatctttgtaacaattttttaaaagtggaaatataattgttggcaatgctaacagctgtagaaatgattacaagatgtggaaaagcataacaggaatgtcaagaatctgtttctggcagtaatatatatggaacattgttcaggacaaaagaggagaaggaagaaaaaaaggagaggggtttatcatctctaagaattttcaaactaaacctcattgcttaataggaaaaaaagattccatatttaaagttaagtcacctctaactactagctaaagcatgacatcaccagcactggagtcagcggaagtgtgtttttgaaggacagtgttgcaggagaatctggacaggttttagagccaggagagagaaaataattctacctctgacagttgaaggaccttaggcaaatcagtttacctctgctagactacactccaaaatttggacattcaaaaatttgatattaataaccacatgaaagtctcgtgttgaggtgaatatgtatttgttggtgaaagatatgttggtttttaaacagacagcactctgcaattgtaggctattgttttgttttgccagttgtcaaattctatccagctatacacacttgtgtggcctcctaatggtgtttttccagtggctaaaggtttatgaataagacacttttcctaatggaattaacccgatgcttttcttaaacatgtaaccttgagttcaccgcaaaaaacaatgcttcgattagagcaatgcatataataaaggttaccctcgtttcttagacactagacatcattcacaaaaagagaactgcttttgaaagggatgtatttgcactggaaagaatagttttctacttctaattataaatgatttattggtgaaagcaaaacaacagcctgtctgagaggcacttctatgagcatcctcacgtgtgatttgcaaggttgaagaagagggaaaaatgcctcaattgtaccaatggtgagaaaacacccaaagtacaaagcaggtttcaaaaaaaccatactcataaccaaggacaataataaagcaatgtgttgacatatactctataagtcttcctccataaatagtttatagaaattttgtaatttctgtaaatgcatcctataataattttgcatcttgctttttttttacatttaatatcaagtagatttctaaagggcaattatttgaaaattatcccaaatacatggggaaatatacatcaagtgaaaaaatgcagtgggtgatagagatatcaggaagcgcctcaaatatttctcatctcgttggagaaaaacaaacatgttctcatttagaatgagtgggagttacctaattgatttaggcctctatatttaacttctagtcaaaaaaggtagttctatctagcaacaatattatggggaacaaaagaaaaaattaactctctaaatttgcagtagggtcttttcttcagaagtaccaaatcccatctattaccagctccatgcttcaggcctaaaatggatctccctgaagcaatgacagaatttttgccaagtgactaggatataaacaccactttggttgcacagtgagacatatgctccaaagaaaactggttcaaaaacaggcaagtgggtttctacagaataaatgagagccctgtcaatggcttcatcttcagggctttgtgtctgtgcttgcgtggtggctcttgtttcatctatggataatggtggcacacagttttcataattccttacattaatgaactgctataaatttgtttttggtattctagagagtcctaacttcagcttctgggcaatgctgaggaggcaccctatattctagacttaccttttgcaaggtgtactctcagcattgtgggcgatttccatgggagaatattctatttaaagaactactgtcccagcataaaacaaaaaatcatttatgaagatgcaggagactcggaaagctctcaattattgtttgcacaagcacaatgtcacagcctcctttccccattccacaagggggtcaggaagagagtactcagctgtgagaaaagacatacagaagaattcatgtggtcatgagagcgaggacatggccgatcccccaaggaggatgtgtcatacacttcatgagcccaagagtgtgctgtagggtctgaagggcaagatgctggttcactgatgtaaaggagagggaaaaaagcttcaaccaactagaaaaacagtctctatgcatgctatttttgattttaaacacaggtatcaattccttctctcagagagtccattttaaaataggatacatttttaaaggaatatttaaaggacacattcattaaaatttattttaaaaacttttcaaaagaaacaaaaggtatgaattttatttaatccttgaggaaatggttcttttctcacacacataaatcactcattttgtttttctttatctcctttattaatctacattagaaaaataaacttttcatacactaagaacaaggaaaccactctcaattgacaaaatgttccaatccaacacaatgattactttcacctttaatttacaggcagccagattcaaaatccttaaagttgcttaaacttaaaaatgacaatgacaacctaaaaggtataatgttgattggaacagacatttaattggaaaattgatgattttccatttccaattaaatctctagatagaaatgaaaaaaattaaaaatcgtatttaagaaaagccaaatcttgggttgtgaggtatctttttaaggatgtttcagcagaaaaaaacaaaggctctcacaattgtgtagctgcctagattaagtgggtatcctgatcaaggagatgggggatgatttggctttagtattccaatgataaagtttataatgagaataacatgttgctacaaaatccagtctcttcctcagatgccttccacagagggcaggaagctttgtcagttttgtttgctgatgatgcctggttccgtcaacaaataacacctgtcacacggtgggtagtcaatatacatttgttgaataaatatgaaaaaaagaaatgtacaatatgtttgtgaagccaactgtgtgtgcattgctattgaggtacacaaaaagtctttgttttaaatttgagaatgaggactttcaatggaatatatctataaaaatgaaaaaaagacattactgtctggacttttgtacagcaagagaagaaaaaccactagccaagagccaactcacctgataggcctggatcaagcatgcagctgtggagaacacccctgggactctaactctggcactctgcaagctgggtacttgggcaggacagcagcagcactcatgaactgggcagcacctgttggtgagggctgatcacatggattctctcatcccagccttacaatcagtccttcaggtacatactttttctgactttgctgatgaggaaactatgcacagaggttacacagcttaacaaagggttctcacctaatgaacaatgaaatgggattttagcctttctttgcatctggtcttagagccaatacccaagaagcactgtactgtatgcattgtctcagagaaacttactcttcctgggcctcagtctttaaaaggtgggcagttgacttaataagaattaaagatcaatgattaaggttcaaggcactccaaaattctggtctttattgaaaaggctacagaagtctcaccttaataataccctatagacttgatattcttggttaattaaatattggaaaccaatttcatagtaattgaggtcagaaaaaagtactcatgacattttagaatatgatgacaaagccatagataaatttcaatgcacctgtaattacttaaaactgttatagcatgcaatgtgttaccacaacagccagagaaatactaatttactcagcctattcttctagaccagtaaacactaggattaaatagatattttcattgaatttgttctacccttcattgccatttatagatagcttacttgtcatagattactttctaattgttttatgtttcctaactagcctgcaatactttggcaaggacctcaaacaatagtagacagtaggtgtaaaatagatggctacattgaacagatgactaaaaggatgcctcctaagtacctatatcttgaaatatatattattgtgccttgctttcaatttgtgattttaaaatctagaaatcacctgttttatgtaataacaataaaatccttctttgttgaaaacatgcacaaataaagtttacaagctcaaaaaattaaacagcagtaacggtcaagctttccaacaataaaatacattttggtaaggttttcattttacaaaaactcaaaatagctttatgagttcacaaaataatatgatatttttcaagatattaacatattcttataccggaagagcatagaataaaatttacttggagattgagcatttgcttctttaagaaatacttcttttagtatttttactttaatattatgaaagctacataattacattcagattcattaactactccagtagttaatttttaaaacttatgatgaatagttttgtttaaaatatataacattggtaatatgcaaatctgaatctgtaataaagaaggatttgcattcctgatttttttttctgatacaaccaatgacaaaataactaatggttccacagaggataaaatgtctcaaatctgttggttctgaaggtgaagcgagatttttgtactgataccgtgtatcactgagataccaggaggaaatggaattaaactcagatagttcaaatggagagattttaatgaagggacgacctacagaggtgtcggcagggttggggggaatcagcgagatatgcttagaacccaccgactggcaaacctccccctgaagatggagaaggaggaaggagtgttactggaatgagagcttgagtccaggggaggaggatgggctgctgaggaggcgacaccatcctgaaagaagaatcctctgccagaggcttttcagggtcatttcttcacactctctgcagggaagcacggagacagcaggaagaaatatcctaacctcactctcttccctctacaggtgcttccattggccaaatccacccagaggccagttggtggcgatcagctctcttcaagtggtatttaaatttcttctttcattttccttctggtaacaaagaagtctgtggctcaaaagatgtttctctaagaccccatcctattaggtctctgagattttagaaatgacccaacttgatccttttattcttcagaatatctctctcaaattttcatttgtttttcattaattgatgaataatgagacattttaggtacctgtccacaaagaaatgaaattttcactttccaggaacctaacaaatgaaaagatagaaatcaattccaacagaatattaccaaagaaatcttttagaatggactgttaaaattatttatttgtatttatctggctctactatttgtggtacatttccacttcaaagctaaacctcaaataacatcatagtgagtggttgacttcatgtttaactgagatcttgaagactgaaaaagaccacgacaaacacacatctattttcttggctactgcatccgtgttcatcaccattctgatagtctgcaatgtattgcagctcaccctttgggaaggactaaagtagacatctgtttgttctgcttactcagcattcctaccctaattttcctttggagaacccctttattctagaccacgtgaagctaatgccaaaccccattccaggggatgcacctgaatccaacctccatcatctaaacagtgccttctccacgttcagagaagagcaagtgactcaaactgccctcataagaacagacctgggacttctgctgcaaatattgaagagtaagtactcttttttcttgctaggactaagctggtagtaccttctatgaggctatcatatggaaacaacttgtctgaaaatgaagccacaactagaaaacagatcctggtaacccggattgatggatccagccctaccttaaatggcaagacctaacccgaggctttttgcatcaaccaataaagtccttaagccagtttgagttggttttgtcacttgcagctaaaagaattctgactctaacaatgtgacaatagcaaaaataaacataactgcttttgaggtttctaatggattttcctccctatatacatgatttcatttaatcctcacaattcaggaaagcacatatctattaacattaaattaatattcattattttgaacacatgctatgtggataagggatgaggaaagccaaggaagtaatcaacgtgaaatctcacttatatgggagggaagtggaggttacatatctcagggcacttaacagatatcatcaaatgaaagaataaacagtgtgtgggagaggcagtaggtgattcttcatcaattcctggatgaaaaattaggagataatgaactccgaacaggcagcctaatgagaatggctcaagcaacaggacatagagagggagttaggttagacatggggttcttgggaattttcacctcgtgggggggcgggggggtcgtgcagctgttgtcagtgggaaagggaaaaaggaaaaggctgagtttggaaggcagggagggaggagacaatgtgagtcagtgaaaaagggcccttagaatgacaagtctggaccagagagaggctaagactgaaaatacaagttgggtaaccactggcatacagatggcagttcaggcttgggcactgcccaccagagcctcagcatgaagagaagagggggaggctggccaccacctccctctaggtaatcgtcatcctgatgctgagctcctgaaaacaggctctttcactcgccccatctcttgctcttgattgcaacccggcattcaggaggcaccctgtaatatctgtggagtgaccgacaacacagcgccagggcactgagaagatcccagggcgccagggactggttctacaagggtgcccctcccggtcccctccagcgcgccgccagagctgccagtcttggctgctacacgggaggcagcctcattatgcagctctcacctcttaaattagttcatgctctcacattaggtgtaatcacagcttgcaacgctttctggggatgtctcagaaagatctgagttgaaaaaatatttttgtgtcattttaatttaaagtaaaattgctgcttcttccccgcccctttctttcctcctggcccacccagcgaccctggccggccgtgctcaacgggggcgggggtcggaggtgagatttcctccacataattccttaaacagctatcaactaagtctcaaagaaaaaaaaaagagatctagaagcagagacgtggctgctggcgatcccaaagctggtgttcgctcttgggggagagcgtaccctgggggaggccgggaggccgggccagaggctagcccagaggcagagggcaggagcgctcagccggcgccccgcgtctctccagctcccgacgctgcgctggctccgctgagcacgccaggatcaaggtcgcctggtggggaccggagcgccaggagcctgtgggaagcgttccagccggcctctgactgggatccggcgccgcgtttctgctttggacttgactgacaggtccccccgccctcccgccgccctactaccagcctgggttcatccttcagggctacgtctaccgcacccgggctggaaagcctggagcgcgcccttcctctcctcatcttctcagctctcctttctccctgccacttggcaaagctgcattttgactttcacgttttggactacgtgtgtgtagttccaagtccatgcgtggcacgaaaatccacttagggtaaaaattattctcgaaaaatcgcccatctcaggatctggtgtctacactcaaggctaggaggtgcaggtacgggtgcgtaaagcatgccgtaagggtgcacagtaaataaaaagtacggatgcaaaatgtaaattttaagtgcaaaacagaaaagcagtactcgttgccgccccgcacgctgggttttaaggggcacgaaggtgggcctcggctgcttttgctcagccccgcgtcctcagcgcccggcccagtacccggtactccgtaggggttcaatgatctcccctgaataagtgaacgaattaacaaatgaatgaatgaccgctcgatccgacctccgcggccggcagagcagtcgctggagaggcgggagagagcgagaggccaagctccaccatcgcggccgccggctggggcagagggacacggagacactcggcgccccggctccgcaccgagtccccg

SEQ ID NO: 17597 - RNA, 11301 nt, Homo sapiens
  source 1..11301: mol_type = other RNA
tcaggccaggcacagtggctcatgcctgtagtcccagcactttgggaggccgaggtgggcagatccacgaggtcaggagatcaagaccatcctaacatggtaaaaccccatctctactaacaatacaaaaaattagtcaggtgtggtggcacgtgcctgtagtcccagctactcaggaggctgaggcaggagaatcgcttgaacctgggaggcggaggttgcagtgagccgagattgtgccactgcaccctagcctaggcaacagagcaagactctgtctcaaaaaaaataaaaaaaaaaaaaagagagaaagagagagagagatgaggagttgctgcactgctgggtgtggagagccgaggaggattcaaagatggtcctgaagtcccagctggaagaagtaggcggcagcaatgtttttaatactgtaaattcatcacgtagcacaggtttggggtggagaaagaaaaattgcattggcttcagggcatgcccagatctttcctcatcttaggcgtttgctaatacatgcattttctaagctgatgtcttgcgtttaatcactgctccattcaaaagagagaaggaggttgtttcaaacctagttgatatcatttgacttccatgctattcacagggctattttatttgaaacaggtataccacagccttaaattgcaagttaatccaggatgttcctaggttggcagttaggaacatgtaattctttggaagggctaaaagtcagctctttaaattatctccatatgaaccttctctccaccttagggtggatccacttatttagtccactgccagtaccacactagaacccgggtggtcactggactccagaaacaacagtagccctctctctgttctgtctctttttgactatctctattctgttcctgaccctgatttctcctgccaagctcaattttgacagctgacaacggcaagccatggcttcccaaaacattattttcaggtcaacttataaatttcaagaacacatttggctccgcttcctgtggtactaagcctacttcttgacagcatttgcctttgttgtaaatagcaaagttcttctagttggatttttgctaagaagtgtgtggatgtggcatgtgacgacatctttagcttggattctagaaaggcactaccattgtgcatttggctaaaggaaacacattttacccgtgaatgccttctatttacaaatgctcagctagcacacaaagctaagtacaagcaataagtactatcctacaatgttactcatttctgaaagcacaaaatgatgactggtatagctttggagatgttttctggaaacccaataaaggaacagatctttgttattccacacctacaaagtcagaagatgcacagtcttttattcatgtttgaacaagcttccttcttgaacaatcaactataaagtgatgtgattctctactagaccaggaactccttgaggacagaatgagggtctaatccatattctaaatccacaccacctggcacaatacatgttgcatggttagggtcaactaagagttggttgaattaatcaataacacacagcaagagaattcacaaagagaggggagtaatcccccagcctcaatcactcggcaagtggaatcgctgggcactgattccagctctgtctcagtgcttgagacagagctgaatgtaatgtgaacatttcaaatgaacaggaaaactagactcacggataagcagtgtagtcatcaagacaacactgtcttggaggtttttctgaagttaaaaccatgctacataagcaataaattatgaaggctgagcatgtgaataaaatttaatgttgtcataaattttataacaaagttaatctgacacatttaatgacatgcataatcattagtatgcagcactgtaatcagacattgataataagcagttcacaccagtgactgtaagagtctttacttgtgttcagccaagccaactgcttggtatatttttctcccttcttagtcgttagttttccatacctacaataactatcagtggtgatgggcttctctgaccatgtgaataatttaatcctcaatgcacagatacagaaacccttgctgaagacagtgtggagcagagaaggctgtctccactccttccacctgaaacacctctgcagatggatatgggagctctgcctacagcccttggacctaaccacttcagtgtgttccagtgagtgtctggacctcggcctgaaagatttttccgaaactaaagaaaatttctctgacctaaagaccttaacctccaccccagaagctctcaccaaggactacagggaactggtggggaaaatccttatcccttactcctcaaggcacagggcagtaatgctgaggcttgtgcgccacacttgctcccagaggtccccagcgggctacctgcggtggtgaatgacctcctaacacgccccttgacggccttcctttccttgcctcacttctccactctcctaccagcattgcagggttcacatcccaaatataccactggcacttgaatcctggtctccaggtctgtttctggaaaaacccaagtaagacattgccccagtaatggggctagatgtctgaggcttcctcaagtatctacctcgaaagctcttactgctgtacacacatgcacatacacacacgtgcgtacaaccagtcacatctaagcaccccgaataccagcctgttgaaggtagcagagagctgcactataagccaaggctgctcccaagagccgctccatcactgaattggcgccccagcaagatgaaggaatgtaatcattggaaggatggagaatgttctctgaatcactgacaaattggaaggggtggagggcaagagtccacctggtggagagatggaaagagcgagagagcctggaatgataatgccattgcttagaaaaggctgctccagatgccatatctacagaaattgtacagcccaaacatctctgagcaataggtctctggtagtcttgatgtctagaccaacaattcccagttcattcttctcagggaaggagccaggatagtccagagactctcattctgctgttagattgaaagggttaggcacaacagccttggcaaagtcacaagggcaaattcacactaaagtgtaaatgacccacaactcctcttctatttttaggttggggaggtgctttagaacataaggaggaactaaagaatattcctgttacatacaaggcagagaaaagggaaactagtggtgacaagacaaatcatccctttgacatttggctggctctacctattacagctctgggggtgaggtgggaacaaaaagatgctgtgtaaagaagtatcttatgccatccctactgtagtgaggtgcagtttagaggggacactgatcaagcagagacccagagtgtttcgttccaagccagaaacagaaatgtataaaacacagcctttccagcatcagaaatgagtagtggtagtggagaactacccaaaacaggaaagaggaccacgtgaggtagagtgtcaaggccctacattccagtgcctctgctcatgactgtaattttgggtaggtcacttaaagtctctggacctcagttttgccatctgtgaaatagggataatactatccagcataaaattggttatgaggctcatgtagggcctgcctgggatgatgtgttgctaatggttaagaacacaacttctggggtctgactggacaggctgaaatccctgcttaacacgttccagcagagccctgggcgatctatttaacttttgttttctcacctgtaagctgagacgaaagtacccactttataagattattccaataattagttgaaataatgcatgcagagaattaagcatggtacttgttatttgttaaactagctattaaaatgtgtaaaatataaagtattgtatggattttaggacaatgcaaagactctttgcttgctgcaatagttcggggccctttcagatggctaaaggcagaatttgtatgtgtaaatatggtgtgcttgtctctgctctggatactgagggcttaccctgttattaaacttatttagtaaatattgaactgtcatgaggcctaacatttagttccagttattagataaaacatttgctttgaatggtatttgaattgccaggttctagattattctggttgacaaactcttcgtattttataaagaggctaaaattggtaagctatcacagaacagatgtgccattttcaaggtatattaaaccatgattcactgtaacattgttcctactggcaacaaattcagagcaggctggactttatttggtgaagaaacattgagtggaagagaaatgacattattttatgtatttacattttcaaattactgtggcttaaacctgttcagccaacattacccaccttcagtctgctaaataaatgattcagtacatttctaatttacagaattttttaacaaaagaaaatgtaatttgatagccaaatcaacgttaaacattatacatttaaaaaaccacaggcaaagacacaaacatgatgacactaacttttgttaaagtatgcttacctatggtttcctctgaggcacgttctttcatgctaagcttccaacataatatgaaaatgaaggagatgcattttgcaaagcaaaacagaccttaagcaaaatattatacttctcaaattaacactgttacaaagttttagaatttaataagttcattaatttaaaagtttggatgtctgagtccttctatcccaaaacaagatcttggagggtcttccacagccatgtaataccatggtcacatgaccctttccaaaattattaatctgaatttactatatgaggataaatctatctttttgaaaatatttaggaaaatgagcttggtatttataaaatgaagctctctttgggtggtatcctaagacacgtcaagccaatcagcctgtaactgtgaaaaaaacattggtaggtacaaaagtggggtgggagaggagtgacttaactttgttaagtgatgggaaagaaacactaatagcattatctcaataaaatgtgatttaaaaaaatttaaaatactaaatcattgaactgacaaagaaatataaatcattcagaaataaactcattaggtcatcaaatcctgttaaatctgcaattaggaagagcaaggtgtacaatccatacatttaaactcacaggctcactttgcacaacgtcaatttactccttaatatgttattaatacgcattttccaaaaggatgtattagtaaatggtacacatctacttcttggcaacatcatataacctggtacaacataagcattcttcttatagttaagaaatgtggatggtatcaaaattagaaaaataaatgccctattatgttgtggtcaggtttaaggcatgtgaattttatcttcatacaaaagattaaaatctagatattaaaaagtagtgcagtatcagtgatgctgcctcagttcccaaaatgtcacatcacaaaaatatcccataattgcctgtagtttattccttggctttcctcttttctctctgcatctttgtaacaattttttaaaagtggaaatataattgttggcaatgctaacagctgtagaaatgattacaagatgtggaaaagcataacaggaatgtcaagaatctgtttctggcagtaatatatatggaacattgttcaggacaaaagaggagaaggaagaaaaaaaggagaggggtttatcatctctaagaattttcaaactaaacctcattgcttaataggaaaaaaagattccatatttaaagttaagtcacctctaactactagctaaagcatgacatcaccagcactggagtcagcggaagtgtgtttttgaaggacagtgttgcaggagaatctggacaggttttagagccaggagagagaaaataattctacctctgacagttgaaggaccttaggcaaatcagtttacctctgctagactacactccaaaatttggacattcaaaaatttgatattaataaccacatgaaagtctcgtgttgaggtgaatatgtatttgttggtgaaagatatgttggtttttaaacagacagcactctgcaattgtaggctattgttttgttttgccagttgtcaaattctatccagctatacacacttgtgtggcctcctaatggtgtttttccagtggctaaaggtttatgaataagacacttttcctaatggaattaacccgatgcttttcttaaacatgtaaccttgagttcaccgcaaaaaacaatgcttcgattagagcaatgcatataataaaggttaccctcgtttcttagacactagacatcattcacaaaaagagaactgcttttgaaagggatgtatttgcactggaaagaatagttttctacttctaattataaatgatttattggtgaaagcaaaacaacagcctgtctgagaggcacttctatgagcatcctcacgtgtgatttgcaaggttgaagaagagggaaaaatgcctcaattgtaccaatggtgagaaaacacccaaagtacaaagcaggtttcaaaaaaaccatactcataaccaaggacaataataaagcaatgtgttgacatatactctataagtcttcctccataaatagtttatagaaattttgtaatttctgtaaatgcatcctataataattttgcatcttgctttttttttacatttaatatcaagtagatttctaaagggcaattatttgaaaattatcccaaatacatggggaaatatacatcaagtgaaaaaatgcagtgggtgatagagatatcaggaagcgcctcaaatatttctcatctcgttggagaaaaacaaacatgttctcatttagaatgagtgggagttacctaattgatttaggcctctatatttaacttctagtcaaaaaaggtagttctatctagcaacaatattatggggaacaaaagaaaaaattaactctctaaatttgcagtagggtcttttcttcagaagtaccaaatcccatctattaccagctccatgcttcaggcctaaaatggatctccctgaagcaatgacagaatttttgccaagtgactaggatataaacaccactttggttgcacagtgagacatatgctccaaagaaaactggttcaaaaacaggcaagtgggtttctacagaataaatgagagccctgtcaatggcttcatcttcagggctttgtgtctgtgcttgcgtggtggctcttgtttcatctatggataatggtggcacacagttttcataattccttacattaatgaactgctataaatttgtttttggtattctagagagtcctaacttcagcttctgggcaatgctgaggaggcaccctatattctagacttaccttttgcaaggtgtactctcagcattgtgggcgatttccatgggagaatattctatttaaagaactactgtcccagcataaaacaaaaaatcatttatgaagatgcaggagactcggaaagctctcaattattgtttgcacaagcacaatgtcacagcctcctttccccattccacaagggggtcaggaagagagtactcagctgtgagaaaagacatacagaagaattcatgtggtcatgagagcgaggacatggccgatcccccaaggaggatgtgtcatacacttcatgagcccaagagtgtgctgtagggtctgaagggcaagatgctggttcactgatgtaaaggagagggaaaaaagcttcaaccaactagaaaaacagtctctatgcatgctatttttgattttaaacacaggtatcaattccttctctcagagagtccattttaaaataggatacatttttaaaggaatatttaaaggacacattcattaaaatttattttaaaaacttttcaaaagaaacaaaaggtatgaattttatttaatccttgaggaaatggttcttttctcacacacataaatcactcattttgtttttctttatctcctttattaatctacattagaaaaataaacttttcatacactaagaacaaggaaaccactctcaattgacaaaatgttccaatccaacacaatgattactttcacctttaatttacaggcagccagattcaaaatccttaaagttgcttaaacttaaaaatgacaatgacaacctaaaaggtataatgttgattggaacagacatttaattggaaaattgatgattttccatttccaattaaatctctagatagaaatgaaaaaaattaaaaatcgtatttaagaaaagccaaatcttgggttgtgaggtatctttttaaggatgtttcagcagaaaaaaacaaaggctctcacaattgtgtagctgcctagattaagtgggtatcctgatcaaggagatgggggatgatttggctttagtattccaatgataaagtttataatgagaataacatgttgctacaaaatccagtctcttcctcagatgccttccacagagggcaggaagctttgtcagttttgtttgctgatgatgcctggttccgtcaacaaataacacctgtcacacggtgggtagtcaatatacatttgttgaataaatatgaaaaaaagaaatgtacaatatgtttgtgaagccaactgtgtgtgcattgctattgaggtacacaaaaagtctttgttttaaatttgagaatgaggactttcaatggaatatatctataaaaatgaaaaaaagacattactgtctggacttttgtacagcaagagaagaaaaaccactagccaagagccaactcacctgataggcctggatcaagcatgcagctgtggagaacacccctgggactctaactctggcactctgcaagctgggtacttgggcaggacagcagcagcactcatgaactgggcagcacctgttggtgagggctgatcacatggattctctcatcccagccttacaatcagtccttcaggtacatactttttctgactttgctgatgaggaaactatgcacagaggttacacagcttaacaaagggttctcacctaatgaacaatgaaatgggattttagcctttctttgcatctggtcttagagccaatacccaagaagcactgtactgtatgcattgtctcagagaaacttactcttcctgggcctcagtctttaaaaggtgggcagttgacttaataagaattaaagatcaatgattaaggttcaaggcactccaaaattctggtctttattgaaaaggctacagaagtctcaccttaataataccctatagacttgatattcttggttaattaaatattggaaaccaatttcatagtaattgaggtcagaaaaaagtactcatgacattttagaatatgatgacaaagccatagataaatttcaatgcacctgtaattacttaaaactgttatagcatgcaatgtgttaccacaacagccagagaaatactaatttactcagcctattcttctagaccagtaaacactaggattaaatagatattttcattgaatttgttctacccttcattgccatttatagatagcttacttgtcatagattactttctaattgttttatgtttcctaactagcctgcaatactttggcaaggacctcaaacaatagtagacagtaggtgtaaaatagatggctacattgaacagatgactaaaaggatgcctcctaagtacctatatcttgaaatatatattattgtgccttgctttcaatttgtgattttaaaatctagaaatcacctgttttatgtaataacaataaaatccttctttgttgaaaacatgcacaaataaagtttacaagctcaaaaaattaaacagcagtaacggtcaagctttccaacaataaaatacattttggtaaggttttcattttacaaaaactcaaaatagctttatgagttcacaaaataatatgatatttttcaagatattaacatattcttataccggaagagcatagaataaaatttacttggagattgagcatttgcttctttaagaaatacttcttttagtatttttactttaatattatgaaagctacataattacattcagattcattaactactccagtagttaatttttaaaacttatgatgaatagttttgtttaaaatatataacattggtaatatgcaaatctgaatctgtaataaagaaggatttgcattcctgatttttttttctgatacaaccaatgacaaaataactaatggttccacagaggataaaatgtctcaaatctgttggttctgaaggtgaagcgagatttttgtactgataccgtgtatcactgagataccaggaggaaatggaattaaactcagatagttcaaatggagagattttaatgaagggacgacctacagaggtgtcggcagggttggggggaatcagcgagatatgcttagaacccaccgactggcaaacctccccctgaagatggagaaggaggaaggagtgttactggaatgagagcttgagtccaggggaggaggatgggctgctgaggaggcgacaccatcctgaaagaagaatcctctgccagaggcttttcagggtcatttcttcacactctctgcagggaagcacggagacagcaggaagaaatatcctaacctcactctcttccctctacaggtgcttccattggccaaatccacccagaggccagttggtggcgatcagctctcttcaagtggtatttaaatttcttctttcattttccttctggtaacaaagaagtctgtggctcaaaagatgtttctctaagaccccatcctattaggtctctgagattttagaaatgacccaacttgatccttttattcttcagaatatctctctcaaattttcatttgtttttcattaattgatgaataatgagacattttaggtacctgtccacaaagaaatgaaattttcactttccaggaacctgagggccgacgagtgggggcgggcaggagggccgagggaggcggaacaggatcgaggcgcgaggcgggagtcgagaaagcgagcggccgaggcgactctcagtgcgcggacgcgggcgcgcgcccgcgctcccttcgtcgactcacggcgagagcccaaccctgctgccgcgcgccacccgcctcgccgcgcct

SEQ ID NO: 17598 - RNA, 11160 nt, Homo sapiens
  source 1..11160: mol_type = other RNA
tcaggccaggcacagtggctcatgcctgtagtcccagcactttgggaggccgaggtgggcagatccacgaggtcaggagatcaagaccatcctaacatggtaaaaccccatctctactaacaatacaaaaaattagtcaggtgtggtggcacgtgcctgtagtcccagctactcaggaggctgaggcaggagaatcgcttgaacctgggaggcggaggttgcagtgagccgagattgtgccactgcaccctagcctaggcaacagagcaagactctgtctcaaaaaaaataaaaaaaaaaaaaagagagaaagagagagagagatgaggagttgctgcactgctgggtgtggagagccgaggaggattcaaagatggtcctgaagtcccagctggaagaagtaggcggcagcaatgtttttaatactgtaaattcatcacgtagcacaggtttggggtggagaaagaaaaattgcattggcttcagggcatgcccagatctttcctcatcttaggcgtttgctaatacatgcattttctaagctgatgtcttgcgtttaatcactgctccattcaaaagagagaaggaggttgtttcaaacctagttgatatcatttgacttccatgctattcacagggctattttatttgaaacaggtataccacagccttaaattgcaagttaatccaggatgttcctaggttggcagttaggaacatgtaattctttggaagggctaaaagtcagctctttaaattatctccatatgaaccttctctccaccttagggtggatccacttatttagtccactgccagtaccacactagaacccgggtggtcactggactccagaaacaacagtagccctctctctgttctgtctctttttgactatctctattctgttcctgaccctgatttctcctgccaagctcaattttgacagctgacaacggcaagccatggcttcccaaaacattattttcaggtcaacttataaatttcaagaacacatttggctccgcttcctgtggtactaagcctacttcttgacagcatttgcctttgttgtaaatagcaaagttcttctagttggatttttgctaagaagtgtgtggatgtggcatgtgacgacatctttagcttggattctagaaaggcactaccattgtgcatttggctaaaggaaacacattttacccgtgaatgccttctatttacaaatgctcagctagcacacaaagctaagtacaagcaataagtactatcctacaatgttactcatttctgaaagcacaaaatgatgactggtatagctttggagatgttttctggaaacccaataaaggaacagatctttgttattccacacctacaaagtcagaagatgcacagtcttttattcatgtttgaacaagcttccttcttgaacaatcaactataaagtgatgtgattctctactagaccaggaactccttgaggacagaatgagggtctaatccatattctaaatccacaccacctggcacaatacatgttgcatggttagggtcaactaagagttggttgaattaatcaataacacacagcaagagaattcacaaagagaggggagtaatcccccagcctcaatcactcggcaagtggaatcgctgggcactgattccagctctgtctcagtgcttgagacagagctgaatgtaatgtgaacatttcaaatgaacaggaaaactagactcacggataagcagtgtagtcatcaagacaacactgtcttggaggtttttctgaagttaaaaccatgctacataagcaataaattatgaaggctgagcatgtgaataaaatttaatgttgtcataaattttataacaaagttaatctgacacatttaatgacatgcataatcattagtatgcagcactgtaatcagacattgataataagcagttcacaccagtgactgtaagagtctttacttgtgttcagccaagccaactgcttggtatatttttctcccttcttagtcgttagttttccatacctacaataactatcagtggtgatgggcttctctgaccatgtgaataatttaatcctcaatgcacagatacagaaacccttgctgaagacagtgtggagcagagaaggctgtctccactccttccacctgaaacacctctgcagatggatatgggagctctgcctacagcccttggacctaaccacttcagtgtgttccagtgagtgtctggacctcggcctgaaagatttttccgaaactaaagaaaatttctctgacctaaagaccttaacctccaccccagaagctctcaccaaggactacagggaactggtggggaaaatccttatcccttactcctcaaggcacagggcagtaatgctgaggcttgtgcgccacacttgctcccagaggtccccagcgggctacctgcggtggtgaatgacctcctaacacgccccttgacggccttcctttccttgcctcacttctccactctcctaccagcattgcagggttcacatcccaaatataccactggcacttgaatcctggtctccaggtctgtttctggaaaaacccaagtaagacattgccccagtaatggggctagatgtctgaggcttcctcaagtatctacctcgaaagctcttactgctgtacacacatgcacatacacacacgtgcgtacaaccagtcacatctaagcaccccgaataccagcctgttgaaggtagcagagagctgcactataagccaaggctgctcccaagagccgctccatcactgaattggcgccccagcaagatgaaggaatgtaatcattggaaggatggagaatgttctctgaatcactgacaaattggaaggggtggagggcaagagtccacctggtggagagatggaaagagcgagagagcctggaatgataatgccattgcttagaaaaggctgctccagatgccatatctacagaaattgtacagcccaaacatctctgagcaataggtctctggtagtcttgatgtctagaccaacaattcccagttcattcttctcagggaaggagccaggatagtccagagactctcattctgctgttagattgaaagggttaggcacaacagccttggcaaagtcacaagggcaaattcacactaaagtgtaaatgacccacaactcctcttctatttttaggttggggaggtgctttagaacataaggaggaactaaagaatattcctgttacatacaaggcagagaaaagggaaactagtggtgacaagacaaatcatccctttgacatttggctggctctacctattacagctctgggggtgaggtgggaacaaaaagatgctgtgtaaagaagtatcttatgccatccctactgtagtgaggtgcagtttagaggggacactgatcaagcagagacccagagtgtttcgttccaagccagaaacagaaatgtataaaacacagcctttccagcatcagaaatgagtagtggtagtggagaactacccaaaacaggaaagaggaccacgtgaggtagagtgtcaaggccctacattccagtgcctctgctcatgactgtaattttgggtaggtcacttaaagtctctggacctcagttttgccatctgtgaaatagggataatactatccagcataaaattggttatgaggctcatgtagggcctgcctgggatgatgtgttgctaatggttaagaacacaacttctggggtctgactggacaggctgaaatccctgcttaacacgttccagcagagccctgggcgatctatttaacttttgttttctcacctgtaagctgagacgaaagtacccactttataagattattccaataattagttgaaataatgcatgcagagaattaagcatggtacttgttatttgttaaactagctattaaaatgtgtaaaatataaagtattgtatggattttaggacaatgcaaagactctttgcttgctgcaatagttcggggccctttcagatggctaaaggcagaatttgtatgtgtaaatatggtgtgcttgtctctgctctggatactgagggcttaccctgttattaaacttatttagtaaatattgaactgtcatgaggcctaacatttagttccagttattagataaaacatttgctttgaatggtatttgaattgccaggttctagattattctggttgacaaactcttcgtattttataaagaggctaaaattggtaagctatcacagaacagatgtgccattttcaaggtatattaaaccatgattcactgtaacattgttcctactggcaacaaattcagagcaggctggactttatttggtgaagaaacattgagtggaagagaaatgacattattttatgtatttacattttcaaattactgtggcttaaacctgttcagccaacattacccaccttcagtctgctaaataaatgattcagtacatttctaatttacagaattttttaacaaaagaaaatgtaatttgatagccaaatcaacgttaaacattatacatttaaaaaaccacaggcaaagacacaaacatgatgacactaacttttgttaaagtatgcttacctatggtttcctctgaggcacgttctttcatgctaagcttccaacataatatgaaaatgaaggagatgcattttgcaaagcaaaacagaccttaagcaaaatattatacttctcaaattaacactgttacaaagttttagaatttaataagttcattaatttaaaagtttggatgtctgagtccttctatcccaaaacaagatcttggagggtcttccacagccatgtaataccatggtcacatgaccctttccaaaattattaatctgaatttactatatgaggataaatctatctttttgaaaatatttaggaaaatgagcttggtatttataaaatgaagctctctttgggtggtatcctaagacacgtcaagccaatcagcctgtaactgtgaaaaaaacattggtaggtacaaaagtggggtgggagaggagtgacttaactttgttaagtgatgggaaagaaacactaatagcattatctcaataaaatgtgatttaaaaaaatttaaaatactaaatcattgaactgacaaagaaatataaatcattcagaaataaactcattaggtcatcaaatcctgttaaatctgcaattaggaagagcaaggtgtacaatccatacatttaaactcacaggctcactttgcacaacgtcaatttactccttaatatgttattaatacgcattttccaaaaggatgtattagtaaatggtacacatctacttcttggcaacatcatataacctggtacaacataagcattcttcttatagttaagaaatgtggatggtatcaaaattagaaaaataaatgccctattatgttgtggtcaggtttaaggcatgtgaattttatcttcatacaaaagattaaaatctagatattaaaaagtagtgcagtatcagtgatgctgcctcagttcccaaaatgtcacatcacaaaaatatcccataattgcctgtagtttattccttggctttcctcttttctctctgcatctttgtaacaattttttaaaagtggaaatataattgttggcaatgctaacagctgtagaaatgattacaagatgtggaaaagcataacaggaatgtcaagaatctgtttctggcagtaatatatatggaacattgttcaggacaaaagaggagaaggaagaaaaaaaggagaggggtttatcatctctaagaattttcaaactaaacctcattgcttaataggaaaaaaagattccatatttaaagttaagtcacctctaactactagctaaagcatgacatcaccagcactggagtcagcggaagtgtgtttttgaaggacagtgttgcaggagaatctggacaggttttagagccaggagagagaaaataattctacctctgacagttgaaggaccttaggcaaatcagtttacctctgctagactacactccaaaatttggacattcaaaaatttgatattaataaccacatgaaagtctcgtgttgaggtgaatatgtatttgttggtgaaagatatgttggtttttaaacagacagcactctgcaattgtaggctattgttttgttttgccagttgtcaaattctatccagctatacacacttgtgtggcctcctaatggtgtttttccagtggctaaaggtttatgaataagacacttttcctaatggaattaacccgatgcttttcttaaacatgtaaccttgagttcaccgcaaaaaacaatgcttcgattagagcaatgcatataataaaggttaccctcgtttcttagacactagacatcattcacaaaaagagaactgcttttgaaagggatgtatttgcactggaaagaatagttttctacttctaattataaatgatttattggtgaaagcaaaacaacagcctgtctgagaggcacttctatgagcatcctcacgtgtgatttgcaaggttgaagaagagggaaaaatgcctcaattgtaccaatggtgagaaaacacccaaagtacaaagcaggtttcaaaaaaaccatactcataaccaaggacaataataaagcaatgtgttgacatatactctataagtcttcctccataaatagtttatagaaattttgtaatttctgtaaatgcatcctataataattttgcatcttgctttttttttacatttaatatcaagtagatttctaaagggcaattatttgaaaattatcccaaatacatggggaaatatacatcaagtgaaaaaatgcagtgggtgatagagatatcaggaagcgcctcaaatatttctcatctcgttggagaaaaacaaacatgttctcatttagaatgagtgggagttacctaattgatttaggcctctatatttaacttctagtcaaaaaaggtagttctatctagcaacaatattatggggaacaaaagaaaaaattaactctctaaatttgcagtagggtcttttcttcagaagtaccaaatcccatctattaccagctccatgcttcaggcctaaaatggatctccctgaagcaatgacagaatttttgccaagtgactaggatataaacaccactttggttgcacagtgagacatatgctccaaagaaaactggttcaaaaacaggcaagtgggtttctacagaataaatgagagccctgtcaatggcttcatcttcagggctttgtgtctgtgcttgcgtggtggctcttgtttcatctatggataatggtggcacacagttttcataattccttacattaatgaactgctataaatttgtttttggtattctagagagtcctaacttcagcttctgggcaatgctgaggaggcaccctatattctagacttaccttttgcaaggtgtactctcagcattgtgggcgatttccatgggagaatattctatttaaagaactactgtcccagcataaaacaaaaaatcatttatgaagatgcaggagactcggaaagctctcaattattgtttgcacaagcacaatgtcacagcctcctttccccattccacaagggggtcaggaagagagtactcagctgtgagaaaagacatacagaagaattcatgtggtcatgagagcgaggacatggccgatcccccaaggaggatgtgtcatacacttcatgagcccaagagtgtgctgtagggtctgaagggcaagatgctggttcactgatgtaaaggagagggaaaaaagcttcaaccaactagaaaaacagtctctatgcatgctatttttgattttaaacacaggtatcaattccttctctcagagagtccattttaaaataggatacatttttaaaggaatatttaaaggacacattcattaaaatttattttaaaaacttttcaaaagaaacaaaaggtatgaattttatttaatccttgaggaaatggttcttttctcacacacataaatcactcattttgtttttctttatctcctttattaatctacattagaaaaataaacttttcatacactaagaacaaggaaaccactctcaattgacaaaatgttccaatccaacacaatgattactttcacctttaatttacaggcagccagattcaaaatccttaaagttgcttaaacttaaaaatgacaatgacaacctaaaaggtataatgttgattggaacagacatttaattggaaaattgatgattttccatttccaattaaatctctagatagaaatgaaaaaaattaaaaatcgtatttaagaaaagccaaatcttgggttgtgaggtatctttttaaggatgtttcagcagaaaaaaacaaaggctctcacaattgtgtagctgcctagattaagtgggtatcctgatcaaggagatgggggatgatttggctttagtattccaatgataaagtttataatgagaataacatgttgctacaaaatccagtctcttcctcagatgccttccacagagggcaggaagctttgtcagttttgtttgctgatgatgcctggttccgtcaacaaataacacctgtcacacggtgggtagtcaatatacatttgttgaataaatatgaaaaaaagaaatgtacaatatgtttgtgaagccaactgtgtgtgcattgctattgaggtacacaaaaagtctttgttttaaatttgagaatgaggactttcaatggaatatatctataaaaatgaaaaaaagacattactgtctggacttttgtacagcaagagaagaaaaaccactagccaagagccaactcacctgataggcctggatcaagcatgcagctgtggagaacacccctgggactctaactctggcactctgcaagctgggtacttgggcaggacagcagcagcactcatgaactgggcagcacctgttggtgagggctgatcacatggattctctcatcccagccttacaatcagtccttcaggtacatactttttctgactttgctgatgaggaaactatgcacagaggttacacagcttaacaaagggttctcacctaatgaacaatgaaatgggattttagcctttctttgcatctggtcttagagccaatacccaagaagcactgtactgtatgcattgtctcagagaaacttactcttcctgggcctcagtctttaaaaggtgggcagttgacttaataagaattaaagatcaatgattaaggttcaaggcactccaaaattctggtctttattgaaaaggctacagaagtctcaccttaataataccctatagacttgatattcttggttaattaaatattggaaaccaatttcatagtaattgaggtcagaaaaaagtactcatgacattttagaatatgatgacaaagccatagataaatttcaatgcacctgtaattacttaaaactgttatagcatgcaatgtgttaccacaacagccagagaaatactaatttactcagcctattcttctagaccagtaaacactaggattaaatagatattttcattgaatttgttctacccttcattgccatttatagatagcttacttgtcatagattactttctaattgttttatgtttcctaactagcctgcaatactttggcaaggacctcaaacaatagtagacagtaggtgtaaaatagatggctacattgaacagatgactaaaaggatgcctcctaagtacctatatcttgaaatatatattattgtgccttgctttcaatttgtgattttaaaatctagaaatcacctgttttatgtaataacaataaaatccttctttgttgaaaacatgcacaaataaagtttacaagctcaaaaaattaaacagcagtaacggtcaagctttccaacaataaaatacattttggtaaggttttcattttacaaaaactcaaaatagctttatgagttcacaaaataatatgatatttttcaagatattaacatattcttataccggaagagcatagaataaaatttacttggagattgagcatttgcttctttaagaaatacttcttttagtatttttactttaatattatgaaagctacataattacattcagattcattaactactccagtagttaatttttaaaacttatgatgaatagttttgtttaaaatatataacattggtaatatgcaaatctgaatctgtaataaagaaggatttgcattcctgatttttttttctgatacaaccaatgacaaaataactaatggttccacagaggataaaatgtctcaaatctgttggttctgaaggtgaagcgagatttttgtactgataccgtgtatcactgagataccaggaggaaatggaattaaactcagatagttcaaatggagagattttaatgaagggacgacctacagaggtgtcggcagggttggggggaatcagcgagatatgcttagaacccaccgactggcaaacctccccctgaagatggagaaggaggaaggagtgttactggaatgagagcttgagtccaggggaggaggatgggctgctgaggaggcgacaccatcctgaaagaagaatcctctgccagaggcttttcagggtcatttcttcacactctctgcagggaagcacggagacagcaggaagaaatatcctaacctcactctcttccctctacaggtgcttccattggccaaatccacccagaggccagttggtggcgatcagctctcttcaagtggtatttaaatttcttctttcattttccttctggtaacaaagaagtctgtggctcaaaagatgtttctctaagaccccatcctattaggtctctgagctgagggccgacgagtgggggcgggcaggagggccgagggaggcggaacaggatcgaggcgcgaggcgggagtcgagaaagcgagcggccgaggcgactctcagtgcgcggacgcgggcgcgcgcccgcgctcccttcgtcgactcacggcgagagcccaaccctgctgccgcgcgccacccgcctcgccgcgcct

SEQ ID NO: 17599 - RNA, 13995 nt, Homo sapiens
  source 1..13995: mol_type = other RNA
tcaggccaggcacagtggctcatgcctgtagtcccagcactttgggaggccgaggtgggcagatccacgaggtcaggagatcaagaccatcctaacatggtaaaaccccatctctactaacaatacaaaaaattagtcaggtgtggtggcacgtgcctgtagtcccagctactcaggaggctgaggcaggagaatcgcttgaacctgggaggcggaggttgcagtgagccgagattgtgccactgcaccctagcctaggcaacagagcaagactctgtctcaaaaaaaataaaaaaaaaaaaaagagagaaagagagagagagatgaggagttgctgcactgctgggtgtggagagccgaggaggattcaaagatggtcctgaagtcccagctggaagaagtaggcggcagcaatgtttttaatactgtaaattcatcacgtagcacaggtttggggtggagaaagaaaaattgcattggcttcagggcatgcccagatctttcctcatcttaggcgtttgctaatacatgcattttctaagctgatgtcttgcgtttaatcactgctccattcaaaagagagaaggaggttgtttcaaacctagttgatatcatttgacttccatgctattcacagggctattttatttgaaacaggtataccacagccttaaattgcaagttaatccaggatgttcctaggttggcagttaggaacatgtaattctttggaagggctaaaagtcagctctttaaattatctccatatgaaccttctctccaccttagggtggatccacttatttagtccactgccagtaccacactagaacccgggtggtcactggactccagaaacaacagtagccctctctctgttctgtctctttttgactatctctattctgttcctgaccctgatttctcctgccaagctcaattttgacagctgacaacggcaagccatggcttcccaaaacattattttcaggtcaacttataaatttcaagaacacatttggctccgcttcctgtggtactaagcctacttcttgacagcatttgcctttgttgtaaatagcaaagttcttctagttggatttttgctaagaagtgtgtggatgtggcatgtgacgacatctttagcttggattctagaaaggcactaccattgtgcatttggctaaaggaaacacattttacccgtgaatgccttctatttacaaatgctcagctagcacacaaagctaagtacaagcaataagtactatcctacaatgttactcatttctgaaagcacaaaatgatgactggtatagctttggagatgttttctggaaacccaataaaggaacagatctttgttattccacacctacaaagtcagaagatgcacagtcttttattcatgtttgaacaagcttccttcttgaacaatcaactataaagtgatgtgattctctactagaccaggaactccttgaggacagaatgagggtctaatccatattctaaatccacaccacctggcacaatacatgttgcatggttagggtcaactaagagttggttgaattaatcaataacacacagcaagagaattcacaaagagaggggagtaatcccccagcctcaatcactcggcaagtggaatcgctgggcactgattccagctctgtctcagtgcttgagacagagctgaatgtaatgtgaacatttcaaatgaacaggaaaactagactcacggataagcagtgtagtcatcaagacaacactgtcttggaggtttttctgaagttaaaaccatgctacataagcaataaattatgaaggctgagcatgtgaataaaatttaatgttgtcataaattttataacaaagttaatctgacacatttaatgacatgcataatcattagtatgcagcactgtaatcagacattgataataagcagttcacaccagtgactgtaagagtctttacttgtgttcagccaagccaactgcttggtatatttttctcccttcttagtcgttagttttccatacctacaataactatcagtggtgatgggcttctctgaccatgtgaataatttaatcctcaatgcacagatacagaaacccttgctgaagacagtgtggagcagagaaggctgtctccactccttccacctgaaacacctctgcagatggatatgggagctctgcctacagcccttggacctaaccacttcagtgtgttccagtgagtgtctggacctcggcctgaaagatttttccgaaactaaagaaaatttctctgacctaaagaccttaacctccaccccagaagctctcaccaaggactacagggaactggtggggaaaatccttatcccttactcctcaaggcacagggcagtaatgctgaggcttgtgcgccacacttgctcccagaggtccccagcgggctacctgcggtggtgaatgacctcctaacacgccccttgacggccttcctttccttgcctcacttctccactctcctaccagcattgcagggttcacatcccaaatataccactggcacttgaatcctggtctccaggtctgtttctggaaaaacccaagtaagacattgccccagtaatggggctagatgtctgaggcttcctcaagtatctacctcgaaagctcttactgctgtacacacatgcacatacacacacgtgcgtacaaccagtcacatctaagcaccccgaataccagcctgttgaaggtagcagagagctgcactataagccaaggctgctcccaagagccgctccatcactgaattggcgccccagcaagatgaaggaatgtaatcattggaaggatggagaatgttctctgaatcactgacaaattggaaggggtggagggcaagagtccacctggtggagagatggaaagagcgagagagcctggaatgataatgccattgcttagaaaaggctgctccagatgccatatctacagaaattgtacagcccaaacatctctgagcaataggtctctggtagtcttgatgtctagaccaacaattcccagttcattcttctcagggaaggagccaggatagtccagagactctcattctgctgttagattgaaagggttaggcacaacagccttggcaaagtcacaagggcaaattcacactaaagtgtaaatgacccacaactcctcttctatttttaggttggggaggtgctttagaacataaggaggaactaaagaatattcctgttacatacaaggcagagaaaagggaaactagtggtgacaagacaaatcatccctttgacatttggctggctctacctattacagctctgggggtgaggtgggaacaaaaagatgctgtgtaaagaagtatcttatgccatccctactgtagtgaggtgcagtttagaggggacactgatcaagcagagacccagagtgtttcgttccaagccagaaacagaaatgtataaaacacagcctttccagcatcagaaatgagtagtggtagtggagaactacccaaaacaggaaagaggaccacgtgaggtagagtgtcaaggccctacattccagtgcctctgctcatgactgtaattttgggtaggtcacttaaagtctctggacctcagttttgccatctgtgaaatagggataatactatccagcataaaattggttatgaggctcatgtagggcctgcctgggatgatgtgttgctaatggttaagaacacaacttctggggtctgactggacaggctgaaatccctgcttaacacgttccagcagagccctgggcgatctatttaacttttgttttctcacctgtaagctgagacgaaagtacccactttataagattattccaataattagttgaaataatgcatgcagagaattaagcatggtacttgttatttgttaaactagctattaaaatgtgtaaaatataaagtattgtatggattttaggacaatgcaaagactctttgcttgctgcaatagttcggggccctttcagatggctaaaggcagaatttgtatgtgtaaatatggtgtgcttgtctctgctctggatactgagggcttaccctgttattaaacttatttagtaaatattgaactgtcatgaggcctaacatttagttccagttattagataaaacatttgctttgaatggtatttgaattgccaggttctagattattctggttgacaaactcttcgtattttataaagaggctaaaattggtaagctatcacagaacagatgtgccattttcaaggtatattaaaccatgattcactgtaacattgttcctactggcaacaaattcagagcaggctggactttatttggtgaagaaacattgagtggaagagaaatgacattattttatgtatttacattttcaaattactgtggcttaaacctgttcagccaacattacccaccttcagtctgctaaataaatgattcagtacatttctaatttacagaattttttaacaaaagaaaatgtaatttgatagccaaatcaacgttaaacattatacatttaaaaaaccacaggcaaagacacaaacatgatgacactaacttttgttaaagtatgcttacctatggtttcctctgaggcacgttctttcatgctaagcttccaacataatatgaaaatgaaggagatgcattttgcaaagcaaaacagaccttaagcaaaatattatacttctcaaattaacactgttacaaagttttagaatttaataagttcattaatttaaaagtttggatgtctgagtccttctatcccaaaacaagatcttggagggtcttccacagccatgtaataccatggtcacatgaccctttccaaaattattaatctgaatttactatatgaggataaatctatctttttgaaaatatttaggaaaatgagcttggtatttataaaatgaagctctctttgggtggtatcctaagacacgtcaagccaatcagcctgtaactgtgaaaaaaacattggtaggtacaaaagtggggtgggagaggagtgacttaactttgttaagtgatgggaaagaaacactaatagcattatctcaataaaatgtgatttaaaaaaatttaaaatactaaatcattgaactgacaaagaaatataaatcattcagaaataaactcattaggtcatcaaatcctgttaaatctgcaattaggaagagcaaggtgtacaatccatacatttaaactcacaggctcactttgcacaacgtcaatttactccttaatatgttattaatacgcattttccaaaaggatgtattagtaaatggtacacatctacttcttggcaacatcatataacctggtacaacataagcattcttcttatagttaagaaatgtggatggtatcaaaattagaaaaataaatgccctattatgttgtggtcaggtttaaggcatgtgaattttatcttcatacaaaagattaaaatctagatattaaaaagtagtgcagtatcagtgatgctgcctcagttcccaaaatgtcacatcacaaaaatatcccataattgcctgtagtttattccttggctttcctcttttctctctgcatctttgtaacaattttttaaaagtggaaatataattgttggcaatgctaacagctgtagaaatgattacaagatgtggaaaagcataacaggaatgtcaagaatctgtttctggcagtaatatatatggaacattgttcaggacaaaagaggagaaggaagaaaaaaaggagaggggtttatcatctctaagaattttcaaactaaacctcattgcttaataggaaaaaaagattccatatttaaagttaagtcacctctaactactagctaaagcatgacatcaccagcactggagtcagcggaagtgtgtttttgaaggacagtgttgcaggagaatctggacaggttttagagccaggagagagaaaataattctacctctgacagttgaaggaccttaggcaaatcagtttacctctgctagactacactccaaaatttggacattcaaaaatttgatattaataaccacatgaaagtctcgtgttgaggtgaatatgtatttgttggtgaaagatatgttggtttttaaacagacagcactctgcaattgtaggctattgttttgttttgccagttgtcaaattctatccagctatacacacttgtgtggcctcctaatggtgtttttccagtggctaaaggtttatgaataagacacttttcctaatggaattaacccgatgcttttcttaaacatgtaaccttgagttcaccgcaaaaaacaatgcttcgattagagcaatgcatataataaaggttaccctcgtttcttagacactagacatcattcacaaaaagagaactgcttttgaaagggatgtatttgcactggaaagaatagttttctacttctaattataaatgatttattggtgaaagcaaaacaacagcctgtctgagaggcacttctatgagcatcctcacgtgtgatttgcaaggttgaagaagagggaaaaatgcctcaattgtaccaatggtgagaaaacacccaaagtacaaagcaggtttcaaaaaaaccatactcataaccaaggacaataataaagcaatgtgttgacatatactctataagtcttcctccataaatagtttatagaaattttgtaatttctgtaaatgcatcctataataattttgcatcttgctttttttttacatttaatatcaagtagatttctaaagggcaattatttgaaaattatcccaaatacatggggaaatatacatcaagtgaaaaaatgcagtgggtgatagagatatcaggaagcgcctcaaatatttctcatctcgttggagaaaaacaaacatgttctcatttagaatgagtgggagttacctaattgatttaggcctctatatttaacttctagtcaaaaaaggtagttctatctagcaacaatattatggggaacaaaagaaaaaattaactctctaaatttgcagtagggtcttttcttcagaagtaccaaatcccatctattaccagctccatgcttcaggcctaaaatggatctccctgaagcaatgacagaatttttgccaagtgactaggatataaacaccactttggttgcacagtgagacatatgctccaaagaaaactggttcaaaaacaggcaagtgggtttctacagaataaatgagagccctgtcaatggcttcatcttcagggctttgtgtctgtgcttgcgtggtggctcttgtttcatctatggataatggtggcacacagttttcataattccttacattaatgaactgctataaatttgtttttggtattctagagagtcctaacttcagcttctgggcaatgctgaggaggcaccctatattctagacttaccttttgcaaggtgtactctcagcattgtgggcgatttccatgggagaatattctatttaaagaactactgtcccagcataaaacaaaaaatcatttatgaagatgcaggagactcggaaagctctcaattattgtttgcacaagcacaatgtcacagcctcctttccccattccacaagggggtcaggaagagagtactcagctgtgagaaaagacatacagaagaattcatgtggtcatgagagcgaggacatggccgatcccccaaggaggatgtgtcatacacttcatgagcccaagagtgtgctgtagggtctgaagggcaagatgctggttcactgatgtaaaggagagggaaaaaagcttcaaccaactagaaaaacagtctctatgcatgctatttttgattttaaacacaggtatcaattccttctctcagagagtccattttaaaataggatacatttttaaaggaatatttaaaggacacattcattaaaatttattttaaaaacttttcaaaagaaacaaaaggtatgaattttatttaatccttgaggaaatggttcttttctcacacacataaatcactcattttgtttttctttatctcctttattaatctacattagaaaaataaacttttcatacactaagaacaaggaaaccactctcaattgacaaaatgttccaatccaacacaatgattactttcacctttaatttacaggcagccagattcaaaatccttaaagttgcttaaacttaaaaatgacaatgacaacctaaaaggtataatgttgattggaacagacatttaattggaaaattgatgattttccatttccaattaaatctctagatagaaatgaaaaaaattaaaaatcgtatttaagaaaagccaaatcttgggttgtgaggtatctttttaaggatgtttcagcagaaaaaaacaaaggctctcacaattgtgtagctgcctagattaagtgggtatcctgatcaaggagatgggggatgatttggctttagtattccaatgataaagtttataatgagaataacatgttgctacaaaatccagtctcttcctcagatgccttccacagagggcaggaagctttgtcagttttgtttgctgatgatgcctggttccgtcaacaaataacacctgtcacacggtgggtagtcaatatacatttgttgaataaatatgaaaaaaagaaatgtacaatatgtttgtgaagccaactgtgtgtgcattgctattgaggtacacaaaaagtctttgttttaaatttgagaatgaggactttcaatggaatatatctataaaaatgaaaaaaagacattactgtctggacttttgtacagcaagagaagaaaaaccactagccaagagccaactcacctgataggcctggatcaagcatgcagctgtggagaacacccctgggactctaactctggcactctgcaagctgggtacttgggcaggacagcagcagcactcatgaactgggcagcacctgttggtgagggctgatcacatggattctctcatcccagccttacaatcagtccttcaggtacatactttttctgactttgctgatgaggaaactatgcacagaggttacacagcttaacaaagggttctcacctaatgaacaatgaaatgggattttagcctttctttgcatctggtcttagagccaatacccaagaagcactgtactgtatgcattgtctcagagaaacttactcttcctgggcctcagtctttaaaaggtgggcagttgacttaataagaattaaagatcaatgattaaggttcaaggcactccaaaattctggtctttattgaaaaggctacagaagtctcaccttaataataccctatagacttgatattcttggttaattaaatattggaaaccaatttcatagtaattgaggtcagaaaaaagtactcatgacattttagaatatgatgacaaagccatagataaatttcaatgcacctgtaattacttaaaactgttatagcatgcaatgtgttaccacaacagccagagaaatactaatttactcagcctattcttctagaccagtaaacactaggattaaatagatattttcattgaatttgttctacccttcattgccatttatagatagcttacttgtcatagattactttctaattgttttatgtttcctaactagcctgcaatactttggcaaggacctcaaacaatagtagacagtaggtgtaaaatagatggctacattgaacagatgactaaaaggatgcctcctaagtacctatatcttgaaatatatattattgtgccttgctttcaatttgtgattttaaaatctagaaatcacctgttttatgtaataacaataaaatccttctttgttgaaaacatgcacaaataaagtttacaagctcaaaaaattaaacagcagtaacggtcaagctttccaacaataaaatacattttggtaaggttttcattttacaaaaactcaaaatagctttatgagttcacaaaataatatgatatttttcaagatattaacatattcttataccggaagagcatagaataaaatttacttggagattgagcatttgcttctttaagaaatacttcttttagtatttttactttaatattatgaaagctacataattacattcagattcattaactactccagtagttaatttttaaaacttatgatgaatagttttgtttaaaatatataacattggtaatatgcaaatctgaatctgtaataaagaaggatttgcattcctgatttttttttctgatacaaccaatgacaaaataactaatggttccacagaggataaaatgtctcaaatctgttggttctgaaggtgaagcgagatttttgtactgataccgtgtatcactgagataccaggaggaaatggaattaaactcagatagttcaaatggagagattttaatgaagggacgacctacagaggtgtcggcagggttggggggaatcagcgagatatgcttagaacccaccgactggcaaacctccccctgaagatggagaaggaggaaggagtgttactggaatgagagcttgagtccaggggaggaggatgggctgctgaggaggcgacaccatcctgaaagaagaatcctctgccagaggcttttcagggtcatttcttcacactctctgcagggaagcacggagacagcaggaagaaatatcctaacctcactctcttccctctacaggtgcttccattggccaaatccacccagaggccagttggtggcgatcagctctcttcaagtggtatttaaatttcttctttcattttccttctggtaacaaagaagtctgtggctcaaaagatgtttctctaagaccccatcctattaggtctctgagctgtccacaaagaaatgaaattttcactttccaggaacctaacaaatgaaaagatagaaatcaattccaacagaatattaccaaagaaatcttttagaatggactgttaaaattatttatttgtatttatctggctctactatttgtggtacatttccacttcaaagctaaacctcaaataacatcatagtgagtggttgacttcatgtttaactgagatcttgaagactgaaaaagaccacgacaaacacacatctattttcttggctactgcatccgtgttcatcaccattctgatagtctgcaatgtattgcagctcaccctttgggaaggactaaagtagacatctgtttgttctgcttactcagcattcctaccctaattttcctttggagaacccctttattctagaccacgtgaagctaatgccaaaccccattccaggggatgcacctgaatccaacctccatcatctaaacagtgccttctccacgttcagagaagagcaagtgactcaaactgccctcataagaacagacctgggacttctgctgcaaatattgaagagtaagtactcttttttcttgctaggactaagctggtagtaccttctatgaggctatcatatggaaacaacttgtctgaaaatgaagccacaactagaaaacagatcctggtaacccggattgatggatccagccctaccttaaatggcaagacctaacccgaggctttttgcatcaaccaataaagtccttaagccagtttgagttggttttgtcacttgcagctaaaagaattctgactctaacaatgtgacaatagcaaaaataaacataactgcttttgaggtttctaatggattttcctccctatatacatgatttcatttaatcctcacaattcaggaaagcacatatctattaacattaaattaatattcattattttgaacacatgctatgtggataagggatgaggaaagccaaggaagtaatcaacgtgaaatctcacttatatgggagggaagtggaggttacatatctcagggcacttaacagatatcatcaaatgaaagaataaacagtgtgtgggagaggcagtaggtgattcttcatcaattcctggatgaaaaattaggagataatgaactccgaacaggcagcctaatgagaatggctcaagcaacaggacatagagagggagttaggttagacatggggttcttgggaattttcacctcgtgggggggcgggggggtcgtgcagctgttgtcagtgggaaagggaaaaaggaaaaggctgagtttggaaggcagggagggaggagacaatgtgagtcagtgaaaaagggcccttagaatgacaagtctggaccagagagaggctaagactgaaaatacaagttgggtaaccactggcatacagatggcagttcaggcttgggcactgcccaccagagcctcagcatgaagagaagagggggaggctggccaccacctccctctaggtaatcgtcatcctgatgctgagctcctgaaaacaggctctttcactcgccccatctcttgctcttgattgcaacccggcattcaggaggcaccctgtaatatctgtggagtgaccgacaacacagcgccagggcactgagaagatcccagggcgccagggactggttctacaagggtgcccctcccggtcccctccagcgcgccgccagagctgccagtcttggctgctacacgggaggcagcctcattatgcagctctcacctcttaaattagttcatgctctcacattaggtgtaatcacagcttgcaacgctttctggggatgtctcagaaagatctgagttgaaaaaatatttttgtgtcattttaatttaaagtaaaattgctgcttcttccccgcccctttctttcctcctggcccacccagcgaccctggccggccgtgctcaacgggggcgggggtcggaggtgagatttcctccacataattccttaaacagctatcaactaagtctcaaagaaaaaaaaaagagatctagaagcagagacgtggctgctggcgatcccaaagctggtgttcgctcttgggggagagcgtaccctgggggaggccgggaggccgggccagaggctagcccagaggcagagggcaggagcgctcagccggcgccccgcgtctctccagctcccgacgctgcgctggctccgctgagcacgccaggatcaaggtcgcctggtggggaccggagcgccaggagcctgtgggaagcgttccagccggcctctgactgggatccggcgccgcgtttctgctttggacttgactgacaggtccccccgccctcccgccgccctactaccagcctgggttcatccttcagggctacgtctaccgcacccgggctggaaagcctggagcgcgcccttcctctcctcatcttctcagctctcctttctccctgccacttggcaaagctgcattttgactttcacgttttggactacgtgtgtgtagttccaagtccatgcgtggcacgaaaatccacttagggtaaaaattattctcgaaaaatcgcccatctcaggatctggtgtctacactcaaggctaggaggtgcaggtacgggtgcgtaaagcatgccgtaagggtgcacagtaaataaaaagtacggatgcaaaatgtaaattttaagtgcaaaacagaaaagcagtactcgttgccgccccgcacgctgggttttaaggggcacgaaggtgggcctcggctgcttttgctcagccccgcgtcctcagcgcccggcccagtacccggtactccgtaggggttcaatgatctcccctgaataagtgaacgaattaacaaatgaatgaatgaccgctcgatccgacctccgcggccggcagagcagtcgctggagaggcgggagagagcgagaggccaagctccaccatcgcggccgccggctggggcagagggacacggagacactcggcgccccggctccgcaccgagtccccg

SEQ ID NO: 17600 - RNA, 11184 nt, Homo sapiens
  source 1..11184: mol_type = other RNA
tcaggccaggcacagtggctcatgcctgtagtcccagcactttgggaggccgaggtgggcagatccacgaggtcaggagatcaagaccatcctaacatggtaaaaccccatctctactaacaatacaaaaaattagtcaggtgtggtggcacgtgcctgtagtcccagctactcaggaggctgaggcaggagaatcgcttgaacctgggaggcggaggttgcagtgagccgagattgtgccactgcaccctagcctaggcaacagagcaagactctgtctcaaaaaaaataaaaaaaaaaaaaagagagaaagagagagagagatgaggagttgctgcactgctgggtgtggagagccgaggaggattcaaagatggtcctgaagtcccagctggaagaagtaggcggcagcaatgtttttaatactgtaaattcatcacgtagcacaggtttggggtggagaaagaaaaattgcattggcttcagggcatgcccagatctttcctcatcttaggcgtttgctaatacatgcattttctaagctgatgtcttgcgtttaatcactgctccattcaaaagagagaaggaggttgtttcaaacctagttgatatcatttgacttccatgctattcacagggctattttatttgaaacaggtataccacagccttaaattgcaagttaatccaggatgttcctaggttggcagttaggaacatgtaattctttggaagggctaaaagtcagctctttaaattatctccatatgaaccttctctccaccttagggtggatccacttatttagtccactgccagtaccacactagaacccgggtggtcactggactccagaaacaacagtagccctctctctgttctgtctctttttgactatctctattctgttcctgaccctgatttctcctgccaagctcaattttgacagctgacaacggcaagccatggcttcccaaaacattattttcaggtcaacttataaatttcaagaacacatttggctccgcttcctgtggtactaagcctacttcttgacagcatttgcctttgttgtaaatagcaaagttcttctagttggatttttgctaagaagtgtgtggatgtggcatgtgacgacatctttagcttggattctagaaaggcactaccattgtgcatttggctaaaggaaacacattttacccgtgaatgccttctatttacaaatgctcagctagcacacaaagctaagtacaagcaataagtactatcctacaatgttactcatttctgaaagcacaaaatgatgactggtatagctttggagatgttttctggaaacccaataaaggaacagatctttgttattccacacctacaaagtcagaagatgcacagtcttttattcatgtttgaacaagcttccttcttgaacaatcaactataaagtgatgtgattctctactagaccaggaactccttgaggacagaatgagggtctaatccatattctaaatccacaccacctggcacaatacatgttgcatggttagggtcaactaagagttggttgaattaatcaataacacacagcaagagaattcacaaagagaggggagtaatcccccagcctcaatcactcggcaagtggaatcgctgggcactgattccagctctgtctcagtgcttgagacagagctgaatgtaatgtgaacatttcaaatgaacaggaaaactagactcacggataagcagtgtagtcatcaagacaacactgtcttggaggtttttctgaagttaaaaccatgctacataagcaataaattatgaaggctgagcatgtgaataaaatttaatgttgtcataaattttataacaaagttaatctgacacatttaatgacatgcataatcattagtatgcagcactgtaatcagacattgataataagcagttcacaccagtgactgtaagagtctttacttgtgttcagccaagccaactgcttggtatatttttctcccttcttagtcgttagttttccatacctacaataactatcagtggtgatgggcttctctgaccatgtgaataatttaatcctcaatgcacagatacagaaacccttgctgaagacagtgtggagcagagaaggctgtctccactccttccacctgaaacacctctgcagatggatatgggagctctgcctacagcccttggacctaaccacttcagtgtgttccagtgagtgtctggacctcggcctgaaagatttttccgaaactaaagaaaatttctctgacctaaagaccttaacctccaccccagaagctctcaccaaggactacagggaactggtggggaaaatccttatcccttactcctcaaggcacagggcagtaatgctgaggcttgtgcgccacacttgctcccagaggtccccagcgggctacctgcggtggtgaatgacctcctaacacgccccttgacggccttcctttccttgcctcacttctccactctcctaccagcattgcagggttcacatcccaaatataccactggcacttgaatcctggtctccaggtctgtttctggaaaaacccaagtaagacattgccccagtaatggggctagatgtctgaggcttcctcaagtatctacctcgaaagctcttactgctgtacacacatgcacatacacacacgtgcgtacaaccagtcacatctaagcaccccgaataccagcctgttgaaggtagcagagagctgcactataagccaaggctgctcccaagagccgctccatcactgaattggcgccccagcaagatgaaggaatgtaatcattggaaggatggagaatgttctctgaatcactgacaaattggaaggggtggagggcaagagtccacctggtggagagatggaaagagcgagagagcctggaatgataatgccattgcttagaaaaggctgctccagatgccatatctacagaaattgtacagcccaaacatctctgagcaataggtctctggtagtcttgatgtctagaccaacaattcccagttcattcttctcagggaaggagccaggatagtccagagactctcattctgctgttagattgaaagggttaggcacaacagccttggcaaagtcacaagggcaaattcacactaaagtgtaaatgacccacaactcctcttctatttttaggttggggaggtgctttagaacataaggaggaactaaagaatattcctgttacatacaaggcagagaaaagggaaactagtggtgacaagacaaatcatccctttgacatttggctggctctacctattacagctctgggggtgaggtgggaacaaaaagatgctgtgtaaagaagtatcttatgccatccctactgtagtgaggtgcagtttagaggggacactgatcaagcagagacccagagtgtttcgttccaagccagaaacagaaatgtataaaacacagcctttccagcatcagaaatgagtagtggtagtggagaactacccaaaacaggaaagaggaccacgtgaggtagagtgtcaaggccctacattccagtgcctctgctcatgactgtaattttgggtaggtcacttaaagtctctggacctcagttttgccatctgtgaaatagggataatactatccagcataaaattggttatgaggctcatgtagggcctgcctgggatgatgtgttgctaatggttaagaacacaacttctggggtctgactggacaggctgaaatccctgcttaacacgttccagcagagccctgggcgatctatttaacttttgttttctcacctgtaagctgagacgaaagtacccactttataagattattccaataattagttgaaataatgcatgcagagaattaagcatggtacttgttatttgttaaactagctattaaaatgtgtaaaatataaagtattgtatggattttaggacaatgcaaagactctttgcttgctgcaatagttcggggccctttcagatggctaaaggcagaatttgtatgtgtaaatatggtgtgcttgtctctgctctggatactgagggcttaccctgttattaaacttatttagtaaatattgaactgtcatgaggcctaacatttagttccagttattagataaaacatttgctttgaatggtatttgaattgccaggttctagattattctggttgacaaactcttcgtattttataaagaggctaaaattggtaagctatcacagaacagatgtgccattttcaaggtatattaaaccatgattcactgtaacattgttcctactggcaacaaattcagagcaggctggactttatttggtgaagaaacattgagtggaagagaaatgacattattttatgtatttacattttcaaattactgtggcttaaacctgttcagccaacattacccaccttcagtctgctaaataaatgattcagtacatttctaatttacagaattttttaacaaaagaaaatgtaatttgatagccaaatcaacgttaaacattatacatttaaaaaaccacaggcaaagacacaaacatgatgacactaacttttgttaaagtatgcttacctatggtttcctctgaggcacgttctttcatgctaagcttccaacataatatgaaaatgaaggagatgcattttgcaaagcaaaacagaccttaagcaaaatattatacttctcaaattaacactgttacaaagttttagaatttaataagttcattaatttaaaagtttggatgtctgagtccttctatcccaaaacaagatcttggagggtcttccacagccatgtaataccatggtcacatgaccctttccaaaattattaatctgaatttactatatgaggataaatctatctttttgaaaatatttaggaaaatgagcttggtatttataaaatgaagctctctttgggtggtatcctaagacacgtcaagccaatcagcctgtaactgtgaaaaaaacattggtaggtacaaaagtggggtgggagaggagtgacttaactttgttaagtgatgggaaagaaacactaatagcattatctcaataaaatgtgatttaaaaaaatttaaaatactaaatcattgaactgacaaagaaatataaatcattcagaaataaactcattaggtcatcaaatcctgttaaatctgcaattaggaagagcaaggtgtacaatccatacatttaaactcacaggctcactttgcacaacgtcaatttactccttaatatgttattaatacgcattttccaaaaggatgtattagtaaatggtacacatctacttcttggcaacatcatataacctggtacaacataagcattcttcttatagttaagaaatgtggatggtatcaaaattagaaaaataaatgccctattatgttgtggtcaggtttaaggcatgtgaattttatcttcatacaaaagattaaaatctagatattaaaaagtagtgcagtatcagtgatgctgcctcagttcccaaaatgtcacatcacaaaaatatcccataattgcctgtagtttattccttggctttcctcttttctctctgcatctttgtaacaattttttaaaagtggaaatataattgttggcaatgctaacagctgtagaaatgattacaagatgtggaaaagcataacaggaatgtcaagaatctgtttctggcagtaatatatatggaacattgttcaggacaaaagaggagaaggaagaaaaaaaggagaggggtttatcatctctaagaattttcaaactaaacctcattgcttaataggaaaaaaagattccatatttaaagttaagtcacctctaactactagctaaagcatgacatcaccagcactggagtcagcggaagtgtgtttttgaaggacagtgttgcaggagaatctggacaggttttagagccaggagagagaaaataattctacctctgacagttgaaggaccttaggcaaatcagtttacctctgctagactacactccaaaatttggacattcaaaaatttgatattaataaccacatgaaagtctcgtgttgaggtgaatatgtatttgttggtgaaagatatgttggtttttaaacagacagcactctgcaattgtaggctattgttttgttttgccagttgtcaaattctatccagctatacacacttgtgtggcctcctaatggtgtttttccagtggctaaaggtttatgaataagacacttttcctaatggaattaacccgatgcttttcttaaacatgtaaccttgagttcaccgcaaaaaacaatgcttcgattagagcaatgcatataataaaggttaccctcgtttcttagacactagacatcattcacaaaaagagaactgcttttgaaagggatgtatttgcactggaaagaatagttttctacttctaattataaatgatttattggtgaaagcaaaacaacagcctgtctgagaggcacttctatgagcatcctcacgtgtgatttgcaaggttgaagaagagggaaaaatgcctcaattgtaccaatggtgagaaaacacccaaagtacaaagcaggtttcaaaaaaaccatactcataaccaaggacaataataaagcaatgtgttgacatatactctataagtcttcctccataaatagtttatagaaattttgtaatttctgtaaatgcatcctataataattttgcatcttgctttttttttacatttaatatcaagtagatttctaaagggcaattatttgaaaattatcccaaatacatggggaaatatacatcaagtgaaaaaatgcagtgggtgatagagatatcaggaagcgcctcaaatatttctcatctcgttggagaaaaacaaacatgttctcatttagaatgagtgggagttacctaattgatttaggcctctatatttaacttctagtcaaaaaaggtagttctatctagcaacaatattatggggaacaaaagaaaaaattaactctctaaatttgcagtagggtcttttcttcagaagtaccaaatcccatctattaccagctccatgcttcaggcctaaaatggatctccctgaagcaatgacagaatttttgccaagtgactaggatataaacaccactttggttgcacagtgagacatatgctccaaagaaaactggttcaaaaacaggcaagtgggtttctacagaataaatgagagccctgtcaatggcttcatcttcagggctttgtgtctgtgcttgcgtggtggctcttgtttcatctatggataatggtggcacacagttttcataattccttacattaatgaactgctataaatttgtttttggtattctagagagtcctaacttcagcttctgggcaatgctgaggaggcaccctatattctagacttaccttttgcaaggtgtactctcagcattgtgggcgatttccatgggagaatattctatttaaagaactactgtcccagcataaaacaaaaaatcatttatgaagatgcaggagactcggaaagctctcaattattgtttgcacaagcacaatgtcacagcctcctttccccattccacaagggggtcaggaagagagtactcagctgtgagaaaagacatacagaagaattcatgtggtcatgagagcgaggacatggccgatcccccaaggaggatgtgtcatacacttcatgagcccaagagtgtgctgtagggtctgaagggcaagatgctggttcactgatgtaaaggagagggaaaaaagcttcaaccaactagaaaaacagtctctatgcatgctatttttgattttaaacacaggtatcaattccttctctcagagagtccattttaaaataggatacatttttaaaggaatatttaaaggacacattcattaaaatttattttaaaaacttttcaaaagaaacaaaaggtatgaattttatttaatccttgaggaaatggttcttttctcacacacataaatcactcattttgtttttctttatctcctttattaatctacattagaaaaataaacttttcatacactaagaacaaggaaaccactctcaattgacaaaatgttccaatccaacacaatgattactttcacctttaatttacaggcagccagattcaaaatccttaaagttgcttaaacttaaaaatgacaatgacaacctaaaaggtataatgttgattggaacagacatttaattggaaaattgatgattttccatttccaattaaatctctagatagaaatgaaaaaaattaaaaatcgtatttaagaaaagccaaatcttgggttgtgaggtatctttttaaggatgtttcagcagaaaaaaacaaaggctctcacaattgtgtagctgcctagattaagtgggtatcctgatcaaggagatgggggatgatttggctttagtattccaatgataaagtttataatgagaataacatgttgctacaaaatccagtctcttcctcagatgccttccacagagggcaggaagctttgtcagttttgtttgctgatgatgcctggttccgtcaacaaataacacctgtcacacggtgggtagtcaatatacatttgttgaataaatatgaaaaaaagaaatgtacaatatgtttgtgaagccaactgtgtgtgcattgctattgaggtacacaaaaagtctttgttttaaatttgagaatgaggactttcaatggaatatatctataaaaatgaaaaaaagacattactgtctggacttttgtacagcaagagaagaaaaaccactagccaagagccaactcacctgataggcctggatcaagcatgcagctgtggagaacacccctgggactctaactctggcactctgcaagctgggtacttgggcaggacagcagcagcactcatgaactgggcagcacctgttggtgagggctgatcacatggattctctcatcccagccttacaatcagtccttcaggtacatactttttctgactttgctgatgaggaaactatgcacagaggttacacagcttaacaaagggttctcacctaatgaacaatgaaatgggattttagcctttctttgcatctggtcttagagccaatacccaagaagcactgtactgtatgcattgtctcagagaaacttactcttcctgggcctcagtctttaaaaggtgggcagttgacttaataagaattaaagatcaatgattaaggttcaaggcactccaaaattctggtctttattgaaaaggctacagaagtctcaccttaataataccctatagacttgatattcttggttaattaaatattggaaaccaatttcatagtaattgaggtcagaaaaaagtactcatgacattttagaatatgatgacaaagccatagataaatttcaatgcacctgtaattacttaaaactgttatagcatgcaatgtgttaccacaacagccagagaaatactaatttactcagcctattcttctagaccagtaaacactaggattaaatagatattttcattgaatttgttctacccttcattgccatttatagatagcttacttgtcatagattactttctaattgttttatgtttcctaactagcctgcaatactttggcaaggacctcaaacaatagtagacagtaggtgtaaaatagatggctacattgaacagatgactaaaaggatgcctcctaagtacctatatcttgaaatatatattattgtgccttgctttcaatttgtgattttaaaatctagaaatcacctgttttatgtaataacaataaaatccttctttgttgaaaacatgcacaaataaagtttacaagctcaaaaaattaaacagcagtaacggtcaagctttccaacaataaaatacattttggtaaggttttcattttacaaaaactcaaaatagctttatgagttcacaaaataatatgatatttttcaagatattaacatattcttataccggaagagcatagaataaaatttacttggagattgagcatttgcttctttaagaaatacttcttttagtatttttactttaatattatgaaagctacataattacattcagattcattaactactccagtagttaatttttaaaacttatgatgaatagttttgtttaaaatatataacattggtaatatgcaaatctgaatctgtaataaagaaggatttgcattcctgatttttttttctgatacaaccaatgacaaaataactaatggttccacagaggataaaatgtctcaaatctgttggttctgaaggtgaagcgagatttttgtactgataccgtgtatcactgagataccaggaggaaatggaattaaactcagatagttcaaatggagagattttaatgaagggacgacctacagaggtgtcggcagggttggggggaatcagcgagatatgcttagaacccaccgactggcaaacctccccctgaagatggagaaggaggaaggagtgttactggaatgagagcttgagtccaggggaggaggatgggctgctgaggaggcgacaccatcctgaaagaagaatcctctgccagaggcttttcagggtcatttcttcacactctctgcagggaagcacggagacagcaggaagaaatatcctaacctcactctcttccctctacaggtgcttccattggccaaatccacccagaggccagttggtggcgatcagctctcttcaagtggtatttaaatttcttctttcattttccttctggtaacaaagaagtctgtggctcaaaagatgtttctctaagaccccatcctattaggtctctgagctgtccacaaagaaatgaaattttcactttccaggaacctgagggccgacgagtgggggcgggcaggagggccgagggaggcggaacaggatcgaggcgcgaggcgggagtcgagaaagcgagcggccgaggcgactctcagtgcgcggacgcgggcgcgcgcccgcgctcccttcgtcgactcacggcgagagcccaaccctgctgccgcgcgccaccc

SEQ ID NO: 17601 - RNA, 12992 nt, Homo sapiens
  source 1..12992: mol_type = other RNA
tcaggccaggcacagtggctcatgcctgtagtcccagcactttgggaggccgaggtgggcagatccacgaggtcaggagatcaagaccatcctaacatggtaaaaccccatctctactaacaatacaaaaaattagtcaggtgtggtggcacgtgcctgtagtcccagctactcaggaggctgaggcaggagaatcgcttgaacctgggaggcggaggttgcagtgagccgagattgtgccactgcaccctagcctaggcaacagagcaagactctgtctcaaaaaaaataaaaaaaaaaaaaagagagaaagagagagagagatgaggagttgctgcactgctgggtgtggagagccgaggaggattcaaagatggtcctgaagtcccagctggaagaagtaggcggcagcaatgtttttaatactgtaaattcatcacgtagcacaggtttggggtggagaaagaaaaattgcattggcttcagggcatgcccagatctttcctcatcttaggcgtttgctaatacatgcattttctaagctgatgtcttgcgtttaatcactgctccattcaaaagagagaaggaggttgtttcaaacctagttgatatcatttgacttccatgctattcacagggctattttatttgaaacaggtataccacagccttaaattgcaagttaatccaggatgttcctaggttggcagttaggaacatgtaattctttggaagggctaaaagtcagctctttaaattatctccatatgaaccttctctccaccttagggtggatccacttatttagtccactgccagtaccacactagaacccgggtggtcactggactccagaaacaacagtagccctctctctgttctgtctctttttgactatctctattctgttcctgaccctgatttctcctgccaagctcaattttgacagctgacaacggcaagccatggcttcccaaaacattattttcaggtcaacttataaatttcaagaacacatttggctccgcttcctgtggtactaagcctacttcttgacagcatttgcctttgttgtaaatagcaaagttcttctagttggatttttgctaagaagtgtgtggatgtggcatgtgacgacatctttagcttggattctagaaaggcactaccattgtgcatttggctaaaggaaacacattttacccgtgaatgccttctatttacaaatgctcagctagcacacaaagctaagtacaagcaataagtactatcctacaatgttactcatttctgaaagcacaaaatgatgactggtatagctttggagatgttttctggaaacccaataaaggaacagatctttgttattccacacctacaaagtcagaagatgcacagtcttttattcatgtttgaacaagcttccttcttgaacaatcaactataaagtgatgtgattctctactagaccaggaactccttgaggacagaatgagggtctaatccatattctaaatccacaccacctggcacaatacatgttgcatggttagggtcaactaagagttggttgaattaatcaataacacacagcaagagaattcacaaagagaggggagtaatcccccagcctcaatcactcggcaagtggaatcgctgggcactgattccagctctgtctcagtgcttgagacagagctgaatgtaatgtgaacatttcaaatgaacaggaaaactagactcacggataagcagtgtagtcatcaagacaacactgtcttggaggtttttctgaagttaaaaccatgctacataagcaataaattatgaaggctgagcatgtgaataaaatttaatgttgtcataaattttataacaaagttaatctgacacatttaatgacatgcataatcattagtatgcagcactgtaatcagacattgataataagcagttcacaccagtgactgtaagagtctttacttgtgttcagccaagccaactgcttggtatatttttctcccttcttagtcgttagttttccatacctacaataactatcagtggtgatgggcttctctgaccatgtgaataatttaatcctcaatgcacagatacagaaacccttgctgaagacagtgtggagcagagaaggctgtctccactccttccacctgaaacacctctgcagatggatatgggagctctgcctacagcccttggacctaaccacttcagtgtgttccagtgagtgtctggacctcggcctgaaagatttttccgaaactaaagaaaatttctctgacctaaagaccttaacctccaccccagaagctctcaccaaggactacagggaactggtggggaaaatccttatcccttactcctcaaggcacagggcagtaatgctgaggcttgtgcgccacacttgctcccagaggtccccagcgggctacctgcggtggtgaatgacctcctaacacgccccttgacggccttcctttccttgcctcacttctccactctcctaccagcattgcagggttcacatcccaaatataccactggcacttgaatcctggtctccaggtctgtttctggaaaaacccaagtaagacattgccccagtaatggggctagatgtctgaggcttcctcaagtatctacctcgaaagctcttactgctgtacacacatgcacatacacacacgtgcgtacaaccagtcacatctaagcaccccgaataccagcctgttgaaggtagcagagagctgcactataagccaaggctgctcccaagagccgctccatcactgaattggcgccccagcaagatgaaggaatgtaatcattggaaggatggagaatgttctctgaatcactgacaaattggaaggggtggagggcaagagtccacctggtggagagatggaaagagcgagagagcctggaatgataatgccattgcttagaaaaggctgctccagatgccatatctacagaaattgtacagcccaaacatctctgagcaataggtctctggtagtcttgatgtctagaccaacaattcccagttcattcttctcagggaaggagccaggatagtccagagactctcattctgctgttagattgaaagggttaggcacaacagccttggcaaagtcacaagggcaaattcacactaaagtgtaaatgacccacaactcctcttctatttttaggttggggaggtgctttagaacataaggaggaactaaagaatattcctgttacatacaaggcagagaaaagggaaactagtggtgacaagacaaatcatccctttgacatttggctggctctacctattacagctctgggggtgaggtgggaacaaaaagatgctgtgtaaagaagtatcttatgccatccctactgtagtgaggtgcagtttagaggggacactgatcaagcagagacccagagtgtttcgttccaagccagaaacagaaatgtataaaacacagcctttccagcatcagaaatgagtagtggtagtggagaactacccaaaacaggaaagaggaccacgtgaggtagagtgtcaaggccctacattccagtgcctctgctcatgactgtaattttgggtaggtcacttaaagtctctggacctcagttttgccatctgtgaaatagggataatactatccagcataaaattggttatgaggctcatgtagggcctgcctgggatgatgtgttgctaatggttaagaacacaacttctggggtctgactggacaggctgaaatccctgcttaacacgttccagcagagccctgggcgatctatttaacttttgttttctcacctgtaagctgagacgaaagtacccactttataagattattccaataattagttgaaataatgcatgcagagaattaagcatggtacttgttatttgttaaactagctattaaaatgtgtaaaatataaagtattgtatggattttaggacaatgcaaagactctttgcttgctgcaatagttcggggccctttcagatggctaaaggcagaatttgtatgtgtaaatatggtgtgcttgtctctgctctggatactgagggcttaccctgttattaaacttatttagtaaatattgaactgtcatgaggcctaacatttagttccagttattagataaaacatttgctttgaatggtatttgaattgccaggttctagattattctggttgacaaactcttcgtattttataaagaggctaaaattggtaagctatcacagaacagatgtgccattttcaaggtatattaaaccatgattcactgtaacattgttcctactggcaacaaattcagagcaggctggactttatttggtgaagaaacattgagtggaagagaaatgacattattttatgtatttacattttcaaattactgtggcttaaacctgttcagccaacattacccaccttcagtctgctaaataaatgattcagtacatttctaatttacagaattttttaacaaaagaaaatgtaatttgatagccaaatcaacgttaaacattatacatttaaaaaaccacaggcaaagacacaaacatgatgacactaacttttgttaaagtatgcttacctatggtttcctctgaggcacgttctttcatgctaagcttccaacataatatgaaaatgaaggagatgcattttgcaaagcaaaacagaccttaagcaaaatattatacttctcaaattaacactgttacaaagttttagaatttaataagttcattaatttaaaagtttggatgtctgagtccttctatcccaaaacaagatcttggagggtcttccacagccatgtaataccatggtcacatgaccctttccaaaattattaatctgaatttactatatgaggataaatctatctttttgaaaatatttaggaaaatgagcttggtatttataaaatgaagctctctttgggtggtatcctaagacacgtcaagccaatcagcctgtaactgtgaaaaaaacattggtaggtacaaaagtggggtgggagaggagtgacttaactttgttaagtgatgggaaagaaacactaatagcattatctcaataaaatgtgatttaaaaaaatttaaaatactaaatcattgaactgacaaagaaatataaatcattcagaaataaactcattaggtcatcaaatcctgttaaatctgcaattaggaagagcaaggtgtacaatccatacatttaaactcacaggctcactttgcacaacgtcaatttactccttaatatgttattaatacgcattttccaaaaggatgtattagtaaatggtacacatctacttcttggcaacatcatataacctggtacaacataagcattcttcttatagttaagaaatgtggatggtatcaaaattagaaaaataaatgccctattatgttgtggtcaggtttaaggcatgtgaattttatcttcatacaaaagattaaaatctagatattaaaaagtagtgcagtatcagtgatgctgcctcagttcccaaaatgtcacatcacaaaaatatcccataattgcctgtagtttattccttggctttcctcttttctctctgcatctttgtaacaattttttaaaagtggaaatataattgttggcaatgctaacagctgtagaaatgattacaagatgtggaaaagcataacaggaatgtcaagaatctgtttctggcagtaatatatatggaacattgttcaggacaaaagaggagaaggaagaaaaaaaggagaggggtttatcatctctaagaattttcaaactaaacctcattgcttaataggaaaaaaagattccatatttaaagttaagtcacctctaactactagctaaagcatgacatcaccagcactggagtcagcggaagtgtgtttttgaaggacagtgttgcaggagaatctggacaggttttagagccaggagagagaaaataattctacctctgacagttgaaggaccttaggcaaatcagtttacctctgctagactacactccaaaatttggacattcaaaaatttgatattaataaccacatgaaagtctcgtgttgaggtgaatatgtatttgttggtgaaagatatgttggtttttaaacagacagcactctgcaattgtaggctattgttttgttttgccagttgtcaaattctatccagctatacacacttgtgtggcctcctaatggtgtttttccagtggctaaaggtttatgaataagacacttttcctaatggaattaacccgatgcttttcttaaacatgtaaccttgagttcaccgcaaaaaacaatgcttcgattagagcaatgcatataataaaggttaccctcgtttcttagacactagacatcattcacaaaaagagaactgcttttgaaagggatgtatttgcactggaaagaatagttttctacttctaattataaatgatttattggtgaaagcaaaacaacagcctgtctgagaggcacttctatgagcatcctcacgtgtgatttgcaaggttgaagaagagggaaaaatgcctcaattgtaccaatggtgagaaaacacccaaagtacaaagcaggtttcaaaaaaaccatactcataaccaaggacaataataaagcaatgtgttgacatatactctataagtcttcctccataaatagtttatagaaattttgtaatttctgtaaatgcatcctataataattttgcatcttgctttttttttacatttaatatcaagtagatttctaaagggcaattatttgaaaattatcccaaatacatggggaaatatacatcaagtgaaaaaatgcagtgggtgatagagatatcaggaagcgcctcaaatatttctcatctcgttggagaaaaacaaacatgttctcatttagaatgagtgggagttacctaattgatttaggcctctatatttaacttctagtcaaaaaaggtagttctatctagcaacaatattatggggaacaaaagaaaaaattaactctctaaatttgcagtagggtcttttcttcagaagtaccaaatcccatctattaccagctccatgcttcaggcctaaaatggatctccctgaagcaatgacagaatttttgccaagtgactaggatataaacaccactttggttgcacagtgagacatatgctccaaagaaaactggttcaaaaacaggcaagtgggtttctacagaataaatgagagccctgtcaatggcttcatcttcagggctttgtgtctgtgcttgcgtggtggctcttgtttcatctatggataatggtggcacacagttttcataattccttacattaatgaactgctataaatttgtttttggtattctagagagtcctaacttcagcttctgggcaatgctgaggaggcaccctatattctagacttaccttttgcaaggtgtactctcagcattgtgggcgatttccatgggagaatattctatttaaagaactactgtcccagcataaaacaaaaaatcatttatgaagatgcaggagactcggaaagctctcaattattgtttgcacaagcacaatgtcacagcctcctttccccattccacaagggggtcaggaagagagtactcagctgtgagaaaagacatacagaagaattcatgtggtcatgagagcgaggacatggccgatcccccaaggaggatgtgtcatacacttcatgagcccaagagtgtgctgtagggtctgaagggcaagatgctggttcactgatgtaaaggagagggaaaaaagcttcaaccaactagaaaaacagtctctatgcatgctatttttgattttaaacacaggtatcaattccttctctcagagagtccattttaaaataggatacatttttaaaggaatatttaaaggacacattcattaaaatttattttaaaaacttttcaaaagaaacaaaaggtatgaattttatttaatccttgaggaaatggttcttttctcacacacataaatcactcattttgtttttctttatctcctttattaatctacattagaaaaataaacttttcatacactaagaacaaggaaaccactctcaattgacaaaatgttccaatccaacacaatgattactttcacctttaatttacaggcagccagattcaaaatccttaaagttgcttaaacttaaaaatgacaatgacaacctaaaaggtataatgttgattggaacagacatttaattggaaaattgatgattttccatttccaattaaatctctagatagaaatgaaaaaaattaaaaatcgtatttaagaaaagccaaatcttgggttgtgaggtatctttttaaggatgtttcagcagaaaaaaacaaaggctctcacaattgtgtagctgcctagattaagtgggtatcctgatcaaggagatgggggatgatttggctttagtattccaatgataaagtttataatgagaataacatgttgctacaaaatccagtctcttcctcagatgccttccacagagggcaggaagctttgtcagttttgtttgctgatgatgcctggttccgtcaacaaataacacctgtcacacggtgggtagtcaatatacatttgttgaataaatatgaaaaaaagaaatgtacaatatgtttgtgaagccaactgtgtgtgcattgctattgaggtacacaaaaagtctttgttttaaatttgagaatgaggactttcaatggaatatatctataaaaatgaaaaaaagacattactgtctggacttttgtacagcaagagaagaaaaaccactagccaagagccaactcacctgataggcctggatcaagcatgcagctgtggagaacacccctgggactctaactctggcactctgcaagctgggtacttgggcaggacagcagcagcactcatgaactgggcagcacctgttggtgagggctgatcacatggattctctcatcccagccttacaatcagtccttcaggtacatactttttctgactttgctgatgaggaaactatgcacagaggttacacagcttaacaaagggttctcacctaatgaacaatgaaatgggattttagcctttctttgcatctggtcttagagccaatacccaagaagcactgtactgtatgcattgtctcagagaaacttactcttcctgggcctcagtctttaaaaggtgggcagttgacttaataagaattaaagatcaatgattaaggttcaaggcactccaaaattctggtctttattgaaaaggctacagaagtctcaccttaataataccctatagacttgatattcttggttaattaaatattggaaaccaatttcatagtaattgaggtcagaaaaaagtactcatgacattttagaatatgatgacaaagccatagataaatttcaatgcacctgtaattacttaaaactgttatagcatgcaatgtgttaccacaacagccagagaaatactaatttactcagcctattcttctagaccagtaaacactaggattaaatagatattttcattgaatttgttctacccttcattgccatttatagatagcttacttgtcatagattactttctaattgttttatgtttcctaactagcctgcaatactttggcaaggacctcaaacaatagtagacagtaggtgtaaaatagatggctacattgaacagatgactaaaaggatgcctcctaagtacctatatcttgaaatatatattattgtgccttgctttcaatttgtgattttaaaatctagaaatcacctgttttatgtaataacaataaaatccttctttgttgaaaacatgcacaaataaagtttacaagctcaaaaaattaaacagcagtaacggtcaagctttccaacaataaaatacattttggtaaggttttcattttacaaaaactcaaaatagctttatgagttcacaaaataatatgatatttttcaagatattaacatattcttataccggaagagcatagaataaaatttacttggagattgagcatttgcttctttaagaaatacttcttttagtatttttactttaatattatgaaagctacataattacattcagattcattaactactccagtagttaatttttaaaacttatgatgaatagttttgtttaaaatatataacattggtaatatgcaaatctgaatctgtaataaagaaggatttgcattcctgatttttttttctgatacaaccaatgacaaaataactaatggttccacagaggataaaatgtctcaaatctgttggttctgaaggtgaagcgagatttttgtactgataccgtgtatcactgagataccaggaggaaatggaattaaactcagatagttcaaatggagagattttaatgaagggacgacctacagaggtgtcggcagggttggggggaatcagcgagatatgcttagaacccaccgactggcaaacctccccctgaagatggagaaggaggaaggagtgttactggaatgagagcttgagtccaggggaggaggatgggctgctgaggaggcgacaccatcctgaaagaagaatcctctgccagaggcttttcagggtcatttcttcacactctctgcagggaagcacggagacagcaggaagaaatatcctaacctcactctcttccctctacaggtgcttccattggccaaatccacccagaggccagttggtggcgatcagctctcttcaagtggtatttaaatttcttctttcattttccttctggtaacaaagaagtctgtggctcaaaagatgtttctctaagaccccatcctattaggtctctgagctgtgggaagtatttatacaattgcttgtgaatataagatccaggaatttccctaagatccctaacaaaattggtgataagtagtcccacatgttaatccagccacccacggatgacagcacttaccatttctttgataaatgtcaaatgcatttgaagtacctacctgaaatatttgtttaaatgctatctaatctattaattttatatatgtgtgagtctgttttgtataccttctgattataggataaatgtaaataaatccaaagagtaatcaaagctaccactttcaagaagccttctttgtagaaccggaagagtcttaaataggcttttcaggtatgcatctcttattatcgctgaactccaagtcctgcaaggcaggcatcatgtgtgggtcacctttacagtaggcacaggccttaaaacagtgacatgcacattgcaggcactccataaatgtttgctgaattggctaaaccttggtttgttcccataatcaaccaccacaaacagcacacagataattacttcttggaaagattccaactagtgtttgatgttacctacgtggtttttctctcaagatcttaagagcagctctgtaggattacattattttctgttttttttttcctttgaccttaatgtcatctacttcaataacagcttcatacaaaattcctaccagcacataccacagcagattcaaggccttgttttaaaaatggtgccagcttctcttaatttggaagatatattgtctctcctgaacatgggctaagaaaatgtataatttggtattaacataagagctgaagacactttaaatgcattgtttcatttttataagataaaaaaaattttaagaatcaaaatgttatcaacagacttgtccttcattaaaaagtaaaactgcatttgcctacattttatgaaagtgtccaattatgaacaattttgaaatgtaacttttaaaaatgtaaacagcaaaaatgttgtatttaaaataaatctggaaaggcagaaaaacaaaaaatacccagaagacagagtttttggtgaaagttaagatatttcatctttgaacaacttagaatctttcctgcattttatagtctagttccaggcattaatttgaaataaccttggaatcctaaatctaacacccttcggaacaaagtagcttttctcttctgctttatgagcaaatggactaaatactagggaatggtactgtctgggcctttgaaccaagattgaaagagatgaaatcctatatgatatgtataaacattagagaatccattttgatttaataaaaggttgaatttgttctatatcctgtgagaaaatggttcccttttcctgaaaatgttacctcattccaacaatagaaagttggtttttttccagggtgtggtgttggcgggggacagagttgccatgaatatggcatctatgaagactgctgttatattcatttctcaaaatgcactgtggtaggaaattcagaacgcagtgagagaaaataaatgtttgacttcaaaatataaggccgcatttaaagcagaaggtaaagtatagaacagttgacagtataaattctttatctgcaatcttgcagttccctaaatctctgtaacacatcacttttaaaagcctcagataagtggttctataataatttaccaataattcaacccctcaaaagtcttagcaagttaaaccttataatcttacattttagaaatgacccaacttgatccttttattcttcagaatatctctctcaaattttcatttgtttttcattaattgatgaataatgagacattttaggtacctgagggccgacgagtgggggcgggcaggagggccgagggaggcggaacaggatcgaggcgcgaggcgggagtcgagaaagcgagcggccgaggcgactctcagtgcgcggacgcgggcgcgcgcccgcgctcccttcgtcgactcacggcgagagcccaaccctgctgccgcgcgccaccc

SEQ ID NO: 17602 - RNA, 14841 nt, Homo sapiens
  source 1..14841: mol_type = other RNA
tcaggccaggcacagtggctcatgcctgtagtcccagcactttgggaggccgaggtgggcagatccacgaggtcaggagatcaagaccatcctaacatggtaaaaccccatctctactaacaatacaaaaaattagtcaggtgtggtggcacgtgcctgtagtcccagctactcaggaggctgaggcaggagaatcgcttgaacctgggaggcggaggttgcagtgagccgagattgtgccactgcaccctagcctaggcaacagagcaagactctgtctcaaaaaaaataaaaaaaaaaaaaagagagaaagagagagagagatgaggagttgctgcactgctgggtgtggagagccgaggaggattcaaagatggtcctgaagtcccagctggaagaagtaggcggcagcaatgtttttaatactgtaaattcatcacgtagcacaggtttggggtggagaaagaaaaattgcattggcttcagggcatgcccagatctttcctcatcttaggcgtttgctaatacatgcattttctaagctgatgtcttgcgtttaatcactgctccattcaaaagagagaaggaggttgtttcaaacctagttgatatcatttgacttccatgctattcacagggctattttatttgaaacaggtataccacagccttaaattgcaagttaatccaggatgttcctaggttggcagttaggaacatgtaattctttggaagggctaaaagtcagctctttaaattatctccatatgaaccttctctccaccttagggtggatccacttatttagtccactgccagtaccacactagaacccgggtggtcactggactccagaaacaacagtagccctctctctgttctgtctctttttgactatctctattctgttcctgaccctgatttctcctgccaagctcaattttgacagctgacaacggcaagccatggcttcccaaaacattattttcaggtcaacttataaatttcaagaacacatttggctccgcttcctgtggtactaagcctacttcttgacagcatttgcctttgttgtaaatagcaaagttcttctagttggatttttgctaagaagtgtgtggatgtggcatgtgacgacatctttagcttggattctagaaaggcactaccattgtgcatttggctaaaggaaacacattttacccgtgaatgccttctatttacaaatgctcagctagcacacaaagctaagtacaagcaataagtactatcctacaatgttactcatttctgaaagcacaaaatgatgactggtatagctttggagatgttttctggaaacccaataaaggaacagatctttgttattccacacctacaaagtcagaagatgcacagtcttttattcatgtttgaacaagcttccttcttgaacaatcaactataaagtgatgtgattctctactagaccaggaactccttgaggacagaatgagggtctaatccatattctaaatccacaccacctggcacaatacatgttgcatggttagggtcaactaagagttggttgaattaatcaataacacacagcaagagaattcacaaagagaggggagtaatcccccagcctcaatcactcggcaagtggaatcgctgggcactgattccagctctgtctcagtgcttgagacagagctgaatgtaatgtgaacatttcaaatgaacaggaaaactagactcacggataagcagtgtagtcatcaagacaacactgtcttggaggtttttctgaagttaaaaccatgctacataagcaataaattatgaaggctgagcatgtgaataaaatttaatgttgtcataaattttataacaaagttaatctgacacatttaatgacatgcataatcattagtatgcagcactgtaatcagacattgataataagcagttcacaccagtgactgtaagagtctttacttgtgttcagccaagccaactgcttggtatatttttctcccttcttagtcgttagttttccatacctacaataactatcagtggtgatgggcttctctgaccatgtgaataatttaatcctcaatgcacagatacagaaacccttgctgaagacagtgtggagcagagaaggctgtctccactccttccacctgaaacacctctgcagatggatatgggagctctgcctacagcccttggacctaaccacttcagtgtgttccagtgagtgtctggacctcggcctgaaagatttttccgaaactaaagaaaatttctctgacctaaagaccttaacctccaccccagaagctctcaccaaggactacagggaactggtggggaaaatccttatcccttactcctcaaggcacagggcagtaatgctgaggcttgtgcgccacacttgctcccagaggtccccagcgggctacctgcggtggtgaatgacctcctaacacgccccttgacggccttcctttccttgcctcacttctccactctcctaccagcattgcagggttcacatcccaaatataccactggcacttgaatcctggtctccaggtctgtttctggaaaaacccaagtaagacattgccccagtaatggggctagatgtctgaggcttcctcaagtatctacctcgaaagctcttactgctgtacacacatgcacatacacacacgtgcgtacaaccagtcacatctaagcaccccgaataccagcctgttgaaggtagcagagagctgcactataagccaaggctgctcccaagagccgctccatcactgaattggcgccccagcaagatgaaggaatgtaatcattggaaggatggagaatgttctctgaatcactgacaaattggaaggggtggagggcaagagtccacctggtggagagatggaaagagcgagagagcctggaatgataatgccattgcttagaaaaggctgctccagatgccatatctacagaaattgtacagcccaaacatctctgagcaataggtctctggtagtcttgatgtctagaccaacaattcccagttcattcttctcagggaaggagccaggatagtccagagactctcattctgctgttagattgaaagggttaggcacaacagccttggcaaagtcacaagggcaaattcacactaaagtgtaaatgacccacaactcctcttctatttttaggttggggaggtgctttagaacataaggaggaactaaagaatattcctgttacatacaaggcagagaaaagggaaactagtggtgacaagacaaatcatccctttgacatttggctggctctacctattacagctctgggggtgaggtgggaacaaaaagatgctgtgtaaagaagtatcttatgccatccctactgtagtgaggtgcagtttagaggggacactgatcaagcagagacccagagtgtttcgttccaagccagaaacagaaatgtataaaacacagcctttccagcatcagaaatgagtagtggtagtggagaactacccaaaacaggaaagaggaccacgtgaggtagagtgtcaaggccctacattccagtgcctctgctcatgactgtaattttgggtaggtcacttaaagtctctggacctcagttttgccatctgtgaaatagggataatactatccagcataaaattggttatgaggctcatgtagggcctgcctgggatgatgtgttgctaatggttaagaacacaacttctggggtctgactggacaggctgaaatccctgcttaacacgttccagcagagccctgggcgatctatttaacttttgttttctcacctgtaagctgagacgaaagtacccactttataagattattccaataattagttgaaataatgcatgcagagaattaagcatggtacttgttatttgttaaactagctattaaaatgtgtaaaatataaagtattgtatggattttaggacaatgcaaagactctttgcttgctgcaatagttcggggccctttcagatggctaaaggcagaatttgtatgtgtaaatatggtgtgcttgtctctgctctggatactgagggcttaccctgttattaaacttatttagtaaatattgaactgtcatgaggcctaacatttagttccagttattagataaaacatttgctttgaatggtatttgaattgccaggttctagattattctggttgacaaactcttcgtattttataaagaggctaaaattggtaagctatcacagaacagatgtgccattttcaaggtatattaaaccatgattcactgtaacattgttcctactggcaacaaattcagagcaggctggactttatttggtgaagaaacattgagtggaagagaaatgacattattttatgtatttacattttcaaattactgtggcttaaacctgttcagccaacattacccaccttcagtctgctaaataaatgattcagtacatttctaatttacagaattttttaacaaaagaaaatgtaatttgatagccaaatcaacgttaaacattatacatttaaaaaaccacaggcaaagacacaaacatgatgacactaacttttgttaaagtatgcttacctatggtttcctctgaggcacgttctttcatgctaagcttccaacataatatgaaaatgaaggagatgcattttgcaaagcaaaacagaccttaagcaaaatattatacttctcaaattaacactgttacaaagttttagaatttaataagttcattaatttaaaagtttggatgtctgagtccttctatcccaaaacaagatcttggagggtcttccacagccatgtaataccatggtcacatgaccctttccaaaattattaatctgaatttactatatgaggataaatctatctttttgaaaatatttaggaaaatgagcttggtatttataaaatgaagctctctttgggtggtatcctaagacacgtcaagccaatcagcctgtaactgtgaaaaaaacattggtaggtacaaaagtggggtgggagaggagtgacttaactttgttaagtgatgggaaagaaacactaatagcattatctcaataaaatgtgatttaaaaaaatttaaaatactaaatcattgaactgacaaagaaatataaatcattcagaaataaactcattaggtcatcaaatcctgttaaatctgcaattaggaagagcaaggtgtacaatccatacatttaaactcacaggctcactttgcacaacgtcaatttactccttaatatgttattaatacgcattttccaaaaggatgtattagtaaatggtacacatctacttcttggcaacatcatataacctggtacaacataagcattcttcttatagttaagaaatgtggatggtatcaaaattagaaaaataaatgccctattatgttgtggtcaggtttaaggcatgtgaattttatcttcatacaaaagattaaaatctagatattaaaaagtagtgcagtatcagtgatgctgcctcagttcccaaaatgtcacatcacaaaaatatcccataattgcctgtagtttattccttggctttcctcttttctctctgcatctttgtaacaattttttaaaagtggaaatataattgttggcaatgctaacagctgtagaaatgattacaagatgtggaaaagcataacaggaatgtcaagaatctgtttctggcagtaatatatatggaacattgttcaggacaaaagaggagaaggaagaaaaaaaggagaggggtttatcatctctaagaattttcaaactaaacctcattgcttaataggaaaaaaagattccatatttaaagttaagtcacctctaactactagctaaagcatgacatcaccagcactggagtcagcggaagtgtgtttttgaaggacagtgttgcaggagaatctggacaggttttagagccaggagagagaaaataattctacctctgacagttgaaggaccttaggcaaatcagtttacctctgctagactacactccaaaatttggacattcaaaaatttgatattaataaccacatgaaagtctcgtgttgaggtgaatatgtatttgttggtgaaagatatgttggtttttaaacagacagcactctgcaattgtaggctattgttttgttttgccagttgtcaaattctatccagctatacacacttgtgtggcctcctaatggtgtttttccagtggctaaaggtttatgaataagacacttttcctaatggaattaacccgatgcttttcttaaacatgtaaccttgagttcaccgcaaaaaacaatgcttcgattagagcaatgcatataataaaggttaccctcgtttcttagacactagacatcattcacaaaaagagaactgcttttgaaagggatgtatttgcactggaaagaatagttttctacttctaattataaatgatttattggtgaaagcaaaacaacagcctgtctgagaggcacttctatgagcatcctcacgtgtgatttgcaaggttgaagaagagggaaaaatgcctcaattgtaccaatggtgagaaaacacccaaagtacaaagcaggtttcaaaaaaaccatactcataaccaaggacaataataaagcaatgtgttgacatatactctataagtcttcctccataaatagtttatagaaattttgtaatttctgtaaatgcatcctataataattttgcatcttgctttttttttacatttaatatcaagtagatttctaaagggcaattatttgaaaattatcccaaatacatggggaaatatacatcaagtgaaaaaatgcagtgggtgatagagatatcaggaagcgcctcaaatatttctcatctcgttggagaaaaacaaacatgttctcatttagaatgagtgggagttacctaattgatttaggcctctatatttaacttctagtcaaaaaaggtagttctatctagcaacaatattatggggaacaaaagaaaaaattaactctctaaatttgcagtagggtcttttcttcagaagtaccaaatcccatctattaccagctccatgcttcaggcctaaaatggatctccctgaagcaatgacagaatttttgccaagtgactaggatataaacaccactttggttgcacagtgagacatatgctccaaagaaaactggttcaaaaacaggcaagtgggtttctacagaataaatgagagccctgtcaatggcttcatcttcagggctttgtgtctgtgcttgcgtggtggctcttgtttcatctatggataatggtggcacacagttttcataattccttacattaatgaactgctataaatttgtttttggtattctagagagtcctaacttcagcttctgggcaatgctgaggaggcaccctatattctagacttaccttttgcaaggtgtactctcagcattgtgggcgatttccatgggagaatattctatttaaagaactactgtcccagcataaaacaaaaaatcatttatgaagatgcaggagactcggaaagctctcaattattgtttgcacaagcacaatgtcacagcctcctttccccattccacaagggggtcaggaagagagtactcagctgtgagaaaagacatacagaagaattcatgtggtcatgagagcgaggacatggccgatcccccaaggaggatgtgtcatacacttcatgagcccaagagtgtgctgtagggtctgaagggcaagatgctggttcactgatgtaaaggagagggaaaaaagcttcaaccaactagaaaaacagtctctatgcatgctatttttgattttaaacacaggtatcaattccttctctcagagagtccattttaaaataggatacatttttaaaggaatatttaaaggacacattcattaaaatttattttaaaaacttttcaaaagaaacaaaaggtatgaattttatttaatccttgaggaaatggttcttttctcacacacataaatcactcattttgtttttctttatctcctttattaatctacattagaaaaataaacttttcatacactaagaacaaggaaaccactctcaattgacaaaatgttccaatccaacacaatgattactttcacctttaatttacaggcagccagattcaaaatccttaaagttgcttaaacttaaaaatgacaatgacaacctaaaaggtataatgttgattggaacagacatttaattggaaaattgatgattttccatttccaattaaatctctagatagaaatgaaaaaaattaaaaatcgtatttaagaaaagccaaatcttgggttgtgaggtatctttttaaggatgtttcagcagaaaaaaacaaaggctctcacaattgtgtagctgcctagattaagtgggtatcctgatcaaggagatgggggatgatttggctttagtattccaatgataaagtttataatgagaataacatgttgctacaaaatccagtctcttcctcagatgccttccacagagggcaggaagctttgtcagttttgtttgctgatgatgcctggttccgtcaacaaataacacctgtcacacggtgggtagtcaatatacatttgttgaataaatatgaaaaaaagaaatgtacaatatgtttgtgaagccaactgtgtgtgcattgctattgaggtacacaaaaagtctttgttttaaatttgagaatgaggactttcaatggaatatatctataaaaatgaaaaaaagacattactgtctggacttttgtacagcaagagaagaaaaaccactagccaagagccaactcacctgataggcctggatcaagcatgcagctgtggagaacacccctgggactctaactctggcactctgcaagctgggtacttgggcaggacagcagcagcactcatgaactgggcagcacctgttggtgagggctgatcacatggattctctcatcccagccttacaatcagtccttcaggtacatactttttctgactttgctgatgaggaaactatgcacagaggttacacagcttaacaaagggttctcacctaatgaacaatgaaatgggattttagcctttctttgcatctggtcttagagccaatacccaagaagcactgtactgtatgcattgtctcagagaaacttactcttcctgggcctcagtctttaaaaggtgggcagttgacttaataagaattaaagatcaatgattaaggttcaaggcactccaaaattctggtctttattgaaaaggctacagaagtctcaccttaataataccctatagacttgatattcttggttaattaaatattggaaaccaatttcatagtaattgaggtcagaaaaaagtactcatgacattttagaatatgatgacaaagccatagataaatttcaatgcacctgtaattacttaaaactgttatagcatgcaatgtgttaccacaacagccagagaaatactaatttactcagcctattcttctagaccagtaaacactaggattaaatagatattttcattgaatttgttctacccttcattgccatttatagatagcttacttgtcatagattactttctaattgttttatgtttcctaactagcctgcaatactttggcaaggacctcaaacaatagtagacagtaggtgtaaaatagatggctacattgaacagatgactaaaaggatgcctcctaagtacctatatcttgaaatatatattattgtgccttgctttcaatttgtgattttaaaatctagaaatcacctgttttatgtaataacaataaaatccttctttgttgaaaacatgcacaaataaagtttacaagctcaaaaaattaaacagcagtaacggtcaagctttccaacaataaaatacattttggtaaggttttcattttacaaaaactcaaaatagctttatgagttcacaaaataatatgatatttttcaagatattaacatattcttataccggaagagcatagaataaaatttacttggagattgagcatttgcttctttaagaaatacttcttttagtatttttactttaatattatgaaagctacataattacattcagattcattaactactccagtagttaatttttaaaacttatgatgaatagttttgtttaaaatatataacattggtaatatgcaaatctgaatctgtaataaagaaggatttgcattcctgatttttttttctgatacaaccaatgacaaaataactaatggttccacagaggataaaatgtctcaaatctgttggttctgaaggtgaagcgagatttttgtactgataccgtgtatcactgagataccaggaggaaatggaattaaactcagatagttcaaatggagagattttaatgaagggacgacctacagaggtgtcggcagggttggggggaatcagcgagatatgcttagaacccaccgactggcaaacctccccctgaagatggagaaggaggaaggagtgttactggaatgagagcttgagtccaggggaggaggatgggctgctgaggaggcgacaccatcctgaaagaagaatcctctgccagaggcttttcagggtcatttcttcacactctctgcagggaagcacggagacagcaggaagaaatatcctaacctcactctcttccctctacaggtgcttccattggccaaatccacccagaggccagttggtggcgatcagctctcttcaagtggtatttaaatttcttctttcattttccttctggtaacaaagaagtctgtggctcaaaagatgtttctctaagaccccatcctattaggtctctgagctgtgggaagtatttatacaattgcttgtgaatataagatccaggaatttccctaagatccctaacaaaattggtgataagtagtcccacatgttaatccagccacccacggatgacagcacttaccatttctttgataaatgtcaaatgcatttgaagtacctacctgaaatatttgtttaaatgctatctaatctattaattttatatatgtgtgagtctgttttgtataccttctgattataggataaatgtaaataaatccaaagagtaatcaaagctaccactttcaagaagccttctttgtagaaccggaagagtcttaaataggcttttcaggtatgcatctcttattatcgctgaactccaagtcctgcaaggcaggcatcatgtgtgggtcacctttacagtaggcacaggccttaaaacagtgacatgcacattgcaggcactccataaatgtttgctgaattggctaaaccttggtttgttcccataatcaaccaccacaaacagcacacagataattacttcttggaaagattccaactagtgtttgatgttacctacgtggtttttctctcaagatcttaagagcagctctgtaggattacattattttctgttttttttttcctttgaccttaatgtcatctacttcaataacagcttcatacaaaattcctaccagcacataccacagcagattcaaggccttgttttaaaaatggtgccagcttctcttaatttggaagatatattgtctctcctgaacatgggctaagaaaatgtataatttggtattaacataagagctgaagacactttaaatgcattgtttcatttttataagataaaaaaaattttaagaatcaaaatgttatcaacagacttgtccttcattaaaaagtaaaactgcatttgcctacattttatgaaagtgtccaattatgaacaattttgaaatgtaacttttaaaaatgtaaacagcaaaaatgttgtatttaaaataaatctggaaaggcagaaaaacaaaaaatacccagaagacagagtttttggtgaaagttaagatatttcatctttgaacaacttagaatctttcctgcattttatagtctagttccaggcattaatttgaaataaccttggaatcctaaatctaacacccttcggaacaaagtagcttttctcttctgctttatgagcaaatggactaaatactagggaatggtactgtctgggcctttgaaccaagattgaaagagatgaaatcctatatgatatgtataaacattagagaatccattttgatttaataaaaggttgaatttgttctatatcctgtgagaaaatggttcccttttcctgaaaatgttacctcattccaacaatagaaagttggtttttttccagggtgtggtgttggcgggggacagagttgccatgaatatggcatctatgaagactgctgttatattcatttctcaaaatgcactgtggtaggaaattcagaacgcagtgagagaaaataaatgtttgacttcaaaatataaggccgcatttaaagcagaaggtaaagtatagaacagttgacagtataaattctttatctgcaatcttgcagttccctaaatctctgtaacacatcacttttaaaagcctcagataagtggttctataataatttaccaataattcaacccctcaaaagtcttagcaagttaaaccttataatcttacattttagaaatgacccaacttgatccttttattcttcagaatatctctctcaaattttcatttgtttttcattaattgatgaataatgagacattttaggtacctgtccacaaagaaatgaaattttcactttccaggaacctaacaaatgaaaagatagaaatcaattccaacagaatattaccaaagaaatcttttagaatggactgttaaaattatttatttgtatttatctggctctactatttgtggtacatttccacttcaaagctaaacctcaaataacatcatagtgagtggttgacttcatgtttaactgagatcttgaagactgaaaaagaccacgacaaacacacatctattttcttggctactgcatccgtgttcatcaccattctgatagtctgcaatgtattgcagctcaccctttgggaaggactaaagtagacatctgtttgttctgcttactcagcattcctaccctaattttcctttggagaacccctttattctagaccacgtgaagctaatgccaaaccccattccaggggatgcacctgaatccaacctccatcatctaaacagtgccttctccacgttcagagaagagcaagtgactcaaactgccctcataagaacagacctgggacttctgctgcaaatattgaagagtaagtactcttttttcttgctaggactaagctggtagtaccttctatgaggctatcatatggaaacaacttgtctgaaaatgaagccacaactagaaaacagatcctggtaacccggattgatggatccagccctaccttaaatggcaagacctaacccgaggctttttgcatcaaccaataaagtccttaagccagtttgagttggttttgtcacttgcagctaaaagaattctgactctaacaatgtgacaatagcaaaaataaacataactgcttttgaggtttctaatggattttcctccctatatacatgatttcatttaatcctcacaattcaggaaagcacatatctattaacattaaattaatattcattattttgaacacatgctatgtggataagggatgaggaaagccaaggaagtaatcaacgtgaaatctcacttatatgggagggaagtggaggttacatatctcagggcacttaacagatatcatcaaatgaaagaataaacagtgtgtgggagaggcagtaggtgattcttcatcaattcctggatgaaaaattaggagataatgaactccgaacaggcagcctaatgagaatggctcaagcaacaggacatagagagggagttaggttagacatggggttcttgggaattttcacctcgtgggggggcgggggggtcgtgcagctgttgtcagtgggaaagggaaaaaggaaaaggctgagtttggaaggcagggagggaggagacaatgtgagtcagtgaaaaagggcccttagaatgacaagtctggaccagagagaggctaagactgaaaatacaagttgggtaaccactggcatacagatggcagttcaggcttgggcactgcccaccagagcctcagcatgaagagaagagggggaggctggccaccacctccctctaggtaatcgtcatcctgatgctgagctcctgaaaacaggctctttcactcgccccatctcttgctcttgattgcaacccggcattcaggaggcaccctgtaatatctgtggagtgaccgacaacacagcgccagggcactgagaagatcccagggcgccagggactggttctacaagggtgcccctcccggtcccctccagcgcgccgccagagctgccagtcttggctgctacacgggaggcagcctcattatgcagctctcacctcttaaattagttcatgctctcacattaggtgtaatcacagcttgcaacgctttctggggatgtctcagaaagatctgagggccgacgagtgggggcgggcaggagggccgagggaggcggaacaggatcgaggcgcgaggcgggagtcgagaaagcgagcggccgaggcgactctcagtgcgcggacgcgggcgcgcgcccgcgctcccttcgtcgactcacggcgagagcccaaccctgctgccgcgcgccaccc

SEQ ID NO: 17603 - RNA, 15841 nt, Homo sapiens
  source 1..15841: mol_type = other RNA
tcaggccaggcacagtggctcatgcctgtagtcccagcactttgggaggccgaggtgggcagatccacgaggtcaggagatcaagaccatcctaacatggtaaaaccccatctctactaacaatacaaaaaattagtcaggtgtggtggcacgtgcctgtagtcccagctactcaggaggctgaggcaggagaatcgcttgaacctgggaggcggaggttgcagtgagccgagattgtgccactgcaccctagcctaggcaacagagcaagactctgtctcaaaaaaaataaaaaaaaaaaaaagagagaaagagagagagagatgaggagttgctgcactgctgggtgtggagagccgaggaggattcaaagatggtcctgaagtcccagctggaagaagtaggcggcagcaatgtttttaatactgtaaattcatcacgtagcacaggtttggggtggagaaagaaaaattgcattggcttcagggcatgcccagatctttcctcatcttaggcgtttgctaatacatgcattttctaagctgatgtcttgcgtttaatcactgctccattcaaaagagagaaggaggttgtttcaaacctagttgatatcatttgacttccatgctattcacagggctattttatttgaaacaggtataccacagccttaaattgcaagttaatccaggatgttcctaggttggcagttaggaacatgtaattctttggaagggctaaaagtcagctctttaaattatctccatatgaaccttctctccaccttagggtggatccacttatttagtccactgccagtaccacactagaacccgggtggtcactggactccagaaacaacagtagccctctctctgttctgtctctttttgactatctctattctgttcctgaccctgatttctcctgccaagctcaattttgacagctgacaacggcaagccatggcttcccaaaacattattttcaggtcaacttataaatttcaagaacacatttggctccgcttcctgtggtactaagcctacttcttgacagcatttgcctttgttgtaaatagcaaagttcttctagttggatttttgctaagaagtgtgtggatgtggcatgtgacgacatctttagcttggattctagaaaggcactaccattgtgcatttggctaaaggaaacacattttacccgtgaatgccttctatttacaaatgctcagctagcacacaaagctaagtacaagcaataagtactatcctacaatgttactcatttctgaaagcacaaaatgatgactggtatagctttggagatgttttctggaaacccaataaaggaacagatctttgttattccacacctacaaagtcagaagatgcacagtcttttattcatgtttgaacaagcttccttcttgaacaatcaactataaagtgatgtgattctctactagaccaggaactccttgaggacagaatgagggtctaatccatattctaaatccacaccacctggcacaatacatgttgcatggttagggtcaactaagagttggttgaattaatcaataacacacagcaagagaattcacaaagagaggggagtaatcccccagcctcaatcactcggcaagtggaatcgctgggcactgattccagctctgtctcagtgcttgagacagagctgaatgtaatgtgaacatttcaaatgaacaggaaaactagactcacggataagcagtgtagtcatcaagacaacactgtcttggaggtttttctgaagttaaaaccatgctacataagcaataaattatgaaggctgagcatgtgaataaaatttaatgttgtcataaattttataacaaagttaatctgacacatttaatgacatgcataatcattagtatgcagcactgtaatcagacattgataataagcagttcacaccagtgactgtaagagtctttacttgtgttcagccaagccaactgcttggtatatttttctcccttcttagtcgttagttttccatacctacaataactatcagtggtgatgggcttctctgaccatgtgaataatttaatcctcaatgcacagatacagaaacccttgctgaagacagtgtggagcagagaaggctgtctccactccttccacctgaaacacctctgcagatggatatgggagctctgcctacagcccttggacctaaccacttcagtgtgttccagtgagtgtctggacctcggcctgaaagatttttccgaaactaaagaaaatttctctgacctaaagaccttaacctccaccccagaagctctcaccaaggactacagggaactggtggggaaaatccttatcccttactcctcaaggcacagggcagtaatgctgaggcttgtgcgccacacttgctcccagaggtccccagcgggctacctgcggtggtgaatgacctcctaacacgccccttgacggccttcctttccttgcctcacttctccactctcctaccagcattgcagggttcacatcccaaatataccactggcacttgaatcctggtctccaggtctgtttctggaaaaacccaagtaagacattgccccagtaatggggctagatgtctgaggcttcctcaagtatctacctcgaaagctcttactgctgtacacacatgcacatacacacacgtgcgtacaaccagtcacatctaagcaccccgaataccagcctgttgaaggtagcagagagctgcactataagccaaggctgctcccaagagccgctccatcactgaattggcgccccagcaagatgaaggaatgtaatcattggaaggatggagaatgttctctgaatcactgacaaattggaaggggtggagggcaagagtccacctggtggagagatggaaagagcgagagagcctggaatgataatgccattgcttagaaaaggctgctccagatgccatatctacagaaattgtacagcccaaacatctctgagcaataggtctctggtagtcttgatgtctagaccaacaattcccagttcattcttctcagggaaggagccaggatagtccagagactctcattctgctgttagattgaaagggttaggcacaacagccttggcaaagtcacaagggcaaattcacactaaagtgtaaatgacccacaactcctcttctatttttaggttggggaggtgctttagaacataaggaggaactaaagaatattcctgttacatacaaggcagagaaaagggaaactagtggtgacaagacaaatcatccctttgacatttggctggctctacctattacagctctgggggtgaggtgggaacaaaaagatgctgtgtaaagaagtatcttatgccatccctactgtagtgaggtgcagtttagaggggacactgatcaagcagagacccagagtgtttcgttccaagccagaaacagaaatgtataaaacacagcctttccagcatcagaaatgagtagtggtagtggagaactacccaaaacaggaaagaggaccacgtgaggtagagtgtcaaggccctacattccagtgcctctgctcatgactgtaattttgggtaggtcacttaaagtctctggacctcagttttgccatctgtgaaatagggataatactatccagcataaaattggttatgaggctcatgtagggcctgcctgggatgatgtgttgctaatggttaagaacacaacttctggggtctgactggacaggctgaaatccctgcttaacacgttccagcagagccctgggcgatctatttaacttttgttttctcacctgtaagctgagacgaaagtacccactttataagattattccaataattagttgaaataatgcatgcagagaattaagcatggtacttgttatttgttaaactagctattaaaatgtgtaaaatataaagtattgtatggattttaggacaatgcaaagactctttgcttgctgcaatagttcggggccctttcagatggctaaaggcagaatttgtatgtgtaaatatggtgtgcttgtctctgctctggatactgagggcttaccctgttattaaacttatttagtaaatattgaactgtcatgaggcctaacatttagttccagttattagataaaacatttgctttgaatggtatttgaattgccaggttctagattattctggttgacaaactcttcgtattttataaagaggctaaaattggtaagctatcacagaacagatgtgccattttcaaggtatattaaaccatgattcactgtaacattgttcctactggcaacaaattcagagcaggctggactttatttggtgaagaaacattgagtggaagagaaatgacattattttatgtatttacattttcaaattactgtggcttaaacctgttcagccaacattacccaccttcagtctgctaaataaatgattcagtacatttctaatttacagaattttttaacaaaagaaaatgtaatttgatagccaaatcaacgttaaacattatacatttaaaaaaccacaggcaaagacacaaacatgatgacactaacttttgttaaagtatgcttacctatggtttcctctgaggcacgttctttcatgctaagcttccaacataatatgaaaatgaaggagatgcattttgcaaagcaaaacagaccttaagcaaaatattatacttctcaaattaacactgttacaaagttttagaatttaataagttcattaatttaaaagtttggatgtctgagtccttctatcccaaaacaagatcttggagggtcttccacagccatgtaataccatggtcacatgaccctttccaaaattattaatctgaatttactatatgaggataaatctatctttttgaaaatatttaggaaaatgagcttggtatttataaaatgaagctctctttgggtggtatcctaagacacgtcaagccaatcagcctgtaactgtgaaaaaaacattggtaggtacaaaagtggggtgggagaggagtgacttaactttgttaagtgatgggaaagaaacactaatagcattatctcaataaaatgtgatttaaaaaaatttaaaatactaaatcattgaactgacaaagaaatataaatcattcagaaataaactcattaggtcatcaaatcctgttaaatctgcaattaggaagagcaaggtgtacaatccatacatttaaactcacaggctcactttgcacaacgtcaatttactccttaatatgttattaatacgcattttccaaaaggatgtattagtaaatggtacacatctacttcttggcaacatcatataacctggtacaacataagcattcttcttatagttaagaaatgtggatggtatcaaaattagaaaaataaatgccctattatgttgtggtcaggtttaaggcatgtgaattttatcttcatacaaaagattaaaatctagatattaaaaagtagtgcagtatcagtgatgctgcctcagttcccaaaatgtcacatcacaaaaatatcccataattgcctgtagtttattccttggctttcctcttttctctctgcatctttgtaacaattttttaaaagtggaaatataattgttggcaatgctaacagctgtagaaatgattacaagatgtggaaaagcataacaggaatgtcaagaatctgtttctggcagtaatatatatggaacattgttcaggacaaaagaggagaaggaagaaaaaaaggagaggggtttatcatctctaagaattttcaaactaaacctcattgcttaataggaaaaaaagattccatatttaaagttaagtcacctctaactactagctaaagcatgacatcaccagcactggagtcagcggaagtgtgtttttgaaggacagtgttgcaggagaatctggacaggttttagagccaggagagagaaaataattctacctctgacagttgaaggaccttaggcaaatcagtttacctctgctagactacactccaaaatttggacattcaaaaatttgatattaataaccacatgaaagtctcgtgttgaggtgaatatgtatttgttggtgaaagatatgttggtttttaaacagacagcactctgcaattgtaggctattgttttgttttgccagttgtcaaattctatccagctatacacacttgtgtggcctcctaatggtgtttttccagtggctaaaggtttatgaataagacacttttcctaatggaattaacccgatgcttttcttaaacatgtaaccttgagttcaccgcaaaaaacaatgcttcgattagagcaatgcatataataaaggttaccctcgtttcttagacactagacatcattcacaaaaagagaactgcttttgaaagggatgtatttgcactggaaagaatagttttctacttctaattataaatgatttattggtgaaagcaaaacaacagcctgtctgagaggcacttctatgagcatcctcacgtgtgatttgcaaggttgaagaagagggaaaaatgcctcaattgtaccaatggtgagaaaacacccaaagtacaaagcaggtttcaaaaaaaccatactcataaccaaggacaataataaagcaatgtgttgacatatactctataagtcttcctccataaatagtttatagaaattttgtaatttctgtaaatgcatcctataataattttgcatcttgctttttttttacatttaatatcaagtagatttctaaagggcaattatttgaaaattatcccaaatacatggggaaatatacatcaagtgaaaaaatgcagtgggtgatagagatatcaggaagcgcctcaaatatttctcatctcgttggagaaaaacaaacatgttctcatttagaatgagtgggagttacctaattgatttaggcctctatatttaacttctagtcaaaaaaggtagttctatctagcaacaatattatggggaacaaaagaaaaaattaactctctaaatttgcagtagggtcttttcttcagaagtaccaaatcccatctattaccagctccatgcttcaggcctaaaatggatctccctgaagcaatgacagaatttttgccaagtgactaggatataaacaccactttggttgcacagtgagacatatgctccaaagaaaactggttcaaaaacaggcaagtgggtttctacagaataaatgagagccctgtcaatggcttcatcttcagggctttgtgtctgtgcttgcgtggtggctcttgtttcatctatggataatggtggcacacagttttcataattccttacattaatgaactgctataaatttgtttttggtattctagagagtcctaacttcagcttctgggcaatgctgaggaggcaccctatattctagacttaccttttgcaaggtgtactctcagcattgtgggcgatttccatgggagaatattctatttaaagaactactgtcccagcataaaacaaaaaatcatttatgaagatgcaggagactcggaaagctctcaattattgtttgcacaagcacaatgtcacagcctcctttccccattccacaagggggtcaggaagagagtactcagctgtgagaaaagacatacagaagaattcatgtggtcatgagagcgaggacatggccgatcccccaaggaggatgtgtcatacacttcatgagcccaagagtgtgctgtagggtctgaagggcaagatgctggttcactgatgtaaaggagagggaaaaaagcttcaaccaactagaaaaacagtctctatgcatgctatttttgattttaaacacaggtatcaattccttctctcagagagtccattttaaaataggatacatttttaaaggaatatttaaaggacacattcattaaaatttattttaaaaacttttcaaaagaaacaaaaggtatgaattttatttaatccttgaggaaatggttcttttctcacacacataaatcactcattttgtttttctttatctcctttattaatctacattagaaaaataaacttttcatacactaagaacaaggaaaccactctcaattgacaaaatgttccaatccaacacaatgattactttcacctttaatttacaggcagccagattcaaaatccttaaagttgcttaaacttaaaaatgacaatgacaacctaaaaggtataatgttgattggaacagacatttaattggaaaattgatgattttccatttccaattaaatctctagatagaaatgaaaaaaattaaaaatcgtatttaagaaaagccaaatcttgggttgtgaggtatctttttaaggatgtttcagcagaaaaaaacaaaggctctcacaattgtgtagctgcctagattaagtgggtatcctgatcaaggagatgggggatgatttggctttagtattccaatgataaagtttataatgagaataacatgttgctacaaaatccagtctcttcctcagatgccttccacagagggcaggaagctttgtcagttttgtttgctgatgatgcctggttccgtcaacaaataacacctgtcacacggtgggtagtcaatatacatttgttgaataaatatgaaaaaaagaaatgtacaatatgtttgtgaagccaactgtgtgtgcattgctattgaggtacacaaaaagtctttgttttaaatttgagaatgaggactttcaatggaatatatctataaaaatgaaaaaaagacattactgtctggacttttgtacagcaagagaagaaaaaccactagccaagagccaactcacctgataggcctggatcaagcatgcagctgtggagaacacccctgggactctaactctggcactctgcaagctgggtacttgggcaggacagcagcagcactcatgaactgggcagcacctgttggtgagggctgatcacatggattctctcatcccagccttacaatcagtccttcaggtacatactttttctgactttgctgatgaggaaactatgcacagaggttacacagcttaacaaagggttctcacctaatgaacaatgaaatgggattttagcctttctttgcatctggtcttagagccaatacccaagaagcactgtactgtatgcattgtctcagagaaacttactcttcctgggcctcagtctttaaaaggtgggcagttgacttaataagaattaaagatcaatgattaaggttcaaggcactccaaaattctggtctttattgaaaaggctacagaagtctcaccttaataataccctatagacttgatattcttggttaattaaatattggaaaccaatttcatagtaattgaggtcagaaaaaagtactcatgacattttagaatatgatgacaaagccatagataaatttcaatgcacctgtaattacttaaaactgttatagcatgcaatgtgttaccacaacagccagagaaatactaatttactcagcctattcttctagaccagtaaacactaggattaaatagatattttcattgaatttgttctacccttcattgccatttatagatagcttacttgtcatagattactttctaattgttttatgtttcctaactagcctgcaatactttggcaaggacctcaaacaatagtagacagtaggtgtaaaatagatggctacattgaacagatgactaaaaggatgcctcctaagtacctatatcttgaaatatatattattgtgccttgctttcaatttgtgattttaaaatctagaaatcacctgttttatgtaataacaataaaatccttctttgttgaaaacatgcacaaataaagtttacaagctcaaaaaattaaacagcagtaacggtcaagctttccaacaataaaatacattttggtaaggttttcattttacaaaaactcaaaatagctttatgagttcacaaaataatatgatatttttcaagatattaacatattcttataccggaagagcatagaataaaatttacttggagattgagcatttgcttctttaagaaatacttcttttagtatttttactttaatattatgaaagctacataattacattcagattcattaactactccagtagttaatttttaaaacttatgatgaatagttttgtttaaaatatataacattggtaatatgcaaatctgaatctgtaataaagaaggatttgcattcctgatttttttttctgatacaaccaatgacaaaataactaatggttccacagaggataaaatgtctcaaatctgttggttctgaaggtgaagcgagatttttgtactgataccgtgtatcactgagataccaggaggaaatggaattaaactcagatagttcaaatggagagattttaatgaagggacgacctacagaggtgtcggcagggttggggggaatcagcgagatatgcttagaacccaccgactggcaaacctccccctgaagatggagaaggaggaaggagtgttactggaatgagagcttgagtccaggggaggaggatgggctgctgaggaggcgacaccatcctgaaagaagaatcctctgccagaggcttttcagggtcatttcttcacactctctgcagggaagcacggagacagcaggaagaaatatcctaacctcactctcttccctctacaggtgcttccattggccaaatccacccagaggccagttggtggcgatcagctctcttcaagtggtatttaaatttcttctttcattttccttctggtaacaaagaagtctgtggctcaaaagatgtttctctaagaccccatcctattaggtctctgagctgtgggaagtatttatacaattgcttgtgaatataagatccaggaatttccctaagatccctaacaaaattggtgataagtagtcccacatgttaatccagccacccacggatgacagcacttaccatttctttgataaatgtcaaatgcatttgaagtacctacctgaaatatttgtttaaatgctatctaatctattaattttatatatgtgtgagtctgttttgtataccttctgattataggataaatgtaaataaatccaaagagtaatcaaagctaccactttcaagaagccttctttgtagaaccggaagagtcttaaataggcttttcaggtatgcatctcttattatcgctgaactccaagtcctgcaaggcaggcatcatgtgtgggtcacctttacagtaggcacaggccttaaaacagtgacatgcacattgcaggcactccataaatgtttgctgaattggctaaaccttggtttgttcccataatcaaccaccacaaacagcacacagataattacttcttggaaagattccaactagtgtttgatgttacctacgtggtttttctctcaagatcttaagagcagctctgtaggattacattattttctgttttttttttcctttgaccttaatgtcatctacttcaataacagcttcatacaaaattcctaccagcacataccacagcagattcaaggccttgttttaaaaatggtgccagcttctcttaatttggaagatatattgtctctcctgaacatgggctaagaaaatgtataatttggtattaacataagagctgaagacactttaaatgcattgtttcatttttataagataaaaaaaattttaagaatcaaaatgttatcaacagacttgtccttcattaaaaagtaaaactgcatttgcctacattttatgaaagtgtccaattatgaacaattttgaaatgtaacttttaaaaatgtaaacagcaaaaatgttgtatttaaaataaatctggaaaggcagaaaaacaaaaaatacccagaagacagagtttttggtgaaagttaagatatttcatctttgaacaacttagaatctttcctgcattttatagtctagttccaggcattaatttgaaataaccttggaatcctaaatctaacacccttcggaacaaagtagcttttctcttctgctttatgagcaaatggactaaatactagggaatggtactgtctgggcctttgaaccaagattgaaagagatgaaatcctatatgatatgtataaacattagagaatccattttgatttaataaaaggttgaatttgttctatatcctgtgagaaaatggttcccttttcctgaaaatgttacctcattccaacaatagaaagttggtttttttccagggtgtggtgttggcgggggacagagttgccatgaatatggcatctatgaagactgctgttatattcatttctcaaaatgcactgtggtaggaaattcagaacgcagtgagagaaaataaatgtttgacttcaaaatataaggccgcatttaaagcagaaggtaaagtatagaacagttgacagtataaattctttatctgcaatcttgcagttccctaaatctctgtaacacatcacttttaaaagcctcagataagtggttctataataatttaccaataattcaacccctcaaaagtcttagcaagttaaaccttataatcttacattttagaaatgacccaacttgatccttttattcttcagaatatctctctcaaattttcatttgtttttcattaattgatgaataatgagacattttaggtacctgtccacaaagaaatgaaattttcactttccaggaacctaacaaatgaaaagatagaaatcaattccaacagaatattaccaaagaaatcttttagaatggactgttaaaattatttatttgtatttatctggctctactatttgtggtacatttccacttcaaagctaaacctcaaataacatcatagtgagtggttgacttcatgtttaactgagatcttgaagactgaaaaagaccacgacaaacacacatctattttcttggctactgcatccgtgttcatcaccattctgatagtctgcaatgtattgcagctcaccctttgggaaggactaaagtagacatctgtttgttctgcttactcagcattcctaccctaattttcctttggagaacccctttattctagaccacgtgaagctaatgccaaaccccattccaggggatgcacctgaatccaacctccatcatctaaacagtgccttctccacgttcagagaagagcaagtgactcaaactgccctcataagaacagacctgggacttctgctgcaaatattgaagagtaagtactcttttttcttgctaggactaagctggtagtaccttctatgaggctatcatatggaaacaacttgtctgaaaatgaagccacaactagaaaacagatcctggtaacccggattgatggatccagccctaccttaaatggcaagacctaacccgaggctttttgcatcaaccaataaagtccttaagccagtttgagttggttttgtcacttgcagctaaaagaattctgactctaacaatgtgacaatagcaaaaataaacataactgcttttgaggtttctaatggattttcctccctatatacatgatttcatttaatcctcacaattcaggaaagcacatatctattaacattaaattaatattcattattttgaacacatgctatgtggataagggatgaggaaagccaaggaagtaatcaacgtgaaatctcacttatatgggagggaagtggaggttacatatctcagggcacttaacagatatcatcaaatgaaagaataaacagtgtgtgggagaggcagtaggtgattcttcatcaattcctggatgaaaaattaggagataatgaactccgaacaggcagcctaatgagaatggctcaagcaacaggacatagagagggagttaggttagacatggggttcttgggaattttcacctcgtgggggggcgggggggtcgtgcagctgttgtcagtgggaaagggaaaaaggaaaaggctgagtttggaaggcagggagggaggagacaatgtgagtcagtgaaaaagggcccttagaatgacaagtctggaccagagagaggctaagactgaaaatacaagttgggtaaccactggcatacagatggcagttcaggcttgggcactgcccaccagagcctcagcatgaagagaagagggggaggctggccaccacctccctctaggtaatcgtcatcctgatgctgagctcctgaaaacaggctctttcactcgccccatctcttgctcttgattgcaacccggcattcaggaggcaccctgtaatatctgtggagtgaccgacaacacagcgccagggcactgagaagatcccagggcgccagggactggttctacaagggtgcccctcccggtcccctccagcgcgccgccagagctgccagtcttggctgctacacgggaggcagcctcattatgcagctctcacctcttaaattagttcatgctctcacattaggtgtaatcacagcttgcaacgctttctggggatgtctcagaaagatctgagttgaaaaaatatttttgtgtcattttaatttaaagtaaaattgctgcttcttccccgcccctttctttcctcctggcccacccagcgaccctggccggccgtgctcaacgggggcgggggtcggaggtgagatttcctccacataattccttaaacagctatcaactaagtctcaaagaaaaaaaaaagagatctagaagcagagacgtggctgctggcgatcccaaagctggtgttcgctcttgggggagagcgtaccctgggggaggccgggaggccgggccagaggctagcccagaggcagagggcaggagcgctcagccggcgccccgcgtctctccagctcccgacgctgcgctggctccgctgagcacgccaggatcaaggtcgcctggtggggaccggagcgccaggagcctgtgggaagcgttccagccggcctctgactgggatccggcgccgcgtttctgctttggacttgactgacaggtccccccgccctcccgccgccctactaccagcctgggttcatccttcagggctacgtctaccgcacccgggctggaaagcctggagcgcgcccttcctctcctcatcttctcagctctcctttctccctgccacttggcaaagctgcattttgactttcacgttttggactacgtgtgtgtagttccaagtccatgcgtggcacgaaaatccacttagggtaaaaattattctcgaaaaatcgcccatctcaggatctggtgtctacactcaaggctaggaggtgcaggtacgggtgcgtaaagcatgccgtaagggtgcacagtaaataaaaagtacggatgcaaaatgtaaattttaagtgcaaaacagaaaagcagtactcgttgccgccccgcacgctgggttttaaggggcacgaaggtgggcctcggctgcttttgctcagccccgcgtcctcagcgcccggcccagtacccggtactccgtaggggttcaatgatctcccctgaataagtgaacgaattaacaaatgaatgaatgaccgctcgatccgacctccgcggccggcagagcagtcgctggagaggcgggagagagcgagaggccaagctccaccatcgcggccgccggctggggcagagggacacggagacactcggcgccccggctccgcaccgagtccccg

SEQ ID NO: 17604 - RNA, 13030 nt, Homo sapiens
  source 1..13030: mol_type = other RNA
tcaggccaggcacagtggctcatgcctgtagtcccagcactttgggaggccgaggtgggcagatccacgaggtcaggagatcaagaccatcctaacatggtaaaaccccatctctactaacaatacaaaaaattagtcaggtgtggtggcacgtgcctgtagtcccagctactcaggaggctgaggcaggagaatcgcttgaacctgggaggcggaggttgcagtgagccgagattgtgccactgcaccctagcctaggcaacagagcaagactctgtctcaaaaaaaataaaaaaaaaaaaaagagagaaagagagagagagatgaggagttgctgcactgctgggtgtggagagccgaggaggattcaaagatggtcctgaagtcccagctggaagaagtaggcggcagcaatgtttttaatactgtaaattcatcacgtagcacaggtttggggtggagaaagaaaaattgcattggcttcagggcatgcccagatctttcctcatcttaggcgtttgctaatacatgcattttctaagctgatgtcttgcgtttaatcactgctccattcaaaagagagaaggaggttgtttcaaacctagttgatatcatttgacttccatgctattcacagggctattttatttgaaacaggtataccacagccttaaattgcaagttaatccaggatgttcctaggttggcagttaggaacatgtaattctttggaagggctaaaagtcagctctttaaattatctccatatgaaccttctctccaccttagggtggatccacttatttagtccactgccagtaccacactagaacccgggtggtcactggactccagaaacaacagtagccctctctctgttctgtctctttttgactatctctattctgttcctgaccctgatttctcctgccaagctcaattttgacagctgacaacggcaagccatggcttcccaaaacattattttcaggtcaacttataaatttcaagaacacatttggctccgcttcctgtggtactaagcctacttcttgacagcatttgcctttgttgtaaatagcaaagttcttctagttggatttttgctaagaagtgtgtggatgtggcatgtgacgacatctttagcttggattctagaaaggcactaccattgtgcatttggctaaaggaaacacattttacccgtgaatgccttctatttacaaatgctcagctagcacacaaagctaagtacaagcaataagtactatcctacaatgttactcatttctgaaagcacaaaatgatgactggtatagctttggagatgttttctggaaacccaataaaggaacagatctttgttattccacacctacaaagtcagaagatgcacagtcttttattcatgtttgaacaagcttccttcttgaacaatcaactataaagtgatgtgattctctactagaccaggaactccttgaggacagaatgagggtctaatccatattctaaatccacaccacctggcacaatacatgttgcatggttagggtcaactaagagttggttgaattaatcaataacacacagcaagagaattcacaaagagaggggagtaatcccccagcctcaatcactcggcaagtggaatcgctgggcactgattccagctctgtctcagtgcttgagacagagctgaatgtaatgtgaacatttcaaatgaacaggaaaactagactcacggataagcagtgtagtcatcaagacaacactgtcttggaggtttttctgaagttaaaaccatgctacataagcaataaattatgaaggctgagcatgtgaataaaatttaatgttgtcataaattttataacaaagttaatctgacacatttaatgacatgcataatcattagtatgcagcactgtaatcagacattgataataagcagttcacaccagtgactgtaagagtctttacttgtgttcagccaagccaactgcttggtatatttttctcccttcttagtcgttagttttccatacctacaataactatcagtggtgatgggcttctctgaccatgtgaataatttaatcctcaatgcacagatacagaaacccttgctgaagacagtgtggagcagagaaggctgtctccactccttccacctgaaacacctctgcagatggatatgggagctctgcctacagcccttggacctaaccacttcagtgtgttccagtgagtgtctggacctcggcctgaaagatttttccgaaactaaagaaaatttctctgacctaaagaccttaacctccaccccagaagctctcaccaaggactacagggaactggtggggaaaatccttatcccttactcctcaaggcacagggcagtaatgctgaggcttgtgcgccacacttgctcccagaggtccccagcgggctacctgcggtggtgaatgacctcctaacacgccccttgacggccttcctttccttgcctcacttctccactctcctaccagcattgcagggttcacatcccaaatataccactggcacttgaatcctggtctccaggtctgtttctggaaaaacccaagtaagacattgccccagtaatggggctagatgtctgaggcttcctcaagtatctacctcgaaagctcttactgctgtacacacatgcacatacacacacgtgcgtacaaccagtcacatctaagcaccccgaataccagcctgttgaaggtagcagagagctgcactataagccaaggctgctcccaagagccgctccatcactgaattggcgccccagcaagatgaaggaatgtaatcattggaaggatggagaatgttctctgaatcactgacaaattggaaggggtggagggcaagagtccacctggtggagagatggaaagagcgagagagcctggaatgataatgccattgcttagaaaaggctgctccagatgccatatctacagaaattgtacagcccaaacatctctgagcaataggtctctggtagtcttgatgtctagaccaacaattcccagttcattcttctcagggaaggagccaggatagtccagagactctcattctgctgttagattgaaagggttaggcacaacagccttggcaaagtcacaagggcaaattcacactaaagtgtaaatgacccacaactcctcttctatttttaggttggggaggtgctttagaacataaggaggaactaaagaatattcctgttacatacaaggcagagaaaagggaaactagtggtgacaagacaaatcatccctttgacatttggctggctctacctattacagctctgggggtgaggtgggaacaaaaagatgctgtgtaaagaagtatcttatgccatccctactgtagtgaggtgcagtttagaggggacactgatcaagcagagacccagagtgtttcgttccaagccagaaacagaaatgtataaaacacagcctttccagcatcagaaatgagtagtggtagtggagaactacccaaaacaggaaagaggaccacgtgaggtagagtgtcaaggccctacattccagtgcctctgctcatgactgtaattttgggtaggtcacttaaagtctctggacctcagttttgccatctgtgaaatagggataatactatccagcataaaattggttatgaggctcatgtagggcctgcctgggatgatgtgttgctaatggttaagaacacaacttctggggtctgactggacaggctgaaatccctgcttaacacgttccagcagagccctgggcgatctatttaacttttgttttctcacctgtaagctgagacgaaagtacccactttataagattattccaataattagttgaaataatgcatgcagagaattaagcatggtacttgttatttgttaaactagctattaaaatgtgtaaaatataaagtattgtatggattttaggacaatgcaaagactctttgcttgctgcaatagttcggggccctttcagatggctaaaggcagaatttgtatgtgtaaatatggtgtgcttgtctctgctctggatactgagggcttaccctgttattaaacttatttagtaaatattgaactgtcatgaggcctaacatttagttccagttattagataaaacatttgctttgaatggtatttgaattgccaggttctagattattctggttgacaaactcttcgtattttataaagaggctaaaattggtaagctatcacagaacagatgtgccattttcaaggtatattaaaccatgattcactgtaacattgttcctactggcaacaaattcagagcaggctggactttatttggtgaagaaacattgagtggaagagaaatgacattattttatgtatttacattttcaaattactgtggcttaaacctgttcagccaacattacccaccttcagtctgctaaataaatgattcagtacatttctaatttacagaattttttaacaaaagaaaatgtaatttgatagccaaatcaacgttaaacattatacatttaaaaaaccacaggcaaagacacaaacatgatgacactaacttttgttaaagtatgcttacctatggtttcctctgaggcacgttctttcatgctaagcttccaacataatatgaaaatgaaggagatgcattttgcaaagcaaaacagaccttaagcaaaatattatacttctcaaattaacactgttacaaagttttagaatttaataagttcattaatttaaaagtttggatgtctgagtccttctatcccaaaacaagatcttggagggtcttccacagccatgtaataccatggtcacatgaccctttccaaaattattaatctgaatttactatatgaggataaatctatctttttgaaaatatttaggaaaatgagcttggtatttataaaatgaagctctctttgggtggtatcctaagacacgtcaagccaatcagcctgtaactgtgaaaaaaacattggtaggtacaaaagtggggtgggagaggagtgacttaactttgttaagtgatgggaaagaaacactaatagcattatctcaataaaatgtgatttaaaaaaatttaaaatactaaatcattgaactgacaaagaaatataaatcattcagaaataaactcattaggtcatcaaatcctgttaaatctgcaattaggaagagcaaggtgtacaatccatacatttaaactcacaggctcactttgcacaacgtcaatttactccttaatatgttattaatacgcattttccaaaaggatgtattagtaaatggtacacatctacttcttggcaacatcatataacctggtacaacataagcattcttcttatagttaagaaatgtggatggtatcaaaattagaaaaataaatgccctattatgttgtggtcaggtttaaggcatgtgaattttatcttcatacaaaagattaaaatctagatattaaaaagtagtgcagtatcagtgatgctgcctcagttcccaaaatgtcacatcacaaaaatatcccataattgcctgtagtttattccttggctttcctcttttctctctgcatctttgtaacaattttttaaaagtggaaatataattgttggcaatgctaacagctgtagaaatgattacaagatgtggaaaagcataacaggaatgtcaagaatctgtttctggcagtaatatatatggaacattgttcaggacaaaagaggagaaggaagaaaaaaaggagaggggtttatcatctctaagaattttcaaactaaacctcattgcttaataggaaaaaaagattccatatttaaagttaagtcacctctaactactagctaaagcatgacatcaccagcactggagtcagcggaagtgtgtttttgaaggacagtgttgcaggagaatctggacaggttttagagccaggagagagaaaataattctacctctgacagttgaaggaccttaggcaaatcagtttacctctgctagactacactccaaaatttggacattcaaaaatttgatattaataaccacatgaaagtctcgtgttgaggtgaatatgtatttgttggtgaaagatatgttggtttttaaacagacagcactctgcaattgtaggctattgttttgttttgccagttgtcaaattctatccagctatacacacttgtgtggcctcctaatggtgtttttccagtggctaaaggtttatgaataagacacttttcctaatggaattaacccgatgcttttcttaaacatgtaaccttgagttcaccgcaaaaaacaatgcttcgattagagcaatgcatataataaaggttaccctcgtttcttagacactagacatcattcacaaaaagagaactgcttttgaaagggatgtatttgcactggaaagaatagttttctacttctaattataaatgatttattggtgaaagcaaaacaacagcctgtctgagaggcacttctatgagcatcctcacgtgtgatttgcaaggttgaagaagagggaaaaatgcctcaattgtaccaatggtgagaaaacacccaaagtacaaagcaggtttcaaaaaaaccatactcataaccaaggacaataataaagcaatgtgttgacatatactctataagtcttcctccataaatagtttatagaaattttgtaatttctgtaaatgcatcctataataattttgcatcttgctttttttttacatttaatatcaagtagatttctaaagggcaattatttgaaaattatcccaaatacatggggaaatatacatcaagtgaaaaaatgcagtgggtgatagagatatcaggaagcgcctcaaatatttctcatctcgttggagaaaaacaaacatgttctcatttagaatgagtgggagttacctaattgatttaggcctctatatttaacttctagtcaaaaaaggtagttctatctagcaacaatattatggggaacaaaagaaaaaattaactctctaaatttgcagtagggtcttttcttcagaagtaccaaatcccatctattaccagctccatgcttcaggcctaaaatggatctccctgaagcaatgacagaatttttgccaagtgactaggatataaacaccactttggttgcacagtgagacatatgctccaaagaaaactggttcaaaaacaggcaagtgggtttctacagaataaatgagagccctgtcaatggcttcatcttcagggctttgtgtctgtgcttgcgtggtggctcttgtttcatctatggataatggtggcacacagttttcataattccttacattaatgaactgctataaatttgtttttggtattctagagagtcctaacttcagcttctgggcaatgctgaggaggcaccctatattctagacttaccttttgcaaggtgtactctcagcattgtgggcgatttccatgggagaatattctatttaaagaactactgtcccagcataaaacaaaaaatcatttatgaagatgcaggagactcggaaagctctcaattattgtttgcacaagcacaatgtcacagcctcctttccccattccacaagggggtcaggaagagagtactcagctgtgagaaaagacatacagaagaattcatgtggtcatgagagcgaggacatggccgatcccccaaggaggatgtgtcatacacttcatgagcccaagagtgtgctgtagggtctgaagggcaagatgctggttcactgatgtaaaggagagggaaaaaagcttcaaccaactagaaaaacagtctctatgcatgctatttttgattttaaacacaggtatcaattccttctctcagagagtccattttaaaataggatacatttttaaaggaatatttaaaggacacattcattaaaatttattttaaaaacttttcaaaagaaacaaaaggtatgaattttatttaatccttgaggaaatggttcttttctcacacacataaatcactcattttgtttttctttatctcctttattaatctacattagaaaaataaacttttcatacactaagaacaaggaaaccactctcaattgacaaaatgttccaatccaacacaatgattactttcacctttaatttacaggcagccagattcaaaatccttaaagttgcttaaacttaaaaatgacaatgacaacctaaaaggtataatgttgattggaacagacatttaattggaaaattgatgattttccatttccaattaaatctctagatagaaatgaaaaaaattaaaaatcgtatttaagaaaagccaaatcttgggttgtgaggtatctttttaaggatgtttcagcagaaaaaaacaaaggctctcacaattgtgtagctgcctagattaagtgggtatcctgatcaaggagatgggggatgatttggctttagtattccaatgataaagtttataatgagaataacatgttgctacaaaatccagtctcttcctcagatgccttccacagagggcaggaagctttgtcagttttgtttgctgatgatgcctggttccgtcaacaaataacacctgtcacacggtgggtagtcaatatacatttgttgaataaatatgaaaaaaagaaatgtacaatatgtttgtgaagccaactgtgtgtgcattgctattgaggtacacaaaaagtctttgttttaaatttgagaatgaggactttcaatggaatatatctataaaaatgaaaaaaagacattactgtctggacttttgtacagcaagagaagaaaaaccactagccaagagccaactcacctgataggcctggatcaagcatgcagctgtggagaacacccctgggactctaactctggcactctgcaagctgggtacttgggcaggacagcagcagcactcatgaactgggcagcacctgttggtgagggctgatcacatggattctctcatcccagccttacaatcagtccttcaggtacatactttttctgactttgctgatgaggaaactatgcacagaggttacacagcttaacaaagggttctcacctaatgaacaatgaaatgggattttagcctttctttgcatctggtcttagagccaatacccaagaagcactgtactgtatgcattgtctcagagaaacttactcttcctgggcctcagtctttaaaaggtgggcagttgacttaataagaattaaagatcaatgattaaggttcaaggcactccaaaattctggtctttattgaaaaggctacagaagtctcaccttaataataccctatagacttgatattcttggttaattaaatattggaaaccaatttcatagtaattgaggtcagaaaaaagtactcatgacattttagaatatgatgacaaagccatagataaatttcaatgcacctgtaattacttaaaactgttatagcatgcaatgtgttaccacaacagccagagaaatactaatttactcagcctattcttctagaccagtaaacactaggattaaatagatattttcattgaatttgttctacccttcattgccatttatagatagcttacttgtcatagattactttctaattgttttatgtttcctaactagcctgcaatactttggcaaggacctcaaacaatagtagacagtaggtgtaaaatagatggctacattgaacagatgactaaaaggatgcctcctaagtacctatatcttgaaatatatattattgtgccttgctttcaatttgtgattttaaaatctagaaatcacctgttttatgtaataacaataaaatccttctttgttgaaaacatgcacaaataaagtttacaagctcaaaaaattaaacagcagtaacggtcaagctttccaacaataaaatacattttggtaaggttttcattttacaaaaactcaaaatagctttatgagttcacaaaataatatgatatttttcaagatattaacatattcttataccggaagagcatagaataaaatttacttggagattgagcatttgcttctttaagaaatacttcttttagtatttttactttaatattatgaaagctacataattacattcagattcattaactactccagtagttaatttttaaaacttatgatgaatagttttgtttaaaatatataacattggtaatatgcaaatctgaatctgtaataaagaaggatttgcattcctgatttttttttctgatacaaccaatgacaaaataactaatggttccacagaggataaaatgtctcaaatctgttggttctgaaggtgaagcgagatttttgtactgataccgtgtatcactgagataccaggaggaaatggaattaaactcagatagttcaaatggagagattttaatgaagggacgacctacagaggtgtcggcagggttggggggaatcagcgagatatgcttagaacccaccgactggcaaacctccccctgaagatggagaaggaggaaggagtgttactggaatgagagcttgagtccaggggaggaggatgggctgctgaggaggcgacaccatcctgaaagaagaatcctctgccagaggcttttcagggtcatttcttcacactctctgcagggaagcacggagacagcaggaagaaatatcctaacctcactctcttccctctacaggtgcttccattggccaaatccacccagaggccagttggtggcgatcagctctcttcaagtggtatttaaatttcttctttcattttccttctggtaacaaagaagtctgtggctcaaaagatgtttctctaagaccccatcctattaggtctctgagctgtgggaagtatttatacaattgcttgtgaatataagatccaggaatttccctaagatccctaacaaaattggtgataagtagtcccacatgttaatccagccacccacggatgacagcacttaccatttctttgataaatgtcaaatgcatttgaagtacctacctgaaatatttgtttaaatgctatctaatctattaattttatatatgtgtgagtctgttttgtataccttctgattataggataaatgtaaataaatccaaagagtaatcaaagctaccactttcaagaagccttctttgtagaaccggaagagtcttaaataggcttttcaggtatgcatctcttattatcgctgaactccaagtcctgcaaggcaggcatcatgtgtgggtcacctttacagtaggcacaggccttaaaacagtgacatgcacattgcaggcactccataaatgtttgctgaattggctaaaccttggtttgttcccataatcaaccaccacaaacagcacacagataattacttcttggaaagattccaactagtgtttgatgttacctacgtggtttttctctcaagatcttaagagcagctctgtaggattacattattttctgttttttttttcctttgaccttaatgtcatctacttcaataacagcttcatacaaaattcctaccagcacataccacagcagattcaaggccttgttttaaaaatggtgccagcttctcttaatttggaagatatattgtctctcctgaacatgggctaagaaaatgtataatttggtattaacataagagctgaagacactttaaatgcattgtttcatttttataagataaaaaaaattttaagaatcaaaatgttatcaacagacttgtccttcattaaaaagtaaaactgcatttgcctacattttatgaaagtgtccaattatgaacaattttgaaatgtaacttttaaaaatgtaaacagcaaaaatgttgtatttaaaataaatctggaaaggcagaaaaacaaaaaatacccagaagacagagtttttggtgaaagttaagatatttcatctttgaacaacttagaatctttcctgcattttatagtctagttccaggcattaatttgaaataaccttggaatcctaaatctaacacccttcggaacaaagtagcttttctcttctgctttatgagcaaatggactaaatactagggaatggtactgtctgggcctttgaaccaagattgaaagagatgaaatcctatatgatatgtataaacattagagaatccattttgatttaataaaaggttgaatttgttctatatcctgtgagaaaatggttcccttttcctgaaaatgttacctcattccaacaatagaaagttggtttttttccagggtgtggtgttggcgggggacagagttgccatgaatatggcatctatgaagactgctgttatattcatttctcaaaatgcactgtggtaggaaattcagaacgcagtgagagaaaataaatgtttgacttcaaaatataaggccgcatttaaagcagaaggtaaagtatagaacagttgacagtataaattctttatctgcaatcttgcagttccctaaatctctgtaacacatcacttttaaaagcctcagataagtggttctataataatttaccaataattcaacccctcaaaagtcttagcaagttaaaccttataatcttacattttagaaatgacccaacttgatccttttattcttcagaatatctctctcaaattttcatttgtttttcattaattgatgaataatgagacattttaggtacctgtccacaaagaaatgaaattttcactttccaggaacctgagggccgacgagtgggggcgggcaggagggccgagggaggcggaacaggatcgaggcgcgaggcgggagtcgagaaagcgagcggccgaggcgactctcagtgcgcggacgcgggcgcgcgcccgcgctcccttcgtcgactcacggcgagagcccaaccctgctgccgcgcgccaccc

SEQ ID NO: 17605 - RNA, 9615 nt, Homo sapiens
  source 1..9615: mol_type = other RNA
tcaggccaggcacagtggctcatgcctgtagtcccagcactttgggaggccgaggtgggcagatccacgaggtcaggagatcaagaccatcctaacatggtaaaaccccatctctactaacaatacaaaaaattagtcaggtgtggtggcacgtgcctgtagtcccagctactcaggaggctgaggcaggagaatcgcttgaacctgggaggcggaggttgcagtgagccgagattgtgccactgcaccctagcctaggcaacagagcaagactctgtctcaaaaaaaataaaaaaaaaaaaaagagagaaagagagagagagatgaggagttgctgcactgctgggtgtggagagccgaggaggattcaaagatggtcctgaagtcccagctggaagaagtaggcggcagcaatgtttttaatactgtaaattcatcacgtagcacaggtttggggtggagaaagaaaaattgcattggcttcagggcatgcccagatctttcctcatcttaggcgtttgctaatacatgcattttctaagctgatgtcttgcgtttaatcactgctccattcaaaagagagaaggaggttgtttcaaacctagttgatatcatttgacttccatgctattcacagggctattttatttgaaacaggtataccacagccttaaattgcaagttaatccaggatgttcctaggttggcagttaggaacatgtaattctttggaagggctaaaagtcagctctttaaattatctccatatgaaccttctctccaccttagggtggatccacttatttagtccactgccagtaccacactagaacccgggtggtcactggactccagaaacaacagtagccctctctctgttctgtctctttttgactatctctattctgttcctgaccctgatttctcctgccaagctcaattttgacagctgacaacggcaagccatggcttcccaaaacattattttcaggtcaacttataaatttcaagaacacatttggctccgcttcctgtggtactaagcctacttcttgacagcatttgcctttgttgtaaatagcaaagttcttctagttggatttttgctaagaagtgtgtggatgtggcatgtgacgacatctttagcttggattctagaaaggcactaccattgtgcatttggctaaaggaaacacattttacccgtgaatgccttctatttacaaatgctcagctagcacacaaagctaagtacaagcaataagtactatcctacaatgttactcatttctgaaagcacaaaatgatgactggtatagctttggagatgttttctggaaacccaataaaggaacagatctttgttattccacacctacaaagtcagaagatgcacagtcttttattcatgtttgaacaagcttccttcttgaacaatcaactataaagtgatgtgattctctactagaccaggaactccttgaggacagaatgagggtctaatccatattctaaatccacaccacctggcacaatacatgttgcatggttagggtcaactaagagttggttgaattaatcaataacacacagcaagagaattcacaaagagaggggagtaatcccccagcctcaatcactcggcaagtggaatcgctgggcactgattccagctctgtctcagtgcttgagacagagctgaatgtaatgtgaacatttcaaatgaacaggaaaactagactcacggataagcagtgtagtcatcaagacaacactgtcttggaggtttttctgaagttaaaaccatgctacataagcaataaattatgaaggctgagcatgtgaataaaatttaatgttgtcataaattttataacaaagttaatctgacacatttaatgacatgcataatcattagtatgcagcactgtaatcagacattgataataagcagttcacaccagtgactgtaagagtctttacttgtgttcagccaagccaactgcttggtatatttttctcccttcttagtcgttagttttccatacctacaataactatcagtggtgatgggcttctctgaccatgtgaataatttaatcctcaatgcacagatacagaaacccttgctgaagacagtgtggagcagagaaggctgtctccactccttccacctgaaacacctctgcagatggatatgggagctctgcctacagcccttggacctaaccacttcagtgtgttccagtgagtgtctggacctcggcctgaaagatttttccgaaactaaagaaaatttctctgacctaaagaccttaacctccaccccagaagctctcaccaaggactacagggaactggtggggaaaatccttatcccttactcctcaaggcacagggcagtaatgctgaggcttgtgcgccacacttgctcccagaggtccccagcgggctacctgcggtggtgaatgacctcctaacacgccccttgacggccttcctttccttgcctcacttctccactctcctaccagcattgcagggttcacatcccaaatataccactggcacttgaatcctggtctccaggtctgtttctggaaaaacccaagtaagacattgccccagtaatggggctagatgtctgaggcttcctcaagtatctacctcgaaagctcttactgctgtacacacatgcacatacacacacgtgcgtacaaccagtcacatctaagcaccccgaataccagcctgttgaaggtagcagagagctgcactataagccaaggctgctcccaagagccgctccatcactgaattggcgccccagcaagatgaaggaatgtaatcattggaaggatggagaatgttctctgaatcactgacaaattggaaggggtggagggcaagagtccacctggtggagagatggaaagagcgagagagcctggaatgataatgccattgcttagaaaaggctgctccagatgccatatctacagaaattgtacagcccaaacatctctgagcaataggtctctggtagtcttgatgtctagaccaacaattcccagttcattcttctcagggaaggagccaggatagtccagagactctcattctgctgttagattgaaagggttaggcacaacagccttggcaaagtcacaagggcaaattcacactaaagtgtaaatgacccacaactcctcttctatttttaggttggggaggtgctttagaacataaggaggaactaaagaatattcctgttacatacaaggcagagaaaagggaaactagtggtgacaagacaaatcatccctttgacatttggctggctctacctattacagctctgggggtgaggtgggaacaaaaagatgctgtgtaaagaagtatcttatgccatccctactgtagtgaggtgcagtttagaggggacactgatcaagcagagacccagagtgtttcgttccaagccagaaacagaaatgtataaaacacagcctttccagcatcagaaatgagtagtggtagtggagaactacccaaaacaggaaagaggaccacgtgaggtagagtgtcaaggccctacattccagtgcctctgctcatgactgtaattttgggtaggtcacttaaagtctctggacctcagttttgccatctgtgaaatagggataatactatccagcataaaattggttatgaggctcatgtagggcctgcctgggatgatgtgttgctaatggttaagaacacaacttctggggtctgactggacaggctgaaatccctgcttaacacgttccagcagagccctgggcgatctatttaacttttgttttctcacctgtaagctgagacgaaagtacccactttataagattattccaataattagttgaaataatgcatgcagagaattaagcatggtacttgttatttgttaaactagctattaaaatgtgtaaaatataaagtattgtatggattttaggacaatgcaaagactctttgcttgctgcaatagttcggggccctttcagatggctaaaggcagaatttgtatgtgtaaatatggtgtgcttgtctctgctctggatactgagggcttaccctgttattaaacttatttagtaaatattgaactgtcatgaggcctaacatttagttccagttattagataaaacatttgctttgaatggtatttgaattgccaggttctagattattctggttgacaaactcttcgtattttataaagaggctaaaattggtaagctatcacagaacagatgtgccattttcaaggtatattaaaccatgattcactgtaacattgttcctactggcaacaaattcagagcaggctggactttatttggtgaagaaacattgagtggaagagaaatgacattattttatgtatttacattttcaaattactgtggcttaaacctgttcagccaacattacccaccttcagtctgctaaataaatgattcagtacatttctaatttacagaattttttaacaaaagaaaatgtaatttgatagccaaatcaacgttaaacattatacatttaaaaaaccacaggcaaagacacaaacatgatgacactaacttttgttaaagtatgcttacctatggtttcctctgaggcacgttctttcatgctaagcttccaacataatatgaaaatgaaggagatgcattttgcaaagcaaaacagaccttaagcaaaatattatacttctcaaattaacactgttacaaagttttagaatttaataagttcattaatttaaaagtttggatgtctgagtccttctatcccaaaacaagatcttggagggtcttccacagccatgtaataccatggtcacatgaccctttccaaaattattaatctgaatttactatatgaggataaatctatctttttgaaaatatttaggaaaatgagcttggtatttataaaatgaagctctctttgggtggtatcctaagacacgtcaagccaatcagcctgtaactgtgaaaaaaacattggtaggtacaaaagtggggtgggagaggagtgacttaactttgttaagtgatgggaaagaaacactaatagcattatctcaataaaatgtgatttaaaaaaatttaaaatactaaatcattgaactgacaaagaaatataaatcattcagaaataaactcattaggtcatcaaatcctgttaaatctgcaattaggaagagcaaggtgtacaatccatacatttaaactcacaggctcactttgcacaacgtcaatttactccttaatatgttattaatacgcattttccaaaaggatgtattagtaaatggtacacatctacttcttggcaacatcatataacctggtacaacataagcattcttcttatagttaagaaatgtggatggtatcaaaattagaaaaataaatgccctattatgttgtggtcaggtttaaggcatgtgaattttatcttcatacaaaagattaaaatctagatattaaaaagtagtgcagtatcagtgatgctgcctcagttcccaaaatgtcacatcacaaaaatatcccataattgcctgtagtttattccttggctttcctcttttctctctgcatctttgtaacaattttttaaaagtggaaatataattgttggcaatgctaacagctgtagaaatgattacaagatgtggaaaagcataacaggaatgtcaagaatctgtttctggcagtaatatatatggaacattgttcaggacaaaagaggagaaggaagaaaaaaaggagaggggtttatcatctctaagaattttcaaactaaacctcattgcttaataggaaaaaaagattccatatttaaagttaagtcacctctaactactagctaaagcatgacatcaccagcactggagtcagcggaagtgtgtttttgaaggacagtgttgcaggagaatctggacaggttttagagccaggagagagaaaataattctacctctgacagttgaaggaccttaggcaaatcagtttacctctgctagactacactccaaaatttggacattcaaaaatttgatattaataaccacatgaaagtctcgtgttgaggtgaatatgtatttgttggtgaaagatatgttggtttttaaacagacagcactctgcaattgtaggctattgttttgttttgccagttgtcaaattctatccagctatacacacttgtgtggcctcctaatggtgtttttccagtggctaaaggtttatgaataagacacttttcctaatggaattaacccgatgcttttcttaaacatgtaaccttgagttcaccgcaaaaaacaatgcttcgattagagcaatgcatataataaaggttaccctcgtttcttagacactagacatcattcacaaaaagagaactgcttttgaaagggatgtatttgcactggaaagaatagttttctacttctaattataaatgatttattggtgaaagcaaaacaacagcctgtctgagaggcacttctatgagcatcctcacgtgtgatttgcaaggttgaagaagagggaaaaatgcctcaattgtaccaatggtgagaaaacacccaaagtacaaagcaggtttcaaaaaaaccatactcataaccaaggacaataataaagcaatgtgttgacatatactctataagtcttcctccataaatagtttatagaaattttgtaatttctgtaaatgcatcctataataattttgcatcttgctttttttttacatttaatatcaagtagatttctaaagggcaattatttgaaaattatcccaaatacatggggaaatatacatcaagtgaaaaaatgcagtgggtgatagagatatcaggaagcgcctcaaatatttctcatctcgttggagaaaaacaaacatgttctcatttagaatgagtgggagttacctaattgatttaggcctctatatttaacttctagtcaaaaaaggtagttctatctagcaacaatattatggggaacaaaagaaaaaattaactctctaaatttgcagtagggtcttttcttcagaagtaccaaatcccatctattaccagctccatgcttcaggcctaaaatggatctccctgaagcaatgacagaatttttgccaagtgactaggatataaacaccactttggttgcacagtgagacatatgctccaaagaaaactggttcaaaaacaggcaagtgggtttctacagaataaatgagagccctgtcaatggcttcatcttcagggctttgtgtctgtgcttgcgtggtggctcttgtttcatctatggataatggtggcacacagttttcataattccttacattaatgaactgctataaatttgtttttggtattctagagagtcctaacttcagcttctgggcaatgctgaggaggcaccctatattctagacttaccttttgcaaggtgtactctcagcattgtgggcgatttccatgggagaatattctatttaaagaactactgtcccagcataaaacaaaaaatcatttatgaagatgcaggagactcggaaagctctcaattattgtttgcacaagcacaatgtcacagcctcctttccccattccacaagggggtcaggaagagagtactcagctgtgagaaaagacatacagaagaattcatgtggtcatgagagcgaggacatggccgatcccccaaggaggatgtgtcatacacttcatgagcccaagagtgtgctgtagggtctgaagggcaagatgctggttcactgatgtaaaggagagggaaaaaagcttcaaccaactagaaaaacagtctctatgcatgctatttttgattttaaacacaggtatcaattccttctctcagagagtccattttaaaataggatacatttttaaaggaatatttaaaggacacattcattaaaatttattttaaaaacttttcaaaagaaacaaaaggtatgaattttatttaatccttgaggaaatggttcttttctcacacacataaatcactcattttgtttttctttatctcctttattaatctacattagaaaaataaacttttcatacactaagaacaaggaaaccactctcaattgacaaaatgttccaatccaacacaatgattactttcacctttaatttacaggcagccagattcaaaatccttaaagttgcttaaacttaaaaatgacaatgacaacctaaaaggtataatgttgattggaacagacatttaattggaaaattgatgattttccatttccaattaaatctctagatagaaatgaaaaaaattaaaaatcgtatttaagaaaagccaaatcttgggttgtgaggtatctttttaaggatgtttcagcagaaaaaaacaaaggctctcacaattgtgtagctgcctagattaagtgggtatcctgatcaaggagatgggggatgatttggctttagtattccaatgataaagtttataatgagaataacatgttgctacaaaatccagtctcttcctcagatgccttccacagagggcaggaagctttgtcagttttgtttgctgatgatgcctggttccgtcaacaaataacacctgtcacacggtgggtagtcaatatacatttgttgaataaatatgaaaaaaagaaatgtacaatatgtttgtgaagccaactgtgtgtgcattgctattgaggtacacaaaaagtctttgttttaaatttgagaatgaggactttcaatggaatatatctataaaaatgaaaaaaagacattactgtctggacttttgtacagcaagagaagaaaaaccactagccaagagccaactcacctgataggcctggatcaagcatgcagctgtggagaacacccctgggactctaactctggcactctgcaagctgggtacttgggcaggacagcagcagcactcatgaactgggcagcacctgttggtgagggctgatcacatggattctctcatcccagccttacaatcagtccttcaggtacatactttttctgactttgctgatgaggaaactatgcacagaggttacacagcttaacaaagggttctcacctctcttcaagtggtatttaaatttcttctttcattttccttctggtaacaaagaagtctgtggctcaaaagatgtttctctaagaccccatcctattaggtctctgagattttagaaatgacccaacttgatccttttattcttcagaatatctctctcaaattttcatttgtttttcattaattgatgaataatgagacattttaggtacctgtccacaaagaaatgaaattttcactttccaggaacctgagggccgacgagtgggggcgggcaggagggccgagggaggcggaacaggatcgaggcgcgaggcgggagtcgagaaagcgagcggccgaggcgactctcagtgcgcggacgcgggcgcgcgcccgcgctcccttcgtcgactcacggcgagagcccaaccctgctgccgcgcgccacccgcctcgccgcgc

SEQ ID NO: 17606 - RNA, 14157 nt, Homo sapiens
  source 1..14157: mol_type = other RNA
tcaggccaggcacagtggctcatgcctgtagtcccagcactttgggaggccgaggtgggcagatccacgaggtcaggagatcaagaccatcctaacatggtaaaaccccatctctactaacaatacaaaaaattagtcaggtgtggtggcacgtgcctgtagtcccagctactcaggaggctgaggcaggagaatcgcttgaacctgggaggcggaggttgcagtgagccgagattgtgccactgcaccctagcctaggcaacagagcaagactctgtctcaaaaaaaataaaaaaaaaaaaaagagagaaagagagagagagatgaggagttgctgcactgctgggtgtggagagccgaggaggattcaaagatggtcctgaagtcccagctggaagaagtaggcggcagcaatgtttttaatactgtaaattcatcacgtagcacaggtttggggtggagaaagaaaaattgcattggcttcagggcatgcccagatctttcctcatcttaggcgtttgctaatacatgcattttctaagctgatgtcttgcgtttaatcactgctccattcaaaagagagaaggaggttgtttcaaacctagttgatatcatttgacttccatgctattcacagggctattttatttgaaacaggtataccacagccttaaattgcaagttaatccaggatgttcctaggttggcagttaggaacatgtaattctttggaagggctaaaagtcagctctttaaattatctccatatgaaccttctctccaccttagggtggatccacttatttagtccactgccagtaccacactagaacccgggtggtcactggactccagaaacaacagtagccctctctctgttctgtctctttttgactatctctattctgttcctgaccctgatttctcctgccaagctcaattttgacagctgacaacggcaagccatggcttcccaaaacattattttcaggtcaacttataaatttcaagaacacatttggctccgcttcctgtggtactaagcctacttcttgacagcatttgcctttgttgtaaatagcaaagttcttctagttggatttttgctaagaagtgtgtggatgtggcatgtgacgacatctttagcttggattctagaaaggcactaccattgtgcatttggctaaaggaaacacattttacccgtgaatgccttctatttacaaatgctcagctagcacacaaagctaagtacaagcaataagtactatcctacaatgttactcatttctgaaagcacaaaatgatgactggtatagctttggagatgttttctggaaacccaataaaggaacagatctttgttattccacacctacaaagtcagaagatgcacagtcttttattcatgtttgaacaagcttccttcttgaacaatcaactataaagtgatgtgattctctactagaccaggaactccttgaggacagaatgagggtctaatccatattctaaatccacaccacctggcacaatacatgttgcatggttagggtcaactaagagttggttgaattaatcaataacacacagcaagagaattcacaaagagaggggagtaatcccccagcctcaatcactcggcaagtggaatcgctgggcactgattccagctctgtctcagtgcttgagacagagctgaatgtaatgtgaacatttcaaatgaacaggaaaactagactcacggataagcagtgtagtcatcaagacaacactgtcttggaggtttttctgaagttaaaaccatgctacataagcaataaattatgaaggctgagcatgtgaataaaatttaatgttgtcataaattttataacaaagttaatctgacacatttaatgacatgcataatcattagtatgcagcactgtaatcagacattgataataagcagttcacaccagtgactgtaagagtctttacttgtgttcagccaagccaactgcttggtatatttttctcccttcttagtcgttagttttccatacctacaataactatcagtggtgatgggcttctctgaccatgtgaataatttaatcctcaatgcacagatacagaaacccttgctgaagacagtgtggagcagagaaggctgtctccactccttccacctgaaacacctctgcagatggatatgggagctctgcctacagcccttggacctaaccacttcagtgtgttccagtgagtgtctggacctcggcctgaaagatttttccgaaactaaagaaaatttctctgacctaaagaccttaacctccaccccagaagctctcaccaaggactacagggaactggtggggaaaatccttatcccttactcctcaaggcacagggcagtaatgctgaggcttgtgcgccacacttgctcccagaggtccccagcgggctacctgcggtggtgaatgacctcctaacacgccccttgacggccttcctttccttgcctcacttctccactctcctaccagcattgcagggttcacatcccaaatataccactggcacttgaatcctggtctccaggtctgtttctggaaaaacccaagtaagacattgccccagtaatggggctagatgtctgaggcttcctcaagtatctacctcgaaagctcttactgctgtacacacatgcacatacacacacgtgcgtacaaccagtcacatctaagcaccccgaataccagcctgttgaaggtagcagagagctgcactataagccaaggctgctcccaagagccgctccatcactgaattggcgccccagcaagatgaaggaatgtaatcattggaaggatggagaatgttctctgaatcactgacaaattggaaggggtggagggcaagagtccacctggtggagagatggaaagagcgagagagcctggaatgataatgccattgcttagaaaaggctgctccagatgccatatctacagaaattgtacagcccaaacatctctgagcaataggtctctggtagtcttgatgtctagaccaacaattcccagttcattcttctcagggaaggagccaggatagtccagagactctcattctgctgttagattgaaagggttaggcacaacagccttggcaaagtcacaagggcaaattcacactaaagtgtaaatgacccacaactcctcttctatttttaggttggggaggtgctttagaacataaggaggaactaaagaatattcctgttacatacaaggcagagaaaagggaaactagtggtgacaagacaaatcatccctttgacatttggctggctctacctattacagctctgggggtgaggtgggaacaaaaagatgctgtgtaaagaagtatcttatgccatccctactgtagtgaggtgcagtttagaggggacactgatcaagcagagacccagagtgtttcgttccaagccagaaacagaaatgtataaaacacagcctttccagcatcagaaatgagtagtggtagtggagaactacccaaaacaggaaagaggaccacgtgaggtagagtgtcaaggccctacattccagtgcctctgctcatgactgtaattttgggtaggtcacttaaagtctctggacctcagttttgccatctgtgaaatagggataatactatccagcataaaattggttatgaggctcatgtagggcctgcctgggatgatgtgttgctaatggttaagaacacaacttctggggtctgactggacaggctgaaatccctgcttaacacgttccagcagagccctgggcgatctatttaacttttgttttctcacctgtaagctgagacgaaagtacccactttataagattattccaataattagttgaaataatgcatgcagagaattaagcatggtacttgttatttgttaaactagctattaaaatgtgtaaaatataaagtattgtatggattttaggacaatgcaaagactctttgcttgctgcaatagttcggggccctttcagatggctaaaggcagaatttgtatgtgtaaatatggtgtgcttgtctctgctctggatactgagggcttaccctgttattaaacttatttagtaaatattgaactgtcatgaggcctaacatttagttccagttattagataaaacatttgctttgaatggtatttgaattgccaggttctagattattctggttgacaaactcttcgtattttataaagaggctaaaattggtaagctatcacagaacagatgtgccattttcaaggtatattaaaccatgattcactgtaacattgttcctactggcaacaaattcagagcaggctggactttatttggtgaagaaacattgagtggaagagaaatgacattattttatgtatttacattttcaaattactgtggcttaaacctgttcagccaacattacccaccttcagtctgctaaataaatgattcagtacatttctaatttacagaattttttaacaaaagaaaatgtaatttgatagccaaatcaacgttaaacattatacatttaaaaaaccacaggcaaagacacaaacatgatgacactaacttttgttaaagtatgcttacctatggtttcctctgaggcacgttctttcatgctaagcttccaacataatatgaaaatgaaggagatgcattttgcaaagcaaaacagaccttaagcaaaatattatacttctcaaattaacactgttacaaagttttagaatttaataagttcattaatttaaaagtttggatgtctgagtccttctatcccaaaacaagatcttggagggtcttccacagccatgtaataccatggtcacatgaccctttccaaaattattaatctgaatttactatatgaggataaatctatctttttgaaaatatttaggaaaatgagcttggtatttataaaatgaagctctctttgggtggtatcctaagacacgtcaagccaatcagcctgtaactgtgaaaaaaacattggtaggtacaaaagtggggtgggagaggagtgacttaactttgttaagtgatgggaaagaaacactaatagcattatctcaataaaatgtgatttaaaaaaatttaaaatactaaatcattgaactgacaaagaaatataaatcattcagaaataaactcattaggtcatcaaatcctgttaaatctgcaattaggaagagcaaggtgtacaatccatacatttaaactcacaggctcactttgcacaacgtcaatttactccttaatatgttattaatacgcattttccaaaaggatgtattagtaaatggtacacatctacttcttggcaacatcatataacctggtacaacataagcattcttcttatagttaagaaatgtggatggtatcaaaattagaaaaataaatgccctattatgttgtggtcaggtttaaggcatgtgaattttatcttcatacaaaagattaaaatctagatattaaaaagtagtgcagtatcagtgatgctgcctcagttcccaaaatgtcacatcacaaaaatatcccataattgcctgtagtttattccttggctttcctcttttctctctgcatctttgtaacaattttttaaaagtggaaatataattgttggcaatgctaacagctgtagaaatgattacaagatgtggaaaagcataacaggaatgtcaagaatctgtttctggcagtaatatatatggaacattgttcaggacaaaagaggagaaggaagaaaaaaaggagaggggtttatcatctctaagaattttcaaactaaacctcattgcttaataggaaaaaaagattccatatttaaagttaagtcacctctaactactagctaaagcatgacatcaccagcactggagtcagcggaagtgtgtttttgaaggacagtgttgcaggagaatctggacaggttttagagccaggagagagaaaataattctacctctgacagttgaaggaccttaggcaaatcagtttacctctgctagactacactccaaaatttggacattcaaaaatttgatattaataaccacatgaaagtctcgtgttgaggtgaatatgtatttgttggtgaaagatatgttggtttttaaacagacagcactctgcaattgtaggctattgttttgttttgccagttgtcaaattctatccagctatacacacttgtgtggcctcctaatggtgtttttccagtggctaaaggtttatgaataagacacttttcctaatggaattaacccgatgcttttcttaaacatgtaaccttgagttcaccgcaaaaaacaatgcttcgattagagcaatgcatataataaaggttaccctcgtttcttagacactagacatcattcacaaaaagagaactgcttttgaaagggatgtatttgcactggaaagaatagttttctacttctaattataaatgatttattggtgaaagcaaaacaacagcctgtctgagaggcacttctatgagcatcctcacgtgtgatttgcaaggttgaagaagagggaaaaatgcctcaattgtaccaatggtgagaaaacacccaaagtacaaagcaggtttcaaaaaaaccatactcataaccaaggacaataataaagcaatgtgttgacatatactctataagtcttcctccataaatagtttatagaaattttgtaatttctgtaaatgcatcctataataattttgcatcttgctttttttttacatttaatatcaagtagatttctaaagggcaattatttgaaaattatcccaaatacatggggaaatatacatcaagtgaaaaaatgcagtgggtgatagagatatcaggaagcgcctcaaatatttctcatctcgttggagaaaaacaaacatgttctcatttagaatgagtgggagttacctaattgatttaggcctctatatttaacttctagtcaaaaaaggtagttctatctagcaacaatattatggggaacaaaagaaaaaattaactctctaaatttgcagtagggtcttttcttcagaagtaccaaatcccatctattaccagctccatgcttcaggcctaaaatggatctccctgaagcaatgacagaatttttgccaagtgactaggatataaacaccactttggttgcacagtgagacatatgctccaaagaaaactggttcaaaaacaggcaagtgggtttctacagaataaatgagagccctgtcaatggcttcatcttcagggctttgtgtctgtgcttgcgtggtggctcttgtttcatctatggataatggtggcacacagttttcataattccttacattaatgaactgctataaatttgtttttggtattctagagagtcctaacttcagcttctgggcaatgctgaggaggcaccctatattctagacttaccttttgcaaggtgtactctcagcattgtgggcgatttccatgggagaatattctatttaaagaactactgtcccagcataaaacaaaaaatcatttatgaagatgcaggagactcggaaagctctcaattattgtttgcacaagcacaatgtcacagcctcctttccccattccacaagggggtcaggaagagagtactcagctgtgagaaaagacatacagaagaattcatgtggtcatgagagcgaggacatggccgatcccccaaggaggatgtgtcatacacttcatgagcccaagagtgtgctgtagggtctgaagggcaagatgctggttcactgatgtaaaggagagggaaaaaagcttcaaccaactagaaaaacagtctctatgcatgctatttttgattttaaacacaggtatcaattccttctctcagagagtccattttaaaataggatacatttttaaaggaatatttaaaggacacattcattaaaatttattttaaaaacttttcaaaagaaacaaaaggtatgaattttatttaatccttgaggaaatggttcttttctcacacacataaatcactcattttgtttttctttatctcctttattaatctacattagaaaaataaacttttcatacactaagaacaaggaaaccactctcaattgacaaaatgttccaatccaacacaatgattactttcacctttaatttacaggcagccagattcaaaatccttaaagttgcttaaacttaaaaatgacaatgacaacctaaaaggtataatgttgattggaacagacatttaattggaaaattgatgattttccatttccaattaaatctctagatagaaatgaaaaaaattaaaaatcgtatttaagaaaagccaaatcttgggttgtgaggtatctttttaaggatgtttcagcagaaaaaaacaaaggctctcacaattgtgtagctgcctagattaagtgggtatcctgatcaaggagatgggggatgatttggctttagtattccaatgataaagtttataatgagaataacatgttgctacaaaatccagtctcttcctcagatgccttccacagagggcaggaagctttgtcagttttgtttgctgatgatgcctggttccgtcaacaaataacacctgtcacacggtgggtagtcaatatacatttgttgaataaatatgaaaaaaagaaatgtacaatatgtttgtgaagccaactgtgtgtgcattgctattgaggtacacaaaaagtctttgttttaaatttgagaatgaggactttcaatggaatatatctataaaaatgaaaaaaagacattactgtctggacttttgtacagcaagagaagaaaaaccactagccaagagccaactcacctgataggcctggatcaagcatgcagctgtggagaacacccctgggactctaactctggcactctgcaagctgggtacttgggcaggacagcagcagcactcatgaactgggcagcacctgttggtgagggctgatcacatggattctctcatcccagccttacaatcagtccttcaggtacatactttttctgactttgctgatgaggaaactatgcacagaggttacacagcttaacaaagggttctcacctctcttcaagtggtatttaaatttcttctttcattttccttctggtaacaaagaagtctgtggctcaaaagatgtttctctaagaccccatcctattaggtctctgagctgtgggaagtatttatacaattgcttgtgaatataagatccaggaatttccctaagatccctaacaaaattggtgataagtagtcccacatgttaatccagccacccacggatgacagcacttaccatttctttgataaatgtcaaatgcatttgaagtacctacctgaaatatttgtttaaatgctatctaatctattaattttatatatgtgtgagtctgttttgtataccttctgattataggataaatgtaaataaatccaaagagtaatcaaagctaccactttcaagaagccttctttgtagaaccggaagagtcttaaataggcttttcaggtatgcatctcttattatcgctgaactccaagtcctgcaaggcaggcatcatgtgtgggtcacctttacagtaggcacaggccttaaaacagtgacatgcacattgcaggcactccataaatgtttgctgaattggctaaaccttggtttgttcccataatcaaccaccacaaacagcacacagataattacttcttggaaagattccaactagtgtttgatgttacctacgtggtttttctctcaagatcttaagagcagctctgtaggattacattattttctgttttttttttcctttgaccttaatgtcatctacttcaataacagcttcatacaaaattcctaccagcacataccacagcagattcaaggccttgttttaaaaatggtgccagcttctcttaatttggaagatatattgtctctcctgaacatgggctaagaaaatgtataatttggtattaacataagagctgaagacactttaaatgcattgtttcatttttataagataaaaaaaattttaagaatcaaaatgttatcaacagacttgtccttcattaaaaagtaaaactgcatttgcctacattttatgaaagtgtccaattatgaacaattttgaaatgtaacttttaaaaatgtaaacagcaaaaatgttgtatttaaaataaatctggaaaggcagaaaaacaaaaaatacccagaagacagagtttttggtgaaagttaagatatttcatctttgaacaacttagaatctttcctgcattttatagtctagttccaggcattaatttgaaataaccttggaatcctaaatctaacacccttcggaacaaagtagcttttctcttctgctttatgagcaaatggactaaatactagggaatggtactgtctgggcctttgaaccaagattgaaagagatgaaatcctatatgatatgtataaacattagagaatccattttgatttaataaaaggttgaatttgttctatatcctgtgagaaaatggttcccttttcctgaaaatgttacctcattccaacaatagaaagttggtttttttccagggtgtggtgttggcgggggacagagttgccatgaatatggcatctatgaagactgctgttatattcatttctcaaaatgcactgtggtaggaaattcagaacgcagtgagagaaaataaatgtttgacttcaaaatataaggccgcatttaaagcagaaggtaaagtatagaacagttgacagtataaattctttatctgcaatcttgcagttccctaaatctctgtaacacatcacttttaaaagcctcagataagtggttctataataatttaccaataattcaacccctcaaaagtcttagcaagttaaaccttataatcttacattttagaaatgacccaacttgatccttttattcttcagaatatctctctcaaattttcatttgtttttcattaattgatgaataatgagacattttaggtacctgtccacaaagaaatgaaattttcactttccaggaacctaacaaatgaaaagatagaaatcaattccaacagaatattaccaaagaaatcttttagaatggactgttaaaattatttatttgtatttatctggctctactatttgtggtacatttccacttcaaagctaaacctcaaataacatcatagtgagtggttgacttcatgtttaactgagatcttgaagactgaaaaagaccacgacaaacacacatctattttcttggctactgcatccgtgttcatcaccattctgatagtctgcaatgtattgcagctcaccctttgggaaggactaaagtagacatctgtttgttctgcttactcagcattcctaccctaattttcctttggagaacccctttattctagaccacgtgaagctaatgccaaaccccattccaggggatgcacctgaatccaacctccatcatctaaacagtgccttctccacgttcagagaagagcaagtgactcaaactgccctcataagaacagacctgggacttctgctgcaaatattgaagagtaagtactcttttttcttgctaggactaagctggtagtaccttctatgaggctatcatatggaaacaacttgtctgaaaatgaagccacaactagaaaacagatcctggtaacccggattgatggatccagccctaccttaaatggcaagacctaacccgaggctttttgcatcaaccaataaagtccttaagccagtttgagttggttttgtcacttgcagctaaaagaattctgactctaacaatgtgacaatagcaaaaataaacataactgcttttgaggtttctaatggattttcctccctatatacatgatttcatttaatcctcacaattcaggaaagcacatatctattaacattaaattaatattcattattttgaacacatgctatgtggataagggatgaggaaagccaaggaagtaatcaacgtgaaatctcacttatatgggagggaagtggaggttacatatctcagggcacttaacagatatcatcaaatgaaagaataaacagtgtgtgggagaggcagtaggtgattcttcatcaattcctggatgaaaaattaggagataatgaactccgaacaggcagcctaatgagaatggctcaagcaacaggacatagagagggagttaggttagacatggggttcttgggaattttcacctcgtgggggggcgggggggtcgtgcagctgttgtcagtgggaaagggaaaaaggaaaaggctgagtttggaaggcagggagggaggagacaatgtgagtcagtgaaaaagggcccttagaatgacaagtctggaccagagagaggctaagactgaaaatacaagttgggtaaccactggcatacagatggcagttcaggcttgggcactgcccaccagagcctcagcatgaagagaagagggggaggctggccaccacctccctctaggtaatcgtcatcctgatgctgagctcctgaaaacaggctctttcactcgccccatctcttgctcttgattgcaacccggcattcaggaggcaccctgtaatatctgtggagtgaccgacaacacagcgccagggcactgagaagatcccagggcgccagggactggttctacaagggtgcccctcccggtcccctccagcgcgccgccagagctgccagtcttggctgctacacgggaggcagcctcattatgcagctctcacctcttaaattagttcatgctctcacattaggtgtaatcacagcttgcaacgctttctggggatgtctcagaaagatctgagttgaaaaaatatttttgtgtcattttaatttaaagtaaaattgctgcttcttccccgcccctttctttcctcctggcccacccagcgaccctggccggccgtgctcaacgggggcgggggtcggaggtgagatttcctccacataattccttaaacagctatcaactaagtctcaaagaaaaaaaaaagagatctagaagcagagacgtggctgctggcgatcccaaagctggtgttcgctcttgggggagagcgtaccctgggggaggccgggaggccgggccagaggctagcccagaggcagagggcaggagcgctcagccggcgccccgcgtctctccagctcccgacgctgcgctggctccgctgagcacgccaggatcaaggtcgcctggtggggaccggagcgccaggagcctgtgggaagcgttccagccggcctctgactgggatccggcgccgcgtttctgctttggacttgactgacaggtccccccgccctcccgccgccctactaccagcctgggttcatccttcagggctacgtctaccgcacccgggctggaaagcctggagcgcgcccttcctctcctcatcttctcagctctcctttctccctgccacttggcaaagctgcattttgactttcacgttttggactacgtgtgtgtagttccaagtccatgcgtggcacgaaaatccacttagggtaaaaattattctcgaaaaatcgcccatctcaggatctggtgtctacactcaaggctaggaggtgcaggtacgggtgcgtaaagcatgccgtaagggtgcacagtaaataaaaagtacggatgcaaaatgtaaattttaagtgcaaaacagaaaagcagtactcgttgccgccccgcacgctgggttttaaggggcacgaaggtgggcctcggctgcttttgctcagccccgcgtcctcagcgcccggcccagtacccggtactccgtaggggttcaatgatctcccctgaataagtgaacgaattaacaaatgaatgaatgaccgctcgatccgacctccgcggccggcagagcagtcgctggagaggcgggagagagcgagaggccaagctccaccatcgcggccgccggctggggcagagggacacggagacactcggcgccccggctccgcaccgagtccccg

SEQ ID NO: 17607 - RNA, 14117 nt, Homo sapiens
  source 1..14117: mol_type = other RNA
tcaggccaggcacagtggctcatgcctgtagtcccagcactttgggaggccgaggtgggcagatccacgaggtcaggagatcaagaccatcctaacatggtaaaaccccatctctactaacaatacaaaaaattagtcaggtgtggtggcacgtgcctgtagtcccagctactcaggaggctgaggcaggagaatcgcttgaacctgggaggcggaggttgcagtgagccgagattgtgccactgcaccctagcctaggcaacagagcaagactctgtctcaaaaaaaataaaaaaaaaaaaaagagagaaagagagagagagatgaggagttgctgcactgctgggtgtggagagccgaggaggattcaaagatggtcctgaagtcccagctggaagaagtaggcggcagcaatgtttttaatactgtaaattcatcacgtagcacaggtttggggtggagaaagaaaaattgcattggcttcagggcatgcccagatctttcctcatcttaggcgtttgctaatacatgcattttctaagctgatgtcttgcgtttaatcactgctccattcaaaagagagaaggaggttgtttcaaacctagttgatatcatttgacttccatgctattcacagggctattttatttgaaacaggtataccacagccttaaattgcaagttaatccaggatgttcctaggttggcagttaggaacatgtaattctttggaagggctaaaagtcagctctttaaattatctccatatgaaccttctctccaccttagggtggatccacttatttagtccactgccagtaccacactagaacccgggtggtcactggactccagaaacaacagtagccctctctctgttctgtctctttttgactatctctattctgttcctgaccctgatttctcctgccaagctcaattttgacagctgacaacggcaagccatggcttcccaaaacattattttcaggtcaacttataaatttcaagaacacatttggctccgcttcctgtggtactaagcctacttcttgacagcatttgcctttgttgtaaatagcaaagttcttctagttggatttttgctaagaagtgtgtggatgtggcatgtgacgacatctttagcttggattctagaaaggcactaccattgtgcatttggctaaaggaaacacattttacccgtgaatgccttctatttacaaatgctcagctagcacacaaagctaagtacaagcaataagtactatcctacaatgttactcatttctgaaagcacaaaatgatgactggtatagctttggagatgttttctggaaacccaataaaggaacagatctttgttattccacacctacaaagtcagaagatgcacagtcttttattcatgtttgaacaagcttccttcttgaacaatcaactataaagtgatgtgattctctactagaccaggaactccttgaggacagaatgagggtctaatccatattctaaatccacaccacctggcacaatacatgttgcatggttagggtcaactaagagttggttgaattaatcaataacacacagcaagagaattcacaaagagaggggagtaatcccccagcctcaatcactcggcaagtggaatcgctgggcactgattccagctctgtctcagtgcttgagacagagctgaatgtaatgtgaacatttcaaatgaacaggaaaactagactcacggataagcagtgtagtcatcaagacaacactgtcttggaggtttttctgaagttaaaaccatgctacataagcaataaattatgaaggctgagcatgtgaataaaatttaatgttgtcataaattttataacaaagttaatctgacacatttaatgacatgcataatcattagtatgcagcactgtaatcagacattgataataagcagttcacaccagtgactgtaagagtctttacttgtgttcagccaagccaactgcttggtatatttttctcccttcttagtcgttagttttccatacctacaataactatcagtggtgatgggcttctctgaccatgtgaataatttaatcctcaatgcacagatacagaaacccttgctgaagacagtgtggagcagagaaggctgtctccactccttccacctgaaacacctctgcagatggatatgggagctctgcctacagcccttggacctaaccacttcagtgtgttccagtgagtgtctggacctcggcctgaaagatttttccgaaactaaagaaaatttctctgacctaaagaccttaacctccaccccagaagctctcaccaaggactacagggaactggtggggaaaatccttatcccttactcctcaaggcacagggcagtaatgctgaggcttgtgcgccacacttgctcccagaggtccccagcgggctacctgcggtggtgaatgacctcctaacacgccccttgacggccttcctttccttgcctcacttctccactctcctaccagcattgcagggttcacatcccaaatataccactggcacttgaatcctggtctccaggtctgtttctggaaaaacccaagtaagacattgccccagtaatggggctagatgtctgaggcttcctcaagtatctacctcgaaagctcttactgctgtacacacatgcacatacacacacgtgcgtacaaccagtcacatctaagcaccccgaataccagcctgttgaaggtagcagagagctgcactataagccaaggctgctcccaagagccgctccatcactgaattggcgccccagcaagatgaaggaatgtaatcattggaaggatggagaatgttctctgaatcactgacaaattggaaggggtggagggcaagagtccacctggtggagagatggaaagagcgagagagcctggaatgataatgccattgcttagaaaaggctgctccagatgccatatctacagaaattgtacagcccaaacatctctgagcaataggtctctggtagtcttgatgtctagaccaacaattcccagttcattcttctcagggaaggagccaggatagtccagagactctcattctgctgttagattgaaagggttaggcacaacagccttggcaaagtcacaagggcaaattcacactaaagtgtaaatgacccacaactcctcttctatttttaggttggggaggtgctttagaacataaggaggaactaaagaatattcctgttacatacaaggcagagaaaagggaaactagtggtgacaagacaaatcatccctttgacatttggctggctctacctattacagctctgggggtgaggtgggaacaaaaagatgctgtgtaaagaagtatcttatgccatccctactgtagtgaggtgcagtttagaggggacactgatcaagcagagacccagagtgtttcgttccaagccagaaacagaaatgtataaaacacagcctttccagcatcagaaatgagtagtggtagtggagaactacccaaaacaggaaagaggaccacgtgaggtagagtgtcaaggccctacattccagtgcctctgctcatgactgtaattttgggtaggtcacttaaagtctctggacctcagttttgccatctgtgaaatagggataatactatccagcataaaattggttatgaggctcatgtagggcctgcctgggatgatgtgttgctaatggttaagaacacaacttctggggtctgactggacaggctgaaatccctgcttaacacgttccagcagagccctgggcgatctatttaacttttgttttctcacctgtaagctgagacgaaagtacccactttataagattattccaataattagttgaaataatgcatgcagagaattaagcatggtacttgttatttgttaaactagctattaaaatgtgtaaaatataaagtattgtatggattttaggacaatgcaaagactctttgcttgctgcaatagttcggggccctttcagatggctaaaggcagaatttgtatgtgtaaatatggtgtgcttgtctctgctctggatactgagggcttaccctgttattaaacttatttagtaaatattgaactgtcatgaggcctaacatttagttccagttattagataaaacatttgctttgaatggtatttgaattgccaggttctagattattctggttgacaaactcttcgtattttataaagaggctaaaattggtaagctatcacagaacagatgtgccattttcaaggtatattaaaccatgattcactgtaacattgttcctactggcaacaaattcagagcaggctggactttatttggtgaagaaacattgagtggaagagaaatgacattattttatgtatttacattttcaaattactgtggcttaaacctgttcagccaacattacccaccttcagtctgctaaataaatgattcagtacatttctaatttacagaattttttaacaaaagaaaatgtaatttgatagccaaatcaacgttaaacattatacatttaaaaaaccacaggcaaagacacaaacatgatgacactaacttttgttaaagtatgcttacctatggtttcctctgaggcacgttctttcatgctaagcttccaacataatatgaaaatgaaggagatgcattttgcaaagcaaaacagaccttaagcaaaatattatacttctcaaattaacactgttacaaagttttagaatttaataagttcattaatttaaaagtttggatgtctgagtccttctatcccaaaacaagatcttggagggtcttccacagccatgtaataccatggtcacatgaccctttccaaaattattaatctgaatttactatatgaggataaatctatctttttgaaaatatttaggaaaatgagcttggtatttataaaatgaagctctctttgggtggtatcctaagacacgtcaagccaatcagcctgtaactgtgaaaaaaacattggtaggtacaaaagtggggtgggagaggagtgacttaactttgttaagtgatgggaaagaaacactaatagcattatctcaataaaatgtgatttaaaaaaatttaaaatactaaatcattgaactgacaaagaaatataaatcattcagaaataaactcattaggtcatcaaatcctgttaaatctgcaattaggaagagcaaggtgtacaatccatacatttaaactcacaggctcactttgcacaacgtcaatttactccttaatatgttattaatacgcattttccaaaaggatgtattagtaaatggtacacatctacttcttggcaacatcatataacctggtacaacataagcattcttcttatagttaagaaatgtggatggtatcaaaattagaaaaataaatgccctattatgttgtggtcaggtttaaggcatgtgaattttatcttcatacaaaagattaaaatctagatattaaaaagtagtgcagtatcagtgatgctgcctcagttcccaaaatgtcacatcacaaaaatatcccataattgcctgtagtttattccttggctttcctcttttctctctgcatctttgtaacaattttttaaaagtggaaatataattgttggcaatgctaacagctgtagaaatgattacaagatgtggaaaagcataacaggaatgtcaagaatctgtttctggcagtaatatatatggaacattgttcaggacaaaagaggagaaggaagaaaaaaaggagaggggtttatcatctctaagaattttcaaactaaacctcattgcttaataggaaaaaaagattccatatttaaagttaagtcacctctaactactagctaaagcatgacatcaccagcactggagtcagcggaagtgtgtttttgaaggacagtgttgcaggagaatctggacaggttttagagccaggagagagaaaataattctacctctgacagttgaaggaccttaggcaaatcagtttacctctgctagactacactccaaaatttggacattcaaaaatttgatattaataaccacatgaaagtctcgtgttgaggtgaatatgtatttgttggtgaaagatatgttggtttttaaacagacagcactctgcaattgtaggctattgttttgttttgccagttgtcaaattctatccagctatacacacttgtgtggcctcctaatggtgtttttccagtggctaaaggtttatgaataagacacttttcctaatggaattaacccgatgcttttcttaaacatgtaaccttgagttcaccgcaaaaaacaatgcttcgattagagcaatgcatataataaaggttaccctcgtttcttagacactagacatcattcacaaaaagagaactgcttttgaaagggatgtatttgcactggaaagaatagttttctacttctaattataaatgatttattggtgaaagcaaaacaacagcctgtctgagaggcacttctatgagcatcctcacgtgtgatttgcaaggttgaagaagagggaaaaatgcctcaattgtaccaatggtgagaaaacacccaaagtacaaagcaggtttcaaaaaaaccatactcataaccaaggacaataataaagcaatgtgttgacatatactctataagtcttcctccataaatagtttatagaaattttgtaatttctgtaaatgcatcctataataattttgcatcttgctttttttttacatttaatatcaagtagatttctaaagggcaattatttgaaaattatcccaaatacatggggaaatatacatcaagtgaaaaaatgcagtgggtgatagagatatcaggaagcgcctcaaatatttctcatctcgttggagaaaaacaaacatgttctcatttagaatgagtgggagttacctaattgatttaggcctctatatttaacttctagtcaaaaaaggtagttctatctagcaacaatattatggggaacaaaagaaaaaattaactctctaaatttgcagtagggtcttttcttcagaagtaccaaatcccatctattaccagctccatgcttcaggcctaaaatggatctccctgaagcaatgacagaatttttgccaagtgactaggatataaacaccactttggttgcacagtgagacatatgctccaaagaaaactggttcaaaaacaggcaagtgggtttctacagaataaatgagagccctgtcaatggcttcatcttcagggctttgtgtctgtgcttgcgtggtggctcttgtttcatctatggataatggtggcacacagttttcataattccttacattaatgaactgctataaatttgtttttggtattctagagagtcctaacttcagcttctgggcaatgctgaggaggcaccctatattctagacttaccttttgcaaggtgtactctcagcattgtgggcgatttccatgggagaatattctatttaaagaactactgtcccagcataaaacaaaaaatcatttatgaagatgcaggagactcggaaagctctcaattattgtttgcacaagcacaatgtcacagcctcctttccccattccacaagggggtcaggaagagagtactcagctgtgagaaaagacatacagaagaattcatgtggtcatgagagcgaggacatggccgatcccccaaggaggatgtgtcatacacttcatgagcccaagagtgtgctgtagggtctgaagggcaagatgctggttcactgatgtaaaggagagggaaaaaagcttcaaccaactagaaaaacagtctctatgcatgctatttttgattttaaacacaggtatcaattccttctctcagagagtccattttaaaataggatacatttttaaaggaatatttaaaggacacattcattaaaatttattttaaaaacttttcaaaagaaacaaaaggtatgaattttatttaatccttgaggaaatggttcttttctcacacacataaatcactcattttgtttttctttatctcctttattaatctacattagaaaaataaacttttcatacactaagaacaaggaaaccactctcaattgacaaaatgttccaatccaacacaatgattactttcacctttaatttacaggcagccagattcaaaatccttaaagttgcttaaacttaaaaatgacaatgacaacctaaaaggtataatgttgattggaacagacatttaattggaaaattgatgattttccatttccaattaaatctctagatagaaatgaaaaaaattaaaaatcgtatttaagaaaagccaaatcttgggttgtgaggtatctttttaaggatgtttcagcagaaaaaaacaaaggctctcacaattgtgtagctgcctagattaagtgggtatcctgatcaaggagatgggggatgatttggctttagtattccaatgataaagtttataatgagaataacatgttgctacaaaatccagtctcttcctcagatgccttccacagagggcaggaagctttgtcagttttgtttgctgatgatgcctggttccgtcaacaaataacacctgtcacacggtgggtagtcaatatacatttgttgaataaatatgaaaaaaagaaatgtacaatatgtttgtgaagccaactgtgtgtgcattgctattgaggtacacaaaaagtctttgttttaaatttgagaatgaggactttcaatggaatatatctataaaaatgaaaaaaagacattactgtctggacttttgtacagcaagagaagaaaaaccactagccaagagccaactcacctgataggcctggatcaagcatgcagctgtggagaacacccctgggactctaactctggcactctgcaagctgggtacttgggcaggacagcagcagcactcatgaactgggcagcacctgttggtgagggctgatcacatggattctctcatcccagccttacaatcagtccttcaggtacatactttttctgactttgctgatgaggaaactctcttcaagtggtatttaaatttcttctttcattttccttctggtaacaaagaagtctgtggctcaaaagatgtttctctaagaccccatcctattaggtctctgagctgtgggaagtatttatacaattgcttgtgaatataagatccaggaatttccctaagatccctaacaaaattggtgataagtagtcccacatgttaatccagccacccacggatgacagcacttaccatttctttgataaatgtcaaatgcatttgaagtacctacctgaaatatttgtttaaatgctatctaatctattaattttatatatgtgtgagtctgttttgtataccttctgattataggataaatgtaaataaatccaaagagtaatcaaagctaccactttcaagaagccttctttgtagaaccggaagagtcttaaataggcttttcaggtatgcatctcttattatcgctgaactccaagtcctgcaaggcaggcatcatgtgtgggtcacctttacagtaggcacaggccttaaaacagtgacatgcacattgcaggcactccataaatgtttgctgaattggctaaaccttggtttgttcccataatcaaccaccacaaacagcacacagataattacttcttggaaagattccaactagtgtttgatgttacctacgtggtttttctctcaagatcttaagagcagctctgtaggattacattattttctgttttttttttcctttgaccttaatgtcatctacttcaataacagcttcatacaaaattcctaccagcacataccacagcagattcaaggccttgttttaaaaatggtgccagcttctcttaatttggaagatatattgtctctcctgaacatgggctaagaaaatgtataatttggtattaacataagagctgaagacactttaaatgcattgtttcatttttataagataaaaaaaattttaagaatcaaaatgttatcaacagacttgtccttcattaaaaagtaaaactgcatttgcctacattttatgaaagtgtccaattatgaacaattttgaaatgtaacttttaaaaatgtaaacagcaaaaatgttgtatttaaaataaatctggaaaggcagaaaaacaaaaaatacccagaagacagagtttttggtgaaagttaagatatttcatctttgaacaacttagaatctttcctgcattttatagtctagttccaggcattaatttgaaataaccttggaatcctaaatctaacacccttcggaacaaagtagcttttctcttctgctttatgagcaaatggactaaatactagggaatggtactgtctgggcctttgaaccaagattgaaagagatgaaatcctatatgatatgtataaacattagagaatccattttgatttaataaaaggttgaatttgttctatatcctgtgagaaaatggttcccttttcctgaaaatgttacctcattccaacaatagaaagttggtttttttccagggtgtggtgttggcgggggacagagttgccatgaatatggcatctatgaagactgctgttatattcatttctcaaaatgcactgtggtaggaaattcagaacgcagtgagagaaaataaatgtttgacttcaaaatataaggccgcatttaaagcagaaggtaaagtatagaacagttgacagtataaattctttatctgcaatcttgcagttccctaaatctctgtaacacatcacttttaaaagcctcagataagtggttctataataatttaccaataattcaacccctcaaaagtcttagcaagttaaaccttataatcttacattttagaaatgacccaacttgatccttttattcttcagaatatctctctcaaattttcatttgtttttcattaattgatgaataatgagacattttaggtacctgtccacaaagaaatgaaattttcactttccaggaacctaacaaatgaaaagatagaaatcaattccaacagaatattaccaaagaaatcttttagaatggactgttaaaattatttatttgtatttatctggctctactatttgtggtacatttccacttcaaagctaaacctcaaataacatcatagtgagtggttgacttcatgtttaactgagatcttgaagactgaaaaagaccacgacaaacacacatctattttcttggctactgcatccgtgttcatcaccattctgatagtctgcaatgtattgcagctcaccctttgggaaggactaaagtagacatctgtttgttctgcttactcagcattcctaccctaattttcctttggagaacccctttattctagaccacgtgaagctaatgccaaaccccattccaggggatgcacctgaatccaacctccatcatctaaacagtgccttctccacgttcagagaagagcaagtgactcaaactgccctcataagaacagacctgggacttctgctgcaaatattgaagagtaagtactcttttttcttgctaggactaagctggtagtaccttctatgaggctatcatatggaaacaacttgtctgaaaatgaagccacaactagaaaacagatcctggtaacccggattgatggatccagccctaccttaaatggcaagacctaacccgaggctttttgcatcaaccaataaagtccttaagccagtttgagttggttttgtcacttgcagctaaaagaattctgactctaacaatgtgacaatagcaaaaataaacataactgcttttgaggtttctaatggattttcctccctatatacatgatttcatttaatcctcacaattcaggaaagcacatatctattaacattaaattaatattcattattttgaacacatgctatgtggataagggatgaggaaagccaaggaagtaatcaacgtgaaatctcacttatatgggagggaagtggaggttacatatctcagggcacttaacagatatcatcaaatgaaagaataaacagtgtgtgggagaggcagtaggtgattcttcatcaattcctggatgaaaaattaggagataatgaactccgaacaggcagcctaatgagaatggctcaagcaacaggacatagagagggagttaggttagacatggggttcttgggaattttcacctcgtgggggggcgggggggtcgtgcagctgttgtcagtgggaaagggaaaaaggaaaaggctgagtttggaaggcagggagggaggagacaatgtgagtcagtgaaaaagggcccttagaatgacaagtctggaccagagagaggctaagactgaaaatacaagttgggtaaccactggcatacagatggcagttcaggcttgggcactgcccaccagagcctcagcatgaagagaagagggggaggctggccaccacctccctctaggtaatcgtcatcctgatgctgagctcctgaaaacaggctctttcactcgccccatctcttgctcttgattgcaacccggcattcaggaggcaccctgtaatatctgtggagtgaccgacaacacagcgccagggcactgagaagatcccagggcgccagggactggttctacaagggtgcccctcccggtcccctccagcgcgccgccagagctgccagtcttggctgctacacgggaggcagcctcattatgcagctctcacctcttaaattagttcatgctctcacattaggtgtaatcacagcttgcaacgctttctggggatgtctcagaaagatctgagttgaaaaaatatttttgtgtcattttaatttaaagtaaaattgctgcttcttccccgcccctttctttcctcctggcccacccagcgaccctggccggccgtgctcaacgggggcgggggtcggaggtgagatttcctccacataattccttaaacagctatcaactaagtctcaaagaaaaaaaaaagagatctagaagcagagacgtggctgctggcgatcccaaagctggtgttcgctcttgggggagagcgtaccctgggggaggccgggaggccgggccagaggctagcccagaggcagagggcaggagcgctcagccggcgccccgcgtctctccagctcccgacgctgcgctggctccgctgagcacgccaggatcaaggtcgcctggtggggaccggagcgccaggagcctgtgggaagcgttccagccggcctctgactgggatccggcgccgcgtttctgctttggacttgactgacaggtccccccgccctcccgccgccctactaccagcctgggttcatccttcagggctacgtctaccgcacccgggctggaaagcctggagcgcgcccttcctctcctcatcttctcagctctcctttctccctgccacttggcaaagctgcattttgactttcacgttttggactacgtgtgtgtagttccaagtccatgcgtggcacgaaaatccacttagggtaaaaattattctcgaaaaatcgcccatctcaggatctggtgtctacactcaaggctaggaggtgcaggtacgggtgcgtaaagcatgccgtaagggtgcacagtaaataaaaagtacggatgcaaaatgtaaattttaagtgcaaaacagaaaagcagtactcgttgccgccccgcacgctgggttttaaggggcacgaaggtgggcctcggctgcttttgctcagccccgcgtcctcagcgcccggcccagtacccggtactccgtaggggttcaatgatctcccctgaataagtgaacgaattaacaaatgaatgaatgaccgctcgatccgacctccgcggccggcagagcagtcgctggagaggcgggagagagcgagaggccaagctccaccatcgcggccgccggctggggcagagggacacggagacactcggcgccccggctccgcaccgagtccccg

SEQ ID NO: 17608 - RNA, 14211 nt, Homo sapiens
  source 1..14211: mol_type = other RNA
tcaggccaggcacagtggctcatgcctgtagtcccagcactttgggaggccgaggtgggcagatccacgaggtcaggagatcaagaccatcctaacatggtaaaaccccatctctactaacaatacaaaaaattagtcaggtgtggtggcacgtgcctgtagtcccagctactcaggaggctgaggcaggagaatcgcttgaacctgggaggcggaggttgcagtgagccgagattgtgccactgcaccctagcctaggcaacagagcaagactctgtctcaaaaaaaataaaaaaaaaaaaaagagagaaagagagagagagatgaggagttgctgcactgctgggtgtggagagccgaggaggattcaaagatggtcctgaagtcccagctggaagaagtaggcggcagcaatgtttttaatactgtaaattcatcacgtagcacaggtttggggtggagaaagaaaaattgcattggcttcagggcatgcccagatctttcctcatcttaggcgtttgctaatacatgcattttctaagctgatgtcttgcgtttaatcactgctccattcaaaagagagaaggaggttgtttcaaacctagttgatatcatttgacttccatgctattcacagggctattttatttgaaacaggtataccacagccttaaattgcaagttaatccaggatgttcctaggttggcagttaggaacatgtaattctttggaagggctaaaagtcagctctttaaattatctccatatgaaccttctctccaccttagggtggatccacttatttagtccactgccagtaccacactagaacccgggtggtcactggactccagaaacaacagtagccctctctctgttctgtctctttttgactatctctattctgttcctgaccctgatttctcctgccaagctcaattttgacagctgacaacggcaagccatggcttcccaaaacattattttcaggtcaacttataaatttcaagaacacatttggctccgcttcctgtggtactaagcctacttcttgacagcatttgcctttgttgtaaatagcaaagttcttctagttggatttttgctaagaagtgtgtggatgtggcatgtgacgacatctttagcttggattctagaaaggcactaccattgtgcatttggctaaaggaaacacattttacccgtgaatgccttctatttacaaatgctcagctagcacacaaagctaagtacaagcaataagtactatcctacaatgttactcatttctgaaagcacaaaatgatgactggtatagctttggagatgttttctggaaacccaataaaggaacagatctttgttattccacacctacaaagtcagaagatgcacagtcttttattcatgtttgaacaagcttccttcttgaacaatcaactataaagtgatgtgattctctactagaccaggaactccttgaggacagaatgagggtctaatccatattctaaatccacaccacctggcacaatacatgttgcatggttagggtcaactaagagttggttgaattaatcaataacacacagcaagagaattcacaaagagaggggagtaatcccccagcctcaatcactcggcaagtggaatcgctgggcactgattccagctctgtctcagtgcttgagacagagctgaatgtaatgtgaacatttcaaatgaacaggaaaactagactcacggataagcagtgtagtcatcaagacaacactgtcttggaggtttttctgaagttaaaaccatgctacataagcaataaattatgaaggctgagcatgtgaataaaatttaatgttgtcataaattttataacaaagttaatctgacacatttaatgacatgcataatcattagtatgcagcactgtaatcagacattgataataagcagttcacaccagtgactgtaagagtctttacttgtgttcagccaagccaactgcttggtatatttttctcccttcttagtcgttagttttccatacctacaataactatcagtggtgatgggcttctctgaccatgtgaataatttaatcctcaatgcacagatacagaaacccttgctgaagacagtgtggagcagagaaggctgtctccactccttccacctgaaacacctctgcagatggatatgggagctctgcctacagcccttggacctaaccacttcagtgtgttccagtgagtgtctggacctcggcctgaaagatttttccgaaactaaagaaaatttctctgacctaaagaccttaacctccaccccagaagctctcaccaaggactacagggaactggtggggaaaatccttatcccttactcctcaaggcacagggcagtaatgctgaggcttgtgcgccacacttgctcccagaggtccccagcgggctacctgcggtggtgaatgacctcctaacacgccccttgacggccttcctttccttgcctcacttctccactctcctaccagcattgcagggttcacatcccaaatataccactggcacttgaatcctggtctccaggtctgtttctggaaaaacccaagtaagacattgccccagtaatggggctagatgtctgaggcttcctcaagtatctacctcgaaagctcttactgctgtacacacatgcacatacacacacgtgcgtacaaccagtcacatctaagcaccccgaataccagcctgttgaaggtagcagagagctgcactataagccaaggctgctcccaagagccgctccatcactgaattggcgccccagcaagatgaaggaatgtaatcattggaaggatggagaatgttctctgaatcactgacaaattggaaggggtggagggcaagagtccacctggtggagagatggaaagagcgagagagcctggaatgataatgccattgcttagaaaaggctgctccagatgccatatctacagaaattgtacagcccaaacatctctgagcaataggtctctggtagtcttgatgtctagaccaacaattcccagttcattcttctcagggaaggagccaggatagtccagagactctcattctgctgttagattgaaagggttaggcacaacagccttggcaaagtcacaagggcaaattcacactaaagtgtaaatgacccacaactcctcttctatttttaggttggggaggtgctttagaacataaggaggaactaaagaatattcctgttacatacaaggcagagaaaagggaaactagtggtgacaagacaaatcatccctttgacatttggctggctctacctattacagctctgggggtgaggtgggaacaaaaagatgctgtgtaaagaagtatcttatgccatccctactgtagtgaggtgcagtttagaggggacactgatcaagcagagacccagagtgtttcgttccaagccagaaacagaaatgtataaaacacagcctttccagcatcagaaatgagtagtggtagtggagaactacccaaaacaggaaagaggaccacgtgaggtagagtgtcaaggccctacattccagtgcctctgctcatgactgtaattttgggtaggtcacttaaagtctctggacctcagttttgccatctgtgaaatagggataatactatccagcataaaattggttatgaggctcatgtagggcctgcctgggatgatgtgttgctaatggttaagaacacaacttctggggtctgactggacaggctgaaatccctgcttaacacgttccagcagagccctgggcgatctatttaacttttgttttctcacctgtaagctgagacgaaagtacccactttataagattattccaataattagttgaaataatgcatgcagagaattaagcatggtacttgttatttgttaaactagctattaaaatgtgtaaaatataaagtattgtatggattttaggacaatgcaaagactctttgcttgctgcaatagttcggggccctttcagatggctaaaggcagaatttgtatgtgtaaatatggtgtgcttgtctctgctctggatactgagggcttaccctgttattaaacttatttagtaaatattgaactgtcatgaggcctaacatttagttccagttattagataaaacatttgctttgaatggtatttgaattgccaggttctagattattctggttgacaaactcttcgtattttataaagaggctaaaattggtaagctatcacagaacagatgtgccattttcaaggtatattaaaccatgattcactgtaacattgttcctactggcaacaaattcagagcaggctggactttatttggtgaagaaacattgagtggaagagaaatgacattattttatgtatttacattttcaaattactgtggcttaaacctgttcagccaacattacccaccttcagtctgctaaataaatgattcagtacatttctaatttacagaattttttaacaaaagaaaatgtaatttgatagccaaatcaacgttaaacattatacatttaaaaaaccacaggcaaagacacaaacatgatgacactaacttttgttaaagtatgcttacctatggtttcctctgaggcacgttctttcatgctaagcttccaacataatatgaaaatgaaggagatgcattttgcaaagcaaaacagaccttaagcaaaatattatacttctcaaattaacactgttacaaagttttagaatttaataagttcattaatttaaaagtttggatgtctgagtccttctatcccaaaacaagatcttggagggtcttccacagccatgtaataccatggtcacatgaccctttccaaaattattaatctgaatttactatatgaggataaatctatctttttgaaaatatttaggaaaatgagcttggtatttataaaatgaagctctctttgggtggtatcctaagacacgtcaagccaatcagcctgtaactgtgaaaaaaacattggtaggtacaaaagtggggtgggagaggagtgacttaactttgttaagtgatgggaaagaaacactaatagcattatctcaataaaatgtgatttaaaaaaatttaaaatactaaatcattgaactgacaaagaaatataaatcattcagaaataaactcattaggtcatcaaatcctgttaaatctgcaattaggaagagcaaggtgtacaatccatacatttaaactcacaggctcactttgcacaacgtcaatttactccttaatatgttattaatacgcattttccaaaaggatgtattagtaaatggtacacatctacttcttggcaacatcatataacctggtacaacataagcattcttcttatagttaagaaatgtggatggtatcaaaattagaaaaataaatgccctattatgttgtggtcaggtttaaggcatgtgaattttatcttcatacaaaagattaaaatctagatattaaaaagtagtgcagtatcagtgatgctgcctcagttcccaaaatgtcacatcacaaaaatatcccataattgcctgtagtttattccttggctttcctcttttctctctgcatctttgtaacaattttttaaaagtggaaatataattgttggcaatgctaacagctgtagaaatgattacaagatgtggaaaagcataacaggaatgtcaagaatctgtttctggcagtaatatatatggaacattgttcaggacaaaagaggagaaggaagaaaaaaaggagaggggtttatcatctctaagaattttcaaactaaacctcattgcttaataggaaaaaaagattccatatttaaagttaagtcacctctaactactagctaaagcatgacatcaccagcactggagtcagcggaagtgtgtttttgaaggacagtgttgcaggagaatctggacaggttttagagccaggagagagaaaataattctacctctgacagttgaaggaccttaggcaaatcagtttacctctgctagactacactccaaaatttggacattcaaaaatttgatattaataaccacatgaaagtctcgtgttgaggtgaatatgtatttgttggtgaaagatatgttggtttttaaacagacagcactctgcaattgtaggctattgttttgttttgccagttgtcaaattctatccagctatacacacttgtgtggcctcctaatggtgtttttccagtggctaaaggtttatgaataagacacttttcctaatggaattaacccgatgcttttcttaaacatgtaaccttgagttcaccgcaaaaaacaatgcttcgattagagcaatgcatataataaaggttaccctcgtttcttagacactagacatcattcacaaaaagagaactgcttttgaaagggatgtatttgcactggaaagaatagttttctacttctaattataaatgatttattggtgaaagcaaaacaacagcctgtctgagaggcacttctatgagcatcctcacgtgtgatttgcaaggttgaagaagagggaaaaatgcctcaattgtaccaatggtgagaaaacacccaaagtacaaagcaggtttcaaaaaaaccatactcataaccaaggacaataataaagcaatgtgttgacatatactctataagtcttcctccataaatagtttatagaaattttgtaatttctgtaaatgcatcctataataattttgcatcttgctttttttttacatttaatatcaagtagatttctaaagggcaattatttgaaaattatcccaaatacatggggaaatatacatcaagtgaaaaaatgcagtgggtgatagagatatcaggaagcgcctcaaatatttctcatctcgttggagaaaaacaaacatgttctcatttagaatgagtgggagttacctaattgatttaggcctctatatttaacttctagtcaaaaaaggtagttctatctagcaacaatattatggggaacaaaagaaaaaattaactctctaaatttgcagtagggtcttttcttcagaagtaccaaatcccatctattaccagctccatgcttcaggcctaaaatggatctccctgaagcaatgacagaatttttgccaagtgactaggatataaacaccactttggttgcacagtgagacatatgctccaaagaaaactggttcaaaaacaggcaagtgggtttctacagaataaatgagagccctgtcaatggcttcatcttcagggctttgtgtctgtgcttgcgtggtggctcttgtttcatctatggataatggtggcacacagttttcataattccttacattaatgaactgctataaatttgtttttggtattctagagagtcctaacttcagcttctgggcaatgctgaggaggcaccctatattctagacttaccttttgcaaggtgtactctcagcattgtgggcgatttccatgggagaatattctatttaaagaactactgtcccagcataaaacaaaaaatcatttatgaagatgcaggagactcggaaagctctcaattattgtttgcacaagcacaatgtcacagcctcctttccccattccacaagggggtcaggaagagagtactcagctgtgagaaaagacatacagaagaattcatgtggtcatgagagcgaggacatggccgatcccccaaggaggatgtgtcatacacttcatgagcccaagagtgtgctgtagggtctgaagggcaagatgctggttcactgatgtaaaggagagggaaaaaagcttcaaccaactagaaaaacagtctctatgcatgctatttttgattttaaacacaggtatcaattccttctctcagagagtccattttaaaataggatacatttttaaaggaatatttaaaggacacattcattaaaatttattttaaaaacttttcaaaagaaacaaaaggtatgaattttatttaatccttgaggaaatggttcttttctcacacacataaatcactcattttgtttttctttatctcctttattaatctacattagaaaaataaacttttcatacactaagaacaaggaaaccactctcaattgacaaaatgttccaatccaacacaatgattactttcacctttaatttacaggcagccagattcaaaatccttaaagttgcttaaacttaaaaatgacaatgacaacctaaaaggtataatgttgattggaacagacatttaattggaaaattgatgattttccatttccaattaaatctctagatagaaatgaaaaaaattaaaaatcgtatttaagaaaagccaaatcttgggttgtgaggtatctttttaaggatgtttcagcagaaaaaaacaaaggctctcacaattgtgtagctgcctagattaagtgggtatcctgatcaaggagatgggggatgatttggctttagtattccaatgataaagtttataatgagaataacatgttgctacaaaatccagtctcttcctcagatgccttccacagagggcaggaagctttgtcagttttgtttgctgatgatgcctggttccgtcaacaaataacacctgtcacacggtgggtagtcaatatacatttgttgaataaatatgaaaaaaagaaatgtacaatatgtttgtgaagccaactgtgtgtgcattgctattgaggtacacaaaaagtctttgttttaaatttgagaatgaggactttcaatggaatatatctgataggcctggatcaagcatgcagctgtggagaacacccctgggactctaactctggcactctgcaagctgggtacttgggcaggacagcagcagcactcatgaactgggcagcaccgactggcaaacctccccctgaagatggagaaggaggaaggagtgttactggaatgagagcttgagtccaggggaggaggatgggctgctgaggaggcgacaccatcctgaaagaagaatcctctgccagaggcttttcagggtcatttcttcacactctctgcagggaagcacggagacagcaggaagaaatatcctaacctcactctcttccctctacaggtgcttccattggccaaatccacccagaggccagttggtggcgatcagctctcttcaagtggtatttaaatttcttctttcattttccttctggtaacaaagaagtctgtggctcaaaagatgtttctctaagaccccatcctattaggtctctgagctgtgggaagtatttatacaattgcttgtgaatataagatccaggaatttccctaagatccctaacaaaattggtgataagtagtcccacatgttaatccagccacccacggatgacagcacttaccatttctttgataaatgtcaaatgcatttgaagtacctacctgaaatatttgtttaaatgctatctaatctattaattttatatatgtgtgagtctgttttgtataccttctgattataggataaatgtaaataaatccaaagagtaatcaaagctaccactttcaagaagccttctttgtagaaccggaagagtcttaaataggcttttcaggtatgcatctcttattatcgctgaactccaagtcctgcaaggcaggcatcatgtgtgggtcacctttacagtaggcacaggccttaaaacagtgacatgcacattgcaggcactccataaatgtttgctgaattggctaaaccttggtttgttcccataatcaaccaccacaaacagcacacagataattacttcttggaaagattccaactagtgtttgatgttacctacgtggtttttctctcaagatcttaagagcagctctgtaggattacattattttctgttttttttttcctttgaccttaatgtcatctacttcaataacagcttcatacaaaattcctaccagcacataccacagcagattcaaggccttgttttaaaaatggtgccagcttctcttaatttggaagatatattgtctctcctgaacatgggctaagaaaatgtataatttggtattaacataagagctgaagacactttaaatgcattgtttcatttttataagataaaaaaaattttaagaatcaaaatgttatcaacagacttgtccttcattaaaaagtaaaactgcatttgcctacattttatgaaagtgtccaattatgaacaattttgaaatgtaacttttaaaaatgtaaacagcaaaaatgttgtatttaaaataaatctggaaaggcagaaaaacaaaaaatacccagaagacagagtttttggtgaaagttaagatatttcatctttgaacaacttagaatctttcctgcattttatagtctagttccaggcattaatttgaaataaccttggaatcctaaatctaacacccttcggaacaaagtagcttttctcttctgctttatgagcaaatggactaaatactagggaatggtactgtctgggcctttgaaccaagattgaaagagatgaaatcctatatgatatgtataaacattagagaatccattttgatttaataaaaggttgaatttgttctatatcctgtgagaaaatggttcccttttcctgaaaatgttacctcattccaacaatagaaagttggtttttttccagggtgtggtgttggcgggggacagagttgccatgaatatggcatctatgaagactgctgttatattcatttctcaaaatgcactgtggtaggaaattcagaacgcagtgagagaaaataaatgtttgacttcaaaatataaggccgcatttaaagcagaaggtaaagtatagaacagttgacagtataaattctttatctgcaatcttgcagttccctaaatctctgtaacacatcacttttaaaagcctcagataagtggttctataataatttaccaataattcaacccctcaaaagtcttagcaagttaaaccttataatcttacattttagaaatgacccaacttgatccttttattcttcagaatatctctctcaaattttcatttgtttttcattaattgatgaataatgagacattttaggtacctgtccacaaagaaatgaaattttcactttccaggaacctaacaaatgaaaagatagaaatcaattccaacagaatattaccaaagaaatcttttagaatggactgttaaaattatttatttgtatttatctggctctactatttgtggtacatttccacttcaaagctaaacctcaaataacatcatagtgagtggttgacttcatgtttaactgagatcttgaagactgaaaaagaccacgacaaacacacatctattttcttggctactgcatccgtgttcatcaccattctgatagtctgcaatgtattgcagctcaccctttgggaaggactaaagtagacatctgtttgttctgcttactcagcattcctaccctaattttcctttggagaacccctttattctagaccacgtgaagctaatgccaaaccccattccaggggatgcacctgaatccaacctccatcatctaaacagtgccttctccacgttcagagaagagcaagtgactcaaactgccctcataagaacagacctgggacttctgctgcaaatattgaagagtaagtactcttttttcttgctaggactaagctggtagtaccttctatgaggctatcatatggaaacaacttgtctgaaaatgaagccacaactagaaaacagatcctggtaacccggattgatggatccagccctaccttaaatggcaagacctaacccgaggctttttgcatcaaccaataaagtccttaagccagtttgagttggttttgtcacttgcagctaaaagaattctgactctaacaatgtgacaatagcaaaaataaacataactgcttttgaggtttctaatggattttcctccctatatacatgatttcatttaatcctcacaattcaggaaagcacatatctattaacattaaattaatattcattattttgaacacatgctatgtggataagggatgaggaaagccaaggaagtaatcaacgtgaaatctcacttatatgggagggaagtggaggttacatatctcagggcacttaacagatatcatcaaatgaaagaataaacagtgtgtgggagaggcagtaggtgattcttcatcaattcctggatgaaaaattaggagataatgaactccgaacaggcagcctaatgagaatggctcaagcaacaggacatagagagggagttaggttagacatggggttcttgggaattttcacctcgtgggggggcgggggggtcgtgcagctgttgtcagtgggaaagggaaaaaggaaaaggctgagtttggaaggcagggagggaggagacaatgtgagtcagtgaaaaagggcccttagaatgacaagtctggaccagagagaggctaagactgaaaatacaagttgggtaaccactggcatacagatggcagttcaggcttgggcactgcccaccagagcctcagcatgaagagaagagggggaggctggccaccacctccctctaggtaatcgtcatcctgatgctgagctcctgaaaacaggctctttcactcgccccatctcttgctcttgattgcaacccggcattcaggaggcaccctgtaatatctgtggagtgaccgacaacacagcgccagggcactgagaagatcccagggcgccagggactggttctacaagggtgcccctcccggtcccctccagcgcgccgccagagctgccagtcttggctgctacacgggaggcagcctcattatgcagctctcacctcttaaattagttcatgctctcacattaggtgtaatcacagcttgcaacgctttctggggatgtctcagaaagatctgagttgaaaaaatatttttgtgtcattttaatttaaagtaaaattgctgcttcttccccgcccctttctttcctcctggcccacccagcgaccctggccggccgtgctcaacgggggcgggggtcggaggtgagatttcctccacataattccttaaacagctatcaactaagtctcaaagaaaaaaaaaagagatctagaagcagagacgtggctgctggcgatcccaaagctggtgttcgctcttgggggagagcgtaccctgggggaggccgggaggccgggccagaggctagcccagaggcagagggcaggagcgctcagccggcgccccgcgtctctccagctcccgacgctgcgctggctccgctgagcacgccaggatcaaggtcgcctggtggggaccggagcgccaggagcctgtgggaagcgttccagccggcctctgactgggatccggcgccgcgtttctgctttggacttgactgacaggtccccccgccctcccgccgccctactaccagcctgggttcatccttcagggctacgtctaccgcacccgggctggaaagcctggagcgcgcccttcctctcctcatcttctcagctctcctttctccctgccacttggcaaagctgcattttgactttcacgttttggactacgtgtgtgtagttccaagtccatgcgtggcacgaaaatccacttagggtaaaaattattctcgaaaaatcgcccatctcaggatctggtgtctacactcaaggctaggaggtgcaggtacgggtgcgtaaagcatgccgtaagggtgcacagtaaataaaaagtacggatgcaaaatgtaaattttaagtgcaaaacagaaaagcagtactcgttgccgccccgcacgctgggttttaaggggcacgaaggtgggcctcggctgcttttgctcagccccgcgtcctcagcgcccggcccagtacccggtactccgtaggggttcaatgatctcccctgaataagtgaacgaattaacaaatgaatgaatgaccgctcgatccgacctccgcggccggcagagcagtcgctggagaggcgggagagagcgagaggccaagctccaccatcgcggccgccggctggggcagagggacacggagacactcggcgccccggctccgcaccgagtccccg

SEQ ID NO: 17609 - RNA, 13941 nt, Homo sapiens
  source 1..13941: mol_type = other RNA
tcaggccaggcacagtggctcatgcctgtagtcccagcactttgggaggccgaggtgggcagatccacgaggtcaggagatcaagaccatcctaacatggtaaaaccccatctctactaacaatacaaaaaattagtcaggtgtggtggcacgtgcctgtagtcccagctactcaggaggctgaggcaggagaatcgcttgaacctgggaggcggaggttgcagtgagccgagattgtgccactgcaccctagcctaggcaacagagcaagactctgtctcaaaaaaaataaaaaaaaaaaaaagagagaaagagagagagagatgaggagttgctgcactgctgggtgtggagagccgaggaggattcaaagatggtcctgaagtcccagctggaagaagtaggcggcagcaatgtttttaatactgtaaattcatcacgtagcacaggtttggggtggagaaagaaaaattgcattggcttcagggcatgcccagatctttcctcatcttaggcgtttgctaatacatgcattttctaagctgatgtcttgcgtttaatcactgctccattcaaaagagagaaggaggttgtttcaaacctagttgatatcatttgacttccatgctattcacagggctattttatttgaaacaggtataccacagccttaaattgcaagttaatccaggatgttcctaggttggcagttaggaacatgtaattctttggaagggctaaaagtcagctctttaaattatctccatatgaaccttctctccaccttagggtggatccacttatttagtccactgccagtaccacactagaacccgggtggtcactggactccagaaacaacagtagccctctctctgttctgtctctttttgactatctctattctgttcctgaccctgatttctcctgccaagctcaattttgacagctgacaacggcaagccatggcttcccaaaacattattttcaggtcaacttataaatttcaagaacacatttggctccgcttcctgtggtactaagcctacttcttgacagcatttgcctttgttgtaaatagcaaagttcttctagttggatttttgctaagaagtgtgtggatgtggcatgtgacgacatctttagcttggattctagaaaggcactaccattgtgcatttggctaaaggaaacacattttacccgtgaatgccttctatttacaaatgctcagctagcacacaaagctaagtacaagcaataagtactatcctacaatgttactcatttctgaaagcacaaaatgatgactggtatagctttggagatgttttctggaaacccaataaaggaacagatctttgttattccacacctacaaagtcagaagatgcacagtcttttattcatgtttgaacaagcttccttcttgaacaatcaactataaagtgatgtgattctctactagaccaggaactccttgaggacagaatgagggtctaatccatattctaaatccacaccacctggcacaatacatgttgcatggttagggtcaactaagagttggttgaattaatcaataacacacagcaagagaattcacaaagagaggggagtaatcccccagcctcaatcactcggcaagtggaatcgctgggcactgattccagctctgtctcagtgcttgagacagagctgaatgtaatgtgaacatttcaaatgaacaggaaaactagactcacggataagcagtgtagtcatcaagacaacactgtcttggaggtttttctgaagttaaaaccatgctacataagcaataaattatgaaggctgagcatgtgaataaaatttaatgttgtcataaattttataacaaagttaatctgacacatttaatgacatgcataatcattagtatgcagcactgtaatcagacattgataataagcagttcacaccagtgactgtaagagtctttacttgtgttcagccaagccaactgcttggtatatttttctcccttcttagtcgttagttttccatacctacaataactatcagtggtgatgggcttctctgaccatgtgaataatttaatcctcaatgcacagatacagaaacccttgctgaagacagtgtggagcagagaaggctgtctccactccttccacctgaaacacctctgcagatggatatgggagctctgcctacagcccttggacctaaccacttcagtgtgttccagtgagtgtctggacctcggcctgaaagatttttccgaaactaaagaaaatttctctgacctaaagaccttaacctccaccccagaagctctcaccaaggactacagggaactggtggggaaaatccttatcccttactcctcaaggcacagggcagtaatgctgaggcttgtgcgccacacttgctcccagaggtccccagcgggctacctgcggtggtgaatgacctcctaacacgccccttgacggccttcctttccttgcctcacttctccactctcctaccagcattgcagggttcacatcccaaatataccactggcacttgaatcctggtctccaggtctgtttctggaaaaacccaagtaagacattgccccagtaatggggctagatgtctgaggcttcctcaagtatctacctcgaaagctcttactgctgtacacacatgcacatacacacacgtgcgtacaaccagtcacatctaagcaccccgaataccagcctgttgaaggtagcagagagctgcactataagccaaggctgctcccaagagccgctccatcactgaattggcgccccagcaagatgaaggaatgtaatcattggaaggatggagaatgttctctgaatcactgacaaattggaaggggtggagggcaagagtccacctggtggagagatggaaagagcgagagagcctggaatgataatgccattgcttagaaaaggctgctccagatgccatatctacagaaattgtacagcccaaacatctctgagcaataggtctctggtagtcttgatgtctagaccaacaattcccagttcattcttctcagggaaggagccaggatagtccagagactctcattctgctgttagattgaaagggttaggcacaacagccttggcaaagtcacaagggcaaattcacactaaagtgtaaatgacccacaactcctcttctatttttaggttggggaggtgctttagaacataaggaggaactaaagaatattcctgttacatacaaggcagagaaaagggaaactagtggtgacaagacaaatcatccctttgacatttggctggctctacctattacagctctgggggtgaggtgggaacaaaaagatgctgtgtaaagaagtatcttatgccatccctactgtagtgaggtgcagtttagaggggacactgatcaagcagagacccagagtgtttcgttccaagccagaaacagaaatgtataaaacacagcctttccagcatcagaaatgagtagtggtagtggagaactacccaaaacaggaaagaggaccacgtgaggtagagtgtcaaggccctacattccagtgcctctgctcatgactgtaattttgggtaggtcacttaaagtctctggacctcagttttgccatctgtgaaatagggataatactatccagcataaaattggttatgaggctcatgtagggcctgcctgggatgatgtgttgctaatggttaagaacacaacttctggggtctgactggacaggctgaaatccctgcttaacacgttccagcagagccctgggcgatctatttaacttttgttttctcacctgtaagctgagacgaaagtacccactttataagattattccaataattagttgaaataatgcatgcagagaattaagcatggtacttgttatttgttaaactagctattaaaatgtgtaaaatataaagtattgtatggattttaggacaatgcaaagactctttgcttgctgcaatagttcggggccctttcagatggctaaaggcagaatttgtatgtgtaaatatggtgtgcttgtctctgctctggatactgagggcttaccctgttattaaacttatttagtaaatattgaactgtcatgaggcctaacatttagttccagttattagataaaacatttgctttgaatggtatttgaattgccaggttctagattattctggttgacaaactcttcgtattttataaagaggctaaaattggtaagctatcacagaacagatgtgccattttcaaggtatattaaaccatgattcactgtaacattgttcctactggcaacaaattcagagcaggctggactttatttggtgaagaaacattgagtggaagagaaatgacattattttatgtatttacattttcaaattactgtggcttaaacctgttcagccaacattacccaccttcagtctgctaaataaatgattcagtacatttctaatttacagaattttttaacaaaagaaaatgtaatttgatagccaaatcaacgttaaacattatacatttaaaaaaccacaggcaaagacacaaacatgatgacactaacttttgttaaagtatgcttacctatggtttcctctgaggcacgttctttcatgctaagcttccaacataatatgaaaatgaaggagatgcattttgcaaagcaaaacagaccttaagcaaaatattatacttctcaaattaacactgttacaaagttttagaatttaataagttcattaatttaaaagtttggatgtctgagtccttctatcccaaaacaagatcttggagggtcttccacagccatgtaataccatggtcacatgaccctttccaaaattattaatctgaatttactatatgaggataaatctatctttttgaaaatatttaggaaaatgagcttggtatttataaaatgaagctctctttgggtggtatcctaagacacgtcaagccaatcagcctgtaactgtgaaaaaaacattggtaggtacaaaagtggggtgggagaggagtgacttaactttgttaagtgatgggaaagaaacactaatagcattatctcaataaaatgtgatttaaaaaaatttaaaatactaaatcattgaactgacaaagaaatataaatcattcagaaataaactcattaggtcatcaaatcctgttaaatctgcaattaggaagagcaaggtgtacaatccatacatttaaactcacaggctcactttgcacaacgtcaatttactccttaatatgttattaatacgcattttccaaaaggatgtattagtaaatggtacacatctacttcttggcaacatcatataacctggtacaacataagcattcttcttatagttaagaaatgtggatggtatcaaaattagaaaaataaatgccctattatgttgtggtcaggtttaaggcatgtgaattttatcttcatacaaaagattaaaatctagatattaaaaagtagtgcagtatcagtgatgctgcctcagttcccaaaatgtcacatcacaaaaatatcccataattgcctgtagtttattccttggctttcctcttttctctctgcatctttgtaacaattttttaaaagtggaaatataattgttggcaatgctaacagctgtagaaatgattacaagatgtggaaaagcataacaggaatgtcaagaatctgtttctggcagtaatatatatggaacattgttcaggacaaaagaggagaaggaagaaaaaaaggagaggggtttatcatctctaagaattttcaaactaaacctcattgcttaataggaaaaaaagattccatatttaaagttaagtcacctctaactactagctaaagcatgacatcaccagcactggagtcagcggaagtgtgtttttgaaggacagtgttgcaggagaatctggacaggttttagagccaggagagagaaaataattctacctctgacagttgaaggaccttaggcaaatcagtttacctctgctagactacactccaaaatttggacattcaaaaatttgatattaataaccacatgaaagtctcgtgttgaggtgaatatgtatttgttggtgaaagatatgttggtttttaaacagacagcactctgcaattgtaggctattgttttgttttgccagttgtcaaattctatccagctatacacacttgtgtggcctcctaatggtgtttttccagtggctaaaggtttatgaataagacacttttcctaatggaattaacccgatgcttttcttaaacatgtaaccttgagttcaccgcaaaaaacaatgcttcgattagagcaatgcatataataaaggttaccctcgtttcttagacactagacatcattcacaaaaagagaactgcttttgaaagggatgtatttgcactggaaagaatagttttctacttctaattataaatgatttattggtgaaagcaaaacaacagcctgtctgagaggcacttctatgagcatcctcacgtgtgatttgcaaggttgaagaagagggaaaaatgcctcaattgtaccaatggtgagaaaacacccaaagtacaaagcaggtttcaaaaaaaccatactcataaccaaggacaataataaagcaatgtgttgacatatactctataagtcttcctccataaatagtttatagaaattttgtaatttctgtaaatgcatcctataataattttgcatcttgctttttttttacatttaatatcaagtagatttctaaagggcaattatttgaaaattatcccaaatacatggggaaatatacatcaagtgaaaaaatgcagtgggtgatagagatatcaggaagcgcctcaaatatttctcatctcgttggagaaaaacaaacatgttctcatttagaatgagtgggagttacctaattgatttaggcctctatatttaacttctagtcaaaaaaggtagttctatctagcaacaatattatggggaacaaaagaaaaaattaactctctaaatttgcagtagggtcttttcttcagaagtaccaaatcccatctattaccagctccatgcttcaggcctaaaatggatctccctgaagcaatgacagaatttttgccaagtgactaggatataaacaccactttggttgcacagtgagacatatgctccaaagaaaactggttcaaaaacaggcaagtgggtttctacagaataaatgagagccctgtcaatggcttcatcttcagggctttgtgtctgtgcttgcgtggtggctcttgtttcatctatggataatggtggcacacagttttcataattccttacattaatgaactgctataaatttgtttttggtattctagagagtcctaacttcagcttctgggcaatgctgaggaggcaccctatattctagacttaccttttgcaaggtgtactctcagcattgtgggcgatttccatgggagaatattctatttaaagaactactgtcccagcataaaacaaaaaatcatttatgaagatgcaggagactcggaaagctctcaattattgtttgcacaagcacaatgtcacagcctcctttccccattccacaagggggtcaggaagagagtactcagctgtgagaaaagacatacagaagaattcatgtggtcatgagagcgaggacatggccgatcccccaaggaggatgtgtcatacacttcatgagcccaagagtgtgctgtagggtctgaagggcaagatgctggttcactgatgtaaaggagagggaaaaaagcttcaaccaactagaaaaacagtctctatgcatgctatttttgattttaaacacaggtatcaattccttctctcagagagtccattttaaaataggatacatttttaaaggaatatttaaaggacacattcattaaaatttattttaaaaacttttcaaaagaaacaaaaggtatgaattttatttaatccttgaggaaatggttcttttctcacacacataaatcactcattttgtttttctttatctcctttattaatctacattagaaaaataaacttttcatacactaagaacaaggaaaccactctcaattgacaaaatgttccaatccaacacaatgattactttcacctttaatttacaggcagccagattcaaaatccttaaagttgcttaaacttaaaaatgacaatgacaacctaaaaggtataatgttgattggaacagacatttaattggaaaattgatgattttccatttccaattaaatctctagatagaaatgaaaaaaattaaaaatcgtatttaagaaaagccaaatcttgggttgtgaggtatctttttaaggatgtttcagcagaaaaaaacaaaggctctcacaattgtgtagctgcctagattaagtgggtatcctgatcaaggagatgggggatgatttggctttagtattccaatgataaagtttataatgagaataacatgttgctacaaaatccagtctcttcctcagatgccttccacagagggcaggaagctttgtcagttttgtttgctgatgatgcctggttccgtcaacaaataacacctgtcacacggtgggtagtcaatatacatttgttgaataaatatgaaaaaaagaaatgtacaatatgtttgtgaagccaactgtgtgtgcattgctattgaggtacacaaaaagtctttgttttaaatttgagaatgaggactttcaatggaatatatctgataggcctggatcaagcatgcagctgtggagaacacccctgggactctaactctggcactctgcaagctgggtacttgggcaggacagcagcagcactcatgaactgggcagcacctctcttcaagtggtatttaaatttcttctttcattttccttctggtaacaaagaagtctgtggctcaaaagatgtttctctaagaccccatcctattaggtctctgagctgtgggaagtatttatacaattgcttgtgaatataagatccaggaatttccctaagatccctaacaaaattggtgataagtagtcccacatgttaatccagccacccacggatgacagcacttaccatttctttgataaatgtcaaatgcatttgaagtacctacctgaaatatttgtttaaatgctatctaatctattaattttatatatgtgtgagtctgttttgtataccttctgattataggataaatgtaaataaatccaaagagtaatcaaagctaccactttcaagaagccttctttgtagaaccggaagagtcttaaataggcttttcaggtatgcatctcttattatcgctgaactccaagtcctgcaaggcaggcatcatgtgtgggtcacctttacagtaggcacaggccttaaaacagtgacatgcacattgcaggcactccataaatgtttgctgaattggctaaaccttggtttgttcccataatcaaccaccacaaacagcacacagataattacttcttggaaagattccaactagtgtttgatgttacctacgtggtttttctctcaagatcttaagagcagctctgtaggattacattattttctgttttttttttcctttgaccttaatgtcatctacttcaataacagcttcatacaaaattcctaccagcacataccacagcagattcaaggccttgttttaaaaatggtgccagcttctcttaatttggaagatatattgtctctcctgaacatgggctaagaaaatgtataatttggtattaacataagagctgaagacactttaaatgcattgtttcatttttataagataaaaaaaattttaagaatcaaaatgttatcaacagacttgtccttcattaaaaagtaaaactgcatttgcctacattttatgaaagtgtccaattatgaacaattttgaaatgtaacttttaaaaatgtaaacagcaaaaatgttgtatttaaaataaatctggaaaggcagaaaaacaaaaaatacccagaagacagagtttttggtgaaagttaagatatttcatctttgaacaacttagaatctttcctgcattttatagtctagttccaggcattaatttgaaataaccttggaatcctaaatctaacacccttcggaacaaagtagcttttctcttctgctttatgagcaaatggactaaatactagggaatggtactgtctgggcctttgaaccaagattgaaagagatgaaatcctatatgatatgtataaacattagagaatccattttgatttaataaaaggttgaatttgttctatatcctgtgagaaaatggttcccttttcctgaaaatgttacctcattccaacaatagaaagttggtttttttccagggtgtggtgttggcgggggacagagttgccatgaatatggcatctatgaagactgctgttatattcatttctcaaaatgcactgtggtaggaaattcagaacgcagtgagagaaaataaatgtttgacttcaaaatataaggccgcatttaaagcagaaggtaaagtatagaacagttgacagtataaattctttatctgcaatcttgcagttccctaaatctctgtaacacatcacttttaaaagcctcagataagtggttctataataatttaccaataattcaacccctcaaaagtcttagcaagttaaaccttataatcttacattttagaaatgacccaacttgatccttttattcttcagaatatctctctcaaattttcatttgtttttcattaattgatgaataatgagacattttaggtacctgtccacaaagaaatgaaattttcactttccaggaacctaacaaatgaaaagatagaaatcaattccaacagaatattaccaaagaaatcttttagaatggactgttaaaattatttatttgtatttatctggctctactatttgtggtacatttccacttcaaagctaaacctcaaataacatcatagtgagtggttgacttcatgtttaactgagatcttgaagactgaaaaagaccacgacaaacacacatctattttcttggctactgcatccgtgttcatcaccattctgatagtctgcaatgtattgcagctcaccctttgggaaggactaaagtagacatctgtttgttctgcttactcagcattcctaccctaattttcctttggagaacccctttattctagaccacgtgaagctaatgccaaaccccattccaggggatgcacctgaatccaacctccatcatctaaacagtgccttctccacgttcagagaagagcaagtgactcaaactgccctcataagaacagacctgggacttctgctgcaaatattgaagagtaagtactcttttttcttgctaggactaagctggtagtaccttctatgaggctatcatatggaaacaacttgtctgaaaatgaagccacaactagaaaacagatcctggtaacccggattgatggatccagccctaccttaaatggcaagacctaacccgaggctttttgcatcaaccaataaagtccttaagccagtttgagttggttttgtcacttgcagctaaaagaattctgactctaacaatgtgacaatagcaaaaataaacataactgcttttgaggtttctaatggattttcctccctatatacatgatttcatttaatcctcacaattcaggaaagcacatatctattaacattaaattaatattcattattttgaacacatgctatgtggataagggatgaggaaagccaaggaagtaatcaacgtgaaatctcacttatatgggagggaagtggaggttacatatctcagggcacttaacagatatcatcaaatgaaagaataaacagtgtgtgggagaggcagtaggtgattcttcatcaattcctggatgaaaaattaggagataatgaactccgaacaggcagcctaatgagaatggctcaagcaacaggacatagagagggagttaggttagacatggggttcttgggaattttcacctcgtgggggggcgggggggtcgtgcagctgttgtcagtgggaaagggaaaaaggaaaaggctgagtttggaaggcagggagggaggagacaatgtgagtcagtgaaaaagggcccttagaatgacaagtctggaccagagagaggctaagactgaaaatacaagttgggtaaccactggcatacagatggcagttcaggcttgggcactgcccaccagagcctcagcatgaagagaagagggggaggctggccaccacctccctctaggtaatcgtcatcctgatgctgagctcctgaaaacaggctctttcactcgccccatctcttgctcttgattgcaacccggcattcaggaggcaccctgtaatatctgtggagtgaccgacaacacagcgccagggcactgagaagatcccagggcgccagggactggttctacaagggtgcccctcccggtcccctccagcgcgccgccagagctgccagtcttggctgctacacgggaggcagcctcattatgcagctctcacctcttaaattagttcatgctctcacattaggtgtaatcacagcttgcaacgctttctggggatgtctcagaaagatctgagttgaaaaaatatttttgtgtcattttaatttaaagtaaaattgctgcttcttccccgcccctttctttcctcctggcccacccagcgaccctggccggccgtgctcaacgggggcgggggtcggaggtgagatttcctccacataattccttaaacagctatcaactaagtctcaaagaaaaaaaaaagagatctagaagcagagacgtggctgctggcgatcccaaagctggtgttcgctcttgggggagagcgtaccctgggggaggccgggaggccgggccagaggctagcccagaggcagagggcaggagcgctcagccggcgccccgcgtctctccagctcccgacgctgcgctggctccgctgagcacgccaggatcaaggtcgcctggtggggaccggagcgccaggagcctgtgggaagcgttccagccggcctctgactgggatccggcgccgcgtttctgctttggacttgactgacaggtccccccgccctcccgccgccctactaccagcctgggttcatccttcagggctacgtctaccgcacccgggctggaaagcctggagcgcgcccttcctctcctcatcttctcagctctcctttctccctgccacttggcaaagctgcattttgactttcacgttttggactacgtgtgtgtagttccaagtccatgcgtggcacgaaaatccacttagggtaaaaattattctcgaaaaatcgcccatctcaggatctggtgtctacactcaaggctaggaggtgcaggtacgggtgcgtaaagcatgccgtaagggtgcacagtaaataaaaagtacggatgcaaaatgtaaattttaagtgcaaaacagaaaagcagtactcgttgccgccccgcacgctgggttttaaggggcacgaaggtgggcctcggctgcttttgctcagccccgcgtcctcagcgcccggcccagtacccggtactccgtaggggttcaatgatctcccctgaataagtgaacgaattaacaaatgaatgaatgaccgctcgatccgacctccgcggccggcagagcagtcgctggagaggcgggagagagcgagaggccaagctccaccatcgcggccgccggctggggcagagggacacggagacactcggcgccccggctccgcaccgagtccccg

SEQ ID NO: 17610 - RNA, 15649 nt, Homo sapiens
  source 1..15649: mol_type = other RNA
tcaggccaggcacagtggctcatgcctgtagtcccagcactttgggaggccgaggtgggcagatccacgaggtcaggagatcaagaccatcctaacatggtaaaaccccatctctactaacaatacaaaaaattagtcaggtgtggtggcacgtgcctgtagtcccagctactcaggaggctgaggcaggagaatcgcttgaacctgggaggcggaggttgcagtgagccgagattgtgccactgcaccctagcctaggcaacagagcaagactctgtctcaaaaaaaataaaaaaaaaaaaaagagagaaagagagagagagatgaggagttgctgcactgctgggtgtggagagccgaggaggattcaaagatggtcctgaagtcccagctggaagaagtaggcggcagcaatgtttttaatactgtaaattcatcacgtagcacaggtttggggtggagaaagaaaaattgcattggcttcagggcatgcccagatctttcctcatcttaggcgtttgctaatacatgcattttctaagctgatgtcttgcgtttaatcactgctccattcaaaagagagaaggaggttgtttcaaacctagttgatatcatttgacttccatgctattcacagggctattttatttgaaacaggtataccacagccttaaattgcaagttaatccaggatgttcctaggttggcagttaggaacatgtaattctttggaagggctaaaagtcagctctttaaattatctccatatgaaccttctctccaccttagggtggatccacttatttagtccactgccagtaccacactagaacccgggtggtcactggactccagaaacaacagtagccctctctctgttctgtctctttttgactatctctattctgttcctgaccctgatttctcctgccaagctcaattttgacagctgacaacggcaagccatggcttcccaaaacattattttcaggtcaacttataaatttcaagaacacatttggctccgcttcctgtggtactaagcctacttcttgacagcatttgcctttgttgtaaatagcaaagttcttctagttggatttttgctaagaagtgtgtggatgtggcatgtgacgacatctttagcttggattctagaaaggcactaccattgtgcatttggctaaaggaaacacattttacccgtgaatgccttctatttacaaatgctcagctagcacacaaagctaagtacaagcaataagtactatcctacaatgttactcatttctgaaagcacaaaatgatgactggtatagctttggagatgttttctggaaacccaataaaggaacagatctttgttattccacacctacaaagtcagaagatgcacagtcttttattcatgtttgaacaagcttccttcttgaacaatcaactataaagtgatgtgattctctactagaccaggaactccttgaggacagaatgagggtctaatccatattctaaatccacaccacctggcacaatacatgttgcatggttagggtcaactaagagttggttgaattaatcaataacacacagcaagagaattcacaaagagaggggagtaatcccccagcctcaatcactcggcaagtggaatcgctgggcactgattccagctctgtctcagtgcttgagacagagctgaatgtaatgtgaacatttcaaatgaacaggaaaactagactcacggataagcagtgtagtcatcaagacaacactgtcttggaggtttttctgaagttaaaaccatgctacataagcaataaattatgaaggctgagcatgtgaataaaatttaatgttgtcataaattttataacaaagttaatctgacacatttaatgacatgcataatcattagtatgcagcactgtaatcagacattgataataagcagttcacaccagtgactgtaagagtctttacttgtgttcagccaagccaactgcttggtatatttttctcccttcttagtcgttagttttccatacctacaataactatcagtggtgatgggcttctctgaccatgtgaataatttaatcctcaatgcacagatacagaaacccttgctgaagacagtgtggagcagagaaggctgtctccactccttccacctgaaacacctctgcagatggatatgggagctctgcctacagcccttggacctaaccacttcagtgtgttccagtgagtgtctggacctcggcctgaaagatttttccgaaactaaagaaaatttctctgacctaaagaccttaacctccaccccagaagctctcaccaaggactacagggaactggtggggaaaatccttatcccttactcctcaaggcacagggcagtaatgctgaggcttgtgcgccacacttgctcccagaggtccccagcgggctacctgcggtggtgaatgacctcctaacacgccccttgacggccttcctttccttgcctcacttctccactctcctaccagcattgcagggttcacatcccaaatataccactggcacttgaatcctggtctccaggtctgtttctggaaaaacccaagtaagacattgccccagtaatggggctagatgtctgaggcttcctcaagtatctacctcgaaagctcttactgctgtacacacatgcacatacacacacgtgcgtacaaccagtcacatctaagcaccccgaataccagcctgttgaaggtagcagagagctgcactataagccaaggctgctcccaagagccgctccatcactgaattggcgccccagcaagatgaaggaatgtaatcattggaaggatggagaatgttctctgaatcactgacaaattggaaggggtggagggcaagagtccacctggtggagagatggaaagagcgagagagcctggaatgataatgccattgcttagaaaaggctgctccagatgccatatctacagaaattgtacagcccaaacatctctgagcaataggtctctggtagtcttgatgtctagaccaacaattcccagttcattcttctcagggaaggagccaggatagtccagagactctcattctgctgttagattgaaagggttaggcacaacagccttggcaaagtcacaagggcaaattcacactaaagtgtaaatgacccacaactcctcttctatttttaggttggggaggtgctttagaacataaggaggaactaaagaatattcctgttacatacaaggcagagaaaagggaaactagtggtgacaagacaaatcatccctttgacatttggctggctctacctattacagctctgggggtgaggtgggaacaaaaagatgctgtgtaaagaagtatcttatgccatccctactgtagtgaggtgcagtttagaggggacactgatcaagcagagacccagagtgtttcgttccaagccagaaacagaaatgtataaaacacagcctttccagcatcagaaatgagtagtggtagtggagaactacccaaaacaggaaagaggaccacgtgaggtagagtgtcaaggccctacattccagtgcctctgctcatgactgtaattttgggtaggtcacttaaagtctctggacctcagttttgccatctgtgaaatagggataatactatccagcataaaattggttatgaggctcatgtagggcctgcctgggatgatgtgttgctaatggttaagaacacaacttctggggtctgactggacaggctgaaatccctgcttaacacgttccagcagagccctgggcgatctatttaacttttgttttctcacctgtaagctgagacgaaagtacccactttataagattattccaataattagttgaaataatgcatgcagagaattaagcatggtacttgttatttgttaaactagctattaaaatgtgtaaaatataaagtattgtatggattttaggacaatgcaaagactctttgcttgctgcaatagttcggggccctttcagatggctaaaggcagaatttgtatgtgtaaatatggtgtgcttgtctctgctctggatactgagggcttaccctgttattaaacttatttagtaaatattgaactgtcatgaggcctaacatttagttccagttattagataaaacatttgctttgaatggtatttgaattgccaggttctagattattctggttgacaaactcttcgtattttataaagaggctaaaattggtaagctatcacagaacagatgtgccattttcaaggtatattaaaccatgattcactgtaacattgttcctactggcaacaaattcagagcaggctggactttatttggtgaagaaacattgagtggaagagaaatgacattattttatgtatttacattttcaaattactgtggcttaaacctgttcagccaacattacccaccttcagtctgctaaataaatgattcagtacatttctaatttacagaattttttaacaaaagaaaatgtaatttgatagccaaatcaacgttaaacattatacatttaaaaaaccacaggcaaagacacaaacatgatgacactaacttttgttaaagtatgcttacctatggtttcctctgaggcacgttctttcatgctaagcttccaacataatatgaaaatgaaggagatgcattttgcaaagcaaaacagaccttaagcaaaatattatacttctcaaattaacactgttacaaagttttagaatttaataagttcattaatttaaaagtttggatgtctgagtccttctatcccaaaacaagatcttggagggtcttccacagccatgtaataccatggtcacatgaccctttccaaaattattaatctgaatttactatatgaggataaatctatctttttgaaaatatttaggaaaatgagcttggtatttataaaatgaagctctctttgggtggtatcctaagacacgtcaagccaatcagcctgtaactgtgaaaaaaacattggtaggtacaaaagtggggtgggagaggagtgacttaactttgttaagtgatgggaaagaaacactaatagcattatctcaataaaatgtgatttaaaaaaatttaaaatactaaatcattgaactgacaaagaaatataaatcattcagaaataaactcattaggtcatcaaatcctgttaaatctgcaattaggaagagcaaggtgtacaatccatacatttaaactcacaggctcactttgcacaacgtcaatttactccttaatatgttattaatacgcattttccaaaaggatgtattagtaaatggtacacatctacttcttggcaacatcatataacctggtacaacataagcattcttcttatagttaagaaatgtggatggtatcaaaattagaaaaataaatgccctattatgttgtggtcaggtttaaggcatgtgaattttatcttcatacaaaagattaaaatctagatattaaaaagtagtgcagtatcagtgatgctgcctcagttcccaaaatgtcacatcacaaaaatatcccataattgcctgtagtttattccttggctttcctcttttctctctgcatctttgtaacaattttttaaaagtggaaatataattgttggcaatgctaacagctgtagaaatgattacaagatgtggaaaagcataacaggaatgtcaagaatctgtttctggcagtaatatatatggaacattgttcaggacaaaagaggagaaggaagaaaaaaaggagaggggtttatcatctctaagaattttcaaactaaacctcattgcttaataggaaaaaaagattccatatttaaagttaagtcacctctaactactagctaaagcatgacatcaccagcactggagtcagcggaagtgtgtttttgaaggacagtgttgcaggagaatctggacaggttttagagccaggagagagaaaataattctacctctgacagttgaaggaccttaggcaaatcagtttacctctgctagactacactccaaaatttggacattcaaaaatttgatattaataaccacatgaaagtctcgtgttgaggtgaatatgtatttgttggtgaaagatatgttggtttttaaacagacagcactctgcaattgtaggctattgttttgttttgccagttgtcaaattctatccagctatacacacttgtgtggcctcctaatggtgtttttccagtggctaaaggtttatgaataagacacttttcctaatggaattaacccgatgcttttcttaaacatgtaaccttgagttcaccgcaaaaaacaatgcttcgattagagcaatgcatataataaaggttaccctcgtttcttagacactagacatcattcacaaaaagagaactgcttttgaaagggatgtatttgcactggaaagaatagttttctacttctaattataaatgatttattggtgaaagcaaaacaacagcctgtctgagaggcacttctatgagcatcctcacgtgtgatttgcaaggttgaagaagagggaaaaatgcctcaattgtaccaatggtgagaaaacacccaaagtacaaagcaggtttcaaaaaaaccatactcataaccaaggacaataataaagcaatgtgttgacatatactctataagtcttcctccataaatagtttatagaaattttgtaatttctgtaaatgcatcctataataattttgcatcttgctttttttttacatttaatatcaagtagatttctaaagggcaattatttgaaaattatcccaaatacatggggaaatatacatcaagtgaaaaaatgcagtgggtgatagagatatcaggaagcgcctcaaatatttctcatctcgttggagaaaaacaaacatgttctcatttagaatgagtgggagttacctaattgatttaggcctctatatttaacttctagtcaaaaaaggtagttctatctagcaacaatattatggggaacaaaagaaaaaattaactctctaaatttgcagtagggtcttttcttcagaagtaccaaatcccatctattaccagctccatgcttcaggcctaaaatggatctccctgaagcaatgacagaatttttgccaagtgactaggatataaacaccactttggttgcacagtgagacatatgctccaaagaaaactggttcaaaaacaggcaagtgggtttctacagaataaatgagagccctgtcaatggcttcatcttcagggctttgtgtctgtgcttgcgtggtggctcttgtttcatctatggataatggtggcacacagttttcataattccttacattaatgaactgctataaatttgtttttggtattctagagagtcctaacttcagcttctgggcaatgctgaggaggcaccctatattctagacttaccttttgcaaggtgtactctcagcattgtgggcgatttccatgggagaatattctatttaaagaactactgtcccagcataaaacaaaaaatcatttatgaagatgcaggagactcggaaagctctcaattattgtttgcacaagcacaatgtcacagcctcctttccccattccacaagggggtcaggaagagagtactcagctgtgagaaaagacatacagaagaattcatgtggtcatgagagcgaggacatggccgatcccccaaggaggatgtgtcatacacttcatgagcccaagagtgtgctgtagggtctgaagggcaagatgctggttcactgatgtaaaggagagggaaaaaagcttcaaccaactagaaaaacagtctctatgcatgctatttttgattttaaacacaggtatcaattccttctctcagagagtccattttaaaataggatacatttttaaaggaatatttaaaggacacattcattaaaatttattttaaaaacttttcaaaagaaacaaaaggtatgaattttatttaatccttgaggaaatggttcttttctcacacacataaatcactcattttgtttttctttatctcctttattaatctacattagaaaaataaacttttcatacactaagaacaaggaaaccactctcaattgacaaaatgttccaatccaacacaatgattactttcacctttaatttacaggcagccagattcaaaatccttaaagttgcttaaacttaaaaatgacaatgacaacctaaaaggtataatgttgattggaacagacatttaattggaaaattgatgattttccatttccaattaaatctctagatagaaatgaaaaaaattaaaaatcgtatttaagaaaagccaaatcttgggttgtgaggtatctttttaaggatgtttcagcagaaaaaaacaaaggctctcacaattgtgtagctgcctagattaagtgggtatcctgatcaaggagatgggggatgatttggctttagtattccaatgataaagtttataatgagaataacatgttgctacaaaatccagtctcttcctcagatgccttccacagagggcaggaagctttgtcagttttgtttgctgatgatgcctggttccgtcaacaaataacacctgtcacacggtgggtagtcaatatacatttgttgaataaatatgaaaaaaagaaatgtacaatatgtttgtgaagccaactgtgtgtgcattgctattgaggtacacaaaaagtctttgttttaaatttgagaatgaggactttcaatggaatatatctgataggcctggatcaagcatgcagctgtggagaacacccctgggactctaactctggcactctgcaagctgggtacttgggcaggacagcagcagcactcatgaactgggcagcacctgttggtgagggctgatcacatggattctctcatcccagccttacaatcagtccttcaggtacatactttttctgactttgctgatgaggaaactatgcacagaggttacacagcttaacaaagggttctcacctaatgaacaatgaaatgggattttagcctttctttgcatctggtcttagagccaatacccaagaagcactgtactgtatgcattgtctcagagaaacttactcttcctgggcctcagtctttaaaaggtgggcagttgacttaataagaattaaagatcaatgattaaggttcaaggcactccaaaattctggtctttattgaaaaggctacagaagtctcaccttaataataccctatagacttgatattcttggttaattaaatattggaaaccaatttcatagtaattgaggtcagaaaaaagtactcatgacattttagaatatgatgacaaagccatagataaatttcaatgcacctgtaattacttaaaactgttatagcatgcaatgtgttaccacaacagccagagaaatactaatttactcagcctattcttctagaccagtaaacactaggattaaatagatattttcattgaatttgttctacccttcattgccatttatagatagcttacttgtcatagattactttctaattgttttatgtttcctaactagcctgcaatactttggcaaggacctcaaacaatagtagacagtaggtgtaaaatagatggctacattgaacagatgactaaaaggatgcctcctaagtacctatatcttgaaatatatattattgtgccttgctttcaatttgtgattttaaaatctagaaatcacctgttttatgtaataacaataaaatccttctttgttgaaaacatgcacaaataaagtttacaagctcaaaaaattaaacagcagtaacggtcaagctttccaacaataaaatacattttggtaaggttttcattttacaaaaactcaaaatagctttatgagttcacaaaataatatgatatttttcaagatattaacatattcttataccggaagagcatagaataaaatttacttggagattgagcatttgcttctttaagaaatacttcttttagtatttttactttaatattatgaaagctacataattacattcagattcattaactactccagtagttaatttttaaaacttatgatgaatagttttgtttaaaatatataacattggtaatatgcaaatctgaatctgtaataaagaaggatttgcattcctgatttttttttctgatacaaccaatgacaaaataactaatggttccacagaggataaaatgtctcaaatctgttggttctgaaggtgaagcgagatttttgtactgataccgtgtatcactgagataccaggaggaaatggaattaaactcagatagttcaaatggagagattttaatgaagggacgacctacagaggtgtcggcagggttggggggaatcagcgagatatgcttagaacccaccgactggcaaacctccccctgaagatggagaaggaggaaggagtgttactggaatgagagcttgagtccaggggaggaggatgggctgctgaggaggcgacaccatcctgaaagaagaatcctctgccagaggcttttcagggtcatttcttcacactctctctcttcaagtggtatttaaatttcttctttcattttccttctggtaacaaagaagtctgtggctcaaaagatgtttctctaagaccccatcctattaggtctctgagctgtgggaagtatttatacaattgcttgtgaatataagatccaggaatttccctaagatccctaacaaaattggtgataagtagtcccacatgttaatccagccacccacggatgacagcacttaccatttctttgataaatgtcaaatgcatttgaagtacctacctgaaatatttgtttaaatgctatctaatctattaattttatatatgtgtgagtctgttttgtataccttctgattataggataaatgtaaataaatccaaagagtaatcaaagctaccactttcaagaagccttctttgtagaaccggaagagtcttaaataggcttttcaggtatgcatctcttattatcgctgaactccaagtcctgcaaggcaggcatcatgtgtgggtcacctttacagtaggcacaggccttaaaacagtgacatgcacattgcaggcactccataaatgtttgctgaattggctaaaccttggtttgttcccataatcaaccaccacaaacagcacacagataattacttcttggaaagattccaactagtgtttgatgttacctacgtggtttttctctcaagatcttaagagcagctctgtaggattacattattttctgttttttttttcctttgaccttaatgtcatctacttcaataacagcttcatacaaaattcctaccagcacataccacagcagattcaaggccttgttttaaaaatggtgccagcttctcttaatttggaagatatattgtctctcctgaacatgggctaagaaaatgtataatttggtattaacataagagctgaagacactttaaatgcattgtttcatttttataagataaaaaaaattttaagaatcaaaatgttatcaacagacttgtccttcattaaaaagtaaaactgcatttgcctacattttatgaaagtgtccaattatgaacaattttgaaatgtaacttttaaaaatgtaaacagcaaaaatgttgtatttaaaataaatctggaaaggcagaaaaacaaaaaatacccagaagacagagtttttggtgaaagttaagatatttcatctttgaacaacttagaatctttcctgcattttatagtctagttccaggcattaatttgaaataaccttggaatcctaaatctaacacccttcggaacaaagtagcttttctcttctgctttatgagcaaatggactaaatactagggaatggtactgtctgggcctttgaaccaagattgaaagagatgaaatcctatatgatatgtataaacattagagaatccattttgatttaataaaaggttgaatttgttctatatcctgtgagaaaatggttcccttttcctgaaaatgttacctcattccaacaatagaaagttggtttttttccagggtgtggtgttggcgggggacagagttgccatgaatatggcatctatgaagactgctgttatattcatttctcaaaatgcactgtggtaggaaattcagaacgcagtgagagaaaataaatgtttgacttcaaaatataaggccgcatttaaagcagaaggtaaagtatagaacagttgacagtataaattctttatctgcaatcttgcagttccctaaatctctgtaacacatcacttttaaaagcctcagataagtggttctataataatttaccaataattcaacccctcaaaagtcttagcaagttaaaccttataatcttacattttagaaatgacccaacttgatccttttattcttcagaatatctctctcaaattttcatttgtttttcattaattgatgaataatgagacattttaggtacctgtccacaaagaaatgaaattttcactttccaggaacctaacaaatgaaaagatagaaatcaattccaacagaatattaccaaagaaatcttttagaatggactgttaaaattatttatttgtatttatctggctctactatttgtggtacatttccacttcaaagctaaacctcaaataacatcatagtgagtggttgacttcatgtttaactgagatcttgaagactgaaaaagaccacgacaaacacacatctattttcttggctactgcatccgtgttcatcaccattctgatagtctgcaatgtattgcagctcaccctttgggaaggactaaagtagacatctgtttgttctgcttactcagcattcctaccctaattttcctttggagaacccctttattctagaccacgtgaagctaatgccaaaccccattccaggggatgcacctgaatccaacctccatcatctaaacagtgccttctccacgttcagagaagagcaagtgactcaaactgccctcataagaacagacctgggacttctgctgcaaatattgaagagtaagtactcttttttcttgctaggactaagctggtagtaccttctatgaggctatcatatggaaacaacttgtctgaaaatgaagccacaactagaaaacagatcctggtaacccggattgatggatccagccctaccttaaatggcaagacctaacccgaggctttttgcatcaaccaataaagtccttaagccagtttgagttggttttgtcacttgcagctaaaagaattctgactctaacaatgtgacaatagcaaaaataaacataactgcttttgaggtttctaatggattttcctccctatatacatgatttcatttaatcctcacaattcaggaaagcacatatctattaacattaaattaatattcattattttgaacacatgctatgtggataagggatgaggaaagccaaggaagtaatcaacgtgaaatctcacttatatgggagggaagtggaggttacatatctcagggcacttaacagatatcatcaaatgaaagaataaacagtgtgtgggagaggcagtaggtgattcttcatcaattcctggatgaaaaattaggagataatgaactccgaacaggcagcctaatgagaatggctcaagcaacaggacatagagagggagttaggttagacatggggttcttgggaattttcacctcgtgggggggcgggggggtcgtgcagctgttgtcagtgggaaagggaaaaaggaaaaggctgagtttggaaggcagggagggaggagacaatgtgagtcagtgaaaaagggcccttagaatgacaagtctggaccagagagaggctaagactgaaaatacaagttgggtaaccactggcatacagatggcagttcaggcttgggcactgcccaccagagcctcagcatgaagagaagagggggaggctggccaccacctccctctaggtaatcgtcatcctgatgctgagctcctgaaaacaggctctttcactcgccccatctcttgctcttgattgcaacccggcattcaggaggcaccctgtaatatctgtggagtgaccgacaacacagcgccagggcactgagaagatcccagggcgccagggactggttctacaagggtgcccctcccggtcccctccagcgcgccgccagagctgccagtcttggctgctacacgggaggcagcctcattatgcagctctcacctcttaaattagttcatgctctcacattaggtgtaatcacagcttgcaacgctttctggggatgtctcagaaagatctgagttgaaaaaatatttttgtgtcattttaatttaaagtaaaattgctgcttcttccccgcccctttctttcctcctggcccacccagcgaccctggccggccgtgctcaacgggggcgggggtcggaggtgagatttcctccacataattccttaaacagctatcaactaagtctcaaagaaaaaaaaaagagatctagaagcagagacgtggctgctggcgatcccaaagctggtgttcgctcttgggggagagcgtaccctgggggaggccgggaggccgggccagaggctagcccagaggcagagggcaggagcgctcagccggcgccccgcgtctctccagctcccgacgctgcgctggctccgctgagcacgccaggatcaaggtcgcctggtggggaccggagcgccaggagcctgtgggaagcgttccagccggcctctgactgggatccggcgccgcgtttctgctttggacttgactgacaggtccccccgccctcccgccgccctactaccagcctgggttcatccttcagggctacgtctaccgcacccgggctggaaagcctggagcgcgcccttcctctcctcatcttctcagctctcctttctccctgccacttggcaaagctgcattttgactttcacgttttggactacgtgtgtgtagttccaagtccatgcgtggcacgaaaatccacttagggtaaaaattattctcgaaaaatcgcccatctcaggatctggtgtctacactcaaggctaggaggtgcaggtacgggtgcgtaaagcatgccgtaagggtgcacagtaaataaaaagtacggatgcaaaatgtaaattttaagtgcaaaacagaaaagcagtactcgttgccgccccgcacgctgggttttaaggggcacgaaggtgggcctcggctgcttttgctcagccccgcgtcctcagcgcccggcccagtacccggtactccgtaggggttcaatgatctcccctgaataagtgaacgaattaacaaatgaatgaatgaccgctcgatccgacctccgcggccggcagagcagtcgctggagaggcgggagagagcgagaggccaagctccaccatcgcggccgccggctggggcagagggacacggagacactcggcgccccggctccgcaccgagtccccg

SEQ ID NO: 17611 - RNA, 11078 nt, Homo sapiens
  source 1..11078: mol_type = other RNA
tcaggccaggcacagtggctcatgcctgtagtcccagcactttgggaggccgaggtgggcagatccacgaggtcaggagatcaagaccatcctaacatggtaaaaccccatctctactaacaatacaaaaaattagtcaggtgtggtggcacgtgcctgtagtcccagctactcaggaggctgaggcaggagaatcgcttgaacctgggaggcggaggttgcagtgagccgagattgtgccactgcaccctagcctaggcaacagagcaagactctgtctcaaaaaaaataaaaaaaaaaaaaagagagaaagagagagagagatgaggagttgctgcactgctgggtgtggagagccgaggaggattcaaagatggtcctgaagtcccagctggaagaagtaggcggcagcaatgtttttaatactgtaaattcatcacgtagcacaggtttggggtggagaaagaaaaattgcattggcttcagggcatgcccagatctttcctcatcttaggcgtttgctaatacatgcattttctaagctgatgtcttgcgtttaatcactgctccattcaaaagagagaaggaggttgtttcaaacctagttgatatcatttgacttccatgctattcacagggctattttatttgaaacaggtataccacagccttaaattgcaagttaatccaggatgttcctaggttggcagttaggaacatgtaattctttggaagggctaaaagtcagctctttaaattatctccatatgaaccttctctccaccttagggtggatccacttatttagtccactgccagtaccacactagaacccgggtggtcactggactccagaaacaacagtagccctctctctgttctgtctctttttgactatctctattctgttcctgaccctgatttctcctgccaagctcaattttgacagctgacaacggcaagccatggcttcccaaaacattattttcaggtcaacttataaatttcaagaacacatttggctccgcttcctgtggtactaagcctacttcttgacagcatttgcctttgttgtaaatagcaaagttcttctagttggatttttgctaagaagtgtgtggatgtggcatgtgacgacatctttagcttggattctagaaaggcactaccattgtgcatttggctaaaggaaacacattttacccgtgaatgccttctatttacaaatgctcagctagcacacaaagctaagtacaagcaataagtactatcctacaatgttactcatttctgaaagcacaaaatgatgactggtatagctttggagatgttttctggaaacccaataaaggaacagatctttgttattccacacctacaaagtcagaagatgcacagtcttttattcatgtttgaacaagcttccttcttgaacaatcaactataaagtgatgtgattctctactagaccaggaactccttgaggacagaatgagggtctaatccatattctaaatccacaccacctggcacaatacatgttgcatggttagggtcaactaagagttggttgaattaatcaataacacacagcaagagaattcacaaagagaggggagtaatcccccagcctcaatcactcggcaagtggaatcgctgggcactgattccagctctgtctcagtgcttgagacagagctgaatgtaatgtgaacatttcaaatgaacaggaaaactagactcacggataagcagtgtagtcatcaagacaacactgtcttggaggtttttctgaagttaaaaccatgctacataagcaataaattatgaaggctgagcatgtgaataaaatttaatgttgtcataaattttataacaaagttaatctgacacatttaatgacatgcataatcattagtatgcagcactgtaatcagacattgataataagcagttcacaccagtgactgtaagagtctttacttgtgttcagccaagccaactgcttggtatatttttctcccttcttagtcgttagttttccatacctacaataactatcagtggtgatgggcttctctgaccatgtgaataatttaatcctcaatgcacagatacagaaacccttgctgaagacagtgtggagcagagaaggctgtctccactccttccacctgaaacacctctgcagatggatatgggagctctgcctacagcccttggacctaaccacttcagtgtgttccagtgagtgtctggacctcggcctgaaagatttttccgaaactaaagaaaatttctctgacctaaagaccttaacctccaccccagaagctctcaccaaggactacagggaactggtggggaaaatccttatcccttactcctcaaggcacagggcagtaatgctgaggcttgtgcgccacacttgctcccagaggtccccagcgggctacctgcggtggtgaatgacctcctaacacgccccttgacggccttcctttccttgcctcacttctccactctcctaccagcattgcagggttcacatcccaaatataccactggcacttgaatcctggtctccaggtctgtttctggaaaaacccaagtaagacattgccccagtaatggggctagatgtctgaggcttcctcaagtatctacctcgaaagctcttactgctgtacacacatgcacatacacacacgtgcgtacaaccagtcacatctaagcaccccgaataccagcctgttgaaggtagcagagagctgcactataagccaaggctgctcccaagagccgctccatcactgaattggcgccccagcaagatgaaggaatgtaatcattggaaggatggagaatgttctctgaatcactgacaaattggaaggggtggagggcaagagtccacctggtggagagatggaaagagcgagagagcctggaatgataatgccattgcttagaaaaggctgctccagatgccatatctacagaaattgtacagcccaaacatctctgagcaataggtctctggtagtcttgatgtctagaccaacaattcccagttcattcttctcagggaaggagccaggatagtccagagactctcattctgctgttagattgaaagggttaggcacaacagccttggcaaagtcacaagggcaaattcacactaaagtgtaaatgacccacaactcctcttctatttttaggttggggaggtgctttagaacataaggaggaactaaagaatattcctgttacatacaaggcagagaaaagggaaactagtggtgacaagacaaatcatccctttgacatttggctggctctacctattacagctctgggggtgaggtgggaacaaaaagatgctgtgtaaagaagtatcttatgccatccctactgtagtgaggtgcagtttagaggggacactgatcaagcagagacccagagtgtttcgttccaagccagaaacagaaatgtataaaacacagcctttccagcatcagaaatgagtagtggtagtggagaactacccaaaacaggaaagaggaccacgtgaggtagagtgtcaaggccctacattccagtgcctctgctcatgactgtaattttgggtaggtcacttaaagtctctggacctcagttttgccatctgtgaaatagggataatactatccagcataaaattggttatgaggctcatgtagggcctgcctgggatgatgtgttgctaatggttaagaacacaacttctggggtctgactggacaggctgaaatccctgcttaacacgttccagcagagccctgggcgatctatttaacttttgttttctcacctgtaagctgagacgaaagtacccactttataagattattccaataattagttgaaataatgcatgcagagaattaagcatggtacttgttatttgttaaactagctattaaaatgtgtaaaatataaagtattgtatggattttaggacaatgcaaagactctttgcttgctgcaatagttcggggccctttcagatggctaaaggcagaatttgtatgtgtaaatatggtgtgcttgtctctgctctggatactgagggcttaccctgttattaaacttatttagtaaatattgaactgtcatgaggcctaacatttagttccagttattagataaaacatttgctttgaatggtatttgaattgccaggttctagattattctggttgacaaactcttcgtattttataaagaggctaaaattggtaagctatcacagaacagatgtgccattttcaaggtatattaaaccatgattcactgtaacattgttcctactggcaacaaattcagagcaggctggactttatttggtgaagaaacattgagtggaagagaaatgacattattttatgtatttacattttcaaattactgtggcttaaacctgttcagccaacattacccaccttcagtctgctaaataaatgattcagtacatttctaatttacagaattttttaacaaaagaaaatgtaatttgatagccaaatcaacgttaaacattatacatttaaaaaaccacaggcaaagacacaaacatgatgacactaacttttgttaaagtatgcttacctatggtttcctctgaggcacgttctttcatgctaagcttccaacataatatgaaaatgaaggagatgcattttgcaaagcaaaacagaccttaagcaaaatattatacttctcaaattaacactgttacaaagttttagaatttaataagttcattaatttaaaagtttggatgtctgagtccttctatcccaaaacaagatcttggagggtcttccacagccatgtaataccatggtcacatgaccctttccaaaattattaatctgaatttactatatgaggataaatctatctttttgaaaatatttaggaaaatgagcttggtatttataaaatgaagctctctttgggtggtatcctaagacacgtcaagccaatcagcctgtaactgtgaaaaaaacattggtaggtacaaaagtggggtgggagaggagtgacttaactttgttaagtgatgggaaagaaacactaatagcattatctcaataaaatgtgatttaaaaaaatttaaaatactaaatcattgaactgacaaagaaatataaatcattcagaaataaactcattaggtcatcaaatcctgttaaatctgcaattaggaagagcaaggtgtacaatccatacatttaaactcacaggctcactttgcacaacgtcaatttactccttaatatgttattaatacgcattttccaaaaggatgtattagtaaatggtacacatctacttcttggcaacatcatataacctggtacaacataagcattcttcttatagttaagaaatgtggatggtatcaaaattagaaaaataaatgccctattatgttgtggtcaggtttaaggcatgtgaattttatcttcatacaaaagattaaaatctagatattaaaaagtagtgcagtatcagtgatgctgcctcagttcccaaaatgtcacatcacaaaaatatcccataattgcctgtagtttattccttggctttcctcttttctctctgcatctttgtaacaattttttaaaagtggaaatataattgttggcaatgctaacagctgtagaaatgattacaagatgtggaaaagcataacaggaatgtcaagaatctgtttctggcagtaatatatatggaacattgttcaggacaaaagaggagaaggaagaaaaaaaggagaggggtttatcatctctaagaattttcaaactaaacctcattgcttaataggaaaaaaagattccatatttaaagttaagtcacctctaactactagctaaagcatgacatcaccagcactggagtcagcggaagtgtgtttttgaaggacagtgttgcaggagaatctggacaggttttagagccaggagagagaaaataattctacctctgacagttgaaggaccttaggcaaatcagtttacctctgctagactacactccaaaatttggacattcaaaaatttgatattaataaccacatgaaagtctcgtgttgaggtgaatatgtatttgttggtgaaagatatgttggtttttaaacagacagcactctgcaattgtaggctattgttttgttttgccagttgtcaaattctatccagctatacacacttgtgtggcctcctaatggtgtttttccagtggctaaaggtttatgaataagacacttttcctaatggaattaacccgatgcttttcttaaacatgtaaccttgagttcaccgcaaaaaacaatgcttcgattagagcaatgcatataataaaggttaccctcgtttcttagacactagacatcattcacaaaaagagaactgcttttgaaagggatgtatttgcactggaaagaatagttttctacttctaattataaatgatttattggtgaaagcaaaacaacagcctgtctgagaggcacttctatgagcatcctcacgtgtgatttgcaaggttgaagaagagggaaaaatgcctcaattgtaccaatggtgagaaaacacccaaagtacaaagcaggtttcaaaaaaaccatactcataaccaaggacaataataaagcaatgtgttgacatatactctataagtcttcctccataaatagtttatagaaattttgtaatttctgtaaatgcatcctataataattttgcatcttgctttttttttacatttaatatcaagtagatttctaaagggcaattatttgaaaattatcccaaatacatggggaaatatacatcaagtgaaaaaatgcagtgggtgatagagatatcaggaagcgcctcaaatatttctcatctcgttggagaaaaacaaacatgttctcatttagaatgagtgggagttacctaattgatttaggcctctatatttaacttctagtcaaaaaaggtagttctatctagcaacaatattatggggaacaaaagaaaaaattaactctctaaatttgcagtagggtcttttcttcagaagtaccaaatcccatctattaccagctccatgcttcaggcctaaaatggatctccctgaagcaatgacagaatttttgccaagtgactaggatataaacaccactttggttgcacagtgagacatatgctccaaagaaaactggttcaaaaacaggcaagtgggtttctacagaataaatgagagccctgtcaatggcttcatcttcagggctttgtgtctgtgcttgcgtggtggctcttgtttcatctatggataatggtggcacacagttttcataattccttacattaatgaactgctataaatttgtttttggtattctagagagtcctaacttcagcttctgggcaatgctgaggaggcaccctatattctagacttaccttttgcaaggtgtactctcagcattgtgggcgatttccatgggagaatattctatttaaagaactactgtcccagcataaaacaaaaaatcatttatgaagatgcaggagactcggaaagctctcaattattgtttgcacaagcacaatgtcacagcctcctttccccattccacaagggggtcaggaagagagtactcagctgtgagaaaagacatacagaagaattcatgtggtcatgagagcgaggacatggccgatcccccaaggaggatgtgtcatacacttcatgagcccaagagtgtgctgtagggtctgaagggcaagatgctggttcactgatgtaaaggagagggaaaaaagcttcaaccaactagaaaaacagtctctatgcatgctatttttgattttaaacacaggtatcaattccttctctcagagagtccattttaaaataggatacatttttaaaggaatatttaaaggacacattcattaaaatttattttaaaaacttttcaaaagaaacaaaaggtatgaattttatttaatccttgaggaaatggttcttttctcacacacataaatcactcattttgtttttctttatctcctttattaatctacattagaaaaataaacttttcatacactaagaacaaggaaaccactctcaattgacaaaatgttccaatccaacacaatgattactttcacctttaatttacaggcagccagattcaaaatccttaaagttgcttaaacttaaaaatgacaatgacaacctaaaaggtataatgttgattggaacagacatttaattggaaaattgatgattttccatttccaattaaatctctagatagaaatgaaaaaaattaaaaatcgtatttaagaaaagccaaatcttgggttgtgaggtatctttttaaggatgtttcagcagaaaaaaacaaaggctctcacaattgtgtagctgcctagattaagtgggtatcctgatcaaggagatgggggatgatttggctttagtattccaatgataaagtttataatgagaataacatgttgctacaaaatccagtctcttcctcagatgccttccacagagggcaggaagctttgtcagttttgtttgctgatgatgcctggttccgtcaacaaataacacctgtcacacggtgggtagtcaatatacatttgttgaataaatatgaaaaaaagaaatgtacaatatgtttgtgaagccaactgtgtgtgcattgctattgaggtacacaaaaagtctttgttttaaatttgagaatgaggactttcaatggaatatatctgataggcctggatcaagcatgcagctgtggagaacacccctgggactctaactctggcactctgcaagctgggtacttgggcaggacagcagcagcactcatgaactgggcagcacctgttggtgagggctgatcacatggattctctcatcccagccttacaatcagtccttcaggtacatactttttctgactttgctgatgaggaaactatgcacagaggttacacagcttaacaaagggttctcacctaatgaacaatgaaatgggattttagcctttctttgcatctggtcttagagccaatacccaagaagcactgtactgtatgcattgtctcagagaaacttactcttcctgggcctcagtctttaaaaggtgggcagttgacttaataagaattaaagatcaatgattaaggttcaaggcactccaaaattctggtctttattgaaaaggctacagaagtctcaccttaataataccctatagacttgatattcttggttaattaaatattggaaaccaatttcatagtaattgaggtcagaaaaaagtactcatgacattttagaatatgatgacaaagccatagataaatttcaatgcacctgtaattacttaaaactgttatagcatgcaatgtgttaccacaacagccagagaaatactaatttactcagcctattcttctagaccagtaaacactaggattaaatagatattttcattgaatttgttctacccttcattgccatttatagatagcttacttgtcatagattactttctaattgttttatgtttcctaactagcctgcaatactttggcaaggacctcaaacaatagtagacagtaggtgtaaaatagatggctacattgaacagatgactaaaaggatgcctcctaagtacctatatcttgaaatatatattattgtgccttgctttcaatttgtgattttaaaatctagaaatcacctgttttatgtaataacaataaaatccttctttgttgaaaacatgcacaaataaagtttacaagctcaaaaaattaaacagcagtaacggtcaagctttccaacaataaaatacattttggtaaggttttcattttacaaaaactcaaaatagctttatgagttcacaaaataatatgatatttttcaagatattaacatattcttataccggaagagcatagaataaaatttacttggagattgagcatttgcttctttaagaaatacttcttttagtatttttactttaatattatgaaagctacataattacattcagattcattaactactccagtagttaatttttaaaacttatgatgaatagttttgtttaaaatatataacattggtaatatgcaaatctgaatctgtaataaagaaggatttgcattcctgatttttttttctgatacaaccaatgacaaaataactaatggttccacagaggataaaatgtctcaaatctgttggttctgaaggtgaagcgagatttttgtactgataccgtgtatcactgagataccaggaggaaatggaattaaactcagatagttcaaatggagagattttaatgaagggacgacctacagaggtgtcggcagggttggggggaatcagcgagatatgcttagaacccaccgactggcaaacctccccctgaagatggagaaggaggaaggagtgttactggaatgagagcttgagtccaggggaggaggatgggctgctgaggaggcgacaccatcctgaaagaagaatcctctgccagaggcttttcagggtcatttcttcacactctctgcagggaagcacggagacagcaggaagaaatatcctaacctcactctcttccctctacaggtgcttccattggccaaatccacccagaggccagttggtggcgatcagctctcttcaagtggtatttaaatttcttctttcattttccttctggtaacaaagaagtctgtggctcaaaagatgtttctctaagaccccatcctattaggtctctgagctgagggccgacgagtgggggcgggcaggagggccgagggaggcggaacaggatcgaggcgcgaggcgggagtcgagaaagcgagcggccgaggcgactctcagtgcgcggacgcgggcgcgcgcccgcgctcccttcgtcgactcacggcgagagcccaaccctgctgccgcgcgccacccgcctcgccgcgcct

SEQ ID NO: 17612 - RNA, 15759 nt, Homo sapiens
  source 1..15759: mol_type = other RNA
tcaggccaggcacagtggctcatgcctgtagtcccagcactttgggaggccgaggtgggcagatccacgaggtcaggagatcaagaccatcctaacatggtaaaaccccatctctactaacaatacaaaaaattagtcaggtgtggtggcacgtgcctgtagtcccagctactcaggaggctgaggcaggagaatcgcttgaacctgggaggcggaggttgcagtgagccgagattgtgccactgcaccctagcctaggcaacagagcaagactctgtctcaaaaaaaataaaaaaaaaaaaaagagagaaagagagagagagatgaggagttgctgcactgctgggtgtggagagccgaggaggattcaaagatggtcctgaagtcccagctggaagaagtaggcggcagcaatgtttttaatactgtaaattcatcacgtagcacaggtttggggtggagaaagaaaaattgcattggcttcagggcatgcccagatctttcctcatcttaggcgtttgctaatacatgcattttctaagctgatgtcttgcgtttaatcactgctccattcaaaagagagaaggaggttgtttcaaacctagttgatatcatttgacttccatgctattcacagggctattttatttgaaacaggtataccacagccttaaattgcaagttaatccaggatgttcctaggttggcagttaggaacatgtaattctttggaagggctaaaagtcagctctttaaattatctccatatgaaccttctctccaccttagggtggatccacttatttagtccactgccagtaccacactagaacccgggtggtcactggactccagaaacaacagtagccctctctctgttctgtctctttttgactatctctattctgttcctgaccctgatttctcctgccaagctcaattttgacagctgacaacggcaagccatggcttcccaaaacattattttcaggtcaacttataaatttcaagaacacatttggctccgcttcctgtggtactaagcctacttcttgacagcatttgcctttgttgtaaatagcaaagttcttctagttggatttttgctaagaagtgtgtggatgtggcatgtgacgacatctttagcttggattctagaaaggcactaccattgtgcatttggctaaaggaaacacattttacccgtgaatgccttctatttacaaatgctcagctagcacacaaagctaagtacaagcaataagtactatcctacaatgttactcatttctgaaagcacaaaatgatgactggtatagctttggagatgttttctggaaacccaataaaggaacagatctttgttattccacacctacaaagtcagaagatgcacagtcttttattcatgtttgaacaagcttccttcttgaacaatcaactataaagtgatgtgattctctactagaccaggaactccttgaggacagaatgagggtctaatccatattctaaatccacaccacctggcacaatacatgttgcatggttagggtcaactaagagttggttgaattaatcaataacacacagcaagagaattcacaaagagaggggagtaatcccccagcctcaatcactcggcaagtggaatcgctgggcactgattccagctctgtctcagtgcttgagacagagctgaatgtaatgtgaacatttcaaatgaacaggaaaactagactcacggataagcagtgtagtcatcaagacaacactgtcttggaggtttttctgaagttaaaaccatgctacataagcaataaattatgaaggctgagcatgtgaataaaatttaatgttgtcataaattttataacaaagttaatctgacacatttaatgacatgcataatcattagtatgcagcactgtaatcagacattgataataagcagttcacaccagtgactgtaagagtctttacttgtgttcagccaagccaactgcttggtatatttttctcccttcttagtcgttagttttccatacctacaataactatcagtggtgatgggcttctctgaccatgtgaataatttaatcctcaatgcacagatacagaaacccttgctgaagacagtgtggagcagagaaggctgtctccactccttccacctgaaacacctctgcagatggatatgggagctctgcctacagcccttggacctaaccacttcagtgtgttccagtgagtgtctggacctcggcctgaaagatttttccgaaactaaagaaaatttctctgacctaaagaccttaacctccaccccagaagctctcaccaaggactacagggaactggtggggaaaatccttatcccttactcctcaaggcacagggcagtaatgctgaggcttgtgcgccacacttgctcccagaggtccccagcgggctacctgcggtggtgaatgacctcctaacacgccccttgacggccttcctttccttgcctcacttctccactctcctaccagcattgcagggttcacatcccaaatataccactggcacttgaatcctggtctccaggtctgtttctggaaaaacccaagtaagacattgccccagtaatggggctagatgtctgaggcttcctcaagtatctacctcgaaagctcttactgctgtacacacatgcacatacacacacgtgcgtacaaccagtcacatctaagcaccccgaataccagcctgttgaaggtagcagagagctgcactataagccaaggctgctcccaagagccgctccatcactgaattggcgccccagcaagatgaaggaatgtaatcattggaaggatggagaatgttctctgaatcactgacaaattggaaggggtggagggcaagagtccacctggtggagagatggaaagagcgagagagcctggaatgataatgccattgcttagaaaaggctgctccagatgccatatctacagaaattgtacagcccaaacatctctgagcaataggtctctggtagtcttgatgtctagaccaacaattcccagttcattcttctcagggaaggagccaggatagtccagagactctcattctgctgttagattgaaagggttaggcacaacagccttggcaaagtcacaagggcaaattcacactaaagtgtaaatgacccacaactcctcttctatttttaggttggggaggtgctttagaacataaggaggaactaaagaatattcctgttacatacaaggcagagaaaagggaaactagtggtgacaagacaaatcatccctttgacatttggctggctctacctattacagctctgggggtgaggtgggaacaaaaagatgctgtgtaaagaagtatcttatgccatccctactgtagtgaggtgcagtttagaggggacactgatcaagcagagacccagagtgtttcgttccaagccagaaacagaaatgtataaaacacagcctttccagcatcagaaatgagtagtggtagtggagaactacccaaaacaggaaagaggaccacgtgaggtagagtgtcaaggccctacattccagtgcctctgctcatgactgtaattttgggtaggtcacttaaagtctctggacctcagttttgccatctgtgaaatagggataatactatccagcataaaattggttatgaggctcatgtagggcctgcctgggatgatgtgttgctaatggttaagaacacaacttctggggtctgactggacaggctgaaatccctgcttaacacgttccagcagagccctgggcgatctatttaacttttgttttctcacctgtaagctgagacgaaagtacccactttataagattattccaataattagttgaaataatgcatgcagagaattaagcatggtacttgttatttgttaaactagctattaaaatgtgtaaaatataaagtattgtatggattttaggacaatgcaaagactctttgcttgctgcaatagttcggggccctttcagatggctaaaggcagaatttgtatgtgtaaatatggtgtgcttgtctctgctctggatactgagggcttaccctgttattaaacttatttagtaaatattgaactgtcatgaggcctaacatttagttccagttattagataaaacatttgctttgaatggtatttgaattgccaggttctagattattctggttgacaaactcttcgtattttataaagaggctaaaattggtaagctatcacagaacagatgtgccattttcaaggtatattaaaccatgattcactgtaacattgttcctactggcaacaaattcagagcaggctggactttatttggtgaagaaacattgagtggaagagaaatgacattattttatgtatttacattttcaaattactgtggcttaaacctgttcagccaacattacccaccttcagtctgctaaataaatgattcagtacatttctaatttacagaattttttaacaaaagaaaatgtaatttgatagccaaatcaacgttaaacattatacatttaaaaaaccacaggcaaagacacaaacatgatgacactaacttttgttaaagtatgcttacctatggtttcctctgaggcacgttctttcatgctaagcttccaacataatatgaaaatgaaggagatgcattttgcaaagcaaaacagaccttaagcaaaatattatacttctcaaattaacactgttacaaagttttagaatttaataagttcattaatttaaaagtttggatgtctgagtccttctatcccaaaacaagatcttggagggtcttccacagccatgtaataccatggtcacatgaccctttccaaaattattaatctgaatttactatatgaggataaatctatctttttgaaaatatttaggaaaatgagcttggtatttataaaatgaagctctctttgggtggtatcctaagacacgtcaagccaatcagcctgtaactgtgaaaaaaacattggtaggtacaaaagtggggtgggagaggagtgacttaactttgttaagtgatgggaaagaaacactaatagcattatctcaataaaatgtgatttaaaaaaatttaaaatactaaatcattgaactgacaaagaaatataaatcattcagaaataaactcattaggtcatcaaatcctgttaaatctgcaattaggaagagcaaggtgtacaatccatacatttaaactcacaggctcactttgcacaacgtcaatttactccttaatatgttattaatacgcattttccaaaaggatgtattagtaaatggtacacatctacttcttggcaacatcatataacctggtacaacataagcattcttcttatagttaagaaatgtggatggtatcaaaattagaaaaataaatgccctattatgttgtggtcaggtttaaggcatgtgaattttatcttcatacaaaagattaaaatctagatattaaaaagtagtgcagtatcagtgatgctgcctcagttcccaaaatgtcacatcacaaaaatatcccataattgcctgtagtttattccttggctttcctcttttctctctgcatctttgtaacaattttttaaaagtggaaatataattgttggcaatgctaacagctgtagaaatgattacaagatgtggaaaagcataacaggaatgtcaagaatctgtttctggcagtaatatatatggaacattgttcaggacaaaagaggagaaggaagaaaaaaaggagaggggtttatcatctctaagaattttcaaactaaacctcattgcttaataggaaaaaaagattccatatttaaagttaagtcacctctaactactagctaaagcatgacatcaccagcactggagtcagcggaagtgtgtttttgaaggacagtgttgcaggagaatctggacaggttttagagccaggagagagaaaataattctacctctgacagttgaaggaccttaggcaaatcagtttacctctgctagactacactccaaaatttggacattcaaaaatttgatattaataaccacatgaaagtctcgtgttgaggtgaatatgtatttgttggtgaaagatatgttggtttttaaacagacagcactctgcaattgtaggctattgttttgttttgccagttgtcaaattctatccagctatacacacttgtgtggcctcctaatggtgtttttccagtggctaaaggtttatgaataagacacttttcctaatggaattaacccgatgcttttcttaaacatgtaaccttgagttcaccgcaaaaaacaatgcttcgattagagcaatgcatataataaaggttaccctcgtttcttagacactagacatcattcacaaaaagagaactgcttttgaaagggatgtatttgcactggaaagaatagttttctacttctaattataaatgatttattggtgaaagcaaaacaacagcctgtctgagaggcacttctatgagcatcctcacgtgtgatttgcaaggttgaagaagagggaaaaatgcctcaattgtaccaatggtgagaaaacacccaaagtacaaagcaggtttcaaaaaaaccatactcataaccaaggacaataataaagcaatgtgttgacatatactctataagtcttcctccataaatagtttatagaaattttgtaatttctgtaaatgcatcctataataattttgcatcttgctttttttttacatttaatatcaagtagatttctaaagggcaattatttgaaaattatcccaaatacatggggaaatatacatcaagtgaaaaaatgcagtgggtgatagagatatcaggaagcgcctcaaatatttctcatctcgttggagaaaaacaaacatgttctcatttagaatgagtgggagttacctaattgatttaggcctctatatttaacttctagtcaaaaaaggtagttctatctagcaacaatattatggggaacaaaagaaaaaattaactctctaaatttgcagtagggtcttttcttcagaagtaccaaatcccatctattaccagctccatgcttcaggcctaaaatggatctccctgaagcaatgacagaatttttgccaagtgactaggatataaacaccactttggttgcacagtgagacatatgctccaaagaaaactggttcaaaaacaggcaagtgggtttctacagaataaatgagagccctgtcaatggcttcatcttcagggctttgtgtctgtgcttgcgtggtggctcttgtttcatctatggataatggtggcacacagttttcataattccttacattaatgaactgctataaatttgtttttggtattctagagagtcctaacttcagcttctgggcaatgctgaggaggcaccctatattctagacttaccttttgcaaggtgtactctcagcattgtgggcgatttccatgggagaatattctatttaaagaactactgtcccagcataaaacaaaaaatcatttatgaagatgcaggagactcggaaagctctcaattattgtttgcacaagcacaatgtcacagcctcctttccccattccacaagggggtcaggaagagagtactcagctgtgagaaaagacatacagaagaattcatgtggtcatgagagcgaggacatggccgatcccccaaggaggatgtgtcatacacttcatgagcccaagagtgtgctgtagggtctgaagggcaagatgctggttcactgatgtaaaggagagggaaaaaagcttcaaccaactagaaaaacagtctctatgcatgctatttttgattttaaacacaggtatcaattccttctctcagagagtccattttaaaataggatacatttttaaaggaatatttaaaggacacattcattaaaatttattttaaaaacttttcaaaagaaacaaaaggtatgaattttatttaatccttgaggaaatggttcttttctcacacacataaatcactcattttgtttttctttatctcctttattaatctacattagaaaaataaacttttcatacactaagaacaaggaaaccactctcaattgacaaaatgttccaatccaacacaatgattactttcacctttaatttacaggcagccagattcaaaatccttaaagttgcttaaacttaaaaatgacaatgacaacctaaaaggtataatgttgattggaacagacatttaattggaaaattgatgattttccatttccaattaaatctctagatagaaatgaaaaaaattaaaaatcgtatttaagaaaagccaaatcttgggttgtgaggtatctttttaaggatgtttcagcagaaaaaaacaaaggctctcacaattgtgtagctgcctagattaagtgggtatcctgatcaaggagatgggggatgatttggctttagtattccaatgataaagtttataatgagaataacatgttgctacaaaatccagtctcttcctcagatgccttccacagagggcaggaagctttgtcagttttgtttgctgatgatgcctggttccgtcaacaaataacacctgtcacacggtgggtagtcaatatacatttgttgaataaatatgaaaaaaagaaatgtacaatatgtttgtgaagccaactgtgtgtgcattgctattgaggtacacaaaaagtctttgttttaaatttgagaatgaggactttcaatggaatatatctgataggcctggatcaagcatgcagctgtggagaacacccctgggactctaactctggcactctgcaagctgggtacttgggcaggacagcagcagcactcatgaactgggcagcacctgttggtgagggctgatcacatggattctctcatcccagccttacaatcagtccttcaggtacatactttttctgactttgctgatgaggaaactatgcacagaggttacacagcttaacaaagggttctcacctaatgaacaatgaaatgggattttagcctttctttgcatctggtcttagagccaatacccaagaagcactgtactgtatgcattgtctcagagaaacttactcttcctgggcctcagtctttaaaaggtgggcagttgacttaataagaattaaagatcaatgattaaggttcaaggcactccaaaattctggtctttattgaaaaggctacagaagtctcaccttaataataccctatagacttgatattcttggttaattaaatattggaaaccaatttcatagtaattgaggtcagaaaaaagtactcatgacattttagaatatgatgacaaagccatagataaatttcaatgcacctgtaattacttaaaactgttatagcatgcaatgtgttaccacaacagccagagaaatactaatttactcagcctattcttctagaccagtaaacactaggattaaatagatattttcattgaatttgttctacccttcattgccatttatagatagcttacttgtcatagattactttctaattgttttatgtttcctaactagcctgcaatactttggcaaggacctcaaacaatagtagacagtaggtgtaaaatagatggctacattgaacagatgactaaaaggatgcctcctaagtacctatatcttgaaatatatattattgtgccttgctttcaatttgtgattttaaaatctagaaatcacctgttttatgtaataacaataaaatccttctttgttgaaaacatgcacaaataaagtttacaagctcaaaaaattaaacagcagtaacggtcaagctttccaacaataaaatacattttggtaaggttttcattttacaaaaactcaaaatagctttatgagttcacaaaataatatgatatttttcaagatattaacatattcttataccggaagagcatagaataaaatttacttggagattgagcatttgcttctttaagaaatacttcttttagtatttttactttaatattatgaaagctacataattacattcagattcattaactactccagtagttaatttttaaaacttatgatgaatagttttgtttaaaatatataacattggtaatatgcaaatctgaatctgtaataaagaaggatttgcattcctgatttttttttctgatacaaccaatgacaaaataactaatggttccacagaggataaaatgtctcaaatctgttggttctgaaggtgaagcgagatttttgtactgataccgtgtatcactgagataccaggaggaaatggaattaaactcagatagttcaaatggagagattttaatgaagggacgacctacagaggtgtcggcagggttggggggaatcagcgagatatgcttagaacccaccgactggcaaacctccccctgaagatggagaaggaggaaggagtgttactggaatgagagcttgagtccaggggaggaggatgggctgctgaggaggcgacaccatcctgaaagaagaatcctctgccagaggcttttcagggtcatttcttcacactctctgcagggaagcacggagacagcaggaagaaatatcctaacctcactctcttccctctacaggtgcttccattggccaaatccacccagaggccagttggtggcgatcagctctcttcaagtggtatttaaatttcttctttcattttccttctggtaacaaagaagtctgtggctcaaaagatgtttctctaagaccccatcctattaggtctctgagctgtgggaagtatttatacaattgcttgtgaatataagatccaggaatttccctaagatccctaacaaaattggtgataagtagtcccacatgttaatccagccacccacggatgacagcacttaccatttctttgataaatgtcaaatgcatttgaagtacctacctgaaatatttgtttaaatgctatctaatctattaattttatatatgtgtgagtctgttttgtataccttctgattataggataaatgtaaataaatccaaagagtaatcaaagctaccactttcaagaagccttctttgtagaaccggaagagtcttaaataggcttttcaggtatgcatctcttattatcgctgaactccaagtcctgcaaggcaggcatcatgtgtgggtcacctttacagtaggcacaggccttaaaacagtgacatgcacattgcaggcactccataaatgtttgctgaattggctaaaccttggtttgttcccataatcaaccaccacaaacagcacacagataattacttcttggaaagattccaactagtgtttgatgttacctacgtggtttttctctcaagatcttaagagcagctctgtaggattacattattttctgttttttttttcctttgaccttaatgtcatctacttcaataacagcttcatacaaaattcctaccagcacataccacagcagattcaaggccttgttttaaaaatggtgccagcttctcttaatttggaagatatattgtctctcctgaacatgggctaagaaaatgtataatttggtattaacataagagctgaagacactttaaatgcattgtttcatttttataagataaaaaaaattttaagaatcaaaatgttatcaacagacttgtccttcattaaaaagtaaaactgcatttgcctacattttatgaaagtgtccaattatgaacaattttgaaatgtaacttttaaaaatgtaaacagcaaaaatgttgtatttaaaataaatctggaaaggcagaaaaacaaaaaatacccagaagacagagtttttggtgaaagttaagatatttcatctttgaacaacttagaatctttcctgcattttatagtctagttccaggcattaatttgaaataaccttggaatcctaaatctaacacccttcggaacaaagtagcttttctcttctgctttatgagcaaatggactaaatactagggaatggtactgtctgggcctttgaaccaagattgaaagagatgaaatcctatatgatatgtataaacattagagaatccattttgatttaataaaaggttgaatttgttctatatcctgtgagaaaatggttcccttttcctgaaaatgttacctcattccaacaatagaaagttggtttttttccagggtgtggtgttggcgggggacagagttgccatgaatatggcatctatgaagactgctgttatattcatttctcaaaatgcactgtggtaggaaattcagaacgcagtgagagaaaataaatgtttgacttcaaaatataaggccgcatttaaagcagaaggtaaagtatagaacagttgacagtataaattctttatctgcaatcttgcagttccctaaatctctgtaacacatcacttttaaaagcctcagataagtggttctataataatttaccaataattcaacccctcaaaagtcttagcaagttaaaccttataatcttacattttagaaatgacccaacttgatccttttattcttcagaatatctctctcaaattttcatttgtttttcattaattgatgaataatgagacattttaggtacctgtccacaaagaaatgaaattttcactttccaggaacctaacaaatgaaaagatagaaatcaattccaacagaatattaccaaagaaatcttttagaatggactgttaaaattatttatttgtatttatctggctctactatttgtggtacatttccacttcaaagctaaacctcaaataacatcatagtgagtggttgacttcatgtttaactgagatcttgaagactgaaaaagaccacgacaaacacacatctattttcttggctactgcatccgtgttcatcaccattctgatagtctgcaatgtattgcagctcaccctttgggaaggactaaagtagacatctgtttgttctgcttactcagcattcctaccctaattttcctttggagaacccctttattctagaccacgtgaagctaatgccaaaccccattccaggggatgcacctgaatccaacctccatcatctaaacagtgccttctccacgttcagagaagagcaagtgactcaaactgccctcataagaacagacctgggacttctgctgcaaatattgaagagtaagtactcttttttcttgctaggactaagctggtagtaccttctatgaggctatcatatggaaacaacttgtctgaaaatgaagccacaactagaaaacagatcctggtaacccggattgatggatccagccctaccttaaatggcaagacctaacccgaggctttttgcatcaaccaataaagtccttaagccagtttgagttggttttgtcacttgcagctaaaagaattctgactctaacaatgtgacaatagcaaaaataaacataactgcttttgaggtttctaatggattttcctccctatatacatgatttcatttaatcctcacaattcaggaaagcacatatctattaacattaaattaatattcattattttgaacacatgctatgtggataagggatgaggaaagccaaggaagtaatcaacgtgaaatctcacttatatgggagggaagtggaggttacatatctcagggcacttaacagatatcatcaaatgaaagaataaacagtgtgtgggagaggcagtaggtgattcttcatcaattcctggatgaaaaattaggagataatgaactccgaacaggcagcctaatgagaatggctcaagcaacaggacatagagagggagttaggttagacatggggttcttgggaattttcacctcgtgggggggcgggggggtcgtgcagctgttgtcagtgggaaagggaaaaaggaaaaggctgagtttggaaggcagggagggaggagacaatgtgagtcagtgaaaaagggcccttagaatgacaagtctggaccagagagaggctaagactgaaaatacaagttgggtaaccactggcatacagatggcagttcaggcttgggcactgcccaccagagcctcagcatgaagagaagagggggaggctggccaccacctccctctaggtaatcgtcatcctgatgctgagctcctgaaaacaggctctttcactcgccccatctcttgctcttgattgcaacccggcattcaggaggcaccctgtaatatctgtggagtgaccgacaacacagcgccagggcactgagaagatcccagggcgccagggactggttctacaagggtgcccctcccggtcccctccagcgcgccgccagagctgccagtcttggctgctacacgggaggcagcctcattatgcagctctcacctcttaaattagttcatgctctcacattaggtgtaatcacagcttgcaacgctttctggggatgtctcagaaagatctgagttgaaaaaatatttttgtgtcattttaatttaaagtaaaattgctgcttcttccccgcccctttctttcctcctggcccacccagcgaccctggccggccgtgctcaacgggggcgggggtcggaggtgagatttcctccacataattccttaaacagctatcaactaagtctcaaagaaaaaaaaaagagatctagaagcagagacgtggctgctggcgatcccaaagctggtgttcgctcttgggggagagcgtaccctgggggaggccgggaggccgggccagaggctagcccagaggcagagggcaggagcgctcagccggcgccccgcgtctctccagctcccgacgctgcgctggctccgctgagcacgccaggatcaaggtcgcctggtggggaccggagcgccaggagcctgtgggaagcgttccagccggcctctgactgggatccggcgccgcgtttctgctttggacttgactgacaggtccccccgccctcccgccgccctactaccagcctgggttcatccttcagggctacgtctaccgcacccgggctggaaagcctggagcgcgcccttcctctcctcatcttctcagctctcctttctccctgccacttggcaaagctgcattttgactttcacgttttggactacgtgtgtgtagttccaagtccatgcgtggcacgaaaatccacttagggtaaaaattattctcgaaaaatcgcccatctcaggatctggtgtctacactcaaggctaggaggtgcaggtacgggtgcgtaaagcatgccgtaagggtgcacagtaaataaaaagtacggatgcaaaatgtaaattttaagtgcaaaacagaaaagcagtactcgttgccgccccgcacgctgggttttaaggggcacgaaggtgggcctcggctgcttttgctcagccccgcgtcctcagcgcccggcccagtacccggtactccgtaggggttcaatgatctcccctgaataagtgaacgaattaacaaatgaatgaatgaccgctcgatccgacctccgcggccggcagagcagtcgctggagaggcgggagagagcgagaggccaagctccaccatcgcggccgccggctggggcagagggacacggagacactcggcgccccggctccgcaccgagtccccg

SEQ ID NO: 17613 - RNA, 12330 nt, Homo sapiens
  source 1..12330: mol_type = other RNA
tcaggccaggcacagtggctcatgcctgtagtcccagcactttgggaggccgaggtgggcagatccacgaggtcaggagatcaagaccatcctaacatggtaaaaccccatctctactaacaatacaaaaaattagtcaggtgtggtggcacgtgcctgtagtcccagctactcaggaggctgaggcaggagaatcgcttgaacctgggaggcggaggttgcagtgagccgagattgtgccactgcaccctagcctaggcaacagagcaagactctgtctcaaaaaaaataaaaaaaaaaaaaagagagaaagagagagagagatgaggagttgctgcactgctgggtgtggagagccgaggaggattcaaagatggtcctgaagtcccagctggaagaagtaggcggcagcaatgtttttaatactgtaaattcatcacgtagcacaggtttggggtggagaaagaaaaattgcattggcttcagggcatgcccagatctttcctcatcttaggcgtttgctaatacatgcattttctaagctgatgtcttgcgtttaatcactgctccattcaaaagagagaaggaggttgtttcaaacctagttgatatcatttgacttccatgctattcacagggctattttatttgaaacaggtataccacagccttaaattgcaagttaatccaggatgttcctaggttggcagttaggaacatgtaattctttggaagggctaaaagtcagctctttaaattatctccatatgaaccttctctccaccttagggtggatccacttatttagtccactgccagtaccacactagaacccgggtggtcactggactccagaaacaacagtagccctctctctgttctgtctctttttgactatctctattctgttcctgaccctgatttctcctgccaagctcaattttgacagctgacaacggcaagccatggcttcccaaaacattattttcaggtcaacttataaatttcaagaacacatttggctccgcttcctgtggtactaagcctacttcttgacagcatttgcctttgttgtaaatagcaaagttcttctagttggatttttgctaagaagtgtgtggatgtggcatgtgacgacatctttagcttggattctagaaaggcactaccattgtgcatttggctaaaggaaacacattttacccgtgaatgccttctatttacaaatgctcagctagcacacaaagctaagtacaagcaataagtactatcctacaatgttactcatttctgaaagcacaaaatgatgactggtatagctttggagatgttttctggaaacccaataaaggaacagatctttgttattccacacctacaaagtcagaagatgcacagtcttttattcatgtttgaacaagcttccttcttgaacaatcaactataaagtgatgtgattctctactagaccaggaactccttgaggacagaatgagggtctaatccatattctaaatccacaccacctggcacaatacatgttgcatggttagggtcaactaagagttggttgaattaatcaataacacacagcaagagaattcacaaagagaggggagtaatcccccagcctcaatcactcggcaagtggaatcgctgggcactgattccagctctgtctcagtgcttgagacagagctgaatgtaatgtgaacatttcaaatgaacaggaaaactagactcacggataagcagtgtagtcatcaagacaacactgtcttggaggtttttctgaagttaaaaccatgctacataagcaataaattatgaaggctgagcatgtgaataaaatttaatgttgtcataaattttataacaaagttaatctgacacatttaatgacatgcataatcattagtatgcagcactgtaatcagacattgataataagcagttcacaccagtgactgtaagagtctttacttgtgttcagccaagccaactgcttggtatatttttctcccttcttagtcgttagttttccatacctacaataactatcagtggtgatgggcttctctgaccatgtgaataatttaatcctcaatgcacagatacagaaacccttgctgaagacagtgtggagcagagaaggctgtctccactccttccacctgaaacacctctgcagatggatatgggagctctgcctacagcccttggacctaaccacttcagtgtgttccagtgagtgtctggacctcggcctgaaagatttttccgaaactaaagaaaatttctctgacctaaagaccttaacctccaccccagaagctctcaccaaggactacagggaactggtggggaaaatccttatcccttactcctcaaggcacagggcagtaatgctgaggcttgtgcgccacacttgctcccagaggtccccagcgggctacctgcggtggtgaatgacctcctaacacgccccttgacggccttcctttccttgcctcacttctccactctcctaccagcattgcagggttcacatcccaaatataccactggcacttgaatcctggtctccaggtctgtttctggaaaaacccaagtaagacattgccccagtaatggggctagatgtctgaggcttcctcaagtatctacctcgaaagctcttactgctgtacacacatgcacatacacacacgtgcgtacaaccagtcacatctaagcaccccgaataccagcctgttgaaggtagcagagagctgcactataagccaaggctgctcccaagagccgctccatcactgaattggcgccccagcaagatgaaggaatgtaatcattggaaggatggagaatgttctctgaatcactgacaaattggaaggggtggagggcaagagtccacctggtggagagatggaaagagcgagagagcctggaatgataatgccattgcttagaaaaggctgctccagatgccatatctacagaaattgtacagcccaaacatctctgagcaataggtctctggtagtcttgatgtctagaccaacaattcccagttcattcttctcagggaaggagccaggatagtccagagactctcattctgctgttagattgaaagggttaggcacaacagccttggcaaagtcacaagggcaaattcacactaaagtgtaaatgacccacaactcctcttctatttttaggttggggaggtgctttagaacataaggaggaactaaagaatattcctgttacatacaaggcagagaaaagggaaactagtggtgacaagacaaatcatccctttgacatttggctggctctacctattacagctctgggggtgaggtgggaacaaaaagatgctgtgtaaagaagtatcttatgccatccctactgtagtgaggtgcagtttagaggggacactgatcaagcagagacccagagtgtttcgttccaagccagaaacagaaatgtataaaacacagcctttccagcatcagaaatgagtagtggtagtggagaactacccaaaacaggaaagaggaccacgtgaggtagagtgtcaaggccctacattccagtgcctctgctcatgactgtaattttgggtaggtcacttaaagtctctggacctcagttttgccatctgtgaaatagggataatactatccagcataaaattggttatgaggctcatgtagggcctgcctgggatgatgtgttgctaatggttaagaacacaacttctggggtctgactggacaggctgaaatccctgcttaacacgttccagcagagccctgggcgatctatttaacttttgttttctcacctgtaagctgagacgaaagtacccactttataagattattccaataattagttgaaataatgcatgcagagaattaagcatggtacttgttatttgttaaactagctattaaaatgtgtaaaatataaagtattgtatggattttaggacaatgcaaagactctttgcttgctgcaatagttcggggccctttcagatggctaaaggcagaatttgtatgtgtaaatatggtgtgcttgtctctgctctggatactgagggcttaccctgttattaaacttatttagtaaatattgaactgtcatgaggcctaacatttagttccagttattagataaaacatttgctttgaatggtatttgaattgccaggttctagattattctggttgacaaactcttcgtattttataaagaggctaaaattggtaagctatcacagaacagatgtgccattttcaaggtatattaaaccatgattcactgtaacattgttcctactggcaacaaattcagagcaggctggactttatttggtgaagaaacattgagtggaagagaaatgacattattttatgtatttacattttcaaattactgtggcttaaacctgttcagccaacattacccaccttcagtctgctaaataaatgattcagtacatttctaatttacagaattttttaacaaaagaaaatgtaatttgatagccaaatcaacgttaaacattatacatttaaaaaaccacaggcaaagacacaaacatgatgacactaacttttgttaaagtatgcttacctatggtttcctctgaggcacgttctttcatgctaagcttccaacataatatgaaaatgaaggagatgcattttgcaaagcaaaacagaccttaagcaaaatattatacttctcaaattaacactgttacaaagttttagaatttaataagttcattaatttaaaagtttggatgtctgagtccttctatcccaaaacaagatcttggagggtcttccacagccatgtaataccatggtcacatgaccctttccaaaattattaatctgaatttactatatgaggataaatctatctttttgaaaatatttaggaaaatgagcttggtatttataaaatgaagctctctttgggtggtatcctaagacacgtcaagccaatcagcctgtaactgtgaaaaaaacattggtaggtacaaaagtggggtgggagaggagtgacttaactttgttaagtgatgggaaagaaacactaatagcattatctcaataaaatgtgatttaaaaaaatttaaaatactaaatcattgaactgacaaagaaatataaatcattcagaaataaactcattaggtcatcaaatcctgttaaatctgcaattaggaagagcaaggtgtacaatccatacatttaaactcacaggctcactttgcacaacgtcaatttactccttaatatgttattaatacgcattttccaaaaggatgtattagtaaatggtacacatctacttcttggcaacatcatataacctggtacaacataagcattcttcttatagttaagaaatgtggatggtatcaaaattagaaaaataaatgccctattatgttgtggtcaggtttaaggcatgtgaattttatcttcatacaaaagattaaaatctagatattaaaaagtagtgcagtatcagtgatgctgcctcagttcccaaaatgtcacatcacaaaaatatcccataattgcctgtagtttattccttggctttcctcttttctctctgcatctttgtaacaattttttaaaagtggaaatataattgttggcaatgctaacagctgtagaaatgattacaagatgtggaaaagcataacaggaatgtcaagaatctgtttctggcagtaatatatatggaacattgttcaggacaaaagaggagaaggaagaaaaaaaggagaggggtttatcatctctaagaattttcaaactaaacctcattgcttaataggaaaaaaagattccatatttaaagttaagtcacctctaactactagctaaagcatgacatcaccagcactggagtcagcggaagtgtgtttttgaaggacagtgttgcaggagaatctggacaggttttagagccaggagagagaaaataattctacctctgacagttgaaggaccttaggcaaatcagtttacctctgctagactacactccaaaatttggacattcaaaaatttgatattaataaccacatgaaagtctcgtgttgaggtgaatatgtatttgttggtgaaagatatgttggtttttaaacagacagcactctgcaattgtaggctattgttttgttttgccagttgtcaaattctatccagctatacacacttgtgtggcctcctaatggtgtttttccagtggctaaaggtttatgaataagacacttttcctaatggaattaacccgatgcttttcttaaacatgtaaccttgagttcaccgcaaaaaacaatgcttcgattagagcaatgcatataataaaggttaccctcgtttcttagacactagacatcattcacaaaaagagaactgcttttgaaagggatgtatttgcactggaaagaatagttttctacttctaattataaatgatttattggtgaaagcaaaacaacagcctgtctgagaggcacttctatgagcatcctcacgtgtgatttgcaaggttgaagaagagggaaaaatgcctcaattgtaccaatggtgagaaaacacccaaagtacaaagcaggtttcaaaaaaaccatactcataaccaaggacaataataaagcaatgtgttgacatatactctataagtcttcctccataaatagtttatagaaattttgtaatttctgtaaatgcatcctataataattttgcatcttgctttttttttacatttaatatcaagtagatttctaaagggcaattatttgaaaattatcccaaatacatggggaaatatacatcaagtgaaaaaatgcagtgggtgatagagatatcaggaagcgcctcaaatatttctcatctcgttggagaaaaacaaacatgttctcatttagaatgagtgggagttacctaattgatttaggcctctatatttaacttctagtcaaaaaaggtagttctatctagcaacaatattatggggaacaaaagaaaaaattaactctctaaatttgcagtagggtcttttcttcagaagtaccaaatcccatctattaccagctccatgcttcaggcctaaaatggatctccctgaagcaatgacagaatttttgccaagtgactaggatataaacaccactttggttgcacagtgagacatatgctccaaagaaaactggttcaaaaacaggcaagtgggtttctacagaataaatgagagccctgtcaatggcttcatcttcagggctttgtgtctgtgcttgcgtggtggctcttgtttcatctatggataatggtggcacacagttttcataattccttacattaatgaactgctataaatttgtttttggtattctagagagtcctaacttcagcttctgggcaatgctgaggaggcaccctatattctagacttaccttttgcaaggtgtactctcagcattgtgggcgatttccatgggagaatattctatttaaagaactactgtcccagcataaaacaaaaaatcatttatgaagatgcaggagactcggaaagctctcaattattgtttgcacaagcacaatgtcacagcctcctttccccattccacaagggggtcaggaagagagtactcagctgtgagaaaagacatacagaagaattcatgtggtcatgagagcgaggacatggccgatcccccaaggaggatgtgtcatacacttcatgagcccaagagtgtgctgtagggtctgaagggcaagatgctggttcactgatgtaaaggagagggaaaaaagcttcaaccaactagaaaaacagtctctatgcatgctatttttgattttaaacacaggtatcaattccttctctcagagagtccattttaaaataggatacatttttaaaggaatatttaaaggacacattcattaaaatttattttaaaaacttttcaaaagaaacaaaaggtatgaattttatttaatccttgaggaaatggttcttttctcacacacataaatcactcattttgtttttctttatctcctttattaatctacattagaaaaataaacttttcatacactaagaacaaggaaaccactctcaattgacaaaatgttccaatccaacacaatgattactttcacctttaatttacaggcagccagattcaaaatccttaaagttgcttaaacttaaaaatgacaatgacaacctaaaaggtataatgttgattggaacagacatttaattggaaaattgatgattttccatttccaattaaatctctagatagaaatgaaaaaaattaaaaatcgtatttaagaaaagccaaatcttgggttgtgaggtatctttttaaggatgtttcagcagaaaaaaacaaaggctctcacaattgtgtagctgcctagattaagtgggtatcctgatcaaggagatgggggatgatttggctttagtattccaatgataaagtttataatgagaataacatgttgctacaaaatccagtctcttcctcagatgccttccacagagggcaggaagctttgtcagttttgtttgctgatgatgcctggttccgtcaacaaataacacctgtcacacggtgggtagtcaatatacatttgttgaataaatatgaaaaaaagaaatgtacaatatgtttgtgaagccaactgtgtgtgcattgctattgaggtacacaaaaagtctttgttttaaatttgagaatgaggactttcaatggaatatatctgataggcctggatcaagcatgcagctgtggagaacacccctgggactctaactctggcactctgcaagctgggtacttgggcaggacagcagcagcactcatgaactgggcagcacctgttggtgagggctgatcacatggattctctcatcccagccttacaatcagtccttcaggtacatactttttctgactttgctgatgaggaaactatgcacagaggttacacagcttaacaaagggttctcacctctcttcaagtggtatttaaatttcttctttcattttccttctggtaacaaagaagtctgtggctcaaaagatgtttctctaagaccccatcctattaggtctctgagattttagaaatgacccaacttgatccttttattcttcagaatatctctctcaaattttcatttgtttttcattaattgatgaataatgagacattttaggtacctgtccacaaagaaatgaaattttcactttccaggaacctaacaaatgaaaagatagaaatcaattccaacagaatattaccaaagaaatcttttagaatggactgttaaaattatttatttgtatttatctggctctactatttgtggtacatttccacttcaaagctaaacctcaaataacatcatagtgagtggttgacttcatgtttaactgagatcttgaagactgaaaaagaccacgacaaacacacatctattttcttggctactgcatccgtgttcatcaccattctgatagtctgcaatgtattgcagctcaccctttgggaaggactaaagtagacatctgtttgttctgcttactcagcattcctaccctaattttcctttggagaacccctttattctagaccacgtgaagctaatgccaaaccccattccaggggatgcacctgaatccaacctccatcatctaaacagtgccttctccacgttcagagaagagcaagtgactcaaactgccctcataagaacagacctgggacttctgctgcaaatattgaagagtaagtactcttttttcttgctaggactaagctggtagtaccttctatgaggctatcatatggaaacaacttgtctgaaaatgaagccacaactagaaaacagatcctggtaacccggattgatggatccagccctaccttaaatggcaagacctaacccgaggctttttgcatcaaccaataaagtccttaagccagtttgagttggttttgtcacttgcagctaaaagaattctgactctaacaatgtgacaatagcaaaaataaacataactgcttttgaggtttctaatggattttcctccctatatacatgatttcatttaatcctcacaattcaggaaagcacatatctattaacattaaattaatattcattattttgaacacatgctatgtggataagggatgaggaaagccaaggaagtaatcaacgtgaaatctcacttatatgggagggaagtggaggttacatatctcagggcacttaacagatatcatcaaatgaaagaataaacagtgtgtgggagaggcagtaggtgattcttcatcaattcctggatgaaaaattaggagataatgaactccgaacaggcagcctaatgagaatggctcaagcaacaggacatagagagggagttaggttagacatggggttcttgggaattttcacctcgtgggggggcgggggggtcgtgcagctgttgtcagtgggaaagggaaaaaggaaaaggctgagtttggaaggcagggagggaggagacaatgtgagtcagtgaaaaagggcccttagaatgacaagtctggaccagagagaggctaagactgaaaatacaagttgggtaaccactggcatacagatggcagttcaggcttgggcactgcccaccagagcctcagcatgaagagaagagggggaggctggccaccacctccctctaggtaatcgtcatcctgatgctgagctcctgaaaacaggctctttcactcgccccatctcttgctcttgattgcaacccggcattcaggaggcaccctgtaatatctgtggagtgaccgacaacacagcgccagggcactgagaagatcccagggcgccagggactggttctacaagggtgcccctcccggtcccctccagcgcgccgccagagctgccagtcttggctgctacacgggaggcagcctcattatgcagctctcacctcttaaattagttcatgctctcacattaggtgtaatcacagcttgcaacgctttctggggatgtctcagaaagatctgagttgaaaaaatatttttgtgtcattttaatttaaagtaaaattgctgcttcttccccgcccctttctttcctcctggcccacccagcgaccctggccggccgtgctcaacgggggcgggggtcggaggtgagatttcctccacataattccttaaacagctatcaactaagtctcaaagaaaaaaaaaagagatctagaagcagagacgtggctgctggcgatcccaaagctggtgttcgctcttgggggagagcgtaccctgggggaggccgggaggccgggccagaggctagcccagaggcagagggcaggagcgctcagccggcgccccgcgtctctccagctcccgacgctgcgctggctccgctgagcacgccaggatcaaggtcgcctggtggggaccggagcgccaggagcctgtgggaagcgttccagccggcctctgactgggatccggcgccgcgtttctgctttggacttgactgacaggtccccccgccctcccgccgccctactaccagcctgggttcatccttcagggctacgtctaccgcacccgggctggaaagcctggagcgcgcccttcctctcctcatcttctcagctctcctttctccctgccacttggcaaagctgcattttgactttcacgttttggactacgtgtgtgtagttccaagtccatgcgtggcacgaaaatccacttagggtaaaaattattctcgaaaaatcgcccatctcaggatctggtgtctacactcaaggctaggaggtgcaggtacgggtgcgtaaagcatgccgtaagggtgcacagtaaataaaaagtacggatgcaaaatgtaaattttaagtgcaaaacagaaaagcagtactcgttgccgccccgcacgctgggttttaaggggcacgaaggtgggcctcggctgcttttgctcagccccgcgtcctcagcgcccggcccagtacccggtactccgtaggggttcaatgatctcccctgaataagtgaacgaattaacaaatgaatgaatgaccgctcgatccgacctccgcggccggcagagcagtcgctggagaggcgggagagagcgagaggccaagctccaccatcgcggccgccggctggggcagagggacacggagacactcggcgccccggctccgcaccgagtccc

SEQ ID NO: 17614 - RNA, 14072 nt, Homo sapiens
  source 1..14072: mol_type = other RNA
tcaggccaggcacagtggctcatgcctgtagtcccagcactttgggaggccgaggtgggcagatccacgaggtcaggagatcaagaccatcctaacatggtaaaaccccatctctactaacaatacaaaaaattagtcaggtgtggtggcacgtgcctgtagtcccagctactcaggaggctgaggcaggagaatcgcttgaacctgggaggcggaggttgcagtgagccgagattgtgccactgcaccctagcctaggcaacagagcaagactctgtctcaaaaaaaataaaaaaaaaaaaaagagagaaagagagagagagatgaggagttgctgcactgctgggtgtggagagccgaggaggattcaaagatggtcctgaagtcccagctggaagaagtaggcggcagcaatgtttttaatactgtaaattcatcacgtagcacaggtttggggtggagaaagaaaaattgcattggcttcagggcatgcccagatctttcctcatcttaggcgtttgctaatacatgcattttctaagctgatgtcttgcgtttaatcactgctccattcaaaagagagaaggaggttgtttcaaacctagttgatatcatttgacttccatgctattcacagggctattttatttgaaacaggtataccacagccttaaattgcaagttaatccaggatgttcctaggttggcagttaggaacatgtaattctttggaagggctaaaagtcagctctttaaattatctccatatgaaccttctctccaccttagggtggatccacttatttagtccactgccagtaccacactagaacccgggtggtcactggactccagaaacaacagtagccctctctctgttctgtctctttttgactatctctattctgttcctgaccctgatttctcctgccaagctcaattttgacagctgacaacggcaagccatggcttcccaaaacattattttcaggtcaacttataaatttcaagaacacatttggctccgcttcctgtggtactaagcctacttcttgacagcatttgcctttgttgtaaatagcaaagttcttctagttggatttttgctaagaagtgtgtggatgtggcatgtgacgacatctttagcttggattctagaaaggcactaccattgtgcatttggctaaaggaaacacattttacccgtgaatgccttctatttacaaatgctcagctagcacacaaagctaagtacaagcaataagtactatcctacaatgttactcatttctgaaagcacaaaatgatgactggtatagctttggagatgttttctggaaacccaataaaggaacagatctttgttattccacacctacaaagtcagaagatgcacagtcttttattcatgtttgaacaagcttccttcttgaacaatcaactataaagtgatgtgattctctactagaccaggaactccttgaggacagaatgagggtctaatccatattctaaatccacaccacctggcacaatacatgttgcatggttagggtcaactaagagttggttgaattaatcaataacacacagcaagagaattcacaaagagaggggagtaatcccccagcctcaatcactcggcaagtggaatcgctgggcactgattccagctctgtctcagtgcttgagacagagctgaatgtaatgtgaacatttcaaatgaacaggaaaactagactcacggataagcagtgtagtcatcaagacaacactgtcttggaggtttttctgaagttaaaaccatgctacataagcaataaattatgaaggctgagcatgtgaataaaatttaatgttgtcataaattttataacaaagttaatctgacacatttaatgacatgcataatcattagtatgcagcactgtaatcagacattgataataagcagttcacaccagtgactgtaagagtctttacttgtgttcagccaagccaactgcttggtatatttttctcccttcttagtcgttagttttccatacctacaataactatcagtggtgatgggcttctctgaccatgtgaataatttaatcctcaatgcacagatacagaaacccttgctgaagacagtgtggagcagagaaggctgtctccactccttccacctgaaacacctctgcagatggatatgggagctctgcctacagcccttggacctaaccacttcagtgtgttccagtgagtgtctggacctcggcctgaaagatttttccgaaactaaagaaaatttctctgacctaaagaccttaacctccaccccagaagctctcaccaaggactacagggaactggtggggaaaatccttatcccttactcctcaaggcacagggcagtaatgctgaggcttgtgcgccacacttgctcccagaggtccccagcgggctacctgcggtggtgaatgacctcctaacacgccccttgacggccttcctttccttgcctcacttctccactctcctaccagcattgcagggttcacatcccaaatataccactggcacttgaatcctggtctccaggtctgtttctggaaaaacccaagtaagacattgccccagtaatggggctagatgtctgaggcttcctcaagtatctacctcgaaagctcttactgctgtacacacatgcacatacacacacgtgcgtacaaccagtcacatctaagcaccccgaataccagcctgttgaaggtagcagagagctgcactataagccaaggctgctcccaagagccgctccatcactgaattggcgccccagcaagatgaaggaatgtaatcattggaaggatggagaatgttctctgaatcactgacaaattggaaggggtggagggcaagagtccacctggtggagagatggaaagagcgagagagcctggaatgataatgccattgcttagaaaaggctgctccagatgccatatctacagaaattgtacagcccaaacatctctgagcaataggtctctggtagtcttgatgtctagaccaacaattcccagttcattcttctcagggaaggagccaggatagtccagagactctcattctgctgttagattgaaagggttaggcacaacagccttggcaaagtcacaagggcaaattcacactaaagtgtaaatgacccacaactcctcttctatttttaggttggggaggtgctttagaacataaggaggaactaaagaatattcctgttacatacaaggcagagaaaagggaaactagtggtgacaagacaaatcatccctttgacatttggctggctctacctattacagctctgggggtgaggtgggaacaaaaagatgctgtgtaaagaagtatcttatgccatccctactgtagtgaggtgcagtttagaggggacactgatcaagcagagacccagagtgtttcgttccaagccagaaacagaaatgtataaaacacagcctttccagcatcagaaatgagtagtggtagtggagaactacccaaaacaggaaagaggaccacgtgaggtagagtgtcaaggccctacattccagtgcctctgctcatgactgtaattttgggtaggtcacttaaagtctctggacctcagttttgccatctgtgaaatagggataatactatccagcataaaattggttatgaggctcatgtagggcctgcctgggatgatgtgttgctaatggttaagaacacaacttctggggtctgactggacaggctgaaatccctgcttaacacgttccagcagagccctgggcgatctatttaacttttgttttctcacctgtaagctgagacgaaagtacccactttataagattattccaataattagttgaaataatgcatgcagagaattaagcatggtacttgttatttgttaaactagctattaaaatgtgtaaaatataaagtattgtatggattttaggacaatgcaaagactctttgcttgctgcaatagttcggggccctttcagatggctaaaggcagaatttgtatgtgtaaatatggtgtgcttgtctctgctctggatactgagggcttaccctgttattaaacttatttagtaaatattgaactgtcatgaggcctaacatttagttccagttattagataaaacatttgctttgaatggtatttgaattgccaggttctagattattctggttgacaaactcttcgtattttataaagaggctaaaattggtaagctatcacagaacagatgtgccattttcaaggtatattaaaccatgattcactgtaacattgttcctactggcaacaaattcagagcaggctggactttatttggtgaagaaacattgagtggaagagaaatgacattattttatgtatttacattttcaaattactgtggcttaaacctgttcagccaacattacccaccttcagtctgctaaataaatgattcagtacatttctaatttacagaattttttaacaaaagaaaatgtaatttgatagccaaatcaacgttaaacattatacatttaaaaaaccacaggcaaagacacaaacatgatgacactaacttttgttaaagtatgcttacctatggtttcctctgaggcacgttctttcatgctaagcttccaacataatatgaaaatgaaggagatgcattttgcaaagcaaaacagaccttaagcaaaatattatacttctcaaattaacactgttacaaagttttagaatttaataagttcattaatttaaaagtttggatgtctgagtccttctatcccaaaacaagatcttggagggtcttccacagccatgtaataccatggtcacatgaccctttccaaaattattaatctgaatttactatatgaggataaatctatctttttgaaaatatttaggaaaatgagcttggtatttataaaatgaagctctctttgggtggtatcctaagacacgtcaagccaatcagcctgtaactgtgaaaaaaacattggtaggtacaaaagtggggtgggagaggagtgacttaactttgttaagtgatgggaaagaaacactaatagcattatctcaataaaatgtgatttaaaaaaatttaaaatactaaatcattgaactgacaaagaaatataaatcattcagaaataaactcattaggtcatcaaatcctgttaaatctgcaattaggaagagcaaggtgtacaatccatacatttaaactcacaggctcactttgcacaacgtcaatttactccttaatatgttattaatacgcattttccaaaaggatgtattagtaaatggtacacatctacttcttggcaacatcatataacctggtacaacataagcattcttcttatagttaagaaatgtggatggtatcaaaattagaaaaataaatgccctattatgttgtggtcaggtttaaggcatgtgaattttatcttcatacaaaagattaaaatctagatattaaaaagtagtgcagtatcagtgatgctgcctcagttcccaaaatgtcacatcacaaaaatatcccataattgcctgtagtttattccttggctttcctcttttctctctgcatctttgtaacaattttttaaaagtggaaatataattgttggcaatgctaacagctgtagaaatgattacaagatgtggaaaagcataacaggaatgtcaagaatctgtttctggcagtaatatatatggaacattgttcaggacaaaagaggagaaggaagaaaaaaaggagaggggtttatcatctctaagaattttcaaactaaacctcattgcttaataggaaaaaaagattccatatttaaagttaagtcacctctaactactagctaaagcatgacatcaccagcactggagtcagcggaagtgtgtttttgaaggacagtgttgcaggagaatctggacaggttttagagccaggagagagaaaataattctacctctgacagttgaaggaccttaggcaaatcagtttacctctgctagactacactccaaaatttggacattcaaaaatttgatattaataaccacatgaaagtctcgtgttgaggtgaatatgtatttgttggtgaaagatatgttggtttttaaacagacagcactctgcaattgtaggctattgttttgttttgccagttgtcaaattctatccagctatacacacttgtgtggcctcctaatggtgtttttccagtggctaaaggtttatgaataagacacttttcctaatggaattaacccgatgcttttcttaaacatgtaaccttgagttcaccgcaaaaaacaatgcttcgattagagcaatgcatataataaaggttaccctcgtttcttagacactagacatcattcacaaaaagagaactgcttttgaaagggatgtatttgcactggaaagaatagttttctacttctaattataaatgatttattggtgaaagcaaaacaacagcctgtctgagaggcacttctatgagcatcctcacgtgtgatttgcaaggttgaagaagagggaaaaatgcctcaattgtaccaatggtgagaaaacacccaaagtacaaagcaggtttcaaaaaaaccatactcataaccaaggacaataataaagcaatgtgttgacatatactctataagtcttcctccataaatagtttatagaaattttgtaatttctgtaaatgcatcctataataattttgcatcttgctttttttttacatttaatatcaagtagatttctaaagggcaattatttgaaaattatcccaaatacatggggaaatatacatcaagtgaaaaaatgcagtgggtgatagagatatcaggaagcgcctcaaatatttctcatctcgttggagaaaaacaaacatgttctcatttagaatgagtgggagttacctaattgatttaggcctctatatttaacttctagtcaaaaaaggtagttctatctagcaacaatattatggggaacaaaagaaaaaattaactctctaaatttgcagtagggtcttttcttcagaagtaccaaatcccatctattaccagctccatgcttcaggcctaaaatggatctccctgaagcaatgacagaatttttgccaagtgactaggatataaacaccactttggttgcacagtgagacatatgctccaaagaaaactggttcaaaaacaggcaagtgggtttctacagaataaatgagagccctgtcaatggcttcatcttcagggctttgtgtctgtgcttgcgtggtggctcttgtttcatctatggataatggtggcacacagttttcataattccttacattaatgaactgctataaatttgtttttggtattctagagagtcctaacttcagcttctgggcaatgctgaggaggcaccctatattctagacttaccttttgcaaggtgtactctcagcattgtgggcgatttccatgggagaatattctatttaaagaactactgtcccagcataaaacaaaaaatcatttatgaagatgcaggagactcggaaagctctcaattattgtttgcacaagcacaatgtcacagcctcctttccccattccacaagggggtcaggaagagagtactcagctgtgagaaaagacatacagaagaattcatgtggtcatgagagcgaggacatggccgatcccccaaggaggatgtgtcatacacttcatgagcccaagagtgtgctgtagggtctgaagggcaagatgctggttcactgatgtaaaggagagggaaaaaagcttcaaccaactagaaaaacagtctctatgcatgctatttttgattttaaacacaggtatcaattccttctctcagagagtccattttaaaataggatacatttttaaaggaatatttaaaggacacattcattaaaatttattttaaaaacttttcaaaagaaacaaaaggtatgaattttatttaatccttgaggaaatggttcttttctcacacacataaatcactcattttgtttttctttatctcctttattaatctacattagaaaaataaacttttcatacactaagaacaaggaaaccactctcaattgacaaaatgttccaatccaacacaatgattactttcacctttaatttacaggcagccagattcaaaatccttaaagttgcttaaacttaaaaatgacaatgacaacctaaaaggtataatgttgattggaacagacatttaattggaaaattgatgattttccatttccaattaaatctctagatagaaatgaaaaaaattaaaaatcgtatttaagaaaagccaaatcttgggttgtgaggtatctttttaaggatgtttcagcagaaaaaaacaaaggctctcacaattgtgtagctgcctagattaagtgggtatcctgatcaaggagatgggggatgatttggctttagtattccaatgataaagtttataatgagaataacatgttgctacaaaatccagtctcttcctcagatgccttccacagagggcaggaagctttgtcagttttgtttgctgatgatgcctggttccgtcaacaaataacacctgtcacacggtgggtagtcaatatacatttgttgaataaatatgaaaaaaagaaatgtacaatatgtttgtgaagccaactgtgtgtgcattgctattgaggtacacaaaaagtctttgttttaaatttgagaatgaggactttcaatggaatatatctgataggcctggatcaagcatgcagctgtggagaacacccctgggactctaactctggcactctgcaagctgggtacttgggcaggacagcagcagcactcatgaactgggcagcacctgttggtgagggctgatcacatggattctctcatcccagccttacaatcagtccttcaggtacatactttttctgactttgctgatgaggaaactatgcacagaggttacacagcttaacaaagggttctcacctctcttcaagtggtatttaaatttcttctttcattttccttctggtaacaaagaagtctgtggctcaaaagatgtttctctaagaccccatcctattaggtctctgagctgtgggaagtatttatacaattgcttgtgaatataagatccaggaatttccctaagatccctaacaaaattggtgataagtagtcccacatgttaatccagccacccacggatgacagcacttaccatttctttgataaatgtcaaatgcatttgaagtacctacctgaaatatttgtttaaatgctatctaatctattaattttatatatgtgtgagtctgttttgtataccttctgattataggataaatgtaaataaatccaaagagtaatcaaagctaccactttcaagaagccttctttgtagaaccggaagagtcttaaataggcttttcaggtatgcatctcttattatcgctgaactccaagtcctgcaaggcaggcatcatgtgtgggtcacctttacagtaggcacaggccttaaaacagtgacatgcacattgcaggcactccataaatgtttgctgaattggctaaaccttggtttgttcccataatcaaccaccacaaacagcacacagataattacttcttggaaagattccaactagtgtttgatgttacctacgtggtttttctctcaagatcttaagagcagctctgtaggattacattattttctgttttttttttcctttgaccttaatgtcatctacttcaataacagcttcatacaaaattcctaccagcacataccacagcagattcaaggccttgttttaaaaatggtgccagcttctcttaatttggaagatatattgtctctcctgaacatgggctaagaaaatgtataatttggtattaacataagagctgaagacactttaaatgcattgtttcatttttataagataaaaaaaattttaagaatcaaaatgttatcaacagacttgtccttcattaaaaagtaaaactgcatttgcctacattttatgaaagtgtccaattatgaacaattttgaaatgtaacttttaaaaatgtaaacagcaaaaatgttgtatttaaaataaatctggaaaggcagaaaaacaaaaaatacccagaagacagagtttttggtgaaagttaagatatttcatctttgaacaacttagaatctttcctgcattttatagtctagttccaggcattaatttgaaataaccttggaatcctaaatctaacacccttcggaacaaagtagcttttctcttctgctttatgagcaaatggactaaatactagggaatggtactgtctgggcctttgaaccaagattgaaagagatgaaatcctatatgatatgtataaacattagagaatccattttgatttaataaaaggttgaatttgttctatatcctgtgagaaaatggttcccttttcctgaaaatgttacctcattccaacaatagaaagttggtttttttccagggtgtggtgttggcgggggacagagttgccatgaatatggcatctatgaagactgctgttatattcatttctcaaaatgcactgtggtaggaaattcagaacgcagtgagagaaaataaatgtttgacttcaaaatataaggccgcatttaaagcagaaggtaaagtatagaacagttgacagtataaattctttatctgcaatcttgcagttccctaaatctctgtaacacatcacttttaaaagcctcagataagtggttctataataatttaccaataattcaacccctcaaaagtcttagcaagttaaaccttataatcttacattttagaaatgacccaacttgatccttttattcttcagaatatctctctcaaattttcatttgtttttcattaattgatgaataatgagacattttaggtacctgtccacaaagaaatgaaattttcactttccaggaacctaacaaatgaaaagatagaaatcaattccaacagaatattaccaaagaaatcttttagaatggactgttaaaattatttatttgtatttatctggctctactatttgtggtacatttccacttcaaagctaaacctcaaataacatcatagtgagtggttgacttcatgtttaactgagatcttgaagactgaaaaagaccacgacaaacacacatctattttcttggctactgcatccgtgttcatcaccattctgatagtctgcaatgtattgcagctcaccctttgggaaggactaaagtagacatctgtttgttctgcttactcagcattcctaccctaattttcctttggagaacccctttattctagaccacgtgaagctaatgccaaaccccattccaggggatgcacctgaatccaacctccatcatctaaacagtgccttctccacgttcagagaagagcaagtgactcaaactgccctcataagaacagacctgggacttctgctgcaaatattgaagagtaagtactcttttttcttgctaggactaagctggtagtaccttctatgaggctatcatatggaaacaacttgtctgaaaatgaagccacaactagaaaacagatcctggtaacccggattgatggatccagccctaccttaaatggcaagacctaacccgaggctttttgcatcaaccaataaagtccttaagccagtttgagttggttttgtcacttgcagctaaaagaattctgactctaacaatgtgacaatagcaaaaataaacataactgcttttgaggtttctaatggattttcctccctatatacatgatttcatttaatcctcacaattcaggaaagcacatatctattaacattaaattaatattcattattttgaacacatgctatgtggataagggatgaggaaagccaaggaagtaatcaacgtgaaatctcacttatatgggagggaagtggaggttacatatctcagggcacttaacagatatcatcaaatgaaagaataaacagtgtgtgggagaggcagtaggtgattcttcatcaattcctggatgaaaaattaggagataatgaactccgaacaggcagcctaatgagaatggctcaagcaacaggacatagagagggagttaggttagacatggggttcttgggaattttcacctcgtgggggggcgggggggtcgtgcagctgttgtcagtgggaaagggaaaaaggaaaaggctgagtttggaaggcagggagggaggagacaatgtgagtcagtgaaaaagggcccttagaatgacaagtctggaccagagagaggctaagactgaaaatacaagttgggtaaccactggcatacagatggcagttcaggcttgggcactgcccaccagagcctcagcatgaagagaagagggggaggctggccaccacctccctctaggtaatcgtcatcctgatgctgagctcctgaaaacaggctctttcactcgccccatctcttgctcttgattgcaacccggcattcaggaggcaccctgtaatatctgtggagtgaccgacaacacagcgccagggcactgagaagatcccagggcgccagggactggttctacaagggtgcccctcccggtcccctccagcgcgccgccagagctgccagtcttggctgctacacgggaggcagcctcattatgcagctctcacctcttaaattagttcatgctctcacattaggtgtaatcacagcttgcaacgctttctggggatgtctcagaaagatctgagttgaaaaaatatttttgtgtcattttaatttaaagtaaaattgctgcttcttccccgcccctttctttcctcctggcccacccagcgaccctggccggccgtgctcaacgggggcgggggtcggaggtgagatttcctccacataattccttaaacagctatcaactaagtctcaaagaaaaaaaaaagagatctagaagcagagacgtggctgctggcgatcccaaagctggtgttcgctcttgggggagagcgtaccctgggggaggccgggaggccgggccagaggctagcccagaggcagagggcaggagcgctcagccggcgccccgcgtctctccagctcccgacgctgcgctggctccgctgagcacgccaggatcaaggtcgcctggtggggaccggagcgccaggagcctgtgggaagcgttccagccggcctctgactgggatccggcgccgcgtttctgctttggacttgactgacaggtccccccgccctcccgccgccctactaccagcctgggttcatccttcagggctacgtctaccgcacccgggctggaaagcctggagcgcgcccttcctctcctcatcttctcagctctcctttctccctgccacttggcaaagctgcattttgactttcacgttttggactacgtgtgtgtagttccaagtccatgcgtggcacgaaaatccacttagggtaaaaattattctcgaaaaatcgcccatctcaggatctggtgtctacactcaaggctaggaggtgcaggtacgggtgcgtaaagcatgccgtaagggtgcacagtaaataaaaagtacggatgcaaaatgtaaattttaagtgcaaaacagaaaagcagtactcgttgccgccccgcacgctgggttttaaggggcacgaaggtgggcctcggctgcttttgctcagccccgcgtcctcagcgcccggcccagtacccggtactccgtaggggttcaatgatctcccctgaataagtgaacgaattaacaaatgaatgaatgaccgctcgatccgacctccgcggccggcagagcagtcgctggagaggcgggagagagcgagaggccaagctccaccatcgcggccgccggctggggcagagggacacggagacactcggcgccccggctccgcaccgagtcc

SEQ ID NO: 17615 - RNA, 14032 nt, Homo sapiens
  source 1..14032: mol_type = other RNA
tcaggccaggcacagtggctcatgcctgtagtcccagcactttgggaggccgaggtgggcagatccacgaggtcaggagatcaagaccatcctaacatggtaaaaccccatctctactaacaatacaaaaaattagtcaggtgtggtggcacgtgcctgtagtcccagctactcaggaggctgaggcaggagaatcgcttgaacctgggaggcggaggttgcagtgagccgagattgtgccactgcaccctagcctaggcaacagagcaagactctgtctcaaaaaaaataaaaaaaaaaaaaagagagaaagagagagagagatgaggagttgctgcactgctgggtgtggagagccgaggaggattcaaagatggtcctgaagtcccagctggaagaagtaggcggcagcaatgtttttaatactgtaaattcatcacgtagcacaggtttggggtggagaaagaaaaattgcattggcttcagggcatgcccagatctttcctcatcttaggcgtttgctaatacatgcattttctaagctgatgtcttgcgtttaatcactgctccattcaaaagagagaaggaggttgtttcaaacctagttgatatcatttgacttccatgctattcacagggctattttatttgaaacaggtataccacagccttaaattgcaagttaatccaggatgttcctaggttggcagttaggaacatgtaattctttggaagggctaaaagtcagctctttaaattatctccatatgaaccttctctccaccttagggtggatccacttatttagtccactgccagtaccacactagaacccgggtggtcactggactccagaaacaacagtagccctctctctgttctgtctctttttgactatctctattctgttcctgaccctgatttctcctgccaagctcaattttgacagctgacaacggcaagccatggcttcccaaaacattattttcaggtcaacttataaatttcaagaacacatttggctccgcttcctgtggtactaagcctacttcttgacagcatttgcctttgttgtaaatagcaaagttcttctagttggatttttgctaagaagtgtgtggatgtggcatgtgacgacatctttagcttggattctagaaaggcactaccattgtgcatttggctaaaggaaacacattttacccgtgaatgccttctatttacaaatgctcagctagcacacaaagctaagtacaagcaataagtactatcctacaatgttactcatttctgaaagcacaaaatgatgactggtatagctttggagatgttttctggaaacccaataaaggaacagatctttgttattccacacctacaaagtcagaagatgcacagtcttttattcatgtttgaacaagcttccttcttgaacaatcaactataaagtgatgtgattctctactagaccaggaactccttgaggacagaatgagggtctaatccatattctaaatccacaccacctggcacaatacatgttgcatggttagggtcaactaagagttggttgaattaatcaataacacacagcaagagaattcacaaagagaggggagtaatcccccagcctcaatcactcggcaagtggaatcgctgggcactgattccagctctgtctcagtgcttgagacagagctgaatgtaatgtgaacatttcaaatgaacaggaaaactagactcacggataagcagtgtagtcatcaagacaacactgtcttggaggtttttctgaagttaaaaccatgctacataagcaataaattatgaaggctgagcatgtgaataaaatttaatgttgtcataaattttataacaaagttaatctgacacatttaatgacatgcataatcattagtatgcagcactgtaatcagacattgataataagcagttcacaccagtgactgtaagagtctttacttgtgttcagccaagccaactgcttggtatatttttctcccttcttagtcgttagttttccatacctacaataactatcagtggtgatgggcttctctgaccatgtgaataatttaatcctcaatgcacagatacagaaacccttgctgaagacagtgtggagcagagaaggctgtctccactccttccacctgaaacacctctgcagatggatatgggagctctgcctacagcccttggacctaaccacttcagtgtgttccagtgagtgtctggacctcggcctgaaagatttttccgaaactaaagaaaatttctctgacctaaagaccttaacctccaccccagaagctctcaccaaggactacagggaactggtggggaaaatccttatcccttactcctcaaggcacagggcagtaatgctgaggcttgtgcgccacacttgctcccagaggtccccagcgggctacctgcggtggtgaatgacctcctaacacgccccttgacggccttcctttccttgcctcacttctccactctcctaccagcattgcagggttcacatcccaaatataccactggcacttgaatcctggtctccaggtctgtttctggaaaaacccaagtaagacattgccccagtaatggggctagatgtctgaggcttcctcaagtatctacctcgaaagctcttactgctgtacacacatgcacatacacacacgtgcgtacaaccagtcacatctaagcaccccgaataccagcctgttgaaggtagcagagagctgcactataagccaaggctgctcccaagagccgctccatcactgaattggcgccccagcaagatgaaggaatgtaatcattggaaggatggagaatgttctctgaatcactgacaaattggaaggggtggagggcaagagtccacctggtggagagatggaaagagcgagagagcctggaatgataatgccattgcttagaaaaggctgctccagatgccatatctacagaaattgtacagcccaaacatctctgagcaataggtctctggtagtcttgatgtctagaccaacaattcccagttcattcttctcagggaaggagccaggatagtccagagactctcattctgctgttagattgaaagggttaggcacaacagccttggcaaagtcacaagggcaaattcacactaaagtgtaaatgacccacaactcctcttctatttttaggttggggaggtgctttagaacataaggaggaactaaagaatattcctgttacatacaaggcagagaaaagggaaactagtggtgacaagacaaatcatccctttgacatttggctggctctacctattacagctctgggggtgaggtgggaacaaaaagatgctgtgtaaagaagtatcttatgccatccctactgtagtgaggtgcagtttagaggggacactgatcaagcagagacccagagtgtttcgttccaagccagaaacagaaatgtataaaacacagcctttccagcatcagaaatgagtagtggtagtggagaactacccaaaacaggaaagaggaccacgtgaggtagagtgtcaaggccctacattccagtgcctctgctcatgactgtaattttgggtaggtcacttaaagtctctggacctcagttttgccatctgtgaaatagggataatactatccagcataaaattggttatgaggctcatgtagggcctgcctgggatgatgtgttgctaatggttaagaacacaacttctggggtctgactggacaggctgaaatccctgcttaacacgttccagcagagccctgggcgatctatttaacttttgttttctcacctgtaagctgagacgaaagtacccactttataagattattccaataattagttgaaataatgcatgcagagaattaagcatggtacttgttatttgttaaactagctattaaaatgtgtaaaatataaagtattgtatggattttaggacaatgcaaagactctttgcttgctgcaatagttcggggccctttcagatggctaaaggcagaatttgtatgtgtaaatatggtgtgcttgtctctgctctggatactgagggcttaccctgttattaaacttatttagtaaatattgaactgtcatgaggcctaacatttagttccagttattagataaaacatttgctttgaatggtatttgaattgccaggttctagattattctggttgacaaactcttcgtattttataaagaggctaaaattggtaagctatcacagaacagatgtgccattttcaaggtatattaaaccatgattcactgtaacattgttcctactggcaacaaattcagagcaggctggactttatttggtgaagaaacattgagtggaagagaaatgacattattttatgtatttacattttcaaattactgtggcttaaacctgttcagccaacattacccaccttcagtctgctaaataaatgattcagtacatttctaatttacagaattttttaacaaaagaaaatgtaatttgatagccaaatcaacgttaaacattatacatttaaaaaaccacaggcaaagacacaaacatgatgacactaacttttgttaaagtatgcttacctatggtttcctctgaggcacgttctttcatgctaagcttccaacataatatgaaaatgaaggagatgcattttgcaaagcaaaacagaccttaagcaaaatattatacttctcaaattaacactgttacaaagttttagaatttaataagttcattaatttaaaagtttggatgtctgagtccttctatcccaaaacaagatcttggagggtcttccacagccatgtaataccatggtcacatgaccctttccaaaattattaatctgaatttactatatgaggataaatctatctttttgaaaatatttaggaaaatgagcttggtatttataaaatgaagctctctttgggtggtatcctaagacacgtcaagccaatcagcctgtaactgtgaaaaaaacattggtaggtacaaaagtggggtgggagaggagtgacttaactttgttaagtgatgggaaagaaacactaatagcattatctcaataaaatgtgatttaaaaaaatttaaaatactaaatcattgaactgacaaagaaatataaatcattcagaaataaactcattaggtcatcaaatcctgttaaatctgcaattaggaagagcaaggtgtacaatccatacatttaaactcacaggctcactttgcacaacgtcaatttactccttaatatgttattaatacgcattttccaaaaggatgtattagtaaatggtacacatctacttcttggcaacatcatataacctggtacaacataagcattcttcttatagttaagaaatgtggatggtatcaaaattagaaaaataaatgccctattatgttgtggtcaggtttaaggcatgtgaattttatcttcatacaaaagattaaaatctagatattaaaaagtagtgcagtatcagtgatgctgcctcagttcccaaaatgtcacatcacaaaaatatcccataattgcctgtagtttattccttggctttcctcttttctctctgcatctttgtaacaattttttaaaagtggaaatataattgttggcaatgctaacagctgtagaaatgattacaagatgtggaaaagcataacaggaatgtcaagaatctgtttctggcagtaatatatatggaacattgttcaggacaaaagaggagaaggaagaaaaaaaggagaggggtttatcatctctaagaattttcaaactaaacctcattgcttaataggaaaaaaagattccatatttaaagttaagtcacctctaactactagctaaagcatgacatcaccagcactggagtcagcggaagtgtgtttttgaaggacagtgttgcaggagaatctggacaggttttagagccaggagagagaaaataattctacctctgacagttgaaggaccttaggcaaatcagtttacctctgctagactacactccaaaatttggacattcaaaaatttgatattaataaccacatgaaagtctcgtgttgaggtgaatatgtatttgttggtgaaagatatgttggtttttaaacagacagcactctgcaattgtaggctattgttttgttttgccagttgtcaaattctatccagctatacacacttgtgtggcctcctaatggtgtttttccagtggctaaaggtttatgaataagacacttttcctaatggaattaacccgatgcttttcttaaacatgtaaccttgagttcaccgcaaaaaacaatgcttcgattagagcaatgcatataataaaggttaccctcgtttcttagacactagacatcattcacaaaaagagaactgcttttgaaagggatgtatttgcactggaaagaatagttttctacttctaattataaatgatttattggtgaaagcaaaacaacagcctgtctgagaggcacttctatgagcatcctcacgtgtgatttgcaaggttgaagaagagggaaaaatgcctcaattgtaccaatggtgagaaaacacccaaagtacaaagcaggtttcaaaaaaaccatactcataaccaaggacaataataaagcaatgtgttgacatatactctataagtcttcctccataaatagtttatagaaattttgtaatttctgtaaatgcatcctataataattttgcatcttgctttttttttacatttaatatcaagtagatttctaaagggcaattatttgaaaattatcccaaatacatggggaaatatacatcaagtgaaaaaatgcagtgggtgatagagatatcaggaagcgcctcaaatatttctcatctcgttggagaaaaacaaacatgttctcatttagaatgagtgggagttacctaattgatttaggcctctatatttaacttctagtcaaaaaaggtagttctatctagcaacaatattatggggaacaaaagaaaaaattaactctctaaatttgcagtagggtcttttcttcagaagtaccaaatcccatctattaccagctccatgcttcaggcctaaaatggatctccctgaagcaatgacagaatttttgccaagtgactaggatataaacaccactttggttgcacagtgagacatatgctccaaagaaaactggttcaaaaacaggcaagtgggtttctacagaataaatgagagccctgtcaatggcttcatcttcagggctttgtgtctgtgcttgcgtggtggctcttgtttcatctatggataatggtggcacacagttttcataattccttacattaatgaactgctataaatttgtttttggtattctagagagtcctaacttcagcttctgggcaatgctgaggaggcaccctatattctagacttaccttttgcaaggtgtactctcagcattgtgggcgatttccatgggagaatattctatttaaagaactactgtcccagcataaaacaaaaaatcatttatgaagatgcaggagactcggaaagctctcaattattgtttgcacaagcacaatgtcacagcctcctttccccattccacaagggggtcaggaagagagtactcagctgtgagaaaagacatacagaagaattcatgtggtcatgagagcgaggacatggccgatcccccaaggaggatgtgtcatacacttcatgagcccaagagtgtgctgtagggtctgaagggcaagatgctggttcactgatgtaaaggagagggaaaaaagcttcaaccaactagaaaaacagtctctatgcatgctatttttgattttaaacacaggtatcaattccttctctcagagagtccattttaaaataggatacatttttaaaggaatatttaaaggacacattcattaaaatttattttaaaaacttttcaaaagaaacaaaaggtatgaattttatttaatccttgaggaaatggttcttttctcacacacataaatcactcattttgtttttctttatctcctttattaatctacattagaaaaataaacttttcatacactaagaacaaggaaaccactctcaattgacaaaatgttccaatccaacacaatgattactttcacctttaatttacaggcagccagattcaaaatccttaaagttgcttaaacttaaaaatgacaatgacaacctaaaaggtataatgttgattggaacagacatttaattggaaaattgatgattttccatttccaattaaatctctagatagaaatgaaaaaaattaaaaatcgtatttaagaaaagccaaatcttgggttgtgaggtatctttttaaggatgtttcagcagaaaaaaacaaaggctctcacaattgtgtagctgcctagattaagtgggtatcctgatcaaggagatgggggatgatttggctttagtattccaatgataaagtttataatgagaataacatgttgctacaaaatccagtctcttcctcagatgccttccacagagggcaggaagctttgtcagttttgtttgctgatgatgcctggttccgtcaacaaataacacctgtcacacggtgggtagtcaatatacatttgttgaataaatatgaaaaaaagaaatgtacaatatgtttgtgaagccaactgtgtgtgcattgctattgaggtacacaaaaagtctttgttttaaatttgagaatgaggactttcaatggaatatatctgataggcctggatcaagcatgcagctgtggagaacacccctgggactctaactctggcactctgcaagctgggtacttgggcaggacagcagcagcactcatgaactgggcagcacctgttggtgagggctgatcacatggattctctcatcccagccttacaatcagtccttcaggtacatactttttctgactttgctgatgaggaaactctcttcaagtggtatttaaatttcttctttcattttccttctggtaacaaagaagtctgtggctcaaaagatgtttctctaagaccccatcctattaggtctctgagctgtgggaagtatttatacaattgcttgtgaatataagatccaggaatttccctaagatccctaacaaaattggtgataagtagtcccacatgttaatccagccacccacggatgacagcacttaccatttctttgataaatgtcaaatgcatttgaagtacctacctgaaatatttgtttaaatgctatctaatctattaattttatatatgtgtgagtctgttttgtataccttctgattataggataaatgtaaataaatccaaagagtaatcaaagctaccactttcaagaagccttctttgtagaaccggaagagtcttaaataggcttttcaggtatgcatctcttattatcgctgaactccaagtcctgcaaggcaggcatcatgtgtgggtcacctttacagtaggcacaggccttaaaacagtgacatgcacattgcaggcactccataaatgtttgctgaattggctaaaccttggtttgttcccataatcaaccaccacaaacagcacacagataattacttcttggaaagattccaactagtgtttgatgttacctacgtggtttttctctcaagatcttaagagcagctctgtaggattacattattttctgttttttttttcctttgaccttaatgtcatctacttcaataacagcttcatacaaaattcctaccagcacataccacagcagattcaaggccttgttttaaaaatggtgccagcttctcttaatttggaagatatattgtctctcctgaacatgggctaagaaaatgtataatttggtattaacataagagctgaagacactttaaatgcattgtttcatttttataagataaaaaaaattttaagaatcaaaatgttatcaacagacttgtccttcattaaaaagtaaaactgcatttgcctacattttatgaaagtgtccaattatgaacaattttgaaatgtaacttttaaaaatgtaaacagcaaaaatgttgtatttaaaataaatctggaaaggcagaaaaacaaaaaatacccagaagacagagtttttggtgaaagttaagatatttcatctttgaacaacttagaatctttcctgcattttatagtctagttccaggcattaatttgaaataaccttggaatcctaaatctaacacccttcggaacaaagtagcttttctcttctgctttatgagcaaatggactaaatactagggaatggtactgtctgggcctttgaaccaagattgaaagagatgaaatcctatatgatatgtataaacattagagaatccattttgatttaataaaaggttgaatttgttctatatcctgtgagaaaatggttcccttttcctgaaaatgttacctcattccaacaatagaaagttggtttttttccagggtgtggtgttggcgggggacagagttgccatgaatatggcatctatgaagactgctgttatattcatttctcaaaatgcactgtggtaggaaattcagaacgcagtgagagaaaataaatgtttgacttcaaaatataaggccgcatttaaagcagaaggtaaagtatagaacagttgacagtataaattctttatctgcaatcttgcagttccctaaatctctgtaacacatcacttttaaaagcctcagataagtggttctataataatttaccaataattcaacccctcaaaagtcttagcaagttaaaccttataatcttacattttagaaatgacccaacttgatccttttattcttcagaatatctctctcaaattttcatttgtttttcattaattgatgaataatgagacattttaggtacctgtccacaaagaaatgaaattttcactttccaggaacctaacaaatgaaaagatagaaatcaattccaacagaatattaccaaagaaatcttttagaatggactgttaaaattatttatttgtatttatctggctctactatttgtggtacatttccacttcaaagctaaacctcaaataacatcatagtgagtggttgacttcatgtttaactgagatcttgaagactgaaaaagaccacgacaaacacacatctattttcttggctactgcatccgtgttcatcaccattctgatagtctgcaatgtattgcagctcaccctttgggaaggactaaagtagacatctgtttgttctgcttactcagcattcctaccctaattttcctttggagaacccctttattctagaccacgtgaagctaatgccaaaccccattccaggggatgcacctgaatccaacctccatcatctaaacagtgccttctccacgttcagagaagagcaagtgactcaaactgccctcataagaacagacctgggacttctgctgcaaatattgaagagtaagtactcttttttcttgctaggactaagctggtagtaccttctatgaggctatcatatggaaacaacttgtctgaaaatgaagccacaactagaaaacagatcctggtaacccggattgatggatccagccctaccttaaatggcaagacctaacccgaggctttttgcatcaaccaataaagtccttaagccagtttgagttggttttgtcacttgcagctaaaagaattctgactctaacaatgtgacaatagcaaaaataaacataactgcttttgaggtttctaatggattttcctccctatatacatgatttcatttaatcctcacaattcaggaaagcacatatctattaacattaaattaatattcattattttgaacacatgctatgtggataagggatgaggaaagccaaggaagtaatcaacgtgaaatctcacttatatgggagggaagtggaggttacatatctcagggcacttaacagatatcatcaaatgaaagaataaacagtgtgtgggagaggcagtaggtgattcttcatcaattcctggatgaaaaattaggagataatgaactccgaacaggcagcctaatgagaatggctcaagcaacaggacatagagagggagttaggttagacatggggttcttgggaattttcacctcgtgggggggcgggggggtcgtgcagctgttgtcagtgggaaagggaaaaaggaaaaggctgagtttggaaggcagggagggaggagacaatgtgagtcagtgaaaaagggcccttagaatgacaagtctggaccagagagaggctaagactgaaaatacaagttgggtaaccactggcatacagatggcagttcaggcttgggcactgcccaccagagcctcagcatgaagagaagagggggaggctggccaccacctccctctaggtaatcgtcatcctgatgctgagctcctgaaaacaggctctttcactcgccccatctcttgctcttgattgcaacccggcattcaggaggcaccctgtaatatctgtggagtgaccgacaacacagcgccagggcactgagaagatcccagggcgccagggactggttctacaagggtgcccctcccggtcccctccagcgcgccgccagagctgccagtcttggctgctacacgggaggcagcctcattatgcagctctcacctcttaaattagttcatgctctcacattaggtgtaatcacagcttgcaacgctttctggggatgtctcagaaagatctgagttgaaaaaatatttttgtgtcattttaatttaaagtaaaattgctgcttcttccccgcccctttctttcctcctggcccacccagcgaccctggccggccgtgctcaacgggggcgggggtcggaggtgagatttcctccacataattccttaaacagctatcaactaagtctcaaagaaaaaaaaaagagatctagaagcagagacgtggctgctggcgatcccaaagctggtgttcgctcttgggggagagcgtaccctgggggaggccgggaggccgggccagaggctagcccagaggcagagggcaggagcgctcagccggcgccccgcgtctctccagctcccgacgctgcgctggctccgctgagcacgccaggatcaaggtcgcctggtggggaccggagcgccaggagcctgtgggaagcgttccagccggcctctgactgggatccggcgccgcgtttctgctttggacttgactgacaggtccccccgccctcccgccgccctactaccagcctgggttcatccttcagggctacgtctaccgcacccgggctggaaagcctggagcgcgcccttcctctcctcatcttctcagctctcctttctccctgccacttggcaaagctgcattttgactttcacgttttggactacgtgtgtgtagttccaagtccatgcgtggcacgaaaatccacttagggtaaaaattattctcgaaaaatcgcccatctcaggatctggtgtctacactcaaggctaggaggtgcaggtacgggtgcgtaaagcatgccgtaagggtgcacagtaaataaaaagtacggatgcaaaatgtaaattttaagtgcaaaacagaaaagcagtactcgttgccgccccgcacgctgggttttaaggggcacgaaggtgggcctcggctgcttttgctcagccccgcgtcctcagcgcccggcccagtacccggtactccgtaggggttcaatgatctcccctgaataagtgaacgaattaacaaatgaatgaatgaccgctcgatccgacctccgcggccggcagagcagtcgctggagaggcgggagagagcgagaggccaagctccaccatcgcggccgccggctggggcagagggacacggagacactcggcgccccggctccgcaccgagtcc

SEQ ID NO: 17616 - RNA, 2065 nt, Homo sapiens
  source 1..2065: mol_type = other RNA
tcaggccaggcacagtggctcatgcctgtagtcccagcactttgggaggctgaggcagggggatcatttgagtcaggagttcgagaccagcctggccaacatggtgaaatcatgtctctactaaaaatagaaaaattagctgggcatggtggcgcatgcctgtaatcccagctactcaggaggctgtggcaggagaatcgcttgaaccggggaggcacaggtttcagtgagctgagatctcgcctctacattccagcctgggtaacgagtgatacttgatctcaaaaaaaaaaaacccaaaacaaaatattgctttaaaatattttttatcttggttgctgagcttttttggtgtcctcttaaaattctgccctggagatgtcaccctagctccagccctgaccttaagagggaggtactagtattatccacatttattttttatttttttaattaaataattaattaattatatttatttttgagacggagtctcgctctgttgcccaggctggagtgcagtggcgctatctcggctcactgcaagctctgcctcccagtttcacgccattctcctgcctcagcctcccaagtagctgggactgcaggtgcccaccaccacacccggctaattttttgtatttttagtagagatggggtttcaccatgttagccaggatggtctcaatctcctgatcttgtgatccacctgcctcggcctcccaaagtgctgggattacaggtgtgagccactgcgcccggcctgttatccacattttataaatgaggaaaccaaggcacagagaggtgaagtgacttgcccaagatcatacagtgggaaaagtggcggagtcaggatttgaatctgggcagcctggctctaggtgctgggctctagatggaaggccctgtctgagctccctgcactaggaacaagtgtggtcaggggctggacggtcagcttttgggtagccattcaagaaatgtattgaaaaacctagagaggcaggctagggagagctgagttggttacatctggggtccatctagggttccatccctggaagagatggtggtggttagggctgtccggagctcctcaggggcaaagacccccagttctgtgatgatgccaccagtgatgaggtcgtggggggtgacatcgaaggcaggattccaaactccaatcccaggtgctgcaatccggaccccattaacatcggtcagctcctggcccggtcgctcttcaataatgatctccttgccggtctccagacggaggtcacatgaagagctgggggcagccacgtagaagggaatgccatggtgcttggcgacaatggccagctggtaggtgcccaccttgttggctgtgtcgccgttggcaaccacgcggtcagctcccacgaccacagctgacacgcccctatgggccatggcagcagccaccatgctgtcggtgataagggtggcggggatctgctcatagaccagctcaaaggccgtcagccgggctccctggttgtagggccgggtctcgagcacagtcccgcccaggggccctcgcagtggcagttccctctgcctggtatgctcttcccaatgctcgcatagctccgtttcacgtctctcccggaccgcctcttccgtagcgccctcccgttcggcctcccgggctgcaacatcagccaggtcgcgggcggcgcgggccatgttgacagcggtgggccgggcggtgacgaggaagctcagcttgtcgcgcacgaaggccacgagcgcggcgagtcccggtcccccggcgcccgcctgcagctccacggcgaggctgagacagcccaccagggctatggccggggcgccccgcaccttcatggcgcggatggcctcccaggcctggtgcaccgagcccaccgcctcgtagcggctctgcttgggcagcagcagctggtctaggatctgcagggagccccgcgagtagcggatcgcctccagggtcatggtgcagcagccaagcccagcgcaactcagagggagctaggggtccgcgcgcacttgggagcggggc

SEQ ID NO: 17617 - RNA, 2119 nt, Homo sapiens
  source 1..2119: mol_type = other RNA
tcaggccaggcacagtggctcatgcctgtagtcccagcactttgggaggctgaggcagggggatcatttgagtcaggagttcgagaccagcctggccaacatggtgaaatcatgtctctactaaaaatagaaaaattagctgggcatggtggcgcatgcctgtaatcccagctactcaggaggctgtggcaggagaatcgcttgaaccggggaggcacaggtttcagtgagctgagatctcgcctctacattccagcctgggtaacgagtgatacttgatctcaaaaaaaaaaaacccaaaacaaaatattgctttaaaatattttttatcttggttgctgagcttttttggtgtcctcttaaaattctgccctggagatgtcaccctagctccagccctgaccttaagagggaggtactagtattatccacatttattttttatttttttaattaaataattaattaattatatttatttttgagacggagtctcgctctgttgcccaggctggagtgcagtggcgctatctcggctcactgcaagctctgcctcccagtttcacgccattctcctgcctcagcctcccaagtagctgggactgcaggtgcccaccaccacacccggctaattttttgtatttttagtagagatggggtttcaccatgttagccaggatggtctcaatctcctgatcttgtgatccacctgcctcggcctcccaaagtgctgggattacaggtgtgagccactgcgcccggcctgttatccacattttataaatgaggaaaccaaggcacagagaggtgaagtgacttgcccaagatcatacagtgggaaaagtggcggagtcaggatttgaatctgggcagcctggctctaggtgctgggctctagatggaaggccctgtctgagctccctgcactaggaacaagtgtggtcaggggctggacggtcagcttttgggtagccattcaagaaatgtattgaaaaacctagagaggcaggctagggagagctgagttggttacatctggggtccatctagggttccatccctggaagagatggtggtggttagggctgtccggagctcctcaggggcaaagacccccagttctgtgatgatgccaccagtgatgaggtcgtggggggtgacatcgaaggcaggattccaaactccaatcccaggtgctgcaatccggaccccattaacatcggtcagctcctggcccggtcgctcttcaataatgatctccttgccggtctccagacggaggtcacatgaagagctgggggcagccacgtagaagggaatgccatggtgcttggcgacaatggccagctggtaggtgcccaccttgttggctgtgtcgccgttggcaaccacgcggtcagctcccacgaccacagctgacacgcccctatgggccatggcagcagccaccatgctgtcggtgataagggtggcggggatctgctcatagaccagctcaaaggccgtcagccgggctccctggttgtagggccgggtctctgtgcagaaggcatgctccaggcggcccaggctgtgcagtgagcgaatcacaccgagcacagtcccgcccaggggccctcgcagtggcagttccctctgcctggtatgctcttcccaatgctcgcatagctccgtttcacgtctctcccggaccgcctcttccgtagcgccctcccgttcggcctcccgggctgcaacatcagccaggtcgcgggcggcgcgggccatgttgacagcggtgggccgggcggtgacgaggaagctcagcttgtcgcgcacgaaggccacgagcgcggcgagtcccggtcccccggcgcccgcctgcagctccacggcgaggctgagacagcccaccagggctatggccggggcgccccgcaccttcatggcgcggatggcctcccaggcctggtgcaccgagcccaccgcctcgtagcggctctgcttgggcagcagcagctggtctaggatctgcagggagccccgcgagtagcggatcgcctccagggtcatggtgcagcagccaagcccagcgcaactcagagggagctaggggtccgcgcgcacttgggagcggggc

SEQ ID NO: 17618 - RNA, 2231 nt, Homo sapiens
  source 1..2231: mol_type = other RNA
tcaggccaggcacagtggctcatgcctgtagtcccagcactttgggaggctgaggcagggggatcatttgagtcaggagttcgagaccagcctggccaacatggtgaaatcatgtctctactaaaaatagaaaaattagctgggcatggtggcgcatgcctgtaatcccagctactcaggaggctgtggcaggagaatcgcttgaaccggggaggcacaggtttcagtgagctgagatctcgcctctacattccagcctgggtaacgagtgatacttgatctcaaaaaaaaaaaacccaaaacaaaatattgctttaaaatattttttatcttggttgctgagcttttttggtgtcctcttaaaattctgccctggagatgtcaccctagctccagccctgaccttaagagggaggtactagtattatccacatttattttttatttttttaattaaataattaattaattatatttatttttgagacggagtctcgctctgttgcccaggctggagtgcagtggcgctatctcggctcactgcaagctctgcctcccagtttcacgccattctcctgcctcagcctcccaagtagctgggactgcaggtgcccaccaccacacccggctaattttttgtatttttagtagagatggggtttcaccatgttagccaggatggtctcaatctcctgatcttgtgatccacctgcctcggcctcccaaagtgctgggattacaggtgtgagccactgcgcccggcctgttatccacattttataaatgaggaaaccaaggcacagagaggtgaagtgacttgcccaagatcatacagtgggaaaagtggcggagtcaggatttgaatctgggcagcctggctctaggtgctgggctctagatggaaggccctgtctgagctccctgcactaggaacaagtgtggtcaggggctggacggtcagcttttgggtagccattcaagaaatgtattgaaaaacctagagaggcaggctagggagagctgagttggttacatctggggtccatctagggttccatccctggaagagatggtggtggttagggctgtccggagctcctcaggggcaaagacccccagttctgtgatgatgccaccagtgatgaggtcgtggggggtgacatcgaaggcaggattccaaactccaatcccaggtgctgcaatccggaccccattaacatcggtcagctcctggcccggtcgctcttcaataatgatctccttgccggtctccagacggaggtcacatgaagagctgggggcagccacgtagaagggaatgccatggtgcttggcgacaatggccagctggtaggtgcccaccttgttggctgtgtcgccgttggcaaccacgcggtcagctcccacgaccacagctgacacgcccctatgggccatggcagcagccaccatgctgtcggtgataagggtggcggggatctgctcatagaccagctcaaaggccgtcagccgggctccctggttgtagggccgggtctctgtgcagaaggcatgctccaggcggcccaggctgtgcagtgagcgaatcacaccgagcacagtcccgcccaggggccctcgcagtggcagttccctctgcctggtatgctcttcccaatgctcgcatagctccgtttcacgtcttgccaccgctgggggccacccgctccaggaggtggcgggctcctaggtccccaatgcttcggttgtctctgaggtctttctccagcatgtcctcggtgcagcagatcactctctcccggaccgcctcttccgtagcgccctcccgttcggcctcccgggctgcaacatcagccaggtcgcgggcggcgcgggccatgttgacagcggtgggccgggcggtgacgaggaagctcagcttgtcgcgcacgaaggccacgagcgcggcgagtcccggtcccccggcgcccgcctgcagctccacggcgaggctgagacagcccaccagggctatggccggggcgccccgcaccttcatggcgcggatggcctcccaggcctggtgcaccgagcccaccgcctcgtagcggctctgcttgggcagcagcagctggtctaggatctgcagggagccccgcgagtagcggatcgcctccagggtcatggtgcagcagccaagcccagcgcaactcagagggagctaggggtccgcgcgcacttgggagcggggc

SEQ ID NO: 17619 - RNA, 2206 nt, Homo sapiens
  source 1..2206: mol_type = other RNA
tcaggccaggcacagtggctcatgcctgtagtcccagcactttgggaggctgaggcagggggatcatttgagtcaggagttcgagaccagcctggccaacatggtgaaatcatgtctctactaaaaatagaaaaattagctgggcatggtggcgcatgcctgtaatcccagctactcaggaggctgtggcaggagaatcgcttgaaccggggaggcacaggtttcagtgagctgagatctcgcctctacattccagcctgggtaacgagtgatacttgatctcaaaaaaaaaaaacccaaaacaaaatattgctttaaaatattttttatcttggttgctgagcttttttggtgtcctcttaaaattctgccctggagatgtcaccctagctccagccctgaccttaagagggaggtactagtattatccacatttattttttatttttttaattaaataattaattaattatatttatttttgagacggagtctcgctctgttgcccaggctggagtgcagtggcgctatctcggctcactgcaagctctgcctcccagtttcacgccattctcctgcctcagcctcccaagtagctgggactgcaggtgcccaccaccacacccggctaattttttgtatttttagtagagatggggtttcaccatgttagccaggatggtctcaatctcctgatcttgtgatccacctgcctcggcctcccaaagtgctgggattacaggtgtgagccactgcgcccggcctgttatccacattttataaatgaggaaaccaaggcacagagaggtgaagtgacttgcccaagatcatacagtgggaaaagtggcggagtcaggatttgaatctgggcagcctggctctaggtgctgggctctagatggaaggccctgtctgagctccctgcactaggaacaagtgtggtcaggggctggacggtcagcttttgggtagccattcaagaaatgtattgaaaaacctagagaggcaggctagggagagctgagttggttacatctggggtccatctagggttccatccctggaagagatggtggtggttagggctgtccggagctcctcaggggcaaagacccccagttctgtgatgatgccaccagtgatgaggtcgtggggggtgacatcgaaggcaggattccaaactccaatcccaggtgctgcaatccggaccccattaacatcggtcagctcctggcccggtcgctcttcaataatgatctccttgccggtctccagacggaggtcacatgaagagctgggggcagccacgtagaagggaatgccatggtgcttggcgacaatggccagctggtaggtgcccaccttgttggctgtgtcgccgttggcaaccacgcggtcagctcccacgaccacagctgacacgcccctatgggccatggcagcagccaccatgctgtcggtgataagggtggcggggatctgctcatagaccagctcaaaggccgtcagccgggctccctggttgtagggccgggtctctgtgcagaaggcatgctccaggcggcccaggctgtgcagtgagcgaatcacacctagggctgtaccatagccagcggtggccagagcaccagtgttacagtgggtcagcacagtcaccttgccaccgctgggggccacccgctccaggaggtggcgggctcctaggtccccaatgcttcggttgtctctgaggtctttctccagcatgtcctcggtgcagcagatcactctctcccggaccgcctcttccgtagcgccctcccgttcggcctcccgggctgcaacatcagccaggtcgcgggcggcgcgggccatgttgacagcggtgggccgggcggtgacgaggaagctcagcttgtcgcgcacgaaggccacgagcgcggcgagtcccggtcccccggcgcccgcctgcagctccacggcgaggctgagacagcccaccagggctatggccggggcgccccgcaccttcatggcgcggatggcctcccaggcctggtgcaccgagcccaccgcctcgtagcggctctgcttgggcagcagcagctggtctaggatctgcagggagccccgcgagtagcggatcgcctccagggtcatggtgcagcagccaagcccagcgcaactcagagggagctaggggtccgcgcgcacttgggagcggggc

SEQ ID NO: 17620 - RNA, 1901 nt, Homo sapiens
  source 1..1901: mol_type = other RNA
tcaggccaggcacagtggctcatgcctgtattgggagggagaggcaatcccatcacttgaggccaggagttccagaccagcctggtgaacatggtgaaaccccatctctactaaaaacacaaaaattagctgggcatggtgaggcatgcctgtaaccccagctactcgggaggctgaggcaggagaatcacttgaacccggaaggcggaggttgcattgagcctagatcgggccactgcactccagcctgtataacagagcaagactctgtctcaaaaagaaaaatcttctaaccctttttcctcgtagcttattttcttctgtgcttcatactttttatttattttttattttttacaataggatccggtttattctgccttggcagggtgatcctgagagtggtgggtgtcaccctctcctgggcagagggaggggccgtgggccagtcaagccaatggtaggagaagcgctggtgaggggtggaatttggggttcaggggtgtaaccccaagaatgcagtgaaaccaggccgaggcccagaggcagctgtggtaggccagggcagggtggaaggcagtggactgggcccgggccgggatgacagggccaaggactcaggccacactggcaccccgggaggcggggcgcagtgtcgcatgacgtagaaaatgaatcacaggcccagggctcacaataagcacatggacaagtgggcacagactcacaggccagatggacctccagccacggccgggccagactcgtggacacaggcgcagtgtcacgtacagaccacggggagacatggcactaggggacaaatggacgtgacaccacaatgcacagggcaggccacagagctcgagggacgtgggcaggggccttttggcatttctgcgctggaatcatgtgagacaagggtggtggccgctctggaggtgcctggggggttccctcattacccctctgggcttagtccatcctccacactgttgtgcagcttctccacctcctggtagaggataaatactgttacccttatccctggtcacatccagggagacgcggtccagcggcccaggcgggggacagtgccgttctagaggtccttgagcccctccttcctcaggatctgcagccataggccggtgtgttccgcgtttgtgctgctccaggccccgcatccggtctcgatcccatccagaggagcgtttcccaagacactggctgcgcccacaatggctccgaagaccccagcgaccagcgggtccatgggcttgctggggttgtcccctcggtaccagctgtgcagggaggtcaggaggagaagcagacggcctggttccagccctgctttagcgtgggtgccatgaggccccggtgagtccccttgttctcgcacaatctctctaacctggtgggagactcctctgcactggaggtctgggaaggtctggccgtggatgaacttcaccttgatggtgtccatggaacatacgaccaccatggcctcggccacgccagcgccctggccgcaccgcagccagcgctgccgtcaggccgtccctgggcatcccgcgtctggctgctgtggaactggaacattcagaacccaacgccgccctggagacaagagccgcagagcagggagccgaggccgcggtgccggcccgggacgccatgaccgcgacagtgcgcacgcgggatccatgcgcggtgcccggctggtgccagcgctcgtccggctgcagctacgacctcccgcgctccgtggggagcggacgcccatttcaatgccgccggccaggccgcctgctggtgtcgccttccccggagcctccgctgggccttcccggacgcggcgcggcgtggccacggcgggcgggaggcgggcgccc

SEQ ID NO: 17621 - RNA, 60 nt, Homo sapiens
  source 1..60: mol_type = other RNA
tcaggccaggcacagtggctcatgcctgtgatcccagcactttaggaggccaaggcggga

SEQ ID NO: 17622 - RNA, 1453 nt, Homo sapiens
  source 1..1453: mol_type = other RNA
tcaggccaggcacagtggctcatgccttgattatggtttgtgggctgtgtccccacccaaatctcatcttgaattgtactcgcataatccccacatgttgtgagagggacccggtgggagataactgaatcatgggagcggtttcccccatactttctcatggtagtgagtaagtatcacgagaactgatggttttataagggatatctgctttcatgtcttcctcatttcctgcttgccgctgccatctaagaagtgccttttgccttctaccataattgtgaggcatccccagccacatggaactgtgagtccaataaacctatttttcttcccagtcttaggtatgtctttatcagcagtgtgaaaatgaactaatacaagcctgtgatcccagcactttgggaagctgaggtgggaggatcccttgaggtcaggagttcgaaaccagcctggccaagaggatgaaaccccatctctacaaaaatacaaaaattagtcaggtgtggtagtgggcacctgtaatcccagccacttgggaggctgagacagaagaatcacttgaacctgggaggtggaagttgcagagagctgagcttgcatcactgcactccagtcagaggaagacttcatctcaaaaacaatacataaataaaattttaaaaaataaaactgttgggggcattagccacacgaacaactgtccaaaagccagggtctctggtttttgttgtttttgtttttacagttttattggttttatttaaaccccaataaaacaaacacattcactgtctattcactttctgcactgtgcaggctggcattggcattggtgactctgatgaccacctgggctgctctttccaagatggctttgcagttcttggaagaaacatcatgagtgatctcaacacagtaagatttgttgctcaccagcagtacttccagctccttaacgttgtggaccaggaacttccagaagccactgggcagtatgtgctttgtctttttgtttctcccataaccaatgttgggcatagatctggccctcaaaccttctatgaaccctgttgttaatacctctgtgtttccaccagttacccttaattttgacatatcagtctgactggttcccagtgaacttggtgctctttttgatgatcttgggcttcgcgagcggtctcaggatggccatgatggaggagatgggtgtcacctccataggcagtgccaaggaagacagctcaggtctttcttaatgaaaccgatatccttcgcgtactgacggaaacactggcggcacatattgaggccatatttccggatcagaccgtgccggtttgaacagacacgacaagagcgagaaccctggccgaattttcgcgggtggctccagtacagctgctggtgacccatcttgctctcagcagtgcaacgaggtaaaaggaag

SEQ ID NO: 17623 - RNA, 535 nt, Homo sapiens
  source 1..535: mol_type = other RNA
tcaggccaggcacagtggctcatgctgtaatcccagcactttagaatagcttgagtccaggagtttgagaccagtctgggcaacatggcaaaaccccatctctgtaccaactgcccaatcctcaaccctcgcctcagcaccaggtggagagcatcctcatctctcctcgtagaacgcttctctgcaaaggccaggaaggtgtgggtggggggtatgtagagcagggctgggatccggtaggtaatccctctgtcatcttcctgccggaacagagggctgttgaaggagcatgttgtcacttcttccatgacctctgcactggaccccggctcctccgtctctgtcggggcagagctggacgccggggattcttccatggggcgcgggggcaggtccgcaggtctcattcgccgaagcccggaagaggcaccggccccaaggctggggagactgagacagaggaggatagagagggagaaacaactgagacggaggacacggagacaagccccgagaagcgaagagcgtgtcgact

SEQ ID NO: 17624 - RNA, 46 nt, Homo sapiens
  source 1..46: mol_type = other RNA
tcaggccaggcacagtggctcatgcttgtaatcccagcactttggg

SEQ ID NO: 17625 - RNA, 192 nt, Homo sapiens
  source 1..192: mol_type = other RNA
tcaggccaggcacagtggctcatgtctatcctcccagcactttgggaggtcaaggatcacttgaagccaggagatcaagaacagcttgggaaagatagcaagaccgggtatctataaaaacaaggtgaaattcacaatgtagatatcaagttaaaaattatcaggcgtgcaaagaagcagagaaatatgacc

SEQ ID NO: 17626 - RNA, 2157 nt, Homo sapiens
  source 1..2157: mol_type = other RNA
tcaggccaggcacagtggctcatgtctgtaaccctagcactttgggaggctgagataggagaattactagggttcaggagtttgagacgaacctgggtgacatagtgagagctcatctctacaaaaaataaaattagctcggcatggtgctgcaagattatagtccctgttagtcgagaggctgaggtgggagaactgcttgagcccaggagggaaagcagcagtgaactgagatcacgccactgcactccagcctgggcgacagtgagaccctgtctcaaaaaaaaaaaaaaaaatgcaagtctggagaaatatagctgggagtcagtaatgccagttttagctgagggagttaagatcatttaatcagtgttaaggaagaaactcaatagtagtgaccaccaatacttaaggaaaaaggataaagtaagaggaatgataaaggctggctgaaatatcttggtgtctagcctaagaaaggaggggttagatgctcatgtttattaatatggatctagagaagcatttattcactaatacattttatttgtgttctctaatttaaaattaccttttcatcttgcttgattttccttcagctaaattagaaatttgtagtttttcccctaaaaaattcaatggcattctttcttataaattacattctctgattttcttgtcagcctgcttcaaggaaatccatgtgttcaaaatgcttgctcgcagtttgctccataccaaatggttgcttaacccaaatatctgagcagcaaattgagctgatccttctggagaaagtacggttgaacagccaagaccactgggtagtcgaagagaagaccacacatcctgaactccccagtctggtgtgaggggaggacagctgataactggatatgcagtgttcccagacatcactggtcccaaaccattacttctgcctgccactgccacaaatacagtaggaatgccatccccttcatactcagctttaatcctcagagtttcatctggtcctttatgcgcagatgttactcgaagttcacatggaatgccaaaatttccacaggccttcttgattttttcacagtgaccaagatcagaagtagagcccatcaacactacaaccctgcactgactttctgatttcaaaagcaactctactctctctgcaacccactcaaagtttttctttaccatttggagcccttcaggagttacttctttgaggtcccgataagactgtttgtctttctgttggcttcgatctcctgatggccagagtctccaggaatcattgtcaataacatcagcaagaacaatttctttggtggttacatcaacaccaaattcaatcttcatatcaaccagtgtacaattctggggcaaccaggatttctccagtatttcaaatatagcctgtgtagcatgactcatgatatccacttcagtctggcctataagaagtccagcaaagcaaaattttgcagcaatcagctgttcctcagaccactgtgggtcattattggcatcatccttgaaaaacaactccactttaggtgggtaaaacttatatccttccttgacaccaggatttcttttgagaaaagaaccagttgctattcttctgcaaacccattcaattggaatcatttcacactgcggtgcaatgaaagctgtctccccacattttctggtgaaggcagttttaatacctgcttcctgtaataactgaaaaatacaactggtgattttatttgagattgcagcttttccttccaggtggttttttctagctgcatttcctgctgtaatctggtccttggactgcaggaggacttttcctggactgtctaacaattcgtagacttcttttgttttaccctcatataattttttaccaatgttcagtacctcagctgtcgccattatcctaagtgggctgagggctgcgaccgcgccgggaagcgaggcagaactcaagtcttgacggcctgggggaagcatgcagggaagggcatatgaaggctaaatgctctgaaagagaaatgaggttaagtccgttactcccattacgctactgttgggtgctggaaaataacggagatttccacgtgcagcaaatacagctttccaggcagctcttaggggaaggct

SEQ ID NO: 17627 - RNA, 1982 nt, Homo sapiens
  source 1..1982: mol_type = other RNA
tcaggccaggcacagtggctcatgtctgtaaccctagcactttgggaggctgagataggagaattactagggttcaggagtttgagacgaacctgggtgacatagtgagagctcatctctacaaaaaataaaattagctcggcatggtgctgcaagattatagtccctgttagtcgagaggctgaggtgggagaactgcttgagcccaggagggaaagcagcagtgaactgagatcacgccactgcactccagcctgggcgacagtgagaccctgtctcaaaaaaaaaaaaaaaaatgcaagtctggagaaatatagctgggagtcagtaatgccagttttagctgagggagttaagatcatttaatcagtgttaaggaagaaactcaatagtagtgaccaccaatacttaaggaaaaaggataaagtaagaggaatgataaaggctggctgaaatatcttggtgtctagcctaagaaaggaggggttagatgctcatgtttattaatatggatctagagaagcatttattcactaatacattttatttgtgttctctaatttaaaattaccttttcatcttgcttgattttccttcagctaaattagaaatttgtagtttttcccctaaaaaattcaatggcattctttcttataaattacattctctgattttcttgtcagcctgcttcaaggaaatccatgtgttcaaaatgcttgctcgcagtttgctccataccaaatggttgcttaacccaaatatctgagcagcaaattgagctgatccttctggagaaagtacggttgaacagccaagaccactgggtagtcgaagagaagaccacacatcctgaactccccagtctggtgtgaggggaggacagctgataactggatatgcagtgttcccagacatcactggtcccaaaccattacttctgcctgccactgccacaaatacagtaggaatgccatccccttcatactcagctttaatcctcagagtttcatctggtcctttatgcgcagatgttactcgaagttcacatggaatgccaaaatttccacaggccttcttgattttttcacagtgaccaagatcagaagtagagcccatcaacactacaaccctgcactgactttctgatttcaaaagcaactctactctctctgcaacccactcaaagtttttctttaccatttggagcccttcaggagttacttctttgaggtcccgataagactgtttgtctttctgttggcttcgatctcctgatggccagagtctccaggaatcattgtcaataacatcagcaagaacaatttctttggtggttacatcaacaccaaattcaatcttcatatcaaccagtgtacaattctggggcaaccaggatttctccagtatttcaaatatagcctgtgtagcatgactcatgatatccacttcagtctggcctataagaagtccagcaaagcaaaattttgcagcaatcagctgttcctcagaccactgtgggtcattattggcatcatccttgaaaaacaactccactttaggtgggtaaaacttatatccttccttgacaccaggatttcttttgagaaaagaaccagttgctattcttctgcaaacccattcaattggaatcatttcacactgcggtgcaatgaaagctgtctccccacattttctggtgaaggcagttttaatacctgcttcctgtaataactgaaaaatacaactggtgattttatttgagattgcagcttttccttccaggtggttttttctagctgcatttcctgctgtaatctggtccttggactgcaggaggacttttcctggactgtctaacaattcgtagacttcttttgttttaccctcatataattttttaccaatgttcagtacctcagctgtcgccattatcctaagtgggctgagggctgcgaccgcgccgggaagcgaggcagaactct

SEQ ID NO: 17628 - RNA, 2003 nt, Homo sapiens
  source 1..2003: mol_type = other RNA
tcaggccaggcacagtggctcatgtctgtaaccctagcactttgggaggctgagataggagaattactagggttcaggagtttgagacgaacctgggtgacatagtgagagctcatctctacaaaaaataaaattagctcggcatggtgctgcaagattatagtccctgttagtcgagaggctgaggtgggagaactgcttgagcccaggagggaaagcagcagtgaactgagatcacgccactgcactccagcctgggcgacagtgagaccctgtctcaaaaaaaaaaaaaaaaatgcaagtctggagaaatatagctgggagtcagtaatgccagttttagctgagggagttaagatcatttaatcagtgttaaggaagaaactcaatagtagtgaccaccaatacttaaggaaaaaggataaagtaagaggaatgataaaggctggctgaaatatcttggtgtctagcctaagaaaggaggggttagatgctcatgtttattaatatggatctagagaagcatttattcactaatacattttatttgtgttctctaatttaaaattaccttttcatcttgcttgattttccttcagctaaattagaaatttgtagtttttcccctaaaaaattcaatggcattctttcttataaattacattctctgattttcttgtcagcctgcttcaaggaaatccatgtgttcaaaatgcttgctcgcagtttgctccataccaaatggttgcttaacccaaatatctgagcagcaaattgagctgatccttctggagaaagtacggttgaacagccaagaccactgggtagtcgaagagaagaccacacatcctgaactccccagtctggtgtgaggggaggacagctgataactggatatgcagtgttcccagacatcactggtcccaaaccattacttctgcctgccactgccacaaatacagtaggaatgccatccccttcatactcagctttaatcctcagagtttcatctggtcctttatgcgcagatgttactcgaagttcacatggaatgccaaaatttccacaggccttcttgattttttcacagtgaccaagatcagaagtagagcccatcaacactacaaccctgcactgactttctgatttcaaaagcaactctactctctctgcaacccactcaaagtttttctttaccatttggagcccttcaggagttacttctttgaggtcccgataagactgtttgtctttctgttggcttcgatctcctgatggccagagtctccaggaatcattgtcaataacatcagcaagaacaatttctttggtggttacatcaacaccaaattcaatcttcatatcaaccagtgtacaattctggggcaaccaggatttctccagtatttcaaatatagcctgtgtagcatgactcatgatatccacttcagtctggcctataagaagtccagcaaagcaaaattttgcagcaatcagctgttcctcagaccactgtgggtcattattggcatcatccttgaaaaacaactccactttaggtgggtaaaacttatatccttccttgacaccaggatttcttttgagaaaagaaccagttgctattcttctgcaaacccattcaattggaatcatttcacactgcggtgcaatgaaagctgtctccccacattttctggtgaaggcagttttaatacgatttgacttatatgaggtaactgcttcctgtaataactgaaaaatacaactggtgattttatttgagattgcagcttttccttccaggtggttttttctagctgcatttcctgctgtaatctggtccttggactgcaggaggacttttcctggactgtctaacaattcgtagacttcttttgttttaccctcatataattttttaccaatgttcagtacctcagctgtcgccattatcctaagtgggctgagggctgcgaccgcgccgggaagcgaggcagaactct

SEQ ID NO: 17629 - RNA, 1821 nt, Homo sapiens
  source 1..1821: mol_type = other RNA
tcaggccaggcacagtggctcatgtctgtaaccctagcactttgggaggctgagataggagaattactagggttcaggagtttgagacgaacctgggtgacatagtgagagctcatctctacaaaaaataaaattagctcggcatggtgctgcaagattatagtccctgttagtcgagaggctgaggtgggagaactgcttgagcccaggagggaaagcagcagtgaactgagatcacgccactgcactccagcctgggcgacagtgagaccctgtctcaaaaaaaaaaaaaaaaatgcaagtctggagaaatatagctgggagtcagtaatgccagttttagctgagggagttaagatcatttaatcagtgttaaggaagaaactcaatagtagtgaccaccaatacttaaggaaaaaggataaagtaagaggaatgataaaggctggctgaaatatcttggtgtctagcctaagaaaggaggggttagatgctcatgtttattaatatggatctagagaagcatttattcactaatacattttatttgtgttctctaatttaaaattaccttttcatcttgcttgattttccttcagctaaattagaaatttgtagtttttcccctaaaaaattcaatggcattctttcttataaattacattctctgattttcttgtcagcctgcttcaaggaaatccatgtgttcaaaatgcttgctcgcagtttgctccataccaaatggttgcttaacccaaatatctgagcagcaaattgagctgatccttctggagaaagtacggttgaacagccaagaccttcatactcagctttaatcctcagagtttcatctggtcctttatgcgcagatgttactcgaagttcacatggaatgccaaaatttccacaggccttcttgattttttcacagtgaccaagatcagaagtagagcccatcaacactacaaccctgcactgactttctgatttcaaaagcaactctactctctctgcaacccactcaaagtttttctttaccatttggagcccttcaggagttacttctttgaggtcccgataagactgtttgtctttctgttggcttcgatctcctgatggccagagtctccaggaatcattgtcaataacatcagcaagaacaatttctttggtggttacatcaacaccaaattcaatcttcatatcaaccagtgtacaattctggggcaaccaggatttctccagtatttcaaatatagcctgtgtagcatgactcatgatatccacttcagtctggcctataagaagtccagcaaagcaaaattttgcagcaatcagctgttcctcagaccactgtgggtcattattggcatcatccttgaaaaacaactccactttaggtgggtaaaacttatatccttccttgacaccaggatttcttttgagaaaagaaccagttgctattcttctgcaaacccattcaattggaatcatttcacactgcggtgcaatgaaagctgtctccccacattttctggtgaaggcagttttaatacctgcttcctgtaataactgaaaaatacaactggtgattttatttgagattgcagcttttccttccaggtggttttttctagctgcatttcctgctgtaatctggtccttggactgcaggaggacttttcctggactgtctaacaattcgtagacttcttttgttttaccctcatataattttttaccaatgttcagtacctcagctgtcgccattatcctaagtgggctgagggctgcgaccgcgccgggaagcgaggcagaact

SEQ ID NO: 17630 - RNA, 2858 nt, Homo sapiens
  source 1..2858: mol_type = other RNA
tcaggccaggcacagtggctcatgtctgtaatcccagcactttgggaggccaaggcgagtggatcacgaggtcaggagttcaagaccattctgggcaacatagtgaaaccccatctctaataaaaatacaaaaattagctggggtgatggcacgtgcctgtagtcccagctacttaggaggctgaggcagaagaatcacttgaacccgggaggcaaaggttgtggtgagccgagatcacgccactgcactgcagcctgggtaacagagtgagactcagtctcaaaaaaaaaaaaaaaagtttggcaaccaagtgaactttttatgtcttcaaataaaatacgtaagatgtttaagatgtatattttaagtgattctcaacttctaccaattacattaataagccaatcaactctttcatcttgatagtgttggatcagaggttttccaccatcctatgattctctgtccagattcaagtgaaaatccaaaaaaacttcaaaagggaagttcaaaaccaaatcattcaaaaaaacttttttccactgagggaatacacacttttcccccctgttgattatatctcctccgggtattttatttaggctactattaaggtccacttgcattttctgcatgtgtgctggtagttgagggtagacacttccccacccatcccccttacaccccacttcaaccccagagtgtgtgggaaggcctcctggccttccagattttccatgggtgatccacacattgggtaatccacatgcccatcatcaaggcctaaccatgttagaaaagggaaggacaatgaagctgcaggaagctcttctagaacatttcactcagctgcctcaaggtcagtcaggggtttgggcatcactttctggagaaagccagagagcaggtgtgaccagctgcagaaagcggaaccctggaattgagaaacctgggctctttagggcagcatctgaagtccttggagctgagcctctggaagaagctgttagggactggccacagcccatgcgatgacattgtggcgtggggtaatgagtaacctacctccacccctagctacacttcttggagagcagcttagattctcatcccactgccaaggtaagagatggatcaggccacaggtaggtagagatgtagcctttggacctgtcccttcatagcccaggattccaaactcaggaacagacactattcatgcaggaacaatctcactgttcatgaggagctggctgcagttaaaggcagaagaagtgtccctctctgagcctcaagttccacatttactagctgaagagagtggatctaaatgtctctctggtcccttccagctgtgcctgcctatgaggctgtgtgtgacccacctgcagtggtgagctcagccagtcactagcaagaaggcataccagccaacaggtcccttctcattggggatgggggtaggggggtgaatgggacatccctgaaattggggtgagaacctaggtcttgccaaaaggcagggcaactgtccccttttagacagaaccaggagatgaggatggggcaatggtctgtcttccaaaaccttgaatctgccagttagggaaggggctgctcctgcagactagcgcaggagagggagagggcggtgccgctctacgacctaactcagctttgtggccagaggaagaggatggggcagggagtcgcttcattttatagcagcgtcttgggatggggccgcctcttgggtctcctcgtcaggcctaggtggggaggttccagggcccggcgctccggtcaccggcctatcattccccctgcagaaggctccgcttctgggcagggaagcggccggggtcagtcggctttgggcgcccggaattcgggcatgctccaggaccgcagtggcggcggtgtgtcccgctccacgtcctcggagatggtcctgatgtcgctggcgaagggcgagatgcgcgcgcgggtcttgaaggtggccaggctgccgcggggccgcaggctccactggcgcgtcagcttgtgggcctcctcttcctgcttcatcctctccaggacctcctgcagcaccgagcggaagagctgggacacctcctgcacctcgggctcctgctccgccagcagctgccggaacctgaggatagcaggcccacaataggatgggtggatcttaacgcagacatcttccagctgcaaccgctcaatggggctgaggtcataggtggaccggggtgtgctggccagccagctgtagtccacaccggtgcagacctttctgaccgcattgctgcgctcccgctgctgcctctcagcctctcgcatctgccccgtcagctccatcataagcgtctccagcaccatctcagcagggctcctggtggacagccgggatggggcctcgttccaccgaagccatgagatgagagacatagcccctggccctctgaggtcagcctctgctcaggtgcagcgtcacagcagggggcctgcgttctgcttcccagtctgggagaagagagtgtctggatattttcaggaaaaaaaaagaaagttgagcagccacagcagggcagggcagtctacatcctcaagtctccctcagcttctctgctgctgccggctggcctcaaattttgcctctctttggttctctgagaagttttaccaagagaagagacaggaggagagatccagcctggactattgtttgtggggtgtgtaggtgtgtgtgtgtgtgtgtgtgtgtgtgtgtgtgtgtgtgtgtgtatgcgtgtatgtatcccgcgaggctggagccacagcttccctgatgaaccatggaggcgggccagctcct

SEQ ID NO: 17631 - RNA, 2861 nt, Homo sapiens
  source 1..2861: mol_type = other RNA
tcaggccaggcacagtggctcatgtctgtaatcccagcactttgggaggccaaggcgagtggatcacgaggtcaggagttcaagaccattctgggcaacatagtgaaaccccatctctaataaaaatacaaaaattagctggggtgatggcacgtgcctgtagtcccagctacttaggaggctgaggcagaagaatcacttgaacccgggaggcaaaggttgtggtgagccgagatcacgccactgcactgcagcctgggtaacagagtgagactcagtctcaaaaaaaaaaaaaaaagtttggcaaccaagtgaactttttatgtcttcaaataaaatacgtaagatgtttaagatgtatattttaagtgattctcaacttctaccaattacattaataagccaatcaactctttcatcttgatagtgttggatcagaggttttccaccatcctatgattctctgtccagattcaagtgaaaatccaaaaaaacttcaaaagggaagttcaaaaccaaatcattcaaaaaaacttttttccactgagggaatacacacttttcccccctgttgattatatctcctccgggtattttatttaggctactattaaggtccacttgcattttctgcatgtgtgctggtagttgagggtagacacttccccacccatcccccttacaccccacttcaaccccagagtgtgtgggaaggcctcctggccttccagattttccatgggtgatccacacattgggtaatccacatgcccatcatcaaggcctaaccatgttagaaaagggaaggacaatgaagctgcaggaagctcttctagaacatttcactcagctgcctcaaggtcagtcaggggtttgggcatcactttctggagaaagccagagagcaggtgtgaccagctgcagaaagcggaaccctggaattgagaaacctgggctctttagggcagcatctgaagtccttggagctgagcctctggaagaagctgttagggactggccacagcccatgcgatgacattgtggcgtggggtaatgagtaacctacctccacccctagctacacttcttggagagcagcttagattctcatcccactgccaaggtaagagatggatcaggccacaggtaggtagagatgtagcctttggacctgtcccttcatagcccaggattccaaactcaggaacagacactattcatgcaggaacaatctcactgttcatgaggagctggctgcagttaaaggcagaagaagtgtccctctctgagcctcaagttccacatttactagctgaagagagtggatctaaatgtctctctggtcccttccagctgtgcctgcctatgaggctgtgtgtgacccacctgcagtggtgagctcagccagtcactagcaagaaggcataccagccaacaggtcccttctcattggggatgggggtaggggggtgaatgggacatccctgaaattggggtgagaacctaggtcttgccaaaaggcagggcaactgtccccttttagacagaaccaggagatgaggatggggcaatggtctgtcttccaaaaccttgaatctgccagttagggaaggggctgctcctgcagactagcgcaggagagggagagggcggtgccgctctacgacctaactcagctttgtggccagaggaagaggatggggcagggagtcgcttcattttatagcagcgtcttgggatggggccgcctcttgggtctcctcgtcaggcctaggtggggaggttccagggcccggcgctccggtcaccggcctatcattccccctgcagaaggctccgcttctgggcagggaagcggccggggtcagtcggctttgggcgcccggaattcgggcatgctccaggaccgcagtggcggcggtgtgtcccgctccacgtcctcggagatggtcctgatgtcgctggcgaagggcgagatgcgcgcgcgggtcttgaaggtggccaggctgccgcggggccgcaggctccactggcgcgtcagcttgtgggcctcctcttcctgcttcatcctctccaggacctcctgcagcaccgagcggaagagctgggacacctcctgcacctcgggctcctgctccgccagcagctgccggaacctgaggatagcaggcccacaataggatgggtggatcttaacgcagacatcttccagctgcaaccgctcaatggggctgaggtcataggtggaccggggtgtgctggccagccagctgtagtccacaccggtgcagacctttctgaccgcattgctgcgctcccgctgctgcctctcagcctctcgcatctgccccgtcagctccatcataagcgtctccagcaccatctcagcagggctcctggtggacagccgggatggggcctcgttccaccgaagccatgagatgagagacatagcccctggccctgctctgaggtcagcctctgctcaggtgcagcgtcacagcagggggcctgcgttctgcttcccagtctgggagaagagagtgtctggatattttcaggaaaaaaaaagaaagttgagcagccacagcagggcagggcagtctacatcctcaagtctccctcagcttctctgctgctgccggctggcctcaaattttgcctctctttggttctctgagaagttttaccaagagaagagacaggaggagagatccagcctggactattgtttgtggggtgtgtaggtgtgtgtgtgtgtgtgtgtgtgtgtgtgtgtgtgtgtgtgtgtatgcgtgtatgtatcccgcgaggctggagccacagcttccctgatgaaccatggaggcgggccagctcct

SEQ ID NO: 17632 - RNA, 2983 nt, Homo sapiens
  source 1..2983: mol_type = other RNA
tcaggccaggcacagtggctcatgtctgtaatcccagcactttgggaggccaaggcgagtggatcacgaggtcaggagttcaagaccattctgggcaacatagtgaaaccccatctctaataaaaatacaaaaattagctggggtgatggcacgtgcctgtagtcccagctacttaggaggctgaggcagaagaatcacttgaacccgggaggcaaaggttgtggtgagccgagatcacgccactgcactgcagcctgggtaacagagtgagactcagtctcaaaaaaaaaaaaaaaagtttggcaaccaagtgaactttttatgtcttcaaataaaatacgtaagatgtttaagatgtatattttaagtgattctcaacttctaccaattacattaataagccaatcaactctttcatcttgatagtgttggatcagaggttttccaccatcctatgattctctgtccagattcaagtgaaaatccaaaaaaacttcaaaagggaagttcaaaaccaaatcattcaaaaaaacttttttccactgagggaatacacacttttcccccctgttgattatatctcctccgggtattttatttaggctactattaaggtccacttgcattttctgcatgtgtgctggtagttgagggtagacacttccccacccatcccccttacaccccacttcaaccccagagtgtgtgggaaggcctcctggccttccagattttccatgggtgatccacacattgggtaatccacatgcccatcatcaaggcctaaccatgttagaaaagggaaggacaatgaagctgcaggaagctcttctagaacatttcactcagctgcctcaaggtcagtcaggggtttgggcatcactttctggagaaagccagagagcaggtgtgaccagctgcagaaagcggaaccctggaattgagaaacctgggctctttagggcagcatctgaagtccttggagctgagcctctggaagaagctgttagggactggccacagcccatgcgatgacattgtggcgtggggtaatgagtaacctacctccacccctagctacacttcttggagagcagcttagattctcatcccactgccaaggtaagagatggatcaggccacaggtaggtagagatgtagcctttggacctgtcccttcatagcccaggattccaaactcaggaacagacactattcatgcaggaacaatctcactgttcatgaggagctggctgcagttaaaggcagaagaagtgtccctctctgagcctcaagttccacatttactagctgaagagagtggatctaaatgtctctctggtcccttccagctgtgcctgcctatgaggctgtgtgtgacccacctgcagtggtgagctcagccagtcactagcaagaaggcataccagccaacaggtcccttctcattggggatgggggtaggggggtgaatgggacatccctgaaattggggtgagaacctaggtcttgccaaaaggcagggcaactgtccccttttagacagaaccaggagatgaggatggggcaatggtctgtcttccaaaaccttgaatctgccagttagggaaggggctgctcctgcagactagcgcaggagagggagagggcggtgccgctctacgacctaactcagctttgtggccagaggaagaggatggggcagggagtcgcttcattttatagcagcgtcttgggatggggccgcctcttgggtctcctcgtcaggcctaggtggggaggttccagggcccggcgctccggtcaccggcctatcattccccctgcagaaggctccgcttctgggcagggaagcggccggggtcagtcggctttgggcgcccggaattcgggcatgctccaggaccgcagtggcggcggtgtgtcccgctccacgtcctcggagatggtcctgatgtcgctggcgaagggcgagatgcgcgcgcgggtcttgaaggtggccaggctgccgcggggccgcaggctccactggcgcgtcagcttgtgggcctcctcttcctgcttcatcctctccaggacctcctgcagcaccgagcggaagagctgggacacctcctgcacctcgggctcctgctccgccagcagctgccggaacctgaggatagcaggcccacaataggatgggtggatcttaacgcagacatcttccagctgcaaccgctcaatggggctgaggtcataggtggaccggggtgtgctggccagccagctgtagtccacaccggtgcagacctttctgaccgcattgctgcgctcccgctgctgcctctcagcctctcgcatctgccccgtcagctccatcataagcgtctccagcaccatctcagcagggctcctggtggacagccgggatggggcctcgttccaccgaagccatgagatgagagacatagcccctggccctgctgagacaggacagatgtgcatctttcctgggcccctctgttagtcagagtggggaacctgggaacccaagggggagagaggagagctgggacccaggagagaagacctgctctgccctaacagttgagtggcctcaagtaggtggcttaatttccctgagcaatcatttctaattctgtaagacaagatagggctgttgtgagaagcagttgtgaataaactttgtacactgtaaacatcacataaaagtaagagactcttgtgattatgatccttaaagcatccccaggattgtgcccagagaaagggcctcctgaatcctcactaactcccaacaaagctggaaacacatggactatggctgagcacaagctttccctatgacttaaggggaacacacacacacacactcagaacagatacatcctatgtcagtctaccaggaaaacaccctcagcttctaaatgcctccagcctattgacgaaagacacttagaactctatggggttggccag

SEQ ID NO: 17633 - RNA, 2339 nt, Homo sapiens
  source 1..2339: mol_type = other RNA
tcaggccaggcacagtggctcatgtctgtaatcccagcactttgggaggctgaggaaggtggatcacttgaggtcaggagttttagaccagtctggtcaacatggtaaaaccccatctctactaagaatacaaaattagccaggcatggtggcgggcacctgtaatcccagctactccggaggctgaggcaggagaattgcttgaactcgggaggcagaggttgcagtgagcaagatcgtaccactgcactccagactgggcgacagagtgagactccatcataggcagtctcctggtgctccacttctcttctcagtctgttgtaatcttctttaacacttcccagctttttgacattcctggaactcaacaccaacagcttgctgaggagtccctccagcccttctctctctgatgttaatgatctaatctcctcggtgaggtctttagccgtccagaaatggtttcctgatatggcatgcattttggcttcaagcaaggctggtagttgggtttcaatatcgttaactttcttcctcagggtgctgcagaatttctcactcatacacaccttagtagtgatttctttaagtgacaagttgagggattttattctttcctggaggctccttatggtttccggtggctctgcatggaagggaatctgaccggctgaggccagggtgtcctgcaaggccttgctgacctcctgcagctgacccagggacagctggcccaccagtggggtcaggtcgcagccctgccactggagttgctgctcttgctcctctatttcccttctcagctgttgatctttggcttccagcacaaacatccttgcttggagagcttcgatttctttctgtagctgctgcttttcctgaagaagccagtctcgtctcgtgatggacacgtgcaagctgtcctgagcagtgggttccaacagcctcggctccattctcagtggggtgtgggtgtcatctccgctggcctgctgagtggccccacggcgcaaggcagcctggacttgtgctgccaggtgacccaggaaactgctaagagctggctgccttgaaggaagttgaaagtgcaggctgattttctcttgttccaggtcttctaatctttgttgtaacgtctcagctttatcataatcatcattctcaactgcatcttcctgaagtttctgaagttttaatcttaaggatattacctccatctgcctccggtttctcagcaggcagtcccgcagcactggctcccatttcctgagcagggtgtcccaagagtgggcatcccctgagccgctgctcccatcaccaccacagccagccagtgagggatccagagaactggaggagccagggtccatgtctggtaaagaatgcatgtcacgctctggcctggagctgttccttgcggcctgggccaagtctgcagagacccgtgtagccaagagactgaagggccgagagagacatcgcgggtcctcgtgaggcccgtccaagctggcagctttggctcccatctcctgggggctctggcaatgggactcagcctctctggatggtgggcagccttctgcttctccacgttccccggcagagccaagcgagagccgaataaagctaaagcttgaggtaaaggcactgtgagagccaggaggggttggggggacctcagggccacagccagggctgcagctgttgctactcaactctgctgatggcagagagcctgctgcccggacacgccttgctccatcgctgcaggctgcctcccagctggcgtccagggtctcagaactatccatggctgcaaactcttgctgccacccagcactcccagggccacacggccagctaagcctgtcaggcaatctggtgccacctctgagctgaatcccaaagtgcgccgaggttcctctcacagaggtcacagtaggggctgctgcactcttggaaacagggctccggaccaagaggcctctcgagtcaaggccacactgtctggccctggactccgagtggtgggactcctcgccagacacccctcctgggaaccggaacagtgtgcccactgctggggaaaggaacccgatcccaggccctgtcgagcttctcatgtagcccggcctccgtgccagccgccgcctccgaaagcacgctgcaggtggtaagcaatcccggctgcctgcgcggtggctcacgccgccgccgccggcggcggctggggcgccctgaggacccccgcctggcatgcgccccgctgccagctcctcccgctccgcctgggctgcctcctgctccttccccgaggccagaggcggggggaaggg

SEQ ID NO: 17634 - RNA, 2055 nt, Homo sapiens
  source 1..2055: mol_type = other RNA
tcaggccaggcacagtggctcatgtctgtaatcccagcactttgggaggctgaggtgggtggaccgcttgagtctaggtgttcaggaccagcctggcagcatggtgaaaccctgtctttacaaaaaatacaaaaaaattacctgagtgtggtgggatgcgcttgtggtcccaagctactcggaaggctgaggtgggaggaccgcttgaggccaggagttggaggttgcagtgagctatgtttgtgccactgcactccagcctgggtgacagagcaagacccttcactgcagcctgcagagacatggactgcagcctggagagacgctcaggactcagctcagccatgcgcagattcccgacccacagaaactgaacaaacttgaagatggcaaatgctggggcgctgtcttcagaatacagaaagcccaagatactaagcagctgggtattaaagcagctgtctccaaggcccaacagaaaactgcagagaatggcaacttctttgctggatttgatgtaagcactgctgtcagttcctttaacaggagcaatcggggcatctccaggcatgttgagaaatattagataaaaagctatgaagtgcaccaggatgcccaacagcacaactggatttctaccaaaacgattgttcttgctcagcaggccgaagaggcttccacctaaaatttctccaatgccgatgaaaatgccagaaagtccaataaggcttttctcttctgctccaaatttatttgtagcaccaatacaggttccatatacaccagagaagaaagttaattccagacctgtataagcagttgtaatactaagaaggagcatctccttggtgacacataacttaaaagactttttaaaagcatctactgcctttgtcagattgttctgggcagactcgttgacttccatgtcctggtcatcagaagactcatcttctcctaggacattttcagaatctggtttccgaatgagaaagaatagaactgtccccacaaggctaatcaccgttagggcaataaacactgttcttcggtcactctctagactgcagaagtgcccagaaaatcccactgtttctcccaatgctgtgctcatccgaattgattgtcaggcagtttccttgtgctgtccaaagcacagcagcagcaattccaatgaaaacagaggctgtgtagaaggaccacgggaaaggctggatgaaaacggcaatgtacatgctgtaaaataaaccactggcaaacatagagagttgaggtcctacaatggcaaccactgacggtgtaatcaaatttgaagcagagaacactccatagataatagccatgctggtatatccactgccgtgaaaatctgtcctatttaagctcctgatgacagtttgcgccacatttccacaagtttgaaaggcagtgaacataaacataaaggcaactcctaaaataatgatgttgaaaagctttttagattccggggacattttggctcagctctgccggaggcagcagcccagggcagtcagctctcctcggggcgaagccactgacaatccggcagttaggatactcctaagaagcgatccgagtacggaagagcacaacccccggagaagcgccaagaatttatccgctccaggttgaggggcccacgaaggggattaaagggccaagtgccagccgcagcagccggcgcggccccgccctcccagcctgactcactgcggccaggcgaccgggtcacctgaccgcagccgcggcgccggccgctcggcccgctgggaaacgtagtcccgggtggcctggcacgcgcaagcgctccgcggggagtccccaccgccaggacgcagagccgacggagctctcgggctctggcgaaagggggttgggaagcggactccggcgaagagcagtcaggaacggctggacggggccgagagacgacgcagcggagtctgagggggccggggtcacagggagaggcaaatgagggcagaagcactcttcagacggagacggggctgacggctgagcaaaaaaggg

SEQ ID NO: 17635 - RNA, 2154 nt, Homo sapiens
  source 1..2154: mol_type = other RNA
tcaggccaggcacagtggctcatgtctgtaatcccagcactttgggaggctgaggtgggtggaccgcttgagtctaggtgttcaggaccagcctggcagcatggtgaaaccctgtctttacaaaaaatacaaaaaaattacctgagtgtggtgggatgcgcttgtggtcccaagctactcggaaggctgaggtgggaggaccgcttgaggccaggagttggaggttgcagtgagctatgtttgtgccactgcactccagcctgggtgacagagcaagacccttcactgcagcctgcagagacatggactgcagcctggagagacgctcaggactcagctcagccatgcgcagattcccgacccacagaaactgaacaaacttgaagatggcaaatgctggggcgctgtcttcagaatacagaaagcccaagatactaagcagctgggtattaaagcagctgtctccaaggcccaacagaaaactgcagagaatggcaacttctttgctggatttgatgtaagcactgctgtcagttcctttaacaggagcaatcggggcatctccaggcatgttgagaaatattagataaaaagctatgaagtgcaccaggatgcccaacagcacaactggatttctaccaaaacgattgttcttgctcagcaggccgaagaggcttccacctaaaatttctccaatgccgatgaaaatgccagaaagtccaataaggcttttctcttctgctccaaatttatttgtagcaccaatacaggttccatatacaccagagaagaaagttaattccagacctgtataagcagttgtaatactaagaaggagcatctccttggtgacacataacttaaaagactttttaaaagcatctactgcctttgtcagattgttctgggcagactcgttgacttccatgtcctggtcatcagaagactcatcttctcctaggacattttcagaatctggtttccgaatgagaaagaatagaactgtccccacaaggctaatcaccgttagggcaataaacactgttcttcggtcactctctgatatctgagttttcccttgccaggcaaaatatatgtagagatttccaaagaacaagctagactgcagaagtgcccagaaaatcccactgtttctcccaatgctgtgctcatccgaattgattgtcaggcagtttccttgtgctgtccaaagcacagcagcagcaattccaatgaaaacagaggctgtgtagaaggaccacgggaaaggctggatgaaaacggcaatgtacatgctaaaatataacaggtcaaggtattacagtcaaacgatacctgtaaaataaaccactggcaaacatagagagttgaggtcctacaatggcaaccactgacggtgtaatcaaatttgaagcagagaacactccatagataatagccatgctggtatatccactgccgtgaaaatctgtcctatttaagctcctgatgacagtttgcgccacatttccacaagtttgaaaggcagtgaacataaacataaaggcaactcctaaaataatgatgttgaaaagctttttagattccggggacattttggctcagctctgccggaggcagcagcccagggcagtcagctctcctcggggcgaagccactgacaatccggcagttaggatactcctaagaagcgatccgagtacggaagagcacaacccccggagaagcgccaagaatttatccgctccaggttgaggggcccacgaaggggattaaagggccaagtgccagccgcagcagccggcgcggccccgccctcccagcctgactcactgcggccaggcgaccgggtcacctgaccgcagccgcggcgccggccgctcggcccgctgggaaacgtagtcccgggtggcctggcacgcgcaagcgctccgcggggagtccccaccgccaggacgcagagccgacggagctctcgggctctggcgaaagggggttgggaagcggactccggcgaagagcagtcaggaacggctggacggggccgagagacgacgcagcggagtctgagggggccggggtcacagggagaggcaaatgagggcagaagcactcttcagacggagacggggctgacggctgagcaaaaaaggg

SEQ ID NO: 17636 - RNA, 2717 nt, Homo sapiens
  source 1..2717: mol_type = other RNA
tcaggccaggcacagtggctcatgtctgtaatcccagcactttgggaggctgaggtgggtggaccgcttgagtctaggtgttcaggaccagcctggcagcatggtgaaaccctgtctttacaaaaaatacaaaaaaattacctgagtgtggtgggatgcgcttgtggtcccaagctactcggaaggctgaggtgggaggaccgcttgaggccaggagttggaggttgcagtgagctatgtttgtgccactgcactccagcctgggtgacagagcaagacccttcactgcagcctgcagagacatggactgcagcctggagagacgctcaggactcagctcagccatgcgcagattcccgacccacagaaactgaacaaacttgaagatggcaaatgctggggcgctgtcttcagaatacagaaagcccaagatactaagcagctgggtattaaagcagctgtctccaaggcccaacagaaaactgcagagaatggcaacttctttgctggatttgatgtaagcactgctgtcagttcctttaacaggagcaatcggggcatctccaggcatgttgagaaatattagataaaaagctatgaagtgcaccaggatgcccaacagcacaactggatttctaccaaaacgattgttcttgctcagcaggccgaagaggcttccacctaaaatttctccaatgccgatgaaaatgccagaaagtccaataaggcttttctcttctgctccaaatttatttgtagcaccaatacaggttccatatacaccagagaagaaagttaattccagacctgtataagcagttgtaatactaagaaggagcatctccttggtgacacataacttaaaagactttttaaaagcatctactgcctttgtcagattgttctgggcagactcgttgacttccatgtcctggtcatcagaagactcatcttctcctaggacattttcagaatctggtttccgaatgagaaagaatagaactgtccccacaaggctaatcaccgttagggcaataaacactgttcttcggtcactctctgatatctgagttttcccttgccaggcaaaatatatgtagagatttccaaagaacaagctagactgcagaagtgcccagaaaatcccactgtttctcccaatgctgtgctcatccgaattgattgtcaggcagtttccttgtgctgtccaaagcacagcagcagcaattccaatgaaaacagaggctgtgtagaaggaccacgggaaaggctggatgaaaacggcaatgtacatgctgtaaaataaaccactggcaaacatagagagttgaggtcctacaatggcaaccactgacggtgtaatcaaatttgaagcagagaacactccatagataatagccatgctggtatatccactgccgtgaaaatctgtcctatttaagctcctgatgacagtttgcgccacatttccacaagtttgaaaggcagtgaacataaacataaaggcaactcctaaaataatgatgttgaaaagctttttagattccggggacattttggctcagctctgccggaggcagcagcccagggcagtcagctctcctcggggcgaagccactgacaatccgccaggacgcagagccgacggagctctcgggctctggcgaaagggggttgggaagcggactccggcgaagagcagtcaggaacggctggacggggccgagagacgacgcagcggagtctgagggggccggggtcacagggagaggcaaatgagggcagaagcactcttcagacggagacggggctgacggctgagcaaaaaaggggcgtgaacttggagtattggcatgaaaaaaaggtgggggcccagatggggagcacctcctcttcctcctgcccaatcgcgatcgtccggcctcccaggcggaaaaagcgtttcgcgggctttccaactgcccgctaattccgctccccctccctccagccgtgactccgcgctttttggcccgcccgccgggctgtgcgcaggcgcttcgggtaggggcggggcgcgcggcagggtcgttacgaagcggggcgcggtgggccaatcagaaggtttcatttccgggtggcgcgggcgccattttgtgaggagcgatataaacgggcgcagaggccggctgcccgcccagttgttactcaggtgcgctagcctgcggagcccgtccgtgctgttctgcggcaaggcctttcccagtgtccccacgcggaaggcaactgcctgagaggcgcggcgtcgcaccgcccagagctgaggaagccggcgccagttcgcggggctccgggccgccactcagagctatgagctacggccgcccccctcccgatgtggagggtatgacctccctcaaggtggacaacctgacctaccgcacctcgcccgacacgctgaggcgcgtcttcgagaagtacgggcgcgtcggcgacgtgtacatcccgcgggaccgctacaccaaggagtcccgcggcttcgccttcgttcgctttcacgacaagcgcgacgctgaggacgctatggatgccatggacggggccgtgctggacggccgcgagctgcgggtgcaaatggcgcgctacggccgccccccggactcacaccacagccgccggggaccgccaccccgcaggtacgggggcggtggctacggacgccggagccgcaggtaaac

SEQ ID NO: 17637 - RNA, 2114 nt, Homo sapiens
  source 1..2114: mol_type = other RNA
tcaggccaggcacagtggctcatgtctgtaatcccagcactttgggaggctgaggtgggtggaccgcttgagtctaggtgttcaggaccagcctggcagcatggtgaaaccctgtctttacaaaaaatacaaaaaaattacctgagtgtggtgggatgcgcttgtggtcccaagctactcggaaggctgaggtgggaggaccgcttgaggccaggagttggaggttgcagtgagctatgtttgtgccactgcactccagcctgggtgacagagcaagacccttcactgcagcctgcagagacatggactgcagcctggagagacgctcaggactcagctcagccatgcgcagattcccgacccacagaaactgaacaaacttgaagatggcaaatgctggggcgctgtcttcagaatacagaaagcccaagatactaagcagctgggtattaaagcagctgtctccaaggcccaacagaaaactgcagagaatggcaacttctttgctggatttgatgtaagcactgctgtcagttcctttaacaggagcaatcggggcatctccaggcatgttgagaaatattagataaaaagctatgaagtgcaccaggatgcccaacagcacaactggatttctaccaaaacgattgttcttgctcagcaggccgaagaggcttccacctaaaatttctccaatgccgatgaaaatgccagaaagtccaataaggcttttctcttctgctccaaatttatttgtagcaccaatacaggttccatatacaccagagaagaaagttaattccagacctgtataagcagttgtaatactaagaaggagcatctccttggtgacacataacttaaaagactttttaaaagcatctactgcctttgtcagattgttctgggcagactcgttgacttccatgtcctggtcatcagaagactcatcttctcctaggacattttcagaatctggtttccgaatgagaaagaatagaactgtccccacaaggctaatcaccgttagggcaataaacactgttcttcggtcactctctgatatctgagttttcccttgccaggcaaaatatatgtagagatttccaaagaacaagctagactgcagaagtgcccagaaaatcccactgtttctcccaatgctgtgctcatccgaattgattgtcaggcagtttccttgtgctgtccaaagcacagcagcagcaattccaatgaaaacagaggctgtgtagaaggaccacgggaaaggctggatgaaaacggcaatgtacatgctgtaaaataaaccactggcaaacatagagagttgaggtcctacaatggcaaccactgacggtgtaatcaaatttgaagcagagaacactccatagataatagccatgctggtatatccactgccgtgaaaatctgtcctatttaagctcctgatgacagtttgcgccacatttccacaagtttgaaaggcagtgaacataaacataaaggcaactcctaaaataatgatgttgaaaagctttttagattccggggacattttggctcagctctgccggaggcagcagcccagggcagtcagctctcctcggggcgaagccactgacaatccggcagttaggatactcctaagaagcgatccgagtacggaagagcacaacccccggagaagcgccaagaatttatccgctccaggttgaggggcccacgaaggggattaaagggccaagtgccagccgcagcagccggcgcggccccgccctcccagcctgactcactgcggccaggcgaccgggtcacctgaccgcagccgcggcgccggccgctcggcccgctgggaaacgtagtcccgggtggcctggcacgcgcaagcgctccgcggggagtccccaccgccaggacgcagagccgacggagctctcgggctctggcgaaagggggttgggaagcggactccggcgaagagcagtcaggaacggctggacggggccgagagacgacgcagcggagtctgagggggccggggtcacagggagaggcaaatgagggcagaagcactcttcagacggagacggggctgacggctgagcaaaaaaggg

SEQ ID NO: 17638 - RNA, 2456 nt, Homo sapiens
  source 1..2456: mol_type = other RNA
tcaggccaggcacagtggctcatgtctgtaatcccagcactttgggaggctgaggtgggtggaccgcttgagtctaggtgttcaggaccagcctggcagcatggtgaaaccctgtctttacaaaaaatacaaaaaaattacctgagtgtggtgggatgcgcttgtggtcccaagctactcggaaggctgaggtgggaggaccgcttgaggccaggagttggaggttgcagtgagctatgtttgtgccactgcactccagcctgggtgacagagcaagacccttcactgcagcctgcagagacatggactgcagcctggagagacgctcaggactcagctcagccatgcgcagattcccgacccacagaaactgaacaaacttgaagatggcaaatgctggggcgctgtcttcagaatacagaaagcccaagatactaagcagctgggtattaaagcagctgtctccaaggcccaacagaaaactgcagagaatggcaacttctttgctggatttgatgtaagcactgctgtcagttcctttaacaggagcaatcggggcatctccaggcatgttgagaaatattagataaaaagctatgaagtgcaccaggatgcccaacagcacaactggatttctaccaaaacgattgttcttgctcagcaggccgaagaggcttccacctaaaatttctccaatgccgatgaaaatgccagaaagtccaataaggcttttctcttctgctccaaatttatttgtagcaccaatacaggttccatatacaccagagaagaaagttaattccagacctgtataagcagttgtaatactaagaaggagcatctccttggtgacacataacttaaaagactttttaaaagcatctactgcctttgtcagattgttctgggcagactcgttgacttccatgtcctggtcatcagaagactcatcttctcctaggacattttcagaatctggtttccgaatgagaaagaatagaactgtccccacaaggctaatcaccgttagggcaataaacactgttcttcggtcactctctgatatctgagttttcccttgccaggcaaaatatatgtagagatttccaaagaacaagctagactgcagaagtgcccagaaaatcccactgtttctcccaatgctgtgctcatccgaattgattgtcaggcagtttccttgtgctgtccaaagcacagcagcagcaattccaatgaaaacagaggctgtgtagaaggaccacgggaaaggctggatgaaaacggcaatgtacatgctgtaaaataaaccactggcaaacatagagagttgaggtcctacaatggcaaccactgacggtgtaatcaaatttgaagcagagaacactccatagataatagccatgctggtatatccactgccgtgaaaatctgtcctatttaagctcctgatgacagtttgcgccacatttccacaagtttgaaaggcagtgaacataaacataaaggcaactcctaaaataatgatgttgaaaagctttttagattccggggacattttggctcagctctgccggaggcagcagcccagggcagtcagctctcctcggggcgaagccactgacaatcctcctcttcctcctgcccaatcgcgatcgtccggcctcccaggcggaaaaagcgtttcgcgggctttccaactgcccgctaattccgctccccctccctccagccgtgactccgcgctttttggcccgcccgccgggctgtgcgcaggcgcttcgggtaggggcggggcgcgcggcagggtcgttacgaagcggggcgcggtgggccaatcagaaggtttcatttccgggtggcgcgggcgccattttgtgaggagcgatataaacgggcgcagaggccggctgcccgcccagttgttactcaggtgcgctagcctgcggagcccgtccgtgctgttctgcggcaaggcctttcccagtgtccccacgcggaaggcaactgcctgagaggcgcggcgtcgcaccgcccagagctgaggaagccggcgccagttcgcggggctccgggccgccactcagagctatgagctacggccgcccccctcccgatgtggagggtatgacctccctcaaggtggacaacctgacctaccgcacctcgcccgacacgctgaggcgcgtcttcgagaagtacgggcgcgtcggcgacgtgtacatcccgcgggaccgctacaccaaggagtcccgcggcttcgccttcgttcgctttcacgacaagcgcgacgctgaggacgctatggatgccatggacggggccgtgctggacggccgcgagctgcgggtgcaaatggcgcgctacggccgccccccggactcacaccacagccgccggggaccgccaccccgcaggtacgggggcggtggctacggacgccggagccgcaggtaaac

SEQ ID NO: 17639 - RNA, 1974 nt, Homo sapiens
  source 1..1974: mol_type = other RNA
tcaggccaggcacagtggctcatgtctgtaatcccagcactttgggaggctgaggtgggtggaccgcttgagtctaggtgttcaggaccagcctggcagcatggtgaaaccctgtctttacaaaaaatacaaaaaaattacctgagtgtggtgggatgcgcttgtggtcccaagctactcggaaggctgaggtgggaggaccgcttgaggccaggagttggaggttgcagtgagctatgtttgtgccactgcactccagcctgggtgacagagcaagacccttcactgcagcctgcagagacatggactgcagcctggagagacgctcaggactcagctcagccatgcgcagattcccgacccacagaaactgaacaaacttgaagatggcaaatgctggggcgctgtcttcagaatacagaaagcccaagatactaagcagctgggtattaaagcagctgtctccaaggcccaacagaaaactgcagagaatggcaacttctttgctggatttgatgtaagcactgctgtcagttcctttaacaggagcaatcggggcatctccaggcatgttgagaaatattagataaaaagctatgaagtgcaccaggatgcccaacagcacaactggatttctaccaaaacgattgttcttgctcagcaggccgaagaggcttccacctaaaatttctccaatgccgatgaaaatgccagaaagtccaataaggcttttctcttctgctccaaatttatttgtagcaccaatacaggttccatatacaccagagaagaaagttaattccagacctgtataagcagttgtaatactaagaaggagcatctccttggtgacacataacttaaaagactttttaaaagcatctactgcctttgtcagattgttctgggcagactcgttgacttccatgtcctggtcatcagaagactcatcttctcctaggacattttcagaatctggtttccgaatgagaaagaatagaactgtccccacaaggctaatcaccgttagggcaataaacactgttcttcggtcactctctgatatctgagttttcccttgccaggcaaaatatatgtagagatttccaaagaacaagctagactgcagaagtgcccagaaaatcccactgtttctcccaatgctgtgctcatccgaattgattgtcaggcagtttccttgtgctgtccaaagcacagcagcagcaattccaatgaaaacagaggctgtgtagaaggaccacgggaaaggctggatgaaaacggcaatgtacatgctgtaaaataaaccactggcaaacatagagagttgaggtcctacaatggcaaccactgacggtgtaatcaaatttgaagcagagaacactccatagataatagccatgctggtatatccactgccgtgaaaatctgtcctatttaagctcctgatgacagtttgcgccacatttccacaagtttgaaaggcagtgaacataaacataaaggcaactcctaaaataatgatgttgaaaagctttttagattccggggacattttggctcagctctgccggaggcagcagcccagggcagtcagctctcctcggggcgaagccactgacaatcctgaccgcagccgcggcgccggccgctcggcccgctgggaaacgtagtcccgggtggcctggcacgcgcaagcgctccgcggggagtccccaccgccaggacgcagagccgacggagctctcgggctctggcgaaagggggttgggaagcggactccggcgaagagcagtcaggaacggctggacggggccgagagacgacgcagcggagtctgagggggccggggtcacagggagaggcaaatgagggcagaagcactcttcagacggagacggggctgacggctgagcaaaaaaggggcgtgaacttggagtattggcatgaaaaaaaggtgggggcccagatggg

SEQ ID NO: 17640 - RNA, 1789 nt, Homo sapiens
  source 1..1789: mol_type = other RNA
tcaggccaggcacagtggctcatgtctgtaatcccagcactttgggaggctgaggtgggtggaccgcttgagtctaggtgttcaggaccagcctggcagcatggtgaaaccctgtctttacaaaaaatacaaaaaaattacctgagtgtggtgggatgcgcttgtggtcccaagctactcggaaggctgaggtgggaggaccgcttgaggccaggagttggaggttgcagtgagctatgtttgtgccactgcactccagcctgggtgacagagcaagacccttcactgcagcctgcagagacatggactgcagcctggagagacgctcaggactcagctcagccatgcgcagattcccgacccacagaaactgaacaaacttgaagatggcaaatgctggggcgctgtcttcagaatacagaaagcccaagatactaagcagctgggtattaaagcagctgtctccaaggcccaacagaaaactgcagagaatggcaacttctttgctggatttgatgtaagcactgctgtcagttcctttaacaggagcaatcggggcatctccaggcatgttgagaaatattagataaaaagctatgaagtgcaccaggatgcccaacagcacaactggatttctaccaaaacgattgttcttgctcagcaggccgaagaggcttccacctaaaatttctccaatgccgatgaaaatgccagaaagtccaataaggcttttctcttctgctccaaatttatttgtagcaccaatacaggttccatatacaccagagaagaaagttaattccagacctgtataagcagttgtaatactaagaaggagcatctccttggtgacacataacttaaaagactttttaaaagcatctactgcctttgtcagattgttctgggcagactcgttgacttccatgtcctggtcatcagaagactcatcttctcctaggacattttcagaatctggtttccgaatgagaaagaatagaactgtccccacaaggctaatcaccgttagggcaataaacactgttcttcggtcactctctgatatctgagttttcccttgccaggcaaaatatatgtagagatttccaaagaacaagctagactgcagaagtgcccagaaaatcccactgtttctcccaatgctgtgctcatccgaattgattgtcaggcagtttccttgtgctgtccaaagcacagcagcagcaattccaatgaaaacagaggctgtgtagaaggaccacgggaaaggctggatgaaaacggcaatgtacatgctgtaaaataaaccactggcaaacatagagagttgaggtcctacaatggcaaccactgacggtgtaatcaaatttgaagcagagaacactccatagataatagccatgctggtatatccactgccgtgaaaatctgtcctatttaagctcctgatgacagtttgcgccacatttccacaagtttgaaaggcagtgaacataaacataaaggcaactcctaaaataatgatgttgaaaagctttttagattccggggacattttggctcagctctgccggaggcagcagcccagggcagtcagctctcctcggggcgaagccactgacaatcctggagaaagaaatgagatggtgagtggagaaggcagatgcaggagccaggcagccaagctgtcaacttccagttcctggatcggaaccccaggtttagggcgaagttctccccaccggcagttaggatactcctaagaagcgatccgagtacggaagagcac

SEQ ID NO: 17641 - RNA, 1916 nt, Homo sapiens
  source 1..1916: mol_type = other RNA
tcaggccaggcacagtggctcatgtctgtaatcccagcactttgggaggctgaggtgggtggaccgcttgagtctaggtgttcaggaccagcctggcagcatggtgaaaccctgtctttacaaaaaatacaaaaaaattacctgagtgtggtgggatgcgcttgtggtcccaagctactcggaaggctgaggtgggaggaccgcttgaggccaggagttggaggttgcagtgagctatgtttgtgccactgcactccagcctgggtgacagagcaagacccttcactgcagcctgcagagacatggactgcagcctggagagacgctcaggactcagctcagccatgcgcagattcccgacccacagaaactgaacaaacttgaagatggcaaatgctggggcgctgtcttcagaatacagaaagcccaagatactaagcagctgggtattaaagcagctgtctccaaggcccaacagaaaactgcagagaatggcaacttctttgctggatttgatgtaagcactgctgtcagttcctttaacaggagcaatcggggcatctccaggcatgttgagaaatattagataaaaagctatgaagtgcaccaggatgcccaacagcacaactggatttctaccaaaacgattgttcttgctcagcaggccgaagaggcttccacctaaaatttctccaatgccgatgaaaatgccagaaagtccaataaggcttttctcttctgctccaaatttatttgtagcaccaatacaggttccatatacaccagagaagaaagttaattccagacctgtataagcagttgtaatactaagaaggagcatctccttggtgacacataacttaaaagactttttaaaagcatctactgcctttgtcagattgttctgggcagactcgttgacttccatgtcctggtcatcagaagactcatcttctcctaggacattttcagaatctggtttccgaatgagaaagaatagaactgtccccacaaggctaatcaccgttagggcaataaacactgttcttcggtcactctctgatatctgagttttcccttgccaggcaaaatatatgtagagatttccaaagaacaagctagactgcagaagtgcccagaaaatcccactgtttctcccaatgctgtgctcatccgaattgattgtcaggcagtttccttgtgctgtccaaagcacagcagcagcaattccaatgaaaacagaggctgtgtagaaggaccacgggaaaggctggatgaaaacggcaatgtacatgctgtaaaataaaccactggcaaacatagagagttgaggtcctacaatggcaaccactgacggtgtaatcaaatttgaagcagagaacactccatagataatagccatgctggtatatccactgccgtgaaaatctgtcctatttaagctcctgatgacagtttgcgccacatttccacaagtttgaaaggcagtgaacataaacataaaggcaactcctaaaataatgatgttgaaaagctttttagattccggggacattttggctcagctctgccggaggcagcagcccagggcagtcagctctcctcggggcgaagccactgacaatcctggcacgcgcaagcgctccgcggggagtccccaccgccaggacgcagagccgacggagctctcgggctctggcgaaagggggttgggaagcggactccggcgaagagcagtcaggaacggctggacggggccgagagacgacgcagcggagtctgagggggccggggtcacagggagaggcaaatgagggcagaagcactcttcagacggagacggggctgacggctgagcaaaaaaggggcgtgaacttggagtattggcatgaaaaaaaggtgggggcccagatggg

SEQ ID NO: 17642 - RNA, 1996 nt, Homo sapiens
  source 1..1996: mol_type = other RNA
tcaggccaggcacagtggctcatgtctgtaatcccagcactttgggaggctgaggtgggtggaccgcttgagtctaggtgttcaggaccagcctggcagcatggtgaaaccctgtctttacaaaaaatacaaaaaaattacctgagtgtggtgggatgcgcttgtggtcccaagctactcggaaggctgaggtgggaggaccgcttgaggccaggagttggaggttgcagtgagctatgtttgtgccactgcactccagcctgggtgacagagcaagacccttcactgcagcctgcagagacatggactgcagcctggagagacgctcaggactcagctcagccatgcgcagattcccgacccacagaaactgaacaaacttgaagatggcaaatgctggggcgctgtcttcagaatacagaaagcccaagatactaagcagctgggtattaaagcagctgtctccaaggcccaacagaaaactgcagagaatggcaacttctttgctggatttgatgtaagcactgctgtcagttcctttaacaggagcaatcggggcatctccaggcatgttgagaaatattagataaaaagctatgaagtgcaccaggatgcccaacagcacaactggatttctaccaaaacgattgttcttgctcagcaggccgaagaggcttccacctaaaatttctccaatgccgatgaaaatgccagaaagtccaataaggcttttctcttctgctccaaatttatttgtagcaccaatacaggttccatatacaccagagaagaaagttaattccagacctgtataagcagttgtaatactaagaaggagcatctccttggtgacacataacttaaaagactttttaaaagcatctactgcctttgtcagattgttctgggcagactcgttgacttccatgtcctggtcatcagaagactcatcttctcctaggacattttcagaatctggtttccgaatgagaaagaatagaactgtccccacaaggctaatcaccgttagggcaataaacactgttcttcggtcactctctgatatctgagttttcccttgccaggcaaaatatatgtagagatttccaaagaacaagctagactgcagaagtgcccagaaaatcccactgtttctcccaatgctgtgctcatccgaattgattgtcaggcagtttccttgtgctgtccaaagcacagcagcagcaattccaatgaaaacagaggctgtgtagaaggaccacgggaaaggctggatgaaaacggcaatgtacatgctgtaaaataaaccactggcaaacatagagagttgaggtcctacaatggcaaccactgacggtgtaatcaaatttgaagcagagaacactccatagataatagccatgctggtatatccactgccgtgaaaatctgtcctatttaagctcctgatgacagtttgcgccacatttccacaagtttgaaaggcagtgaacataaacataaaggcaactcctaaaataatgatgttgaaaagctttttagattccggggacattttggctcagctctgccggaggcagcagcccagggcagtcagctctcctcggggcgaagccactgacaatctgcggccaggcgaccgggtcacctgaccgcagccgcggcgccggccgctcggcccgctgggaaacgtagtcccgggtggcctggcacgcgcaagcgctccgcggggagtccccaccgccaggacgcagagccgacggagctctcgggctctggcgaaagggggttgggaagcggactccggcgaagagcagtcaggaacggctggacggggccgagagacgacgcagcggagtctgagggggccggggtcacagggagaggcaaatgagggcagaagcactcttcagacggagacggggctgacggctgagcaaaaaaggggcgtgaacttggagtattggcatgaaaaaaaggtgggggcccagatggg

SEQ ID NO: 17643 - RNA, 1590 nt, Homo sapiens
  source 1..1590: mol_type = other RNA
tcaggccaggcacagtggctcatgtctgtaattccagcactttgggaggccgaggcatacttttctgtattaaaaatacaaaagtatttgtctctactaaaaatatccaccccccccgcccaaaaaagaaaaattagttgagcatggtggtgtgtacctgtaatcccagctactcgggaggctgaggcaggagaatcacttgaaggatgggaggcaggggttgcagtgagcccagatcacgccactgcactccagcctggtgacagagcaaaacttcatctcaagaaaaaaaaaaaaaagagtgagcatattgaactaccctcagctcatagtaaggcaaataggtcaacagaataataattcatgctattgcattggaaaagcaattaaaagaaatttaaaaatgtgtaagcagaaattcagttgcatgtaagaaaatccaattccccgtgagaaagagaaagagctggagtcctttaaaaattaactgcctgtttttctgtggctagtgagccttatctctcctcctttcccaggcattgtaaataccctgtttctctagctgtgcagctgcaaggtaactagacagataaactcaagtcgtaaaacatgattttccttgaaaagtaagaaatgatgtaatgcatgtctcagttaattgaataactgtctttcttgcttctgtaatatgcttccccctgcacagattccccccaacccccgcggccccacaaaatgcttaaaaggtaacttaactctgttcagggttcagtcctttggatgttaatctgactgggctggtgcacctaaataataaatatctccctgaactccatcagtctctctgattccttaaaaatcccgctacattttgtgtaatgaactggcaacaagagaaagttggtcgaagaaaggcagaggaactgtgtcttgtaagaattagaatcgaggggctccataatcatctggcatccgttcaatgttgtatctatggttagaaatgtacatgataggaactccaggaatcttacggattcttcttttcaggtcccggtcaactgtggccacaatgtaacacttatgctgagttactctctgtactaagcagtcatctgcataggttcctttgtgtgtacatggtaatcgttcaaatcttggatccttggcaatccttagagccactcgatacttctgccccaatttctcaatttcagccattacacaatcggttatacatgggatacacttggcatacagacagtccatcattgactgcactaagtccagtttggcttttatggaaaagttgataaagttggtatcaacgaggatgtggtaaggtgggcccagctgtgtattatattggaaaaataagcaggaagggtgttggggaacttctctttcctttaatgcgctgggatccttcttttctttctttttaggttttaatctatccttttctttaagcctctgatctctgagactaagcattcgcttcatggtcgcatacttccttgttttcttttgcttccccatggtcacgccaaactcctggttcttccgtaatcaccaacggcgcaatacttctac

SEQ ID NO: 17644 - RNA, 1649 nt, Homo sapiens
  source 1..1649: mol_type = other RNA
tcaggccaggcacagtggctcatgtctgtaattccagcactttgggaggccgaggcatacttttctgtattaaaaatacaaaagtatttgtctctactaaaaatatccaccccccccgcccaaaaaagaaaaattagttgagcatggtggtgtgtacctgtaatcccagctactcgggaggctgaggcaggagaatcacttgaaggatgggaggcaggggttgcagtgagcccagatcacgccactgcactccagcctggtgacagagcaaaacttcatctcaagaaaaaaaaaaaaaagagtgagcatattgaactaccctcagctcatagtaaggcaaataggtcaacagaataataattcatgctattgcattggaaaagcaattaaaagaaatttaaaaatgtgtaagcagaaattcagttgcatgtaagaaaatccaattccccgtgagaaagagaaagagctggagtcctttaaaaattaactgcctgtttttctgtggctagtgagccttatctctcctcctttcccaggcattgtaaataccctgtttctctagctgtgcagctgcaaggtaactagacagataaactcaagtcgtaaaacatgattttccttgaaaagtaagaaatgatgtaatgcatgtctcagttaattgaataactgtctttcttgcttctgtaatatgcttccccctgcacagattccccccaacccccgcggccccacaaaatgcttaaaaggtaacttaactctgttcagggttcagtcctttggatgttaatctgactgggctggtgcacctaaataataaatatctccctgaactccatcagtctctctgattccttaaaaatcccgctacattttgtgtaatgaactggcaacaagagaaagttggtcgaagaaaggcagaggaactgtgtcttgtaagaattagaatcgaggggctccataatcatctggcatccgttcaatgttgtatctatggttagaaatgtacatgataggaactccaggaatcttacggattcttcttttcaggtcccggtcaactgtggccacaatgtaacacttatgctgagttactctctgtactaagcagtcatctgcataggttcctttgtgtgtacatggtaatcgttcaaatcttggatccttggcaatccttagagccactcgatacttctgccccaatttctcaatttcagccattacacaatcggttatacatgggatacacttggcatacagacagtccatcattgactgcactaagtccagtttggcttttatggaaaagttgataaagttggtatcaacgaggatgtggtaaggtgggcccagctgtgtattatattggaaaaataagcaggaagggtgttggggaacttctctttcctttaatgcgctgggatccttcttttctttctttttaggttttaatctatccttttctttaagcctctgatctctgagactaagcattcgcttcatggtcgcatacttccttgttttcttttgcttcccctccttctccacccaaaaagtggcctgataacgtcccttcttggaccgtcttctctcaccatggtcacgccaaactcctggttcttccgtaatcaccaacggcgcaatacttctac

SEQ ID NO: 17645 - RNA, 81 nt, Homo sapiens
  source 1..81: mol_type = other RNA
tcaggccaggcacagtggctcattcttctaatctcagcaatttgggaggctgaggcaagtggatagcttgagctcaggagc

SEQ ID NO: 17646 - RNA, 4551 nt, Homo sapiens
  source 1..4551: mol_type = other RNA
tcaggtgtggaaactgaggcagaaataattttagtggctttcataaagtcctaccatatgctatctgtgacagtcttccatgtagaaggaattgtcacctcatacacatttagcactcataggtcaccatattaaaaagtttccatggagactcccccaaactgttaaattttgcagctcattagtgaggaaagatgcttcaattttttgctactgcatgtacatctgacagaaaaaaaatcttttctgcaaccactaaagcaggagtgaagagaaaatagagagtgctcaagatcctcactagcacaagcagggcaatttttctttcctcattattaatacatcgcattaccttgtgaagcaagtgtcccaacataggtctagttgcttaatgtctcagacaataacctatcatacaagcaaggaggcttagaatccagatctagtagtaaggcttcttagaatcctattaatggggttccaatttgcaatatattcaatgtattcaataacataaaggcttcaatattcaataggaaggggcagagttgacagtcacagcctcttaaaaccatgtgtgtctctgagttctttttttcctacgtacggaataaaaataagaaacacagagtgccagatctcaatgagtttcaataatcattttgaaaggagaaagtcaggcatctatagtgaaatttgttcctgtaaagacaacttattttttaaagaaagagagagagagtgacatgaggcactaaagaaaatgttactatcagagcatctttaagaatcatatcaaatttgaaataactatatagtaagaattacaatgattgctaaattatagtaaagaagtggatatgggaaaatagaacataaattccatttgctgttctgtaatagagtatggttaccaaatacccgctttatgatgccaaattatcattttgaaaaagccattgctgaggactcctttagtgcctaatgttttttgttttttttttcatctcttttttgttaatggtctaaattttaactaagtcactaatgcaataatagaatgacattcttaattattaatttttagaaaataacaaatactagcatattctatatactgaatgcccctaaagttgttaggtattctgaatatgtttaatagctagatagataaatagatgtaatgctatggttagcatgattcagtagaataatgtgaataaaacaaaagtgtccttgcaacatgcatttctcacactctttacaggagataataaaaaccactaacaatctattcaggagaaagtaaagtaagtattgcggtattcgcaaacagagatataacaggctgattttggctccctgtgatggaatgtgaatgtctttaagaggtgtaaaataatacaagcagaaatgatagattgagaatttctgcttggagcaatgcatggaacatattatccaaatcaccctctgtgaaagtatatgtggttcgctgtgtaaaagcaaaaggagaaaatcaatatatagttagagaatatagtgttaatagttcagttgtttctttttttcaggcttactttttcaaatatgtttttacatgataaattgtacttaagtctatattaatgttcttgagattttaacattgtgctttttctcaagtacaaaattagtgtaatgcaatatatcatggtttcctaggtaattcctgactcagatatagtgggagcacttagtaaatttcaaatttcaggctgcaattccaggactgctgagtagaattttcaaaggtaatcacactatattgctcaggaaattctgatgcctaccaaatatacgtttccttttgctactttgacaaactgccacaaatgtagtagcttaaacaacacaaatttatctcctacagatctggaagttagagtctgaaaatacgtttcactgagctaatgtcaaggcatcagtagggctgtttctatctggaagttctagggagaattcatttcctcatcttctgcagcttcgaaaggctgccttgcctgatttcctcagattttaaccccttcctctgtctttgaatctagtaaggtagcatcttcaaatctctcactacttctgctttcgtagccactttatgtgtgtctgtgtgtttcattctgaacttttgccttcctcttttaaggaacattgttcattgtaatttcattgagttcacttagaataatatttctgtcttaagatcattaacttaattacatctgcaaagtctctttgttacataaggtaacatattccaggtttgggaggttaggactaggccatccttaagggaccattgttctgtttgccacaccaaatttgggtagaacttgatgatcctactaagcaattagattctacaatcctatatatctaccaacatttttgttgctgcatttaactatttatttatttattcattcatcattaaataagtacttgtttcacagctactgggtgtaaagcacagagccaatccatggagacatgaaaataatttaaaagtaaaatccctacccttatgcaattctatctttcaatataattcctaagccaaattgagatatgtgggtattacctaattatgtgcaaaatatgatctatttacaaataaaaaagacatacttatgtagtagacagagaatgtgatatgttgtttccattgaaatttccatgattattctagaaatagattgtaaaatagcataaaaagagacatccatgggaatacatcatagaattggtaagttaaaaaaaaaaagaaaaaagaaagtctgcaagactacagcctagggagatatactgagcaattgacatactgttagggtgtcaataaaatcaaacgttgccagttagaagaataatgagctcttttctctctgtacccaaaggagattaattcaagaatatatattttctgcatgttgctcacctctcccgataaaatgaaagtgctaaaaatggtcatctgggggtggttttgactttactttttattctctctactaagaagaaacaagttacataactcctattacacacagaattccatgacagacattttgttatttggattcctggccaagtgatttaatgaatgttcagttaaagaatatgtgttttaaaattaccatatcagaactgacagaagagttcctctactgttaaaaatgtcccaagttaggcaaaaatctgttaatgccacacacacacaaaattgaaattagcaagtcactgaaagaaaacaggaactcccactctccatagtcaggcttttctgaaattcagacccagaaacccttatcttgccttgggctcactctatctgcttctctaaatttctgttttccctgatgcttccatgcatgtttaccatagctactgtcgactcttcttctcctgggatagcagcagagatgcttcaggtacaattttagccctgtactacacgagcaattcttttcacttctgccgtttcatcttcaggtaccttgtgctttgaaggtgctccctaggtatttagatatacttttgagtttgcttcatgctttgaactttcctgagctcttctgtttcttcaaattcatctgtcctgtttcccactttctttacatttgaaagaagaaagtcaggggaagtgatttgagttttatgttaatatgtgctcctggtttcatatgattatgctctcagaaaacatgtttttattttaacaggagccatcaataccaaaggcctgtgctcctcaaactatgtaactcaaacatctgttgaatagtatattcagtaaatcaaaagctaaacatcatgcattttgtctgaagcatgcattttaattcattctaaataaagcattgcttttgtattattgaatataatatacaatttatattagatgcttttaagccaagtctcccacttcaagtaaattttctccttgtgatatgttattttaggttcataaagctctaaatcttctttgtacagaaccccacagaaaacatatttaactcatttgctattctggatatttcagtataaaagtatgagaataactgcgttaaaagacgggaacttagctttgttgaaagatcctcatgatccatctgaatcaccagcgaggttcagcctttttttttcctttctctgaagtcctggttagcatgcttataacagttctagagtgattgttttcctcttttctaggaatcttcttgtcccaacttccagaaccttgccccaggactcagttccaggacttcctgggcacctacttgcgaaggattgatacacatctgcaagatcctatgatgtccactgaggagcaacagctcaaataagccatgatccctaagtcatattgagaggtgacggcgtgctggcagcactcacaggcctcgctcgctctccgcgcctccttggcctaggcgcccactcttgccgcgcttcagcagcccttcagcccgccgctgcactgcgggagcccttttctgggctggccgaggccgg

SEQ ID NO: 17647 - RNA, 4660 nt, Homo sapiens
  source 1..4660: mol_type = other RNA
tcaggtgtggaaactgaggcagaaataattttagtggctttcataaagtcctaccatatgctatctgtgacagtcttccatgtagaaggaattgtcacctcatacacatttagcactcataggtcaccatattaaaaagtttccatggagactcccccaaactgttaaattttgcagctcattagtgaggaaagatgcttcaattttttgctactgcatgtacatctgacagaaaaaaaatcttttctgcaaccactaaagcaggagtgaagagaaaatagagagtgctcaagatcctcactagcacaagcagggcaatttttctttcctcattattaatacatcgcattaccttgtgaagcaagtgtcccaacataggtctagttgcttaatgtctcagacaataacctatcatacaagcaaggaggcttagaatccagatctagtagtaaggcttcttagaatcctattaatggggttccaatttgcaatatattcaatgtattcaataacataaaggcttcaatattcaataggaaggggcagagttgacagtcacagcctcttaaaaccatgtgtgtctctgagttctttttttcctacgtacggaataaaaataagaaacacagagtgccagatctcaatgagtttcaataatcattttgaaaggagaaagtcaggcatctatagtgaaatttgttcctgtaaagacaacttattttttaaagaaagagagagagagtgacatgaggcactaaagaaaatgttactatcagagcatctttaagaatcatatcaaatttgaaataactatatagtaagaattacaatgattgctaaattatagtaaagaagtggatatgggaaaatagaacataaattccatttgctgttctgtaatagagtatggttaccaaatacccgctttatgatgccaaattatcattttgaaaaagccattgctgaggactcctttagtgcctaatgttttttgttttttttttcatctcttttttgttaatggtctaaattttaactaagtcactaatgcaataatagaatgacattcttaattattaatttttagaaaataacaaatactagcatattctatatactgaatgcccctaaagttgttaggtattctgaatatgtttaatagctagatagataaatagatgtaatgctatggttagcatgattcagtagaataatgtgaataaaacaaaagtgtccttgcaacatgcatttctcacactctttacaggagataataaaaaccactaacaatctattcaggagaaagtaaagtaagtattgcggtattcgcaaacagagatataacaggctgattttggctccctgtgatggaatgtgaatgtctttaagaggtgtaaaataatacaagcagaaatgatagattgagaatttctgcttggagcaatgcatggaacatattatccaaatcaccctctgtgaaagtatatgtggttcgctgtgtaaaagcaaaaggagaaaatcaatatatagttagagaatatagtgttaatagttcagttgtttctttttttcaggcttactttttcaaatatgtttttacatgataaattgtacttaagtctatattaatgttcttgagattttaacattgtgctttttctcaagtacaaaattagtgtaatgcaatatatcatggtttcctaggtaattcctgactcagatatagtgggagcacttagtaaatttcaaatttcaggctgcaattccaggactgctgagtagaattttcaaaggtaatcacactatattgctcaggaaattctgatgcctaccaaatatacgtttccttttgctactttgacaaactgccacaaatgtagtagcttaaacaacacaaatttatctcctacagatctggaagttagagtctgaaaatacgtttcactgagctaatgtcaaggcatcagtagggctgtttctatctggaagttctagggagaattcatttcctcatcttctgcagcttcgaaaggctgccttgcctgatttcctcagattttaaccccttcctctgtctttgaatctagtaaggtagcatcttcaaatctctcactacttctgctttcgtagccactttatgtgtgtctgtgtgtttcattctgaacttttgccttcctcttttaaggaacattgttcattgtaatttcattgagttcacttagaataatatttctgtcttaagatcattaacttaattacatctgcaaagtctctttgttacataaggtaacatattccaggtttgggaggttaggactaggccatccttaagggaccattgttctgtttgccacaccaaatttgggtagaacttgatgatcctactaagcaattagattctacaatcctatatatctaccaacatttttgttgctgcatttaactatttatttatttattcattcatcattaaataagtacttgtttcacagctactgggtgtaaagcacagagccaatccatggagacatgaaaataatttaaaagtaaaatccctacccttatgcaattctatctttcaatataattcctaagccaaattgagatatgtgggtattacctaattatgtgcaaaatatgatctatttacaaataaaaaagacatacttatgtagtagacagagaatgtgatatgttgtttccattgaaatttccatgattattctagaaatagattgtaaaatagcataaaaagagacatccatgggaatacatcatagaattggtaagttaaaaaaaaaaagaaaaaagaaagtctgcaagactacagcctagggagatatactgagcaattgacatactgttagggtgtcaataaaatcaaacgttgccagttagaagaataatgagctcttttctctctgtacccaaaggagattaattcaagaatatatattttctgcatgttgctcacctctcccgataaaatgaaagtgctaaaaatggtcatctgggggtggttttgactttactttttattctctctactaagaagaaacaagttacataactcctattacacacagaattccatgacagacattttgttatttggattcctggccaagtgatttaatgaatgttcagttaaagaatatgtgttttaaaattaccatatcagaactgacagaagagttcctctactgttaaaaatgtcccaagttaggcaaaaatctgttaatgccacacacacacaaaattgaaattagcaagtcactgaaagaaaacaggaactcccactctccatagtcaggcttttctgaaattcagacccagaaacccttatcttgccttgggctcactctatctgcttctctaaatttctgttttccctgatgcttccatgcatgtttaccatagctactgtcgactcttcttctcctgggatagcagcagagatgcttcaggtacaattttagccctgtactacacgagcaattcttttcacttctgccgtttcatcttcaggtaccttgtgctttgaaggtgctccctaggtatttagatatacttttgagtttgcttcatgctttgaactttcctgagctcttctgtttcttcaaattcatctgtcctgtttcccactttctttacatttgaaagaagaaagtcaggggaagtgatttgagttttatgttaatatgtgctcctggtttcatatgattatgctctcagaaaacatgtttttattttaacaggagccatcaataccaaaggcctgtgctcctcaaactatgtaactcaaacatctgttgaatagtatattcagtaaatcaaaagctaaacatcatgcattttgtctgaagcatgcattttaattcattctaaataaagcattgcttttgtattattgaatataatatacaatttatattagatgcttttaagccaagtctcccacttcaagtaaattttctccttgtgatatgttattttaggttcataaagctctaaatcttctttgtacagaaccccacagaaaacatatttaactcatttgctattctggatatttcagtataaaagtatgagaataactgcgttaaaagacgggaacttagctttgttgaaagatcctcatgatccatctgaatcaccagcgaggttcagcctttttttttcctttctctgaagtcctggttagcatgcttataacagttctagagtgattgttttcctcttttctaggaatcttcttgtcccaacttccagaaccttgccccaggactcagttccaggacttcctgggcacctttttcaatcagtctattcgtcctccaaataggtcagttcagttaaacagctctgtctcttttcaggaggagcattgcagatgggacccatcaaggttaggtctctttgcagtgtaagaataaggaaatttaaaagagacttttctatgtaaacaaacaaaaactcgcaaagcctaacgtctggagtattctccaagctactttctgagtctgaatagcagctcactgagaagatttctgaacctgagctaaagtattttcagctggagcagagcaggcagtggcaaactgacagaatttcctggtttgcagtttcaatgttataaagcttgtccatctgcaagcca

SEQ ID NO: 17648 - RNA, 4391 nt, Homo sapiens
  source 1..4391: mol_type = other RNA
tcaggtgtggaaactgaggcagaaataattttagtggctttcataaagtcctaccatatgctatctgtgacagtcttccatgtagaaggaattgtcacctcatacacatttagcactcataggtcaccatattaaaaagtttccatggagactcccccaaactgttaaattttgcagctcattagtgaggaaagatgcttcaattttttgctactgcatgtacatctgacagaaaaaaaatcttttctgcaaccactaaagcaggagtgaagagaaaatagagagtgctcaagatcctcactagcacaagcagggcaatttttctttcctcattattaatacatcgcattaccttgtgaagcaagtgtcccaacataggtctagttgcttaatgtctcagacaataacctatcatacaagcaaggaggcttagaatccagatctagtagtaaggcttcttagaatcctattaatggggttccaatttgcaatatattcaatgtattcaataacataaaggcttcaatattcaataggaaggggcagagttgacagtcacagcctcttaaaaccatgtgtgtctctgagttctttttttcctacgtacggaataaaaataagaaacacagagtgccagatctcaatgagtttcaataatcattttgaaaggagaaagtcaggcatctatagtgaaatttgttcctgtaaagacaacttattttttaaagaaagagagagagagtgacatgaggcactaaagaaaatgttactatcagagcatctttaagaatcatatcaaatttgaaataactatatagtaagaattacaatgattgctaaattatagtaaagaagtggatatgggaaaatagaacataaattccatttgctgttctgtaatagagtatggttaccaaatacccgctttatgatgccaaattatcattttgaaaaagccattgctgaggactcctttagtgcctaatgttttttgttttttttttcatctcttttttgttaatggtctaaattttaactaagtcactaatgcaataatagaatgacattcttaattattaatttttagaaaataacaaatactagcatattctatatactgaatgcccctaaagttgttaggtattctgaatatgtttaatagctagatagataaatagatgtaatgctatggttagcatgattcagtagaataatgtgaataaaacaaaagtgtccttgcaacatgcatttctcacactctttacaggagataataaaaaccactaacaatctattcaggagaaagtaaagtaagtattgcggtattcgcaaacagagatataacaggctgattttggctccctgtgatggaatgtgaatgtctttaagaggtgtaaaataatacaagcagaaatgatagattgagaatttctgcttggagcaatgcatggaacatattatccaaatcaccctctgtgaaagtatatgtggttcgctgtgtaaaagcaaaaggagaaaatcaatatatagttagagaatatagtgttaatagttcagttgtttctttttttcaggcttactttttcaaatatgtttttacatgataaattgtacttaagtctatattaatgttcttgagattttaacattgtgctttttctcaagtacaaaattagtgtaatgcaatatatcatggtttcctaggtaattcctgactcagatatagtgggagcacttagtaaatttcaaatttcaggctgcaattccaggactgctgagtagaattttcaaaggtaatcacactatattgctcaggaaattctgatgcctaccaaatatacgtttccttttgctactttgacaaactgccacaaatgtagtagcttaaacaacacaaatttatctcctacagatctggaagttagagtctgaaaatacgtttcactgagctaatgtcaaggcatcagtagggctgtttctatctggaagttctagggagaattcatttcctcatcttctgcagcttcgaaaggctgccttgcctgatttcctcagattttaaccccttcctctgtctttgaatctagtaaggtagcatcttcaaatctctcactacttctgctttcgtagccactttatgtgtgtctgtgtgtttcattctgaacttttgccttcctcttttaaggaacattgttcattgtaatttcattgagttcacttagaataatatttctgtcttaagatcattaacttaattacatctgcaaagtctctttgttacataaggtaacatattccaggtttgggaggttaggactaggccatccttaagggaccattgttctgtttgccacaccaaatttgggtagaacttgatgatcctactaagcaattagattctacaatcctatatatctaccaacatttttgttgctgcatttaactatttatttatttattcattcatcattaaataagtacttgtttcacagctactgggtgtaaagcacagagccaatccatggagacatgaaaataatttaaaagtaaaatccctacccttatgcaattctatctttcaatataattcctaagccaaattgagatatgtgggtattacctaattatgtgcaaaatatgatctatttacaaataaaaaagacatacttatgtagtagacagagaatgtgatatgttgtttccattgaaatttccatgattattctagaaatagattgtaaaatagcataaaaagagacatccatgggaatacatcatagaattggtaagttaaaaaaaaaaagaaaaaagaaagtctgcaagactacagcctagggagatatactgagcaattgacatactgttagggtgtcaataaaatcaaacgttgccagttagaagaataatgagctcttttctctctgtacccaaaggagattaattcaagaatatatattttctgcatgttgctcacctctcccgataaaatgaaagtgctaaaaatggtcatctgggggtggttttgactttactttttattctctctactaagaagaaacaagttacataactcctattacacacagaattccatgacagacattttgttatttggattcctggccaagtgatttaatgaatgttcagttaaagaatatgtgttttaaaattaccatatcagaactgacagaagagttcctctactgttaaaaatgtcccaagttaggcaaaaatctgttaatgccacacacacacaaaattgaaattagcaagtcactgaaagaaaacaggaactcccactctccatagtcaggcttttctgaaattcagacccagaaacccttatcttgccttgggctcactctatctgcttctctaaatttctgttttccctgatgcttccatgcatgtttaccatagctactgtcgactcttcttctcctgggatagcagcagagatgcttcaggtacaattttagccctgtactacacgagcaattcttttcacttctgccgtttcatcttcaggtaccttgtgctttgaaggtgctccctaggtatttagatatacttttgagtttgcttcatgctttgaactttcctgagctcttctgtttcttcaaattcatctgtcctgtttcccactttctttacatttgaaagaagaaagtcaggggaagtgatttgagttttatgttaatatgtgctcctggtttcatatgattatgctctcagaaaacatgtttttattttaacaggagccatcaataccaaaggcctgtgctcctcaaactatgtaactcaaacatctgttgaatagtatattcagtaaatcaaaagctaaacatcatgcattttgtctgaagcatgcattttaattcattctaaataaagcattgcttttgtattattgaatataatatacaatttatattagatgcttttaagccaagtctcccacttcaagtaaattttctccttgtgatatgttattttaggttcataaagctctaaatcttctttgtacagaaccccacagaaaacatatttaactcatttgctattctggatatttcagtataaaagtatgagaataactgcgttaaaagacgggaacttagctttgttgaaagatcctcatgatccatctgaatcaccagcgaggttcagcctttttttttcctttctctgaagtcctggttagcatgcttataacagttctagagtgattgttttcctcttttctaggaatcttcttgtcccaacttccagaaccttgccccaggactcagttccaggacttcctgggcacttctcatcctttaattcttgttaattgaagttcccaaggagacatccaataaacgaaatcatttccccacatatattct

SEQ ID NO: 17649 - RNA, 169 nt, Homo sapiens
  source 1..169: mol_type = other RNA
tcaggtgtggaaactgaggcagaatcaggagatccactgccgaaggtgcccagcaatcatgcctggtgggatcaagtctaaagctgctatttgtaccctggctggaatgcagtggcatgatctcgactcactggaacctccacctcccagattcaagcaattctcctgc

SEQ ID NO: 17650 - RNA, 403 nt, Homo sapiens
  source 1..403: mol_type = other RNA
tcaggtgtggaaactgaggcaggagaattgcttgaaccctgggaggcagaggttgcagagctgagatcgagccacactactccagcttgggcgactaagcaagactccatctacgaaggatccggggatgggcagcgccacccggcccgctccagagtcagcatgggtaagggcgcccgcctgccgcagccggggcttgggcccctcaccctgttcccgaccatagcccggccggggtgtaggtgaacgccccctccttgtctgcccctcggaagtgtacgtttcttaccgcgccctttgtggagcccggactggagttctcgcagggagggcagggtcagggaatatgaggcgggaggggattccacgggagactttatccctgtcttgtcttagaggatct

SEQ ID NO: 17651 - RNA, 1315 nt, Homo sapiens
  source 1..1315: mol_type = other RNA
tcaggtgtggaaactgaggcaggatcaggcccttcccaggagtttcctcctctgcagggggacctcggctcccctctccaggcctttctgctgaccagtcagcctccccaccccgacgaggttatgcaggatgatctcctctacgacagggtaatggggggtgttcgtctcatttacagaatacgttcacggcagcaccgcgtaaccgagcatggtggcctggccaggggactcccaagcctgactgtctcagtctactcttggacctgccaccctccacattgcctgagtcttatactcgtctccagatcaagacagcagcaaagtcacactgctgcccgaaacacaagtatgctgcacgcaactgaaaacatgctccctttccccagaagatgaatgtctgggtgatgtccaggcttatcctggatgtcctgcagcagaaatgagggaggcctgtacatgagagtcgccccagccggtacagtcacccccatcttcgcatgctggttctgtggcacagggagtccaaggcaggcctcactttcagttcaatggaatcactgctgtgtctcctggtggaagcatttctcccttgggaactgacacctttctccttcagatgttgctgtttggagctgaggcagccgtcctgtgaccatcccgttgtccctgcaggccctggctgggcatgaactgggcgccttcatcccagcgccgtgtccgggtgcgcgccgaaaaggccgaattccggtttcttgcagccagcaggggggccttggctttccatcaagattttttcccaggaggatattatctcacgtgaacaaaactcaggaggagtcagaataggctccggaagaactctgtgctctctgactttttaaaaccttacagaaacagcagcccaccccaggctcctggtgctgtgaaggctgattccgattcccaggaggtgggcagtgtctcctggcgtctgtttctgcccctgctaatagggctggatgcggagcttttctgacattaaatcaccactcttagttgaatttgaggagtgtggtagcagacttgctgaaaatatttcttccctcctaattttttgataccttttccaatttatcccagatctcatctcttccacacagcctgctccgtcctttctcaagagtgaaatgatggctctccttcatctccacctttcacagtctctctgccctgcccactaggggaagagtgcctgggcactacaagaatttagtaccaattgcccttccttccttccttccttcctctttcccttcctctttcccttcctttt

SEQ ID NO: 17652 - RNA, 1555 nt, Homo sapiens
  source 1..1555: mol_type = other RNA
tcaggtgtggaaactgaggcaggtgttccaggagcagactgagagaagaggaggagggcagagtggggaactaggcaagcacatggggacagcctccagaagcctcccagggggagagcttttactccaccatccctgacccttgtgtgatacaggaaaagaggcatttagacacaggcggaactcctggttattctattctatatggttttggggtccttcaggtaaggagcgcttcagttttcactcctgccagtgggcagtggcttattcatgtggcctcgttctagtcacatacatttctgccttcacggggctattttcaggatccagcgataaatgcacacaggatgtctgacatggtctgttgttgctctcctatggatcccatctcggcctgccagtatttccccagaagaagatactcagtttaactcttttctctgagaaggatgcactttctcaccacgatgtcttatttctccaggttccacaatcttcaacacccttttctgggagtgttggaaagaaccacacataagcatgaaacccaagtgtctgatgctagaaagaggaagtcccagcatggggcgagcaggatgcttctgtagtgggagctctgtccaggtcaggccaaaattgtatggtccagggcaaaactgagcaggagaagtatcaggtgtgccttctgcatgtcacagcccccacaagagaattacggtgaaaagcattgagctgtctgtatttcatgccaaccccaagtggctggtggaatgaaggaccaagcatgtttggggctgtaacttcttttctgaggcacaaatgcccacccaagattattagaggaacgagggcagtgggcaggaaggtgagacgctgactttagaaatagccggtgattacagatttaattcatgttattaactccctgccttttacctcctccctcctcccttggcacaactgccagatggatgtggctggaagtcagaggacattctcgtgggttcgtgggcctagggtacaaatgacctcagcgtgacagcaaacaggacagagaagaccaggctcttactcaggaatccaccagccaggagaatgacaatgttgaacaccggaaccccttggtcaccaccaagcggatgcgatcgaacagcatgtgaggctccttgggaggctggtagatcacacactgatacagtccagaatcttccacttgaaggttgaccattcggacgcgcagtaaaccatgatcatggtagtcttctagtatgatcctccccacttggactggatgggaattctttgaaggcctctctgtgcatgccagggtcttgggcatctctccgtcccttattatctgccaagctttctggctgctggcaaacttctctagcgtgtagtcacatttcacatccagggtctgcccctctttcagttcatacttttcctcagttaatttagttgcagctcggagttctgagacaaagagcatccacagcagcccccagagcctggtcttcctcatccttcctgtgcaccagctccaactgct

SEQ ID NO: 17653 - RNA, 1748 nt, Homo sapiens
  source 1..1748: mol_type = other RNA
tcaggtgtggaaactgaggcaggtgttccaggagcagactgagagaagaggaggagggcagagtggggaactaggcaagcacatggggacagcctccagaagcctcccagggggagagcttttactccaccatccctgacccttgtgtgatacaggaaaagaggcatttagacacaggcggaactcctggttattctattctatatggttttggggtccttcaggtaaggagcgcttcagttttcactcctgccagtgggcagtggcttattcatgtggcctcgttctagtcacatacatttctgccttcacggggctattttcaggatccagcgataaatgcacacaggatgtctgacatggtctgttgttgctctcctatggatcccatctcggcctgccagtatttccccagaagaagatactcagtttaactcttttctctgagaaggatgcactttctcaccacgatgtcttatttctccaggttccacaatcttcaacacccttttctgggagtgttggaaagaaccacacataagcatgaaacccaagtgtctgatgctagaaagaggaagtcccagcatggggcgagcaggatgcttctgtagtgggagctctgtccaggtcaggccaaaattgtatggtccagggcaaaactgagcaggagaagtatcaggtgtgccttctgcatgtcacagcccccacaagagaattacggtgaaaagcattgagctgtctgtatttcatgccaaccccaagtggctggtggaatgaaggaccaagcatgtttggggctgtaacttcttttctgaggcacaaatgcccacccaagattattagaggaacgagggcagtgggcaggaaggtgagacgctgactttagaaatagccggtgattacagatttaattcatgttattaactccctgccttttacctcctccctcctcccttggcacaactgccagatggatgtggctggaagtcagaggacattctcgtgggttcgtgggcctagggtacaaatgacctcagcgtgacagcaaacaggacagagaagaccaggctcttactcaggaatccaccagccaggagaatgacaatgttgaacaccggaaccctgatgatatctgtcacatttgtaaggttgatttcagagtcaggagtggagacatcggcagttgacttgggtggagcttgggtcacagttctggggctggtatagagtgggcacaaggccttagtggtggtaggaggaatcttatacacattctgggtagaattctcattggagccaggggtccctgaaaaacccttggtcaccaccaagcggatgcgatcgaacagcatgtgaggctccttgggaggctggtagatcacacactgatacagtccagaatcttccacttgaaggttgaccattcggacgcgcagtaaaccatgatcatggtagtcttctagtatgatcctccccacttggactggatgggaattctttgaaggcctctctgtgcatgccagggtcttgggcatctctccgtcccttattatctgccaagctttctggctgctggcaaacttctctagcgtgtagtcacatttcacatccagggtctgcccctctttcagttcatacttttcctcagttaatttagttgcagctcggagttctgagacaaagagcatccacagcagcccccagagcctggtcttcctcatccttcctgtgcaccagctccaactgct

SEQ ID NO: 17654 - RNA, 1758 nt, Homo sapiens
  source 1..1758: mol_type = other RNA
tcaggtgtggaaactgaggcaggtgttccaggagcagactgagagaagaggaggagggcagagtggggaactaggcaagcacatggggacagcctccagaagcctcccagggggagagcttttactccaccatccctgacccttgtgtgatacaggaaaagaggcatttagacacaggcggaactcctggttattctattctatatggttttggggtccttcaggtaaggagcgcttcagttttcactcctgccagtgggcagtggcttattcatgtggcctcgttctagtcacatacatttctgccttcacggggctattttcaggatccagcgataaatgcacacaggatgtctgacatggtctgttgttgctctcctatggatcccatctcggcctgccagtatttccccagaagaagatactcagtttaactcttttctctgagaaggatgcactttctcaccacgatgtcttatttctccaggttccacaatcttcaacacccttttctgggagtgttggaaagaaccacacataagcatgaaacccaagtgtctgatgctagaaagaggaagtcccagcatggggcgagcaggatgcttctgtagtgggagctctgtccaggtcaggccaaaattgtatggtccagggcaaaactgagcaggagaagtatcaggtgtgccttctgcatgtcacagcccccacaagagaattacggtgaaaagcattgagctgtctgtatttcatgccaaccccaagtggctggtggaatgaaggaccaagcatgtttggggctgtaacttcttttctgaggcacaaatgcccacccaagattattagaggaacgagggcagtgggcaggaaggtgagacgctgactttagaaatagccggtgattacagatttaattcatgttattaactccctgccttttacctcctccctcctcccttggcacaactgccagatggatgtggctggaagtcagaggacattctcgtgggttcgtgggcctagggtacaaatgacctcagcgtgacagcaaacaggacagagaagaccaggctcttactcaggaatccaccagccaggagaatgacaatgttgaacaccggaaccctgatgatatctgtcacatttgtaaggttgatttcagagtcaggagtggagacatcggcagttgacttgggtggagcttgggtcacagttctggggctggtatagagtgggcacaaggccttagtggtggtaggaggaatcttatacacattctgggtagaattctcattggagccaggggtccctgaaaaacccttggtcaccaccaagcggatgcgatcgaacagcatgtgaggctccttgggaggctggtagatcacacactgatacagtccagaatcttccacttgaaggttgaccattcggacgcgcagtaaaccatgatcatggtagtcttctagtatgatcctccccacttggactggatgggaattctttgaaggcctctctgtgcatgccagggtcttgggcatctctccgtcccttattatctgccaagctttctggctgctggcaaacttctctagcgtgtagtcacatttcacatccagggtctgcccctctttcagttcatacttttcctcagttaatttagttgcagctcggagttctgagacaaagagcatccacagcagcccccagagcctggtcttcctcatccttcctgtgcaccagctccaactgctgctgagggct

SEQ ID NO: 17655 - RNA, 7818 nt, Homo sapiens
  source 1..7818: mol_type = other RNA
tcagtaaatgtttattagatgaaagaacacatgaatatgtcattaattagctttccagtttcaaaattagtgtcaatagcatggacgtaagattattgcaaactgagaaagggacttaggggactcagaaattataaatctttttcttctttttctttttttggagatgaagtctcgctctgttgcccaggctggagtgcaatggcatgatctcagctcactgcaacttctgcctcctgggttcaagggattctcccacctcagcctcccgagtagctgggaccacaggcgcgcaccaccatgcccagctaactttttgtatttttagtagagatggggtttcaccatgttggccaggctggtctcaaactccttacctcaggtgatccacccaccttgggctcccaaagtactgggaatacaggcatgagccaccgcacccggccagaaattataaatctaaccaggattcccaaacctacaatacaatgaaatatcatttctctcttataggtttttggttttaaccaatctattttaaaaggggcaattcaaggattatggtttatatggtggatttctgttgaatatgatcaaatgttcactggagaacaagcaataatttgcaaaaggcatatttatgccttacattaaatgtggatcctcttctaaaactagaataagcatcagttcagtcacccaacgtgggaagaaagaatagaggtggcaagaaatgaagctcaagtttgttttgaaacaaaagaagaaacttattaaaagattcttctgagttactacataacaaccattcttctagttggcagtttagctagtcagagagacaaaaaaaaacaaaaccaaaaccaaaaacaaaaacagatgtcctctatgtgcctatttattgtgccttatccttaacttgaaattctatcctttaagagaatgaatttgtgtcactcatctgccagatgtttttgtttttttagagaaaggtttcaaatcagccacttaagcagtctattactagtgtaaaataaattccatttaacatcacagcataggaataatgatattgctcaaaaatacagaaccctgatatatagcataattattttagaactatcatcacacatttatcgagtgtctatgtatccagcacagtgaaagatttagcttaaagggtggaggcgggcagattgctacaattggtttttaaagacagtatgtggaaagtcagaataattttagattaccaagcaattagggggcacagagaaagaacagcaggagatggcagactgctctacttccatcttcagtggggttaaaaaaaaaaaaaagccacaataacaacagaaatttaactgaaagtgatgtccaaactcaaagtagagtataataccacctggtaattaatgtcatacctgacagagatatataaaaagaatgaatgactacagtcaaattcaacttaaagtttaagcagaatcccaaatttaagtaagtctcttttcattacatagatatttgatctgatcagagcaatttgctttgagaccaaagagatctggcattttacttattcattaggaattgaaaaaagaagacctttggctttctaaccagccatttcattcatggcatcaacagccgatggcagccacatggaaatgtatgctggatatttggatagtttaaatattatgtacaaggaatagcttataaccagtgaaaataataagaacataattcagcataagtgtccaagataagatacaaaaaagcagagaaagtgcttgagtctacaggtcttccctgaaagtttcaaaaatgtttaattcttaagcaggtaggccttttaatagaatttgcatagcagcatacaaggtaatttgcattaaaatatatgaacagagattcttccatggctttgaaaacaaatatatccacatgcatataagttaagcaagaagacctggaatttctcacaaaattaaaaaaaagaatctattataaccttttctcacactttcgcccatcaaaaccatttacagcaaaacctgtttctaggagaaacatagccttgtccagattccacacagcttaattttttttttaagcataatttctggggccaggtgcagtggctcacatctgtaatcccagcactttgggaggctgaggcagaaggactgcttgagtgccaagagttcaagaccagcctgggcaacatggcgaaaaaaaaaaaagaaaaaaaaatccataaaaattagccaggtgtggtggcacacacctgtggtcccagctactcaggaggctgaggtgaaaggatcatttgagcccagaaggttgaggctgcagtcagctatgatcataccactgcactccaacctcggtgacagagtgagaacctgtctcaaaaaaaaaagaaggaaaaaaaagaacaaattctggtttatcagctaagtgcattcattcagctggaaaagctttgttaccattcaacttaggaggataaattaggaaaacaatcagtaataatgttaggtatttgttgtttagaaagatttttttacttataaaaatataagaaataaataatccaatctctcctgccatgcaataattttgagtaacaaagtttgtgagagtacagaacataaaaacaggcactatcagaccttctttggcctaaaaagtgctaaaacatggctttaaaataggtgaatgacatttaaagtagtatttttgactgcctatatatgttccagtatttaacctgaaactcttatctactagggaggtgagtttacagttacaactatctaataaatactgcaggaacttatatttaagtatttcttcatatacaacattagaaactaatttccagataatgtttcatttgatgacttcaggaaaggacttacctttttcagaaaaagaaaaactgaatgtttttcttttgttcctttccttttctttttatggagagaaaggagagaagttttaggagaaaaggtgggagacttttcatataccaactcgctgctcctaggcatctgtgtggaatgtggagaagctgtcgaagccccgggtctggggggcacaggaagcagtccctctgaatggggagcagacactattctgcagtttcctttccattccacacactggaacccaccacatcctcaacaattttcttaattcaaaatgaaaaagaaatgaaaagtgagctggttctataaaaaaggtagaatatcgaaaattcccatttgtagttatcatttggaaataatttgccatactttggcatctaaatataaatacatatttatcatggtgtcccattcattagagagcacttcatttgcggactgaaaatcccacaaacacatttgattgaagaacaaccttggtcatcatgactggagagctgttaggtatgtaagaaaagcagcaaaagggttctggttcttggggctgctaatggacaaaggaaacctcccacactttcatttcacagcaagactcaaaagatattaagaaccctacagacctcagtgctatacatgtcagtttaaccttgaccaaaatgagtgaaaatgcacacatgccttgcctttcctgctcacattttaattccacctattttacatcctcatataaccaacaagcagggtggctcagaagctcccctgcaaatctcagtggcttagcttttcacattaacacagaaaacctcaaccaaatggctttgctgctgaagtctgtaaaggcatcattcaacatctcatattaataatgctctcactgcatagagggttcaagattgcctacctgagggtattacatattgaaattctgattccagaaatcatttctggacgttcaagagatttttttccttctctgaaatgaaaatttattgtgggccaggcacgggggctcacacctataatcccagcactttgggaggccaaggcaggtggatcacttgaggtcgggagttcaagaccagcctagccaacatggtgaaaacctgcctctactaaaaatacaaaaattagctgggtgtggtggtgggtagctataaccccagctactcaggagaatcacttgaacctaggaggtggaggttgcagtgagccgagatcatgccactgcactccagcctgggagacagaacgagactccgtctcaaaaaaaaaaagaaaagaaaatttatctcagatggagccaatcttaggtttatgaactttcaaaacataaaaagctcttgaaagacatattcttgtctagattttaatttccagttttaagcagttcagataattcatttttggaactttgacaattatatgaagctgggggaagaacaggcatctctccccaacctctgcatattgttggtttcactgtaatgaggaaggaggactgacttatgggtgaaggaggacaatggagttacaatgttgacctagaactctctctgctcatgggtcctccccatcggtcaggccgcactgaaaccaaatagctcattttgcacacaggtgtgtttttctcttcttttctccccctgtgcctgccccatctgaagtgacaccctcctccaccctccacagcgctcacattcttccgtggcactcttgatcaatcaagcaaacaagaactttccctagacctttcttcagagagcataaagaacatccaagtcaatattacctattctttgagatccagggactgtgctaattttgacattttatatgatattataccattttaaatgtttgcagatatataccaccttcaaaattaggaaaaacaagctgagttcattttctaacactacaaaatcagcattcttgctgctactgtgtcctaatgatatctggcaatcttaaccaaaagcaggtagctgttccacggtctcatcaccctgctcactgtagggtgtgctgtgaagccaatagtaagtctcgaattagcagttgcttgtccatgccactgctgccacaaagggccaggccacagccaggatgctgcatcctgttgtttttgggcagcccaaaacaattcaacatgacgtttgtgcggaattgctggcttcacccaccaagtctactcctcaagcaggctggctctttaggatttatcttgttcaaacagatctgcctactagaagagatgccattaaggaaacccacctcaatgactattcctcaaaactaggataggtgatctcctggaaatggcagtgatttccagttattcaaatagtgactaataaagctccactaaccctaaccaaaggcacatttggtaagcaataaaaaaaatggcttaacctaggaagaggattttcatttaaaataaatcttatcccctggctcctaacaaaaataaaattggaaaaacctaaaccaagcaaaacttttctttaaaagcagtggcttccaacttgcttttcaactcagtcaccactagaaaggaagtagaaggcaaggcaaatcaaatttacaagttctaagtcctagagacagtggcaaagcttgggataaggtgggaagtgatggccaggctgagatagagggagatccagggcaaatggaacaaccctttggtgatacaattcaaggacttcctatggtggaaggagctagtgaggacagtaaattccaagacatacgacctatctggaatgctcaggaagcaacaggctgctgcaagctagcacctgggaagggacaattgttctgaacaagagatcaaggctaagcacaacacaaatcctacagggagaagaaaaagaaaacaatgcttgggtatttgattatgtctaaaaatgaaaacaatgaaaaaaaaagaaaacaatgagccattctttttagcagtagaaataaacctaattactcataaaccatattttgaaatgagaataaatcaacagcttcattttggagccttttagagtgctagaatatctggccaaggtagactgtgaaaggtaggctcttctttaaacacggttatggttcagcagttatttgcaggtccttgggaaggcactgtgctgaaggagagcaaagagtttctttttgtgcttttttttttttgaggtggaaatatttcttgtgacagtcaaggctcttttctgattttttgttgctcatacaagcagtcccatacgagtgactttggccgataaaaacgtgtgcaacacaaatacaatcggcttcggacaagagtgcaggtccatggtcagttctccctcgggaccaccaaaatccaagtatagatttcggatgccatcatcagcagacatcttcagcctttcaaaggggtagcggtacaatatgctgctggagcctccattttcccttgagatggtgaacccattttcatagtgaatagtaagcctcacctcttggccatttaacatgcagcctagagagacttccttgatcagctcagcagcagcatggcaaccctgaacaagtatcctggtccaggatgacagatcccgatgtgtctccaccctgaagagatgcatctcaatgccctgtcgagagcctgtcctggtagcaaatgtaaggtcagatccaagggagggggatcgacatccggagccagaatgaaccaacctggtggcaacaagtgggtagctgtggcatggtgacgcccaggcatctcttgtccacggcatacagtcatagagcagcaaatccttctcagtcacagccatgaggacaggtctccattgctgtcttccaccatctagttttgcctgttctgccagccaggcaatatgcttcacctctttactgcctcctgctgtactggttgccccaagcatggcgttgagttcagccaacacctgtgggaggagagccattatgttggtgtggatagctacgaaccaggagtgtgctgtggctgtatctttgcagcgtaggatcaacgtgttcctgctatcaggagaatgtagctctatcaatctgttttccagatccggcatgcttaggtttctagcagcaaagcacattttgagagggatgatcttcctgtccttggtgctgttctggtgttttggcgaaccagagtcctcactgccactaaagcttggtgactggggggctgcaccttcccacggcagatctgatactaatgatggcttcttgatatatggtgttacttctcggatgaacttgacctccagcagcacctccttgcccgcgcgcttcagcgcctgcacggcctggtcgtgggtggcctggcgcaggtcggtgccgttcaccgacaggatggcgtcgcccagccgcagcgcccggctctggtcggcagccagcccggggaagatcttggagatgaggatcggcatccggttctcgcggccgcccttgatgctgatgcccaggccgcccgcctcttgcttcaccacccgcacccggcgcacgggcggcgacgcgcccgcctcacccgcggggccccgaggcggcgccggcgggctcgggggccccaggccgcggcttgggctcccgggcagcgagtcgcccgcgccgccgccgtttgggaggccgttgaaggcggcggccgcgggtcccagagcgggctccagctcggccgcggcggcgtcgcccgtcaggctcaggctctccccgctcagctcggccaccactcggacccagcgctccctcaggagcagctccaccagccccgctttggtggcccgcgtccacaccgccatggccggccccgctccagccgccgcagtcgccgcagctaccctcattccagtcaggcagcctcggc

SEQ ID NO: 17656 - RNA, 5302 nt, Homo sapiens
  source 1..5302: mol_type = other RNA
tcagtaaatgtttattagatgaatacatgactgcatgcgtggaagtactcaagattatttgagtagttagtgacctccacagtgtgatacgaagtttgccacccttatctatttgcctttgcttaaagccatttttcctggttttgaaatagtcctatccttgaacattgactacaaaaactacccaaacattatcagtgaggatttagtgaatacagaaaactttctaacacaaattaggatgccaaatttaaggtaactcataggttgccaagacaacatttcttcagtctcacagttttactgaaatctaattctgaaaactcctttatagagaatttcatgttctacctcacaatgcttaatgtttattttaatgacatcctcaatatctctttatagatatcatctaactcagtgattccatctaatgatgcccgtgaactctggaggggttcttataatactttatgctacagtgctatagaccatctgaaaaaaaaaaaaaagaagaagaaagcgtacgatagtcacactgataaaagaatgctaaaagtatggtgaatgctttcttttgttgagcccatttcagaaatgaactattattatccaagctatggtcttcttaaggctgagtggaatcaagacataaaataaaactaaaataaaccacttgcagcaggccactgaaattgccagtcattctcaaaacagctttctataaccagagtagaatttttgcttaaattttcaattctgtctagtttccccaggtagacagaggctaaggggttggacaattcacagaaagaaaaacatttacaaggcgtaaagctaataactagcatgtaaggggagtttttttctctgataatccaactacttttaaaattaaaccttatataaagagatgtgtaaaaatatgaaccactactgctattcttactattttttgtttagagaacacggctatttttcattaaactgttattgtgtttatctacttgtgtttattatggctgtctaaaataaaattgtaagtgatttcatttaagttagttgccttcattttaattatttgacctaaataaatgtgggtttttgaaagggattcagatcccaggcagaaaaaggattaagatattaacgatgttgctaatgtcacagagaggagatttcagatttcactgtagcttagtctcttgtgacattctggatgctttatcatttgtagtgaatttcaaacatgaccaccataattcatagctccttccatgaaaacatgggaggggggactcgttttttccatatattgaatacaagtttgtcttcagactggctttgataaaagaaatgagtcaaaaatgtaattgcccctctgaatctaggcttcaagaggacttgcaatttttattaagttcttggaactcctaccatctgctgccatgtgaacaaactctccctagactgttggatgatgagagacatggtatagccaccttcattagccaggctagtagagagagaaacatcagctgtgacaataagaccatttcagatatcatggcccatgaccaagtccattactgaccacagaagcacgagtgagcccagcaacgatcagcttagtctgacaagatcagcagaaatgctcacatgaccaacagactcatgaacaatgataacgattagttttaagcaccaactttgtgggtggtttgttacatgtcataaaccagctgatgcaatcttcatttttacattcaatgactatactgttgagcaccaatttatttatggtatgtaagccattgtattaagaactggaaatacagaagtgaacaagtcatagtcgctggcttcaaagtcatcaccaccttttgggagacacatttaagcaaataagcatcttaacacaatacaatacgtactatgatagggacaaacagagtgttctatgggccatccaagtgctccatccaagagtgtccatgaaactgtccatccaaattatgcacatataaatgacttcttatttacagacttctataaagtcaaaatagccaaactgatattctgtttaaatgcagtgtgctgaactaaccctcttcctttctcaattactaaataaaagaattaaacaaaaattacatcacattctactcttcctggttagaaaaagcagagctctttacaatcaggcagggagaggaaaaagccaacttttattcaaaaccataatgcaggtttctagtattacaaaaagtacaaaatcaaggccatgccaatggaattatttattccaatttgacttagattctctagttccatggaatgaaactgtttcccttgactagatgctcttatttcttaattatttagaaagaaaattagaaacagttttctttggtggggaaagtgaactcatgctgatgctcacatatggaactggatttaattcgcttattcttccttgccttcactttcaaccaataatgtccaaggaaaatctcattattcttcagggaagatctccatattccccatttgtggtcaagtgtttgatctggttctggaagagcctcaggatgcatgtttggtgaggctggggaagggttagcatttcctagtcctaatcattgtgagaggttctaatggagttagtactagagaagcaaaggcttccttgtctgtctcactggatttgggcagtaatgataaaagcatgtgcaagcattggtctcatcccactcccatgacgaccaactcagagactgacaatctgtaaatacaggattctgactcacttgcttacacaaagattcaatttctatgctcaatgtttgaagttattctcatcagctaacccgaagtagaagatatctgttatagatgtagatgcaacttaggaaaagattgtgttcccatggttaaggtacagtttgggagttggagacgtcaaatattttaccatataaaaactattttcaaacaaaaggttaagccctctcaattatttcaattaggttgaacattgtttatagaatttcacatcaatttctacctaaggtagaaatcagctagattgtactaggtacatgttgttcaaccttgatagcaatagtctgttgggagaggcaagtctgaaagtcaggaagttttaaaatttttagcttctgtacagaatgagacactaatattcttagactctgcacataaagattctttaatgcaaataggaaatataaacacttatgtatagtcctggttgtggaaacattattcttaatgtataaagtaacaaaagggaaatatacaattttattgtatttgtacaaaaaaacccatcatgtatttttttcatgttataattaaacacacgtaaacctaatagtaacagaaagaaattgatgccagttacttaactatgttatcagttgacaatcaagtggctcttcttgtagatcaagtaggggaacactcttttaaccataatttcttctaagtaatctcttataaaagacattccattagatatagtttatatttttattgctttattctttagtgctggcttatgtactgatattatggaaaacctaagggaatcttcgtggtgtgatacatgcaatgtgaattccttagtaaatttaatattatagtaaccattctggtttctagaagtgaaacaagttgatatggtcaaataattgccaggagccagaagtaatgatgtaaacctatacattttttaagtgatgttgatgttatacaaaatctatagcagtcacagtttgaaaatatcaacttgaaaatatgtctcattcaaatactagagtaaacatttgatatgcagctaatctttaagtttcttgttttgctttttctcacatcagcaaatgtgcagtcaatacagtatgtgcaaagactcatatacaattacgtatataacagattgtaaataccctttcactttattcaatgtgcaaatactatagtaaacatttgatatgcagctaatctttaagtttcttgttttgctttttctcacatcagcaaatgtgcagtcaatacagtatgtgcaaagactcatatacaattatgtacataacagattgtaaataccctttcactttcctctgattaagatatttttatgtgcacagaatattcatgaataaacacatgatacccaaagaaggttacagataggaataaatcatctttattttaatgaagcaaacttcttcttgcacttctaacccttgtgctcagattaaagagtaaacgaaagcacttcctagactagtttcataaatgtatacacatacacgaacacacacactcacatacttggattcacttgtgtgtcagccctctgccagaaaatgtccaggatgcagggactatgagtctaattatgtaactactcatgggggaggcatccttttctagggtgagtgcaatgagagaagggtacataggttatcatggggatgctgggggaggaatgaaactcaacctagcagaaagaagacttgggaaggaaatgacatatgagtccgcacctggcctagtgcctggctagaataaacactagagaaatttttgtctagtagattcttgaagatgcattgaagcagttacatgtaattagtatggaccttcatacaaaatcaattgaattacctcattttatttttgttgctgccctagaaaagtatgcctttggtgcaattattttgatcattttgatttagtattgtaataatttttaattgttaattgtgacaaatgaagagctcctggcaggacaagaaatgtcagctccaatattcccttattttcttatagaaaagtcttgactctgtggtttctttgtatgtactttctaggccatggggttatttgtgatggttagttgatggaaaattctaataatataatccactaatttagttaagcaggtaaagataaactaccatacactgaaagagatttaataaatgaggacattatgttcaaatttccctctgtgaagcatttattctttcttcttgataatgcaaattctttcgagtcatgtgaattgaactgacatattgagcaagaaatcacaccaattcccatctgcatattgaatacaagaaaagctcaaattattccttaccattttagagaaaataaatagaatttctaaatcatctttttggcccacaatgcattatcttgcatgccccagggaatgcaaagtttccactggtctttttattgatatgacacttcttttgtattgctgagt

SEQ ID NO: 17657 - RNA, 1389 nt, Homo sapiens
  source 1..1389: mol_type = other RNA
tcagtaaatgtttattagatgaatgagagaatcctgacatgagcagacacctcgtgctgtgttgtggaggcggacaggccctgtggggagtggggacacactcgtgtggcagcttcccccagccccaacgccccacccctgcttccctaggctgcaggccaacttcaccatccgggaagatgccaaccccagctcccgacagcgaggactcaagcgcttccaggctaacccggaggccaactggggtccccggcctcgtgcccggccagggtgagtggtggtaaggtgggggtggggctcagccagggaaagaaggggtaaagggcagatggggtcccacctactcctcccctcgcacaggggcaaggcggccgacgaagctatggaggagagacgcaggctgcttcagaacaagcggaaggagccgccggaagatgtggcccagcgggctgcccggctcaagacatttccttgcaagaggtttaaggaggtgaggtccctcctccctttcctccactgcaggacacatgagtctcccctttgggcaacagggagagaattgggggagctggggccaggcaagtgtttgggagtgggcttcccatcccaggaaaggatcccatcaggggctgctgagctccgggcaggggttcacacccaccatcttcccaccagggcacctgtcaacgcggggaccagtgctgctactcccacagccccccgacacccagggtttctgctgatgctgcccctgactgtccagagacctccaaccagaccccccctggacctggggctgccgctgggccaggcatagactgaaccaataaagagatgtcacgtcaccttctcccgattgcctgtggtttgtgtattggtccatacagctgcatgactgggatctgttcctctggggatcgttcgcccctgcctggctggagtgttgagtcttcagcgctctccaggccacgggcttgcgcatagtggggcgctcctgcccggtagcccccacgtgtcttcgcgccgctgcctcctcgccgcctggtttctttggcccagctctccaggggccacagtggcggaagctggaccggaaccaggcgccctgtgcatccgctccagaccaggtgcttcctgccctgaggcccggggcgaggggggcgtgcacacaaagagggacctcgcaggctgctgcccagacacccagtgagggggagctgtacccctccctgccctccagagtggggtttagtaacgttaacgaagagtcctggggcaggatcccctctctggctcctgctcccttcatccccatctgtaatgaggctaatcttaggaccctccttgtagcgatatcagagttagcgcttaattttttttttttttttt

SEQ ID NO: 17658 - RNA, 1915 nt, Homo sapiens
  source 1..1915: mol_type = other RNA
tcagtgcatcacagaactttgtgtgccaggtttctcctctgtaaaacggagtgggaggaataatgtatccacctcccagggcttacctgaggatagaaaatgggcacctagtgttctggggcactaggaagggaacttggagaccttttgggcagggcccacacggcaggcactctgagtggggaccctgatgccagggagtggggcctgggcacagagggcaggatggtatggtaactgggaggggaggtggaaacatgggcccagggaggatcagagttggaaatggagaaacagagtggtttggtcgtggggagatactgcctggagggagttgcagtataggggaggtcctcccctgaaggtgaaggtggggagaaaacctggtcaaatcaccctgagtatgagcaatgaagccacctggccctgacaggctggagaaaagatctctgacaccccctgcccacagcatggtcatcgttttatacctgagtcgaaagtaccagatacggggacactggtacccacctgagctgcaagcccgcacctgcgtggatgagtacttggcgtggaagcatgtcaccatccagctgcctgccaccaatgtctacctgtgcaaggtgagcttcctaggccctgtcatgcaggctggggcaggggcctggacccccagagatggaaggcaccagttggtacatattacatattagcttcacttccactgtcctcagcagacataactaatctatcacagtactccttcccctaagcctgaatgaatccttagaaaccttctgaacacagagccccagaggacatcactaatgagtggcagccgggaagggatggagaggaggcccaagaggcttccaagagtctgggttaagttgctcctctcctcccagcccagtctctcctgccccacttctccggacagcctgcagatgctgcacagctggagcggctgttggggaggctgatgccagccctgcagcacctggattggggggtgctggtggccaggcccttcctggcaatggagcagatctccctggaagacttggtgctgacggaggtgatgcaggtgaagctttcctacccacctgccctctggggggactctgggcatggggctgagccccaaccccagctgccctgtcttcccagcccactgccgttggctgcgacctcttccaagactgccccggctggcagtgtggcaggcccgtgtggcggctgcccttggtactgagctcttgctggaggcccacaagctcatactccagcctctgaaccacagtgaggcttggcgggacccccagctggcccagaagcaggtgcagtgggtgcagcccactccactgcaccctgctgtctgcaataaacacactgcatgctcttcgcttgtctccaggcttactctgtcaccagaagtggggtcagtcccatttctcagcctagacctattagatcacagcatagagtgagtggcactcagtcctctacgtggggctctagttaccttccttggccaccaggtacacagtctggccactgcagccccaaccaaggccaggaagtttctaggctcctctgtgtggcacacaccggctgagtgccccctgacttcctggtggtggtgtccccattgctcccaaagctcacagtttcctgtgtctctttctcccagttcctttctagtcatagttcaggctcgattcacctgtgtctctttctcccaattcctttctagtcatagttcaggctcgatttacctgtggatactcccagcctctacttctagaatcctccagggataattctcattgcctcctcttcattctggaccctgcaaagcccctttcgtcaggttctttgccacgggcctctccccagcctactcctgggcctcctt

SEQ ID NO: 17659 - RNA, 606 nt, Homo sapiens
  source 1..606: mol_type = other RNA
tcagtgcatcacagaactttgtgttaagtttctgagacatctatcaggcccgcagcatccctgggtgaggagtgtgtggcagagggaaccaagggtgaattttcacgtctagttgttcaaaggggcctgggaggccagttgaactccaaatttagagttcagagcaaaggatgaaggaactgtgccaaatggggccttggaggcgttcagtgggatgtaacggggcagggggccatgtaggttctatgctcagtttgagtctcgcagaagcaaagagtaggcgctgaggactggggcaccgaggactttgtcaaagtctccgggtcgggtgggcgcgtctgtcagatggggcagggctgaagtgagtttccgcaccggacggaccggaaccgtggcaagggacgctcccggggctccaaagggggcaagggacatctgtcagacggggcaaaggtctcgaggagcggcggaggagtgtttctgaggcctgggaccctgcgagcggcgacagaaggccctgggcccacacaactaaagggcctgggggaggggggggtcccgcagactggacggaaggcgtcgggggcggcggcaccggcaggcggg

SEQ ID NO: 17660 - RNA, 3328 nt, Homo sapiens
  source 1..3328: mol_type = other RNA
tcatagccctgtacaatgctgctggtattctgaattgttttttagacacacctttcatcatgctgataatgattcatggagacagaagccgtcagttaaaaattcctctcagatacaaacagaagcaagtactctccaatttactgaatttgccagatgatggactttagctttatcgggagctcagggttgggttccaagtcccaccaccaaggtaacagtgccgtggctgggagtgccccacaacccctgcctctaggaaccagcccttatgggagcacatgggctggggtgagggcaccgtggcagcctttggggccactcaagtcctccatggaaccgagactttatcaaggggagttagcgtccccttcccagtgctcatatccaatcattaaaatagactttaaaaaaatataaaatccgcctgagaacgatgggaatcagggacagtggtcagcccctaccctgctgagcattcaataccacctatgtgcacctggacataatgtgaaacctacacgggagagggacatgaatgtggtggggaagccccaacagagtggggaaatttcagttgtgccaatttgaagatggtgatctggcatagatcagccacaagtgcgctccttttaaacgtggattattatgtattttaaccatctttctccccattttcccctcttcttcattccgtattgtacctattggttagggagtgattggaattaatctacagatactgacagttcttttcccttgagtcaatactgtaagcaaagcaatgcattcgttcgcatttttttctggtagcaataaagataaaaaaattagtgtaaatatagaaagaggccgtaaatggaggtattttaatcaattacccaagtagggggaagaagattggaaaaacattaaggtcaagaaatgaaccatcctttaaggctgattaaaacacctctctgcatgtttttaaaacctgaaggaaattttatttttcttcccactgaggtgtgatccaccctcttggtggggcctggagagcttctttaaacaatccacgtttaaaagtgccttgcgctagaatttctgacaccccgaggggcagacagtgttgggccaattgggtgggtgtttggggctgagagatcagggttcctcactggaacatctttctcaatcaagtgggcaaacctgatctacagcccggcccaggtgtcccggattcccactcattctcaggcctgccggggagagcacactctcgatttctgcccgttgttgtcctggactcgaagggacagggaggggctggtcacttcctccgtgcctgggcctggttactctgtcccttctgatgctgctgcttaacctgggccaggatgtctcggatcttccgttgagccatctgactggcatagaaatgtccgatgattttcacgatgacctggtcgttctcatcaggggtctggtctcttggtactaccacctcagctgccgtcaaattctgcaactcgttcaccgtttttccacctttgccaatgacccggccagctgctgatgctggcacacgtatgtgggtctccagcttcacttcctccttgggaccaaagaagttctcctccttgagtttgccatagattcttccctgagccttgaattgggcctctggcggtccagtgatgataaccatacgaactttggagtcaggtgtttcgggtggtgcaatcttgatggaggcgctggcaaaccgggagagctgtttgatgtgctgccccttcttgccgatgatggcgcccactgcctgggcggggataaacacctgcaccatctcctgctcgggagccataaaggagctatagggagcagccccagtaacgctgctgggaggcggcgggactgcgctggatgaagctgggaaaagacctacagcagccaggttcaggccagggatcaggtgagactgcaggctcatggcagccacatcattctcataggcctcccgaactttcttcattatttcctgctcggccctgcaacaattctcgatggcccccttcacagtgatggtcctctcagggttgtaaagggtaaggtcttgcaacgaggagatggtgatttttgtctcggtatcttgctctaccttcttcaggttccgtccttccttgccaatgagacgccctacaaagttattatgggccaggatcttcaggggaacctcgtcagccgttttggtgtccttagcctctttatgcataatctccaagatcatcttacaagcggaggagcagccctcaggggtggagtgcacactgatggctttttcagctgcacctgcgttctccttcctatgcacgtctatcttggactgggtctgttttgtgatgttgcggatggtggccccctccttgccaataatggcacccacatactgggtgggcaccaggagccgaagggggatgtccacttgctgctgcttggctggggcccccgctgccacaggtgagccctggcggggctgaccccgagagccaaagccccctcggcgcccattctcaggtccctgtgctatctgctcatcggggatgtaggagaccttcagggcatggttctccaactggtggccattcagcttcatgatggcttgcctggtctgctcccggttggaataggtgacattcaccactgccgtctcactctcggtgttcacttgctcacagttctctactgtaccatactgagccagcaggctgtccagtacttcccatcggagctggggtggaatatttcggatttgaattttccggctcctttgttttttgggcaccgaatgttcaatctctaagcgttttccttgtaattctactttcccggagaaagtttcgatggccttcatcgcccagtgctcgtccgggcagtccacgaaggcgtagccggatttgaccaagaactggccgctgtaggagatcttgtgctccgcaaacactttctccaagtccgcgggggtcacgctctcgttgaggttgccgatgtaaagcttgttcatggtggcggtctcggggcaggacgcggtcccgggcaaggccgaacgagcgggcgcgggcggcgagcctcctaggccaagaggcggagaggccggcggcaggagccgcaaactttctttgcaccccaccccagaagttgtcccgagcccagggcggggaaggcggcctgagggcgcgcagaggtcgcgggagagttcggggagagcccaggagaagtgcccgcggcgcgcagggagacggacgacacggcgcagcttcttcccttcggtccgaaacccctccgagag

SEQ ID NO: 17661 - RNA, 3103 nt, Homo sapiens
  source 1..3103: mol_type = other RNA
tcatagccctgtacaatgctgctggtattctgaattgttttttagacacacctttcatcatgctgataatgattcatggagacagaagccgtcagttaaaaattcctctcagatacaaacagaagcaagtactctccaatttactgaatttgccagatgatggactttagctttatcgggagctcagggttgggttccaagtcccaccaccaaggtaacagtgccgtggctgggagtgccccacaacccctgcctctaggaaccagcccttatgggagcacatgggctggggtgagggcaccgtggcagcctttggggccactcaagtcctccatggaaccgagactttatcaaggggagttagcgtccccttcccagtgctcatatccaatcattaaaatagactttaaaaaaatataaaatccgcctgagaacgatgggaatcagggacagtggtcagcccctaccctgctgagcattcaataccacctatgtgcacctggacataatgtgaaacctacacgggagagggacatgaatgtggtggggaagccccaacagagtggggaaatttcagttgtgccaatttgaagatggtgatctggcatagatcagccacaagtgcgctccttttaaacgtggattattatgtattttaaccatctttctccccattttcccctcttcttcattccgtattgtacctattggttagggagtgattggaattaatctacagatactgacagttcttttcccttgagtcaatactgtaagcaaagcaatgcattcgttcgcatttttttctggtagcaataaagataaaaaaattagtgtaaatatagaaagaggccgtaaatggaggtattttaatcaattacccaagtagggggaagaagattggaaaaacattaaggtcaagaaatgaaccatcctttaaggctgattaaaacacctctctgcatgtttttaaaacctgaaggaaattttatttttcttcccactgaggtgtgatccaccctcttggtggggcctggagagcttctttaaacaatccacgtttaaaagtgccttgcgctagaatttctgacaccccgaggggcagacagtgttgggccaattgggtgggtgtttggggctgagagatcagggttcctcactggaacatctttctcaatcaagtgggcaaacctgatctacagcccggcccaggtgtcccggattcccactcattctcaggcctgccggggagagcacactctcgatttctgcccgttgttgtcctggactcgaagggacagggaggggctggtcacttcctccgtgcctgggcctggttactctgtcccttctgatgctgctgcttaacctgggccaggatgtctcggatcttccgttgagccatctgactggcatagaaatgtccgatgattttcacgatgacctggtcgttctcatcaggggtctggtctcttggtactaccacctcagctgccgtcaaattctgcaactcgttcaccgtttttccacctttgccaatgacccggccagctgctgatgctggcacacgtatgtgggtctccagcttcacttcctccttgggaccaaagaagttctcctccttgagtttgccatagattcttccctgagccttgaattgggcctctggcggtccagtgatgataaccatacgaactttggagtcaggtgtttcgggtggtgcaatcttgatggaggcgctggcaaaccgggagagctgtttgatgtgctgccccttcttgccgatgatggcgcccactgcctgggcggggataaacacctgcaccatctcctgctcgggagcctgcataaaggagctatagggagcagccccagtaacgctgctgggaggcggcgggactgcgctggatgaagctgggaaaagacctacagcagccaggttcaggccagggatcaggtgagactgcaggctcatggcagccacatcattctcataggcctcccgaactttcttcattatttcctgctcggccctgcaacaattctcgatggcccccttcacagtgatggtcctctcagggttgtaaagggtaaggtcttgcaacgaggagatggtgatttttgtctcggtatcttgctctaccttcttcaggttccgtccttccttgccaatgagacgccctacaaagttattatgggccaggatcttcaggggaacctcgtcagccgttttggtgtccttagcctctttatgcataatctccaagatcatcttacaagcggaggagcagccctcaggggtggagtgcacactgatggctttttcagctgcacctgcgttctccttcctatgcacgtctatcttggactgggtctgttttgtgatgttgcggatggtggccccctccttgccaataatggcacccacatactgggtgggcaccaggagccgaagggggatgtccacttgctgctgcttggctggggcccccgctgccacaggtgagccctggcggggctgaccccgagagccaaagccccctcggcgcccattctcaggtccctgtgctatctgctcatcggggatgtaggagaccttcagggcatggttctccaactggtggccattcagcttcatgatggcttgcctggtctgctcccggttggaataggtgacattcaccactgccgtctcactctcggtgttcacttgctcacagttctctactgtaccatactgagccagcaggctgtccagtacttcccatcggagctggggtggaatatttcggatttgaattttccggctccttgaaaacagacagagtcgggctctgtcctccagagggaacagccgaggtggccctctcaggagccaggagaggaaaccagaccagcctccaaagcaatctgtcttcggcagcttcccaccgcaccatgagaaggacccggcagacatccccgtgctcctcggggtccttagtgccccctgatgacgatgggcaaacatctgggcaccagccccgcaagcgtctgcgtgtccataagtggcggccgctgcgcagtagccctcagggatccgcgtctccccctagctgccaac

SEQ ID NO: 17662 - RNA, 3407 nt, Homo sapiens
  source 1..3407: mol_type = other RNA
tcatagccctgtacaatgctgctggtattctgaattgttttttagacacacctttcatcatgctgataatgattcatggagacagaagccgtcagttaaaaattcctctcagatacaaacagaagcaagtactctccaatttactgaatttgccagatgatggactttagctttatcgggagctcagggttgggttccaagtcccaccaccaaggtaacagtgccgtggctgggagtgccccacaacccctgcctctaggaaccagcccttatgggagcacatgggctggggtgagggcaccgtggcagcctttggggccactcaagtcctccatggaaccgagactttatcaaggggagttagcgtccccttcccagtgctcatatccaatcattaaaatagactttaaaaaaatataaaatccgcctgagaacgatgggaatcagggacagtggtcagcccctaccctgctgagcattcaataccacctatgtgcacctggacataatgtgaaacctacacgggagagggacatgaatgtggtggggaagccccaacagagtggggaaatttcagttgtgccaatttgaagatggtgatctggcatagatcagccacaagtgcgctccttttaaacgtggattattatgtattttaaccatctttctccccattttcccctcttcttcattccgtattgtacctattggttagggagtgattggaattaatctacagatactgacagttcttttcccttgagtcaatactgtaagcaaagcaatgcattcgttcgcatttttttctggtagcaataaagataaaaaaattagtgtaaatatagaaagaggccgtaaatggaggtattttaatcaattacccaagtagggggaagaagattggaaaaacattaaggtcaagaaatgaaccatcctttaaggctgattaaaacacctctctgcatgtttttaaaacctgaaggaaattttatttttcttcccactgaggtgtgatccaccctcttggtggggcctggagagcttctttaaacaatccacgtttaaaagtgccttgcgctagaatttctgacaccccgaggggcagacagtgttgggccaattgggtgggtgtttggggctgagagatcagggttcctcactggaacatctttctcaatcaagtgggcaaacctgatctacagcccggcccaggtgtcccggattcccactcattctcaggcctgccggggagagcacactctcgatttctgcccgttgttgtcctggactcgaagggacagggaggggctggtcacttcctccgtgcctgggcctggttactctgtcccttctgatgctgctgcttaacctgggccaggatgtctcggatcttccgttgagccatctgactggcatagaaatgtccgatgattttcacgatgacctggtcgttctcatcaggggtctggtctcttggtactaccacctcagctgccgtcaaattctgcaactcgttcaccgtttttccacctttgccaatgacccggccagctgctgatgctggcacacgtatgtgggtctccagcttcacttcctccttgggaccaaagaagttctcctccttgagtttgccatagattcttccctgagccttgaattgggcctctggcggtccagtgatgataaccatacgaactttggagtcaggtgtttcgggtggtgcaatcttgatggaggcgctggcaaaccgggagagctgtttgatgtgctgccccttcttgccgatgatggcgcccactgcctgggcggggataaacacctgcaccatctcctgctcgggagcctgcataaaggagctatagggagcagccccagtaacgctgctgggaggcggcgggactgcgctggatgaagctgggaaaagacctacagcagccaggttcaggccagggatcaggtgagactgcaggctcatggcagccacatcattctcataggcctcccgaactttcttcattatttcctgctcggccctgcaacaattctcgatggcccccttcacagtgatggtcctctcagggttgtaaagggtaaggtcttgcaacgaggagatggtgatttttgtctcggtatcttgctctaccttcttcaggttccgtccttccttgccaatgagacgccctacaaagttattatgggccaggatcttcaggggaacctcgtcagccgttttggtgtccttagcctctttatgcataatctccaagatcatcttacaagcggaggagcagccctcaggggtggagtgcacactgatggctttttcagctgcacctgcgttctccttcctatgcacgtctatcttggactgggtctgttttgtgatgttgcggatggtggccccctccttgccaataatggcacccacatactgggtgggcaccaggagccgaagggggatgtccacttgctgctgcttggctggggcccccgctgccacaggtgagccctggcggggctgaccccgagagccaaagccccctcggcgcccattctcaggtccctgtgctatctgctcatcggggatgtaggagaccttcagggcatggttctccaactggtggccattcagcttcatgatggcttgcctggtctgctcccggttggaataggtgacattcaccactgccgtctcactctcggtgttcacttgctcacagttctctactgtaccatactgagccagcaggctgtccagtacttcccatcggagctggggtggaatatttcggatttgaattttccggctcctttgttttttgggcaccgaatgttcaatctctaagcgttttccttgtaattctactttcccggagaaagtttcgatggccttcatcgcccagtgctcgtccgggcagtccacgaaggcgtagccggatttgaccaagaactggccgctgtaggagatcttgtgctccgcaaacactttctccaagtccgcgggggtcacgctctcgttgaggttgccgatgtaaagcttgttcatggtggcggtctcggggcaggacgcggtcccgggcaaggccgaacgagcgggcgcgggcggcgagcctcctaggccaagaggcggagaggccggcggcaggagccgcaaactttctttgcaccccaccccagaagttgtcccgagcccagggcggggaaggcggcctgagggcgcgcagaggtcgcgggagagttcggggagagcccaggagaagtgcccgcggcgcgcagggagacggacgacacggcgcagcttcttcccttcggtccgaaacccctccgagagggctggtgtgtcacgtttctccgcggccgccctggcgccgcctctaaataaaatcgacttgaaaaaaaatggagcg

SEQ ID NO: 17663 - RNA, 2990 nt, Homo sapiens
  source 1..2990: mol_type = other RNA
tcatagccctgtacaatgctgctggtattctgaattgttttttagacacacctttcatcatgctgataatgattcatggagacagaagccgtcagttaaaaattcctctcagatacaaacagaagcaagtactctccaatttactgaatttgccagatgatggactttagctttatcgggagctcagggttgggttccaagtcccaccaccaaggtaacagtgccgtggctgggagtgccccacaacccctgcctctaggaaccagcccttatgggagcacatgggctggggtgagggcaccgtggcagcctttggggccactcaagtcctccatggaaccgagactttatcaaggggagttagcgtccccttcccagtgctcatatccaatcattaaaatagactttaaaaaaatataaaatccgcctgagaacgatgggaatcagggacagtggtcagcccctaccctgctgagcattcaataccacctatgtgcacctggacataatgtgaaacctacacgggagagggacatgaatgtggtggggaagccccaacagagtggggaaatttcagttgtgccaatttgaagatggtgatctggcatagatcagccacaagtgcgctccttttaaacgtggattattatgtattttaaccatctttctccccattttcccctcttcttcattccgtattgtacctattggttagggagtgattggaattaatctacagatactgacagttcttttcccttgagtcaatactgtaagcaaagcaatgcattcgttcgcatttttttctggtagcaataaagataaaaaaattagtgtaaatatagaaagaggccgtaaatggaggtattttaatcaattacccaagtagggggaagaagattggaaaaacattaaggtcaagaaatgaaccatcctttaaggctgattaaaacacctctctgcatgtttttaaaacctgaaggaaattttatttttcttcccactgaggtgtgatccaccctcttggtggggcctggagagcttctttaaacaatccacgtttaaaagtgccttgcgctagaatttctgacaccccgaggggcagacagtgttgggccaattgggtgggtgtttggggctgagagatcagggttcctcactggaacatctttctcaatcaagtgggcaaacctgatctacagcccggcccaggtgtcccggattcccactcattctcaggcctgccggggagagcacactctcgatttctgcccgttgttgtcctggactcgaagggacagggaggggctggtcacttcctccgtgcctgggcctggttactctgtcccttctgatgctgctgcttaacctgggccaggatgtctcggatcttccgttgagccatctgactggcatagaaatgtccgatgattttcacgatgacctggtcgttctcatcaggggtctggtctcttggtactaccacctcagctgccgtcaaattctgcaactcgttcaccgtttttccacctttgccaatgacccggccagctgctgatgctggcacacgtatgtgggtctccagcttcacttcctccttgggaccaaagaagttctcctccttgagtttgccatagattcttccctgagccttgaattgggcctctggcggtccagtgatgataaccatacgaactttggagtcaggtgtttcgggtggtgcaatcttgatggaggcgctggcaaaccgggagagctgtttgatgtgctgccccttcttgccgatgatggcgcccactgcctgggcggggataaacacctgcaccatctcctgctcgggagcctgcataaaggagctatagggagcagccccagtaacgctgctgggaggcggcgggactgcgctggatgaagctgggaaaagacctacagcagccaggttcaggccagggatcaggtgagactgcaggctcatggcagccacatcattctcataggcctcccgaactttcttcattatttcctgctcggccctgcaacaattctcgatggcccccttcacagtgatggtcctctcagggttgtaaagggtaaggtcttgcaacgaggagatggtgatttttgtctcggtatcttgctctaccttcttcaggttccgtccttccttgccaatgagacgccctacaaagttattatgggccaggatcttcaggggaacctcgtcagcctgcctggtctgctcccggttggaataggtgacattcaccactgccgtctcactctcggtgttcacttgctcacagttctctactgtaccatactgagccagcaggctgtccagtacttcccatcggagctggggtggaatatttcggatttgaattttccggctcctttgttttttgggcaccgaatgttcaatctctaagcgttttccttgtaattctactttcccggagaaagtttcgatggccttcatcgcccagtgctcgtccgggcagtccacgaaggcgtagccggatttgaccaagaactggccgctgtaggagatcttgtgctccgcaaacactttctccaagtccgcgggggtcacgctctcgttgaggttgccgatgtaaagcttgttcatggtggcggtctcggggcaggacgcggtcccgggcaaggccgaacgagcgggcgcgggcggcgagcctcctaggccaagaggcggagaggccggcggcaggagccgcaaactttctttgcaccccaccccagaagttgtcccgagcccagggcggggaaggcggcctgagggcgcgcagaggtcgcgggagagttcggggagagcccaggagaagtgcccgcggcgcgcagggagacggacgacacggcgcagcttcttcccttcggtccgaaacccctccgagagggctggtgtgtcacgtttctccgcggccgccctggcgccgcctctaaataaaatcgacttgaaaaaaaatggagcg

SEQ ID NO: 17664 - RNA, 3325 nt, Homo sapiens
  source 1..3325: mol_type = other RNA
tcatagccctgtacaatgctgctggtattctgaattgttttttagacacacctttcatcatgctgataatgattcatggagacagaagccgtcagttaaaaattcctctcagatacaaacagaagcaagtactctccaatttactgaatttgccagatgatggactttagctttatcgggagctcagggttgggttccaagtcccaccaccaaggtaacagtgccgtggctgggagtgccccacaacccctgcctctaggaaccagcccttatgggagcacatgggctggggtgagggcaccgtggcagcctttggggccactcaagtcctccatggaaccgagactttatcaaggggagttagcgtccccttcccagtgctcatatccaatcattaaaatagactttaaaaaaatataaaatccgcctgagaacgatgggaatcagggacagtggtcagcccctaccctgctgagcattcaataccacctatgtgcacctggacataatgtgaaacctacacgggagagggacatgaatgtggtggggaagccccaacagagtggggaaatttcagttgtgccaatttgaagatggtgatctggcatagatcagccacaagtgcgctccttttaaacgtggattattatgtattttaaccatctttctccccattttcccctcttcttcattccgtattgtacctattggttagggagtgattggaattaatctacagatactgacagttcttttcccttgagtcaatactgtaagcaaagcaatgcattcgttcgcatttttttctggtagcaataaagataaaaaaattagtgtaaatatagaaagaggccgtaaatggaggtattttaatcaattacccaagtagggggaagaagattggaaaaacattaaggtcaagaaatgaaccatcctttaaggctgattaaaacacctctctgcatgtttttaaaacctgaaggaaattttatttttcttcccactgaggtgtgatccaccctcttggtggggcctggagagcttctttaaacaatccacgtttaaaagtgccttgcgctagaatttctgacaccccgaggggcagacagtgttgggccaattgggtgggtgtttggggctgagagatcagggttcctcactggaacatctttctcaatcaagtgggcaaacctgatctacagcccggcccaggtgtcccggattcccactcattctcaggcctgccggggagagcacactctcgatttctgcccgttgttgtcctggactcgaagggacagggaggggctggtcacttcctccgtgcctgggcctggttactctgtcccttctgatgctgctgcttaacctgggccaggatgtctcggatcttccgttgagccatctgactggcatagaaatgtccgatgattttcacgatgacctggtcgttctcatcaggggtctggtctcttggtactaccacctcagctgccgtcaaattctgcaactcgttcaccgtttttccacctttgccaatgacccggccagctgctgatgctggcacacgtatgtgggtctccagcttcacttcctccttgggaccaaagaagttctcctccttgagtttgccatagattcttccctgagccttgaattgggcctctggcggtccagtgatgataaccatacgaactttggagtcaggtgtttcgggtggtgcaatcttgatggaggcgctggcaaaccgggagagctgtttgatgtgctgccccttcttgccgatgatggcgcccactgcctgggcggggataaacacctgcaccatctcctgctcgggagcctgcataaaggagctatagggagcagccccagtaacgctgctgggaggcggcgggactgcgctggatgaagctgggaaaagacctacagcagccaggttcaggccagggatcaggtgagagctcatggcagccacatcattctcataggcctcccgaactttcttcattatttcctgctcggccctgcaacaattctcgatggcccccttcacagtgatggtcctctcagggttgtaaagggtaaggtcttgcaacgaggagatggtgatttttgtctcggtatcttgctctaccttcttcaggttccgtccttccttgccaatgagacgccctacaaagttattatgggccaggatcttcaggggaacctcgtcagccgttttggtgtccttagcctctttatgcataatctccaagatcatcttacaagcggaggagcagccctcaggggtggagtgcacactgatggctttttcagctgcacctgcgttctccttcctatgcacgtctatcttggactgggtctgttttgtgatgttgcggatggtggccccctccttgccaataatggcacccacatactgggtgggcaccaggagccgaagggggatgtccacttgctgctgcttggctggggcccccgctgccacaggtgagccctggcggggctgaccccgagagccaaagccccctcggcgcccattctcaggtccctgtgctatctgctcatcggggatgtaggagaccttcagggcatggttctccaactggtggccattcagcttcatgatggcttgcctggtctgctcccggttggaataggtgacattcaccactgccgtctcactctcggtgttcacttgctcacagttctctactgtaccatactgagccagcaggctgtccagtacttcccatcggagctggggtggaatatttcggatttgaattttccggctcctttgttttttgggcaccgaatgttcaatctctaagcgttttccttgtaattctactttcccggagaaagtttcgatggccttcatcgcccagtgctcgtccgggcagtccacgaaggcgtagccggatttgaccaagaactggccgctgtaggagatcttgtgctccgcaaacactttctccaagtccgcgggggtcacgctctcgttgaggttgccgatgtaaagcttgttcatggtggcggtctcggggcaggacgcggtcccgggcaaggccgaacgagcgggcgcgggcggcgagcctcctaggccaagaggcggagaggccggcggcaggagccgcaaactttctttgcaccccaccccagaagttgtcccgagcccagggcggggaaggcggcctgagggcgcgcagaggtcgcgggagagttcggggagagcccaggagaagtgcccgcggcgcgcagggagacggacgacacggcgcagcttcttcccttcggtccgaaacccctccgagag

SEQ ID NO: 17665 - RNA, 72 nt, Homo sapiens
  source 1..72: mol_type = other RNA
tcatagccctgtacaatgctgcttgaactccatgccacaaggcaacactgtaaagaagctgaaagcagagag

SEQ ID NO: 17666 - RNA, 70 nt, Homo sapiens
  source 1..70: mol_type = other RNA
tcatagccctgtacaatgctgcttgacctgaatgctacaaggcagcactgtaaagaagctgaaagcacaa

SEQ ID NO: 17667 - RNA, 70 nt, Homo sapiens
  source 1..70: mol_type = other RNA
tcatagccctgtacaatgctgcttgatccatatgcaacaaggcagcactgtaaagaagccgagggcagta

SEQ ID NO: 17668 - RNA, 5434 nt, Homo sapiens
  source 1..5434: mol_type = other RNA
tcatattgcttctttctaatgccaagaaagaagagtataagaacttcctcccagaagcctagacattttaatacattttctatttcaacttacaatgaaactttaatcctgaatcttgatttatctaaatcaaaaatctcacattacgaacacaaggaatgccatatgtaaggccacatcttaataaatttataatttttggttgaatatttattgaaaaaatcagtctaaggcttctaagagtcaagttgcttaaaaaaataaatacaccagtgtttaaactgaagttaaggttaaaaaaacgcatacacacacacacacacacacacacacactgtaagaacagaaaaatagaatgctttgctacaaaaatcccacttaatatattttagcacaaaaatgtctaatatacactggataagcgtgcatttacgtacatacaactaggggaaacatttacagagggctacgggatgcaaatgaacttaatgagtaataaaaaccagttgttatctgtaaaacagagaatctcaatactgtattctcagtcaagaattagaacataaacttcctcttaagctgaagcttaaaacacaaaattggagccattttagaaaatacagaaaatgcaatgatcattcaggtatgaaaaccaaaatgtcgagagcactccaacagaaaagtcttgtaatgcatctcattgtataaaacagtatgtatttagattggcacagttaaatacataagggaaagagaaagtctttgccctttccacaattttccttcactataaaatattatacaacattcattaaaacctccatgtttattttaataactgacctgaaactagtaaaaaataaagcaatattctccacaggagaattaaatgaaaatagtatcttaagctacaagttatctgtgtattccaaattgtcattaactgcttaagaacattctaggtaaaaggaccattaaatgggctaaactatgatcaaaagccactgcaacttactccaaaccttatgaaaagtgacaaaaaaaaaaaacacacatctgcaaatttacactggaatatgctttccacaacatagttcctttaaccaaaagcagcactttcaatccaaagtgttgcctcagaagcagtaccattcaggtactgtatcactcatctgtttaactttactactggctgaaaggaatgtgactgtatagcactaataaatgctatgttttaaaattcaactcgtttgttttcacatccactacagttattaactaaggaaaaaatgaaaaggtctctgagacactgtttttggtgtctatgcaaggatttatctctttggattgtttttacacattaaaaaaaggaagagttttcaaataacattaacccataaacaactgaagggggtatgaagaacaaaacaaggcctgcaattttcacctttactgctatacattcacgtgttatcaggtagagaaggactttgcaaaattacttggtcaaaccaagaagttatttccttctgacaacacttaaaataacggattagcagcaaacaaatctagtacactcacactgtctgtaacgaaagtcatgtaatgagatcagccaagcaaggagaagagtgatatagaaggagcaattaaaaggttccattgataaaatatgaaaaggtaaataaaggatttaattagtataaaatttccagtttcatttcaagtgcagttagatttttgtgattccatttttaaactgttcaaagaaaattttattttcatggacattttacttaccttttaaccctttactattaactaatttctcttgtaatatttatatgtccatacttcttcgcattagggcattgtagtcaaaatattaaaaagccaagaaatgacacaacaatatacagaaaacaggaaaattttgatacaactctaaaataatgttaaaaaagcaaccgcattttcaacaaaatgctttaaaaaatcatttctgaaagtgaacagttctgataaacatcaacgatcccatgcacagatacttcaaacacaaaatattttaaaataaaactggcagtgatatgggtaattcaaaacagctaattttgtcagaagtggtttgatagcagacaagatgaaagtgaagaacagcagtggaaatttctggagggtttctacagttgcacataacacagtatctagggtattttaacactttaagcattgtcctagaatttgggtactctttaacaaccaatgtgtattaacagaagatctctcaaagataatcagatcttaaaaacatattaacgtgctcaagaattttaagtcaaatttctgaagtagtgatttcaaattacattcccataaaaacacctaatcaagttgacaccctgcctctgccaattttgcaatcaagaacacatgctagtcaggtgcttttaaagtgggcctatatgtaaggcaggtttgaaaaaaatctttgattaagtaactatagcatgaatcaatacggtgcatgaatatacatagtattccttaaactgtgcagacacggtttatctgtaatttcccattacaaatactggggaatacaaccgaatgttaatgaacatcacatccttcaaaaatttataccaattggaaaatataaggctctctttactcacatttacctgctgcagggctgtatttacactgactatggcttaagaaataaaccataagatcaataaaaacagcaagtaattgcagcatcaaatcggaattgtcaaaatttcttcaatgttagcggttcacaattaagtgtttcggtacatctgtgttgtaattaacctgcattacacatcaaatatgtacgggtttttacttatgtgttaaaacctctgtttttttgaccccttacacattgactagattgctatgtctgtcaaatctctatttttacaagtttacataccattcagcaaagtcacaagctaactaggtaaaaacagctagaaaagcagaatatagaaatattaaatatccatgtaatcacctattctaatatcaaaatcaagggcaaaagacacttaattactatgtttaattcactgaacgcaagattagattgaggcatatccaaaaacgctattgcaatgctttaaaggacagtaaaaatgttgtcatagtaacattatctttagatattgctgaacacaagactttccctgaggtgtaaacatcaaataacttgaacagctttacacatcagccccattaaacagtttattacaacactacatctattgtaatcaaagtgatgctgtttacagacattatcatataaacatttttaacaagaacaaactactacaaaaacaagcatttacttgactttttttccaattgcttgcacatcataatggccaaatgtatataaccagtaataaagttgcaaaagctataactttttaaatcacacaggtttccttcaaataaaacagttaagcaacataaaaaataaaagtagagctactggttaccatttatgcagatttgctttattcagatctattcctgttcattttatccatgaatccttacaggttcagttcaatcacaagaagcaaactgctggacaagcgtcatttttcccccatgaagactgttttgtcttggaaggtgatcctcttccttcagcttctaacgatgacgatattcgcgctctcggtcacgctctcggtcacggtctcggtcacgatcccggtgcctctctcgttctctgcttctctctctgtaataatcgtcatgacggtctctactacgggatttatgacgtcgactcttttctcgtgatctactatggtccctctctcttgatcgttcacgtcttcttgatccagaaccataagacttggactcaattccatgaaggcaatcttgcaaagaactaataagaactttgcaacgatcatcagcagatactttggattgtttaattaaagaaattgcagttaccagtgtctcaatagcactcccataatcaccagcactggcatcagacacagctctcgaaatagcactgcttgagattgccctatttctattcatgatttcttcaaattcagcttcactcaatggcgttcttgcagtatccatttcccttccaggggggccatagtcacccctatcatatggtggaggtcgcccatatggatctgttggtggtggacctcggctatctgatgtaggcatgccactgttagttggtggaggaaagaaagctgggttcacatgcggagctggcggtggggcacctggaggtggtccaggaagatgcggaggaggagctagtgtaaggggtggcccaagtggaccgggtggacgaggtggaaaggggcctggaggtggaggtggtccctgttgtggaggtggtgggccaggaggggggccgtagcctggaactggaggtggagggccaggaggaagtggacccaatggaggctgcccaaaaggttgtccaggaaaaagaactggtggtggagggcgatctcctcgattaggaggcccagctagaggaggaggcagaacctgaccaggaggtggaggacctggtggaccaggtgggcctggaggacctaagggtggacgtggtggagtctgtccagctggaaaaggtgggggtggccctcctggtcctgctggcccaggaaatctgtccccaccaggaacagcccctggaaaacggccccgtcctctaccaccttgtggaaatgctgcacgggaactgcctcctggaggaccagctttaccttccccagacatttgtcctgattgtgtagttttcctggactgcatttcaaattgactcaggaactgtttattgcatggagttacaacaggattctgaccatgaagttctcttttaggtaacagatccattaacttttttgaagatgcttcagatccaacaccaacaagggcaaacccctttgactggccatttgcccgattttcaaaaaattttatctccaaaatatcatttactcccaaagaatgaactgcttcagttaagtcttcatctgttgtccaccatgttagatttccaatatataatgcaattctctttccagtatatgtatagacaacatttggtgctgctcctttacccacatcatcaccaacagttggtgggagagtatccatgtaatctcggtcttctggggcatctccattatttgcagatggagatatgacatcgtcatacaaatctatctgatcatgcccaccatattcagcttcctggttgaactcttcgccgacatccgcgtaaatgtctatgtggtccacgccgtccgccatcttccttcagcctcggccgccgccgccgccgccgcctcctgcaggtctgcccgccgcggcagcagcagcggatctagcg

SEQ ID NO: 17669 - RNA, 5545 nt, Homo sapiens
  source 1..5545: mol_type = other RNA
tcatattgcttctttctaatgccaagaaagaagagtataagaacttcctcccagaagcctagacattttaatacattttctatttcaacttacaatgaaactttaatcctgaatcttgatttatctaaatcaaaaatctcacattacgaacacaaggaatgccatatgtaaggccacatcttaataaatttataatttttggttgaatatttattgaaaaaatcagtctaaggcttctaagagtcaagttgcttaaaaaaataaatacaccagtgtttaaactgaagttaaggttaaaaaaacgcatacacacacacacacacacacacacacactgtaagaacagaaaaatagaatgctttgctacaaaaatcccacttaatatattttagcacaaaaatgtctaatatacactggataagcgtgcatttacgtacatacaactaggggaaacatttacagagggctacgggatgcaaatgaacttaatgagtaataaaaaccagttgttatctgtaaaacagagaatctcaatactgtattctcagtcaagaattagaacataaacttcctcttaagctgaagcttaaaacacaaaattggagccattttagaaaatacagaaaatgcaatgatcattcaggtatgaaaaccaaaatgtcgagagcactccaacagaaaagtcttgtaatgcatctcattgtataaaacagtatgtatttagattggcacagttaaatacataagggaaagagaaagtctttgccctttccacaattttccttcactataaaatattatacaacattcattaaaacctccatgtttattttaataactgacctgaaactagtaaaaaataaagcaatattctccacaggagaattaaatgaaaatagtatcttaagctacaagttatctgtgtattccaaattgtcattaactgcttaagaacattctaggtaaaaggaccattaaatgggctaaactatgatcaaaagccactgcaacttactccaaaccttatgaaaagtgacaaaaaaaaaaaacacacatctgcaaatttacactggaatatgctttccacaacatagttcctttaaccaaaagcagcactttcaatccaaagtgttgcctcagaagcagtaccattcaggtactgtatcactcatctgtttaactttactactggctgaaaggaatgtgactgtatagcactaataaatgctatgttttaaaattcaactcgtttgttttcacatccactacagttattaactaaggaaaaaatgaaaaggtctctgagacactgtttttggtgtctatgcaaggatttatctctttggattgtttttacacattaaaaaaaggaagagttttcaaataacattaacccataaacaactgaagggggtatgaagaacaaaacaaggcctgcaattttcacctttactgctatacattcacgtgttatcaggtagagaaggactttgcaaaattacttggtcaaaccaagaagttatttccttctgacaacacttaaaataacggattagcagcaaacaaatctagtacactcacactgtctgtaacgaaagtcatgtaatgagatcagccaagcaaggagaagagtgatatagaaggagcaattaaaaggttccattgataaaatatgaaaaggtaaataaaggatttaattagtataaaatttccagtttcatttcaagtgcagttagatttttgtgattccatttttaaactgttcaaagaaaattttattttcatggacattttacttaccttttaaccctttactattaactaatttctcttgtaatatttatatgtccatacttcttcgcattagggcattgtagtcaaaatattaaaaagccaagaaatgacacaacaatatacagaaaacaggaaaattttgatacaactctaaaataatgttaaaaaagcaaccgcattttcaacaaaatgctttaaaaaatcatttctgaaagtgaacagttctgataaacatcaacgatcccatgcacagatacttcaaacacaaaatattttaaaataaaactggcagtgatatgggtaattcaaaacagctaattttgtcagaagtggtttgatagcagacaagatgaaagtgaagaacagcagtggaaatttctggagggtttctacagttgcacataacacagtatctagggtattttaacactttaagcattgtcctagaatttgggtactctttaacaaccaatgtgtattaacagaagatctctcaaagataatcagatcttaaaaacatattaacgtgctcaagaattttaagtcaaatttctgaagtagtgatttcaaattacattcccataaaaacacctaatcaagttgacaccctgcctctgccaattttgcaatcaagaacacatgctagtcaggtgcttttaaagtgggcctatatgtaaggcaggtttgaaaaaaatctttgattaagtaactatagcatgaatcaatacggtgcatgaatatacatagtattccttaaactgtgcagacacggtttatctgtaatttcccattacaaatactggggaatacaaccgaatgttaatgaacatcacatccttcaaaaatttataccaattggaaaatataaggctctctttactcacatttacctgctgcagggctgtatttacactgactatggcttaagaaataaaccataagatcaataaaaacagcaagtaattgcagcatcaaatcggaattgtcaaaatttcttcaatgttagcggttcacaattaagtgtttcggtacatctgtgttgtaattaacctgcattacacatcaaatatgtacgggtttttacttatgtgttaaaacctctgtttttttgaccccttacacattgactagattgctatgtctgtcaaatctctatttttacaagtttacataccattcagcaaagtcacaagctaactaggtaaaaacagctagaaaagcagaatatagaaatattaaatatccatgtaatcacctattctaatatcaaaatcaagggcaaaagacacttaattactatgtttaattcactgaacgcaagattagattgaggcatatccaaaaacgctattgcaatgctttaaaggacagtaaaaatgttgtcatagtaacattatctttagatattgctgaacacaagactttccctgaggtgtaaacatcaaataacttgaacagctttacacatcagccccattaaacagtttattacaacactacatctattgtaatcaaagtgatgctgtttacagacattatcatataaacatttttaacaagaacaaactactacaaaaacaagcatttacttgactttttttccaattgcttgcacatcataatggccaaatgtatataaccagtaataaagttgcaaaagctataactttttaaatcacacaggtttccttcaaataaaacagttaagcaacataaaaaataaaagtagagctactggttaccatttatgcagatttgctttattcagatctattcctgttcattttatccatgaatccttacaggttcagttcaatcacaagaagcaaactgctggacaagcgtcatttttcccccatgaagactgttttgtcttggaaggtgatcctcttccttcagcttctaacgatgacgatattcgcgctctcggtcacgctctcggtcacggtctcggtcacgatcccggtgcctctctcgttctctgcttctctctctgtaataatcgtcatgacggtctctactacgggatttatgacgtcgactcttttctcgtgatctactatggtccctctctcttgatcgttcacgtcttcttgatccagaaccataagacttggactcaattccatgaaggcaatcttgcaaagaactaataagaactttgcaacgatcatcagcagatactttggattgtttaattaaagaaattgcagttaccagtgtctcaatagcactcccataatcaccagcactggcatcagacacagctctcgaaatagcactgcttgagattgccctatttctattcatgatttcttcaaattcagcttcactcaatggcgttcttgcagtatccatttcccttccaggggggccatagtcacccctatcatatggtggaggtcgcccatatggatctgttggtggtggacctcggctatctgatgtaggcatgccactgttagttggtggaggaaagaaagctgggttcacatgcggagctggcggtggggcacctggaggtggtccaggaagatgcggaggaggagctagtgtaaggggtggcccaagtggaccgggtggacgaggtggaaaggggcctggaggtggaggtggtccctgttgtggaggtggtgggccaggaggggggccgtagcctggaactggaggtggagggccaggaggaagtggacccaatggaggctgcccaaaaggttgtccaggaaaaagaactggtggtggagggcgatctcctcgattaggaggcccagctagaggaggaggcagaacctgaccaggaggtggaggacctggtggaccaggtgggcctggaggacctaagggtggacgtggtggagtctgtccagcttttaggccaaaaatgggtatttcctctatgctgtgccccatatgccatggaatcctagtttccaggaacaaaggccgagttcctttaacaagatgcttgatcaaatttcctggaaaaggtgggggtggccctcctggtcctgctggcccaggaaatctgtccccaccaggaacagcccctggaaaacggccccgtcctctaccaccttgtggaaatgctgcacgggaactgcctcctggaggaccagctttaccttccccagacatttgtcctgattgtgtagttttcctggactgcatttcaaattgactcaggaactgtttattgcatggagttacaacaggattctgaccatgaagttctcttttaggtaacagatccattaacttttttgaagatgcttcagatccaacaccaacaagggcaaacccctttgactggccatttgcccgattttcaaaaaattttatctccaaaatatcatttactcccaaagaatgaactgcttcagttaagtcttcatctgttgtccaccatgttagatttccaatatataatgcaattctctttccagtatatgtatagacaacatttggtgctgctcctttacccacatcatcaccaacagttggtgggagagtatccatgtaatctcggtcttctggggcatctccattatttgcagatggagatatgacatcgtcatacaaatctatctgatcatgcccaccatattcagcttcctggttgaactcttcgccgacatccgcgtaaatgtctatgtggtccacgccgtccgccatcttccttcagcctcggccgccgccgccgccgccgcctcctgcaggtctgcccgccgcggcagcagcagcggatctagcg

SEQ ID NO: 17670 - RNA, 5430 nt, Homo sapiens
  source 1..5430: mol_type = other RNA
tcatattgcttctttctaatgccaagaaagaagagtataagaacttcctcccagaagcctagacattttaatacattttctatttcaacttacaatgaaactttaatcctgaatcttgatttatctaaatcaaaaatctcacattacgaacacaaggaatgccatatgtaaggccacatcttaataaatttataatttttggttgaatatttattgaaaaaatcagtctaaggcttctaagagtcaagttgcttaaaaaaataaatacaccagtgtttaaactgaagttaaggttaaaaaaacgcatacacacacacacacacacacacacacactgtaagaacagaaaaatagaatgctttgctacaaaaatcccacttaatatattttagcacaaaaatgtctaatatacactggataagcgtgcatttacgtacatacaactaggggaaacatttacagagggctacgggatgcaaatgaacttaatgagtaataaaaaccagttgttatctgtaaaacagagaatctcaatactgtattctcagtcaagaattagaacataaacttcctcttaagctgaagcttaaaacacaaaattggagccattttagaaaatacagaaaatgcaatgatcattcaggtatgaaaaccaaaatgtcgagagcactccaacagaaaagtcttgtaatgcatctcattgtataaaacagtatgtatttagattggcacagttaaatacataagggaaagagaaagtctttgccctttccacaattttccttcactataaaatattatacaacattcattaaaacctccatgtttattttaataactgacctgaaactagtaaaaaataaagcaatattctccacaggagaattaaatgaaaatagtatcttaagctacaagttatctgtgtattccaaattgtcattaactgcttaagaacattctaggtaaaaggaccattaaatgggctaaactatgatcaaaagccactgcaacttactccaaaccttatgaaaagtgacaaaaaaaaaaaacacacatctgcaaatttacactggaatatgctttccacaacatagttcctttaaccaaaagcagcactttcaatccaaagtgttgcctcagaagcagtaccattcaggtactgtatcactcatctgtttaactttactactggctgaaaggaatgtgactgtatagcactaataaatgctatgttttaaaattcaactcgtttgttttcacatccactacagttattaactaaggaaaaaatgaaaaggtctctgagacactgtttttggtgtctatgcaaggatttatctctttggattgtttttacacattaaaaaaaggaagagttttcaaataacattaacccataaacaactgaagggggtatgaagaacaaaacaaggcctgcaattttcacctttactgctatacattcacgtgttatcaggtagagaaggactttgcaaaattacttggtcaaaccaagaagttatttccttctgacaacacttaaaataacggattagcagcaaacaaatctagtacactcacactgtctgtaacgaaagtcatgtaatgagatcagccaagcaaggagaagagtgatatagaaggagcaattaaaaggttccattgataaaatatgaaaaggtaaataaaggatttaattagtataaaatttccagtttcatttcaagtgcagttagatttttgtgattccatttttaaactgttcaaagaaaattttattttcatggacattttacttaccttttaaccctttactattaactaatttctcttgtaatatttatatgtccatacttcttcgcattagggcattgtagtcaaaatattaaaaagccaagaaatgacacaacaatatacagaaaacaggaaaattttgatacaactctaaaataatgttaaaaaagcaaccgcattttcaacaaaatgctttaaaaaatcatttctgaaagtgaacagttctgataaacatcaacgatcccatgcacagatacttcaaacacaaaatattttaaaataaaactggcagtgatatgggtaattcaaaacagctaattttgtcagaagtggtttgatagcagacaagatgaaagtgaagaacagcagtggaaatttctggagggtttctacagttgcacataacacagtatctagggtattttaacactttaagcattgtcctagaatttgggtactctttaacaaccaatgtgtattaacagaagatctctcaaagataatcagatcttaaaaacatattaacgtgctcaagaattttaagtcaaatttctgaagtagtgatttcaaattacattcccataaaaacacctaatcaagttgacaccctgcctctgccaattttgcaatcaagaacacatgctagtcaggtgcttttaaagtgggcctatatgtaaggcaggtttgaaaaaaatctttgattaagtaactatagcatgaatcaatacggtgcatgaatatacatagtattccttaaactgtgcagacacggtttatctgtaatttcccattacaaatactggggaatacaaccgaatgttaatgaacatcacatccttcaaaaatttataccaattggaaaatataaggctctctttactcacatttacctgctgcagggctgtatttacactgactatggcttaagaaataaaccataagatcaataaaaacagcaagtaattgcagcatcaaatcggaattgtcaaaatttcttcaatgttagcggttcacaattaagtgtttcggtacatctgtgttgtaattaacctgcattacacatcaaatatgtacgggtttttacttatgtgttaaaacctctgtttttttgaccccttacacattgactagattgctatgtctgtcaaatctctatttttacaagtttacataccattcagcaaagtcacaagctaactaggtaaaaacagctagaaaagcagaatatagaaatattaaatatccatgtaatcacctattctaatatcaaaatcaagggcaaaagacacttaattactatgtttaattcactgaacgcaagattagattgaggcatatccaaaaacgctattgcaatgctttaaaggacagtaaaaatgttgtcatagtaacattatctttagatattgctgaacacaagactttccctgaggtgtaaacatcaaataacttgaacagctttacacatcagccccattaaacagtttattacaacactacatctattgtaatcaaagtgatgctgtttacagacattatcatataaacatttttaacaagaacaaactactacaaaaacaagcatttacttgactttttttccaattgcttgcacatcataatggccaaatgtatataaccagtaataaagttgcaaaagctataactttttaaatcacacaggtttccttcaaataaaacagttaagcaacataaaaaataaaagtagagctactggttaccatttatgcagatttgctttattcagatctattcctgttcattttatccatgaatccttacaggttcagttcaatcacaagaagcaaactgctggacaagcgtcatttttcccccatgaagactgttttgtcttggaaggtgatcctcttccttcagcttctaacgatgacgatattcgcgctctcggtcacgctctcggtcacggtctcggtcacgatcccggtgcctctctcgttctctgcttctctctctgtaataatcgtcatgacggtctctactacgggatttatgacgtcgactcttttctcgtgatctactatggtccctctctcttgatcgttcacgtcttgatccagaaccataagacttggactcaattccatgaaggcaatcttgcaaagaactaataagaactttgcaacgatcatcagcagatactttggattgtttaattaaagaaattgcagttaccagtgtctcaatagcactcccataatcaccagcactggcatcagacacagctctcgaaatagcactgcttgagattgccctatttctattcatgatttcttcaaattcagcttcactcaatggcgttcttgcagtatccatttcccttccaggggggccatagtcacccctatcatatggtggaggtcgcccatatggatctgttggtggtggacctcggctatctgatgtaggcatgccactgttagttggtggaggaaagaaagctgggttcacatgcggagctggcggtggggcacctggaggtggtccaggaagatgcggaggaggagctagtgtaaggggtggcccaagtggaccgggtggacgaggtggaaaggggcctggaggtggaggtggtccctgttgtggaggtggtgggccaggaggggggccgtagcctggaactggaggtggagggccaggaggaagtggacccaatggaggctgcccaaaaggttgtccaggaaaaagaactggtggtggagggcgatctcctcgattaggaggcccagctagaggaggaggcagaacctgaccaggaggtggaggacctggtggaccaggtgggcctggaggacctaagggtggacgtggtggagtctgtccagctggaaaaggtgggggtggccctcctggtcctgctggcccaggaaatctgtccccaccaggaacagcccctggaaaacggccccgtcctctaccaccttgtggaaatgctgcacgggaactgcctcctggaggaccagctttaccttccccagacatttgtcctgattgtgtagttttcctggactgcatttcaaattgactcaggaactgtttattgcatggagttacaacaggattctgaccatgaagttctcttttaggtaacagatccattaacttttttgaagatgcttcagatccaacaccaacaagggcaaacccctttgactggccatttgcccgattttcaaaaaattttatctccaaaatatcatttactcccaaagaatgaactgcttcagttaagtcttcatctgttgtccaccatgttagatttccaatatataatgcaattctctttccagtatatgtatagacaacatttggtgctgctcctttacccacatcatcaccaacagttggtgggagagtatccatgtaatctcggtcttctggggcatctccattatttgcagatggagatatgacatcgtcatacaaatctatctgatcatgcccaccatattcagcttcctggttgaactcttcgccgacatccgcgtaaatgtctatgtggtccacgccgtccgccatcttccttcagcctcggccgccgccgccgccgccgcctcctgcaggtctgcccgccgcggcagcagcagcggatctagc

SEQ ID NO: 17671 - RNA, 5541 nt, Homo sapiens
  source 1..5541: mol_type = other RNA
tcatattgcttctttctaatgccaagaaagaagagtataagaacttcctcccagaagcctagacattttaatacattttctatttcaacttacaatgaaactttaatcctgaatcttgatttatctaaatcaaaaatctcacattacgaacacaaggaatgccatatgtaaggccacatcttaataaatttataatttttggttgaatatttattgaaaaaatcagtctaaggcttctaagagtcaagttgcttaaaaaaataaatacaccagtgtttaaactgaagttaaggttaaaaaaacgcatacacacacacacacacacacacacacactgtaagaacagaaaaatagaatgctttgctacaaaaatcccacttaatatattttagcacaaaaatgtctaatatacactggataagcgtgcatttacgtacatacaactaggggaaacatttacagagggctacgggatgcaaatgaacttaatgagtaataaaaaccagttgttatctgtaaaacagagaatctcaatactgtattctcagtcaagaattagaacataaacttcctcttaagctgaagcttaaaacacaaaattggagccattttagaaaatacagaaaatgcaatgatcattcaggtatgaaaaccaaaatgtcgagagcactccaacagaaaagtcttgtaatgcatctcattgtataaaacagtatgtatttagattggcacagttaaatacataagggaaagagaaagtctttgccctttccacaattttccttcactataaaatattatacaacattcattaaaacctccatgtttattttaataactgacctgaaactagtaaaaaataaagcaatattctccacaggagaattaaatgaaaatagtatcttaagctacaagttatctgtgtattccaaattgtcattaactgcttaagaacattctaggtaaaaggaccattaaatgggctaaactatgatcaaaagccactgcaacttactccaaaccttatgaaaagtgacaaaaaaaaaaaacacacatctgcaaatttacactggaatatgctttccacaacatagttcctttaaccaaaagcagcactttcaatccaaagtgttgcctcagaagcagtaccattcaggtactgtatcactcatctgtttaactttactactggctgaaaggaatgtgactgtatagcactaataaatgctatgttttaaaattcaactcgtttgttttcacatccactacagttattaactaaggaaaaaatgaaaaggtctctgagacactgtttttggtgtctatgcaaggatttatctctttggattgtttttacacattaaaaaaaggaagagttttcaaataacattaacccataaacaactgaagggggtatgaagaacaaaacaaggcctgcaattttcacctttactgctatacattcacgtgttatcaggtagagaaggactttgcaaaattacttggtcaaaccaagaagttatttccttctgacaacacttaaaataacggattagcagcaaacaaatctagtacactcacactgtctgtaacgaaagtcatgtaatgagatcagccaagcaaggagaagagtgatatagaaggagcaattaaaaggttccattgataaaatatgaaaaggtaaataaaggatttaattagtataaaatttccagtttcatttcaagtgcagttagatttttgtgattccatttttaaactgttcaaagaaaattttattttcatggacattttacttaccttttaaccctttactattaactaatttctcttgtaatatttatatgtccatacttcttcgcattagggcattgtagtcaaaatattaaaaagccaagaaatgacacaacaatatacagaaaacaggaaaattttgatacaactctaaaataatgttaaaaaagcaaccgcattttcaacaaaatgctttaaaaaatcatttctgaaagtgaacagttctgataaacatcaacgatcccatgcacagatacttcaaacacaaaatattttaaaataaaactggcagtgatatgggtaattcaaaacagctaattttgtcagaagtggtttgatagcagacaagatgaaagtgaagaacagcagtggaaatttctggagggtttctacagttgcacataacacagtatctagggtattttaacactttaagcattgtcctagaatttgggtactctttaacaaccaatgtgtattaacagaagatctctcaaagataatcagatcttaaaaacatattaacgtgctcaagaattttaagtcaaatttctgaagtagtgatttcaaattacattcccataaaaacacctaatcaagttgacaccctgcctctgccaattttgcaatcaagaacacatgctagtcaggtgcttttaaagtgggcctatatgtaaggcaggtttgaaaaaaatctttgattaagtaactatagcatgaatcaatacggtgcatgaatatacatagtattccttaaactgtgcagacacggtttatctgtaatttcccattacaaatactggggaatacaaccgaatgttaatgaacatcacatccttcaaaaatttataccaattggaaaatataaggctctctttactcacatttacctgctgcagggctgtatttacactgactatggcttaagaaataaaccataagatcaataaaaacagcaagtaattgcagcatcaaatcggaattgtcaaaatttcttcaatgttagcggttcacaattaagtgtttcggtacatctgtgttgtaattaacctgcattacacatcaaatatgtacgggtttttacttatgtgttaaaacctctgtttttttgaccccttacacattgactagattgctatgtctgtcaaatctctatttttacaagtttacataccattcagcaaagtcacaagctaactaggtaaaaacagctagaaaagcagaatatagaaatattaaatatccatgtaatcacctattctaatatcaaaatcaagggcaaaagacacttaattactatgtttaattcactgaacgcaagattagattgaggcatatccaaaaacgctattgcaatgctttaaaggacagtaaaaatgttgtcatagtaacattatctttagatattgctgaacacaagactttccctgaggtgtaaacatcaaataacttgaacagctttacacatcagccccattaaacagtttattacaacactacatctattgtaatcaaagtgatgctgtttacagacattatcatataaacatttttaacaagaacaaactactacaaaaacaagcatttacttgactttttttccaattgcttgcacatcataatggccaaatgtatataaccagtaataaagttgcaaaagctataactttttaaatcacacaggtttccttcaaataaaacagttaagcaacataaaaaataaaagtagagctactggttaccatttatgcagatttgctttattcagatctattcctgttcattttatccatgaatccttacaggttcagttcaatcacaagaagcaaactgctggacaagcgtcatttttcccccatgaagactgttttgtcttggaaggtgatcctcttccttcagcttctaacgatgacgatattcgcgctctcggtcacgctctcggtcacggtctcggtcacgatcccggtgcctctctcgttctctgcttctctctctgtaataatcgtcatgacggtctctactacgggatttatgacgtcgactcttttctcgtgatctactatggtccctctctcttgatcgttcacgtcttgatccagaaccataagacttggactcaattccatgaaggcaatcttgcaaagaactaataagaactttgcaacgatcatcagcagatactttggattgtttaattaaagaaattgcagttaccagtgtctcaatagcactcccataatcaccagcactggcatcagacacagctctcgaaatagcactgcttgagattgccctatttctattcatgatttcttcaaattcagcttcactcaatggcgttcttgcagtatccatttcccttccaggggggccatagtcacccctatcatatggtggaggtcgcccatatggatctgttggtggtggacctcggctatctgatgtaggcatgccactgttagttggtggaggaaagaaagctgggttcacatgcggagctggcggtggggcacctggaggtggtccaggaagatgcggaggaggagctagtgtaaggggtggcccaagtggaccgggtggacgaggtggaaaggggcctggaggtggaggtggtccctgttgtggaggtggtgggccaggaggggggccgtagcctggaactggaggtggagggccaggaggaagtggacccaatggaggctgcccaaaaggttgtccaggaaaaagaactggtggtggagggcgatctcctcgattaggaggcccagctagaggaggaggcagaacctgaccaggaggtggaggacctggtggaccaggtgggcctggaggacctaagggtggacgtggtggagtctgtccagcttttaggccaaaaatgggtatttcctctatgctgtgccccatatgccatggaatcctagtttccaggaacaaaggccgagttcctttaacaagatgcttgatcaaatttcctggaaaaggtgggggtggccctcctggtcctgctggcccaggaaatctgtccccaccaggaacagcccctggaaaacggccccgtcctctaccaccttgtggaaatgctgcacgggaactgcctcctggaggaccagctttaccttccccagacatttgtcctgattgtgtagttttcctggactgcatttcaaattgactcaggaactgtttattgcatggagttacaacaggattctgaccatgaagttctcttttaggtaacagatccattaacttttttgaagatgcttcagatccaacaccaacaagggcaaacccctttgactggccatttgcccgattttcaaaaaattttatctccaaaatatcatttactcccaaagaatgaactgcttcagttaagtcttcatctgttgtccaccatgttagatttccaatatataatgcaattctctttccagtatatgtatagacaacatttggtgctgctcctttacccacatcatcaccaacagttggtgggagagtatccatgtaatctcggtcttctggggcatctccattatttgcagatggagatatgacatcgtcatacaaatctatctgatcatgcccaccatattcagcttcctggttgaactcttcgccgacatccgcgtaaatgtctatgtggtccacgccgtccgccatcttccttcagcctcggccgccgccgccgccgccgcctcctgcaggtctgcccgccgcggcagcagcagcggatctagc

SEQ ID NO: 17672 - RNA, 1493 nt, Homo sapiens
  source 1..1493: mol_type = other RNA
tcatattgcttctttctgtttattttgttaacagctacttgaggttcagttactgaataatgagggacaccagaatctaaacttgtttttgaaccactgaattcagtacttctaccttggaattcagcgtgcttttctctttgaagccatgtttctttgacaattacttcaggtttgtgagtcgctgcctgaagagggacatcagaatccaaacttgtttcaaaaacactcttattttctaagtacatgtgctcttttgtgtgaaggcttatttctttaatgggatcttcagaacgtccagtcactgaatgaaaaatgatattataatccaaacttacttcagaatcaataggttcattttccttattttctaagtgtacctgctcttctttttgaggatttagctttttaacagctacttcgggagaattagtcactgaatgaagaggggcatgggaatccgaacttatttcagaaccactgggttcatcattcttcctttctaagtgaatgtactcttctttctgaattacttctttaacagctacttcagggtgatcatttcagctctcatcttccaggtcaatgtgccgttcttttccttcagcatccagatgagactgctcagtaactgacagaagaggcgggtcagaatcaaaagtcaactcagagctggagcaatcatagctcctaacttccatgtcaatatttaactctttaagatttacttcatccaaagcttcttgaggctcatcatgagctgaatgataaagagaagccggagaatcagaactcagagaagaacggctagactgaacactcttattctcaaggtcaacatccactttctgacgctctatttcggctacttgagactggtcagctaattgagcatcagcctgaaaacccatttcaggaccatgggattcacagttcatatccataaggtcagcattcttctccttcagaagatttatcttttcaacagccctctgggattcatctgcaactgtcccaagtgagacatcacaatcaagatgtgctttagcactactgggtttacgcttcttatgttttaggtggacttgtctacctttcaggtttcttcctttgacagtcagttggggatgatcaactactgactcaagagaaacatcacaatcaaaacttgtttcagaacaactcgatccatagttatcaaccaagctggtatgagccttcttccgaagttttgtttctgtgacagccactgggggtctgtcaaccactgactgcagtgggaaaacagaatcagcacttacttcagagctactggaaccatagttcttatcaaccaaaccaatgtgcacttccttaggaaggtttacttctgttacagattgttgggggtagtcactagtggactgaggtgaagcatcacaatcaaaattcgtttcagaactactagattcatagctttggtcaaccaggctaatatgccttgcattctgaag

SEQ ID NO: 17673 - RNA, 4635 nt, Homo sapiens
  source 1..4635: mol_type = other RNA
tcatattgcttctttctgtttattttgttaacagctacttgaggttcagttactgaataatgagggacaccagaatctaaacttgtttttgaaccactgaattcagtacttctaccttggaattcagcgtgcttttctctttgaagccatgtttctttgacaattacttcaggtttgtgagtcgctgcctgaagagggacatcagaatccaaacttgtttcaaaaacactcttattttctaagtacatgtgctcttttgtgtgaaggcttatttctttaatgggatcttcagaacgtccagtcactgaatgaaaaatgatattataatccaaacttacttcagaatcaataggttcattttccttattttctaagtgtacctgctcttctttttgaggatttagctttttaacagctacttcgggagaattagtcactgaatgaagaggggcatgggaatccgaacttatttcagaaccactgggttcatcattcttcctttctaagtgaatgtactcttctttctgaattacttctttaacagctacttcagggtgatcatttcctgaatgaagaggaatatcagaatcaaaagttatttcagagacacaagattcattacttttactttccagatcaacagtttcttcctcataaacagctacttcaggttggtcaattactgaataaagaggaatatcagaatcaaaagttatttcagaactatctgactcacagctctcatcttccaggtcaatgtgccgttcttttccttcagcatccagatgagactgctcagtaactgacagaagaggcgggtcagaatcaaaagtcaactcagagctggagcaatcatagctcctaacttccatgtcaatatttaactctttaagatttacttcatccaaagcttcttgaggctcatcatgagctgaatgataaagagaagccggagaatcagaactcagagaagaacggctagactgaacactcttattctcaaggtcaacatccactttctgacgctctatttcggctacttgagactggtcagctaattgagcatcagcctgaaaacccatttcaggaccatgggattcacagttcatatccataaggtcagcattcttctccttcagaagatttatcttttcaacagccctctgggattcatctgcaactgtcccaagtgagacatcacaatcaagatgtgctttagcactactgggtttacgcttcttatgttttaggtggacttgtctacctttcaggtttcttcctttgacagtcagttggggatgatcaactactgactcaagagaaacatcacaatcaaaacttgtttcagaacaactcgatccatagttatcaaccaagctggtatgagccttcttccgaagttttgtttctgtgacagccactgggggtctgtcaaccactgactgcagtgggaaaacagaatcagcacttacttcagagctactggaaccatagttcttatcaaccaaaccaatgtgcacttccttaggaaggtttacttctgttacagattgttgggggtagtcactagtggactgaggtgaagcatcacaatcaaaattcgtttcagaactactagattcatagctttggtcaaccaggctaatatgccttgcattctgaagacttatttctttaacaatcatttgggattggttggtaaccaagtgaagaatgtcatcacaatcagaacttattttagaaacataagatttattattcttatactgtacatcagtacgtacttccttggaaaggtttacttctttggcactcactttagattggtcagtcagtgaatgaaaagaggaactgcaatcaaaactcatttctgaacctctagactcatagttatcttcttggtcaatttgctcctccttccaaagacttaagtcttgtgcagtctcttggggctgatcagatgctgactgaagagagatacaatcaaacttcatttcagaactcactgagcacttctgttcccaaaaggctgtcttgttaaaaaccaaatgcttttcttcttgggtacaatccatgttagaaaagaattcctcatggttctttgcaatagtatcttcaaagattcctttattagaaggcatgtcagttttattcgggtttactgctaatttggaaggagatttaactcttaaggagcccttagtacccatgcgttcatggaatttcaagccagctgataaagttttaccctgagattttacatctttccacaaaaccaacttatctgaattcatgcgtaaagatttcctatttgattctttatgtttctgatacgaaaatgaagtagtttctacatgggatgatggcacaggatttctagaggccccatctggctgttcaagatatttctcaactttgtttgggtcacatttgctaactgaatccaaatgagctgctggtggtaaactagttgtattagctgtaactggtctatcgttagagctttcaggtaaacaactagcaggagcattacaaatcactggggggcgtaccaagttgcttctattatttgtagcctgaccaatatctactaggttacattttctcacactggccccaattttatgaacaaactccaagggctgctgctgtcccttctccagtttttgaataactgatggtcgaactgaaacctcctgcgtgccttcctgagatttatgaggtctggaatgtaactcttcaataggttctgaaacctcggatggtctctcttcggtagcatcctcatcctcaaccttatcctcatcctcttcctcttcttcagaaaaagcatcatccaaatgcaccacttcagacgatgacccagtattcacatgtgtctcatcttgtgttgaactgctctcttgacaatgatatgggtggtgctgcagtacatcctgtaagaaacgttccatcaaactactggtacatatttgacgtctactctgtctggtcaaactcctgtgctgagcactgaacaaatgctgttccaggttattatactgcacacggcaataactgcaatatccttgtcttttctgcatcttgaataaataactgaagtcagatggctactgtctttgaatactcaagctattacttcttattatgagaaattgattttctgacttctcacatttatgaggaaaattaatcaattaaaccagcctctggagcagaaaaggtcaggtatttcatcagctgtattagttctggcaagtatctccgcggaggctgcccggattccttccgggccgcggtggagaccgaggaccgagccgggcgctctcccttcttattccggttccgcggcggcgcccgaatcccagaccgtccgagcgccacggccccgctgcccgcggagccagaaataggcgacttcggcccctgcggtccggaggcgagaagcggcgcgggagcgcgtctctcaggacgcgggccccgagtcgcgactccactcacgcaggcatccaaggcaacgtggcgttgcaaccctgatggaggtttgacgtcagggaaggtgcgaaaaccagaccccttctgacgcaggagcggcgggaccgccccctgcccgcccacccactcactcactctcccacccgggcggaggagccccttcctcccctccagaagctcttaaagcggacacttcctccctggtcagggccccactccggagcttgggaaatctatcgcgttccaacaaaaatgactagactcataagcacagttgggacgcgaagtagagaccaaggttttagcgtttgagggtccaaataaaaactgcttgccaattcaaagcaacgtatgaatgtagaaaagaaaacggggctaagagagctagtcgtttccgtttccatgcctatttcatagtgaggtgcatctcacaaaagctgctgttcaatgagcgcttgctctgtgctaggcaccgtttaaggtttctatacattattgcatttcatttcagagtaactctgaatgaatcctattattgtccccctttgacaaattgagaaaactgaggcttaaggaagttaggtattcaaagatctatcctgcacattaaagggttacaaatattaacaaacaacattaggtcatgcaattatattcactgcgctaccccattacgaatatagttgtgagcaaaaacagtttaagtgtaacggagatcacaaacctaaatgaatcacactactgaatatgaaattataatctgcgataagaaggttctgaaacacctaaaccaattttactaaaatggagagaggccctgttgcaaagcttatgtctaatgtaaaaataatcttaaaatgagctactttgctctttggctgtagctgtaattgtcgttaccctttttagtaagcttgtgattttgtccctttaaagaacaacaacaaaaaaacttgcctattgcttttgcgtccattgtttttattctttctgtatttctcagctccttcttcccccactacatctttctctcactttaaagttgggctcctgcaactgttcgatttataacctcccttagatttaacataccaaaaagtacggatttcttttaaggcaagttttttccacatcccaact

SEQ ID NO: 17674 - RNA, 3341 nt, Homo sapiens
  source 1..3341: mol_type = other RNA
tcatattgcttctttctgtttattttgttaacagctacttgaggttcagttactgaataatgagggacaccagaatctaaacttgtttttgaaccactgaattcagtacttctaccttggaattcagcgtgcttttctctttgaagccatgtttctttgacaattacttcaggtttgtgagtcgctgcctgaagagggacatcagaatccaaacttgtttcaaaaacactcttattttctaagtacatgtgctcttttgtgtgaaggcttatttctttaatgggatcttcagaacgtccagtcactgaatgaaaaatgatattataatccaaacttacttcagaatcaataggttcattttccttattttctaagtgtacctgctcttctttttgaggatttagctttttaacagctacttcgggagaattagtcactgaatgaagaggggcatgggaatccgaacttatttcagaaccactgggttcatcattcttcctttctaagtgaatgtactcttctttctgaattacttctttaacagctacttcagggtgatcatttcctgaatgaagaggaatatcagaatcaaaagttatttcagagacacaagattcattacttttactttccagatcaacagtttcttcctcataaacagctacttcaggttggtcaattactgaataaagaggaatatcagaatcaaaagttatttcagaactatctgactcacagctctcatcttccaggtcaatgtgccgttcttttccttcagcatccagatgagactgctcagtaactgacagaagaggcgggtcagaatcaaaagtcaactcagagctggagcaatcatagctcctaacttccatgtcaatatttaactctttaagatttacttcatccaaagcttcttgaggctcatcatgagctgaatgataaagagaagccggagaatcagaactcagagaagaacggctagactgaacactcttattctcaaggtcaacatccactttctgacgctctatttcggctacttgagactggtcagctaattgagcatcagcctgaaaacccatttcaggaccatgggattcacagttcatatccataaggtcagcattcttctccttcagaagatttatcttttcaacagccctctgggattcatctgcaactgtcccaagtgagacatcacaatcaagatgtgctttagcactactgggtttacgcttcttatgttttaggtggacttgtctacctttcaggtttcttcctttgacagtcagttggggatgatcaactactgactcaagagaaacatcacaatcaaaacttgtttcagaacaactcgatccatagttatcaaccaagctggtatgagccttcttccgaagttttgtttctgtgacagccactgggggtctgtcaaccactgactgcagtgggaaaacagaatcagcacttacttcagagctactggaaccatagttcttatcaaccaaaccaatgtgcacttccttaggaaggtttacttctgttacagattgttgggggtagtcactagtggactgaggtgaagcatcacaatcaaaattcgtttcagaactactagattcatagctttggtcaaccaggctaatatgccttgcattctgaagacttatttctttaacaatcatttgggattggttggtaaccaagtgaagaatgtcatcacaatcagaacttattttagaaacataagatttattattcttatactgtacatcagtacgtacttccttggaaaggtttacttctttggcactcactttagattggtcagtcagtgaatgaaaagaggaactgcaatcaaaactcatttctgaacctctagactcatagttatcttcttggtcaatttgctcctccttccaaagacttaagtcttgtgcagtctcttggggctgatcagatgctgactgaagagagatacaatcaaacttcatttcagaactcactgagcacttctgttcccaaaaggctgtcttgttaaaaaccaaatgcttttcttcttgggtacaatccatgttagaaaagaattcctcatggttctttgcaatagtatcttcaaagattcctttattagaaggcatgtcagttttattcgggtttactgctaatttggaaggagatttaactcttaaggagcccttagtacccatgcgttcatggaatttcaagccagctgataaagttttaccctgagattttacatctttccacaaaaccaacttatctgaattcatgcgtaaagatttcctatttgattctttatgtttctgatacgaaaatgaagtagtttctacatgggatgatggcacaggatttctagaggccccatctggctgttcaagatatttctcaactttgtttgggtcacatttgctaactgaatccaaatgagctgctggtggtaaactagttgtattagctgtaactggtctatcgttagagctttcaggtaaacaactagcaggagcattacaaatcactggggggcgtaccaagttgcttctattatttgtagcctgaccaatatctactaggttacattttctcacactggccccaattttatgaacaaactccaagggctgctgctgtcccttctccagtttttgaataactgatggtcgaactgaaacctcctgcgtgccttcctgagatttatgaggtctggaatgtaactcttcaataggttctgaaacctcggatggtctctcttcggtagcatcctcatcctcaaccttatcctcatcctcttcctcttcttcagaaaaagcatcatccaaatgcaccacttcagacgatgacccagtattcacatgtgtctcatcttgtgttgaactgctctcttgacaatgatatgggtggtgctgcagtacatcctgtaagaaacgttccatcaaactactggtacatatttgacgtctactctgtctggtcaaactcctgtgctgagcactgaacaaatgctgttccaggttattatactgcacacggcaataactgcaatatccttgtcttttctgcatcttgaataaataactgaagtcagatggctactgtctttgaatactcaagctattacttcttattatgagaaattgattttctgacttctcacatttatgaggaaaattaatcaattaaaccagcctctggagcagaaaaggtcaggtatttcatcagctgtattagttctggcaagtatctgcgaggcggccgcgggagcccagcgagcggtcctggcgtccctcgggaagaaggcgccccgggcgcccggcgagcag

SEQ ID NO: 17675 - RNA, 3469 nt, Homo sapiens
  source 1..3469: mol_type = other RNA
tcatattgcttctttctgtttattttgttaacagctacttgaggttcagttactgaataatgagggacaccagaatctaaacttgtttttgaaccactgaattcagtacttctaccttggaattcagcgtgcttttctctttgaagccatgtttctttgacaattacttcaggtttgtgagtcgctgcctgaagagggacatcagaatccaaacttgtttcaaaaacactcttattttctaagtacatgtgctcttttgtgtgaaggcttatttctttaatgggatcttcagaacgtccagtcactgaatgaaaaatgatattataatccaaacttacttcagaatcaataggttcattttccttattttctaagtgtacctgctcttctttttgaggatttagctttttaacagctacttcgggagaattagtcactgaatgaagaggggcatgggaatccgaacttatttcagaaccactgggttcatcattcttcctttctaagtgaatgtactcttctttctgaattacttctttaacagctacttcagggtgatcatttcctgaatgaagaggaatatcagaatcaaaagttatttcagagacacaagattcattacttttactttccagatcaacagtttcttcctcataaacagctacttcaggttggtcaattactgaataaagaggaatatcagaatcaaaagttatttcagaactatctgactcacagctctcatcttccaggtcaatgtgccgttcttttccttcagcatccagatgagactgctcagtaactgacagaagaggcgggtcagaatcaaaagtcaactcagagctggagcaatcatagctcctaacttccatgtcaatatttaactctttaagatttacttcatccaaagcttcttgaggctcatcatgagctgaatgataaagagaagccggagaatcagaactcagagaagaacggctagactgaacactcttattctcaaggtcaacatccactttctgacgctctatttcggctacttgagactggtcagctaattgagcatcagcctgaaaacccatttcaggaccatgggattcacagttcatatccataaggtcagcattcttctccttcagaagatttatcttttcaacagccctctgggattcatctgcaactgtcccaagtgagacatcacaatcaagatgtgctttagcactactgggtttacgcttcttatgttttaggtggacttgtctacctttcaggtttcttcctttgacagtcagttggggatgatcaactactgactcaagagaaacatcacaatcaaaacttgtttcagaacaactcgatccatagttatcaaccaagctggtatgagccttcttccgaagttttgtttctgtgacagccactgggggtctgtcaaccactgactgcagtgggaaaacagaatcagcacttacttcagagctactggaaccatagttcttatcaaccaaaccaatgtgcacttccttaggaaggtttacttctgttacagattgttgggggtagtcactagtggactgaggtgaagcatcacaatcaaaattcgtttcagaactactagattcatagctttggtcaaccaggctaatatgccttgcattctgaagacttatttctttaacaatcatttgggattggttggtaaccaagtgaagaatgtcatcacaatcagaacttattttagaaacataagatttattattcttatactgtacatcagtacgtacttccttggaaaggtttacttctttggcactcactttagattggtcagtcagtgaatgaaaagaggaactgcaatcaaaactcatttctgaacctctagactcatagttatcttcttggtcaatttgctcctccttccaaagacttaagtcttgtgcagtctcttggggctgatcagatgctgactgaagagagatacaatcaaacttcatttcagaactcactgagcacttctgttcccaaaaggctgtcttgttaaaaaccaaatgcttttcttcttgggtacaatccatgttagaaaagaattcctcatggttctttgcaatagtatcttcaaagattcctttattagaaggcatgtcagttttattcgggtttactgctaatttggaaggagatttaactcttaaggagcccttagtacccatgcgttcatggaatttcaagccagctgataaagttttaccctgagattttacatctttccacaaaaccaacttatctgaattcatgcgtaaagatttcctatttgattctttatgtttctgatacgaaaatgaagtagtttctacatgggatgatggcacaggatttctagaggccccatctggctgttcaagatatttctcaactttgtttgggtcacatttgctaactgaatccaaatgagctgctggtggtaaactagttgtattagctgtaactggtctatcgttagagctttcaggtaaacaactagcaggagcattacaaatcactggggggcgtaccaagttgcttctattatttgtagcctgaccaatatctactaggttacattttctcacactggccccaattttatgaacaaactccaagggctgctgctgtcccttctccagtttttgaataactgatggtcgaactgaaacctcctgcgtgccttcctgagatttatgaggtctggaatgtaactcttcaataggttctgaaacctcggatggtctctcttcggtagcatcctcatcctcaaccttatcctcatcctcttcctcttcttcagaaaaagcatcatccaaatgcaccacttcagacgatgacccagtattcacatgtgtctcatcttgtgttgaactgctctcttgacaatgatatgggtggtgctgcagtacatcctgtaagaaacgttccatcaaactactggtacatatttgacgtctactctgtctggtcaaactcctgtgctgagcactgaacaaatgctgttccaggttattatactgcacacggcaataactgcaatatccttgtcttttctgcatcttgaataaataactgaagtcagatggctactgtctttgaatactcaagctggagcagaaaaggtcaggtatttcatcagctgtattagttctggcaagtatctccgcggaggctgcccggattccttccgggccgcggtggagaccgaggaccgagccgggcgctctcccttcttattccggttccgcggcggcgcccgaatcccagaccgtccgagcgccacggccccgctgcccgcggagccagaaataggcgacttcggcccctgcggtccggaggcgagaagcggcgcgggagcgcgtctctcaggacgcgggccccgagtcgcgactccactcacgcaggcatccaaggcaacgtggcgttgcaaccctgatggaggttt

SEQ ID NO: 17676 - RNA, 3269 nt, Homo sapiens
  source 1..3269: mol_type = other RNA
tcatattgcttctttctgtttattttgttaacagctacttgaggttcagttactgaataatgagggacaccagaatctaaacttgtttttgaaccactgaattcagtacttctaccttggaattcagcgtgcttttctctttgaagccatgtttctttgacaattacttcaggtttgtgagtcgctgcctgaagagggacatcagaatccaaacttgtttcaaaaacactcttattttctaagtacatgtgctcttttgtgtgaaggcttatttctttaatgggatcttcagaacgtccagtcactgaatgaaaaatgatattataatccaaacttacttcagaatcaataggttcattttccttattttctaagtgtacctgctcttctttttgaggatttagctttttaacagctacttcgggagaattagtcactgaatgaagaggggcatgggaatccgaacttatttcagaaccactgggttcatcattcttcctttctaagtgaatgtactcttctttctgaattacttctttaacagctacttcagggtgatcatttcctgaatgaagaggaatatcagaatcaaaagttatttcagagacacaagattcattacttttactttccagatcaacagtttcttcctcataaacagctacttcaggttggtcaattactgaataaagaggaatatcagaatcaaaagttatttcagaactatctgactcacagctctcatcttccaggtcaatgtgccgttcttttccttcagcatccagatgagactgctcagtaactgacagaagaggcgggtcagaatcaaaagtcaactcagagctggagcaatcatagctcctaacttccatgtcaatatttaactctttaagatttacttcatccaaagcttcttgaggctcatcatgagctgaatgataaagagaagccggagaatcagaactcagagaagaacggctagactgaacactcttattctcaaggtcaacatccactttctgacgctctatttcggctacttgagactggtcagctaattgagcatcagcctgaaaacccatttcaggaccatgggattcacagttcatatccataaggtcagcattcttctccttcagaagatttatcttttcaacagccctctgggattcatctgcaactgtcccaagtgagacatcacaatcaagatgtgctttagcactactgggtttacgcttcttatgttttaggtggacttgtctacctttcaggtttcttcctttgacagtcagttggggatgatcaactactgactcaagagaaacatcacaatcaaaacttgtttcagaacaactcgatccatagttatcaaccaagctggtatgagccttcttccgaagttttgtttctgtgacagccactgggggtctgtcaaccactgactgcagtgggaaaacagaatcagcacttacttcagagctactggaaccatagttcttatcaaccaaaccaatgtgcacttccttaggaaggtttacttctgttacagattgttgggggtagtcactagtggactgaggtgaagcatcacaatcaaaattcgtttcagaactactagattcatagctttggtcaaccaggctaatatgccttgcattctgaagacttatttctttaacaatcatttgggattggttggtaaccaagtgaagaatgtcatcacaatcagaacttattttagaaacataagatttattattcttatactgtacatcagtacgtacttccttggaaaggtttacttctttggcactcactttagattggtcagtcagtgaatgaaaagaggaactgcaatcaaaactcatttctgaacctctagactcatagttatcttcttggtcaatttgctcctccttccaaagacttaagtcttgtgcagtctcttggggctgatcagatgctgactgaagagagatacaatcaaacttcatttcagaactcactgagcacttctgttcccaaaaggctgtcttgttaaaaaccaaatgcttttcttcttgggtacaatccatgttagaaaagaattcctcatggttctttgcaatagtatcttcaaagattcctttattagaaggcatgtcagttttattcgggtttactgctaatttggaaggagatttaactcttaaggagcccttagtacccatgcgttcatggaatttcaagccagctgataaagttttaccctgagattttacatctttccacaaaaccaacttatctgaattcatgcgtaaagatttcctatttgattctttatgtttctgatacgaaaatgaagtagtttctacatgggatgatggcacaggatttctagaggccccatctggctgttcaagatatttctcaactttgtttgggtcacatttgctaactgaatccaaatgagctgctggtggtaaactagttgtattagctgtaactggtctatcgttagagctttcaggtaaacaactagcaggagcattacaaatcactggggggcgtaccaagttgcttctattatttgtagcctgaccaatatctactaggttacattttctcacactggccccaattttatgaacaaactccaagggctgctgctgtcccttctccagtttttgaataactgatggtcgaactgaaacctcctgcgtgccttcctgagatttatgaggtctggaatgtaactcttcaataggttctgaaacctcggatggtctctcttcggtagcatcctcatcctcaaccttatcctcatcctcttcctcttcttcagaaaaagcatcatccaaatgcaccacttcagacgatgacccagtattcacatgtgtctcatcttgtgttgaactgctctcttgacaatgatatgggtggtgctgcagtacatcctgtaagaaacgttccatcaaactactggtacatatttgacgtctactctgtctggtcaaactcctgtgctgagcactgaacaaatgctgttccaggttattatactgcacacggcaataactgcaatatccttgtcttttctgcatcttgaataaataactgaagtcagatggctactgtctttgaatactcaagctggagcagaaaaggtcaggtatttcatcagctgtattagttctggcaagtatctccttccctcgccccgccacctcgatcccggcccggagccgccgacacctctcacgcagcaggggcagaaagggacgcggggt

SEQ ID NO: 17677 - RNA, 3264 nt, Homo sapiens
  source 1..3264: mol_type = other RNA
tcatattgcttctttctgtttattttgttaacagctacttgaggttcagttactgaataatgagggacaccagaatctaaacttgtttttgaaccactgaattcagtacttctaccttggaattcagcgtgcttttctctttgaagccatgtttctttgacaattacttcaggtttgtgagtcgctgcctgaagagggacatcagaatccaaacttgtttcaaaaacactcttattttctaagtacatgtgctcttttgtgtgaaggcttatttctttaatgggatcttcagaacgtccagtcactgaatgaaaaatgatattataatccaaacttacttcagaatcaataggttcattttccttattttctaagtgtacctgctcttctttttgaggatttagctttttaacagctacttcgggagaattagtcactgaatgaagaggggcatgggaatccgaacttatttcagaaccactgggttcatcattcttcctttctaagtgaatgtactcttctttctgaattacttctttaacagctacttcagggtgatcatttcctgaatgaagaggaatatcagaatcaaaagttatttcagagacacaagattcattacttttactttccagatcaacagtttcttcctcataaacagctacttcaggttggtcaattactgaataaagaggaatatcagaatcaaaagttatttcagaactatctgactcacagctctcatcttccaggtcaatgtgccgttcttttccttcagcatccagatgagactgctcagtaactgacagaagaggcgggtcagaatcaaaagtcaactcagagctggagcaatcatagctcctaacttccatgtcaatatttaactctttaagatttacttcatccaaagcttcttgaggctcatcatgagctgaatgataaagagaagccggagaatcagaactcagagaagaacggctagactgaacactcttattctcaaggtcaacatccactttctgacgctctatttcggctacttgagactggtcagctaattgagcatcagcctgaaaacccatttcaggaccatgggattcacagttcatatccataaggtcagcattcttctccttcagaagatttatcttttcaacagccctctgggattcatctgcaactgtcccaagtgagacatcacaatcaagatgtgctttagcactactgggtttacgcttcttatgttttaggtggacttgtctacctttcaggtttcttcctttgacagtcagttggggatgatcaactactgactcaagagaaacatcacaatcaaaacttgtttcagaacaactcgatccatagttatcaaccaagctggtatgagccttcttccgaagttttgtttctgtgacagccactgggggtctgtcaaccactgactgcagtgggaaaacagaatcagcacttacttcagagctactggaaccatagttcttatcaaccaaaccaatgtgcacttccttaggaaggtttacttctgttacagattgttgggggtagtcactagtggactgaggtgaagcatcacaatcaaaattcgtttcagaactactagattcatagctttggtcaaccaggctaatatgccttgcattctgaagacttatttctttaacaatcatttgggattggttggtaaccaagtgaagaatgtcatcacaatcagaacttattttagaaacataagatttattattcttatactgtacatcagtacgtacttccttggaaaggtttacttctttggcactcactttagattggtcagtcagtgaatgaaaagaggaactgcaatcaaaactcatttctgaacctctagactcatagttatcttcttggtcaatttgctcctccttccaaagacttaagtcttgtgcagtctcttggggctgatcagatgctgactgaagagagatacaatcaaacttcatttcagaactcactgagcacttctgttcccaaaaggctgtcttgttaaaaaccaaatgcttttcttcttgggtacaatccatgttagaaaagaattcctcatggttctttgcaatagtatcttcaaagattcctttattagaaggcatgtcagttttattcgggtttactgctaatttggaaggagatttaactcttaaggagcccttagtacccatgcgttcatggaatttcaagccagctgataaagttttaccctgagattttacatctttccacaaaaccaacttatctgaattcatgcgtaaagatttcctatttgattctttatgtttctgatacgaaaatgaagtagtttctacatgggatgatggcacaggatttctagaggccccatctggctgttcaagatatttctcaactttgtttgggtcacatttgctaactgaatccaaatgagctgctggtggtaaactagttgtattagctgtaactggtctatcgttagagctttcaggtaaacaactagcaggagcattacaaatcactggggggcgtaccaagttgcttctattatttgtagcctgaccaatatctactaggttacattttctcacactggccccaattttatgaacaaactccaagggctgctgctgtcccttctccagtttttgaataactgatggtcgaactgaaacctcctgcgtgccttcctgagatttatgaggtctggaatgtaactcttcaataggttctgaaacctcggatggtctctcttcggtagcatcctcatcctcaaccttatcctcatcctcttcctcttcttcagaaaaagcatcatccaaatgcaccacttcagacgatgacccagtattcacatgtgtctcatcttgtgttgaactgctctcttgacaatgatatgggtggtgctgcagtacatcctgtaagaaacgttccatcaaactactggtacatatttgacgtctactctgtctggtcaaactcctgtgctgagcactgaacaaatgctgttccaggttattatactgcacacggcaataactgcaatatccttgtcttttctgcatcttgaataaataactgaagtcagatggctactgtctttgaatactcaagctggagcagaaaaggtcaggtatttcatcagctgtattagttctggcaagtatctgcgaggcggccgcgggagcccagcgagcggtcctggcgtccctcgggaagaaggcgccccgggcgcccggcgagcag

SEQ ID NO: 17678 - RNA, 3513 nt, Homo sapiens
  source 1..3513: mol_type = other RNA
tcatattgcttctttctgtttattttgttaacagctacttgaggttcagttactgaataatgagggacaccagaatctaaacttgtttttgaaccactgaattcagtacttctaccttggaattcagcgtgcttttctctttgaagccatgtttctttgacaattacttcaggtttgtgagtcgctgcctgaagagggacatcagaatccaaacttgtttcaaaaacactcttattttctaagtacatgtgctcttttgtgtgaaggcttatttctttaatgggatcttcagaacgtccagtcactgaatgaaaaatgatattataatccaaacttacttcagaatcaataggttcattttccttattttctaagtgtacctgctcttctttttgaggatttagctttttaacagctacttcgggagaattagtcactgaatgaagaggggcatgggaatccgaacttatttcagaaccactgggttcatcattcttcctttctaagtgaatgtactcttctttctgaattacttctttaacagctacttcagggtgatcatttcctgaatgaagaggaatatcagaatcaaaagttatttcagagacacaagattcattacttttactttccagatcaacagtttcttcctcataaacagctacttcaggttggtcaattactgaataaagaggaatatcagaatcaaaagttatttcagaactatctgactcacagctctcatcttccaggtcaatgtgccgttcttttccttcagcatccagatgagactgctcagtaactgacagaagaggcgggtcagaatcaaaagtcaactcagagctggagcaatcatagctcctaacttccatgtcaatatttaactctttaagatttacttcatccaaagcttcttgaggctcatcatgagctgaatgataaagagaagccggagaatcagaactcagagaagaacggctagactgaacactcttattctcaaggtcaacatccactttctgacgctctatttcggctacttgagactggtcagctaattgagcatcagcctgaaaacccatttcaggaccatgggattcacagttcatatccataaggtcagcattcttctccttcagaagatttatcttttcaacagccctctgggattcatctgcaactgtcccaagtgagacatcacaatcaagatgtgctttagcactactgggtttacgcttcttatgttttaggtggacttgtctacctttcaggtttcttcctttgacagtcagttggggatgatcaactactgactcaagagaaacatcacaatcaaaacttgtttcagaacaactcgatccatagttatcaaccaagctggtatgagccttcttccgaagttttgtttctgtgacagccactgggggtctgtcaaccactgactgcagtgggaaaacagaatcagcacttacttcagagctactggaaccatagttcttatcaaccaaaccaatgtgcacttccttaggaaggtttacttctgttacagattgttgggggtagtcactagtggactgaggtgaagcatcacaatcaaaattcgtttcagaactactagattcatagctttggtcaaccaggctaatatgccttgcattctgaagacttatttctttaacaatcatttgggattggttggtaaccaagtgaagaatgtcatcacaatcagaacttattttagaaacataagatttattattcttatactgtacatcagtacgtacttccttggaaaggtttacttctttggcactcactttagattggtcagtcagtgaatgaaaagaggaactgcaatcaaaactcatttctgaacctctagactcatagttatcttcttggtcaatttgctcctccttccaaagacttaagtcttgtgcagtctcttggggctgatcagatgctgactgaagagagatacaatcaaacttcatttcagaactcactgagcacttctgttcccaaaaggctgtcttgttaaaaaccaaatgcttttcttcttgggtacaatccatgttagaaaagaattcctcatggttctttgcaatagtatcttcaaagattcctttattagaaggcatgtcagttttattcgggtttactgctaatttggaaggagatttaactcttaaggagcccttagtacccatgcgttcatggaatttcaagccagctgataaagttttaccctgagattttacatctttccacaaaaccaacttatctgaattcatgcgtaaagatttcctatttgattctttatgtttctgatacgaaaatgaagtagtttctacatgggatgatggcacaggatttctagaggccccatctggctgttcaagatatttctcaactttgtttgggtcacatttgctaactgaatccaaatgagctgctggtggtaaactagttgtattagctgtaactggtctatcgttagagctttcaggtaaacaactagcaggagcattacaaatcactggggggcgtaccaagttgcttctattatttgtagcctgaccaatatctactaggttacattttctcacactggccccaattttatgaacaaactccaagggctgctgctgtcccttctccagtttttgaataactgatggtcgaactgaaacctcctgcgtgccttcctgagatttatgaggtctggaatgtaactcttcaataggttctgaaacctcggatggtctctcttcggtagcatcctcatcctcaaccttatcctcatcctcttcctcttcttcagaaaaagcatcatccaaatgcaccacttcagacgatgacccagtattcacatgtgtctcatcttgtgttgaactgctctcttgacaatgatatgggtggtgctgcagtacatcctgtaagaaacgttccatcaaactactggtacatatttgacgtctactctgtctggtcaaactcctgtgctgagcactgaacaaatgctgttccaggttattatactgcacacggcaataactgcaatatccttgtcttttctgcatcttgaataaataactgaagtcagatggctactgtctttgaatactcaagttaaaatttggtctcttttccactaatttacttcacttattaacctggagcagaaaaggtcaggtatttcatcagctgtattagttctggcaagtatctccgcggaggctgcccggattccttccgggccgcggtggagaccgaggaccgagccgggcgctctcccttcttattccggttccgcggcggcgcccgaatcccagaccgtccgagcgccacggccccgctgcccgcggagccagaaataggcgacttcggcccctgcggtccggaggcgagaagcggcgcgggagcgcgtctctcaggacgcgggccccgagtcgcgactccactcacgcaggcatccaaggcaacgtggcgttgcaaccctgatggaggttt

SEQ ID NO: 17679 - RNA, 4604 nt, Homo sapiens
  source 1..4604: mol_type = other RNA
tcatattgcttctttctgtttattttgttaacagctacttgaggttcagttactgaataatgagggacaccagaatctaaacttgtttttgaaccactgaattcagtacttctaccttggaattcagcgtgcttttctctttgaagccatgtttctttgacaattacttcaggtttgtgagtcgctgcctgaagagggacatcagaatccaaacttgtttcaaaaacactcttattttctaagtacatgtgctcttttgtgtgaaggcttatttctttaatgggatcttcagaacgtccagtcactgaatgaaaaatgatattataatccaaacttacttcagaatcaataggttcattttccttattttctaagtgtacctgctcttctttttgaggatttagctttttaacagctacttcgggagaattagtcactgaatgaagaggggcatgggaatccgaacttatttcagaaccactgggttcatcattcttcctttctaagtgaatgtactcttctttctgaattacttctttaacagctacttcagggtgatcatttcctgaatgaagaggaatatcagaatcaaaagttatttcagagacacaagattcattacttttactttccagatcaacagtttcttcctcataaacagctacttcaggttggtcaattactgaataaagaggaatatcagaatcaaaagttatttcagaactatctgactcacagctctcatcttccaggtcaatgtgccgttcttttccttcagcatccagatgagactgctcagtaactgacagaagaggcgggtcagaatcaaaagtcaactcagagctggagcaatcatagctcctaacttccatgtcaatatttaactctttaagatttacttcatccaaagcttcttgaggctcatcatgagctgaatgataaagagaagccggagaatcagaactcagagaagaacggctagactgaacactcttattctcaaggtcaacatccactttctgacgctctatttcggctacttgagactggtcagctaattgagcatcagcctgaaaacccatttcaggaccatgggattcacagttcatatccataaggtcagcattcttctccttcagaagatttatcttttcaacagccctctgggattcatctgcaactgtcccaagtgagacatcacaatcaagatgtgctttagcactactgggtttacgcttcttatgttttaggtggacttgtctacctttcaggtttcttcctttgacagtcagttggggatgatcaactactgactcaagagaaacatcacaatcaaaacttgtttcagaacaactcgatccatagttatcaaccaagctggtatgagccttcttccgaagttttgtttctgtgacagccactgggggtctgtcaaccactgactgcagtgggaaaacagaatcagcacttacttcagagctactggaaccatagttcttatcaaccaaaccaatgtgcacttccttaggaaggtttacttctgttacagattgttgggggtagtcactagtggactgaggtgaagcatcacaatcaaaattcgtttcagaactactagattcatagctttggtcaaccaggctaatatgccttgcattctgaagacttatttctttaacaatcatttgggattggttggtaaccaagtgaagaatgtcatcacaatcagaacttattttagaaacataagatttattattcttatactgtacatcagtacgtacttccttggaaaggtttacttctttggcactcactttagattggtcagtcagtgaatgaaaagaggaactgcaatcaaaactcatttctgaacctctagactcatagttatcttcttggtcaatttgctcctccttccaaagacttaagtcttgtgcagtctcttggggctgatcagatgctgactgaagagagatacaatcaaacttcatttcagaactcactgagcacttctgttcccaaaaggctgtcttgttaaaaaccaaatgcttttcttcttgggtacaatccatgttagaaaagaattcctcatggttctttgcaatagtatcttcaaagattcctttattagaaggcatgtcagttttattcgggtttactgctaatttggaaggagatttaactcttaaggagcccttagtacccatgcgttcatggaatttcaagccagctgataaagttttaccctgagattttacatctttccacaaaaccaacttatctgaattcatgcgtaaagatttcctatttgattctttatgtttctgatacgaaaatgaagtagtttctacatgggatgatggcacaggatttctagaggccccatctggctgttcaagatatttctcaactttgtttgggtcacatttgctaactgaatccaaatgagctgctggtggtaaactagttgtattagctgtaactggtctatcgttagagctttcaggtaaacaactagcaggagcattacaaatcactggggggcgtaccaagttgcttctattatttgtagcctgaccaatatctactaggttacattttctcacactggccccaattttatgaacaaactccaagggctgctgctgtcccttctccagtttttgaataactgatggtcgaactgaaacctcctgcgtgccttcctgagatttatgaggtctggaatgtaactcttcaataggttctgaaacctcggatggtctctcttcggtagcatcctcatcctcaaccttatcctcatcctcttcctcttcttcagaaaaagcatcatccaaatgcaccacttcagacgatgacccagtattcacatgtgtctcatcttgtgttgaactgctctcttgacaatgatatgggtggtgctgcagtacatcctgtaagaaacgttccatcaaactactggtacatatttgacgtctactctgtctggtcaaactcctgtgctgagcactgaacaaatgctgttccaggttattatactgcacacggcaataactgcaatatccttgtcttttctgcatcttgaataaataactgaagtcagatggctactgtctttgaatactcaagttaaaatttggtctcttttccactaatttacttcacttattaacctggagcagaaaaggtcaggtatttcatcagctgtattagttctggcaagtatctccgcggaggctgcccggattccttccgggccgcggtggagaccgaggaccgagccgggcgctctcccttcttattccggttccgcggcggcgcccgaatcccagaccgtccgagcgccacggccccgctgcccgcggagccagaaataggcgacttcggcccctgcggtccggaggcgagaagcggcgcgggagcgcgtctctcaggacgcgggccccgagtcgcgactccactcacgcaggcatccaaggcaacgtggcgttgcaaccctgatggaggtttgacgtcagggaaggtgcgaaaaccagaccccttctgacgcaggagcggcgggaccgccccctgcccgcccacccactcactcactctcccacccgggcggaggagccccttcctcccctccagaagctcttaaagcggacacttcctccctggtcagggccccactccggagcttgggaaatctatcgcgttccaacaaaaatgactagactcataagcacagttgggacgcgaagtagagaccaaggttttagcgtttgagggtccaaataaaaactgcttgccaattcaaagcaacgtatgaatgtagaaaagaaaacggggctaagagagctagtcgtttccgtttccatgcctatttcatagtgaggtgcatctcacaaaagctgctgttcaatgagcgcttgctctgtgctaggcaccgtttaaggtttctatacattattgcatttcatttcagagtaactctgaatgaatcctattattgtccccctttgacaaattgagaaaactgaggcttaaggaagttaggtattcaaagatctatcctgcacattaaagggttacaaatattaacaaacaacattaggtcatgcaattatattcactgcgctaccccattacgaatatagttgtgagcaaaaacagtttaagtgtaacggagatcacaaacctaaatgaatcacactactgaatatgaaattataatctgcgataagaaggttctgaaacacctaaaccaattttactaaaatggagagaggccctgttgcaaagcttatgtctaatgtaaaaataatcttaaaatgagctactttgctctttggctgtagctgtaattgtcgttaccctttttagtaagcttgtgattttgtccctttaaagaacaacaacaaaaaaacttgcctattgcttttgcgtccattgtttttattctttctgtatttctcagctccttcttcccccactacatctttctctcactttaaagttgggctcctgcaactgttcgatttataacctcccttagatttaacataccaaaaagtacggatttcttttaaggcaagttttttccacatcccaacttt

SEQ ID NO: 17680 - RNA, 3313 nt, Homo sapiens
  source 1..3313: mol_type = other RNA
tcatattgcttctttctgtttattttgttaacagctacttgaggttcagttactgaataatgagggacaccagaatctaaacttgtttttgaaccactgaattcagtacttctaccttggaattcagcgtgcttttctctttgaagccatgtttctttgacaattacttcaggtttgtgagtcgctgcctgaagagggacatcagaatccaaacttgtttcaaaaacactcttattttctaagtacatgtgctcttttgtgtgaaggcttatttctttaatgggatcttcagaacgtccagtcactgaatgaaaaatgatattataatccaaacttacttcagaatcaataggttcattttccttattttctaagtgtacctgctcttctttttgaggatttagctttttaacagctacttcgggagaattagtcactgaatgaagaggggcatgggaatccgaacttatttcagaaccactgggttcatcattcttcctttctaagtgaatgtactcttctttctgaattacttctttaacagctacttcagggtgatcatttcctgaatgaagaggaatatcagaatcaaaagttatttcagagacacaagattcattacttttactttccagatcaacagtttcttcctcataaacagctacttcaggttggtcaattactgaataaagaggaatatcagaatcaaaagttatttcagaactatctgactcacagctctcatcttccaggtcaatgtgccgttcttttccttcagcatccagatgagactgctcagtaactgacagaagaggcgggtcagaatcaaaagtcaactcagagctggagcaatcatagctcctaacttccatgtcaatatttaactctttaagatttacttcatccaaagcttcttgaggctcatcatgagctgaatgataaagagaagccggagaatcagaactcagagaagaacggctagactgaacactcttattctcaaggtcaacatccactttctgacgctctatttcggctacttgagactggtcagctaattgagcatcagcctgaaaacccatttcaggaccatgggattcacagttcatatccataaggtcagcattcttctccttcagaagatttatcttttcaacagccctctgggattcatctgcaactgtcccaagtgagacatcacaatcaagatgtgctttagcactactgggtttacgcttcttatgttttaggtggacttgtctacctttcaggtttcttcctttgacagtcagttggggatgatcaactactgactcaagagaaacatcacaatcaaaacttgtttcagaacaactcgatccatagttatcaaccaagctggtatgagccttcttccgaagttttgtttctgtgacagccactgggggtctgtcaaccactgactgcagtgggaaaacagaatcagcacttacttcagagctactggaaccatagttcttatcaaccaaaccaatgtgcacttccttaggaaggtttacttctgttacagattgttgggggtagtcactagtggactgaggtgaagcatcacaatcaaaattcgtttcagaactactagattcatagctttggtcaaccaggctaatatgccttgcattctgaagacttatttctttaacaatcatttgggattggttggtaaccaagtgaagaatgtcatcacaatcagaacttattttagaaacataagatttattattcttatactgtacatcagtacgtacttccttggaaaggtttacttctttggcactcactttagattggtcagtcagtgaatgaaaagaggaactgcaatcaaaactcatttctgaacctctagactcatagttatcttcttggtcaatttgctcctccttccaaagacttaagtcttgtgcagtctcttggggctgatcagatgctgactgaagagagatacaatcaaacttcatttcagaactcactgagcacttctgttcccaaaaggctgtcttgttaaaaaccaaatgcttttcttcttgggtacaatccatgttagaaaagaattcctcatggttctttgcaatagtatcttcaaagattcctttattagaaggcatgtcagttttattcgggtttactgctaatttggaaggagatttaactcttaaggagcccttagtacccatgcgttcatggaatttcaagccagctgataaagttttaccctgagattttacatctttccacaaaaccaacttatctgaattcatgcgtaaagatttcctatttgattctttatgtttctgatacgaaaatgaagtagtttctacatgggatgatggcacaggatttctagaggccccatctggctgttcaagatatttctcaactttgtttgggtcacatttgctaactgaatccaaatgagctgctggtggtaaactagttgtattagctgtaactggtctatcgttagagctttcaggtaaacaactagcaggagcattacaaatcactggggggcgtaccaagttgcttctattatttgtagcctgaccaatatctactaggttacattttctcacactggccccaattttatgaacaaactccaagggctgctgctgtcccttctccagtttttgaataactgatggtcgaactgaaacctcctgcgtgccttcctgagatttatgaggtctggaatgtaactcttcaataggttctgaaacctcggatggtctctcttcggtagcatcctcatcctcaaccttatcctcatcctcttcctcttcttcagaaaaagcatcatccaaatgcaccacttcagacgatgacccagtattcacatgtgtctcatcttgtgttgaactgctctcttgacaatgatatgggtggtgctgcagtacatcctgtaagaaacgttccatcaaactactggtacatatttgacgtctactctgtctggtcaaactcctgtgctgagcactgaacaaatgctgttccaggttattatactgcacacggcaataactgcaatatccttgtcttttctgcatcttgaataaataactgaagtcagatggctactgtctttgaatactcaagttaaaatttggtctcttttccactaatttacttcacttattaacctggagcagaaaaggtcaggtatttcatcagctgtattagttctggcaagtatctccttccctcgccccgccacctcgatcccggcccggagccgccgacacctctcacgcagcaggggcagaaagggacgcggggt

SEQ ID NO: 17681 - RNA, 3308 nt, Homo sapiens
  source 1..3308: mol_type = other RNA
tcatattgcttctttctgtttattttgttaacagctacttgaggttcagttactgaataatgagggacaccagaatctaaacttgtttttgaaccactgaattcagtacttctaccttggaattcagcgtgcttttctctttgaagccatgtttctttgacaattacttcaggtttgtgagtcgctgcctgaagagggacatcagaatccaaacttgtttcaaaaacactcttattttctaagtacatgtgctcttttgtgtgaaggcttatttctttaatgggatcttcagaacgtccagtcactgaatgaaaaatgatattataatccaaacttacttcagaatcaataggttcattttccttattttctaagtgtacctgctcttctttttgaggatttagctttttaacagctacttcgggagaattagtcactgaatgaagaggggcatgggaatccgaacttatttcagaaccactgggttcatcattcttcctttctaagtgaatgtactcttctttctgaattacttctttaacagctacttcagggtgatcatttcctgaatgaagaggaatatcagaatcaaaagttatttcagagacacaagattcattacttttactttccagatcaacagtttcttcctcataaacagctacttcaggttggtcaattactgaataaagaggaatatcagaatcaaaagttatttcagaactatctgactcacagctctcatcttccaggtcaatgtgccgttcttttccttcagcatccagatgagactgctcagtaactgacagaagaggcgggtcagaatcaaaagtcaactcagagctggagcaatcatagctcctaacttccatgtcaatatttaactctttaagatttacttcatccaaagcttcttgaggctcatcatgagctgaatgataaagagaagccggagaatcagaactcagagaagaacggctagactgaacactcttattctcaaggtcaacatccactttctgacgctctatttcggctacttgagactggtcagctaattgagcatcagcctgaaaacccatttcaggaccatgggattcacagttcatatccataaggtcagcattcttctccttcagaagatttatcttttcaacagccctctgggattcatctgcaactgtcccaagtgagacatcacaatcaagatgtgctttagcactactgggtttacgcttcttatgttttaggtggacttgtctacctttcaggtttcttcctttgacagtcagttggggatgatcaactactgactcaagagaaacatcacaatcaaaacttgtttcagaacaactcgatccatagttatcaaccaagctggtatgagccttcttccgaagttttgtttctgtgacagccactgggggtctgtcaaccactgactgcagtgggaaaacagaatcagcacttacttcagagctactggaaccatagttcttatcaaccaaaccaatgtgcacttccttaggaaggtttacttctgttacagattgttgggggtagtcactagtggactgaggtgaagcatcacaatcaaaattcgtttcagaactactagattcatagctttggtcaaccaggctaatatgccttgcattctgaagacttatttctttaacaatcatttgggattggttggtaaccaagtgaagaatgtcatcacaatcagaacttattttagaaacataagatttattattcttatactgtacatcagtacgtacttccttggaaaggtttacttctttggcactcactttagattggtcagtcagtgaatgaaaagaggaactgcaatcaaaactcatttctgaacctctagactcatagttatcttcttggtcaatttgctcctccttccaaagacttaagtcttgtgcagtctcttggggctgatcagatgctgactgaagagagatacaatcaaacttcatttcagaactcactgagcacttctgttcccaaaaggctgtcttgttaaaaaccaaatgcttttcttcttgggtacaatccatgttagaaaagaattcctcatggttctttgcaatagtatcttcaaagattcctttattagaaggcatgtcagttttattcgggtttactgctaatttggaaggagatttaactcttaaggagcccttagtacccatgcgttcatggaatttcaagccagctgataaagttttaccctgagattttacatctttccacaaaaccaacttatctgaattcatgcgtaaagatttcctatttgattctttatgtttctgatacgaaaatgaagtagtttctacatgggatgatggcacaggatttctagaggccccatctggctgttcaagatatttctcaactttgtttgggtcacatttgctaactgaatccaaatgagctgctggtggtaaactagttgtattagctgtaactggtctatcgttagagctttcaggtaaacaactagcaggagcattacaaatcactggggggcgtaccaagttgcttctattatttgtagcctgaccaatatctactaggttacattttctcacactggccccaattttatgaacaaactccaagggctgctgctgtcccttctccagtttttgaataactgatggtcgaactgaaacctcctgcgtgccttcctgagatttatgaggtctggaatgtaactcttcaataggttctgaaacctcggatggtctctcttcggtagcatcctcatcctcaaccttatcctcatcctcttcctcttcttcagaaaaagcatcatccaaatgcaccacttcagacgatgacccagtattcacatgtgtctcatcttgtgttgaactgctctcttgacaatgatatgggtggtgctgcagtacatcctgtaagaaacgttccatcaaactactggtacatatttgacgtctactctgtctggtcaaactcctgtgctgagcactgaacaaatgctgttccaggttattatactgcacacggcaataactgcaatatccttgtcttttctgcatcttgaataaataactgaagtcagatggctactgtctttgaatactcaagttaaaatttggtctcttttccactaatttacttcacttattaacctggagcagaaaaggtcaggtatttcatcagctgtattagttctggcaagtatctgcgaggcggccgcgggagcccagcgagcggtcctggcgtccctcgggaagaaggcgccccgggcgcccggcgagcag

SEQ ID NO: 17682 - RNA, 4709 nt, Homo sapiens
  source 1..4709: mol_type = other RNA
tcatattgcttctttctgtttattttgttaacagctacttgaggttcagttactgaataatgagggacaccagaatctaaacttgtttttgaaccactgaattcagtacttctaccttggaattcagcgtgcttttctctttgaagccatgtttctttgacaattacttcaggtttgtgagtcgctgcctgaagagggacatcagaatccaaacttgtttcaaaaacactcttattttctaagtacatgtgctcttttgtgtgaaggcttatttctttaatgggatcttcagaacgtccagtcactgaatgaaaaatgatattataatccaaacttacttcagaatcaataggttcattttccttattttctaagtgtacctgctcttctttttgaggatttagctttttaacagctacttcgggagaattagtcactgaatgaagaggggcatgggaatccgaacttatttcagaaccactgggttcatcattcttcctttctaagtgaatgtactcttctttctgaattacttctttaacagctacttcagggtgatcatttcctgaatgaagaggaatatcagaatcaaaagttatttcagagacacaagattcattacttttactttccagatcaacagtttcttcctcataaacagctacttcaggttggtcaattactgaataaagaggaatatcagaatcaaaagttatttcagaactatctgactcacagctctcatcttccaggtcaatgtgccgttcttttccttcagcatccagatgagactgctcagtaactgacagaagaggcgggtcagaatcaaaagtcaactcagagctggagcaatcatagctcctaacttccatgtcaatatttaactctttaagatttacttcatccaaagcttcttgaggctcatcatgagctgaatgataaagagaagccggagaatcagaactcagagaagaacggctagactgaacactcttattctcaaggtcaacatccactttctgacgctctatttcggctacttgagactggtcagctaattgagcatcagcctgaaaacccatttcaggaccatgggattcacagttcatatccataaggtcagcattcttctccttcagaagatttatcttttcaacagccctctgggattcatctgcaactgtcccaagtgagacatcacaatcaagatgtgctttagcactactgggtttacgcttcttatgttttaggtggacttgtctacctttcaggtttcttcctttgacagtcagttggggatgatcaactactgactcaagagaaacatcacaatcaaaacttgtttcagaacaactcgatccatagttatcaaccaagctggtatgagccttcttccgaagttttgtttctgtgacagccactgggggtctgtcaaccactgactgcagtgggaaaacagaatcagcacttacttcagagctactggaaccatagttcttatcaaccaaaccaatgtgcacttccttaggaaggtttacttctgttacagattgttgggggtagtcactagtggactgaggtgaagcatcacaatcaaaattcgtttcagaactactagattcatagctttggtcaaccaggctaatatgccttgcattctgaagacttatttctttaacaatcatttgggattggttggtaaccaagtgaagaatgtcatcacaatcagaacttattttagaaacataagatttattattcttatactgtacatcagtacgtacttccttggaaaggtttacttctttggcactcactttagattggtcagtcagtgaatgaaaagaggaactgcaatcaaaactcatttctgaacctctagactcatagttatcttcttggtcaatttgctcctccttccaaagacttaagtcttgtgcagtctcttggggctgatcagatgctgactgaagagagatacaatcaaacttcatttcagaactcactgagcacttctgttcccaaaaggctgtcttgttaaaaaccaaatgcttttcttcttgggtacaatccatgttagaaaagaattcctcatggttctttgcaatagtatcttcaaagattcctttattagaaggcatgtcagttttattcgggtttactgctaatttggaaggagatttaactcttaaggagcccttagtacccatgcgttcatggaatttcaagccagctgataaagttttaccctgagattttacatctttccacaaaaccaacttatctgaattcatgcgtaaagatttcctatttgattctttatgtttctgatacgaaaatgaagtagtttctacatgggatgatggcacaggatttctagaggccccatctggctgttcaagatatttctcaactttgtttgggtcacatttgctaactgaatccaaatgagctgctggtggtaaactagttgtattagctgtaactggtctatcgttagagctttcaggtaaacaactagcaggagcattacaaatcactggggggcgtaccaagttgcttctattatttgtagcctgaccaatatctactaggttacattttctcacactggccccaattttatgaacaaactccaagggctgctgctgtcccttctccagtttttgaataactgatggtcgaactgaaacctcctgcgtgccttcctgagatttatgaggtctggaatgtaactcttcaataggttctgaaacctcggatggtctctcttcggtagcatcctcatcctcaaccttatcctcatcctcttcctcttcttcagaaaaagcatcatccaaatgcaccacttcagacgatgacccagtattcacatgtgtctcatcttgtgttgaactgctctcttgacaatgatatgggtggtgctgcagtacatcctgtaagaaacgttccatcaaactactggtacatatttgacgtctactctgtctggtcaaactcctgtgctgagcactgaacaaatgctttccactgttcttcattacttcctgtatctctgagcttccatcgggaatcattttccttctgcctgaagaactcctttttagtttttcctttagtgagagtctgctgttccaggttattatactgcacacggcaataactgcaatatccttgtcttttctgcatcttgaataaataactgaagtcagatggctactgtctttgaatactcaagttaaaatttggtctcttttccactaatttacttcacttattaacctggagcagaaaaggtcaggtatttcatcagctgtattagttctggcaagtatctccgcggaggctgcccggattccttccgggccgcggtggagaccgaggaccgagccgggcgctctcccttcttattccggttccgcggcggcgcccgaatcccagaccgtccgagcgccacggccccgctgcccgcggagccagaaataggcgacttcggcccctgcggtccggaggcgagaagcggcgcgggagcgcgtctctcaggacgcgggccccgagtcgcgactccactcacgcaggcatccaaggcaacgtggcgttgcaaccctgatggaggtttgacgtcagggaaggtgcgaaaaccagaccccttctgacgcaggagcggcgggaccgccccctgcccgcccacccactcactcactctcccacccgggcggaggagccccttcctcccctccagaagctcttaaagcggacacttcctccctggtcagggccccactccggagcttgggaaatctatcgcgttccaacaaaaatgactagactcataagcacagttgggacgcgaagtagagaccaaggttttagcgtttgagggtccaaataaaaactgcttgccaattcaaagcaacgtatgaatgtagaaaagaaaacggggctaagagagctagtcgtttccgtttccatgcctatttcatagtgaggtgcatctcacaaaagctgctgttcaatgagcgcttgctctgtgctaggcaccgtttaaggtttctatacattattgcatttcatttcagagtaactctgaatgaatcctattattgtccccctttgacaaattgagaaaactgaggcttaaggaagttaggtattcaaagatctatcctgcacattaaagggttacaaatattaacaaacaacattaggtcatgcaattatattcactgcgctaccccattacgaatatagttgtgagcaaaaacagtttaagtgtaacggagatcacaaacctaaatgaatcacactactgaatatgaaattataatctgcgataagaaggttctgaaacacctaaaccaattttactaaaatggagagaggccctgttgcaaagcttatgtctaatgtaaaaataatcttaaaatgagctactttgctctttggctgtagctgtaattgtcgttaccctttttagtaagcttgtgattttgtccctttaaagaacaacaacaaaaaaacttgcctattgcttttgcgtccattgtttttattctttctgtatttctcagctccttcttcccccactacatctttctctcactttaaagttgggctcctgcaactgttcgatttataacctcccttagatttaacataccaaaaagtacggatttcttttaaggcaagttttttccacatcccaactt

SEQ ID NO: 17683 - RNA, 3523 nt, Homo sapiens
  source 1..3523: mol_type = other RNA
tcatattgcttctttctgtttattttgttaacagctacttgaggttcagttactgaataatgagggacaccagaatctaaacttgtttttgaaccactgaattcagtacttctaccttggaattcagcgtgcttttctctttgaagccatgtttctttgacaattacttcaggtttgtgagtcgctgcctgaagagggacatcagaatccaaacttgtttcaaaaacactcttattttctaagtacatgtgctcttttgtgtgaaggcttatttctttaatgggatcttcagaacgtccagtcactgaatgaaaaatgatattataatccaaacttacttcagaatcaataggttcattttccttattttctaagtgtacctgctcttctttttgaggatttagctttttaacagctacttcgggagaattagtcactgaatgaagaggggcatgggaatccgaacttatttcagaaccactgggttcatcattcttcctttctaagtgaatgtactcttctttctgaattacttctttaacagctacttcagggtgatcatttcctgaatgaagaggaatatcagaatcaaaagttatttcagagacacaagattcattacttttactttccagatcaacagtttcttcctcataaacagctacttcaggttggtcaattactgaataaagaggaatatcagaatcaaaagttatttcagaactatctgactcacagctctcatcttccaggtcaatgtgccgttcttttccttcagcatccagatgagactgctcagtaactgacagaagaggcgggtcagaatcaaaagtcaactcagagctggagcaatcatagctcctaacttccatgtcaatatttaactctttaagatttacttcatccaaagcttcttgaggctcatcatgagctgaatgataaagagaagccggagaatcagaactcagagaagaacggctagactgaacactcttattctcaaggtcaacatccactttctgacgctctatttcggctacttgagactggtcagctaattgagcatcagcctgaaaacccatttcaggaccatgggattcacagttcatatccataaggtcagcattcttctccttcagaagatttatcttttcaacagccctctgggattcatctgcaactgtcccaagtgagacatcacaatcaagatgtgctttagcactactgggtttacgcttcttatgttttaggtggacttgtctacctttcaggtttcttcctttgacagtcagttggggatgatcaactactgactcaagagaaacatcacaatcaaaacttgtttcagaacaactcgatccatagttatcaaccaagctggtatgagccttcttccgaagttttgtttctgtgacagccactgggggtctgtcaaccactgactgcagtgggaaaacagaatcagcacttacttcagagctactggaaccatagttcttatcaaccaaaccaatgtgcacttccttaggaaggtttacttctgttacagattgttgggggtagtcactagtggactgaggtgaagcatcacaatcaaaattcgtttcagaactactagattcatagctttggtcaaccaggctaatatgccttgcattctgaagacttatttctttaacaatcatttgggattggttggtaaccaagtgaagaatgtcatcacaatcagaacttattttagaaacataagatttattattcttatactgtacatcagtacgtacttccttggaaaggtttacttctttggcactcactttagattggtcagtcagtgaatgaaaagaggaactgcaatcaaaactcatttctgaacctctagactcatagttatcttcttggtcaatttgctcctccttccaaagacttaagtcttgtgcagtctcttggggctgatcagatgctgactgaagagagatacaatcaaacttcatttcagaactcactgagcacttctgttcccaaaaggctgtcttgttaaaaaccaaatgcttttcttcttgggtacaatccatgttagaaaagaattcctcatggttctttgcaatagtatcttcaaagattcctttattagaaggcatgtcagttttattcgggtttactgctaatttggaaggagatttaactcttaaggagcccttagtacccatgcgttcatggaatttcaagccagctgataaagttttaccctgagattttacatctttccacaaaaccaacttatctgaattcatgcgtaaagatttcctatttgattctttatgtttctgatacgaaaatgaagtagtttctacatgggatgatggcacaggatttctagaggccccatctggctgttcaagatatttctcaactttgtttgggtcacatttgctaactgaatccaaatgagctgctggtggtaaactagttgtattagctgtaactggtctatcgttagagctttcaggtaaacaactagcaggagcattacaaatcactggggggcgtaccaagttgcttctattatttgtagcctgaccaatatctactaggttacattttctcacactggccccaattttatgaacaaactccaagggctgctgctgtcccttctccagtttttgaataactgatggtcgaactgaaacctcctgcgtgccttcctgagatttatgaggtctggaatgtaactcttcaataggttctgaaacctcggatggtctctcttcggtagcatcctcatcctcaaccttatcctcatcctcttcctcttcttcagaaaaagcatcatccaaatgcaccacttcagacgatgacccagtattcacatgtgtctcatcttgtgttgaactgctctcttgacaatgatatgggtggtgctgcagtacatcctgtaagaaacgttccatcaaactactggtacatatttgacgtctactctgtctggtcaaactcctgtgctgagcactgaacaaatgctttccactgttcttcattacttcctgtatctctgagcttccatcgggaatcattttccttctgcctgaagaactcctttttagtttttcctttagtgagagtctgctgttccaggttattatactgcacacggcaataactgcaatatccttgtcttttctgcatcttgaataaataactgaagtcagatggctactgtctttgaatactcaagttaaaatttggtctcttttccactaatttacttcacttattaacctggagcagaaaaggtcaggtatttcatcagctgtattagttctggcaagtatctccttccctcgccccgccacctcgatcccggcccggagccgccgacacctctcacgcagcaggggcagaaagggacgcggggtggggggaagccgaggacctgcgaggcggccgcgggagcccagcgagcggtcctggcgtccctcgggaagaaggcgccccgggcgcccggcgagcaggccccgcc

SEQ ID NO: 17684 - RNA, 3402 nt, Homo sapiens
  source 1..3402: mol_type = other RNA
tcatattgcttctttctgtttattttgttaacagctacttgaggttcagttactgaataatgagggacaccagaatctaaacttgtttttgaaccactgaattcagtacttctaccttggaattcagcgtgcttttctctttgaagccatgtttctttgacaattacttcaggtttgtgagtcgctgcctgaagagggacatcagaatccaaacttgtttcaaaaacactcttattttctaagtacatgtgctcttttgtgtgaaggcttatttctttaatgggatcttcagaacgtccagtcactgaatgaaaaatgatattataatccaaacttacttcagaatcaataggttcattttccttattttctaagtgtacctgctcttctttttgaggatttagctttttaacagctacttcgggagaattagtcactgaatgaagaggggcatgggaatccgaacttatttcagaaccactgggttcatcattcttcctttctaagtgaatgtactcttctttctgaattacttctttaacagctacttcagggtgatcatttcctgaatgaagaggaatatcagaatcaaaagttatttcagagacacaagattcattacttttactttccagatcaacagtttcttcctcataaacagctacttcaggttggtcaattactgaataaagaggaatatcagaatcaaaagttatttcagaactatctgactcacagctctcatcttccaggtcaatgtgccgttcttttccttcagcatccagatgagactgctcagtaactgacagaagaggcgggtcagaatcaaaagtcaactcagagctggagcaatcatagctcctaacttccatgtcaatatttaactctttaagatttacttcatccaaagcttcttgaggctcatcatgagctgaatgataaagagaagccggagaatcagaactcagagaagaacggctagactgaacactcttattctcaaggtcaacatccactttctgacgctctatttcggctacttgagactggtcagctaattgagcatcagcctgaaaacccatttcaggaccatgggattcacagttcatatccataaggtcagcattcttctccttcagaagatttatcttttcaacagccctctgggattcatctgcaactgtcccaagtgagacatcacaatcaagatgtgctttagcactactgggtttacgcttcttatgttttaggtggacttgtctacctttcaggtttcttcctttgacagtcagttggggatgatcaactactgactcaagagaaacatcacaatcaaaacttgtttcagaacaactcgatccatagttatcaaccaagctggtatgagccttcttccgaagttttgtttctgtgacagccactgggggtctgtcaaccactgactgcagtgggaaaacagaatcagcacttacttcagagctactggaaccatagttcttatcaaccaaaccaatgtgcacttccttaggaaggtttacttctgttacagattgttgggggtagtcactagtggactgaggtgaagcatcacaatcaaaattcgtttcagaactactagattcatagctttggtcaaccaggctaatatgccttgcattctgaagacttatttctttaacaatcatttgggattggttggtaaccaagtgaagaatgtcatcacaatcagaacttattttagaaacataagatttattattcttatactgtacatcagtacgtacttccttggaaaggtttacttctttggcactcactttagattggtcagtcagtgaatgaaaagaggaactgcaatcaaaactcatttctgaacctctagactcatagttatcttcttggtcaatttgctcctccttccaaagacttaagtcttgtgcagtctcttggggctgatcagatgctgactgaagagagatacaatcaaacttcatttcagaactcactgagcacttctgttcccaaaaggctgtcttgttaaaaaccaaatgcttttcttcttgggtacaatccatgttagaaaagaattcctcatggttctttgcaatagtatcttcaaagattcctttattagaaggcatgtcagttttattcgggtttactgctaatttggaaggagatttaactcttaaggagcccttagtacccatgcgttcatggaatttcaagccagctgataaagttttaccctgagattttacatctttccacaaaaccaacttatctgaattcatgcgtaaagatttcctatttgattctttatgtttctgatacgaaaatgaagtagtttctacatgggatgatggcacaggatttctagaggccccatctggctgttcaagatatttctcaactttgtttgggtcacatttgctaactgaatccaaatgagctgctggtggtaaactagttgtattagctgtaactggtctatcgttagagctttcaggtaaacaactagcaggagcattacaaatcactggggggcgtaccaagttgcttctattatttgtagcctgaccaatatctactaggttacattttctcacactggccccaattttatgaacaaactccaagggctgctgctgtcccttctccagtttttgaataactgatggtcgaactgaaacctcctgcgtgccttcctgagatttatgaggtctggaatgtaactcttcaataggttctgaaacctcggatggtctctcttcggtagcatcctcatcctcaaccttatcctcatcctcttcctcttcttcagaaaaagcatcatccaaatgcaccacttcagacgatgacccagtattcacatgtgtctcatcttgtgttgaactgctctcttgacaatgatatgggtggtgctgcagtacatcctgtaagaaacgttccatcaaactactggtacatatttgacgtctactctgtctggtcaaactcctgtgctgagcactgaacaaatgctttccactgttcttcattacttcctgtatctctgagcttccatcgggaatcattttccttctgcctgaagaactcctttttagtttttcctttagtgagagtctgttccaggttattatactgcacacggcaataactgcaatatccttgtcttttctgcatcttgaataaataactgaagtcagatggctactgtctttgaatactcaagttaaaatttggtctcttttccactaatttacttcacttattaacctggagcagaaaaggtcaggtatttcatcagctgtattagttctggcaagtatctgcgaggcggccgcgggagcccagcgagcggtcctggcgtccctcgggaagaaggcgccccgggcgccc

SEQ ID NO: 17685 - RNA, 11888 nt, Homo sapiens
  source 1..11888: mol_type = other RNA
tcatattgcttctttcttgttgtttattatctgtcttccccaccagaatgcaagctccatttgggcagtggccaccttgtttactgtgtacctgtctgtatccatgaagtctgacataatgcctggcatatattatgagctcaataactattgagtgaatgaaataatgagaaaatcctgtttgatcacttgccagccatataatgctagtcaattttttccacttcagtttctgcatctgtgaaactggataacacaaatgctcaccttgtggcattgttggaataattacctgaaatcatgatgtaaattcatagcataatattggaagtgttagggctcagaatgtgataccccacagtatggtgtcttggtgtgatgagtgctttgaactgaaggaaactgaaagagcttcagaaacaaagtctttctggccttctcccacctttctttctcctgctctcctttcttccccaaggcagaccagagaaactagaattccttttccccaaggtgggtcatagaaaccagagctcttccctaaagacagccataaaacctagacatattactctaacgttcccctgcctttctgtgtaggggctggccataaagaaattctctgacctaacttgtctgatacatgatcatgagaccctcattccagaatgagtcctgccctaaacccaggagaaagagctgccacacagagaggcaaagaagaatgtgaacagacaggtcttgcggggtttcctccctctgcctgctaccattagaccataccctttttgtccaatcaaatttgacacagctgtctgttcttcactgaatctgagcatacaaatggacaattttccttgatatttgggtcttcatttcttaaagctcctgtgacgtgtacaactttgatcaaataaattcgtacgttttctcctattaatctttctctgccaaccctaggcaggttgaggaaactttctctttgacaggcacatcataagagctgaactaatattagctcctttatttcctaagatgaacctctgtctgagtgcatgccagtcagtagaagaaatcagatgggctattcccattttgcctccaatgaatatattgttttgaagaaggtaaatgaatgtgtaaaactccaggcagggcatccttctctctcattgggcacagtgccctgcctggtaaaactgaatttggtaaaaccttctgtgctctcatagtaacttgttcaaatgaccacacagatggaattatgtttacttgtctatttcctgagttggtctgtgtgggggaaggaagatactttactaattttgtaatcctgctgcctagcatggtgcctgcttcctagtgcttagtcatggacattcagtgaaaagtgatatttgagctgagttttatagataaagaaggcatatccagcagacaaatgcagggagggcctaggcagggcacatggcataagcaaaggcatggcagcctaaaaggcaaggcatgctccaggaggaaagttgaggaggttggtagaatagcaagggaggagggagtcggcttctgaaggtgaagatttccgaggtgaggggacgatttctggatatttcaggattgggattgtcgctacaagttacccaggtctattaaagtgtaaagcactgggaacgggtaagtcaaagcattgtgaggctgaggtccagactgggtgatctatgaggatgctgaagtcatcaggaaggtgcagaagtggggaaggagatggcaactgagttaagtgccaagggttctaataaatatggaatgatctgaatggcagagccatagccaaagtgcatgtgtcccaagtgaaggtgacaacactggcctgcaagctgtgctttgaatggttttctcagcagtcggcgagggagaacactgactcatctctacttcttcatgaagaccaccactcacatcttcaggactcaagcaagggtacaaatggaagccctgccctgcagagctccttttctgtgtgtgccctggttgcactgagcatgcattatgccactcagcctgcacctctgagttccatttacacactgcaaacagccatccttaggcctgtagtgtgcacactgtgggtgtaatccaccctcgggtggagagggtcaaggcaaaccttgagtactcaggcaggagattttggggcctcaagtatcagaacatgttcagtgcaaatttgggtgctcatgtgccgttggcctcatgggctcccagattccttgcctatgggtaaggcatggccagaggagggcaagagagagcagggtcctctaaagcatggtgtccaggaaggggaccacatatctgcccttaacttgcttcattacaaaccagcacctaaatgtaaaatgcctgattgcagcagagaaaatagccacggccaggcaatggtcttattctcttccagcaaatggtctcttttagggatgaacaaagacatgcttaaattaaaggttattctcctctggaggaaacaccttagagctgtcaaattctttcttaactacactggctcacagtcaagtttggcccatgagttagggctctcctgagccacagtacatttcattgacttttatttttctctcttcctggcttctgctgagctcaactgcgtgccagtcagggggtgccctgtgcttgggatcaggaggagaaaaggtattacagggaattagaaaaagctctgctcactggatcactgggctttgctttgtgactctattttccttgttcatctgattaaattcacatcatcaaggcttcagcatggacagtgagcatcagctgtgtgagaatacagtccctggtcagctgctggcctggtcttgctgccagaagtgtctgaactaggttgctgcccttattcatgttaaggctggtgtttccaatacctctacttttatgtgaccctgggaagtggacacattcagttgtgacagtcattaaagagacagtccagactggaaccaagggatttgaattctgcgcttattctgtcattgtataggtgcacaacctagagaggtcacttaacctttgaatgctaatttcttcttttataacaaggaaaccctgtcctcctttctacctcacaggaatgttttgaggatctaatgagccaatgcaagccaaagtcttctggaatttgtaaaaaaaacccattgaaatataggagattattatcaccgtggtgtgaaccatgtatcatattctttagaaagtgacagccccacaggagagcagctttgctgtggggtggttggagagatgatggcaggagagaattagagtgagggctgggaaaccaggagagagtggaaaagggggaggattaggtgcagcaagctgttaaaagaaatgaaaagtgactgaaattcaaaatttcctagtgttaaatactaggctaggcaatctacacacacaagctcaattaatacttattacaacctttcaggtgtcttttttttttattcttaatcaccctgcttccacccttttagaaatagagaaattgaaatgatatagcttcctgtacttttttgtcttcatttcttgctactctccctcacccctttttctctgctccagccacaccgatcttgtttttctggagcaaagcaggtttactgtccctgggcttttgcacttgctgttccctttgcctggagcactcttccctcagtatccacacgtctcactttccattccctccaggtctactcaagtcacgttctcagggaggcccccaatgtcgcacatcatatccctcttccctgatttattttttgtcaccagcacttgtcactgcctagcaccaatgcattttactgagtttgtatgtcattggtcacctctactagaatatagagtctccaaggacagaaattttttatttactactttatatccagtgactggaatagtgcttggtttaaagtaggcactcaataaatatttgttgaatgagggaatgcataagtggaaaatagaattgtgtgggcttgttcagagttagtttttgatttctctaggtggctcccagtgatataatttaccccaacaccaaatatttttatagttccaaatactgacccttatctctttggttagactccgtctcactttttgaactagatctgggggccccacaccatggtatgtagagccctgggaaacctagaccatcatgatatgtccattgggcttttctactgggatctaaaactgagctcattcagtgttttgaattgaactctttgcaacaagttggaaaggttttcttaagacaaagataaacaagtatctgcacaaagggacatgatcagggcatggctttctttcacattgcccctttccttgatatttgtcttgccattctctcttttcctcatgtctcctccttcctatcctagtgcatttcttttcttacttctttttcctcttgtctcttttctttctttttttccttttccattcctattcccaaacaggatttcatggacaatgtgtgactccaatggttgcctttagatctgagtagtctctaaggtttgtttcagggagggatggaacagactacatggagaggaggagctgcactgcaggttataatggagggagggtgacagaggaatgaagacaggagatgtgaggtgtaaaggtgccatatgtattctgaccttgaatcccactggcttcatcccatgagagaggatttgggttggctcacgttggaggatgaggttgcctacccattcattccccctcttctagtacctgcttccacattcctgactgacagaacttgcctttcactatagaggctgaatgtggcagaggctcattttgtgacctctcttgcaaccagggcagcagtcctggatagtgaatagaaaggaggctttctcatggcctttaatgagacattctattccctttgaaaagagagatgcacagaagaaaagacatctcttctttgtttctggatttggtcatgtctgcttggggcatctggaactgctatagcaacctactatcatgagggaagacatggctgaagactccaaagatgacagagcaaaaagatggaaaggtcctgggtctttgagatcattgagctgccaatccaagcctggaacattttatataactggccttactgtttaaggcttttttaaaataagagttctgcttcttgccactgaaagcactttgatgagggtcagcaaataccaccttatagttgagctttattttgtgtggacgtttatttagtctctttaatgggttcagttatattttaaacaaacaacacatcctatatatttgtcttctttcttcaatgtcccttagtatgtagtagctgaaagtttattccctgcttgtgcctttacaaactttcctaataaaatactttatgaacctgaaggttgtggccatcagtttcaatgatctttttctgatttttctaatgccatgtgatactgacctaaataaggtgtagtgctgcctgtggtaagagttgcagtatcttagtgatgcaagtgcagggggctttttctcttattctcttcctccctccatttgctcttgcagaaacaaggtatgaagggttccccatgatcagcacatggagacttttagtgaaatagtactctccagtgccccccattccatccccttcaccaaaactaatgcatctgtatgtgacaagataaaaatttttgatcaacttgtgtacctagttcatctcttcactctgacccattcactctggatttatccattcagtcaccttgctccaaccccaccaaggaggatcctaccttgtcagattttcttgggatttagtcaaaggagtatatggaggaaagttggtggagaagggaagacaaaatgagaggctttccaggatggggctgaataaatttatgatgagtgaaaatctgaggaaatagacatgggagcaggtccagtgtgtggtcagggataggaggcaaagatttcattttgcaccaggatggccaaagccaatatccatcatgagagatcagtatttgtattgatattttcagtattacccatggagatatgggtactttaagtaatctctgggagctattgtcctcttcatggtttttgagatttgcaatacaaacttaaaaaatagaaaaaacaaacttgtattaatctgaaacttcgtgcacgcgcgtgcgcgtgtgtgtgtgtgtgtgttccctctgggtcaccactatgggactgaactgccactccaggaggtacaactttaggggtgttacctgtataatcacctttagggggaagagtgatttcaatggtttttattataatacaggaagtgtaggatgtttttctttccctttagatttgtctaaagggtttagaagcactgagtttagctacccataaatatgtttgcttatttgagaaaagtctcatctcttaccaggaagtattatagtgatggaaaaaatgtcttctgagtgtctcttgctgtatatttgtctctgagcacattcttgcctctcagagccatgatttcttaaaccgatgtgtcatcagcagctatgttgtggaataattaatactctatcgtatttttaatttagctgcaacttgcttttgagtccaaattcagaaatacattgcctctggtcaaaaataaggaagatgaatgactgcagatggagctgggacagcccagcagtgcagcaaacgagtgtgtgggggctggggagaaaatgctagctgaaagccctgcatttttgtatagttctagatcagtgccctccaattgaaataaactgcaagccataaatgcaagccacataagtaatttaaaattttcttgtagctacattaaaaaatgtaaaaataaataagtgaaactaatttttaaatgtatttgtcctgatacctccaaaacaatattgtcctagtatgtaatcaataaaataattattgagctattttatgattttttatatgaagtatttggaatcccatgtgtattttacacttacagcacatctaaattcaggctagccacggttcaagtgcccagtagccacatgtggctagcagccactgtgctagacagtaaagctctagactctttacaaggacaattattttattttgcacttgatgctcacagtatatcaaaatggtgccaggtcagatgggaagagacgattgctttttcttctggctctctaaggacttcctccaaaatgcttttgggatcaagtttttaaatgtttgccaaagggtaagaggaggaagggctggcttctgacatagaaagagaagacgcagagctttgtctgctagccaaggcacagagcttggtggaatttatagttgatatttatgaccgaaattatccagatggggtcatttataaaatagatgtgggtagtatggttatttattgagagcaatatgctataatggaatgagttctagactgagggtcaggagagggcactagaccaggcacaggtctgggaggagagaagtgaactaacgtttaccatgccagttacagcactaggctcttcacaaccattttcttatctacttcttacaataagctcaaaagttagctatataaccgtctctagtttacagaaatggcagctgagcctagtgaggtcaggtcctggcttattatggagtcctaataaaatcgcagtgctgtctgattccaaactgctgtgttcttaacattacgatccatatgcatgtcatataataggtgttagggttcaagtagagaagcagaaccagtgatatatttgcatgcatgtaaatatatataggtggtaaatatttgttacaggctcacacagttgtggggagctggttaacctgtctttgtaaggatgtctccacagctgatgccagaactagaagtcctcagggtgggcgatcataaagggaagatcacagcatgctggaagcagcagcacaggtagaactccacaagcacaccctgagccctgcttacattcttgttgcctctgaccttggtgatgaaagtgccgtacagaagttggagcctttatcatggagcttaacaaatatacctggcccaggacgagtctgagaacctgaaggaggatccagggaaaggtggagcaattggagacccagccgttgcttcacagcagtgagctgagtcagcatcagcaacagagtgtgctgagctacaaaatggctgccattttcctctgccctcctgttttcctagagtcctcactatggcccacactaactggaaacacatgaggaagggaaatctgggaaatgtatttcagcctatccacactgacgcattacaaaggcttcagatgggtgttcaattaatatttgttgaatgaatgaatgaatgaataccatggtgcttctctgggaaattctctgggagtcggaatacctaatcctggctctgcctcttacaaactaaacaattttgaacaagtcacttaactctttgagtcgtggtttcctcatttgtaaaactccaagaataatccctgtcctgcttatttaacagggatcacttgagatatctgaacaaaagcactttgaacataacgtgcaaaaataacatatataaggataaaatatgtaatacagtattgcattctttaattattattgttgttactaataattcagcttcctaatgtatcacatggaattaatagttcctgaccaatttaccttaaaggtatgccaggaatattaaattagatgaaatgtgtagaagcactgtcagctctttgtgacatacccttcaaaggcaagactgaattatcattcaatactcagatacattttcacattgtgttttagttttgggctaaatgacttagagggacaagtatgtaagtggaaccactggtgactctgggagctgaagagcagtggccattccttggatgggtgttgtggacagtggatgaagtttctgtcctataaatttgggcttgcatttcatagcagccacacttgctcagcagaatgaagaaatctctgcgaaagtttttggtaaagatggcatagaggaaggggttggcacaggagttgatggggtgaaacagaaccagcagaatctttgctttggacacagtgatgaggggcaccttgagggaggcagaaatggcaaagaaagaaatgggtgccatgcagaggaagtcagtgaagatgagcatggccatgcgcttggcgatcctggtgtcactagaggaggacacgatgttggggttccgcactgtgaggtagatgtggatatagcagccacagatgaccacaaaggccaggacattgagcacaaggagggacatgacatacagctgtgacaaagggctgtcaatatccatgggcaggcagatgctcaccttcatgtagctgctgatgccaaagatgggaaagagggcagctgcaaaagcaaaaatccagcccatcaccatgacactggcagcatggcggagctgcaccttgcagtccagctgcatggcatgcgtgatggtatgccatctttccaaggtgatagctgtcagagtgtagactgacagctcactggcaaagacagtgaaaaagccagcagcatcacagcctgccccagtttgccagtcaatggcatagttgtgatattggctcttggtatggatatcaactgatgcaatgagcagcaggtagattccaatgcagagatcagcaaaggccaggttgcacataaggaacctggggactgtgagtttatattggctggtagttaggatcactagcactatgatgttcccagtgatggccaggatgctgataaaccatatcaggactctgaggatgttgtaccccatgatatcttcacatgggttgaatgcatctggcttaggggagcaggtcacgtcaaccacttcattgcataagtcatagtcaaactcagtgtacgtcatgtcaaatcctctgctgtagctggactcattgtcttctgccagagaggatctctgacccctagcctgagtcatataatcaacttcttgccttaaaatagatttgttgcaaattggatgaagctcagagatttgccgtctccagtttgcaaaggcacagcaatggctgggataggtgaggctggcttccatgagggcgacaagcttttccagagtaggcagcttttttaagttgtaagtcgacctggccctcagcttcttaagattttctaagccatagctaggcagggaatggatccttgttcttgaaatatctagaatgactggtccagaggctccgtggaaaacatcattaggcaattcttctaaattattattatcgcttagattcagctcatctagttgggttccattgaatgcacagttgtgtatttcttgaatcccattcttattcagccatagaatcacactttcaaagctcagccccacgaaagaatttctttcaattgtgtggatgtttatgttatcttgaatgtcaagtaaaactttttggagagaatgaatcttgtgaacatctggaaggtgcttaatacctgtgttggatattaaccttttcagagtctcagtttctctctgtaaaatgattttgtgtaagaaattatgtgagacagtaggaaagcctggtttcttgccttttcgatctcacattttcaaaactagaagtatttaactctcatatttaactggaactctttgtctcagtctccatggaaaccaaactccttagtaatcaggggaaatttaaggagctcaagggtaacatttcctagaggagaggtcagtcctatcggcttggctgcagattctgttcggacctagcatcctagatttgcaatcagcctctgtttttgagcagggcatgtagcatagcttcaaaggtaagagctctggtgccagatggtctggtttcaagtcctcctggccttatcattttttaagatgtgtagccttaggggttagttggagtctccagggctcagatctcttatattttacacagggaaataagatttaccttttaggacaacttagccccgtgaccaggaattgttactgctgtggtcatgctccagccttgtattccagttgccatatctgagattctgatttccttgatccactaggacctgggtcatgtcttacatctccctagttctcttgggtgctcaaatgctgtttccttgcctgagtccctgtgggacttatatgacacttcagtaggctggtctgttaccttctacctgaggctccttgagctctgctgagaacattggaagtcacagtggactttcccagattcctcctgccctcgttctctaattgccttctgcttccttctgataaacctgcctggatcaacctttttacctttttacctgtctgactctgtttagcctctggctcctgggttttctgatcaggatcatactatcacttagaggtttgttgaagtcaaggaaaactactacctagagttgataaattaaagatgacttatacatttttttttcaaaaagacaagtgatccaaatttgttgagtttttctttgacaaatggctgtcagaaataatggtacaaagcagatattttctaattagacatacttgatttgtctttttaagtgaaaggtggtatattaatgaggaggaaggcaacaggatttgaaaaaaaaatctgtgctatggataaagcattgggaaacatgtatggaaattgttaatttattgctgaaagtgatgtatgtcattatatatgaaaactctcatagtatatgttttaaacataaggaa

SEQ ID NO: 17686 - RNA, 11221 nt, Homo sapiens
  source 1..11221: mol_type = other RNA
tcatattgcttctttcttgttgtttattatctgtcttccccaccagaatgcaagctccatttgggcagtggccaccttgtttactgtgtacctgtctgtatccatgaagtctgacataatgcctggcatatattatgagctcaataactattgagtgaatgaaataatgagaaaatcctgtttgatcacttgccagccatataatgctagtcaattttttccacttcagtttctgcatctgtgaaactggataacacaaatgctcaccttgtggcattgttggaataattacctgaaatcatgatgtaaattcatagcataatattggaagtgttagggctcagaatgtgataccccacagtatggtgtcttggtgtgatgagtgctttgaactgaaggaaactgaaagagcttcagaaacaaagtctttctggccttctcccacctttctttctcctgctctcctttcttccccaaggcagaccagagaaactagaattccttttccccaaggtgggtcatagaaaccagagctcttccctaaagacagccataaaacctagacatattactctaacgttcccctgcctttctgtgtaggggctggccataaagaaattctctgacctaacttgtctgatacatgatcatgagaccctcattccagaatgagtcctgccctaaacccaggagaaagagctgccacacagagaggcaaagaagaatgtgaacagacaggtcttgcggggtttcctccctctgcctgctaccattagaccataccctttttgtccaatcaaatttgacacagctgtctgttcttcactgaatctgagcatacaaatggacaattttccttgatatttgggtcttcatttcttaaagctcctgtgacgtgtacaactttgatcaaataaattcgtacgttttctcctattaatctttctctgccaaccctaggcaggttgaggaaactttctctttgacaggcacatcataagagctgaactaatattagctcctttatttcctaagatgaacctctgtctgagtgcatgccagtcagtagaagaaatcagatgggctattcccattttgcctccaatgaatatattgttttgaagaaggtaaatgaatgtgtaaaactccaggcagggcatccttctctctcattgggcacagtgccctgcctggtaaaactgaatttggtaaaaccttctgtgctctcatagtaacttgttcaaatgaccacacagatggaattatgtttacttgtctatttcctgagttggtctgtgtgggggaaggaagatactttactaattttgtaatcctgctgcctagcatggtgcctgcttcctagtgcttagtcatggacattcagtgaaaagtgatatttgagctgagttttatagataaagaaggcatatccagcagacaaatgcagggagggcctaggcagggcacatggcataagcaaaggcatggcagcctaaaaggcaaggcatgctccaggaggaaagttgaggaggttggtagaatagcaagggaggagggagtcggcttctgaaggtgaagatttccgaggtgaggggacgatttctggatatttcaggattgggattgtcgctacaagttacccaggtctattaaagtgtaaagcactgggaacgggtaagtcaaagcattgtgaggctgaggtccagactgggtgatctatgaggatgctgaagtcatcaggaaggtgcagaagtggggaaggagatggcaactgagttaagtgccaagggttctaataaatatggaatgatctgaatggcagagccatagccaaagtgcatgtgtcccaagtgaaggtgacaacactggcctgcaagctgtgctttgaatggttttctcagcagtcggcgagggagaacactgactcatctctacttcttcatgaagaccaccactcacatcttcaggactcaagcaagggtacaaatggaagccctgccctgcagagctccttttctgtgtgtgccctggttgcactgagcatgcattatgccactcagcctgcacctctgagttccatttacacactgcaaacagccatccttaggcctgtagtgtgcacactgtgggtgtaatccaccctcgggtggagagggtcaaggcaaaccttgagtactcaggcaggagattttggggcctcaagtatcagaacatgttcagtgcaaatttgggtgctcatgtgccgttggcctcatgggctcccagattccttgcctatgggtaaggcatggccagaggagggcaagagagagcagggtcctctaaagcatggtgtccaggaaggggaccacatatctgcccttaacttgcttcattacaaaccagcacctaaatgtaaaatgcctgattgcagcagagaaaatagccacggccaggcaatggtcttattctcttccagcaaatggtctcttttagggatgaacaaagacatgcttaaattaaaggttattctcctctggaggaaacaccttagagctgtcaaattctttcttaactacactggctcacagtcaagtttggcccatgagttagggctctcctgagccacagtacatttcattgacttttatttttctctcttcctggcttctgctgagctcaactgcgtgccagtcagggggtgccctgtgcttgggatcaggaggagaaaaggtattacagggaattagaaaaagctctgctcactggatcactgggctttgctttgtgactctattttccttgttcatctgattaaattcacatcatcaaggcttcagcatggacagtgagcatcagctgtgtgagaatacagtccctggtcagctgctggcctggtcttgctgccagaagtgtctgaactaggttgctgcccttattcatgttaaggctggtgtttccaatacctctacttttatgtgaccctgggaagtggacacattcagttgtgacagtcattaaagagacagtccagactggaaccaagggatttgaattctgcgcttattctgtcattgtataggtgcacaacctagagaggtcacttaacctttgaatgctaatttcttcttttataacaaggaaaccctgtcctcctttctacctcacaggaatgttttgaggatctaatgagccaatgcaagccaaagtcttctggaatttgtaaaaaaaacccattgaaatataggagattattatcaccgtggtgtgaaccatgtatcatattctttagaaagtgacagccccacaggagagcagctttgctgtggggtggttggagagatgatggcaggagagaattagagtgagggctgggaaaccaggagagagtggaaaagggggaggattaggtgcagcaagctgttaaaagaaatgaaaagtgactgaaattcaaaatttcctagtgttaaatactaggctaggcaatctacacacacaagctcaattaatacttattacaacctttcaggtgtcttttttttttattcttaatcaccctgcttccacccttttagaaatagagaaattgaaatgatatagcttcctgtacttttttgtcttcatttcttgctactctccctcacccctttttctctgctccagccacaccgatcttgtttttctggagcaaagcaggtttactgtccctgggcttttgcacttgctgttccctttgcctggagcactcttccctcagtatccacacgtctcactttccattccctccaggtctactcaagtcacgttctcagggaggcccccaatgtcgcacatcatatccctcttccctgatttattttttgtcaccagcacttgtcactgcctagcaccaatgcattttactgagtttgtatgtcattggtcacctctactagaatatagagtctccaaggacagaaattttttatttactactttatatccagtgactggaatagtgcttggtttaaagtaggcactcaataaatatttgttgaatgagggaatgcataagtggaaaatagaattgtgtgggcttgttcagagttagtttttgatttctctaggtggctcccagtgatataatttaccccaacaccaaatatttttatagttccaaatactgacccttatctctttggttagactccgtctcactttttgaactagatctgggggccccacaccatggtatgtagagccctgggaaacctagaccatcatgatatgtccattgggcttttctactgggatctaaaactgagctcattcagtgttttgaattgaactctttgcaacaagttggaaaggttttcttaagacaaagataaacaagtatctgcacaaagggacatgatcagggcatggctttctttcacattgcccctttccttgatatttgtcttgccattctctcttttcctcatgtctcctccttcctatcctagtgcatttcttttcttacttctttttcctcttgtctcttttctttctttttttccttttccattcctattcccaaacaggatttcatggacaatgtgtgactccaatggttgcctttagatctgagtagtctctaaggtttgtttcagggagggatggaacagactacatggagaggaggagctgcactgcaggttataatggagggagggtgacagaggaatgaagacaggagatgtgaggtgtaaaggtgccatatgtattctgaccttgaatcccactggcttcatcccatgagagaggatttgggttggctcacgttggaggatgaggttgcctacccattcattccccctcttctagtacctgcttccacattcctgactgacagaacttgcctttcactatagaggctgaatgtggcagaggctcattttgtgacctctcttgcaaccagggcagcagtcctggatagtgaatagaaaggaggctttctcatggcctttaatgagacattctattccctttgaaaagagagatgcacagaagaaaagacatctcttctttgtttctggatttggtcatgtctgcttggggcatctggaactgctatagcaacctactatcatgagggaagacatggctgaagactccaaagatgacagagcaaaaagatggaaaggtcctgggtctttgagatcattgagctgccaatccaagcctggaacattttatataactggccttactgtttaaggcttttttaaaataagagttctgcttcttgccactgaaagcactttgatgagggtcagcaaataccaccttatagttgagctttattttgtgtggacgtttatttagtctctttaatgggttcagttatattttaaacaaacaacacatcctatatatttgtcttctttcttcaatgtcccttagtatgtagtagctgaaagtttattccctgcttgtgcctttacaaactttcctaataaaatactttatgaacctgaaggttgtggccatcagtttcaatgatctttttctgatttttctaatgccatgtgatactgacctaaataaggtgtagtgctgcctgtggtaagagttgcagtatcttagtgatgcaagtgcagggggctttttctcttattctcttcctccctccatttgctcttgcagaaacaaggtatgaagggttccccatgatcagcacatggagacttttagtgaaatagtactctccagtgccccccattccatccccttcaccaaaactaatgcatctgtatgtgacaagataaaaatttttgatcaacttgtgtacctagttcatctcttcactctgacccattcactctggatttatccattcagtcaccttgctccaaccccaccaaggaggatcctaccttgtcagattttcttgggatttagtcaaaggagtatatggaggaaagttggtggagaagggaagacaaaatgagaggctttccaggatggggctgaataaatttatgatgagtgaaaatctgaggaaatagacatgggagcaggtccagtgtgtggtcagggataggaggcaaagatttcattttgcaccaggatggccaaagccaatatccatcatgagagatcagtatttgtattgatattttcagtattacccatggagatatgggtactttaagtaatctctgggagctattgtcctcttcatggtttttgagatttgcaatacaaacttaaaaaatagaaaaaacaaacttgtattaatctgaaacttcgtgcacgcgcgtgcgcgtgtgtgtgtgtgtgtgttccctctgggtcaccactatgggactgaactgccactccaggaggtacaactttaggggtgttacctgtataatcacctttagggggaagagtgatttcaatggtttttattataatacaggaagtgtaggatgtttttctttccctttagatttgtctaaagggtttagaagcactgagtttagctacccataaatatgtttgcttatttgagaaaagtctcatctcttaccaggaagtattatagtgatggaaaaaatgtcttctgagtgtctcttgctgtatatttgtctctgagcacattcttgcctctcagagccatgatttcttaaaccgatgtgtcatcagcagctatgttgtggaataattaatactctatcgtatttttaatttagctgcaacttgcttttgagtccaaattcagaaatacattgcctctggtcaaaaataaggaagatgaatgactgcagatggagctgggacagcccagcagtgcagcaaacgagtgtgtgggggctggggagaaaatgctagctgaaagccctgcatttttgtatagttctagatcagtgccctccaattgaaataaactgcaagccataaatgcaagccacataagtaatttaaaattttcttgtagctacattaaaaaatgtaaaaataaataagtgaaactaatttttaaatgtatttgtcctgatacctccaaaacaatattgtcctagtatgtaatcaataaaataattattgagctattttatgattttttatatgaagtatttggaatcccatgtgtattttacacttacagcacatctaaattcaggctagccacggttcaagtgcccagtagccacatgtggctagcagccactgtgctagacagtaaagctctagactctttacaaggacaattattttattttgcacttgatgctcacagtatatcaaaatggtgccaggtcagatgggaagagacgattgctttttcttctggctctctaaggacttcctccaaaatgcttttgggatcaagtttttaaatgtttgccaaagggtaagaggaggaagggctggcttctgacatagaaagagaagacgcagagctttgtctgctagccaaggcacagagcttggtggaatttatagttgatatttatgaccgaaattatccagatggggtcatttataaaatagatgtgggtagtatggttatttattgagagcaatatgctataatggaatgagttctagactgagggtcaggagagggcactagaccaggcacaggtctgggaggagagaagtgaactaacgtttaccatgccagttacagcactaggctcttcacaaccattttcttatctacttcttacaataagctcaaaagttagctatataaccgtctctagtttacagaaatggcagctgagcctagtgaggtcaggtcctggcttattatggagtcctaataaaatcgcagtgctgtctgattccaaactgctgtgttcttaacattacgatccatatgcatgtcatataataggtgttagggttcaagtagagaagcagaaccagtgatatatttgcatgcatgtaaatatatataggtggtaaatatttgttacaggctcacacagttgtggggagctggttaacctgtctttgtaaggatgtctccacagctgatgccagaactagaagtcctcagggtgggcgatcataaagggaagatcacagcatgctggaagcagcagcacaggtagaactccacaagcacaccctgagccctgcttacattcttgttgcctctgaccttggtgatgaaagtgccgtacagaagttggagcctttatcatggagcttaacaaatatacctggcccaggacgagtctgagaacctgaaggaggatccagggaaaggtggagcaattggagacccagccgttgcttcacagcagtgagctgagtcagcatcagcaacagagtgtgctgagctacaaaatggctgccattttcctctgccctcctgttttcctagagtcctcactatggcccacactaactggaaacacatgaggaagggaaatctgggaaatgtatttcagcctatccacactgacgcattacaaaggcttcagatgggtgttcaattaatatttgttgaatgaatgaatgaatgaataccatggtgcttctctgggaaattctctgggagtcggaatacctaatcctggctctgcctcttacaaactaaacaattttgaacaagtcacttaactctttgagtcgtggtttcctcatttgtaaaactccaagaataatccctgtcctgcttatttaacagggatcacttgagatatctgaacaaaagcactttgaacataacgtgcaaaaataacatatataaggataaaatatgtaatacagtattgcattctttaattattattgttgttactaataattcagcttcctaatgtatcacatggaattaatagttcctgaccaatttaccttaaaggtatgccaggaatattaaattagatgaaatgtgtagaagcactgtcagctctttgtgacatacccttcaaaggcaagactgaattatcattcaatactcagatacattttcacattgtgttttagttttgggctaaatgacttagagggacaagtatgtaagtggaaccactggtgactctgggagctgaagagcagtggccattccttggatgggtgttgtggacagtggatgaagtttctgtcctataaatttgggcttgcatttcatagcagccacacttgctcagcagaatgaagaaatctctgcgaaagtttttggtaaagatggcatagaggaaggggttggcacaggagttgatggggtgaaacagaaccagcagaatctttgctttggacacagtgatgaggggcaccttgagggaggcagaaatggcaaagaaagaaatgggtgccatgcagaggaagtcagtgaagatgagcatggccatgcgcttggcgatcctggtgtcactagaggaggacacgatgttggggttccgcactgtgaggtagatgtggatatagcagccacagatgaccacaaaggccaggacattgagcacaaggagggacatgacatacagctgtgacaaagggctgtcaatatccatgggcaggcagatgctcaccttcatgtagctgctgatgccaaagatgggaaagagggcagctgcaaaagcaaaaatccagcccatcaccatgacactggcagcatggcggagctgcaccttgcagtccagctgcatggcatgcgtgatggtatgccatctttccaaggtgatagctgtcagagtgtagactgacagctcactggcaaagacagtgaaaaagccagcagcatcacagcctgccccagtttgccagtcaatggcatagttgtgatattggctcttggtatggatatcaactgatgcaatgagcagcaggtagattccaatgcagagatcagcaaaggccaggttgcacataaggaacctggggactgtgagtttatattggctggtagttaggatcactagcactatgatgttcccagtgatggccaggatgctgataaaccatatcaggactctgaggatgttgtaccccatgatatcttcacatgggttgaatgcatctggcttaggggagcaggtcacgtcaaccacttcattgcataagtcatagtcaaactcagtgtacgtcatgtcaaatcctctgctgtagctggactcattgtcttctgccagagaggatctctgacccctagcctgagtcatataatcaacttcttgccttaaaatagatttgttgcaaattggatgaagctcagagatttgccgtctccagtttgcaaaggcacagcaatggctgggataggtgaggctggcttccatgagggcgacaagcttttccagagtaggcagcttttttaagttgtaagtcgacctggccctcagcttcttaagattttctaagccatagctaggcagggaatggatccttgttcttgaaatatctatggatgaggagagagactccggttcctccaacacaccttggccagatggatatttggctaataggacatttggttctgtaggagtcctggtccttctgttcagaatgactggtccagaggctccgtggaaaacatcattaggcaattcttctaaattattattatcgcttagattcagctcatctagttgggttccattgaatgcacagttgtgtatttcttgaatcccattcttattcagccatagaatcacactttcaaagctcagccccacgaaagaatttctttcaattgtgtggatgtttatgttatcttgaatgtcaagtaaaactttttggagagaatgaatcttgtgaacatctggaaggtgcttaatacctgtgttggatattaacagatattgaaggttgggaaggttctggaaggcctcagggttgatgtagagcaggttgttggccttttcaattctaatttcatgtaatttgggaaggttggagaacacatctgcctctatcacctccaagacatcattctgagagatctctattttctccaggtccccaaatcctgaaaatgcacctttttggatgactcgaagcttggtgaggacaaacctcagttcaatggcattcctcgggaggtcagaaggaatctctgtcaccttgctctcttggcagagaaaaaccctgttagagcagtgacagatccgatgatgacatcctgagcccaagctcaggaatgccagcaaagagaccaggagcagggccataattatgcatccatccacctgatttcttcctgcatttgcagagaaaaacctccacagatctcagaagctccacacagtgcccttatgagaagagatct

SEQ ID NO: 17687 - RNA, 11484 nt, Homo sapiens
  source 1..11484: mol_type = other RNA
tcatattgcttctttcttgttgtttattatctgtcttccccaccagaatgcaagctccatttgggcagtggccaccttgtttactgtgtacctgtctgtatccatgaagtctgacataatgcctggcatatattatgagctcaataactattgagtgaatgaaataatgagaaaatcctgtttgatcacttgccagccatataatgctagtcaattttttccacttcagtttctgcatctgtgaaactggataacacaaatgctcaccttgtggcattgttggaataattacctgaaatcatgatgtaaattcatagcataatattggaagtgttagggctcagaatgtgataccccacagtatggtgtcttggtgtgatgagtgctttgaactgaaggaaactgaaagagcttcagaaacaaagtctttctggccttctcccacctttctttctcctgctctcctttcttccccaaggcagaccagagaaactagaattccttttccccaaggtgggtcatagaaaccagagctcttccctaaagacagccataaaacctagacatattactctaacgttcccctgcctttctgtgtaggggctggccataaagaaattctctgacctaacttgtctgatacatgatcatgagaccctcattccagaatgagtcctgccctaaacccaggagaaagagctgccacacagagaggcaaagaagaatgtgaacagacaggtcttgcggggtttcctccctctgcctgctaccattagaccataccctttttgtccaatcaaatttgacacagctgtctgttcttcactgaatctgagcatacaaatggacaattttccttgatatttgggtcttcatttcttaaagctcctgtgacgtgtacaactttgatcaaataaattcgtacgttttctcctattaatctttctctgccaaccctaggcaggttgaggaaactttctctttgacaggcacatcataagagctgaactaatattagctcctttatttcctaagatgaacctctgtctgagtgcatgccagtcagtagaagaaatcagatgggctattcccattttgcctccaatgaatatattgttttgaagaaggtaaatgaatgtgtaaaactccaggcagggcatccttctctctcattgggcacagtgccctgcctggtaaaactgaatttggtaaaaccttctgtgctctcatagtaacttgttcaaatgaccacacagatggaattatgtttacttgtctatttcctgagttggtctgtgtgggggaaggaagatactttactaattttgtaatcctgctgcctagcatggtgcctgcttcctagtgcttagtcatggacattcagtgaaaagtgatatttgagctgagttttatagataaagaaggcatatccagcagacaaatgcagggagggcctaggcagggcacatggcataagcaaaggcatggcagcctaaaaggcaaggcatgctccaggaggaaagttgaggaggttggtagaatagcaagggaggagggagtcggcttctgaaggtgaagatttccgaggtgaggggacgatttctggatatttcaggattgggattgtcgctacaagttacccaggtctattaaagtgtaaagcactgggaacgggtaagtcaaagcattgtgaggctgaggtccagactgggtgatctatgaggatgctgaagtcatcaggaaggtgcagaagtggggaaggagatggcaactgagttaagtgccaagggttctaataaatatggaatgatctgaatggcagagccatagccaaagtgcatgtgtcccaagtgaaggtgacaacactggcctgcaagctgtgctttgaatggttttctcagcagtcggcgagggagaacactgactcatctctacttcttcatgaagaccaccactcacatcttcaggactcaagcaagggtacaaatggaagccctgccctgcagagctccttttctgtgtgtgccctggttgcactgagcatgcattatgccactcagcctgcacctctgagttccatttacacactgcaaacagccatccttaggcctgtagtgtgcacactgtgggtgtaatccaccctcgggtggagagggtcaaggcaaaccttgagtactcaggcaggagattttggggcctcaagtatcagaacatgttcagtgcaaatttgggtgctcatgtgccgttggcctcatgggctcccagattccttgcctatgggtaaggcatggccagaggagggcaagagagagcagggtcctctaaagcatggtgtccaggaaggggaccacatatctgcccttaacttgcttcattacaaaccagcacctaaatgtaaaatgcctgattgcagcagagaaaatagccacggccaggcaatggtcttattctcttccagcaaatggtctcttttagggatgaacaaagacatgcttaaattaaaggttattctcctctggaggaaacaccttagagctgtcaaattctttcttaactacactggctcacagtcaagtttggcccatgagttagggctctcctgagccacagtacatttcattgacttttatttttctctcttcctggcttctgctgagctcaactgcgtgccagtcagggggtgccctgtgcttgggatcaggaggagaaaaggtattacagggaattagaaaaagctctgctcactggatcactgggctttgctttgtgactctattttccttgttcatctgattaaattcacatcatcaaggcttcagcatggacagtgagcatcagctgtgtgagaatacagtccctggtcagctgctggcctggtcttgctgccagaagtgtctgaactaggttgctgcccttattcatgttaaggctggtgtttccaatacctctacttttatgtgaccctgggaagtggacacattcagttgtgacagtcattaaagagacagtccagactggaaccaagggatttgaattctgcgcttattctgtcattgtataggtgcacaacctagagaggtcacttaacctttgaatgctaatttcttcttttataacaaggaaaccctgtcctcctttctacctcacaggaatgttttgaggatctaatgagccaatgcaagccaaagtcttctggaatttgtaaaaaaaacccattgaaatataggagattattatcaccgtggtgtgaaccatgtatcatattctttagaaagtgacagccccacaggagagcagctttgctgtggggtggttggagagatgatggcaggagagaattagagtgagggctgggaaaccaggagagagtggaaaagggggaggattaggtgcagcaagctgttaaaagaaatgaaaagtgactgaaattcaaaatttcctagtgttaaatactaggctaggcaatctacacacacaagctcaattaatacttattacaacctttcaggtgtcttttttttttattcttaatcaccctgcttccacccttttagaaatagagaaattgaaatgatatagcttcctgtacttttttgtcttcatttcttgctactctccctcacccctttttctctgctccagccacaccgatcttgtttttctggagcaaagcaggtttactgtccctgggcttttgcacttgctgttccctttgcctggagcactcttccctcagtatccacacgtctcactttccattccctccaggtctactcaagtcacgttctcagggaggcccccaatgtcgcacatcatatccctcttccctgatttattttttgtcaccagcacttgtcactgcctagcaccaatgcattttactgagtttgtatgtcattggtcacctctactagaatatagagtctccaaggacagaaattttttatttactactttatatccagtgactggaatagtgcttggtttaaagtaggcactcaataaatatttgttgaatgagggaatgcataagtggaaaatagaattgtgtgggcttgttcagagttagtttttgatttctctaggtggctcccagtgatataatttaccccaacaccaaatatttttatagttccaaatactgacccttatctctttggttagactccgtctcactttttgaactagatctgggggccccacaccatggtatgtagagccctgggaaacctagaccatcatgatatgtccattgggcttttctactgggatctaaaactgagctcattcagtgttttgaattgaactctttgcaacaagttggaaaggttttcttaagacaaagataaacaagtatctgcacaaagggacatgatcagggcatggctttctttcacattgcccctttccttgatatttgtcttgccattctctcttttcctcatgtctcctccttcctatcctagtgcatttcttttcttacttctttttcctcttgtctcttttctttctttttttccttttccattcctattcccaaacaggatttcatggacaatgtgtgactccaatggttgcctttagatctgagtagtctctaaggtttgtttcagggagggatggaacagactacatggagaggaggagctgcactgcaggttataatggagggagggtgacagaggaatgaagacaggagatgtgaggtgtaaaggtgccatatgtattctgaccttgaatcccactggcttcatcccatgagagaggatttgggttggctcacgttggaggatgaggttgcctacccattcattccccctcttctagtacctgcttccacattcctgactgacagaacttgcctttcactatagaggctgaatgtggcagaggctcattttgtgacctctcttgcaaccagggcagcagtcctggatagtgaatagaaaggaggctttctcatggcctttaatgagacattctattccctttgaaaagagagatgcacagaagaaaagacatctcttctttgtttctggatttggtcatgtctgcttggggcatctggaactgctatagcaacctactatcatgagggaagacatggctgaagactccaaagatgacagagcaaaaagatggaaaggtcctgggtctttgagatcattgagctgccaatccaagcctggaacattttatataactggccttactgtttaaggcttttttaaaataagagttctgcttcttgccactgaaagcactttgatgagggtcagcaaataccaccttatagttgagctttattttgtgtggacgtttatttagtctctttaatgggttcagttatattttaaacaaacaacacatcctatatatttgtcttctttcttcaatgtcccttagtatgtagtagctgaaagtttattccctgcttgtgcctttacaaactttcctaataaaatactttatgaacctgaaggttgtggccatcagtttcaatgatctttttctgatttttctaatgccatgtgatactgacctaaataaggtgtagtgctgcctgtggtaagagttgcagtatcttagtgatgcaagtgcagggggctttttctcttattctcttcctccctccatttgctcttgcagaaacaaggtatgaagggttccccatgatcagcacatggagacttttagtgaaatagtactctccagtgccccccattccatccccttcaccaaaactaatgcatctgtatgtgacaagataaaaatttttgatcaacttgtgtacctagttcatctcttcactctgacccattcactctggatttatccattcagtcaccttgctccaaccccaccaaggaggatcctaccttgtcagattttcttgggatttagtcaaaggagtatatggaggaaagttggtggagaagggaagacaaaatgagaggctttccaggatggggctgaataaatttatgatgagtgaaaatctgaggaaatagacatgggagcaggtccagtgtgtggtcagggataggaggcaaagatttcattttgcaccaggatggccaaagccaatatccatcatgagagatcagtatttgtattgatattttcagtattacccatggagatatgggtactttaagtaatctctgggagctattgtcctcttcatggtttttgagatttgcaatacaaacttaaaaaatagaaaaaacaaacttgtattaatctgaaacttcgtgcacgcgcgtgcgcgtgtgtgtgtgtgtgtgttccctctgggtcaccactatgggactgaactgccactccaggaggtacaactttaggggtgttacctgtataatcacctttagggggaagagtgatttcaatggtttttattataatacaggaagtgtaggatgtttttctttccctttagatttgtctaaagggtttagaagcactgagtttagctacccataaatatgtttgcttatttgagaaaagtctcatctcttaccaggaagtattatagtgatggaaaaaatgtcttctgagtgtctcttgctgtatatttgtctctgagcacattcttgcctctcagagccatgatttcttaaaccgatgtgtcatcagcagctatgttgtggaataattaatactctatcgtatttttaatttagctgcaacttgcttttgagtccaaattcagaaatacattgcctctggtcaaaaataaggaagatgaatgactgcagatggagctgggacagcccagcagtgcagcaaacgagtgtgtgggggctggggagaaaatgctagctgaaagccctgcatttttgtatagttctagatcagtgccctccaattgaaataaactgcaagccataaatgcaagccacataagtaatttaaaattttcttgtagctacattaaaaaatgtaaaaataaataagtgaaactaatttttaaatgtatttgtcctgatacctccaaaacaatattgtcctagtatgtaatcaataaaataattattgagctattttatgattttttatatgaagtatttggaatcccatgtgtattttacacttacagcacatctaaattcaggctagccacggttcaagtgcccagtagccacatgtggctagcagccactgtgctagacagtaaagctctagactctttacaaggacaattattttattttgcacttgatgctcacagtatatcaaaatggtgccaggtcagatgggaagagacgattgctttttcttctggctctctaaggacttcctccaaaatgcttttgggatcaagtttttaaatgtttgccaaagggtaagaggaggaagggctggcttctgacatagaaagagaagacgcagagctttgtctgctagccaaggcacagagcttggtggaatttatagttgatatttatgaccgaaattatccagatggggtcatttataaaatagatgtgggtagtatggttatttattgagagcaatatgctataatggaatgagttctagactgagggtcaggagagggcactagaccaggcacaggtctgggaggagagaagtgaactaacgtttaccatgccagttacagcactaggctcttcacaaccattttcttatctacttcttacaataagctcaaaagttagctatataaccgtctctagtttacagaaatggcagctgagcctagtgaggtcaggtcctggcttattatggagtcctaataaaatcgcagtgctgtctgattccaaactgctgtgttcttaacattacgatccatatgcatgtcatataataggtgttagggttcaagtagagaagcagaaccagtgatatatttgcatgcatgtaaatatatataggtggtaaatatttgttacaggctcacacagttgtggggagctggttaacctgtctttgtaaggatgtctccacagctgatgccagaactagaagtcctcagggtgggcgatcataaagggaagatcacagcatgctggaagcagcagcacaggtagaactccacaagcacaccctgagccctgcttacattcttgttgcctctgaccttggtgatgaaagtgccgtacagaagttggagcctttatcatggagcttaacaaatatacctggcccaggacgagtctgagaacctgaaggaggatccagggaaaggtggagcaattggagacccagccgttgcttcacagcagtgagctgagtcagcatcagcaacagagtgtgctgagctacaaaatggctgccattttcctctgccctcctgttttcctagagtcctcactatggcccacactaactggaaacacatgaggaagggaaatctgggaaatgtatttcagcctatccacactgacgcattacaaaggcttcagatgggtgttcaattaatatttgttgaatgaatgaatgaatgaataccatggtgcttctctgggaaattctctgggagtcggaatacctaatcctggctctgcctcttacaaactaaacaattttgaacaagtcacttaactctttgagtcgtggtttcctcatttgtaaaactccaagaataatccctgtcctgcttatttaacagggatcacttgagatatctgaacaaaagcactttgaacataacgtgcaaaaataacatatataaggataaaatatgtaatacagtattgcattctttaattattattgttgttactaataattcagcttcctaatgtatcacatggaattaatagttcctgaccaatttaccttaaaggtatgccaggaatattaaattagatgaaatgtgtagaagcactgtcagctctttgtgacatacccttcaaaggcaagactgaattatcattcaatactcagatacattttcacattgtgttttagttttgggctaaatgacttagagggacaagtatgtaagtggaaccactggtgactctgggagctgaagagcagtggccattccttggatgggtgttgtggacagtggatgaagtttctgtcctataaatttgggcttgcatttcatagcagccacacttgctcagcagaatgaagaaatctctgcgaaagtttttggtaaagatggcatagaggaaggggttggcacaggagttgatggggtgaaacagaaccagcagaatctttgctttggacacagtgatgaggggcaccttgagggaggcagaaatggcaaagaaagaaatgggtgccatgcagaggaagtcagtgaagatgagcatggccatgcgcttggcgatcctggtgtcactagaggaggacacgatgttggggttccgcactgtgaggtagatgtggatatagcagccacagatgaccacaaaggccaggacattgagcacaaggagggacatgacatacagctgtgacaaagggctgtcaatatccatgggcaggcagatgctcaccttcatgtagctgctgatgccaaagatgggaaagagggcagctgcaaaagcaaaaatccagcccatcaccatgacactggcagcatggcggagctgcaccttgcagtccagctgcatggcatgcgtgatggtatgccatctttccaaggtgatagctgtcagagtgtagactgacagctcactggcaaagacagtgaaaaagccagcagcatcacagcctgccccagtttgccagtcaatggcatagttgtgatattggctcttggtatggatatcaactgatgcaatgagcagcaggtagattccaatgcagagatcagcaaaggccaggttgcacataaggaacctggggactgtgagtttatattggctggtagttaggatcactagcactatgatgttcccagtgatggccaggatgctgataaaccatatcaggactctgaggatgttgtaccccatgatatcttcacatgggttgaatgcatctggcttaggggagcaggtcacgtcaaccacttcattgcataagtcatagtcaaactcagtgtacgtcatgtcaaatcctctgctgtagctggactcattgtcttctgccagagaggatctctgacccctagcctgagtcatataatcaacttcttgccttaaaatagatttgttgcaaattggatgaagctcagagatttgccgtctccagtttgcaaaggcacagcaatggctgggataggtgaggctggcttccatgagggcgacaagcttttccagagtaggcagcttttttaagttgtaagtcgacctggccctcagcttcttaagattttctaagccatagctaggcagggaatggatccttgttcttgaaatatctatggatgaggagagagactccggttcctccaacacaccttggccagatggatatttggctaataggacatttggttctgtaggagtcctggtccttctgttcagaatgactggtccagaggctccgtggaaaacatcattaggcaattcttctaaattattattatcgcttagattcagctcatctagttgggttccattgaatgcacagttgtgtatttcttgaatcccattcttattcagccatagaatcacactttcaaagctcagccccacgaaagaatttctttcaattgtgtggatgtttatgttatcttgaatgtcaagtaaaactttttggagagaatgaatcttgtgaacatctggaaggtgcttaatacctgtgttggatattaacctgtttccaatccgcattttcagatatgctattattatcatgggctagggatatctatgtgaagagctggttttcttcttgggtttgtccttggcaggagtgctttgcattagccatatgtgatagtttatgaatgaaagtgtctctggggatgcctcttcatgtcctagagagcatttgttctgtcactgaaggctctatgatccccattttccactttggcattctccaaaacaaaagaagagaaggatagatattgaaggttgggaaggttctggaaggcctcagggttgatgtagagcaggttgttggccttttcaattctaatttcatgtaatttgggaaggttggagaacacatctgcctctatcacctccaagacatcattctgagagatctctattttctccaggtccccaaatcctgaaaatgcacctttttggatgactcgaagcttggtgaggacaaacctcagttcaatggcattcctcgggaggtcagaaggaatctctgtcaccttgctctcttggcagagaaaaaccctgttagagcagtgacagatccgatgatgacatcctgagcccaagctcaggaatgccagcaaagagaccaggagcagggccataattatgcatccatccacctgatttcttcctgcatttgcagagaaaaacctccacagatctcagaagctccacacagtgcccttatgagaagagatctgacttgagaact

SEQ ID NO: 17688 - RNA, 10814 nt, Homo sapiens
  source 1..10814: mol_type = other RNA
tcatattgcttctttcttgttgtttattatctgtcttccccaccagaatgcaagctccatttgggcagtggccaccttgtttactgtgtacctgtctgtatccatgaagtctgacataatgcctggcatatattatgagctcaataactattgagtgaatgaaataatgagaaaatcctgtttgatcacttgccagccatataatgctagtcaattttttccacttcagtttctgcatctgtgaaactggataacacaaatgctcaccttgtggcattgttggaataattacctgaaatcatgatgtaaattcatagcataatattggaagtgttagggctcagaatgtgataccccacagtatggtgtcttggtgtgatgagtgctttgaactgaaggaaactgaaagagcttcagaaacaaagtctttctggccttctcccacctttctttctcctgctctcctttcttccccaaggcagaccagagaaactagaattccttttccccaaggtgggtcatagaaaccagagctcttccctaaagacagccataaaacctagacatattactctaacgttcccctgcctttctgtgtaggggctggccataaagaaattctctgacctaacttgtctgatacatgatcatgagaccctcattccagaatgagtcctgccctaaacccaggagaaagagctgccacacagagaggcaaagaagaatgtgaacagacaggtcttgcggggtttcctccctctgcctgctaccattagaccataccctttttgtccaatcaaatttgacacagctgtctgttcttcactgaatctgagcatacaaatggacaattttccttgatatttgggtcttcatttcttaaagctcctgtgacgtgtacaactttgatcaaataaattcgtacgttttctcctattaatctttctctgccaaccctaggcaggttgaggaaactttctctttgacaggcacatcataagagctgaactaatattagctcctttatttcctaagatgaacctctgtctgagtgcatgccagtcagtagaagaaatcagatgggctattcccattttgcctccaatgaatatattgttttgaagaaggtaaatgaatgtgtaaaactccaggcagggcatccttctctctcattgggcacagtgccctgcctggtaaaactgaatttggtaaaaccttctgtgctctcatagtaacttgttcaaatgaccacacagatggaattatgtttacttgtctatttcctgagttggtctgtgtgggggaaggaagatactttactaattttgtaatcctgctgcctagcatggtgcctgcttcctagtgcttagtcatggacattcagtgaaaagtgatatttgagctgagttttatagataaagaaggcatatccagcagacaaatgcagggagggcctaggcagggcacatggcataagcaaaggcatggcagcctaaaaggcaaggcatgctccaggaggaaagttgaggaggttggtagaatagcaagggaggagggagtcggcttctgaaggtgaagatttccgaggtgaggggacgatttctggatatttcaggattgggattgtcgctacaagttacccaggtctattaaagtgtaaagcactgggaacgggtaagtcaaagcattgtgaggctgaggtccagactgggtgatctatgaggatgctgaagtcatcaggaaggtgcagaagtggggaaggagatggcaactgagttaagtgccaagggttctaataaatatggaatgatctgaatggcagagccatagccaaagtgcatgtgtcccaagtgaaggtgacaacactggcctgcaagctgtgctttgaatggttttctcagcagtcggcgagggagaacactgactcatctctacttcttcatgaagaccaccactcacatcttcaggactcaagcaagggtacaaatggaagccctgccctgcagagctccttttctgtgtgtgccctggttgcactgagcatgcattatgccactcagcctgcacctctgagttccatttacacactgcaaacagccatccttaggcctgtagtgtgcacactgtgggtgtaatccaccctcgggtggagagggtcaaggcaaaccttgagtactcaggcaggagattttggggcctcaagtatcagaacatgttcagtgcaaatttgggtgctcatgtgccgttggcctcatgggctcccagattccttgcctatgggtaaggcatggccagaggagggcaagagagagcagggtcctctaaagcatggtgtccaggaaggggaccacatatctgcccttaacttgcttcattacaaaccagcacctaaatgtaaaatgcctgattgcagcagagaaaatagccacggccaggcaatggtcttattctcttccagcaaatggtctcttttagggatgaacaaagacatgcttaaattaaaggttattctcctctggaggaaacaccttagagctgtcaaattctttcttaactacactggctcacagtcaagtttggcccatgagttagggctctcctgagccacagtacatttcattgacttttatttttctctcttcctggcttctgctgagctcaactgcgtgccagtcagggggtgccctgtgcttgggatcaggaggagaaaaggtattacagggaattagaaaaagctctgctcactggatcactgggctttgctttgtgactctattttccttgttcatctgattaaattcacatcatcaaggcttcagcatggacagtgagcatcagctgtgtgagaatacagtccctggtcagctgctggcctggtcttgctgccagaagtgtctgaactaggttgctgcccttattcatgttaaggctggtgtttccaatacctctacttttatgtgaccctgggaagtggacacattcagttgtgacagtcattaaagagacagtccagactggaaccaagggatttgaattctgcgcttattctgtcattgtataggtgcacaacctagagaggtcacttaacctttgaatgctaatttcttcttttataacaaggaaaccctgtcctcctttctacctcacaggaatgttttgaggatctaatgagccaatgcaagccaaagtcttctggaatttgtaaaaaaaacccattgaaatataggagattattatcaccgtggtgtgaaccatgtatcatattctttagaaagtgacagccccacaggagagcagctttgctgtggggtggttggagagatgatggcaggagagaattagagtgagggctgggaaaccaggagagagtggaaaagggggaggattaggtgcagcaagctgttaaaagaaatgaaaagtgactgaaattcaaaatttcctagtgttaaatactaggctaggcaatctacacacacaagctcaattaatacttattacaacctttcaggtgtcttttttttttattcttaatcaccctgcttccacccttttagaaatagagaaattgaaatgatatagcttcctgtacttttttgtcttcatttcttgctactctccctcacccctttttctctgctccagccacaccgatcttgtttttctggagcaaagcaggtttactgtccctgggcttttgcacttgctgttccctttgcctggagcactcttccctcagtatccacacgtctcactttccattccctccaggtctactcaagtcacgttctcagggaggcccccaatgtcgcacatcatatccctcttccctgatttattttttgtcaccagcacttgtcactgcctagcaccaatgcattttactgagtttgtatgtcattggtcacctctactagaatatagagtctccaaggacagaaattttttatttactactttatatccagtgactggaatagtgcttggtttaaagtaggcactcaataaatatttgttgaatgagggaatgcataagtggaaaatagaattgtgtgggcttgttcagagttagtttttgatttctctaggtggctcccagtgatataatttaccccaacaccaaatatttttatagttccaaatactgacccttatctctttggttagactccgtctcactttttgaactagatctgggggccccacaccatggtatgtagagccctgggaaacctagaccatcatgatatgtccattgggcttttctactgggatctaaaactgagctcattcagtgttttgaattgaactctttgcaacaagttggaaaggttttcttaagacaaagataaacaagtatctgcacaaagggacatgatcagggcatggctttctttcacattgcccctttccttgatatttgtcttgccattctctcttttcctcatgtctcctccttcctatcctagtgcatttcttttcttacttctttttcctcttgtctcttttctttctttttttccttttccattcctattcccaaacaggatttcatggacaatgtgtgactccaatggttgcctttagatctgagtagtctctaaggtttgtttcagggagggatggaacagactacatggagaggaggagctgcactgcaggttataatggagggagggtgacagaggaatgaagacaggagatgtgaggtgtaaaggtgccatatgtattctgaccttgaatcccactggcttcatcccatgagagaggatttgggttggctcacgttggaggatgaggttgcctacccattcattccccctcttctagtacctgcttccacattcctgactgacagaacttgcctttcactatagaggctgaatgtggcagaggctcattttgtgacctctcttgcaaccagggcagcagtcctggatagtgaatagaaaggaggctttctcatggcctttaatgagacattctattccctttgaaaagagagatgcacagaagaaaagacatctcttctttgtttctggatttggtcatgtctgcttggggcatctggaactgctatagcaacctactatcatgagggaagacatggctgaagactccaaagatgacagagcaaaaagatggaaaggtcctgggtctttgagatcattgagctgccaatccaagcctggaacattttatataactggccttactgtttaaggcttttttaaaataagagttctgcttcttgccactgaaagcactttgatgagggtcagcaaataccaccttatagttgagctttattttgtgtggacgtttatttagtctctttaatgggttcagttatattttaaacaaacaacacatcctatatatttgtcttctttcttcaatgtcccttagtatgtagtagctgaaagtttattccctgcttgtgcctttacaaactttcctaataaaatactttatgaacctgaaggttgtggccatcagtttcaatgatctttttctgatttttctaatgccatgtgatactgacctaaataaggtgtagtgctgcctgtggtaagagttgcagtatcttagtgatgcaagtgcagggggctttttctcttattctcttcctccctccatttgctcttgcagaaacaaggtatgaagggttccccatgatcagcacatggagacttttagtgaaatagtactctccagtgccccccattccatccccttcaccaaaactaatgcatctgtatgtgacaagataaaaatttttgatcaacttgtgtacctagttcatctcttcactctgacccattcactctggatttatccattcagtcaccttgctccaaccccaccaaggaggatcctaccttgtcagattttcttgggatttagtcaaaggagtatatggaggaaagttggtggagaagggaagacaaaatgagaggctttccaggatggggctgaataaatttatgatgagtgaaaatctgaggaaatagacatgggagcaggtccagtgtgtggtcagggataggaggcaaagatttcattttgcaccaggatggccaaagccaatatccatcatgagagatcagtatttgtattgatattttcagtattacccatggagatatgggtactttaagtaatctctgggagctattgtcctcttcatggtttttgagatttgcaatacaaacttaaaaaatagaaaaaacaaacttgtattaatctgaaacttcgtgcacgcgcgtgcgcgtgtgtgtgtgtgtgtgttccctctgggtcaccactatgggactgaactgccactccaggaggtacaactttaggggtgttacctgtataatcacctttagggggaagagtgatttcaatggtttttattataatacaggaagtgtaggatgtttttctttccctttagatttgtctaaagggtttagaagcactgagtttagctacccataaatatgtttgcttatttgagaaaagtctcatctcttaccaggaagtattatagtgatggaaaaaatgtcttctgagtgtctcttgctgtatatttgtctctgagcacattcttgcctctcagagccatgatttcttaaaccgatgtgtcatcagcagctatgttgtggaataattaatactctatcgtatttttaatttagctgcaacttgcttttgagtccaaattcagaaatacattgcctctggtcaaaaataaggaagatgaatgactgcagatggagctgggacagcccagcagtgcagcaaacgagtgtgtgggggctggggagaaaatgctagctgaaagccctgcatttttgtatagttctagatcagtgccctccaattgaaataaactgcaagccataaatgcaagccacataagtaatttaaaattttcttgtagctacattaaaaaatgtaaaaataaataagtgaaactaatttttaaatgtatttgtcctgatacctccaaaacaatattgtcctagtatgtaatcaataaaataattattgagctattttatgattttttatatgaagtatttggaatcccatgtgtattttacacttacagcacatctaaattcaggctagccacggttcaagtgcccagtagccacatgtggctagcagccactgtgctagacagtaaagctctagactctttacaaggacaattattttattttgcacttgatgctcacagtatatcaaaatggtgccaggtcagatgggaagagacgattgctttttcttctggctctctaaggacttcctccaaaatgcttttgggatcaagtttttaaatgtttgccaaagggtaagaggaggaagggctggcttctgacatagaaagagaagacgcagagctttgtctgctagccaaggcacagagcttggtggaatttatagttgatatttatgaccgaaattatccagatggggtcatttataaaatagatgtgggtagtatggttatttattgagagcaatatgctataatggaatgagttctagactgagggtcaggagagggcactagaccaggcacaggtctgggaggagagaagtgaactaacgtttaccatgccagttacagcactaggctcttcacaaccattttcttatctacttcttacaataagctcaaaagttagctatataaccgtctctagtttacagaaatggcagctgagcctagtgaggtcaggtcctggcttattatggagtcctaataaaatcgcagtgctgtctgattccaaactgctgtgttcttaacattacgatccatatgcatgtcatataataggtgttagggttcaagtagagaagcagaaccagtgatatatttgcatgcatgtaaatatatataggtggtaaatatttgttacaggctcacacagttgtggggagctggttaacctgtctttgtaaggatgtctccacagctgatgccagaactagaagtcctcagggtgggcgatcataaagggaagatcacagcatgctggaagcagcagcacaggtagaactccacaagcacaccctgagccctgcttacattcttgttgcctctgaccttggtgatgaaagtgccgtacagaagttggagcctttatcatggagcttaacaaatatacctggcccaggacgagtctgagaacctgaaggaggatccagggaaaggtggagcaattggagacccagccgttgcttcacagcagtgagctgagtcagcatcagcaacagagtgtgctgagctacaaaatggctgccattttcctctgccctcctgttttcctagagtcctcactatggcccacactaactggaaacacatgaggaagggaaatctgggaaatgtatttcagcctatccacactgacgcattacaaaggcttcagatgggtgttcaattaatatttgttgaatgaatgaatgaatgaataccatggtgcttctctgggaaattctctgggagtcggaatacctaatcctggctctgcctcttacaaactaaacaattttgaacaagtcacttaactctttgagtcgtggtttcctcatttgtaaaactccaagaataatccctgtcctgcttatttaacagggatcacttgagatatctgaacaaaagcactttgaacataacgtgcaaaaataacatatataaggataaaatatgtaatacagtattgcattctttaattattattgttgttactaataattcagcttcctaatgtatcacatggaattaatagttcctgaccaatttaccttaaaggtatgccaggaatattaaattagatgaaatgtgtagaagcactgtcagctctttgtgacatacccttcaaaggcaagactgaattatcattcaatactcagatacattttcacattgtgttttagttttgggctaaatgacttagagggacaagtatgtaagtggaaccactggtgactctgggagctgaagagcagtggccattccttggatgggtgttgtggacagtggatgaagtttctgtcctataaatttgggcttgcatttcatagcagccacacttgctcagcagaatgaagaaatctctgcgaaagtttttggtaaagatggcatagaggaaggggttggcacaggagttgatggggtgaaacagaaccagcagaatctttgctttggacacagtgatgaggggcaccttgagggaggcagaaatggcaaagaaagaaatgggtgccatgcagaggaagtcagtgaagatgagcatggccatgcgcttggcgatcctggtgtcactagaggaggacacgatgttggggttccgcactgtgaggtagatgtggatatagcagccacagatgaccacaaaggccaggacattgagcacaaggagggacatgacatacagctgtgacaaagggctgtcaatatccatgggcaggcagatgctcaccttcatgtagctgctgatgccaaagatgggaaagagggcagctgcaaaagcaaaaatccagcccatcaccatgacactggcagcatggcggagctgcaccttgcagtccagctgcatggcatgcgtgatggtatgccatctttccaaggtgatagctgtcagagtgtagactgacagctcactggcaaagacagtgaaaaagccagcagcatcacagcctgccccagtttgccagtcaatggcatagttgtgatattggctcttggtatggatatcaactgatgcaatgagcagcaggtagattccaatgcagagatcagcaaaggccaggttgcacataaggaacctggggactgtgagtttatattggctggtagttaggatcactagcactatgatgttcccagtgatggccaggatgctgataaaccatatcaggactctgaggatgttgtaccccatgatatcttcacatgggttgaatgcatctggcttaggggagcaggtcacgtcaaccacttcattgcataagtcatagtcaaactcagtgtacgtcatgtcaaatcctctgctgtagctggactcattgtcttctgccagagaggatctctgacccctagcctgagtcatataatcaacttcttgccttaaaatagatttgttgcaaattggatgaagctcagagatttgccgtctccagtttgcaaaggcacagcaatggctgggataggtgaggctggcttccatgagggcgacaagcttttccagagtaggcagcttttttaagttgtaagtcgacctggccctcagcttcttaagattttctaagccatagctaggcagggaatggatccttgttcttgaaatatctatggatgaggagagagactccggttcctccaacacaccttggccagatggatatttggctaataggacatttggttctgtaggagtcctggtccttctgttcagaatgactggtccagaggctccgtggaaaacatcattaggcaattcttctaaattattattatcgcttagattcagctcatctagttgggttccattgaatgcacagttgtgtatttcttgaatcccattcttattcagccatagaatcacactttcaaagctcagccccacgaaagaatttctttcaattgtgtggatgtttatgttatcttgaatgtcaagtaaaactttttggagagaatgaatcttgtgaacatctggaaggtgcttaatacctgtgttggatattaaccttttcagagtctcagtttctctctgtaaaatgattttgtgtaagaaattatgtgagacagtagg

SEQ ID NO: 17689 - RNA, 843 nt, Homo sapiens
  source 1..843: mol_type = other RNA
tccactctcctggcccccagccacacctagccccacctggccctggactttcacttgctagcaaaaaaggcccctacagttaccagggcccccagtgccacggcccccgtcagcactgtcctcactgatgcccagttcccctcccgcagacgccgcgcctcctccagggccccgtccccgtatagagctgtgaactccgcccagcccccactgctgtggatccagtcagccagctgcgtctccaggtaggccaccatccactcctgcacttgtcccaccagtggttccatctccttgttgacactctcagcacacagtgcagccccaaagacaaagaaggctacaaggcggccccagttggggcccccttgaaaaagttcatcggagacctgggtgaagcgttgttgggctgagcctggggtcacatgcagctgagccgccagatcagagaaggtgcgccggaagcgggtctcgaactcatctccagctgcccgcatggcttggtgcagcgggtcagctgctgggccctccccggggccagctccacagacataacccttctgcctcagcttataacctacaaagtctgccaccagagcccgtgtgtctggggccgaggctggggtcgccatccgggcggccagccgggatggcagctcttaagacacagcactggtggcaaggagcccccagctggggcctttcatcctcctggccagcgtggagccccccacctcagccagtctccaaccccgcccgcctgccaggttagggatctcacgggtcaggccgctgccgggatccgggccgtttcctggtgcaggagctgggagggagggagag

SEQ ID NO: 17690 - RNA, 790 nt, Homo sapiens
  source 1..790: mol_type = other RNA
tccactctcctggcccccagccacacctagccccacctggccctggactttcacttgctagcaaaaaaggcccctacagttaccagggcccccagtgccacggcccccgtcagcactgtcctcactgatgcccagttcccctcccgcagacgccgcgcctcctccagggccccgtccccgtatagagctgtgaactccgcccagcccccactgctgtggatccagtcagccagctgcgtctccaggtaggccaccatccactcctgcacttgtcccaccagtggttccatctccttgttgacactctcagcacacagtgcagccccaaagacaaagaaggctacaaggcggccccagttggggcccccttgaaaaagttcatcggagacctgggtgaagcgttgttgggctgagcctggggtcacatgcagctgagccgccagatcagagaaggtgcgccggaagcgggtctcgaactcatctccagctgcccgcatggcttggtgcagcgggtcagctgctgggccctccccggggccagctccacagacataacccttctgcctcagcttataacctacaaagtctgccaccagagcccgtgtgtctggggccgaggctggggtcgccatccgggcggccagccgggatggcagctcttaagacacagcactggtggcaaggagcccccagctggggcctttcatcctcctggccagcgtggagccgggtcaggccgctgccgggatccgggccgtttcctggtgcaggagctgggagggagggagag

SEQ ID NO: 17691 - RNA, 32 nt, Homo sapiens
  source 1..32: mol_type = other RNA
tccagcatcagtgattttgttgaagagggcag

SEQ ID NO: 17692 - RNA, 1698 nt, Homo sapiens
  source 1..1698: mol_type = other RNA
tccagctcggtggcacatgatgaccacaaagccgatggctcagagctggtcacatcccttggaactgagtggcttgtggggccagccatcccagaagagggtggagtggagggaaggacaccactcagaatactgagcaaatccccacactgcgagagatcccggggcctccaatagagaagagcaaggtcctgacttccacactgcccgacacaacagcctttgcaggcaggtgtcccttggtagcctacgggctgtcttatgtcagctgcttaactagggcgtgccggggaagtaaatgatctcactgacactttgctccacatataaaataagtcacttaccccagttcttcacagaaggtcaccagggcatcaaaggccatgatagtggctttatcagatgctttgtttcctctcttttcctggagttttgctacttccttcctgatcaggaagctgacttggtcccggtcattcctggagtaatagagacggcaccaggaaggcttcccatccctgccagcccggccagactcctggtagtacccagccatagacttggcaatattccaatgggcgacaaacctgacattggctttatccactcccatcccaaaactaatggttgcaacaattacagggaccttctcctccatccagtcgttctgcaccagcgttctttcagaggccttcagccctgcatggtaagccttggcgttcacacccctgcagctgagctctatggccagctgttcacaagcctctctagtcctgcagtacacaatgccgcagccagataaccctttatcagcctcctgtccaagagccttaaggcagaagtccttcaggttcccatagggatcagaaatcagttccttgaattgcacatcatagaagaggttggcccggaagcagggagtcttgaagatggcaactggtttcttcaggtgcagggcagcaaacacgtcctcttggacctgtggggtggctgtggcggtcagagccacacaaggggcatgtcccaggcgggagcgcagggcacccagacgcaagtagtcaggacgaaagtcatgcccccattgggaaacacaatgagcttcatccaccaccaagtaagacagcaggtggcgggacaccagggagttcagggtgggctggaaggaggatgaagctgccatctctggggtgatgtacagaatcttggtctggggcttttctcgctccaggtcagcaagcagctccttcctttcctgtgcagagagcttcgagttcagggaacttactcgtacctttagggttagcaagtggtccacttggtcctgaatcaaagcaatgagaggagagactacaatggtgatgcctttggccaacagagcagggagctgatagcatagggattttcctgcccctgtgggcatgcacacaaagacgtccttgttaccttttactacagccatggtcgcactctcctgtaaaggcgtcttaaaagagtcaaacccaaagaccttcttcagcgtactccggactcgccgctcagggtcaaaaggaaaggtggtatggtggctgctcatcttagccaagaacacagaaccggccgtggtccgcccaagaattaaaggctgctggctggttccggaactgttcgaagacccctatacacaaccccaactcagagaagccaaagcgctgggaattc

SEQ ID NO: 17693 - RNA, 76 nt, Homo sapiens
  source 1..76: mol_type = other RNA
tccagtacaggtctctcatttcaaagtagtattcctaatcatgaaggaaatgagagacctgtactggaatcctgtc

SEQ ID NO: 17694 - RNA, 2177 nt, Homo sapiens
  source 1..2177: mol_type = other RNA
tccagtacaggtctctcatttcagcctcccaagtagctgagactatgggtgtgggccactgtgcccagtttaggaggtaaagtcttggccaggcatgaaacagtgttcctctgaatctctaacctcatgagaaaaccatttcagcttggaaaacactacataggaaatccccttcttaaagatggacaaaacatgttagcatataagaagttctcagaagttctgcattatgaagaacaaatgtgacttgatttaaatctagcctttctcaaacgcatcagggcacagacaccagttttgggcataacaactatttctttggcatggaatggctgttttgcaaaaacatcctttggaaagcgctgctctggctgggctatttttaattaattataacagcctgaaagacttcagtcaaagtaaatattatgaaaagaagtcaactaattccttccaaacaaataatctaacattatccaatctccttaaattttaattatttgattatttttgttcagagaggaggacctaaagatagtattttttaaagcctgtaagttgacaaatcaaatgctgagaattttattcttaaattaacaacaaaaggatgacttcaaacagtacatgctgtttgtagatgggtggctttcggtaaatgttgattccttgatctggaacatggaaatgtttaggggcctgagcgtaagttggagttagagggcggctgtctggccggtaagggagaggggagttccggccgctggacggctcattgcctttgatatggggaatgaagtggtgtcggaaaggggggttggggcgggagtcgctgtgggtggggctgaggctgctggtgcgcaggtacgacaacctctgcacaccaggagacaaaagctcaggtctgtggaaatgctggggagagcgggacgtggttggagtgtagctgtggcggctgtacacaggggagttgatggagccctggctcgtggaccgatggatcatccgatcccgaacatcctggtacccttctgctgatggagtaggagacaaagtcctcggagactctccaaggctctgtctctcctgtttgtcatcatagcccgaagtgtagaaaggctcataggtaataagatctggacgttcaatgtcataaattgccttgaccttcggaatggctgctaaatccttgtaatccaggatctcattgtctacttttgcatagatagtatgacctggtgagccaggaatactggagcctggcctagaataaatactttccgaggatgtcctggtaggctgcagagacggagaccgtcctgtgcgtcgaatcagacttttggaataaaagaaatcggatgaagaacgccgaatgtttggcagccgcagcttttcctcggtcttcgtagattgcttacagtcgggatgccaaacggtggagccttgaagatacatttcctctccttctgtgaacatctggttgcatctgctgcatcgtgcacagctggggtggtaatgtttgtcacctgcctccaggactttccctgtgataaactggtgacacgcctcacatttcaccccaaagagtccctggtagtccttttcacagtacggagcaccatccttgctgatgtactccccggtgaggaccttcccgcaggacttgcatttaaagcaccccaagtgccactgcttatccagcgccagcagcgcctgcccattcttgatatctcttccgcagccggcacaattgctggagaaggtggtttctttcggactggacgacatcggctgtgcacagagttgacaaaggcagtctctcccattgaatgtgactcggtctccgggtggaaacgggcgcttgcagatagtacaagcaaagcaattgggatggtaggtcttgcccagagcagtcaccacttcgccctccacgaactccccacagccatggcagcgtgtcccgtacatccgctggtagtccagggtgcagagatactctccgttctttatgaagaagcccccttgtgccaggtcacagccacacactttgcaggtgaaacacttgatgtggaaatgtttggtctggacccgaagcacttcacccttgcaaggctccccacatttatggcagtgaatgacaggcttctctgatgggtggtgagggtcctgagggtgggcca

SEQ ID NO: 17695 - RNA, 903 nt, Homo sapiens
  source 1..903: mol_type = other RNA
tccagtgccctcctctccaggccgccggtggtagaccagctctccacccagggccaggcaaggcgtgatgctctggaggtagtgggctacgaggattcctgaacccacgaggacgtctgggttccccagggtgacggctgctgtgaagtcagagccccgatactccccgtccacctgccagttcacaaacttcgactgctgggtctggatggccatcttggacctgagaccggggcccagctggtgaatgacctgagcgttgagactgccactgttgtccatgtcacccaccagtacagggaacgcctctgtgggactcagctgctttgtccccacatatgtgaccccgaagtggtagttggactccccgattgtgctgagggctactgtgtggttgacctgaaaatggttactcaaccctttgttgactgtgagcttgacaccctccatctgaatgggaaacagctccttgcacttccggtggcactcctcgaatgtgcccgggttgggcaggcagccgcaggccccatcctcggcggcccctgaggcgctggcggttgcagccccgggggtccgttccgaacttcgactcgtactggtgccggcgcccaggctgcctcccagcggcggcagcgtgaagcccggcggcgagggcggaggtggcggcagccccacgagggccggcgcaggcggcggtggcggccctgcgggcggcgagctggcagccaacacgttccccatggtcgcctgctaggggagaggtcagagggcagaggtcagggcccgcgcgcccccgactcagccccagcaaatccgcacccggctccggccccggttctcactggcggcggcgcctgctcccggcctgggctccgctcccaccccgtgcgccacgcgcaaccg

SEQ ID NO: 17696 - RNA, 811 nt, Homo sapiens
  source 1..811: mol_type = other RNA
tccagtgccctcctctccaggccgccggtggtagaccagctctccacccagggccaggcaaggcgtgatgctctggaggtagtgggctacgaggattcctgaacccacgaggacgtctgggttccccagggtgacggctgctgtgaagtcagagccccgatactccccgtccacctgccagttcacaaacttcgactgctgggtctggatggccatcttggacctgagaccggggcccagctggtgaatgacctgagcgttgagactgccactgttgtccatgtcacccaccagtacagggaacgcctctgtgggactcagctgctttgtccccacatatgtgaccccgaagtggtagttggactccccgattgtgctgagggctactgtgtggttgacctgaaaatggttactcaaccctttgttgactgtgagcttgacaccctccatctgaatgggaaacagctccttgcacttccggtggcactcctcgaatgtgcccgggttgggcaggcagccgcaggccccatcctcggcggcccctgaggcgctggcggttgcagccccgggggtccgttccgaacttcgactcgtactggtgccggcgcccaggctgcctcccagcggcggcagcgtgaagcccggcggcgagggcggaggtggcggcagccccacgagggccggcgcaggcggcggtggcggccctgcgggcggcgagctggcagccaacacgttccccatggtcgcctgtggcggcggcgcctgctcccggcctgggctccgctcccaccccgtgcgccacgcgcaaccg

SEQ ID NO: 17697 - RNA, 839 nt, Homo sapiens
  source 1..839: mol_type = other RNA
tccagtgccctcctctccaggccgccggtggtagaccagctctccacccagggccaggcaaggcgtgatgctctggaggtagtgggctacgaggattcctgaacccacgaggacgtctgggttccccagggtgacggctgctgtgaagtcagagccccgatactccccgtccacctgccagttcacaaacttcgactgctgggtctggatggccatcttggacctgagaccggggcccagctggtgaatgacctgagcgttgagactgccactgttgtccatgtcacccaccagtacagggaacgcctctgtgggactcagctgctttgtccccacatatgtgaccccgaagtggtagttggactccccgattgtgctgagggctactgtgtggttgacctgaaaatggttactcaaccctttgttgactgtgagcttgacaccctccatctgaatgggaaacagctccttgcacttccggtggcactcctcgaatgtgcccgggttgggcaggcagccgcaggccccatcctcggcggcccctgaggcgctggcggttgcagccccgggggtccgttccgaacttcgactcgtactggtgccggcgcccaggctgcctcccagcggcggcagcgtgaagcccggcggcgagggcggaggtggcggcagccccacgagggccggcgcaggcggcggtggcggccctgcgggcggcgagctggcagccaacacgttccccatggtcgcctgtggcggcggcgcctgctcccggcctgggctccgctcccaccccgtgcgccacgcgcaaccgaacccgctgccgccgccgccaccaccgt

SEQ ID NO: 17698 - RNA, 808 nt, Homo sapiens
  source 1..808: mol_type = other RNA
tccagtgccctcctctccaggccgccggtggtagaccagctctccacccagggccaggcaaggcgtgatgctctggaggtagtgggctacgaggattcctgaacccacgaggacgtctgggttccccagggtgacggctgctgtgaagtcagagccccgatactccccgtccacctgccagttcacaaacttcgactgctgggtctggatggccatcttggacctgagaccggggcccagctggtgaatgacctgagcgttgagactgccactgttgtccatgtcacccaccagtacagggaacgcctctgtgggactcagctgctttgtccccacatatgtgaccccgaagtggtagttggactccccgattgtgctgagggctactgtgtggttgacctgaaaatggttactcaaccctttgttgactgtgagcttgacaccctccatctgaatgggaaacagctccttgcacttccggtggcactcctcgaatgtgcccgggttgggcaggcagccgcaggccccatcctcggcggcccctgaggcgctggcggttgcagccccgggggtccgttccgaacttcgactcgtactggtgccggcgcccaggctgcctcccagcggcggcagcgtgaagcccggcggcgagggcggaggtggcggcagccccacgagggccggcgcaggcggcggtggcggccctgcgggcggcgagctggcagccaacacgttccccatggtcgctggcggcggcgcctgctcccggcctgggctccgctcccaccccgtgcgccacgcgcaaccg

SEQ ID NO: 17699 - RNA, 758 nt, Homo sapiens
  source 1..758: mol_type = other RNA
tccatgtttccttcccccttctcctcgaaaagcctgttcatctgtggcgtggggactgtcattagtgagcactgactaaggtaggctggacaaggatgcagcctacaagccgcgtggcatcttttccttccctgtggacctctggggtgattcccttgtctctgtctctgctcctcagaaacgcccctatcaggctgtgcgcggtggctcacgcctgtaatcccagcactctggaggctgaggtgggcagatcacttgaggtcaggagtttgagaccagcctggccaacatggtgaaacccctgttaaaaatacaaaaaattagctgggcgtggtggcatgcacctctaatcccagctactcgggaggctgaggcaggagacgcacttgaacccagcagaggttgcagtgagccgagatagcaccaccgtactccatgctgggcaacagagcgagactccatcaaaaaacaagaaaaaaagaaaagccgcaatctgtgtgtcctgcctccccccaggaccaggcctgccaggcagcagtgggagttgacctttcagcagatccacaaactgaaagttgaactggatgtcatgcttcttcgagaagatgtagacggcacggcagggtgctgacagcaggtccatgtagagctccagtgccatgttgagacacatgccaggccccacagccgcagttggccagccacagacctgggcctatgtctggccagagtccctggccctgtgccctctccgatct

SEQ ID NO: 17700 - RNA, 8797 nt, Homo sapiens
  source 1..8797: mol_type = other RNA
tccatgtttccttcccccttctttgccttgggctttctttttcgtttcttctttttatcttctttttcaaaattttttggtgttttctcagtggaacatcatgggataacgtgtgtgtgtgcatgtatgtgtatgcatttatggggatggggagctgggaattcagtgaggaaaaggaagatagaaccaaggatatattttgtgtgtggtaggcagacatgtatgaataatcagggtgccaagatgggtgtatgtgtctgtgaagatgggcaagggctacatctgcaaggagctgaggaggaggatcaatgtgtgtgtctgtggggattgggaggaggcaggactctgctggaagtggggtgtgtggtgcccactgagggtgggaactgaacagttcctgtgaggtgggcggggccagggggtggggtgagggatttgagctcccaccgaacaccccttggggtaaaagagggagccctgaggccctcccctctccccatcttggttaatctgtttataaagctagaagtgtagaggtagtcgtagtttttgggttggagtccgtgtgaggtaatcttgcttcctctttggcaaaagccacagcagccgaggcagcagtggcggcgttggtgatggagatgggtgggcccccttgaggtggggctgccttgcgcctgtgggccgaggagcgcaggtgggaggctagggcttcacgcccactcagcagcacctcacatgccaggcagtggtaggtgcagatgggcacccgcaatgggggtggcatggagcccccagagccccgcccaaagaagcagaaggatctctggtgggcagtagccggggcctccccgtcaaatgccatcttgcactggcggcacaggtagcgatgggttacatccacggtggagatgccagtgctgcctgtcagcagctcatcaacctcaccagcttccccctcccctggagcaggcagttcaggaggctttggaggtgctgtggctgtgggctcagggggctggggtggcggctggaggagggcattggggagcagcccaatgagggtctgaggtatcatggggttcatgggaaatagccccttcttcatgccatagagctgttggaagtaggccccctgtagctgggggccaaagacagctggcggtgctgttcccccagcagggggcaatggaaagggcaggaactggccccccaacagggctgggacagtggtcttcaatgctttgaggttcttgagggcatcattggaggagctggtggggcctgcaactggctttcgctcactggagaccttgtcccccaagggctcagtaggagggcctgggacagggtcagtggtgcctgctgtggaggtgttggtttggtcgggcatgggtctctgaggtaaggggcggcctgggccagcagtctggaccactgtggtggtaggcaggaccgaagtggcgaggccgaggaggcctgaggaggctgccgggcctgaattgaaaggagctaagttgcccagcgggggctgagccagagctgggccagataagaggaccggcgccaggcgaggcaaggttggggcagccccgaggggcatggaggcaggtgtggtggcaggtggggccttgagagctgggggagcctcaggtgctggggccaagtcgtagcacttgctttcactcttcagctgggctcgaaccgcctccttgagcttggccaggtgctgacgggaaaagagatggcctcggcaggagacatagaaatcatacttgacatcacaataggggcagtcagtgcgctgggctgctaagaggccctcactgctgcccccagtgctcccagcggctgtcccctgtagtttggccttcttttccttggcacgagcattctggaaccagacctggatgactctcttgggcagcccaatctcctctcccagcacctcacactcctgcatggtgggggtgcggtaagcttcatagcaggctttcatgatcttcagctgcaggctgctcatctgggtcctgtagcgccgctgccccattccatctggaaccccagtcccacctccaggtcccccactggtccctccagccccaggggattctggttcagctaggctggaagcagatgaatcactcagatctcctgcagagagactgcaagcctcactctctggagaagctttaggtggttcctctgggccctcttcctcactgggtggagggggaggtaggagaggtagaggtggctctggtgttggggtggtggcctctttcccaggtggtaggaaaggctggggcccagaagcaagcgtggcagtggggtagggaaaagcaggtgcttccctctttggggcttccctcccagtgccatcatctaccttgcctaataagaggttgaacttgggcaaggatgcaggggtggctgtggcaggcggtttcactgctggactaggcacccccccaggggtgcttcgaaactggcctttcctctcccgggccctggtattctggaaccagacctgtaccactcgctttttgagccccacctcctcggagatgcagtcgagcatcttgcgtgttgggttggaatcctgcatgtaccaacggtacaggatctctagctgctcaggcaagatggtggtgcgcaggcgcttgtccctggggggctcgccctcccctcctccccctgcttcactgcctgtgggagacaagctgccgtcctcatgcttccgtttgagaggtggacctggcattggtgaggtggctgccaccagggggtttctctccccaaacaccagcaagggcagatctaggagttgggggggagcactgggctgcagagatggcaggaaatgtagtcggcggtgactggtcaggaggtcctggctggagaaagaaatggcacactggtcacaggtatgggctggggaaggtgatggagtagccttctcttcaggctctttgcctcctgcctttgttgcctctgcttggctcagctcctccccatctggaggctctggtaatgggccctcaggccctgctggaggttcaaggccctgttcctcctctacttcttcttcttccacctcttcctcctcttcccctctctctgcctcttcctcctcctcttcaagggtctggtcatcatagcacttcttgaggtggcgcaccaactcaaaaacacaggagaaagtggcgtggcaacgcctgcagccggaggctcccccagtgcctcctccggttggcatggacccaccctcacaggcatttttgcgtgctttctggcgggcattctggaaccacaccaccaccacacggctagccagacccaacagacttgcgagtcgctccacctctccgtctttggggtaggcgctagtctcaaagaaagactgcagggcttgggtctggaactctgtgaacttggttctggagaaccggcggccggcaggcaccaggggaggaagattccctctggagctttcttcctcttctatgggccagtgtccccctgctcgacttcgctcttcaggggcacgggtcccccctgcctcaggctctgggaccaggaagggtgggcccagatggggaacaggtgaatccagagacccatcaggaggtttgggaggctctgcaaggggcgggtataggctgtcatagctctttcgaaactgagcagcataacggctcagggcttcaaagggcagaaagcggcggtggacatgttcctcgtgtgtcttgaggataagcatattggagaagagtttcccacaggccccacaggccagcttgtccccacccccgagggcctcaggtgggggtggggtagggggagggggcacagcttgcttcccttcattgtactggatcaccagctcaaagccaaagttttctagaagggctttggctgcagtgcgggcagcctcgttgggcaatgggtcggggggtgaggaaggccctgcctcattaccctctttggccatggggggccgctcccactcccgctcagccagctcagccttgggaggttggggtggaggaggaggggtggcagctggcagggacagcacaggtgcaggcccagctagtgtcagcttgggccccaccttgagatcgtggaggtagaagggcaggagcagctgctgctgctggagcttaagcagtgattcgggcaccagagggaaggggggcaggactggtggggtgaagagaggggctgggaatcggtgcaggtccaagggaggtgggggaggggacaggaaaggcaatccagatatgaagccactggtgtcagggcccttcttctcagtgcccacctccccctctgtctcgccttccttgggctcttcttggctgcgttctggcccttcaatcttggaatcagtcttggttccccgagagcgagtctgatgcagaactgaccgcatgtggatctccagggtggagctctggttgtaggagactctgcagactgtgcacttaaagggcttgtctgtggcagcagtggtggtgggtggggcaccggcctctccccgtgcaggggcagaggggtcaatggcagccttcttcatcttgtgaaggtgggagacagaattataatgaaccaacagaatattcttctgggtgaaggactccttacacacagtgcacttatagggccgggcagggtcgagaaacttgtccagggcaaagttggtggttttccgataggtcagagggtggcgagagtcagctggagctggctctgcagagcggagctccccagtggtcccctcttcctcctcagccatggtgggcggaggagctacgtcttcagcttgggcatcaggttcagggactggagatggggctggagaagggggttggccagggcttcctgagggtttgtctgggacctcaactgaggccaggggaggctcaggaagaggatctggactggcttctggggtcaggttagggccttctgctgcctggtctctgctcggtgtaggctctggcccatgagtggggggttcttggccattgtccagagggcttaatgtgggtgcagacagcactttggttgtaaatgtcatttctacagttgtagctacaagcagcagcttctcaacgcactcgggcaccacgttgtgaaggtggctaaggtggaagtgcagggcaggccggcccaccagctgttcctggcacagtgggcatctgtacttgggctgcactgcatgctgggagagtgtatgagccctcacctggctggactctgggctcaggaagctgcagtatggacagcagtataccccaattctgaccgtggtctggttggcactgtctctggaagggccagtcttgttttctgtctcttctgaagccaattgttctgtcttgttctgggcatctttctcaggggtgggtggctcagctaagggggtgacaggagccttcccgggagtccggagctgcccgtggctgaagctcaggatgctctgaagagctgcgagtccttcctcagtggttgggccattctgtagcagctgcagacgcctctgggcctgggcatcgcggtgggcaggtgtgcgcaggtgttgcagcacagccaagcgggagggtgtctcccacgcacacaacaggcagtggtatagccccagctctgcccctgcctccgctccctccatgtccagcagaaacttatagatttggctgttttcttcgtgggctgcacccctggcatgcagctgcatcttctccttgctgttggactcaaagtcacagatgttgcagcgcaggtgtagtggggagacagacccataaggagccccatctcccagggatgctggggaaggggtgcccatggctccacccccctcccgcaggtgggctgccagctggtacttctgagcatgtttgtcagtcttgaggtggagttggaagttggccttgagctgggtgccatagcagcaaagcttgcagcggtgggtgtcaccagccacctccttccattcagcttccgggaggctccggcctatgctgcagtggtagagcagcagctccaggctgtctgtgctgaaggcctggcacactaggcagcggaacaccttcagggacaggctgtcgtcggatgtggggaacttgcgggcaggtgctcctacgtggtggaaaccattgagaagtagctgggcttccaggggcttgtctggcctcagccccgggccagccaagggagtctgaggctgccctagggcctggggcccaaagtactggaagagttcaggggggctagtgggggtagcccctggtgggggaggagggcctggccccatcaatccaggtggcaggcccagcggcagcccctggtgcagcattaggacattctgcatgtgcttctcagaggtcatatggatgcgcaggttacgggagatgtttgtctcgtagctgcacaccttgcactgccaggatgatttggtcttaggctctttgtctcccgcggagggtgggagtgatgcctctggtggacttccctgcccaccagggcccgcctggaagccctgtaggttggccaggtgcttgtcagactgcatatggatgctgaggttgcctttggtggttgtagagtagttgcagacgtcacagcggtagggtttgtagccacagttgtagctctctccacgagcaaggcgggggtgggcgcccccagcactgcagtagctgcagtgactgttgctctcagggtgcttctctcgcatgtgcacatccagggtctgctggtacttgtagtgccagttgcacttgggacacttgagtgtcttgcaggagttgcgtgagtggagcagggacatgtggctggacaggctgaggccctggaaggctgcaggggctggggtgtagtcatcagctaggcgatagggctggggtgggtcactggggtcttcgggggagcccactggggcagggagagtgcccccctccttggaggtgggtgagctttggttgagtggggggcagagccctccatcctcttcttgcccctcagggaaccaatctggccctgcctcgcctgctgctactggcgattctttggcttgggttgggctggggtcccaggtggctgtgggtggagagggtgggctgagggccataacttcttcatccaggaggataagggcctggacttctgcctcaggggggccatcctctgtctgggccacattcgcctccatgttcactgtgctgctgttgtcaaggggtatgtcagaagaggggcgagcagggagttttggctccagaaagcttatgagggccttgcagccttcatctccctcctggagtacagctgggctacctgacaggccctgatattgggcaggggttagcttcaccccatgagactgtgtgtgatccataaaggcctggggcttgctgaaacccaggcggcacagaaggcagagccagaagaccgccacgtggttgcccccgctgttccccatggggccatctttgggatctccgggtggatttggagccagctggtagctccagaaagctccatgcctttcctcacaggcagccggagatggtgctgaggtatcatgggacagaatttggtcagaagagctaaagccttggattgggtcaaagccatgttggatgtgaagggcagtgaggtgtgaggggggtgggtaggcaaggaagggcagactgggctcttccttgatgcccgcctcaccccaggggaagccctttggtaacaggagttcactgccacctggcagggacagcttggccactaggtaggcctcacctccagctgtgaagaataagtggttgcttaggtccatgggagggagcccttcttcttcctcctcctgctccttgtccttttccacccctgggtcatttggtgggaagtgaccacagtcaggcccttcctggggctccccaatctcctttggtgggacgaggccacagcccgactccaggagctgtccccctggctctgaggacctcatgttctcagaggtggaggaggcagcagggggatctttggtgacaggatcagagggggtgctggaggagaaggtgtccgaaggcagggacggggcattgtgcccaggggagggggtggtaccagtggtagaggctgagttaagggtggccatggtagacggaggagtgctgggggctcatgtcagcgtgacagccagtaccctgcgcttagctggctgctatagcagatatctgttggacggtgtgaatggcttgtattccaggcccatctgcctgcgttgggggtgcggcggggggtgttggagacgggactggggcttgagctccttgcacccgactctccccgccgccttgtagccccagttcagctttaggtagagtaccgcaggcaccaagtgcagctttcctgtcgccatagcgacgggcggggcgagatggcaaagtctccctttggaactacatctcccatcatgcatccgcgcctcggggtgcctggctcagcctcaggcatgagacctgtaccagcccccgggagccgtgcggggccaacaatgaggagcagaatgcaaggggcggcctcgctcccctggccaccgcgggggtcgcggcctcccattacatagcgcgtgtctcgagccctggcctgctctcggcaccgccacaacgggcgtaatatggccgctggtgccgggacctgccgggcgcgcggagggtcgggccgaggtccgggatccggaactgctcccggcattcctcgcgagtgtatggcgtgggctcccttccccctctgtggg

SEQ ID NO: 17701 - RNA, 8268 nt, Homo sapiens
  source 1..8268: mol_type = other RNA
tccatgtttccttcccccttctttgccttgggctttctttttcgtttcttctttttatcttctttttcaaaattttttggtgttttctcagtggaacatcatgggataacgtgtgtgtgtgcatgtatgtgtatgcatttatggggatggggagctgggaattcagtgaggaaaaggaagatagaaccaaggatatattttgtgtgtggtaggcagacatgtatgaataatcagggtgccaagatgggtgtatgtgtctgtgaagatgggcaagggctacatctgcaaggagctgaggaggaggatcaatgtgtgtgtctgtggggattgggaggaggcaggactctgctggaagtggggtgtgtggtgcccactgagggtgggaactgaacagttcctgtgaggtgggcggggccagggggtggggtgagggatttgagctcccaccgaacaccccttggggtaaaagagggagccctgaggccctcccctctccccatcttggttaatctgtttataaagctagaagtgtagaggtagtcgtagtttttgggttggagtccgtgtgaggtaatcttgcttcctctttggcaaaagccacagcagccgaggcagcagtggcggcgttggtgatggagatgggtgggcccccttgaggtggggctgccttgcgcctgtgggccgaggagcgcaggtgggaggctagggcttcacgcccactcagcagcacctcacatgccaggcagtggtaggtgcagatgggcacccgcaatgggggtggcatggagcccccagagccccgcccaaagaagcagaaggatctctggtgggcagtagccggggcctccccgtcaaatgccatcttgcactggcggcacaggtagcgatgggttacatccacggtggagatgccagtgctgcctgtcagcagctcatcaacctcaccagcttccccctcccctggagcaggcagttcaggaggctttggaggtgctgtggctgtgggctcagggggctggggtggcggctggaggagggcattggggagcagcccaatgagggtctgaggtatcatggggttcatgggaaatagccccttcttcatgccatagagctgttggaagtaggccccctgtagctgggggccaaagacagctggcggtgctgttcccccagcagggggcaatggaaagggcaggaactggccccccaacagggctgggacagtggtcttcaatgctttgaggttcttgagggcatcattggaggagctggtggggcctgcaactggctttcgctcactggagaccttgtcccccaagggctcagtaggagggcctgggacagggtcagtggtgcctgctgtggaggtgttggtttggtcgggcatgggtctctgaggtaaggggcggcctgggccagcagtctggaccactgtggtggtaggcaggaccgaagtggcgaggccgaggaggcctgaggaggctgccgggcctgaattgaaaggagctaagttgcccagcgggggctgagccagagctgggccagataagaggaccggcgccaggcgaggcaaggttggggcagccccgaggggcatggaggcaggtgtggtggcaggtggggccttgagagctgggggagcctcaggtgctggggccaagtcgtagcacttgctttcactcttcagctgggctcgaaccgcctccttgagcttggccaggtgctgacgggaaaagagatggcctcggcaggagacatagaaatcatacttgacatcacaataggggcagtcagtgcgctgggctgctaagaggccctcactgctgcccccagtgctcccagcggctgtcccctgtagtttggccttcttttccttggcacgagcattctggaaccagacctggatgactctcttgggcagcccaatctcctctcccagcacctcacactcctgcatggtgggggtgcggtaagcttcatagcaggctttcatgatcttcagctgcaggctgctcatctgggtcctgtagcgccgctgccccattccatctggaaccccagtcccacctccaggtcccccactggtccctccagccccaggggattctggttcagctaggctggaagcagatgaatcactcagatctcctgcagagagactgcaagcctcactctctggagaagctttaggtggttcctctgggccctcttcctcactgggtggagggggaggtaggagaggtagaggtggctctggtgttggggtggtggcctctttcccaggtggtaggaaaggctggggcccagaagcaagcgtggcagtggggtagggaaaagcaggtgcttccctctttggggcttccctcccagtgccatcatctaccttgcctaataagaggttgaacttgggcaaggatgcaggggtggctgtggcaggcggtttcactgctggactaggcacccccccaggggtgcttcgaaactggcctttcctctcccgggccctggtattctggaaccagacctgtaccactcgctttttgagccccacctcctcggagatgcagtcgagcatcttgcgtgttgggttggaatcctgcatgtaccaacggtacaggatctctagctgctcaggcaagatggtggtgcgcaggcgcttgtccctggggggctcgccctcccctcctccccctgcttcactgcctgtgggagacaagctgccgtcctcatgcttccgtttgagaggtggacctggcattggtgaggtggctgccaccagggggtttctctccccaaacaccagcaagggcagatctaggagttgggggggagcactgggctgcagagatggcaggaaatgtagtcggcggtgactggtcaggaggtcctggctggagaaagaaatggcacactggtcacaggtatgggctggggaaggtgatggagtagccttctcttcaggctctttgcctcctgcctttgttgcctctgcttggctcagctcctccccatctggaggctctggtaatgggccctcaggccctgctggaggttcaaggccctgttcctcctctacttcttcttcttccacctcttcctcctcttcccctctctctgcctcttcctcctcctcttcaagggtctggtcatcatagcacttcttgaggtggcgcaccaactcaaaaacacaggagaaagtggcgtggcaacgcctgcagccggaggctcccccagtgcctcctccggttggcatggacccaccctcacaggcatttttgcgtgctttctggcgggcattctggaaccacaccaccaccacacggctagccagacccaacagacttgcgagtcgctccacctctccgtctttggggtaggcgctagtctcaaagaaagactgcagggcttgggtctggaactctgtgaacttggttctggagaaccggcggccggcaggcaccaggggaggaagattccctctggagctttcttcctcttctatgggccagtgtccccctgctcgacttcgctcttcaggggcacgggtcccccctgcctcaggctctgggaccaggaagggtgggcccagatggggaacaggtgaatccagagacccatcaggaggtttgggaggctctgcaaggggcgggtataggctgtcatagctctttcgaaactgagcagcataacggctcagggcttcaaagggcagaaagcggcggtggacatgttcctcgtgtgtcttgaggataagcatattggagaagagtttcccacaggccccacaggccagcttgtccccacccccgagggcctcaggtgggggtggggtagggggagggggcacagcttgcttcccttcattgtactggatcaccagctcaaagccaaagttttctagaagggctttggctgcagtgcgggcagcctcgttgggcaatgggtcggggggtgaggaaggccctgcctcattaccctctttggccatggggggccgctcccactcccgctcagccagctcagccttgggaggttggggtggaggaggaggggtggcagctggcagggacagcacaggtgcaggcccagctagtgtcagcttgggccccaccttgagatcgtggaggtagaagggcaggagcagctgctgctgctggagcttaagcagtgattcgggcaccagagggaaggggggcaggactggtggggtgaagagaggggctgggaatcggtgcaggtccaagggaggtgggggaggggacaggaaaggcaatccagatatgaagccactggtgtcagggcccttcttctcagtgcccacctccccctctgtctcgccttccttgggctcttcttggctgcgttctggcccttcaatcttggaatcagtcttggttccccgagagcgagtctgatgcagaactgaccgcatgtggatctccagggtggagctctggttgtaggagactctgcagactgtgcacttaaagggcttgtctgtggcagcagtggtggtgggtggggcaccggcctctccccgtgcaggggcagaggggtcaatggcagccttcttcatcttgtgaaggtgggagacagaattataatgaaccaacagaatattcttctgggtgaaggactccttacacacagtgcacttatagggccgggcagggtcgagaaacttgtccagggcaaagttggtggttttccgataggtcagagggtggcgagagtcagctggagctggctctgcagagcggagctccccagtggtcccctcttcctcctcagccatggtgggcggaggagctacgtcttcagcttgggcatcaggttcagggactggagatggggctggagaagggggttggccagggcttcctgagggtttgtctgggacctcaactgaggccaggggaggctcaggaagaggatctggactggcttctggggtcaggttagggccttctgctgcctggtctctgctcggtgtaggctctggcccatgagtggggggttcttggccattgtccagagggcttaatgtgggtgcagacagcactttggttgtaaatgtcatttctacagttgtagctacaagcagcagcttctcaacgcactcgggcaccacgttgtgaaggtggctaaggtggaagtgcagggcaggccggcccaccagctgttcctggcacagtgggcatctgtacttgggctgcactgcatgctgggagagtgtatgagccctcacctggctggactctgggctcaggaagctgcagtatggacagcagtataccccaattctgaccgtggtctggttggcactgtctctggaagggccagtcttgttttctgtctcttctgaagccaattgttctgtcttgttctgggcatctttctcaggggtgggtggctcagctaagggggtgacaggagccttcccgggagtccggagctgcccgtggctgaagctcaggatgctctgaagagctgcgagtccttcctcagtggttgggccattctgtagcagctgcagacgcctctgggcctgggcatcgcggtgggcaggtgtgcgcaggtgttgcagcacagccaagcgggagggtgtctcccacgcacacaacaggcagtggtatagccccagctctgcccctgcctccgctccctccatgtccagcagaaacttatagatttggctgttttcttcgtgggctgcacccctggcatgcagctgcatcttctccttgctgttggactcaaagtcacagatgttgcagcgcaggtgtagtggggagacagacccataaggagccccatctcccagggatgctggggaaggggtgcccatggctccacccccctcccgcaggtgggctgccagctggtacttctgagcatgtttgtcagtcttgaggtggagttggaagttggccttgagctgggtgccatagcagcaaagcttgcagcggtgggtgtcaccagccacctccttccattcagcttccgggaggctccggcctatgctgcagtggtagagcagcagctccaggctgtctgtgctgaaggcctggcacactaggcagcggaacaccttcagggacaggctgtcgtctgggggtggtgaggtgggcaggctgtcagatgaggaacccaggagctgacttggaggcaggtgggcatcaggggataggcttccaggggcggatgtggggaacttgcgggcaggtgctcctacgtggtggaaaccattgagaagtagctgggcttccaggggcttgtctggcctcagccccgggccagccaagggagtctgaggctgccctagggcctggggcccaaagtactggaagagttcaggggggctagtgggggtagcccctggtgggggaggagggcctggccccatcaatccaggtggcaggcccagcggcagcccctggtgcagcattaggacattctgcatgtgcttctcagaggtcatatggatgcgcaggttacgggagatgtttgtctcgtagctgcacaccttgcactgccaggatgatttggtcttaggctctttgtctcccgcggagggtgggagtgatgcctctggtggacttccctgcccaccagggcccgcctggaagccctgtaggttggccaggtgcttgtcagactgcatatggatgctgaggttgcctttggtggttgtagagtagttgcagacgtcacagcggtagggtttgtagccacagttgtagctctctccacgagcaaggcgggggtgggcgcccccagcactgcagtagctgcagtgactgttgctctcagggtgcttctctcgcatgtgcacatccagggtctgctggtacttgtagtgccagttgcacttgggacacttgagtgtcttgcaggagttgcgtgagtggagcagggacatgtggctggacaggctgaggccctggaaggctgcaggggctggggtgtagtcatcagctaggcgatagggctggggtgggtcactggggtcttcgggggagcccactggggcagggagagtgcccccctccttggaggtgggtgagctttggttgagtggggggcagagccctccatcctcttcttgcccctcagggaaccaatctggccctgcctcgcctgctgctactggcgattctttggcttgggttgggctggggtcccaggtggctgtgggtggagagggtgggctgagggccataacttcttcatccaggaggataagggcctggacttctgcctcaggggggccatcctctgtctgggccacattcgcctccatgttcactgtgctgctgttgtcaaggggtatgtcagaagaggggcgagcagggagttttggctccagaaagcttatgagggccttgcagccttcatctccctcctggagtacagctgggctacctgacaggccctgatattgggcaggggttagcttcaccccatgagactgtgtgtgatccataaaggcctggggcttgctgaaacccaggcggcacagaaggcagagccagaagaccgccacgtggttgcccccgctgttccccatggggccatctttgggatctccgggtggatttggagccagctggtagctccagaaagctccatgcctttcctcacaggcagccggagatggtgctgaggtatcatgggacagaatttggtcagaagagctaaagccttggattgggtcaaagccatgttggatgtgaagggcagtgaggtgtgaggggggtgggtaggcaaggaagggcagactgggctcttccttgatgcccgcctcaccccaggggaagccctttggtaacaggagttcactgccacctggcagggacagcttggccactaggtaggcctcacctccagctgtgaagaataagtggttgcttaggtccatgggagggagcccttcttcttcctcctcctgctccttgtccttttccacccctgggtcatttggtgggaagtgaccacagtcaggcccttcctggggctccccaatctcctttggtgggacgaggccacagcccgactccaggagctgtccccctggctctgaggacctcatgttctcagaggtggaggaggcagcagggggatctttggtgacaggatcagagggggtgctggaggagaaggtgtccgaaggcagggacggggcattgtgcccaggggagggggtggtaccagtggtagaggctgagttaagggtggccatggtagacggaggagtgctggggg

SEQ ID NO: 17702 - RNA, 5564 nt, Homo sapiens
  source 1..5564: mol_type = other RNA
tccatgtttccttcccccttctttgccttgggctttctttttcgtttcttctttttatcttctttttcaaaattttttggtgttttctcagtggaacatcatgggataacgtgtgtgtgtgcatgtatgtgtatgcatttatggggatggggagctgggaattcagtgaggaaaaggaagatagaaccaaggatatattttgtgtgtggtaggcagacatgtatgaataatcagggtgccaagatgggtgtatgtgtctgtgaagatgggcaagggctacatctgcaaggagctgaggaggaggatcaatgtgtgtgtctgtggggattgggaggaggcaggactctgctggaagtggggtgtgtggtgcccactgagggtgggaactgaacagttcctgtgaggtgggcggggccagggggtggggtgagggatttgagctcccaccgaacaccccttggggtaaaagagggagccctgaggccctcccctctccccatcttggttaatctgtttataaagctagaagtgtagaggtagtcgtagtttttgggttggagtccgtgtgaggtaatcttgcttcctctttggcaaaagccacagcagccgaggcagcagtggcggcgttggtgatggagatgggtgggcccccttgaggtggggctgccttgcgcctgtgggccgaggagcgcaggtgggaggctagggcttcacgcccactcagcagcacctcacatgccaggcagtggtaggtgcagatgggcacccgcaatgggggtggcatggagcccccagagccccgcccaaagaagcagaaggatctctggtgggcagtagccggggcctccccgtcaaatgccatcttgcactggcggcacaggtagcgatgggttacatccacggtggagatgccagtgctgcctgtcagcagctcatcaacctcaccagcttccccctcccctggagcaggcagttcaggaggctttggaggtgctgtggctgtgggctcagggggctggggtggcggctggaggagggcattggggagcagcccaatgagggtctgaggtatcatggggttcatgggaaatagccccttcttcatgccatagagctgttggaagtaggccccctgtagctgggggccaaagacagctggcggtgctgttcccccagcagggggcaatggaaagggcaggaactggccccccaacagggctgggacagtggtcttcaatgctttgaggttcttgagggcatcattggaggagctggtggggcctgcaactggctttcgctcactggagaccttgtcccccaagggctcagtaggagggcctgggacagggtcagtggtgcctgctgtggaggtgttggtttggtcgggcatgggtctctgaggtaaggggcggcctgggccagcagtctggaccactgtggtggtaggcaggaccgaagtggcgaggccgaggaggcctgaggaggctgccgggcctgaattgaaaggagctaagttgcccagcgggggctgagccagagctgggccagataagaggaccggcgccaggcgaggcaaggttggggcagccccgaggggcatggaggcaggtgtggtggcaggtggggccttgagagctgggggagcctcaggtgctggggccaagtcgtagcacttgctttcactcttcagctgggctcgaaccgcctccttgagcttggccaggtgctgacgggaaaagagatggcctcggcaggagacatagaaatcatacttgacatcacaataggggcagtcagtgcgctgggctgctaagaggccctcactgctgcccccagtgctcccagcggctgtcccctgtagtttggccttcttttccttggcacgagcattctggaaccagacctggatgactctcttgggcagcccaatctcctctcccagcacctcacactcctgcatggtgggggtgcggtaagcttcatagcaggctttcatgatcttcagctgcaggctgctcatctgggtcctgtagcgccgctgccccattccatctggaaccccagtcccacctccaggtcccccactggtccctccagccccaggggattctggttcagctaggctggaagcagatgaatcactcagatctcctgcagagagactgcaagcctcactctctggagaagctttaggtggttcctctgggccctcttcctcactgggtggagggggaggtaggagaggtagaggtggctctggtgttggggtggtggcctctttcccaggtggtaggaaaggctggggcccagaagcaagcgtggcagtggggtagggaaaagcaggtgcttccctctttggggcttccctcccagtgccatcatctaccttgcctaataagaggttgaacttgggcaaggatgcaggggtggctgtggcaggcggtttcactgctggactaggcacccccccaggggtgcttcgaaactggcctttcctctcccgggccctggtattctggaaccagacctgtaccactcgctttttgagccccacctcctcggagatgcagtcgagcatcttgcgtgttgggttggaatcctgcatgtaccaacggtacaggatctctagctgctcaggcaagatggtggtgcgcaggcgcttgtccctggggggctcgccctcccctcctccccctgcttcactgcctgtgggagacaagctgccgtcctcatgcttccgtttgagaggtggacctggcattggtgaggtggctgccaccagggggtttctctccccaaacaccagcaagggcagatctaggagttgggggggagcactgggctgcagagatggcaggaaatgtagtcggcggtgactggtcaggaggtcctggctggagaaagaaatggcacactggtcacaggtatgggctggggaaggtgatggagtagccttctcttcaggctctttgcctcctgcctttgttgcctctgcttggctcagctcctccccatctggaggctctggtaatgggccctcaggccctgctggaggttcaaggccctgttcctcctctacttcttcttcttccacctcttcctcctcttcccctctctctgcctcttcctcctcctcttcaagggtctggtcatcatagcacttcttgaggtggcgcaccaactcaaaaacacaggagaaagtggcgtggcaacgcctgcagccggaggctcccccagtgcctcctccggttggcatggacccaccctcacaggcatttttgcgtgctttctggcgggcattctggaaccacaccaccaccacacggctagccagacccaacagacttgcgagtcgctccacctctccgtctttggggtaggcgctagtctcaaagaaagactgcagggcttgggtctggaactctgtgaacttggttctggagaaccggcggccggcaggcaccaggggaggaagattccctctggagctttcttcctcttctatgggccagtgtccccctgctcgacttcgctcttcaggggcacgggtcccccctgcctcaggctctgggaccaggaagggtgggcccagatggggaacaggtgaatccagagacccatcaggaggtttgggaggctctgcaaggggcgggtataggctgtcatagctctttcgaaactgagcagcataacggctcagggcttcaaagggcagaaagcggcggtggacatgttcctcgtgtgtcttgaggataagcatattggagaagagtttcccacaggccccacaggccagcttgtccccacccccgagggcctcaggtgggggtggggtagggggagggggcacagcttgcttcccttcattgtactggatcaccagctcaaagccaaagttttctagaagggctttggctgcagtgcgggcagcctcgttgggcaatgggtcggggggtgaggaaggccctgcctcattaccctctttggccatggggggccgctcccactcccgctcagccagctcagccttgggaggttggggtggaggaggaggggtggcagctggcagggacagcacaggtgcaggcccagctagtgtcagcttgggccccaccttgagatcgtggaggtagaagggcaggagcagctgctgctgctggagcttaagcagtgattcgggcaccagagggaaggggggcaggactggtggggtgaagagaggggctgggaatcggtgcaggtccaagggaggtgggggaggggacaggaaaggcaatccagatatgaagccactggtgtcagggcccttcttctcagtgcccacctccccctctgtctcgccttccttgggctcttcttggctgcgttctggcccttcaatcttggaatcagtcttggttccccgagagcgagtctgatgcagaactgaccgcatgtggatctccagggtggagctctggttgtaggagactctgcagactgtgcacttaaagggcttgtctgtggcagcagtggtggtgggtggggcaccggcctctccccgtgcaggggcagaggggtcaatggcagccttcttcatcttgtgaaggtgggagacagaattataatgaaccaacagaatattcttctgggtgaaggactccttacacacagtgcacttatagggccgggcagggtcgagaaacttgtccagggcaaagttggtggttttccgataggtcagagggtggcgagagtcagctggagctggctctgcagagcggagctccccagtggtcccctcttcctcctcagccatggtgggcggaggagctacgtcttcagcttgggcatcaggttcagggactggagatggggctggagaagggggttggccagggcttcctgagggtttgtctgggacctcaactgaggccaggggaggctcaggaagaggatctggactggcttctggggtcaggttagggccttctgctgcctggtctctgctcggtgtaggctctggcccatgagtggggggttcttggccattgtccagagggcttaatgtgggtgcagacagcactttggttgtaaatgtcatttctacagttgtagctacaagcagcagcttctcaacgcactcgggcaccacgttgtgaaggtggctaaggtggaagtgcagggcaggccggcccaccagctgttcctggcacagtgggcatctgtacttgggctgcactgcatgctgggagagtgtatgagccctcacctggctggactctgggctcaggaagctgcagtatggacagcagtataccccaattctgaccgtggtctggttggcactgtctctggaagggccagtcttgttttctgtctcttctgaagccaattgttctgtcttgttctgggcatctttctcaggggtgggtggctcagctaagggggtgacaggagccttccctctggcagccccttgcaggctcttctcctgtaccctctggatcaatggtgcctggctggctgttcccggcctctgctggtacaacctcagctgcctaagggtgactctaagcccagcc

SEQ ID NO: 17703 - RNA, 8705 nt, Homo sapiens
  source 1..8705: mol_type = other RNA
tccatgtttccttcccccttctttgccttgggctttctttttcgtttcttctttttatcttctttttcaaaattttttggtgttttctcagtggaacatcatgggataacgtgtgtgtgtgcatgtatgtgtatgcatttatggggatggggagctgggaattcagtgaggaaaaggaagatagaaccaaggatatattttgtgtgtggtaggcagacatgtatgaataatcagggtgccaagatgggtgtatgtgtctgtgaagatgggcaagggctacatctgcaaggagctgaggaggaggatcaatgtgtgtgtctgtggggattgggaggaggcaggactctgctggaagtggggtgtgtggtgcccactgagggtgggaactgaacagttcctgtgaggtgggcggggccagggggtggggtgagggatttgagctcccaccgaacaccccttggggtaaaagagggagccctgaggccctcccctctccccatcttggttaatctgtttataaagctagaagtgtagaggtagtcgtagtttttgggttggagtccgtgtgaggtaatcttgcttcctctttggcaaaagccacagcagccgaggcagcagtggcggcgttggtgatggagatgggtgggcccccttgaggtggggctgccttgcgcctgtgggccgaggagcgcaggtgggaggctagggcttcacgcccactcagcagcacctcacatgccaggcagtggtaggtgcagatgggcacccgcaatgggggtggcatggagcccccagagccccgcccaaagaagcagaaggatctctggtgggcagtagccggggcctccccgtcaaatgccatcttgcactggcggcacaggtagcgatgggttacatccacggtggagatgccagtgctgcctgtcagcagctcatcaacctcaccagcttccccctcccctggagcaggcagttcaggaggctttggaggtgctgtggctgtgggctcagggggctggggtggcggctggaggagggcattggggagcagcccaatgagggtctgaggtatcatggggttcatgggaaatagccccttcttcatgccatagagctgttggaagtaggccccctgtagctgggggccaaagacagctggcggtgctgttcccccagcagggggcaatggaaagggcaggaactggccccccaacagggctgggacagtggtcttcaatgctttgaggttcttgagggcatcattggaggagctggtggggcctgcaactggctttcgctcactggagaccttgtcccccaagggctcagtaggagggcctgggacagggtcagtggtgcctgctgtggaggtgttggtttggtcgggcatgggtctctgaggtaaggggcggcctgggccagcagtctggaccactgtggtggtaggcaggaccgaagtggcgaggccgaggaggcctgaggaggctgccgggcctgaattgaaaggagctaagttgcccagcgggggctgagccagagctgggccagataagaggaccggcgccaggcgaggcaaggttggggcagccccgaggggcatggaggcaggtgtggtggcaggtggggccttgagagctgggggagcctcaggtgctggggccaagtcgtagcacttgctttcactcttcagctgggctcgaaccgcctccttgagcttggccaggtgctgacgggaaaagagatggcctcggcaggagacatagaaatcatacttgacatcacaataggggcagtcagtgcgctgggctgctaagaggccctcactgctgcccccagtgctcccagcggctgtcccctgtagtttggccttcttttccttggcacgagcattctggaaccagacctggatgactctcttgggcagcccaatctcctctcccagcacctcacactcctgcatggtgggggtgcggtaagcttcatagcaggctttcatgatcttcagctgcaggctgctcatctgggtcctgtagcgccgctgccccattccatctggaaccccagtcccacctccaggtcccccactggtccctccagccccaggggattctggttcagctaggctggaagcagatgaatcactcagatctcctgcagagagactgcaagcctcactctctggagaagctttaggtggttcctctgggccctcttcctcactgggtggagggggaggtaggagaggtagaggtggctctggtgttggggtggtggcctctttcccaggtggtaggaaaggctggggcccagaagcaagcgtggcagtggggtagggaaaagcaggtgcttccctctttggggcttccctcccagtgccatcatctaccttgcctaataagaggttgaacttgggcaaggatgcaggggtggctgtggcaggcggtttcactgctggactaggcacccccccaggggtgcttcgaaactggcctttcctctcccgggccctggtattctggaaccagacctgtaccactcgctttttgagccccacctcctcggagatgcagtcgagcatcttgcgtgttgggttggaatcctgcatgtaccaacggtacaggatctctagctgctcaggcaagatggtggtgcgcaggcgcttgtccctggggggctcgccctcccctcctccccctgcttcactgcctgtgggagacaagctgccgtcctcatgcttccgtttgagaggtggacctggcattggtgaggtggctgccaccagggggtttctctccccaaacaccagcaagggcagatctaggagttgggggggagcactgggctgcagagatggcaggaaatgtagtcggcggtgactggtcaggaggtcctggctggagaaagaaatggcacactggtcacaggtatgggctggggaaggtgatggagtagccttctcttcaggctctttgcctcctgcctttgttgcctctgcttggctcagctcctccccatctggaggctctggtaatgggccctcaggccctgctggaggttcaaggccctgttcctcctctacttcttcttcttccacctcttcctcctcttcccctctctctgcctcttcctcctcctcttcaagggtctggtcatcatagcacttcttgaggtggcgcaccaactcaaaaacacaggagaaagtggcgtggcaacgcctgcagccggaggctcccccagtgcctcctccggttggcatggacccaccctcacaggcatttttgcgtgctttctggcgggcattctggaaccacaccaccaccacacggctagccagacccaacagacttgcgagtcgctccacctctccgtctttggggtaggcgctagtctcaaagaaagactgcagggcttgggtctggaactctgtgaacttggttctggagaaccggcggccggcaggcaccaggggaggaagattccctctggagctttcttcctcttctatgggccagtgtccccctgctcgacttcgctcttcaggggcacgggtcccccctgcctcaggctctgggaccaggaagggtgggcccagatggggaacaggtgaatccagagacccatcaggaggtttgggaggctctgcaaggggcgggtataggctgtcatagctctttcgaaactgagcagcataacggctcagggcttcaaagggcagaaagcggcggtggacatgttcctcgtgtgtcttgaggataagcatattggagaagagtttcccacaggccccacaggccagcttgtccccacccccgagggcctcaggtgggggtggggtagggggagggggcacagcttgcttcccttcattgtactggatcaccagctcaaagccaaagttttctagaagggctttggctgcagtgcgggcagcctcgttgggcaatgggtcggggggtgaggaaggccctgcctcattaccctctttggccatggggggccgctcccactcccgctcagccagctcagccttgggaggttggggtggaggaggaggggtggcagctggcagggacagcacaggtgcaggcccagctagtgtcagcttgggccccaccttgagatcgtggaggtagaagggcaggagcagctgctgctgctggagcttaagcagtgattcgggcaccagagggaaggggggcaggactggtggggtgaagagaggggctgggaatcggtgcaggtccaagggaggtgggggaggggacaggaaaggcaatccagatatgaagccactggtgtcagggcccttcttctcagtgcccacctccccctctgtctcgccttccttgggctcttcttggctgcgttctggcccttcaatcttggaatcagtcttggttccccgagagcgagtctgatgcagaactgaccgcatgtggatctccagggtggagctctggttgtaggagactctgcagactgtgcacttaaagggcttgtctgtggcagcagtggtggtgggtggggcaccggcctctccccgtgcaggggcagaggggtcaatggcagccttcttcatcttgtgaaggtgggagacagaattataatgaaccaacagaatattcttctgggtgaaggactccttacacacagtgcacttatagggccgggcagggtcgagaaacttgtccagggcaaagttggtggttttccgataggtcagagggtggcgagagtcagctggagctggctctgcagagcggagctccccagtggtcccctcttcctcctcagccatggtgggcggaggagctacgtcttcagcttgggcatcaggttcagggactggagatggggctggagaagggggttggccagggcttcctgagggtttgtctgggacctcaactgaggccaggggaggctcaggaagaggatctggactggcttctggggtcaggttagggccttctgctgcctggtctctgctcggtgtaggctctggcccatgagtggggggttcttggccattgtccagagggcttaatgtgggtgcagacagcactttggttgtaaatgtcatttctacagttgtagctacaagcagcagcttctcaacgcactcgggcaccacgttgtgaaggtggctaaggtggaagtgcagggcaggccggcccaccagctgttcctggcacagtgggcatctgtacttgggctgcactgcatgctgggagagtgtatgagccctcacctggctggactctgggctcaggaagctgcagtatggacagcagtataccgtggtctggttggcactgtctctggaagggccagtcttgttttctgtctcttctgaagccaattgttctgtcttgttctgggcatctttctcaggggtgggtggctcagctaagggggtgacaggagccttcccgggagtccggagctgcccgtggctgaagctcaggatgctctgaagagctgcgagtccttcctcagtggttgggccattctgtagcagctgcagacgcctctgggcctgggcatcgcggtgggcaggtgtgcgcaggtgttgcagcacagccaagcgggagggtgtctcccacgcacacaacaggcagtggtatagccccagctctgcccctgcctccgctccctccatgtccagcagaaacttatagatttggctgttttcttcgtgggctgcacccctggcatgcagctgcatcttctccttgctgttggactcaaagtcacagatgttgcagcgcaggtgtagtggggagacagacccataaggagccccatctcccagggatgctggggaaggggtgcccatggctccacccccctcccgcaggtgggctgccagctggtacttctgagcatgtttgtcagtcttgaggtggagttggaagttggccttgagctgggtgccatagcagcaaagcttgcagcggtgggtgtcaccagccacctccttccattcagcttccgggaggctccggcctatgctgcagtggtagagcagcagctccaggctgtctgtgctgaaggcctggcacactaggcagcggaacaccttcagggacaggctgtcgtctgggggtggtgaggtgggcaggctgtcagatgaggaacccaggagctgacttggaggcaggtgggcatcaggggataggcttccaggggcggatgtggggaacttgcgggcaggtgctcctacgtggtggaaaccattgagaagtagctgggcttccaggggcttgtctggcctcagccccgggccagccaagggagtctgaggctgccctagggcctggggcccaaagtactggaagagttcaggggggctagtgggggtagcccctggtgggggaggagggcctggccccatcaatccaggtggcaggcccagcggcagcccctggtgcagcattaggacattctgcatgtgcttctcagaggtcatatggatgcgcaggttacgggagatgtttgtctcgtagctgcacaccttgcactgccaggatgatttggtcttaggctctttgtctcccgcggagggtgggagtgatgcctctggtggacttccctgcccaccagggcccgcctggaagccctgtaggttggccaggtgcttgtcagactgcatatggatgctgaggttgcctttggtggttgtagagtagttgcagacgtcacagcggtagggtttgtagccacagttgtagctctctccacgagcaaggcgggggtgggcgcccccagcactgcagtagctgcagtgactgttgctctcagggtgcttctctcgcatgtgcacatccagggtctgctggtacttgtagtgccagttgcacttgggacacttgagtgtcttgcaggagttgcgtgagtggagcagggacatgtggctggacaggctgaggccctggaaggctgcaggggctggggtgtagtcatcagctaggcgatagggctggggtgggtcactggggtcttcgggggagcccactggggcagggagagtgcccccctccttggaggtgggtgagctttggttgagtggggggcagagccctccatcctcttcttgcccctcagggaaccaatctggccctgcctcgcctgctgctactggcgattctttggcttgggttgggctggggtcccaggtggctgtgggtggagagggtgggctgagggccataacttcttcatccaggaggataagggcctggacttctgcctcaggggggccatcctctgtctgggccacattcgcctccatgttcactgtgctgctgttgtcaaggggtatgtcagaagaggggcgagcagggagttttggctccagaaagcttatgagggccttgcagccttcatctccctcctggagtacagctgggctacctgacaggccctgatattgggcaggggttagcttcaccccatgagactgtgtgtgatccataaaggcctggggcttgctgaaacccaggcggcacagaaggcagagccagaagaccgccacgtggttgcccccgctgttccccatggggccatctttgggatctccgggtggatttggagccagctggtagctccagaaagctccatgcctttcctcacaggcagccggagatggtgctgaggtatcatgggacagaatttggtcagaagagctaaagccttggattgggtcaaagccatgttggatgtgaagggcagtgaggtgtgaggggggtgggtaggcaaggaagggcagactgggctcttccttgatgcccgcctcaccccaggggaagccctttggtaacaggagttcactgccacctggcagggacagcttggccactaggtaggcctcacctccagctgtgaagaataagtggttgcttaggtccatgggagggagcccttcttcttcctcctcctgctccttgtccttttccacccctgggtcatttggtgggaagtgaccacagtcaggcccttcctggggctccccaatctcctttggtgggacgaggccacagcccgactccaggagctgtccccctggctctgaggacctcatgttctcagaggtggaggaggcagcagggggatctttggtgacaggatcagagggggtgctggaggagaaggtgtccgaaggcagggacggggcattgtgcccaggggagggggtggtaccagtggtagaggctgagttaagggtggccatggtagacggaggagtgctgggggctcatgtcagcgtgacagccagtaccacctcagctggaagcagggacgggagtcgaaccgcggccaccgagcagcgcgaggcggggaggggagggggcggctcttggaagggacttctccgatgtgttgattcctcttttttcccctcctcctccctccctccagcgctcgctccggggcgtcagggacggagacggaaaaaaataaataaataaattcacggcggtgagggaagtgaaggaaaataatcaatgctatttggctgcggctgaagtgtttccccggcttcgtgagggggtttccattgattcaccctgggcactcgctcgctccctgcctcctcctcctcctcctccttctcctcctcgccctcctcctcctcctcctcctcgccctcactcctccgcctcattcactggctggagtctaggcgtcccacacaatggaat

SEQ ID NO: 17704 - RNA, 10946 nt, Homo sapiens
  source 1..10946: mol_type = other RNA
tccatgtttccttcccccttctttgccttgggctttctttttcgtttcttctttttatcttctttttcaaaattttttggtgttttctcagtggaacatcatgggataacgtgtgtgtgtgcatgtatgtgtatgcatttatggggatggggagctgggaattcagtgaggaaaaggaagatagaaccaaggatatattttgtgtgtggtaggcagacatgtatgaataatcagggtgccaagatgggtgtatgtgtctgtgaagatgggcaagggctacatctgcaaggagctgaggaggaggatcaatgtgtgtgtctgtggggattgggaggaggcaggactctgctggaagtggggtgtgtggtgcccactgagggtgggaactgaacagttcctgtgaggtgggcggggccagggggtggggtgagggatttgagctcccaccgaacaccccttggggtaaaagagggagccctgaggccctcccctctccccatcttggttaatctgtttataaagctagaagtgtagaggtagtcgtagtttttgggttggagtccgtgtgaggtaatcttgcttcctctttggcaaaagccacagcagccgaggcagcagtggcggcgttggtgatggagatgggtgggcccccttgaggtggggctgccttgcgcctgtgggccgaggagcgcaggtgggaggctagggcttcacgcccactcagcagcacctcacatgccaggcagtggtaggtgcagatgggcacccgcaatgggggtggcatggagcccccagagccccgcccaaagaagcagaaggatctctggtgggcagtagccggggcctccccgtcaaatgccatcttgcactggcggcacaggtagcgatgggttacatccacggtggagatgccagtgctgcctgtcagcagctcatcaacctcaccagcttccccctcccctggagcaggcagttcaggaggctttggaggtgctgtggctgtgggctcagggggctggggtggcggctggaggagggcattggggagcagcccaatgagggtctgaggtatcatggggttcatgggaaatagccccttcttcatgccatagagctgttggaagtaggccccctgtagctgggggccaaagacagctggcggtgctgttcccccagcagggggcaatggaaagggcaggaactggccccccaacagggctgggacagtggtcttcaatgctttgaggttcttgagggcatcattggaggagctggtggggcctgcaactggctttcgctcactggagaccttgtcccccaagggctcagtaggagggcctgggacagggtcagtggtgcctgctgtggaggtgttggtttggtcgggcatgggtctctgaggtaaggggcggcctgggccagcagtctggaccactgtggtggtaggcaggaccgaagtggcgaggccgaggaggcctgaggaggctgccgggcctgaattgaaaggagctaagttgcccagcgggggctgagccagagctgggccagataagaggaccggcgccaggcgaggcaaggttggggcagccccgaggggcatggaggcaggtgtggtggcaggtggggccttgagagctgggggagcctcaggtgctggggccaagtcgtagcacttgctttcactcttcagctgggctcgaaccgcctccttgagcttggccaggtgctgacgggaaaagagatggcctcggcaggagacatagaaatcatacttgacatcacaataggggcagtcagtgcgctgggctgctaagaggccctcactgctgcccccagtgctcccagcggctgtcccctgtagtttggccttcttttccttggcacgagcattctggaaccagacctggatgactctcttgggcagcccaatctcctctcccagcacctcacactcctgcatggtgggggtgcggtaagcttcatagcaggctttcatgatcttcagctgcaggctgctcatctgggtcctgtagcgccgctgccccattccatctggaaccccagtcccacctccaggtcccccactggtccctccagccccaggggattctggttcagctaggctggaagcagatgaatcactcagatctcctgcagagagactgcaagcctcactctctggagaagctttaggtggttcctctgggccctcttcctcactgggtggagggggaggtaggagaggtagaggtggctctggtgttggggtggtggcctctttcccaggtggtaggaaaggctggggcccagaagcaagcgtggcagtggggtagggaaaagcaggtgcttccctctttggggcttccctcccagtgccatcatctaccttgcctaataagaggttgaacttgggcaaggatgcaggggtggctgtggcaggcggtttcactgctggactaggcacccccccaggggtgcttcgaaactggcctttcctctcccgggccctggtattctggaaccagacctgtaccactcgctttttgagccccacctcctcggagatgcagtcgagcatcttgcgtgttgggttggaatcctgcatgtaccaacggtacaggatctctagctgctcaggcaagatggtggtgcgcaggcgcttgtccctggggggctcgccctcccctcctccccctgcttcactgcctgtgggagacaagctgccgtcctcatgcttccgtttgagaggtggacctggcattggtgaggtggctgccaccagggggtttctctccccaaacaccagcaagggcagatctaggagttgggggggagcactgggctgcagagatggcaggaaatgtagtcggcggtgactggtcaggaggtcctggctggagaaagaaatggcacactggtcacaggtatgggctggggaaggtgatggagtagccttctcttcaggctctttgcctcctgcctttgttgcctctgcttggctcagctcctccccatctggaggctctggtaatgggccctcaggccctgctggaggttcaaggccctgttcctcctctacttcttcttcttccacctcttcctcctcttcccctctctctgcctcttcctcctcctcttcaagggtctggtcatcatagcacttcttgaggtggcgcaccaactcaaaaacacaggagaaagtggcgtggcaacgcctgcagccggaggctcccccagtgcctcctccggttggcatggacccaccctcacaggcatttttgcgtgctttctggcgggcattctggaaccacaccaccaccacacggctagccagacccaacagacttgcgagtcgctccacctctccgtctttggggtaggcgctagtctcaaagaaagactgcagggcttgggtctggaactctgtgaacttggttctggagaaccggcggccggcaggcaccaggggaggaagattccctctggagctttcttcctcttctatgggccagtgtccccctgctcgacttcgctcttcaggggcacgggtcccccctgcctcaggctctgggaccaggaagggtgggcccagatggggaacaggtgaatccagagacccatcaggaggtttgggaggctctgcaaggggcgggtataggctgtcatagctctttcgaaactgagcagcataacggctcagggcttcaaagggcagaaagcggcggtggacatgttcctcgtgtgtcttgaggataagcatattggagaagagtttcccacaggccccacaggccagcttgtccccacccccgagggcctcaggtgggggtggggtagggggagggggcacagcttgcttcccttcattgtactggatcaccagctcaaagccaaagttttctagaagggctttggctgcagtgcgggcagcctcgttgggcaatgggtcggggggtgaggaaggccctgcctcattaccctctttggccatggggggccgctcccactcccgctcagccagctcagccttgggaggttggggtggaggaggaggggtggcagctggcagggacagcacaggtgcaggcccagctagtgtcagcttgggccccaccttgagatcgtggaggtagaagggcaggagcagctgctgctgctggagcttaagcagtgattcgggcaccagagggaaggggggcaggactggtggggtgaagagaggggctgggaatcggtgcaggtccaagggaggtgggggaggggacaggaaaggcaatccagatatgaagccactggtgtcagggcccttcttctcagtgcccacctccccctctgtctcgccttccttgggctcttcttggctgcgttctggcccttcaatcttggaatcagtcttggttccccgagagcgagtctgatgcagaactgaccgcatgtggatctccagggtggagctctggttgtaggagactctgcagactgtgcacttaaagggcttgtctgtggcagcagtggtggtgggtggggcaccggcctctccccgtgcaggggcagaggggtcaatggcagccttcttcatcttgtgaaggtgggagacagaattataatgaaccaacagaatattcttctgggtgaaggactccttacacacagtgcacttatagggccgggcagggtcgagaaacttgtccagggcaaagttggtggttttccgataggtcagagggtggcgagagtcagctggagctggctctgcagagcggagctccccagtggtcccctcttcctcctcagccatggtgggcggaggagctacgtcttcagcttgggcatcaggttcagggactggagatggggctggagaagggggttggccagggcttcctgagggtttgtctgggacctcaactgaggccaggggaggctcaggaagaggatctggactggcttctggggtcaggttagggccttctgctgcctggtctctgctcggtgtaggctctggcccatgagtggggggttcttggccattgtccagagggcttaatgtgggtgcagacagcactttggttgtaaatgtcatttctacagttgtagctacaagcagcagcttctcaacgcactcgggcaccacgttgtgaaggtggctaaggtggaagtgcagggcaggccggcccaccagctgttcctggcacagtgggcatctgtacttgggctgcactgcatgctgggagagtgtatgagccctcacctggctggactctgggctcaggaagctgcagtatggacagcagtataccgtggtctggttggcactgtctctggaagggccagtcttgttttctgtctcttctgaagccaattgttctgtcttgttctgggcatctttctcaggggtgggtggctcagctaagggggtgacaggagccttcccgggagtccggagctgcccgtggctgaagctcaggatgctctgaagagctgcgagtccttcctcagtggttgggccattctgtagcagctgcagacgcctctgggcctgggcatcgcggtgggcaggtgtgcgcaggtgttgcagcacagccaagcgggagggtgtctcccacgcacacaacaggcagtggtatagccccagctctgcccctgcctccgctccctccatgtccagcagaaacttatagatttggctgttttcttcgtgggctgcacccctggcatgcagctgcatcttctccttgctgttggactcaaagtcacagatgttgcagcgcaggtgtagtggggagacagacccataaggagccccatctcccagggatgctggggaaggggtgcccatggctccacccccctcccgcaggtgggctgccagctggtacttctgagcatgtttgtcagtcttgaggtggagttggaagttggccttgagctgggtgccatagcagcaaagcttgcagcggtgggtgtcaccagccacctccttccattcagcttccgggaggctccggcctatgctgcagtggtagagcagcagctccaggctgtctgtgctgaaggcctggcacactaggcagcggaacaccttcagggacaggctgtcgtctgggggtggtgaggtgggcaggctgtcagatgaggaacccaggagctgacttggaggcaggtgggcatcaggggataggcttccaggggcggatgtggggaacttgcgggcaggtgctcctacgtggtggaaaccattgagaagtagctgggcttccaggggcttgtctggcctcagccccgggccagccaagggagtctgaggctgccctagggcctggggcccaaagtactggaagagttcaggggggctagtgggggtagcccctggtgggggaggagggcctggccccatcaatccaggtggcaggcccagcggcagcccctggtgcagcattaggacattctgcatgtgcttctcagaggtcatatggatgcgcaggttacgggagatgtttgtctcgtagctgcacaccttgcactgccaggatgatttggtcttaggctctttgtctcccgcggagggtgggagtgatgcctctggtggacttccctgcccaccagggcccgcctggaagccctgtaggttggccaggtgcttgtcagactgcatatggatgctgaggttgcctttggtggttgtagagtagttgcagacgtcacagcggtagggtttgtagccacagttgtagctctctccacgagcaaggcgggggtgggcgcccccagcactgcagtagctgcagtgactgttgctctcagggtgcttctctcgcatgtgcacatccagggtctgctggtacttgtagtgccagttgcacttgggacacttgagtgtcttgcaggagttgcgtgagtggagcagggacatgtggctggacaggctgaggccctggaaggctgcaggggctggggtgtagtcatcagctaggcgatagggctggggtgggtcactggggtcttcgggggagcccactggggcagggagagtgcccccctccttggaggtgggtgagctttggttgagtggggggcagagccctccatcctcttcttgcccctcagggaaccaatctggccctgcctcgcctgctgctactggcgattctttggcttgggttgggctggggtcccaggtggctgtgggtggagagggtgggctgagggccataacttcttcatccaggaggataagggcctggacttctgcctcaggggggccatcctctgtctgggccacattcgcctccatgttcactgtgctgctgttgtcaaggggtatgtcagaagaggggcgagcagggagttttggctccagaaagcttatgagggccttgcagccttcatctccctcctggagtacagctgggctacctgacaggccctgatattgggcaggggttagcttcaccccatgagactgtgtgtgatccataaaggcctggggcttgctgaaacccaggcggcacagaaggcagagccagaagaccgccacgtggttgcccccgctgttccccatggggccatctttgggatctccgggtggatttggagccagctggtagctccagaaagctccatgcctttcctcacaggcagccggagatggtgctgaggtatcatgggacagaatttggtcagaagagctaaagccttggattgggtcaaagccatgttggatgtgaagggcagtgaggtgtgaggggggtgggtaggcaaggaagggcagactgggctcttccttgatgcccgcctcaccccaggggaagccctttggtaacaggagttcactgccacctggcagggacagcttggccactaggtaggcctcacctccagctgtgaagaataagtggttgcttaggtccatgggagggagcccttcttcttcctcctcctgctccttgtccttttccacccctgggtcatttggtgggaagtgaccacagtcaggcccttcctggggctccccaatctcctttggtgggacgaggccacagcccgactccaggagctgtccccctggctctgaggacctcatgttctcagaggtggaggaggcagcagggggatctttggtgacaggatcagagggggtgctggaggagaaggtgtccgaaggcagggacggggcattgtgcccaggggagggggtggtaccagtggtagaggctgagttaagggtggccatggtagacggaggagtgctgggggctcatgtcagcgtgacagccagtacccaattcgacccaggccctggcccgtaggtgatacagcaccccggcaaagcagcaagtgattcctgtatgggtctcaaggtaacaccagctgcctctgacatcatggagggaggaaccctgtcaggttgccaaggcaataccagcaatttatgacatcagaggcttgaggtctttggttctcaggggctgggaagattcaagttcctctcagctgaagtttatgggaattctactttttcatctctttgcttgtgttctggcttgggaatgaaatacaaaggcctttcgtgggggtagtgagtgattaggccaatgaaatgaatgctcgtgaggttctctctctctctgtctcttccctggatatttctgctttctctccctctcttgggcatttctctcttctggggcttcgcccagtggtattcctgctatttgtgctatgctttttttccaaccccccggcgcccccgcagtgctctcgctctcttcgcatcagtcacgctgtgtcctcctcacaccagaggcatttgtttcctttgatacctcatcctctcctcttttcctcctaccaagctctgtgcagctctgatctgcctcagcactccttcgtttgccatccatttaccttctttgtaccatactctcttcccatctcatcttgttcagcaattcctcccttccccctctttactactgtattaatttcatagtgctttttctgttgacctccactttaggaatattctatcatttctcttccttttaccttctgtattgctatcaacacgttttgtttcattcttccaatttcttattaatcaccccttggttcctcccctgcccccgagtccgcatagattttcctcccttcctttgcacatccctcacgtcatacatttctctaccccatgtgtttattgcaccgaccacccctttctttctttaattctgttcacctctgaaatcgtccatcttctgcccatgtctgcctgctccttttacctttccaagctcctgaggtttggaaaaacaatgatgggctaaaaactaaggtaaactctccagatcctttatccacccttactgttcttcaggctaaatgaacttggctccttacatacgatagcttttattacactaataaacactgcctcattaaaaaaaaatggtgctggatctaaatatgatagtagcaggggcctaggaagaagatgaactaaaaagtgaagaaaaagcaactgatatctagaatgaactgaaggatggggggcaaccaggcagggtggagcttagagtcctagggaatgtccccttacaaaatcaaagttgacagttaactgacataatggcactgactgatggaggggttatatgcccctggaagctcattaaatttatttcttggcctgtttatgtgccttcacaaaccataccccacacctctcccagccctttgcttgctggtactttctgctgctggggttaaaatgctggataagaggaaaagggataaaagaaactagaaacttagggtgatcaagaagaaaaggtaggaagagggcagattatgggaacaaaggtggaaactcagagctcatgggaaacagatggaaaaaaggggtgaagcaaaatggggaaataaaaaatatacaatgatacagtgggggaagggagtaaaattaagtcagcagggaagaggttttgttgtgcgaagctcctggaaaggcagatgacacgcatgagaccagaaggtgaggttctgatgagggagacaggcacatggcaaaggggacagtcaacaatgctaggaagttccaaagcttctctggtgatggtggaagaggaggctgtcctggccatgctgaaggcactagaggctttggcgaagacacatttgctccatcatcccactcctccaggccctgactgtgaccaccacaatcatgactgataagcaaattccaaagtagcctgaaaaggccagagatatccagacagactctgaaggagagggcatggaatcctagaccgacagaacaggcagccaaggcgtgacacatagtgatagagacacacaaggagaggatcactcagatgggaagggtcacaagtggagacagtgacatacagatccagagatggatgggatggaagagacaagatgaagaacagcaaaaccaaaagtcagggacacatggacagagatcagcggggctacaggcacagcgaggaagcgtggtcctgtgcttgaaaatgatagggctgctcagaggggcagacgagcggatgggggtggtaggatgggcgtgcaggacagacacgcttcaccttgaatgggcttatggcctcccctcacctactcaacactttcaaaaaaaggaatggaaagcccaacttcagccaaaaacgaacgaagactgagagtatccacgtcccctcccactccacgccccagcgcgctagcccatccatcagcccgccggccgcggttctcccatcccacagccggcggggggccgccgagacccaggaccctccaggctgacagctctgagccctcacactcaccgggcctccccttccccccgggatccccgctccctgcccaactcggcgcggtccgtctaggctttccatacccttcgtctgtccggcgggcctctg

SEQ ID NO: 17705 - RNA, 8504 nt, Homo sapiens
  source 1..8504: mol_type = other RNA
tccatgtttccttcccccttctttgccttgggctttctttttcgtttcttctttttatcttctttttcaaaattttttggtgttttctcagtggaacatcatgggataacgtgtgtgtgtgcatgtatgtgtatgcatttatggggatggggagctgggaattcagtgaggaaaaggaagatagaaccaaggatatattttgtgtgtggtaggcagacatgtatgaataatcagggtgccaagatgggtgtatgtgtctgtgaagatgggcaagggctacatctgcaaggagctgaggaggaggatcaatgtgtgtgtctgtggggattgggaggaggcaggactctgctggaagtggggtgtgtggtgcccactgagggtgggaactgaacagttcctgtgaggtgggcggggccagggggtggggtgagggatttgagctcccaccgaacaccccttggggtaaaagagggagccctgaggccctcccctctccccatcttggttaatctgtttataaagctagaagtgtagaggtagtcgtagtttttgggttggagtccgtgtgaggtaatcttgcttcctctttggcaaaagccacagcagccgaggcagcagtggcggcgttggtgatggagatgggtgggcccccttgaggtggggctgccttgcgcctgtgggccgaggagcgcaggtgggaggctagggcttcacgcccactcagcagcacctcacatgccaggcagtggtaggtgcagatgggcacccgcaatgggggtggcatggagcccccagagccccgcccaaagaagcagaaggatctctggtgggcagtagccggggcctccccgtcaaatgccatcttgcactggcggcacaggtagcgatgggttacatccacggtggagatgccagtgctgcctgtcagcagctcatcaacctcaccagcttccccctcccctggagcaggcagttcaggaggctttggaggtgctgtggctgtgggctcagggggctggggtggcggctggaggagggcattggggagcagcccaatgagggtctgaggtatcatggggttcatgggaaatagccccttcttcatgccatagagctgttggaagtaggccccctgtagctgggggccaaagacagctggcggtgctgttcccccagcagggggcaatggaaagggcaggaactggccccccaacagggctgggacagtggtcttcaatgctttgaggttcttgagggcatcattggaggagctggtggggcctgcaactggctttcgctcactggagaccttgtcccccaagggctcagtaggagggcctgggacagggtcagtggtgcctgctgtggaggtgttggtttggtcgggcatgggtctctgaggtaaggggcggcctgggccagcagtctggaccactgtggtggtaggcaggaccgaagtggcgaggccgaggaggcctgaggaggctgccgggcctgaattgaaaggagctaagttgcccagcgggggctgagccagagctgggccagataagaggaccggcgccaggcgaggcaaggttggggcagccccgaggggcatggaggcaggtgtggtggcaggtggggccttgagagctgggggagcctcaggtgctggggccaagtcgtagcacttgctttcactcttcagctgggctcgaaccgcctccttgagcttggccaggtgctgacgggaaaagagatggcctcggcaggagacatagaaatcatacttgacatcacaataggggcagtcagtgcgctgggctgctaagaggccctcactgctgcccccagtgctcccagcggctgtcccctgtagtttggccttcttttccttggcacgagcattctggaaccagacctggatgactctcttgggcagcccaatctcctctcccagcacctcacactcctgcatggtgggggtgcggtaagcttcatagcaggctttcatgatcttcagctgcaggctgctcatctgggtcctgtagcgccgctgccccattccatctggaaccccagtcccacctccaggtcccccactggtccctccagccccaggggattctggttcagctaggctggaagcagatgaatcactcagatctcctgcagagagactgcaagcctcactctctggagaagctttaggtggttcctctgggccctcttcctcactgggtggagggggaggtaggagaggtagaggtggctctggtgttggggtggtggcctctttcccaggtggtaggaaaggctggggcccagaagcaagcgtggcagtggggtagggaaaagcaggtgcttccctctttggggcttccctcccagtgccatcatctaccttgcctaataagaggttgaacttgggcaaggatgcaggggtggctgtggcaggcggtttcactgctggactaggcacccccccaggggtgcttcgaaactggcctttcctctcccgggccctggtattctggaaccagacctgtaccactcgctttttgagccccacctcctcggagatgcagtcgagcatcttgcgtgttgggttggaatcctgcatgtaccaacggtacaggatctctagctgctcaggcaagatggtggtgcgcaggcgcttgtccctggggggctcgccctcccctcctccccctgcttcactgcctgtgggagacaagctgccgtcctcatgcttccgtttgagaggtggacctggcattggtgaggtggctgccaccagggggtttctctccccaaacaccagcaagggcagatctaggagttgggggggagcactgggctgcagagatggcaggaaatgtagtcggcggtgactggtcaggaggtcctggctggagaaagaaatggcacactggtcacaggtatgggctggggaaggtgatggagtagccttctcttcaggctctttgcctcctgcctttgttgcctctgcttggctcagctcctccccatctggaggctctggtaatgggccctcaggccctgctggaggttcaaggccctgttcctcctctacttcttcttcttccacctcttcctcctcttcccctctctctgcctcttcctcctcctcttcaagggtctggtcatcatagcacttcttgaggtggcgcaccaactcaaaaacacaggagaaagtggcgtggcaacgcctgcagccggaggctcccccagtgcctcctccggttggcatggacccaccctcacaggcatttttgcgtgctttctggcgggcattctggaaccacaccaccaccacacggctagccagacccaacagacttgcgagtcgctccacctctccgtctttggggtaggcgctagtctcaaagaaagactgcagggcttgggtctggaactctgtgaacttggttctggagaaccggcggccggcaggcaccaggggaggaagattccctctggagctttcttcctcttctatgggccagtgtccccctgctcgacttcgctcttcaggggcacgggtcccccctgcctcaggctctgggaccaggaagggtgggcccagatggggaacaggtgaatccagagacccatcaggaggtttgggaggctctgcaaggggcgggtataggctgtcatagctctttcgaaactgagcagcataacggctcagggcttcaaagggcagaaagcggcggtggacatgttcctcgtgtgtcttgaggataagcatattggagaagagtttcccacaggccccacaggccagcttgtccccacccccgagggcctcaggtgggggtggggtagggggagggggcacagcttgcttcccttcattgtactggatcaccagctcaaagccaaagttttctagaagggctttggctgcagtgcgggcagcctcgttgggcaatgggtcggggggtgaggaaggccctgcctcattaccctctttggccatggggggccgctcccactcccgctcagccagctcagccttgggaggttggggtggaggaggaggggtggcagctggcagggacagcacaggtgcaggcccagctagtgtcagcttgggccccaccttgagatcgtggaggtagaagggcaggagcagctgctgctgctggagcttaagcagtgattcgggcaccagagggaaggggggcaggactggtggggtgaagagaggggctgggaatcggtgcaggtccaagggaggtgggggaggggacaggaaaggcaatccagatatgaagccactggtgtcagggcccttcttctcagtgcccacctccccctctgtctcgccttccttgggctcttcttggctgcgttctggcccttcaatcttggaatcagtcttggttccccgagagcgagtctgatgcagaactgaccgcatgtggatctccagggtggagctctggttgtaggagactctgcagactgtgcacttaaagggcttgtctgtggcagcagtggtggtgggtggggcaccggcctctccccgtgcaggggcagaggggtcaatggcagccttcttcatcttgtgaaggtgggagacagaattataatgaaccaacagaatattcttctgggtgaaggactccttacacacagtgcacttatagggccgggcagggtcgagaaacttgtccagggcaaagttggtggttttccgataggtcagagggtggcgagagtcagctggagctggctctgcagagcggagctccccagtggtcccctcttcctcctcagccatggtgggcggaggagctacgtcttcagcttgggcatcaggttcagggactggagatggggctggagaagggggttggccagggcttcctgagggtttgtctgggacctcaactgaggccaggggaggctcaggaagaggatctggactggcttctggggtcaggttagggccttctgctgcctggtctctgctcggtgtaggctctggcccatgagtggggggttcttggccattgtccagagggcttaatgtgggtgcagacagcactttggttgtaaatgtcatttctacagttgtagctacaagcagcagcttctcaacgcactcgggcaccacgttgtgaaggtggctaaggtggaagtgcagggcaggccggcccaccagctgttcctggcacagtgggcatctgtacttgggctgcactgcatgctgggagagtgtatgagccctcacctggctggactctgggctcaggaagctgcagtatggacagcagtataccgtggtctggttggcactgtctctggaagggccagtcttgttttctgtctcttctgaagccaattgttctgtcttgttctgggcatctttctcaggggtgggtggctcagctaagggggtgacaggagccttcccgggagtccggagctgcccgtggctgaagctcaggatgctctgaagagctgcgagtccttcctcagtggttgggccattctgtagcagctgcagacgcctctgggcctgggcatcgcggtgggcaggtgtgcgcaggtgttgcagcacagccaagcgggagggtgtctcccacgcacacaacaggcagtggtatagccccagctctgcccctgcctccgctccctccatgtccagcagaaacttatagatttggctgttttcttcgtgggctgcacccctggcatgcagctgcatcttctccttgctgttggactcaaagtcacagatgttgcagcgcaggtgtagtggggagacagacccataaggagccccatctcccagggatgctggggaaggggtgcccatggctccacccccctcccgcaggtgggctgccagctggtacttctgagcatgtttgtcagtcttgaggtggagttggaagttggccttgagctgggtgccatagcagcaaagcttgcagcggtgggtgtcaccagccacctccttccattcagcttccgggaggctccggcctatgctgcagtggtagagcagcagctccaggctgtctgtgctgaaggcctggcacactaggcagcggaacaccttcagggacaggctgtcgtctgggggtggtgaggtgggcaggctgtcagatgaggaacccaggagctgacttggaggcaggtgggcatcaggggataggcttccaggggcggatgtggggaacttgcgggcaggtgctcctacgtggtggaaaccattgagaagtagctgggcttccaggggcttgtctggcctcagccccgggccagccaagggagtctgaggctgccctagggcctggggcccaaagtactggaagagttcaggggggctagtgggggtagcccctggtgggggaggagggcctggccccatcaatccaggtggcaggcccagcggcagcccctggtgcagcattaggacattctgcatgtgcttctcagaggtcatatggatgcgcaggttacgggagatgtttgtctcgtagctgcacaccttgcactgccaggatgatttggtcttaggctctttgtctcccgcggagggtgggagtgatgcctctggtggacttccctgcccaccagggcccgcctggaagccctgtaggttggccaggtgcttgtcagactgcatatggatgctgaggttgcctttggtggttgtagagtagttgcagacgtcacagcggtagggtttgtagccacagttgtagctctctccacgagcaaggcgggggtgggcgcccccagcactgcagtagctgcagtgactgttgctctcagggtgcttctctcgcatgtgcacatccagggtctgctggtacttgtagtgccagttgcacttgggacacttgagtgtcttgcaggagttgcgtgagtggagcagggacatgtggctggacaggctgaggccctggaaggctgcaggggctggggtgtagtcatcagctaggcgatagggctggggtgggtcactggggtcttcgggggagcccactggggcagggagagtgcccccctccttggaggtgggtgagctttggttgagtggggggcagagccctccatcctcttcttgcccctcagggaaccaatctggccctgcctcgcctgctgctactggcgattctttggcttgggttgggctggggtcccaggtggctgtgggtggagagggtgggctgagggccataacttcttcatccaggaggataagggcctggacttctgcctcaggggggccatcctctgtctgggccacattcgcctccatgttcactgtgctgctgttgtcaaggggtatgtcagaagaggggcgagcagggagttttggctccagaaagcttatgagggccttgcagccttcatctccctcctggagtacagctgggctacctgacaggccctgatattgggcaggggttagcttcaccccatgagactgtgtgtgatccataaaggcctggggcttgctgaaacccaggcggcacagaaggcagagccagaagaccgccacgtggttgcccccgctgttccccatggggccatctttgggatctccgggtggatttggagccagctggtagctccagaaagctccatgcctttcctcacaggcagccggagatggtgctgaggtatcatgggacagaatttggtcagaagagctaaagccttggattgggtcaaagccatgttggatgtgaagggcagtgaggtgtgaggggggtgggtaggcaaggaagggcagactgggctcttccttgatgcccgcctcaccccaggggaagccctttggtaacaggagttcactgccacctggcagggacagcttggccactaggtaggcctcacctccagctgtgaagaataagtggttgcttaggtccatgggagggagcccttcttcttcctcctcctgctccttgtccttttccacccctgggtcatttggtgggaagtgaccacagtcaggcccttcctggggctccccaatctcctttggtgggacgaggccacagcccgactccaggagctgtccccctggctctgaggacctcatgttctcagaggtggaggaggcagcagggggatctttggtgacaggatcagagggggtgctggaggagaaggtgtccgaaggcagggacggggcattgtgcccaggggagggggtggtaccagtggtagaggctgagttaagggtggccatggtagacggaggagtgctgggggctcatgtcagcgtgacagccagtaccccaggcgcccggggctgccccactgagcaggtgcagcgacccgcccgccgcggcgcatgccgggagttgtagtctgttcgcgcccgcccgcctgcctcgcgggacccagggccgggggcaggccggccagcccaccaggtcgcctccaggttcaagccggtgcctgcaaagagggcaggcccctttaaactcttttccgtctcctctcctcttcatcctgtg

SEQ ID NO: 17706 - RNA, 9524 nt, Homo sapiens
  source 1..9524: mol_type = other RNA
tccatgtttccttcccccttctttgccttgggctttctttttcgtttcttctttttatcttctttttcaaaattttttggtgttttctcagtggaacatcatgggataacgtgtgtgtgtgcatgtatgtgtatgcatttatggggatggggagctgggaattcagtgaggaaaaggaagatagaaccaaggatatattttgtgtgtggtaggcagacatgtatgaataatcagggtgccaagatgggtgtatgtgtctgtgaagatgggcaagggctacatctgcaaggagctgaggaggaggatcaatgtgtgtgtctgtggggattgggaggaggcaggactctgctggaagtggggtgtgtggtgcccactgagggtgggaactgaacagttcctgtgaggtgggcggggccagggggtggggtgagggatttgagctcccaccgaacaccccttggggtaaaagagggagccctgaggccctcccctctccccatcttggttaatctgtttataaagctagaagtgtagaggtagtcgtagtttttgggttggagtccgtgtgaggtaatcttgcttcctctttggcaaaagccacagcagccgaggcagcagtggcggcgttggtgatggagatgggtgggcccccttgaggtggggctgccttgcgcctgtgggccgaggagcgcaggtgggaggctagggcttcacgcccactcagcagcacctcacatgccaggcagtggtaggtgcagatgggcacccgcaatgggggtggcatggagcccccagagccccgcccaaagaagcagaaggatctctggtgggcagtagccggggcctccccgtcaaatgccatcttgcactggcggcacaggtagcgatgggttacatccacggtggagatgccagtgctgcctgtcagcagctcatcaacctcaccagcttccccctcccctggagcaggcagttcaggaggctttggaggtgctgtggctgtgggctcagggggctggggtggcggctggaggagggcattggggagcagcccaatgagggtctgaggtatcatggggttcatgggaaatagccccttcttcatgccatagagctgttggaagtaggccccctgtagctgggggccaaagacagctggcggtgctgttcccccagcagggggcaatggaaagggcaggaactggccccccaacagggctgggacagtggtcttcaatgctttgaggttcttgagggcatcattggaggagctggtggggcctgcaactggctttcgctcactggagaccttgtcccccaagggctcagtaggagggcctgggacagggtcagtggtgcctgctgtggaggtgttggtttggtcgggcatgggtctctgaggtaaggggcggcctgggccagcagtctggaccactgtggtggtaggcaggaccgaagtggcgaggccgaggaggcctgaggaggctgccgggcctgaattgaaaggagctaagttgcccagcgggggctgagccagagctgggccagataagaggaccggcgccaggcgaggcaaggttggggcagccccgaggggcatggaggcaggtgtggtggcaggtggggccttgagagctgggggagcctcaggtgctggggccaagtcgtagcacttgctttcactcttcagctgggctcgaaccgcctccttgagcttggccaggtgctgacgggaaaagagatggcctcggcaggagacatagaaatcatacttgacatcacaataggggcagtcagtgcgctgggctgctaagaggccctcactgctgcccccagtgctcccagcggctgtcccctgtagtttggccttcttttccttggcacgagcattctggaaccagacctggatgactctcttgggcagcccaatctcctctcccagcacctcacactcctgcatggtgggggtgcggtaagcttcatagcaggctttcatgatcttcagctgcaggctgctcatctgggtcctgtagcgccgctgccccattccatctggaaccccagtcccacctccaggtcccccactggtccctccagccccaggggattctggttcagctaggctggaagcagatgaatcactcagatctcctgcagagagactgcaagcctcactctctggagaagctttaggtggttcctctgggccctcttcctcactgggtggagggggaggtaggagaggtagaggtggctctggtgttggggtggtggcctctttcccaggtggtaggaaaggctggggcccagaagcaagcgtggcagtggggtagggaaaagcaggtgcttccctctttggggcttccctcccagtgccatcatctaccttgcctaataagaggttgaacttgggcaaggatgcaggggtggctgtggcaggcggtttcactgctggactaggcacccccccaggggtgcttcgaaactggcctttcctctcccgggccctggtattctggaaccagacctgtaccactcgctttttgagccccacctcctcggagatgcagtcgagcatcttgcgtgttgggttggaatcctgcatgtaccaacggtacaggatctctagctgctcaggcaagatggtggtgcgcaggcgcttgtccctggggggctcgccctcccctcctccccctgcttcactgcctgtgggagacaagctgccgtcctcatgcttccgtttgagaggtggacctggcattggtgaggtggctgccaccagggggtttctctccccaaacaccagcaagggcagatctaggagttgggggggagcactgggctgcagagatggcaggaaatgtagtcggcggtgactggtcaggaggtcctggctggagaaagaaatggcacactggtcacaggtatgggctggggaaggtgatggagtagccttctcttcaggctctttgcctcctgcctttgttgcctctgcttggctcagctcctccccatctggaggctctggtaatgggccctcaggccctgctggaggttcaaggccctgttcctcctctacttcttcttcttccacctcttcctcctcttcccctctctctgcctcttcctcctcctcttcaagggtctggtcatcatagcacttcttgaggtggcgcaccaactcaaaaacacaggagaaagtggcgtggcaacgcctgcagccggaggctcccccagtgcctcctccggttggcatggacccaccctcacaggcatttttgcgtgctttctggcgggcattctggaaccacaccaccaccacacggctagccagacccaacagacttgcgagtcgctccacctctccgtctttggggtaggcgctagtctcaaagaaagactgcagggcttgggtctggaactctgtgaacttggttctggagaaccggcggccggcaggcaccaggggaggaagattccctctggagctttcttcctcttctatgggccagtgtccccctgctcgacttcgctcttcaggggcacgggtcccccctgcctcaggctctgggaccaggaagggtgggcccagatggggaacaggtgaatccagagacccatcaggaggtttgggaggctctgcaaggggcgggtataggctgtcatagctctttcgaaactgagcagcataacggctcagggcttcaaagggcagaaagcggcggtggacatgttcctcgtgtgtcttgaggataagcatattggagaagagtttcccacaggccccacaggccagcttgtccccacccccgagggcctcaggtgggggtggggtagggggagggggcacagcttgcttcccttcattgtactggatcaccagctcaaagccaaagttttctagaagggctttggctgcagtgcgggcagcctcgttgggcaatgggtcggggggtgaggaaggccctgcctcattaccctctttggccatggggggccgctcccactcccgctcagccagctcagccttgggaggttggggtggaggaggaggggtggcagctggcagggacagcacaggtgcaggcccagctagtgtcagcttgggccccaccttgagatcgtggaggtagaagggcaggagcagctgctgctgctggagcttaagcagtgattcgggcaccagagggaaggggggcaggactggtggggtgaagagaggggctgggaatcggtgcaggtccaagggaggtgggggaggggacaggaaaggcaatccagatatgaagccactggtgtcagggcccttcttctcagtgcccacctccccctctgtctcgccttccttgggctcttcttggctgcgttctggcccttcaatcttggaatcagtcttggttccccgagagcgagtctgatgcagaactgaccgcatgtggatctccagggtggagctctggttgtaggagactctgcagactgtgcacttaaagggcttgtctgtggcagcagtggtggtgggtggggcaccggcctctccccgtgcaggggcagaggggtcaatggcagccttcttcatcttgtgaaggtgggagacagaattataatgaaccaacagaatattcttctgggtgaaggactccttacacacagtgcacttatagggccgggcagggtcgagaaacttgtccagggcaaagttggtggttttccgataggtcagagggtggcgagagtcagctggagctggctctgcagagcggagctccccagtggtcccctcttcctcctcagccatggtgggcggaggagctacgtcttcagcttgggcatcaggttcagggactggagatggggctggagaagggggttggccagggcttcctgagggtttgtctgggacctcaactgaggccaggggaggctcaggaagaggatctggactggcttctggggtcaggttagggccttctgctgcctggtctctgctcggtgtaggctctggcccatgagtggggggttcttggccattgtccagagggcttaatgtgggtgcagacagcactttggttgtaaatgtcatttctacagttgtagctacaagcagcagcttctcaacgcactcgggcaccacgttgtgaaggtggctaaggtggaagtgcagggcaggccggcccaccagctgttcctggcacagtgggcatctgtacttgggctgcactgcatgctgggagagtgtatgagccctcacctggctggactctgggctcaggaagctgcagtatggacagcagtataccgtggtctggttggcactgtctctggaagggccagtcttgttttctgtctcttctgaagccaattgttctgtcttgttctgggcatctttctcaggggtgggtggctcagctaagggggtgacaggagccttcccgggagtccggagctgcccgtggctgaagctcaggatgctctgaagagctgcgagtccttcctcagtggttgggccattctgtagcagctgcagacgcctctgggcctgggcatcgcggtgggcaggtgtgcgcaggtgttgcagcacagccaagcgggagggtgtctcccacgcacacaacaggcagtggtatagccccagctctgcccctgcctccgctccctccatgtccagcagaaacttatagatttggctgttttcttcgtgggctgcacccctggcatgcagctgcatcttctccttgctgttggactcaaagtcacagatgttgcagcgcaggtgtagtggggagacagacccataaggagccccatctcccagggatgctggggaaggggtgcccatggctccacccccctcccgcaggtgggctgccagctggtacttctgagcatgtttgtcagtcttgaggtggagttggaagttggccttgagctgggtgccatagcagcaaagcttgcagcggtgggtgtcaccagccacctccttccattcagcttccgggaggctccggcctatgctgcagtggtagagcagcagctccaggctgtctgtgctgaaggcctggcacactaggcagcggaacaccttcagggacaggctgtcgtctgggggtggtgaggtgggcaggctgtcagatgaggaacccaggagctgacttggaggcaggtgggcatcaggggataggcttccaggggcggatgtggggaacttgcgggcaggtgctcctacgtggtggaaaccattgagaagtagctgggcttccaggggcttgtctggcctcagccccgggccagccaagggagtctgaggctgccctagggcctggggcccaaagtactggaagagttcaggggggctagtgggggtagcccctggtgggggaggagggcctggccccatcaatccaggtggcaggcccagcggcagcccctggtgcagcattaggacattctgcatgtgcttctcagaggtcatatggatgcgcaggttacgggagatgtttgtctcgtagctgcacaccttgcactgccaggatgatttggtcttaggctctttgtctcccgcggagggtgggagtgatgcctctggtggacttccctgcccaccagggcccgcctggaagccctgtaggttggccaggtgcttgtcagactgcatatggatgctgaggttgcctttggtggttgtagagtagttgcagacgtcacagcggtagggtttgtagccacagttgtagctctctccacgagcaaggcgggggtgggcgcccccagcactgcagtagctgcagtgactgttgctctcagggtgcttctctcgcatgtgcacatccagggtctgctggtacttgtagtgccagttgcacttgggacacttgagtgtcttgcaggagttgcgtgagtggagcagggacatgtggctggacaggctgaggccctggaaggctgcaggggctggggtgtagtcatcagctaggcgatagggctggggtgggtcactggggtcttcgggggagcccactggggcagggagagtgcccccctccttggaggtgggtgagctttggttgagtggggggcagagccctccatcctcttcttgcccctcagggaaccaatctggccctgcctcgcctgctgctactggcgattctttggcttgggttgggctggggtcccaggtggctgtgggtggagagggtgggctgagggccataacttcttcatccaggaggataagggcctggacttctgcctcaggggggccatcctctgtctgggccacattcgcctccatgttcactgtgctgctgttgtcaaggggtatgtcagaagaggggcgagcagggagttttggctccagaaagcttatgagggccttgcagccttcatctccctcctggagtacagctgggctacctgacaggccctgatattgggcaggggttagcttcaccccatgagactgtgtgtgatccataaaggcctggggcttgctgaaacccaggcggcacagaaggcagagccagaagaccgccacgtggttgcccccgctgttccccatggggccatctttgggatctccgggtggatttggagccagctggtagctccagaaagctccatgcctttcctcacaggcagccggagatggtgctgaggtatcatgggacagaatttggtcagaagagctaaagccttggattgggtcaaagccatgttggatgtgaagggcagtgaggtgtgaggggggtgggtaggcaaggaagggcagactgggctcttccttgatgcccgcctcaccccaggggaagccctttggtaacaggagttcactgccacctggcagggacagcttggccactaggtaggcctcacctccagctgtgaagaataagtggttgcttaggtccatgggagggagcccttcttcttcctcctcctgctccttgtccttttccacccctgggtcatttggtgggaagtgaccacagtcaggcccttcctggggctccccaatctcctttggtgggacgaggccacagcccgactccaggagctgtccccctggctctgaggacctcatgttctcagaggtggaggaggcagcagggggatctttggtgacaggatcagagggggtgctggaggagaaggtgtccgaaggcagggacggggcattgtgcccaggggagggggtggtaccagtggtagaggctgagttaagggtggccatggtagacggaggagtgctgggggctcatgtcagcgtgacagccagtaccctctggagtctttcaacaatggagagtcagatgtcaaggccatccctcacagggttctttacatcaagatctgggcagcagtaacttctccctcctttggccttttggcccacatggccaatgctgccttcgttgtattaataattacctggcttgggataggtgtttagaatgggtctggtattgatttatgaactccttatttgcggccattgtatatatacggttatgaccaattcaattgtagtttcatgattgggaatggggtggggatgctacttttaattcacatttgccaactctctctttggaaacaactctcaaccttttctggaaaccgcctcctttctcttccctcctccacatcttcctcttgggctcctagggctgttcattcatgttttcctccaattatcactacaaagactctgcacatgagccctgagagttcccctggctgcctccaagtgtgaccctaacccagtctctcctgtctgcctcagatctcactgtcactggttaactaccctccagccattccctccggtttctgatttcccagtttgcccattaatgtagacttaggtggggggagtgggtgaaaattaggtgggcaactctttcccccagcctctccctactaattcaacgtttgatcagtagatatttattaagccttttctgtgtgacagacactgtgctaggtgctggaaaacaattggaaactagacagatgtagccactcctcagatgaccatgtgactaaccctgagtctctcaccagacagctaagtctctcagactaggggactctgtcccatttcccccctttctgtacagccaaattccactgtgccctctggcatttcacaacccttcccttttctcaatccctgaatgagtttacactcacacagccccgatcccttccctctgcattctagctttagtctccattcctaaacccaaagccattacactttcaacaactctcctccccactcacaaagcccttctcctttcacattctgtaactgccatttctagtcctcctcttccgtctctgcctgccttttgatccaaccatcctgacctcaatgccctgtcttaggttccttcctcttgctactgtcaggctctagcaaacctcaggtgctcacaaacaggagttatttgtgacaactgttgttctgagctgggaagagctccagggaggcaaggtcaagctaccagagtcagaaa

SEQ ID NO: 17707 - RNA, 8875 nt, Homo sapiens
  source 1..8875: mol_type = other RNA
tccatgtttccttcccccttctttgccttgggctttctttttcgtttcttctttttatcttctttttcaaaattttttggtgttttctcagtggaacatcatgggataacgtgtgtgtgtgcatgtatgtgtatgcatttatggggatggggagctgggaattcagtgaggaaaaggaagatagaaccaaggatatattttgtgtgtggtaggcagacatgtatgaataatcagggtgccaagatgggtgtatgtgtctgtgaagatgggcaagggctacatctgcaaggagctgaggaggaggatcaatgtgtgtgtctgtggggattgggaggaggcaggactctgctggaagtggggtgtgtggtgcccactgagggtgggaactgaacagttcctgtgaggtgggcggggccagggggtggggtgagggatttgagctcccaccgaacaccccttggggtaaaagagggagccctgaggccctcccctctccccatcttggttaatctgtttataaagctagaagtgtagaggtagtcgtagtttttgggttggagtccgtgtgaggtaatcttgcttcctctttggcaaaagccacagcagccgaggcagcagtggcggcgttggtgatggagatgggtgggcccccttgaggtggggctgccttgcgcctgtgggccgaggagcgcaggtgggaggctagggcttcacgcccactcagcagcacctcacatgccaggcagtggtaggtgcagatgggcacccgcaatgggggtggcatggagcccccagagccccgcccaaagaagcagaaggatctctggtgggcagtagccggggcctccccgtcaaatgccatcttgcactggcggcacaggtagcgatgggttacatccacggtggagatgccagtgctgcctgtcagcagctcatcaacctcaccagcttccccctcccctggagcaggcagttcaggaggctttggaggtgctgtggctgtgggctcagggggctggggtggcggctggaggagggcattggggagcagcccaatgagggtctgaggtatcatggggttcatgggaaatagccccttcttcatgccatagagctgttggaagtaggccccctgtagctgggggccaaagacagctggcggtgctgttcccccagcagggggcaatggaaagggcaggaactggccccccaacagggctgggacagtggtcttcaatgctttgaggttcttgagggcatcattggaggagctggtggggcctgcaactggctttcgctcactggagaccttgtcccccaagggctcagtaggagggcctgggacagggtcagtggtgcctgctgtggaggtgttggtttggtcgggcatgggtctctgaggtaaggggcggcctgggccagcagtctggaccactgtggtggtaggcaggaccgaagtggcgaggccgaggaggcctgaggaggctgccgggcctgaattgaaaggagctaagttgcccagcgggggctgagccagagctgggccagataagaggaccggcgccaggcgaggcaaggttggggcagccccgaggggcatggaggcaggtgtggtggcaggtggggccttgagagctgggggagcctcaggtgctggggccaagtcgtagcacttgctttcactcttcagctgggctcgaaccgcctccttgagcttggccaggtgctgacgggaaaagagatggcctcggcaggagacatagaaatcatacttgacatcacaataggggcagtcagtgcgctgggctgctaagaggccctcactgctgcccccagtgctcccagcggctgtcccctgtagtttggccttcttttccttggcacgagcattctggaaccagacctggatgactctcttgggcagcccaatctcctctcccagcacctcacactcctgcatggtgggggtgcggtaagcttcatagcaggctttcatgatcttcagctgcaggctgctcatctgggtcctgtagcgccgctgccccattccatctggaaccccagtcccacctccaggtcccccactggtccctccagccccaggggattctggttcagctaggctggaagcagatgaatcactcagatctcctgcagagagactgcaagcctcactctctggagaagctttaggtggttcctctgggccctcttcctcactgggtggagggggaggtaggagaggtagaggtggctctggtgttggggtggtggcctctttcccaggtggtaggaaaggctggggcccagaagcaagcgtggcagtggggtagggaaaagcaggtgcttccctctttggggcttccctcccagtgccatcatctaccttgcctaataagaggttgaacttgggcaaggatgcaggggtggctgtggcaggcggtttcactgctggactaggcacccccccaggggtgcttcgaaactggcctttcctctcccgggccctggtattctggaaccagacctgtaccactcgctttttgagccccacctcctcggagatgcagtcgagcatcttgcgtgttgggttggaatcctgcatgtaccaacggtacaggatctctagctgctcaggcaagatggtggtgcgcaggcgcttgtccctggggggctcgccctcccctcctccccctgcttcactgcctgtgggagacaagctgccgtcctcatgcttccgtttgagaggtggacctggcattggtgaggtggctgccaccagggggtttctctccccaaacaccagcaagggcagatctaggagttgggggggagcactgggctgcagagatggcaggaaatgtagtcggcggtgactggtcaggaggtcctggctggagaaagaaatggcacactggtcacaggtatgggctggggaaggtgatggagtagccttctcttcaggctctttgcctcctgcctttgttgcctctgcttggctcagctcctccccatctggaggctctggtaatgggccctcaggccctgctggaggttcaaggccctgttcctcctctacttcttcttcttccacctcttcctcctcttcccctctctctgcctcttcctcctcctcttcaagggtctggtcatcatagcacttcttgaggtggcgcaccaactcaaaaacacaggagaaagtggcgtggcaacgcctgcagccggaggctcccccagtgcctcctccggttggcatggacccaccctcacaggcatttttgcgtgctttctggcgggcattctggaaccacaccaccaccacacggctagccagacccaacagacttgcgagtcgctccacctctccgtctttggggtaggcgctagtctcaaagaaagactgcagggcttgggtctggaactctgtgaacttggttctggagaaccggcggccggcaggcaccaggggaggaagattccctctggagctttcttcctcttctatgggccagtgtccccctgctcgacttcgctcttcaggggcacgggtcccccctgcctcaggctctgggaccaggaagggtgggcccagatggggaacaggtgaatccagagacccatcaggaggtttgggaggctctgcaaggggcgggtataggctgtcatagctctttcgaaactgagcagcataacggctcagggcttcaaagggcagaaagcggcggtggacatgttcctcgtgtgtcttgaggataagcatattggagaagagtttcccacaggccccacaggccagcttgtccccacccccgagggcctcaggtgggggtggggtagggggagggggcacagcttgcttcccttcattgtactggatcaccagctcaaagccaaagttttctagaagggctttggctgcagtgcgggcagcctcgttgggcaatgggtcggggggtgaggaaggccctgcctcattaccctctttggccatggggggccgctcccactcccgctcagccagctcagccttgggaggttggggtggaggaggaggggtggcagctggcagggacagcacaggtgcaggcccagctagtgtcagcttgggccccaccttgagatcgtggaggtagaagggcaggagcagctgctgctgctggagcttaagcagtgattcgggcaccagagggaaggggggcaggactggtggggtgaagagaggggctgggaatcggtgcaggtccaagggaggtgggggaggggacaggaaaggcaatccagatatgaagccactggtgtcagggcccttcttctcagtgcccacctccccctctgtctcgccttccttgggctcttcttggctgcgttctggcccttcaatcttggaatcagtcttggttccccgagagcgagtctgatgcagaactgaccgcatgtggatctccagggtggagctctggttgtaggagactctgcagactgtgcacttaaagggcttgtctgtggcagcagtggtggtgggtggggcaccggcctctccccgtgcaggggcagaggggtcaatggcagccttcttcatcttgtgaaggtgggagacagaattataatgaaccaacagaatattcttctgggtgaaggactccttacacacagtgcacttatagggccgggcagggtcgagaaacttgtccagggcaaagttggtggttttccgataggtcagagggtggcgagagtcagctggagctggctctgcagagcggagctccccagtggtcccctcttcctcctcagccatggtgggcggaggagctacgtcttcagcttgggcatcaggttcagggactggagatggggctggagaagggggttggccagggcttcctgagggtttgtctgggacctcaactgaggccaggggaggctcaggaagaggatctggactggcttctggggtcaggttagggccttctgctgcctggtctctgctcggtgtaggctctggcccatgagtggggggttcttggccattgtccagagggcttaatgtgggtgcagacagcactttggttgtaaatgtcatttctacagttgtagctacaagcagcagcttctcaacgcactcgggcaccacgttgtgaaggtggctaaggtggaagtgcagggcaggccggcccaccagctgttcctggcacagtgggcatctgtacttgggctgcactgcatgctgggagagtgtatgagccctcacctggctggactctgggctcaggaagctgcagtatggacagcagtataccgtggtctggttggcactgtctctggaagggccagtcttgttttctgtctcttctgaagccaattgttctgtcttgttctgggcatctttctcaggggtgggtggctcagctaagggggtgacaggagccttcccgggagtccggagctgcccgtggctgaagctcaggatgctctgaagagctgcgagtccttcctcagtggttgggccattctgtagcagctgcagacgcctctgggcctgggcatcgcggtgggcaggtgtgcgcaggtgttgcagcacagccaagcgggagggtgtctcccacgcacacaacaggcagtggtatagccccagctctgcccctgcctccgctccctccatgtccagcagaaacttatagatttggctgttttcttcgtgggctgcacccctggcatgcagctgcatcttctccttgctgttggactcaaagtcacagatgttgcagcgcaggtgtagtggggagacagacccataaggagccccatctcccagggatgctggggaaggggtgcccatggctccacccccctcccgcaggtgggctgccagctggtacttctgagcatgtttgtcagtcttgaggtggagttggaagttggccttgagctgggtgccatagcagcaaagcttgcagcggtgggtgtcaccagccacctccttccattcagcttccgggaggctccggcctatgctgcagtggtagagcagcagctccaggctgtctgtgctgaaggcctggcacactaggcagcggaacaccttcagggacaggctgtcgtctgggggtggtgaggtgggcaggctgtcagatgaggaacccaggagctgacttggaggcaggtgggcatcaggggataggcttccaggggcggatgtggggaacttgcgggcaggtgctcctacgtggtggaaaccattgagaagtagctgggcttccaggggcttgtctggcctcagccccgggccagccaagggagtctgaggctgccctagggcctggggcccaaagtactggaagagttcaggggggctagtgggggtagcccctggtgggggaggagggcctggccccatcaatccaggtggcaggcccagcggcagcccctggtgcagcattaggacattctgcatgtgcttctcagaggtcatatggatgcgcaggttacgggagatgtttgtctcgtagctgcacaccttgcactgccaggatgatttggtcttaggctctttgtctcccgcggagggtgggagtgatgcctctggtggacttccctgcccaccagggcccgcctggaagccctgtaggttggccaggtgcttgtcagactgcatatggatgctgaggttgcctttggtggttgtagagtagttgcagacgtcacagcggtagggtttgtagccacagttgtagctctctccacgagcaaggcgggggtgggcgcccccagcactgcagtagctgcagtgactgttgctctcagggtgcttctctcgcatgtgcacatccagggtctgctggtacttgtagtgccagttgcacttgggacacttgagtgtcttgcaggagttgcgtgagtggagcagggacatgtggctggacaggctgaggccctggaaggctgcaggggctggggtgtagtcatcagctaggcgatagggctggggtgggtcactggggtcttcgggggagcccactggggcagggagagtgcccccctccttggaggtgggtgagctttggttgagtggggggcagagccctccatcctcttcttgcccctcagggaaccaatctggccctgcctcgcctgctgctactggcgattctttggcttgggttgggctggggtcccaggtggctgtgggtggagagggtgggctgagggccataacttcttcatccaggaggataagggcctggacttctgcctcaggggggccatcctctgtctgggccacattcgcctccatgttcactgtgctgctgttgtcaaggggtatgtcagaagaggggcgagcagggagttttggctccagaaagcttatgagggccttgcagccttcatctccctcctggagtacagctgggctacctgacaggccctgatattgggcaggggttagcttcaccccatgagactgtgtgtgatccataaaggcctggggcttgctgaaacccaggcggcacagaaggcagagccagaagaccgccacgtggttgcccccgctgttccccatggggccatctttgggatctccgggtggatttggagccagctggtagctccagaaagctccatgcctttcctcacaggcagccggagatggtgctgaggtatcatgggacagaatttggtcagaagagctaaagccttggattgggtcaaagccatgttggatgtgaagggcagtgaggtgtgaggggggtgggtaggcaaggaagggcagactgggctcttccttgatgcccgcctcaccccaggggaagccctttggtaacaggagttcactgccacctggcagggacagcttggccactaggtaggcctcacctccagctgtgaagaataagtggttgcttaggtccatgggagggagcccttcttcttcctcctcctgctccttgtccttttccacccctgggtcatttggtgggaagtgaccacagtcaggcccttcctggggctccccaatctcctttggtgggacgaggccacagcccgactccaggagctgtccccctggctctgaggacctcatgttctcagaggtggaggaggcagcagggggatctttggtgacaggatcagagggggtgctggaggagaaggtgtccgaaggcagggacggggcattgtgcccaggggagggggtggtaccagtggtagaggctgagttaagggtggccatggtagacggaggagtgctgggggctcatgtcagcgtgacagccagtaccctgcgcttagctggctgctatagcagatatctgttggacggtgtgaatggcttgtattccaggcccatctgcctgcgttgggggtgcggcggggggtgttggagacgggactggggcttgagctccttgcacccgactctccccgccgccttgtagccccagttcagctttaggtagagtaccgcaggcaccaagtgcagctttcctgtcgccatagcgacgggcggggcgagatggcaaagtctccctttggaactacatctcccatcatgcatccgcgcctcggggtgcctggctcagcctcaggcatgagacctgtaccagcccccgggagccgtgcggggccaacaatgaggagcagaatgcaaggggcggcctcgctcccctggccaccgcgggggtcgcggcctcccattacatagcgcgtgtctcgagccctggcctgctctcggcaccgccacaacgggcgtaatatggccgctggtgccgggacctgccgggcgcgcggagggtcgggccgaggtccgggatccggaactgctcccggcattcctcgcgagtgtatggcgtgggctcccttccccctctgtggg

SEQ ID NO: 17708 - RNA, 5727 nt, Homo sapiens
  source 1..5727: mol_type = other RNA
tccatgtttccttcccccttctttgccttgggctttctttttcgtttcttctttttatcttctttttcaaaattttttggtgttttctcagtggaacatcatgggataacgtgtgtgtgtgcatgtatgtgtatgcatttatggggatggggagctgggaattcagtgaggaaaaggaagatagaaccaaggatatattttgtgtgtggtaggcagacatgtatgaataatcagggtgccaagatgggtgtatgtgtctgtgaagatgggcaagggctacatctgcaaggagctgaggaggaggatcaatgtgtgtgtctgtggggattgggaggaggcaggactctgctggaagtggggtgtgtggtgcccactgagggtgggaactgaacagttcctgtgaggtgggcggggccagggggtggggtgagggatttgagctcccaccgaacaccccttggggtaaaagagggagccctgaggccctcccctctccccatcttggttaatctgtttataaagctagaagtgtagaggtagtcgtagtttttgggttggagtccgtgtgaggtaatcttgcttcctctttggcaaaagccacagcagccgaggcagcagtggcggcgttggtgatggagatgggtgggcccccttgaggtggggctgccttgcgcctgtgggccgaggagcgcaggtgggaggctagggcttcacgcccactcagcagcacctcacatgccaggcagtggtaggtgcagatgggcacccgcaatgggggtggcatggagcccccagagccccgcccaaagaagcagaaggatctctggtgggcagtagccggggcctccccgtcaaatgccatcttgcactggcggcacaggtagcgatgggttacatccacggtggagatgccagtgctgcctgtcagcagctcatcaacctcaccagcttccccctcccctggagcaggcagttcaggaggctttggaggtgctgtggctgtgggctcagggggctggggtggcggctggaggagggcattggggagcagcccaatgagggtctgaggtatcatggggttcatgggaaatagccccttcttcatgccatagagctgttggaagtaggccccctgtagctgggggccaaagacagctggcggtgctgttcccccagcagggggcaatggaaagggcaggaactggccccccaacagggctgggacagtggtcttcaatgctttgaggttcttgagggcatcattggaggagctggtggggcctgcaactggctttcgctcactggagaccttgtcccccaagggctcagtaggagggcctgggacagggtcagtggtgcctgctgtggaggtgttggtttggtcgggcatgggtctctgaggtaaggggcggcctgggccagcagtctggaccactgtggtggtaggcaggaccgaagtggcgaggccgaggaggcctgaggaggctgccgggcctgaattgaaaggagctaagttgcccagcgggggctgagccagagctgggccagataagaggaccggcgccaggcgaggcaaggttggggcagccccgaggggcatggaggcaggtgtggtggcaggtggggccttgagagctgggggagcctcaggtgctggggccaagtcgtagcacttgctttcactcttcagctgggctcgaaccgcctccttgagcttggccaggtgctgacgggaaaagagatggcctcggcaggagacatagaaatcatacttgacatcacaataggggcagtcagtgcgctgggctgctaagaggccctcactgctgcccccagtgctcccagcggctgtcccctgtagtttggccttcttttccttggcacgagcattctggaaccagacctggatgactctcttgggcagcccaatctcctctcccagcacctcacactcctgcatggtgggggtgcggtaagcttcatagcaggctttcatgatcttcagctgcaggctgctcatctgggtcctgtagcgccgctgccccattccatctggaaccccagtcccacctccaggtcccccactggtccctccagccccaggggattctggttcagctaggctggaagcagatgaatcactcagatctcctgcagagagactgcaagcctcactctctggagaagctttaggtggttcctctgggccctcttcctcactgggtggagggggaggtaggagaggtagaggtggctctggtgttggggtggtggcctctttcccaggtggtaggaaaggctggggcccagaagcaagcgtggcagtggggtagggaaaagcaggtgcttccctctttggggcttccctcccagtgccatcatctaccttgcctaataagaggttgaacttgggcaaggatgcaggggtggctgtggcaggcggtttcactgctggactaggcacccccccaggggtgcttcgaaactggcctttcctctcccgggccctggtattctggaaccagacctgtaccactcgctttttgagccccacctcctcggagatgcagtcgagcatcttgcgtgttgggttggaatcctgcatgtaccaacggtacaggatctctagctgctcaggcaagatggtggtgcgcaggcgcttgtccctggggggctcgccctcccctcctccccctgcttcactgcctgtgggagacaagctgccgtcctcatgcttccgtttgagaggtggacctggcattggtgaggtggctgccaccagggggtttctctccccaaacaccagcaagggcagatctaggagttgggggggagcactgggctgcagagatggcaggaaatgtagtcggcggtgactggtcaggaggtcctggctggagaaagaaatggcacactggtcacaggtatgggctggggaaggtgatggagtagccttctcttcaggctctttgcctcctgcctttgttgcctctgcttggctcagctcctccccatctggaggctctggtaatgggccctcaggccctgctggaggttcaaggccctgttcctcctctacttcttcttcttccacctcttcctcctcttcccctctctctgcctcttcctcctcctcttcaagggtctggtcatcatagcacttcttgaggtggcgcaccaactcaaaaacacaggagaaagtggcgtggcaacgcctgcagccggaggctcccccagtgcctcctccggttggcatggacccaccctcacaggcatttttgcgtgctttctggcgggcattctggaaccacaccaccaccacacggctagccagacccaacagacttgcgagtcgctccacctctccgtctttggggtaggcgctagtctcaaagaaagactgcagggcttgggtctggaactctgtgaacttggttctggagaaccggcggccggcaggcaccaggggaggaagattccctctggagctttcttcctcttctatgggccagtgtccccctgctcgacttcgctcttcaggggcacgggtcccccctgcctcaggctctgggaccaggaagggtgggcccagatggggaacaggtgaatccagagacccatcaggaggtttgggaggctctgcaaggggcgggtataggctgtcatagctctttcgaaactgagcagcataacggctcagggcttcaaagggcagaaagcggcggtggacatgttcctcgtgtgtcttgaggataagcatattggagaagagtttcccacaggccccacaggccagcttgtccccacccccgagggcctcaggtgggggtggggtagggggagggggcacagcttgcttcccttcattgtactggatcaccagctcaaagccaaagttttctagaagggctttggctgcagtgcgggcagcctcgttgggcaatgggtcggggggtgaggaaggccctgcctcattaccctctttggccatggggggccgctcccactcccgctcagccagctcagccttgggaggttggggtggaggaggaggggtggcagctggcagggacagcacaggtgcaggcccagctagtgtcagcttgggccccaccttgagatcgtggaggtagaagggcaggagcagctgctgctgctggagcttaagcagtgattcgggcaccagagggaaggggggcaggactggtggggtgaagagaggggctgggaatcggtgcaggtccaagggaggtgggggaggggacaggaaaggcaatccagatatgaagccactggtgtcagggcccttcttctcagtgcccacctccccctctgtctcgccttccttgggctcttcttggctgcgttctggcccttcaatcttggaatcagtcttggttccccgagagcgagtctgatgcagaactgaccgcatgtggatctccagggtggagctctggttgtaggagactctgcagactgtgcacttaaagggcttgtctgtggcagcagtggtggtgggtggggcaccggcctctccccgtgcaggggcagaggggtcaatggcagccttcttcatcttgtgaaggtgggagacagaattataatgaaccaacagaatattcttctgggtgaaggactccttacacacagtgcacttatagggccgggcagggtcgagaaacttgtccagggcaaagttggtggttttccgataggtcagagggtggcgagagtcagctggagctggctctgcagagcggagctccccagtggtcccctcttcctcctcagccatggtgggcggaggagctacgtcttcagcttgggcatcaggttcagggactggagatggggctggagaagggggttggccagggcttcctgagggtttgtctgggacctcaactgaggccaggggaggctcaggaagaggatctggactggcttctggggtcaggttagggccttctgctgcctggtctctgctcggtgtaggctctggcccatgagtggggggttcttggccattgtccagagggcttaatgtgggtgcagacagcactttggttgtaaatgtcatttctacagttgtagctacaagcagcagcttctcaacgcactcgggcaccacgttgtgaaggtggctaaggtggaagtgcagggcaggccggcccaccagctgttcctggcacagtgggcatctgtacttgggctgcactgcatgctgggagagtgtatgagccctcacctggctggactctgggctcaggaagctgcagtatggacagcagtatacctgtctgctcagaagccagctcatcctccctcaggctcagcagctcccaccttattttccatctttctttttccttcttctttttcccttagtaagaggatgccaggacagttccatccaggctcagggcgttttgtagggtaggaacaccggtgtcttgtctttctgctcctaactaagggataaagagctgggcagtagctggttgtttgcttttgcctttctcctcccctccttccagcatgtacccccactctttcctactctcagcacaattcctttattcatctttccctcaagttcctgctgtctccctcctatcatctccctctgtgcttgaccctgctgggccagctctgcccccgaaagtgctgaacatgtggaactggatctgggtggaatttcttaactgtgctattctgagtgaa

SEQ ID NO: 17709 - RNA, 5752 nt, Homo sapiens
  source 1..5752: mol_type = other RNA
tccatgtttccttcccccttctttgccttgggctttctttttcgtttcttctttttatcttctttttcaaaattttttggtgttttctcagtggaacatcatgggataacgtgtgtgtgtgcatgtatgtgtatgcatttatggggatggggagctgggaattcagtgaggaaaaggaagatagaaccaaggatatattttgtgtgtggtaggcagacatgtatgaataatcagggtgccaagatgggtgtatgtgtctgtgaagatgggcaagggctacatctgcaaggagctgaggaggaggatcaatgtgtgtgtctgtggggattgggaggaggcaggactctgctggaagtggggtgtgtggtgcccactgagggtgggaactgaacagttcctgtgaggtgggcggggccagggggtggggtgagggatttgagctcccaccgaacaccccttggggtaaaagagggagccctgaggccctcccctctccccatcttggttaatctgtttataaagctagaagtgtagaggtagtcgtagtttttgggttggagtccgtgtgaggtaatcttgcttcctctttggcaaaagccacagcagccgaggcagcagtggcggcgttggtgatggagatgggtgggcccccttgaggtggggctgccttgcgcctgtgggccgaggagcgcaggtgggaggctagggcttcacgcccactcagcagcacctcacatgccaggcagtggtaggtgcagatgggcacccgcaatgggggtggcatggagcccccagagccccgcccaaagaagcagaaggatctctggtgggcagtagccggggcctccccgtcaaatgccatcttgcactggcggcacaggtagcgatgggttacatccacggtggagatgccagtgctgcctgtcagcagctcatcaacctcaccagcttccccctcccctggagcaggcagttcaggaggctttggaggtgctgtggctgtgggctcagggggctggggtggcggctggaggagggcattggggagcagcccaatgagggtctgaggtatcatggggttcatgggaaatagccccttcttcatgccatagagctgttggaagtaggccccctgtagctgggggccaaagacagctggcggtgctgttcccccagcagggggcaatggaaagggcaggaactggccccccaacagggctgggacagtggtcttcaatgctttgaggttcttgagggcatcattggaggagctggtggggcctgcaactggctttcgctcactggagaccttgtcccccaagggctcagtaggagggcctgggacagggtcagtggtgcctgctgtggaggtgttggtttggtcgggcatgggtctctgaggtaaggggcggcctgggccagcagtctggaccactgtggtggtaggcaggaccgaagtggcgaggccgaggaggcctgaggaggctgccgggcctgaattgaaaggagctaagttgcccagcgggggctgagccagagctgggccagataagaggaccggcgccaggcgaggcaaggttggggcagccccgaggggcatggaggcaggtgtggtggcaggtggggccttgagagctgggggagcctcaggtgctggggccaagtcgtagcacttgctttcactcttcagctgggctcgaaccgcctccttgagcttggccaggtgctgacgggaaaagagatggcctcggcaggagacatagaaatcatacttgacatcacaataggggcagtcagtgcgctgggctgctaagaggccctcactgctgcccccagtgctcccagcggctgtcccctgtagtttggccttcttttccttggcacgagcattctggaaccagacctggatgactctcttgggcagcccaatctcctctcccagcacctcacactcctgcatggtgggggtgcggtaagcttcatagcaggctttcatgatcttcagctgcaggctgctcatctgggtcctgtagcgccgctgccccattccatctggaaccccagtcccacctccaggtcccccactggtccctccagccccaggggattctggttcagctaggctggaagcagatgaatcactcagatctcctgcagagagactgcaagcctcactctctggagaagctttaggtggttcctctgggccctcttcctcactgggtggagggggaggtaggagaggtagaggtggctctggtgttggggtggtggcctctttcccaggtggtaggaaaggctggggcccagaagcaagcgtggcagtggggtagggaaaagcaggtgcttccctctttggggcttccctcccagtgccatcatctaccttgcctaataagaggttgaacttgggcaaggatgcaggggtggctgtggcaggcggtttcactgctggactaggcacccccccaggggtgcttcgaaactggcctttcctctcccgggccctggtattctggaaccagacctgtaccactcgctttttgagccccacctcctcggagatgcagtcgagcatcttgcgtgttgggttggaatcctgcatgtaccaacggtacaggatctctagctgctcaggcaagatggtggtgcgcaggcgcttgtccctggggggctcgccctcccctcctccccctgcttcactgcctgtgggagacaagctgccgtcctcatgcttccgtttgagaggtggacctggcattggtgaggtggctgccaccagggggtttctctccccaaacaccagcaagggcagatctaggagttgggggggagcactgggctgcagagatggcaggaaatgtagtcggcggtgactggtcaggaggtcctggctggagaaagaaatggcacactggtcacaggtatgggctggggaaggtgatggagtagccttctcttcaggctctttgcctcctgcctttgttgcctctgcttggctcagctcctccccatctggaggctctggtaatgggccctcaggccctgctggaggttcaaggccctgttcctcctctacttcttcttcttccacctcttcctcctcttcccctctctctgcctcttcctcctcctcttcaagggtctggtcatcatagcacttcttgaggtggcgcaccaactcaaaaacacaggagaaagtggcgtggcaacgcctgcagccggaggctcccccagtgcctcctccggttggcatggacccaccctcacaggcatttttgcgtgctttctggcgggcattctggaaccacaccaccaccacacggctagccagacccaacagacttgcgagtcgctccacctctccgtctttggggtaggcgctagtctcaaagaaagactgcagggcttgggtctggaactctgtgaacttggttctggagaaccggcggccggcaggcaccaggggaggaagattccctctggagctttcttcctcttctatgggccagtgtccccctgctcgacttcgctcttcaggggcacgggtcccccctgcctcaggctctgggaccaggaagggtgggcccagatggggaacaggtgaatccagagacccatcaggaggtttgggaggctctgcaaggggcgggtataggctgtcatagctctttcgaaactgagcagcataacggctcagggcttcaaagggcagaaagcggcggtggacatgttcctcgtgtgtcttgaggataagcatattggagaagagtttcccacaggccccacaggccagcttgtccccacccccgagggcctcaggtgggggtggggtagggggagggggcacagcttgcttcccttcattgtactggatcaccagctcaaagccaaagttttctagaagggctttggctgcagtgcgggcagcctcgttgggcaatgggtcggggggtgaggaaggccctgcctcattaccctctttggccatggggggccgctcccactcccgctcagccagctcagccttgggaggttggggtggaggaggaggggtggcagctggcagggacagcacaggtgcaggcccagctagtgtcagcttgggccccaccttgagatcgtggaggtagaagggcaggagcagctgctgctgctggagcttaagcagtgattcgggcaccagagggaaggggggcaggactggtggggtgaagagaggggctgggaatcggtgcaggtccaagggaggtgggggaggggacaggaaaggcaatccagatatgaagccactggtgtcagggcccttcttctcagtgcccacctccccctctgtctcgccttccttgggctcttcttggctgcgttctggcccttcaatcttggaatcagtcttggttccccgagagcgagtctgatgcagaactgaccgcatgtggatctccagggtggagctctggttgtaggagactctgcagactgtgcacttaaagggcttgtctgtggcagcagtggtggtgggtggggcaccggcctctccccgtgcaggggcagaggggtcaatggcagccttcttcatcttgtgaaggtgggagacagaattataatgaaccaacagaatattcttctgggtgaaggactccttacacacagtgcacttatagggccgggcagggtcgagaaacttgtccagggcaaagttggtggttttccgataggtcagagggtggcgagagtcagctggagctggctctgcagagcggagctccccagtggtcccctcttcctcctcagccatggtgggcggaggagctacgtcttcagcttgggcatcaggttcagggactggagatggggctggagaagggggttggccagggcttcctgagggtttgtctgggacctcaactgaggccaggggaggctcaggaagaggatctggactggcttctggggtcaggttagggccttctgctgcctggtctctgctcggtgtaggctctggcccatgagtggggggttcttggccattgtccagagggcttaatgtgggtgcagacagcactttggttgtaaatgtcatttctacagttgtagctacaagcagcagcttctcaacgcactcgggcaccacgttgtgaaggtggctaaggtggaagtgcagggcaggccggcccaccagctgttcctggcacagtgggcatctgtacttgggctgcactgcatgctgggagagtgtatgagccctcacctggctggactctgggctcaggaagctgcagtatggacagcagtatacctgtctgctcagaagccagctcatcctccctcaggctcagcagctcccaccttattttccatctttctttttccttcttctttttccgtggtctggttggcactgtctctggaagggccagtcttgttttctgtctcttctgaagctgaggatgaaagaagaggagattaaggaaccctgacagccctcaagatgatttgtagcagagagcttccagggtagggagttgggcactagagaaagggcaggaaactcagtagataggtgaggcttggcaagggctgactccgggtcagtaggatggtcaggtctgagttctcaaagagggcggaagtgcctagcctctcgtggctcagcctcccttccccctgatgagccctttctttaatcagttttgctccttgagcacagacattgctgggctcctggattactgcaaggtcccgtgagcgt

SEQ ID NO: 17710 - RNA, 1062 nt, Homo sapiens
  source 1..1062: mol_type = other RNA
tccattacactaccctgcctcttgtctggagcatgttggttcataattcagtaggtaatgaggtttgggattgcagaaggcctgtgattgatggcacaaaaacctgacgtagtccaattcaattctgtttggaaaagtagtcccaggtcatcaaactgccctcgcattgcagaaagcaccataaaatggaagagaccacaggacatgaaagaactacttttctttctgtagccaacacacattaaaggtcactattctgcgttaacttgaaaagagcaaaagcactgtttaacacaggctgtccagactcaattttagaggcaggaaacagaaattagtcaagtcctctaatttatagatggaaaaactattgtccaaaagtttctttcaatgaatctgttttgaacatttattgtgagatattaccaagatgcatgattgtatgtctcttcaagccagcagaatatttatcacacactatatttcctcaagaaattcttaataagtaaacaaatgaatgaattcacagacttgccccatgttagaaattagtaactagaagaactagagctagaacacccatctcctgacttcctgtttactacttctgggtgagaccaaaaatgcttgaaaatagctaggaaaactcaagcagttttcttagattagcttctgaatcactgatttaagcccatgcagaaaacacaaatgaagcactctgccaccagcccatgactgaaggttgtgtcatagtgtctctgaatcagtcccttcctgggaatgatgatgtccatactaatgccttctataaaagggcttttgcctcctttcacctcttaaacagctctcatttcacttcagagggcctctttgtttcaaagtcaaagtatacagaaccagaattttatcagtcagccagtattaaaaggtgtacaatggattaatgaggcaagaattctctcatttactcttaagggacaagaaagagaggcaaatgtcattgcttacaggtattcgggcccacaatgctcagagagtactaagtgtctaaaatccatttct

SEQ ID NO: 17711 - RNA, 2404 nt, Homo sapiens
  source 1..2404: mol_type = other RNA
tcccacgttgtggcccagcaggacggtgatctgtccctcgtacaggttgaggttcaggtctctgacggccgccctgtccttatttcccaccctgaacaccttggacaggtgcttgatcttgatccccgccaccaggtcctctggctcggcttcaaagtactcgtttctgagtgctttctcggggtcactgtcttcttcctccttccctgcaaccgcccttggcttcccacaccaataggagggcatgatgaagaagtaccagggctgaggcacgccgaactgccctgggaagacggcctccatgtaccaggtcaccaggccatagagcacagagtccagcagcagcatccccagcacctgcccgaagcagaagtcgtcgtccacgttgacgggactcaggaggtctcgccactggatgcccatgcctttcgcctcaaatttcccaatgagctgggctcccattgccatggcgacattagacaggaggcaggagcagagcttctggctcagagtcatccagttgtaccgaggggccacgaagaagtaggggatgtaggtgaagaagtagaggaagcctccgaaggctgctgccatgttggctttgctgaagaaggtgctgaccatgaagctgaaggagatggtagagatggcgaagcacagcaggaaggcgagcaccagggaggggtcgctgcgggacagcacggctacatttggcttcaccttgacacagaagagcagggtcatgaaggaggcggcgatgaggaggaagaggaagaacaagaggaaccaggcactccagtgcagccagctgctgagccccatcatgcgcatgtactccttcagcctcctttccttctcctgcacgacagcacgggcaatggtgagcgcggtgtaggtgaagctgagcagcagcagcaggggcagctggtactggatggccacgaggaaggggtctgcgatgaacggcgggtacgggaacctcttgatggtcaccgtcagtctctggaacagctggcgtgtggcggcatcggcatggtactccatgatggcccggtccacagcatgctgcacggccaggaagccttcccggatgtacccaggttctccgccatcaggggatgtaggttcccttggtcctgggtttgggaaaagcgggaaaagggaagtagtgtgccagccttctgtctctttcaggaaaaaggagcctgtttgggtccacatgtaatttctccgtgtgtaactgaaccgtaggtgatatttcaccgccagcggcaggggctccttgctgtggttgaaggggtgctcgaagaccacggcggccagcacgctggacgagcagttgtcgtacctaatgtagtcctcaaagtccttctcggagggaaagccgcgcactcgcatgttgatcacaagtgccctgcgcactgtctcagtgacggtcttggcagcgtcactgtgagaagggatgtaggcaagctcccaggtgtctcctggcggagggaaggtgaagaacagaggcagctcctggatggactggcccgggtagatggtggcgttgggcacattttccgactgaatcttcaagcggagccagatgaggatcccagaaaacagcaatggcaggaagagttccaggaccgtcaccaggaccttccgcttctgcagggtgtagttcttccagaggaggagcgccagctgcctgagcacagccatcgtcttgctgaaagggacgcccagtgctgctagagaagtaggtggtctgagtaagttcaagtaggcgctgcaacccgcaggaaataggagaaacgtgctctgaaaactgagtgtaaagagggcgaggtgtgcagacgtggctgctctgtcctggagaggcagggaaggcgatggaggaggggcagtctagagagcccctggtgctggtccactcgctacaactgcaggcagagaggagtccttcccgctcagcgtccttcatgtgcggaaaagcctccttgactcacagtggaagagtttcaggttcagttgctcagctccacactcatggctgggtcccagaagaggctccacacagcaggtctcccttcaggactactggggaactggccaggaggaggcggctccgcacagagggctccggggtggggcctgagagcctctggagtggggcagggcaaccctgaggtttgggaacaccgtgacctcgcaggacatcaggaggtgcccagggctcacaggcatgactctccagcaccgagcctgggcgccggggcggcggcggccggcgcgcggccctctcgcggggtcccctccctcggccacccgggctccgctccagcctcgcagtggcggcggcactgacagctgcgtggccgccctggaggggagggtgcgcctgcaacccgctact

SEQ ID NO: 17712 - RNA, 1532 nt, Homo sapiens
  source 1..1532: mol_type = other RNA
tcccctgctcccttgttccccaggatgtgccagagcccggggcctgtccgtcctgttcctgcccctccaccttcctccctgggcatgcaggagtctgagcaggagttacgcggccgttctggttgggccggtacacgctgcccacgctgaggcggccctgctgcgcgccgttccgctccccacccggcgggggcgtgtcggagctgcgcaccggcaggtagggcggctccagcgcgcgcggcggcccgtacgcctcgggcggcgggttggcgtagggcgggtaccagcccaggcgtgggtctccgccatgggcctgcgccgcctcgggaccggggtcagggtaggcctgctcgaagccgggggtgccctcgctgtacagactgtgcgagtagcggcggtccaggccgtcggggggcggcggcggcggcggcacgtagggcctctcgggggccgggtagaagccctgaggcgggtactcgggcagctcttcgccgccgccgtactcctcgtagcgcgcccggggctggtaggggtagatgacccccgccgaggccacggccgccgcccccgcgcccacgccgccgcccgcgggccggtagtacacgaaaccctggtcgtaggtccgcgacgcggggtcgtagttctcgtactggctgacgaagggcgcctgcgggtaggggaactgctgcgggtaggagggctgctggcggtaggtgctggcgaaggccgaagccgagaccgaggaggcggagcccccgtgccgttgctgggagacggaggtgcgggcccgggccatgcccgtgctgtccccgacggccacctcgcgccagttgtcgggcacctggccaaagccgaatgggtgccgcgcctggccgcgcacggtgtccgagcccacgcgccccggcaggggcagggacggcgcctgccgacgccgggggctcccgtggctgcgccgctgctgggcctggggcgcgccggccagcagcacccgggagctactctcggagcgctgaggtccggccggcacgtactctgagcccgagttgagcaagctgtacacctgcccgttgttctcccactggatcagctgccgccagcgggcggggtccgagccctgcccgggctgcgcctgctgcccgtgcaccagcacgcacaggcaggcgccccacaccagggcccccagctgccggctgcctcgggccagagccatggtgacccctctgcagaggcctggtggacagagaggctctcaggagtggccccctgggcgtgcttctcttcccacggcctcgaggacaggaaggctccttgcttgccccagctctagctttgtccatgctggccttgtcccgagcgggacggctcctccgatgacagcatttcaaggccaaggggtcagggcagggcaggggcggtgcccagggctgcacgaggctctccgcagggcaccgggcgggcaggaccgcctgtgggccttacatggccagccccgcactggctggccgctcggctggcgctttcccactctgaat

SEQ ID NO: 17713 - RNA, 1662 nt, Homo sapiens
  source 1..1662: mol_type = other RNA
tcccctgctcccttgttccccagtgtgtttgcaatgcctgtcttcacgttgtcagtacagatgtggctgatccggttctcgtgctcaggcttggccagcaccacgatgcggatgttccagagcgtgtggatggcgactgttttaaaagtcacactggtgatttcttgcagggagtgtttgaggatctccagccactccttctcactcagggggtcctcttgggtgccgatcacgtaaatgtcatgggggatgtagtccgcagagtcgtcccgcgtctttccctgcccccatgttccaggtgccgatgaagatggtgatcatgtcgggctccggctgctctgagtgcttgttcttcatctgctgcaggagctggcagaagccttctctctttttggagtcagcaaaaacatattccttccgcaggatcttctccttctctgtttccaccaagatcaccaacttattcagaaatttctgtgacttaatgagctgcaggattttcttgtggctgtagaacttgtcctcagaaccatccttggacttcttaatgatcagtttcccagactcaacgtcgactttgagctgcattttctgaggaatccccagagactctgccttcacctcaaaggtgactggagggataagggagggccggtgcggagactcaggaccctcgtgcagcaaggccttgaccttgtcttcaatggacgacaacaggcttgtcagttggctgagcttggacaccatgttgatgggattggcctcaccaggaacctgaggacgtggacggaggcccggggagagctgctggtcaaataacctctgcagagactccagggatgggagggtccggatgacttctccatagagctccttgcagagcagtgtggtcagtttcttcaggtgaggaagactgctggaccctgtcttcacaaattcagagtcctgggcgagctgagtgcttaaataatcttggatggccttaagatgctcttctggaagcccactggtgtccatgctttgcagtcgctggaacaatgtctcggagaggctcggccggctggtctcggtcgctcggggattctcgtttgaaaaaggaacctccttggcctcacaggagctggcagtcagcgggatgtttcttgggggcagctcgggtggagacacgacactttctactgtgtcctcctcagggtcgtcgcctgtgtcctcttcctccagcggcacagggtattgcagatgggtcaccagccccatgttttccttcttgtaaaactcgatgagctggtccagcttggtgaagaacctcatggagacgccttcggatgcctgaacagtgaatttatcatcttcattgggcagaattctgtaagtgtaaacgcaattccgatacagcacgcagagcgcgtatgcccgggagatggactcgctggcacgcacgaggaagctcccgtccttgcctgtcctggaaagcagctcctccgccttggagcgggtgatgttgccatggttccagcaggggaccatggtgggcgtgggcctcctcggccgggccggcaggcacccccaggacccacacaccaccgaggggagcggaggcccctccactgcaacctgccgcccgttgcctcttggtggcctcggctgctgccaccagcttaa

SEQ ID NO: 17714 - RNA, 1711 nt, Homo sapiens
  source 1..1711: mol_type = other RNA
tcccctgctcccttgttccccagtgtgtttgcaatgcctgtcttcacgttgtcagtacagatgtggctgatccggttctcgtgctcaggcttggccagcaccacgatgcggatgttccagagcgtgtggatggcgactgttttaaaagtcacactggtgatttcttgcagggagtgtttgaggatctccagccactccttctcactcagggggtcctcttgggtgccgatcacgtaaatgtcatgggggatgtagtccgcagagtcgtcccgcgtctttccctgccccttggagagaaaccaggacgtgatcttcttgggagggggggcgttacccatgttccaggtgccgatgaagatggtgatcatgtcgggctccggctgctctgagtgcttgttcttcatctgctgcaggagctggcagaagccttctctctttttggagtcagcaaaaacatattccttccgcaggatcttctccttctctgtttccaccaagatcaccaacttattcagaaatttctgtgacttaatgagctgcaggattttcttgtggctgtagaacttgtcctcagaaccatccttggacttcttaatgatcagtttcccagactcaacgtcgactttgagctgcattttctgaggaatccccagagactctgccttcacctcaaaggtgactggagggataagggagggccggtgcggagactcaggaccctcgtgcagcaaggccttgaccttgtcttcaatggacgacaacaggcttgtcagttggctgagcttggacaccatgttgatgggattggcctcaccaggaacctgaggacgtggacggaggcccggggagagctgctggtcaaataacctctgcagagactccagggatgggagggtccggatgacttctccatagagctccttgcagagcagtgtggtcagtttcttcaggtgaggaagactgctggaccctgtcttcacaaattcagagtcctgggcgagctgagtgcttaaataatcttggatggccttaagatgctcttctggaagcccactggtgtccatgctttgcagtcgctggaacaatgtctcggagaggctcggccggctggtctcggtcgctcggggattctcgtttgaaaaaggaacctccttggcctcacaggagctggcagtcagcgggatgtttcttgggggcagctcgggtggagacacgacactttctactgtgtcctcctcagggtcgtcgcctgtgtcctcttcctccagcggcacagggtattgcagatgggtcaccagccccatgttttccttcttgtaaaactcgatgagctggtccagcttggtgaagaacctcatggagacgccttcggatgcctgaacagtgaatttatcatcttcattgggcagaattctgtaagtgtaaacgcaattccgatacagcacgcagagcgcgtatgcccgggagatggactcgctggcacgcacgaggaagctcccgtccttgcctgtcctggaaagcagctcctccgccttggagcgggtgatgttgccatggttccagcaggggaccatggtgggcgtgggcctcctcggccgggccggcaggcacccccaggacccacacaccaccgaggggagcggaggcccctccactgcaacctgccgcccgttgcctcttggtggcctcggctgctgccaccagcttaact

SEQ ID NO: 17715 - RNA, 1708 nt, Homo sapiens
  source 1..1708: mol_type = other RNA
tcccctgctcccttgttccccagtgtgtttgcaatgcctgtcttcacgttgtcagtacagatgtggctgatccggttctcgtgctcaggcttggccagcaccacgatgcggatgttccagagcgtgtggatggcgactgttttaaaagtcacactggtgatttcttgcagggagtgtttgaggatctccagccactccttctcactcagggggtcctcttgggtgccgatcacgtaaatgtcatgggggatgtagtccgcagagtcgtcccgcgtctttccctgccccttggagagaaaccaggacgtgatcttcttgggagggggggcgttacccatgttccaggtgccgatgaagatggtgatcatgtcgggctccggctgctctgagtgcttgttcttcatctgctgcaggagctggcagaagccttctctctttttggagtcagcaaaaacatattccttccgcaggatcttctccttctctgtttccaccaagatcaccaacttattcagaaatttctgtgacttaatgagctgcaggattttcttgtggctgtagaacttgtcctcagaaccatccttggacttcttaatgatcagtttcccagactcaacgtcgactttgagctgcattttctgaggaatccccagagactctgccttcacctcaaaggtgactggagggataagggagggccggtgcggagactcaggaccctcgtgcagcaaggccttgaccttgtcttcaatggacgacaacaggcttgtcagttggctgagcttggacaccatgttgatgggattggcctcaccaggaacctgaggacgtggacggaggcccggggagagctgctggtcaaataacctctgcagagactccagggatgggagggtccggatgacttctccatagagctccttgcagagcagtgtggtcagtttcttcaggtgaggaagactgctggaccctgtcttcacaaattcagagtcctgggcgagctgagtgcttaaataatcttggatggccttaagatgctcttctggaagcccactggtgtccatgctttgcagtcgctggaacaatgtctcggagaggctcggccggctggtctcggtcgctcggggattctcgtttgaaaaaggaacctccttggcctcacaggagctggcagtcagcgggatgtttcttgggggcagctcgggtggagacacgacactttctgtgtcctcctcagggtcgtcgcctgtgtcctcttcctccagcggcacagggtattgcagatgggtcaccagccccatgttttccttcttgtaaaactcgatgagctggtccagcttggtgaagaacctcatggagacgccttcggatgcctgaacagtgaatttatcatcttcattgggcagaattctgtaagtgtaaacgcaattccgatacagcacgcagagcgcgtatgcccgggagatggactcgctggcacgcacgaggaagctcccgtccttgcctgtcctggaaagcagctcctccgccttggagcgggtgatgttgccatggttccagcaggggaccatggtgggcgtgggcctcctcggccgggccggcaggcacccccaggacccacacaccaccgaggggagcggaggcccctccactgcaacctgccgcccgttgcctcttggtggcctcggctgctgccaccagcttaact

SEQ ID NO: 17716 - RNA, 9816 nt, Homo sapiens
  source 1..9816: mol_type = other RNA
tccccttcctccctgcccagactcccgtgtggtggcattgaagagtgtccttcatggggggacagctgggccacataccccggcggcagcatggaggccccagggacagtggcagcagacggcttagcctcaactaatagcaaacaggactttcaacctctttctcactggcaagttttcagggtttaagacgtattgtctttagaagcgagggactctgtgtgtgctccaagaatgggttactagtccagcaggaaagaacaatgagtacaggcaggactccttccttttttagtttggaaattaactcatctttagtcattttacagtctaaaatcctttttggaataagaaacctaaaaaacctaaaaacactcaatataatcagcagtggccaatgatatagacggctgtgtttgcattgaacaaatctgcagatttgtcagccttgccttctatccaaagaaggtggctggtttacaaggacatgagatacacacccaagtgggcacaactgcatttttggtcaatacaaacagaactctgagattttatcagaaagtctgagcagcaagcgtgagacttgtaggtgcgtataagactttttgaacctccaccctggatggtagatgcggctggactgaagtcactaccgccttataagaacataatagacttcaagttgaaggctaatttatgacaaaccaggccagattcctgcctgtctaattccccacgctgcgatgcctggctgtttaccccagcttctcatgagaggagccccttctccagctcaggggttcccacctttgtcaagacaggacacatctctgcatttgcatcttaatgctcccccatgttaagaatggcaactggcgaataaacaacgggcagagtgttctgattccaaatccggaagagatgaaagagacagcttcctcgtgatgtagaggggaattcaaggacaacaagatcaaagtttgcagctcgcaggtgggaactgaaagcccatgataaagcaaactctcgctcctcagcaccaccgtgcaatgcgacgtggagtgactcccagggacacaatagcaccaccgcccgttcttagatcttagttttgctccgctgctaatgcttccacctcacatatttggagcagggggtgaggaggacaggttcacacaaggagttagacctatgcatctaaatgttaatttcaaatatttttttctagtcctttcgcttgtgggtaatgaaatagaaatgggttcgttgatattcccccttgcctccttgggttctctatcaccaaaaccaaggggagacctggaactatcatgtctggccactgggtaaggcatcctcccgtgactgggactgcttcagaatggtcagccggaactccttccttcatcatcaatacagtcaatttataggcagagacaggaacaagcacatcataacgtaaaatgcctgatttcttcatgtggtttatcaatattggtaaattaacatgtttgcagcttatttaggtcaaaaaaaagcaaagagaagagagagagaatggacaacatcaacataaagcattctccttcaccgtggcctgcgagatcctgcgaggtgttctgtgattgccatcttgggaaggagtctgacttgctaagagaactcttggtttccttccgccttttgttacagcataaagttgctacaaatggataaaagcagatttaggcaggaggcaagccgaatgccactcccctcggaaggattccatcggtttcagtccaggaagggcaccaggctctgtcactggctaaaggaaggcagtgcagcatggaaggaacctcaggggaggatgtggcaggggcgaaagccaaactcatcgatgactcatcagatgagtttctttccaacaaaaacagaatattcacctttgaaaatctccaattaaagacttttcatgaactatatgtttgaaaccagcaaccagcagcccaatggcaaactcgaaggattggcttccctttgggtccagaagcctccaaggatattactgttaagcaagcccacttacacaagtgctttgaggccagaggcgagcccagagcatgcgactgtcctgcagaatggggtcaaggttaaggagctcagggaggtcctgcttcccagggcaacacacttgtcagacttgggagatacacagaaggaagaacgagccatgccagagcagcctctcactgtagtttagcctgttcagccagcagatttgggcatgtctcctgtttgcacctttgcatagaagcagactcttatggaaagtgcaaagccagactcgtgacccagggagctggcttccaaagcacatgagccaacagggccacctgaaccctgttctgataacaaaggatcaggtcatgtgaagctcacaagacttcggttcccatttaccgagttcagccagctgtgtgggctgcagtgtccagaggtacactgaccaagaaacgtagtgtttttttccccgcttggggagtggctggggctgagttgttggttaataaagacagcctagcttggaaataaataggctcatgaagatatgctgcatttgagggcaaaagggaagcgtgctctgcacacgcctaagtaccatcctcgatgcgaaggctgcagggactcttagattctgggctgcactatcatcagcaccacagcttttatcagggaaatcccttgaccactctgtaccccaggtttctatcaatcactaaaatgggtatcataattcctaagggaattgttatagggaggaacatctgaatttgaggtcctgagttgttgggagccaagacctggacatccatagtcttcagctatgttctgcctatccagggtcgtgtgagttatggaggggaagctctctctgcctttgggcaggagcaaagactgagaggacaagcctgtcccttcttggcatagaggctttgggacacaggagagctgaaatccttgtactctggacaacagacaagatgtacagtctcaagaatccttcttctaatccaatacagttgaagtctctgaacaagcctgagaaggtctctcagctggggaaaaacccactttaatcaatctacaacacaacactagaaaatactaaagaaagaaatatggctctggtgaattggttccagctttcgttcaagactttttggaataaaaatgaatatgaattttgagggccacgcaaactgtggatttgtgggtcaaggaaccacatgtgtggaggacttgaggggggcaaacggtctacagaacatacggcccacctcccaggagcagggagggcccaggtcgcaaaggactcctcctcccctgtgctgcaggtgccgtctcctcacctgttctctaaagcacctgccccacaatcaaccttctgggtctacctgaccacgctgcttgttgggatgtggcatcgaggtcacctgctgctccaaacctactttggaaacacacacactggctcgtgccgagggaagtctctctgtttgagtggcctcaccagaataaccataaaagacaggtaatatttattcataagcaatactgattaagaaatagctctacaaacacaacttacttagaaacagcaagtcagaaataggataaaacaccaagagaaaaagagctgtgaatacatttccaaaatgtttttcttgtttgttttgttgttttcatcttgactagcaccatctgtacacaagaaagtatgaacataaatgtttggataataataaagatttgcaaggcacttaatcagtcattctgggttgttttgtgttcgctttccacagcaatcctacatccacgcccctcctttctcacgaaagcaagagaagagtgaggtctcttttgctagcagttcttatgtacaaacaaggtctttaaggttcctcaaagtgctttttcagtctcacagggcttggacacccctcgggcttcccatccttttctccttccacggtgtttgacgtttgcacctttcctacagaaaacaaaagaaaactcgccttccgctcaacgcccgctccagacttgccaccaaccttcatcctcattcattgtctttgatgccccagcacagagggcctaggggcgtgcaacatctctgaagtcctggggagcgggggaccactaggacaagggtctggctcatctaccggcgcctggaggtgatgtcgaagcaggtgatcatcatgagatgggccttgcagaagttgacacggctctccaggcgctccgtcacacactccagtgcctccaggtactccagggaatccagctcccaaacctgctccaagtcaaattcactgagccacttgttgggatccagcatcagatactgtttggtcgcctccagctccttcatcagccactcgtacttcgcgcggacctcggcgatcctctgctggcggtgttccagaatcttcagctttgcattgaagcacatggcctccttgctggcaccccctcgtcgccgctgcaggcgctccacgtcatcgatttcatagactttaatctcaaagggttccccaaggcccctcgggctgctccgcaaggggccatccacccagcggacgcctgtgctgttggggggttttctcacaggggaagaggtgtccagggatagtgctgggataagcctccgtctctgagaacctggattggagcgtttcttcggggtcttgaggctccggcacctgccgcccacggagctgctgttctcgctcgtggagtcctgcgccgaggacgcgctgccggtggcctcgctgtcccgcatcacgctctcgtagccgctgctgccgccgctgtggtagaacagggccgtcttccccatggccggcgggagctccccgctcagcacgctgctgttgtcgctgccgtggccgctgctgcagcggtggggcctccgcgggggcgtgatcttgctgtagggcgacgggagcaggtgcgcggccgcgggctcgtcctcggccagggcccccccgcgcgcctccgcctcgggcccggcccgcagctgcaagccccgggcgcccgcgccaccctgcagcagctccgagatgcgcccgctgacggcccgcaggggaagcttggaggccaggcccgagctcctgttcctgctgagggactgcgtggaccagggcgtgtgcttcccaccggggggcgagctggagccctggcccaccgcctgcggcagggacttggtggagaagctgagggttttggtggtggaggcggacgggccgcgcgctctggggctggccaggaggagtctgctcacggcggagatcttggactggccggccttgggcgaggccccggagctggggggcgaggtcccggcgctgcggcccaggctcctccccgcgcggggcatggtgccgtccttgcccgcgtgcagccgggagctcacggaggacaggctctcggcccgctccagggagaggcattcgtagtggctgactgtcgccctgcccagcgagttgcttctgctggccagctgctccagcttggcactgaagagcttgctgctgctgctggcgtccttcgtcttgccgctaggctcgtctgggaggcccgccgggaaggcggctggttggttcagggggctgctggtgccgctgccgctggcactgtgctgagggctggcccggttcttctggtccaggctggactttcggacagggggcagagggggagtccctttgggccgagccagaacacagtgcttgggggaagccaccttcccctccagggtagccttggagggcggggtgcccgaggctgcacccaccccgttggtctcagcagcgcagtaataggagaggctgtccggctcctcctgccggctggccttctgaaaggccctgggaaggctgctggacttgacgcttttgttgggatgcacggggctctgggtggccaaaccgggcagggccatctcacacccatccacgaccctcctgaagttgtcagtgaccggggaggccgacacctctccgctgctgctgctgagcctgtctcccggactgggctttccgtcctgctcctgctctgctctggtctcagcattcgaggggcccgtggcagtctcacacctcatcatcccttcttcattgggatgagccgtctcttttttcacttcctcttctcgtttcagccacgggtcctcaaatttcatctctttctttgcactgttttccttactctcccgggactgggctaatgtggggcctgctttgggggtggcggtgggggcctccggctcttggatgttccgggggctcatggcaatgcaggggtaaactgtgatattggtcttcatggggatgtacccctcgcagctgctcagattggccgtgttggagatggtgaccatggccttgctcactgtggatattttgcagcctttgatgggggctgctttgttgaaagagtcatctcccatctcagacaggatgagcaagttgtcggggctggccttgggcttctctctgcacaccacagcggtgttctggaggctgctgacaaactccgaggccacaggttctgccattgcctccccgtgcccaaaacacgtctgggctatgaaactgtggcacgactgctcaccctcactgcccgcgctcatctcgctcagccaggagctgatggaagagcgtctgctccctgcgtcctgggccttctcatccaggctcatcttcgggaggggcaagaactgtgtgatgctgacctcggagacgggggccgtgctggagtagcactccaggtcctcgctgatgctgctgatgatgctgacgggccgcgagcccgaggccagggcccgtgcagagcagtcgctgttgaagctgatgatgctggtggggcggccgctgtccaggaccccgctgatggtcagctcctccaccagcgtgaacaccagctcgtcctcaccgttcagctccagtggctgctgcaccgtcaccatcgtggtgctcaggatctccttcttggactctgaaggagtagctgcctgctgctcatcatcgacaggagtttccgggaacccttcgctcccagcagacatggattttttcaaaacctgggggctcattccaaccgggggcgtacgcacctcgggctgcagcaaggactccctagacgccacgccggaatccttgctcgagggaggcagtggggcgggagacggcaggacccccttctgggtgtagactttgcatctctgggaaggagagctgggtggcttgtactccgaggtcttggacaggctggcgatgcccagccggggggagcccatgggcctgggcttgccttccacgaagccgcaggagttgaggctctcccggctgctctggaggctggggctctgcacgagtggggaggcgctgtgctggctactgctgcccgggacgctcctgggtgaggccgggctggggctgtgggcgggtgccgcggcgggcacaggtgagtgactcctctgcatcttggaggctgggagttcagggccttctctgttggtcagctgaccttcggacccattatcttccttatcagactcagagagtgggcttgcccccgctgcttggcttaaccgggggcctctgcttgcctgctctggcccaaactgagcaggcagttcttcgaaaggaaagctgctgggctcctcgctgccgtcgatgcagtccagcctctcctgcagctcggcaaacgtgttgcacttcaggcagtccctttctgacttgccggctgcagcctctcctgcctctgcgggccggctgtcgccccgggtcttctgcagggctggcacgatagggacaaagtctggggggccctcgttgtcggtgagctccttgtcagagagggccgtgccgttgggcccgatgtagatgacggtgtcgcaggactgctcgctgctggaggagtagtcggggtcgctggacaggtgagcgatggggaagtcagggtccaccgtggccctggtgtggaagggtctcagctgggtgggcctgcgcatgcggccttcttcgcaggagctctccccgccggacgagctggatgtgtacttcgtcttctttttcttcatcctcaagactctcgatgcaatctggatggtggacagggtctccgcgtagctcccgaccgcggccgagatgtgcgcgatcatggtggtacggcagttcatgttccccagagactcccgcagcaacatggcgagcttgctctctttgtatggaatgtgtttgctgccattgacgagagccaggatgacattgcccagagcagacagcgagagacacagccctgagcctccttctcgatttttgctaagagctttcacacagctgccgagatcaatgagatgcaggcggctgcgacctccagacattccccctttcccgctcttctccatccggtactggtagatgtgcagtgtgaagaacacgtgtgagttgcggtggtcgtcctcatcacagtcctgttggtggctcctgcgggaggcaatggcggcatccaggaaaaaggcagccttctctgcggtgggggcccgcagctcgctctggttctgcagctgcgtgccgcagatggggtcctcacagaggtacacgcccggggactggccgtcctgcaggctgcccgtggccacctccgacagcaggtcccgcaggttctcctccttcccccacacttccacggcggaaacccggactgagaaacgggcgccggtcttttccttgcgttcgtttatgagcttgaagagccaagagatggcacagggaatgatgcccaggttctgcatggaatcatcctttccgatcatggtgtaggattttcccagtttggcgtggccgaaacagaacacgcagccatctgccccgttgaccacagactggatcacctctgccacggtgcctgcacacacttcagcctgagaagcgtcttgtggaaaaactgcatcgaaggcaaacatctttggaggaacctggttgcctctcttttggaaggcattttgacctccacaagtcaggggatcgtacaaggtgatctgcttcttccgtgggtccacctttaagaaagagctggattctgaagtatctcgagccaaggtggaacagatgcgaagcatgactttcaccttgcccagccccggggtgtccttcaccttgttgacagccctcagcaggcagggtggggctgggggaggggaggtctgcagaatcccactgaagctggttgcaaagagcggtggttcggcagcggaagaagtggaaggccgatgtttcttctttttagaagacagatttaacttctgggcagctactgctttccaatccatcatcattgataagtcatggctaaataatcaagtgcagaatccatttcttcacgtctgctaataaatagcttctctcaaatgtctcttgcagatctggggccatctcaggagaaagtaaaattgtgcgaaggtgaaggaggaaaggctggaaaattctaaaatccatgggggtctgagaactctcagagcagaccctggtgaaacattcttgtgattccagcctttggctaaaccatgatcctggcctcactgagctcccagccaccttcccagtgcagctcagcccctgctccaacattgcatttccctccaagaacagtgcatggatgggagaggagctcacacaatcctgccaatccgcacatgcaagcacgcttctcaaaggaagctgcaccagtttcactctggtgtctgctatctcagagaga

SEQ ID NO: 17717 - RNA, 11529 nt, Homo sapiens
  source 1..11529: mol_type = other RNA
tccccttcctccctgcccagactcccgtgtggtggcattgaagagtgtccttcatggggggacagctgggccacataccccggcggcagcatggaggccccagggacagtggcagcagacggcttagcctcaactaatagcaaacaggactttcaacctctttctcactggcaagttttcagggtttaagacgtattgtctttagaagcgagggactctgtgtgtgctccaagaatgggttactagtccagcaggaaagaacaatgagtacaggcaggactccttccttttttagtttggaaattaactcatctttagtcattttacagtctaaaatcctttttggaataagaaacctaaaaaacctaaaaacactcaatataatcagcagtggccaatgatatagacggctgtgtttgcattgaacaaatctgcagatttgtcagccttgccttctatccaaagaaggtggctggtttacaaggacatgagatacacacccaagtgggcacaactgcatttttggtcaatacaaacagaactctgagattttatcagaaagtctgagcagcaagcgtgagacttgtaggtgcgtataagactttttgaacctccaccctggatggtagatgcggctggactgaagtcactaccgccttataagaacataatagacttcaagttgaaggctaatttatgacaaaccaggccagattcctgcctgtctaattccccacgctgcgatgcctggctgtttaccccagcttctcatgagaggagccccttctccagctcaggggttcccacctttgtcaagacaggacacatctctgcatttgcatcttaatgctcccccatgttaagaatggcaactggcgaataaacaacgggcagagtgttctgattccaaatccggaagagatgaaagagacagcttcctcgtgatgtagaggggaattcaaggacaacaagatcaaagtttgcagctcgcaggtgggaactgaaagcccatgataaagcaaactctcgctcctcagcaccaccgtgcaatgcgacgtggagtgactcccagggacacaatagcaccaccgcccgttcttagatcttagttttgctccgctgctaatgcttccacctcacatatttggagcagggggtgaggaggacaggttcacacaaggagttagacctatgcatctaaatgttaatttcaaatatttttttctagtcctttcgcttgtgggtaatgaaatagaaatgggttcgttgatattcccccttgcctccttgggttctctatcaccaaaaccaaggggagacctggaactatcatgtctggccactgggtaaggcatcctcccgtgactgggactgcttcagaatggtcagccggaactccttccttcatcatcaatacagtcaatttataggcagagacaggaacaagcacatcataacgtaaaatgcctgatttcttcatgtggtttatcaatattggtaaattaacatgtttgcagcttatttaggtcaaaaaaaagcaaagagaagagagagagaatggacaacatcaacataaagcattctccttcaccgtggcctgcgagatcctgcgaggtgttctgtgattgccatcttgggaaggagtctgacttgctaagagaactcttggtttccttccgccttttgttacagcataaagttgctacaaatggataaaagcagatttaggcaggaggcaagccgaatgccactcccctcggaaggattccatcggtttcagtccaggaagggcaccaggctctgtcactggctaaaggaaggcagtgcagcatggaaggaacctcaggggaggatgtggcaggggcgaaagccaaactcatcgatgactcatcagatgagtttctttccaacaaaaacagaatattcacctttgaaaatctccaattaaagacttttcatgaactatatgtttgaaaccagcaaccagcagcccaatggcaaactcgaaggattggcttccctttgggtccagaagcctccaaggatattactgttaagcaagcccacttacacaagtgctttgaggccagaggcgagcccagagcatgcgactgtcctgcagaatggggtcaaggttaaggagctcagggaggtcctgcttcccagggcaacacacttgtcagacttgggagatacacagaaggaagaacgagccatgccagagcagcctctcactgtagtttagcctgttcagccagcagatttgggcatgtctcctgtttgcacctttgcatagaagcagactcttatggaaagtgcaaagccagactcgtgacccagggagctggcttccaaagcacatgagccaacagggccacctgaaccctgttctgataacaaaggatcaggtcatgtgaagctcacaagacttcggttcccatttaccgagttcagccagctgtgtgggctgcagtgtccagaggtacactgaccaagaaacgtagtgtttttttccccgcttggggagtggctggggctgagttgttggttaataaagacagcctagcttggaaataaataggctcatgaagatatgctgcatttgagggcaaaagggaagcgtgctctgcacacgcctaagtaccatcctcgatgcgaaggctgcagggactcttagattctgggctgcactatcatcagcaccacagcttttatcagggaaatcccttgaccactctgtaccccaggtttctatcaatcactaaaatgggtatcataattcctaagggaattgttatagggaggaacatctgaatttgaggtcctgagttgttgggagccaagacctggacatccatagtcttcagctatgttctgcctatccagggtcgtgtgagttatggaggggaagctctctctgcctttgggcaggagcaaagactgagaggacaagcctgtcccttcttggcatagaggctttgggacacaggagagctgaaatccttgtactctggacaacagacaagatgtacagtctcaagaatccttcttctaatccaatacagttgaagtctctgaacaagcctgagaaggtctctcagctggggaaaaacccactttaatcaatctacaacacaacactagaaaatactaaagaaagaaatatggctctggtgaattggttccagctttcgttcaagactttttggaataaaaatgaatatgaattttgagggccacgcaaactgtggatttgtgggtcaaggaaccacatgtgtggaggacttgaggggggcaaacggtctacagaacatacggcccacctcccaggagcagggagggcccaggtcgcaaaggactcctcctcccctgtgctgcaggtgccgtctcctcacctgttctctaaagcacctgccccacaatcaaccttctgggtctacctgaccacgctgcttgttgggatgtggcatcgaggtcacctgctgctccaaacctactttggaaacacacacactggctcgtgccgagggaagtctctctgtttgagtggcctcaccagaataaccataaaagacaggtaatatttattcataagcaatactgattaagaaatagctctacaaacacaacttacttagaaacagcaagtcagaaataggataaaacaccaagagaaaaagagctgtgaatacatttccaaaatgtttttcttgtttgttttgttgttttcatcttgactagcaccatctgtacacaagaaagtatgaacataaatgtttggataataataaagatttgcaaggcacttaatcagtcattctgggttgttttgtgttcgctttccacagcaatcctacatccacgcccctcctttctcacgaaagcaagagaagagtgaggtctcttttgctagcagttcttatgtacaaacaaggtctttaaggttcctcaaagtgctttttcagtctcacagggcttggacacccctcgggcttcccatccttttctccttccacggtgtttgacgtttgcacctttcctacagaaaacaaaagaaaactcgccttccgctcaacgcccgctccagacttgccaccaaccttcatcctcattcattgtctttgatgccccagcacagagggcctaggggcgtgcaacatctctgaagtcctggggagcgggggaccactaggacaagggtctggctcatctaccggcgcctggaggtgatgtcgaagcaggtgatcatcatgagatgggccttgcagaagttgacacggctctccaggcgctccgtcacacactccagtgcctccaggtactccagggaatccagctcccaaacctgctccaagtcaaattcactgagccacttgttgggatccagcatcagatactgtttggtcgcctccagctccttcatcagccactcgtacttcgcgcggacctcggcgatcctctgctggcggtgttccagaatcttcagctttgcattgaagcacatggcctccttgctggcaccccctcgtcgccgctgcaggcgctccacgtcatcgatttcatagactttaatctcaaagggttccccaaggcccctcgggctgctccgcaaggggccatccacccagcggacgcctgtgctgttggggggttttctcacaggggaagaggtgtccagggatagtgctgggataagcctccgtctctgagaacctggattggagcgtttcttcggggtcttgaggctccggcacctgccgcccacggagctgctgttctcgctcgtggagtcctgcgccgaggacgcgctgccggtggcctcgctgtcccgcatcacgctctcgtagccgctgctgccgccgctgtggtagaacagggccgtcttccccatggccggcgggagctccccgctcagcacgctgctgttgtcgctgccgtggccgctgctgcagcggtggggcctccgcgggggcgtgatcttgctgtagggcgacgggagcaggtgcgcggccgcgggctcgtcctcggccagggcccccccgcgcgcctccgcctcgggcccggcccgcagctgcaagccccgggcgcccgcgccaccctgcagcagctccgagatgcgcccgctgacggcccgcaggggaagcttggaggccaggcccgagctcctgttcctgctgagggactgcgtggaccagggcgtgtgcttcccaccggggggcgagctggagccctggcccaccgcctgcggcagggacttggtggagaagctgagggttttggtggtggaggcggacgggccgcgcgctctggggctggccaggaggagtctgctcacggcggagatcttggactggccggccttgggcgaggccccggagctggggggcgaggtcccggcgctgcggcccaggctcctccccgcgcggggcatggtgccgtccttgcccgcgtgcagccgggagctcacggaggacaggctctcggcccgctccagggagaggcattcgtagtggctgactgtcgccctgcccagcgagttgcttctgctggccagctgctccagcttggcactgaagagcttgctgctgctgctggcgtccttcgtcttgccgctaggctcgtctgggaggcccgccgggaaggcggctggttggttcagggggctgctggtgccgctgccgctggcactgtgctgagggctggcccggttcttctggtccaggctggactttcggacagggggcagagggggagtccctttgggccgagccagaacacagtgcttgggggaagccaccttcccctccagggtagccttggagggcggggtgcccgaggctgcacccaccccgttggtctcagcagcgcagtaataggagaggctgtccggctcctcctgccggctggccttctgaaaggccctgggaaggctgctggacttgacgcttttgttgggatgcacggggctctgggtggccaaaccgggcagggccatctcacacccatccacgaccctcctgaagttgtcagtgaccggggaggccgacacctctccgctgctgctgctgagcctgtctcccggactgggctttccgtcctgctcctgctctgctctggtctcagcattcgaggggcccgtggcagtctcacacctcatcatcccttcttcattgggatgagccgtctcttttttcacttcctcttctcgtttcagccacgggtcctcaaatttcatctctttctttgcactgttttccttactctcccgggactgggctaatgtggggcctgctttgggggtggcggtgggggcctccggctcttggatgttccgggggctcatggcaatgcaggggtaaactgtgatattggtcttcatggggatgtacccctcgcagctgctcagattggccgtgttggagatggtgaccatggccttgctcactgtggatattttgcagcctttgatgggggctgctttgttgaaagagtcatctcccatctcagacaggatgagcaagttgtcggggctggccttgggcttctctctgcacaccacagcggtgttctggaggctgctgacaaactccgaggccacaggttctgccattgcctccccgtgcccaaaacacgtctgggctatgaaactgtggcacgactgctcaccctcactgcccgcgctcatctcgctcagccaggagctgatggaagagcgtctgctccctgcgtcctgggccttctcatccaggctcatcttcgggaggggcaagaactgtgtgatgctgacctcggagacgggggccgtgctggagtagcactccaggtcctcgctgatgctgctgatgatgctgacgggccgcgagcccgaggccagggcccgtgcagagcagtcgctgttgaagctgatgatgctggtggggcggccgctgtccaggaccccgctgatggtcagctcctccaccagcgtgaacaccagctcgtcctcaccgttcagctccagtggctgctgcaccgtcaccatcgtggtgctcaggatctccttcttggactctgaaggagtagctgcctgctgctcatcatcgacaggagtttccgggaacccttcgctcccagcagacatggattttttcaaaacctgggggctcattccaaccgggggcgtacgcacctcgggctgcagcaaggactccctagacgccacgccggaatccttgctcgagggaggcagtggggcgggagacggcaggacccccttctgggtgtagactttgcatctctgggaaggagagctgggtggcttgtactccgaggtcttggacaggctggcgatgcccagccggggggagcccatgggcctgggcttgccttccacgaagccgcaggagttgaggctctcccggctgctctggaggctggggctctgcacgagtggggaggcgctgtgctggctactgctgcccgggacgctcctgggtgaggccgggctggggctgtgggcgggtgccgcggcgggcacaggtgagtgactcctctgcatcttggaggctgggagttcagggccttctctgttggtcagctgaccttcggacccattatcttccttatcagactcagagagtgggcttgcccccgctgcttggcttaaccgggggcctctgcttgcctgctctggcccaaactgagcaggcagttcttcgaaaggaaagctgctgggctcctcgctgccgtcgatgcagtccagcctctcctgcagctcggcaaacgtgttgcacttcaggcagtccctttctgacttgccggctgcagcctctcctgcctctgcgggccggctgtcgccccgggtcttctgcagggctggcacgatagggacaaagtctggggggccctcgttgtcggtgagctccttgtcagagagggccgtgccgttgggcccgatgtagatgacggtgtcgcaggactgctcgctgctggaggagtagtcggggtcgctggacaggtgagcgatggggaagtcagggtccaccgtggccctggtgtggaagggtctcagctgggtgggcctgcgcatgcggccttcttcgcaggagctctccccgccggacgagctggatgtgtacttcgtcttctttttcttcatcctcaagactctcgatgcaatctggatggtggacagggtctccgcgtagctcccgaccgcggccgagatgtgcgcgatcatggtggtacggcagttcatgttccccagagactcccgcagcaacatggcgagcttgctctctttgtatggaatgtgtttgctgccattgacgagagccaggatgacattgcccagagcagacagcgagagacacagccctgagcctccttctcgatttttgctaagagctttcacacagctgccgagatcaatgagatgcaggcggctgcgacctccagacattccccctttcccgctcttctccatccggtactggtagatgtgcagtgtgaagaacacgtgtgagttgcggtggtcgtcctcatcacagtcctgttggtggctcctgcgggaggcaatggcggcatccaggaaaaaggcagccttctctgcggtgggggcccgcagctcgctctggttctgcagctgcgtgccgcagatggggtcctcacagaggtacacgcccggggactggccgtcctgcaggctgcccgtggccacctccgacagcaggtcccgcaggttctcctccttcccccacacttccacggcggaaacccggactgagaaacgggcgccggtcttttccttgcgttcgtttatgagcttgaagagccaagagatggcacagggaatgatgcccaggttctgcatggaatcatcctttccgatcatggtgtaggattttcccagtttggcgtggccgaaacagaacacgcagccatctgccccgttgaccacagactggatcacctctgccacggtgcctgcacacacttcagcctgagaagcgtcttgtggaaaaactgcatcgaaggcaaacatctttggaggaacctggttgcctctcttttggaaggcattttgacctccacaagtcaggggatcgtacaaggtgatctgcttcttccgtgggtccacctttaagaaagagctggattctgaagtatctcgagccaaggtggaacagatgcgaagcatgactttcaccttgcccagccccggggtgtccttcaccttgttgacagccctcagcaggcagggtggggctgggggaggggaggtctgcagaatcccactgaagctggttgcaaagagcggtggttcggcagcggaagaagtggaaggccgatgtttcttctttttagaagacagatttaacttctgggcagctcgtgcaaagaaggaggcggccaccgatgtgcctgtggaagtctcgctggccacgcaggagccctgcgaggctgggacactgcaggcggaaggcttgtctgcattgtagcggttcagcactgcttctgttagtccctcccggctactctctgtcatcagctgggagatctggtatgggtacagggtgaccccgttggttctcgacagggaccaggtgccatccaggtactggtgagcctggatggccaccgaattgaggatgttcccattgcttggactggtggccatctggaggctgaccttggcctggtgggttggggacccgctcttcttttccgccccattgctgaccccaaggctgctgggtttgctgccgtgcttgttggcgaagcctgtgtagttggaggtggcacagggggcgggcacaaaggcccagtctctgggctgctggagcccacccacgtgccgggaccccaccagggtggggatgttggagagcggtggcggggagcagggcgaggcgtcgtagtgctcactgccggctgcctgctccaacgtcagcaccatctggatggcctcctgcttcaactggttcaggtgagtggcgcaaatgtcacagcggttgtcccggtcgttccatgccttccggatggtgttggggacctggagtttgtcgtgaatcacagccgagaaagcagggtcctgtgaggtccagaatttcaccgtccatcctgagacatcgtgtttgcttatttggggactgatgaattaatcctaggctactcagccacacttcttacccctctttcttccataatgatccttagtgaaaaggtctgaactgaaaattcactgagatgagcaaagcatcaccaaagcagctttaaatacagcaggatggtggtggggagggcgggaggagcaggaagcatttctccaggaacttggccacacctctctgccagctccagtcagtaactgtcattcttgagaagtcagttgcaaccaactattacacacccacgaagtcagagaaccggccagccattctcagcttagacccccacctcatgaatcatgacctgggtggctgcagggcaatgaggatttctgggcctgaccacaaggatgtgccacgatccgaatcttcctcggtgtgtgccacccctaccgcccctccaccaaataaagctaacctctttagaggctgccatctttactggcttctcagagaactttcatggtagggagagccggcagaacatcttgagcgtctgagcaaaggctgaggctgtcttttttgaatgaaccttctagatgttcccacaccacctcaaccacaacaagcccaagctagtatgtgaaagagggagagggggtgagtaaaccaggacccctctccctgctgcctctagtcattccaacacacaggagcctagagtttgacagagcacagctgtacttctctgctatactgttaaactgatttgtcctcacattttaaaagacagccttctgactatctttaacagatcctgtaagatacagatttgaatcaatcaattcatatacattgtctacttatataaattaattctacaagaaacttaaaacgatagccactacaactccaaaacctctaacgtgataatcgtatgaataatatgagcagactcagtggaaaagagtaaaaagcaaaagtctatagcaagagagccacttctcaccttttccctactctacacacccacccacgcccaccacacacacacacacacacacgtgtacatctctttaggaagaaaccactaagatagttctagtcgtggggttggggaacccgtactagtaagacaggctcaggagttgagattcccaaaaatgcgaagaaaactcacctccccgtccccacctgcctctatcacttttccttgaatcgattctgaaaaagttaaaaaaatgttcgtaaagtgattgttgtggtccaaaaaaggattaaaatgacaaaactgtactccaagtatttcccaggtgactttaaactggaagtaggtgggccaggcacagtggttcacgcctataatctcagcacttggcgaggccaaggttgatggattactttcagttaggagtttgagaccaacctggccaacattgtg

SEQ ID NO: 17718 - RNA, 10977 nt, Homo sapiens
  source 1..10977: mol_type = other RNA
tccccttcctccctgcccagactcccgtgtggtggcattgaagagtgtccttcatggggggacagctgggccacataccccggcggcagcatggaggccccagggacagtggcagcagacggcttagcctcaactaatagcaaacaggactttcaacctctttctcactggcaagttttcagggtttaagacgtattgtctttagaagcgagggactctgtgtgtgctccaagaatgggttactagtccagcaggaaagaacaatgagtacaggcaggactccttccttttttagtttggaaattaactcatctttagtcattttacagtctaaaatcctttttggaataagaaacctaaaaaacctaaaaacactcaatataatcagcagtggccaatgatatagacggctgtgtttgcattgaacaaatctgcagatttgtcagccttgccttctatccaaagaaggtggctggtttacaaggacatgagatacacacccaagtgggcacaactgcatttttggtcaatacaaacagaactctgagattttatcagaaagtctgagcagcaagcgtgagacttgtaggtgcgtataagactttttgaacctccaccctggatggtagatgcggctggactgaagtcactaccgccttataagaacataatagacttcaagttgaaggctaatttatgacaaaccaggccagattcctgcctgtctaattccccacgctgcgatgcctggctgtttaccccagcttctcatgagaggagccccttctccagctcaggggttcccacctttgtcaagacaggacacatctctgcatttgcatcttaatgctcccccatgttaagaatggcaactggcgaataaacaacgggcagagtgttctgattccaaatccggaagagatgaaagagacagcttcctcgtgatgtagaggggaattcaaggacaacaagatcaaagtttgcagctcgcaggtgggaactgaaagcccatgataaagcaaactctcgctcctcagcaccaccgtgcaatgcgacgtggagtgactcccagggacacaatagcaccaccgcccgttcttagatcttagttttgctccgctgctaatgcttccacctcacatatttggagcagggggtgaggaggacaggttcacacaaggagttagacctatgcatctaaatgttaatttcaaatatttttttctagtcctttcgcttgtgggtaatgaaatagaaatgggttcgttgatattcccccttgcctccttgggttctctatcaccaaaaccaaggggagacctggaactatcatgtctggccactgggtaaggcatcctcccgtgactgggactgcttcagaatggtcagccggaactccttccttcatcatcaatacagtcaatttataggcagagacaggaacaagcacatcataacgtaaaatgcctgatttcttcatgtggtttatcaatattggtaaattaacatgtttgcagcttatttaggtcaaaaaaaagcaaagagaagagagagagaatggacaacatcaacataaagcattctccttcaccgtggcctgcgagatcctgcgaggtgttctgtgattgccatcttgggaaggagtctgacttgctaagagaactcttggtttccttccgccttttgttacagcataaagttgctacaaatggataaaagcagatttaggcaggaggcaagccgaatgccactcccctcggaaggattccatcggtttcagtccaggaagggcaccaggctctgtcactggctaaaggaaggcagtgcagcatggaaggaacctcaggggaggatgtggcaggggcgaaagccaaactcatcgatgactcatcagatgagtttctttccaacaaaaacagaatattcacctttgaaaatctccaattaaagacttttcatgaactatatgtttgaaaccagcaaccagcagcccaatggcaaactcgaaggattggcttccctttgggtccagaagcctccaaggatattactgttaagcaagcccacttacacaagtgctttgaggccagaggcgagcccagagcatgcgactgtcctgcagaatggggtcaaggttaaggagctcagggaggtcctgcttcccagggcaacacacttgtcagacttgggagatacacagaaggaagaacgagccatgccagagcagcctctcactgtagtttagcctgttcagccagcagatttgggcatgtctcctgtttgcacctttgcatagaagcagactcttatggaaagtgcaaagccagactcgtgacccagggagctggcttccaaagcacatgagccaacagggccacctgaaccctgttctgataacaaaggatcaggtcatgtgaagctcacaagacttcggttcccatttaccgagttcagccagctgtgtgggctgcagtgtccagaggtacactgaccaagaaacgtagtgtttttttccccgcttggggagtggctggggctgagttgttggttaataaagacagcctagcttggaaataaataggctcatgaagatatgctgcatttgagggcaaaagggaagcgtgctctgcacacgcctaagtaccatcctcgatgcgaaggctgcagggactcttagattctgggctgcactatcatcagcaccacagcttttatcagggaaatcccttgaccactctgtaccccaggtttctatcaatcactaaaatgggtatcataattcctaagggaattgttatagggaggaacatctgaatttgaggtcctgagttgttgggagccaagacctggacatccatagtcttcagctatgttctgcctatccagggtcgtgtgagttatggaggggaagctctctctgcctttgggcaggagcaaagactgagaggacaagcctgtcccttcttggcatagaggctttgggacacaggagagctgaaatccttgtactctggacaacagacaagatgtacagtctcaagaatccttcttctaatccaatacagttgaagtctctgaacaagcctgagaaggtctctcagctggggaaaaacccactttaatcaatctacaacacaacactagaaaatactaaagaaagaaatatggctctggtgaattggttccagctttcgttcaagactttttggaataaaaatgaatatgaattttgagggccacgcaaactgtggatttgtgggtcaaggaaccacatgtgtggaggacttgaggggggcaaacggtctacagaacatacggcccacctcccaggagcagggagggcccaggtcgcaaaggactcctcctcccctgtgctgcaggtgccgtctcctcacctgttctctaaagcacctgccccacaatcaaccttctgggtctacctgaccacgctgcttgttgggatgtggcatcgaggtcacctgctgctccaaacctactttggaaacacacacactggctcgtgccgagggaagtctctctgtttgagtggcctcaccagaataaccataaaagacaggtaatatttattcataagcaatactgattaagaaatagctctacaaacacaacttacttagaaacagcaagtcagaaataggataaaacaccaagagaaaaagagctgtgaatacatttccaaaatgtttttcttgtttgttttgttgttttcatcttgactagcaccatctgtacacaagaaagtatgaacataaatgtttggataataataaagatttgcaaggcacttaatcagtcattctgggttgttttgtgttcgctttccacagcaatcctacatccacgcccctcctttctcacgaaagcaagagaagagtgaggtctcttttgctagcagttcttatgtacaaacaaggtctttaaggttcctcaaagtgctttttcagtctcacagggcttggacacccctcgggcttcccatccttttctccttccacggtgtttgacgtttgcacctttcctacagaaaacaaaagaaaactcgccttccgctcaacgcccgctccagacttgccaccaaccttcatcctcattcattgtctttgatgccccagcacagagggcctaggggcgtgcaacatctctgaagtcctggggagcgggggaccactaggacaagggtctggctcatctaccggcgcctggaggtgatgtcgaagcaggtgatcatcatgagatgggccttgcagaagttgacacggctctccaggcgctccgtcacacactccagtgcctccaggtactccagggaatccagctcccaaacctgctccaagtcaaattcactgagccacttgttgggatccagcatcagatactgtttggtcgcctccagctccttcatcagccactcgtacttcgcgcggacctcggcgatcctctgctggcggtgttccagaatcttcagctttgcattgaagcacatggcctccttgctggcaccccctcgtcgccgctgcaggcgctccacgtcatcgatttcatagactttaatctcaaagggttccccaaggcccctcgggctgctccgcaaggggccatccacccagcggacgcctgtgctgttggggggttttctcacaggggaagaggtgtccagggatagtgctgggataagcctccgtctctgagaacctggattggagcgtttcttcggggtcttgaggctccggcacctgccgcccacggagctgctgttctcgctcgtggagtcctgcgccgaggacgcgctgccggtggcctcgctgtcccgcatcacgctctcgtagccgctgctgccgccgctgtggtagaacagggccgtcttccccatggccggcgggagctccccgctcagcacgctgctgttgtcgctgccgtggccgctgctgcagcggtggggcctccgcgggggcgtgatcttgctgtagggcgacgggagcaggtgcgcggccgcgggctcgtcctcggccagggcccccccgcgcgcctccgcctcgggcccggcccgcagctgcaagccccgggcgcccgcgccaccctgcagcagctccgagatgcgcccgctgacggcccgcaggggaagcttggaggccaggcccgagctcctgttcctgctgagggactgcgtggaccagggcgtgtgcttcccaccggggggcgagctggagccctggcccaccgcctgcggcagggacttggtggagaagctgagggttttggtggtggaggcggacgggccgcgcgctctggggctggccaggaggagtctgctcacggcggagatcttggactggccggccttgggcgaggccccggagctggggggcgaggtcccggcgctgcggcccaggctcctccccgcgcggggcatggtgccgtccttgcccgcgtgcagccgggagctcacggaggacaggctctcggcccgctccagggagaggcattcgtagtggctgactgtcgccctgcccagcgagttgcttctgctggccagctgctccagcttggcactgaagagcttgctgctgctgctggcgtccttcgtcttgccgctaggctcgtctgggaggcccgccgggaaggcggctggttggttcagggggctgctggtgccgctgccgctggcactgtgctgagggctggcccggttcttctggtccaggctggactttcggacagggggcagagggggagtccctttgggccgagccagaacacagtgcttgggggaagccaccttcccctccagggtagccttggagggcggggtgcccgaggctgcacccaccccgttggtctcagcagcgcagtaataggagaggctgtccggctcctcctgccggctggccttctgaaaggccctgggaaggctgctggacttgacgcttttgttgggatgcacggggctctgggtggccaaaccgggcagggccatctcacacccatccacgaccctcctgaagttgtcagtgaccggggaggccgacacctctccgctgctgctgctgagcctgtctcccggactgggctttccgtcctgctcctgctctgctctggtctcagcattcgaggggcccgtggcagtctcacacctcatcatcccttcttcattgggatgagccgtctcttttttcacttcctcttctcgtttcagccacgggtcctcaaatttcatctctttctttgcactgttttccttactctcccgggactgggctaatgtggggcctgctttgggggtggcggtgggggcctccggctcttggatgttccgggggctcatggcaatgcaggggtaaactgtgatattggtcttcatggggatgtacccctcgcagctgctcagattggccgtgttggagatggtgaccatggccttgctcactgtggatattttgcagcctttgatgggggctgctttgttgaaagagtcatctcccatctcagacaggatgagcaagttgtcggggctggccttgggcttctctctgcacaccacagcggtgttctggaggctgctgacaaactccgaggccacaggttctgccattgcctccccgtgcccaaaacacgtctgggctatgaaactgtggcacgactgctcaccctcactgcccgcgctcatctcgctcagccaggagctgatggaagagcgtctgctccctgcgtcctgggccttctcatccaggctcatcttcgggaggggcaagaactgtgtgatgctgacctcggagacgggggccgtgctggagtagcactccaggtcctcgctgatgctgctgatgatgctgacgggccgcgagcccgaggccagggcccgtgcagagcagtcgctgttgaagctgatgatgctggtggggcggccgctgtccaggaccccgctgatggtcagctcctccaccagcgtgaacaccagctcgtcctcaccgttcagctccagtggctgctgcaccgtcaccatcgtggtgctcaggatctccttcttggactctgaaggagtagctgcctgctgctcatcatcgacaggagtttccgggaacccttcgctcccagcagacatggattttttcaaaacctgggggctcattccaaccgggggcgtacgcacctcgggctgcagcaaggactccctagacgccacgccggaatccttgctcgagggaggcagtggggcgggagacggcaggacccccttctgggtgtagactttgcatctctgggaaggagagctgggtggcttgtactccgaggtcttggacaggctggcgatgcccagccggggggagcccatgggcctgggcttgccttccacgaagccgcaggagttgaggctctcccggctgctctggaggctggggctctgcacgagtggggaggcgctgtgctggctactgctgcccgggacgctcctgggtgaggccgggctggggctgtgggcgggtgccgcggcgggcacaggtgagtgactcctctgcatcttggaggctgggagttcagggccttctctgttggtcagctgaccttcggacccattatcttccttatcagactcagagagtgggcttgcccccgctgcttggcttaaccgggggcctctgcttgcctgctctggcccaaactgagcaggcagttcttcgaaaggaaagctgctgggctcctcgctgccgtcgatgcagtccagcctctcctgcagctcggcaaacgtgttgcacttcaggcagtccctttctgacttgccggctgcagcctctcctgcctctgcgggccggctgtcgccccgggtcttctgcagggctggcacgatagggacaaagtctggggggccctcgttgtcggtgagctccttgtcagagagggccgtgccgttgggcccgatgtagatgacggtgtcgcaggactgctcgctgctggaggagtagtcggggtcgctggacaggtgagcgatggggaagtcagggtccaccgtggccctggtgtggaagggtctcagctgggtgggcctgcgcatgcggccttcttcgcaggagctctccccgccggacgagctggatgtgtacttcgtcttctttttcttcatcctcaagactctcgatgcaatctggatggtggacagggtctccgcgtagctcccgaccgcggccgagatgtgcgcgatcatggtggtacggcagttcatgttccccagagactcccgcagcaacatggcgagcttgctctctttgtatggaatgtgtttgctgccattgacgagagccaggatgacattgcccagagcagacagcgagagacacagccctgagcctccttctcgatttttgctaagagctttcacacagctgccgagatcaatgagatgcaggcggctgcgacctccagacattccccctttcccgctcttctccatccggtactggtagatgtgcagtgtgaagaacacgtgtgagttgcggtggtcgtcctcatcacagtcctgttggtggctcctgcgggaggcaatggcggcatccaggaaaaaggcagccttctctgcggtgggggcccgcagctcgctctggttctgcagctgcgtgccgcagatggggtcctcacagaggtacacgcccggggactggccgtcctgcaggctgcccgtggccacctccgacagcaggtcccgcaggttctcctccttcccccacacttccacggcggaaacccggactgagaaacgggcgccggtcttttccttgcgttcgtttatgagcttgaagagccaagagatggcacagggaatgatgcccaggttctgcatggaatcatcctttccgatcatggtgtaggattttcccagtttggcgtggccgaaacagaacacgcagccatctgccccgttgaccacagactggatcacctctgccacggtgcctgcacacacttcagcctgagaagcgtcttgtggaaaaactgcatcgaaggcaaacatctttggaggaacctggttgcctctcttttggaaggcattttgacctccacaagtcaggggatcgtacaaggtgatctgcttcttccgtgggtccacctttaagaaagagctggattctgaagtatctcgagccaaggtggaacagatgcgaagcatgactttcaccttgcccagccccggggtgtccttcaccttgttgacagccctcagcaggcagggtggggctgggggaggggaggtctgcagaatcccactgaagctggttgcaaagagcggtggttcggcagcggaagaagtggaaggccgatgtttcttctttttagaagacagatttaacttctgggcagctcgtgcaaagaaggaggcggccaccgatgtgcctgtggaagtctcgctggccacgcaggagccctgcgaggctgggacactgcaggcggaaggcttgtctgcattgtagcggttcagcactgcttctgttagtccctcccggctactctctgtcatcagctgggagatctggtatgggtacagggtgaccccgttggttctcgacagggaccaggtgccatccaggtactggtgagcctggatggccaccgaattgaggatgttcccattgcttggactggtggccatctggaggctgaccttggcctggtgggttggggacccgctcttcttttccgccccattgctgaccccaaggctgctgggtttgctgccgtgcttgttggcgaagcctgtgtagttggaggtggcacagggggcgggcacaaaggcccagtctctgggctgctggagcccacccacgtgccgggaccccaccagggtggggatgttggagagcggtggcggggagcagggcgaggcgtcgtagtgctcactgccggctgcctgctccaacgtcagcaccatctggatggcctcctgcttcaactggttcaggtgagtggcgcaaatgtcacagcggttgtcccggtcgttccatgccttccggatggtgttggggacctggagtttgtcgtgaatcacagccgagaaagcagggtccttgcccgggaagggccccgggaggagcaacctcagggcctgcctcttgagctccaccaggcgggcgttgcagttctcgcaccagacgccgcggtccgagccgggggaggagccgccgccgctgccggagcccggggagcctgtgccgaagcccggagagccgcccaaggagcccggcgaactagtgccgatgccgggggaggcgggtcccggggagccggtgaacgagctcggggacgaggtgcccgagccgggagacggggtccccgaggagccgagcgctgagcccgcgccctcaggagtgggccggctgccggcgcgcgactcctcgtatgctttccggtaccagctttccggggagaagggcgctgcgggcttggtgggcgagcagacttcattcaccccgtatttcttgcccctggtggagaccgcaagcctctctttattcccagctaccgaattcatggtggcttttccagaggagagtatctaaaggttccaccgacgctacatccagaaggtcctccaacccagaagcgtcccccggctgcagggggctggctctcagccctcagggcaaggtttcttcagcggtggggtgggagggaatgaaagcaaatggatcccacaagtaatagcaccaatttgcagaaagggttggggtcgctggtttattcttctcttcaaagcatgcttttcctcgtccccttctgcctcttccagccgcacgtcctcttgtcacggccacatccacagaactggcattttcttcagccaagtcagtccgtgctcccccacgaggaaagcgagggatacaatcagggctcgcggccgctgccgggaaggtgggagagccgagccgagtcagctgtgggaacttgtctccttcaccgagcttggtaact

SEQ ID NO: 17719 - RNA, 1799 nt, Homo sapiens
  source 1..1799: mol_type = other RNA
tccccttcctccctgcccagccccaccccgacctgctctactcatagggccacagagagtaagtccaatctctaatccaaagaccagcctgtctgacacctcacaatttacatggtggcaccaggcactccaatttgtttaagtattctcatgtagaatattttattctacagcatcctgtttgctgaaggaagtccagcctatttgcatcctccctaaaagatgtgactggctatgatctgactatcgcaacaaaaaatagaaatgatctctttcagtcaagactctgtatttccattaatgactgcattaacttgggttgttcatataacaataactcctttgagtttttagcaataggcagtgtgatgagggttcctgagatctgttatgaataatgggtaagtcaaaagtataacagagactctaggttacagaaaaagtttagaaattctagcctggacatcagctctacataaagtagttactccttttggcccattttgccttcctttttaaaaacattttgaaatatttaattgataaataaagatggaatatatccaaggtgtacaatgtgatgatttgttatacatatgcatcgtgtaatgaatgtcacaatcaaattaattaacacatccgtcatcacccatactatatagtagagcgccagaacttgttcatcttataacttaaagtttgtaccctttaaccaacatctcctcaattatcccaagcccttgacaaccactattctactcgctgcttctatgagtttgacttttttagattccacatgtaagtgagatcatgtggtttttgtcttcctatatctagcttatttcacttagtatgatgtcctctgggttcattaatgtcttgagaaatgacaggatttccttcctttttatgtctgaataatattccactgtatatgtgtaccatgatttctttatccattcatttgctgatggacacttcgattgctcccatatcttggttattacaaaaaaggatgcaatggatatggggtgcaaatatctatttgagatactgatttcatttcctttgattatgtgtccagaagaaggattgatggatcatttggcaattttatttttaattttttgagaatccttcatattgcctttgatagtggctttaccaacttacattcccaccaacagtgtgcaaagattttattttctccttaccctcaccaacacttctttcttgtctacttgataacagcaatcctaaacagcatgaggtgatattttattgtggttttgactcacatttccctgattataagtgaggttgagcataatttgttttatacaaaattatgttccacctcagactgcccaggagcaaaattggtgaggggccaacaactggcagaaaacctgcaggatgagggtggaaaatatgtctacagtcacgatggattgttttggcagcaatgttgtcctttcattgtgcaagactccaattctccccttcatcctggatacacaaaggagcaggatggcaggagtgatcataatttccttctgtggttgatggagcttcttctccattcggaagatagtccttgacttccaatttccttattattgcttggccccgtagaaattacttccattctataaaataactcctgcctggctatctttgaagctgggctcctcagacagcaggaaggggattataacctgtaatttctcatctcggttagcaggtgacaggctcccataacatggcatccatatggcgtcaccccttctgttgagcac

SEQ ID NO: 17720 - RNA, 519 nt, Homo sapiens
  source 1..519: mol_type = other RNA
tccccttcctccctgcccagctaccctgctgtgttcttacaatgagtcagagagcctccagctctgacccccagcttcagggatgagggtgaggaaacgagaggcctgacatccttcatagactttatctcacaggattcctaagctggagcaaaggaagagtaagatggggcagagttggggagatgctgatatgggggccacagttgggcatctgtcttttccaaagcaggctctgggccaatgtacagcctccctagggaatgtgtcatagagacacagggtgtgtggtgtaggcgggaagttatggttaggagagctgtgtgtgtctgatatttttctaattaaatccaaaaggtgtcagctccccagggcaactacagcctgctccaaaggagaggacccaggtcttgagaaggatctaggagagtggagcccccctccacacatctaggttggggttccctgccgagggctgagagcaagtgtgaaagccctcaccattagggcctcagccgg

SEQ ID NO: 17721 - RNA, 467 nt, Homo sapiens
  source 1..467: mol_type = other RNA
tccccttcctccctgcccagggcaccagcccagtgaccctgcagggagggtggaggggaagccctaatgaaagagaaaaaaaagcagcagcagcacatgacagggaaactgagtcacggagcaggccccaggagggtttgtgtagaagctgccttcagctccagggtagagggggacaggcgccggctcactgatgacattcacggacatcctccttcccaagctgccgtccttcccaatgaccagagacatctttgcaagcatagcatggctggaggatgcgtttcaccaaacgcgatgtaagcaccaccaggtgcccagcgcggaggtggatgtgggcgaaccctggacgccccacaaaggacagctgcggcctgggaagggaaggagatggagcggggagagggggaagaggttgctccgcgttttccgcccgcccgcctgctttccgcgaggcactgaggcct

SEQ ID NO: 17722 - RNA, 264 nt, Homo sapiens
  source 1..264: mol_type = other RNA
tccctacccctccactccccagaaccatcattgcttcctcatctcctgtctcctccctgccccaaggccctccctgtgctcaccctggctcctccccctgctccatgcccagcctctgcagagcagcccaggcccagagacttgggcagaagcttccgtcccaccagctgcagaaccttccctacagaaccaggccagtccctgtgtctcatatttgtagagatcccaatcaccctcagagatgacgggtgggaaaccagccca

SEQ ID NO: 17723 - RNA, 4563 nt, Homo sapiens
  source 1..4563: mol_type = other RNA
tccctccttctgtccccacagagatgcttctgctcagggccaagggctcccaggtcacagatgtggaaacagcctcccgtggagctagcagtgcccagatttgaacctggagctgtggtctttccagtatatgaggcctgccttgactatactgcctccttcattatatcctgcatacagttggtactctgtaattgctttctggacacaagaataaagaaacaggattcagaaacaggggaatgggaaggacaagaagaacctcggggttggctggagtggctctggagaggacctgagctgagagccagtggattaagttgaactggaatcaacgagccccctatactccaggctttacggtaactggaacaggctccgactccctggagcgccaggtccagggtgacatctgagctcagcgaaccgaattttgaatctaaaactcgacactcgattcagttattggacaacactgaagtatgtttggaacaacttgggtctgagaatctgctttttcaactgtaaatcttatgatagctaaattcagatcaagtatttccaataaaacttcggcatctgaatggagatgtgctgtaagtaaaaaatgcatacttttgtgctctccaaagagagtccgaaacatgtaaagcaactcaatatttttatattgattgcatactgaaatggtaattttgaacatgttggatgaaattatcatttatttgcaactgtttgttctttaatgtagctactagaaaatttatatcacatatgtggttcacagtcatagcttctattggacaatgccaccttgaagcctatgatattttgataaaatggaaataaagagtttgcggaaattttatgattgttttttactcatctaggcagagtacttggaatgccctagttcaatccccttgttttacaaataggaaacctgaggccagagaaggcaagtaagttgcctgggtcacacagcatgtggatggagctgggcccataacttggcacttgctccaggcatgcttggaggtgccggctgctgtagaccaacctaaaccaggctcccccatcccccttttttcagatatgccttgcaagaacacagatctgcaggccactagaaccaagcaagatgccaacatgcctgacacccaacctgggtcagaagattaccccagggcaagtagcaaggagacatcataagggcttttcctggttggtgaagaccacaggctgctgcccaagggaagggcctggagtccctgacacttggccatctgtgcaccgtgctcaaagcctcaccttccaactacaaagagaaaaatgttccctctgtgaaaaggtgggctgtatccagcagagggtaacctgtccagctcacgttaccgcaggagcaattcctcctctctgaacagagtgcagcatcgtgggggtggagacccggctgaggggggtgggcctcctccccctgcccgctgctccatcgtggacgtcttctctcagagcctcgattttcccattagaggcagggcagcgtgaagccaaggagaaggcgggcactcagctggcaccacgtggccttgagccacagattgccagatgccatcagaagctggagggggcaggaagggctctcctctagagcctctggaggggcacagcccgaccgacgcctggggctcagacttgtggtccccagaaccagccctgcgactcggtcttcgctcctggtctggatccggcatctctcctgctggacccaggctcctgagaggctgggactgttgccgccagtgttgtctggaatcctggtctccaggacagtgcccacatgtgctgggtgccccagagagtacactgcctctccagacacagctgcccccttggccggactgggctcccccagggcagggagtctggaatccatttctgggtcttcgtgcctagcacggggccctggcagacactctccaggcttctggaattctgaacggcattcccatttgcaaacacaaaaacagaggcttggagcaccttagccagctgcccaagcagccgtcgttactgagcagggagaccagaccccgtgtgtctgactcaagcctgagggccccctttggtttggggccttacaacacaggaaggacaggctgggatctgaagagggttcgggtcttcgtggcagaacagaaggcctacgaatggcccccactcccatcccaggctttctttcccacaggctgtgctcagggatggcctagatccagcttgggagagacccaggccctcgacaggacaggatgcagaggtgggcattctcacagcttccctccatggctcccgcgggtgtacaatgcaccccaaggggcagctgagaagcgaaggcagccagcacattactcctaggaggtctcatggttcatcaccggtcggggcaccttgtaagctctgatgccatccaagggccctctgtagaacaagcacagacacatcagttggatacaagaccccctgaggcccactcacggatcaccagaggctctgcgggcctgaggccaggatgcccccgaagggaaagaggaggcctgggacccacggtcgtctcaggcatgaatctgccatgggcctgtgggccagtcactgggcctctcggggcctccatttctccatcataaaacaggagcctgaagtctaacccccaagtccaaggactcttcctcctgcttcccagtggggtgggcttccctgacatcctggaaagaccatcattcccaccagcagcccaggcctgggcactgtggggacacactttcctccgctcatgccccgaggccaggcagcgggctggagacagctccaggcagagatgggagggcctcgaacctgcgtcctgtgtcaaggaggcaccaacagaaaaccataaagggctcaagctggttcccgggcaggcagcccctctcgtccctagacactgcagtgggagtgcaatccagggtctccacctctcctgacccttccaagccccggctctggctccaaggggctgtgggcaaggagagcgtgatgagtattgaccctgcattcaatgggcaatcactcatgttattttgggtaacagaccttgggtgaagccaatttagtggcaatttgtaataaaaataacagatgggctcagccagcaaggcagacatccagtgaacgcggctgcagggaggtgtcgaacctgctggagccgcctgaaacccaggccctcacgccctgcatctgctccactgcactttgtcacggagcagctgtaacgaccttggctatcattttttgagcacctaggacagatgaggaagtggtagatcagagaggtcggaagccttggacaaagccacacagccaggaaacagggggctgagacttcctccaggtcggcctgactccaatgcccgggctccctgctctgcaccacgctgcctcacaggaggctgcacacgcggggcctgggtgtggggaactggacgcatcccacccctgtgtctgagctcacgggagtcagcctccggggctggggaagaaccaggtcactggtgcagctgaagggctttacaagtcctggttttggtgctttgtggccaaaactgacagcattctcttttgtgaattttcccctctgtgcagggcttccaagttgcctcccaataaatactgtcccctctgctttagcaacaaaactctttgaagataggggtagccagagaaacgaaagcagaaatcagtgaaagaggcttctgggctatctctaaaagctgagaggaggcccacctttgcctcttgcccttccccttattcctgaataaaacaggaatgtgagagctggtgcttcagcagccattctgtgacctggaggatgaaacttatccactaaggatggccaaaaaaaaaaaagcaagatagaaggagtccctgggttcctggccacactagccctgggctgcccacctcccactgtggtcagtgccctgtcagcagccaaacacagattctgactggcccagtttacaagagcctcctgtattagggtattgactctatttcttaaatggaagccaagtcatggtagcttacacaagacagaaagttttgtttgtttctcacaaacaaataaatgagtgaagctggtaaaccatccaggaggtaggacagctctgccccaggtcaccagggacctggctccttctatccgaggctctgctttgctgtaactaaattgtcctcacctgaccatcacagccccattccaggcagccaagaaggagagtttgagggtcacccaacttcctgataagtcaaagatctatccagatgttgcccgctgcacatctcatgctcactggtcagaaccacatcatgtgaccgggctgagctgcaagggaggctgggaaatgtagtctttagctaagtgcccaactgaaatccagaagggttcaattagtaaaaggtaaaaggggagaatgcggctgggcatggtggctcacacctgtaatcccagcactttggcaggcc

SEQ ID NO: 17724 - RNA, 5152 nt, Homo sapiens
  source 1..5152: mol_type = other RNA
tccctccttctgtccccacagagatgcttctgctcagggccaagggctcccaggtcacagatgtggaaacagcctcccgtggagctagcagtgcccagatttgaacctggagctgtggtctttccagtatatgaggcctgccttgactatactgcctccttcattatatcctgcatacagttggtactctgtaattgctttctggacacaagaataaagaaacaggattcagaaacaggggaatgggaaggacaagaagaacctcggggttggctggagtggctctggagaggacctgagctgagagccagtggattaagttgaactggaatcaacgagccccctatactccaggctttacggtaactggaacaggctccgactccctggagcgccaggtccagggtgacatctgagctcagcgaaccgaattttgaatctaaaactcgacactcgattcagttattggacaacactgaagtatgtttggaacaacttgggtctgagaatctgctttttcaactgtaaatcttatgatagctaaattcagatcaagtatttccaataaaacttcggcatctgaatggagatgtgctgtaagtaaaaaatgcatacttttgtgctctccaaagagagtccgaaacatgtaaagcaactcaatatttttatattgattgcatactgaaatggtaattttgaacatgttggatgaaattatcatttatttgcaactgtttgttctttaatgtagctactagaaaatttatatcacatatgtggttcacagtcatagcttctattggacaatgccaccttgaagcctatgatattttgataaaatggaaataaagagtttgcggaaattttatgattgttttttactcatctaggcagagtacttggaatgccctagttcaatccccttgttttacaaataggaaacctgaggccagagaaggcaagtaagttgcctgggtcacacagcatgtggatggagctgggcccataacttggcacttgctccaggcatgcttggaggtgccggctgctgtagaccaacctaaaccaggctcccccatcccccttttttcagatatgccttgcaagaacacagatctgcaggccactagaaccaagcaagatgccaacatgcctgacacccaacctgggtcagaagattaccccagggcaagtagcaaggagacatcataagggcttttcctggttggtgaagaccacaggctgctgcccaagggaagggcctggagtccctgacacttggccatctgtgcaccgtgctcaaagcctcaccttccaactacaaagagaaaaatgttccctctgtgaaaaggtgggctgtatccagcagagggtaacctgtccagctcacgttaccgcaggagcaattcctcctctctgaacagagtgcagcatcgtgggggtggagacccggctgaggggggtgggcctcctccccctgcccgctgctccatcgtggacgtcttctctcagagcctcgattttcccattagaggcagggcagcgtgaagccaaggagaaggcgggcactcagctggcaccacgtggccttgagccacagattgccagatgccatcagaagctggagggggcaggaagggctctcctctagagcctctggaggggcacagcccgaccgacgcctggggctcagacttgtggtccccagaactgcaagataaaacatttcaattgtctgaagcccattgcctgtggcccttggtcccggcagccccaggacactcacggagacacacgcagggcagctctcctggggtccccccggccccagcgtgcggtcttcaactgtcatcaggcccatgtggatgcaaccccaggggtttttctccctctcttccaatcctctgcccttgctgggtagggcaggaagaaatggggaccctcacaggaggtctctgagctggaacagcccctccgggcatcgggtgtggtctgccatttgtcatttaactccaccctcagcccggagtcttcagatgagggttctctgcccttgcttcctgtcaggggggcccgatgggagggacacaggtgggcaggtgacaaaggaagtggccaagggtgtgtcccaaaccctgtgggtgttggtttctctgggcctccttctcccacagccccacaacccccctcagcccacccatgtgccgaagagtgtctcacgtggcaagcctggcacctgataggcacacggtgagtctgttgactgaatgagtgaaggtagacagggtgctggctggggccagccctgcgactcggtcttcgctcctggtctggatccggcatctctcctgctggacccaggctcctgagaggctgggactgttgccgccagtgttgtctggaatcctggtctccaggacagtgcccacatgtgctgggtgccccagagagtacactgcctctccagacacagctgcccccttggccggactgggctcccccagggcagggagtctggaatccatttctgggtcttcgtgcctagcacggggccctggcagacactctccaggcttctggaattctgaacggcattcccatttgcaaacacaaaaacagaggcttggagcaccttagccagctgcccaagcagccgtcgttactgagcagggagaccagaccccgtgtgtctgactcaagcctgagggccccctttggtttggggccttacaacacaggaaggacaggctgggatctgaagagggttcgggtcttcgtggcagaacagaaggcctacgaatggcccccactcccatcccaggctttctttcccacaggctgtgctcagggatggcctagatccagcttgggagagacccaggccctcgacaggacaggatgcagaggtgggcattctcacagcttccctccatggctcccgcgggtgtacaatgcaccccaaggggcagctgagaagcgaaggcagccagcacattactcctaggaggtctcatggttcatcaccggtcggggcaccttgtaagctctgatgccatccaagggccctctgtagaacaagcacagacacatcagttggatacaagaccccctgaggcccactcacggatcaccagaggctctgcgggcctgaggccaggatgcccccgaagggaaagaggaggcctgggacccacggtcgtctcaggcatgaatctgccatgggcctgtgggccagtcactgggcctctcggggcctccatttctccatcataaaacaggagcctgaagtctaacccccaagtccaaggactcttcctcctgcttcccagtggggtgggcttccctgacatcctggaaagaccatcattcccaccagcagcccaggcctgggcactgtggggacacactttcctccgctcatgccccgaggccaggcagcgggctggagacagctccaggcagagatgggagggcctcgaacctgcgtcctgtgtcaaggaggcaccaacagaaaaccataaagggctcaagctggttcccgggcaggcagcccctctcgtccctagacactgcagtgggagtgcaatccagggtctccacctctcctgacccttccaagccccggctctggctccaaggggctgtgggcaaggagagcgtgatgagtattgaccctgcattcaatgggcaatcactcatgttattttgggtaacagaccttgggtgaagccaatttagtggcaatttgtaataaaaataacagatgggctcagccagcaaggcagacatccagtgaacgcggctgcagggaggtgtcgaacctgctggagccgcctgaaacccaggccctcacgccctgcatctgctccactgcactttgtcacggagcagctgtaacgaccttggctatcattttttgagcacctaggacagatgaggaagtggtagatcagagaggtcggaagccttggacaaagccacacagccaggaaacagggggctgagacttcctccaggtcggcctgactccaatgcccgggctccctgctctgcaccacgctgcctcacaggaggctgcacacgcggggcctgggtgtggggaactggacgcatcccacccctgtgtctgagctcacgggagtcagcctccggggctggggaagaaccaggtcactggtgcagctgaagggctttacaagtcctggttttggtgctttgtggccaaaactgacagcattctcttttgtgaattttcccctctgtgcagggcttccaagttgcctcccaataaatactgtcccctctgctttagcaacaaaactctttgaagataggggtagccagagaaacgaaagcagaaatcagtgaaagaggcttctgggctatctctaaaagctgagaggaggcccacctttgcctcttgcccttccccttattcctgaataaaacaggaatgtgagagctggtgcttcagcagccattctgtgacctggaggatgaaacttatccactaaggatggccaaaaaaaaaaaagcaagatagaaggagtccctgggttcctggccacactagccctgggctgcccacctcccactgtggtcagtgccctgtcagcagccaaacacagattctgactggcccagtttacaagagcctcctgtattagggtattgactctatttcttaaatggaagccaagtcatggtagcttacacaagacagaaagttttgtttgtttctcacaaacaaataaatgagtgaagctggtaaaccatccaggaggtaggacagctctgccccaggtcaccagggacctggctccttctatccgaggctctgctttgctgtaactaaattgtcctcacctgaccatcacagccccattccaggcagccaagaaggagagtttgagggtcacccaacttcctgataagtcaaagatctatccagatgttgcccgctgcacatctcatgctcactggtcagaaccacatcatgtgaccgggctgagctgcaagggaggctgggaaatgtagtctttagctaagtgcccaactgaaatccagaagggttcaattagtaaaaggtaaaaggggagaatgcggctgggcatggtggctcacacctgtaatcccagcactttggcaggcc

SEQ ID NO: 17725 - RNA, 2790 nt, Homo sapiens
  source 1..2790: mol_type = other RNA
tccctccttctgtccccacagagtctgctagatcttcctcttctgagtcatcctcttcttcctcctctggtgctgacgaactggaggtgggccctttgcaggttttcaggtggcgggtgagatggtatttggttagataagcctttgtacatttttcacagacataatcccgttttccttcatgagaattgagatgcttctttaagtgatttgttctcaagaacagcttatcacacttgggacacttgatctggcgttcttgagtgtggatgagcacgtgctgcttgaggtcctgcctccgcataaacaacttgtcacagtaatcacacttaagattcttctccccagtgtggataaccatgtgggactccaggtgagccttctgggtgaaagacttgtcacacaaggtacacctgtagttcttctgacctgtatgtatcttgaggtgggtccgcaggttgctgggatcactaaaagccttgctacagaaatcacacttgtggggcttcatacccatgtgacccataaagtggacatgaagtttggaaggagagataaaagcttgggggcacattgagcacttccacttcctttctttgctgtgacttggcccatggctgccgctatgtccctgggtaggaagatggttatggatgtggctggtcagatgggctttgaactctgtgtaagaattgcactccttgccacagttacagagatgcacatctgggtgttcaggaacaccaatctgttgagcataatctcggctataataaaaaagcagttcattttcaggagggatatcttgtgaggtgcagaaaaagatttttccatcatgaggataagccaccaaattctgctcttcccggttcctggctttgcgcacaaacatcatccaattacattcattttcatcagttgtaatgatgcagaattctaggacaccattgtggtatatcttccagatatggttaactgccttgtctgtccattctgctacttccatggagtgactctgctggccaattagaggtccaaagcaagtccgcacaggaatggtttctccagtccatacaccaacttctgctcccacaattgactgacggagaacaagctgctttgggagagaaagccttgctctgctctctattggagtgtcaggaacaaaagtcactggtccatgttcgggacagtccgagggataggcgcggtcacacagagtacaccaaattgtaaacaaggttgccatgttctccttgtttgaattggagtcttccatttgcagtgaaggtgatacaaaagaaagactgtctgaagatacatctacatgacctgtccccatagcaacctcctgggtgatggaggagacagccacaggttctaggctgaggccaacttcatggagggaaacagattctagggaggcaaggttgtgtgaggtagagagtgccacgcttacagagttggtgctcatggccacagtgtgaatggagtcactgagggcactgtcagacatgccattgacccgacttgcaatgtggtctgtctccatgaccacagggagctccaggccattcccatgcatgggtatcacaccaccatgtcctacagcgtctgctgcaaggttgttgctcacagaatccacagacagaggttcatgacttctggagccatttgggatttgggaatgctcgcctgcaacaccgtccatcgtaagctcctctgccattccatctgtcgaaattgggctggtaaccctagaaacgttctccatagtgattgctgtgtccaaggccacctcatggccatcactgggatgaagactttgggcaccatgtgtgttcacagagcgagagtctattgaaacaatgcctggttctaatccaacatttccattggactgatagggatctagtgctgaagggttattggtgatagataatgctgtattaccatcaacatttatagagttagggtggatgtactgtggaggtggtctgtcagctaaataagataaaatgccaggtagaatggttctgaaataactgctctccaggtgagggtaaggtggtggaggtagggtgtagtttctttcaggtaacccacacatcacccctcgatccccaatacccattggtagcattaaagacagagcagaaggcagagagctcagggagggacccaggtttggaattgccactgggaggcctggggcagggatggcactgtgagtgggtgaggcagccaatcccaggtgacttcctgagactggcaaggcattgctcacagaggatgaagtcagctgctccatccccactggactcaggttcatttcattcatcctgtgatgcatcggcttggggccaaatatcagagaaaggagcgctcgggtggtggggaacaggcatcagggtttgcgttccagggtcacgtgctaccacatcttgctcacaaccgctgcaccgacgcggccactcgtccccggggtcgcccggggccgcccaacttctcccgagggccggtggccgtgcaccccgccacgggttggggcatctcggggaacacctggggccttccgtccagaagcttcgggaagggggctgcccaacctgccagctgcgctgggggcgcacgcgcctgccccactgctttgttcctcatccgggcagagttcgcctcggggccctgcccgtccgctcggccccctcaccccgggggccgctgccctaacgtttcccgtcccgcccggcccttcccggcccgcggcctcctctgggccgcaccctctgc

SEQ ID NO: 17726 - RNA, 2772 nt, Homo sapiens
  source 1..2772: mol_type = other RNA
tccctccttctgtccccacagagtctgctagatcttcctcttctgagtcatcctcttcttcctcctctggtgctgacgaactggaggtgggccctttgcaggttttcaggtggcgggtgagatggtatttggttagataagcctttgtacatttttcacagacataatcccgttttccttcatgagaattgagatgcttctttaagtgatttgttctcaagaacagcttatcacacttgggacacttgatctggcgttcttgagtgtggatgagcacgtgctgcttgaggtcctgcctccgcataaacaacttgtcacagtaatcacacttaagattcttctccccagtgtggataaccatgtgggactccaggtgagccttctgggtgaaagacttgtcacacaaggtacacctgtagttcttctgacctgtatgtatcttgaggtgggtccgcaggttgctgggatcactaaaagccttgctacagaaatcacacttgtggggcttcatacccatgtgacccataaagtggacatgaagtttggaaggagagataaaagcttgggggcacattgagcacttccacttcctttctttgctgtgacttggcccatggctgccgctatgtccctgggtaggaagatggttatggatgtggctggtcagatgggctttgaactctgtgtaagaattgcactccttgccacagttacagagatgcacatctgggtgttcaggaacaccaatctgttgagcataatctcggctataataaaaaagcagttcattttcaggagggatatcttgtgaggtgcagaaaaagatttttccatcatgaggataagccaccaaattctgctcttcccggttcctggctttgcgcacaaacatcatccaattacattcattttcatcagttgtaatgatgcagaattctaggacaccattgtggtatatcttccagatatggttaactgccttgtctgtccattctgctacttccatggagtgactctgctggccaattagaggtccaaagcaagtccgcacaggaatggtttctccagtccatacacctgtcagtggaaggacaccaacaacttctgctcccacaattgactgacggagaacaagctgctttgggagagaaagccttgctctgctctctattggagtgtcaggaacaaaagtcactggtccatgttcgggacagtccgagggataggcgcggtcacacagagtacaccaaattgtaaacaaggttgccatgttctccttgtttgaattggagtcttccatttgcagtgaaggtgatacaaaagaaagactgtctgaagatacatctacatgacctgtccccatagcaacctcctgggtgatggaggagacagccacaggttctaggctgaggccaacttcatggagggaaacagattctagggaggcaaggttgtgtgaggtagagagtgccacgcttacagagttggtgctcatggccacagtgtgaatggagtcactgagggcactgtcagacatgccattgacccgacttgcaatgtggtctgtctccatgaccacagggagctccaggccattcccatgcatgggtatcacaccaccatgtcctacagcgtctgctgcaaggttgttgctcacagaatccacagacagaggttcatgacttctggagccatttgggatttgggaatgctcgcctgcaacaccgtccatcgtaagctcctctgccattccatctgtcgaaattgggctggtaaccctagaaacgttctccatagtgattgctgtgtccaaggccacctcatggccatcactgggatgaagactttgggcaccatgtgtgttcacagagcgagagtctattgaaacaatgcctggttctaatccaacatttccattggactgatagggatctagtgctgaagggttattggtgatagataatgctgtattaccatcaacatttatagagttagggtggatgtactgtggaggtggtctgtcagctaaataagataaaatgccaggtagaatggttctgaaataactgctctccaggtgagggtaaggtggtggaggtagggtgtagtttctttcaggtaacccacacatcacccctcgatccccaatacccattggtagcattaaagacagagcagaaggcagagagctcagggagggacccaggtttggaattgccactgggaggcctggggcagggatggcactgtgagtgggtgaggcagccaatcccaggtgacttcctgagactggcaaggcattgctcacagaggatgaagtcagctgctccatccccactggactcaggttcatttcattcatcctgtgatgcatcggcttggggccaaatatcagagaaaggagcgctcgggtggtggggaacaggcatcagggtttgcgttccagggtcacgtgctaccacatcttgctcacaaccgctgcaccgacgcggccactcgtccccggggtcgcccggggccgcccaacttctcccgagggccggtggccgtgcaccccgccacgggttggggcatctcggggaacacctggggccttccgtccagaagcttcgggaagggggctgcccaaccctctgcggcgcgtttccggatcctcagccactctcagcgcccgccgctccgcccctcgtgcgtgcgccctccccgccgcggcccgcaagcggcgcccgcgcaccgcgtcgcccttctcccagcccaggcccctccgcgcgt

SEQ ID NO: 17727 - RNA, 2809 nt, Homo sapiens
  source 1..2809: mol_type = other RNA
tccctccttctgtccccacagagtctgctagatcttcctcttctgagtcatcctcttcttcctcctctggtgctgacgaactggaggtgggccctttgcaggttttcaggtggcgggtgagatggtatttggttagataagcctttgtacatttttcacagacataatcccgttttccttcatgagaattgagatgcttctttaagtgatttgttctcaagaacagcttatcacacttgggacacttgatctggcgttcttgagtgtggatgagcacgtgctgcttgaggtcctgcctccgcataaacaacttgtcacagtaatcacacttaagattcttctccccagtgtggataaccatgtgggactccaggtgagccttctgggtgaaagacttgtcacacaaggtacacctgtagttcttctgacctgtatgtatcttgaggtgggtccgcaggttgctgggatcactaaaagccttgctacagaaatcacacttgtggggcttcatacccatgtgacccataaagtggacatgaagtttggaaggagagataaaagcttgggggcacattgagcacttccacttcctttctttgctgtgacttggcccatggctgccgctatgtccctgggtaggaagatggttatggatgtggctggtcagatgggctttgaactctgtgtaagaattgcactccttgccacagttacagagatgcacatctgggtgttcaggaacaccaatctgttgagcataatctcggctataataaaaaagcagttcattttcaggagggatatcttgtgaggtgcagaaaaagatttttccatcatgaggataagccaccaaattctgctcttcccggttcctggctttgcgcacaaacatcatccaattacattcattttcatcagttgtaatgatgcagaattctaggacaccattgtggtatatcttccagatatggttaactgccttgtctgtccattctgctacttccatggagtgactctgctggccaattagaggtccaaagcaagtccgcacaggaatggtttctccagtccatacacctgtcagtggaaggacaccaacaacttctgctcccacaattgactgacggagaacaagctgctttgggagagaaagccttgctctgctctctattggagtgtcaggaacaaaagtcactggtccatgttcgggacagtccgagggataggcgcggtcacacagagtacaccaaattgtaaacaaggttgccatgttctccttgtttgaattggagtcttccatttgcagtgaaggtgatacaaaagaaagactgtctgaagatacatctacatgacctgtccccatagcaacctcctgggtgatggaggagacagccacaggttctaggctgaggccaacttcatggagggaaacagattctagggaggcaaggttgtgtgaggtagagagtgccacgcttacagagttggtgctcatggccacagtgtgaatggagtcactgagggcactgtcagacatgccattgacccgacttgcaatgtggtctgtctccatgaccacagggagctccaggccattcccatgcatgggtatcacaccaccatgtcctacagcgtctgctgcaaggttgttgctcacagaatccacagacagaggttcatgacttctggagccatttgggatttgggaatgctcgcctgcaacaccgtccatcgtaagctcctctgccattccatctgtcgaaattgggctggtaaccctagaaacgttctccatagtgattgctgtgtccaaggccacctcatggccatcactgggatgaagactttgggcaccatgtgtgttcacagagcgagagtctattgaaacaatgcctggttctaatccaacatttccattggactgatagggatctagtgctgaagggttattggtgatagataatgctgtattaccatcaacatttatagagttagggtggatgtactgtggaggtggtctgtcagctaaataagataaaatgccaggtagaatggttctgaaataactgctctccaggtgagggtaaggtggtggaggtagggtgtagtttctttcaggtaacccacacatcacccctcgatccccaatacccattggtagcattaaagacagagcagaaggcagagagctcagggagggacccaggtttggaattgccactgggaggcctggggcagggatggcactgtgagtgggtgaggcagccaatcccaggtgacttcctgagactggcaaggcattgctcacagaggatgaagtcagctgctccatccccactggactcaggttcatttcattcatcctgtgatgcatcggcttggggccaaatatcagagaaaggagcgctcgggtggtggggaacaggcatcagggtttgcgttccagggtcacgtgctaccacatcttgctcacaaccgctgcaccgacgcggccactcgtccccggggtcgcccggggccgcccaacttctcccgagggccggtggccgtgcaccccgccacgggttggggcatctcggggaacacctggggccttccgtccagaagcttcgggaagggggctgcccaacctgccagctgcgctgggggcgcacgcgcctgccccactgctttgttcctcatccgggcagagttcgcctcggggccctgcccgtccgctcggccccctcaccccgggggccgctgccctaacgtttcccgtcccgcccggcccttcccggcccgcggcctcctctgggccgcaccctct

SEQ ID NO: 17728 - RNA, 2702 nt, Homo sapiens
  source 1..2702: mol_type = other RNA
tccctccttctgtccccacagagtctgctagatcttcctcttctgagtcatcctcttcttcctcctctggtgctgacgaactggaggtgggccctttgcaggttttcaggtggcgggtgagatggtatttggttagataagcctttgtacatttttcacagacataatcccgttttccttcatgagaattgagatgcttctttaagtgatttgttctcaagaacagcttatcacacttgggacacttgatctggcgttcttgagtgtggatgagcacgtgctgcttgaggtcctgcctccgcataaacaacttgtcacagtaatcacacttaagattcttctccccagtgtggataaccatgtgggactccaggtgagccttctgggtgaaagacttgtcacacaaggtacacctgtagttcttctgacctgtatgtatcttgaggtgggtccgcaggttgctgggatcactaaaagccttgctacagaaatcacacttgtggggcttcatacccatgtgacccataaagtggacatgaagtttggaaggagagataaaagcttgggggcacattgagcacttccacttcctttctttgctgtgacttggcccatggctgccgctatgtccctgggtaggaagatggttatggatgtggctggtcagatgggctttgaactctgtgtaagaattgcactccttgccacagttacagagatgcacatctgggtgttcaggaacaccaatctgttgagcataatctcggctataataaaaaagcagttcattttcaggagggatatcttgtgaggtgcagaaaaagatttttccatcatgaggataagccaccaaattctgctcttcccggttccttccagatatggttaactgccttgtctgtccattctgctacttccatggagtgactctgctggccaattagaggtccaaagcaagtccgcacaggaatggtttctccagtccatacaccaacttctgctcccacaattgactgacggagaacaagctgctttgggagagaaagccttgctctgctctctattggagtgtcaggaacaaaagtcactggtccatgttcgggacagtccgagggataggcgcggtcacacagagtacaccaaattgtaaacaaggttgccatgttctccttgtttgaattggagtcttccatttgcagtgaaggtgatacaaaagaaagactgtctgaagatacatctacatgacctgtccccatagcaacctcctgggtgatggaggagacagccacaggttctaggctgaggccaacttcatggagggaaacagattctagggaggcaaggttgtgtgaggtagagagtgccacgcttacagagttggtgctcatggccacagtgtgaatggagtcactgagggcactgtcagacatgccattgacccgacttgcaatgtggtctgtctccatgaccacagggagctccaggccattcccatgcatgggtatcacaccaccatgtcctacagcgtctgctgcaaggttgttgctcacagaatccacagacagaggttcatgacttctggagccatttgggatttgggaatgctcgcctgcaacaccgtccatcgtaagctcctctgccattccatctgtcgaaattgggctggtaaccctagaaacgttctccatagtgattgctgtgtccaaggccacctcatggccatcactgggatgaagactttgggcaccatgtgtgttcacagagcgagagtctattgaaacaatgcctggttctaatccaacatttccattggactgatagggatctagtgctgaagggttattggtgatagataatgctgtattaccatcaacatttatagagttagggtggatgtactgtggaggtggtctgtcagctaaataagataaaatgccaggtagaatggttctgaaataactgctctccaggtgagggtaaggtggtggaggtagggtgtagtttctttcaggtaacccacacatcacccctcgatccccaatacccattggtagcattaaagacagagcagaaggcagagagctcagggagggacccaggtttggaattgccactgggaggcctggggcagggatggcactgtgagtgggtgaggcagccaatcccaggtgacttcctgagactggcaaggcattgctcacagaggatgaagtcagctgctccatccccactggactcaggttcatttcattcatcctgtgatgcatcggcttggggccaaatatcagagaaaggagcgctcgggtggtggggaacaggcatcagggtttgcgttccagggtcacgtgctaccacatcttgctcacaaccgctgcaccgacgcggccactcgtccccggggtcgcccggggccgcccaacttctcccgagggccggtggccgtgcaccccgccacgggttggggcatctcggggaacacctggggccttccgtccagaagcttcgggaagggggctgcccaacctgccagctgcgctgggggcgcacgcgcctgccccactgctttgttcctcatccgggcagagttcgcctcggggccctgcccgtccgctcggccccctcaccccgggggccgctgccctaacgtttcccgtcccgcccggcccttcccggcccgcggcctcctctgggccgcaccctct

SEQ ID NO: 17729 - RNA, 2723 nt, Homo sapiens
  source 1..2723: mol_type = other RNA
tccctccttctgtccccacagagtctgctagatcttcctcttctgagtcatcctcttcttcctcctctggtgctgacgaactggaggtgggccctttgcaggttttcaggtggcgggtgagatggtatttggttagataagcctttgtacatttttcacagacataatcccgttttccttcatgagaattgagatgcttctttaagtgatttgttctcaagaacagcttatcacacttgggacacttgatctggcgttcttgagtgtggatgagcacgtgctgcttgaggtcctgcctccgcataaacaacttgtcacagtaatcacacttaagattcttctccccagtgtggataaccatgtgggactccaggtgagccttctgggtgaaagacttgtcacacaaggtacacctgtagttcttctgacctgtatgtatcttgaggtgggtccgcaggttgctgggatcactaaaagccttgctacagaaatcacacttgtggggcttcatacccatgtgacccataaagtggacatgaagtttggaaggagagataaaagcttgggggcacattgagcacttccacttcctttctttgctgtgacttggcccatggctgccgctatgtccctgggtaggaagatggttatggatgtggctggtcagatgggctttgaactctgtgtaagaattgcactccttgccacagttacagagatgcacatctgggtgttcaggaacaccaatctgttgagcataatctcggctataataaaaaagcagttcattttcaggagggatatcttgtgaggtgcagaaaaagatttttccatcatgaggataagccaccaaattctgctcttcccggttccttccagatatggttaactgccttgtctgtccattctgctacttccatggagtgactctgctggccaattagaggtccaaagcaagtccgcacaggaatggtttctccagtccatacacctgtcagtggaaggacaccaacaacttctgctcccacaattgactgacggagaacaagctgctttgggagagaaagccttgctctgctctctattggagtgtcaggaacaaaagtcactggtccatgttcgggacagtccgagggataggcgcggtcacacagagtacaccaaattgtaaacaaggttgccatgttctccttgtttgaattggagtcttccatttgcagtgaaggtgatacaaaagaaagactgtctgaagatacatctacatgacctgtccccatagcaacctcctgggtgatggaggagacagccacaggttctaggctgaggccaacttcatggagggaaacagattctagggaggcaaggttgtgtgaggtagagagtgccacgcttacagagttggtgctcatggccacagtgtgaatggagtcactgagggcactgtcagacatgccattgacccgacttgcaatgtggtctgtctccatgaccacagggagctccaggccattcccatgcatgggtatcacaccaccatgtcctacagcgtctgctgcaaggttgttgctcacagaatccacagacagaggttcatgacttctggagccatttgggatttgggaatgctcgcctgcaacaccgtccatcgtaagctcctctgccattccatctgtcgaaattgggctggtaaccctagaaacgttctccatagtgattgctgtgtccaaggccacctcatggccatcactgggatgaagactttgggcaccatgtgtgttcacagagcgagagtctattgaaacaatgcctggttctaatccaacatttccattggactgatagggatctagtgctgaagggttattggtgatagataatgctgtattaccatcaacatttatagagttagggtggatgtactgtggaggtggtctgtcagctaaataagataaaatgccaggtagaatggttctgaaataactgctctccaggtgagggtaaggtggtggaggtagggtgtagtttctttcaggtaacccacacatcacccctcgatccccaatacccattggtagcattaaagacagagcagaaggcagagagctcagggagggacccaggtttggaattgccactgggaggcctggggcagggatggcactgtgagtgggtgaggcagccaatcccaggtgacttcctgagactggcaaggcattgctcacagaggatgaagtcagctgctccatccccactggactcaggttcatttcattcatcctgtgatgcatcggcttggggccaaatatcagagaaaggagcgctcgggtggtggggaacaggcatcagggtttgcgttccagggtcacgtgctaccacatcttgctcacaaccgctgcaccgacgcggccactcgtccccggggtcgcccggggccgcccaacttctcccgagggccggtggccgtgcaccccgccacgggttggggcatctcggggaacacctggggccttccgtccagaagcttcgggaagggggctgcccaacctgccagctgcgctgggggcgcacgcgcctgccccactgctttgttcctcatccgggcagagttcgcctcggggccctgcccgtccgctcggccccctcaccccgggggccgctgccctaacgtttcccgtcccgcccggcccttcccggcccgcggcctcctctgggccgcaccctct

SEQ ID NO: 17730 - RNA, 1691 nt, Homo sapiens
  source 1..1691: mol_type = other RNA
tccctcgccttctcaccctcagccaccacaggccttcttccagatccttgaaaaacttcagtgtctgcagctgtctttccttgcttacagctctttctgttctcttcactagctaagacctcacccttcaggtctctggctgtttgactttcccagcataatttaagagccattatgtaacaggcatgccatttcctcagagaggcctttctggacccctgagatgaggctaactcctttgggaacactcaccactcattaactaatcatgagcccaatgtatgcgagggctccccagggtgggccatgtctgtttacaccactgaactgcagacaccaaggcctggcacatggctcacggacaccttcagtgcctatgggctgtatgaatatcctgggttaaagcagcctctcttctggtatctccaatcaggacaaaacctgagtatccccctcactgccaaccaatcatcaagtcctcatgattccacctcatagacaaatctccctatagtgtacccaggctccccatcctcatcaccatgatccacctgagatactgcctacggcctctaaaactgcttcctggcctctggcctcccccttagtcagcctccacaatttggttagaaggctctttttaaagtgcaaatcccatccagctactctcctaattaaccccctcaattgttccctgatgctcttgtgataaacttataaaggccagaacaacctgtccctccctggtcctccctcctgacctctttcccttccaactctcccaacacacacttcagtttttcatttctggaattaaaacacgccaccctgtctcacttggagcctgaagcacactctctcccatttgcccggccagctcctgtcctttagagctcatttatactctcactcagcgaaagcctttcctgacctcctcccacctcaaatctggggcaggtgaccctgctacctgccagtgcatactccaggcacccttcggcactgtcccatcaacacagagctgggagtgtgtccctgtcccacggtctttctaggcctgacttggggagagcacgtaacaggaagagagacctctgagccctggccaccaggctgcaggctgttcgactgttcctttcactgagaatgctactcttgagacccagcaaatgagaaaacgcgcctacagaaataccacaacagtaggctttaggaagctttttcttctggagagaactaggctccatctccacaacccaggccttgggggtaactcggctttttttgcctgtgggttcctgccatcgtgggtctggctttcttggctttttgctatggtatttcccctggaggaatttcacactgtgcaaacagtctttctcttggctattttggtcagctcagctgggccgtaagccaacaaagcagtttctaagcccaggcttttccagttgcctagcctggaagaattcagagctggtgagggaaaagcatgccctggctggttttagagaacaaagttggacctcaaagaaagctcacaaatggggtatgagaatccatttggatgaagaaagcagcaaccttggtagtgaaagactccaaattgtgctgaatatttcaatgagaggcaaacctcagcaatcataataactattataaggtgggcacggtggctcatgcctgtaata

SEQ ID NO: 17731 - RNA, 1696 nt, Homo sapiens
  source 1..1696: mol_type = other RNA
tccctcgccttctcaccctcagccaccacaggccttcttccagatccttgaaaaacttcagtgtctgcagctgtctttccttgcttacagctctttctgttctcttcactagctaagacctcacccttcaggtctctggctgtttgactttcccagcataatttaagagccattatgtaacaggcatgccatttcctcagagaggcctttctggacccctgagatgaggctaactcctttgggaacactcaccactcattaactaatcatgagcccaatgtatgcgagggctccccagggtgggccatgtctgtttacaccactgaactgcagacaccaaggcctggcacatggctcacggacaccttcagtgcctatgggctgtatgaatatcctgggttaaagcagcctctcttctggtatctccaatcaggacaaaacctgagtatccccctcactgccaaccaatcatcaagtcctcatgattccacctcatagacaaatctccctatagtgtacccaggctccccatcctcatcaccatgatccacctgagatactgcctacggcctctaaaactgcttcctggcctctggcctcccccttagtcagcctccacaatttggttagaaggctctttttaaagtgcaaatcccatccagctactctcctaattaaccccctcaattgttccctgatgctcttgtgataaacttataaaggccagaacaacctgtccctccctggtcctccctcctgacctctttcccttccaactctcccaacacacacttcagtttttcatttctggaattaaaacacgccaccctgtctcacttggagcctgaagcacactctctcccatttgcccggccagctcctgtcctttagagctcatttatactctcactcagcgaaagcctttcctgacctcctcccacctcaaatctggggcaggtgaccctgctacctgccagtgcatactccaggcacccttcggcactgtcccatcaacacagagctgggagtgtgtccctgtcccacggtctttctaggcctgacttggggagagcacgtaacaggaagagagacctctgagccctggccaccaggctgcaggctgttcgactgttcctttcactgagaatgctactcttgagacccagcaaatgagaaaacgcgcctacagaaataccacaacagtaggctttaggaagctttttcttctggagagaactaggctccatctccacaacccaggccttgggggtaactcggctttttttgcctgtgggttcctgccatcgtgggtctggctttcttggctttttgctatggtatttcccctggaggaatttcacactgtgcaaacagtctttctcttggctattttggtcagctcagctgggccgtaagccaacaaagcagtttctaagcccaggcttttccagttgcctagcctggaagaattcagagctggtgagggaaaagcatgccctggctggttttagagaacaaagttggacctcaaagaaagctcacaaatggggtatgagaatccatttggatgaagaaagcagcaaccttggtagtgaaagactccaaattgtgctgaatatttcaatgagaggcaaacctcagcaatcataataactattataaggtgggcacggtggctcatgcctgtaataccagc

SEQ ID NO: 17732 - RNA, 42 nt, Homo sapiens
  source 1..42: mol_type = other RNA
tccctcgccttctcaccctcagcgcccgatgccggtagaact

SEQ ID NO: 17733 - RNA, 185 nt, Homo sapiens
  source 1..185: mol_type = other RNA
tccctcgccttctcaccctcagcgcccgatgccggtagaactggtgcgcggctcgcccctcccccaaacttcctgagaactcttcaaagaggggtgagtccaaacccagcttttccagactgctgggttttccagggagtctggggctgcgctgccctgtctccagggcgttattctccagcgct

SEQ ID NO: 17734 - RNA, 158 nt, Homo sapiens
  source 1..158: mol_type = other RNA
tccctcgccttctcaccctcagcgggtttcctaagtcccaacccctgcgtacagatcaaggacttttcactttctcaaggcagcttctctgagaaatgtacaagccacgccgcgaaccgcccgcccggaaagctctggcggctgaggtggtgcctccc

SEQ ID NO: 17735 - RNA, 3004 nt, Homo sapiens
  source 1..3004: mol_type = other RNA
tccctctcccaccccttgcagtggtgccgcctggcagcccagcagacaggctcccacccccatcggcagacctgtcccctccacctgcgccctgcaaaaagccagcccggagctgggcccaggcctgccccctagcctgctcctgatggtgcctggggcggggtgggcaggtgggtggggctggaacctcctttcctgttttcctgagtgatccctccccactggggaagagaagagaaaggaggaagaagaggaggaggaggaagagaaaaacaagaaactgagttggaagagggccctggagcaatcaggacgtcaaaagtttgcattccgactagctataggaaatagtttttttctctttttattatttcaagttttcataaaaatccataattattgaaacccaagttacagagaaagttcgtaacttttttattgaattattgactctgccgcgtgtcggttcgtcggctttcaactccagtctgtcaatgcccctgtgtaggtggggtccccaggtctgggcttctgaggtcctggtagaaggagggcaggtggtgagggctggcggggggcagcaggggacggaggcgggagggagaaagagaacgtgtgtagaagggtagggaggaggtgggaaggactggagagtgagcaggtggcggccaggccccttcccctgcccggccgcccgggggtccctgccccccgccccggcctcatatcatcttcatgttgaacttgcggggcgcgtcggcggagctgatgcctgcgtccgactttcggggcacatactcgatctcgatgttgtgctttgtgttgcccttgccccggctccagagaaacagcagcaccaggcagaagaggacgacgcccaggaaagagatgaagcccatggtggtggcgatgatgagggtcttgatgtcgaaggggaaaggcacagtggcgcgggtgctgttggcctctccctcgcccggctggttggagatgaaagcgaaggtcttgttgggctgatggggccagtcgggcgagtagctgcgcacatgcaggtgggcgggcatggagtcgttgccgcccgcgttggccgcgatgcacaggtacgtgccgttgtcctgtacctgggcgtagcgcacctccagcgtgccatcagggaagactgtgagccgcccattgctcttggctgagaccaggtgctttcggggtgagagccagaggatggcgggcggcgggtcgccatcggcccggcacacaaactgcaccgtgtggccctcgtccacaaacacctgctgggccttgcggtcccggatgcgggcgcggcggcaggtgaagtagttgggcagtagcacatcagggaagtccttgaactccttgccctggacaaactcgggcgtggcgcacgtgggctgctgccggttgaagttgagccgccagcggcgccggaacacccacaggagccgacagtcgcaggccagcgggttggagtccaggatgagtgtctccaggttgcccaccgagtggaagactgattcctccagtgtggtcagctggttgccagagacattgagcacgcgcaggtagttgaggccgcggaaggcatagggctccaccacggccagctgcccgcccaccagctggatctcctgcagccggagcagctcatgcaacatggagccctcaatggtgctgatggggttgtaggagaggttgaggaagcggagatagactaggtggcggacggccaggtagggcacagcggtcagattgcagtgtgtgatggacagggacgtcaggttgaggccgtagaggcagttgggtgtcatggtgtccaagtagggccagtgggagatctccaagaccttgagtcggtacagcctcttgaaggagtagtcccggatggcattgatgttgaggtgccggagcctcaggacgatgaggccgtgcaggtgggacagcgcctcggtggggatggaggtcaggttgcatttctccagcgtcagctgctccaggctgttgaggccgctgaaggcgcggtgagagatgtagacgaggtcattgtcgccaacctccagtgacttgaggttgtacaggtcctgaaacatgtagtccagtaggataacgatcttgttctcgctgatgtccagcttggtcaggttgctgaggccagtgaagacgcctagcgggatgagcttcaggcggttgctgcggagacccagcgtccggaggttgaagaggttgttgaaggcgccgggctccacggcgctcacgatgttctcgttgagctccagctcctccaggtgcgggaagctggcgaactcgtcctggttgagcgttttgatgcggttcttgcctaggtccagcaggcgcgtctcggtggggatgccctcggggactgccacaaagcgcttgcggtggcacagcacagcgcggtcctgggcggagcactcgcagcggggcgggcagcccgtggccgagcctgacagcactgagcccagcaccagcaggaggatgggctgccagcaggccaggagggggctgggcatgctcctcacgccccccgccagcatcctcttgctcaccctgactgctgctgtgtcctgctgggtcccaaagcttgagaagtccccttggcccaggctggggtcaggagtagacttgggagctggtccaggagctggatagagtcagagccctggagatgcaggctgaaggctgtgtagccccacagactcaaggtagccaggtcatggtcataagatcctcaagcatcgtctcagggctcagggctccgggctcaagatcagggcctcctcggtgggacacttcacaaagcctctgcttcctcttctataagaagggtggtggtagctgcctctcagctgctgtgaagatgggaagcacccagccaggcctggcactttcagggcactctgcacactggtcagccccgcaggacctgaggctgagcctctcgtgggacacccgcagacactcagctccaact

SEQ ID NO: 17736 - RNA, 3182 nt, Homo sapiens
  source 1..3182: mol_type = other RNA
tccctctcccaccccttgcagtggtgccgcctggcagcccagcagacaggctcccacccccatcggcagacctgtcccctccacctgcgccctgcaaaaagccagcccggagctgggcccaggcctgccccctagcctgctcctgatggtgcctggggcggggtgggcaggtgggtggggctggaacctcctttcctgttttcctgagtgatccctccccactggggaagagaagagaaaggaggaagaagaggaggaggaggaagagaaaaacaagaaactgagttggaagagggccctggagcaatcaggacgtcaaaagtttgcattccgactagctataggaaatagtttttttctctttttattatttcaagttttcataaaaatccataattattgaaacccaagttacagagaaagttcgtaacttttttattgaattattgactctgccgcgtgtcggttcgtcggctttcaactccagtctgtcaatgcccctgtgtaggtggggtccccaggtctgggcttctgaggtcctggtagaaggagggcaggtggtgagggctggcggggggcagcaggggacggaggcgggagggagaaagagaacgtgtgtagaagggtagggaggaggtgggaaggactggagagtgagcaggtggcggccaggccccttcccctgcccggccgcccgggggtccctgccccccgccccggcctcatatcatcttcatgttgaacttgcggggcgcgtcggcggagctgatgcctgcgtccgactttcggggcacatactcgatctcgatgttgtgctttgtgttgcccttgccccggctccagagaaacagcagcaccaggcagaagaggacgacgcccaggaaagagatgaagcccatggtggtggcgatgatgagggtcttgatgtcgaaggggaaaggcacagtggcgcgggtgctgttggcctctccctcgcccggctggttggagatgaaagcgaaggtcttgttgggctgatggggccagtcgggcgagtagctgcgcacatgcaggtgggcgggcatggagtcgttgccgcccgcgttggccgcgatgcacaggtacgtgccgttgtcctgtacctgggcgtagcgcacctccagcgtgccatcagggaagactgtgagccgcccattgctcttggctgagaccaggtgctttcggggtgagagccagaggatggcgggcggcgggtcgccatcggcccggcacacaaactgcaccgtgtggccctcgtccacaaacacctgctgggccttgcggtcccggatgcgggcgcggcggcaggtgaagtagttgggcagtagcacatcagggaagtccttgaactccttgccctggacaaactcgggcgtggcgcacgtgggctgctgccggttgaagttgagccgccagcggcgccggaacacccacaggagccgacagtcgcaggccagcgggttggagtccaggatgagtgtctccaggttgcccaccgagtggaagactgattcctccagtgtggtcagctggttgccagagacattgagcacgcgcaggtagttgaggccgcggaaggcatagggctccaccacggccagctgcccgcccaccagctggatctcctgcagccggagcagctcatgcaacatggagccctcaatggtgctgatggggttgtaggagaggttgaggaagcggagatagactaggtggcggacggccaggtagggcacagcggtcagattgcagtgtgtgatggacagggacgtcaggttgaggccgtagaggcagttgggtgtcatggtgtccaagtagggccagtgggagatctccaagaccttgagtcggtacagcctcttgaaggagtagtcccggatggcattgatgttgaggtgccggagcctcaggacgatgaggccgtgcaggtgggacagcgcctcggtggggatggaggtcaggttgcatttctccagcgtcagctgctccaggctgttgaggccgctgaaggcgcggtgagagatgtagacgaggtcattgtcgccaacctccagtgacttgaggttgtacaggtcctgaaacatgtagtccagtaggataacgatcttgttctcgctgatgtccagcttggtcaggttgctgaggccagtgaagacgcctagcgggatgagcttcaggcggttgctgcggagacccagcgtccggaggttgaagaggttgttgaaggcgccgggctccacggcgctcacgatgttctcgttgagctccagctcctccaggtgcgggaagctggcgaactcgtcctggttgagcgttttgatgcggttcttgcctaggtccagcaggcgcgtctcggtggggatgccctcggggactgccacaaagcgcttgcggtggcacagcacagcgcggtcctgggcggagcactcgcagcggggcgggcagcccgtggccgagcctgacagcactgagcccagcaccagcaggaggatgggctgccagcaggccaggagggggctgggcatgctcctcacgccccccgccagcatcctcttgctcacctgcatctcgggcgcgccttcggtccgctcggctcggtcaccaatcgcatgtctctccagccggcccgaccaggccccagcccctgcccagccccctcctccgtttcctcctcctccgacacctccgcccggcagtccgcgcgccctcgcggggctggctgtccgtctgtccgccccgcgcgggcgggagccgagccggagccggggccggggctcgggagtggggaggcgggaggccgcggccccggcgggcggatgggcgggcgcgctcaggccgcgggacaggggctgcgcgagcctgcttctgccccctgggccggcccggagccgccgccgccgcctctgccgctggggccggggtcgaggccgggcgcgctccgccgcggggccggggccggcgggcagcggccgcgcatgctgctcggcgccccgcgtcgggagaggggccggagcggcgcgggtggggactccgcgccctccggggccgggaccaggacccaccgccgccgccgccgcctgcgctgtcgcccgccgcccgctccggctcccgcgccggctcccgctcgggctccgcgctctgcagcggcgcggggagggagcact

SEQ ID NO: 17737 - RNA, 2709 nt, Homo sapiens
  source 1..2709: mol_type = other RNA
tccctctcccaccccttgcagtggtgccgcctggcagcccagcagacaggctcccacccccatcggcagacctgtcccctccacctgcgccctgcaaaaagccagcccggagctgggcccaggcctgccccctagcctgctcctgatggtgcctggggcggggtgggcaggtgggtggggctggaacctcctttcctgttttcctgagtgatccctccccactggggaagagaagagaaaggaggaagaagaggaggaggaggaagagaaaaacaagaaactgagttggaagagggccctggagcaatcaggacgtcaaaagtttgcattccgactagctataggaaatagtttttttctctttttattatttcaagttttcataaaaatccataattattgaaacccaagttacagagaaagttcgtaacttttttattgaattattgactctgccgcgtgtcggttcgtcggctttcaactccagtctgtcaatgcccctgtgtaggtggggtccccaggtctgggcttctgaggtcctggtagaaggagggcaggtggtgagggctggcggggggcagcaggggacggaggcgggagggagaaagagaacgtgtgtagaagggtagggaggaggtgggaaggactggagagtgagcaggtggcggccaggccccttcccctgcccggccgcccgggggtccctgccccccgccccggcctcatatcatcttcatgttgaacttgcggggcgcgtcggcggagctgatgcctgcgtccgactttcggggcacatactcgatctcgatgttgtgctttgtgttgcccttgccccggctccagagaaacagcagcaccaggcagaagaggacgacgcccaggaaagagatgaagcccatggtggtggcgatgatgagggtcttgatgtcgaaggggaaaggcacagtggcgcgggtgctgttggcctctccctcgcccggctggttggagatgaaagcgaaggtcttgttgggctgatggggccagtcgggcgagtagctgcgcacatgcaggtgggcgggcatggagtcgttgccgcccgcgttggccgcgatgcacaggtacgtgccgttgtcctgtacctgggcgtagcgcacctccagcgtgccatcagggaagactgtgagccgcccattgctcttggctgagaccaggtgctttcggggtgagagccagaggatggcgggcggcgggtcgccatcggcccggcacacaaactgcaccgtgtggccctcgtccacaaacacctgctgggccttgcggtcccggatgcgggcgcggcggcaggtgaagtagttgggcagtagcacatcagggaagtccttgaactccttgccctggacaaactcgggcgtggcgcacgtgggctgctgccggttgaagttgagccgccagcggcgccggaacacccacaggagccgacagtcgcaggccagcgggttggagtccaggatgagtgtctccaggttgcccaccgagtggaagactgattcctccagtgtggtcagctggttgccagagacattgagcacgcgcaggtagttgaggccgcggaaggcatagggctccaccacggccagctgcccgcccaccagctggatctcctgcagccggagcagctcatgcaacatggagccctcaatggtgctgatggggttgtaggagaggttgaggaagcggagatagactaggtggcggacggccaggtagggcacagcggtcagattgcagtgtgtgatggacagggacgtcaggttgaggccgtagaggcagttgggtgtcatggtgtccaagtagggccagtgggagatctccaagaccttgagtcggtacagcctcttgaaggagtagtcccggatggcattgatgttgaggtgccggagcctcaggacgatgaggccgtgcaggtgggacagcgcctcggtggggatggaggtcaggttgcatttctccagcgtcagctgctccaggctgttgaggccgctgaaggcgcggtgagagatgtagacgaggtcattgtcgccaacctccagtgacttgaggttgtacaggtcctgaaacatgtagtccagtaggataacgatcttgttctcgctgatgtccagcttggtcaggttgctgaggccagtgaagacgcctagcgggatgagcttcaggcggttgctgcggagacccagcgtccggaggttgaagaggttgttgaaggcgccgggctccacggcgctcacgatgttctcgttgagctccagctcctccaggtgcgggaagctggcgaactcgtcctggttgagcgttttgatgcggttcttgcctaggtccagcaggcgcgtctcggtggggatgccctcggggactgccacaaagcgcttgcggtggcacagcacagcgcggtcctgggcggagcactcgcagcggggcgggcagcccgtggccgagcctgacagcactgagcccagcaccagcaggaggatgggctgccagcaggccaggagggggctgggcatgctcctcacgccccccgccagcatcctcttgctcacctgggcctcctgctgtgtcccagttcagcctaaggagctcagccaccctcctgggtgagacttccagggtcagacccttctgactgtggttacagactgagtcttgaccctggcagggtggactggcccc

SEQ ID NO: 17738 - RNA, 2779 nt, Homo sapiens
  source 1..2779: mol_type = other RNA
tccctctcccaccccttgcagtggtgccgcctggcagcccagcagacaggctcccacccccatcggcagacctgtcccctccacctgcgccctgcaaaaagccagcccggagctgggcccaggcctgccccctagcctgctcctgatggtgcctggggcggggtgggcaggtgggtggggctggaacctcctttcctgttttcctgagtgatccctccccactggggaagagaagagaaaggaggaagaagaggaggaggaggaagagaaaaacaagaaactgagttggaagagggccctggagcaatcaggacgtcaaaagtttgcattccgactagctataggaaatagtttttttctctttttattatttcaagttttcataaaaatccataattattgaaacccaagttacagagaaagttcgtaacttttttattgaattattgactctgccgcgtgtcggttcgtcggctttcaactccagtctgtcaatgcccctgtgtaggtggggtccccaggtctgggcttctgaggtcctggtagaaggagggcaggtggtgagggctggcggggggcagcaggggacggaggcgggagggagaaagagaacgtgtgtagaagggtagggaggaggtgggaaggactggagagtgagcaggtggcggccaggccccttcccctgcccggccgcccgggggtccctgccccccgccccggcctcatatcatcttcatgttgaacttgcggggcgcgtcggcggagctgatgcctgcgtccgactttcggggcacatactcgatctcgatgttgtgctttgtgttgcccttgccccggctccagagaaacagcagcaccaggcagaagaggacgacgcccaggaaagagatgaagcccatggtggtggcgatgatgagggtcttgatgtcgaaggggaaaggcacagtggcgcgggtgctgttggcctctccctcgcccggctggttggagatgaaagcgaaggtcttgttgggctgatggggccagtcgggcgagtagctgcgcacatgcaggtgggcgggcatggagtcgttgccgcccgcgttggccgcgatgcacaggtacgtgccgttgtcctgtacctgggcgtagcgcacctccagcgtgccatcagggaagactgtgagccgcccattgctcttggctgagaccaggtgctttcggggtgagagccagaggatggcgggcggcgggtcgccatcggcccggcacacaaactgcaccgtgtggccctcgtccacaaacacctgctgggccttgcggtcccggatgcgggcgcggcggcaggtgaagtagttgggcagtagcacatcagggaagtccttgaactccttgccctggacaaactcgggcgtggcgcacgtgggctgctgccggttgaagttgagccgccagcggcgccggaacacccacaggagccgacagtcgcaggccagcgggttggagtccaggatgagtgtctccaggttgcccaccgagtggaagactgattcctccagtgtggtcagctggttgccagagacattgagcacgcgcaggtagttgaggccgcggaaggcatagggctccaccacggccagctgcccgcccaccagctggatctcctgcagccggagcagctcatgcaacatggagccctcaatggtgctgatggggttgtaggagaggttgaggaagcggagatagactaggtggcggacggccaggtagggcacagcggtcagattgcagtgtgtgatggacagggacgtcaggttgaggccgtagaggcagttgggtgtcatggtgtccaagtagggccagtgggagatctccaagaccttgagtcggtacagcctcttgaaggagtagtcccggatggcattgatgttgaggtgccggagcctcaggacgatgaggccgtgcaggtgggacagcgcctcggtggggatggaggtcaggttgcatttctccagcgtcagctgctccaggctgttgaggccgctgaaggcgcggtgagagatgtagacgaggtcattgtcgccaacctccagtgacttgaggttgtacaggtcctgaaacatgtagtccagtaggataacgatcttgttctcgctgatgtccagcttggtcaggttgctgaggccagtgaagacgcctagcgggatgagcttcaggcggttgctgcggagacccagcgtccggaggttgaagaggttgttgaaggcgccgggctccacggcgctcacgatgttctcgttgagctccagctcctccaggtgcgggaagctggcgaactcgtcctggttgagcgttttgatgcggttcttgcctaggtccagcaggcgcgtctcggtggggatgccctcggggactgccacaaagcgcttgcggtggcacagcacagcgcggtcctgggcggagcactcgcagcggggcgggcagcccgtggccgagcctgacagcactgagcccagcaccagcaggaggatgggctgccagcaggccaggagggggctgggcatgctcctcacgccccccgccagcatcctcttgctcacctgggtcagatggcgttgggaggcaaacagactggcctctgggggcctggggtgcggcagcctgtccgtcgcggtcccagcatgcacatgactcttgaagcacaaatgatcccaaccattctgcagatgagaaaacagctcagaatggccacatggcttgcccaaggtggcaccgccagcaagagatggagcttaaaatc

SEQ ID NO: 17739 - RNA, 2982 nt, Homo sapiens
  source 1..2982: mol_type = other RNA
tccctctcccaccccttgcagtggtgccgcctggcagcccagcagacaggctcccacccccatcggcagacctgtcccctccacctgcgccctgcaaaaagccagcccggagctgggcccaggcctgccccctagcctgctcctgatggtgcctggggcggggtgggcaggtgggtggggctggaacctcctttcctgttttcctgagtgatccctccccactggggaagagaagagaaaggaggaagaagaggaggaggaggaagagaaaaacaagaaactgagttggaagagggccctggagcaatcaggacgtcaaaagtttgcattccgactagctataggaaatagtttttttctctttttattatttcaagttttcataaaaatccataattattgaaacccaagttacagagaaagttcgtaacttttttattgaattattgactctgccgcgtgtcggttcgtcggctttcaactccagtctgtcaatgcccctgtgtaggtggggtccccaggtctgggcttctgaggtcctggtagaaggagggcaggtggtgagggctggcggggggcagcaggggacggaggcgggagggagaaagagaacgtgtgtagaagggtagggaggaggtgggaaggactggagagtgagcaggtggcggccaggccccttcccctgcccggccgcccgggggtccctgccccccgccccggcctcatatcatcttcatgttgaacttgcggggcgcgtcggcggagctgatgcctgcgtccgactttcggggcacatactcgatctcgatgttgtgctttgtgttgcccttgccccggctccagagaaacagcagcaccaggcagaagaggacgacgcccaggaaagagatgaagcccatggtggtggcgatgatgagggtcttgatgtcgaaggggaaaggcacagtggcgcgggtgctgttggcctctccctcgcccggctggttggagatgaaagcgaaggtcttgttgggctgatggggccagtcgggcgagtagctgcgcacatgcaggtgggcgggcatggagtcgttgccgcccgcgttggccgcgatgcacaggtacgtgccgttgtcctgtacctgggcgtagcgcacctccagcgtgccatcagggaagactgtgagccgcccattgctcttggctgagaccaggtgctttcggggtgagagccagaggatggcgggcggcgggtcgccatcggcccggcacacaaactgcaccgtgtggccctcgtccacaaacacctgctgggccttgcggtcccggatgcgggcgcggcggcaggtgaagtagttgggcagtagcacatcagggaagtccttgaactccttgccctggacaaactcgggcgtggcgcacgtgggctgctgccggttgaagttgagccgccagcggcgccggaacacccacaggagccgacagtcgcaggccagcgggttggagtccaggatgagtgtctccaggttgcccaccgagtggaagactgattcctccagtgtggtcagctggttgccagagacattgagcacgcgcaggtagttgaggccgcggaaggcatagggctccaccacggccagctgcccgcccaccagctggatctcctgcagccggagcagctcatgcaacatggagccctcaatggtgctgatggggttgtaggagaggttgaggaagcggagatagactaggtggcggacggccaggtagggcacagcggtcagattgcagtgtgtgatggacagggacgtcaggttgaggccgtagaggcagttgggtgtcatggtgtccaagtagggccagtgggagatctccaagaccttgagtcggtacagcctcttgaaggagtagtcccggatggcattgatgttgaggtgccggagcctcaggacgatgaggccgtgcaggtgggacagcgcctcggtggggatggaggtcaggttgcatttctccagcgtcagctgctccaggctgttgaggccgctgaaggcgcggtgagagatgtagacgaggtcattgtcgccaacctccagtgacttgaggttgtacaggtcctgaaacatgtagtccagtaggataacgatcttgttctcgctgatgtccagcttggtcaggttgctgaggccagtgaagacgcctagcgggatgagcttcaggcggttgctgcggagacccagcgtccggaggttgaagaggttgttgaaggcgccgggctccacggcgctcacgatgttctcgttgagctccagctcctccaggtgcgggaagctggcgaactcgtcctggttgagcgttttgatgcggttcttgcctaggtccagcaggcgcgtctcggtggggatgccctcggggactgccacaaagcgcttgcggtggcacagcacagcgcggtcctgggcggagcactcgcagcggggcgggcagcccgtggccgagcctgacagcactgagcccagcaccagcaggaggatgggctgccagcaggccaggagggggctgggcatgctcctcacgccccccgccagcatcctcttgctcacctgggtcagatggcgttgggaggcaaacagactggcctctgggggcctggggtgcggcagcctgtccgtcgcggtcccagcatgcacctgactgctgctgtgtcctgctgggtcccaaagcttgagaagtccccttggcccaggctggggtcaggagtagacttgggagctggtccaggagctggatagagtcagagccctggagatgcaggctgaaggctgtgtagccccacagactcaaggtagccaggtcatggtcataagatcccccatagatacttttcagactaaagatgtaagctgtcacaatcagtcataattaagtcaagcaagctatttttttttttcttgagctcccttcccctctcgggcacccgctcctccttgggttagatctcagagt

SEQ ID NO: 17740 - RNA, 3025 nt, Homo sapiens
  source 1..3025: mol_type = other RNA
tccctctcccaccccttgcagtggtgccgcctggcagcccagcagacaggctcccacccccatcggcagacctgtcccctccacctgcgccctgcaaaaagccagcccggagctgggcccaggcctgccccctagcctgctcctgatggtgcctggggcggggtgggcaggtgggtggggctggaacctcctttcctgttttcctgagtgatccctccccactggggaagagaagagaaaggaggaagaagaggaggaggaggaagagaaaaacaagaaactgagttggaagagggccctggagcaatcaggacgtcaaaagtttgcattccgactagctataggaaatagtttttttctctttttattatttcaagttttcataaaaatccataattattgaaacccaagttacagagaaagttcgtaacttttttattgaattattgactctgccgcgtgtcggttcgtcggctttcaactccagtctgtcaatgcccctgtgtaggtggggtccccaggtctgggcttctgaggtcctggtagaaggagggcaggtggtgagggctggcggggggcagcaggggacggaggcgggagggagaaagagaacgtgtgtagaagggtagggaggaggtgggaaggactggagagtgagcaggtggcggccaggccccttcccctgcccggccgcccgggggtccctgccccccgccccggcctcatatcatcttcatgttgaacttgcggggcgcgtcggcggagctgatgcctgcgtccgactttcggggcacatactcgatctcgatgttgtgctttgtgttgcccttgccccggctccagagaaacagcagcaccaggcagaagaggacgacgcccaggaaagagatgaagcccatggtggtggcgatgatgagggtcttgatgtcgaaggggaaaggcacagtggcgcgggtgctgttggcctctccctcgcccggctggttggagatgaaagcgaaggtcttgttgggctgatggggccagtcgggcgagtagctgcgcacatgcaggtgggcgggcatggagtcgttgccgcccgcgttggccgcgatgcacaggtacgtgccgttgtcctgtacctgggcgtagcgcacctccagcgtgccatcagggaagactgtgagccgcccattgctcttggctgagaccaggtgctttcggggtgagagccagaggatggcgggcggcgggtcgccatcggcccggcacacaaactgcaccgtgtggccctcgtccacaaacacctgctgggccttgcggtcccggatgcgggcgcggcggcaggtgaagtagttgggcagtagcacatcagggaagtccttgaactccttgccctggacaaactcgggcgtggcgcacgtgggctgctgccggttgaagttgagccgccagcggcgccggaacacccacaggagccgacagtcgcaggccagcgggttggagtccaggatgagtgtctccaggttgcccaccgagtggaagactgattcctccagtgtggtcagctggttgccagagacattgagcacgcgcaggtagttgaggccgcggaaggcatagggctccaccacggccagctgcccgcccaccagctggatctcctgcagccggagcagctcatgcaacatggagccctcaatggtgctgatggggttgtaggagaggttgaggaagcggagatagactaggtggcggacggccaggtagggcacagcggtcagattgcagtgtgtgatggacagggacgtcaggttgaggccgtagaggcagttgggtgtcatggtgtccaagtagggccagtgggagatctccaagaccttgagtcggtacagcctcttgaaggagtagtcccggatggcattgatgttgaggtgccggagcctcaggacgatgaggccgtgcaggtgggacagcgcctcggtggggatggaggtcaggttgcatttctccagcgtcagctgctccaggctgttgaggccgctgaaggcgcggtgagagatgtagacgaggtcattgtcgccaacctccagtgacttgaggttgtacaggtcctgaaacatgtagtccagtaggataacgatcttgttctcgctgatgtccagcttggtcaggttgctgaggccagtgaagacgcctagcgggatgagcttcaggcggttgctgcggagacccagcgtccggaggttgaagaggttgttgaaggcgccgggctccacggcgctcacgatgttctcgttgagctccagctcctccaggtgcgggaagctggcgaactcgtcctggttgagcgttttgatgcggttcttgcctaggtccagcaggcgcgtctcggtggggatgccctcggggactgccacaaagcgcttgcggtggcacagcacagcgcggtcctgggcggagcactcgcagcggggcgggcagcccgtggccgagcctgacagcactgagcccagcaccagcaggaggatgggctgccagcaggccaggagggggctgggcatgctcctcacgccccccgccagcatcctcttgctcacctgggtcagatggcgttgggaggcaaacagactggcctctgggggcctggggtgcggcagcctgtccgtcgcggtcccagcatgcacctgactgctgctgtgtcctgctgggtcccaaagcttgagaagtccccttggcccaggctggggtcaggagtagacttgggagctggtccaggagctggatagagtcagagccctggagatgcaggctgaaggctgtgtagccccacagactcaaggtagccaggtcatggtcataagatcccccatcattgcagtcaaggtcacaggcaccggcacagggcgggctgggcaaggagcctttaatctgggagttcaggctgaggaaactacacgcttgaagccggagtacattactgccctgaatgatctgtcggcttctattaggctaaatatctctgtataatggggaattatcctct

SEQ ID NO: 17741 - RNA, 3425 nt, Homo sapiens
  source 1..3425: mol_type = other RNA
tccctctcccaccccttgcagtggtgccgcctggcagcccagcagacaggctcccacccccatcggcagacctgtcccctccacctgcgccctgcaaaaagccagcccggagctgggcccaggcctgccccctagcctgctcctgatggtgcctggggcggggtgggcaggtgggtggggctggaacctcctttcctgttttcctgagtgatccctccccactggggaagagaagagaaaggaggaagaagaggaggaggaggaagagaaaaacaagaaactgagttggaagagggccctggagcaatcaggacgtcaaaagtttgcattccgactagctataggaaatagtttttttctctttttattatttcaagttttcataaaaatccataattattgaaacccaagttacagagaaagttcgtaacttttttattgaattattgactctgccgcgtgtcggttcgtcggctttcaactccagtctgtcaatgcccctgtgtaggtggggtccccaggtctgggcttctgaggtcctggtagaaggagggcaggtggtgagggctggcggggggcagcaggggacggaggcgggagggagaaagagaacgtgtgtagaagggtagggaggaggtgggaaggactggagagtgagcaggtggcggccaggccccttcccctgcccggccgcccgggggtccctgccccccgccccggcctcatatcatcttcatgttgaacttgcggggcgcgtcggcggagctgatgcctgcgtccgactttcggggcacatactcgatctcgatgttgtgctttgtgttgcccttgccccggctccagagaaacagcagcaccaggcagaagaggacgacgcccaggaaagagatgaagcccatggtggtggcgatgatgagggtcttgatgtcgaaggggaaaggcacagtggcgcgggtgctgttggcctctccctcgcccggctggttggagatgaaagcgaaggtcttgttgggctgatggggccagtcgggcgagtagctgcgcacatgcaggtgggcgggcatggagtcgttgccgcccgcgttggccgcgatgcacaggtacgtgccgttgtcctgtacctgggcgtagcgcacctccagcgtgccatcagggaagactgtgagccgcccattgctcttggctgagaccaggtgctttcggggtgagagccagaggatggcgggcggcgggtcgccatcggcccggcacacaaactgcaccgtgtggccctcgtccacaaacacctgctgggccttgcggtcccggatgcgggcgcggcggcaggtgaagtagttgggcagtagcacatcagggaagtccttgaactccttgccctggacaaactcgggcgtggcgcacgtgggctgctgccggttgaagttgagccgccagcggcgccggaacacccacaggagccgacagtcgcaggccagcgggttggagtccaggatgagtgtctccaggttgcccaccgagtggaagactgattcctccagtgtggtcagctggttgccagagacattgagcacgcgcaggtagttgaggccgcggaaggcatagggctccaccacggccagctgcccgcccaccagctggatctcctgcagccggagcagctcatgcaacatggagccctcaatggtgctgatggggttgtaggagaggttgaggaagcggagatagactaggtggcggacggccaggtagggcacagcggtcagattgcagtgtgtgatggacagggacgtcaggttgaggccgtagaggcagttgggtgtcatggtgtccaagtagggccagtgggagatctccaagaccttgagtcggtacagcctcttgaaggagtagtcccggatggcattgatgttgaggtgccggagcctcaggacgatgaggccgtgcaggtgggacagcgcctcggtggggatggaggtcaggttgcatttctccagcgtcagctgctccaggctgttgaggccgctgaaggcgcggtgagagatgtagacgaggtcattgtcgccaacctccagtgacttgaggttgtacaggtcctgaaacatgtagtccagtaggataacgatcttgttctcgctgatgtccagcttggtcaggttgctgaggccagtgaagacgcctagcgggatgagcttcaggcggttgctgcggagacccagcgtccggaggttgaagaggttgttgaaggcgccgggctccacggcgctcacgatgttctcgttgagctccagctcctccaggtgcgggaagctggcgaactcgtcctggttgagcgttttgatgcggttcttgcctaggtccagcaggcgcgtctcggtggggatgccctcggggactgccacaaagcgcttgcggtggcacagcacagcgcggtcctgggcggagcactcgcagcggggcgggcagcccgtggccgagcctgacagcactgagcccagcaccagcaggaggatgggctgccagcaggccaggagggggctgggcatgctcctcacgccccccgccagcatcctcttgctcacctgggtcagatggcgttgggaggcaaacagactggcctctgggggcctggggtgcggcagcctgtccgtcgcggtcccagcatgcacctgactgctgctgtgtcctgctgggtcccaaagcttgagaagtccccttggcccaggctggggtcaggagtagacttgggagctggtccaggagctggatagagtcagagccctggagatgcaggctgaaggctgtgtagccccacagactcaaggtagccaggtcatggtcataagatccctccaccttggccttagtattctccaaatatcctttctgcctgtccccaacaggtgcccagggccaccctcctctccattcatctcaggacaagtgctgggaccacttcctccaggaaggtgtccctggctgctctgaagggggctgggctcctctccactggcacgctgtgcacatcaggtgtttgaggctggtacggctctggtgtctcacggtcagtcaagcatcgtctcagggctcagggctccgggctcaagatcagggcctcctcggtgggacacctcgggttgggtgggtgtctggggagtacagctgggcagggctcagcctgggctggactcagtcgccctctctgcctgtgggcactggagcctcagggcctgtgggtgccggaggcgtcccgggcgcgccgtccgcgcgcggctccgctccgggccggcatcccccggctcggctgcctccggtccccgctccggcctcggttcccgctccgcagggctcggctccgcgatggtggccgcggcggcgagcgcggcagggagggcgtgtgtatgcgcgtgagagcgcgcagcgtgtgc

SEQ ID NO: 17742 - RNA, 3144 nt, Homo sapiens
  source 1..3144: mol_type = other RNA
tccctctcccaccccttgcagtggtgccgcctggcagcccagcagacaggctcccacccccatcggcagacctgtcccctccacctgcgccctgcaaaaagccagcccggagctgggcccaggcctgccccctagcctgctcctgatggtgcctggggcggggtgggcaggtgggtggggctggaacctcctttcctgttttcctgagtgatccctccccactggggaagagaagagaaaggaggaagaagaggaggaggaggaagagaaaaacaagaaactgagttggaagagggccctggagcaatcaggacgtcaaaagtttgcattccgactagctataggaaatagtttttttctctttttattatttcaagttttcataaaaatccataattattgaaacccaagttacagagaaagttcgtaacttttttattgaattattgactctgccgcgtgtcggttcgtcggctttcaactccagtctgtcaatgcccctgtgtaggtggggtccccaggtctgggcttctgaggtcctggtagaaggagggcaggtggtgagggctggcggggggcagcaggggacggaggcgggagggagaaagagaacgtgtgtagaagggtagggaggaggtgggaaggactggagagtgagcaggtggcggccaggccccttcccctgcccggccgcccgggggtccctgccccccgccccggcctcatatcatcttcatgttgaacttgcggggcgcgtcggcggagctgatgcctgcgtccgactttcggggcacatactcgatctcgatgttgtgctttgtgttgcccttgccccggctccagagaaacagcagcaccaggcagaagaggacgacgcccaggaaagagatgaagcccatggtggtggcgatgatgagggtcttgatgtcgaaggggaaaggcacagtggcgcgggtgctgttggcctctccctcgcccggctggttggagatgaaagcgaaggtcttgttgggctgatggggccagtcgggcgagtagctgcgcacatgcaggtgggcgggcatggagtcgttgccgcccgcgttggccgcgatgcacaggtacgtgccgttgtcctgtacctgggcgtagcgcacctccagcgtgccatcagggaagactgtgagccgcccattgctcttggctgagaccaggtgctttcggggtgagagccagaggatggcgggcggcgggtcgccatcggcccggcacacaaactgcaccgtgtggccctcgtccacaaacacctgctgggccttgcggtcccggatgcgggcgcggcggcaggtgaagtagttgggcagtagcacatcagggaagtccttgaactccttgccctggacaaactcgggcgtggcgcacgtgggctgctgccggttgaagttgagccgccagcggcgccggaacacccacaggagccgacagtcgcaggccagcgggttggagtccaggatgagtgtctccaggttgcccaccgagtggaagactgattcctccagtgtggtcagctggttgccagagacattgagcacgcgcaggtagttgaggccgcggaaggcatagggctccaccacggccagctgcccgcccaccagctggatctcctgcagccggagcagctcatgcaacatggagccctcaatggtgctgatggggttgtaggagaggttgaggaagcggagatagactaggtggcggacggccaggtagggcacagcggtcagattgcagtgtgtgatggacagggacgtcaggttgaggccgtagaggcagttgggtgtcatggtgtccaagtagggccagtgggagatctccaagaccttgagtcggtacagcctcttgaaggagtagtcccggatggcattgatgttgaggtgccggagcctcaggacgatgaggccgtgcaggtgggacagcgcctcggtggggatggaggtcaggttgcatttctccagcgtcagctgctccaggctgttgaggccgctgaaggcgcggtgagagatgtagacgaggtcattgtcgccaacctccagtgacttgaggttgtacaggtcctgaaacatgtagtccagtaggataacgatcttgttctcgctgatgtccagcttggtcaggttgctgaggccagtgaagacgcctagcgggatgagcttcaggcggttgctgcggagacccagcgtccggaggttgaagaggttgttgaaggcgccgggctccacggcgctcacgatgttctcgttgagctccagctcctccaggtgcgggaagctggcgaactcgtcctggttgagcgttttgatgcggttcttgcctaggtccagcaggcgcgtctcggtggggatgccctcggggactgccacaaagcgcttgcggtggcacagcacagcgcggtcctgggcggagcactcgcagcggggcgggcagcccgtggccgagcctgacagcactgagcccagcaccagcaggaggatgggctgccagcaggccaggagggggctgggcatgctcctcacgccccccgccagcatcctcttgctcacctgggtcagatggcgttgggaggcaaacagactggcctctgggggcctggggtgcggcagcctgtccgtcgcggtcccagcatgcacctgactgctgctgtgtcctgctgggtcccaaagcttgagaagtccccttggcccaggctggggtcaggagtagacttgggagctggtccaggagctggatagagtcagagccctggagatgcaggctgaaggctgtgtagccccacagactcaaggtagccaggtcatggtcataagatccctcgggttgggtgggtgtctggggagtacagctgggcagggctcagcctgggctggactcagtcgccctctctgcctgtgggcactggagcctcagggcctgtgggtgccggaggcgtcccgggcgcgccgtccgcgcgcggctccgctccgggccggcatcccccggctcggctgcctccggtccccgctccggcctcggttcccgctccgcagggctcggctccgcgatggtggccgcggcggcgagcgcggcagggagggcgtgtgtatgcgcgtgagagcgcgcagcgtgtgc

SEQ ID NO: 17743 - RNA, 2952 nt, Homo sapiens
  source 1..2952: mol_type = other RNA
tccctctcccaccccttgcagtggtgccgcctggcagcccagcagacaggctcccacccccatcggcagacctgtcccctccacctgcgccctgcaaaaagccagcccggagctgggcccaggcctgccccctagcctgctcctgatggtgcctggggcggggtgggcaggtgggtggggctggaacctcctttcctgttttcctgagtgatccctccccactggggaagagaagagaaaggaggaagaagaggaggaggaggaagagaaaaacaagaaactgagttggaagagggccctggagcaatcaggacgtcaaaagtttgcattccgactagctataggaaatagtttttttctctttttattatttcaagttttcataaaaatccataattattgaaacccaagttacagagaaagttcgtaacttttttattgaattattgactctgccgcgtgtcggttcgtcggctttcaactccagtctgtcaatgcccctgtgtaggtggggtccccaggtctgggcttctgaggtcctggtagaaggagggcaggtggtgagggctggcggggggcagcaggggacggaggcgggagggagaaagagaacgtgtgtagaagggtagggaggaggtgggaaggactggagagtgagcaggtggcggccaggccccttcccctgcccggccgcccgggggtccctgccccccgccccggcctcatatcatcttcatgttgaacttgcggggcgcgtcggcggagctgatgcctgcgtccgactttcggggcacatactcgatctcgatgttgtgctttgtgttgcccttgccccggctccagagaaacagcagcaccaggcagaagaggacgacgcccaggaaagagatgaagcccatggtggtggcgatgatgagggtcttgatgtcgaaggggaaaggcacagtggcgcgggtgctgttggcctctccctcgcccggctggttggagatgaaagcgaaggtcttgttgggctgatggggccagtcgggcgagtagctgcgcacatgcaggtgggcgggcatggagtcgttgccgcccgcgttggccgcgatgcacaggtacgtgccgttgtcctgtacctgggcgtagcgcacctccagcgtgccatcagggaagactgtgagccgcccattgctcttggctgagaccaggtgctttcggggtgagagccagaggatggcgggcggcgggtcgccatcggcccggcacacaaactgcaccgtgtggccctcgtccacaaacacctgctgggccttgcggtcccggatgcgggcgcggcggcaggtgaagtagttgggcagtagcacatcagggaagtccttgaactccttgccctggacaaactcgggcgtggcgcacgtgggctgctgccggttgaagttgagccgccagcggcgccggaacacccacaggagccgacagtcgcaggccagcgggttggagtccaggatgagtgtctccaggttgcccaccgagtggaagactgattcctccagtgtggtcagctggttgccagagacattgagcacgcgcaggtagttgaggccgcggaaggcatagggctccaccacggccagctgcccgcccaccagctggatctcctgcagccggagcagctcatgcaacatggagccctcaatggtgctgatggggttgtaggagaggttgaggaagcggagatagactaggtggcggacggccaggtagggcacagcggtcagattgcagtgtgtgatggacagggacgtcaggttgaggccgtagaggcagttgggtgtcatggtgtccaagtagggccagtgggagatctccaagaccttgagtcggtacagcctcttgaaggagtagtcccggatggcattgatgttgaggtgccggagcctcaggacgatgaggccgtgcaggtgggacagcgcctcggtggggatggaggtcaggttgcatttctccagcgtcagctgctccaggctgttgaggccgctgaaggcgcggtgagagatgtagacgaggtcattgtcgccaacctccagtgacttgaggttgtacaggtcctgaaacatgtagtccagtaggataacgatcttgttctcgctgatgtccagcttggtcaggttgctgaggccagtgaagacgcctagcgggatgagcttcaggcggttgctgcggagacccagcgtccggaggttgaagaggttgttgaaggcgccgggctccacggcgctcacgatgttctcgttgagctccagctcctccaggtgcgggaagctggcgaactcgtcctggttgagcgttttgatgcggttcttgcctaggtccagcaggcgcgtctcggtggggatgccctcggggactgccacaaagcgcttgcggtggcacagcacagcgcggtcctgggcggagcactcgcagcggggcgggcagcccgtggccgagcctgacagcactgagcccagcaccagcaggaggatgggctgccagcaggccaggagggggctgggcatgctcctcacgccccccgccagcatcctcttgctcacctgggtcagatggcgttgggaggcaaacagactggcctctgggggcctggggtgcggcagcctgtccgtcgcggtcccagcatgcacctgactgctgctgtgtcctgctgggtcccaaagcttgagaagtccccttggcccaggctggggtcaggagtagacttgggagctggtccaggagctggatagagtcagagccctggagatgcaggctgaaggctgtgtagccccacagactcaaggtagccaggtcatggtcataagatccctgggtggaggcctgacaaggccactggtcagccaggtgaccccgggcaagtccctgagcctcttggaatctccgtcttcctgtctcttagatggagctaataat

SEQ ID NO: 17744 - RNA, 3192 nt, Homo sapiens
  source 1..3192: mol_type = other RNA
tccctctcccaccccttgcagtggtgccgcctggcagcccagcagacaggctcccacccccatcggcagacctgtcccctccacctgcgccctgcaaaaagccagcccggagctgggcccaggcctgccccctagcctgctcctgatggtgcctggggcggggtgggcaggtgggtggggctggaacctcctttcctgttttcctgagtgatccctccccactggggaagagaagagaaaggaggaagaagaggaggaggaggaagagaaaaacaagaaactgagttggaagagggccctggagcaatcaggacgtcaaaagtttgcattccgactagctataggaaatagtttttttctctttttattatttcaagttttcataaaaatccataattattgaaacccaagttacagagaaagttcgtaacttttttattgaattattgactctgccgcgtgtcggttcgtcggctttcaactccagtctgtcaatgcccctgtgtaggtggggtccccaggtctgggcttctgaggtcctggtagaaggagggcaggtggtgagggctggcggggggcagcaggggacggaggcgggagggagaaagagaacgtgtgtagaagggtagggaggaggtgggaaggactggagagtgagcaggtggcggccaggccccttcccctgcccggccgcccgggggtccctgccccccgccccggcctcatatcatcttcatgttgaacttgcggggcgcgtcggcggagctgatgcctgcgtccgactttcggggcacatactcgatctcgatgttgtgctttgtgttgcccttgccccggctccagagaaacagcagcaccaggcagaagaggacgacgcccaggaaagagatgaagcccatggtggtggcgatgatgagggtcttgatgtcgaaggggaaaggcacagtggcgcgggtgctgttggcctctccctcgcccggctggttggagatgaaagcgaaggtcttgttgggctgatggggccagtcgggcgagtagctgcgcacatgcaggtgggcgggcatggagtcgttgccgcccgcgttggccgcgatgcacaggtacgtgccgttgtcctgtacctgggcgtagcgcacctccagcgtgccatcagggaagactgtgagccgcccattgctcttggctgagaccaggtgctttcggggtgagagccagaggatggcgggcggcgggtcgccatcggcccggcacacaaactgcaccgtgtggccctcgtccacaaacacctgctgggccttgcggtcccggatgcgggcgcggcggcaggtgaagtagttgggcagtagcacatcagggaagtccttgaactccttgccctggacaaactcgggcgtggcgcacgtgggctgctgccggttgaagttgagccgccagcggcgccggaacacccacaggagccgacagtcgcaggccagcgggttggagtccaggatgagtgtctccaggttgcccaccgagtggaagactgattcctccagtgtggtcagctggttgccagagacattgagcacgcgcaggtagttgaggccgcggaaggcatagggctccaccacggccagctgcccgcccaccagctggatctcctgcagccggagcagctcatgcaacatggagccctcaatggtgctgatggggttgtaggagaggttgaggaagcggagatagactaggtggcggacggccaggtagggcacagcggtcagattgcagtgtgtgatggacagggacgtcaggttgaggccgtagaggcagttgggtgtcatggtgtccaagtagggccagtgggagatctccaagaccttgagtcggtacagcctcttgaaggagtagtcccggatggcattgatgttgaggtgccggagcctcaggacgatgaggccgtgcaggtgggacagcgcctcggtggggatggaggtcaggttgcatttctccagcgtcagctgctccaggctgttgaggccgctgaaggcgcggtgagagatgtagacgaggtcattgtcgccaacctccagtgacttgaggttgtacaggtcctgaaacatgtagtccagtaggataacgatcttgttctcgctgatgtccagcttggtcaggttgctgaggccagtgaagacgcctagcgggatgagcttcaggcggttgctgcggagacccagcgtccggaggttgaagaggttgttgaaggcgccgggctccacggcgctcacgatgttctcgttgagctccagctcctccaggtgcgggaagctggcgaactcgtcctggttgagcgttttgatgcggttcttgcctaggtccagcaggcgcgtctcggtggggatgccctcggggactgccacaaagcgcttgcggtggcacagcacagcgcggtcctgggcggagcactcgcagcggggcgggcagcccgtggccgagcctgacagcactgagcccagcaccagcaggaggatgggctgccagcaggccaggagggggctgggcatgctcctcacgccccccgccagcatcctcttgctcacctgggtcagatggcgttgggaggcaaacagactggcctctgggggcctggggtgcggcagcctgtccgtcgcggtcccagcatgcacctgactgctgctgtgtcctgctgggtcccaaagcttgagaagtccccttggcccaggctggggtcaggagtagacttgggagctggtccaggagctggatagagtcagagccctggagatgcaggctgaaggctgtgtagccccacagactcaaggtagccaggtcatggtcataagatcctcaagcatcgtctcagggctcagggctccgggctcaagatcagggcctcctcggtgggacacctcgggttgggtgggtgtctggggagtacagctgggcagggctcagcctgggctggactcagtcgccctctctgcctgtgggcactggagcctcagggcctgtgggtgccggaggattctccgcattacagcgggtgccgcccgccgctcgcggggcccagggttcgagcgcgcagtgggcggcgaggggacccgccacgcccggccccgccgccccctccgctctccgcggctccgcggctgctagctccggcctggcgctagggtggcgacgtcccgcgct

SEQ ID NO: 17745 - RNA, 3082 nt, Homo sapiens
  source 1..3082: mol_type = other RNA
tccctctcccaccccttgcagtggtgccgcctggcagcccagcagacaggctcccacccccatcggcagacctgtcccctccacctgcgccctgcaaaaagccagcccggagctgggcccaggcctgccccctagcctgctcctgatggtgcctggggcggggtgggcaggtgggtggggctggaacctcctttcctgttttcctgagtgatccctccccactggggaagagaagagaaaggaggaagaagaggaggaggaggaagagaaaaacaagaaactgagttggaagagggccctggagcaatcaggacgtcaaaagtttgcattccgactagctataggaaatagtttttttctctttttattatttcaagttttcataaaaatccataattattgaaacccaagttacagagaaagttcgtaacttttttattgaattattgactctgccgcgtgtcggttcgtcggctttcaactccagtctgtcaatgcccctgtgtaggtggggtccccaggtctgggcttctgaggtcctggtagaaggagggcaggtggtgagggctggcggggggcagcaggggacggaggcgggagggagaaagagaacgtgtgtagaagggtagggaggaggtgggaaggactggagagtgagcaggtggcggccaggccccttcccctgcccggccgcccgggggtccctgccccccgccccggcctcatatcatcttcatgttgaacttgcggggcgcgtcggcggagctgatgcctgcgtccgactttcggggcacatactcgatctcgatgttgtgctttgtgttgcccttgccccggctccagagaaacagcagcaccaggcagaagaggacgacgcccaggaaagagatgaagcccatggtggtggcgatgatgagggtcttgatgtcgaaggggaaaggcacagtggcgcgggtgctgttggcctctccctcgcccggctggttggagatgaaagcgaaggtcttgttgggctgatggggccagtcgggcgagtagctgcgcacatgcaggtgggcgggcatggagtcgttgccgcccgcgttggccgcgatgcacaggtacgtgccgttgtcctgtacctgggcgtagcgcacctccagcgtgccatcagggaagactgtgagccgcccattgctcttggctgagaccaggtgctttcggggtgagagccagaggatggcgggcggcgggtcgccatcggcccggcacacaaactgcaccgtgtggccctcgtccacaaacacctgctgggccttgcggtcccggatgcgggcgcggcggcaggtgaagtagttgggcagtagcacatcagggaagtccttgaactccttgccctggacaaactcgggcgtggcgcacgtgggctgctgccggttgaagttgagccgccagcggcgccggaacacccacaggagccgacagtcgcaggccagcgggttggagtccaggatgagtgtctccaggttgcccaccgagtggaagactgattcctccagtgtggtcagctggttgccagagacattgagcacgcgcaggtagttgaggccgcggaaggcatagggctccaccacggccagctgcccgcccaccagctggatctcctgcagccggagcagctcatgcaacatggagccctcaatggtgctgatggggttgtaggagaggttgaggaagcggagatagactaggtggcggacggccaggtagggcacagcggtcagattgcagtgtgtgatggacagggacgtcaggttgaggccgtagaggcagttgggtgtcatggtgtccaagtagggccagtgggagatctccaagaccttgagtcggtacagcctcttgaaggagtagtcccggatggcattgatgttgaggtgccggagcctcaggacgatgaggccgtgcaggtgggacagcgcctcggtggggatggaggtcaggttgcatttctccagcgtcagctgctccaggctgttgaggccgctgaaggcgcggtgagagatgtagacgaggtcattgtcgccaacctccagtgacttgaggttgtacaggtcctgaaacatgtagtccagtaggataacgatcttgttctcgctgatgtccagcttggtcaggttgctgaggccagtgaagacgcctagcgggatgagcttcaggcggttgctgcggagacccagcgtccggaggttgaagaggttgttgaaggcgccgggctccacggcgctcacgatgttctcgttgagctccagctcctccaggtgcgggaagctggcgaactcgtcctggttgagcgttttgatgcggttcttgcctaggtccagcaggcgcgtctcggtggggatgccctcggggactgccacaaagcgcttgcggtggcacagcacagcgcggtcctgggcggagcactcgcagcggggcgggcagcccgtggccgagcctgacagcactgagcccagcaccagcaggaggatgggctgccagcaggccaggagggggctgggcatgctcctcacgccccccgccagcatcctcttgctcacctgggtcagatggcgttgggaggcaaacagactggcctctgggggcctggggtgcggcagcctgtccgtcgcggtcccagcatgcacctgactgctgctgtgtcctgctgggtcccaaagcttgagaagtccccttggcccaggctggggtcaggagtagacttgggagctggtccaggagctggatagagtcagagccctggagatgcaggctgaaggctgtgtagccccacagactcaaggtagccaggtcatggtcataagatcctcaagcatcgtctcagggctcagggctccgggctcaagatcagggcctcctcggtgggacacctcgggttgggtgggtgtctggggagtacagctgggcagggctcagcctgggctggactcagtcgccctctctgcctgtgggcactggagcctcagggcctgtgggtgccggaggcaggactggtctgcctcctccttccaactgcctcatcagggaaaccagggaacgaggt

SEQ ID NO: 17746 - RNA, 3099 nt, Homo sapiens
  source 1..3099: mol_type = other RNA
tccctctcccaccccttgcagtggtgccgcctggcagcccagcagacaggctcccacccccatcggcagacctgtcccctccacctgcgccctgcaaaaagccagcccggagctgggcccaggcctgccccctagcctgctcctgatggtgcctggggcggggtgggcaggtgggtggggctggaacctcctttcctgttttcctgagtgatccctccccactggggaagagaagagaaaggaggaagaagaggaggaggaggaagagaaaaacaagaaactgagttggaagagggccctggagcaatcaggacgtcaaaagtttgcattccgactagctataggaaatagtttttttctctttttattatttcaagttttcataaaaatccataattattgaaacccaagttacagagaaagttcgtaacttttttattgaattattgactctgccgcgtgtcggttcgtcggctttcaactccagtctgtcaatgcccctgtgtaggtggggtccccaggtctgggcttctgaggtcctggtagaaggagggcaggtggtgagggctggcggggggcagcaggggacggaggcgggagggagaaagagaacgtgtgtagaagggtagggaggaggtgggaaggactggagagtgagcaggtggcggccaggccccttcccctgcccggccgcccgggggtccctgccccccgccccggcctcatatcatcttcatgttgaacttgcggggcgcgtcggcggagctgatgcctgcgtccgactttcggggcacatactcgatctcgatgttgtgctttgtgttgcccttgccccggctccagagaaacagcagcaccaggcagaagaggacgacgcccaggaaagagatgaagcccatggtggtggcgatgatgagggtcttgatgtcgaaggggaaaggcacagtggcgcgggtgctgttggcctctccctcgcccggctggttggagatgaaagcgaaggtcttgttgggctgatggggccagtcgggcgagtagctgcgcacatgcaggtgggcgggcatggagtcgttgccgcccgcgttggccgcgatgcacaggtacgtgccgttgtcctgtacctgggcgtagcgcacctccagcgtgccatcagggaagactgtgagccgcccattgctcttggctgagaccaggtgctttcggggtgagagccagaggatggcgggcggcgggtcgccatcggcccggcacacaaactgcaccgtgtggccctcgtccacaaacacctgctgggccttgcggtcccggatgcgggcgcggcggcaggtgaagtagttgggcagtagcacatcagggaagtccttgaactccttgccctggacaaactcgggcgtggcgcacgtgggctgctgccggttgaagttgagccgccagcggcgccggaacacccacaggagccgacagtcgcaggccagcgggttggagtccaggatgagtgtctccaggttgcccaccgagtggaagactgattcctccagtgtggtcagctggttgccagagacattgagcacgcgcaggtagttgaggccgcggaaggcatagggctccaccacggccagctgcccgcccaccagctggatctcctgcagccggagcagctcatgcaacatggagccctcaatggtgctgatggggttgtaggagaggttgaggaagcggagatagactaggtggcggacggccaggtagggcacagcggtcagattgcagtgtgtgatggacagggacgtcaggttgaggccgtagaggcagttgggtgtcatggtgtccaagtagggccagtgggagatctccaagaccttgagtcggtacagcctcttgaaggagtagtcccggatggcattgatgttgaggtgccggagcctcaggacgatgaggccgtgcaggtgggacagcgcctcggtggggatggaggtcaggttgcatttctccagcgtcagctgctccaggctgttgaggccgctgaaggcgcggtgagagatgtagacgaggtcattgtcgccaacctccagtgacttgaggttgtacaggtcctgaaacatgtagtccagtaggataacgatcttgttctcgctgatgtccagcttggtcaggttgctgaggccagtgaagacgcctagcgggatgagcttcaggcggttgctgcggagacccagcgtccggaggttgaagaggttgttgaaggcgccgggctccacggcgctcacgatgttctcgttgagctccagctcctccaggtgcgggaagctggcgaactcgtcctggttgagcgttttgatgcggttcttgcctaggtccagcaggcgcgtctcggtggggatgccctcggggactgccacaaagcgcttgcggtggcacagcacagcgcggtcctgggcggagcactcgcagcggggcgggcagcccgtggccgagcctgacagcactgagcccagcaccagcaggaggatgggctgccagcaggccaggagggggctgggcatgctcctcacgccccccgccagcatcctcttgctcacctgggtcagatggcgttgggaggcaaacagactggcctctgggggcctggggtgcggcagcctgtccgtcgcggtcccagcatgcacctgactgctgctgtgtcctgctgggtcccaaagcttgagaagtccccttggcccaggctggggtcaggagtagacttgggagctggtccaggagctggatagagtcagagccctggagatgcaggctgaaggctgtgtagccccacagactcaaggtagccaggtcatggtcataagatcctcaagcatcgtctcagggctcagggctccgggctcaagatcagggcctcctcggtgggacacctcgggttgggtgggtgtctggggagtacagctgggcagggctcagcctgggctggactcagtcgccctctctgcctgtgggcactggagcctcagggcctgtgggtgccggaggccggctcgaccggccccacccgggggccccggggaagggacctcgctgcgcgggaacagtccggggcggtggcac

SEQ ID NO: 17747 - RNA, 3206 nt, Homo sapiens
  source 1..3206: mol_type = other RNA
tccctctcccaccccttgcagtggtgccgcctggcagcccagcagacaggctcccacccccatcggcagacctgtcccctccacctgcgccctgcaaaaagccagcccggagctgggcccaggcctgccccctagcctgctcctgatggtgcctggggcggggtgggcaggtgggtggggctggaacctcctttcctgttttcctgagtgatccctccccactggggaagagaagagaaaggaggaagaagaggaggaggaggaagagaaaaacaagaaactgagttggaagagggccctggagcaatcaggacgtcaaaagtttgcattccgactagctataggaaatagtttttttctctttttattatttcaagttttcataaaaatccataattattgaaacccaagttacagagaaagttcgtaacttttttattgaattattgactctgccgcgtgtcggttcgtcggctttcaactccagtctgtcaatgcccctgtgtaggtggggtccccaggtctgggcttctgaggtcctggtagaaggagggcaggtggtgagggctggcggggggcagcaggggacggaggcgggagggagaaagagaacgtgtgtagaagggtagggaggaggtgggaaggactggagagtgagcaggtggcggccaggccccttcccctgcccggccgcccgggggtccctgccccccgccccggcctcatatcatcttcatgttgaacttgcggggcgcgtcggcggagctgatgcctgcgtccgactttcggggcacatactcgatctcgatgttgtgctttgtgttgcccttgccccggctccagagaaacagcagcaccaggcagaagaggacgacgcccaggaaagagatgaagcccatggtggtggcgatgatgagggtcttgatgtcgaaggggaaaggcacagtggcgcgggtgctgttggcctctccctcgcccggctggttggagatgaaagcgaaggtcttgttgggctgatggggccagtcgggcgagtagctgcgcacatgcaggtgggcgggcatggagtcgttgccgcccgcgttggccgcgatgcacaggtacgtgccgttgtcctgtacctgggcgtagcgcacctccagcgtgccatcagggaagactgtgagccgcccattgctcttggctgagaccaggtgctttcggggtgagagccagaggatggcgggcggcgggtcgccatcggcccggcacacaaactgcaccgtgtggccctcgtccacaaacacctgctgggccttgcggtcccggatgcgggcgcggcggcaggtgaagtagttgggcagtagcacatcagggaagtccttgaactccttgccctggacaaactcgggcgtggcgcacgtgggctgctgccggttgaagttgagccgccagcggcgccggaacacccacaggagccgacagtcgcaggccagcgggttggagtccaggatgagtgtctccaggttgcccaccgagtggaagactgattcctccagtgtggtcagctggttgccagagacattgagcacgcgcaggtagttgaggccgcggaaggcatagggctccaccacggccagctgcccgcccaccagctggatctcctgcagccggagcagctcatgcaacatggagccctcaatggtgctgatggggttgtaggagaggttgaggaagcggagatagactaggtggcggacggccaggtagggcacagcggtcagattgcagtgtgtgatggacagggacgtcaggttgaggccgtagaggcagttgggtgtcatggtgtccaagtagggccagtgggagatctccaagaccttgagtcggtacagcctcttgaaggagtagtcccggatggcattgatgttgaggtgccggagcctcaggacgatgaggccgtgcaggtgggacagcgcctcggtggggatggaggtcaggttgcatttctccagcgtcagctgctccaggctgttgaggccgctgaaggcgcggtgagagatgtagacgaggtcattgtcgccaacctccagtgacttgaggttgtacaggtcctgaaacatgtagtccagtaggataacgatcttgttctcgctgatgtccagcttggtcaggttgctgaggccagtgaagacgcctagcgggatgagcttcaggcggttgctgcggagacccagcgtccggaggttgaagaggttgttgaaggcgccgggctccacggcgctcacgatgttctcgttgagctccagctcctccaggtgcgggaagctggcgaactcgtcctggttgagcgttttgatgcggttcttgcctaggtccagcaggcgcgtctcggtggggatgccctcggggactgccacaaagcgcttgcggtggcacagcacagcgcggtcctgggcggagcactcgcagcggggcgggcagcccgtggccgagcctgacagcactgagcccagcaccagcaggaggatgggctgccagcaggccaggagggggctgggcatgctcctcacgccccccgccagcatcctcttgctcacctgggtcagatggcgttgggaggcaaacagactggcctctgggggcctggggtgcggcagcctgtccgtcgcggtcccagcatgcacctgactgctgctgtgtcctgctgggtcccaaagcttgagaagtccccttggcccaggctggggtcaggagtagacttgggagctggtccaggagctggatagagtcagagccctggagatgcaggctgaaggctgtgtagccccacagactcaaggtagccaggtcatggtcataagatcctcaagcatcgtctcagggctcagggctccgggctcaagatcagggcctcctcggtgggacacctcgggttgggtgggtgtctggggagtacagctgggcagggctcagcctgggctggactcagtcgccctctctgcctgtgggcactggagcctcagggcctgtgggtgccggaggcgtcccgggcgcgccgtccgcgcgcggctccgctccgggccggcatcccccggctcggctgcctccggtccccgctccggcctcggttcccgctccgcagggctcggctccgcgatggtggccgcggcggcgagcgcggcagggagggcgtgtgtatgcgcgtgagagcgcgcagcgtgtgc

SEQ ID NO: 17748 - RNA, 3051 nt, Homo sapiens
  source 1..3051: mol_type = other RNA
tccctctcccaccccttgcagtggtgccgcctggcagcccagcagacaggctcccacccccatcggcagacctgtcccctccacctgcgccctgcaaaaagccagcccggagctgggcccaggcctgccccctagcctgctcctgatggtgcctggggcggggtgggcaggtgggtggggctggaacctcctttcctgttttcctgagtgatccctccccactggggaagagaagagaaaggaggaagaagaggaggaggaggaagagaaaaacaagaaactgagttggaagagggccctggagcaatcaggacgtcaaaagtttgcattccgactagctataggaaatagtttttttctctttttattatttcaagttttcataaaaatccataattattgaaacccaagttacagagaaagttcgtaacttttttattgaattattgactctgccgcgtgtcggttcgtcggctttcaactccagtctgtcaatgcccctgtgtaggtggggtccccaggtctgggcttctgaggtcctggtagaaggagggcaggtggtgagggctggcggggggcagcaggggacggaggcgggagggagaaagagaacgtgtgtagaagggtagggaggaggtgggaaggactggagagtgagcaggtggcggccaggccccttcccctgcccggccgcccgggggtccctgccccccgccccggcctcatatcatcttcatgttgaacttgcggggcgcgtcggcggagctgatgcctgcgtccgactttcggggcacatactcgatctcgatgttgtgctttgtgttgcccttgccccggctccagagaaacagcagcaccaggcagaagaggacgacgcccaggaaagagatgaagcccatggtggtggcgatgatgagggtcttgatgtcgaaggggaaaggcacagtggcgcgggtgctgttggcctctccctcgcccggctggttggagatgaaagcgaaggtcttgttgggctgatggggccagtcgggcgagtagctgcgcacatgcaggtgggcgggcatggagtcgttgccgcccgcgttggccgcgatgcacaggtacgtgccgttgtcctgtacctgggcgtagcgcacctccagcgtgccatcagggaagactgtgagccgcccattgctcttggctgagaccaggtgctttcggggtgagagccagaggatggcgggcggcgggtcgccatcggcccggcacacaaactgcaccgtgtggccctcgtccacaaacacctgctgggccttgcggtcccggatgcgggcgcggcggcaggtgaagtagttgggcagtagcacatcagggaagtccttgaactccttgccctggacaaactcgggcgtggcgcacgtgggctgctgccggttgaagttgagccgccagcggcgccggaacacccacaggagccgacagtcgcaggccagcgggttggagtccaggatgagtgtctccaggttgcccaccgagtggaagactgattcctccagtgtggtcagctggttgccagagacattgagcacgcgcaggtagttgaggccgcggaaggcatagggctccaccacggccagctgcccgcccaccagctggatctcctgcagccggagcagctcatgcaacatggagccctcaatggtgctgatggggttgtaggagaggttgaggaagcggagatagactaggtggcggacggccaggtagggcacagcggtcagattgcagtgtgtgatggacagggacgtcaggttgaggccgtagaggcagttgggtgtcatggtgtccaagtagggccagtgggagatctccaagaccttgagtcggtacagcctcttgaaggagtagtcccggatggcattgatgttgaggtgccggagcctcaggacgatgaggccgtgcaggtgggacagcgcctcggtggggatggaggtcaggttgcatttctccagcgtcagctgctccaggctgttgaggccgctgaaggcgcggtgagagatgtagacgaggtcattgtcgccaacctccagtgacttgaggttgtacaggtcctgaaacatgtagtccagtaggataacgatcttgttctcgctgatgtccagcttggtcaggttgctgaggccagtgaagacgcctagcgggatgagcttcaggcggttgctgcggagacccagcgtccggaggttgaagaggttgttgaaggcgccgggctccacggcgctcacgatgttctcgttgagctccagctcctccaggtgcgggaagctggcgaactcgtcctggttgagcgttttgatgcggttcttgcctaggtccagcaggcgcgtctcggtggggatgccctcggggactgccacaaagcgcttgcggtggcacagcacagcgcggtcctgggcggagcactcgcagcggggcgggcagcccgtggccgagcctgacagcactgagcccagcaccagcaggaggatgggctgccagcaggccaggagggggctgggcatgctcctcacgccccccgccagcatcctcttgctcacctgggtcagatggcgttgggaggcaaacagactggcctctgggggcctggggtgcggcagcctgtccgtcgcggtcccagcatgcacctgactgctgctgtgtcctgctgggtcccaaagcttgagaagtccccttggcccaggctggggtcaggagtagacttgggagctggtccaggagctggatagagtcagagccctggagatgcaggctgaaggctgtgtagccccacagactcaaggtagccaggtcatggtcataagatcctcaagcatcgtctcagggctcagggctccgggctcaagatcagggcctcctcggtgggacacttcacaaagcctctgcttcctcttctataagaagggtggtggtagctgcctctcagctgctgtgaagatgggaagcacccagccaggcctggcactttcagggcactctgcacactggtcagccccgcaggacctgaggctg

SEQ ID NO: 17749 - RNA, 2962 nt, Homo sapiens
  source 1..2962: mol_type = other RNA
tccctctcccaccccttgcagtggtgccgcctggcagcccagcagacaggctcccacccccatcggcagacctgtcccctccacctgcgccctgcaaaaagccagcccggagctgggcccaggcctgccccctagcctgctcctgatggtgcctggggcggggtgggcaggtgggtggggctggaacctcctttcctgttttcctgagtgatccctccccactggggaagagaagagaaaggaggaagaagaggaggaggaggaagagaaaaacaagaaactgagttggaagagggccctggagcaatcaggacgtcaaaagtttgcattccgactagctataggaaatagtttttttctctttttattatttcaagttttcataaaaatccataattattgaaacccaagttacagagaaagttcgtaacttttttattgaattattgactctgccgcgtgtcggttcgtcggctttcaactccagtctgtcaatgcccctgtgtaggtggggtccccaggtctgggcttctgaggtcctggtagaaggagggcaggtggtgagggctggcggggggcagcaggggacggaggcgggagggagaaagagaacgtgtgtagaagggtagggaggaggtgggaaggactggagagtgagcaggtggcggccaggccccttcccctgcccggccgcccgggggtccctgccccccgccccggcctcatatcatcttcatgttgaacttgcggggcgcgtcggcggagctgatgcctgcgtccgactttcggggcacatactcgatctcgatgttgtgctttgtgttgcccttgccccggctccagagaaacagcagcaccaggcagaagaggacgacgcccaggaaagagatgaagcccatggtggtggcgatgatgagggtcttgatgtcgaaggggaaaggcacagtggcgcgggtgctgttggcctctccctcgcccggctggttggagatgaaagcgaaggtcttgttgggctgatggggccagtcgggcgagtagctgcgcacatgcaggtgggcgggcatggagtcgttgccgcccgcgttggccgcgatgcacaggtacgtgccgttgtcctgtacctgggcgtagcgcacctccagcgtgccatcagggaagactgtgagccgcccattgctcttggctgagaccaggtgctttcggggtgagagccagaggatggcgggcggcgggtcgccatcggcccggcacacaaactgcaccgtgtggccctcgtccacaaacacctgctgggccttgcggtcccggatgcgggcgcggcggcaggtgaagtagttgggcagtagcacatcagggaagtccttgaactccttgccctggacaaactcgggcgtggcgcacgtgggctgctgccggttgaagttgagccgccagcggcgccggaacacccacaggagccgacagtcgcaggccagcgggttggagtccaggatgagtgtctccaggttgcccaccgagtggaagactgattcctccagtgtggtcagctggttgccagagacattgagcacgcgcaggtagttgaggccgcggaaggcatagggctccaccacggccagctgcccgcccaccagctggatctcctgcagccggagcagctcatgcaacatggagccctcaatggtgctgatggggttgtaggagaggttgaggaagcggagatagactaggtggcggacggccaggtagggcacagcggtcagattgcagtgtgtgatggacagggacgtcaggttgaggccgtagaggcagttgggtgtcatggtgtccaagtagggccagtgggagatctccaagaccttgagtcggtacagcctcttgaaggagtagtcccggatggcattgatgttgaggtgccggagcctcaggacgatgaggccgtgcaggtgggacagcgcctcggtggggatggaggtcaggttgcatttctccagcgtcagctgctccaggctgttgaggccgctgaaggcgcggtgagagatgtagacgaggtcattgtcgccaacctccagtgacttgaggttgtacaggtcctgaaacatgtagtccagtaggataacgatcttgttctcgctgatgtccagcttggtcaggttgctgaggccagtgaagacgcctagcgggatgagcttcaggcggttgctgcggagacccagcgtccggaggttgaagaggttgttgaaggcgccgggctccacggcgctcacgatgttctcgttgagctccagctcctccaggtgcgggaagctggcgaactcgtcctggttgagcgttttgatgcggttcttgcctaggtccagcaggcgcgtctcggtggggatgccctcggggactgccacaaagcgcttgcggtggcacagcacagcgcggtcctgggcggagcactcgcagcggggcgggcagcccgtggccgagcctgacagcactgagcccagcaccagcaggaggatgggctgccagcaggccaggagggggctgggcatgctcctcacgccccccgccagcatcctcttgctcacctgggtcagatggcgttgggaggcaaacagactggcctctgggggcctggggtgcggcagcctgtccgtcgcggtcccagcatgcactcgggttgggtgggtgtctggggagtacagctgggcagggctcagcctgggctggactcagtcgccctctctgcctgtgggcactggagcctcagggcctgtgggtgccggaggcgtcccgggcgcgccgtccgcgcgcggctccgctccgggccggcatcccccggctcggctgcctccggtccccgctccggcctcggttcccgctccgcagggctcggctccgcgatggtggccgcggcggcgagcgcggcagggagggcgtgtgtatgcgcgtgagagcgcgcagcgtgtgc

SEQ ID NO: 17750 - RNA, 189 nt, Homo sapiens
  source 1..189: mol_type = other RNA
tccctgagaccctttaacctgtgaggacatccagggtcacaggtgaggttcttgggagcctggcgtctggcccaaccacacacctggggaattgctggcctgacttctgacccctgactcctcatacccttcctccagagcatgacatttgaccaccaactgaaacctgacctctgaccccagaccact

SEQ ID NO: 17751 - RNA, 2023 nt, Homo sapiens
  source 1..2023: mol_type = other RNA
tccctgagcaaagccacgcccgtgcacgggaagtgcagcaccaccaacctgcagccggagccaaagatctgggcatccacgtctgatcctttgccctccctccctctcgggtcctgccagagccttcgggtggcagaacctgataaggaccagaccaccgaggggacccctccgatgctgcaccaggagaccagccctgcagggcacagagctcagcaggaagagggaagcccagacctggcaggagaagagaggatttggacacagatgagtggcaagtgcacacacacatcacagaagaaaacacgcgtttgctacagtcagtttctgctgcaagttcccagcttagagctggtttttgacttcttactcttttaccagctatgcctcctttatcgtaatccagcggcttggctggcaattgttacctgctaagtgggactaaacctctcctcttgagccctgggaggtgctgcctgaatggagttgttcattgctttccaatctggagttgacaatgctgccaagtattccagaaaatcatctgggatgacaaatgcttcttcctgcctgcagtgtggtggaacgatctcattttcagcaccccattaatcaactgacccccagaaccccgcaaccagtgggattgtgtaaatttcccacacagcacagaacacattgtagagctgagatccaatcacacacaggaagatagaaatggcacatctgggagcccttgctacattgttcgactttccaacaaccagcttttgatattaatacctacaaaatagtggaactgataaattattagcattgaattactgtacaatattatccttcttttcttgacagcagcaaagttggtcaaaaagagaatattgggcatgtgatcagtcaatatggttactgttagaatgcttccaattaataaaacataattctctacacccactggctctgcactcctttgaatagtttatttcagaaccaacagaggggatggtgtgagtgaatataaaataattaggtttagagtaatgtaacaaatcattatttaaatgttctgagatttgtagtctaaagtaactaacagtcaacagaaagacaacatccaaaattgtatagactgctactatgccattcacaagggggaaatgatagccactgtgttcatgtaatttgtttcattttttttgaattgtagtaagtcaagaaatgtacatcatctagatatcagtttaatgacacaaatttcagctcagaagctagaatgcaagtccgcaaggacagtcctgactgcatatttctgaagttaatttacactaggtgctgattctatttttccttcaattttgattggcttgtctgcaagtacttgtgacttttttcctacttgatgctgaacatgattctatttcccaagaacctttgtgccgtcagtccagtgtgatgagtcgccaacaggtttgaatttggcgtccatggtgagataagccacgagtgcagtgcaaagctgtgtctgtctttgcttgtcctcttgtatttccccttggcccgtttatttacgtaattttaaaagtttgtttcctgtctcttcaatcgttgtggagcaggaagaagacttcataagtaagactagaataaaatcaggtcatccacgtgaataattcccatgattttctatctgcattcttactcacaagctccactttgatgcaactgtttgcatcaagatctagaaaaaggcatacgttttcatttaaatgaaaaatatctcaaagaactaagaatgaccaaagatgcttcctcatacctaattccaaaatttactgtgctccatcagaagctattctgtgagtttatgtgtggctgcgaacacaaactcttccctttcatcctcacaatcccatttcttcaagataccactcgtagcaaatacacatacatacacacacaaacacacatgcacacatatacacgcgaatgcacacacacaacatacacacagagagagacacaa

SEQ ID NO: 17752 - RNA, 3640 nt, Homo sapiens
  source 1..3640: mol_type = other RNA
tccctgagcaaagccacgcccgtgcacgggaagtgcagcaccaccaacctgcagccggagccaaagatctgggcatccacgtctgatcctttgccctccctccctctcgggtcctgccagagccttcgggtggcagaacctgataaggaccagaccaccgaggggacccctccgatgctgcaccaggagaccagccctgcagggcacagagctcagcaggaagagggaagcccagacctggcaggagaagagaggatttggacacagatgagtggcaagtgcacacacacatcacagaagaaaacacgcgtttgctacagtcagtttctgctgcaagttcccagcttagagctggtttttgacttcttactcttttaccagctatgcctcctttatcgtaatccagcggcttggctggcaattgttacctgctaagtgggactaaacctctcctcttgagccctgggaggtgctgcctgaatggagttgttcattgctttccaatctggagttgacaatgctgccaagtattccagaaaatcatctgggatgacaaatgcttcttcctgcctgcagtgtggtggaacgatctcattttcagcaccccattaatcaactgacccccagaaccccgcaaccagtgggattgtgtaaatttcccacacagcacagaacacattgtagagctgagatccaatcacacacaggaagatagaaatggcacatctgggagcccttgctacattgttcgactttccaacaaccagcttttgatattaatacctacaaaatagtggaactgataaattattagcattgaattactgtacaatattatccttcttttcttgacagcagcaaagttggtcaaaaagagaatattgggcatgtgatcagtcaatatggttactgttagaatgcttccaattaataaaacataattctctacacccactggctctgcactcctttgaatagtttatttcagaaccaacagaggggatggtgtgagtgaatataaaataattaggtttagagtaatgtaacaaatcattatttaaatgttctgagatttgtagtctaaagtaactaacagtcaacagaaagacaacatccaaaattgtatagactggtactatgccattcacaagggggaaatgatagccactgtgttcatgtaatttgtttcattttttttgaattgtagtaagtcaagaaatgtacatcatctagatatcagtttaatgacacaaatttcagctcagaagctagaatgcaagtccgcaaggacagtcctgactgcatatttctgaagttaatttacactaggtgctgattctatttttccttcaattttgattggcttgtctgcaagtacttgtgacttttttcctacttgatgctgaacatgattctatttcccaagaacctttgtgccgtcagtccagtgtgatgagtcgccaacaggtttgaatttggcgtccatggtgagataagccacgagtgcagtgcaaagctgtgtctgtctttgcttgtcctcttgtatttccccttggcccgtttatttacgtaattttaaaagtttgtttcctgtctcttcaatcgttgtggagcaggaagaagacttcataagtaagactagaataaaatcaggtcatccacgtgaataattcccatgattttctatctgcattcttactcacaagctccactttgatgcaactgtttgcatcaagatctagaaaaaggcatacgttttcatttaaatgaaaaatatctcaaagaactaagaatgaccaaagatgcttcctcatacctaattccaaaatttactgtgctccatcagaagctattctgtgagtttatgtgtggctgcgaacacaaactcttccctttcatcctcacaatcccatttcttcaagataccactcgtagcaaatacacatacatacacacacaaacacacatgcacacatatacacgcgaatgcacacacacaacatacacacagagagagacacaaacacatgcacacacatacatgtacatacgtacacaaacacacatgcacacatatacacatgcacacatggacagcatcatgcacatcctttgtttagcccccacaaaactacaaagcaacggcccacctgcacacacacaacatgcacacagacacaaacacatgtgcgcacatatgtacatatgtacacaaatatacatgcacatgtatatactcatgcacacacagacacacatgcacacacatagacataaacacatgtacatatgtacacatatacatacatacctgcatatatacacatgcacatgtacacacatgtacatatgtacacacatacacacctgcacattgcataacatgtacacataaatatagcatgcacatggacacacatacatgtacctatgtacacaatgcacatgcactcatataaacacacatgcatacgcacatacacatgcacagagacacacctataaatatgcacacacatacacacattcccatgcatacacacatgcatatacaaatgcacacactagcacacactcatacatatacacacatacacatgcacgcacacacacgcatatcacctacacagtgcacacacacacatataaacacatatgtatgcacacactcacacactccacccaggaggacgcagaaatttctactccccatagtattagagaatgtaagagccaggcctaaggaactggaaatggaaaataaccgtgaagatctcgtgaaaacatcctccagtcaccaaggacagcagagccttcacagctccctcattaagcgcctgcctgatggcaatttttatagaggtatattaaactgtttacgattaaaatggatctttgaagtaattaatagtttgccctggtaatttcatcacattttgctgccggatggcaattatgatttaattatgatctcctgatgaagaacatattagataattcttcagataatttcccttttattcctgattagggagcaaggttaggagagatacagggttatggctttgctgtaatctaattttccgactttgaaaatagaaggttttccgggctttaaagtttgctaagaggagacagaaatggcgacagacgtcacatctgaacagtgtcctctgtcctttagaacaacgacaggtcccgaggactctcggcactgcaggaaactggatggctgctctttcattaacgtggagactcagaaaatgcaacagatggggacgcaacagatacttctccctggatttccttccctgagatatgaggggttcagaaatacagaagaaaaacctgcagtaatgaaaacagcagggcaattcccaccgcggccggaggtctccgggtaggaatgcaggcgggcatggaggggaactgactccacgcgcacctgccactcacaggtgaagctcacagacggtcatgggaggtaggggagcctttccagttcccagtcagactcagctccctgaatgcagggccccgctttacaccccgactgtgactcagaattcctggtgctctgagacaagctatgagtagcttgtcattaaatacctgaggagttgaatgcatgataataaat

SEQ ID NO: 17753 - RNA, 1279 nt, Homo sapiens
  source 1..1279: mol_type = other RNA
tccctgtcctccaggagctcacggtagcgctcatactcctcatccgtgaggcccgggacgtcgccccctcccagccccgccccctcggccagcagagagtccatgctgaaatggaagtcccggctctgcagggcgtccccttgcaggccaaacttgcgcaggcttcccggggtgttggtggagctcgggggttcgtcccccagcaggtcgtgctcagagctctcttcgttccgggtgctctcgtcagtccggcccaccccgctgtccagctcctggctgttgctcaggcctgggccggcatcgggagcccccttctcctcttcgtttccgggctgctgggcagggggtgatttcagtttacgagcacgcagctccccctcattctcagagccaaagtcatccaggaagtcatcccggtcgctgtccttccaccttttcgccagctgactctcaggtcgggccaccagcagggagatgttggtgttctcttcctggctcaggatggccaccgcctcttcccggttctggacgtctacaccgttaatctggatgatgcggtctccctcacggatccggccgtctttggctgcaatgctgttgggatttacctctccgacataaatgcccaggtcctcctcgtcgtccgtgcggtagcaaaccatcaggcccagcttgtcccggtggctgcttttatacagctccacctcctcatactccagctcatccaagcggtctgcctcctgcgggccgccctccataaactccgccgggtcataatactcatggctgattggggggagctcagagaggacgtacggctccaggatgaccatgggcggggtgggcggacgcagcttgcccagcgccatgatatgctcgaaggtgatgtcggtctgagtgccactgtccaccagctgcaggtcgtgacaggagctgtccccccggaggcgggggctgcgtctcagcacctggatcaccaggggctccttggaggagcgcagggcctgcagagtttgctcctgagacagcttggagagctccttcccgttcacccgagacgcctaaggcccgggagcccatcgttcgggcagggccaggcgggagtgggtgtcggggtgggcacccagcccccggacggacttggaccgcgcccggggacgcccacgcactcccacgctccaggcccgccgggatctagattcggcgccccccgcacggcgggagcctggctccctcccccgccctgggtcctgcggggagagcgtgtgcggggaactgc

SEQ ID NO: 17754 - RNA, 1358 nt, Homo sapiens
  source 1..1358: mol_type = other RNA
tccctgtcctccaggagctcacggtagcgctcatactcctcatccgtgaggcccgggacgtcgccccctcccagccccgccccctcggccagcagagagtccatgctgaaatggaagtcccggctctgcagggcgtccccttgcaggccaaacttgcgcaggcttcccggggtgttggtggagctcgggggttcgtcccccagcaggtcgtgctcagagctctcttcgttccgggtgctctcgtcagtccggcccaccccgctgtccagctcctggctgttgctcaggcctgggccggcatcgggagcccccttctcctcttcgtttccgggctgctgggcagggggtgatttcagtttacgagcacgcagctccccctcattctcagagccaaagtcatccaggaagtcatcccggtcgctgtccttccaccttttcgccagctgactctcaggtcgggccaccagcagggagatgttggtgttctcttcctggctcaggatggccaccgcctcttcccggttctggacgtctacaccgttaatctggatgatgcggtctccctcacggatccggccgtctttggctgcaatgctgttgggatttacctctccgacataaatgcccaggtcctcctcgtcgtccgtgcggtagcaaaccatcaggcccagcttgtcccggtggctgcttttatacagctccacctcctcatactccagctcatccaagcggtctgcctcctgcgggccgccctccataaactccgccgggtcataatactcatggctgattggggggagctcagagaggacgtacggctccaggatgaccatgggcggggtgggcggacgcagcttgcccagcgccatgatatgctcgaaggtgatgtcggtctgagtgccactgtccaccagctgcaggtcgtgacaggagctgtccccccggaggcgggggctgcgtctcagcacctggatcaccaggggctccttggaggagcgcagggcctgcagagtttgctcctgagacagcttggagagctccttcccgttcacctgcagcatcactttgtactgctcctccggtttctggaccacgcacatattacatcccatgttgctggccggcgagaggaggcggagggcgggaacgggaagacgcctttcactgacccgggcgcgggacctcgggtcccgggccggggccaggggccataccctggcgcggggggcgggccgcctagcgggggaggggggcacgcccccgaggtgggggcagcggctcgcccctcaggttaactcttcgctggccgaggccaggcgcgggcatgctccctcgcacccggccaggagaaaaagggc

SEQ ID NO: 17755 - RNA, 1601 nt, Homo sapiens
  source 1..1601: mol_type = other RNA
tccctgtcctccaggagctcacggtagcgctcatactcctcatccgtgaggcccgggacgtcgccccctcccagccccgccccctcggccagcagagagtccatgctgaaatggaagtcccggctctgcagggcgtccccttgcaggccaaacttgcgcaggcttcccggggtgttggtggagctcgggggttcgtcccccagcaggtcgtgctcagagctctcttcgttccgggtgctctcgtcagtccggcccaccccgctgtccagctcctggctgttgctcaggcctgggccggcatcgggagcccccttctcctcttcgtttccgggctgctgggcagggggtgatttcagtttacgagcacgcagctccccctcattctcagagccaaagtcatccaggaagtcatcccggtcgctgtccttccaccttttcgccagctgactctcaggtcgggccaccagcagggagatgttggtgttctcttcctggctcaggatggccaccgcctcttcccggttctggacgtctacaccgttaatctggatgatgcggtctccctcacggatccggccgtctttggctgcaatgctgttgggatttacctctccgacataaatgcccaggtcctcctcgtcgtccgtgcggtagcaaaccatcaggcccagcttgtcccggtggctgcttttatacagctccacctcctcatactccagctcatccaagcggtctgcctcctgcgggccgccctccataaactccgccgggtcataatactcatggctgattgggggggcggtcatgagccaccaggcctggatgaaaggcccttcttccggtcgggccaaagaaagaagctgaagagatggaggaaattcagagcaggtagaggaatgagacagacaagggatgcaagaagattcaaggagtgatgcttgtgaggcggcagaggagagaggatggaggaggaggagctgaggccctcaaccctggcacttccggcagcgacgtcccggacaggagggtcctccctcggccagctcagagaggacgtacggctccaggatgaccatgggcggggtgggcggacgcagcttgcccagcgccatgatatgctcgaaggtgatgtcggtctgagtgccactgtccaccagctgcaggtcgtgacaggagctgtccccccggaggcgggggctgcgtctcagcacctggatcaccaggggctccttggaggagcgcagggcctgcagagtttgctcctgagacagcttggagagctccttcccgttcacctgcagcatcactttgtactgctcctccggtttctggaccacgcacatattacatcccatgttgctggccggcgagaggaggcggagggcgggaacgggaagacgcctttcactgacccgggcgcgggacctcgggtcccgggccggggccaggggccataccctggcgcggggggcgggccgcctagcgggggaggggggcacgcccccgaggtgggggcagcggctcgcccctcaggttaactcttcgctggccgaggccaggcgcgggcatgctccctcgcacccggccaggagaaaaagggc

SEQ ID NO: 17756 - RNA, 1261 nt, Homo sapiens
  source 1..1261: mol_type = other RNA
tccctgtcctccaggagctcacggtagcgctcatactcctcatccgtgaggcccgggacgtcgccccctcccagccccgccccctcggccagcagagagtccatgctgaaatggaagtcccggctctgcagggcgtccccttgcaggccaaacttgcgcaggcttcccggggtgttggtggagctcgggggttcgtcccccagcaggtcgtgctcagagctctcttcgttccgggtgctctcgtcagtccggcccaccccgctgtccagctcctggctgttgctcaggcctgggccggcatcgggagcccccttctcctcttcgtttccgggctgctgggcagggggtgatttcagtttacgagcacgcagctccccctcattctcagagccaaagtcatccaggaagtcatcccggtcgctgtccttccaccttttcgccagctgactctcaggtcgggccaccagcagggagatgttggtgttctcttcctggctcaggatggccaccgcctcttcccggttctggacgtctacaccgttaatctggatgatgcggtctccctcacggatccggccgtctttggctgcaatgctgttgggatttacctctccgacataaatgcccaggtcctcctcgtcgtccgtgcggtagcaaaccatcaggcccagcttgtcccggtggctgcttttatacagctccacctcctcatactccagctcatccaagcggtctgcctcctgcgggccgccctccataaactccgccgggtcataatactcatggctgattggggggggctccaggatgaccatgggcggggtgggcggacgcagcttgcccagcgccatgatatgctcgaaggtgatgtcggtctgagtgccactgtccaccagctgcaggtcgtgacaggagctgtccccccggaggcgggggctgcgtctcagcacctggatcaccaggggctccttggaggagcgcagggcctgcagagtttgctcctgagacagcttggagagctccttcccgttcacccgagacgcctaaggcccgggagcccatcgttcgggcagggccaggcgggagtgggtgtcggggtgggcacccagcccccggacggacttggaccgcgcccggggacgcccacgcactcccacgctccaggcccgccgggatctagattcggcgccccccgcacggcgggagcctggctccctcccccgccctgggtcctgcggggagagcgtgtgcggggaactgc

SEQ ID NO: 17757 - RNA, 1340 nt, Homo sapiens
  source 1..1340: mol_type = other RNA
tccctgtcctccaggagctcacggtagcgctcatactcctcatccgtgaggcccgggacgtcgccccctcccagccccgccccctcggccagcagagagtccatgctgaaatggaagtcccggctctgcagggcgtccccttgcaggccaaacttgcgcaggcttcccggggtgttggtggagctcgggggttcgtcccccagcaggtcgtgctcagagctctcttcgttccgggtgctctcgtcagtccggcccaccccgctgtccagctcctggctgttgctcaggcctgggccggcatcgggagcccccttctcctcttcgtttccgggctgctgggcagggggtgatttcagtttacgagcacgcagctccccctcattctcagagccaaagtcatccaggaagtcatcccggtcgctgtccttccaccttttcgccagctgactctcaggtcgggccaccagcagggagatgttggtgttctcttcctggctcaggatggccaccgcctcttcccggttctggacgtctacaccgttaatctggatgatgcggtctccctcacggatccggccgtctttggctgcaatgctgttgggatttacctctccgacataaatgcccaggtcctcctcgtcgtccgtgcggtagcaaaccatcaggcccagcttgtcccggtggctgcttttatacagctccacctcctcatactccagctcatccaagcggtctgcctcctgcgggccgccctccataaactccgccgggtcataatactcatggctgattggggggggctccaggatgaccatgggcggggtgggcggacgcagcttgcccagcgccatgatatgctcgaaggtgatgtcggtctgagtgccactgtccaccagctgcaggtcgtgacaggagctgtccccccggaggcgggggctgcgtctcagcacctggatcaccaggggctccttggaggagcgcagggcctgcagagtttgctcctgagacagcttggagagctccttcccgttcacctgcagcatcactttgtactgctcctccggtttctggaccacgcacatattacatcccatgttgctggccggcgagaggaggcggagggcgggaacgggaagacgcctttcactgacccgggcgcgggacctcgggtcccgggccggggccaggggccataccctggcgcggggggcgggccgcctagcgggggaggggggcacgcccccgaggtgggggcagcggctcgcccctcaggttaactcttcgctggccgaggccaggcgcgggcatgctccctcgcacccggccaggagaaaaagggc

SEQ ID NO: 17758 - RNA, 1013 nt, Homo sapiens
  source 1..1013: mol_type = other RNA
tccctgtcctccaggagctcacggtagcgctcatactcctcatccgtgaggcccgggacgtcgccccctcccagccccgccccctcggccagcagagagtccatgctgaaatggaagtcccggctctgcagggcgtccccttgcaggccaaacttgcgcaggcttcccggggtgttggtggagctcgggggttcgtcccccagcaggtcgtgctcagagctctcttcgttccgggtgctctcgtcagtccggcccaccccgctgtccagctcctggctgttgctcaggcctgggccggcatcgggagcccccttctcctcttcgtttccgggctgctgggcagggggtgatttcagtttacgagcacgcagctccccctcattctcagagccaaagtcatccaggaagtcatcccggtcgctgtccttccaccttttcgccagctgactctcaggtcgggccaccagcagggagatgttggtgttctcttcctggctcaggatggccaccgcctcttcccggttctggacgtctacaccgttaatctggatgatgcggtctccctcacggatccggccgtctttggctgcaatgctgttgggatttacctctccgacataaatgcccaggtcctcctcgtcgtccgtgcggtagcaaaccatcaggcccagcttgtcccggtggctgcttttatacagctccacctcctgcagcatcactttgtactgctcctccggtttctggaccacgcacatattacatcccatgttgctggccggcgagaggaggcggagggcgggaacgggaagacgcctttcactgacccgggcgcgggacctcgggtcccgggccggggccaggggccataccctggcgcggggggcgggccgcctagcgggggaggggggcacgcccccgaggtgggggcagcggctcgcccctcaggttaactcttcgctggccgaggccaggcgcgggcatgctccctcgcacccggccaggagaaaaagggc

SEQ ID NO: 17759 - RNA, 708 nt, Homo sapiens
  source 1..708: mol_type = other RNA
tccgaactctccattcctctgcattgctcaaagtccccagcacagtgtctgctctgctttcttaagtcaatggtgagaaatatccaagttgattgagttatcaagtgggtccccgagtgtgttgactcagtggctgaaccacgacaacaggggctgaggttctcagtttctctgttgaagttcgtgatggtttcctctacaggttggtagcaagagggtggcagaagttccaggagctccatagagttacggaaatattcacagaactgtttccttctttctcggcttttcacagaagctgggagagagggcagccatcttccttgtaaacgatattccaaaaggatgagtcccaggttcataagaaaagacattcctggtcataaagctggaaaagacttctttagctaatgctgaccaaactggatttagtgacaaccctggggcaaaatatagaatgagagccctggaaattgagagctaaataccactttcccagagcttaagaaaagacagctagagcgagcaagagagaagccactggctctagcgccatcataaatgggggcacatccaggtcctcctccgtgtttctaagtcctccttggttcaagagttttcttctccatgtcctcttgacagcaccgtcccattccttgggtgttctccagttctggaggctggaagtgtgagctcaggtgttggcag

SEQ ID NO: 17760 - RNA, 501 nt, Homo sapiens
  source 1..501: mol_type = other RNA
tccgaactctccattcctctgcattgctcaaagtccccagcacagtgtctgctctgctttcttaagtcaatggtgagaaatatccaagttgattgagttatcaagtgggtccccgagtgtgttgactcagtggctgaaccacgacaacaggggctgaggttctcagtttctctgttgaagttcgtgatggtttcctctacaggttggtagcaagagggtggcagaagttccaggagctccatagagttacggaaatattcacagaactgtttccttctttctcggcttttcacagaagctgggagagagggcagccatcttccttgtaaacgatattccaaaaggatgagtcccaggttcataagaaaagacattcctggtcataaagctggaaaagacttctttagcttttaaagagatttacatacatttcaaagagacagagaaaaacaattacaattaggaaatctctaaagtgctctaagaaaaggaaggaggtat

SEQ ID NO: 17761 - RNA, 191 nt, Homo sapiens
  source 1..191: mol_type = other RNA
tccgaactctccattcctctgcattgctcaaagtccccagcacagtgtctgctctgctttcttaagtcaatggtgagaaatatccaagttgattgagttatcagtaagataaattgctgatgattaaagtgtaaatcttggtgccctaagttgatgatctctgcgggttttgtgcaccatttgtaaatggc

SEQ ID NO: 17762 - RNA, 317 nt, Homo sapiens
  source 1..317: mol_type = other RNA
tccgaactctccattcctctgcattgctcaaagtccccagcacagtgtctgctctgctttcttaagtcaatggtgagaaatatccaagttgattgagttatcttttcacagaagctgggagagagggcagccatcttccttgtaaacgatattccaaaaggatgagtcccaggttcataagaaaagacattcctggtcataaagctggaaaagacttctttagcttttaaagagatttacatacatttcaaagagacagagaaaaacaattacaattaggaaatctctaaagtgctctaagaaaaggaaggaggtat

SEQ ID NO: 17763 - RNA, 9458 nt, Homo sapiens
  source 1..9458: mol_type = other RNA
tccgagcctgggtctccctcttcctttcttttcccttctcattcattttttatacttccctgttggcaactgaatttgaaaccccagacacggtccaaatctcttcatattacacacagtgagactgagctctagggagaggcagaaccagaggcagaatccaggtttccacacctctggtctctaacactatcctcaaaactagccctttccaacctgttgcactagggttcacctaaaagaaaatgccaagatatcattatcacaggctttcaagagccacccaggatgggtgaacaattaagtctgtgacttcaccccaaatgaatcagatttggaagtggtatttaagtagcaaatgggaataagcttaaacagagacttatctgggagtctaactgtggcctagatttgatcaggtttactcccagcagtggaggtgggacatgggacggctccatgtccgacaaggggagagcatctggggtcagcctcctgctgagtagacttgccactgttaaactctgaaatggcgggagcccagcagcaaaaataacctctgctctcgatgccaggccacctgcttcttgtctatggctgatgatctttgcttaggaggctaagtgccatatgggatcctgaacccctatttttctgtgatatttatgcaaacaagccagaatgcatttttgtatggagctgagtcaatgccttactttctccgttaaccatcttggttaaattcctacctggggatgaagtataaagaaaaacagaaataaggcatgttccttttttagaaaaatatattttaagaggtcacaatatctccagagccaaaagcaagcagctccatatggctttacagtggctgtcagacaatggtatctctactattccattaagagaatttccctgcactctccacaaacactgaagagtgagatttctccttcctaaaagtttgcattttcttcctaagaacactagctgagagggatggatgtacctaaaatgtagagctgattgaaatgtaggcagtatgcacagcctctgggaaccacgcaggctttatccaccaacatttgagtctgtggctgatgggaaaatgtgatagctgaaagtaaccaatgaaatgaatctggttcagtccctacatttaattaatgaagaagctgagagtcacagaggtgaactagttaataactacatattattaccaatttattgtcttggatttcaatactcaaggcaacttaatatctacatggcatcattttagttccatgccaccattctgagttgaagagaagcaactccattttgcagatggggagacagattactagaaataaaaaactcatttttagttcagagagatgaaggatgatattggacaagtatttccaatatcttcaacacacgtattgaaaatacttgtccaatatcatactttccaatacaagtactggaaatttccaatactccgagccttagtttcctcacctaaacgaggataataatattgtctaacaggactgttaggaagattcaagaatacatgaagaatgctgaaagagcatttcagcacaggataaatatttgttgtagttgttaagctattattaagcaaagggcagtgccaataataggacccctgtctccatatgactggctcagtgcctttccattagaccatgctacatgaaactcagattatacatcatttgtcgttaaaacatgcaccaagcagagtggtgaaggagggaaggggggaggcaatgaataaaaaccatctaagacatggagattagctgttaccaaaatatggcatcaggcaatcatcatccaaatttgtgactgcatttcatagaacagcgcggatgggattttattagatggcttctgccaaaaacatattggcagatacagccctgagcttgtggttcaccagacacaaaagagcccctcttcgggaaggggatcctgcttaggccctggcccaactccgagttaacacacagttaaaagtagcagctgcagcactgctgagacagggggtcccctagaggaaggccttgccaagggggctgttcccaaattatttatcaattgttataaagagaactttaaaaatacacacatatacacaaagcaaacaaaacctccacaaaatttaaccttagaaaatacagatgttgtaagaacaaatacaattagtcgacagattaacgggaaaacctcaagaaatgcaaactcaaacatcaatgaagtccaattttcacctaccagtttagaaggaaaaacctcaaaaatataataatgcttcaaggataaatgtatactttgctgattgcagtgtaaattggtgcaacgcttttggaaagcaatctggtaatatgtaccaaaagccataaaaacgttcatatcttttgacttagtaatcttccttttagattctaaggatctaatccaaaaaaaggagaaagcggtataagcaaatatgtaattgcagcattacttataactatgttaaatcaaaagcaacttaaaggtccaacaataaggaaatgattttgcatattgtaatacatcctctacatggaatatccagtagccattataaatcatataaagaaactgcttctaacagtaagtgaaaaatcacaggctcctatgattacaactattttaaaacatgtatataaaatgtatatgcagtaaataaagacccaaagggaaacatctaaacatattaatagttgtttggggctcagtttcttactattattaagaaaagtttccacactgtctattatttagaatattcccacttatgttctgcattatgtatataagtgtgtgcaaactagcaacccgtaaagtacatccaactacagttgagttttatctgcatgttttaaaacagtgaattatctgccaacactgaaaactcaaaaagtgtcacactggcggctttcaccgaaaaatctagtcttgcaatcctgggcccacacctctgtaaggtaataactgtttggagttggaagcaactgtcccttgtagacagcataagtgcccacctgtttgccatacccaccaccatccctgttgtctttttcttttttcttttctttttttttttttttttgagatggagtctcgccctgttgcccaggctggagtacaatggtgcaatctcggctcactatgacctctgcctcacaggttcaagcaattctccctgcctcagcctcccgagtagttgggattataggcgcccaccaccacaaccggcttatttttgtatttttagtagagatggggattctccatgtcagccaagctggtctcgaactcctgacctcaggggatccacccgccttggcctcccaaagtgctgggattacaggcttgagctaccgcgcccagcccctgttgtttttcacccaagtcggcttccctcttgtatgtcacctgcccaattcctagtccatatgattaagggaggcaaatgatgatggagaactgtaaataatttgaattcccttttaaacgggaatcattgcctattaaacttgagctttagtttggtttgttaggtcaccagaaaattacggtccaatctactactctcctcaccatgcaacaggcaatttcagggtctttcttatcaacaaaagaaccattggccacacctcgcctcctccgttggacatgctcctcagtccagagtctgctggtgcactcttttcctcttttcttgaagttagtctgtggcaaggccctggctagcctcctcctccgtgcttagcaactacagaggcgagcacacagcacacttttaggcagcagttcacagccacgttaccctaactgcttttctatattacagagacaaattattttctgcgtttcctgagacagagatagagcaggttacgggcgaggctttctttctccctatacatattctagctatcacctggcagaactctggctctgtttgctgtaggcagatgtttgcatttttcttttcccaggggcagaaggtatagaaacagagagtgtgcagtagtagagaggtgacactggaggatataggtcctgtcacatctattgcataaagatgcagtgtggtgagaatgtctgggaactcgctgtttgtgagtcgccacaaaaaaagcacaaactaccaatgacagtatatattatgttcatttacttacacgcatgcaaaaggccataatgttggtagatgaattaatagaaaacaagccccccccaaaaaataagcaagtaattttctagtctacatgtctgatctagtgaaggctgagggacagctcctggaccaaggacctttagtaaacatcagggctctgggccgaatgtccttacctgtttcctaaggcttgggaaactgttattcaggcaagagagttatttcagataaaggacaaatgctgtcctttaattaacaatatctatctctgggacaagcacatcaggtatacaatacagaagattcttttaatataaaggacagatggcaacttcactcctgggactttcaaggctgccccagaaaaacacacaattttaaaaggctttgagaattctctaaggagaaccagtcaggagataagaatgcttcattgccccatttacaaagtaaaccagaaagtgtctcagaatcattcagaaacacttgaagaagggtcaggtaaatctgagagaggaaaataataacttttgccccatagtgtagttgtgaatatcgtgaaagtttcctttcctctgagccaaacagtactagatgaaaaggagtttgaatgtgctgtactgactaacagtttgggcttcatgatcacataacaacaaagcaaaacaaaactttcaaatatcctccttatgctaatattgaaaacatcccaccaggacactgccacccagctgagcactggtttacttggtaaaaggataggatgaggtccccagctcaagtgaaatgtctctccttttatggttctcattaatctgactcaacacacacatgtgttggtacaagattcctacagcatgtgttatacctgcctaactgggtgctaacattataaaccacacatcaacacttcttgtccgagagtgttaatgtctattaatgtcctgctggggaaaaggctcttagagccagcccacagccacaattcaagactgcctgccacgagtcctagacttggcctgctgattttagatggtgtatttcattaccagaatttctggaggagggtggcgatgatggtgctgtacttggttttatgttgccaagattatcttcatatatgaaacttaaaaagccatatgaatctgaaggaacttaggactgaggaatcaaccatgtagaatttggctactgataccccagataccaaattaggcttttctgcttctgcactgtgatgttttgcaacacattgatatggggaggaaaggggcttgccaatgtcacagtgagcttccttgtctgcacattttctatacatcctatgaagtcatgcacattatctcaagctggatttactaagttcctaagtgcacatacaatgtgcttgtatgtgcaatgtgtatatatgtatatcactgatagacccgaatcaagtatatatggtgaatttcttttatatacatatgaaggctgcataatatgtgaacacacacatatacatacatataaattaaaacaaattaattaaatgataatttcataaattttgtgatgttttctcaagatttgctaggcagcacaaaaagtgtatatttaaaccacacaactccattcctgcaaataataataaaaaaagatgtacacacaagcacaaccgtcaaaaccggatttgcccttctctaaattaatccaattattcaaatgtcagttatatctgtcacagcccggctccttgggccgaaccaaactgttaaaaattaaaactgttttacttcgtttagtctttctgcctttttagtgtaaaacccacagtctcgacaaaaagttgtgggatttgacacccagtgcaacacaaccctattgctgtcatccatgcataattcactttggaaatatgcacttgctttaaaatattactaaaaaatacatgtaacatatgctaatttcactgcgttggcttgtaagctctagccactaggttatatgtaaactttgccaagtgcacacactgtacataaagggattataaatgaaaggaaatatctctgtccctagctctctgtctccatccttggccaaactgacagccccaaatcccagcaccatctaacatgcccttcccgtggagaagacagcctgttctcagagtcttaattacatcccagctgactacccagcgttgccaaaatcaggcaacaaacgctggcccttcactcacaatatggtctgctaaacagactcctggtcacacagaaagaaactttcacaacgtggagaaataaagggacaagcaggagatcaagggagagcacaaacagtaacctaggggatggaagagagagaaacaattcatccccaccgtgcaaaaaaaggggaaaataaaaagaaaaaccttttcccagaatccttaggcaccactgcgcagcggaattttaacaaagctatccttattataatgaaatcaaagaccgactcatccagccaagaactgctgctcctcaagatgggaggctgatacgaagactcagtagattaacgattgttaagcaggactcacccactccacacggatcaggccattataattacagaagaacagcatgcaacattctaccattgcaaatggtatcatacgttttcctggctggctttcggggaagggtttagctcatttgacatggcagaaggtcctggagccatgcattcatagctacctgtctttcatatctagcggcataaaattaagtttctttctttttgtgattgcatcacttgtatatgactgcaaagatggtcactgaacttggaggctattcttggcttggtccacctctaaatagaattagctattaaaaagaaaatttactttaaaagggagctttggaaggcagttgttctccagagcaactgaaaccaagatcaacaaaagatcttgagaatgtgctaatagagaaagacctgctctatgaattaaaatgttgtagactgagaaatcaaactgtggtttcaaatgtggcccacaaatcagaagttataaaggcagctgcttggaattttccttgttgattttggtatttgagattgtgattgtggggatgccatttattcaacacaatgggaacactgctgcctggcattctgtcataatcaaactgcttttcatatgggcaattccacatagaatgttccaagattaatagcactatggatttacttattttaatgatggtacaagattctccagaacagggtaggggcagacaattaaacagtaaaaataacaaatacattataaacacaatttgcaaagcacttaaatatacatcctcattaagtttcaaaattacagctgccatggtggctcacacctgtaatcccagcactttgggaggacaaggtgggcggatcacttgaggccaggagttcgagatcagcctggccaacatggtgaaaccccatctctactaaaaacacaaaaattagttaggcgtggtggcgtatgcctgtaatcccagctacttaggaggctgaggcaggagaatctcttgaatccgggaggcagaggttgcagtgagccgagatcgtgccactgcactccagcctgggtgacagaggaagactctaactcaaaaaaaaaaaaaaaaagtttcaaaattactctataaggttggcattattattctgattttacacaagatgaaactgaaggtcaaggaagttaaatggcttttccaagataacaggggttttgactccaaaactcattctttttccactgccctatgtcgttgctctggcatgccattctctcctcaggttctggcgtgcagtgagcgaggcaaggatggcagtcaagatttcattcctttgttccacggggagcccctctcttttaacttcatgaagcacagcatttgtcacaccctccatcttcttccacagtgcttccagttgagccatgggttgacaccaccagtcagtgcactttctgtatcgattgccttgaaaccaaaactgcctcagccactcaaactcgacctcattatgaatttcttctccttgtttcaaaactgcaggctcaaaggatttcaaagagacatcatcattgtccacatcgtcacagacattctgcagagccaactgacagcgttgtaaaatataatccaaggttcctgttgagcactctgccactcggtgggtggaactaaaccgaggttgtgaaccggccaaaacacagtgttggtgggtggcattgagatcatcaagcatgaaatagcagtctccttggtgaaggggtatcgccaaaccaggtgtctctatgtcccatgagatcttaaaaccaacatgccaaatatcaggatccctgccttcgagatgagagtcatcctcactttcctcttcagggcagggctgctttttccaagagcagactgtaccttcacagctataactgtacactgccaccgctgacctgtccaccagattttcatcatgatgccagctcactgccattttccccatgccaaaataaggttcctctttcaggtatggcattttctgaggatccatgaaattcagcaaagttacgttgtatgctgctctgctcttaatgtccacttcatcttgtccgttgtaggatgaacccatcccaaccctggggaaatctgcagacatacacaatggcacagcatcctcattagccttctctttggcagcaagttcttccaaagcctggatggtttctatctgcaggtagtcattgagcttgaggaaggtctcacaagcagcggctatttcagcctcggtgtgttttatattagaccctttcactggccaggggaccgtaaagagcctggtgttcaggtacttgtaggtgcagcctggattaccaatgaggatgcgagataccggagtgagcagatctttgccttggatcctaaccaggtcccgaaataagcagccatgcttgtgcagtgtgagaaaggcttcttgaacctctttatggagctcctcagatacactgctggcttctcggagaattagtttaggatatttcagctgccactgctgatagaattcatcatctttgggggtcagataagggagccaagtgtcttcaagctcttcaagaagcctcagtttcttagcttcgcgctctcgttcctcggcagtcggggtgcgcttcatgctgccactaaagccgccttcgccaccgcaagctgcgtagatc

SEQ ID NO: 17764 - RNA, 486 nt, Homo sapiens
  source 1..486: mol_type = other RNA
tccgagcctgggtctccctcttcttgtgatgatgggagatgatgcaatgcctacatgatgtgaatggaggtgaatgatccaggcattgtgacatagcatcgggccactcctgagtttctgatgatgtcggaagggaggatcatctgcctcagttgattctggatcctcaagccatgatgatgtccacggttgaatgtcaggagcagacgacgtcaatgacaaagggatgttccatgtccggggcaggacagcacaagatttcatcatgctcctcagaatggtgtgcaatttaaaacttttgaagtgtttattcctggaattttccaagttgactacagaactgaaccctcagaaagcaaaaccttgggtaagaggggactattctatcacaagctcagtagcttaaaacaacagacatttattctgccacagttctagaggctatgcatcagaaatcaaggtgtcagcaggaccgtgctccctctg

SEQ ID NO: 17765 - RNA, 1836 nt, Homo sapiens
  source 1..1836: mol_type = other RNA
tcctcttctccctcctcccagcaccccacttggcttcaacctccagtgactgcacagagcccacccagggtctaaagctagggaaggcagctcaaactcacctttcttctcccttcttccacctcccacctcattcccatctcttgtatgatgctgcagttctgggggctctgggttcgggggctggagttgcccaggaggtaggagcgggtgaccagattgtccccgaagctgccacccccactgccccccacactgcggtagctgcgagtgaccgtgacactggaggcagaagagccagaggagatgggtccgcccacctgggctcctgagccgctggcagatgccttgtcggcaggctgcccgcaggtcccgcacagcacggtgcgcgagcgcaggttgtactcagcggggtcccccgagctgctgcagtgggagccgtggtggtgatggagcaggtcatctccatcctcatcctcgtcgtcctcaaccacagtcactgagcgcaccagcttgcgcatggccacttcttccccagtggagttgatgagagccgtacgcaggctgttcccgcagccccaggtgttctgtgccttccacaccaggtcggtaggggggctgtgggtggccccagctcctgcagcccagatcgtcaccacctgcccagccttcagggtgaactttggtgggaaccggtaagtcagcaagggatcatctccattctggcgcttgatctgccaattgcccatggactggtcctcattggacttgttgcgcagccggacaaacttgccctcctcatccacctcctccacggccacgcgcccgctagtgcgtgcgtgctgtgagaagctgctgcggctctcagtggactccagtttgcgctttttggtgacgctgcccccaccctgtgtctgggatgagtgagaggaagcacggccacggctgcgctgcgaggtagggctgggggacaggcgtagcctctcctcctcgccctccaagagcttgcggtaggcgtggatctccatgtccagggccagcttgatgtccagaagctcctggtactcgtccagctgctgctgcatccttgcccgcatctcggccatctcccgctccttttccgccagcagccgccggctggtgtcccgctcacgggccagtgagtcctccaggtctcgaagcttcgcctccttggctgccagctgcttctggagctggctgagctgggcagagaggctgtcgatgcggatgcgcgactgctgcagctcctcgtgggcagcccccaccaggttgctgttcctctcagcagactgcctggcattgtccagcttggcagaataagtcttctccagctccttcttatactgctccacctggtcctcatgctgggcccgcagttcctgcagcgcatccgccagccggctctcaaactcacgctgcttcccattgtcaatctccaccagtcgggtctcatgacggcgcttggtctcacgcagctcctcactgtagatgttcttctggaagtccagttcctccttcatggtctgcagcctgttctcagcatccacccgccgcagcatctcatcctgaagttgcttcttggcctcacctagggctgcctcaagcttggccacctggccccgcagatcatgcagctcgccctccagcgtgcgcttctcactgagagcagtgctcagtgcggcctccttggagttcagcagagcctccaggtccttcagccgagcctgagcagctatcaggtcaccctccttcttggtattgcagccctcagagttccccattgccaggcagcacacaggaagggagcagaagagc

SEQ ID NO: 17766 - RNA, 2863 nt, Homo sapiens
  source 1..2863: mol_type = other RNA
tcctcttctccctcctcccagcaccccacttggcttcaacctccagtgactgcacagagcccacccagggtctaaagctagggaaggcagctcaaactcacctttcttctcccttcttccacctcccacctcattcccatctcttgtctaaataaaatacagaaaagcaagcgcagctggtacctgggagaatggactcaccccggggctgggggcaggggtggggactgggggcggggcaggcagaggaacctcagccaggtgtagtggaatcacagcaggccaagcccaggggcccggctcaagctgtcctctctctctctctctccctctcggaggctggcctggcagtgagcctgccgtccagaggaggctggcggagaagcctctatgcctgcctctcaggcaccatgtcacagggtccccggggtgggggcagcagccagggcagaaaagcagaagctagcctctataaaagcacccctttcccttggcttctagaggaagccctctttggttttaaggcagatgtggagtttcctggaagcagggaaaaggaagggaggagaaattaggattgagatagatgagatagatgcttttttttttttttgcttgtgtttttccttcagtataaaaccactgtagaaaataacttctcttagaaaaaaaaatacagaagaaaaaaaccaaagggttatttttctttggcttcaagccccctcccatgacgtgcagggcagggggtgggcatgaggtgaggaggacgcaggaagcctccacccccacccctgcctggcaggtcccagattacatgatgctgcagttctgggggctctgggctcctgagccgctggcagatgccttgtcggcaggctgcccgcaggtcccgcacagcacggtgcgcgagcgcaggttgtactcagcggggtcccccgagctgctgcagtgggagccgtggtggtgatggagcaggtcatctccatcctcatcctcgtcgtcctcaaccacagtcactgagcgcaccagcttgcgcatggccacttcttccccagtggagttgatgagagccgtacgcaggctgttcccgcagccccaggtgttctgtgccttccacaccaggtcggtaggggggctgtgggtggccccagctcctgcagcccagatcgtcaccacctgcccagccttcagggtgaactttggtgggaaccggtaagtcagcaagggatcatctccattctggcgcttgatctgccaattgcccatggactggtcctcattggacttgttgcgcagccggacaaacttgccctcctcatccacctcctccacggccacgcgcccgctagtgcgtgcgtgctgtgagaagctgctgcggctctcagtggactccagtttgcgctttttggtgacgctgcccccaccctgtgtctgggatgagtgagaggaagcacggccacggctgcgctgcgaggtagggctgggggacaggcgtagcctctcctcctcgccctccaagagcttgcggtaggcgtggatctccatgtccagggccagcttgatgtccagaagctcctggtactcgtccagctgctgctgcatccttgcccgcatctcggccatctcccgctccttttccgccagcagccgccggctggtgtcccgctcacgggccagtgagtcctccaggtctcgaagcttcgcctccttggctgccagctgcttctggagctggctgagctgggcagagaggctgtcgatgcggatgcgcgactgctgcagctcctcgtgggcagcccccaccaggttgctgttcctctcagcagactgcctggcattgtccagcttggcagaataagtcttctccagctccttcttatactgctccacctggtcctcatgctgggcccgcagttcctgcagcgcatccgccagccggctctcaaactcacgctgcttcccattgtcaatctccaccagtcgggtctcatgacggcgcttggtctcacgcagctcctcactgtagatgttcttctggaagtccagttcctccttcatggtctgcagcctgttctcagcatccacccgccgcagcatctcatcctgaagttgcttcttggcctcacctagggctgcctcaagcttggccacctggccccgcagatcatgcagctcgccctccagcgtgcgcttctcactgagagcagtgctcagtgcggcctccttggagttcagcagagcctccaggtccttcagccgagcctgagcagctatcaggtcaccctccttcttggtattgcgcgctttcagctccttaaactcctcacgcactttgctcagctccagctgcaggcgggcgcgctccttggctactgagtcaagggtcttgcgggcatccccgagctcggcctcgtaggcggccttgatgccggacacctcgcggctgaccacctcttcagactcggtgatgcgaaggcgcagccctgcgttctccgtttccagcgagcgcacacggtcgatgtagaccgccaagcgatcattgagctcctgcaggtcctccttctcctgcagccgggtgatgcgggtgggcgacagcggagtggagctggcctgcgccccgctgcgggtggcgcgccgctgggacggggtctccatggccggcaggttggcagcgctgcccgcggggcaggggtcccggaaagggcgcggggctcgggtcgaaggacagagactgctcggagtcggagtgcgccggccggctggctctcggcttgctcctggcaggcgtggggatctgggccgggcgctgtcggacctcgggatctgggttggctggtgtaggtgcggcgctcccgcgaacact

SEQ ID NO: 17767 - RNA, 2591 nt, Homo sapiens
  source 1..2591: mol_type = other RNA
tcctcttctccctcctcccagcaccccacttggcttcaacctccagtgactgcacagagcccacccagggtctaaagctagggaaggcagctcaaactcacctttcttctcccttcttccacctcccacctcattcccatctcttgtctaaataaaatacagaaaagcaagcgcagctggtacctgggagaatggactcaccccggggctgggggcaggggtggggactgggggcggggcaggcagaggaacctcagccaggtgtagtggaatcacagcaggccaagcccaggggcccggctcaagctgtcctctctctctctctctccctctcggaggctggcctggcagtgagcctgccgtccagaggaggctggcggagaagcctctatgcctgcctctcaggcaccatgtcacagggtccccggggtgggggcagcagccagggcagaaaagcagaagctagcctctataaaagcacccctttcccttggcttctagaggaagccctctttggttttaaggcagatgtggagtttcctggaagcagggaaaaggaagggaggagaaattaggattgagatagatgagatagatgcttttttttttttttgcttgtgtttttccttcagtataaaaccactgtagaaaataacttctcttagaaaaaaaaatacagaagaaaaaaaccaaagggttatttttctttggcttcaagccccctcccatgacgtgcagggcagggggtgggcatgaggtgaggaggacgcaggaagcctccacccccacccctgcctggcaggtcccagattacatgatgctgcagttctgggggctctgggttcgggggctggagttgcccaggaggtaggagcgggtgaccagattgtccccgaagctgccacccccactgccccccacactgcggtagctgcgagtgaccgtgacactggaggcagaagagccagaggagatgggtccgcccacctgggctcctgagccgctggcagatgccttgtcggcaggctgcccgcaggtcccgcacagcacggtgcgcgagcgcaggttgtactcagcggggtcccccgagctgctgcagtgggagccgtggtggtgatggagcaggtcatctccatcctcatcctcgtcgtcctcaaccacagtcactgagcgcaccagcttgcgcatggccacttcttccccagtggagttgatgagagccgtacgcaggctgttcccgcagccccaggtgttctgtgccttccacaccaggtcggtaggggggctgtgggtggccccagctcctgcagcccagatcgtcaccacctgcccagccttcagggtgaactttggtgggaaccggtaagtcagcaagggatcatctccattctggcgcttgatctgccaattgcccatggactggtcctcattggacttgttgcgcagccggacaaacttgccctcctcatccacctcctccacggccacgcgcccgctagtgcgtgcgtgctgtgagaagctgctgcggctctcagtggactccagtttgcgctttttggtgacgctgcccccaccctgtgtctgggatgagtgagaggaagcacggccacggctgcgctgcgaggtagggctgggggacaggcgtagcctctcctcctcgccctccaagagcttgcggtaggcgtggatctccatgtccagggccagcttgatgtccagaagctcctggtactcgtccagctgctgctgcatccttgcccgcatctcggccatctcccgctccttttccgccagcagccgccggctggtgtcccgctcacgggccagtgagtcctccaggtctcgaagcttcgcctccttggctgccagctgaaggggggtgggagggtttggtgagctcccaagggccctgcttctggagctggctgagctgggcagagaggctgtcgatgcggatgcgcgactgctgcagctcctcgtgggcagcccccaccaggttgctgttcctctcagcagactgcctggcattgtccagcttggcagaataagtcttctccagctccttcttatactgctccacctggtcctcatgctgggcccgcagttcctgcagcgcatccgccagccggctctcaaactcacgctgcttcccattgtcaatctccaccagtcgggtctcatgacggcgcttggtctcacgcagctcctcactgtagatgttcttctggaagtccagttcctccttcatggtctgcagcctgttctcagcatccacccgccgcagcatctcatcctgaagttgcttcttggcctcacctagggctgcctcaagcttggccacctggccccgcagatcatgcagctcgccctccagcgtgcgcttctcactgagagcagtgctcagtgcggcctccttggagttcagcagagcctccaggtccttcagccgagcctgagcagctatcaggtcaccctccttcttggtattgcagccctcagagttccccattgccaggcagcacacaggaagggagcagaagagcagagggtctcccagcccctgggcatttcctgtctcccaggaacatcgc

SEQ ID NO: 17768 - RNA, 3092 nt, Homo sapiens
  source 1..3092: mol_type = other RNA
tcctcttctccctcctcccagcaccccacttggcttcaacctccagtgactgcacagagcccacccagggtctaaagctagggaaggcagctcaaactcacctttcttctcccttcttccacctcccacctcattcccatctcttgtctaaataaaatacagaaaagcaagcgcagctggtacctgggagaatggactcaccccggggctgggggcaggggtggggactgggggcggggcaggcagaggaacctcagccaggtgtagtggaatcacagcaggccaagcccaggggcccggctcaagctgtcctctctctctctctctccctctcggaggctggcctggcagtgagcctgccgtccagaggaggctggcggagaagcctctatgcctgcctctcaggcaccatgtcacagggtccccggggtgggggcagcagccagggcagaaaagcagaagctagcctctataaaagcacccctttcccttggcttctagaggaagccctctttggttttaaggcagatgtggagtttcctggaagcagggaaaaggaagggaggagaaattaggattgagatagatgagatagatgcttttttttttttttgcttgtgtttttccttcagtataaaaccactgtagaaaataacttctcttagaaaaaaaaatacagaagaaaaaaaccaaagggttatttttctttggcttcaagccccctcccatgacgtgcagggcagggggtgggcatgaggtgaggaggacgcaggaagcctccacccccacccctgcctggcaggtcccagattacatgatgctgcagttctgggggctctgggttcgggggctggagttgcccaggaggtaggagcgggtgaccagattgtccccgaagctgccacccccactgccccccacactgcggtagctgcgagtgaccgtgacactggaggcagaagagccagaggagatgggtccgcccacctgggctcctgagccgctggcagatgccttgtcggcaggctgcccgcaggtcccgcacagcacggtgcgcgagcgcaggttgtactcagcggggtcccccgagctgctgcagtgggagccgtggtggtgatggagcaggtcatctccatcctcatcctcgtcgtcctcaaccacagtcactgagcgcaccagcttgcgcatggccacttcttccccagtggagttgatgagagccgtacgcaggctgttcccgcagccccaggtgttctgtgccttccacaccaggtcggtaggggggctgtgggtggccccagctcctgcagcccagatcgtcaccacctgcccagccttcagggtgaactttggtgggaaccggtaagtcagcaagggatcatctccattctggcgcttgatctgccaattgcccatggactggtcctcattggacttgttgcgcagccggacaaacttgccctcctcatccacctcctccacggccacgcgcccgctagtgcgtgcgtgctgtgagaagctgctgcggctctcagtggactccagtttgcgctttttggtgacgctgcccccaccctgtgtctgggatgagtgagaggaagcacggccacggctgcgctgcgaggtagggctgggggacaggcgtagcctctcctcctcgccctccaagagcttgcggtaggcgtggatctccatgtccagggccagcttgatgtccagaagctcctggtactcgtccagctgctgctgcatccttgcccgcatctcggccatctcccgctccttttccgccagcagccgccggctggtgtcccgctcacgggccagtgagtcctccaggtctcgaagcttcgcctccttggctgccagctgaaggggggtgggagggtttggtgagctcccaagggccctgcttctggagctggctgagctgggcagagaggctgtcgatgcggatgcgcgactgctgcagctcctcgtgggcagcccccaccaggttgctgttcctctcagcagactgcctggcattgtccagcttggcagaataagtcttctccagctccttcttatactgctccacctggtcctcatgctgggcccgcagttcctgcagcgcatccgccagccggctctcaaactcacgctgcttcccattgtcaatctccaccagtcgggtctcatgacggcgcttggtctcacgcagctcctcactgtagatgttcttctggaagtccagttcctccttcatggtctgcagcctgttctcagcatccacccgccgcagcatctcatcctgaagttgcttcttggcctcacctagggctgcctcaagcttggccacctggccccgcagatcatgcagctcgccctccagcgtgcgcttctcactgagagcagtgctcagtgcggcctccttggagttcagcagagcctccaggtccttcagccgagcctgagcagctatcaggtcaccctccttcttggtattgcgcgctttcagctccttaaactcctcacgcactttgctcagctccagctgcaggcgggcgcgctccttggctactgagtcaagggtcttgcgggcatccccgagctcggcctcgtaggcggccttgatgccggacacctcgcggctgaccacctcttcagactcggtgatgcgaaggcgcagccctgcgttctccgtttccagcgagcgcacacggtcgatgtagaccgccaagcgatcattgagctcctgcaggtcctccttctcctgcagccgggtgatgcgggtgggcgacagcggagtggagctggcctgcgccccgctgcgggtggcgcgccgctgggacggggtctccatggccggcaggttggcagcgctgcccgcggggcaggggtcccggaaagggcgcggggctcgggtcgaaggacagagactgctcggagtcggagtgcgccggccggctggctctcggcttgctcctggcaggcgtggggatctgggccgggcgctgtcggacctcgggatctgggttggctggtgtaggtgcggcgctcccgcgaacactgagtcaccgacgccggggcaaaggctctaataggtcctc

SEQ ID NO: 17769 - RNA, 2551 nt, Homo sapiens
  source 1..2551: mol_type = other RNA
tcctcttctccctcctcccagcaccccacttggcttcaacctccagtgactgcacagagcccacccagggtctaaagctagggaaggcagctcaaactcacctttcttctcccttcttccacctcccacctcattcccatctcttgtctaaataaaatacagaaaagcaagcgcagctggtacctgggagaatggactcaccccggggctgggggcaggggtggggactgggggcggggcaggcagaggaacctcagccaggtgtagtggaatcacagcaggccaagcccaggggcccggctcaagctgtcctctctctctctctctccctctcggaggctggcctggcagtgagcctgccgtccagaggaggctggcggagaagcctctatgcctgcctctcaggcaccatgtcacagggtccccggggtgggggcagcagccagggcagaaaagcagaagctagcctctataaaagcacccctttcccttggcttctagaggaagccctctttggttttaaggcagatgtggagtttcctggaagcagggaaaaggaagggaggagaaattaggattgagatagatgagatagatgcttttttttttttttgcttgtgtttttccttcagtataaaaccactgtagaaaataacttctcttagaaaaaaaaatacagaagaaaaaaaccaaagggttatttttctttggcttcaagccccctcccatgacgtgcagggcagggggtgggcatgaggtgaggaggacgcaggaagcctccacccccacccctgcctggcaggtcccagattacatgatgctgcagttctgggggctctgggttcgggggctggagttgcccaggaggtaggagcgggtgaccagattgtccccgaagctgccacccccactgccccccacactgcggtagctgcgagtgaccgtgacactggaggcagaagagccagaggagatgggtccgcccacctgggctcctgagccgctggcagatgccttgtcggcaggctgcccgcaggtcccgcacagcacggtgcgcgagcgcaggttgtactcagcggggtcccccgagctgctgcagtgggagccgtggtggtgatggagcaggtcatctccatcctcatcctcgtcgtcctcaaccacagtcactgagcgcaccagcttgcgcatggccacttcttccccagtggagttgatgagagccgtacgcaggctgttcccgcagccccaggtgttctgtgccttccacaccaggtcggtaggggggctgtgggtggccccagctcctgcagcccagatcgtcaccacctgcccagccttcagggtgaactttggtgggaaccggtaagtcagcaagggatcatctccattctggcgcttgatctgccaattgcccatggactggtcctcattggacttgttgcgcagccggacaaacttgccctcctcatccacctcctccacggccacgcgcccgctagtgcgtgcgtgctgtgagaagctgctgcggctctcagtggactccagtttgcgctttttggtgacgctgcccccaccctgtgtctgggatgagtgagaggaagcacggccacggctgcgctgcgaggtagggctgggggacaggcgtagcctctcctcctcgccctccaagagcttgcggtaggcgtggatctccatgtccagggccagcttgatgtccagaagctcctggtactcgtccagctgctgctgcatccttgcccgcatctcggccatctcccgctccttttccgccagcagccgccggctggtgtcccgctcacgggccagtgagtcctccaggtctcgaagcttcgcctccttggctgccagctgcttctggagctggctgagctgggcagagaggctgtcgatgcggatgcgcgactgctgcagctcctcgtgggcagcccccaccaggttgctgttcctctcagcagactgcctggcattgtccagcttggcagaataagtcttctccagctccttcttatactgctccacctggtcctcatgctgggcccgcagttcctgcagcgcatccgccagccggctctcaaactcacgctgcttcccattgtcaatctccaccagtcgggtctcatgacggcgcttggtctcacgcagctcctcactgtagatgttcttctggaagtccagttcctccttcatggtctgcagcctgttctcagcatccacccgccgcagcatctcatcctgaagttgcttcttggcctcacctagggctgcctcaagcttggccacctggccccgcagatcatgcagctcgccctccagcgtgcgcttctcactgagagcagtgctcagtgcggcctccttggagttcagcagagcctccaggtccttcagccgagcctgagcagctatcaggtcaccctccttcttggtattgcagccctcagagttccccattgccaggcagcacacaggaagggagcagaagagcagagggtctcccagcccctgggcatttcctgtctcccaggaacatcgc

SEQ ID NO: 17770 - RNA, 3013 nt, Homo sapiens
  source 1..3013: mol_type = other RNA
tcctcttctccctcctcccagcaccccacttggcttcaacctccagtgactgcacagagcccacccagggtctaaagctagggaaggcagctcaaactcacctttcttctcccttcttccacctcccacctcattcccatctcttgtctaaataaaatacagaaaagcaagcgcagctggtacctgggagaatggactcaccccggggctgggggcaggggtggggactgggggcggggcaggcagaggaacctcagccaggtgtagtggaatcacagcaggccaagcccaggggcccggctcaagctgtcctctctctctctctctccctctcggaggctggcctggcagtgagcctgccgtccagaggaggctggcggagaagcctctatgcctgcctctcaggcaccatgtcacagggtccccggggtgggggcagcagccagggcagaaaagcagaagctagcctctataaaagcacccctttcccttggcttctagaggaagccctctttggttttaaggcagatgtggagtttcctggaagcagggaaaaggaagggaggagaaattaggattgagatagatgagatagatgcttttttttttttttgcttgtgtttttccttcagtataaaaccactgtagaaaataacttctcttagaaaaaaaaatacagaagaaaaaaaccaaagggttatttttctttggcttcaagccccctcccatgacgtgcagggcagggggtgggcatgaggtgaggaggacgcaggaagcctccacccccacccctgcctggcaggtcccagattacatgatgctgcagttctgggggctctgggttcgggggctggagttgcccaggaggtaggagcgggtgaccagattgtccccgaagctgccacccccactgccccccacactgcggtagctgcgagtgaccgtgacactggaggcagaagagccagaggagatgggtccgcccacctgggctcctgagccgctggcagatgccttgtcggcaggctgcccgcaggtcccgcacagcacggtgcgcgagcgcaggttgtactcagcggggtcccccgagctgctgcagtgggagccgtggtggtgatggagcaggtcatctccatcctcatcctcgtcgtcctcaaccacagtcactgagcgcaccagcttgcgcatggccacttcttccccagtggagttgatgagagccgtacgcaggctgttcccgcagccccaggtgttctgtgccttccacaccaggtcggtaggggggctgtgggtggccccagctcctgcagcccagatcgtcaccacctgcccagccttcagggtgaactttggtgggaaccggtaagtcagcaagggatcatctccattctggcgcttgatctgccaattgcccatggactggtcctcattggacttgttgcgcagccggacaaacttgccctcctcatccacctcctccacggccacgcgcccgctagtgcgtgcgtgctgtgagaagctgctgcggctctcagtggactccagtttgcgctttttggtgacgctgcccccaccctgtgtctgggatgagtgagaggaagcacggccacggctgcgctgcgaggtagggctgggggacaggcgtagcctctcctcctcgccctccaagagcttgcggtaggcgtggatctccatgtccagggccagcttgatgtccagaagctcctggtactcgtccagctgctgctgcatccttgcccgcatctcggccatctcccgctccttttccgccagcagccgccggctggtgtcccgctcacgggccagtgagtcctccaggtctcgaagcttcgcctccttggctgccagctgcttctggagctggctgagctgggcagagaggctgtcgatgcggatgcgcgactgctgcagctcctcgtgggcagcccccaccaggttgctgttcctctcagcagactgcctggcattgtccagcttggcagaataagtcttctccagctccttcttatactgctccacctggtcctcatgctgggcccgcagttcctgcagcgcatccgccagccggctctcaaactcacgctgcttcccattgtcaatctccaccagtcgggtctcatgacggcgcttggtctcacgcagctcctcactgtagatgttcttctggaagtccagttcctccttcatggtctgcagcctgttctcagcatccacccgccgcagcatctcatcctgaagttgcttcttggcctcacctagggctgcctcaagcttggccacctggccccgcagatcatgcagctcgccctccagcgtgcgcttctcactgagagcagtgctcagtgcggcctccttggagttcagcagagcctccaggtccttcagccgagcctgagcagctatcaggtcaccctccttcttggtattgcgcgctttcagctccttaaactcctcacgcactttgctcagctccagctgcaggcgggcgcgctccttggctactgagtcaagggtcttgcgggcatccccgagctcggcctcgtaggcggccttgatgccggacacctcgcggctgaccacctcttcagactcggtgatgcgaaggcgcagccctgcgttctccgtttccagcgagcgcacacggtcgatgtagaccgccaagcgatcattgagctcctgcaggtcctccttctcctgcagccgggtgatgcgggtgggcgacagcggagtggagctggcctgcgccccgctgcgggtggcgcgccgctgggacggggtctccatggccggcaggttggcagcgctgcccgcggggcaggggtcccggaaagggcgcggggctcgggtcgaaggacagagactgctcggagtcggagtgcgccggccggctggctctcggcttgctcctggcaggcgtggggatctgggccgggcgctgtcggacctcgggatctgggttggctggtgtaggtgcggcgctcccgcgaacact

SEQ ID NO: 17771 - RNA, 2923 nt, Homo sapiens
  source 1..2923: mol_type = other RNA
tcctcttctccctcctcccagcaccccacttggcttcaacctccagtgactgcacagagcccacccagggtctaaagctagggaaggcagctcaaactcacctttcttctcccttcttccacctcccacctcattcccatctcttgtctaaataaaatacagaaaagcaagcgcagctggtacctgggagaatggactcaccccggggctgggggcaggggtggggactgggggcggggcaggcagaggaacctcagccaggtgtagtggaatcacagcaggccaagcccaggggcccggctcaagctgtcctctctctctctctctccctctcggaggctggcctggcagtgagcctgccgtccagaggaggctggcggagaagcctctatgcctgcctctcaggcaccatgtcacagggtccccggggtgggggcagcagccagggcagaaaagcagaagctagcctctataaaagcacccctttcccttggcttctagaggaagccctctttggttttaaggcagatgtggagtttcctggaagcagggaaaaggaagggaggagaaattaggattgagatagatgagatagatgcttttttttttttttgcttgtgtttttccttcagtataaaaccactgtagaaaataacttctcttagaaaaaaaaatacagaagaaaaaaaccaaagggttatttttctttggcttcaagccccctcccatgacgtgcagggcagggggtgggcatgaggtgaggaggacgcaggaagcctccacccccacccctgcctggcaggtcccagattacatgatgctgcagttctgggggctctgggttcgggggctggagttgcccaggaggtaggagcgggtgaccagattgtccccgaagctgccacccccactgccccccacactgcggtagctgcgagtgaccgtgacactggaggcagaagagccagaggagatgggtccgcccacctgggctcctgagccgctggcagatgccttgtcggcaggctgcccgcaggtcccgcacagcacggtgcgcgagcgcaggttgtactcagcggggtcccccgagctgctgcagtgggagccttccccagtggagttgatgagagccgtacgcaggctgttcccgcagccccaggtgttctgtgccttccacaccaggtcggtaggggggctgtgggtggccccagctcctgcagcccagatcgtcaccacctgcccagccttcagggtgaactttggtgggaaccggtaagtcagcaagggatcatctccattctggcgcttgatctgccaattgcccatggactggtcctcattggacttgttgcgcagccggacaaacttgccctcctcatccacctcctccacggccacgcgcccgctagtgcgtgcgtgctgtgagaagctgctgcggctctcagtggactccagtttgcgctttttggtgacgctgcccccaccctgtgtctgggatgagtgagaggaagcacggccacggctgcgctgcgaggtagggctgggggacaggcgtagcctctcctcctcgccctccaagagcttgcggtaggcgtggatctccatgtccagggccagcttgatgtccagaagctcctggtactcgtccagctgctgctgcatccttgcccgcatctcggccatctcccgctccttttccgccagcagccgccggctggtgtcccgctcacgggccagtgagtcctccaggtctcgaagcttcgcctccttggctgccagctgcttctggagctggctgagctgggcagagaggctgtcgatgcggatgcgcgactgctgcagctcctcgtgggcagcccccaccaggttgctgttcctctcagcagactgcctggcattgtccagcttggcagaataagtcttctccagctccttcttatactgctccacctggtcctcatgctgggcccgcagttcctgcagcgcatccgccagccggctctcaaactcacgctgcttcccattgtcaatctccaccagtcgggtctcatgacggcgcttggtctcacgcagctcctcactgtagatgttcttctggaagtccagttcctccttcatggtctgcagcctgttctcagcatccacccgccgcagcatctcatcctgaagttgcttcttggcctcacctagggctgcctcaagcttggccacctggccccgcagatcatgcagctcgccctccagcgtgcgcttctcactgagagcagtgctcagtgcggcctccttggagttcagcagagcctccaggtccttcagccgagcctgagcagctatcaggtcaccctccttcttggtattgcgcgctttcagctccttaaactcctcacgcactttgctcagctccagctgcaggcgggcgcgctccttggctactgagtcaagggtcttgcgggcatccccgagctcggcctcgtaggcggccttgatgccggacacctcgcggctgaccacctcttcagactcggtgatgcgaaggcgcagccctgcgttctccgtttccagcgagcgcacacggtcgatgtagaccgccaagcgatcattgagctcctgcaggtcctccttctcctgcagccgggtgatgcgggtgggcgacagcggagtggagctggcctgcgccccgctgcgggtggcgcgccgctgggacggggtctccatggccggcaggttggcagcgctgcccgcggggcaggggtcccggaaagggcgcggggctcgggtcgaaggacagagactgctcggagtcggagtgcgccggccggctggctctcggcttgctcctggcaggcgtggggatctgggccgggcgctgtcggacctcgggatctgggttggctggtgtaggtgcggcgctcccgcgaacact

SEQ ID NO: 17772 - RNA, 2409 nt, Homo sapiens
  source 1..2409: mol_type = other RNA
tcctcttctccctcctcccagcccaggcctgcaggccaggtagtgatggataagacgggtcattgcacctggtgctgcactcgcctcctgttccttccaggagggtcttctccagccctgccgggaagaccctggtgcacacaggccttccagcatggcctgcctagctcctcgccctcctgggtcctcacagccccggcctcctccctccatggtcgtgctcttctgctgtcagccccaggcctcgcagtatcggccagaaaagcccatgcccctgggcaagccctgagtcagggcccctccacagaacccgggacccctccacagaacccagggacccctccacagaacccagggcccctccacagaacccaggacccttccacagaacccagggcccctccacagaacacagggcccctccacagaacccagggacccctccacagaacccagggcccctccacagaacccagggcccctccacagaacccagggcccctccacagaacccagggacccctccacagaacccaggacccctccatagaacccaggacccctccatagaacccagggcccctccacagaacccagggaccctccacagaacccagggacccctccatagaacccagggcccctccacagaacgcaggacccctccacagaacccagggaccctccacagaacccagggcccctccacagaacccaggacccctccacagaacccaggacccttccacagaacccaggacccctccatagaacccaggacccttccacagaacccagggcccctccacagaacccagggacccctccatagaacccagggcccctctacagaacccagggcccctctacagaactcaggacccctctacagaacccaggacccctctacagaatgcaggacccctccatagaacccaggacccctctacagaactcaggacccctctacagaacccagaacccatctacagaactcaggacccctctacagaacccaggacccctctacagaacgcaggacccctccatagaacccaggacccctctacagaacccaggacccctctacagaacccaggacccctctacagaacccagggcccctctacagaactcaggacccctctacagaacccaggacccctctacagaactcaggacccctctacagaactcaggacccctctacagaacccagaacccatctacagaacccaggacccctctacagaacccaggacccttctacagaacccagaacccatctacagaacccaggacccctccacagaacccaggacccctctatagaacccaggacccctctacagaacccaggacccctctacagaaccgaggacccctctacagaacccaggacccctctacaggacccagggcccctctgtagaacccaggacccctctacaggacccagggcccctctatagaacccagggcccctctacagaacccaggacccctctacaggacccaggaccgttctacggaacccagcgcttgtcccctggcccctgcaggtgtgtcctgctctgcactgcacaggcagtgggaagagtggggtagttgcgggacgccccgattctcttcaggaggaggtgtcacctgcctcacagaggactaggtgagcagtggatgcagggtttgttttaaaacaacacacaagcctttctgatctcatgttcctttctaagaatgggtctggccaagacctgcgcctcctgagggtcgctgtggaaataaattctctctccgcagccgaccgaggccacgtccagtggccaccacagtgtcagtttctgctgtttgcctttcttctgttggtcagcacactccgtccctcaaagctgcgcagagaaaatgcagcgatcacagggcccagggctgcatttcggaagccacaggcaagacgacagctcagctttgcagccgcacacggtcctgcgctgctgagagggaatggcgattttctcactttttatgtcaccgcatctcagggtttgcaggcaaaagtcagcagactcaccctcccgcacgccgccgtccatctcctaggccagcgtgattcttctgagtgcagctgggtctcctcctgggagatccggtggctctagcagcgtgggtgctgggaacaggaccagcctcgccggcggacagtgtggacgcctgagggcaaaccctggaccactctctccccgggggactccgttcccgcctccagggagctgcgaacgctccttctgggacacctgttggcaagaaaccagttcaatcgtctcacttccagaaacgattctgtgttttgacagaagttttcaggcagcagaactcagccaaaaggatgtctgtgggcggcccttccggggg

SEQ ID NO: 17773 - RNA, 2412 nt, Homo sapiens
  source 1..2412: mol_type = other RNA
tcctcttctccctcctcccagcccaggcctgcaggccaggtagtgatggataagacgggtcattgcacctggtgctgcactcgcctcctgttccttccaggagggtcttctccagccctgccgggaagaccctggtgcacacaggccttccagcatggcctgcctagctcctcgccctcctgggtcctcacagccccggcctcctccctccatggtcgtgctcttctgctgtcagccccaggcctcgcagtatcggccagaaaagcccatgcccctgggcaagccctgagtcagggcccctccacagaacccgggacccctccacagaacccagggacccctccacagaacccagggcccctccacagaacccaggacccttccacagaacccagggcccctccacagaacacagggcccctccacagaacccagggacccctccacagaacccagggcccctccacagaacccagggcccctccacagaacccagggcccctccacagaacccagggacccctccacagaacccaggacccctccatagaacccaggacccctccatagaacccagggcccctccacagaacccagggaccctccacagaacccagggacccctccatagaacccagggcccctccacagaacgcaggacccctccacagaacccagggaccctccacagaacccagggcccctccacagaacccaggacccctccacagaacccaggacccttccacagaacccaggacccctccatagaacccaggacccttccacagaacccagggcccctccacagaacccagggacccctccatagaacccagggcccctctacagaacccagggcccctctacagaactcaggacccctctacagaacccaggacccctctacagaatgcaggacccctccatagaacccaggacccctctacagaactcaggacccctctacagaacccagaacccatctacagaactcaggacccctctacagaacccaggacccctctacagaacgcaggacccctccatagaacccaggacccctctacagaacccaggacccctctacagaacccaggacccctctacagaacccagggcccctctacagaactcaggacccctctacagaacccaggacccctctacagaactcaggacccctctacagaactcaggacccctctacagaacccagaacccatctacagaacccaggacccctctacagaacccaggacccttctacagaacccagaacccatctacagaacccaggacccctccacagaacccaggacccctctatagaacccaggacccctctacagaacccaggacccctctacagaaccgaggacccctctacagaacccaggacccctctacaggacccagggcccctctgtagaacccaggacccctctacaggacccagggcccctctatagaacccagggcccctctacagaacccaggacccctctacaggacccaggaccgttctacggaacccagcgcttgtcccctggcccctgcaggtgtgtcctgctctgcactgcacaggcagtgggaagagtggggtagttgcgggacgccccgattctcttcaggaggaggtgtcacctgcctcacagaggactaggtgagcagtggatgcagggtttgttttaaaacaacacacaagcctttctgatctcatgttcctttctaagaatgggtctggccaagacctgcgcctcctgagggtcgctgtggaaataaattctctctccgcagccgaccgaggccacgtccagtggccaccacagtgtcagtttctgctgtttgcctttcttctgttggtcagcacactccgtccctcaaagctgcgcagagaaaatgcagcgatcacagggcccagggctgcatttcggaagccacaggcaagacgacagctcagctttgcagccgcacacggtcctgctgcgctgctgagagggaatggcgattttctcactttttatgtcaccgcatctcagggtttgcaggcaaaagtcagcagactcaccctcccgcacgccgccgtccatctcctaggccagcgtgattcttctgagtgcagctgggtctcctcctgggagatccggtggctctagcagcgtgggtgctgggaacaggaccagcctcgccggcggacagtgtggacgcctgagggcaaaccctggaccactctctccccgggggactccgttcccgcctccagggagctgcgaacgctccttctgggacacctgttggcaagaaaccagttcaatcgtctcacttccagaaacgattctgtgttttgacagaagttttcaggcagcagaactcagccaaaaggatgtctgtgggcggcccttccggggg

SEQ ID NO: 17774 - RNA, 2439 nt, Homo sapiens
  source 1..2439: mol_type = other RNA
tcctcttctccctcctcccagcccaggcctgcctgctctccctcctcccagcccaggcctgcaggccaggtagtgatggataagacgggtcattgcacctggtgctgcactcgcctcctgttccttccaggagggtcttctccagccctgccgggaagaccctggtgcacacaggccttccagcatggcctgcctagctcctcgccctcctgggtcctcacagccccggcctcctccctccatggtcgtgctcttctgctgtcagccccaggcctcgcagtatcggccagaaaagcccatgcccctgggcaagccctgagtcagggcccctccacagaacccgggacccctccacagaacccagggacccctccacagaacccagggcccctccacagaacccaggacccttccacagaacccagggcccctccacagaacacagggcccctccacagaacccagggacccctccacagaacccagggcccctccacagaacccagggcccctccacagaacccagggcccctccacagaacccagggacccctccacagaacccaggacccctccatagaacccaggacccctccatagaacccagggcccctccacagaacccagggaccctccacagaacccagggacccctccatagaacccagggcccctccacagaacgcaggacccctccacagaacccagggaccctccacagaacccagggcccctccacagaacccaggacccctccacagaacccaggacccttccacagaacccaggacccctccatagaacccaggacccttccacagaacccagggcccctccacagaacccagggacccctccatagaacccagggcccctctacagaacccagggcccctctacagaactcaggacccctctacagaacccaggacccctctacagaatgcaggacccctccatagaacccaggacccctctacagaactcaggacccctctacagaacccagaacccatctacagaactcaggacccctctacagaacccaggacccctctacagaacgcaggacccctccatagaacccaggacccctctacagaacccaggacccctctacagaacccaggacccctctacagaacccagggcccctctacagaactcaggacccctctacagaacccaggacccctctacagaactcaggacccctctacagaactcaggacccctctacagaacccagaacccatctacagaacccaggacccctctacagaacccaggacccttctacagaacccagaacccatctacagaacccaggacccctccacagaacccaggacccctctatagaacccaggacccctctacagaacccaggacccctctacagaaccgaggacccctctacagaacccaggacccctctacaggacccagggcccctctgtagaacccaggacccctctacaggacccagggcccctctatagaacccagggcccctctacagaacccaggacccctctacaggacccaggaccgttctacggaacccagcgcttgtcccctggcccctgcaggtgtgtcctgctctgcactgcacaggcagtgggaagagtggggtagttgcgggacgccccgattctcttcaggaggaggtgtcacctgcctcacagaggactaggtgagcagtggatgcagggtttgttttaaaacaacacacaagcctttctgatctcatgttcctttctaagaatgggtctggccaagacctgcgcctcctgagggtcgctgtggaaataaattctctctccgcagccgaccgaggccacgtccagtggccaccacagtgtcagtttctgctgtttgcctttcttctgttggtcagcacactccgtccctcaaagctgcgcagagaaaatgcagcgatcacagggcccagggctgcatttcggaagccacaggcaagacgacagctcagctttgcagccgcacacggtcctgcgctgctgagagggaatggcgattttctcactttttatgtcaccgcatctcagggtttgcaggcaaaagtcagcagactcaccctcccgcacgccgccgtccatctcctaggccagcgtgattcttctgagtgcagctgggtctcctcctgggagatccggtggctctagcagcgtgggtgctgggaacaggaccagcctcgccggcggacagtgtggacgcctgagggcaaaccctggaccactctctccccgggggactccgttcccgcctccagggagctgcgaacgctccttctgggacacctgttggcaagaaaccagttcaatcgtctcacttccagaaacgattctgtgttttgacagaagttttcaggcagcagaactcagccaaaaggatgtctgtgggcggcccttccggggg

SEQ ID NO: 17775 - RNA, 2442 nt, Homo sapiens
  source 1..2442: mol_type = other RNA
tcctcttctccctcctcccagcccaggcctgcctgctctccctcctcccagcccaggcctgcaggccaggtagtgatggataagacgggtcattgcacctggtgctgcactcgcctcctgttccttccaggagggtcttctccagccctgccgggaagaccctggtgcacacaggccttccagcatggcctgcctagctcctcgccctcctgggtcctcacagccccggcctcctccctccatggtcgtgctcttctgctgtcagccccaggcctcgcagtatcggccagaaaagcccatgcccctgggcaagccctgagtcagggcccctccacagaacccgggacccctccacagaacccagggacccctccacagaacccagggcccctccacagaacccaggacccttccacagaacccagggcccctccacagaacacagggcccctccacagaacccagggacccctccacagaacccagggcccctccacagaacccagggcccctccacagaacccagggcccctccacagaacccagggacccctccacagaacccaggacccctccatagaacccaggacccctccatagaacccagggcccctccacagaacccagggaccctccacagaacccagggacccctccatagaacccagggcccctccacagaacgcaggacccctccacagaacccagggaccctccacagaacccagggcccctccacagaacccaggacccctccacagaacccaggacccttccacagaacccaggacccctccatagaacccaggacccttccacagaacccagggcccctccacagaacccagggacccctccatagaacccagggcccctctacagaacccagggcccctctacagaactcaggacccctctacagaacccaggacccctctacagaatgcaggacccctccatagaacccaggacccctctacagaactcaggacccctctacagaacccagaacccatctacagaactcaggacccctctacagaacccaggacccctctacagaacgcaggacccctccatagaacccaggacccctctacagaacccaggacccctctacagaacccaggacccctctacagaacccagggcccctctacagaactcaggacccctctacagaacccaggacccctctacagaactcaggacccctctacagaactcaggacccctctacagaacccagaacccatctacagaacccaggacccctctacagaacccaggacccttctacagaacccagaacccatctacagaacccaggacccctccacagaacccaggacccctctatagaacccaggacccctctacagaacccaggacccctctacagaaccgaggacccctctacagaacccaggacccctctacaggacccagggcccctctgtagaacccaggacccctctacaggacccagggcccctctatagaacccagggcccctctacagaacccaggacccctctacaggacccaggaccgttctacggaacccagcgcttgtcccctggcccctgcaggtgtgtcctgctctgcactgcacaggcagtgggaagagtggggtagttgcgggacgccccgattctcttcaggaggaggtgtcacctgcctcacagaggactaggtgagcagtggatgcagggtttgttttaaaacaacacacaagcctttctgatctcatgttcctttctaagaatgggtctggccaagacctgcgcctcctgagggtcgctgtggaaataaattctctctccgcagccgaccgaggccacgtccagtggccaccacagtgtcagtttctgctgtttgcctttcttctgttggtcagcacactccgtccctcaaagctgcgcagagaaaatgcagcgatcacagggcccagggctgcatttcggaagccacaggcaagacgacagctcagctttgcagccgcacacggtcctgctgcgctgctgagagggaatggcgattttctcactttttatgtcaccgcatctcagggtttgcaggcaaaagtcagcagactcaccctcccgcacgccgccgtccatctcctaggccagcgtgattcttctgagtgcagctgggtctcctcctgggagatccggtggctctagcagcgtgggtgctgggaacaggaccagcctcgccggcggacagtgtggacgcctgagggcaaaccctggaccactctctccccgggggactccgttcccgcctccagggagctgcgaacgctccttctgggacacctgttggcaagaaaccagttcaatcgtctcacttccagaaacgattctgtgttttgacagaagttttcaggcagcagaactcagccaaaaggatgtctgtgggcggcccttccggggg

SEQ ID NO: 17776 - RNA, 2469 nt, Homo sapiens
  source 1..2469: mol_type = other RNA
tcctcttctccctcctcccagcccaggcctgtgtgctctccctcctcccagcccaggcctgcctgctctccctcctcccagcccaggcctgcaggccaggtagtgatggataagacgggtcattgcacctggtgctgcactcgcctcctgttccttccaggagggtcttctccagccctgccgggaagaccctggtgcacacaggccttccagcatggcctgcctagctcctcgccctcctgggtcctcacagccccggcctcctccctccatggtcgtgctcttctgctgtcagccccaggcctcgcagtatcggccagaaaagcccatgcccctgggcaagccctgagtcagggcccctccacagaacccgggacccctccacagaacccagggacccctccacagaacccagggcccctccacagaacccaggacccttccacagaacccagggcccctccacagaacacagggcccctccacagaacccagggacccctccacagaacccagggcccctccacagaacccagggcccctccacagaacccagggcccctccacagaacccagggacccctccacagaacccaggacccctccatagaacccaggacccctccatagaacccagggcccctccacagaacccagggaccctccacagaacccagggacccctccatagaacccagggcccctccacagaacgcaggacccctccacagaacccagggaccctccacagaacccagggcccctccacagaacccaggacccctccacagaacccaggacccttccacagaacccaggacccctccatagaacccaggacccttccacagaacccagggcccctccacagaacccagggacccctccatagaacccagggcccctctacagaacccagggcccctctacagaactcaggacccctctacagaacccaggacccctctacagaatgcaggacccctccatagaacccaggacccctctacagaactcaggacccctctacagaacccagaacccatctacagaactcaggacccctctacagaacccaggacccctctacagaacgcaggacccctccatagaacccaggacccctctacagaacccaggacccctctacagaacccaggacccctctacagaacccagggcccctctacagaactcaggacccctctacagaacccaggacccctctacagaactcaggacccctctacagaactcaggacccctctacagaacccagaacccatctacagaacccaggacccctctacagaacccaggacccttctacagaacccagaacccatctacagaacccaggacccctccacagaacccaggacccctctatagaacccaggacccctctacagaacccaggacccctctacagaaccgaggacccctctacagaacccaggacccctctacaggacccagggcccctctgtagaacccaggacccctctacaggacccagggcccctctatagaacccagggcccctctacagaacccaggacccctctacaggacccaggaccgttctacggaacccagcgcttgtcccctggcccctgcaggtgtgtcctgctctgcactgcacaggcagtgggaagagtggggtagttgcgggacgccccgattctcttcaggaggaggtgtcacctgcctcacagaggactaggtgagcagtggatgcagggtttgttttaaaacaacacacaagcctttctgatctcatgttcctttctaagaatgggtctggccaagacctgcgcctcctgagggtcgctgtggaaataaattctctctccgcagccgaccgaggccacgtccagtggccaccacagtgtcagtttctgctgtttgcctttcttctgttggtcagcacactccgtccctcaaagctgcgcagagaaaatgcagcgatcacagggcccagggctgcatttcggaagccacaggcaagacgacagctcagctttgcagccgcacacggtcctgcgctgctgagagggaatggcgattttctcactttttatgtcaccgcatctcagggtttgcaggcaaaagtcagcagactcaccctcccgcacgccgccgtccatctcctaggccagcgtgattcttctgagtgcagctgggtctcctcctgggagatccggtggctctagcagcgtgggtgctgggaacaggaccagcctcgccggcggacagtgtggacgcctgagggcaaaccctggaccactctctccccgggggactccgttcccgcctccagggagctgcgaacgctccttctgggacacctgttggcaagaaaccagttcaatcgtctcacttccagaaacgattctgtgttttgacagaagttttcaggcagcagaactcagccaaaaggatgtctgtgggcggcccttccggggg

SEQ ID NO: 17777 - RNA, 2472 nt, Homo sapiens
  source 1..2472: mol_type = other RNA
tcctcttctccctcctcccagcccaggcctgtgtgctctccctcctcccagcccaggcctgcctgctctccctcctcccagcccaggcctgcaggccaggtagtgatggataagacgggtcattgcacctggtgctgcactcgcctcctgttccttccaggagggtcttctccagccctgccgggaagaccctggtgcacacaggccttccagcatggcctgcctagctcctcgccctcctgggtcctcacagccccggcctcctccctccatggtcgtgctcttctgctgtcagccccaggcctcgcagtatcggccagaaaagcccatgcccctgggcaagccctgagtcagggcccctccacagaacccgggacccctccacagaacccagggacccctccacagaacccagggcccctccacagaacccaggacccttccacagaacccagggcccctccacagaacacagggcccctccacagaacccagggacccctccacagaacccagggcccctccacagaacccagggcccctccacagaacccagggcccctccacagaacccagggacccctccacagaacccaggacccctccatagaacccaggacccctccatagaacccagggcccctccacagaacccagggaccctccacagaacccagggacccctccatagaacccagggcccctccacagaacgcaggacccctccacagaacccagggaccctccacagaacccagggcccctccacagaacccaggacccctccacagaacccaggacccttccacagaacccaggacccctccatagaacccaggacccttccacagaacccagggcccctccacagaacccagggacccctccatagaacccagggcccctctacagaacccagggcccctctacagaactcaggacccctctacagaacccaggacccctctacagaatgcaggacccctccatagaacccaggacccctctacagaactcaggacccctctacagaacccagaacccatctacagaactcaggacccctctacagaacccaggacccctctacagaacgcaggacccctccatagaacccaggacccctctacagaacccaggacccctctacagaacccaggacccctctacagaacccagggcccctctacagaactcaggacccctctacagaacccaggacccctctacagaactcaggacccctctacagaactcaggacccctctacagaacccagaacccatctacagaacccaggacccctctacagaacccaggacccttctacagaacccagaacccatctacagaacccaggacccctccacagaacccaggacccctctatagaacccaggacccctctacagaacccaggacccctctacagaaccgaggacccctctacagaacccaggacccctctacaggacccagggcccctctgtagaacccaggacccctctacaggacccagggcccctctatagaacccagggcccctctacagaacccaggacccctctacaggacccaggaccgttctacggaacccagcgcttgtcccctggcccctgcaggtgtgtcctgctctgcactgcacaggcagtgggaagagtggggtagttgcgggacgccccgattctcttcaggaggaggtgtcacctgcctcacagaggactaggtgagcagtggatgcagggtttgttttaaaacaacacacaagcctttctgatctcatgttcctttctaagaatgggtctggccaagacctgcgcctcctgagggtcgctgtggaaataaattctctctccgcagccgaccgaggccacgtccagtggccaccacagtgtcagtttctgctgtttgcctttcttctgttggtcagcacactccgtccctcaaagctgcgcagagaaaatgcagcgatcacagggcccagggctgcatttcggaagccacaggcaagacgacagctcagctttgcagccgcacacggtcctgctgcgctgctgagagggaatggcgattttctcactttttatgtcaccgcatctcagggtttgcaggcaaaagtcagcagactcaccctcccgcacgccgccgtccatctcctaggccagcgtgattcttctgagtgcagctgggtctcctcctgggagatccggtggctctagcagcgtgggtgctgggaacaggaccagcctcgccggcggacagtgtggacgcctgagggcaaaccctggaccactctctccccgggggactccgttcccgcctccagggagctgcgaacgctccttctgggacacctgttggcaagaaaccagttcaatcgtctcacttccagaaacgattctgtgttttgacagaagttttcaggcagcagaactcagccaaaaggatgtctgtgggcggcccttccggggg

SEQ ID NO: 17778 - RNA, 3341 nt, Homo sapiens
  source 1..3341: mol_type = other RNA
tcctcttctccctcctcccagcctccaccctcaagtaggccatggtgtctctttttccgctttttgtgttcatgtgttctcatggtgtatctcccacttataagtgagagcatgcagtatctggttttctgtttctgcattagtttgcttaggataatggcctctagctccatccatattgctgcaaaggacatgatctttttcttttttatggctgcttagtattctgtggtgaatatgtaccatattttctttattcagtctactattgatgggcatataggttgattccatgtctttgctattgtgaatagtgctgcaatgaacatacatgtgcatgtgtttttatggcaggatgatttacattccactgggtatatgcccaataatgggattgctgggttgaacggtaattctattttaagtttttcaaggaattgctacgctacttttcacaatggctgaactaatttacattcccaccagcagtgtataagcgttacaaaagattatttatgaagacagagattatatgggagtattcttttctttagcatgttcctctttattttctagattttttttgcagtgagcataccttacttcatgatgaggaaaaaaattgttatttctccaaaatgactgagcagtttgtatgaacacaatactgcaataagtaattacgggaattaaaaaaaaactttttttcttttttggagctttcaatattcacaaataaattgacgctatgtgataatatttgtattgcctgttatgtatcagatacttctcccatttaatttcacatactctatctcctttaatccaaatatagagaatacatgtaaatccactccatgttattgtaaataatgttgacaatgaacatagagatgcatattttataatagtaagttacaaacacaaagtaaaaataggcagacagaaagctatgcataaagactaaagggaaagcagtctagatagtgataatttttttctaccaactaaatttactagtaggagcatgtatccttcccataatgggagaaaaaatgaacttttaatgatttttaacatatatgacagccatggaacaattctgtgctaactttggggtacttatgtgcagcatattggacatttagtgaaaagagagaccactgtgagatgatgaagctggagaaggcttcaagaagcaatgcagggctccctgagtactttaaaggaagggaaagtttctttaagaatgtggaaggaggacaaggaggacgttatagaaagaaaataacttgtacaacagcaacaagaactggtccatttataaaacaggagcttgctcaggtggtggctatgaggattaagtaagttggtgcacctggcatcatgcctgaatgaaaggtgctcaggaaatattagccatcatgatgatggtgctggtgagaatggagaagagggatgaattcaagacacagtccaaaggactaaatggtaaacttgttcacagtctggttccttgaatagaaataaaagtgccaaataggccttcattgtttctctcccaagagagcagaaggagagtgcccgtgtcagaaggggaacaggctggggagctgggcagcaggggtaggtgatgagacaagtttgggacactcagagttaaaagtttgggaggtaaaggaagtgtggccagtgaggcggagaacacagaggtggcatcagagaaacaagagagggaagatttttcagggatgtcatcaactcttcagccagcggaatgcaggcggagttgaagaagtggaaagagaagtccctcagtgctatactaattgtgtcaccacttgaagcaccctgctttccctattcttgcatctaattgcagtacgctaccatgaaaccagttcattctgtgctcaatttgctgttctgcttaaagggacttaaacttgatacctgaaggccagttgctacgggccattacatttatttccttccaggcattgtatgtagataagcaattagatgagggaaaagaagttgagagtcatttatcatggagaaaaaaaaaaaaaaccattcaacaaggctgtacaagcaaacctatttagattgaagaaaacataacgtttaattctcagaaacaaatgcaagcctcggtccaagtcttccttcccaaacctttgtcatttagggattgagaagctgagttgggtgaaaggttgaatagaaaacaaaaaggaaagctagaaacacgctgagctcatggagatgcagcttcttctgtagctcctaaagcccagctgaggtatcatctaatgagaattctctctatgccaggcactgcgctaagcatttcacatcattaaccaatgtgagttttaggcaaccccgaagcaggcagtctgttcatcccaattgcagctgagaaacagggtgagtgaggccaagcagctggcccaaggtcccctgcctggtaagtggcacagcctgcagccctgccaggtggtcctgctaaccaagccggcgcttttctgtcaccatgccgtatcgcctcccgtactatcaaaatgtactatcaaatttacctcaaaagaaaaccctctgtcttctgagaagctccggaaggtccaacacgttgcctgtctttctgaaaagtgtcttgtctgttaatgtcatatgagcccctgtggtggtagaagaatgctataaattttggatccacagaactaaagtacgagagggaatttttcacaggaaagatggttgatacttgtccttagtatcagaacaatctccagtggattcaacagagcatctgccgttttcttgaacaaaggtttcttagggctggaacaccagtaaagcttctcttctctggaaaaagtttaggtctctgaagttttctcagtgcatcataactgacagcagcaggaatatggttttgcttttatcctggcccagacgcggctggggcggacgggacctctcgcgctctgcctcctcctcttgcttcatggagccatgcgcctgggtgggggctcccgagagaagctggcctgcgggcgggccggacgcgctgcgcggacgggacggggcgaaggaggccggcaggcggaggaggaagcggcggggcggcggcggcggcggcggccgggaagaactagaggtattccccgggcggctggaggactgagtcgagccgggacccgagtcctccggtatcccagcagccaccggaggcagtgaggtaatggaggaagaatgtagggagtcctccggtggaccacactccttctagcgagccgcggaaaccatagagatcagggctcagccggagggcc

SEQ ID NO: 17779 - RNA, 65 nt, Homo sapiens
  source 1..65: mol_type = other RNA
tcctcttctccctcctcccagctgaataggagccggtgtcagtcacgctgctccaggggagagtc

SEQ ID NO: 17780 - RNA, 4325 nt, Homo sapiens
  source 1..4325: mol_type = other RNA
tcctcttctccctcctcccaggcagagatgctcctctgtgcggcgcagtcaccacctctgggaaatccatgctcaacatctgtcttgatttcccatccttgctgggatgggtctcccaaacttctaggcccagtagggccagctgctcttctcctgggctggtatctcctctcccacagctggacagttacagcaccctccgctgaaaagccttttccagcctgaacgcggcggctatggagtcatttggatggactccttaagcctcagtctcagtgctgaatggtggtgctgccgtcagcaccagtgggcccgtcccttgctcctcctgcctctctgcctttagaccccaaggcagccactccccacgagcacttgcagagcacctcctgtgttccgggcttggttccgggcacaggggatggaggtgactgagaccctgccacaggcctccacagctttggtggcggatgagtgagtggaggggtcagagggcccctatgggggtggggcagggccgtgctcatgacctgggtgtgcagctgggcctgtggggtcatggccagtgagctccgttcatcacgggcaaccatctagtggagacgcatgtgctcagtgggtctgtgggagcagctggtacccaggcccaaggggtgggtagggaagagggtgtggggacaccccaccctgaccacccactgcaggtagctctggggtgggggcaggtgggctgagctgggccacctggcaggtgtggcgcttgccctctcccggcctctcccaggtgacctgtcgggggatttcaggtcatgtcacacatacttcccggtaggcatcctcccgactcacagccaagccagaggagggcctatggctccatcctgtcccagagagtgtgtcaggtgggaacacctaccggcaggcagacagagagcctctggggctgctcctggagagggtgggtggtctcaggggaagaggcagatactgaggccaacaacttcgggcccctgtgttttggagtctggtgcagagctgccttcccatggcccatccggtggccaggcacgaccaccaccccttgctggccttatcttttgtgggactgcccagcgggcccaggcctgcccagccaataggggccacttctgaggcatccagaatctcaggcccagtgtgcctgtgttcctggggcggtggcccaggtctgcgacgtttacttaagagctcgggtgtggcctcttggaaaacagcacccgctcacatcccgtccatccaggcctggcgcacctcttactcaagaggagaattaatccatgggcctcaggtgaaataccagcttccacccccgggactcatgtgtgcggctcccagatgtgtgagcacctgctgcgtgcagatgctgggccagctgcaaggacactgcagggtcatgcccaggggctctcctggagggggcacagtgtcttaggggggccaaacagcaggagcagaaaccacaggagcacttgaacccagatggaaaccccccccggaggctttctgccagagggggcaccggggcgaggtggaggcaccagggtaaggtggaggctgttgtagcagctctgggatctgcgccttccctgagaataaaaacacggcacacggcatttggagaacgcttgtggtttatacagcgcttgcaccgccagactctcctgggtgccccgctgggcccctgagatgggttttctggtcccagcagactcatgaatgccggtctcgggggaaaggggctccagaacgtctctgtgaattgtctcaacattcttgtgaggcaggtatgatcatccccattctacagattagaaaactgaggctcagacagctggagggctgtgttcaccgtctttgccctcgctgctccacatcccggtggccaccccagactcctccggcttttcccgggagcttttgcctggcatattttgctctcctgactttgagcacaccccaagactttccttctgctcattaccagggcagcggagggtctggggtgcaaggagagagagggaccctgtagtggctgagacatggggggggactgctccgaagcccagcagcccttggagaatgtgaccaaagccccagacctctccccggaaatgtccagggatacgtgcttgtcatacacacctttggcagccacccccagggactccaggttgagaagctctggcctgagcgagacccagactcccacccccggctgttggcaagaggtaatgaccctactagtgatgggccctcgaagcctccgtccacccctgcctccgctcaccccggccatgaccccagcctggctcacagccagatgtccatccagcagaaggtaaaggggcacctgagcccatgggcaggctctcatgggaccaccggcaacatctcagccttggagatgagagggcagccttggctgggtcagggagcggggcacatgagtgtgttccggtccagtagagatgctttcaagggcaaagctgtgcggcaccgttgttaagagagaggctttcgggatcaggaatacttggttttgaacttcagctctgctccttcccagcctccctcctcagagcttcagtttttcatttgtgaaatggggatggggaaagcacccacctcatgggcctcgctagcaggctctgggtctctggcagccacggtcacgcgtgttccccagcgtggaggtgcatctctttccatacatgcttctggcagtgttgcacagcgttgcacagcttggcggcctcctggctcctgcaccagaagcttgggcccagggcacactggtcggtgcccagcagtggggtcctggggccgtggcaggcccccaccttcttgcacacagccacggggtccatcatgtccttgagactctcaatgagcacgggctcgtactgggtgacgaagtgcttgcactggatcatatagggcagcggcaggatgctgcagccacccttgaaggccaccaggatgtctcgcttggtgctcttgctctccaagttgtgggaggacaccgtgagcagcctcttgcacccattgcagaagctgccctggttctccgcgtcccactctggggacggcacgatggcataggcatcatggactgcccgggcccgcctccggttgccacacagacggatgaacttgcacaccttctctggggtgattttggccacaagctgcaccaaggaggggctgtaggtgtccaccaagatgatgcactccttcgtgatagaggcaggcattaccgagcacacgcgctccagggcatgggtgatcatgagctcagagctgttggacatgagccagtggtccagcttctgcaccacgttcatgcacacctcacaggtcacaccggccttcatctgcatctcgctctgtttccttggcaaccccagctccagggaggggaccccgtccatggccactacttgagtcaaacgggcaggtgcccctagctcctcacagaatccccccttcctgcagagctcctgcggggggagaagcctcagtgcttggtcagcagggacaaaaaactggaagaggtagttcttgcagaggacggccaggccaggccccaaggactcacactgctcctggatgttcaagtcggccaaggtcaagttggaccggacagcctcctggagtcgggagacctgccgtacacagtcttggcacagagctccttcaggcgcctggcgggggtggaaggtaaggggcccattggccatgaacggagccacagcctcaaaggtgtcctctttggagagtggcctcagggtggccaggtgcctctgcagcggctcacagaggctgagcgctgtgcacacctgtgccggggcactgtccggggccccacggagcatgctcaggatggccgaactgtgggcatccaccatccacttgcatccggctgaagactcctggctggggagccactcacaggtcttcatcaccaaagccaggatgtcagactccgtggcgtcagggttcagcccattgccagcggcggctgctatgtcctggcatacgtcgcagggcagagacttcgcggtgggtttgttccatacggccccttggcagtaccccacagccccgcacctggcagctgtctgcagatcctgacaccacaccgtggagccctttgcacactcctgggggcctgaggtggggctggccctggtggcccccaggaggctgggcaggaggagcagggcacacagcatgctgcccagggactctctggctccagagtacccagcagtggctgctgctat

SEQ ID NO: 17781 - RNA, 2550 nt, Homo sapiens
  source 1..2550: mol_type = other RNA
tcctgccttcctctgcaccagtagcctgcatagatgcaatgatggcttctaccctctgagatttttctagtagacgcctgtcaaacaaacacaactctgagacatcttccctaacctgggagattctcttaccacgtgtgtctgaggcactacccaccaccctttaccattttcctgatcaaagtagataatgtcaccttctaaggacattttctacaaacttatttggaaatataacttcactcctgaaattcttattgcctctcatttgcacttaaaagtttggtgcttttgtacgtttctcacaaatttaatctgaaaaattatttcactgggagcatgttagaaaagtgtagactaatgcatgatttacactaatctaagccaatgattcaatgcaagtagactggttgctatctctactggttcctacttctcaaaaaaaaaatttttttttttgagatggagtctcactttgtcgcccaggctggagtgcagtggcgtgatcttggttcactgcaacctccactcactgggtttaagtgattctcctgccttagcctcccgagtagctgggactataggtgcccgccaccatgcccagctaatttttgtatttttagtgaagacagggtttcaccatgttggccaggttggtctcaaactcctgacctcaagtgatccacctgcctcagcctcccgaagtgctgggattacaggcatgagccaccctgccaggcccagcgtctattgattcctatttctagaggaaatttcccctgaggcccttgatcttgaaagatgtaaataactcaactgaaaatgttacttacttattctctttggtttcaaattgcctcctttctatcaagttggctatgctctgaggaaagagaagacagacaaggaatgcacatagttctatttcagcagctcagggcgaagtgggcacatgaggggtacttgaccgtatggaggaaatggggagaaggtccagattgagttaccttgtagcacctgtgcaacaacattcgggcagctgacaggatgttcacagtatataaatagaaggtcctggatggggcatggtctggtgttttgggaatttcctggagtgacatgaaattttctgagagcatcttatatagcatatcctttgcctcctttgcaggaatcattgcaaagtcttccacttgcttctgctctatgtgtttcttctgcaaaactagacggaatattctagcacagcgagacccaaattggatcatctgccagcagagtgagatactgatcaagaacttgcttagagatgttatagccaacaggtagggatctgaagatctcattggaagacaatggctgggtgaagggagcactagaggaagtggtaatctcactcattcggagcatggttcgcacaatctcgctgcttgtctgtttgaaaagtaaactggtccatcctgttagcaactgcgctcacaatggcttggtcacggaagtgttggtggaatctgtcaaggttggcctgccaataaatcccatcatctggaatgggctccttgttatctgtagtatattttggtctcttggccttgggctccccagcagcatcttcatcagatgatctcctccttttacctttccctatcaagctgagtttaggaaccaggtacatgtccttttcattaatgacaagtgtgggggcaggtggtggtggcccagggtctgaattctcagtggtaggtaccgaagggcagcgttgtacaaagtgtgtgtctgccagtcgcacaaatgtgtttgatacttcagcatagtccatggtcttgccatcctccatggtctctgtgagccggtctgccactttcttcacaacagctgacattgtcagtttgccgttcaacagaagctcctcaacaatcagctctccagtgtcactgtacagagttttggtagtatagatgtaccggggatatctaagcattcgcaatacccggctgcactgggcttcatactccaccacaccacgtttgtgcacttgataactcaccaggttatgttggacgaggacacacagggctttcttcacctgatccagtgatgttcctgtgtcatgggcaattactcttagtggctggctgccggttcttatcagatggactccaattttttctacaatctctccaaaatgctcttgcagcaacaaagaacagagcttaatttctgcttgagtcattgtactggggagtctgagagctcagggtcagcgcaatccgggggctccaactccaattcggctgagcttcccgcgacggcttcctacggctcccgctggccttctaggccgaggtggagcccaccgccctttctaggacgcggatcgccaccgaagaagacgcggaaaagcaaaaagcgcgtgccactctaccccagagtttcggcggcttccggggacgctctttctttcttctcgctggaagactggaggaccagcgaggggctgtttgtggagccggcgggcgggccgtttgtctctccttcctgcgcctcttt

SEQ ID NO: 17782 - RNA, 1338 nt, Homo sapiens
  source 1..1338: mol_type = other RNA
tcctgccttcctctgcaccagtagcctgcatagatgcaatgatggcttctaccctctgagatttttctagtagacgcttattctctttggtttcaaattgcctcctttctatcaagttggctatgctcttgtagcacctgtgcaacaacattcgggcagctgacaggatgttcacagtatataaatagaaggtcctggatggggcatggtctggtgttttgggaatttcctggagtgacatgaaattttctgagagcatcttatatagcatatcctttgcctcctttgcaggaatcattgcaaagtcttccacttgcttctgctctatgtgtttcttctgcaaaactagacggaatattctagcacagcgagacccaaatctcattggaagacaatggctgggtgaagggagcactagaggaagtggtaatctcactcattcggagcatggttcgcacaatctcgctgcttgtctggtccatcctgttagcaactgcgctcacaatggcttggtcacggaagtgttggtggaatctgtcaaggttggcctgccaataaatcccatcatctggaatgggctccttgttatctgtagtatattttggtctcttggccttgggctccccagcagcatcttcatcagatgatctcctccttttacctttccctatcaagctgagtttaggaaccaggtacatgtccttttcattaatgacaagtgtgggggcaggtggtggtggcccagggtctgaattctcagtggtaggtaccgaagggcagcgttgtacaaagtgtgtgtctgccagtcgcacaaatgtgtttgatacttcagcatagtccatggtcttgccatcctccatggtctctgtgagccggtctgccactttcttcacaacagctgacattgtcagtttgccgttcaacagaagctcctcaacaatcagctctccagtgtcactgtacagagttttggtagtatagatgtaccggggatatctaagcattcgcaatacccggctgcactgggcttcatactccaccacaccacgtttgtgcacttgataactcaccaggttatgttggacgaggacacacagggctttcttcacctgatccagtgatgttcctgtgtcatgggcaattactcttagtggctggctgccggttcttatcagatggactccaattttttctacaatctctccaaaatgctcttgcagcaacaaagaacagagcttaatttctgcttgagtcattgtactggggagtctgagagctatttcgtccatccacatatctttggagaagcattcccagatcctttgccatcctcggaaa

SEQ ID NO: 17783 - RNA, 1570 nt, Homo sapiens
  source 1..1570: mol_type = other RNA
tcctgccttcctctgcaccagtagcctgcatagatgcaatgatggcttctaccctctgagatttttctagtagacgcttattctctttggtttcaaattgcctcctttctatcaagttggctatgctcttgtagcacctgtgcaacaacattcgggcagctgacaggatgttcacagtatataaatagaaggtcctggatggggcatggtctggtgttttgggaatttcctggagtgacatgaaattttctgagagcatcttatatagcatatcctttgcctcctttgcaggaatcattgcaaagtcttccacttgcttctgctctatgtgtttcttctgcaaaactagacggaatattctagcacagcgagacccaaatctcattggaagacaatggctgggtgaagggagcactagaggaagtggtaatctcactcattcggagcatggttcgcacaatctcgctgcttgtctggtccatcctgttagcaactgcgctcacaatggcttggtcacggaagtgttggtggaatctgtcaaggttggcctgccaataaatcccatcatctggaatgggctccttgttatctgtagtatattttggtctcttggccttgggctccccagcagcatcttcatcagatgatctcctccttttacctttccctatcaagctgagtttaggaaccaggtacatgtccttttcattaatgacaagtgtgggggcaggtggtggtggcccagggtctgaattctcagtggtaggtaccgaagggcagcgttgtacaaagtgtgtgtctgccagtcgcacaaatgtgtttgatacttcagcatagtccatggtcttgccatcctccatggtctctgtgagccggtctgccactttcttcacaacagctgacattgtcagtttgccgttcaacagaagctcctcaacaatcagctctccagtgtcactgtacagagttttggtagtatagatgtaccggggatatctaagcattcgcaatacccggctgcactgggcttcatactccaccacaccacgtttgtgcacttgataactcaccaggttatgttggacgaggacacacagggctttcttcacctgatccagtgatgttcctgtgtcatgggcaattactcttagtggctggctgccggttcttatcagatggactccaattttttctacaatctctccaaaatgctcttgcagcaacaaagaacagagcttaatttctgcttgagtcattgtactggggagtctgagagctcagggtcagcgcaatccgggggctccaactccaattcggctgagcttcccgcgacggcttcctacggctcccgctggccttctaggccgaggtggagcccaccgccctttctaggacgcggatcgccaccgaagaagacgcggaaaagcaaaaagcgcgtgccactctaccccagagtttcggcggcttccggggacgctctttctttcttctcgctggaagactggaggaccagcgaggggctgtttgtggagccggcgggcgggccgtttgtctctccttcctgcgcctc

SEQ ID NO: 17784 - RNA, 2023 nt, Homo sapiens
  source 1..2023: mol_type = other RNA
tcctgccttcctctgcaccagtagcctgcatagatgcaatgatggcttctaccctctgagatttttctagtagacgcttattctctttggtttcaaattgcctcctttctatcaagttggctatgctcttgtagcacctgtgcaacaacattcgggcagctgacaggatgttcacagtatataaatagaaggtcctggatggggcatggtctggtgttttgggaatttcctggagtgacatgaaattttctgagagcatcttatatagcatatcctttgcctcctttgcaggaatcattgcaaagtcttccacttgcttctgctctatgtgtttcttctgcaaaactagacggaatattctagcacagcgagacccaaatctctcctgtacgacggactccagagtggctgtggctagggatgctaatgccttatggaggttgatgacatacattcctccaccactgtcgccagactttccaacaaactctagctattaagaaaaagagagagtgttaactgaacggaaagtccagtgattctgtttccaatggaacaaatctgaccaaaagtctgcagcaggtagccctcctatcaaatgatgtggagaaattgtctgggctggctaggtagagaataactctgcaggaggatgacactaggtatcagtgcagaaataaattatcaacagtacaggctaaagaaaaaagaaaaaaagcaaaaacagacttactggatcatctgccagcagagtgagatactgatcaagaacttgcttagagatgttatagccaacaggtagggatctgaagatctcattggaagacaatggctgggtgaagggagcactagaggaagtggtaatctcactcattcggagcatggttcgcacaatctcgctgcttgtctgtttgaaaagtaaactggtccatcctgttagcaactgcgctcacaatggcttggtcacggaagtgttggtggaatctgtcaaggttggcctgccaataaatcccatcatctggaatgggctccttgttatctgtagtatattttggtctcttggccttgggctccccagcagcatcttcatcagatgatctcctccttttacctttccctatcaagctgagtttaggaaccaggtacatgtccttttcattaatgacaagtgtgggggcaggtggtggtggcccagggtctgaattctcagtggtaggtaccgaagggcagcgttgtacaaagtgtgtgtctgccagtcgcacaaatgtgtttgatacttcagcatagtccatggtcttgccatcctccatggtctctgtgagccggtctgccactttcttcacaacagctgacattgtcagtttgccgttcaacagaagctcctcaacaatcagctctccagtgtcactgtacagagttttggtagtatagatgtaccggggatatctaagcattcgcaatacccggctgcactgggcttcatactccaccacaccacgtttgtgcacttgataactcaccaggttatgttggacgaggacacacagggctttcttcacctgatccagtgatgttcctgtgtcatgggcaattactcttagtggctggctgccggttcttatcagatggactccaattttttctacaatctctccaaaatgctcttgcagcaacaaagaacagagcttaatttctgcttgagtcattgtactggggagtctgagagctcagggtcagcgcaatccgggggctccaactccaattcggctgagcttcccgcgacggcttcctacggctcccgctggccttctaggccgaggtggagcccaccgccctttctaggacgcggatcgccaccgaagaagacgcggaaaagcaaaaagcgcgtgccactctaccccagagtttcggcggcttccggggacgctctttctttcttctcgctggaagactggaggaccagcgaggggctgtttgtggagccggcgggcgggccgtttgtctctccttcctgcgcctcttt

SEQ ID NO: 17785 - RNA, 1460 nt, Homo sapiens
  source 1..1460: mol_type = other RNA
tcctgccttcctctgcaccagtagcctgcatagatgcaatgatggcttctaccctctgagatttttctagtagacgcttattctctttggtttcaaattgcctcctttctatcaagttggctatgctcttgtagcacctgtgcaacaacattcgggcagctgacaggatgttcacagtatataaatagaaggtcctggatggggcatggtctggtgttttgggaatttcctggagtgacatgaaattttctgagagcatcttatatagcatatcctttgcctcctttgcaggaatcattgcaaagtcttccacttgcttctgctctatgtgtttcttctgcaaaactagacggaatattctagcacagcgagacccaaatctctcctgtacgacggactccagagtggctgtggctagggatgctaatgccttatggaggttgatgacatacattcctccaccactgtcgccagactttccaacaaactctagtggatcatctgccagcagagtgagatactgatcaagaacttgcttagagatgttatagccaacaggtagggatctgaagatctcattggaagacaatggctgggtgaagggagcactagaggaagtggtaatctcactcattcggagcatggttcgcacaatctcgctgcttgtctggtccatcctgttagcaactgcgctcacaatggcttggtcacggaagtgttggtggaatctgtcaaggttggcctgccaataaatcccatcatctggaatgggctccttgttatctgtagtatattttggtctcttggccttgggctccccagcagcatcttcatcagatgatctcctccttttacctttccctatcaagctgagtttaggaaccaggtacatgtccttttcattaatgacaagtgtgggggcaggtggtggtggcccagggtctgaattctcagtggtaggtaccgaagggcagcgttgtacaaagtgtgtgtctgccagtcgcacaaatgtgtttgatacttcagcatagtccatggtcttgccatcctccatggtctctgtgagccggtctgccactttcttcacaacagctgacattgtcagtttgccgttcaacagaagctcctcaacaatcagctctccagtgtcacaggttatgttggacgaggacacacagggctttcttcacctgatccagtgatgttcctgtgtcatgggcaattactcttagtggctggctgccggttcttatcagatggactccaattttttctacaatctctccaaaatgctcttgcagcaacaaagaacagagcttaatttctgcttgagtcattgtactggggagtctgagagctatttcgtccatccacatatctttggagaagcattcccagatcctttgccatcctcggaaagggcttccaaggcgcttggctcctagctctacacttccttt

SEQ ID NO: 17786 - RNA, 2544 nt, Homo sapiens
  source 1..2544: mol_type = other RNA
tcctgccttcctctgcaccagtagcctgcatagatgcaatgatggcttctaccctctgagatttttctagtagacgcttattctctttggtttcaaattgcctcctttctatcaagttggctatgctcttgtagcacctgtgcaacaacattcgggcagctgacaggatgttcacagtatataaatagaaggtcctggatggggcatggtctggtgttttgggaatttcctggagtgacatgaaattttctgagagcatcttatatagcatatcctttgcctcctttgcaggaatcattgcaaagtcttccacttgcttctgctctatgtgtttcttctgcaaaactagacggaatattctagcacagcgagacccaaatctctcctgtacgacggactccagagtggctgtggctagggatgctaatgccttatggaggttgatgacatacattcctccaccactgtcgccagactttccaacaaactctagtggatcatctgccagcagagtgagatactgatcaagaacttgcttagagatgttatagccaacaggtagggatctgaagatctcattggaagacaatggctgggtgaagggagcactagaggaagtggtaatctcactcattcggagcatggttcgcacaatctcgctgcttgtctggtccatcctgttagcaactgcgctcacaatggcttggtcacggaagtgttggtggaatctgtcaaggttggcctgccaataaatcccatcatctggaatgggctccttgttatctgtagtatattttggtctcttggccttgggctccccagcagcatcttcatcagatgatctcctccttttacctttccctatcaagctgagtttaggaaccaggtacatgtccttttcattaatgacaagtgtgggggcaggtggtggtggcccagggtctgaattctcagtggtaggtaccgaagggcagcgttgtacaaagtgtgtgtctgccagtcgcacaaatgtgtttgatacttcagcatagtccatggtcttgccatcctccatggtctctgtgagccggtctgccactttcttcacaacagctgacattgtcagtttgccgttcaacagaagctcctcaacaatcagctctccagtgtcacaggttatgttggacgaggacacacagggctttcttcacctgatccagtgatgttcctgtgtcatgggcaattactcttagtggctggctgccggttcttatcagatggactccaattttttctacaatctctccaaaatgctcttgcagcaacaaagaacagagcttaatttctgcttgagtcattgtactggggagtctgagagctcagggtcagcgcaatccgggggctccaactccaattcggctgagcttcccgcgacggcttcctacggctcccgctggccttctaggccgaggtggagcccaccgccctttctaggacgcggatcgccaccgaagaagacgcggaaaagcaaaaagcgcgtgccactctaccccagagtttcggcggcttccggggacgctctttctttcttctcgctggaagactggaggaccagcgaggggctgtttgtggagccggcgggcgggccgtttgtctctccttcctgcgcctctttggtgctgggaggcgggccgcagggtagctgttggcgccgccgcgtttctgggcctggccaactcacgtgaccgacgcgggctctgaagcggtgggccgcaccgaggcggcggcggcggcgacgactgcagctcgggaggtagcggcctggcgagggacgggccggctgccctctcggacggccgcggcggagggcaaaaatggcggaggcttcggcggccggggcggactcgggcgccgctgtagccgcccaccggtttttctgccacttttgcaagggcgaggtcagccccaaactaccggtaagagcgctgtgttctctatacttgggaacctcatagattcctggccccgatttcccggaactgggtctggagctttctgcacatcattgactcgcccgacatcggtctgccgaatacctgctgcccacttctaagccgccggccctaaaccctgggcatcacggcctcggccccgtacctcctgcccacctcttaattcatcctgggctgctccacctgacctcacctctttacctcccgtgtccttaatttttttttttcttagcaagtttccctctgataactctcccctcaattttcttgcattcttttatacctggtctttttcctacgatgacctccccccacacttcttccactgtgtcttctcaccttcctctgtgttcttttccacttttcaccccccaccgcccccgccacctcccttgtcagtgaagcgaaatagcggattgctgaggattgtcactcttcggttttttctagggaaggaagcacagaaagggggttggaaggtatctgtggggcgaaaagggggattttgctcttcagtggtttccagggtccttgtgacagtgaagacagcagc

SEQ ID NO: 17787 - RNA, 1573 nt, Homo sapiens
  source 1..1573: mol_type = other RNA
tcctgccttcctctgcaccagtagcctgcatagatgcaatgatggcttctaccctctgagatttttctagtagacgcttattctctttggtttcaaattgcctcctttctatcaagttggctatgctcttgtagcacctgtgcaacaacattcgggcagctgacaggatgttcacagtatataaatagaaggtcctggatggggcatggtctggtgttttgggaatttcctggagtgacatgaaattttctgagagcatcttatatagcatatcctttgcctcctttgcaggaatcattgcaaagtcttccacttgcttctgctctatgtgtttcttctgcaaaactagacggaatattctagcacagcgagacccaaatctctcctgtacgacggactccagagtggctgtggctagggatgctaatgccttatggaggttgatgacatacattcctccaccactgtcgccagactttccaacaaactctagtggatcatctgccagcagagtgagatactgatcaagaacttgcttagagatgttatagccaacaggtagggatctgaagatctcattggaagacaatggctgggtgaagggagcactagaggaagtggtaatctcactcattcggagcatggttcgcacaatctcgctgcttgtctggtccatcctgttagcaactgcgctcacaatggcttggtcacggaagtgttggtggaatctgtcaaggttggcctgccaataaatcccatcatctggaatgggctccttgttatctgtagtatattttggtctcttggccttgggctccccagcagcatcttcatcagatgatctcctccttttacctttccctatcaagctgagtttaggaaccaggtacatgtccttttcattaatgacaagtgtgggggcaggtggtggtggcccagggtctgaattctcagtggtaggtaccgaagggcagcgttgtacaaagtgtgtgtctgccagtcgcacaaatgtgtttgatacttcagcatagtccatggtcttgccatcctccatggtctctgtgagccggtctgccactttcttcacaacagctgacattgtcagtttgccgttcaacagaagctcctcaacaatcagctctccagtgtcactgtacagagttttggtagtatagatgtaccggggatatctaagcattcgcaatacccggctgcactgggcttcatactccaccacaccacgtttgtgcacttgataactcaccaggttatgttggacgaggacacacagggctttcttcacctgatccagtgatgttcctgtgtcatgggcaattactcttagtggctggctgccggttcttatcagatggactccaattttttctacaatctctccaaaatgctcttgcagcaacaaagaacagagcttaatttctgcttgagtcattgtactggggagtctgagagctatttcgtccatccacatatctttggagaagcattcccagatcctttgccatcctcggaaagggcttccaaggcgcttggctcctagctctacacttccttt

SEQ ID NO: 17788 - RNA, 1640 nt, Homo sapiens
  source 1..1640: mol_type = other RNA
tcctgccttcctctgcaccagtagcctgcatagatgcaatgatggcttctaccctctgagatttttctagtagacgcttattctctttggtttcaaattgcctcctttctatcaagttggctatgctcttgtagcacctgtgcaacaacattcgggcagctgacaggatgttcacagtatataaatagaaggtcctggatggggcatggtctggtgttttgggaatttcctggagtgacatgaaattttctgagagcatcttatatagcatatcctttgcctcctttgcaggaatcattgcaaagtcttccacttgcttctgctctatgtgtttcttctgcaaaactagacggaatattctagcacagcgagacccaaatctctcctgtacgacggactccagagtggctgtggctagggatgctaatgccttatggaggttgatgacatacattcctccaccactgtcgccagactttccaacaaactctagtggatcatctgccagcagagtgagatactgatcaagaacttgcttagagatgttatagccaacaggtagggatctgaagatctcattggaagacaatggctgggtgaagggagcactagaggaagtggtaatctcactcattcggagcatggttcgcacaatctcgctgcttgtctggtccatcctgttagcaactgcgctcacaatggcttggtcacggaagtgttggtggaatctgtcaaggttggcctgccaataaatcccatcatctggaatgggctccttgttatctgtagtatattttggtctcttggccttgggctccccagcagcatcttcatcagatgatctcctccttttacctttccctatcaagctgagtttaggaaccaggtacatgtccttttcattaatgacaagtgtgggggcaggtggtggtggcccagggtctgaattctcagtggtaggtaccgaagggcagcgttgtacaaagtgtgtgtctgccagtcgcacaaatgtgtttgatacttcagcatagtccatggtcttgccatcctccatggtctctgtgagccggtctgccactttcttcacaacagctgacattgtcagtttgccgttcaacagaagctcctcaacaatcagctctccagtgtcactgtacagagttttggtagtatagatgtaccggggatatctaagcattcgcaatacccggctgcactgggcttcatactccaccacaccacgtttgtgcacttgataactcaccaggttatgttggacgaggacacacagggctttcttcacctgatccagtgatgttcctgtgtcatgggcaattactcttagtggctggctgccggttcttatcagatggactccaattttttctacaatctctccaaaatgctcttgcagcaacaaagaacagagcttaatttctgcttgagtcattgtactggggagtctgagagctcagggtcagcgcaatccgggggctccaactccaattcggctgagcttcccgcgacggcttcctacggctcccgctggccttctaggccgaggtggagcccaccgccctttctaggacgcggatcgccaccgaagaagacgcggaaaagcaaaaagcgcgtgccactct

SEQ ID NO: 17789 - RNA, 1548 nt, Homo sapiens
  source 1..1548: mol_type = other RNA
tcctgccttcctctgcaccagtagcctgcatagatgcaatgatggcttctaccctctgagatttttctagtagacgcttattctctttggtttcaaattgcctcctttctatcaagttggctatgctcttgtagcacctgtgcaacaacattcgggcagctgacaggatgttcacagtatataaatagaaggtcctggatggggcatggtctggtgttttgggaatttcctggagtgacatgaaattttctgagagcatcttatatagcatatcctttgcctcctttgcaggaatcattgcaaagtcttccacttgcttctgctctatgtgtttcttctgcaaaactagacggaatattctagcacagcgagacccaaatctctcctgtacgacggactccagagtggctgtggctagggatgctaatgccttatggaggttgatgacatacattcctccaccactgtcgccagactttccaacaaactctagtggatcatctgccagcagagtgagatactgatcaagaacttgcttagagatgttatagccaacaggtagggatctgaagatctcattggaagacaatggctgggtgaagggagcactagaggaagtggtaatctcactcattcggagcatggttcgcacaatctcgctgcttgtctgtttgaaaagtaaactggtccatcctgttagcaactgcgctcacaatggcttggtcacggaagtgttggtggaatctgtcaaggttggcctgccaataaatcccatcatctggaatgggctccttgttatctgtagtatattttggtctcttggccttgggctccccagcagcatcttcatcagatgatctcctccttttacctttccctatcaagctgagtttaggaaccaggtacatgtccttttcattaatgacaagtgtgggggcaggtggtggtggcccagggtctgaattctcagtggtaggtaccgaagggcagcgttgtacaaagtgtgtgtctgccagtcgcacaaatgtgtttgatacttcagcatagtccatggtcttgccatcctccatggtctctgtgagccggtctgccactttcttcacaacagctgacattgtcagtttgccgttcaacagaagctcctcaacaatcagctctccagtgtcactgtacagagttttggtagtatagatgtaccggggatatctaagcattcgcaatacccggctgcactgggcttcatactccaccacaccacgtttgtgcacttgataactcaccaggttatgttggacgaggacacacagggctttcttcacctgatccagtgatgttcctgtgtcatgggcaattactcttagtggctggctgccggttcttatcagatggactccaattttttctacaatctctccaaaatgctcttgcagcaacaaagaacagagcttaatttctgcttgagtcattgtactggggagtctgagagctatttcgtccatccacatatctttggagaagcattcccagatcctttgccatcctcggaaa

SEQ ID NO: 17790 - RNA, 1419 nt, Homo sapiens
  source 1..1419: mol_type = other RNA
tcctgccttcctctgcaccagtagcctgcatagatgcaatgatggcttctaccctctgagatttttctagtagacgcttattctctttggtttcaaattgcctcctttctatcaagttggctatgctcttgtagcacctgtgcaacaacattcgggcagctgacaggatgttcacagtatataaatagaaggtcctggatggggcatggtctggtgttttgggaatttcctggagtgacatgaaattttctgagagcatcttatatagcatatcctttgcctcctttgcaggaatcattgcaaagtcttccacttgcttctgctctatgtgtttcttctgcaaaactagacggaatattctagcacagcgagacccaaattggatcatctgccagcagagtgagatactgatcaagaacttgcttagagatgttatagccaacaggtagggatctgaagatctcattggaagacaatggctgggtgaagggagcactagaggaagtggtaatctcactcattcggagcatggttcgcacaatctcgctgcttgtctggtccatcctgttagcaactgcgctcacaatggcttggtcacggaagtgttggtggaatctgtcaaggttggcctgccaataaatcccatcatctggaatgggctccttgttatctgtagtatattttggtctcttggccttgggctccccagcagcatcttcatcagatgatctcctccttttacctttccctatcaagctgagtttaggaaccaggtacatgtccttttcattaatgacaagtgtgggggcaggtggtggtggcccagggtctgaattctcagtggtaggtaccgaagggcagcgttgtacaaagtgtgtgtctgccagtcgcacaaatgtgtttgatacttcagcatagtccatggtcttgccatcctccatggtctctgtgagccggtctgccactttcttcacaacagctgacattgtcagtttgccgttcaacagaagctcctcaacaatcagctctccagtgtcactgtacagagttttggtagtatagatgtaccggggatatctaagcattcgcaatacccggctgcactgggcttcatactccaccacaccacgtttgtgcacttgataactcaccaggttatgttggacgaggacacacagggctttcttcacctgatccagtgatgttcctgtgtcatgggcaattactcttagtggctggctgccggttcttatcagatggactccaattttttctacaatctctccaaaatgctcttgcagcaacaaagaacagagcttaatttctgcttgagtcattgtactggggagtctgagagctatttcgtccatccacatatctttggagaagcattcccagatcctttgccatcctcggaaa

SEQ ID NO: 17791 - RNA, 1639 nt, Homo sapiens
  source 1..1639: mol_type = other RNA
tcctgccttcctctgcaccagtagcctgcatagatgcaatgatggcttctaccctctgagatttttctagtagacgcttattctctttggtttcaaattgcctcctttctatcaagttggctatgctcttgtagcacctgtgcaacaacattcgggcagctgacaggatgttcacagtatataaatagaaggtcctggatggggcatggtctggtgttttgggaatttcctggagtgacatgaaattttctgagagcatcttatatagcatatcctttgcctcctttgcaggaatcattgcaaagtcttccacttgcttctgctctatgtgtttcttctgcaaaactagacggaatattctagcacagcgagacccaaattggatcatctgccagcagagtgagatactgatcaagaacttgcttagagatgttatagccaacaggtagggatctgaagatctcattggaagacaatggctgggtgaagggagcactagaggaagtggtaatctcactcattcggagcatggttcgcacaatctcgctgcttgtctggtccatcctgttagcaactgcgctcacaatggcttggtcacggaagtgttggtggaatctgtcaaggttggcctgccaataaatcccatcatctggaatgggctccttgttatctgtagtatattttggtctcttggccttgggctccccagcagcatcttcatcagatgatctcctccttttacctttccctatcaagctgagtttaggaaccaggtacatgtccttttcattaatgacaagtgtgggggcaggtggtggtggcccagggtctgaattctcagtggtaggtaccgaagggcagcgttgtacaaagtgtgtgtctgccagtcgcacaaatgtgtttgatacttcagcatagtccatggtcttgccatcctccatggtctctgtgagccggtctgccactttcttcacaacagctgacattgtcagtttgccgttcaacagaagctcctcaacaatcagctctccagtgtcactgtacagagttttggtagtatagatgtaccggggatatctaagcattcgcaatacccggctgcactgggcttcatactccaccacaccacgtttgtgcacttgataactcaccaggttatgttggacgaggacacacagggctttcttcacctgatccagtgatgttcctgtgtcatgggcaattactcttagtggctggctgccggttcttatcagatggactccaattttttctacaatctctccaaaatgctcttgcagcaacaaagaacagagcttaatttctgcttgagtcattgtactggggagtctgagagctcagggtcagcgcaatccgggggctccaactccaattcggctgagcttcccgcgacggcttcctacggctcccgctggccttctaggccgaggtggagcccaccgccctttctaggacgcggatcgccaccgaagaagacgcggaaaagcaaaaagcgcgtgccactctaccccagagtttcggcggcttccggggacgctctttctttcttctcgctggaagactggaggaccagcgaggggctgtttgtggagccggcgggcgggccgtttgtctctcc

SEQ ID NO: 17792 - RNA, 101 nt, Homo sapiens
  source 1..101: mol_type = other RNA
tcctgtactgagctgccccgagactaccccaccaaagtcttcttggtggcgaccacccaagcaccacgacgccggcaccctgacaggaccataacagtgac

SEQ ID NO: 17793 - RNA, 65 nt, Homo sapiens
  source 1..65: mol_type = other RNA
tcctgtactgagctgccccgagctgggcagcatgaagggcctcggggcagctcagtacaggatgc

SEQ ID NO: 17794 - RNA, 62 nt, Homo sapiens
  source 1..62: mol_type = other RNA
tcctgtactgagctgccccgaggcccttcatgctgcccagctcggggcagctcagtacagga

SEQ ID NO: 17795 - RNA, 778 nt, Homo sapiens
  source 1..778: mol_type = other RNA
tccttcattccaccggagtctgaggagtgggagctccgagaagcaccagtccctgcggtggagacgtcagagctgccaggggagggggctcctgcgccacagctgccggggtggtaggggctggcttgctgaccgtcgtccagcagctcctgggcaaaggggctgccctggtcaaagggccctgggtctagggcctcctggaaggccatgccatccttctccagcagctcaatgatccaactgagctcatcagaagagctggaagtgaggtctcgcagctgggcatggagttggtcccccagaggcccaaagaccagacgcagctcctcaagggcacaattgcagagggtggcgccatccatgtcacatcgtgagaagtcaatggcgcttgcgtcgtacttgttcttctccacttggtagctgatccagtccagaacctgcgtcttcgaccagaactggggctgttcccccaaccagctggccttctctgtaccctccaatgacatctgggggttgctcagggtcagtaccaagtcatcggccccaaaggtggcagcagggggaacagaggccagggtggagtcctccgagctgtacatcgcactgaagtagttgctaaaaatgttgctaatctcacaggttgcagccatgaggctaccggagtggcggagtccggctgtggcaggcaggccggcaggcgggagagaaatccagttccgccaggtagcgctgaggtatctggccgctgcgctcccctacccggctctaaatagagcct

SEQ ID NO: 17796 - RNA, 892 nt, Homo sapiens
  source 1..892: mol_type = other RNA
tccttcattccaccggagtctgaggagtgggagctccgagaagcaccagtccctgcggtggagacgtcagagctgccaggggagggggctcctgcgccacagctgccggggtggtaggggctggcttgctgaccgtcgtccagcagctcctgggcaaaggggctgccctggtcaaagggccctgggtctagggcctcctggaaggccatgccatccttctccagcagctcaatgatccaactgagctcatcagaagagctggaagtgaggtctcgcagctgggcatggagttggtcccccagaggcccaaagaccagacgcagctcctcaagggcacaattgcagagggtggcgccatccatgtcacatcgtgagaagtcaatggcgcttgcgtcgtacttgttcttctccacttggtagctgatccagtccagaacctgcgtcttcgaccagaactggggctgttcccccaaccagctggccttctctgtaccctccaatgacatctgggggttgctcagggtcagtaccaagtcatcggccccaaaggtggcagcagggggaacagaggccagggtggagtcctccgagctgtacatcgcactgaagtagttgctaaaaatgttgctaatctcacaggttgcagccatgaggctacgctcttgctcggagatcctagactggagtgtgcaggttcagaactgcaaatcctctggacccctctgcagtttcccaagagctgggctagggaatgacaggcggggaatcctaccggagtggcggagtccggctgtggcaggcaggccggcaggcgggagagaaatccagttccgccaggtagcgctgaggtatctggccgctgcgctcccctacccggctctaaatagagcct

SEQ ID NO: 17797 - RNA, 878 nt, Homo sapiens
  source 1..878: mol_type = other RNA
tccttcattccaccggagtctgaggagtgggagctccgagaagcaccagtccctggggggcggggtcagagtaagtcccctgccggcccaccctctgctcaaccacgctgctggctctcaggacacacttcccagcctgttcctgttcctgcggtggagacgtcagagctgccaggggagggggctcctgcgccacagctgccggggtggtaggggctggcttgctgaccgtcgtccagcagctcctgggcaaaggggctgccctggtcaaagggccctgggtctagggcctcctggaaggccatgccatccttctccagcagctcaatgatccaactgagctcatcagaagagctggaagtgaggtctcgcagctgggcatggagttggtcccccagaggcccaaagaccagacgcagctcctcaagggcacaattgcagagggtggcgccatccatgtcacatcgtgagaagtcaatggcgcttgcgtcgtacttgttcttctccacttggtagctgatccagtccagaacctgcgtcttcgaccagaactggggctgttcccccaaccagctggccttctctgtaccctccaatgacatctgggggttgctcagggtcagtaccaagtcatcggccccaaaggtggcagcagggggaacagaggccagggtggagtcctccgagctgtacatcgcactgaagtagttgctaaaaatgttgctaatctcacaggttgcagccatgaggctaccggagtggcggagtccggctgtggcaggcaggccggcaggcgggagagaaatccagttccgccaggtagcgctgaggtatctggccgctgcgctcccctacccggctctaaatagagcctggag

SEQ ID NO: 17798 - RNA, 574 nt, Homo sapiens
  source 1..574: mol_type = other RNA
tccttctgctccgtcccccaggacagagcctggaatgatgcagccaatcacagagtgacttatcacctttctgtgttctatgggcaaggtagcaggacttgggaaacactttgggctttcgacatcgacactgacaaagcatgagaacaagtccacagggcccagcagtgaaccaacctgctctggggccaggccagggctgaggtcatcctgtgacactgggggccagagagcggccttggccttgctccccaccctgcctccaagcccctgtctgcctctgggctgccagcctccacctgcctgcgacggtggccccggggtgatggcctggctgtgccccatgcacaggtggttcgttaggcactcggcggctattattaacccagcagtgacgtcaccggcagccaatgggaggcaggtttatttccagggctgacagcttgatagcggttaattttagctgcatcttctttcccgaggctcgtgaaaccctagccagccaaagaaggggttgcctgtgtctccccaaacagctcagggatgggtcctgggggctctgggaggcggcaag

SEQ ID NO: 17799 - RNA, 303 nt, Homo sapiens
  source 1..303: mol_type = other RNA
tcgacagcacgacactgccttcattacttcagttgaaatcgtctccaggtacctctgcgcgcgggggtcgggccgggcggggcatcacggccctggtcgtgccaggcctgcggtggcaacctcggctttccctgctcaggagcctcgtgtctttctccgcagcgctttgccagccggccggctttccccttccaccacacacctccacccttctctctgtaagctcggccgctgctaggagtcgcctctcttttcttccttcttttccctgtcttcccttcctcttttatctcttctttcttt

SEQ ID NO: 17800 - RNA, 2142 nt, Homo sapiens
  source 1..2142: mol_type = other RNA
tcgaggagctcacagtctaacgctgtctatgtcgattaggctgctgtgccgtcggttcccttcttggtctagcagagccttcagctccttgatctgctcagccaactccgggttcaagtcaaactccgctgggaaggcggagatccagtacctgaccaggtggcacgttttcacctgcagggaattggagttgtccttccgggattgttggtagatgtggagcagcttggccgccagcgaaggcttcgatgcacccgcggagcagctcctccaccgtgcagcccttgtccaggtccagggtgcctgccatggccgccggcgcggggtgggctgggcccaggctgcgctccgggagcctcccaccgggctcggaccgaacccctgtcccgggagaggcagagcgggagtctgcggagtcgcgggcgggggagcggccccgcgggcagaaacggggcggggcgggcacgccccctgctggacaggggcggagttgtcccccgcggccactcccggggttaaacggtctggcccgggatggtgcaacccgccagttgggaaacggacccgcagagaggcttccggcccaccctcggagtcgcgggaaggccgaggggcttcacgaggatggggacgaaccaagatcccaggactggctggcgcccagccccccgcagggcgccttctcctcgcgccctctccccagaggcacctgcagcaccccgcagctcggctctgcgcccctcccgcttccctccctccacagcctcccttcccccgcagggttattttgggaacccagagcctgaggggacctcggaggaatttctccctggtatgggaggtggggggagagaacccaggcgtcctgcccgcctcgccccctcccgggagcccaggaaggcgaggcggggctgcggcagcccccagggggcctgccctaggggaggcggactggatgggagaggaacattcctggggcggggggagcccgctgcggccaggaggcgtcagcgggaagcctgagcctgggaactgagcgctcccaggccacctccgcaaaggtcccaggggtcccggctcagcttgtccacaggccctcttcctccctatccccggctcctgaccctggccccggccccgcacaggcgaactgtgagcgcgcacggagcagggtgtccagaggggggcgctcgcgccaagggtggccggtgggtgcatgacaccattagcaactccggtcactggcggggtcatacgcaccctggcaggggcaaacactccacacccaagttattcgtcggaggccggggacctaagtggaggtgcaggcgtccgcacttacacgcaccgggccacaggcaccggcctcccatcctccgtctctcacacacaatggcacccacaccctgtgcacacctgcacgaagaaaccctcaggcacacatacccagctcgtccaccccagaatgcaaacccgcggacgaggtcgcctcctggacgtgctgttcacttgagccaggccagccttgagtcccgcggccacacaggcgctgacatcctcacacgtgtgcacacacgcaaggcagtgcctctccacgcatgtacactcccacacacatgcacacacccccatgggtgcgcacgcccattccgtcgcccccctcccatttgcggtgcagggcccgccctgcggccccagctccctgactcccctcactcccagattttggcagagccttgccccacggaaaggtaccccggccctacacatactcactcccccaggctggaggacaggggagctcctgtacggagttctcaggcggacttttcctaagagccacccagagccgtccccgcctggctctaccgcttcctcgtgtgaccttgagaatcacttggcctctgggagcctcaattttctcatctgccaaatgggggtacgcgggggagggccccgctggaaggtggctgggaaaagctgggtgcaccgtggaggtcctccgccctccggggatccagcgcgccttagctctcgtggccgctgccccctctcccagacccgggccgcagactccccacccgctcgccgcccccagcccgcccgcgccgccctgggcggggggggagtcgctgggggccg

SEQ ID NO: 17801 - RNA, 332 nt, Homo sapiens
  source 1..332: mol_type = other RNA
tcgaggagctcacagtctaacgctgtctatgtcgattaggctgctgtgccgtcggttcccttcttggtctagcagagccttcagctccttgatctgctcagccaactccgggttcaagtcaaactccgctgggaaggcggagatccagtacctgaccaggtggcacgttttcacctgcagggaattggagttgtccttccgggattgttggtagatgtggagcagcttggccgccagctgagaggaggggatgtaccaggggtgcatcatgaggaacatgcgcaccagctgcgggtcccgcaccttcccggagtcatcgaaggcttcgatgc

SEQ ID NO: 17802 - RNA, 1952 nt, Homo sapiens
  source 1..1952: mol_type = other RNA
tcgaggagctcacagtctaatggtaaactacagagtaaactgaggcacagagtggtaaatgacttacccaatgaggtagaaacagctaggtatgtgaaaatgtgggagcagagctggagagagggcaaggtacaacttgtcctaagtaaaaccccttggactgactcaacagcaaggctgcatacacaaacattacaaaatctacttgcaaaaacctgaaaggagtttccaattatcaccatgactgaattcatgtttcacaatgaattcagctatttcctgatggcatttctatccttgcccccaaagccactgggcatgccaccagtctgctgggagacagcaattaggtagacagcttaaaaccaagaagtatctgactccaattttagcactgaaaaccatattaaaatactttaattaaatccacaaacataaatgtgtagcacatttatgatacttctacatgtagaagtttggaaaaagtctcttctaaccctcatccagaggattctaataagttataggtaccaaagagattagagaatttgtctgtcactttccatatatacattattttggctgtacaagggtgaaaagtgtcactcagacatatttcgtaagtaatctcaacattatacagatatatacaaagacatcacatttaaattcgtgtgtacatctatgcaatgtacaacagtaactgcaaacatgaaccagtgtaaggcaatttcttttgtgatatatgacatactccttgaagggaagggtagagtccacaaagaactgtccatttcagcctgactgtctgtcttcatgacactctgtgatgaagctacttcaggaggcaagatgtctatttcactgacaaaaagcagtgaataattataaaaggagttgttttcaaatgtggaaaccacaattactcagtaatctaagtggtgaactcctcaaagacactactggccatgatgccgctactgagaacgagagcacttcatggataatttattgctctgagaatcaaatttgatgcgtaattctccacgaagatattcccaaaaaactcagtgatacataaattctcaaatgccatcagttgcttacttcaagcaattcttcactttgctgaggattttcttcttcctcagggccttctggatgagtgctctcagatgaagaggtcccgacaccttcagaccttttgttactggtctgaccctgctccacttcacacaaatagacatcgataggtccgttggtgctccttatgtgcactgtgatagagtcatccatctaatatggttcttggatttcttttcaacgaggtcgattccatctaagacattggtgatgtcatacactctccgctttcggactcccagtttcgttgcaaccttgtttaagtcaagaatacccccgggagcagatctgacaagatccataaattttcgagttaaataaaccagcgatacatcaaaacgaggtctcttcacttttagagcttttctcatggacacatattgtacattatcttctaaattaatccttatttttgatggcagcaggccctccacgttgatggggtctcggcaccgacggcgaaccgtctcctccgtcgggtccaggaggagactgggtaacttcctcgccggccgctgctgactcatgctgcccggccgggcgtcctgctcccctcgcaccccacgagctctcccgccctctcgcgctcagctcgagcaccgccccccacgcgccgatttccaagggcccagcacctaaggggtccgcggcttcctccgaggcgccgcccggctaggccgtcccgcccgccagtaaacgcggcacggcctcacgtgcccgggagctcccgacgcagacggaaaaagaggagggagacccgcggatctcaagtcgcccggcccgccatcttcccgcatgcgcagtacacc

SEQ ID NO: 17803 - RNA, 2227 nt, Homo sapiens
  source 1..2227: mol_type = other RNA
tcgaggagctcacagtctaatggtaaactacagagtaaactgaggcacagagtggtaaatgacttacccaatgaggtagaaacagctaggtatgtgaaaatgtgggagcagagctggagagagggcaaggtacaacttgtcctaagtaaaaccccttggactgactcaacagcaaggctgcatacacaaacattacaaaatctacttgcaaaaacctgaaaggagtttccaattatcaccatgactgaattcatgtttcacaatgaattcagctatttcctgatggcatttctatccttgcccccaaagccactgggcatgccaccagtctgctgggagacagcaattaggtagacagcttaaaaccaagaagtatctgactccaattttagcactgaaaaccatattaaaatactttaattaaatccacaaacataaatgtgtagcacatttatgatacttctacatgtagaagtttggaaaaagtctcttctaaccctcatccagaggattctaataagttataggtaccaaagagattagagaatttgtctgtcactttccatatatacattattttggctgtacaagggtgaaaagtgtcactcagacatatttcgtaagtaatctcaacattatacagatatatacaaagacatcacatttaaattcgtgtgtacatctatgcaatgtacaacagtaactgcaaacatgaaccagtgtaaggcaatttcttttgtgatatatgacatactccttgaagggaagggtagagtccacaaagaactgtccatttcagcctgactgtctgtcttcatgacactctgtgatgaagctacttcaggaggcaagatgtctatttcactgacaaaaagcagtgaataattataaaaggagttgttttcaaatgtggaaaccacaattactcagtaatctaagtggtgaactcctcaaagacactactggccatgatgccgctactgagaacgagagcacttcatggataatttattgctctgagaatcaaatttgatgcgtaattctccacgaagatattcccaaaaaactcagtgatacataaattctcaaatgccatcagttgcttacttcaagcaattcttcactttgctgaggattttcttcttcctcagggccttctggatgagtgctctcagatgaagaggtcccgacaccttcagaccttttgttactggtctgaccctgctccacttcacacaaatagacatcgataggtccgttggtgctccttatgtgcactgtgatagagtcctacttctctgggagctggaacatccaatctggtttctgctggagctttaactgcaatgacgatctgttcatggaaggcctgaatgctatgaatgtcttgataggtcacatatgctagtctttcattttctttgtcatctgttaactcaaacagctgctgagcacaatccttaattaactcatccaaagcatcttccattgctgataagtcagaaagttcctcctgtagcttcttttgttggggaactgctccaaaattgctaagatcagatcctatccatctaatatggttcttggatttcttttcaacgaggtcgattccatctaagacattggtgatgtcatacactctccgctttcggactcccagtttcgttgcaaccttgtttaagtcaagaatacccccgggagcagatctgacaagatccataaattttcgagttaaataaaccagcgatacatcaaaacgaggtctcttcacttttagagcttttctcatggacacatattgtacattatcttctaaattaatccttatttttgatggcagcaggccctccacgttgatggggtctcggcaccgacggcgaaccgtctcctccgtcgggtccaggaggagactgggtaacttcctcgccggccgctgctgactcatgctgcccggccgggcgtcctgctcccctcgcaccccacgagctctcccgccctctcgcgctcagctcgagcaccgccccccacgcgccgatttccaagggcccagcacctaaggggtccgcggcttcctccgaggcgccgcccggctaggccgtcccgcccgccagtaaacgcggcacggcctcacgtgcccgggagctcccgacgcagacggaaaaagaggagggagacccgcggatctcaagtcgcccggcccgccatcttcccgcatgcgcagtacacc

SEQ ID NO: 17804 - RNA, 2168 nt, Homo sapiens
  source 1..2168: mol_type = other RNA
tcgaggagctcacagtctaatggtaaactacagagtaaactgaggcacagagtggtaaatgacttacccaatgaggtagaaacagctaggtatgtgaaaatgtgggagcagagctggagagagggcaaggtacaacttgtcctaagtaaaaccccttggactgactcaacagcaaggctgcatacacaaacattacaaaatctacttgcaaaaacctgaaaggagtttccaattatcaccatgactgaattcatgtttcacaatgaattcagctatttcctgatggcatttctatccttgcccccaaagccactgggcatgccaccagtctgctgggagacagcaattaggtagacagcttaaaaccaagaagtatctgactccaattttagcactgaaaaccatattaaaatactttaattaaatccacaaacataaatgtgtagcacatttatgatacttctacatgtagaagtttggaaaaagtctcttctaaccctcatccagaggattctaataagttataggtaccaaagagattagagaatttgtctgtcactttccatatatacattattttggctgtacaagggtgaaaagtgtcactcagacatatttcgtaagtaatctcaacattatacagatatatacaaagacatcacatttaaattcgtgtgtacatctatgcaatgtacaacagtaactgcaaacatgaaccagtgtaaggcaatttcttttgtgatatatgacatactccttgaagggaagggtagagtccacaaagaactgtccatttcagcctgactgtctgtcttcatgacactctgtgatgaagctacttcaggaggcaagatgtctatttcactgacaaaaagcagtgaataattataaaaggagttgttttcaaatgtggaaaccacaattactcagtaatctaagtggtgaactcctcaaagacactactggccatgatgccgctactgagaacgagagcacttcatggataatttattgctctgagaatcaaatttgatgcgtaattctccacgaagatattcccaaaaaactcagtgatacataaattctcaaatgccatcagttgcttacttcaagcaattcttcactttgctgaggattttcttcttcctcagggccttctggatgagtgctctcagatgaagaggtcccgacaccttcagaccttttgttactggtctgaccctgctccacttcacacaaatagacatcgataggtccgttggtgctccttatgtgcactgtgatagagtcttctctgggagctggaacatccaatctggtttctgctggagctttaactgcaatgacgatctgttcatggaaggcctgaatgctatgaatgtcttgataggtcacatatgctagtctttcattttctttgtcatctgttaactcaaacagctgctgagcacaatccttaattaactcatccaaagcatcttccattgctgataagtcagaaagttcctcctgtagcttcttttgttggggaactgctccaaaattgctaagatcagatcctatccatctaatatggttcttggatttcttttcaacgaggtcgattccatctaagacattggtgatgtcatacactctccgctttcggactcccagtttcgttgcaaccttgtttaagtcaagaatacccccgggagcagatctgacaagatccataaattttcgagttaaataaaccagcgatacatcaaaacgaggtctcttcacttttagagcttcagcaggccctccacgttgatggggtctcggcaccgacggcgaaccgtctcctccgtcgggtccaggaggagactgggtaacttcctcgccggccgctgctgactcatgctgcccggccgggcgtcctgctcccctcgcaccccacgagctctcccgccctctcgcgctcagctcgagcaccgccccccacgcgccgatttccaagggcccagcacctaaggggtccgcggcttcctccgaggcgccgcccggctaggccgtcccgcccgccagtaaacgcggcacggcctcacgtgcccgggagctcccgacgcagacggaaaaagaggagggagacccgcggatctcaagtcgcccggcccgccatcttcccgcatgcgcagtacacc

SEQ ID NO: 17805 - RNA, 2427 nt, Homo sapiens
  source 1..2427: mol_type = other RNA
tcgaggagctcacagtctaatggtaaactacagagtaaactgaggcacagagtggtaaatgacttacccaatgaggtagaaacagctaggtatgtgaaaatgtgggagcagagctggagagagggcaaggtacaacttgtcctaagtaaaaccccttggactgactcaacagcaaggctgcatacacaaacattacaaaatctacttgcaaaaacctgaaaggagtttccaattatcaccatgactgaattcatgtttcacaatgaattcagctatttcctgatggcatttctatccttgcccccaaagccactgggcatgccaccagtctgctgggagacagcaattaggtagacagcttaaaaccaagaagtatctgactccaattttagcactgaaaaccatattaaaatactttaattaaatccacaaacataaatgtgtagcacatttatgatacttctacatgtagaagtttggaaaaagtctcttctaaccctcatccagaggattctaataagttataggtaccaaagagattagagaatttgtctgtcactttccatatatacattattttggctgtacaagggtgaaaagtgtcactcagacatatttcgtaagtaatctcaacattatacagatatatacaaagacatcacatttaaattcgtgtgtacatctatgcaatgtacaacagtaactgcaaacatgaaccagtgtaaggcaatttcttttgtgatatatgacatactccttgaagggaagggtagagtccacaaagaactgtccatttcagcctgactgtctgtcttcatgacactctgtgatgaagctacttcaggaggcaagatgtctatttcactgacaaaaagcagtgaataattataaaaggagttgttttcaaatgtggaaaccacaattactcagtaatctaagtggtgaactcctcaaagacactactggccatgatgccgctactgagaacgagagcacttcatggataatttattgctctgagaatcaaatttgatgcgtaattctccacgaagatattcccaaaaaactcagtgatacataaattctcaaatgccatcagttgcttacttcaagcaattcttcactttgctgaggattttcttcttcctcagggccttctggatgagtgctctcagatgaagaggtcccgacaccttcagaccttttgttactggtctgaccctgctccacttcacacaaatagacatcgataggtccgttggtgctccttatgtgcactgtgatagagtcttctctgggagctggaacatccaatctggtttctgctggagctttaactgcaatgacgatctgttcatggaaggcctgaatgctatgaatgtcttgataggtcacatatgctagtctttcattttctttgtcatctgttaactcaaacagctgctgagcacaatccttaattaactcatccaaagcatcttccattgctgataagtcagaaagttcctcctgtagcttcttttgttggggaactgctccaaaattgctaagatcagatcctatccatctaatatggttcttggatttcttttcaacgaggtcgattccatctaagacattggtgatgtcatacactctccgctttcggactcccagtttcgttgcaaccttgtttaagtcaagaatacccccgggagcagatctgacaagatccataaattttcgagttaaataaaccagcgatacatcaaaacgaggtctcttcacttttagagcttcttcagtcagaaatgtccttactcagaacctccacaatgtcacatttagtttaaagaccactggcggttacttcaggaacaaaggtacatatttcataatataaatgtcttctctctggagcccattcctacattctcatggacacatattgtacattatcttctaaattaatccttatttttgatggagaaggattcatggcgaaggcagccctcagctgagcctagcccagcaagccagatttgcctgaataaacaacagcaggccctccacgttgatggggtctcggcaccgacggcgaaccgtctcctccgtcgggtccaggaggagactgggtaacttcctcgccggccgctgctgactcatgctgcccggccgggcgtcctgctcccctcgcaccccacgagctctcccgccctctcgcgctcagctcgagcaccgccccccacgcgccgatttccaagggcccagcacctaaggggtccgcggcttcctccgaggcgccgcccggctaggccgtcccgcccgccagtaaacgcggcacggcctcacgtgcccgggagctcccgacgcagacggaaaaagaggagggagacccgcggatctcaagtcgcccggcccgccatcttcccgcatgcgcagtacacc

SEQ ID NO: 17806 - RNA, 2356 nt, Homo sapiens
  source 1..2356: mol_type = other RNA
tcgaggagctcacagtctaatggtaaactacagagtaaactgaggcacagagtggtaaatgacttacccaatgaggtagaaacagctaggtatgtgaaaatgtgggagcagagctggagagagggcaaggtacaacttgtcctaagtaaaaccccttggactgactcaacagcaaggctgcatacacaaacattacaaaatctacttgcaaaaacctgaaaggagtttccaattatcaccatgactgaattcatgtttcacaatgaattcagctatttcctgatggcatttctatccttgcccccaaagccactgggcatgccaccagtctgctgggagacagcaattaggtagacagcttaaaaccaagaagtatctgactccaattttagcactgaaaaccatattaaaatactttaattaaatccacaaacataaatgtgtagcacatttatgatacttctacatgtagaagtttggaaaaagtctcttctaaccctcatccagaggattctaataagttataggtaccaaagagattagagaatttgtctgtcactttccatatatacattattttggctgtacaagggtgaaaagtgtcactcagacatatttcgtaagtaatctcaacattatacagatatatacaaagacatcacatttaaattcgtgtgtacatctatgcaatgtacaacagtaactgcaaacatgaaccagtgtaaggcaatttcttttgtgatatatgacatactccttgaagggaagggtagagtccacaaagaactgtccatttcagcctgactgtctgtcttcatgacactctgtgatgaagctacttcaggaggcaagatgtctatttcactgacaaaaagcagtgaataattataaaaggagttgttttcaaatgtggaaaccacaattactcagtaatctaagtggtgaactcctcaaagacactactggccatgatgccgctactgagaacgagagcacttcatggataatttattgctctgagaatcaaatttgatgcgtaattctccacgaagatattcccaaaaaactcagtgatacataaattctcaaatgccatcagttgcttacttcaagcaattcttcactttgctgaggattttcttcttcctcagggccttctggatgagtgctctcagatgaagaggtcccgacaccttcagaccttttgttactggtctgaccctgctccacttcacacaaatagacatcgataggtccgttggtgctccttatgtgcactgtgatagagtcttctctgggagctggaacatccaatctggtttctgctggagctttaactgcaatgacgatctgttcatggaaggcctgaatgctatgaatgtcttgataggtcacatatgctagtctttcattttctttgtcatctgttaactcaaacagctgctgagcacaatccttaattaactcatccaaagcatcttccattgctgataagtcagaaagttcctcctgtagcttcttttgttggggaactgctccaaaattgctaagatcagatcctatccatctaatatggttcttggatttcttttcaacgaggtcgattccatctaagacattggtgatgtcatacactctccgctttcggactcccagtttcgttgcaaccttgtttaagtcaagaatacccccgggagcagatctgacaagatccataaattttcgagttaaataaaccagcgatacatcaaaacgaggtctcttcacttttagagcttcttcagtcagaaatgtccttactcagaacctccacaatgtcacatttagtttaaagaccactggcggttacttcaggaacaaaggtacatatttcataatataaatgtcttctctctggagcccattcctacattctcatggacacatattgtacattatcttctaaattaatccttatttttgatggcagcaggccctccacgttgatggggtctcggcaccgacggcgaaccgtctcctccgtcgggtccaggaggagactgggtaacttcctcgccggccgctgctgactcatgctgcccggccgggcgtcctgctcccctcgcaccccacgagctctcccgccctctcgcgctcagctcgagcaccgccccccacgcgccgatttccaagggcccagcacctaaggggtccgcggcttcctccgaggcgccgcccggctaggccgtcccgcccgccagtaaacgcggcacggcctcacgtgcccgggagctcccgacgcagacggaaaaagaggagggagacccgcggatctcaagtcgcccggcccgccatcttcccgcatgcgcagtacacc

SEQ ID NO: 17807 - RNA, 2294 nt, Homo sapiens
  source 1..2294: mol_type = other RNA
tcgaggagctcacagtctaatggtaaactacagagtaaactgaggcacagagtggtaaatgacttacccaatgaggtagaaacagctaggtatgtgaaaatgtgggagcagagctggagagagggcaaggtacaacttgtcctaagtaaaaccccttggactgactcaacagcaaggctgcatacacaaacattacaaaatctacttgcaaaaacctgaaaggagtttccaattatcaccatgactgaattcatgtttcacaatgaattcagctatttcctgatggcatttctatccttgcccccaaagccactgggcatgccaccagtctgctgggagacagcaattaggtagacagcttaaaaccaagaagtatctgactccaattttagcactgaaaaccatattaaaatactttaattaaatccacaaacataaatgtgtagcacatttatgatacttctacatgtagaagtttggaaaaagtctcttctaaccctcatccagaggattctaataagttataggtaccaaagagattagagaatttgtctgtcactttccatatatacattattttggctgtacaagggtgaaaagtgtcactcagacatatttcgtaagtaatctcaacattatacagatatatacaaagacatcacatttaaattcgtgtgtacatctatgcaatgtacaacagtaactgcaaacatgaaccagtgtaaggcaatttcttttgtgatatatgacatactccttgaagggaagggtagagtccacaaagaactgtccatttcagcctgactgtctgtcttcatgacactctgtgatgaagctacttcaggaggcaagatgtctatttcactgacaaaaagcagtgaataattataaaaggagttgttttcaaatgtggaaaccacaattactcagtaatctaagtggtgaactcctcaaagacactactggccatgatgccgctactgagaacgagagcacttcatggataatttattgctctgagaatcaaatttgatgcgtaattctccacgaagatattcccaaaaaactcagtgatacataaattctcaaatgccatcagttgcttacttcaagcaattcttcactttgctgaggattttcttcttcctcagggccttctggatgagtgctctcagatgaagaggtcccgacaccttcagaccttttgttactggtctgaccctgctccacttcacacaaatagacatcgataggtccgttggtgctccttatgtgcactgtgatagagtcttctctgggagctggaacatccaatctggtttctgctggagctttaactgcaatgacgatctgttcatggaaggcctgaatgctatgaatgtcttgataggtcacatatgctagtctttcattttctttgtcatctgttaactcaaacagctgctgagcacaatccttaattaactcatccaaagcatcttccattgctgataagtcagaaagttcctcctgtagcttcttttgttggggaactgctccaaaattgctaagatcagatcctatccatctaatatggttcttggatttcttttcaacgaggtcgattccatctaagacattggtgatgtcatacactctccgctttcggactcccagtttcgttgcaaccttgtttaagtcaagaatacccccgggagcagatctgacaagatccataaattttcgagttaaataaaccagcgatacatcaaaacgaggtctcttcacttttagagcttttctcatggacacatattgtacattatcttctaaattaatccttatttttgatggagaaggattcatggcgaaggcagccctcagctgagcctagcccagcaagccagatttgcctgaataaacaacagcaggccctccacgttgatggggtctcggcaccgacggcgaaccgtctcctccgtcgggtccaggaggagactgggtaacttcctcgccggccgctgctgactcatgctgcccggccgggcgtcctgctcccctcgcaccccacgagctctcccgccctctcgcgctcagctcgagcaccgccccccacgcgccgatttccaagggcccagcacctaaggggtccgcggcttcctccgaggcgccgcccggctaggccgtcccgcccgccagtaaacgcggcacggcctcacgtgcccgggagctcccgacgcagacggaaaaagaggagggagacccgcggatctcaagtcgcccggcccgccatcttcccgcatgcgcagtacacc

SEQ ID NO: 17808 - RNA, 2223 nt, Homo sapiens
  source 1..2223: mol_type = other RNA
tcgaggagctcacagtctaatggtaaactacagagtaaactgaggcacagagtggtaaatgacttacccaatgaggtagaaacagctaggtatgtgaaaatgtgggagcagagctggagagagggcaaggtacaacttgtcctaagtaaaaccccttggactgactcaacagcaaggctgcatacacaaacattacaaaatctacttgcaaaaacctgaaaggagtttccaattatcaccatgactgaattcatgtttcacaatgaattcagctatttcctgatggcatttctatccttgcccccaaagccactgggcatgccaccagtctgctgggagacagcaattaggtagacagcttaaaaccaagaagtatctgactccaattttagcactgaaaaccatattaaaatactttaattaaatccacaaacataaatgtgtagcacatttatgatacttctacatgtagaagtttggaaaaagtctcttctaaccctcatccagaggattctaataagttataggtaccaaagagattagagaatttgtctgtcactttccatatatacattattttggctgtacaagggtgaaaagtgtcactcagacatatttcgtaagtaatctcaacattatacagatatatacaaagacatcacatttaaattcgtgtgtacatctatgcaatgtacaacagtaactgcaaacatgaaccagtgtaaggcaatttcttttgtgatatatgacatactccttgaagggaagggtagagtccacaaagaactgtccatttcagcctgactgtctgtcttcatgacactctgtgatgaagctacttcaggaggcaagatgtctatttcactgacaaaaagcagtgaataattataaaaggagttgttttcaaatgtggaaaccacaattactcagtaatctaagtggtgaactcctcaaagacactactggccatgatgccgctactgagaacgagagcacttcatggataatttattgctctgagaatcaaatttgatgcgtaattctccacgaagatattcccaaaaaactcagtgatacataaattctcaaatgccatcagttgcttacttcaagcaattcttcactttgctgaggattttcttcttcctcagggccttctggatgagtgctctcagatgaagaggtcccgacaccttcagaccttttgttactggtctgaccctgctccacttcacacaaatagacatcgataggtccgttggtgctccttatgtgcactgtgatagagtcttctctgggagctggaacatccaatctggtttctgctggagctttaactgcaatgacgatctgttcatggaaggcctgaatgctatgaatgtcttgataggtcacatatgctagtctttcattttctttgtcatctgttaactcaaacagctgctgagcacaatccttaattaactcatccaaagcatcttccattgctgataagtcagaaagttcctcctgtagcttcttttgttggggaactgctccaaaattgctaagatcagatcctatccatctaatatggttcttggatttcttttcaacgaggtcgattccatctaagacattggtgatgtcatacactctccgctttcggactcccagtttcgttgcaaccttgtttaagtcaagaatacccccgggagcagatctgacaagatccataaattttcgagttaaataaaccagcgatacatcaaaacgaggtctcttcacttttagagcttttctcatggacacatattgtacattatcttctaaattaatccttatttttgatggcagcaggccctccacgttgatggggtctcggcaccgacggcgaaccgtctcctccgtcgggtccaggaggagactgggtaacttcctcgccggccgctgctgactcatgctgcccggccgggcgtcctgctcccctcgcaccccacgagctctcccgccctctcgcgctcagctcgagcaccgccccccacgcgccgatttccaagggcccagcacctaaggggtccgcggcttcctccgaggcgccgcccggctaggccgtcccgcccgccagtaaacgcggcacggcctcacgtgcccgggagctcccgacgcagacggaaaaagaggagggagacccgcggatctcaagtcgcccggcccgccatcttcccgcatgcgcagtacacc

SEQ ID NO: 17809 - RNA, 2147 nt, Homo sapiens
  source 1..2147: mol_type = other RNA
tcgaggagctcacagtctaatggtaaactacagagtaaactgaggcacagagtggtaaatgacttacccaatgaggtagaaacagctaggtatgtgaaaatgtgggagcagagctggagagagggcaaggtacaacttgtcctaagtaaaaccccttggactgactcaacagcaaggctgcatacacaaacattacaaaatctacttgcaaaaacctgaaaggagtttccaattatcaccatgactgaattcatgtttcacaatgaattcagctatttcctgatggcatttctatccttgcccccaaagccactgggcatgccaccagtctgctgggagacagcaattaggtagacagcttaaaaccaagaagtatctgactccaattttagcactgaaaaccatattaaaatactttaattaaatccacaaacataaatgtgtagcacatttatgatacttctacatgtagaagtttggaaaaagtctcttctaaccctcatccagaggattctaataagttataggtaccaaagagattagagaatttgtctgtcactttccatatatacattattttggctgtacaagggtgaaaagtgtcactcagacatatttcgtaagtaatctcaacattatacagatatatacaaagacatcacatttaaattcgtgtgtacatctatgcaatgtacaacagtaactgcaaacatgaaccagtgtaaggcaatttcttttgtgatatatgacatactccttgaagggaagggtagagtccacaaagaactgtccatttcagcctgactgtctgtcttcatgacactctgtgatgaagctacttcaggaggcaagatgtctatttcactgacaaaaagcagtgaataattataaaaggagttgttttcaaatgtggaaaccacaattactcagtaatctaagtggtgaactcctcaaagacactactggccatgatgccgctactgagaacgagagcacttcatggataatttattgctctgagaatcaaatttgatgcgtaattctccacgaagatattcccaaaaaactcagtgatacataaattctcaaatgccatcagttgcttacttcaagcaattcttcactttgctgaggattttcttcttcctcagggccttctggatgagtgctctcagatgaagaggtcccgacaccttcagaccttttgttactggtctgaccctgctccacttcacacaaatagacatcgataggtccgttggtgctccttatgtgcactgtgatagagtcttctctgggagctggaacatccaatctggtttctgctggagctttaactgcaatgacgatctgttcatggaaggcctgaatgctatgaatgtcttgataggtcacatatgctagtctttcattttctttgtcatctgttaactcaaacagctgctgagcacaatccttaattaactcatccaaagcatcttccattgctgataagtcagaaagttcctcctgtagcttcttttgttggggaactgctccaaaattgctaagatcagatcctatccatctaatatggttcttggatttcttttcaacgaggtcgattccatctaagacattggtgatgtcatacactctccgctttcggactcccagtttcgttgcaaccttgtttaagtcaagaatacccccgggagcagatttctcatggacacatattgtacattatcttctaaattaatccttatttttgatggcagcaggccctccacgttgatggggtctcggcaccgacggcgaaccgtctcctccgtcgggtccaggaggagactgggtaacttcctcgccggccgctgctgactcatgctgcccggccgggcgtcctgctcccctcgcaccccacgagctctcccgccctctcgcgctcagctcgagcaccgccccccacgcgccgatttccaagggcccagcacctaaggggtccgcggcttcctccgaggcgccgcccggctaggccgtcccgcccgccagtaaacgcggcacggcctcacgtgcccgggagctcccgacgcagacggaaaaagaggagggagacccgcggatctcaagtcgcccggcccgccatcttcccgcatgcgcagtacacc

SEQ ID NO: 17810 - RNA, 1969 nt, Homo sapiens
  source 1..1969: mol_type = other RNA
tcgaggagctcacagtctaatggtaaactacagagtaaactgaggcacagagtggtaaatgacttacccaatgaggtagaaatagctaggtatgtgaaaatgtgggagcagagctggagagagggcaaggtacaacttgtcctaagtaaaaccccttggactgactcaacagcaaggctgcatacacaaacattacaaaatctacttgcaaaaacctgaaaggagtttccaattatcaccatgactgaattcatgtttcacaatgaattcagctatttcctgatgacatttctatccttgcccccaaagccactgggcatgccaccgatctgctgggagacagcaattaggtagacagcttaaaaccaagaagtatctgactccaattttagcactgaaaaccatattaaaatactttaattaaatccacaaacataaatgtgtagcacatttatgatacttctacatgtagaagtttggaaaaagtctcttctaaccctcatccagaggattctaataagttatagataccaaagagattagagaatttgtctgtcactttccatatatacattattttggctgtacgagagtgaaaagtgtcactcagacatatttcgtaagtaatctcaacattatacagatatatacaaagacatcacatttaaattcgtgtgtacatctatgcaatgtacaacagtaactgcaaacatgaaccagtgtaaggcaatttcttttgtgacatatgacatactccttgaagggaagggtagagtccacaaagaactgtccttttcagcctgactgtctgtcttcatgacactctgtgatgaagctacttcaggaggcaagatgtctatttcactgacaaaaagcagtgaataattataaaaggagttgttttcaaatgtggaaaccacaattactcagtaatctaagtggtgaactcctcaaagacactactggccatgatgctgctactgagaacgagagcacttcatggataatttattgctctgagaatcaaatttgatgcgtaattctccaggaagatattcccaaaaaactcagtgatacataaattctcaaatgccatcagttgcttacttcaagcaattcttcactttgctgaggattttcttcttcctcagggccttctggatgagtgctctcagatgaagaggtcctgacaccttcagaccttttgttactggtctgaccctgctccacttctcacaaatagacatcgataggtccgttggtgctccttatgtgcactgtgatagagtcttctctgggagctggaacatccaatctggtttctgctggagctttaactgcaatgacgatctgttcatggaaggcctgaatgctatgaatgtcttgataggtcacatatgctagtctttcattttctttgtcatctgttaactcaaacagctgctgagcacaatccttaattaactcatccaaagcatcttccattgctgataagtcagaaagttcctcctgtagcttcttttgttggggaactgctccaaaattgctaagatcagatcctatccatctaatatggttcttggatttcttttcaacgaggtcgattccatctaagacatcggtgatgtcatacactctccgctttcggactcccagtttcgttgcaaccttgtttaagtcaagaatacccccgggagcagatttctcatggacacatattgtacattatcttctaaattaatccttatttttgatggcagcaggccctccacgttgatggggtctcctccgtcgggtgcaggaggagactgggtaatctcctcgccggccgctgctgactcatgctgcccggccgggcgtcctgctcccctcgcaccccacgagctctcccgccctctcgcgctcagctcgagcaccgccccccacgcgccgatttccaagggcccagcacctaaggggtccgcggcct

SEQ ID NO: 17811 - RNA, 1843 nt, Homo sapiens
  source 1..1843: mol_type = other RNA
tcgaggagctcacagtctaatggtaaactacagagtaaactgaggcacagagtggtaaatgacttacccaatgaggtagaaatagctaggtatgtgaaaatgtgggagcagagctggagagagggcaaggtacaacttgtcctaagtaaaaccccttggactgactcaacagcaaggctgcatacacaaacattacaaaatctacttgcaaaaacctgaaaggagtttccaattatcaccatgactgaattcatgtttcacaatgaattcagctatttcctgatggcatttctatccttgcccccaaagccactgggcatgccaccgatctgctgggagacagcaattaggtagacagcttaaaaccaagaagtatctgactccaattttagcactgaaaaccatattaaaatactttaattaaatccacaaacataaatgtgtagcacatttatgatacttctacatgtagaagtttggaaaaagtctcttctaaccctcatccagaggattctaataagttatagataccaaagagattagagaatttgtctgtcattttccatatatacattattttggctgtacaagagtgaaaagtgtcactcagacatatttcgtaagtaatctcaacattatacagatatatacaaagacatcacatttaaattcgtgtgtacatctatgcaatgtacaacagtaactgcaaacatgaaccagtgtaaggcaatttcttttgtgacatatgacatactccttgaagggaagggtagagtccacaaagaactgtccttttcagcctgactgtctgtcttcatgacactctgtgatgaagctacttcaggaggcaagatgtctatttcactgacaaaaagcagtgaataattataaaaggagttgttttcaaatgtggaaaccacaattactcagtaatctaagtggtgaactcctcaaagacactactggccatgatgccgctactgagaacgagagcacttcatggataatttattgctctgagaatcaaatttgatgcgtaattctccacgaagatattcccaaaaaactcagtgatacataaattctcaaatgccatcagttgcttacttcaagcaattcttcactttgctgaggattttcttcttcctcagggccttctggatgagtgctctcagatgaagaggtcctgacaccttcagaccttttgttactggtctgaccctgctccacttctcacaaatagacatcgataggtccgttggtgctccttatgtgcactgtgatagagtcttctctgggagctggaacatccaatctggtttctgctggagctttaactgcaatgacgatctgttcatggaaggcctgaatgctatgaatgtcttgataggtcacatatgctagtctttcattttctttgtcatctgttaactcaaacagctgctgagcacaatccttaattaactcatccaaagcatcttccattgctgataagtcagaaagttcctcctgtagcttcttttgttggggaactgctccaaaattgctaagatcagatcctatccatctaatatggttcttggatttcttttcaacgaggtcgattccatctaagacatcggtgatgtcatacactctccgctttcggactcccagtttcgttgcaaccttgtttaagtcaagaatacccccgggagcagatttctcatggacacatattgtacattatcttctaaattaatccttatttttgatggcagcaggccctccacgttgatggggtctcctccgtcgggtgcaggaggagactgggtaatctcctcgccggccgctgctgactcat

SEQ ID NO: 17812 - RNA, 6983 nt, Homo sapiens
  source 1..6983: mol_type = other RNA
tcgaggagctcacagtctagaaagggcagcaagacagtacacaatcagtggcagcagcaccagccagagtggcaagtgctcaaagcgagacacaaagtgctgtgcggtcacaacatcatggggatgcttctggcagaagcactggaaaggagacgaggactcaggctgggccttccaggagggaagccatttgggagaagggcatctctagcggagagaggtccatctgcagagcccacaggtcatgggaaacatgtggctgcagggagagtttggggacagtcaagtatggctgggaggtggacagccacggacactaagctcaggagatgtgaactttgtggtctggtcaaacagccactgcagatcacttcgcaggaggaggggtgactagaagtatgttactggaaggtaaatctggccacactgcagcatctggacggcagagggcagcgctgggaggggccagccagttagggcccaccacccctgggtgtctgagagtgggagtagcgggcaggggccagcaaagcacgagggcagagcaggggaccatacggagggtgggtgtggaagaagggaggggccccatgcaagctgcaggtctggggagcctgaggatgtcatagggcttcctggtagagtggaaagtgcactcctgaaggtcagggccagtcactacagagaggggacagcgaggagagggacggtgtggccctaagggtgactgcagtttctcaacatgtggtccgtggatcacctgcatgggaactgcctggggaatgcgctcatttgcagattcccgggccttcctccagaactactgggcaagcatctgccgggtcatgcccggtaacctacattcttaacaccagctgccctctccaccaccacgagccccaaaggtggggaaaagtctgcaagccacctgcagaggaagaatagggtgttaaggactggctttaggcaaaaagaagagacaaaaagaatgagggaggtctgggagtgagggaagtggtgggaagcagggaaagtccggtcaagccatgtgcaccaagacagagccccagcgcggccttgcagccaggcaccgggccgtccccaagggctgctctcagtccgctttcacttggtgggcgaaagccacatttgcaaactgggaagtggagagtgggaggtgaggggaagcactagcaatgaatgaagaggattcttccgggaatcaggctgtttcaatctaaaacatccaagataagtggaaacactggggaggaaggtgatgaacagacggaggtgagccagagacacctcctgggcaagtcggccaggaggcgggaggcgtgggtcagagacactgcaggaactgggtgaggacaaggaggtgcgaggaaaggggttgggggatggtcccacaggcagccacacctgaggcgtgggaggcaggtaggagctgggggagggcggggagaagaggggtttctgtgtgtagatctgagtcctccctcacatcccagccgtgccacaagccgcatcggcatgaggccggctctcccttcttcactggtctcaaaagccacccaggcccaagtcccggccagacagccgagcctgcctagcaacgctgaccggccgcccaggatggcccagacaccttctgtctcctgaatgcagcctacaggggttcaaacagactgcttgcattaaggtcagacaaggctcttttacttccagagacagcggcctggagcctcgggaagaatgtaggcccaggaatcacccagcccctcaggacaacctctctgagcaacagacatcctccctgttgaatgagagtgacatctctgccctgccacctactttacatggatgccacgaagtgggagagcctgagcagtagacagggaagaggcgagcggccccactgcaggaggtagacaggctacagatacttatgcagcagccacactgaggctagtactggaggaggctgagaaccagtaatgagttcttaatggtttgataatttgggtttttaaatattaaatattaaatatcaggggtttcggaaggaatgatgaattccgtctcatgctgtaactgatgaaggcaaccaatgagcaatccttccttcccatagccgagaaagggaaaggggacaggccaatccctctgaagcagtaagtcagaacacgaagacttacagaactcaaacatcaaaggtcaagtagcttctagccaggaaaagtggtggccccctcagcctagccagcaccaaccagcatgggtggagactcagcctggcagtaagggcatttcctgggtttcctctgaagcagaggagaaatagtgggtcagccaggctgctggactgaaccatgagccagaaggccagaatcactgcaagacagctccagcccgcacacctcagttgtgcttttgaaaacaggtacaaagctgaggcatgggagctgtgactgaagtcgccctcctggctggcctcgtcttctacctctgcttccacagctgggtgacttggccataggcccaaacaatggacaaccagttccacattaggaggcatcacggacgcatctgagaggaaacatgattgaaggacaagcttggcctcatggagggctctggattcatcccttgaagaacgcagtgatcaaacaaaaccaagaagcaggcctggagggagcactctgggatgcccccaagtcccctcaccatttacaaaccagcactgagttctcagcctccgctcctcaggactaggagacaagatccggacaggcaggacaggcagcaagccgactgtgagcagcctgggggcgcaggtgtaaaatacaaagccctttgaaggtccagacaataagagtaaagatgttaagattgcccaggaaaagaacttcactgacactgaatttgggcaacacctagaacagacaatattaagatatcaattctgagaaagactcacaggaaaggctgtttaggaggacactagagacaaacacagggaaaataaatacaggggctctgggatccccccacagaagctactaatgctatttattggcttgggtcacttttgagaatagaaaaccattttttggcaaagctgtacaaactccacatcagggcgtctcctgcagttggggacacaagatggccacagtgaccgggctcttcattaaacttcctcataacccgctacggtgttcagaagctaagacgtgacttccagagccaggccaggcatgtggaggcccctgactgtgggcgtgtcaagccctggctggggagcctgctgcctgcccggccactcctcagctgtggctgtggctgtgggcatggccggacggcgtgcacactgggccgtccccttttgcgcagggtggaagggggaaggagggtgggactccatgggctccacgatgtcttctagccctggtattctgtgagactaacttcgccctggtcattcaccatggctaggcaccaagtgccatctagtggcaccgcgggtccactttcacaacactccaaccaaagactgcagaacaaaccaactcttacccactttaactccgggggtgagggcagaggaggctggaagggtgagcacacttcatggtagtgatgggacatactcatctcaagaaaatatactttaagacgtcttgctttccttaagaaagcaacacttttttttttatttatttataaaggctaaccatatccatttgtcaatattttcggctttaaggaaaatagtttaaaaaacataaaaaggtaaatacactcaagagtaactgctattaaacagttctgaacaggcagaaaatgtagactttcctttaacagaaaatgttaaatctgtaatagcagcataatttatatatagaaaaaagctggttttgaaaacccagatttatacccaaaacattttttttctgtacaactgcgtttacactgggaaataagtttcttcacattatgttcattcccatcaggtacaggtgtgagcttgagtttgatcagccagccctgagcgcaagctcagcgctcagcacaatcttcaatccaacaccatggcagaaagcgcatttagatctttcatgtatgggtgggccaccaagatctggtctattttcagtctttgctctgagtcagggaagatcttcagaagggcttccctcagctcgttggtttctgcagaagatctctgagctggcatgggcaggttctgctggagactggggagggctggcagcagtgggaagtggggctgctgagggagccagtggcttgaaggggctccctgaatccgggtcggaggctggtggctggtgctggctgcctgggtgccagggactctgaagctggggtcaaacatgcccacatttggcagggcactgagtaggggctgcatatctctaagacagacttccttctgaagaaactcctctaatcgaggtccacttcttcccagaggatcatcgggaaccataaatatgtcccccacgaacgtgtactgcagcagcctttttgtaataatttctctccaagagactgactcattcacaaattctctgaaattatcatttgtcacaattatgccaccagttttgtccgctaagtgtagtagaaacctgtcatcatgagaagcaattctttctccaaagaccatccgggcaggagttaaagataatattccgagctcctggagctgggttaagaagtgctgttctgtgacattaggatcacgccttgttctccactgagggacaaatacagtgatgtttctgttgccaagcttccaaaaatattcaactgcaattgcaattccacgacaagaaaagaactttttcagaccatgggtaattgcaacattgctcccatctataacaatgtgtttcaaatccgttctccctggttcattttttaattccagcttgtagggtatttttagagtatctcgaaacctttgaaccccagtaactgaggaatcaatatgatcagaaggtcctgccgaccttgcatcagtaaccgaaggtaacagctggggcagtggcattggtggagaaagggttgagcaatttggcttagaatgaggagaactacaacatcctaaacgtttttcacaggcagatttcatattatttggaagcaagggttctggctgctggtgtaaaccattttcaggaaaaagtggaactctgggctggtgacttgaagctccccttgaaacaaaattgacttctttgggacttggagaggcaacagaaggtgaaaggccatcagtttcagggtctgtgttacaaatgtagttctggtttgaaccccagacttcatgtttctgttctattggcactgttctgaaagtattaattctacaatttgaggtacatggtttagcttccactttgaatggtaactgagaaaatttttctaccatattttgctgtgtgtgagcctgtgttttctttggagtggaatcagttgtaagctcatttgtgctgctataaacacctttatttttggttttgttggtctctggatacactgtaccagctgaaaattctctgtcttcttggaatcttttattttctttttcaatttcctctaagagcaataatggttcagtagatggtccatacaccttaatgaccttttcaacaatttcttgggagtagcccatggttttaaaaaagtttacgaggatgttgtattccatttcctcagtagtttcttttatatctggacttaaattttcagaatcagcagaagaatcagataggtcagctattacatttccagccaatgtcttagcatcgtgtaaaatctccccctcctgaacattttccaaagaaaactgcttcttcgtatgcctttcttcagaatcagaaaatctccttttctgacaaattctctcattggaaagtgcctcttcatctggggttagaccatttattggatcaaaaagcacatctggtgagctagaaaggactgtgtccatttgttttgtaagctcagaaacaggagtcccagctttatttcttgcctcttcctgcaaaacagtttcatctctagaaatattcagccctgtggcagcattctgtgtaaactctgtttgttgagaatctctcatttcaataacctcatcatctcctgtttcaaagagattctcctcaccttgtgtgagtgtcaaaagttcttttttcaaggaagtgggcaaaatcaacaaatccattgtgtaattgtctgcatgggcttcaacaaattgtttgaattcccttttcacctctgattctttctgactactgggtaggttctctttattttcaaagagctttacaaattgttgaatgtgactcctagccatgaccacagcctcagcacttcctctgatgccaagaaggccaatgtccagaatgcagaggtcagcacaagtatcctgaatcaagcttttcagaaacaggctctctgccccaacaaaaatgcagtgcatgtccttggggtaacattctctttcttctagttcaggttcacagattcctttaatatattccttggcgctgtgcaccgcctcctgcgccccgcagagctgcagccagatgcgcgcgggcagcggctcctcagcccctagcgcgccgagcacggctaggctcacgccaaacaggccctcgatacggccgcggctctgctccagcagctccgccttctcagctggcgcagtgaactcgtccagcaccgcccgggccgccatggcgggcgcggcctcccgcggcggcgccgggggccggcggcggcgacgccccctcagcttgctgccgctgctcccaagccagtcaggcggcgtcggcccttcccggccgcctcgcccccgcccgcgccccgccgcccgccctcaggcccggctataccatcccgccacgaccgcagcagcttggcaattgctggcagcgaacccctcc

SEQ ID NO: 17813 - RNA, 6920 nt, Homo sapiens
  source 1..6920: mol_type = other RNA
tcgaggagctcacagtctagaaagggcagcaagacagtacacaatcagtggcagcagcaccagccagagtggcaagtgctcaaagcgagacacaaagtgctgtgcggtcacaacatcatggggatgcttctggcagaagcactggaaaggagacgaggactcaggctgggccttccaggagggaagccatttgggagaagggcatctctagcggagagaggtccatctgcagagcccacaggtcatgggaaacatgtggctgcagggagagtttggggacagtcaagtatggctgggaggtggacagccacggacactaagctcaggagatgtgaactttgtggtctggtcaaacagccactgcagatcacttcgcaggaggaggggtgactagaagtatgttactggaaggtaaatctggccacactgcagcatctggacggcagagggcagcgctgggaggggccagccagttagggcccaccacccctgggtgtctgagagtgggagtagcgggcaggggccagcaaagcacgagggcagagcaggggaccatacggagggtgggtgtggaagaagggaggggccccatgcaagctgcaggtctggggagcctgaggatgtcatagggcttcctggtagagtggaaagtgcactcctgaaggtcagggccagtcactacagagaggggacagcgaggagagggacggtgtggccctaagggtgactgcagtttctcaacatgtggtccgtggatcacctgcatgggaactgcctggggaatgcgctcatttgcagattcccgggccttcctccagaactactgggcaagcatctgccgggtcatgcccggtaacctacattcttaacaccagctgccctctccaccaccacgagccccaaaggtggggaaaagtctgcaagccacctgcagaggaagaatagggtgttaaggactggctttaggcaaaaagaagagacaaaaagaatgagggaggtctgggagtgagggaagtggtgggaagcagggaaagtccggtcaagccatgtgcaccaagacagagccccagcgcggccttgcagccaggcaccgggccgtccccaagggctgctctcagtccgctttcacttggtgggcgaaagccacatttgcaaactgggaagtggagagtgggaggtgaggggaagcactagcaatgaatgaagaggattcttccgggaatcaggctgtttcaatctaaaacatccaagataagtggaaacactggggaggaaggtgatgaacagacggaggtgagccagagacacctcctgggcaagtcggccaggaggcgggaggcgtgggtcagagacactgcaggaactgggtgaggacaaggaggtgcgaggaaaggggttgggggatggtcccacaggcagccacacctgaggcgtgggaggcaggtaggagctgggggagggcggggagaagaggggtttctgtgtgtagatctgagtcctccctcacatcccagccgtgccacaagccgcatcggcatgaggccggctctcccttcttcactggtctcaaaagccacccaggcccaagtcccggccagacagccgagcctgcctagcaacgctgaccggccgcccaggatggcccagacaccttctgtctcctgaatgcagcctacaggggttcaaacagactgcttgcattaaggtcagacaaggctcttttacttccagagacagcggcctggagcctcgggaagaatgtaggcccaggaatcacccagcccctcaggacaacctctctgagcaacagacatcctccctgttgaatgagagtgacatctctgccctgccacctactttacatggatgccacgaagtgggagagcctgagcagtagacagggaagaggcgagcggccccactgcaggaggtagacaggctacagatacttatgcagcagccacactgaggctagtactggaggaggctgagaaccagtaatgagttcttaatggtttgataatttgggtttttaaatattaaatattaaatatcaggggtttcggaaggaatgatgaattccgtctcatgctgtaactgatgaaggcaaccaatgagcaatccttccttcccatagccgagaaagggaaaggggacaggccaatccctctgaagcagtaagtcagaacacgaagacttacagaactcaaacatcaaaggtcaagtagcttctagccaggaaaagtggtggccccctcagcctagccagcaccaaccagcatgggtggagactcagcctggcagtaagggcatttcctgggtttcctctgaagcagaggagaaatagtgggtcagccaggctgctggactgaaccatgagccagaaggccagaatcactgcaagacagctccagcccgcacacctcagttgtgcttttgaaaacaggtacaaagctgaggcatgggagctgtgactgaagtcgccctcctggctggcctcgtcttctacctctgcttccacagctgggtgacttggccataggcccaaacaatggacaaccagttccacattaggaggcatcacggacgcatctgagaggaaacatgattgaaggacaagcttggcctcatggagggctctggattcatcccttgaagaacgcagtgatcaaacaaaaccaagaagcaggcctggagggagcactctgggatgcccccaagtcccctcaccatttacaaaccagcactgagttctcagcctccgctcctcaggactaggagacaagatccggacaggcaggacaggcagcaagccgactgtgagcagcctgggggcgcaggtgtaaaatacaaagccctttgaaggtccagacaataagagtaaagatgttaagattgcccaggaaaagaacttcactgacactgaatttgggcaacacctagaacagacaatattaagatatcaattctgagaaagactcacaggaaaggctgtttaggaggacactagagacaaacacagggaaaataaatacaggggctctgggatccccccacagaagctactaatgctatttattggcttgggtcacttttgagaatagaaaaccattttttggcaaagctgtacaaactccacatcagggcgtctcctgcagttggggacacaagatggccacagtgaccgggctcttcattaaacttcctcataacccgctacggtgttcagaagctaagacgtgacttccagagccaggccaggcatgtggaggcccctgactgtgggcgtgtcaagccctggctggggagcctgctgcctgcccggccactcctcagctgtggctgtggctgtgggcatggccggacggcgtgcacactgggccgtccccttttgcgcagggtggaagggggaaggagggtgggactccatgggctccacgatgtcttctagccctggtattctgtgagactaacttcgccctggtcattcaccatggctaggcaccaagtgccatctagtggcaccgcgggtccactttcacaacactccaaccaaagactgcagaacaaaccaactcttacccactttaactccgggggtgagggcagaggaggctggaagggtgagcacacttcatggtagtgatgggacatactcatctcaagaaaatatactttaagacgtcttgctttccttaagaaagcaacacttttttttttatttatttataaaggctaaccatatccatttgtcaatattttcggctttaaggaaaatagtttaaaaaacataaaaaggtaaatacactcaagagtaactgctattaaacagttctgaacaggcagaaaatgtagactttcctttaacagaaaatgttaaatctgtaatagcagcataatttatatatagaaaaaagctggttttgaaaacccagatttatacccaaaacattttttttctgtacaactgcgtttacactgggaaataagtttcttcacattatgttcattcccatcaggtacaggtgtgagcttgagtttgatcagccagccctgagcgcaagctcagcgctcagcacaatcttcaatccaacaccatggcagaaagcgcatttagatctttcatgtatgggtgggccaccaagatctggtctattttcagtctttgctctgagtcagggaagatcttcagaagggcttccctcagctcgttggtttctgcagaagatctctgagctggcatgggcaggttctgctggagactggggagggctggcagcagtgggaagtggggctgctgagggagccagtggcttgaaggggctccctgaatccgggtcggaggctggtggctggtgctggctgcctgggtgccagggactctgaagctggggtcaaacatgcccacatttggcagggcactgagtaggggctgcatatctctaagacagacttccttctgaagaaactcctctaatcgaggtccacttcttcccagaggatcatcgggaaccataaatatgtcccccacgaacgtgtactgcagcagcctttttgtaataatttctctccaagagactgactcattcacaaattctctgaaattatcatttgtcacaattatgccaccagttttgtccgctaagtgtagtagaaacctgtgacattaggatcacgccttgttctccactgagggacaaatacagtgatgtttctgttgccaagcttccaaaaatattcaactgcaattgcaattccacgacaagaaaagaactttttcagaccatgggtaattgcaacattgctcccatctataacaatgtgtttcaaatccgttctccctggttcattttttaattccagcttgtagggtatttttagagtatctcgaaacctttgaaccccagtaactgaggaatcaatatgatcagaaggtcctgccgaccttgcatcagtaaccgaaggtaacagctggggcagtggcattggtggagaaagggttgagcaatttggcttagaatgaggagaactacaacatcctaaacgtttttcacaggcagatttcatattatttggaagcaagggttctggctgctggtgtaaaccattttcaggaaaaagtggaactctgggctggtgacttgaagctccccttgaaacaaaattgacttctttgggacttggagaggcaacagaaggtgaaaggccatcagtttcagggtctgtgttacaaatgtagttctggtttgaaccccagacttcatgtttctgttctattggcactgttctgaaagtattaattctacaatttgaggtacatggtttagcttccactttgaatggtaactgagaaaatttttctaccatattttgctgtgtgtgagcctgtgttttctttggagtggaatcagttgtaagctcatttgtgctgctataaacacctttatttttggttttgttggtctctggatacactgtaccagctgaaaattctctgtcttcttggaatcttttattttctttttcaatttcctctaagagcaataatggttcagtagatggtccatacaccttaatgaccttttcaacaatttcttgggagtagcccatggttttaaaaaagtttacgaggatgttgtattccatttcctcagtagtttcttttatatctggacttaaattttcagaatcagcagaagaatcagataggtcagctattacatttccagccaatgtcttagcatcgtgtaaaatctccccctcctgaacattttccaaagaaaactgcttcttcgtatgcctttcttcagaatcagaaaatctccttttctgacaaattctctcattggaaagtgcctcttcatctggggttagaccatttattggatcaaaaagcacatctggtgagctagaaaggactgtgtccatttgttttgtaagctcagaaacaggagtcccagctttatttcttgcctcttcctgcaaaacagtttcatctctagaaatattcagccctgtggcagcattctgtgtaaactctgtttgttgagaatctctcatttcaataacctcatcatctcctgtttcaaagagattctcctcaccttgtgtgagtgtcaaaagttcttttttcaaggaagtgggcaaaatcaacaaatccattgtgtaattgtctgcatgggcttcaacaaattgtttgaattcccttttcacctctgattctttctgactactgggtaggttctctttattttcaaagagctttacaaattgttgaatgtgactcctagccatgaccacagcctcagcacttcctctgatgccaagaaggccaatgtccagaatgcagaggtcagcacaagtatcctgaatcaagcttttcagaaacaggctctctgccccaacaaaaatgcagtgcatgtccttggggtaacattctctttcttctagttcaggttcacagattcctttaatatattccttggcgctgtgcaccgcctcctgcgccccgcagagctgcagccagatgcgcgcgggcagcggctcctcagcccctagcgcgccgagcacggctaggctcacgccaaacaggccctcgatacggccgcggctctgctccagcagctccgccttctcagctggcgcagtgaactcgtccagcaccgcccgggccgccatggcgggcgcggcctcccgcggcggcgccgggggccggcggcggcgacgccccctcagcttgctgccgctgctcccaagccagtcaggcggcgtcggcccttcccggccgcctcgcccccgcccgcgccccgccgcccgccctcaggcccggctataccatcccgccacgaccgcagcagcttggcaattgctggcagcgaacccctccgcccctttgccgccgccgcgggccgggccccgcc

SEQ ID NO: 17814 - RNA, 6909 nt, Homo sapiens
  source 1..6909: mol_type = other RNA
tcgaggagctcacagtctagaaagggcagcaagacagtacacaatcagtggcagcagcaccagccagagtggcaagtgctcaaagcgagacacaaagtgctgtgcggtcacaacatcatggggatgcttctggcagaagcactggaaaggagacgaggactcaggctgggccttccaggagggaagccatttgggagaagggcatctctagcggagagaggtccatctgcagagcccacaggtcatgggaaacatgtggctgcagggagagtttggggacagtcaagtatggctgggaggtggacagccacggacactaagctcaggagatgtgaactttgtggtctggtcaaacagccactgcagatcacttcgcaggaggaggggtgactagaagtatgttactggaaggtaaatctggccacactgcagcatctggacggcagagggcagcgctgggaggggccagccagttagggcccaccacccctgggtgtctgagagtgggagtagcgggcaggggccagcaaagcacgagggcagagcaggggaccatacggagggtgggtgtggaagaagggaggggccccatgcaagctgcaggtctggggagcctgaggatgtcatagggcttcctggtagagtggaaagtgcactcctgaaggtcagggccagtcactacagagaggggacagcgaggagagggacggtgtggccctaagggtgactgcagtttctcaacatgtggtccgtggatcacctgcatgggaactgcctggggaatgcgctcatttgcagattcccgggccttcctccagaactactgggcaagcatctgccgggtcatgcccggtaacctacattcttaacaccagctgccctctccaccaccacgagccccaaaggtggggaaaagtctgcaagccacctgcagaggaagaatagggtgttaaggactggctttaggcaaaaagaagagacaaaaagaatgagggaggtctgggagtgagggaagtggtgggaagcagggaaagtccggtcaagccatgtgcaccaagacagagccccagcgcggccttgcagccaggcaccgggccgtccccaagggctgctctcagtccgctttcacttggtgggcgaaagccacatttgcaaactgggaagtggagagtgggaggtgaggggaagcactagcaatgaatgaagaggattcttccgggaatcaggctgtttcaatctaaaacatccaagataagtggaaacactggggaggaaggtgatgaacagacggaggtgagccagagacacctcctgggcaagtcggccaggaggcgggaggcgtgggtcagagacactgcaggaactgggtgaggacaaggaggtgcgaggaaaggggttgggggatggtcccacaggcagccacacctgaggcgtgggaggcaggtaggagctgggggagggcggggagaagaggggtttctgtgtgtagatctgagtcctccctcacatcccagccgtgccacaagccgcatcggcatgaggccggctctcccttcttcactggtctcaaaagccacccaggcccaagtcccggccagacagccgagcctgcctagcaacgctgaccggccgcccaggatggcccagacaccttctgtctcctgaatgcagcctacaggggttcaaacagactgcttgcattaaggtcagacaaggctcttttacttccagagacagcggcctggagcctcgggaagaatgtaggcccaggaatcacccagcccctcaggacaacctctctgagcaacagacatcctccctgttgaatgagagtgacatctctgccctgccacctactttacatggatgccacgaagtgggagagcctgagcagtagacagggaagaggcgagcggccccactgcaggaggtagacaggctacagatacttatgcagcagccacactgaggctagtactggaggaggctgagaaccagtaatgagttcttaatggtttgataatttgggtttttaaatattaaatattaaatatcaggggtttcggaaggaatgatgaattccgtctcatgctgtaactgatgaaggcaaccaatgagcaatccttccttcccatagccgagaaagggaaaggggacaggccaatccctctgaagcagtaagtcagaacacgaagacttacagaactcaaacatcaaaggtcaagtagcttctagccaggaaaagtggtggccccctcagcctagccagcaccaaccagcatgggtggagactcagcctggcagtaagggcatttcctgggtttcctctgaagcagaggagaaatagtgggtcagccaggctgctggactgaaccatgagccagaaggccagaatcactgcaagacagctccagcccgcacacctcagttgtgcttttgaaaacaggtacaaagctgaggcatgggagctgtgactgaagtcgccctcctggctggcctcgtcttctacctctgcttccacagctgggtgacttggccataggcccaaacaatggacaaccagttccacattaggaggcatcacggacgcatctgagaggaaacatgattgaaggacaagcttggcctcatggagggctctggattcatcccttgaagaacgcagtgatcaaacaaaaccaagaagcaggcctggagggagcactctgggatgcccccaagtcccctcaccatttacaaaccagcactgagttctcagcctccgctcctcaggactaggagacaagatccggacaggcaggacaggcagcaagccgactgtgagcagcctgggggcgcaggtgtaaaatacaaagccctttgaaggtccagacaataagagtaaagatgttaagattgcccaggaaaagaacttcactgacactgaatttgggcaacacctagaacagacaatattaagatatcaattctgagaaagactcacaggaaaggctgtttaggaggacactagagacaaacacagggaaaataaatacaggggctctgggatccccccacagaagctactaatgctatttattggcttgggtcacttttgagaatagaaaaccattttttggcaaagctgtacaaactccacatcagggcgtctcctgcagttggggacacaagatggccacagtgaccgggctcttcattaaacttcctcataacccgctacggtgttcagaagctaagacgtgacttccagagccaggccaggcatgtggaggcccctgactgtgggcgtgtcaagccctggctggggagcctgctgcctgcccggccactcctcagctgtggctgtggctgtgggcatggccggacggcgtgcacactgggccgtccccttttgcgcagggtggaagggggaaggagggtgggactccatgggctccacgatgtcttctagccctggtattctgtgagactaacttcgccctggtcattcaccatggctaggcaccaagtgccatctagtggcaccgcgggtccactttcacaacactccaaccaaagactgcagaacaaaccaactcttacccactttaactccgggggtgagggcagaggaggctggaagggtgagcacacttcatggtagtgatgggacatactcatctcaagaaaatatactttaagacgtcttgctttccttaagaaagcaacacttttttttttatttatttataaaggctaaccatatccatttgtcaatattttcggctttaaggaaaatagtttaaaaaacataaaaaggtaaatacactcaagagtaactgctattaaacagttctgaacaggcagaaaatgtagactttcctttaacagaaaatgttaaatctgtaatagcagcataatttatatatagaaaaaagctggttttgaaaacccagatttatacccaaaacattttttttctgtacaactgcgtttacactgggaaataagtttcttcacattatgttcattcccatcaggtacaggtgtgagcttgagtttgatcagccagccctgagcgcaagctcagcgctcagcacaatcttcaatccaacaccatggcagaaagcgcatttagatctttcatgtatgggtgggccaccaagatctggtctattttcagtctttgctctgagtcagggaagatcttcagaagggcttccctcagctcgttggtttctgcagaagatctctgagctggcatgggcaggttctgctggagactggggagggctggcagcagtgggaagtggggctgctgagggagccagtggcttgaaggggctccctgaatccgggtcggaggctggtggctggtgctggctgcctgggtgccagggactctgaagctggggtcaaacatgcccacatttggcagggcactgagtaggggctgcatatctctttttgtaataatttctctccaagagactgactcattcacaaattctctgaaattatcatttgtcacaattatgccaccagttttgtccgctaagtgtagtagaaacctgtcatcatgagaagcaattctttctccaaagaccatccgggcaggagttaaagataatattccgagctcctggagctgggttaagaagtgctgttctgtgacattaggatcacgccttgttctccactgagggacaaatacagtgatgtttctgttgccaagcttccaaaaatattcaactgcaattgcaattccacgacaagaaaagaactttttcagaccatgggtaattgcaacattgctcccatctataacaatgtgtttcaaatccgttctccctggttcattttttaattccagcttgtagggtatttttagagtatctcgaaacctttgaaccccagtaactgaggaatcaatatgatcagaaggtcctgccgaccttgcatcagtaaccgaaggtaacagctggggcagtggcattggtggagaaagggttgagcaatttggcttagaatgaggagaactacaacatcctaaacgtttttcacaggcagatttcatattatttggaagcaagggttctggctgctggtgtaaaccattttcaggaaaaagtggaactctgggctggtgacttgaagctccccttgaaacaaaattgacttctttgggacttggagaggcaacagaaggtgaaaggccatcagtttcagggtctgtgttacaaatgtagttctggtttgaaccccagacttcatgtttctgttctattggcactgttctgaaagtattaattctacaatttgaggtacatggtttagcttccactttgaatggtaactgagaaaatttttctaccatattttgctgtgtgtgagcctgtgttttctttggagtggaatcagttgtaagctcatttgtgctgctataaacacctttatttttggttttgttggtctctggatacactgtaccagctgaaaattctctgtcttcttggaatcttttattttctttttcaatttcctctaagagcaataatggttcagtagatggtccatacaccttaatgaccttttcaacaatttcttgggagtagcccatggttttaaaaaagtttacgaggatgttgtattccatttcctcagtagtttcttttatatctggacttaaattttcagaatcagcagaagaatcagataggtcagctattacatttccagccaatgtcttagcatcgtgtaaaatctccccctcctgaacattttccaaagaaaactgcttcttcgtatgcctttcttcagaatcagaaaatctccttttctgacaaattctctcattggaaagtgcctcttcatctggggttagaccatttattggatcaaaaagcacatctggtgagctagaaaggactgtgtccatttgttttgtaagctcagaaacaggagtcccagctttatttcttgcctcttcctgcaaaacagtttcatctctagaaatattcagccctgtggcagcattctgtgtaaactctgtttgttgagaatctctcatttcaataacctcatcatctcctgtttcaaagagattctcctcaccttgtgtgagtgtcaaaagttcttttttcaaggaagtgggcaaaatcaacaaatccattgtgtaattgtctgcatgggcttcaacaaattgtttgaattcccttttcacctctgattctttctgactactgggtaggttctctttattttcaaagagctttacaaattgttgaatgtgactcctagccatgaccacagcctcagcacttcctctgatgccaagaaggccaatgtccagaatgcagaggtcagcacaagtatcctgaatcaagcttttcagaaacaggctctctgccccaacaaaaatgcagtgcatgtccttggggtaacattctctttcttctagttcaggttcacagattcctttaatatattccttggcgctgtgcaccgcctcctgcgccccgcagagctgcagccagatgcgcgcgggcagcggctcctcagcccctagcgcgccgagcacggctaggctcacgccaaacaggccctcgatacggccgcggctctgctccagcagctccgccttctcagctggcgcagtgaactcgtccagcaccgcccgggccgccatggcgggcgcggcctcccgcggcggcgccgggggccggcggcggcgacgccccctcagcttgctgccgctgctcccaagccagtcaggcggcgtcggcccttcccggccgcctcgcccccgcccgcgccccgccgcccgccctcaggcccggctataccatcccgccacgaccgcagcagcttggcaattgctggcagcgaacccctccgcccctttgccgccgccgcgggccgggccccgcc

SEQ ID NO: 17815 - RNA, 6812 nt, Homo sapiens
  source 1..6812: mol_type = other RNA
tcgaggagctcacagtctagaaagggcagcaagacagtacacaatcagtggcagcagcaccagccagagtggcaagtgctcaaagcgagacacaaagtgctgtgcggtcacaacatcatggggatgcttctggcagaagcactggaaaggagacgaggactcaggctgggccttccaggagggaagccatttgggagaagggcatctctagcggagagaggtccatctgcagagcccacaggtcatgggaaacatgtggctgcagggagagtttggggacagtcaagtatggctgggaggtggacagccacggacactaagctcaggagatgtgaactttgtggtctggtcaaacagccactgcagatcacttcgcaggaggaggggtgactagaagtatgttactggaaggtaaatctggccacactgcagcatctggacggcagagggcagcgctgggaggggccagccagttagggcccaccacccctgggtgtctgagagtgggagtagcgggcaggggccagcaaagcacgagggcagagcaggggaccatacggagggtgggtgtggaagaagggaggggccccatgcaagctgcaggtctggggagcctgaggatgtcatagggcttcctggtagagtggaaagtgcactcctgaaggtcagggccagtcactacagagaggggacagcgaggagagggacggtgtggccctaagggtgactgcagtttctcaacatgtggtccgtggatcacctgcatgggaactgcctggggaatgcgctcatttgcagattcccgggccttcctccagaactactgggcaagcatctgccgggtcatgcccggtaacctacattcttaacaccagctgccctctccaccaccacgagccccaaaggtggggaaaagtctgcaagccacctgcagaggaagaatagggtgttaaggactggctttaggcaaaaagaagagacaaaaagaatgagggaggtctgggagtgagggaagtggtgggaagcagggaaagtccggtcaagccatgtgcaccaagacagagccccagcgcggccttgcagccaggcaccgggccgtccccaagggctgctctcagtccgctttcacttggtgggcgaaagccacatttgcaaactgggaagtggagagtgggaggtgaggggaagcactagcaatgaatgaagaggattcttccgggaatcaggctgtttcaatctaaaacatccaagataagtggaaacactggggaggaaggtgatgaacagacggaggtgagccagagacacctcctgggcaagtcggccaggaggcgggaggcgtgggtcagagacactgcaggaactgggtgaggacaaggaggtgcgaggaaaggggttgggggatggtcccacaggcagccacacctgaggcgtgggaggcaggtaggagctgggggagggcggggagaagaggggtttctgtgtgtagatctgagtcctccctcacatcccagccgtgccacaagccgcatcggcatgaggccggctctcccttcttcactggtctcaaaagccacccaggcccaagtcccggccagacagccgagcctgcctagcaacgctgaccggccgcccaggatggcccagacaccttctgtctcctgaatgcagcctacaggggttcaaacagactgcttgcattaaggtcagacaaggctcttttacttccagagacagcggcctggagcctcgggaagaatgtaggcccaggaatcacccagcccctcaggacaacctctctgagcaacagacatcctccctgttgaatgagagtgacatctctgccctgccacctactttacatggatgccacgaagtgggagagcctgagcagtagacagggaagaggcgagcggccccactgcaggaggtagacaggctacagatacttatgcagcagccacactgaggctagtactggaggaggctgagaaccagtaatgagttcttaatggtttgataatttgggtttttaaatattaaatattaaatatcaggggtttcggaaggaatgatgaattccgtctcatgctgtaactgatgaaggcaaccaatgagcaatccttccttcccatagccgagaaagggaaaggggacaggccaatccctctgaagcagtaagtcagaacacgaagacttacagaactcaaacatcaaaggtcaagtagcttctagccaggaaaagtggtggccccctcagcctagccagcaccaaccagcatgggtggagactcagcctggcagtaagggcatttcctgggtttcctctgaagcagaggagaaatagtgggtcagccaggctgctggactgaaccatgagccagaaggccagaatcactgcaagacagctccagcccgcacacctcagttgtgcttttgaaaacaggtacaaagctgaggcatgggagctgtgactgaagtcgccctcctggctggcctcgtcttctacctctgcttccacagctgggtgacttggccataggcccaaacaatggacaaccagttccacattaggaggcatcacggacgcatctgagaggaaacatgattgaaggacaagcttggcctcatggagggctctggattcatcccttgaagaacgcagtgatcaaacaaaaccaagaagcaggcctggagggagcactctgggatgcccccaagtcccctcaccatttacaaaccagcactgagttctcagcctccgctcctcaggactaggagacaagatccggacaggcaggacaggcagcaagccgactgtgagcagcctgggggcgcaggtgtaaaatacaaagccctttgaaggtccagacaataagagtaaagatgttaagattgcccaggaaaagaacttcactgacactgaatttgggcaacacctagaacagacaatattaagatatcaattctgagaaagactcacaggaaaggctgtttaggaggacactagagacaaacacagggaaaataaatacaggggctctgggatccccccacagaagctactaatgctatttattggcttgggtcacttttgagaatagaaaaccattttttggcaaagctgtacaaactccacatcagggcgtctcctgcagttggggacacaagatggccacagtgaccgggctcttcattaaacttcctcataacccgctacggtgttcagaagctaagacgtgacttccagagccaggccaggcatgtggaggcccctgactgtgggcgtgtcaagccctggctggggagcctgctgcctgcccggccactcctcagctgtggctgtggctgtgggcatggccggacggcgtgcacactgggccgtccccttttgcgcagggtggaagggggaaggagggtgggactccatgggctccacgatgtcttctagccctggtattctgtgagactaacttcgccctggtcattcaccatggctaggcaccaagtgccatctagtggcaccgcgggtccactttcacaacactccaaccaaagactgcagaacaaaccaactcttacccactttaactccgggggtgagggcagaggaggctggaagggtgagcacacttcatggtagtgatgggacatactcatctcaagaaaatatactttaagacgtcttgctttccttaagaaagcaacacttttttttttatttatttataaaggctaaccatatccatttgtcaatattttcggctttaaggaaaatagtttaaaaaacataaaaaggtaaatacactcaagagtaactgctattaaacagttctgaacaggcagaaaatgtagactttcctttaacagaaaatgttaaatctgtaatagcagcataatttatatatagaaaaaagctggttttgaaaacccagatttatacccaaaacattttttttctgtacaactgcgtttacactgggaaataagtttcttcacattatgttcattcccatcaggtacaggtgtgagcttgagtttgatcagccagccctgagcgcaagctcagcgctcagcacaatcttcaatccaacaccatggcagaaagcgcatttagatctttcatgtatgggtgggccaccaagatctggtctattttcagtctttgctctgagtcagggaagatcttcagaagggcttccctcagctcgttggtttctgcagaagatctctgagctggcatgggcaggttctgctggagactggggagggctggcagcagtgggaagtggggctgctgagggagccagtggcttgaaggggctccctgaatccgggtcggaggctggtggctggtgctggctgcctgggtgccagggactctgaagctggggtcaaacatgcccacatttggcagggcactgagtaggggctgcatatctctttttgtaataatttctctccaagagactgactcattcacaaattctctgaaattatcatttgtcacaattatgccaccagttttgtccgctaagtgtagtagaaacctgtgacattaggatcacgccttgttctccactgagggacaaatacagtgatgtttctgttgccaagcttccaaaaatattcaactgcaattgcaattccacgacaagaaaagaactttttcagaccatgggtaattgcaacattgctcccatctataacaatgtgtttcaaatccgttctccctggttcattttttaattccagcttgtagggtatttttagagtatctcgaaacctttgaaccccagtaactgaggaatcaatatgatcagaaggtcctgccgaccttgcatcagtaaccgaaggtaacagctggggcagtggcattggtggagaaagggttgagcaatttggcttagaatgaggagaactacaacatcctaaacgtttttcacaggcagatttcatattatttggaagcaagggttctggctgctggtgtaaaccattttcaggaaaaagtggaactctgggctggtgacttgaagctccccttgaaacaaaattgacttctttgggacttggagaggcaacagaaggtgaaaggccatcagtttcagggtctgtgttacaaatgtagttctggtttgaaccccagacttcatgtttctgttctattggcactgttctgaaagtattaattctacaatttgaggtacatggtttagcttccactttgaatggtaactgagaaaatttttctaccatattttgctgtgtgtgagcctgtgttttctttggagtggaatcagttgtaagctcatttgtgctgctataaacacctttatttttggttttgttggtctctggatacactgtaccagctgaaaattctctgtcttcttggaatcttttattttctttttcaatttcctctaagagcaataatggttcagtagatggtccatacaccttaatgaccttttcaacaatttcttgggagtagcccatggttttaaaaaagtttacgaggatgttgtattccatttcctcagtagtttcttttatatctggacttaaattttcagaatcagcagaagaatcagataggtcagctattacatttccagccaatgtcttagcatcgtgtaaaatctccccctcctgaacattttccaaagaaaactgcttcttcgtatgcctttcttcagaatcagaaaatctccttttctgacaaattctctcattggaaagtgcctcttcatctggggttagaccatttattggatcaaaaagcacatctggtgagctagaaaggactgtgtccatttgttttgtaagctcagaaacaggagtcccagctttatttcttgcctcttcctgcaaaacagtttcatctctagaaatattcagccctgtggcagcattctgtgtaaactctgtttgttgagaatctctcatttcaataacctcatcatctcctgtttcaaagagattctcctcaccttgtgtgagtgtcaaaagttcttttttcaaggaagtgggcaaaatcaacaaatccattgtgtaattgtctgcatgggcttcaacaaattgtttgaattcccttttcacctctgattctttctgactactgggtaggttctctttattttcaaagagctttacaaattgttgaatgtgactcctagccatgaccacagcctcagcacttcctctgatgccaagaaggccaatgtccagaatgcagaggtcagcacaagtatcctgaatcaagcttttcagaaacaggctctctgccccaacaaaaatgcagtgcatgtccttggggtaacattctctttcttctagttcaggttcacagattcctttaatatattccttggcgctgtgcaccgcctcctgcgccccgcagagctgcagccagatgcgcgcgggcagcggctcctcagcccctagcgcgccgagcacggctaggctcacgccaaacaggccctcgatacggccgcggctctgctccagcagctccgccttctcagctggcgcagtgaactcgtccagcaccgcccgggccgccatggcgggcgcggcctcccgcggcggcgccgggggccggcggcggcgacgccccctcagcttgctgccgctgctcccaagccagtcaggcggcgtcggcccttcccggccgcctcgcccccgcccgcgccccgccgcccgccctcaggcccggctataccatcccgccacgaccgcagcagcttggcaattgctggcagcgaacccctccgcccctttgccgccgccgcgggccgggccccgcc

SEQ ID NO: 17816 - RNA, 6777 nt, Homo sapiens
  source 1..6777: mol_type = other RNA
tcgaggagctcacagtctagaaatggagatggaaacataaacaaataaatcacacattggggtagtgtgacaataaaaggtatatacaaggcacaggtttagcatagagaaggtccctagcttgaactagggatgggaggattaggaaagacttgctggattagatgatgataagtcatctcgctctgtttccttaatttcattgtgagctctttgagaacaagggttatgtcttattcactttagtgtcctcatcacctaacataatacctagcacattgtagatagtcaagatctatcagtggaatttacttgaacgtgtaggaagctggttctaaaaggcaaagtgtctagaggcccagttttttaatattcaaaatcttctttttgtttggtttggttccagctttgcctctgcctgtgtgtgcctgcatgtttgaaatgataacaaagctgttttccttggttacgttgattgcgaaactgtccttactatatgggctgtcacatatgctgattttattctctctttcatttagatattttcttaatttattaacttgaaaaattatgttcatttaattaactagtttaagaaaatttttagagatcaaacaaactaatgagattttacagatttttgaaaaataatgttttcttctttatggaaacatgtatttgcaaacattaacattgacttcaaataattattacaaatcaagttaaaagtatagatgtccttggtgttagaccagtttaacatgttattacacgatacgggggtgttgaatcctatttaagtctgtctttgaaaccatgaaacctgatacagtttcattaaattgaatggaaattgtgttttaaaatgagctaataaaacaaagattttaacatattatactagtggctccatattaataaaatgcttgtctgtgacctttaagataagcaatttcaataacagtcatctgacatctttgtggatcctgaataaaaccaaactgattatgaaaatgacacattataaaaatttatccctacatttcctttttaggtatgacattaaaaagaacaatacttaatttaaagggcataaaaattcacatcatcaccataaatatagaacccagtttacagatgactacaatgaagaaatctgttagctaattatgtagcaacctgactctggttctcaacattttatgagcttatgttccttaacaccatatgttatagggaacagtaaagacatctgaattcaaatattttgaagaaatgtgtatttagcaagtgaatacatgctaaaaggaataatttacagcagcagtttcattacatttttctctccagtttttctagttcccatctgaaatgcaatgataagtaaagatatggaacatatttcctacctggcaaaaaacatgcttattgaacgggcacgcaccttccgcccttaaatagtacataaaccaccttgtcacctgcgtgggaaaatcttgccttttaggatgatgttgaacacattgaaatggagtacttatagaaagttttattttacactgttcttcctctttttctcccaaattatttacatcttttttttgcctaatgtgtaggtagcaaaaatattaaacacataccactgcaaattactaaataatacataaaatgaagtgtgcatttacatgcatttacattttacatttgatatcaactgggccataatgtctctgctgtgatgcatctttttcatactttaagactgctgttgtaattttcgtaaggtcacatgagtctctcaaacagtttcatctctgatgattcatgcatatgacaaagtctatttaaagctgaattattaaatgggccaataattctttttcgtgcaaactgccccctctcaatacacatgggcagagattatgactgtaatgagttatctgcaagttatatctacaattttctttgaaaacttagacctgatggtatataaagacatgcctgtagatttgtttgtttgtgtaacttttaattgaagtcgagacttttttctattgtcatttcataacactaaacaaaatgcattcaaattctgaaagtcttctataaatttatcatataatctctatcccttcaaatcctttatttctgaggatgaataataagatatttctgctatcgcaaataaatttatttcagctgcaaatttagaatgaaacacaacactgaatgttagtacagtttagatactttatgaaaataaaagaatgacctattttttggagcactctttgttcttcgatttatatttgaaacactactttctgtacagtggtgtgtccttcaaataatttaacaatttggcttccatgtgaggatatacagtacttccaaaagcaacaccatattagtcaatggagcctaaaattgaatgtagattatttttaggcttttgtttgaaacaagtggcaacaacttgtttattcaaggcagtcattaaaactgaaacatgagcttccatctgtgaaatatttcagctgataggaaataaaaattcactgtagtctgaggtgagaaattgatgctgagttaattagaatccaaagacagctagagttagaatttcaatgttgcttcattaattactaataagatgttttctttgcatttttgtgcatgatgaggaacctgggggaggagtcctgaataggtgagtgcagtgcaaaagaaaccacagtataatgctgaaagttttaaatatctcaaagtcagtgattctcaacgaatcgtcttaggacaatgaaggaagcaaatcttgaattttagtcttttaccttattttgtaagttgttgcaggaaacaaagaattttacattgtttaaatgtgggttgcatcctggaaaatactttgtagaaaagtccctcccattgatatgaaaagagtcatgtgtttcttgtacaaataattgtcttaaataaggaaaggtaagaggcacctgatacagatgtaaatgattggaaactttgcctttaacatgttgctctgaatagttattgatctctctcttttaaaaaaattaagtgacacagatataattcttggtagaatcataagagagatcttagtctcaaatatcatgcagggattcaagcacggaattaagacacattttctattaacagtatattaagacaatgcttattattttcatgaaatatgcagttccttttcccttcattgattcattatagtaaaatgcacttaaaaatcaacttgtttcttccttttttcctgcttaaatgttctgtttttttttctaagaacattatgcaagtaaaaattaatttagataatgcttaaagaaggggaggtgtgaacagcttccatttgtttgattttctcagagaaataaagcataatttatatcctggttttagagattcactcttaatgatgtatatgtgtttctagaacaatgtcatctatccctcttatagaattgaaaataaaatgtccaaagaaagcagcacaccattggaatttttaaaacaaaaactacatagcacaataattgtaagacaaatcctactctagcttagaaaacaactaatttttactgcatatttttcatggtacatttaaattatagttttaataaaatacatctttagatcaaagctgaaagaagacatcagtagtagatcagtgtattccatttttcttctggatgatggatggcttatgtttttttttttttttaatatttccacagaacatttcattcagtatcattttactcattttactcctcaagtacatacaaacatgagggccggtagacaaaatatatccttgaatccaaccacgttttggaatattcatcagcttagtaaatccatgcagttcattttaaacttttagttcaatacaatggctttgctgatgcagtttttctcctttagatggcaatatggcaaatgacatttttatttctcaggcaaagaagaaagacaaacctgtacagtgaaatctcataggaaacattaagtctgctaaagtgaacatctgcattcacctgtgttctctgttaggtggtggtattaggaaaaaaagcctattaggaaagttactcatggatttaatttataattggtggaactcagctgaatttcccaccattgtaaacatccacataatgccatgaaaaaagttcatgtatattgcatttgtttttccagttattgtctaggcaagtttctacttgtttgaggtttctagaggtaatgcagctcagacactcctgggtgccctctcaaattcgtgggtcctcctgtttctacctttcttattttcttgtaagtgcttccatttgttactgttccctggggtatgtcctggcctttgccgacgttgttttcggtcccttttccaaacttgttcacagaactcatccattgtgttgagattggggtggttgatgagctgcatgaagtctctgtaccagaccttctggctaggtgtcatgctattggacatttctttggtcttagagccatctccatcatcatctttatgaagaagttcttccaaatgctctgtgtcaatgacttccagggttaccttaagaagagtttgtatgaacccatgttccaccgcatggcagaggtaattgcctgaatccttctgttgtagactacgtagcagaaggccttgatctgtcctgatgatatgatcatccactctgatctcttcttttcgctcttcatttcgcctctggaattgccaatagaccagcgctctctgcgacttcggactgcattccaaaaatgtgctactattctctacaccatagatgattctctcttcagggctgtggccatggtgattatcatggtgtaagtctgaacagtgagtcagtgggtctccatttcttatatcttgtcgtcttgtgcgtctctttgcagtgggaaaatagcgagaacatgcagaaccatcccaagcacagtaagggtctcgggcgaggcaacactcagcacacgctttcccgtaaatatcacaccggtgtaaagggagctgggcaaccccagccgttgaaccaatatatagttgttgctgcttagtggaaagctccattgctgaaatagcagtcggttcccgaaaaactgtcatttcttccagcagaacctcttctaaatcataccaagtctccttaggaattgaaactactttaagaacggtcccaacatctgttccgataaacataacatcatactgtccatcttctgcatccactcggtctacgacaatttgtgtaaattgataatttacatccgttttgatcactattgggcgattgttcataggaaacactggattgtacatggctggatgacttcttgcaaaggttataacatcatcaggaaggtcctttgtagagtcaaaaccaccaaatgttttgctgggacaagttcctggccgtggataggggactcttccttgataaggcacccattgatagttgggtccatccctgtgggcatatggaccaaggaacacccttctcacatcactcatgctatacatacacacggctgatcccttgaaaatgttactggaagtcgtaaacactccatatacaactggatttttaggatctttaaagttcattaggaatacatcctgcagttcatcaaaatgagtgtcaatgccatttggacctggcactgagcaaatcagacgagctttgaggaatgttgtccatttattcaccagacttctgtgccctccaaagtcattcttgcatatctgacctattctagcgtgagtagcttttccagagtgttctccatctattgcattttcacggaagaaaaagtatactttgtcatcttcaggattgtcactctctgagatgaggtgggcactaatgaactttggatcattgagccacctggaatcatgctgctctgtcctgattgggtggtggtgcccaagagttcggaagatagcaaagtctcgccccataaaatcagctgcagttccagagtataattctccatctattaaaagggatgctgtcagcagcttagggtcatatggactcttcccacggccgttttcaaaatgtgagttctccagcttaaaaatattgtcctcaggatgatgtccaatttcaatgtaggtgcaaattggatgaaaagcccccgttccacaggcgtacaagtgagtctgattatatgccttaagtaccttgatgaaattagcacattctttcaggatgtcttttccagcccacttgcattcatctcttctggtgtaagatactggccacacaatcttttgaaaatccttgatattaaccaggtcgaatgaaaatatgtgatcctttgctccaacatacagcctactccgttcctcatccaaaaggaaggtatgataactggagctgttggccaagccattgaaagtgatcacattgttggattccaacatttctttgtaggataatttcagccttggcacattgttcttcccattctgatagtttgctcttgctgtaagtaatactccccagaaaagacagacaatcctagttaaccagcccatgctgcagacgctgtaggtccctttgctgctttagtcttccttcctgtattgtgcggccagagaagttcaaacaatctggaaaaaaatttacaattcatgctcattatacaatcctgctgaacttgtgcattgtatgtgtgcgtgtgtgtgtgtgtgtgtgtgtgtgtgtc

SEQ ID NO: 17817 - RNA, 6810 nt, Homo sapiens
  source 1..6810: mol_type = other RNA
tcgaggagctcacagtctagaaatggagatggaaacataaacaaataaatcacacattggggtagtgtgacaataaaaggtatatacaaggcacaggtttagcatagagaaggtccctagcttgaactagggatgggaggattaggaaagacttgctggattagatgatgataagtcatctcgctctgtttccttaatttcattgtgagctctttgagaacaagggttatgtcttattcactttagtgtcctcatcacctaacataatacctagcacattgtagatagtcaagatctatcagtggaatttacttgaacgtgtaggaagctggttctaaaaggcaaagtgtctagaggcccagttttttaatattcaaaatcttctttttgtttggtttggttccagctttgcctctgcctgtgtgtgcctgcatgtttgaaatgataacaaagctgttttccttggttacgttgattgcgaaactgtccttactatatgggctgtcacatatgctgattttattctctctttcatttagatattttcttaatttattaacttgaaaaattatgttcatttaattaactagtttaagaaaatttttagagatcaaacaaactaatgagattttacagatttttgaaaaataatgttttcttctttatggaaacatgtatttgcaaacattaacattgacttcaaataattattacaaatcaagttaaaagtatagatgtccttggtgttagaccagtttaacatgttattacacgatacgggggtgttgaatcctatttaagtctgtctttgaaaccatgaaacctgatacagtttcattaaattgaatggaaattgtgttttaaaatgagctaataaaacaaagattttaacatattatactagtggctccatattaataaaatgcttgtctgtgacctttaagataagcaatttcaataacagtcatctgacatctttgtggatcctgaataaaaccaaactgattatgaaaatgacacattataaaaatttatccctacatttcctttttaggtatgacattaaaaagaacaatacttaatttaaagggcataaaaattcacatcatcaccataaatatagaacccagtttacagatgactacaatgaagaaatctgttagctaattatgtagcaacctgactctggttctcaacattttatgagcttatgttccttaacaccatatgttatagggaacagtaaagacatctgaattcaaatattttgaagaaatgtgtatttagcaagtgaatacatgctaaaaggaataatttacagcagcagtttcattacatttttctctccagtttttctagttcccatctgaaatgcaatgataagtaaagatatggaacatatttcctacctggcaaaaaacatgcttattgaacgggcacgcaccttccgcccttaaatagtacataaaccaccttgtcacctgcgtgggaaaatcttgccttttaggatgatgttgaacacattgaaatggagtacttatagaaagttttattttacactgttcttcctctttttctcccaaattatttacatcttttttttgcctaatgtgtaggtagcaaaaatattaaacacataccactgcaaattactaaataatacataaaatgaagtgtgcatttacatgcatttacattttacatttgatatcaactgggccataatgtctctgctgtgatgcatctttttcatactttaagactgctgttgtaattttcgtaaggtcacatgagtctctcaaacagtttcatctctgatgattcatgcatatgacaaagtctatttaaagctgaattattaaatgggccaataattctttttcgtgcaaactgccccctctcaatacacatgggcagagattatgactgtaatgagttatctgcaagttatatctacaattttctttgaaaacttagacctgatggtatataaagacatgcctgtagatttgtttgtttgtgtaacttttaattgaagtcgagacttttttctattgtcatttcataacactaaacaaaatgcattcaaattctgaaagtcttctataaatttatcatataatctctatcccttcaaatcctttatttctgaggatgaataataagatatttctgctatcgcaaataaatttatttcagctgcaaatttagaatgaaacacaacactgaatgttagtacagtttagatactttatgaaaataaaagaatgacctattttttggagcactctttgttcttcgatttatatttgaaacactactttctgtacagtggtgtgtccttcaaataatttaacaatttggcttccatgtgaggatatacagtacttccaaaagcaacaccatattagtcaatggagcctaaaattgaatgtagattatttttaggcttttgtttgaaacaagtggcaacaacttgtttattcaaggcagtcattaaaactgaaacatgagcttccatctgtgaaatatttcagctgataggaaataaaaattcactgtagtctgaggtgagaaattgatgctgagttaattagaatccaaagacagctagagttagaatttcaatgttgcttcattaattactaataagatgttttctttgcatttttgtgcatgatgaggaacctgggggaggagtcctgaataggtgagtgcagtgcaaaagaaaccacagtataatgctgaaagttttaaatatctcaaagtcagtgattctcaacgaatcgtcttaggacaatgaaggaagcaaatcttgaattttagtcttttaccttattttgtaagttgttgcaggaaacaaagaattttacattgtttaaatgtgggttgcatcctggaaaatactttgtagaaaagtccctcccattgatatgaaaagagtcatgtgtttcttgtacaaataattgtcttaaataaggaaaggtaagaggcacctgatacagatgtaaatgattggaaactttgcctttaacatgttgctctgaatagttattgatctctctcttttaaaaaaattaagtgacacagatataattcttggtagaatcataagagagatcttagtctcaaatatcatgcagggattcaagcacggaattaagacacattttctattaacagtatattaagacaatgcttattattttcatgaaatatgcagttccttttcccttcattgattcattatagtaaaatgcacttaaaaatcaacttgtttcttccttttttcctgcttaaatgttctgtttttttttctaagaacattatgcaagtaaaaattaatttagataatgcttaaagaaggggaggtgtgaacagcttccatttgtttgattttctcagagaaataaagcataatttatatcctggttttagagattcactcttaatgatgtatatgtgtttctagaacaatgtcatctatccctcttatagaattgaaaataaaatgtccaaagaaagcagcacaccattggaatttttaaaacaaaaactacatagcacaataattgtaagacaaatcctactctagcttagaaaacaactaatttttactgcatatttttcatggtacatttaaattatagttttaataaaatacatctttagatcaaagctgaaagaagacatcagtagtagatcagtgtattccatttttcttctggatgatggatggcttatgtttttttttttttttaatatttccacagaacatttcattcagtatcattttactcattttactcctcaagtacatacaaacatgagggccggtagacaaaatatatccttgaatccaaccacgttttggaatattcatcagcttagtaaatccatgcagttcattttaaacttttagttcaatacaatggctttgctgatgcagtttttctcctttagatggcaatatggcaaatgacatttttatttctcaggcaaagaagaaagacaaacctgtacagtgaaatctcataggaaacattaagtctgctaaagtgaacatctgcattcacctgtgttctctgttaggtggtggtattaggaaaaaaagcctattaggaaagttactcatggatttaatttataattggtggaactcagctgaatttcccaccattgtaaacatccacataatgccatgaaaaaagttcatgtatattgcatttgtttttccagttattgtctaggcaagtttctacttgtttgaggtttctagaggtaatgcagctcagacactcctgggtgccctctcaaattcgtgggtcctcctgtttctacctttcttattttcttgtaagtgcttccatttgttactgttccctggggtatgtcctggcctttgccgacgttgttttcggtcccttttccaaacttgttcacagaactcatccattgtgttgagattggggtggttgatgagctgcatgaagtctctgtaccagaccttctggctaggtgtcatgctattggacatttctttggtcttagagccatctccatcatcatctttatgaagaagttcttccaaatgctctgtgtcaatgacttccagggttaccttaagaagagtttgtatgaacccatgttccaccgcatggcagaggtaattgcctgaatccttctgttgtagactacgtagcagaaggccttgatctgtcctgatgatatgatcatccactctgatctcttcttttcgctcttcatttcgcctctggaattgccaatagaccagcgctctctgcgacttcggactgcattccaaaaatgtgctactattctctacaccatagatgattctctcttcagggctgtggccatggtgattatcatggtgtaagtctgaacagtgagtcagtgggtctccatttcttatatcttgtcgtcttgtgcgtctctttgcagtgggaaaatagcgagaacatgcagaaccatcccaagcacagtaagggtctcgggcgaggcaacactcagcacacgctttcccgtaaatatcacaccggtgtaaagggagctgggcaaccccagccgttgaaccaatatatagttgttgctgcttagtggaaagctccattgctgaaatagcagtcggttcccgaaaaactgtcatttcttccagcagaacctcttctaaatcataccaagtctccttaggaattgaaactactttaagaacggtcccaacatctgttccgataaacataacatcatactgtccatcttctgcatccactcggtctacgacaatttgtgtaaattgataatttacatccgttttgatcactattgggcgattgttcataggaaacactggattgtacatggctggatgacttcttgcaaaggttataacatcatcaggaaggtcctttgtagagtcaaaaccaccaaatgttttgctgggacaagttcctggccgtggataggggactcttccttgataaggcacccattgatagttgggtccatccctgtgggcatatggaccaaggaacacccttctcacatcactcatgctatacatacacacggctgatcccttgaaaatgttactggaagtcgtaaacactccatatacaactggatttttaggatctttaaagttcattaggaatacatcctgcagttcatcaaaatgagtgtcaatgccatttggacctggcactgagcaaatcagacgagctttgaggaatgttgtccatttattcaccagacttctgtgccctccaaagtcattcttgcatatctgacctattctagcgtgagtagcttttccagagtgttctccatctattgcattttcacggaagaaaaagtatactttgtcatcttcaggattgtcactctctgagatgaggtgggcactaatgaactttggatcattgagccacctggaatcatgctgctctgtcctgattgggtggtggtgcccaagagttcggaagatagcaaagtctcgccccataaaatcagctgcagttccagagtataattctccatctattaaaagggatgctgtcagcagcttagggtcatatggactcttcccacggccgttttcaaaatgtgagttctccagcttaaaaatattgtcctcaggatgatgtccaatttcaatgtaggtgcaaattggatgaaaagcccccgttccacaggcgtacaagtgagtctgattatatgccttaagtaccttgatgaaattagcacattctttcaggatgtcttttccagcccacttgcattcatctcttctggtgtaagatactggccacacaatcttttgaaaatccttgatattaaccaggtcgaatgaaaatatgtgatcctttgctccaacatacagcctactccgttcctcatccaaaaggaaggtatgataactggagctgttggccaagccattgaaagtgatcacattgttggattccaacatttctttgtaggataatttcagccttggcacattgttcttcccattctgatagtttgctcttgctgtaagtaatactccccagaaaagacagacaatcctagttaaccagcccatgctgcagacgctgtaggtccctttgctgctttagtcttccttcctgtattgtgcggccagagaagttcaaacaatctggaaactggaggtaacaggtgatttaggtcagtttcattcataaatgcagacaatcaagacctcatggcaacactaacacctcttcttctgtaacagtcactgaagcacagaaacttcaaaccctc

SEQ ID NO: 17818 - RNA, 6957 nt, Homo sapiens
  source 1..6957: mol_type = other RNA
tcgaggagctcacagtctagaaatggagatggaaacataaacaaataaatcacacattggggtagtgtgacaataaaaggtatatacaaggcacaggtttagcatagagaaggtccctagcttgaactagggatgggaggattaggaaagacttgctggattagatgatgataagtcatctcgctctgtttccttaatttcattgtgagctctttgagaacaagggttatgtcttattcactttagtgtcctcatcacctaacataatacctagcacattgtagatagtcaagatctatcagtggaatttacttgaacgtgtaggaagctggttctaaaaggcaaagtgtctagaggcccagttttttaatattcaaaatcttctttttgtttggtttggttccagctttgcctctgcctgtgtgtgcctgcatgtttgaaatgataacaaagctgttttccttggttacgttgattgcgaaactgtccttactatatgggctgtcacatatgctgattttattctctctttcatttagatattttcttaatttattaacttgaaaaattatgttcatttaattaactagtttaagaaaatttttagagatcaaacaaactaatgagattttacagatttttgaaaaataatgttttcttctttatggaaacatgtatttgcaaacattaacattgacttcaaataattattacaaatcaagttaaaagtatagatgtccttggtgttagaccagtttaacatgttattacacgatacgggggtgttgaatcctatttaagtctgtctttgaaaccatgaaacctgatacagtttcattaaattgaatggaaattgtgttttaaaatgagctaataaaacaaagattttaacatattatactagtggctccatattaataaaatgcttgtctgtgacctttaagataagcaatttcaataacagtcatctgacatctttgtggatcctgaataaaaccaaactgattatgaaaatgacacattataaaaatttatccctacatttcctttttaggtatgacattaaaaagaacaatacttaatttaaagggcataaaaattcacatcatcaccataaatatagaacccagtttacagatgactacaatgaagaaatctgttagctaattatgtagcaacctgactctggttctcaacattttatgagcttatgttccttaacaccatatgttatagggaacagtaaagacatctgaattcaaatattttgaagaaatgtgtatttagcaagtgaatacatgctaaaaggaataatttacagcagcagtttcattacatttttctctccagtttttctagttcccatctgaaatgcaatgataagtaaagatatggaacatatttcctacctggcaaaaaacatgcttattgaacgggcacgcaccttccgcccttaaatagtacataaaccaccttgtcacctgcgtgggaaaatcttgccttttaggatgatgttgaacacattgaaatggagtacttatagaaagttttattttacactgttcttcctctttttctcccaaattatttacatcttttttttgcctaatgtgtaggtagcaaaaatattaaacacataccactgcaaattactaaataatacataaaatgaagtgtgcatttacatgcatttacattttacatttgatatcaactgggccataatgtctctgctgtgatgcatctttttcatactttaagactgctgttgtaattttcgtaaggtcacatgagtctctcaaacagtttcatctctgatgattcatgcatatgacaaagtctatttaaagctgaattattaaatgggccaataattctttttcgtgcaaactgccccctctcaatacacatgggcagagattatgactgtaatgagttatctgcaagttatatctacaattttctttgaaaacttagacctgatggtatataaagacatgcctgtagatttgtttgtttgtgtaacttttaattgaagtcgagacttttttctattgtcatttcataacactaaacaaaatgcattcaaattctgaaagtcttctataaatttatcatataatctctatcccttcaaatcctttatttctgaggatgaataataagatatttctgctatcgcaaataaatttatttcagctgcaaatttagaatgaaacacaacactgaatgttagtacagtttagatactttatgaaaataaaagaatgacctattttttggagcactctttgttcttcgatttatatttgaaacactactttctgtacagtggtgtgtccttcaaataatttaacaatttggcttccatgtgaggatatacagtacttccaaaagcaacaccatattagtcaatggagcctaaaattgaatgtagattatttttaggcttttgtttgaaacaagtggcaacaacttgtttattcaaggcagtcattaaaactgaaacatgagcttccatctgtgaaatatttcagctgataggaaataaaaattcactgtagtctgaggtgagaaattgatgctgagttaattagaatccaaagacagctagagttagaatttcaatgttgcttcattaattactaataagatgttttctttgcatttttgtgcatgatgaggaacctgggggaggagtcctgaataggtgagtgcagtgcaaaagaaaccacagtataatgctgaaagttttaaatatctcaaagtcagtgattctcaacgaatcgtcttaggacaatgaaggaagcaaatcttgaattttagtcttttaccttattttgtaagttgttgcaggaaacaaagaattttacattgtttaaatgtgggttgcatcctggaaaatactttgtagaaaagtccctcccattgatatgaaaagagtcatgtgtttcttgtacaaataattgtcttaaataaggaaaggtaagaggcacctgatacagatgtaaatgattggaaactttgcctttaacatgttgctctgaatagttattgatctctctcttttaaaaaaattaagtgacacagatataattcttggtagaatcataagagagatcttagtctcaaatatcatgcagggattcaagcacggaattaagacacattttctattaacagtatattaagacaatgcttattattttcatgaaatatgcagttccttttcccttcattgattcattatagtaaaatgcacttaaaaatcaacttgtttcttccttttttcctgcttaaatgttctgtttttttttctaagaacattatgcaagtaaaaattaatttagataatgcttaaagaaggggaggtgtgaacagcttccatttgtttgattttctcagagaaataaagcataatttatatcctggttttagagattcactcttaatgatgtatatgtgtttctagaacaatgtcatctatccctcttatagaattgaaaataaaatgtccaaagaaagcagcacaccattggaatttttaaaacaaaaactacatagcacaataattgtaagacaaatcctactctagcttagaaaacaactaatttttactgcatatttttcatggtacatttaaattatagttttaataaaatacatctttagatcaaagctgaaagaagacatcagtagtagatcagtgtattccatttttcttctggatgatggatggcttatgtttttttttttttttaatatttccacagaacatttcattcagtatcattttactcattttactcctcaagtacatacaaacatgagggccggtagacaaaatatatccttgaatccaaccacgttttggaatattcatcagcttagtaaatccatgcagttcattttaaacttttagttcaatacaatggctttgctgatgcagtttttctcctttagatggcaatatggcaaatgacatttttatttctcaggcaaagaagaaagacaaacctgtacagtgaaatctcataggaaacattaagtctgctaaagtgaacatctgcattcacctgtgttctctgttaggtggtggtattaggaaaaaaagcctattaggaaagttactcatggatttaatttataattggtggaactcagctgaatttcccaccattgtaaacatccacataatgccatgaaaaaagttcatgtatattgcatttgtttttccagttattgtctaggcaagtttctacttgtttgaggtttctagaggtaatgcagctcagacactcctgggtgccctctcaaattcgtgggtcctcctgtttctacctttcttattttcttgtaagtgcttccatttgttactgttccctggggtatgtcctggcctttgccgacgttgttttcggtcccttttccaaacttgttcacagaactcatccattgtgttgagattggggtggttgatgagctgcatgaagtctctgtaccagaccttctggctaggtgtcatgctattggacatttctttggtcttagagccatctccatcatcatctttatgaagaagttcttccaaatgctctgtgtcaatgacttccagggttaccttaagaagagtttgtatgaacccatgttccaccgcatggcagaggtaattgcctgaatccttctgttgtagactacgtagcagaaggccttgatctgtcctgatgatatgatcatccactctgatctcttcttttcgctcttcatttcgcctctggaattgccaatagaccagcgctctctgcgacttcggactgcattccaaaaatgtgctactattctctacaccatagatgattctctcttcagggctgtggccatggtgattatcatggtgtaagtctgaacagtgagtcagtgggtctccatttcttatatcttgtcgtcttgtgcgtctctttgcagtgggaaaatagcgagaacatgcagaaccatcccaagcacagtaagggtctcgggcgaggcaacactcagcacacgctttcccgtaaatatcacaccggtgtaaagggagctgggcaaccccagccgttgaaccaatatatagttgttgctgcttagtggaaagctccattgctgaaatagcagtcggttcccgaaaaactgtcatttcttccagcagaacctcttctaaatcataccaagtctccttaggaattgaaactactttaagaacggtcccaacatctgttccgataaacataacatcatactgtccatcttctgcatccactcggtctacgacaatttgtgtaaattgataatttacatccgttttgatcactattgggcgattgttcataggaaacactggattgtacatggctggatgacttcttgcaaaggttataacatcatcaggaaggtcctttgtagagtcaaaaccaccaaatgttttgctgggacaagttcctggccgtggataggggactcttccttgataaggcacccattgatagttgggtccatccctgtgggcatatggaccaaggaacacccttctcacatcactcatgctatacatacacacggctgatcccttgaaaatgttactggaagtcgtaaacactccatatacaactggatttttaggatctttaaagttcattaggaatacatcctgcagttcatcaaaatgagtgtcaatgccatttggacctggcactgagcaaatcagacgagctttgaggaatgttgtccatttattcaccagacttctgtgccctccaaagtcattcttgcatatctgacctattctagcgtgagtagcttttccagagtgttctccatctattgcattttcacggaagaaaaagtatactttgtcatcttcaggattgtcactctctgagatgaggtgggcactaatgaactttggatcattgagccacctggaatcatgctgctctgtcctgattgggtggtggtgcccaagagttcggaagatagcaaagtctcgccccataaaatcagctgcagttccagagtataattctccatctattaaaagggatgctgtcagcagcttagggtcatatggactcttcccacggccgttttcaaaatgtgagttctccagcttaaaaatattgtcctcaggatgatgtccaatttcaatgtaggtgcaaattggatgaaaagcccccgttccacaggcgtacaagtgagtctgattatatgccttaagtaccttgatgaaattagcacattctttcaggatgtcttttccagcccacttgcattcatctcttctggtgtaagatactggccacacaatcttttgaaaatccttgatattaaccaggtcgaatgaaaatatgtgatcctttgctccaacatacagcctactccgttcctcatccaaaaggaaggtatgataactggagctgttggccaagccattgaaagtgatcacattgttggattccaacatttctttgtaggataatttcagccttggcacattgttcttcccattctgatagtttgctcttgctgtaagtaatactccccagaaaagacagacaatcctagttaaccagcccatgctgcagacgctgtaggtccctttgctgctttagtcttccttcctgtattgtgcggccagagaagttcaaacaatctggaaacttcttttaggaaaaattcttaattcctgagatacaatgtgttcagtccaacttgttattgtaagtacctgggcactttaaatacccatttaagagctcctgtgaatcttctctcctgttacttgatgatatttttataaagtggatttttttatcttccataatcacattctattactttattttaaagctataatccagaagcagatttttttttccaaaactgttagtggtccaagaaaataaaggacaaggagaggttgcgggg

SEQ ID NO: 17819 - RNA, 7142 nt, Homo sapiens
  source 1..7142: mol_type = other RNA
tcgaggagctcacagtctagaaatggagatggaaacataaacaaataaatcacacattggggtagtgtgacaataaaaggtatatacaaggcacaggtttagcatagagaaggtccctagcttgaactagggatgggaggattaggaaagacttgctggattagatgatgataagtcatctcgctctgtttccttaatttcattgtgagctctttgagaacaagggttatgtcttattcactttagtgtcctcatcacctaacataatacctagcacattgtagatagtcaagatctatcagtggaatttacttgaacgtgtaggaagctggttctaaaaggcaaagtgtctagaggcccagttttttaatattcaaaatcttctttttgtttggtttggttccagctttgcctctgcctgtgtgtgcctgcatgtttgaaatgataacaaagctgttttccttggttacgttgattgcgaaactgtccttactatatgggctgtcacatatgctgattttattctctctttcatttagatattttcttaatttattaacttgaaaaattatgttcatttaattaactagtttaagaaaatttttagagatcaaacaaactaatgagattttacagatttttgaaaaataatgttttcttctttatggaaacatgtatttgcaaacattaacattgacttcaaataattattacaaatcaagttaaaagtatagatgtccttggtgttagaccagtttaacatgttattacacgatacgggggtgttgaatcctatttaagtctgtctttgaaaccatgaaacctgatacagtttcattaaattgaatggaaattgtgttttaaaatgagctaataaaacaaagattttaacatattatactagtggctccatattaataaaatgcttgtctgtgacctttaagataagcaatttcaataacagtcatctgacatctttgtggatcctgaataaaaccaaactgattatgaaaatgacacattataaaaatttatccctacatttcctttttaggtatgacattaaaaagaacaatacttaatttaaagggcataaaaattcacatcatcaccataaatatagaacccagtttacagatgactacaatgaagaaatctgttagctaattatgtagcaacctgactctggttctcaacattttatgagcttatgttccttaacaccatatgttatagggaacagtaaagacatctgaattcaaatattttgaagaaatgtgtatttagcaagtgaatacatgctaaaaggaataatttacagcagcagtttcattacatttttctctccagtttttctagttcccatctgaaatgcaatgataagtaaagatatggaacatatttcctacctggcaaaaaacatgcttattgaacgggcacgcaccttccgcccttaaatagtacataaaccaccttgtcacctgcgtgggaaaatcttgccttttaggatgatgttgaacacattgaaatggagtacttatagaaagttttattttacactgttcttcctctttttctcccaaattatttacatcttttttttgcctaatgtgtaggtagcaaaaatattaaacacataccactgcaaattactaaataatacataaaatgaagtgtgcatttacatgcatttacattttacatttgatatcaactgggccataatgtctctgctgtgatgcatctttttcatactttaagactgctgttgtaattttcgtaaggtcacatgagtctctcaaacagtttcatctctgatgattcatgcatatgacaaagtctatttaaagctgaattattaaatgggccaataattctttttcgtgcaaactgccccctctcaatacacatgggcagagattatgactgtaatgagttatctgcaagttatatctacaattttctttgaaaacttagacctgatggtatataaagacatgcctgtagatttgtttgtttgtgtaacttttaattgaagtcgagacttttttctattgtcatttcataacactaaacaaaatgcattcaaattctgaaagtcttctataaatttatcatataatctctatcccttcaaatcctttatttctgaggatgaataataagatatttctgctatcgcaaataaatttatttcagctgcaaatttagaatgaaacacaacactgaatgttagtacagtttagatactttatgaaaataaaagaatgacctattttttggagcactctttgttcttcgatttatatttgaaacactactttctgtacagtggtgtgtccttcaaataatttaacaatttggcttccatgtgaggatatacagtacttccaaaagcaacaccatattagtcaatggagcctaaaattgaatgtagattatttttaggcttttgtttgaaacaagtggcaacaacttgtttattcaaggcagtcattaaaactgaaacatgagcttccatctgtgaaatatttcagctgataggaaataaaaattcactgtagtctgaggtgagaaattgatgctgagttaattagaatccaaagacagctagagttagaatttcaatgttgcttcattaattactaataagatgttttctttgcatttttgtgcatgatgaggaacctgggggaggagtcctgaataggtgagtgcagtgcaaaagaaaccacagtataatgctgaaagttttaaatatctcaaagtcagtgattctcaacgaatcgtcttaggacaatgaaggaagcaaatcttgaattttagtcttttaccttattttgtaagttgttgcaggaaacaaagaattttacattgtttaaatgtgggttgcatcctggaaaatactttgtagaaaagtccctcccattgatatgaaaagagtcatgtgtttcttgtacaaataattgtcttaaataaggaaaggtaagaggcacctgatacagatgtaaatgattggaaactttgcctttaacatgttgctctgaatagttattgatctctctcttttaaaaaaattaagtgacacagatataattcttggtagaatcataagagagatcttagtctcaaatatcatgcagggattcaagcacggaattaagacacattttctattaacagtatattaagacaatgcttattattttcatgaaatatgcagttccttttcccttcattgattcattatagtaaaatgcacttaaaaatcaacttgtttcttccttttttcctgcttaaatgttctgtttttttttctaagaacattatgcaagtaaaaattaatttagataatgcttaaagaaggggaggtgtgaacagcttccatttgtttgattttctcagagaaataaagcataatttatatcctggttttagagattcactcttaatgatgtatatgtgtttctagaacaatgtcatctatccctcttatagaattgaaaataaaatgtccaaagaaagcagcacaccattggaatttttaaaacaaaaactacatagcacaataattgtaagacaaatcctactctagcttagaaaacaactaatttttactgcatatttttcatggtacatttaaattatagttttaataaaatacatctttagatcaaagctgaaagaagacatcagtagtagatcagtgtattccatttttcttctggatgatggatggcttatgtttttttttttttttaatatttccacagaacatttcattcagtatcattttactcattttactcctcaagtacatacaaacatgagggccggtagacaaaatatatccttgaatccaaccacgttttggaatattcatcagcttagtaaatccatgcagttcattttaaacttttagttcaatacaatggctttgctgatgcagtttttctcctttagatggcaatatggcaaatgacatttttatttctcaggcaaagaagaaagacaaacctgtacagtgaaatctcataggaaacattaagtctgctaaagtgaacatctgcattcacctgtgttctctgttaggtggtggtattaggaaaaaaagcctattaggaaagttactcatggatttaatttataattggtggaactcagctgaatttcccaccattgtaaacatccacataatgccatgaaaaaagttcatgtatattgcatttgtttttccagttattgtctaggcaagtttctacttgtttgaggtttctagaggtaatgcagctcagacactcctgggtgccctctcaaattcgtgggtcctcctgtttctacctttcttattttcttgtaagtgcttccatttgttactgttccctggggtatgtcctggcctttgccgacgttgttttcggtcccttttccaaacttgttcacagaactcatccattgtgttgagattggggtggttgatgagctgcatgaagtctctgtaccagaccttctggctaggtgtcatgctattggacatttctttggtcttagagccatctccatcatcatctttatgaagaagttcttccaaatgctctgtgtcaatgacttccagggttaccttaagaagagtttgtatgaacccatgttccaccgcatggcagaggtaattgcctgaatccttctgttgtagactacgtagcagaaggccttgatctgtcctgatgatatgatcatccactctgatctcttcttttcgctcttcatttcgcctctggaattgccaatagaccagcgctctctgcgacttcggactgcattccaaaaatgtgctactattctctacaccatagatgattctctcttcagggctgtggccatggtgattatcatggtgtaagtctgaacagtgagtcagtgggtctccatttcttatatcttgtcgtcttgtgcgtctctttgcagtgggaaaatagcgagaacatgcagaaccatcccaagcacagtaagggtctcgggcgaggcaacactcagcacacgctttcccgtaaatatcacaccggtgtaaagggagctgggcaaccccagccgttgaaccaatatatagttgttgctgcttagtggaaagctccattgctgaaatagcagtcggttcccgaaaaactgtcatttcttccagcagaacctcttctaaatcataccaagtctccttaggaattgaaactactttaagaacggtcccaacatctgttccgataaacataacatcatactgtccatcttctgcatccactcggtctacgacaatttgtgtaaattgataatttacatccgttttgatcactattgggcgattgttcataggaaacactggattgtacatggctggatgacttcttgcaaaggttataacatcatcaggaaggtcctttgtagagtcaaaaccaccaaatgttttgctgggacaagttcctggccgtggataggggactcttccttgataaggcacccattgatagttgggtccatccctgtgggcatatggaccaaggaacacccttctcacatcactcatgctatacatacacacggctgatcccttgaaaatgttactggaagtcgtaaacactccatatacaactggatttttaggatctttaaagttcattaggaatacatcctgcagttcatcaaaatgagtgtcaatgccatttggacctggcactgagcaaatcagacgagctttgaggaatgttgtccatttattcaccagacttctgtgccctccaaagtcattcttgcatatctgacctattctagcgtgagtagcttttccagagtgttctccatctattgcattttcacggaagaaaaagtatactttgtcatcttcaggattgtcactctctgagatgaggtgggcactaatgaactttggatcattgagccacctggaatcatgctgctctgtcctgattgggtggtggtgcccaagagttcggaagatagcaaagtctcgccccataaaatcagctgcagttccagagtataattctccatctattaaaagggatgctgtcagcagcttagggtcatatggactcttcccacggccgttttcaaaatgtgagttctccagcttaaaaatattgtcctcaggatgatgtccaatttcaatgtaggtgcaaattggatgaaaagcccccgttccacaggcgtacaagtgagtctgattatatgccttaagtaccttgatgaaattagcacattctttcaggatgtcttttccagcccacttgcattcatctcttctggtgtaagatactggccacacaatcttttgaaaatccttgatattaaccaggtcgaatgaaaatatgtgatcctttgctccaacatacagcctactccgttcctcatccaaaaggaaggtatgataactggagctgttggccaagccattgaaagtgatcacattgttggattccaacatttctttgtaggataatttcagccttggcacattgttcttcccattctgatagtttgctcttgctgtaagtaatactccccagaaaagacagacaatcctagttaaccagcccatgctgcagacgctgtaggtccctttgctgctttagtcttccttcctgtattgtgcggccagagaagttcaaacaatctggaaacttcttttaggaaaaattcttaattcctgagatacaatgtgttcagtccaacttgttattgtaagtacctgggcactttaaataccctgctaaagggcctcttcttgatgaataattccctttgttatgttagactgtcccatggatggtttttttaaatattagttctgtgggttgactggactctgcagtatccttctagcttagggtttttcacatggtgacagtcagatggaagctggcattgtagttatctaaaggtgcagctggattggatgtccaagattgttcatgtacacagctggcagttgatactagctgttgcccaggacctggagccatctagcagagcacctatacctgatcttctcatggtatggtgactaacttcatataggaaacattccaagagcaagcatttcaagacgtccaagcaaaatctgcaagtcttct

SEQ ID NO: 17820 - RNA, 7117 nt, Homo sapiens
  source 1..7117: mol_type = other RNA
tcgaggagctcacagtctagaaatggagatggaaacataaacaaataaatcacacattggggtagtgtgacaataaaaggtatatacaaggcacaggtttagcatagagaaggtccctagcttgaactagggatgggaggattaggaaagacttgctggattagatgatgataagtcatctcgctctgtttccttaatttcattgtgagctctttgagaacaagggttatgtcttattcactttagtgtcctcatcacctaacataatacctagcacattgtagatagtcaagatctatcagtggaatttacttgaacgtgtaggaagctggttctaaaaggcaaagtgtctagaggcccagttttttaatattcaaaatcttctttttgtttggtttggttccagctttgcctctgcctgtgtgtgcctgcatgtttgaaatgataacaaagctgttttccttggttacgttgattgcgaaactgtccttactatatgggctgtcacatatgctgattttattctctctttcatttagatattttcttaatttattaacttgaaaaattatgttcatttaattaactagtttaagaaaatttttagagatcaaacaaactaatgagattttacagatttttgaaaaataatgttttcttctttatggaaacatgtatttgcaaacattaacattgacttcaaataattattacaaatcaagttaaaagtatagatgtccttggtgttagaccagtttaacatgttattacacgatacgggggtgttgaatcctatttaagtctgtctttgaaaccatgaaacctgatacagtttcattaaattgaatggaaattgtgttttaaaatgagctaataaaacaaagattttaacatattatactagtggctccatattaataaaatgcttgtctgtgacctttaagataagcaatttcaataacagtcatctgacatctttgtggatcctgaataaaaccaaactgattatgaaaatgacacattataaaaatttatccctacatttcctttttaggtatgacattaaaaagaacaatacttaatttaaagggcataaaaattcacatcatcaccataaatatagaacccagtttacagatgactacaatgaagaaatctgttagctaattatgtagcaacctgactctggttctcaacattttatgagcttatgttccttaacaccatatgttatagggaacagtaaagacatctgaattcaaatattttgaagaaatgtgtatttagcaagtgaatacatgctaaaaggaataatttacagcagcagtttcattacatttttctctccagtttttctagttcccatctgaaatgcaatgataagtaaagatatggaacatatttcctacctggcaaaaaacatgcttattgaacgggcacgcaccttccgcccttaaatagtacataaaccaccttgtcacctgcgtgggaaaatcttgccttttaggatgatgttgaacacattgaaatggagtacttatagaaagttttattttacactgttcttcctctttttctcccaaattatttacatcttttttttgcctaatgtgtaggtagcaaaaatattaaacacataccactgcaaattactaaataatacataaaatgaagtgtgcatttacatgcatttacattttacatttgatatcaactgggccataatgtctctgctgtgatgcatctttttcatactttaagactgctgttgtaattttcgtaaggtcacatgagtctctcaaacagtttcatctctgatgattcatgcatatgacaaagtctatttaaagctgaattattaaatgggccaataattctttttcgtgcaaactgccccctctcaatacacatgggcagagattatgactgtaatgagttatctgcaagttatatctacaattttctttgaaaacttagacctgatggtatataaagacatgcctgtagatttgtttgtttgtgtaacttttaattgaagtcgagacttttttctattgtcatttcataacactaaacaaaatgcattcaaattctgaaagtcttctataaatttatcatataatctctatcccttcaaatcctttatttctgaggatgaataataagatatttctgctatcgcaaataaatttatttcagctgcaaatttagaatgaaacacaacactgaatgttagtacagtttagatactttatgaaaataaaagaatgacctattttttggagcactctttgttcttcgatttatatttgaaacactactttctgtacagtggtgtgtccttcaaataatttaacaatttggcttccatgtgaggatatacagtacttccaaaagcaacaccatattagtcaatggagcctaaaattgaatgtagattatttttaggcttttgtttgaaacaagtggcaacaacttgtttattcaaggcagtcattaaaactgaaacatgagcttccatctgtgaaatatttcagctgataggaaataaaaattcactgtagtctgaggtgagaaattgatgctgagttaattagaatccaaagacagctagagttagaatttcaatgttgcttcattaattactaataagatgttttctttgcatttttgtgcatgatgaggaacctgggggaggagtcctgaataggtgagtgcagtgcaaaagaaaccacagtataatgctgaaagttttaaatatctcaaagtcagtgattctcaacgaatcgtcttaggacaatgaaggaagcaaatcttgaattttagtcttttaccttattttgtaagttgttgcaggaaacaaagaattttacattgtttaaatgtgggttgcatcctggaaaatactttgtagaaaagtccctcccattgatatgaaaagagtcatgtgtttcttgtacaaataattgtcttaaataaggaaaggtaagaggcacctgatacagatgtaaatgattggaaactttgcctttaacatgttgctctgaatagttattgatctctctcttttaaaaaaattaagtgacacagatataattcttggtagaatcataagagagatcttagtctcaaatatcatgcagggattcaagcacggaattaagacacattttctattaacagtatattaagacaatgcttattattttcatgaaatatgcagttccttttcccttcattgattcattatagtaaaatgcacttaaaaatcaacttgtttcttccttttttcctgcttaaatgttctgtttttttttctaagaacattatgcaagtaaaaattaatttagataatgcttaaagaaggggaggtgtgaacagcttccatttgtttgattttctcagagaaataaagcataatttatatcctggttttagagattcactcttaatgatgtatatgtgtttctagaacaatgtcatctatccctcttatagaattgaaaataaaatgtccaaagaaagcagcacaccattggaatttttaaaacaaaaactacatagcacaataattgtaagacaaatcctactctagcttagaaaacaactaatttttactgcatatttttcatggtacatttaaattatagttttaataaaatacatctttagatcaaagctgaaagaagacatcagtagtagatcagtgtattccatttttcttctggatgatggatggcttatgtttttttttttttttaatatttccacagaacatttcattcagtatcattttactcattttactcctcaagtacatacaaacatgagggccggtagacaaaatatatccttgaatccaaccacgttttggaatattcatcagcttagtaaatccatgcagttcattttaaacttttagttcaatacaatggctttgctgatgcagtttttctcctttagatggcaatatggcaaatgacatttttatttctcaggcaaagaagaaagacaaacctgtacagtgaaatctcataggaaacattaagtctgctaaagtgaacatctgcattcacctgtgttctctgttaggtggtggtattaggaaaaaaagcctattaggaaagttactcatggatttaatttataattggtggaactcagctgaatttcccaccattgtaaacatccacataatgccatgaaaaaagttcatgtatattgcatttgtttttccagttattgtctaggcaagtttctacttgtttgaggtttctagaggtaatgcagctcagacactcctgggtgccctctcaaattcgtgggtcctcctgtttctacctttcttattttcttgtaagtgcttccatttgttactgttccctggggtatgtcctggcctttgccgacgttgttttcggtcccttttccaaacttgttcacagaactcatccattgtgttgagattggggtggttgatgagctgcatgaagtctctgtaccagaccttctggctaggtgtcatgctattggacatttctttggtcttagagccatctccatcatcatctttatgaagaagttcttccaaatgctctgtgtcaatgacttccagggttaccttaagaagagtttgtatgaacccatgttccaccgcatggcagaggtaattgcctgaatccttctgttgtagactacgtagcagaaggccttgatctgtcctgatgatatgatcatccactctgatctcttcttttcgctcttcatttcgcctctggaattgccaatagaccagcgctctctgcgacttcggactgcattccaaaaatgtgctactattctctacaccatagatgattctctcttcagggctgtggccatggtgattatcatggtgtaagtctgaacagtgagtcagtgggtctccatttcttatatcttgtcgtcttgtgcgtctctttgcagtgggaaaatagcgagaacatgcagaaccatcccaagcacagtaagggtctcgggcgaggcaacactcagcacacgctttcccgtaaatatcacaccggtgtaaagggagctgggcaaccccagccgttgaaccaatatatagttgttgctgcttagtggaaagctccattgctgaaatagcagtcggttcccgaaaaactgtcatttcttccagcagaacctcttctaaatcataccaagtctccttaggaattgaaactactttaagaacggtcccaacatctgttccgataaacataacatcatactgtccatcttctgcatccactcggtctacgacaatttgtgtaaattgataatttacatccgttttgatcactattgggcgattgttcataggaaacactggattgtacatggctggatgacttcttgcaaaggttataacatcatcaggaaggtcctttgtagagtcaaaaccaccaaatgttttgctgggacaagttcctggccgtggataggggactcttccttgataaggcacccattgatagttgggtccatccctgtgggcatatggaccaaggaacacccttctcacatcactcatgctatacatacacacggctgatcccttgaaaatgttactggaagtcgtaaacactccatatacaactggatttttaggatctttaaagttcattaggaatacatcctgcagttcatcaaaatgagtgtcaatgccatttggacctggcactgagcaaatcagacgagctttgaggaatgttgtccatttattcaccagacttctgtgccctccaaagtcattcttgcatatctgacctattctagcgtgagtagcttttccagagtgttctccatctattgcattttcacggaagaaaaagtatactttgtcatcttcaggattgtcactctctgagatgaggtgggcactaatgaactttggatcattgagccacctggaatcatgctgctctgtcctgattgggtggtggtgcccaagagttcggaagatagcaaagtctcgccccataaaatcagctgcagttccagagtataattctccatctattaaaagggatgctgtcagcagcttagggtcatatggactcttcccacggccgttttcaaaatgtgagttctccagcttaaaaatattgtcctcaggatgatgtccaatttcaatgtaggtgcaaattggatgaaaagcccccgttccacaggcgtacaagtgagtctgattatatgccttaagtaccttgatgaaattagcacattctttcaggatgtcttttccagcccacttgcattcatctcttctggtgtaagatactggccacacaatcttttgaaaatccttgatattaaccaggtcgaatgaaaatatgtgatcctttgctccaacatacagcctactccgttcctcatccaaaaggaaggtatgataactggagctgttggccaagccattgaaagtgatcacattgttggattccaacatttctttgtaggataatttcagccttggcacattgttcttcccattctgatagtttgctcttgctgtaagtaatactccccagaaaagacagacaatcctagttaaccagcccatgctgcagacgctgtaggtccctttgctgctttagtcttccttcctgtattgtgcggccagagaagttcaaacaatctggaaacttcttttaggaaaaattcttaattcctgagatacaatgtgttcagtccaacttgttattgtaagtacctgggcactttaaataccctgctaaagggcctcttcttgatgaataattccctttgttatgttagactgtcccatggatggtttttttaaatatttgcctttgttgtcctttgtccatgcgttgaagtcaaagggctgttctgttcttacctagctccaggttgccctccagattagggataaatgtgagcagcaagaagcatgttcactttgtaactgtaccaggagcagcccatcacactgatgctagagagccagtcaagacacagcactaaacttcagcatgagagcacagaatctattacccctgaggctctaccatttcacctacacctgggcggatctatcaggcttcatctc

SEQ ID NO: 17821 - RNA, 6860 nt, Homo sapiens
  source 1..6860: mol_type = other RNA
tcgaggagctcacagtctagaaatggagatggaaacataaacaaataaatcacacattggggtagtgtgacaataaaaggtatatacaaggcacaggtttagcatagagaaggtccctagcttgaactagggatgggaggattaggaaagacttgctggattagatgatgataagtcatctcgctctgtttccttaatttcattgtgagctctttgagaacaagggttatgtcttattcactttagtgtcctcatcacctaacataatacctagcacattgtagatagtcaagatctatcagtggaatttacttgaacgtgtaggaagctggttctaaaaggcaaagtgtctagaggcccagttttttaatattcaaaatcttctttttgtttggtttggttccagctttgcctctgcctgtgtgtgcctgcatgtttgaaatgataacaaagctgttttccttggttacgttgattgcgaaactgtccttactatatgggctgtcacatatgctgattttattctctctttcatttagatattttcttaatttattaacttgaaaaattatgttcatttaattaactagtttaagaaaatttttagagatcaaacaaactaatgagattttacagatttttgaaaaataatgttttcttctttatggaaacatgtatttgcaaacattaacattgacttcaaataattattacaaatcaagttaaaagtatagatgtccttggtgttagaccagtttaacatgttattacacgatacgggggtgttgaatcctatttaagtctgtctttgaaaccatgaaacctgatacagtttcattaaattgaatggaaattgtgttttaaaatgagctaataaaacaaagattttaacatattatactagtggctccatattaataaaatgcttgtctgtgacctttaagataagcaatttcaataacagtcatctgacatctttgtggatcctgaataaaaccaaactgattatgaaaatgacacattataaaaatttatccctacatttcctttttaggtatgacattaaaaagaacaatacttaatttaaagggcataaaaattcacatcatcaccataaatatagaacccagtttacagatgactacaatgaagaaatctgttagctaattatgtagcaacctgactctggttctcaacattttatgagcttatgttccttaacaccatatgttatagggaacagtaaagacatctgaattcaaatattttgaagaaatgtgtatttagcaagtgaatacatgctaaaaggaataatttacagcagcagtttcattacatttttctctccagtttttctagttcccatctgaaatgcaatgataagtaaagatatggaacatatttcctacctggcaaaaaacatgcttattgaacgggcacgcaccttccgcccttaaatagtacataaaccaccttgtcacctgcgtgggaaaatcttgccttttaggatgatgttgaacacattgaaatggagtacttatagaaagttttattttacactgttcttcctctttttctcccaaattatttacatcttttttttgcctaatgtgtaggtagcaaaaatattaaacacataccactgcaaattactaaataatacataaaatgaagtgtgcatttacatgcatttacattttacatttgatatcaactgggccataatgtctctgctgtgatgcatctttttcatactttaagactgctgttgtaattttcgtaaggtcacatgagtctctcaaacagtttcatctctgatgattcatgcatatgacaaagtctatttaaagctgaattattaaatgggccaataattctttttcgtgcaaactgccccctctcaatacacatgggcagagattatgactgtaatgagttatctgcaagttatatctacaattttctttgaaaacttagacctgatggtatataaagacatgcctgtagatttgtttgtttgtgtaacttttaattgaagtcgagacttttttctattgtcatttcataacactaaacaaaatgcattcaaattctgaaagtcttctataaatttatcatataatctctatcccttcaaatcctttatttctgaggatgaataataagatatttctgctatcgcaaataaatttatttcagctgcaaatttagaatgaaacacaacactgaatgttagtacagtttagatactttatgaaaataaaagaatgacctattttttggagcactctttgttcttcgatttatatttgaaacactactttctgtacagtggtgtgtccttcaaataatttaacaatttggcttccatgtgaggatatacagtacttccaaaagcaacaccatattagtcaatggagcctaaaattgaatgtagattatttttaggcttttgtttgaaacaagtggcaacaacttgtttattcaaggcagtcattaaaactgaaacatgagcttccatctgtgaaatatttcagctgataggaaataaaaattcactgtagtctgaggtgagaaattgatgctgagttaattagaatccaaagacagctagagttagaatttcaatgttgcttcattaattactaataagatgttttctttgcatttttgtgcatgatgaggaacctgggggaggagtcctgaataggtgagtgcagtgcaaaagaaaccacagtataatgctgaaagttttaaatatctcaaagtcagtgattctcaacgaatcgtcttaggacaatgaaggaagcaaatcttgaattttagtcttttaccttattttgtaagttgttgcaggaaacaaagaattttacattgtttaaatgtgggttgcatcctggaaaatactttgtagaaaagtccctcccattgatatgaaaagagtcatgtgtttcttgtacaaataattgtcttaaataaggaaaggtaagaggcacctgatacagatgtaaatgattggaaactttgcctttaacatgttgctctgaatagttattgatctctctcttttaaaaaaattaagtgacacagatataattcttggtagaatcataagagagatcttagtctcaaatatcatgcagggattcaagcacggaattaagacacattttctattaacagtatattaagacaatgcttattattttcatgaaatatgcagttccttttcccttcattgattcattatagtaaaatgcacttaaaaatcaacttgtttcttccttttttcctgcttaaatgttctgtttttttttctaagaacattatgcaagtaaaaattaatttagataatgcttaaagaaggggaggtgtgaacagcttccatttgtttgattttctcagagaaataaagcataatttatatcctggttttagagattcactcttaatgatgtatatgtgtttctagaacaatgtcatctatccctcttatagaattgaaaataaaatgtccaaagaaagcagcacaccattggaatttttaaaacaaaaactacatagcacaataattgtaagacaaatcctactctagcttagaaaacaactaatttttactgcatatttttcatggtacatttaaattatagttttaataaaatacatctttagatcaaagctgaaagaagacatcagtagtagatcagtgtattccatttttcttctggatgatggatggcttatgtttttttttttttttaatatttccacagaacatttcattcagtatcattttactcattttactcctcaagtacatacaaacatgagggccggtagacaaaatatatccttgaatccaaccacgttttggaatattcatcagcttagtaaatccatgcagttcattttaaacttttagttcaatacaatggctttgctgatgcagtttttctcctttagatggcaatatggcaaatgacatttttatttctcaggcaaagaagaaagacaaacctgtacagtgaaatctcataggaaacattaagtctgctaaagtgaacatctgcattcacctgtgttctctgttaggtggtggtattaggaaaaaaagcctattaggaaagttactcatggatttaatttataattggtggaactcagctgaatttcccaccattgtaaacatccacataatgccatgaaaaaagttcatgtatattgcatttgtttttccagttattgtctaggcaagtttctacttgtttgaggtttctagaggtaatgcagctcagacactcctgggtgccctctcaaattcgtgggtcctcctgtttctacctttcttattttcttgtaagtgcttccatttgttactgttccctggggtatgtcctggcctttgccgacgttgttttcggtcccttttccaaacttgttcacagaactcatccattgtgttgagattggggtggttgatgagctgcatgaagtctctgtaccagaccttctggctaggtgtcatgctattggacatttctttggtcttagagccatctccatcatcatctttatgaagaagttcttccaaatgctctgtgtcaatgacttccagggttaccttaagaagagtttgtatgaacccatgttccaccgcatggcagaggtaattgcctgaatccttctgttgtagactacgtagcagaaggccttgatctgtcctgatgatatgatcatccactctgatctcttcttttcgctcttcatttcgcctctggaattgccaatagaccagcgctctctgcgacttcggactgcattccaaaaatgtgctactattctctacaccatagatgattctctcttcagggctgtggccatggtgattatcatggtgtaagtctgaacagtgagtcagtgggtctccatttcttatatcttgtcgtcttgtgcgtctctttgcagtgggaaaatagcgagaacatgcagaaccatcccaagcacagtaagggtctcgggcgaggcaacactcagcacacgctttcccgtaaatatcacaccggtgtaaagggagctgggcaaccccagccgttgaaccaatatatagttgttgctgcttagtggaaagctccattgctgaaatagcagtcggttcccgaaaaactgtcatttcttccagcagaacctcttctaaatcataccaagtctccttaggaattgaaactactttaagaacggtcccaacatctgttccgataaacataacatcatactgtccatcttctgcatccactcggtctacgacaatttgtgtaaattgataatttacatccgttttgatcactattgggcgattgttcataggaaacactggattgtacatggctggatgacttcttgcaaaggttataacatcatcaggaaggtcctttgtagagtcaaaaccaccaaatgttttgctgggacaagttcctggccgtggataggggactcttccttgataaggcacccattgatagttgggtccatccctgtgggcatatggaccaaggaacacccttctcacatcactcatgctatacatacacacggctgatcccttgaaaatgttactggaagtcgtaaacactccatatacaactggatttttaggatctttaaagttcattaggaatacatcctgcagttcatcaaaatgagtgtcaatgccatttggacctggcactgagcaaatcagacgagctttgaggaatgttgtccatttattcaccagacttctgtgccctccaaagtcattcttgcatatctgacctattctagcgtgagtagcttttccagagtgttctccatctattgcattttcacggaagaaaaagtatactttgtcatcttcaggattgtcactctctgagatgaggtgggcactaatgaactttggatcattgagccacctggaatcatgctgctctgtcctgattgggtggtggtgcccaagagttcggaagatagcaaagtctcgccccataaaatcagctgcagttccagagtataattctccatctattaaaagggatgctgtcagcagcttagggtcatatggactcttcccacggccgttttcaaaatgtgagttctccagcttaaaaatattgtcctcaggatgatgtccaatttcaatgtaggtgcaaattggatgaaaagcccccgttccacaggcgtacaagtgagtctgattatatgccttaagtaccttgatgaaattagcacattctttcaggatgtcttttccagcccacttgcattcatctcttctggtgtaagatactggccacacaatcttttgaaaatccttgatattaaccaggtcgaatgaaaatatgtgatcctttgctccaacatacagcctactccgttcctcatccaaaaggaaggtatgataactggagctgttggccaagccattgaaagtgatcacattgttggattccaacatttctttgtaggataatttcagccttggcacattgttcttcccattctgatagtttgctcttgctgtaagtaatactccccagaaaagacagacaatcctagttaaccagcccatgctgcagacgctgtaggtccctttgctgctttagtcttccttcctgtattgtgcggccagagaagttcaaacaatctggaaatagactggctgacaatgggagaacaggcgagctcaacctactccccttccctcctgtcacacaacacatgcaaaaaacatctcgtagagattagagccgggagcagaaccctcaggcgtgcctgtgaaaggcatgtagctataaatttacttcccaaggcaagcgttgttt

SEQ ID NO: 17822 - RNA, 7169 nt, Homo sapiens
  source 1..7169: mol_type = other RNA
tcgaggagctcacagtctagaaatggagatggaaacataaacaaataaatcacacattggggtagtgtgacaataaaaggtatatacaaggcacaggtttagcatagagaaggtccctagcttgaactagggatgggaggattaggaaagacttgctggattagatgatgataagtcatctcgctctgtttccttaatttcattgtgagctctttgagaacaagggttatgtcttattcactttagtgtcctcatcacctaacataatacctagcacattgtagatagtcaagatctatcagtggaatttacttgaacgtgtaggaagctggttctaaaaggcaaagtgtctagaggcccagttttttaatattcaaaatcttctttttgtttggtttggttccagctttgcctctgcctgtgtgtgcctgcatgtttgaaatgataacaaagctgttttccttggttacgttgattgcgaaactgtccttactatatgggctgtcacatatgctgattttattctctctttcatttagatattttcttaatttattaacttgaaaaattatgttcatttaattaactagtttaagaaaatttttagagatcaaacaaactaatgagattttacagatttttgaaaaataatgttttcttctttatggaaacatgtatttgcaaacattaacattgacttcaaataattattacaaatcaagttaaaagtatagatgtccttggtgttagaccagtttaacatgttattacacgatacgggggtgttgaatcctatttaagtctgtctttgaaaccatgaaacctgatacagtttcattaaattgaatggaaattgtgttttaaaatgagctaataaaacaaagattttaacatattatactagtggctccatattaataaaatgcttgtctgtgacctttaagataagcaatttcaataacagtcatctgacatctttgtggatcctgaataaaaccaaactgattatgaaaatgacacattataaaaatttatccctacatttcctttttaggtatgacattaaaaagaacaatacttaatttaaagggcataaaaattcacatcatcaccataaatatagaacccagtttacagatgactacaatgaagaaatctgttagctaattatgtagcaacctgactctggttctcaacattttatgagcttatgttccttaacaccatatgttatagggaacagtaaagacatctgaattcaaatattttgaagaaatgtgtatttagcaagtgaatacatgctaaaaggaataatttacagcagcagtttcattacatttttctctccagtttttctagttcccatctgaaatgcaatgataagtaaagatatggaacatatttcctacctggcaaaaaacatgcttattgaacgggcacgcaccttccgcccttaaatagtacataaaccaccttgtcacctgcgtgggaaaatcttgccttttaggatgatgttgaacacattgaaatggagtacttatagaaagttttattttacactgttcttcctctttttctcccaaattatttacatcttttttttgcctaatgtgtaggtagcaaaaatattaaacacataccactgcaaattactaaataatacataaaatgaagtgtgcatttacatgcatttacattttacatttgatatcaactgggccataatgtctctgctgtgatgcatctttttcatactttaagactgctgttgtaattttcgtaaggtcacatgagtctctcaaacagtttcatctctgatgattcatgcatatgacaaagtctatttaaagctgaattattaaatgggccaataattctttttcgtgcaaactgccccctctcaatacacatgggcagagattatgactgtaatgagttatctgcaagttatatctacaattttctttgaaaacttagacctgatggtatataaagacatgcctgtagatttgtttgtttgtgtaacttttaattgaagtcgagacttttttctattgtcatttcataacactaaacaaaatgcattcaaattctgaaagtcttctataaatttatcatataatctctatcccttcaaatcctttatttctgaggatgaataataagatatttctgctatcgcaaataaatttatttcagctgcaaatttagaatgaaacacaacactgaatgttagtacagtttagatactttatgaaaataaaagaatgacctattttttggagcactctttgttcttcgatttatatttgaaacactactttctgtacagtggtgtgtccttcaaataatttaacaatttggcttccatgtgaggatatacagtacttccaaaagcaacaccatattagtcaatggagcctaaaattgaatgtagattatttttaggcttttgtttgaaacaagtggcaacaacttgtttattcaaggcagtcattaaaactgaaacatgagcttccatctgtgaaatatttcagctgataggaaataaaaattcactgtagtctgaggtgagaaattgatgctgagttaattagaatccaaagacagctagagttagaatttcaatgttgcttcattaattactaataagatgttttctttgcatttttgtgcatgatgaggaacctgggggaggagtcctgaataggtgagtgcagtgcaaaagaaaccacagtataatgctgaaagttttaaatatctcaaagtcagtgattctcaacgaatcgtcttaggacaatgaaggaagcaaatcttgaattttagtcttttaccttattttgtaagttgttgcaggaaacaaagaattttacattgtttaaatgtgggttgcatcctggaaaatactttgtagaaaagtccctcccattgatatgaaaagagtcatgtgtttcttgtacaaataattgtcttaaataaggaaaggtaagaggcacctgatacagatgtaaatgattggaaactttgcctttaacatgttgctctgaatagttattgatctctctcttttaaaaaaattaagtgacacagatataattcttggtagaatcataagagagatcttagtctcaaatatcatgcagggattcaagcacggaattaagacacattttctattaacagtatattaagacaatgcttattattttcatgaaatatgcagttccttttcccttcattgattcattatagtaaaatgcacttaaaaatcaacttgtttcttccttttttcctgcttaaatgttctgtttttttttctaagaacattatgcaagtaaaaattaatttagataatgcttaaagaaggggaggtgtgaacagcttccatttgtttgattttctcagagaaataaagcataatttatatcctggttttagagattcactcttaatgatgtatatgtgtttctagaacaatgtcatctatccctcttatagaattgaaaataaaatgtccaaagaaagcagcacaccattggaatttttaaaacaaaaactacatagcacaataattgtaagacaaatcctactctagcttagaaaacaactaatttttactgcatatttttcatggtacatttaaattatagttttaataaaatacatctttagatcaaagctgaaagaagacatcagtagtagatcagtgtattccatttttcttctggatgatggatggcttatgtttttttttttttttaatatttccacagaacatttcattcagtatcattttactcattttactcctcaagtacatacaaacatgagggccggtagacaaaatatatccttgaatccaaccacgttttggaatattcatcagcttagtaaatccatgcagttcattttaaacttttagttcaatacaatggctttgctgatgcagtttttctcctttagatggcaatatggcaaatgacatttttatttctcaggcaaagaagaaagacaaacctgtacagtgaaatctcataggaaacattaagtctgctaaagtgaacatctgcattcacctgtgttctctgttaggtggtggtattaggaaaaaaagcctattaggaaagttactcatggatttaatttataattggtggaactcagctgaatttcccaccattgtaaacatccacataatgccatgaaaaaagttcatgtatattgcatttgtttttccagttattgtctaggcaagtttctacttgtttgaggtttctagaggtaatgcagctcagacactcctgggtgccctctcaaattcgtgggtcctcctgtttctacctttcttattttcttgtaagtgcttccatttgttactgttccctggggtatgtcctggcctttgccgacgttgttttcggtcccttttccaaacttgttcacagaactcatccattgtgttgagattggggtggttgatgagctgcatgaagtctctgtaccagaccttctggctaggtgtcatgctattggacatttctttggtcttagagccatctccatcatcatctttatgaagaagttcttccaaatgctctgtgtcaatgacttccagggttaccttaagaagagtttgtatgaacccatgttccaccgcatggcagaggtaattgcctgaatccttctgttgtagactacgtagcagaaggccttgatctgtcctgatgatatgatcatccactctgatctcttcttttcgctcttcatttcgcctctggaattgccaatagaccagcgctctctgcgacttcggactgcattccaaaaatgtgctactattctctacaccatagatgattctctcttcagggctgtggccatggtgattatcatggtgtaagtctgaacagtgagtcagtgggtctccatttcttatatcttgtcgtcttgtgcgtctctttgcagtgggaaaatagcgagaacatgcagaaccatcccaagcacagtaagggtctcgggcgaggcaacactcagcacacgctttcccgtaaatatcacaccggtgtaaagggagctgggcaaccccagccgttgaaccaatatatagttgttgctgcttagtggaaagctccattgctgaaatagcagtcggttcccgaaaaactgtcatttcttccagcagaacctcttctaaatcataccaagtctccttaggaattgaaactactttaagaacggtcccaacatctgttccgataaacataacatcatactgtccatcttctgcatccactcggtctacgacaatttgtgtaaattgataatttacatccgttttgatcactattgggcgattgttcataggaaacactggattgtacatggctggatgacttcttgcaaaggttataacatcatcaggaaggtcctttgtagagtcaaaaccaccaaatgttttgctgggacaagttcctggccgtggataggggactcttccttgataaggcacccattgatagttgggtccatccctgtgggcatatggaccaaggaacacccttctcacatcactcatgctatacatacacacggctgatcccttgaaaatgttactggaagtcgtaaacactccatatacaactggatttttaggatctttaaagttcattaggaatacatcctgcagttcatcaaaatgagtgtcaatgccatttggacctggcactgagcaaatcagacgagctttgaggaatgttgtccatttattcaccagacttctgtgccctccaaagtcattcttgcatatctgacctattctagcgtgagtagcttttccagagtgttctccatctattgcattttcacggaagaaaaagtatactttgtcatcttcaggattgtcactctctgagatgaggtgggcactaatgaactttggatcattgagccacctggaatcatgctgctctgtcctgattgggtggtggtgcccaagagttcggaagatagcaaagtctcgccccataaaatcagctgcagttccagagtataattctccatctattaaaagggatgctgtcagcagcttagggtcatatggactcttcccacggccgttttcaaaatgtgagttctccagcttaaaaatattgtcctcaggatgatgtccaatttcaatgtaggtgcaaattggatgaaaagcccccgttccacaggcgtacaagtgagtctgattatatgccttaagtaccttgatgaaattagcacattctttcaggatgtcttttccagcccacttgcattcatctcttctggtgtaagatactggccacacaatcttttgaaaatccttgatattaaccaggtcgaatgaaaatatgtgatcctttgctccaacatacagcctactccgttcctcatccaaaaggaaggtatgataactggagctgttggccaagccattgaaagtgatcacattgttggattccaacatttctttgtaggataatttcagccttggcacattgttcttcccattctgatagtttgctcttgctgtaagtaatactccccagaaaagacagacaatcctagttaaccagcccatgctgcagacgctgtaggtccctttgctgctttagtcttccttcctgtattgtgcggccagagaagttcaaacaatctggaaattttagtattatgttcattccatccaaacttggcaattgaagactgtgtggaatttcaactaacacatctcagatgtgcatgatctcagccttcttttaggaaaaattcttaattcctgagatacaatgtgttcagtccaacttgttattgtaagtacctgggcactttaaataccctgctaaagggcctcttcttgatgaataattccctttgttatgttagactgtcccatggatggtttttttaaatattagttctgtgggttgactggactctgcagtatccttctagcttagggtttttcacatggtgacagtcagatggaagctggcattgtagttatctaaaggtgcagctggattggatgtccaagattgttcatgtacacagctggcagttgatactagctgttgcccaggacctggagccatctagcagagcacctatacctgatcttctcatggtatggtgactaactt

SEQ ID NO: 17823 - RNA, 11148 nt, Homo sapiens
  source 1..11148: mol_type = other RNA
tcgaggagctcacagtctagtaagaaagagatgaatttgaaaatatatttgaaactgtaggcaaaataagtaccctcacagagaaattcaacatttggtttcaaatttgttatgcagtgaaaattagaaactacaaccaagatttttttaaaacattatgttcatataacgctgtagtatacctgaaaggcaagaacttaaacaagtgtgctgaaaaacaaattaggaatatttgaacaaaatatactttaaaaatgatcaacaacgtaaaatattcctgatttaaataaatctaagttattttatttagtttaagcaaaatatgtatccatatgaaaatgccagttctttcatttttggttaattcctttacacatattatttgctaagttcagaaatgctatatatacaaaaatttcaaaaataaataagtatcccaagatcacataacaatactttaagtacattcatgtgtaagaaggcaaaaaaagaaggttctatcttatattttaaaactttgacaggtattttaaatgtattattttatactttattttctttaaaaatgaaataatacagccatgatttaagtcatgtaaaaacaactgtttggatcatttaggtgtcaagcaaaactatcctctttatttcactatcatagtaaccatagttgatagaccatgtggcaatatgatcatttgttcagtggtcattaagatatctatagaataaacaagacaactacattttatttttttcacttaaaaatcacaaaaatacagcctaaaatataatttatattttaaaaataattctaaacattaacccctaaatctaatcccttaaaaaattcttgcaaaagttagctggatgtggctgttgccaaggaatgtcttttattagcaacaagtgactatctataacttttattccaacaatcttattttaaatatttgtttcaatttaatgctgggattagaaaaacatatttgttcaaagtatgtaagtagtaagtaaaacaatttcaaaaatctatcaaaaaaggagaattattcattctaggaaataattaacatactggtttaaaatatctgggagaagaacttttacataaaaagcttcaaatttagtcagttgtagcaagcacttgaaaagaccctgctctttcatctgcaatatcaggaattactatatctgactcatatttgattaagttacaatctcatttttgttgtcactacaaagaaggatccttatattagtaaatgcactcactgcaactactgaggcctgcctcctgtcagaatgacaatgcagtcttagcatacgggtgtcggtttggctgaatctaaccaaacacatcacgtactacagatgtttttagggcccacccaattcataaaagattttactgcgatacatgagtttacccaaatttttattaaaatgtgtttttagggtaaatatcttgatgaactaggcaaacaaatactgaatgcagattactgtttttacagttttaccgggaaaactcctaatagcaacccctcttccccttcaccacagatctttaatttaggtgtgatttttgtttgttctctacatgggaataaaggagaaagtttagaaagactgtatctagctagataagatgcagaggtagatggaatctctaacataaaagaagctctaattacactgttgccagacagctgttatggattttagtattgtttattaggtgaagaaaacattcataaaataagaaatttttgagatagaacttactctaataatttcattaacatatgttcaggttcttagatcaagaaatactgtagaggtgttctcctcaagactatgctatggcaataatttcttgcatacaatttaataatttaaacttgaactgtgtgttctgtgctctggcgttctacttcagaaaaaaatgaacactgcttctaaaataaaaaggaacataaaataaaaaaggaattaatgagatattgacatgttttctattaatacaatattgatgttttaaatgattttgatattgctataacaacatatattgtgcaaaataattaatctcactaaatattatttctgatttgccacgaattatctgccgtggcaatcaggaaatagtcttcaaagtaagtttgcaaacatgattttgcaaaccatgattggaaaaatatattcatttgggctataaactatcaagtagggttgttatatatatttctaggaaaatattttatttactctacaaagatcatcattatgaccttacggcttctgtagtgcaatggagaaaaaagtgtgttagaagttaaaagacctgaattctatctccaaccctgcatttattcagagtattggtataggtttaggcaaaatccttaatccagtctagttttatatggtaaaaatgtggatacctatcaaaactgagggttgagaggatgaaatgaattcattaaacatatcttctgagacataaatatatcaaaacaaatcaaaatacaattagatctaatgtttagaaataaatattttaattcatatttgctatttcactaaatctagaaatactaatgctttagttaaatatagaaagttgatgatagaaaaataaaatccatcgtaccattgaaaagcttgtcagaaatatgtactcttgagattcggaggatgagaaaaaaaatgtgtactctaacgaggaagctatataaactgagtctaactcaaaacatttattttagatgcatataagaattaaagtcttagtcaaaagaatgttttaaaatttcatcctaaatttatgtgagataaaatgccattcttttgtttttctgaacagaggagcttttatcaacttattctattttatttttatttttattattttattttattttatttattattattatactttaagttttagggtacatgtgcacaatgtgcaggttagttacatatgtatacatgtgccatgctggtgcgctgcacccactaactcgtcacctagcattaggtatatctcccaatgctatccctcccccctcccccgaccccaccacagtccccagagtgtgatgttccccttcctgtgtccatgtgttctcattgttcagttcccacctatgagtgagaatatgcggtgtttggttttttgttcttgcgatagtttactgagaatgatgatttctaatttcatccatgtccctacacgaacttattctattttaatagaatgttcagtatcagtgttttcacactgagattctctagcttattttgccatatttaaattaaaaagaaacaaaaaatcctgtttgatcatgtgaaaaatatttactgaaatgtgaataaatttatgatcattaattgcctactgaaatattcctgaatattgctcaccttattaacaagtatatatggagactgaaaaacatgtagatcatgcaaacaagtgtaactaactataccaaagaaacaaaagtccatactaaatatgtccataattaaataaaaaatgctaaacaagttttacctagatattataaaaacatagaaaggaaaacatttaggagatgatgaagaagcaggagattgggatgggagatgtaatttgatctaaattcccatatgcttctgtaaaatcaaaaattcattttgcaatattaattttgctcttaaggtagagacttttaaaatgaccattctcaatactacagcaattcttccctgatttgcacataaatgaattaaagtgaagaaaaagcagtagaggagagaagactaaaataaaccagattgtagcaccctgtaaagagctaaaatctccagtgtacaaacaactgataggaaagaagagaaaatcagaactataaaaaagtgacataagctcagaaaattactcatttttaattgtatcaacaaagataatttgtaattttgatcatgcaagcattataattactgataattgggcctttcagcttttaagtgccttctcaaacatgagttctgcatatggttgtgcagaaatcaaaatcttaaagagagatgagtaaagtcaagtttgtaatattaatcttatattctcaatatagatgctaattagtgctctgaatggttgtggttagaaatcttgttggtatgatgtatcagtgatgtcactgcattgatggagacagaataatacataatggtgcaatgtggtgatggtaagctttgttactcaatattgtcaggcactttaagaaaatcagaaacattcaggatagtgccaaagaagatcagtttttcaagactctaaaatcatattcaattatatgtgtatgtaattataaatatgtgcatcatggctgactttgagaagaatgcagcgccttgcaagtgcactatttgaatagagctaaggagaactatagtctaaggactgcaaaagtctagatggagaagacaaaagcaatgacacttgttttctctacagaacaaatagacaaagaggtgaatgacaacaaagatgttcagagaaacttgaaaaataagctacggtgtagggtaagttgtattaaatgatgaaaattaatatgtaactgtatgggtaaaccaaatcatttgtatcttataatcttttttttggtagctacggataatattataaatggaataatcactaaaattctaaatataatgttttctagtaagaacattttattttttttttaatagagacagattctcactctattgcctaggctggactgcaagtggggccattatagctcactgaagcctcaacttcctgggctcaaatgaccctctcgtctcagcctcccgagtagctgggactacaggtgcacatcaccacatccaggtaattattttactttttgaatcatgatatgtagcaaccaatctgggaattatttattcataaaagataacattttcctgctaactccaacctcagaaaaaatgtattatgcctgactcaaatatgtcattatttttatgagaaaaagagtcatattgaagtaattatgtctatatgtaataattatcattatttgagataatttgcattggggagaaaagcaggcaatcagaaattacatattcaaggctgggcgcagtggctcacgcctgtaatcccagcactttgggaggcagaggcgagtgaatcacctgaggtcagagttcaagaccagcctgaccaacaaggagaaaccccatctctactaaaacaaaacaaaacaaaacaaaacaaaaaaagccacaaaattagccgggcatggtggcacatgcctgtaattccagttactcgggaggctgaggcaggagaattgcttgaacctgggaggcagaggttgtagtaagccgagattgtgccactgcacgccagcctgggcgacaagaacgagactcagtctcaaaaaaaaaaaaaaagaaagaaagaaagaaattacatattcaggttctagcaaatgcagttctctaataaacactaaataaatcataatacaagttacagttaaacctaattgttttactatataggatgtatcttttttgtacctatattttatcttcctttgcttctctggcctctattgggaggcagcacggtagtgaacacctcggggatctttctggttacgtaaacctgagttttaattttggttcatactaccttttaactttgggtagtctgctgagcttgttttttgttttcactcatctgtcatatcaagctagtaataattctgccatggttttggttttcatattgaaaggcattacataagcaaaatgcataacatataaatattagttccctttccactatgcatccaatctccctattaaattaagcctaaaaataataatttttgttttattaaaagccttccacattctacatatgaaagggattttttaaaggtgttttagataaaaaatgtttcaaccaactgaccaagaatatctcttcatatttatgtcatctacataaaaacttacatttatatcatatatcttttagtcttcttttctatattcttgattgtcatgttgtacagccagaaaagaatgagtataaattatctagattttttaaagtgcacattcaaacatagaaaatctaattattttacttgtttcttagtattaggctgaggccaatgagtccatgagctaaagggttgaaacttggcaccaaaaaagtgattgtttatgagtcctgtagatttatactgagaaaacatcatgtcttccaatgtgaaatacactaaaacctgattttttgtctcttaaggtgtgctaggtgaatgcaaaaaggatcaggaaagggggtgaggataggtcaggaaaagtgcaaacacaatgttctattcataaattagtgatggcatatttaaggttaagtagtaaaaaatatggggggctcagttaacacgaatgaaaaaatagttaaagtagccatgaattatctggataccttgatttaatgacaccctttcttctgtacaatttcataatgtgggaatagagattagtggggattgtagtggtataccctgactttgcttcatgatatctcaaatgtttaaaacctattattccctagagaaagaaatatgttcatactaattgttgcagaggcagaagccaaatatatctcctcctccatttatgtgactatatagtaatgaaaatcctaggttgatacacttttctcaatcttggaaagattctgctaaagcagcaaatcttctaacaagttcaagagggtggggagagtgaacaagtagaataatttatattaccctggaacaattctgaatcctgtaggtatttatgtcactgtttcaattgtgttctggtttaactgtcaatatttatgcatagcagttaacgtgtgtgcatatttgtaactgtgcagtgctactgccaggtgtgactgtacaaatcatgtgctttgaatgtgcaagttttactttcttttctaacaatttaatacagtgttagaaataaataacgaatgaagacaaccaaagagcagccagacaaatgtgaactggttttgacgtgacgagaaactcatcagtaagtaaataaacctcctccctggagaaggccactgaaatgcacccaggaggatgtctctactagaaggtaataaaaaatatatataatgtagtctttgacctaaaacctcatgattattactttgccatttatttccccctggtatctgatgttcatattagtttaatgtgccttttcagagaattcaagacactttttggaaagtagaatttttttttgaaaatttatgattggagaggtactacacaatttagaggttacatttcttgacaaatctgagttgaataaaaaagaactaaaaatataaacatagctaattcaagaatcaagatcgggtgaaactaaattaaaaacagccataaagtcccacattttccctaatttatttacctatgatattggcacatcttgttttacttaacatttgaaaaatacaaatatctcttcatatgcaaaagagcaaatgttaaatgaaaaactgaattttatatagcttcctaaatatgagccacatgcttaagcagtgaattaactttatgaatcaaatgtttaatgttaactattacaaaagcctggtatccaggtgcaatctcaccagaaaaaaatagcacctgcctttattacaataaaaaaaatggctaattccctttgacatcttaagagtgacactactttgtcaagcactaaatactttttaaattaatcatgttaaacttcagatttatagatataaatattgtatttataactttagtcataatgtacaatttctttcttgtttaaaagtactttctcactcaaaatggtatttatagtttaaaaagaatatgcctctgtattcaggagtgattcaaattcccagatgttttcacatagttatgaaaatgggaaagtgctgaattaaactgggctgcaatatttcaagttttttgctatcaggttataaactatacctacgattgcaagtcatacagtgcctctatttctagaaggcttttaaagtttcctggcttagttatgtccaaaggcagcaggaagtctcatcagtagagggcagaattttcaagtgctgccattcttatcccaggaggcatttccagtggttgagcacaaggcctgtttgtagtttgcttttgctcttgcattttgtggaagggaaggaactgagagagcttagagggttcattaaaaccacccctcactctcttagtcgtagtcagatggagtattcataacagtaacctccaattaccactatgtgttgggaaaaattagaattcggtctacttacaatcctgccaactaggattttactttgatatttcagtataacagtgaatctggattgatgcctgattaaaataaaatccctgattattactttctggattacgaactaaaatccctgtaaaatcaatggatgtgactcattgttaagagtcatgcagacttttacatattaggtaagaattctaaaaattatttgagggttctattctctagcaccaggtactaatgctccctactcaaaaaaaatcatgtgcatggattaatcaagtctaacagtgctcagatttaatggtttaacattgattttcttttctttgtcaaacttatatatgcaaatatttttatagtagtcagatgttatttttgaataaggatcaccctcatttttacccatgtgcttatctttaaaaccaacattgtaaagtagcacgcagacatatgtttcttttatcttcatggattatttttaccttaaaaataaattatcatttttttttttgaatttgggttttattctccagatactctgtgtacatgtgggtaagtatgtgggagtatgtgtgtttgtgtgtaagaggggataattaattgtctctcaactctatctcatactttaatatcaaataaaaaatgaaatgtataaagggtcactttgtaggattaggcatcctccttctacctacttaaaccaggggtttgggattcagaattctccatataaccaagaccgaaagtcactggaagactttaaaattagtattttaaccaccacacccagagtcaggtatggaaataaacctatagcatggattctttctatgcataatctcaaaatttaactacccaaataagtaagtttttaaaaactaatttaaaatttgccattgaggaaaatatcacctccatccttaattgtgactcctcatttcagctaaaaccttttctaatactttaaaaaaacaaaatgaaaaacaaactcctagataaagtcataaacactgaaatcagagatgtgattcttgttaaatgttagtttctctttctgaggttacactctgtgcatttgaaactttgacgttaacatcttccgaatgtttagatttgctcaagggttcagattctctggtcttctgccttgcattttcctccttcctttcctttgcaagcaatctatagttgatagcattgccaatgagcagccacacgcttgctgctaccacaatagccccacaggacatgtacatgtatttatattctccagttaaatccaccaatttacctgcaagaggagggccaagaagaactgggccacactccacaattgtgacaagtccgacggcactggaaaatcttggtgcacccacgaggtccatgagagtttcaaagagaacactgctaacactcccaaatccaaggccaaaaaatacagcatataataccaggcttgtgtagtcctgtgccagtgggcacaagaggtgacacactccattgaacatgattgcaaaactgaagaagtactgaattcgaggtcgaatatatttggagtttgcaattaatcctacagaaggcctagcaaacatatcaacgaaagccataacagatagcagaaaagctgccgagtactcatcaattccttggtctttagcatatggagccaagaatataatgggggcaaaaaaacctaggaacataatgacatttccagacagatatatcagaaatcctctatgcttaaaaagggagaaatctaaatacttattaactttttcccaagttgatttcttcgttttgattttctttgggcttgaatcatcttctgttttgccagtcttatttttagacttagaagtggtttgattgggtccaaggggtctcatgagggaaccagccacacaggcattcaaaagtagacttcccaaaatcaggaagcttcctttccagccaaaagtattaaaaaggtactgattgaaaggagccaatgaacttaagaaaacaggacttcctgccatggccaatccatttgccatgggtcgcttcctatagaagtatttgccaattatggttaaggcgggttgcaggttgaaggctaaacctaaacctgtaatgaatcccatagtgaggtacagctgtaccacgctgctactaaaggaggccaacaccattccaagacagcataataagcctcctgctatcaccaccggccggctgccgtatttattcaccaaaacactacttacaggacctaggcatgatcctgattgagtaaagctgcactgaatcctcaaggatgtgaagatcaaaaagctttcaaatattctacctcaagtagatggtgatctctttaaagggtgaatgatgcattccgcttctccttttttcctcctgcgtacataacagccagcataatggatgaaatccatgctatttcactgtaggtagtgtggaatatttgctgaatttctttgaagaatacggtgacagctttggggaatgcataggaaaatccaatggagataaaagctgctccaaccacaatccaaccccatcctccatctggaggtggatgcacaggtggggcacttggcattggtggcatttctgctcctctagtggaaattcaagtaacctggcgacaggtgtttagaaacatggtcttccatttcaccaagacataagtttccctgatctatggactcctctccccacctgaggcagaagtttccttgt

SEQ ID NO: 17824 - RNA, 11390 nt, Homo sapiens
  source 1..11390: mol_type = other RNA
tcgaggagctcacagtctagtaagaaagagatgaatttgaaaatatatttgaaactgtaggcaaaataagtaccctcacagagaaattcaacatttggtttcaaatttgttatgcagtgaaaattagaaactacaaccaagatttttttaaaacattatgttcatataacgctgtagtatacctgaaaggcaagaacttaaacaagtgtgctgaaaaacaaattaggaatatttgaacaaaatatactttaaaaatgatcaacaacgtaaaatattcctgatttaaataaatctaagttattttatttagtttaagcaaaatatgtatccatatgaaaatgccagttctttcatttttggttaattcctttacacatattatttgctaagttcagaaatgctatatatacaaaaatttcaaaaataaataagtatcccaagatcacataacaatactttaagtacattcatgtgtaagaaggcaaaaaaagaaggttctatcttatattttaaaactttgacaggtattttaaatgtattattttatactttattttctttaaaaatgaaataatacagccatgatttaagtcatgtaaaaacaactgtttggatcatttaggtgtcaagcaaaactatcctctttatttcactatcatagtaaccatagttgatagaccatgtggcaatatgatcatttgttcagtggtcattaagatatctatagaataaacaagacaactacattttatttttttcacttaaaaatcacaaaaatacagcctaaaatataatttatattttaaaaataattctaaacattaacccctaaatctaatcccttaaaaaattcttgcaaaagttagctggatgtggctgttgccaaggaatgtcttttattagcaacaagtgactatctataacttttattccaacaatcttattttaaatatttgtttcaatttaatgctgggattagaaaaacatatttgttcaaagtatgtaagtagtaagtaaaacaatttcaaaaatctatcaaaaaaggagaattattcattctaggaaataattaacatactggtttaaaatatctgggagaagaacttttacataaaaagcttcaaatttagtcagttgtagcaagcacttgaaaagaccctgctctttcatctgcaatatcaggaattactatatctgactcatatttgattaagttacaatctcatttttgttgtcactacaaagaaggatccttatattagtaaatgcactcactgcaactactgaggcctgcctcctgtcagaatgacaatgcagtcttagcatacgggtgtcggtttggctgaatctaaccaaacacatcacgtactacagatgtttttagggcccacccaattcataaaagattttactgcgatacatgagtttacccaaatttttattaaaatgtgtttttagggtaaatatcttgatgaactaggcaaacaaatactgaatgcagattactgtttttacagttttaccgggaaaactcctaatagcaacccctcttccccttcaccacagatctttaatttaggtgtgatttttgtttgttctctacatgggaataaaggagaaagtttagaaagactgtatctagctagataagatgcagaggtagatggaatctctaacataaaagaagctctaattacactgttgccagacagctgttatggattttagtattgtttattaggtgaagaaaacattcataaaataagaaatttttgagatagaacttactctaataatttcattaacatatgttcaggttcttagatcaagaaatactgtagaggtgttctcctcaagactatgctatggcaataatttcttgcatacaatttaataatttaaacttgaactgtgtgttctgtgctctggcgttctacttcagaaaaaaatgaacactgcttctaaaataaaaaggaacataaaataaaaaaggaattaatgagatattgacatgttttctattaatacaatattgatgttttaaatgattttgatattgctataacaacatatattgtgcaaaataattaatctcactaaatattatttctgatttgccacgaattatctgccgtggcaatcaggaaatagtcttcaaagtaagtttgcaaacatgattttgcaaaccatgattggaaaaatatattcatttgggctataaactatcaagtagggttgttatatatatttctaggaaaatattttatttactctacaaagatcatcattatgaccttacggcttctgtagtgcaatggagaaaaaagtgtgttagaagttaaaagacctgaattctatctccaaccctgcatttattcagagtattggtataggtttaggcaaaatccttaatccagtctagttttatatggtaaaaatgtggatacctatcaaaactgagggttgagaggatgaaatgaattcattaaacatatcttctgagacataaatatatcaaaacaaatcaaaatacaattagatctaatgtttagaaataaatattttaattcatatttgctatttcactaaatctagaaatactaatgctttagttaaatatagaaagttgatgatagaaaaataaaatccatcgtaccattgaaaagcttgtcagaaatatgtactcttgagattcggaggatgagaaaaaaaatgtgtactctaacgaggaagctatataaactgagtctaactcaaaacatttattttagatgcatataagaattaaagtcttagtcaaaagaatgttttaaaatttcatcctaaatttatgtgagataaaatgccattcttttgtttttctgaacagaggagcttttatcaacttattctattttatttttatttttattattttattttattttatttattattattatactttaagttttagggtacatgtgcacaatgtgcaggttagttacatatgtatacatgtgccatgctggtgcgctgcacccactaactcgtcacctagcattaggtatatctcccaatgctatccctcccccctcccccgaccccaccacagtccccagagtgtgatgttccccttcctgtgtccatgtgttctcattgttcagttcccacctatgagtgagaatatgcggtgtttggttttttgttcttgcgatagtttactgagaatgatgatttctaatttcatccatgtccctacacgaacttattctattttaatagaatgttcagtatcagtgttttcacactgagattctctagcttattttgccatatttaaattaaaaagaaacaaaaaatcctgtttgatcatgtgaaaaatatttactgaaatgtgaataaatttatgatcattaattgcctactgaaatattcctgaatattgctcaccttattaacaagtatatatggagactgaaaaacatgtagatcatgcaaacaagtgtaactaactataccaaagaaacaaaagtccatactaaatatgtccataattaaataaaaaatgctaaacaagttttacctagatattataaaaacatagaaaggaaaacatttaggagatgatgaagaagcaggagattgggatgggagatgtaatttgatctaaattcccatatgcttctgtaaaatcaaaaattcattttgcaatattaattttgctcttaaggtagagacttttaaaatgaccattctcaatactacagcaattcttccctgatttgcacataaatgaattaaagtgaagaaaaagcagtagaggagagaagactaaaataaaccagattgtagcaccctgtaaagagctaaaatctccagtgtacaaacaactgataggaaagaagagaaaatcagaactataaaaaagtgacataagctcagaaaattactcatttttaattgtatcaacaaagataatttgtaattttgatcatgcaagcattataattactgataattgggcctttcagcttttaagtgccttctcaaacatgagttctgcatatggttgtgcagaaatcaaaatcttaaagagagatgagtaaagtcaagtttgtaatattaatcttatattctcaatatagatgctaattagtgctctgaatggttgtggttagaaatcttgttggtatgatgtatcagtgatgtcactgcattgatggagacagaataatacataatggtgcaatgtggtgatggtaagctttgttactcaatattgtcaggcactttaagaaaatcagaaacattcaggatagtgccaaagaagatcagtttttcaagactctaaaatcatattcaattatatgtgtatgtaattataaatatgtgcatcatggctgactttgagaagaatgcagcgccttgcaagtgcactatttgaatagagctaaggagaactatagtctaaggactgcaaaagtctagatggagaagacaaaagcaatgacacttgttttctctacagaacaaatagacaaagaggtgaatgacaacaaagatgttcagagaaacttgaaaaataagctacggtgtagggtaagttgtattaaatgatgaaaattaatatgtaactgtatgggtaaaccaaatcatttgtatcttataatcttttttttggtagctacggataatattataaatggaataatcactaaaattctaaatataatgttttctagtaagaacattttattttttttttaatagagacagattctcactctattgcctaggctggactgcaagtggggccattatagctcactgaagcctcaacttcctgggctcaaatgaccctctcgtctcagcctcccgagtagctgggactacaggtgcacatcaccacatccaggtaattattttactttttgaatcatgatatgtagcaaccaatctgggaattatttattcataaaagataacattttcctgctaactccaacctcagaaaaaatgtattatgcctgactcaaatatgtcattatttttatgagaaaaagagtcatattgaagtaattatgtctatatgtaataattatcattatttgagataatttgcattggggagaaaagcaggcaatcagaaattacatattcaaggctgggcgcagtggctcacgcctgtaatcccagcactttgggaggcagaggcgagtgaatcacctgaggtcagagttcaagaccagcctgaccaacaaggagaaaccccatctctactaaaacaaaacaaaacaaaacaaaacaaaaaaagccacaaaattagccgggcatggtggcacatgcctgtaattccagttactcgggaggctgaggcaggagaattgcttgaacctgggaggcagaggttgtagtaagccgagattgtgccactgcacgccagcctgggcgacaagaacgagactcagtctcaaaaaaaaaaaaaaagaaagaaagaaagaaattacatattcaggttctagcaaatgcagttctctaataaacactaaataaatcataatacaagttacagttaaacctaattgttttactatataggatgtatcttttttgtacctatattttatcttcctttgcttctctggcctctattgggaggcagcacggtagtgaacacctcggggatctttctggttacgtaaacctgagttttaattttggttcatactaccttttaactttgggtagtctgctgagcttgttttttgttttcactcatctgtcatatcaagctagtaataattctgccatggttttggttttcatattgaaaggcattacataagcaaaatgcataacatataaatattagttccctttccactatgcatccaatctccctattaaattaagcctaaaaataataatttttgttttattaaaagccttccacattctacatatgaaagggattttttaaaggtgttttagataaaaaatgtttcaaccaactgaccaagaatatctcttcatatttatgtcatctacataaaaacttacatttatatcatatatcttttagtcttcttttctatattcttgattgtcatgttgtacagccagaaaagaatgagtataaattatctagattttttaaagtgcacattcaaacatagaaaatctaattattttacttgtttcttagtattaggctgaggccaatgagtccatgagctaaagggttgaaacttggcaccaaaaaagtgattgtttatgagtcctgtagatttatactgagaaaacatcatgtcttccaatgtgaaatacactaaaacctgattttttgtctcttaaggtgtgctaggtgaatgcaaaaaggatcaggaaagggggtgaggataggtcaggaaaagtgcaaacacaatgttctattcataaattagtgatggcatatttaaggttaagtagtaaaaaatatggggggctcagttaacacgaatgaaaaaatagttaaagtagccatgaattatctggataccttgatttaatgacaccctttcttctgtacaatttcataatgtgggaatagagattagtggggattgtagtggtataccctgactttgcttcatgatatctcaaatgtttaaaacctattattccctagagaaagaaatatgttcatactaattgttgcagaggcagaagccaaatatatctcctcctccatttatgtgactatatagtaatgaaaatcctaggttgatacacttttctcaatcttggaaagattctgctaaagcagcaaatcttctaacaagttcaagagggtggggagagtgaacaagtagaataatttatattaccctggaacaattctgaatcctgtaggtatttatgtcactgtttcaattgtgttctggtttaactgtcaatatttatgcatagcagttaacgtgtgtgcatatttgtaactgtgcagtgctactgccaggtgtgactgtacaaatcatgtgctttgaatgtgcaagttttactttcttttctaacaatttaatacagtgttagaaataaataacgaatgaagacaaccaaagagcagccagacaaatgtgaactggttttgacgtgacgagaaactcatcagtaagtaaataaacctcctccctggagaaggccactgaaatgcacccaggaggatgtctctactagaaggtaataaaaaatatatataatgtagtctttgacctaaaacctcatgattattactttgccatttatttccccctggtatctgatgttcatattagtttaatgtgccttttcagagaattcaagacactttttggaaagtagaatttttttttgaaaatttatgattggagaggtactacacaatttagaggttacatttcttgacaaatctgagttgaataaaaaagaactaaaaatataaacatagctaattcaagaatcaagatcgggtgaaactaaattaaaaacagccataaagtcccacattttccctaatttatttacctatgatattggcacatcttgttttacttaacatttgaaaaatacaaatatctcttcatatgcaaaagagcaaatgttaaatgaaaaactgaattttatatagcttcctaaatatgagccacatgcttaagcagtgaattaactttatgaatcaaatgtttaatgttaactattacaaaagcctggtatccaggtgcaatctcaccagaaaaaaatagcacctgcctttattacaataaaaaaaatggctaattccctttgacatcttaagagtgacactactttgtcaagcactaaatactttttaaattaatcatgttaaacttcagatttatagatataaatattgtatttataactttagtcataatgtacaatttctttcttgtttaaaagtactttctcactcaaaatggtatttatagtttaaaaagaatatgcctctgtattcaggagtgattcaaattcccagatgttttcacatagttatgaaaatgggaaagtgctgaattaaactgggctgcaatatttcaagttttttgctatcaggttataaactatacctacgattgcaagtcatacagtgcctctatttctagaaggcttttaaagtttcctggcttagttatgtccaaaggcagcaggaagtctcatcagtagagggcagaattttcaagtgctgccattcttatcccaggaggcatttccagtggttgagcacaaggcctgtttgtagtttgcttttgctcttgcattttgtggaagggaaggaactgagagagcttagagggttcattaaaaccacccctcactctcttagtcgtagtcagatggagtattcataacagtaacctccaattaccactatgtgttgggaaaaattagaattcggtctacttacaatcctgccaactaggattttactttgatatttcagtataacagtgaatctggattgatgcctgattaaaataaaatccctgattattactttctggattacgaactaaaatccctgtaaaatcaatggatgtgactcattgttaagagtcatgcagacttttacatattaggtaagaattctaaaaattatttgagggttctattctctagcaccaggtactaatgctccctactcaaaaaaaatcatgtgcatggattaatcaagtctaacagtgctcagatttaatggtttaacattgattttcttttctttgtcaaacttatatatgcaaatatttttatagtagtcagatgttatttttgaataaggatcaccctcatttttacccatgtgcttatctttaaaaccaacattgtaaagtagcacgcagacatatgtttcttttatcttcatggattatttttaccttaaaaataaattatcatttttttttttgaatttgggttttattctccagatactctgtgtacatgtgggtaagtatgtgggagtatgtgtgtttgtgtgtaagaggggataattaattgtctctcaactctatctcatactttaatatcaaataaaaaatgaaatgtataaagggtcactttgtaggattaggcatcctccttctacctacttaaaccaggggtttgggattcagaattctccatataaccaagaccgaaagtcactggaagactttaaaattagtattttaaccaccacacccagagtcaggtatggaaataaacctatagcatggattctttctatgcataatctcaaaatttaactacccaaataagtaagtttttaaaaactaatttaaaatttgccattgaggaaaatatcacctccatccttaattgtgactcctcatttcagctaaaaccttttctaatactttaaaaaaacaaaatgaaaaacaaactcctagataaagtcataaacactgaaatcagagatgtgattcttgttaaatgttagtttctctttctgaggttacactctgtgcatttgaaactttgacgttaacatcttccgaatgtttagatttgctcaagggttcagattctctggtcttctgccttgcattttcctccttcctttcctttgcaagcaatctatagttgatagcattgccaatgagcagccacacgcttgctgctaccacaatagccccacaggacatgtacatgtatttatattctccagttaaatccaccaatttacctgcaagaggagggccaagaagaactgggccacactccacaattgtgacaagtccgacggcactggaaaatcttggtgcacccacgaggtccatgagagtttcaaagagaacactgctaacactcccaaatccaaggccaaaaaatacagcatataataccaggcttgtgtagtcctgtgccagtgggcacaagaggtgacacactccattgaacatgattgcaaaactgaagaagtactgaattcgaggtcgaatatatttggagtttgcaattaatcctacagaaggcctagcaaacatatcaacgaaagccataacagatagcagaaaagctgccgagtactcatcaattccttggtctttagcatatggagccaagaatataatgggggcaaaaaaacctaggaacataatgacatttccagacagatatatcagaaatcctctatgcttaaaaagggagaaatctaaatacttattaactttttcccaagttgatttcttcgttttgattttctttgggcttgaatcatcttctgttttgccagtcttatttttagacttagaagtggtttgattgggtccaaggggtctcatgagggaaccagccacacaggcattcaaaagtagacttcccaaaatcaggaagcttcctttccagccaaaagtattaaaaaggtactgattgaaaggagccaatgaacttaagaaaacaggacttcctgccatggccaatccatttgccatgggtcgcttcctatagaagtatttgccaattatggttaaggcgggttgcaggttgaaggctaaacctaaacctgtaatgaatcccatagtgaggtacagctgtaccacgctgctactaaaggaggccaacaccattccaagacagcataataagcctcctgctatcaccaccggccggctgccgtatttattcaccaaaacactacttacaggacctaggcatgatcctgattgagtaaagctgcactgaatcctcaaggatgtgaagatcaaaaagctttcaaatattctacctcctgcgtacataacagccagcataatggatgaaatccatgctatttcactgtaggtagtgtggaatatttgctgaatttctttgaagaatacggtgacagctttggggaatgcataggaaaatccaatggagataaaagctgctccaaccacaatccaaccccatcctccatctggaggtggatgcacaggtggggcacttggcattggtggcatttctgctcctctagtggaaattcaagtaacagagtaactctgttggcaccaagagtcccagagtctttggttccccagatcaccttgtttcaggtttcacaggaaagtatcacatcttaagattgactctttatctggtctctggcgcagggtgggcgctgcagccctccgttcccagcaaaccgcagccgattcgcctcgctgtcaacgggtgaatggaattatttatttatttatggcccctgacgtgtcctcgcccgccacagccagcggagaaggaggcggtggcgggaaggggaggcgcggctgctgaacgcccttgtgggtgcggaggagcgcgcgccaggggtgggggccggacaggctgcggtggaggccggcccggggggtggtgggggggagccgcctcccggtgcctggagaccgactgag

SEQ ID NO: 17825 - RNA, 12015 nt, Homo sapiens
  source 1..12015: mol_type = other RNA
tcgaggagctcacagtctagtaagaaagagatgaatttgaaaatatatttgaaactgtaggcaaaataagtaccctcacagagaaattcaacatttggtttcaaatttgttatgcagtgaaaattagaaactacaaccaagatttttttaaaacattatgttcatataacgctgtagtatacctgaaaggcaagaacttaaacaagtgtgctgaaaaacaaattaggaatatttgaacaaaatatactttaaaaatgatcaacaacgtaaaatattcctgatttaaataaatctaagttattttatttagtttaagcaaaatatgtatccatatgaaaatgccagttctttcatttttggttaattcctttacacatattatttgctaagttcagaaatgctatatatacaaaaatttcaaaaataaataagtatcccaagatcacataacaatactttaagtacattcatgtgtaagaaggcaaaaaaagaaggttctatcttatattttaaaactttgacaggtattttaaatgtattattttatactttattttctttaaaaatgaaataatacagccatgatttaagtcatgtaaaaacaactgtttggatcatttaggtgtcaagcaaaactatcctctttatttcactatcatagtaaccatagttgatagaccatgtggcaatatgatcatttgttcagtggtcattaagatatctatagaataaacaagacaactacattttatttttttcacttaaaaatcacaaaaatacagcctaaaatataatttatattttaaaaataattctaaacattaacccctaaatctaatcccttaaaaaattcttgcaaaagttagctggatgtggctgttgccaaggaatgtcttttattagcaacaagtgactatctataacttttattccaacaatcttattttaaatatttgtttcaatttaatgctgggattagaaaaacatatttgttcaaagtatgtaagtagtaagtaaaacaatttcaaaaatctatcaaaaaaggagaattattcattctaggaaataattaacatactggtttaaaatatctgggagaagaacttttacataaaaagcttcaaatttagtcagttgtagcaagcacttgaaaagaccctgctctttcatctgcaatatcaggaattactatatctgactcatatttgattaagttacaatctcatttttgttgtcactacaaagaaggatccttatattagtaaatgcactcactgcaactactgaggcctgcctcctgtcagaatgacaatgcagtcttagcatacgggtgtcggtttggctgaatctaaccaaacacatcacgtactacagatgtttttagggcccacccaattcataaaagattttactgcgatacatgagtttacccaaatttttattaaaatgtgtttttagggtaaatatcttgatgaactaggcaaacaaatactgaatgcagattactgtttttacagttttaccgggaaaactcctaatagcaacccctcttccccttcaccacagatctttaatttaggtgtgatttttgtttgttctctacatgggaataaaggagaaagtttagaaagactgtatctagctagataagatgcagaggtagatggaatctctaacataaaagaagctctaattacactgttgccagacagctgttatggattttagtattgtttattaggtgaagaaaacattcataaaataagaaatttttgagatagaacttactctaataatttcattaacatatgttcaggttcttagatcaagaaatactgtagaggtgttctcctcaagactatgctatggcaataatttcttgcatacaatttaataatttaaacttgaactgtgtgttctgtgctctggcgttctacttcagaaaaaaatgaacactgcttctaaaataaaaaggaacataaaataaaaaaggaattaatgagatattgacatgttttctattaatacaatattgatgttttaaatgattttgatattgctataacaacatatattgtgcaaaataattaatctcactaaatattatttctgatttgccacgaattatctgccgtggcaatcaggaaatagtcttcaaagtaagtttgcaaacatgattttgcaaaccatgattggaaaaatatattcatttgggctataaactatcaagtagggttgttatatatatttctaggaaaatattttatttactctacaaagatcatcattatgaccttacggcttctgtagtgcaatggagaaaaaagtgtgttagaagttaaaagacctgaattctatctccaaccctgcatttattcagagtattggtataggtttaggcaaaatccttaatccagtctagttttatatggtaaaaatgtggatacctatcaaaactgagggttgagaggatgaaatgaattcattaaacatatcttctgagacataaatatatcaaaacaaatcaaaatacaattagatctaatgtttagaaataaatattttaattcatatttgctatttcactaaatctagaaatactaatgctttagttaaatatagaaagttgatgatagaaaaataaaatccatcgtaccattgaaaagcttgtcagaaatatgtactcttgagattcggaggatgagaaaaaaaatgtgtactctaacgaggaagctatataaactgagtctaactcaaaacatttattttagatgcatataagaattaaagtcttagtcaaaagaatgttttaaaatttcatcctaaatttatgtgagataaaatgccattcttttgtttttctgaacagaggagcttttatcaacttattctattttatttttatttttattattttattttattttatttattattattatactttaagttttagggtacatgtgcacaatgtgcaggttagttacatatgtatacatgtgccatgctggtgcgctgcacccactaactcgtcacctagcattaggtatatctcccaatgctatccctcccccctcccccgaccccaccacagtccccagagtgtgatgttccccttcctgtgtccatgtgttctcattgttcagttcccacctatgagtgagaatatgcggtgtttggttttttgttcttgcgatagtttactgagaatgatgatttctaatttcatccatgtccctacacgaacttattctattttaatagaatgttcagtatcagtgttttcacactgagattctctagcttattttgccatatttaaattaaaaagaaacaaaaaatcctgtttgatcatgtgaaaaatatttactgaaatgtgaataaatttatgatcattaattgcctactgaaatattcctgaatattgctcaccttattaacaagtatatatggagactgaaaaacatgtagatcatgcaaacaagtgtaactaactataccaaagaaacaaaagtccatactaaatatgtccataattaaataaaaaatgctaaacaagttttacctagatattataaaaacatagaaaggaaaacatttaggagatgatgaagaagcaggagattgggatgggagatgtaatttgatctaaattcccatatgcttctgtaaaatcaaaaattcattttgcaatattaattttgctcttaaggtagagacttttaaaatgaccattctcaatactacagcaattcttccctgatttgcacataaatgaattaaagtgaagaaaaagcagtagaggagagaagactaaaataaaccagattgtagcaccctgtaaagagctaaaatctccagtgtacaaacaactgataggaaagaagagaaaatcagaactataaaaaagtgacataagctcagaaaattactcatttttaattgtatcaacaaagataatttgtaattttgatcatgcaagcattataattactgataattgggcctttcagcttttaagtgccttctcaaacatgagttctgcatatggttgtgcagaaatcaaaatcttaaagagagatgagtaaagtcaagtttgtaatattaatcttatattctcaatatagatgctaattagtgctctgaatggttgtggttagaaatcttgttggtatgatgtatcagtgatgtcactgcattgatggagacagaataatacataatggtgcaatgtggtgatggtaagctttgttactcaatattgtcaggcactttaagaaaatcagaaacattcaggatagtgccaaagaagatcagtttttcaagactctaaaatcatattcaattatatgtgtatgtaattataaatatgtgcatcatggctgactttgagaagaatgcagcgccttgcaagtgcactatttgaatagagctaaggagaactatagtctaaggactgcaaaagtctagatggagaagacaaaagcaatgacacttgttttctctacagaacaaatagacaaagaggtgaatgacaacaaagatgttcagagaaacttgaaaaataagctacggtgtagggtaagttgtattaaatgatgaaaattaatatgtaactgtatgggtaaaccaaatcatttgtatcttataatcttttttttggtagctacggataatattataaatggaataatcactaaaattctaaatataatgttttctagtaagaacattttattttttttttaatagagacagattctcactctattgcctaggctggactgcaagtggggccattatagctcactgaagcctcaacttcctgggctcaaatgaccctctcgtctcagcctcccgagtagctgggactacaggtgcacatcaccacatccaggtaattattttactttttgaatcatgatatgtagcaaccaatctgggaattatttattcataaaagataacattttcctgctaactccaacctcagaaaaaatgtattatgcctgactcaaatatgtcattatttttatgagaaaaagagtcatattgaagtaattatgtctatatgtaataattatcattatttgagataatttgcattggggagaaaagcaggcaatcagaaattacatattcaaggctgggcgcagtggctcacgcctgtaatcccagcactttgggaggcagaggcgagtgaatcacctgaggtcagagttcaagaccagcctgaccaacaaggagaaaccccatctctactaaaacaaaacaaaacaaaacaaaacaaaaaaagccacaaaattagccgggcatggtggcacatgcctgtaattccagttactcgggaggctgaggcaggagaattgcttgaacctgggaggcagaggttgtagtaagccgagattgtgccactgcacgccagcctgggcgacaagaacgagactcagtctcaaaaaaaaaaaaaaagaaagaaagaaagaaattacatattcaggttctagcaaatgcagttctctaataaacactaaataaatcataatacaagttacagttaaacctaattgttttactatataggatgtatcttttttgtacctatattttatcttcctttgcttctctggcctctattgggaggcagcacggtagtgaacacctcggggatctttctggttacgtaaacctgagttttaattttggttcatactaccttttaactttgggtagtctgctgagcttgttttttgttttcactcatctgtcatatcaagctagtaataattctgccatggttttggttttcatattgaaaggcattacataagcaaaatgcataacatataaatattagttccctttccactatgcatccaatctccctattaaattaagcctaaaaataataatttttgttttattaaaagccttccacattctacatatgaaagggattttttaaaggtgttttagataaaaaatgtttcaaccaactgaccaagaatatctcttcatatttatgtcatctacataaaaacttacatttatatcatatatcttttagtcttcttttctatattcttgattgtcatgttgtacagccagaaaagaatgagtataaattatctagattttttaaagtgcacattcaaacatagaaaatctaattattttacttgtttcttagtattaggctgaggccaatgagtccatgagctaaagggttgaaacttggcaccaaaaaagtgattgtttatgagtcctgtagatttatactgagaaaacatcatgtcttccaatgtgaaatacactaaaacctgattttttgtctcttaaggtgtgctaggtgaatgcaaaaaggatcaggaaagggggtgaggataggtcaggaaaagtgcaaacacaatgttctattcataaattagtgatggcatatttaaggttaagtagtaaaaaatatggggggctcagttaacacgaatgaaaaaatagttaaagtagccatgaattatctggataccttgatttaatgacaccctttcttctgtacaatttcataatgtgggaatagagattagtggggattgtagtggtataccctgactttgcttcatgatatctcaaatgtttaaaacctattattccctagagaaagaaatatgttcatactaattgttgcagaggcagaagccaaatatatctcctcctccatttatgtgactatatagtaatgaaaatcctaggttgatacacttttctcaatcttggaaagattctgctaaagcagcaaatcttctaacaagttcaagagggtggggagagtgaacaagtagaataatttatattaccctggaacaattctgaatcctgtaggtatttatgtcactgtttcaattgtgttctggtttaactgtcaatatttatgcatagcagttaacgtgtgtgcatatttgtaactgtgcagtgctactgccaggtgtgactgtacaaatcatgtgctttgaatgtgcaagttttactttcttttctaacaatttaatacagtgttagaaataaataacgaatgaagacaaccaaagagcagccagacaaatgtgaactggttttgacgtgacgagaaactcatcagtaagtaaataaacctcctccctggagaaggccactgaaatgcacccaggaggatgtctctactagaaggtaataaaaaatatatataatgtagtctttgacctaaaacctcatgattattactttgccatttatttccccctggtatctgatgttcatattagtttaatgtgccttttcagagaattcaagacactttttggaaagtagaatttttttttgaaaatttatgattggagaggtactacacaatttagaggttacatttcttgacaaatctgagttgaataaaaaagaactaaaaatataaacatagctaattcaagaatcaagatcgggtgaaactaaattaaaaacagccataaagtcccacattttccctaatttatttacctatgatattggcacatcttgttttacttaacatttgaaaaatacaaatatctcttcatatgcaaaagagcaaatgttaaatgaaaaactgaattttatatagcttcctaaatatgagccacatgcttaagcagtgaattaactttatgaatcaaatgtttaatgttaactattacaaaagcctggtatccaggtgcaatctcaccagaaaaaaatagcacctgcctttattacaataaaaaaaatggctaattccctttgacatcttaagagtgacactactttgtcaagcactaaatactttttaaattaatcatgttaaacttcagatttatagatataaatattgtatttataactttagtcataatgtacaatttctttcttgtttaaaagtactttctcactcaaaatggtatttatagtttaaaaagaatatgcctctgtattcaggagtgattcaaattcccagatgttttcacatagttatgaaaatgggaaagtgctgaattaaactgggctgcaatatttcaagttttttgctatcaggttataaactatacctacgattgcaagtcatacagtgcctctatttctagaaggcttttaaagtttcctggcttagttatgtccaaaggcagcaggaagtctcatcagtagagggcagaattttcaagtgctgccattcttatcccaggaggcatttccagtggttgagcacaaggcctgtttgtagtttgcttttgctcttgcattttgtggaagggaaggaactgagagagcttagagggttcattaaaaccacccctcactctcttagtcgtagtcagatggagtattcataacagtaacctccaattaccactatgtgttgggaaaaattagaattcggtctacttacaatcctgccaactaggattttactttgatatttcagtataacagtgaatctggattgatgcctgattaaaataaaatccctgattattactttctggattacgaactaaaatccctgtaaaatcaatggatgtgactcattgttaagagtcatgcagacttttacatattaggtaagaattctaaaaattatttgagggttctattctctagcaccaggtactaatgctccctactcaaaaaaaatcatgtgcatggattaatcaagtctaacagtgctcagatttaatggtttaacattgattttcttttctttgtcaaacttatatatgcaaatatttttatagtagtcagatgttatttttgaataaggatcaccctcatttttacccatgtgcttatctttaaaaccaacattgtaaagtagcacgcagacatatgtttcttttatcttcatggattatttttaccttaaaaataaattatcatttttttttttgaatttgggttttattctccagatactctgtgtacatgtgggtaagtatgtgggagtatgtgtgtttgtgtgtaagaggggataattaattgtctctcaactctatctcatactttaatatcaaataaaaaatgaaatgtataaagggtcactttgtaggattaggcatcctccttctacctacttaaaccaggggtttgggattcagaattctccatataaccaagaccgaaagtcactggaagactttaaaattagtattttaaccaccacacccagagtcaggtatggaaataaacctatagcatggattctttctatgcataatctcaaaatttaactacccaaataagtaagtttttaaaaactaatttaaaatttgccattgaggaaaatatcacctccatccttaattgtgactcctcatttcagctaaaaccttttctaatactttaaaaaaacaaaatgaaaaacaaactcctagataaagtcataaacactgaaatcagagatgtgattcttgttaaatgttagtttctctttctgaggttacactctgtgcatttgaaactttgacgttaacatcttccgaatgtttagatttgctcaagggttcagattctctggtcttctgccttgcattttcctccttcctttcctttgcaagcaatctatagttgatagcattgccaatgagcagccacacgcttgctgctaccacaatagccccacaggacatgtacatgtatttatattctccagttaaatccaccaatttacctgcaagaggagggccaagaagaactgggccacactccacaattgtgacaagtccgacggcactggaaaatcttggtgcacccacgaggtccatgagagtttcaaagagaacactgctaacactcccaaatccaaggccaaaaaatacagcatataataccaggcttgtgtagtcctgtgccagtgggcacaagaggtgacacactccattgaacatgattgcaaaactgaagaagtactgaattcgaggtcgaatatatttggagtttgcaattaatcctacagaaggcctagcaaacatatcaacgaaagccataacagatagcagaaaagctgccgagtactcatcaattccttggtctttagcatatggagccaagaatataatgggggcaaaaaaacctaggaacataatgacatttccagacagatatatcagaaatcctctatgcttaaaaagggagaaatctaaatacttattaactttttcccaagttgatttcttcgttttgattttctttgggcttgaatcatcttctgttttgccagtcttatttttagacttagaagtggtttgattgggtccaaggggtctcatgagggaaccagccacacaggcattcaaaagtagacttcccaaaatcaggaagcttcctttccagccaaaagtattaaaaaggtactgattgaaaggagccaatgaacttaagaaaacaggacttcctgccatggccaatccatttgccatgggtcgcttcctatagaagtatttgccaattatggttaaggcgggttgcaggttgaaggctaaacctaaacctgtaatgaatcccatagtgaggtacagctgtaccacgctgctactaaaggaggccaacaccattccaagacagcataataagcctcctgctatcaccaccggccggctgccgtatttattcaccaaaacactacttacaggacctaggcatgatcctgattgagtaaagctgcactgaatcctcaaggatgtgaagatcaaaaagctttcaaatattctacctcctgcgtacataacagccagcataatggatgaaatccatgctatttcactgtaggtagtgtggaatatttgctgaatttctttgaagaatacggtgacagctttggggaatgcataggaaaatccaatggagataaaagctgctccaaccacaatccaaccccatcctccatctggaggtggatgcacaggtggggcacttggcattggtggcatttctgctcctctagtggaaattcaagtaacatacatatctccagagactctgctttgccctcccctctctcttctctcaaatagggcaaagttagttatttctctttttcaagaacctgctttgacgtgcactattagttcatacttttcagagtctaaagtaagcttggcttaaattatatcatgggtcaaagaaggtggccaagtctggcaatttgaactgctaaatttaaccttctcatgtgttgtgttgatgtagccacattttcaagcacattttccattgcgtgatttaatatgcataaaacatattgcaaaaatactgtactatatacattaatagtttagtgactcttcactgagtctgagactaggtaatttgtaagttatgaacaataacaaagaggccagggtcaaagtgttgaatctcttgtgggccagtttaatctatttcttgatcacacataacactccctacatggtcagccactctgtaaatgcatgctctctgtcccaaagagtccccaaccctgtgtgagggtgaatctggtgatagatcattagtaccatcttcgttttagaagaaattactataacctttggaaaaatgcagtggtgtaatttattaaatgcttctcatattctaggtaagcattttgccaaacaatttatacccactaccccattctctaaatgatacatgatagacattatgataaatattttcctatggggacactgaagctcagcgttttgattacttatgtaaggccatatagctgtaaaatatggggtcctggattccaactctagattgtctagattcgaggctcatgttcctctctatcaaacagcatgccagactcctctatcagtggatgagaaatatctgatttcctatgtgaaagatacaattatttagatctaagcactaagcagtagccacttgtaaaatatgcttcccaaagatttgggaaggctgcatttctaaatgtgtataataatgaaataataataaccaggtaataacataaataacctctagaaattttatcta

SEQ ID NO: 17826 - RNA, 11080 nt, Homo sapiens
  source 1..11080: mol_type = other RNA
tcgaggagctcacagtctagtaagaaagagatgaatttgaaaatatatttgaaactgtaggcaaaataagtaccctcacagagaaattcaacatttggtttcaaatttgttatgcagtgaaaattagaaactacaaccaagatttttttaaaacattatgttcatataacgctgtagtatacctgaaaggcaagaacttaaacaagtgtgctgaaaaacaaattaggaatatttgaacaaaatatactttaaaaatgatcaacaacgtaaaatattcctgatttaaataaatctaagttattttatttagtttaagcaaaatatgtatccatatgaaaatgccagttctttcatttttggttaattcctttacacatattatttgctaagttcagaaatgctatatatacaaaaatttcaaaaataaataagtatcccaagatcacataacaatactttaagtacattcatgtgtaagaaggcaaaaaaagaaggttctatcttatattttaaaactttgacaggtattttaaatgtattattttatactttattttctttaaaaatgaaataatacagccatgatttaagtcatgtaaaaacaactgtttggatcatttaggtgtcaagcaaaactatcctctttatttcactatcatagtaaccatagttgatagaccatgtggcaatatgatcatttgttcagtggtcattaagatatctatagaataaacaagacaactacattttatttttttcacttaaaaatcacaaaaatacagcctaaaatataatttatattttaaaaataattctaaacattaacccctaaatctaatcccttaaaaaattcttgcaaaagttagctggatgtggctgttgccaaggaatgtcttttattagcaacaagtgactatctataacttttattccaacaatcttattttaaatatttgtttcaatttaatgctgggattagaaaaacatatttgttcaaagtatgtaagtagtaagtaaaacaatttcaaaaatctatcaaaaaaggagaattattcattctaggaaataattaacatactggtttaaaatatctgggagaagaacttttacataaaaagcttcaaatttagtcagttgtagcaagcacttgaaaagaccctgctctttcatctgcaatatcaggaattactatatctgactcatatttgattaagttacaatctcatttttgttgtcactacaaagaaggatccttatattagtaaatgcactcactgcaactactgaggcctgcctcctgtcagaatgacaatgcagtcttagcatacgggtgtcggtttggctgaatctaaccaaacacatcacgtactacagatgtttttagggcccacccaattcataaaagattttactgcgatacatgagtttacccaaatttttattaaaatgtgtttttagggtaaatatcttgatgaactaggcaaacaaatactgaatgcagattactgtttttacagttttaccgggaaaactcctaatagcaacccctcttccccttcaccacagatctttaatttaggtgtgatttttgtttgttctctacatgggaataaaggagaaagtttagaaagactgtatctagctagataagatgcagaggtagatggaatctctaacataaaagaagctctaattacactgttgccagacagctgttatggattttagtattgtttattaggtgaagaaaacattcataaaataagaaatttttgagatagaacttactctaataatttcattaacatatgttcaggttcttagatcaagaaatactgtagaggtgttctcctcaagactatgctatggcaataatttcttgcatacaatttaataatttaaacttgaactgtgtgttctgtgctctggcgttctacttcagaaaaaaatgaacactgcttctaaaataaaaaggaacataaaataaaaaaggaattaatgagatattgacatgttttctattaatacaatattgatgttttaaatgattttgatattgctataacaacatatattgtgcaaaataattaatctcactaaatattatttctgatttgccacgaattatctgccgtggcaatcaggaaatagtcttcaaagtaagtttgcaaacatgattttgcaaaccatgattggaaaaatatattcatttgggctataaactatcaagtagggttgttatatatatttctaggaaaatattttatttactctacaaagatcatcattatgaccttacggcttctgtagtgcaatggagaaaaaagtgtgttagaagttaaaagacctgaattctatctccaaccctgcatttattcagagtattggtataggtttaggcaaaatccttaatccagtctagttttatatggtaaaaatgtggatacctatcaaaactgagggttgagaggatgaaatgaattcattaaacatatcttctgagacataaatatatcaaaacaaatcaaaatacaattagatctaatgtttagaaataaatattttaattcatatttgctatttcactaaatctagaaatactaatgctttagttaaatatagaaagttgatgatagaaaaataaaatccatcgtaccattgaaaagcttgtcagaaatatgtactcttgagattcggaggatgagaaaaaaaatgtgtactctaacgaggaagctatataaactgagtctaactcaaaacatttattttagatgcatataagaattaaagtcttagtcaaaagaatgttttaaaatttcatcctaaatttatgtgagataaaatgccattcttttgtttttctgaacagaggagcttttatcaacttattctattttatttttatttttattattttattttattttatttattattattatactttaagttttagggtacatgtgcacaatgtgcaggttagttacatatgtatacatgtgccatgctggtgcgctgcacccactaactcgtcacctagcattaggtatatctcccaatgctatccctcccccctcccccgaccccaccacagtccccagagtgtgatgttccccttcctgtgtccatgtgttctcattgttcagttcccacctatgagtgagaatatgcggtgtttggttttttgttcttgcgatagtttactgagaatgatgatttctaatttcatccatgtccctacacgaacttattctattttaatagaatgttcagtatcagtgttttcacactgagattctctagcttattttgccatatttaaattaaaaagaaacaaaaaatcctgtttgatcatgtgaaaaatatttactgaaatgtgaataaatttatgatcattaattgcctactgaaatattcctgaatattgctcaccttattaacaagtatatatggagactgaaaaacatgtagatcatgcaaacaagtgtaactaactataccaaagaaacaaaagtccatactaaatatgtccataattaaataaaaaatgctaaacaagttttacctagatattataaaaacatagaaaggaaaacatttaggagatgatgaagaagcaggagattgggatgggagatgtaatttgatctaaattcccatatgcttctgtaaaatcaaaaattcattttgcaatattaattttgctcttaaggtagagacttttaaaatgaccattctcaatactacagcaattcttccctgatttgcacataaatgaattaaagtgaagaaaaagcagtagaggagagaagactaaaataaaccagattgtagcaccctgtaaagagctaaaatctccagtgtacaaacaactgataggaaagaagagaaaatcagaactataaaaaagtgacataagctcagaaaattactcatttttaattgtatcaacaaagataatttgtaattttgatcatgcaagcattataattactgataattgggcctttcagcttttaagtgccttctcaaacatgagttctgcatatggttgtgcagaaatcaaaatcttaaagagagatgagtaaagtcaagtttgtaatattaatcttatattctcaatatagatgctaattagtgctctgaatggttgtggttagaaatcttgttggtatgatgtatcagtgatgtcactgcattgatggagacagaataatacataatggtgcaatgtggtgatggtaagctttgttactcaatattgtcaggcactttaagaaaatcagaaacattcaggatagtgccaaagaagatcagtttttcaagactctaaaatcatattcaattatatgtgtatgtaattataaatatgtgcatcatggctgactttgagaagaatgcagcgccttgcaagtgcactatttgaatagagctaaggagaactatagtctaaggactgcaaaagtctagatggagaagacaaaagcaatgacacttgttttctctacagaacaaatagacaaagaggtgaatgacaacaaagatgttcagagaaacttgaaaaataagctacggtgtagggtaagttgtattaaatgatgaaaattaatatgtaactgtatgggtaaaccaaatcatttgtatcttataatcttttttttggtagctacggataatattataaatggaataatcactaaaattctaaatataatgttttctagtaagaacattttattttttttttaatagagacagattctcactctattgcctaggctggactgcaagtggggccattatagctcactgaagcctcaacttcctgggctcaaatgaccctctcgtctcagcctcccgagtagctgggactacaggtgcacatcaccacatccaggtaattattttactttttgaatcatgatatgtagcaaccaatctgggaattatttattcataaaagataacattttcctgctaactccaacctcagaaaaaatgtattatgcctgactcaaatatgtcattatttttatgagaaaaagagtcatattgaagtaattatgtctatatgtaataattatcattatttgagataatttgcattggggagaaaagcaggcaatcagaaattacatattcaaggctgggcgcagtggctcacgcctgtaatcccagcactttgggaggcagaggcgagtgaatcacctgaggtcagagttcaagaccagcctgaccaacaaggagaaaccccatctctactaaaacaaaacaaaacaaaacaaaacaaaaaaagccacaaaattagccgggcatggtggcacatgcctgtaattccagttactcgggaggctgaggcaggagaattgcttgaacctgggaggcagaggttgtagtaagccgagattgtgccactgcacgccagcctgggcgacaagaacgagactcagtctcaaaaaaaaaaaaaaagaaagaaagaaagaaattacatattcaggttctagcaaatgcagttctctaataaacactaaataaatcataatacaagttacagttaaacctaattgttttactatataggatgtatcttttttgtacctatattttatcttcctttgcttctctggcctctattgggaggcagcacggtagtgaacacctcggggatctttctggttacgtaaacctgagttttaattttggttcatactaccttttaactttgggtagtctgctgagcttgttttttgttttcactcatctgtcatatcaagctagtaataattctgccatggttttggttttcatattgaaaggcattacataagcaaaatgcataacatataaatattagttccctttccactatgcatccaatctccctattaaattaagcctaaaaataataatttttgttttattaaaagccttccacattctacatatgaaagggattttttaaaggtgttttagataaaaaatgtttcaaccaactgaccaagaatatctcttcatatttatgtcatctacataaaaacttacatttatatcatatatcttttagtcttcttttctatattcttgattgtcatgttgtacagccagaaaagaatgagtataaattatctagattttttaaagtgcacattcaaacatagaaaatctaattattttacttgtttcttagtattaggctgaggccaatgagtccatgagctaaagggttgaaacttggcaccaaaaaagtgattgtttatgagtcctgtagatttatactgagaaaacatcatgtcttccaatgtgaaatacactaaaacctgattttttgtctcttaaggtgtgctaggtgaatgcaaaaaggatcaggaaagggggtgaggataggtcaggaaaagtgcaaacacaatgttctattcataaattagtgatggcatatttaaggttaagtagtaaaaaatatggggggctcagttaacacgaatgaaaaaatagttaaagtagccatgaattatctggataccttgatttaatgacaccctttcttctgtacaatttcataatgtgggaatagagattagtggggattgtagtggtataccctgactttgcttcatgatatctcaaatgtttaaaacctattattccctagagaaagaaatatgttcatactaattgttgcagaggcagaagccaaatatatctcctcctccatttatgtgactatatagtaatgaaaatcctaggttgatacacttttctcaatcttggaaagattctgctaaagcagcaaatcttctaacaagttcaagagggtggggagagtgaacaagtagaataatttatattaccctggaacaattctgaatcctgtaggtatttatgtcactgtttcaattgtgttctggtttaactgtcaatatttatgcatagcagttaacgtgtgtgcatatttgtaactgtgcagtgctactgccaggtgtgactgtacaaatcatgtgctttgaatgtgcaagttttactttcttttctaacaatttaatacagtgttagaaataaataacgaatgaagacaaccaaagagcagccagacaaatgtgaactggttttgacgtgacgagaaactcatcagtaagtaaataaacctcctccctggagaaggccactgaaatgcacccaggaggatgtctctactagaaggtaataaaaaatatatataatgtagtctttgacctaaaacctcatgattattactttgccatttatttccccctggtatctgatgttcatattagtttaatgtgccttttcagagaattcaagacactttttggaaagtagaatttttttttgaaaatttatgattggagaggtactacacaatttagaggttacatttcttgacaaatctgagttgaataaaaaagaactaaaaatataaacatagctaattcaagaatcaagatcgggtgaaactaaattaaaaacagccataaagtcccacattttccctaatttatttacctatgatattggcacatcttgttttacttaacatttgaaaaatacaaatatctcttcatatgcaaaagagcaaatgttaaatgaaaaactgaattttatatagcttcctaaatatgagccacatgcttaagcagtgaattaactttatgaatcaaatgtttaatgttaactattacaaaagcctggtatccaggtgcaatctcaccagaaaaaaatagcacctgcctttattacaataaaaaaaatggctaattccctttgacatcttaagagtgacactactttgtcaagcactaaatactttttaaattaatcatgttaaacttcagatttatagatataaatattgtatttataactttagtcataatgtacaatttctttcttgtttaaaagtactttctcactcaaaatggtatttatagtttaaaaagaatatgcctctgtattcaggagtgattcaaattcccagatgttttcacatagttatgaaaatgggaaagtgctgaattaaactgggctgcaatatttcaagttttttgctatcaggttataaactatacctacgattgcaagtcatacagtgcctctatttctagaaggcttttaaagtttcctggcttagttatgtccaaaggcagcaggaagtctcatcagtagagggcagaattttcaagtgctgccattcttatcccaggaggcatttccagtggttgagcacaaggcctgtttgtagtttgcttttgctcttgcattttgtggaagggaaggaactgagagagcttagagggttcattaaaaccacccctcactctcttagtcgtagtcagatggagtattcataacagtaacctccaattaccactatgtgttgggaaaaattagaattcggtctacttacaatcctgccaactaggattttactttgatatttcagtataacagtgaatctggattgatgcctgattaaaataaaatccctgattattactttctggattacgaactaaaatccctgtaaaatcaatggatgtgactcattgttaagagtcatgcagacttttacatattaggtaagaattctaaaaattatttgagggttctattctctagcaccaggtactaatgctccctactcaaaaaaaatcatgtgcatggattaatcaagtctaacagtgctcagatttaatggtttaacattgattttcttttctttgtcaaacttatatatgcaaatatttttatagtagtcagatgttatttttgaataaggatcaccctcatttttacccatgtgcttatctttaaaaccaacattgtaaagtagcacgcagacatatgtttcttttatcttcatggattatttttaccttaaaaataaattatcatttttttttttgaatttgggttttattctccagatactctgtgtacatgtgggtaagtatgtgggagtatgtgtgtttgtgtgtaagaggggataattaattgtctctcaactctatctcatactttaatatcaaataaaaaatgaaatgtataaagggtcactttgtaggattaggcatcctccttctacctacttaaaccaggggtttgggattcagaattctccatataaccaagaccgaaagtcactggaagactttaaaattagtattttaaccaccacacccagagtcaggtatggaaataaacctatagcatggattctttctatgcataatctcaaaatttaactacccaaataagtaagtttttaaaaactaatttaaaatttgccattgaggaaaatatcacctccatccttaattgtgactcctcatttcagctaaaaccttttctaatactttaaaaaaacaaaatgaaaaacaaactcctagataaagtcataaacactgaaatcagagatgtgattcttgttaaatgttagtttctctttctgaggttacactctgtgcatttgaaactttgacgttaacatcttccgaatgtttagatttgctcaagggttcagattctctggtcttctgccttgcattttcctccttcctttcctttgcaagcaatctatagttgatagcattgccaatgagcagccacacgcttgctgctaccacaatagccccacaggacatgtacatgtatttatattctccagttaaatccaccaatttacctgcaagaggagggccaagaagaactgggccacactccacaattgtgacaagtccgacggcactggaaaatcttggtgcacccacgaggtccatgagagtttcaaagagaacactgctaacactcccaaatccaaggccaaaaaatacagcatataataccaggcttgtgtagtcctgtgccagtgggcacaagaggtgacacactccattgaacatgattgcaaaactgaagaagtactgaattcgaggtcgaatatatttggagtttgcaattaatcctacagaaggcctagcaaacatatcaacgaaagccataacagatagcagaaaagctgccgagtactcatcaattccttggtctttagcatatggagccaagaatataatgggggcaaaaaaacctaggaacataatgacatttccagacagatatatcagaaatcctctatgcttaaaaagggagaaatctaaatacttattaactttttcccaagttgatttcttcgttttgattttctttgggcttgaatcatcttctgttttgccagtcttatttttagacttagaagtggtttgattgggtccaaggggtctcatgagggaaccagccacacaggcattcaaaagtagacttcccaaaatcaggaagcttcctttccagccaaaagtattaaaaaggtactgattgaaaggagccaatgaacttaagaaaacaggacttcctgccatggccaatccatttgccatgggtcgcttcctatagaagtatttgccaattatggttaaggcgggttgcaggttgaaggctaaacctaaacctgtaatgaatcccatagtgaggtacagctgtaccacgctgctactaaaggaggccaacaccattccaagacagcataataagcctcctgctatcaccaccggccggctgccgtatttattcaccaaaacactacttacaggacctaggcatgatcctgattgagtaaagctgcactgaatcctcaaggatgtgaagatcaaaaagctttcaaatattctacctcctgcgtacataacagccagcataatggatgaaatccatgctatttcactgtaggtagtgtggaatatttgctgaatttctttgaagaatacggtgacagctttggggaatgcataggaaaatccaatggagataaaagctgctccaaccacaatccaaccccatcctccatctggaggtggatgcacaggtggggcacttggcattggtggcatttctgctcctctagtggaaattcaagtaacctgaatagagagagaacctgcgtttgacacttttctccaggctcagggctaagaagagaggcaactgatcattaacttttagccacaagcaa

SEQ ID NO: 17827 - RNA, 11284 nt, Homo sapiens
  source 1..11284: mol_type = other RNA
tcgaggagctcacagtctagtaagaaagagatgaatttgaaaatatatttgaaactgtaggcaaaataagtaccctcacagagaaattcaacatttggtttcaaatttgttatgcagtgaaaattagaaactacaaccaagatttttttaaaacattatgttcatataacgctgtagtatacctgaaaggcaagaacttaaacaagtgtgctgaaaaacaaattaggaatatttgaacaaaatatactttaaaaatgatcaacaacgtaaaatattcctgatttaaataaatctaagttattttatttagtttaagcaaaatatgtatccatatgaaaatgccagttctttcatttttggttaattcctttacacatattatttgctaagttcagaaatgctatatatacaaaaatttcaaaaataaataagtatcccaagatcacataacaatactttaagtacattcatgtgtaagaaggcaaaaaaagaaggttctatcttatattttaaaactttgacaggtattttaaatgtattattttatactttattttctttaaaaatgaaataatacagccatgatttaagtcatgtaaaaacaactgtttggatcatttaggtgtcaagcaaaactatcctctttatttcactatcatagtaaccatagttgatagaccatgtggcaatatgatcatttgttcagtggtcattaagatatctatagaataaacaagacaactacattttatttttttcacttaaaaatcacaaaaatacagcctaaaatataatttatattttaaaaataattctaaacattaacccctaaatctaatcccttaaaaaattcttgcaaaagttagctggatgtggctgttgccaaggaatgtcttttattagcaacaagtgactatctataacttttattccaacaatcttattttaaatatttgtttcaatttaatgctgggattagaaaaacatatttgttcaaagtatgtaagtagtaagtaaaacaatttcaaaaatctatcaaaaaaggagaattattcattctaggaaataattaacatactggtttaaaatatctgggagaagaacttttacataaaaagcttcaaatttagtcagttgtagcaagcacttgaaaagaccctgctctttcatctgcaatatcaggaattactatatctgactcatatttgattaagttacaatctcatttttgttgtcactacaaagaaggatccttatattagtaaatgcactcactgcaactactgaggcctgcctcctgtcagaatgacaatgcagtcttagcatacgggtgtcggtttggctgaatctaaccaaacacatcacgtactacagatgtttttagggcccacccaattcataaaagattttactgcgatacatgagtttacccaaatttttattaaaatgtgtttttagggtaaatatcttgatgaactaggcaaacaaatactgaatgcagattactgtttttacagttttaccgggaaaactcctaatagcaacccctcttccccttcaccacagatctttaatttaggtgtgatttttgtttgttctctacatgggaataaaggagaaagtttagaaagactgtatctagctagataagatgcagaggtagatggaatctctaacataaaagaagctctaattacactgttgccagacagctgttatggattttagtattgtttattaggtgaagaaaacattcataaaataagaaatttttgagatagaacttactctaataatttcattaacatatgttcaggttcttagatcaagaaatactgtagaggtgttctcctcaagactatgctatggcaataatttcttgcatacaatttaataatttaaacttgaactgtgtgttctgtgctctggcgttctacttcagaaaaaaatgaacactgcttctaaaataaaaaggaacataaaataaaaaaggaattaatgagatattgacatgttttctattaatacaatattgatgttttaaatgattttgatattgctataacaacatatattgtgcaaaataattaatctcactaaatattatttctgatttgccacgaattatctgccgtggcaatcaggaaatagtcttcaaagtaagtttgcaaacatgattttgcaaaccatgattggaaaaatatattcatttgggctataaactatcaagtagggttgttatatatatttctaggaaaatattttatttactctacaaagatcatcattatgaccttacggcttctgtagtgcaatggagaaaaaagtgtgttagaagttaaaagacctgaattctatctccaaccctgcatttattcagagtattggtataggtttaggcaaaatccttaatccagtctagttttatatggtaaaaatgtggatacctatcaaaactgagggttgagaggatgaaatgaattcattaaacatatcttctgagacataaatatatcaaaacaaatcaaaatacaattagatctaatgtttagaaataaatattttaattcatatttgctatttcactaaatctagaaatactaatgctttagttaaatatagaaagttgatgatagaaaaataaaatccatcgtaccattgaaaagcttgtcagaaatatgtactcttgagattcggaggatgagaaaaaaaatgtgtactctaacgaggaagctatataaactgagtctaactcaaaacatttattttagatgcatataagaattaaagtcttagtcaaaagaatgttttaaaatttcatcctaaatttatgtgagataaaatgccattcttttgtttttctgaacagaggagcttttatcaacttattctattttatttttatttttattattttattttattttatttattattattatactttaagttttagggtacatgtgcacaatgtgcaggttagttacatatgtatacatgtgccatgctggtgcgctgcacccactaactcgtcacctagcattaggtatatctcccaatgctatccctcccccctcccccgaccccaccacagtccccagagtgtgatgttccccttcctgtgtccatgtgttctcattgttcagttcccacctatgagtgagaatatgcggtgtttggttttttgttcttgcgatagtttactgagaatgatgatttctaatttcatccatgtccctacacgaacttattctattttaatagaatgttcagtatcagtgttttcacactgagattctctagcttattttgccatatttaaattaaaaagaaacaaaaaatcctgtttgatcatgtgaaaaatatttactgaaatgtgaataaatttatgatcattaattgcctactgaaatattcctgaatattgctcaccttattaacaagtatatatggagactgaaaaacatgtagatcatgcaaacaagtgtaactaactataccaaagaaacaaaagtccatactaaatatgtccataattaaataaaaaatgctaaacaagttttacctagatattataaaaacatagaaaggaaaacatttaggagatgatgaagaagcaggagattgggatgggagatgtaatttgatctaaattcccatatgcttctgtaaaatcaaaaattcattttgcaatattaattttgctcttaaggtagagacttttaaaatgaccattctcaatactacagcaattcttccctgatttgcacataaatgaattaaagtgaagaaaaagcagtagaggagagaagactaaaataaaccagattgtagcaccctgtaaagagctaaaatctccagtgtacaaacaactgataggaaagaagagaaaatcagaactataaaaaagtgacataagctcagaaaattactcatttttaattgtatcaacaaagataatttgtaattttgatcatgcaagcattataattactgataattgggcctttcagcttttaagtgccttctcaaacatgagttctgcatatggttgtgcagaaatcaaaatcttaaagagagatgagtaaagtcaagtttgtaatattaatcttatattctcaatatagatgctaattagtgctctgaatggttgtggttagaaatcttgttggtatgatgtatcagtgatgtcactgcattgatggagacagaataatacataatggtgcaatgtggtgatggtaagctttgttactcaatattgtcaggcactttaagaaaatcagaaacattcaggatagtgccaaagaagatcagtttttcaagactctaaaatcatattcaattatatgtgtatgtaattataaatatgtgcatcatggctgactttgagaagaatgcagcgccttgcaagtgcactatttgaatagagctaaggagaactatagtctaaggactgcaaaagtctagatggagaagacaaaagcaatgacacttgttttctctacagaacaaatagacaaagaggtgaatgacaacaaagatgttcagagaaacttgaaaaataagctacggtgtagggtaagttgtattaaatgatgaaaattaatatgtaactgtatgggtaaaccaaatcatttgtatcttataatcttttttttggtagctacggataatattataaatggaataatcactaaaattctaaatataatgttttctagtaagaacattttattttttttttaatagagacagattctcactctattgcctaggctggactgcaagtggggccattatagctcactgaagcctcaacttcctgggctcaaatgaccctctcgtctcagcctcccgagtagctgggactacaggtgcacatcaccacatccaggtaattattttactttttgaatcatgatatgtagcaaccaatctgggaattatttattcataaaagataacattttcctgctaactccaacctcagaaaaaatgtattatgcctgactcaaatatgtcattatttttatgagaaaaagagtcatattgaagtaattatgtctatatgtaataattatcattatttgagataatttgcattggggagaaaagcaggcaatcagaaattacatattcaaggctgggcgcagtggctcacgcctgtaatcccagcactttgggaggcagaggcgagtgaatcacctgaggtcagagttcaagaccagcctgaccaacaaggagaaaccccatctctactaaaacaaaacaaaacaaaacaaaacaaaaaaagccacaaaattagccgggcatggtggcacatgcctgtaattccagttactcgggaggctgaggcaggagaattgcttgaacctgggaggcagaggttgtagtaagccgagattgtgccactgcacgccagcctgggcgacaagaacgagactcagtctcaaaaaaaaaaaaaaagaaagaaagaaagaaattacatattcaggttctagcaaatgcagttctctaataaacactaaataaatcataatacaagttacagttaaacctaattgttttactatataggatgtatcttttttgtacctatattttatcttcctttgcttctctggcctctattgggaggcagcacggtagtgaacacctcggggatctttctggttacgtaaacctgagttttaattttggttcatactaccttttaactttgggtagtctgctgagcttgttttttgttttcactcatctgtcatatcaagctagtaataattctgccatggttttggttttcatattgaaaggcattacataagcaaaatgcataacatataaatattagttccctttccactatgcatccaatctccctattaaattaagcctaaaaataataatttttgttttattaaaagccttccacattctacatatgaaagggattttttaaaggtgttttagataaaaaatgtttcaaccaactgaccaagaatatctcttcatatttatgtcatctacataaaaacttacatttatatcatatatcttttagtcttcttttctatattcttgattgtcatgttgtacagccagaaaagaatgagtataaattatctagattttttaaagtgcacattcaaacatagaaaatctaattattttacttgtttcttagtattaggctgaggccaatgagtccatgagctaaagggttgaaacttggcaccaaaaaagtgattgtttatgagtcctgtagatttatactgagaaaacatcatgtcttccaatgtgaaatacactaaaacctgattttttgtctcttaaggtgtgctaggtgaatgcaaaaaggatcaggaaagggggtgaggataggtcaggaaaagtgcaaacacaatgttctattcataaattagtgatggcatatttaaggttaagtagtaaaaaatatggggggctcagttaacacgaatgaaaaaatagttaaagtagccatgaattatctggataccttgatttaatgacaccctttcttctgtacaatttcataatgtgggaatagagattagtggggattgtagtggtataccctgactttgcttcatgatatctcaaatgtttaaaacctattattccctagagaaagaaatatgttcatactaattgttgcagaggcagaagccaaatatatctcctcctccatttatgtgactatatagtaatgaaaatcctaggttgatacacttttctcaatcttggaaagattctgctaaagcagcaaatcttctaacaagttcaagagggtggggagagtgaacaagtagaataatttatattaccctggaacaattctgaatcctgtaggtatttatgtcactgtttcaattgtgttctggtttaactgtcaatatttatgcatagcagttaacgtgtgtgcatatttgtaactgtgcagtgctactgccaggtgtgactgtacaaatcatgtgctttgaatgtgcaagttttactttcttttctaacaatttaatacagtgttagaaataaataacgaatgaagacaaccaaagagcagccagacaaatgtgaactggttttgacgtgacgagaaactcatcagtaagtaaataaacctcctccctggagaaggccactgaaatgcacccaggaggatgtctctactagaaggtaataaaaaatatatataatgtagtctttgacctaaaacctcatgattattactttgccatttatttccccctggtatctgatgttcatattagtttaatgtgccttttcagagaattcaagacactttttggaaagtagaatttttttttgaaaatttatgattggagaggtactacacaatttagaggttacatttcttgacaaatctgagttgaataaaaaagaactaaaaatataaacatagctaattcaagaatcaagatcgggtgaaactaaattaaaaacagccataaagtcccacattttccctaatttatttacctatgatattggcacatcttgttttacttaacatttgaaaaatacaaatatctcttcatatgcaaaagagcaaatgttaaatgaaaaactgaattttatatagcttcctaaatatgagccacatgcttaagcagtgaattaactttatgaatcaaatgtttaatgttaactattacaaaagcctggtatccaggtgcaatctcaccagaaaaaaatagcacctgcctttattacaataaaaaaaatggctaattccctttgacatcttaagagtgacactactttgtcaagcactaaatactttttaaattaatcatgttaaacttcagatttatagatataaatattgtatttataactttagtcataatgtacaatttctttcttgtttaaaagtactttctcactcaaaatggtatttatagtttaaaaagaatatgcctctgtattcaggagtgattcaaattcccagatgttttcacatagttatgaaaatgggaaagtgctgaattaaactgggctgcaatatttcaagttttttgctatcaggttataaactatacctacgattgcaagtcatacagtgcctctatttctagaaggcttttaaagtttcctggcttagttatgtccaaaggcagcaggaagtctcatcagtagagggcagaattttcaagtgctgccattcttatcccaggaggcatttccagtggttgagcacaaggcctgtttgtagtttgcttttgctcttgcattttgtggaagggaaggaactgagagagcttagagggttcattaaaaccacccctcactctcttagtcgtagtcagatggagtattcataacagtaacctccaattaccactatgtgttgggaaaaattagaattcggtctacttacaatcctgccaactaggattttactttgatatttcagtataacagtgaatctggattgatgcctgattaaaataaaatccctgattattactttctggattacgaactaaaatccctgtaaaatcaatggatgtgactcattgttaagagtcatgcagacttttacatattaggtaagaattctaaaaattatttgagggttctattctctagcaccaggtactaatgctccctactcaaaaaaaatcatgtgcatggattaatcaagtctaacagtgctcagatttaatggtttaacattgattttcttttctttgtcaaacttatatatgcaaatatttttatagtagtcagatgttatttttgaataaggatcaccctcatttttacccatgtgcttatctttaaaaccaacattgtaaagtagcacgcagacatatgtttcttttatcttcatggattatttttaccttaaaaataaattatcatttttttttttgaatttgggttttattctccagatactctgtgtacatgtgggtaagtatgtgggagtatgtgtgtttgtgtgtaagaggggataattaattgtctctcaactctatctcatactttaatatcaaataaaaaatgaaatgtataaagggtcactttgtaggattaggcatcctccttctacctacttaaaccaggggtttgggattcagaattctccatataaccaagaccgaaagtcactggaagactttaaaattagtattttaaccaccacacccagagtcaggtatggaaataaacctatagcatggattctttctatgcataatctcaaaatttaactacccaaataagtaagtttttaaaaactaatttaaaatttgccattgaggaaaatatcacctccatccttaattgtgactcctcatttcagctaaaaccttttctaatactttaaaaaaacaaaatgaaaaacaaactcctagataaagtcataaacactgaaatcagagatgtgattcttgttaaatgttagtttctctttctgaggttacactctgtgcatttgaaactttgacgttaacatcttccgaatgtttagatttgctcaagggttcagattctctggtcttctgccttgcattttcctccttcctttcctttgcaagcaatctatagttgatagcattgccaatgagcagccacacgcttgctgctaccacaatagccccacaggacatgtacatgtatttatattctccagttaaatccaccaatttacctgcaagaggagggccaagaagaactgggccacactccacaattgtgacaagtccgacggcactggaaaatcttggtgcacccacgaggtccatgagagtttcaaagagaacactgctaacactcccaaatccaaggccaaaaaatacagcatataataccaggcttgtgtagtcctgtgccagtgggcacaagaggtgacacactccattgaacatgattgcaaaactgaagaagtactgaattcgaggtcgaatatatttggagtttgcaattaatcctacagaaggcctagcaaacatatcaacgaaagccataacagatagcagaaaagctgccgagtactcatcaattccttggtctttagcatatggagccaagaatataatgggggcaaaaaaacctaggaacataatgacatttccagacagatatatcagaaatcctctatgcttaaaaagggagaaatctaaatacttattaactttttcccaagttgatttcttcgttttgattttctttgggcttgaatcatcttctgttttgccagtcttatttttagacttagaagtggtttgattgggtccaaggggtctcatgagggaaccagccacacaggcattcaaaagtagacttcccaaaatcaggaagcttcctttccagccaaaagtattaaaaaggtactgattgaaaggagccaatgaacttaagaaaacaggacttcctgccatggccaatccatttgccatgggtcgcttcctatagaagtatttgccaattatggttaaggcgggttgcaggttgaaggctaaacctaaacctgtaatgaatcccatagtgaggtacagctgtaccacgctgctactaaaggaggccaacaccattccaagacagcataataagcctcctgctatcaccaccggccggctgccgtatttattcaccaaaacactacttacaggacctaggcatgatcctgattgagtaaagctgcactgaatcctcaaggatgtgaagatcaaaaagctttcaaatattctacctcctgcgtacataacagccagcataatggatgaaatccatgctatttcactgtaggtagtgtggaatatttgctgaatttctttgaagaatacggtgacagctttggggaatgcataggaaaatccaatggagataaaagctgctccaaccacaatccaaccccatcctccatctggaggtggatgcacaggtggggcacttggcattggtggcatttctgctcctctagtggaaattcaagtaacctggcgacaggtgtttagaaacatggtcttccatttcaccaagacataagtttccctgatctatggactcctctccccacctgaggcagaagtttccttgtgaaccattgctctttttagaatcctgaacatacttagttccatctatctctttgtcactcaacactttgtcagctagtctcaggattctatgaccccttcccctagctcacttgagtaatcataatatgggaaaactaatctaaatgccaactctgagaagcggttgcatatattactgtcattcacttgataaa

SEQ ID NO: 17828 - RNA, 11197 nt, Homo sapiens
  source 1..11197: mol_type = other RNA
tcgaggagctcacagtctagtaagaaagagatgaatttgaaaatatatttgaaactgtaggcaaaataagtaccctcacagagaaattcaacatttggtttcaaatttgttatgcagtgaaaattagaaactacaaccaagatttttttaaaacattatgttcatataacgctgtagtatacctgaaaggcaagaacttaaacaagtgtgctgaaaaacaaattaggaatatttgaacaaaatatactttaaaaatgatcaacaacgtaaaatattcctgatttaaataaatctaagttattttatttagtttaagcaaaatatgtatccatatgaaaatgccagttctttcatttttggttaattcctttacacatattatttgctaagttcagaaatgctatatatacaaaaatttcaaaaataaataagtatcccaagatcacataacaatactttaagtacattcatgtgtaagaaggcaaaaaaagaaggttctatcttatattttaaaactttgacaggtattttaaatgtattattttatactttattttctttaaaaatgaaataatacagccatgatttaagtcatgtaaaaacaactgtttggatcatttaggtgtcaagcaaaactatcctctttatttcactatcatagtaaccatagttgatagaccatgtggcaatatgatcatttgttcagtggtcattaagatatctatagaataaacaagacaactacattttatttttttcacttaaaaatcacaaaaatacagcctaaaatataatttatattttaaaaataattctaaacattaacccctaaatctaatcccttaaaaaattcttgcaaaagttagctggatgtggctgttgccaaggaatgtcttttattagcaacaagtgactatctataacttttattccaacaatcttattttaaatatttgtttcaatttaatgctgggattagaaaaacatatttgttcaaagtatgtaagtagtaagtaaaacaatttcaaaaatctatcaaaaaaggagaattattcattctaggaaataattaacatactggtttaaaatatctgggagaagaacttttacataaaaagcttcaaatttagtcagttgtagcaagcacttgaaaagaccctgctctttcatctgcaatatcaggaattactatatctgactcatatttgattaagttacaatctcatttttgttgtcactacaaagaaggatccttatattagtaaatgcactcactgcaactactgaggcctgcctcctgtcagaatgacaatgcagtcttagcatacgggtgtcggtttggctgaatctaaccaaacacatcacgtactacagatgtttttagggcccacccaattcataaaagattttactgcgatacatgagtttacccaaatttttattaaaatgtgtttttagggtaaatatcttgatgaactaggcaaacaaatactgaatgcagattactgtttttacagttttaccgggaaaactcctaatagcaacccctcttccccttcaccacagatctttaatttaggtgtgatttttgtttgttctctacatgggaataaaggagaaagtttagaaagactgtatctagctagataagatgcagaggtagatggaatctctaacataaaagaagctctaattacactgttgccagacagctgttatggattttagtattgtttattaggtgaagaaaacattcataaaataagaaatttttgagatagaacttactctaataatttcattaacatatgttcaggttcttagatcaagaaatactgtagaggtgttctcctcaagactatgctatggcaataatttcttgcatacaatttaataatttaaacttgaactgtgtgttctgtgctctggcgttctacttcagaaaaaaatgaacactgcttctaaaataaaaaggaacataaaataaaaaaggaattaatgagatattgacatgttttctattaatacaatattgatgttttaaatgattttgatattgctataacaacatatattgtgcaaaataattaatctcactaaatattatttctgatttgccacgaattatctgccgtggcaatcaggaaatagtcttcaaagtaagtttgcaaacatgattttgcaaaccatgattggaaaaatatattcatttgggctataaactatcaagtagggttgttatatatatttctaggaaaatattttatttactctacaaagatcatcattatgaccttacggcttctgtagtgcaatggagaaaaaagtgtgttagaagttaaaagacctgaattctatctccaaccctgcatttattcagagtattggtataggtttaggcaaaatccttaatccagtctagttttatatggtaaaaatgtggatacctatcaaaactgagggttgagaggatgaaatgaattcattaaacatatcttctgagacataaatatatcaaaacaaatcaaaatacaattagatctaatgtttagaaataaatattttaattcatatttgctatttcactaaatctagaaatactaatgctttagttaaatatagaaagttgatgatagaaaaataaaatccatcgtaccattgaaaagcttgtcagaaatatgtactcttgagattcggaggatgagaaaaaaaatgtgtactctaacgaggaagctatataaactgagtctaactcaaaacatttattttagatgcatataagaattaaagtcttagtcaaaagaatgttttaaaatttcatcctaaatttatgtgagataaaatgccattcttttgtttttctgaacagaggagcttttatcaacttattctattttatttttatttttattattttattttattttatttattattattatactttaagttttagggtacatgtgcacaatgtgcaggttagttacatatgtatacatgtgccatgctggtgcgctgcacccactaactcgtcacctagcattaggtatatctcccaatgctatccctcccccctcccccgaccccaccacagtccccagagtgtgatgttccccttcctgtgtccatgtgttctcattgttcagttcccacctatgagtgagaatatgcggtgtttggttttttgttcttgcgatagtttactgagaatgatgatttctaatttcatccatgtccctacacgaacttattctattttaatagaatgttcagtatcagtgttttcacactgagattctctagcttattttgccatatttaaattaaaaagaaacaaaaaatcctgtttgatcatgtgaaaaatatttactgaaatgtgaataaatttatgatcattaattgcctactgaaatattcctgaatattgctcaccttattaacaagtatatatggagactgaaaaacatgtagatcatgcaaacaagtgtaactaactataccaaagaaacaaaagtccatactaaatatgtccataattaaataaaaaatgctaaacaagttttacctagatattataaaaacatagaaaggaaaacatttaggagatgatgaagaagcaggagattgggatgggagatgtaatttgatctaaattcccatatgcttctgtaaaatcaaaaattcattttgcaatattaattttgctcttaaggtagagacttttaaaatgaccattctcaatactacagcaattcttccctgatttgcacataaatgaattaaagtgaagaaaaagcagtagaggagagaagactaaaataaaccagattgtagcaccctgtaaagagctaaaatctccagtgtacaaacaactgataggaaagaagagaaaatcagaactataaaaaagtgacataagctcagaaaattactcatttttaattgtatcaacaaagataatttgtaattttgatcatgcaagcattataattactgataattgggcctttcagcttttaagtgccttctcaaacatgagttctgcatatggttgtgcagaaatcaaaatcttaaagagagatgagtaaagtcaagtttgtaatattaatcttatattctcaatatagatgctaattagtgctctgaatggttgtggttagaaatcttgttggtatgatgtatcagtgatgtcactgcattgatggagacagaataatacataatggtgcaatgtggtgatggtaagctttgttactcaatattgtcaggcactttaagaaaatcagaaacattcaggatagtgccaaagaagatcagtttttcaagactctaaaatcatattcaattatatgtgtatgtaattataaatatgtgcatcatggctgactttgagaagaatgcagcgccttgcaagtgcactatttgaatagagctaaggagaactatagtctaaggactgcaaaagtctagatggagaagacaaaagcaatgacacttgttttctctacagaacaaatagacaaagaggtgaatgacaacaaagatgttcagagaaacttgaaaaataagctacggtgtagggtaagttgtattaaatgatgaaaattaatatgtaactgtatgggtaaaccaaatcatttgtatcttataatcttttttttggtagctacggataatattataaatggaataatcactaaaattctaaatataatgttttctagtaagaacattttattttttttttaatagagacagattctcactctattgcctaggctggactgcaagtggggccattatagctcactgaagcctcaacttcctgggctcaaatgaccctctcgtctcagcctcccgagtagctgggactacaggtgcacatcaccacatccaggtaattattttactttttgaatcatgatatgtagcaaccaatctgggaattatttattcataaaagataacattttcctgctaactccaacctcagaaaaaatgtattatgcctgactcaaatatgtcattatttttatgagaaaaagagtcatattgaagtaattatgtctatatgtaataattatcattatttgagataatttgcattggggagaaaagcaggcaatcagaaattacatattcaaggctgggcgcagtggctcacgcctgtaatcccagcactttgggaggcagaggcgagtgaatcacctgaggtcagagttcaagaccagcctgaccaacaaggagaaaccccatctctactaaaacaaaacaaaacaaaacaaaacaaaaaaagccacaaaattagccgggcatggtggcacatgcctgtaattccagttactcgggaggctgaggcaggagaattgcttgaacctgggaggcagaggttgtagtaagccgagattgtgccactgcacgccagcctgggcgacaagaacgagactcagtctcaaaaaaaaaaaaaaagaaagaaagaaagaaattacatattcaggttctagcaaatgcagttctctaataaacactaaataaatcataatacaagttacagttaaacctaattgttttactatataggatgtatcttttttgtacctatattttatcttcctttgcttctctggcctctattgggaggcagcacggtagtgaacacctcggggatctttctggttacgtaaacctgagttttaattttggttcatactaccttttaactttgggtagtctgctgagcttgttttttgttttcactcatctgtcatatcaagctagtaataattctgccatggttttggttttcatattgaaaggcattacataagcaaaatgcataacatataaatattagttccctttccactatgcatccaatctccctattaaattaagcctaaaaataataatttttgttttattaaaagccttccacattctacatatgaaagggattttttaaaggtgttttagataaaaaatgtttcaaccaactgaccaagaatatctcttcatatttatgtcatctacataaaaacttacatttatatcatatatcttttagtcttcttttctatattcttgattgtcatgttgtacagccagaaaagaatgagtataaattatctagattttttaaagtgcacattcaaacatagaaaatctaattattttacttgtttcttagtattaggctgaggccaatgagtccatgagctaaagggttgaaacttggcaccaaaaaagtgattgtttatgagtcctgtagatttatactgagaaaacatcatgtcttccaatgtgaaatacactaaaacctgattttttgtctcttaaggtgtgctaggtgaatgcaaaaaggatcaggaaagggggtgaggataggtcaggaaaagtgcaaacacaatgttctattcataaattagtgatggcatatttaaggttaagtagtaaaaaatatggggggctcagttaacacgaatgaaaaaatagttaaagtagccatgaattatctggataccttgatttaatgacaccctttcttctgtacaatttcataatgtgggaatagagattagtggggattgtagtggtataccctgactttgcttcatgatatctcaaatgtttaaaacctattattccctagagaaagaaatatgttcatactaattgttgcagaggcagaagccaaatatatctcctcctccatttatgtgactatatagtaatgaaaatcctaggttgatacacttttctcaatcttggaaagattctgctaaagcagcaaatcttctaacaagttcaagagggtggggagagtgaacaagtagaataatttatattaccctggaacaattctgaatcctgtaggtatttatgtcactgtttcaattgtgttctggtttaactgtcaatatttatgcatagcagttaacgtgtgtgcatatttgtaactgtgcagtgctactgccaggtgtgactgtacaaatcatgtgctttgaatgtgcaagttttactttcttttctaacaatttaatacagtgttagaaataaataacgaatgaagacaaccaaagagcagccagacaaatgtgaactggttttgacgtgacgagaaactcatcagtaagtaaataaacctcctccctggagaaggccactgaaatgcacccaggaggatgtctctactagaaggtaataaaaaatatatataatgtagtctttgacctaaaacctcatgattattactttgccatttatttccccctggtatctgatgttcatattagtttaatgtgccttttcagagaattcaagacactttttggaaagtagaatttttttttgaaaatttatgattggagaggtactacacaatttagaggttacatttcttgacaaatctgagttgaataaaaaagaactaaaaatataaacatagctaattcaagaatcaagatcgggtgaaactaaattaaaaacagccataaagtcccacattttccctaatttatttacctatgatattggcacatcttgttttacttaacatttgaaaaatacaaatatctcttcatatgcaaaagagcaaatgttaaatgaaaaactgaattttatatagcttcctaaatatgagccacatgcttaagcagtgaattaactttatgaatcaaatgtttaatgttaactattacaaaagcctggtatccaggtgcaatctcaccagaaaaaaatagcacctgcctttattacaataaaaaaaatggctaattccctttgacatcttaagagtgacactactttgtcaagcactaaatactttttaaattaatcatgttaaacttcagatttatagatataaatattgtatttataactttagtcataatgtacaatttctttcttgtttaaaagtactttctcactcaaaatggtatttatagtttaaaaagaatatgcctctgtattcaggagtgattcaaattcccagatgttttcacatagttatgaaaatgggaaagtgctgaattaaactgggctgcaatatttcaagttttttgctatcaggttataaactatacctacgattgcaagtcatacagtgcctctatttctagaaggcttttaaagtttcctggcttagttatgtccaaaggcagcaggaagtctcatcagtagagggcagaattttcaagtgctgccattcttatcccaggaggcatttccagtggttgagcacaaggcctgtttgtagtttgcttttgctcttgcattttgtggaagggaaggaactgagagagcttagagggttcattaaaaccacccctcactctcttagtcgtagtcagatggagtattcataacagtaacctccaattaccactatgtgttgggaaaaattagaattcggtctacttacaatcctgccaactaggattttactttgatatttcagtataacagtgaatctggattgatgcctgattaaaataaaatccctgattattactttctggattacgaactaaaatccctgtaaaatcaatggatgtgactcattgttaagagtcatgcagacttttacatattaggtaagaattctaaaaattatttgagggttctattctctagcaccaggtactaatgctccctactcaaaaaaaatcatgtgcatggattaatcaagtctaacagtgctcagatttaatggtttaacattgattttcttttctttgtcaaacttatatatgcaaatatttttatagtagtcagatgttatttttgaataaggatcaccctcatttttacccatgtgcttatctttaaaaccaacattgtaaagtagcacgcagacatatgtttcttttatcttcatggattatttttaccttaaaaataaattatcatttttttttttgaatttgggttttattctccagatactctgtgtacatgtgggtaagtatgtgggagtatgtgtgtttgtgtgtaagaggggataattaattgtctctcaactctatctcatactttaatatcaaataaaaaatgaaatgtataaagggtcactttgtaggattaggcatcctccttctacctacttaaaccaggggtttgggattcagaattctccatataaccaagaccgaaagtcactggaagactttaaaattagtattttaaccaccacacccagagtcaggtatggaaataaacctatagcatggattctttctatgcataatctcaaaatttaactacccaaataagtaagtttttaaaaactaatttaaaatttgccattgaggaaaatatcacctccatccttaattgtgactcctcatttcagctaaaaccttttctaatactttaaaaaaacaaaatgaaaaacaaactcctagataaagtcataaacactgaaatcagagatgtgattcttgttaaatgttagtttctctttctgaggttacactctgtgcatttgaaactttgacgttaacatcttccgaatgtttagatttgctcaagggttcagattctctggtcttctgccttgcattttcctccttcctttcctttgcaagcaatctatagttgatagcattgccaatgagcagccacacgcttgctgctaccacaatagccccacaggacatgtacatgtatttatattctccagttaaatccaccaatttacctgcaagaggagggccaagaagaactgggccacactccacaattgtgacaagtccgacggcactggaaaatcttggtgcacccacgaggtccatgagagtttcaaagagaacactgctaacactcccaaatccaaggccaaaaaatacagcatataataccaggcttgtgtagtcctgtgccagtgggcacaagaggtgacacactccattgaacatgattgcaaaactgaagaagtactgaattcgaggtcgaatatatttggagtttgcaattaatcctacagaaggcctagcaaacatatcaacgaaagccataacagatagcagaaaagctgccgagtactcatcaattccttggtctttagcatatggagccaagaatataatgggggcaaaaaaacctaggaacataatgacatttccagacagatatatcagaaatcctctatgcttaaaaagggagaaatctaaatacttattaactttttcccaagttgatttcttcgttttgattttctttgggcttgaatcatcttctgttttgccagtcttatttttagacttagaagtggtttgattgggtccaaggggtctcatgagggaaccagccacacaggcattcaaaagtagacttcccaaaatcaggaagcttcctttccagccaaaagtattaaaaaggtactgattgaaaggagccaatgaacttaagaaaacaggacttcctgccatggccaatccatttgccatgggtcgcttcctatagaagtatttgccaattatggttaaggcgggttgcaggttgaaggctaaacctaaacctgtaatgaatcccatagtgaggtacagctgtaccacgctgctactaaaggaggccaacaccattccaagacagcataataagcctcctgctatcaccaccggccggctgccgtatttattcaccaaaacactacttacaggacctcctgcgtacataacagccagcataatggatgaaatccatgctatttcactgtaggtagtgtggaatatttgctgaatttctttgaagaatacggtgacagctttggggaatgcataggaaaatccaatggagataaaagctgctccaaccacaatccaaccccatcctccatctggaggtggatgcacaggtggggcacttggcattggtggcatttctgctcctagagtaactctgttggcaccaagagtcccagagtctttggttccccagatcaccttgtttcaggtttcacaggaaagtatcacatcttaagattgactctttatctggtctctggcgcagggtgggcgctgcagccctccgttcccagcaaaccgcagccgattcgcctcgctgtcaacgggtgaatggaattatttatttatttatggcccctgacgtgtcctcgcccgccacagccagcggagaaggaggcggtggcgggaaggggaggcgcggctgctgaacgcccttgtgggtgcggaggagc

SEQ ID NO: 17829 - RNA, 11217 nt, Homo sapiens
  source 1..11217: mol_type = other RNA
tcgaggagctcacagtctagtaagaaagagatgaatttgaaaatatatttgaaactgtaggcaaaataagtaccctcacagagaaattcaacatttggtttcaaatttgttatgcagtgaaaattagaaactacaaccaagatttttttaaaacattatgttcatataacgctgtagtatacctgaaaggcaagaacttaaacaagtgtgctgaaaaacaaattaggaatatttgaacaaaatatactttaaaaatgatcaacaacgtaaaatattcctgatttaaataaatctaagttattttatttagtttaagcaaaatatgtatccatatgaaaatgccagttctttcatttttggttaattcctttacacatattatttgctaagttcagaaatgctatatatacaaaaatttcaaaaataaataagtatcccaagatcacataacaatactttaagtacattcatgtgtaagaaggcaaaaaaagaaggttctatcttatattttaaaactttgacaggtattttaaatgtattattttatactttattttctttaaaaatgaaataatacagccatgatttaagtcatgtaaaaacaactgtttggatcatttaggtgtcaagcaaaactatcctctttatttcactatcatagtaaccatagttgatagaccatgtggcaatatgatcatttgttcagtggtcattaagatatctatagaataaacaagacaactacattttatttttttcacttaaaaatcacaaaaatacagcctaaaatataatttatattttaaaaataattctaaacattaacccctaaatctaatcccttaaaaaattcttgcaaaagttagctggatgtggctgttgccaaggaatgtcttttattagcaacaagtgactatctataacttttattccaacaatcttattttaaatatttgtttcaatttaatgctgggattagaaaaacatatttgttcaaagtatgtaagtagtaagtaaaacaatttcaaaaatctatcaaaaaaggagaattattcattctaggaaataattaacatactggtttaaaatatctgggagaagaacttttacataaaaagcttcaaatttagtcagttgtagcaagcacttgaaaagaccctgctctttcatctgcaatatcaggaattactatatctgactcatatttgattaagttacaatctcatttttgttgtcactacaaagaaggatccttatattagtaaatgcactcactgcaactactgaggcctgcctcctgtcagaatgacaatgcagtcttagcatacgggtgtcggtttggctgaatctaaccaaacacatcacgtactacagatgtttttagggcccacccaattcataaaagattttactgcgatacatgagtttacccaaatttttattaaaatgtgtttttagggtaaatatcttgatgaactaggcaaacaaatactgaatgcagattactgtttttacagttttaccgggaaaactcctaatagcaacccctcttccccttcaccacagatctttaatttaggtgtgatttttgtttgttctctacatgggaataaaggagaaagtttagaaagactgtatctagctagataagatgcagaggtagatggaatctctaacataaaagaagctctaattacactgttgccagacagctgttatggattttagtattgtttattaggtgaagaaaacattcataaaataagaaatttttgagatagaacttactctaataatttcattaacatatgttcaggttcttagatcaagaaatactgtagaggtgttctcctcaagactatgctatggcaataatttcttgcatacaatttaataatttaaacttgaactgtgtgttctgtgctctggcgttctacttcagaaaaaaatgaacactgcttctaaaataaaaaggaacataaaataaaaaaggaattaatgagatattgacatgttttctattaatacaatattgatgttttaaatgattttgatattgctataacaacatatattgtgcaaaataattaatctcactaaatattatttctgatttgccacgaattatctgccgtggcaatcaggaaatagtcttcaaagtaagtttgcaaacatgattttgcaaaccatgattggaaaaatatattcatttgggctataaactatcaagtagggttgttatatatatttctaggaaaatattttatttactctacaaagatcatcattatgaccttacggcttctgtagtgcaatggagaaaaaagtgtgttagaagttaaaagacctgaattctatctccaaccctgcatttattcagagtattggtataggtttaggcaaaatccttaatccagtctagttttatatggtaaaaatgtggatacctatcaaaactgagggttgagaggatgaaatgaattcattaaacatatcttctgagacataaatatatcaaaacaaatcaaaatacaattagatctaatgtttagaaataaatattttaattcatatttgctatttcactaaatctagaaatactaatgctttagttaaatatagaaagttgatgatagaaaaataaaatccatcgtaccattgaaaagcttgtcagaaatatgtactcttgagattcggaggatgagaaaaaaaatgtgtactctaacgaggaagctatataaactgagtctaactcaaaacatttattttagatgcatataagaattaaagtcttagtcaaaagaatgttttaaaatttcatcctaaatttatgtgagataaaatgccattcttttgtttttctgaacagaggagcttttatcaacttattctattttatttttatttttattattttattttattttatttattattattatactttaagttttagggtacatgtgcacaatgtgcaggttagttacatatgtatacatgtgccatgctggtgcgctgcacccactaactcgtcacctagcattaggtatatctcccaatgctatccctcccccctcccccgaccccaccacagtccccagagtgtgatgttccccttcctgtgtccatgtgttctcattgttcagttcccacctatgagtgagaatatgcggtgtttggttttttgttcttgcgatagtttactgagaatgatgatttctaatttcatccatgtccctacacgaacttattctattttaatagaatgttcagtatcagtgttttcacactgagattctctagcttattttgccatatttaaattaaaaagaaacaaaaaatcctgtttgatcatgtgaaaaatatttactgaaatgtgaataaatttatgatcattaattgcctactgaaatattcctgaatattgctcaccttattaacaagtatatatggagactgaaaaacatgtagatcatgcaaacaagtgtaactaactataccaaagaaacaaaagtccatactaaatatgtccataattaaataaaaaatgctaaacaagttttacctagatattataaaaacatagaaaggaaaacatttaggagatgatgaagaagcaggagattgggatgggagatgtaatttgatctaaattcccatatgcttctgtaaaatcaaaaattcattttgcaatattaattttgctcttaaggtagagacttttaaaatgaccattctcaatactacagcaattcttccctgatttgcacataaatgaattaaagtgaagaaaaagcagtagaggagagaagactaaaataaaccagattgtagcaccctgtaaagagctaaaatctccagtgtacaaacaactgataggaaagaagagaaaatcagaactataaaaaagtgacataagctcagaaaattactcatttttaattgtatcaacaaagataatttgtaattttgatcatgcaagcattataattactgataattgggcctttcagcttttaagtgccttctcaaacatgagttctgcatatggttgtgcagaaatcaaaatcttaaagagagatgagtaaagtcaagtttgtaatattaatcttatattctcaatatagatgctaattagtgctctgaatggttgtggttagaaatcttgttggtatgatgtatcagtgatgtcactgcattgatggagacagaataatacataatggtgcaatgtggtgatggtaagctttgttactcaatattgtcaggcactttaagaaaatcagaaacattcaggatagtgccaaagaagatcagtttttcaagactctaaaatcatattcaattatatgtgtatgtaattataaatatgtgcatcatggctgactttgagaagaatgcagcgccttgcaagtgcactatttgaatagagctaaggagaactatagtctaaggactgcaaaagtctagatggagaagacaaaagcaatgacacttgttttctctacagaacaaatagacaaagaggtgaatgacaacaaagatgttcagagaaacttgaaaaataagctacggtgtagggtaagttgtattaaatgatgaaaattaatatgtaactgtatgggtaaaccaaatcatttgtatcttataatcttttttttggtagctacggataatattataaatggaataatcactaaaattctaaatataatgttttctagtaagaacattttattttttttttaatagagacagattctcactctattgcctaggctggactgcaagtggggccattatagctcactgaagcctcaacttcctgggctcaaatgaccctctcgtctcagcctcccgagtagctgggactacaggtgcacatcaccacatccaggtaattattttactttttgaatcatgatatgtagcaaccaatctgggaattatttattcataaaagataacattttcctgctaactccaacctcagaaaaaatgtattatgcctgactcaaatatgtcattatttttatgagaaaaagagtcatattgaagtaattatgtctatatgtaataattatcattatttgagataatttgcattggggagaaaagcaggcaatcagaaattacatattcaaggctgggcgcagtggctcacgcctgtaatcccagcactttgggaggcagaggcgagtgaatcacctgaggtcagagttcaagaccagcctgaccaacaaggagaaaccccatctctactaaaacaaaacaaaacaaaacaaaacaaaaaaagccacaaaattagccgggcatggtggcacatgcctgtaattccagttactcgggaggctgaggcaggagaattgcttgaacctgggaggcagaggttgtagtaagccgagattgtgccactgcacgccagcctgggcgacaagaacgagactcagtctcaaaaaaaaaaaaaaagaaagaaagaaagaaattacatattcaggttctagcaaatgcagttctctaataaacactaaataaatcataatacaagttacagttaaacctaattgttttactatataggatgtatcttttttgtacctatattttatcttcctttgcttctctggcctctattgggaggcagcacggtagtgaacacctcggggatctttctggttacgtaaacctgagttttaattttggttcatactaccttttaactttgggtagtctgctgagcttgttttttgttttcactcatctgtcatatcaagctagtaataattctgccatggttttggttttcatattgaaaggcattacataagcaaaatgcataacatataaatattagttccctttccactatgcatccaatctccctattaaattaagcctaaaaataataatttttgttttattaaaagccttccacattctacatatgaaagggattttttaaaggtgttttagataaaaaatgtttcaaccaactgaccaagaatatctcttcatatttatgtcatctacataaaaacttacatttatatcatatatcttttagtcttcttttctatattcttgattgtcatgttgtacagccagaaaagaatgagtataaattatctagattttttaaagtgcacattcaaacatagaaaatctaattattttacttgtttcttagtattaggctgaggccaatgagtccatgagctaaagggttgaaacttggcaccaaaaaagtgattgtttatgagtcctgtagatttatactgagaaaacatcatgtcttccaatgtgaaatacactaaaacctgattttttgtctcttaaggtgtgctaggtgaatgcaaaaaggatcaggaaagggggtgaggataggtcaggaaaagtgcaaacacaatgttctattcataaattagtgatggcatatttaaggttaagtagtaaaaaatatggggggctcagttaacacgaatgaaaaaatagttaaagtagccatgaattatctggataccttgatttaatgacaccctttcttctgtacaatttcataatgtgggaatagagattagtggggattgtagtggtataccctgactttgcttcatgatatctcaaatgtttaaaacctattattccctagagaaagaaatatgttcatactaattgttgcagaggcagaagccaaatatatctcctcctccatttatgtgactatatagtaatgaaaatcctaggttgatacacttttctcaatcttggaaagattctgctaaagcagcaaatcttctaacaagttcaagagggtggggagagtgaacaagtagaataatttatattaccctggaacaattctgaatcctgtaggtatttatgtcactgtttcaattgtgttctggtttaactgtcaatatttatgcatagcagttaacgtgtgtgcatatttgtaactgtgcagtgctactgccaggtgtgactgtacaaatcatgtgctttgaatgtgcaagttttactttcttttctaacaatttaatacagtgttagaaataaataacgaatgaagacaaccaaagagcagccagacaaatgtgaactggttttgacgtgacgagaaactcatcagtaagtaaataaacctcctccctggagaaggccactgaaatgcacccaggaggatgtctctactagaaggtaataaaaaatatatataatgtagtctttgacctaaaacctcatgattattactttgccatttatttccccctggtatctgatgttcatattagtttaatgtgccttttcagagaattcaagacactttttggaaagtagaatttttttttgaaaatttatgattggagaggtactacacaatttagaggttacatttcttgacaaatctgagttgaataaaaaagaactaaaaatataaacatagctaattcaagaatcaagatcgggtgaaactaaattaaaaacagccataaagtcccacattttccctaatttatttacctatgatattggcacatcttgttttacttaacatttgaaaaatacaaatatctcttcatatgcaaaagagcaaatgttaaatgaaaaactgaattttatatagcttcctaaatatgagccacatgcttaagcagtgaattaactttatgaatcaaatgtttaatgttaactattacaaaagcctggtatccaggtgcaatctcaccagaaaaaaatagcacctgcctttattacaataaaaaaaatggctaattccctttgacatcttaagagtgacactactttgtcaagcactaaatactttttaaattaatcatgttaaacttcagatttatagatataaatattgtatttataactttagtcataatgtacaatttctttcttgtttaaaagtactttctcactcaaaatggtatttatagtttaaaaagaatatgcctctgtattcaggagtgattcaaattcccagatgttttcacatagttatgaaaatgggaaagtgctgaattaaactgggctgcaatatttcaagttttttgctatcaggttataaactatacctacgattgcaagtcatacagtgcctctatttctagaaggcttttaaagtttcctggcttagttatgtccaaaggcagcaggaagtctcatcagtagagggcagaattttcaagtgctgccattcttatcccaggaggcatttccagtggttgagcacaaggcctgtttgtagtttgcttttgctcttgcattttgtggaagggaaggaactgagagagcttagagggttcattaaaaccacccctcactctcttagtcgtagtcagatggagtattcataacagtaacctccaattaccactatgtgttgggaaaaattagaattcggtctacttacaatcctgccaactaggattttactttgatatttcagtataacagtgaatctggattgatgcctgattaaaataaaatccctgattattactttctggattacgaactaaaatccctgtaaaatcaatggatgtgactcattgttaagagtcatgcagacttttacatattaggtaagaattctaaaaattatttgagggttctattctctagcaccaggtactaatgctccctactcaaaaaaaatcatgtgcatggattaatcaagtctaacagtgctcagatttaatggtttaacattgattttcttttctttgtcaaacttatatatgcaaatatttttatagtagtcagatgttatttttgaataaggatcaccctcatttttacccatgtgcttatctttaaaaccaacattgtaaagtagcacgcagacatatgtttcttttatcttcatggattatttttaccttaaaaataaattatcatttttttttttgaatttgggttttattctccagatactctgtgtacatgtgggtaagtatgtgggagtatgtgtgtttgtgtgtaagaggggataattaattgtctctcaactctatctcatactttaatatcaaataaaaaatgaaatgtataaagggtcactttgtaggattaggcatcctccttctacctacttaaaccaggggtttgggattcagaattctccatataaccaagaccgaaagtcactggaagactttaaaattagtattttaaccaccacacccagagtcaggtatggaaataaacctatagcatggattctttctatgcataatctcaaaatttaactacccaaataagtaagtttttaaaaactaatttaaaatttgccattgaggaaaatatcacctccatccttaattgtgactcctcatttcagctaaaaccttttctaatactttaaaaaaacaaaatgaaaaacaaactcctagataaagtcataaacactgaaatcagagatgtgattcttgttaaatgttagtttctctttctgaggttacactctgtgcatttgaaactttgacgttaacatcttccgaatgtttagatttgctcaagggttcagattctctggtcttctgccttgcattttcctccttcctttcctttgcaagcaatctatagttgatagcattgccaatgagcagccacacgcttgctgctaccacaatagccccacaggacatgtacatgtatttatattctccagttaaatccaccaatttacctgcaagaggagggccaagaagaactgggccacactccacaattgtgacaagtccgacggcactggaaaatcttggtgcacccacgaggtccatgagagtttcaaagagaacactgctaacactcccaaatccaaggccaaaaaatacagcatataataccaggcttgtgtagtcctgtgccagtgggcacaagaggtgacacactccattgaacatgattgcaaaactgaagaagtactgaattcgaggtcgaatatatttggagtttgcaattaatcctacagaaggcctagcaaacatatcaacgaaagccataacagatagcagaaaagctgccgagtactcatcaattccttggtctttagcatatggagccaagaatataatgggggcaaaaaaacctaggaacataatgacatttccagacagatatatcagaaatcctctatgcttaaaaagggagaaatctaaatacttattaactttttcccaagttgatttcttcgttttgattttctttgggcttgaatcatcttctgttttgccagtcttatttttagacttagaagtggtttgattgggtccaaggggtctcatgagggaaccagccacacaggcattcaaaagtagacttcccaaaatcaggaagcttcctttccagccaaaagtattaaaaaggtactgattgaaaggagccaatgaacttaagaaaacaggacttcctgccatggccaatccatttgccatgggtcgcttcctatagaagtatttgccaattatggttaaggcgggttgcaggttgaaggctaaacctaaacctgtaatgaatcccatagtgaggtacagctgtaccacgctgctactaaaggaggccaacaccattccaagacagcataataagcctcctgctatcaccaccggccggctgccgtatttattcaccaaaacactacttacaggacctcctgcgtacataacagccagcataatggatgaaatccatgctatttcactgtaggtagtgtggaatatttgctgaatttctttgaagaatacggtgacagctttggggaatgcataggaaaatccaatggagataaaagctgctccaaccacaatccaaccccatcctccatctggaggtggatgcacaggtggggcacttggcattggtggcatttctgctcctctagtggaaattcaagtaacagagtaactctgttggcaccaagagtcccagagtctttggttccccagatcaccttgtttcaggtttcacaggaaagtatcacatcttaagattgactctttatctggtctctggcgcagggtgggcgctgcagccctccgttcccagcaaaccgcagccgattcgcctcgctgtcaacgggtgaatggaattatttatttatttatggcccctgacgtgtcctcgcccgccacagccagcggagaaggaggcggtggcgggaaggggaggcgcggctgctgaacgcccttgtgggtgcggaggagc

SEQ ID NO: 17830 - RNA, 11930 nt, Homo sapiens
  source 1..11930: mol_type = other RNA
tcgaggagctcacagtctagtaagaaagagatgaatttgaaaatatatttgaaactgtaggcaaaataagtaccctcacagagaaattcaacatttggtttcaaatttgttatgcagtgaaaattagaaactacaaccaagatttttttaaaacattatgttcatataacgctgtagtatacctgaaaggcaagaacttaaacaagtgtgctgaaaaacaaattaggaatatttgaacaaaatatactttaaaaatgatcaacaacgtaaaatattcctgatttaaataaatctaagttattttatttagtttaagcaaaatatgtatccatatgaaaatgccagttctttcatttttggttaattcctttacacatattatttgctaagttcagaaatgctatatatacaaaaatttcaaaaataaataagtatcccaagatcacataacaatactttaagtacattcatgtgtaagaaggcaaaaaaagaaggttctatcttatattttaaaactttgacaggtattttaaatgtattattttatactttattttctttaaaaatgaaataatacagccatgatttaagtcatgtaaaaacaactgtttggatcatttaggtgtcaagcaaaactatcctctttatttcactatcatagtaaccatagttgatagaccatgtggcaatatgatcatttgttcagtggtcattaagatatctatagaataaacaagacaactacattttatttttttcacttaaaaatcacaaaaatacagcctaaaatataatttatattttaaaaataattctaaacattaacccctaaatctaatcccttaaaaaattcttgcaaaagttagctggatgtggctgttgccaaggaatgtcttttattagcaacaagtgactatctataacttttattccaacaatcttattttaaatatttgtttcaatttaatgctgggattagaaaaacatatttgttcaaagtatgtaagtagtaagtaaaacaatttcaaaaatctatcaaaaaaggagaattattcattctaggaaataattaacatactggtttaaaatatctgggagaagaacttttacataaaaagcttcaaatttagtcagttgtagcaagcacttgaaaagaccctgctctttcatctgcaatatcaggaattactatatctgactcatatttgattaagttacaatctcatttttgttgtcactacaaagaaggatccttatattagtaaatgcactcactgcaactactgaggcctgcctcctgtcagaatgacaatgcagtcttagcatacgggtgtcggtttggctgaatctaaccaaacacatcacgtactacagatgtttttagggcccacccaattcataaaagattttactgcgatacatgagtttacccaaatttttattaaaatgtgtttttagggtaaatatcttgatgaactaggcaaacaaatactgaatgcagattactgtttttacagttttaccgggaaaactcctaatagcaacccctcttccccttcaccacagatctttaatttaggtgtgatttttgtttgttctctacatgggaataaaggagaaagtttagaaagactgtatctagctagataagatgcagaggtagatggaatctctaacataaaagaagctctaattacactgttgccagacagctgttatggattttagtattgtttattaggtgaagaaaacattcataaaataagaaatttttgagatagaacttactctaataatttcattaacatatgttcaggttcttagatcaagaaatactgtagaggtgttctcctcaagactatgctatggcaataatttcttgcatacaatttaataatttaaacttgaactgtgtgttctgtgctctggcgttctacttcagaaaaaaatgaacactgcttctaaaataaaaaggaacataaaataaaaaaggaattaatgagatattgacatgttttctattaatacaatattgatgttttaaatgattttgatattgctataacaacatatattgtgcaaaataattaatctcactaaatattatttctgatttgccacgaattatctgccgtggcaatcaggaaatagtcttcaaagtaagtttgcaaacatgattttgcaaaccatgattggaaaaatatattcatttgggctataaactatcaagtagggttgttatatatatttctaggaaaatattttatttactctacaaagatcatcattatgaccttacggcttctgtagtgcaatggagaaaaaagtgtgttagaagttaaaagacctgaattctatctccaaccctgcatttattcagagtattggtataggtttaggcaaaatccttaatccagtctagttttatatggtaaaaatgtggatacctatcaaaactgagggttgagaggatgaaatgaattcattaaacatatcttctgagacataaatatatcaaaacaaatcaaaatacaattagatctaatgtttagaaataaatattttaattcatatttgctatttcactaaatctagaaatactaatgctttagttaaatatagaaagttgatgatagaaaaataaaatccatcgtaccattgaaaagcttgtcagaaatatgtactcttgagattcggaggatgagaaaaaaaatgtgtactctaacgaggaagctatataaactgagtctaactcaaaacatttattttagatgcatataagaattaaagtcttagtcaaaagaatgttttaaaatttcatcctaaatttatgtgagataaaatgccattcttttgtttttctgaacagaggagcttttatcaacttattctattttatttttatttttattattttattttattttatttattattattatactttaagttttagggtacatgtgcacaatgtgcaggttagttacatatgtatacatgtgccatgctggtgcgctgcacccactaactcgtcacctagcattaggtatatctcccaatgctatccctcccccctcccccgaccccaccacagtccccagagtgtgatgttccccttcctgtgtccatgtgttctcattgttcagttcccacctatgagtgagaatatgcggtgtttggttttttgttcttgcgatagtttactgagaatgatgatttctaatttcatccatgtccctacacgaacttattctattttaatagaatgttcagtatcagtgttttcacactgagattctctagcttattttgccatatttaaattaaaaagaaacaaaaaatcctgtttgatcatgtgaaaaatatttactgaaatgtgaataaatttatgatcattaattgcctactgaaatattcctgaatattgctcaccttattaacaagtatatatggagactgaaaaacatgtagatcatgcaaacaagtgtaactaactataccaaagaaacaaaagtccatactaaatatgtccataattaaataaaaaatgctaaacaagttttacctagatattataaaaacatagaaaggaaaacatttaggagatgatgaagaagcaggagattgggatgggagatgtaatttgatctaaattcccatatgcttctgtaaaatcaaaaattcattttgcaatattaattttgctcttaaggtagagacttttaaaatgaccattctcaatactacagcaattcttccctgatttgcacataaatgaattaaagtgaagaaaaagcagtagaggagagaagactaaaataaaccagattgtagcaccctgtaaagagctaaaatctccagtgtacaaacaactgataggaaagaagagaaaatcagaactataaaaaagtgacataagctcagaaaattactcatttttaattgtatcaacaaagataatttgtaattttgatcatgcaagcattataattactgataattgggcctttcagcttttaagtgccttctcaaacatgagttctgcatatggttgtgcagaaatcaaaatcttaaagagagatgagtaaagtcaagtttgtaatattaatcttatattctcaatatagatgctaattagtgctctgaatggttgtggttagaaatcttgttggtatgatgtatcagtgatgtcactgcattgatggagacagaataatacataatggtgcaatgtggtgatggtaagctttgttactcaatattgtcaggcactttaagaaaatcagaaacattcaggatagtgccaaagaagatcagtttttcaagactctaaaatcatattcaattatatgtgtatgtaattataaatatgtgcatcatggctgactttgagaagaatgcagcgccttgcaagtgcactatttgaatagagctaaggagaactatagtctaaggactgcaaaagtctagatggagaagacaaaagcaatgacacttgttttctctacagaacaaatagacaaagaggtgaatgacaacaaagatgttcagagaaacttgaaaaataagctacggtgtagggtaagttgtattaaatgatgaaaattaatatgtaactgtatgggtaaaccaaatcatttgtatcttataatcttttttttggtagctacggataatattataaatggaataatcactaaaattctaaatataatgttttctagtaagaacattttattttttttttaatagagacagattctcactctattgcctaggctggactgcaagtggggccattatagctcactgaagcctcaacttcctgggctcaaatgaccctctcgtctcagcctcccgagtagctgggactacaggtgcacatcaccacatccaggtaattattttactttttgaatcatgatatgtagcaaccaatctgggaattatttattcataaaagataacattttcctgctaactccaacctcagaaaaaatgtattatgcctgactcaaatatgtcattatttttatgagaaaaagagtcatattgaagtaattatgtctatatgtaataattatcattatttgagataatttgcattggggagaaaagcaggcaatcagaaattacatattcaaggctgggcgcagtggctcacgcctgtaatcccagcactttgggaggcagaggcgagtgaatcacctgaggtcagagttcaagaccagcctgaccaacaaggagaaaccccatctctactaaaacaaaacaaaacaaaacaaaacaaaaaaagccacaaaattagccgggcatggtggcacatgcctgtaattccagttactcgggaggctgaggcaggagaattgcttgaacctgggaggcagaggttgtagtaagccgagattgtgccactgcacgccagcctgggcgacaagaacgagactcagtctcaaaaaaaaaaaaaaagaaagaaagaaagaaattacatattcaggttctagcaaatgcagttctctaataaacactaaataaatcataatacaagttacagttaaacctaattgttttactatataggatgtatcttttttgtacctatattttatcttcctttgcttctctggcctctattgggaggcagcacggtagtgaacacctcggggatctttctggttacgtaaacctgagttttaattttggttcatactaccttttaactttgggtagtctgctgagcttgttttttgttttcactcatctgtcatatcaagctagtaataattctgccatggttttggttttcatattgaaaggcattacataagcaaaatgcataacatataaatattagttccctttccactatgcatccaatctccctattaaattaagcctaaaaataataatttttgttttattaaaagccttccacattctacatatgaaagggattttttaaaggtgttttagataaaaaatgtttcaaccaactgaccaagaatatctcttcatatttatgtcatctacataaaaacttacatttatatcatatatcttttagtcttcttttctatattcttgattgtcatgttgtacagccagaaaagaatgagtataaattatctagattttttaaagtgcacattcaaacatagaaaatctaattattttacttgtttcttagtattaggctgaggccaatgagtccatgagctaaagggttgaaacttggcaccaaaaaagtgattgtttatgagtcctgtagatttatactgagaaaacatcatgtcttccaatgtgaaatacactaaaacctgattttttgtctcttaaggtgtgctaggtgaatgcaaaaaggatcaggaaagggggtgaggataggtcaggaaaagtgcaaacacaatgttctattcataaattagtgatggcatatttaaggttaagtagtaaaaaatatggggggctcagttaacacgaatgaaaaaatagttaaagtagccatgaattatctggataccttgatttaatgacaccctttcttctgtacaatttcataatgtgggaatagagattagtggggattgtagtggtataccctgactttgcttcatgatatctcaaatgtttaaaacctattattccctagagaaagaaatatgttcatactaattgttgcagaggcagaagccaaatatatctcctcctccatttatgtgactatatagtaatgaaaatcctaggttgatacacttttctcaatcttggaaagattctgctaaagcagcaaatcttctaacaagttcaagagggtggggagagtgaacaagtagaataatttatattaccctggaacaattctgaatcctgtaggtatttatgtcactgtttcaattgtgttctggtttaactgtcaatatttatgcatagcagttaacgtgtgtgcatatttgtaactgtgcagtgctactgccaggtgtgactgtacaaatcatgtgctttgaatgtgcaagttttactttcttttctaacaatttaatacagtgttagaaataaataacgaatgaagacaaccaaagagcagccagacaaatgtgaactggttttgacgtgacgagaaactcatcagtaagtaaataaacctcctccctggagaaggccactgaaatgcacccaggaggatgtctctactagaaggtaataaaaaatatatataatgtagtctttgacctaaaacctcatgattattactttgccatttatttccccctggtatctgatgttcatattagtttaatgtgccttttcagagaattcaagacactttttggaaagtagaatttttttttgaaaatttatgattggagaggtactacacaatttagaggttacatttcttgacaaatctgagttgaataaaaaagaactaaaaatataaacatagctaattcaagaatcaagatcgggtgaaactaaattaaaaacagccataaagtcccacattttccctaatttatttacctatgatattggcacatcttgttttacttaacatttgaaaaatacaaatatctcttcatatgcaaaagagcaaatgttaaatgaaaaactgaattttatatagcttcctaaatatgagccacatgcttaagcagtgaattaactttatgaatcaaatgtttaatgttaactattacaaaagcctggtatccaggtgcaatctcaccagaaaaaaatagcacctgcctttattacaataaaaaaaatggctaattccctttgacatcttaagagtgacactactttgtcaagcactaaatactttttaaattaatcatgttaaacttcagatttatagatataaatattgtatttataactttagtcataatgtacaatttctttcttgtttaaaagtactttctcactcaaaatggtatttatagtttaaaaagaatatgcctctgtattcaggagtgattcaaattcccagatgttttcacatagttatgaaaatgggaaagtgctgaattaaactgggctgcaatatttcaagttttttgctatcaggttataaactatacctacgattgcaagtcatacagtgcctctatttctagaaggcttttaaagtttcctggcttagttatgtccaaaggcagcaggaagtctcatcagtagagggcagaattttcaagtgctgccattcttatcccaggaggcatttccagtggttgagcacaaggcctgtttgtagtttgcttttgctcttgcattttgtggaagggaaggaactgagagagcttagagggttcattaaaaccacccctcactctcttagtcgtagtcagatggagtattcataacagtaacctccaattaccactatgtgttgggaaaaattagaattcggtctacttacaatcctgccaactaggattttactttgatatttcagtataacagtgaatctggattgatgcctgattaaaataaaatccctgattattactttctggattacgaactaaaatccctgtaaaatcaatggatgtgactcattgttaagagtcatgcagacttttacatattaggtaagaattctaaaaattatttgagggttctattctctagcaccaggtactaatgctccctactcaaaaaaaatcatgtgcatggattaatcaagtctaacagtgctcagatttaatggtttaacattgattttcttttctttgtcaaacttatatatgcaaatatttttatagtagtcagatgttatttttgaataaggatcaccctcatttttacccatgtgcttatctttaaaaccaacattgtaaagtagcacgcagacatatgtttcttttatcttcatggattatttttaccttaaaaataaattatcatttttttttttgaatttgggttttattctccagatactctgtgtacatgtgggtaagtatgtgggagtatgtgtgtttgtgtgtaagaggggataattaattgtctctcaactctatctcatactttaatatcaaataaaaaatgaaatgtataaagggtcactttgtaggattaggcatcctccttctacctacttaaaccaggggtttgggattcagaattctccatataaccaagaccgaaagtcactggaagactttaaaattagtattttaaccaccacacccagagtcaggtatggaaataaacctatagcatggattctttctatgcataatctcaaaatttaactacccaaataagtaagtttttaaaaactaatttaaaatttgccattgaggaaaatatcacctccatccttaattgtgactcctcatttcagctaaaaccttttctaatactttaaaaaaacaaaatgaaaaacaaactcctagataaagtcataaacactgaaatcagagatgtgattcttgttaaatgttagtttctctttctgaggttacactctgtgcatttgaaactttgacgttaacatcttccgaatgtttagatttgctcaagggttcagattctctggtcttctgccttgcattttcctccttcctttcctttgcaagcaatctatagttgatagcattgccaatgagcagccacacgcttgctgctaccacaatagccccacaggacatgtacatgtatttatattctccagttaaatccaccaatttacctgcaagaggagggccaagaagaactgggccacactccacaattgtgacaagtccgacggcactggaaaatcttggtgcacccacgaggtccatgagagtttcaaagagaacactgctaacactcccaaatccaaggccaaaaaatacagcatataataccaggcttgtgtagtcctgtgccagtgggcacaagaggtgacacactccattgaacatgattgcaaaactgaagaagtactgaattcgaggtcgaatatatttggagtttgcaattaatcctacagaaggcctagcaaacatatcaacgaaagccataacagatagcagaaaagctgccgagtactcatcaattccttggtctttagcatatggagccaagaatataatgggggcaaaaaaacctaggaacataatgacatttccagacagatatatcagaaatcctctatgcttaaaaagggagaaatctaaatacttattaactttttcccaagttgatttcttcgttttgattttctttgggcttgaatcatcttctgttttgccagtcttatttttagacttagaagtggtttgattgggtccaaggggtctcatgagggaaccagccacacaggcattcaaaagtagacttcccaaaatcaggaagcttcctttccagccaaaagtattaaaaaggtactgattgaaaggagccaatgaacttaagaaaacaggacttcctgccatggccaatccatttgccatgggtcgcttcctatagaagtatttgccaattatggttaaggcgggttgcaggttgaaggctaaacctaaacctgtaatgaatcccatagtgaggtacagctgtaccacgctgctactaaaggaggccaacaccattccaagacagcataataagcctcctgctatcaccaccggccggctgccgtatttattcaccaaaacactacttacaggacctcctgcgtacataacagccagcataatggatgaaatccatgctatttcactgtaggtagtgtggaatatttgctgaatttctttgaagaatacggtgacagctttggggaatgcataggaaaatccaatggagataaaagctgctccaaccacaatccaaccccatcctccatctggaggtggatgcacaggtggggcacttggcattggtggcatttctgctcctctagtggaaattcaagtaacatacatatctccagagactctgctttgccctcccctctctcttctctcaaatagggcaaagttagttatttctctttttcaagaacctgctttgacgtgcactattagttcatacttttcagagtctaaagtaagcttggcttaaattatatcatgggtcaaagaaggtggccaagtctggcaatttgaactgctaaatttaaccttctcatgtgttgtgttgatgtagccacattttcaagcacattttccattgcgtgatttaatatgcataaaacatattgcaaaaatactgtactatatacattaatagtttagtgactcttcactgagtctgagactaggtaatttgtaagttatgaacaataacaaagaggccagggtcaaagtgttgaatctcttgtgggccagtttaatctatttcttgatcacacataacactccctacatggtcagccactctgtaaatgcatgctctctgtcccaaagagtccccaaccctgtgtgagggtgaatctggtgatagatcattagtaccatcttcgttttagaagaaattactataacctttggaaaaatgcagtggtgtaatttattaaatgcttctcatattctaggtaagcattttgccaaacaatttatacccactaccccattctctaaatgatacatgatagacattatgataaatattttcctatggggacactgaagctcagcgttttgattacttatgtaaggccatatagctgtaaaatatggggtcctggattccaactctagattgtctagattcgaggctcatgttcctctctatcaaacagcatgccagactcctctatcagtggatgagaaatatctgatttcctatgtgaaagatacaattatttagatctaagcactaagcagtagccacttgtaaaatatgcttcccaaagatttgggaaggctgcatttctaaatgtgtataataatgaaataataataaccaggtaataacataaataacctctagaaatt

SEQ ID NO: 17831 - RNA, 10980 nt, Homo sapiens
  source 1..10980: mol_type = other RNA
tcgaggagctcacagtctagtaagaaagagatgaatttgaaaatatatttgaaactgtaggcaaaataagtaccctcacagagaaattcaacatttggtttcaaatttgttatgcagtgaaaattagaaactacaaccaagatttttttaaaacattatgttcatataacgctgtagtatacctgaaaggcaagaacttaaacaagtgtgctgaaaaacaaattaggaatatttgaacaaaatatactttaaaaatgatcaacaacgtaaaatattcctgatttaaataaatctaagttattttatttagtttaagcaaaatatgtatccatatgaaaatgccagttctttcatttttggttaattcctttacacatattatttgctaagttcagaaatgctatatatacaaaaatttcaaaaataaataagtatcccaagatcacataacaatactttaagtacattcatgtgtaagaaggcaaaaaaagaaggttctatcttatattttaaaactttgacaggtattttaaatgtattattttatactttattttctttaaaaatgaaataatacagccatgatttaagtcatgtaaaaacaactgtttggatcatttaggtgtcaagcaaaactatcctctttatttcactatcatagtaaccatagttgatagaccatgtggcaatatgatcatttgttcagtggtcattaagatatctatagaataaacaagacaactacattttatttttttcacttaaaaatcacaaaaatacagcctaaaatataatttatattttaaaaataattctaaacattaacccctaaatctaatcccttaaaaaattcttgcaaaagttagctggatgtggctgttgccaaggaatgtcttttattagcaacaagtgactatctataacttttattccaacaatcttattttaaatatttgtttcaatttaatgctgggattagaaaaacatatttgttcaaagtatgtaagtagtaagtaaaacaatttcaaaaatctatcaaaaaaggagaattattcattctaggaaataattaacatactggtttaaaatatctgggagaagaacttttacataaaaagcttcaaatttagtcagttgtagcaagcacttgaaaagaccctgctctttcatctgcaatatcaggaattactatatctgactcatatttgattaagttacaatctcatttttgttgtcactacaaagaaggatccttatattagtaaatgcactcactgcaactactgaggcctgcctcctgtcagaatgacaatgcagtcttagcatacgggtgtcggtttggctgaatctaaccaaacacatcacgtactacagatgtttttagggcccacccaattcataaaagattttactgcgatacatgagtttacccaaatttttattaaaatgtgtttttagggtaaatatcttgatgaactaggcaaacaaatactgaatgcagattactgtttttacagttttaccgggaaaactcctaatagcaacccctcttccccttcaccacagatctttaatttaggtgtgatttttgtttgttctctacatgggaataaaggagaaagtttagaaagactgtatctagctagataagatgcagaggtagatggaatctctaacataaaagaagctctaattacactgttgccagacagctgttatggattttagtattgtttattaggtgaagaaaacattcataaaataagaaatttttgagatagaacttactctaataatttcattaacatatgttcaggttcttagatcaagaaatactgtagaggtgttctcctcaagactatgctatggcaataatttcttgcatacaatttaataatttaaacttgaactgtgtgttctgtgctctggcgttctacttcagaaaaaaatgaacactgcttctaaaataaaaaggaacataaaataaaaaaggaattaatgagatattgacatgttttctattaatacaatattgatgttttaaatgattttgatattgctataacaacatatattgtgcaaaataattaatctcactaaatattatttctgatttgccacgaattatctgccgtggcaatcaggaaatagtcttcaaagtaagtttgcaaacatgattttgcaaaccatgattggaaaaatatattcatttgggctataaactatcaagtagggttgttatatatatttctaggaaaatattttatttactctacaaagatcatcattatgaccttacggcttctgtagtgcaatggagaaaaaagtgtgttagaagttaaaagacctgaattctatctccaaccctgcatttattcagagtattggtataggtttaggcaaaatccttaatccagtctagttttatatggtaaaaatgtggatacctatcaaaactgagggttgagaggatgaaatgaattcattaaacatatcttctgagacataaatatatcaaaacaaatcaaaatacaattagatctaatgtttagaaataaatattttaattcatatttgctatttcactaaatctagaaatactaatgctttagttaaatatagaaagttgatgatagaaaaataaaatccatcgtaccattgaaaagcttgtcagaaatatgtactcttgagattcggaggatgagaaaaaaaatgtgtactctaacgaggaagctatataaactgagtctaactcaaaacatttattttagatgcatataagaattaaagtcttagtcaaaagaatgttttaaaatttcatcctaaatttatgtgagataaaatgccattcttttgtttttctgaacagaggagcttttatcaacttattctattttatttttatttttattattttattttattttatttattattattatactttaagttttagggtacatgtgcacaatgtgcaggttagttacatatgtatacatgtgccatgctggtgcgctgcacccactaactcgtcacctagcattaggtatatctcccaatgctatccctcccccctcccccgaccccaccacagtccccagagtgtgatgttccccttcctgtgtccatgtgttctcattgttcagttcccacctatgagtgagaatatgcggtgtttggttttttgttcttgcgatagtttactgagaatgatgatttctaatttcatccatgtccctacacgaacttattctattttaatagaatgttcagtatcagtgttttcacactgagattctctagcttattttgccatatttaaattaaaaagaaacaaaaaatcctgtttgatcatgtgaaaaatatttactgaaatgtgaataaatttatgatcattaattgcctactgaaatattcctgaatattgctcaccttattaacaagtatatatggagactgaaaaacatgtagatcatgcaaacaagtgtaactaactataccaaagaaacaaaagtccatactaaatatgtccataattaaataaaaaatgctaaacaagttttacctagatattataaaaacatagaaaggaaaacatttaggagatgatgaagaagcaggagattgggatgggagatgtaatttgatctaaattcccatatgcttctgtaaaatcaaaaattcattttgcaatattaattttgctcttaaggtagagacttttaaaatgaccattctcaatactacagcaattcttccctgatttgcacataaatgaattaaagtgaagaaaaagcagtagaggagagaagactaaaataaaccagattgtagcaccctgtaaagagctaaaatctccagtgtacaaacaactgataggaaagaagagaaaatcagaactataaaaaagtgacataagctcagaaaattactcatttttaattgtatcaacaaagataatttgtaattttgatcatgcaagcattataattactgataattgggcctttcagcttttaagtgccttctcaaacatgagttctgcatatggttgtgcagaaatcaaaatcttaaagagagatgagtaaagtcaagtttgtaatattaatcttatattctcaatatagatgctaattagtgctctgaatggttgtggttagaaatcttgttggtatgatgtatcagtgatgtcactgcattgatggagacagaataatacataatggtgcaatgtggtgatggtaagctttgttactcaatattgtcaggcactttaagaaaatcagaaacattcaggatagtgccaaagaagatcagtttttcaagactctaaaatcatattcaattatatgtgtatgtaattataaatatgtgcatcatggctgactttgagaagaatgcagcgccttgcaagtgcactatttgaatagagctaaggagaactatagtctaaggactgcaaaagtctagatggagaagacaaaagcaatgacacttgttttctctacagaacaaatagacaaagaggtgaatgacaacaaagatgttcagagaaacttgaaaaataagctacggtgtagggtaagttgtattaaatgatgaaaattaatatgtaactgtatgggtaaaccaaatcatttgtatcttataatcttttttttggtagctacggataatattataaatggaataatcactaaaattctaaatataatgttttctagtaagaacattttattttttttttaatagagacagattctcactctattgcctaggctggactgcaagtggggccattatagctcactgaagcctcaacttcctgggctcaaatgaccctctcgtctcagcctcccgagtagctgggactacaggtgcacatcaccacatccaggtaattattttactttttgaatcatgatatgtagcaaccaatctgggaattatttattcataaaagataacattttcctgctaactccaacctcagaaaaaatgtattatgcctgactcaaatatgtcattatttttatgagaaaaagagtcatattgaagtaattatgtctatatgtaataattatcattatttgagataatttgcattggggagaaaagcaggcaatcagaaattacatattcaaggctgggcgcagtggctcacgcctgtaatcccagcactttgggaggcagaggcgagtgaatcacctgaggtcagagttcaagaccagcctgaccaacaaggagaaaccccatctctactaaaacaaaacaaaacaaaacaaaacaaaaaaagccacaaaattagccgggcatggtggcacatgcctgtaattccagttactcgggaggctgaggcaggagaattgcttgaacctgggaggcagaggttgtagtaagccgagattgtgccactgcacgccagcctgggcgacaagaacgagactcagtctcaaaaaaaaaaaaaaagaaagaaagaaagaaattacatattcaggttctagcaaatgcagttctctaataaacactaaataaatcataatacaagttacagttaaacctaattgttttactatataggatgtatcttttttgtacctatattttatcttcctttgcttctctggcctctattgggaggcagcacggtagtgaacacctcggggatctttctggttacgtaaacctgagttttaattttggttcatactaccttttaactttgggtagtctgctgagcttgttttttgttttcactcatctgtcatatcaagctagtaataattctgccatggttttggttttcatattgaaaggcattacataagcaaaatgcataacatataaatattagttccctttccactatgcatccaatctccctattaaattaagcctaaaaataataatttttgttttattaaaagccttccacattctacatatgaaagggattttttaaaggtgttttagataaaaaatgtttcaaccaactgaccaagaatatctcttcatatttatgtcatctacataaaaacttacatttatatcatatatcttttagtcttcttttctatattcttgattgtcatgttgtacagccagaaaagaatgagtataaattatctagattttttaaagtgcacattcaaacatagaaaatctaattattttacttgtttcttagtattaggctgaggccaatgagtccatgagctaaagggttgaaacttggcaccaaaaaagtgattgtttatgagtcctgtagatttatactgagaaaacatcatgtcttccaatgtgaaatacactaaaacctgattttttgtctcttaaggtgtgctaggtgaatgcaaaaaggatcaggaaagggggtgaggataggtcaggaaaagtgcaaacacaatgttctattcataaattagtgatggcatatttaaggttaagtagtaaaaaatatggggggctcagttaacacgaatgaaaaaatagttaaagtagccatgaattatctggataccttgatttaatgacaccctttcttctgtacaatttcataatgtgggaatagagattagtggggattgtagtggtataccctgactttgcttcatgatatctcaaatgtttaaaacctattattccctagagaaagaaatatgttcatactaattgttgcagaggcagaagccaaatatatctcctcctccatttatgtgactatatagtaatgaaaatcctaggttgatacacttttctcaatcttggaaagattctgctaaagcagcaaatcttctaacaagttcaagagggtggggagagtgaacaagtagaataatttatattaccctggaacaattctgaatcctgtaggtatttatgtcactgtttcaattgtgttctggtttaactgtcaatatttatgcatagcagttaacgtgtgtgcatatttgtaactgtgcagtgctactgccaggtgtgactgtacaaatcatgtgctttgaatgtgcaagttttactttcttttctaacaatttaatacagtgttagaaataaataacgaatgaagacaaccaaagagcagccagacaaatgtgaactggttttgacgtgacgagaaactcatcagtaagtaaataaacctcctccctggagaaggccactgaaatgcacccaggaggatgtctctactagaaggtaataaaaaatatatataatgtagtctttgacctaaaacctcatgattattactttgccatttatttccccctggtatctgatgttcatattagtttaatgtgccttttcagagaattcaagacactttttggaaagtagaatttttttttgaaaatttatgattggagaggtactacacaatttagaggttacatttcttgacaaatctgagttgaataaaaaagaactaaaaatataaacatagctaattcaagaatcaagatcgggtgaaactaaattaaaaacagccataaagtcccacattttccctaatttatttacctatgatattggcacatcttgttttacttaacatttgaaaaatacaaatatctcttcatatgcaaaagagcaaatgttaaatgaaaaactgaattttatatagcttcctaaatatgagccacatgcttaagcagtgaattaactttatgaatcaaatgtttaatgttaactattacaaaagcctggtatccaggtgcaatctcaccagaaaaaaatagcacctgcctttattacaataaaaaaaatggctaattccctttgacatcttaagagtgacactactttgtcaagcactaaatactttttaaattaatcatgttaaacttcagatttatagatataaatattgtatttataactttagtcataatgtacaatttctttcttgtttaaaagtactttctcactcaaaatggtatttatagtttaaaaagaatatgcctctgtattcaggagtgattcaaattcccagatgttttcacatagttatgaaaatgggaaagtgctgaattaaactgggctgcaatatttcaagttttttgctatcaggttataaactatacctacgattgcaagtcatacagtgcctctatttctagaaggcttttaaagtttcctggcttagttatgtccaaaggcagcaggaagtctcatcagtagagggcagaattttcaagtgctgccattcttatcccaggaggcatttccagtggttgagcacaaggcctgtttgtagtttgcttttgctcttgcattttgtggaagggaaggaactgagagagcttagagggttcattaaaaccacccctcactctcttagtcgtagtcagatggagtattcataacagtaacctccaattaccactatgtgttgggaaaaattagaattcggtctacttacaatcctgccaactaggattttactttgatatttcagtataacagtgaatctggattgatgcctgattaaaataaaatccctgattattactttctggattacgaactaaaatccctgtaaaatcaatggatgtgactcattgttaagagtcatgcagacttttacatattaggtaagaattctaaaaattatttgagggttctattctctagcaccaggtactaatgctccctactcaaaaaaaatcatgtgcatggattaatcaagtctaacagtgctcagatttaatggtttaacattgattttcttttctttgtcaaacttatatatgcaaatatttttatagtagtcagatgttatttttgaataaggatcaccctcatttttacccatgtgcttatctttaaaaccaacattgtaaagtagcacgcagacatatgtttcttttatcttcatggattatttttaccttaaaaataaattatcatttttttttttgaatttgggttttattctccagatactctgtgtacatgtgggtaagtatgtgggagtatgtgtgtttgtgtgtaagaggggataattaattgtctctcaactctatctcatactttaatatcaaataaaaaatgaaatgtataaagggtcactttgtaggattaggcatcctccttctacctacttaaaccaggggtttgggattcagaattctccatataaccaagaccgaaagtcactggaagactttaaaattagtattttaaccaccacacccagagtcaggtatggaaataaacctatagcatggattctttctatgcataatctcaaaatttaactacccaaataagtaagtttttaaaaactaatttaaaatttgccattgaggaaaatatcacctccatccttaattgtgactcctcatttcagctaaaaccttttctaatactttaaaaaaacaaaatgaaaaacaaactcctagataaagtcataaacactgaaatcagagatgtgattcttgttaaatgttagtttctctttctgaggttacactctgtgcatttgaaactttgacgttaacatcttccgaatgtttagatttgctcaagggttcagattctctggtcttctgccttgcattttcctccttcctttcctttgcaagcaatctatagttgatagcattgccaatgagcagccacacgcttgctgctaccacaatagccccacaggacatgtacatgtatttatattctccagttaaatccaccaatttacctgcaagaggagggccaagaagaactgggccacactccacaattgtgacaagtccgacggcactggaaaatcttggtgcacccacgaggtccatgagagtttcaaagagaacactgctaacactcccaaatccaaggccaaaaaatacagcatataataccaggcttgtgtagtcctgtgccagtgggcacaagaggtgacacactccattgaacatgattgcaaaactgaagaagtactgaattcgaggtcgaatatatttggagtttgcaattaatcctacagaaggcctagcaaacatatcaacgaaagccataacagatagcagaaaagctgccgagtactcatcaattccttggtctttagcatatggagccaagaatataatgggggcaaaaaaacctaggaacataatgacatttccagacagatatatcagaaatcctctatgcttaaaaagggagaaatctaaatacttattaactttttcccaagttgatttcttcgttttgattttctttgggcttgaatcatcttctgttttgccagtcttatttttagacttagaagtggtttgattgggtccaaggggtctcatgagggaaccagccacacaggcattcaaaagtagacttcccaaaatcaggaagcttcctttccagccaaaagtattaaaaaggtactgattgaaaggagccaatgaacttaagaaaacaggacttcctgccatggccaatccatttgccatgggtcgcttcctatagaagtatttgccaattatggttaaggcgggttgcaggttgaaggctaaacctaaacctgtaatgaatcccatagtgaggtacagctgtaccacgctgctactaaaggaggccaacaccattccaagacagcataataagcctcctgctatcaccaccggccggctgccgtatttattcaccaaaacactacttacaggacctcctgcgtacataacagccagcataatggatgaaatccatgctatttcactgtaggtagtgtggaatatttgctgaatttctttgaagaatacggtgacagctttggggaatgcataggaaaatccaatggagataaaagctgctccaaccacaatccaaccccatcctccatctggaggtggatgcacaggtggggcacttggcattggtggcatttctgctcctctagtggaaattcaagtaacctgaatagagagagaacctgcgtttgacacttttctccaggctcagggctaagaagagaggcaactgatc

SEQ ID NO: 17832 - RNA, 11011 nt, Homo sapiens
  source 1..11011: mol_type = other RNA
tcgaggagctcacagtctagtaagaaagagatgaatttgaaaatatatttgaaactgtaggcaaaataagtaccctcacagagaaattcaacatttggtttcaaatttgttatgcagtgaaaattagaaactacaaccaagatttttttaaaacattatgttcatataacgctgtagtatacctgaaaggcaagaacttaaacaagtgtgctgaaaaacaaattaggaatatttgaacaaaatatactttaaaaatgatcaacaacgtaaaatattcctgatttaaataaatctaagttattttatttagtttaagcaaaatatgtatccatatgaaaatgccagttctttcatttttggttaattcctttacacatattatttgctaagttcagaaatgctatatatacaaaaatttcaaaaataaataagtatcccaagatcacataacaatactttaagtacattcatgtgtaagaaggcaaaaaaagaaggttctatcttatattttaaaactttgacaggtattttaaatgtattattttatactttattttctttaaaaatgaaataatacagccatgatttaagtcatgtaaaaacaactgtttggatcatttaggtgtcaagcaaaactatcctctttatttcactatcatagtaaccatagttgatagaccatgtggcaatatgatcatttgttcagtggtcattaagatatctatagaataaacaagacaactacattttatttttttcacttaaaaatcacaaaaatacagcctaaaatataatttatattttaaaaataattctaaacattaacccctaaatctaatcccttaaaaaattcttgcaaaagttagctggatgtggctgttgccaaggaatgtcttttattagcaacaagtgactatctataacttttattccaacaatcttattttaaatatttgtttcaatttaatgctgggattagaaaaacatatttgttcaaagtatgtaagtagtaagtaaaacaatttcaaaaatctatcaaaaaaggagaattattcattctaggaaataattaacatactggtttaaaatatctgggagaagaacttttacataaaaagcttcaaatttagtcagttgtagcaagcacttgaaaagaccctgctctttcatctgcaatatcaggaattactatatctgactcatatttgattaagttacaatctcatttttgttgtcactacaaagaaggatccttatattagtaaatgcactcactgcaactactgaggcctgcctcctgtcagaatgacaatgcagtcttagcatacgggtgtcggtttggctgaatctaaccaaacacatcacgtactacagatgtttttagggcccacccaattcataaaagattttactgcgatacatgagtttacccaaatttttattaaaatgtgtttttagggtaaatatcttgatgaactaggcaaacaaatactgaatgcagattactgtttttacagttttaccgggaaaactcctaatagcaacccctcttccccttcaccacagatctttaatttaggtgtgatttttgtttgttctctacatgggaataaaggagaaagtttagaaagactgtatctagctagataagatgcagaggtagatggaatctctaacataaaagaagctctaattacactgttgccagacagctgttatggattttagtattgtttattaggtgaagaaaacattcataaaataagaaatttttgagatagaacttactctaataatttcattaacatatgttcaggttcttagatcaagaaatactgtagaggtgttctcctcaagactatgctatggcaataatttcttgcatacaatttaataatttaaacttgaactgtgtgttctgtgctctggcgttctacttcagaaaaaaatgaacactgcttctaaaataaaaaggaacataaaataaaaaaggaattaatgagatattgacatgttttctattaatacaatattgatgttttaaatgattttgatattgctataacaacatatattgtgcaaaataattaatctcactaaatattatttctgatttgccacgaattatctgccgtggcaatcaggaaatagtcttcaaagtaagtttgcaaacatgattttgcaaaccatgattggaaaaatatattcatttgggctataaactatcaagtagggttgttatatatatttctaggaaaatattttatttactctacaaagatcatcattatgaccttacggcttctgtagtgcaatggagaaaaaagtgtgttagaagttaaaagacctgaattctatctccaaccctgcatttattcagagtattggtataggtttaggcaaaatccttaatccagtctagttttatatggtaaaaatgtggatacctatcaaaactgagggttgagaggatgaaatgaattcattaaacatatcttctgagacataaatatatcaaaacaaatcaaaatacaattagatctaatgtttagaaataaatattttaattcatatttgctatttcactaaatctagaaatactaatgctttagttaaatatagaaagttgatgatagaaaaataaaatccatcgtaccattgaaaagcttgtcagaaatatgtactcttgagattcggaggatgagaaaaaaaatgtgtactctaacgaggaagctatataaactgagtctaactcaaaacatttattttagatgcatataagaattaaagtcttagtcaaaagaatgttttaaaatttcatcctaaatttatgtgagataaaatgccattcttttgtttttctgaacagaggagcttttatcaacttattctattttatttttatttttattattttattttattttatttattattattatactttaagttttagggtacatgtgcacaatgtgcaggttagttacatatgtatacatgtgccatgctggtgcgctgcacccactaactcgtcacctagcattaggtatatctcccaatgctatccctcccccctcccccgaccccaccacagtccccagagtgtgatgttccccttcctgtgtccatgtgttctcattgttcagttcccacctatgagtgagaatatgcggtgtttggttttttgttcttgcgatagtttactgagaatgatgatttctaatttcatccatgtccctacacgaacttattctattttaatagaatgttcagtatcagtgttttcacactgagattctctagcttattttgccatatttaaattaaaaagaaacaaaaaatcctgtttgatcatgtgaaaaatatttactgaaatgtgaataaatttatgatcattaattgcctactgaaatattcctgaatattgctcaccttattaacaagtatatatggagactgaaaaacatgtagatcatgcaaacaagtgtaactaactataccaaagaaacaaaagtccatactaaatatgtccataattaaataaaaaatgctaaacaagttttacctagatattataaaaacatagaaaggaaaacatttaggagatgatgaagaagcaggagattgggatgggagatgtaatttgatctaaattcccatatgcttctgtaaaatcaaaaattcattttgcaatattaattttgctcttaaggtagagacttttaaaatgaccattctcaatactacagcaattcttccctgatttgcacataaatgaattaaagtgaagaaaaagcagtagaggagagaagactaaaataaaccagattgtagcaccctgtaaagagctaaaatctccagtgtacaaacaactgataggaaagaagagaaaatcagaactataaaaaagtgacataagctcagaaaattactcatttttaattgtatcaacaaagataatttgtaattttgatcatgcaagcattataattactgataattgggcctttcagcttttaagtgccttctcaaacatgagttctgcatatggttgtgcagaaatcaaaatcttaaagagagatgagtaaagtcaagtttgtaatattaatcttatattctcaatatagatgctaattagtgctctgaatggttgtggttagaaatcttgttggtatgatgtatcagtgatgtcactgcattgatggagacagaataatacataatggtgcaatgtggtgatggtaagctttgttactcaatattgtcaggcactttaagaaaatcagaaacattcaggatagtgccaaagaagatcagtttttcaagactctaaaatcatattcaattatatgtgtatgtaattataaatatgtgcatcatggctgactttgagaagaatgcagcgccttgcaagtgcactatttgaatagagctaaggagaactatagtctaaggactgcaaaagtctagatggagaagacaaaagcaatgacacttgttttctctacagaacaaatagacaaagaggtgaatgacaacaaagatgttcagagaaacttgaaaaataagctacggtgtagggtaagttgtattaaatgatgaaaattaatatgtaactgtatgggtaaaccaaatcatttgtatcttataatcttttttttggtagctacggataatattataaatggaataatcactaaaattctaaatataatgttttctagtaagaacattttattttttttttaatagagacagattctcactctattgcctaggctggactgcaagtggggccattatagctcactgaagcctcaacttcctgggctcaaatgaccctctcgtctcagcctcccgagtagctgggactacaggtgcacatcaccacatccaggtaattattttactttttgaatcatgatatgtagcaaccaatctgggaattatttattcataaaagataacattttcctgctaactccaacctcagaaaaaatgtattatgcctgactcaaatatgtcattatttttatgagaaaaagagtcatattgaagtaattatgtctatatgtaataattatcattatttgagataatttgcattggggagaaaagcaggcaatcagaaattacatattcaaggctgggcgcagtggctcacgcctgtaatcccagcactttgggaggcagaggcgagtgaatcacctgaggtcagagttcaagaccagcctgaccaacaaggagaaaccccatctctactaaaacaaaacaaaacaaaacaaaacaaaaaaagccacaaaattagccgggcatggtggcacatgcctgtaattccagttactcgggaggctgaggcaggagaattgcttgaacctgggaggcagaggttgtagtaagccgagattgtgccactgcacgccagcctgggcgacaagaacgagactcagtctcaaaaaaaaaaaaaaagaaagaaagaaagaaattacatattcaggttctagcaaatgcagttctctaataaacactaaataaatcataatacaagttacagttaaacctaattgttttactatataggatgtatcttttttgtacctatattttatcttcctttgcttctctggcctctattgggaggcagcacggtagtgaacacctcggggatctttctggttacgtaaacctgagttttaattttggttcatactaccttttaactttgggtagtctgctgagcttgttttttgttttcactcatctgtcatatcaagctagtaataattctgccatggttttggttttcatattgaaaggcattacataagcaaaatgcataacatataaatattagttccctttccactatgcatccaatctccctattaaattaagcctaaaaataataatttttgttttattaaaagccttccacattctacatatgaaagggattttttaaaggtgttttagataaaaaatgtttcaaccaactgaccaagaatatctcttcatatttatgtcatctacataaaaacttacatttatatcatatatcttttagtcttcttttctatattcttgattgtcatgttgtacagccagaaaagaatgagtataaattatctagattttttaaagtgcacattcaaacatagaaaatctaattattttacttgtttcttagtattaggctgaggccaatgagtccatgagctaaagggttgaaacttggcaccaaaaaagtgattgtttatgagtcctgtagatttatactgagaaaacatcatgtcttccaatgtgaaatacactaaaacctgattttttgtctcttaaggtgtgctaggtgaatgcaaaaaggatcaggaaagggggtgaggataggtcaggaaaagtgcaaacacaatgttctattcataaattagtgatggcatatttaaggttaagtagtaaaaaatatggggggctcagttaacacgaatgaaaaaatagttaaagtagccatgaattatctggataccttgatttaatgacaccctttcttctgtacaatttcataatgtgggaatagagattagtggggattgtagtggtataccctgactttgcttcatgatatctcaaatgtttaaaacctattattccctagagaaagaaatatgttcatactaattgttgcagaggcagaagccaaatatatctcctcctccatttatgtgactatatagtaatgaaaatcctaggttgatacacttttctcaatcttggaaagattctgctaaagcagcaaatcttctaacaagttcaagagggtggggagagtgaacaagtagaataatttatattaccctggaacaattctgaatcctgtaggtatttatgtcactgtttcaattgtgttctggtttaactgtcaatatttatgcatagcagttaacgtgtgtgcatatttgtaactgtgcagtgctactgccaggtgtgactgtacaaatcatgtgctttgaatgtgcaagttttactttcttttctaacaatttaatacagtgttagaaataaataacgaatgaagacaaccaaagagcagccagacaaatgtgaactggttttgacgtgacgagaaactcatcagtaagtaaataaacctcctccctggagaaggccactgaaatgcacccaggaggatgtctctactagaaggtaataaaaaatatatataatgtagtctttgacctaaaacctcatgattattactttgccatttatttccccctggtatctgatgttcatattagtttaatgtgccttttcagagaattcaagacactttttggaaagtagaatttttttttgaaaatttatgattggagaggtactacacaatttagaggttacatttcttgacaaatctgagttgaataaaaaagaactaaaaatataaacatagctaattcaagaatcaagatcgggtgaaactaaattaaaaacagccataaagtcccacattttccctaatttatttacctatgatattggcacatcttgttttacttaacatttgaaaaatacaaatatctcttcatatgcaaaagagcaaatgttaaatgaaaaactgaattttatatagcttcctaaatatgagccacatgcttaagcagtgaattaactttatgaatcaaatgtttaatgttaactattacaaaagcctggtatccaggtgcaatctcaccagaaaaaaatagcacctgcctttattacaataaaaaaaatggctaattccctttgacatcttaagagtgacactactttgtcaagcactaaatactttttaaattaatcatgttaaacttcagatttatagatataaatattgtatttataactttagtcataatgtacaatttctttcttgtttaaaagtactttctcactcaaaatggtatttatagtttaaaaagaatatgcctctgtattcaggagtgattcaaattcccagatgttttcacatagttatgaaaatgggaaagtgctgaattaaactgggctgcaatatttcaagttttttgctatcaggttataaactatacctacgattgcaagtcatacagtgcctctatttctagaaggcttttaaagtttcctggcttagttatgtccaaaggcagcaggaagtctcatcagtagagggcagaattttcaagtgctgccattcttatcccaggaggcatttccagtggttgagcacaaggcctgtttgtagtttgcttttgctcttgcattttgtggaagggaaggaactgagagagcttagagggttcattaaaaccacccctcactctcttagtcgtagtcagatggagtattcataacagtaacctccaattaccactatgtgttgggaaaaattagaattcggtctacttacaatcctgccaactaggattttactttgatatttcagtataacagtgaatctggattgatgcctgattaaaataaaatccctgattattactttctggattacgaactaaaatccctgtaaaatcaatggatgtgactcattgttaagagtcatgcagacttttacatattaggtaagaattctaaaaattatttgagggttctattctctagcaccaggtactaatgctccctactcaaaaaaaatcatgtgcatggattaatcaagtctaacagtgctcagatttaatggtttaacattgattttcttttctttgtcaaacttatatatgcaaatatttttatagtagtcagatgttatttttgaataaggatcaccctcatttttacccatgtgcttatctttaaaaccaacattgtaaagtagcacgcagacatatgtttcttttatcttcatggattatttttaccttaaaaataaattatcatttttttttttgaatttgggttttattctccagatactctgtgtacatgtgggtaagtatgtgggagtatgtgtgtttgtgtgtaagaggggataattaattgtctctcaactctatctcatactttaatatcaaataaaaaatgaaatgtataaagggtcactttgtaggattaggcatcctccttctacctacttaaaccaggggtttgggattcagaattctccatataaccaagaccgaaagtcactggaagactttaaaattagtattttaaccaccacacccagagtcaggtatggaaataaacctatagcatggattctttctatgcataatctcaaaatttaactacccaaataagtaagtttttaaaaactaatttaaaatttgccattgaggaaaatatcacctccatccttaattgtgactcctcatttcagctaaaaccttttctaatactttaaaaaaacaaaatgaaaaacaaactcctagataaagtcataaacactgaaatcagagatgtgattcttgttaaatgttagtttctctttctgaggttacactctgtgcatttgaaactttgacgttaacatcttccgaatgtttagatttgctcaagggttcagattctctggtcttctgccttgcattttcctccttcctttcctttgcaagcaatctatagttgatagcattgccaatgagcagccacacgcttgctgctaccacaatagccccacaggacatgtacatgtatttatattctccagttaaatccaccaatttacctgcaagaggagggccaagaagaactgggccacactccacaattgtgacaagtccgacggcactggaaaatcttggtgcacccacgaggtccatgagagtttcaaagagaacactgctaacactcccaaatccaaggccaaaaaatacagcatataataccaggcttgtgtagtcctgtgccagtgggcacaagaggtgacacactccattgaacatgattgcaaaactgaagaagtactgaattcgaggtcgaatatatttggagtttgcaattaatcctacagaaggcctagcaaacatatcaacgaaagccataacagatagcagaaaagctgccgagtactcatcaattccttggtctttagcatatggagccaagaatataatgggggcaaaaaaacctaggaacataatgacatttccagacagatatatcagaaatcctctatgcttaaaaagggagaaatctaaatacttattaactttttcccaagttgatttcttcgttttgattttctttgggcttgaatcatcttctgttttgccagtcttatttttagacttagaagtggtttgattgggtccaaggggtctcatgagggaaccagccacacaggcattcaaaagtagacttcccaaaatcaggaagcttcctttccagccaaaagtattaaaaaggtactgattgaaaggagccaatgaacttaagaaaacaggacttcctgccatggccaatccatttgccatgggtcgcttcctatagaagtatttgccaattatggttaaggcgggttgcaggttgaaggctaaacctaaacctgtaatgaatcccatagtgaggtacagctgtaccacgctgctactaaaggaggccaacaccattccaagacagcataataagcctcctgctatcaccaccggccggctgccgtatttattcaccaaaacactacttacaggacctcctgcgtacataacagccagcataatggatgaaatccatgctatttcactgtaggtagtgtggaatatttgctgaatttctttgaagaatacggtgacagctttggggaatgcataggaaaatccaatggagataaaagctgctccaaccacaatccaaccccatcctccatctggaggtggatgcacaggtggggcacttggcattggtggcatttctgctcctctagtggaaattcaagtaacctggcgacaggtgtttagaaacatggtcttccatttcaccaagacataagtttccctgatctatggactcctctccccacctgaggcagaagtttccttgt

SEQ ID NO: 17833 - RNA, 11287 nt, Homo sapiens
  source 1..11287: mol_type = other RNA
tcgaggagctcacagtctagtaagaaagagatgaatttgaaaatatatttgaaactgtaggcaaaataagtaccctcacagagaaattcaacatttggtttcaaatttgttatgcagtgaaaattagaaactacaaccaagatttttttaaaacattatgttcatataacgctgtagtatacctgaaaggcaagaacttaaacaagtgtgctgaaaaacaaattaggaatatttgaacaaaatatactttaaaaatgatcaacaacgtaaaatattcctgatttaaataaatctaagttattttatttagtttaagcaaaatatgtatccatatgaaaatgccagttctttcatttttggttaattcctttacacatattatttgctaagttcagaaatgctatatatacaaaaatttcaaaaataaataagtatcccaagatcacataacaatactttaagtacattcatgtgtaagaaggcaaaaaaagaaggttctatcttatattttaaaactttgacaggtattttaaatgtattattttatactttattttctttaaaaatgaaataatacagccatgatttaagtcatgtaaaaacaactgtttggatcatttaggtgtcaagcaaaactatcctctttatttcactatcatagtaaccatagttgatagaccatgtggcaatatgatcatttgttcagtggtcattaagatatctatagaataaacaagacaactacattttatttttttcacttaaaaatcacaaaaatacagcctaaaatataatttatattttaaaaataattctaaacattaacccctaaatctaatcccttaaaaaattcttgcaaaagttagctggatgtggctgttgccaaggaatgtcttttattagcaacaagtgactatctataacttttattccaacaatcttattttaaatatttgtttcaatttaatgctgggattagaaaaacatatttgttcaaagtatgtaagtagtaagtaaaacaatttcaaaaatctatcaaaaaaggagaattattcattctaggaaataattaacatactggtttaaaatatctgggagaagaacttttacataaaaagcttcaaatttagtcagttgtagcaagcacttgaaaagaccctgctctttcatctgcaatatcaggaattactatatctgactcatatttgattaagttacaatctcatttttgttgtcactacaaagaaggatccttatattagtaaatgcactcactgcaactactgaggcctgcctcctgtcagaatgacaatgcagtcttagcatacgggtgtcggtttggctgaatctaaccaaacacatcacgtactacagatgtttttagggcccacccaattcataaaagattttactgcgatacatgagtttacccaaatttttattaaaatgtgtttttagggtaaatatcttgatgaactaggcaaacaaatactgaatgcagattactgtttttacagttttaccgggaaaactcctaatagcaacccctcttccccttcaccacagatctttaatttaggtgtgatttttgtttgttctctacatgggaataaaggagaaagtttagaaagactgtatctagctagataagatgcagaggtagatggaatctctaacataaaagaagctctaattacactgttgccagacagctgttatggattttagtattgtttattaggtgaagaaaacattcataaaataagaaatttttgagatagaacttactctaataatttcattaacatatgttcaggttcttagatcaagaaatactgtagaggtgttctcctcaagactatgctatggcaataatttcttgcatacaatttaataatttaaacttgaactgtgtgttctgtgctctggcgttctacttcagaaaaaaatgaacactgcttctaaaataaaaaggaacataaaataaaaaaggaattaatgagatattgacatgttttctattaatacaatattgatgttttaaatgattttgatattgctataacaacatatattgtgcaaaataattaatctcactaaatattatttctgatttgccacgaattatctgccgtggcaatcaggaaatagtcttcaaagtaagtttgcaaacatgattttgcaaaccatgattggaaaaatatattcatttgggctataaactatcaagtagggttgttatatatatttctaggaaaatattttatttactctacaaagatcatcattatgaccttacggcttctgtagtgcaatggagaaaaaagtgtgttagaagttaaaagacctgaattctatctccaaccctgcatttattcagagtattggtataggtttaggcaaaatccttaatccagtctagttttatatggtaaaaatgtggatacctatcaaaactgagggttgagaggatgaaatgaattcattaaacatatcttctgagacataaatatatcaaaacaaatcaaaatacaattagatctaatgtttagaaataaatattttaattcatatttgctatttcactaaatctagaaatactaatgctttagttaaatatagaaagttgatgatagaaaaataaaatccatcgtaccattgaaaagcttgtcagaaatatgtactcttgagattcggaggatgagaaaaaaaatgtgtactctaacgaggaagctatataaactgagtctaactcaaaacatttattttagatgcatataagaattaaagtcttagtcaaaagaatgttttaaaatttcatcctaaatttatgtgagataaaatgccattcttttgtttttctgaacagaggagcttttatcaacttattctattttatttttatttttattattttattttattttatttattattattatactttaagttttagggtacatgtgcacaatgtgcaggttagttacatatgtatacatgtgccatgctggtgcgctgcacccactaactcgtcacctagcattaggtatatctcccaatgctatccctcccccctcccccgaccccaccacagtccccagagtgtgatgttccccttcctgtgtccatgtgttctcattgttcagttcccacctatgagtgagaatatgcggtgtttggttttttgttcttgcgatagtttactgagaatgatgatttctaatttcatccatgtccctacacgaacttattctattttaatagaatgttcagtatcagtgttttcacactgagattctctagcttattttgccatatttaaattaaaaagaaacaaaaaatcctgtttgatcatgtgaaaaatatttactgaaatgtgaataaatttatgatcattaattgcctactgaaatattcctgaatattgctcaccttattaacaagtatatatggagactgaaaaacatgtagatcatgcaaacaagtgtaactaactataccaaagaaacaaaagtccatactaaatatgtccataattaaataaaaaatgctaaacaagttttacctagatattataaaaacatagaaaggaaaacatttaggagatgatgaagaagcaggagattgggatgggagatgtaatttgatctaaattcccatatgcttctgtaaaatcaaaaattcattttgcaatattaattttgctcttaaggtagagacttttaaaatgaccattctcaatactacagcaattcttccctgatttgcacataaatgaattaaagtgaagaaaaagcagtagaggagagaagactaaaataaaccagattgtagcaccctgtaaagagctaaaatctccagtgtacaaacaactgataggaaagaagagaaaatcagaactataaaaaagtgacataagctcagaaaattactcatttttaattgtatcaacaaagataatttgtaattttgatcatgcaagcattataattactgataattgggcctttcagcttttaagtgccttctcaaacatgagttctgcatatggttgtgcagaaatcaaaatcttaaagagagatgagtaaagtcaagtttgtaatattaatcttatattctcaatatagatgctaattagtgctctgaatggttgtggttagaaatcttgttggtatgatgtatcagtgatgtcactgcattgatggagacagaataatacataatggtgcaatgtggtgatggtaagctttgttactcaatattgtcaggcactttaagaaaatcagaaacattcaggatagtgccaaagaagatcagtttttcaagactctaaaatcatattcaattatatgtgtatgtaattataaatatgtgcatcatggctgactttgagaagaatgcagcgccttgcaagtgcactatttgaatagagctaaggagaactatagtctaaggactgcaaaagtctagatggagaagacaaaagcaatgacacttgttttctctacagaacaaatagacaaagaggtgaatgacaacaaagatgttcagagaaacttgaaaaataagctacggtgtagggtaagttgtattaaatgatgaaaattaatatgtaactgtatgggtaaaccaaatcatttgtatcttataatcttttttttggtagctacggataatattataaatggaataatcactaaaattctaaatataatgttttctagtaagaacattttattttttttttaatagagacagattctcactctattgcctaggctggactgcaagtggggccattatagctcactgaagcctcaacttcctgggctcaaatgaccctctcgtctcagcctcccgagtagctgggactacaggtgcacatcaccacatccaggtaattattttactttttgaatcatgatatgtagcaaccaatctgggaattatttattcataaaagataacattttcctgctaactccaacctcagaaaaaatgtattatgcctgactcaaatatgtcattatttttatgagaaaaagagtcatattgaagtaattatgtctatatgtaataattatcattatttgagataatttgcattggggagaaaagcaggcaatcagaaattacatattcaaggctgggcgcagtggctcacgcctgtaatcccagcactttgggaggcagaggcgagtgaatcacctgaggtcagagttcaagaccagcctgaccaacaaggagaaaccccatctctactaaaacaaaacaaaacaaaacaaaacaaaaaaagccacaaaattagccgggcatggtggcacatgcctgtaattccagttactcgggaggctgaggcaggagaattgcttgaacctgggaggcagaggttgtagtaagccgagattgtgccactgcacgccagcctgggcgacaagaacgagactcagtctcaaaaaaaaaaaaaaagaaagaaagaaagaaattacatattcaggttctagcaaatgcagttctctaataaacactaaataaatcataatacaagttacagttaaacctaattgttttactatataggatgtatcttttttgtacctatattttatcttcctttgcttctctggcctctattgggaggcagcacggtagtgaacacctcggggatctttctggttacgtaaacctgagttttaattttggttcatactaccttttaactttgggtagtctgctgagcttgttttttgttttcactcatctgtcatatcaagctagtaataattctgccatggttttggttttcatattgaaaggcattacataagcaaaatgcataacatataaatattagttccctttccactatgcatccaatctccctattaaattaagcctaaaaataataatttttgttttattaaaagccttccacattctacatatgaaagggattttttaaaggtgttttagataaaaaatgtttcaaccaactgaccaagaatatctcttcatatttatgtcatctacataaaaacttacatttatatcatatatcttttagtcttcttttctatattcttgattgtcatgttgtacagccagaaaagaatgagtataaattatctagattttttaaagtgcacattcaaacatagaaaatctaattattttacttgtttcttagtattaggctgaggccaatgagtccatgagctaaagggttgaaacttggcaccaaaaaagtgattgtttatgagtcctgtagatttatactgagaaaacatcatgtcttccaatgtgaaatacactaaaacctgattttttgtctcttaaggtgtgctaggtgaatgcaaaaaggatcaggaaagggggtgaggataggtcaggaaaagtgcaaacacaatgttctattcataaattagtgatggcatatttaaggttaagtagtaaaaaatatggggggctcagttaacacgaatgaaaaaatagttaaagtagccatgaattatctggataccttgatttaatgacaccctttcttctgtacaatttcataatgtgggaatagagattagtggggattgtagtggtataccctgactttgcttcatgatatctcaaatgtttaaaacctattattccctagagaaagaaatatgttcatactaattgttgcagaggcagaagccaaatatatctcctcctccatttatgtgactatatagtaatgaaaatcctaggttgatacacttttctcaatcttggaaagattctgctaaagcagcaaatcttctaacaagttcaagagggtggggagagtgaacaagtagaataatttatattaccctggaacaattctgaatcctgtaggtatttatgtcactgtttcaattgtgttctggtttaactgtcaatatttatgcatagcagttaacgtgtgtgcatatttgtaactgtgcagtgctactgccaggtgtgactgtacaaatcatgtgctttgaatgtgcaagttttactttcttttctaacaatttaatacagtgttagaaataaataacgaatgaagacaaccaaagagcagccagacaaatgtgaactggttttgacgtgacgagaaactcatcagtaagtaaataaacctcctccctggagaaggccactgaaatgcacccaggaggatgtctctactagaaggtaataaaaaatatatataatgtagtctttgacctaaaacctcatgattattactttgccatttatttccccctggtatctgatgttcatattagtttaatgtgccttttcagagaattcaagacactttttggaaagtagaatttttttttgaaaatttatgattggagaggtactacacaatttagaggttacatttcttgacaaatctgagttgaataaaaaagaactaaaaatataaacatagctaattcaagaatcaagatcgggtgaaactaaattaaaaacagccataaagtcccacattttccctaatttatttacctatgatattggcacatcttgttttacttaacatttgaaaaatacaaatatctcttcatatgcaaaagagcaaatgttaaatgaaaaactgaattttatatagcttcctaaatatgagccacatgcttaagcagtgaattaactttatgaatcaaatgtttaatgttaactattacaaaagcctggtatccaggtgcaatctcaccagaaaaaaatagcacctgcctttattacaataaaaaaaatggctaattccctttgacatcttaagagtgacactactttgtcaagcactaaatactttttaaattaatcatgttaaacttcagatttatagatataaatattgtatttataactttagtcataatgtacaatttctttcttgtttaaaagtactttctcactcaaaatggtatttatagtttaaaaagaatatgcctctgtattcaggagtgattcaaattcccagatgttttcacatagttatgaaaatgggaaagtgctgaattaaactgggctgcaatatttcaagttttttgctatcaggttataaactatacctacgattgcaagtcatacagtgcctctatttctagaaggcttttaaagtttcctggcttagttatgtccaaaggcagcaggaagtctcatcagtagagggcagaattttcaagtgctgccattcttatcccaggaggcatttccagtggttgagcacaaggcctgtttgtagtttgcttttgctcttgcattttgtggaagggaaggaactgagagagcttagagggttcattaaaaccacccctcactctcttagtcgtagtcagatggagtattcataacagtaacctccaattaccactatgtgttgggaaaaattagaattcggtctacttacaatcctgccaactaggattttactttgatatttcagtataacagtgaatctggattgatgcctgattaaaataaaatccctgattattactttctggattacgaactaaaatccctgtaaaatcaatggatgtgactcattgttaagagtcatgcagacttttacatattaggtaagaattctaaaaattatttgagggttctattctctagcaccaggtactaatgctccctactcaaaaaaaatcatgtgcatggattaatcaagtctaacagtgctcagatttaatggtttaacattgattttcttttctttgtcaaacttatatatgcaaatatttttatagtagtcagatgttatttttgaataaggatcaccctcatttttacccatgtgcttatctttaaaaccaacattgtaaagtagcacgcagacatatgtttcttttatcttcatggattatttttaccttaaaaataaattatcatttttttttttgaatttgggttttattctccagatactctgtgtacatgtgggtaagtatgtgggagtatgtgtgtttgtgtgtaagaggggataattaattgtctctcaactctatctcatactttaatatcaaataaaaaatgaaatgtataaagggtcactttgtaggattaggcatcctccttctacctacttaaaccaggggtttgggattcagaattctccatataaccaagaccgaaagtcactggaagactttaaaattagtattttaaccaccacacccagagtcaggtatggaaataaacctatagcatggattctttctatgcataatctcaaaatttaactacccaaataagtaagtttttaaaaactaatttaaaatttgccattgaggaaaatatcacctccatccttaattgtgactcctcatttcagctaaaaccttttctaatactttaaaaaaacaaaatgaaaaacaaactcctagataaagtcataaacactgaaatcagagatgtgattcttgttaaatgttagtttctctttctgaggttacactctgtgcatttgaaactttgacgttaacatcttccgaatgtttagatttgctcaagggttcagattctctggtcttctgccttgcattttcctccttcctttcctttgcaagcaatctatagttgatagcattgccaatgagcagccacacgcttgctgctaccacaatagccccacaggacatgtacatgtatttatattctccagttaaatccaccaatttacctgcaagaggagggccaagaagaactgggccacactccacaattgtgacaagtccgacggcactggaaaatcttggtgcacccacgaggtccatgagagtttcaaagagaacactgctaacactcccaaatccaaggccaaaaaatacagcatataataccaggcttgtgtagtcctgtgccagtgggcacaagaggtgacacactccattgaacatgattgcaaaactgaagaagtactgaattcgaggtcgaatatatttggagtttgcaattaatcctacagaaggcctagcaaacatatcaacgaaagccataacagatagcagaaaagctgccgagtactcatcaattccttggtctttagcatatggagccaagaatataatgggggcaaaaaaacctaggaacataatgacatttccagacagatatatcagaaatcctctatgcttaaaaagggagaaatctaaatacttattaactttttcccaagttgatttcttcgttttgattttctttgggcttgaatcatcttctgttttgccagtcttatttttagacttagaagtggtttgattgggtccaaggggtctcatgagggaaccagccacacaggcattcaaaagtagacttcccaaaatcaggaagcttcctttccagccaaaagtattaaaaaggtactgattgaaaggagccaatgaacttaagaaaacaggacttcctgccatggccaatccatttgccatgggtcgcttcctatagaagtatttgccaattatggttaaggcgggttgcaggttgaaggctaaacctaaacctgtaatgaatcccatagtgaggtacagctgtaccacgctgctactaaaggaggccaacaccattccaagacagcataataagcctcctgctatcaccaccggccggctgccgtatttattcaccaaaacactacttacaggacttcactgaagtcctgagcctcttaaagtcacccatgaggattgaaataaacttcttccaaacttctgttaatgttggtattttgacctcctcccataacagtgaatgatcgtgatgttatctagaatagcaaatcctttccagaagattttccatctccttttcccagattcatcagaggagtcattatgtacggcagctaggcatgatcctgattgagtaaagctgcactgaatcctcaaggatgtgaagatcaaaaagctttcaaatattctacctcctgcgtacataacagccagcataatggatgaaatccatgctatttcactgtaggtagtgtggaatatttgctgaatttctttgaagaatacggtgacagctttggggaatgcataggaaaatccaatggagataaaagctgctccaaccacaatccaaccccatcctccatctggaggtggatgcacaggtggggcacttggcattggtggcatttctgctcctctagtggaaattcaagtaacctggcgacaggtgtttagaaacatggtcttccatttcaccaagacataagtttccctgatctatggactcctctccccacctgaggcagaagtttccttgt

SEQ ID NO: 17834 - RNA, 11375 nt, Homo sapiens
  source 1..11375: mol_type = other RNA
tcgaggagctcacagtctagtaagaaagagatgaatttgaaaatatatttgaaactgtaggcaaaataagtaccctcacagagaaattcaacatttggtttcaaatttgttatgcagtgaaaattagaaactacaaccaagatttttttaaaacattatgttcatataacgctgtagtatacctgaaaggcaagaacttaaacaagtgtgctgaaaaacaaattaggaatatttgaacaaaatatactttaaaaatgatcaacaacgtaaaatattcctgatttaaataaatctaagttattttatttagtttaagcaaaatatgtatccatatgaaaatgccagttctttcatttttggttaattcctttacacatattatttgctaagttcagaaatgctatatatacaaaaatttcaaaaataaataagtatcccaagatcacataacaatactttaagtacattcatgtgtaagaaggcaaaaaaagaaggttctatcttatattttaaaactttgacaggtattttaaatgtattattttatactttattttctttaaaaatgaaataatacagccatgatttaagtcatgtaaaaacaactgtttggatcatttaggtgtcaagcaaaactatcctctttatttcactatcatagtaaccatagttgatagaccatgtggcaatatgatcatttgttcagtggtcattaagatatctatagaataaacaagacaactacattttatttttttcacttaaaaatcacaaaaatacagcctaaaatataatttatattttaaaaataattctaaacattaacccctaaatctaatcccttaaaaaattcttgcaaaagttagctggatgtggctgttgccaaggaatgtcttttattagcaacaagtgactatctataacttttattccaacaatcttattttaaatatttgtttcaatttaatgctgggattagaaaaacatatttgttcaaagtatgtaagtagtaagtaaaacaatttcaaaaatctatcaaaaaaggagaattattcattctaggaaataattaacatactggtttaaaatatctgggagaagaacttttacataaaaagcttcaaatttagtcagttgtagcaagcacttgaaaagaccctgctctttcatctgcaatatcaggaattactatatctgactcatatttgattaagttacaatctcatttttgttgtcactacaaagaaggatccttatattagtaaatgcactcactgcaactactgaggcctgcctcctgtcagaatgacaatgcagtcttagcatacgggtgtcggtttggctgaatctaaccaaacacatcacgtactacagatgtttttagggcccacccaattcataaaagattttactgcgatacatgagtttacccaaatttttattaaaatgtgtttttagggtaaatatcttgatgaactaggcaaacaaatactgaatgcagattactgtttttacagttttaccgggaaaactcctaatagcaacccctcttccccttcaccacagatctttaatttaggtgtgatttttgtttgttctctacatgggaataaaggagaaagtttagaaagactgtatctagctagataagatgcagaggtagatggaatctctaacataaaagaagctctaattacactgttgccagacagctgttatggattttagtattgtttattaggtgaagaaaacattcataaaataagaaatttttgagatagaacttactctaataatttcattaacatatgttcaggttcttagatcaagaaatactgtagaggtgttctcctcaagactatgctatggcaataatttcttgcatacaatttaataatttaaacttgaactgtgtgttctgtgctctggcgttctacttcagaaaaaaatgaacactgcttctaaaataaaaaggaacataaaataaaaaaggaattaatgagatattgacatgttttctattaatacaatattgatgttttaaatgattttgatattgctataacaacatatattgtgcaaaataattaatctcactaaatattatttctgatttgccacgaattatctgccgtggcaatcaggaaatagtcttcaaagtaagtttgcaaacatgattttgcaaaccatgattggaaaaatatattcatttgggctataaactatcaagtagggttgttatatatatttctaggaaaatattttatttactctacaaagatcatcattatgaccttacggcttctgtagtgcaatggagaaaaaagtgtgttagaagttaaaagacctgaattctatctccaaccctgcatttattcagagtattggtataggtttaggcaaaatccttaatccagtctagttttatatggtaaaaatgtggatacctatcaaaactgagggttgagaggatgaaatgaattcattaaacatatcttctgagacataaatatatcaaaacaaatcaaaatacaattagatctaatgtttagaaataaatattttaattcatatttgctatttcactaaatctagaaatactaatgctttagttaaatatagaaagttgatgatagaaaaataaaatccatcgtaccattgaaaagcttgtcagaaatatgtactcttgagattcggaggatgagaaaaaaaatgtgtactctaacgaggaagctatataaactgagtctaactcaaaacatttattttagatgcatataagaattaaagtcttagtcaaaagaatgttttaaaatttcatcctaaatttatgtgagataaaatgccattcttttgtttttctgaacagaggagcttttatcaacttattctattttatttttatttttattattttattttattttatttattattattatactttaagttttagggtacatgtgcacaatgtgcaggttagttacatatgtatacatgtgccatgctggtgcgctgcacccactaactcgtcacctagcattaggtatatctcccaatgctatccctcccccctcccccgaccccaccacagtccccagagtgtgatgttccccttcctgtgtccatgtgttctcattgttcagttcccacctatgagtgagaatatgcggtgtttggttttttgttcttgcgatagtttactgagaatgatgatttctaatttcatccatgtccctacacgaacttattctattttaatagaatgttcagtatcagtgttttcacactgagattctctagcttattttgccatatttaaattaaaaagaaacaaaaaatcctgtttgatcatgtgaaaaatatttactgaaatgtgaataaatttatgatcattaattgcctactgaaatattcctgaatattgctcaccttattaacaagtatatatggagactgaaaaacatgtagatcatgcaaacaagtgtaactaactataccaaagaaacaaaagtccatactaaatatgtccataattaaataaaaaatgctaaacaagttttacctagatattataaaaacatagaaaggaaaacatttaggagatgatgaagaagcaggagattgggatgggagatgtaatttgatctaaattcccatatgcttctgtaaaatcaaaaattcattttgcaatattaattttgctcttaaggtagagacttttaaaatgaccattctcaatactacagcaattcttccctgatttgcacataaatgaattaaagtgaagaaaaagcagtagaggagagaagactaaaataaaccagattgtagcaccctgtaaagagctaaaatctccagtgtacaaacaactgataggaaagaagagaaaatcagaactataaaaaagtgacataagctcagaaaattactcatttttaattgtatcaacaaagataatttgtaattttgatcatgcaagcattataattactgataattgggcctttcagcttttaagtgccttctcaaacatgagttctgcatatggttgtgcagaaatcaaaatcttaaagagagatgagtaaagtcaagtttgtaatattaatcttatattctcaatatagatgctaattagtgctctgaatggttgtggttagaaatcttgttggtatgatgtatcagtgatgtcactgcattgatggagacagaataatacataatggtgcaatgtggtgatggtaagctttgttactcaatattgtcaggcactttaagaaaatcagaaacattcaggatagtgccaaagaagatcagtttttcaagactctaaaatcatattcaattatatgtgtatgtaattataaatatgtgcatcatggctgactttgagaagaatgcagcgccttgcaagtgcactatttgaatagagctaaggagaactatagtctaaggactgcaaaagtctagatggagaagacaaaagcaatgacacttgttttctctacagaacaaatagacaaagaggtgaatgacaacaaagatgttcagagaaacttgaaaaataagctacggtgtagggtaagttgtattaaatgatgaaaattaatatgtaactgtatgggtaaaccaaatcatttgtatcttataatcttttttttggtagctacggataatattataaatggaataatcactaaaattctaaatataatgttttctagtaagaacattttattttttttttaatagagacagattctcactctattgcctaggctggactgcaagtggggccattatagctcactgaagcctcaacttcctgggctcaaatgaccctctcgtctcagcctcccgagtagctgggactacaggtgcacatcaccacatccaggtaattattttactttttgaatcatgatatgtagcaaccaatctgggaattatttattcataaaagataacattttcctgctaactccaacctcagaaaaaatgtattatgcctgactcaaatatgtcattatttttatgagaaaaagagtcatattgaagtaattatgtctatatgtaataattatcattatttgagataatttgcattggggagaaaagcaggcaatcagaaattacatattcaaggctgggcgcagtggctcacgcctgtaatcccagcactttgggaggcagaggcgagtgaatcacctgaggtcagagttcaagaccagcctgaccaacaaggagaaaccccatctctactaaaacaaaacaaaacaaaacaaaacaaaaaaagccacaaaattagccgggcatggtggcacatgcctgtaattccagttactcgggaggctgaggcaggagaattgcttgaacctgggaggcagaggttgtagtaagccgagattgtgccactgcacgccagcctgggcgacaagaacgagactcagtctcaaaaaaaaaaaaaaagaaagaaagaaagaaattacatattcaggttctagcaaatgcagttctctaataaacactaaataaatcataatacaagttacagttaaacctaattgttttactatataggatgtatcttttttgtacctatattttatcttcctttgcttctctggcctctattgggaggcagcacggtagtgaacacctcggggatctttctggttacgtaaacctgagttttaattttggttcatactaccttttaactttgggtagtctgctgagcttgttttttgttttcactcatctgtcatatcaagctagtaataattctgccatggttttggttttcatattgaaaggcattacataagcaaaatgcataacatataaatattagttccctttccactatgcatccaatctccctattaaattaagcctaaaaataataatttttgttttattaaaagccttccacattctacatatgaaagggattttttaaaggtgttttagataaaaaatgtttcaaccaactgaccaagaatatctcttcatatttatgtcatctacataaaaacttacatttatatcatatatcttttagtcttcttttctatattcttgattgtcatgttgtacagccagaaaagaatgagtataaattatctagattttttaaagtgcacattcaaacatagaaaatctaattattttacttgtttcttagtattaggctgaggccaatgagtccatgagctaaagggttgaaacttggcaccaaaaaagtgattgtttatgagtcctgtagatttatactgagaaaacatcatgtcttccaatgtgaaatacactaaaacctgattttttgtctcttaaggtgtgctaggtgaatgcaaaaaggatcaggaaagggggtgaggataggtcaggaaaagtgcaaacacaatgttctattcataaattagtgatggcatatttaaggttaagtagtaaaaaatatggggggctcagttaacacgaatgaaaaaatagttaaagtagccatgaattatctggataccttgatttaatgacaccctttcttctgtacaatttcataatgtgggaatagagattagtggggattgtagtggtataccctgactttgcttcatgatatctcaaatgtttaaaacctattattccctagagaaagaaatatgttcatactaattgttgcagaggcagaagccaaatatatctcctcctccatttatgtgactatatagtaatgaaaatcctaggttgatacacttttctcaatcttggaaagattctgctaaagcagcaaatcttctaacaagttcaagagggtggggagagtgaacaagtagaataatttatattaccctggaacaattctgaatcctgtaggtatttatgtcactgtttcaattgtgttctggtttaactgtcaatatttatgcatagcagttaacgtgtgtgcatatttgtaactgtgcagtgctactgccaggtgtgactgtacaaatcatgtgctttgaatgtgcaagttttactttcttttctaacaatttaatacagtgttagaaataaataacgaatgaagacaaccaaagagcagccagacaaatgtgaactggttttgacgtgacgagaaactcatcagtaagtaaataaacctcctccctggagaaggccactgaaatgcacccaggaggatgtctctactagaaggtaataaaaaatatatataatgtagtctttgacctaaaacctcatgattattactttgccatttatttccccctggtatctgatgttcatattagtttaatgtgccttttcagagaattcaagacactttttggaaagtagaatttttttttgaaaatttatgattggagaggtactacacaatttagaggttacatttcttgacaaatctgagttgaataaaaaagaactaaaaatataaacatagctaattcaagaatcaagatcgggtgaaactaaattaaaaacagccataaagtcccacattttccctaatttatttacctatgatattggcacatcttgttttacttaacatttgaaaaatacaaatatctcttcatatgcaaaagagcaaatgttaaatgaaaaactgaattttatatagcttcctaaatatgagccacatgcttaagcagtgaattaactttatgaatcaaatgtttaatgttaactattacaaaagcctggtatccaggtgcaatctcaccagaaaaaaatagcacctgcctttattacaataaaaaaaatggctaattccctttgacatcttaagagtgacactactttgtcaagcactaaatactttttaaattaatcatgttaaacttcagatttatagatataaatattgtatttataactttagtcataatgtacaatttctttcttgtttaaaagtactttctcactcaaaatggtatttatagtttaaaaagaatatgcctctgtattcaggagtgattcaaattcccagatgttttcacatagttatgaaaatgggaaagtgctgaattaaactgggctgcaatatttcaagttttttgctatcaggttataaactatacctacgattgcaagtcatacagtgcctctatttctagaaggcttttaaagtttcctggcttagttatgtccaaaggcagcaggaagtctcatcagtagagggcagaattttcaagtgctgccattcttatcccaggaggcatttccagtggttgagcacaaggcctgtttgtagtttgcttttgctcttgcattttgtggaagggaaggaactgagagagcttagagggttcattaaaaccacccctcactctcttagtcgtagtcagatggagtattcataacagtaacctccaattaccactatgtgttgggaaaaattagaattcggtctacttacaatcctgccaactaggattttactttgatatttcagtataacagtgaatctggattgatgcctgattaaaataaaatccctgattattactttctggattacgaactaaaatccctgtaaaatcaatggatgtgactcattgttaagagtcatgcagacttttacatattaggtaagaattctaaaaattatttgagggttctattctctagcaccaggtactaatgctccctactcaaaaaaaatcatgtgcatggattaatcaagtctaacagtgctcagatttaatggtttaacattgattttcttttctttgtcaaacttatatatgcaaatatttttatagtagtcagatgttatttttgaataaggatcaccctcatttttacccatgtgcttatctttaaaaccaacattgtaaagtagcacgcagacatatgtttcttttatcttcatggattatttttaccttaaaaataaattatcatttttttttttgaatttgggttttattctccagatactctgtgtacatgtgggtaagtatgtgggagtatgtgtgtttgtgtgtaagaggggataattaattgtctctcaactctatctcatactttaatatcaaataaaaaatgaaatgtataaagggtcactttgtaggattaggcatcctccttctacctacttaaaccaggggtttgggattcagaattctccatataaccaagaccgaaagtcactggaagactttaaaattagtattttaaccaccacacccagagtcaggtatggaaataaacctatagcatggattctttctatgcataatctcaaaatttaactacccaaataagtaagtttttaaaaactaatttaaaatttgccattgaggaaaatatcacctccatccttaattgtgactcctcatttcagctaaaaccttttctaatactttaaaaaaacaaaatgaaaaacaaactcctagataaagtcataaacactgaaatcagagatgtgattcttgttaaatgttagtttctctttctgaggttacactctgtgcatttgaaactttgacgttaacatcttccgaatgtttagatttgctcaagggttcagattctctggtcttctgccttgcattttcctccttcctttcctttgcaagcaatctatagttgatagcattgccaatgagcagccacacgcttgctgctaccacaatagccccacaggacatgtacatgtatttatattctccagttaaatccaccaatttacctgcaagaggagggccaagaagaactgggccacactccacaattgtgacaagtccgacggcactggaaaatcttggtgcacccacgaggtccatgagagtttcaaagagaacactgctaacactcccaaatccaaggccaaaaaatacagcatataataccaggcttgtgtagtcctgtgccagtgggcacaagaggtgacacactccattgaacatgattgcaaaactgaagaagtactgaattcgaggtcgaatatatttggagtttgcaattaatcctacagaaggcctagcaaacatatcaacgaaagccataacagatagcagaaaagctgccgagtactcatcaattccttggtctttagcatatggagccaagaatataatgggggcaaaaaaacctaggaacataatgacatttccagacagatatatcagaaatcctctatgcttaaaaagggagaaatctaaatacttattaactttttcccaagttgatttcttcgttttgattttctttgggcttgaatcatcttctgttttgccagtcttatttttagacttagaagtggtttgattgggtccaaggggtctcatgagggaaccagccacacaggcattcaaaagtagacttcccaaaatcaggaagcttcctttccagccaaaagtattaaaaaggtactgattgaaaggagccaatgaacttaagaaaacaggacttcctgccatggccaatccatttgccatgggtcgcttcctatagaagtatttgccaattatggttaaggcgggttgcaggttgaaggctaaacctaaacctgtaatgaatcccatagtgaggtacagctgtaccacgctgctactaaaggaggccaacaccattccaagacagcataataagcctcctgctatcaccaccggccggctgccgtatttattcaccaaaacactacttacaggacttcactgaagtcctgagcctcttaaagtcacccatgaggattgaaataaacttcttccaaacttctgttaatgttggtattttgacctcctcccataacagtgaatgatcgtgatgttatctagaatagcaaatcctttccagaagattttccatctccttttcccagattcatcagaggagtcattatgtacggcagctgtaagctaggcatgatcctgattgagtaaagctgcactgaatcctcaaggatgtgaagatcaaaaagctttcaaatattctacctcaagtagatggtgatctctttaaagggtgaatgatgcattccgcttctccttttttcctcctgcgtacataacagccagcataatggatgaaatccatgctatttcactgtaggtagtgtggaatatttgctgaatttctttgaagaatacggtgacagctttggggaatgcataggaaaatccaatggagataaaagctgctccaaccacaatccaaccccatcctccatctggaggtggatgcacaggtggggcacttggcattggtggcatttctgctcctctagtggaaattcaagtaacctggcgacaggtgtttagaaacatggtcttccatttcaccaagacataagtttccctgatctatggactcctctccccacctgaggcagaagtttccttgtgaaccattgctctttttagaat

SEQ ID NO: 17835 - RNA, 11701 nt, Homo sapiens
  source 1..11701: mol_type = other RNA
tcgaggagctcacagtctagtaagaaagagatgaatttgaaaatatatttgaaactgtaggcaaaataagtaccctcacagagaaattcaacatttggtttcaaatttgttatgcagtgaaaattagaaactacaaccaagatttttttaaaacattatgttcatataacgctgtagtatacctgaaaggcaagaacttaaacaagtgtgctgaaaaacaaattaggaatatttgaacaaaatatactttaaaaatgatcaacaacgtaaaatattcctgatttaaataaatctaagttattttatttagtttaagcaaaatatgtatccatatgaaaatgccagttctttcatttttggttaattcctttacacatattatttgctaagttcagaaatgctatatatacaaaaatttcaaaaataaataagtatcccaagatcacataacaatactttaagtacattcatgtgtaagaaggcaaaaaaagaaggttctatcttatattttaaaactttgacaggtattttaaatgtattattttatactttattttctttaaaaatgaaataatacagccatgatttaagtcatgtaaaaacaactgtttggatcatttaggtgtcaagcaaaactatcctctttatttcactatcatagtaaccatagttgatagaccatgtggcaatatgatcatttgttcagtggtcattaagatatctatagaataaacaagacaactacattttatttttttcacttaaaaatcacaaaaatacagcctaaaatataatttatattttaaaaataattctaaacattaacccctaaatctaatcccttaaaaaattcttgcaaaagttagctggatgtggctgttgccaaggaatgtcttttattagcaacaagtgactatctataacttttattccaacaatcttattttaaatatttgtttcaatttaatgctgggattagaaaaacatatttgttcaaagtatgtaagtagtaagtaaaacaatttcaaaaatctatcaaaaaaggagaattattcattctaggaaataattaacatactggtttaaaatatctgggagaagaacttttacataaaaagcttcaaatttagtcagttgtagcaagcacttgaaaagaccctgctctttcatctgcaatatcaggaattactatatctgactcatatttgattaagttacaatctcatttttgttgtcactacaaagaaggatccttatattagtaaatgcactcactgcaactactgaggcctgcctcctgtcagaatgacaatgcagtcttagcatacgggtgtcggtttggctgaatctaaccaaacacatcacgtactacagatgtttttagggcccacccaattcataaaagattttactgcgatacatgagtttacccaaatttttattaaaatgtgtttttagggtaaatatcttgatgaactaggcaaacaaatactgaatgcagattactgtttttacagttttaccgggaaaactcctaatagcaacccctcttccccttcaccacagatctttaatttaggtgtgatttttgtttgttctctacatgggaataaaggagaaagtttagaaagactgtatctagctagataagatgcagaggtagatggaatctctaacataaaagaagctctaattacactgttgccagacagctgttatggattttagtattgtttattaggtgaagaaaacattcataaaataagaaatttttgagatagaacttactctaataatttcattaacatatgttcaggttcttagatcaagaaatactgtagaggtgttctcctcaagactatgctatggcaataatttcttgcatacaatttaataatttaaacttgaactgtgtgttctgtgctctggcgttctacttcagaaaaaaatgaacactgcttctaaaataaaaaggaacataaaataaaaaaggaattaatgagatattgacatgttttctattaatacaatattgatgttttaaatgattttgatattgctataacaacatatattgtgcaaaataattaatctcactaaatattatttctgatttgccacgaattatctgccgtggcaatcaggaaatagtcttcaaagtaagtttgcaaacatgattttgcaaaccatgattggaaaaatatattcatttgggctataaactatcaagtagggttgttatatatatttctaggaaaatattttatttactctacaaagatcatcattatgaccttacggcttctgtagtgcaatggagaaaaaagtgtgttagaagttaaaagacctgaattctatctccaaccctgcatttattcagagtattggtataggtttaggcaaaatccttaatccagtctagttttatatggtaaaaatgtggatacctatcaaaactgagggttgagaggatgaaatgaattcattaaacatatcttctgagacataaatatatcaaaacaaatcaaaatacaattagatctaatgtttagaaataaatattttaattcatatttgctatttcactaaatctagaaatactaatgctttagttaaatatagaaagttgatgatagaaaaataaaatccatcgtaccattgaaaagcttgtcagaaatatgtactcttgagattcggaggatgagaaaaaaaatgtgtactctaacgaggaagctatataaactgagtctaactcaaaacatttattttagatgcatataagaattaaagtcttagtcaaaagaatgttttaaaatttcatcctaaatttatgtgagataaaatgccattcttttgtttttctgaacagaggagcttttatcaacttattctattttatttttatttttattattttattttattttatttattattattatactttaagttttagggtacatgtgcacaatgtgcaggttagttacatatgtatacatgtgccatgctggtgcgctgcacccactaactcgtcacctagcattaggtatatctcccaatgctatccctcccccctcccccgaccccaccacagtccccagagtgtgatgttccccttcctgtgtccatgtgttctcattgttcagttcccacctatgagtgagaatatgcggtgtttggttttttgttcttgcgatagtttactgagaatgatgatttctaatttcatccatgtccctacacgaacttattctattttaatagaatgttcagtatcagtgttttcacactgagattctctagcttattttgccatatttaaattaaaaagaaacaaaaaatcctgtttgatcatgtgaaaaatatttactgaaatgtgaataaatttatgatcattaattgcctactgaaatattcctgaatattgctcaccttattaacaagtatatatggagactgaaaaacatgtagatcatgcaaacaagtgtaactaactataccaaagaaacaaaagtccatactaaatatgtccataattaaataaaaaatgctaaacaagttttacctagatattataaaaacatagaaaggaaaacatttaggagatgatgaagaagcaggagattgggatgggagatgtaatttgatctaaattcccatatgcttctgtaaaatcaaaaattcattttgcaatattaattttgctcttaaggtagagacttttaaaatgaccattctcaatactacagcaattcttccctgatttgcacataaatgaattaaagtgaagaaaaagcagtagaggagagaagactaaaataaaccagattgtagcaccctgtaaagagctaaaatctccagtgtacaaacaactgataggaaagaagagaaaatcagaactataaaaaagtgacataagctcagaaaattactcatttttaattgtatcaacaaagataatttgtaattttgatcatgcaagcattataattactgataattgggcctttcagcttttaagtgccttctcaaacatgagttctgcatatggttgtgcagaaatcaaaatcttaaagagagatgagtaaagtcaagtttgtaatattaatcttatattctcaatatagatgctaattagtgctctgaatggttgtggttagaaatcttgttggtatgatgtatcagtgatgtcactgcattgatggagacagaataatacataatggtgcaatgtggtgatggtaagctttgttactcaatattgtcaggcactttaagaaaatcagaaacattcaggatagtgccaaagaagatcagtttttcaagactctaaaatcatattcaattatatgtgtatgtaattataaatatgtgcatcatggctgactttgagaagaatgcagcgccttgcaagtgcactatttgaatagagctaaggagaactatagtctaaggactgcaaaagtctagatggagaagacaaaagcaatgacacttgttttctctacagaacaaatagacaaagaggtgaatgacaacaaagatgttcagagaaacttgaaaaataagctacggtgtagggtaagttgtattaaatgatgaaaattaatatgtaactgtatgggtaaaccaaatcatttgtatcttataatcttttttttggtagctacggataatattataaatggaataatcactaaaattctaaatataatgttttctagtaagaacattttattttttttttaatagagacagattctcactctattgcctaggctggactgcaagtggggccattatagctcactgaagcctcaacttcctgggctcaaatgaccctctcgtctcagcctcccgagtagctgggactacaggtgcacatcaccacatccaggtaattattttactttttgaatcatgatatgtagcaaccaatctgggaattatttattcataaaagataacattttcctgctaactccaacctcagaaaaaatgtattatgcctgactcaaatatgtcattatttttatgagaaaaagagtcatattgaagtaattatgtctatatgtaataattatcattatttgagataatttgcattggggagaaaagcaggcaatcagaaattacatattcaaggctgggcgcagtggctcacgcctgtaatcccagcactttgggaggcagaggcgagtgaatcacctgaggtcagagttcaagaccagcctgaccaacaaggagaaaccccatctctactaaaacaaaacaaaacaaaacaaaacaaaaaaagccacaaaattagccgggcatggtggcacatgcctgtaattccagttactcgggaggctgaggcaggagaattgcttgaacctgggaggcagaggttgtagtaagccgagattgtgccactgcacgccagcctgggcgacaagaacgagactcagtctcaaaaaaaaaaaaaaagaaagaaagaaagaaattacatattcaggttctagcaaatgcagttctctaataaacactaaataaatcataatacaagttacagttaaacctaattgttttactatataggatgtatcttttttgtacctatattttatcttcctttgcttctctggcctctattgggaggcagcacggtagtgaacacctcggggatctttctggttacgtaaacctgagttttaattttggttcatactaccttttaactttgggtagtctgctgagcttgttttttgttttcactcatctgtcatatcaagctagtaataattctgccatggttttggttttcatattgaaaggcattacataagcaaaatgcataacatataaatattagttccctttccactatgcatccaatctccctattaaattaagcctaaaaataataatttttgttttattaaaagccttccacattctacatatgaaagggattttttaaaggtgttttagataaaaaatgtttcaaccaactgaccaagaatatctcttcatatttatgtcatctacataaaaacttacatttatatcatatatcttttagtcttcttttctatattcttgattgtcatgttgtacagccagaaaagaatgagtataaattatctagattttttaaagtgcacattcaaacatagaaaatctaattattttacttgtttcttagtattaggctgaggccaatgagtccatgagctaaagggttgaaacttggcaccaaaaaagtgattgtttatgagtcctgtagatttatactgagaaaacatcatgtcttccaatgtgaaatacactaaaacctgattttttgtctcttaaggtgtgctaggtgaatgcaaaaaggatcaggaaagggggtgaggataggtcaggaaaagtgcaaacacaatgttctattcataaattagtgatggcatatttaaggttaagtagtaaaaaatatggggggctcagttaacacgaatgaaaaaatagttaaagtagccatgaattatctggataccttgatttaatgacaccctttcttctgtacaatttcataatgtgggaatagagattagtggggattgtagtggtataccctgactttgcttcatgatatctcaaatgtttaaaacctattattccctagagaaagaaatatgttcatactaattgttgcagaggcagaagccaaatatatctcctcctccatttatgtgactatatagtaatgaaaatcctaggttgatacacttttctcaatcttggaaagattctgctaaagcagcaaatcttctaacaagttcaagagggtggggagagtgaacaagtagaataatttatattaccctggaacaattctgaatcctgtaggtatttatgtcactgtttcaattgtgttctggtttaactgtcaatatttatgcatagcagttaacgtgtgtgcatatttgtaactgtgcagtgctactgccaggtgtgactgtacaaatcatgtgctttgaatgtgcaagttttactttcttttctaacaatttaatacagtgttagaaataaataacgaatgaagacaaccaaagagcagccagacaaatgtgaactggttttgacgtgacgagaaactcatcagtaagtaaataaacctcctccctggagaaggccactgaaatgcacccaggaggatgtctctactagaaggtaataaaaaatatatataatgtagtctttgacctaaaacctcatgattattactttgccatttatttccccctggtatctgatgttcatattagtttaatgtgccttttcagagaattcaagacactttttggaaagtagaatttttttttgaaaatttatgattggagaggtactacacaatttagaggttacatttcttgacaaatctgagttgaataaaaaagaactaaaaatataaacatagctaattcaagaatcaagatcgggtgaaactaaattaaaaacagccataaagtcccacattttccctaatttatttacctatgatattggcacatcttgttttacttaacatttgaaaaatacaaatatctcttcatatgcaaaagagcaaatgttaaatgaaaaactgaattttatatagcttcctaaatatgagccacatgcttaagcagtgaattaactttatgaatcaaatgtttaatgttaactattacaaaagcctggtatccaggtgcaatctcaccagaaaaaaatagcacctgcctttattacaataaaaaaaatggctaattccctttgacatcttaagagtgacactactttgtcaagcactaaatactttttaaattaatcatgttaaacttcagatttatagatataaatattgtatttataactttagtcataatgtacaatttctttcttgtttaaaagtactttctcactcaaaatggtatttatagtttaaaaagaatatgcctctgtattcaggagtgattcaaattcccagatgttttcacatagttatgaaaatgggaaagtgctgaattaaactgggctgcaatatttcaagttttttgctatcaggttataaactatacctacgattgcaagtcatacagtgcctctatttctagaaggcttttaaagtttcctggcttagttatgtccaaaggcagcaggaagtctcatcagtagagggcagaattttcaagtgctgccattcttatcccaggaggcatttccagtggttgagcacaaggcctgtttgtagtttgcttttgctcttgcattttgtggaagggaaggaactgagagagcttagagggttcattaaaaccacccctcactctcttagtcgtagtcagatggagtattcataacagtaacctccaattaccactatgtgttgggaaaaattagaattcggtctacttacaatcctgccaactaggattttactttgatatttcagtataacagtgaatctggattgatgcctgattaaaataaaatccctgattattactttctggattacgaactaaaatccctgtaaaatcaatggatgtgactcattgttaagagtcatgcagacttttacatattaggtaagaattctaaaaattatttgagggttctattctctagcaccaggtactaatgctccctactcaaaaaaaatcatgtgcatggattaatcaagtctaacagtgctcagatttaatggtttaacattgattttcttttctttgtcaaacttatatatgcaaatatttttatagtagtcagatgttatttttgaataaggatcaccctcatttttacccatgtgcttatctttaaaaccaacattgtaaagtagcacgcagacatatgtttcttttatcttcatggattatttttaccttaaaaataaattatcatttttttttttgaatttgggttttattctccagatactctgtgtacatgtgggtaagtatgtgggagtatgtgtgtttgtgtgtaagaggggataattaattgtctctcaactctatctcatactttaatatcaaataaaaaatgaaatgtataaagggtcactttgtaggattaggcatcctccttctacctacttaaaccaggggtttgggattcagaattctccatataaccaagaccgaaagtcactggaagactttaaaattagtattttaaccaccacacccagagtcaggtatggaaataaacctatagcatggattctttctatgcataatctcaaaatttaactacccaaataagtaagtttttaaaaactaatttaaaatttgccattgaggaaaatatcacctccatccttaattgtgactcctcatttcagctaaaaccttttctaatactttaaaaaaacaaaatgaaaaacaaactcctagataaagtcataaacactgaaatcagagatgtgattcttgttaaatgttagtttctctttctgaggttacactctgtgcatttgaaactttgacgttaacatcttccgaatgtttagatttgctcaagggttcagattctctggtcttctgccttgcattttcctccttcctttcctttgcaagcaatctatagttgatagcattgccaatgagcagccacacgcttgctgctaccacaatagccccacaggacatgtacatgtatttatattctccagttaaatccaccaatttacctgcaagaggagggccaagaagaactgggccacactccacaattgtgacaagtccgacggcactggaaaatcttggtgcacccacgaggtccatgagagtttcaaagagaacactgctaacactcccaaatccaaggccaaaaaatacagcatataataccaggcttgtgtagtcctgtgccagtgggcacaagaggtgacacactccattgaacatgattgcaaaactgaagaagtactgaattcgaggtcgaatatatttggagtttgcaattaatcctacagaaggcctagcaaacatatcaacgaaagccataacagatagcagaaaagctgccgagtactcatcaattccttggtctttagcatatggagccaagaatataatgggggcaaaaaaacctaggaacataatgacatttccagacagatatatcagaaatcctctatgcttaaaaagggagaaatctaaatacttattaactttttcccaagttgatttcttcgttttgattttctttgggcttgaatcatcttctgttttgccagtcttatttttagacttagaagtggtttgattgggtccaaggggtctcatgagggaaccagccacacaggcattcaaaagtagacttcccaaaatcaggaagcttcctttccagccaaaagtattaaaaaggtactgattgaaaggagccaatgaacttaagaaaacaggacttcctgccatggccaatccatttgccatgggtcgcttcctatagaagtatttgccaattatggttaaggcgggttgcaggttgaaggctaaacctaaacctgtaatgaatcccatagtgaggtacagctgtaccacgctgctactaaaggaggccaacaccattccaagacagcataataagcctcctgctatcaccaccggccggctgccgtatttattcaccaaaacactacttacaggacttcactgaagtcctgagcctcttaaagtcacccatgaggattgaaataaacttcttccaaacttctgttaatgttggtattttgacctcctcccataacagtgaatgatcgtgatgttatctagaatagcaaatcctttccagaagattttccatctccttttcccagattcatcagaggagtcattatgtacggcagctgtaagcttcagtagaattgaagacagttagggccctgctctggattaggctctggcttagggaatgttgtgggtggtttgatcttgtatccaaacttctaaaactttcttcacttttcctttgcattcacaacttggctaaccttagtgctagacacctagctttcagcctgtgctttcagcacctttctcattaaggtgaatcatttctagcttttgatttcaaatgagagacttgcaactcttcctttcacttgaacacttagaagccactgtaggtttattaagtggcctaatttcaatactgttgtatctcagacagtagagaggccctaggcatgatcctgattgagtaaagctgcactgaatcctcaaggatgtgaagatcaaaaagctttcaaatattctacctcaagtagatggtgatctctttaaagggtgaatgatgcattccgcttctccttttttcctcctgcgtacataacagccagcataatggatgaaatccatgctatttcactgtaggtagtgtggaatatttgctgaatttctttgaagaatacggtgacagctttggggaatgcataggaaaatccaatggagataaaagctgctccaaccacaatccaaccccatcctccatctggaggtggatgcacaggtggggcacttggcattggtggcatttctgctcctctagtggaaattcaagtaacctggcgacaggtgtttagaaacatggtcttccatttcaccaagacataagtttccctgatctatggactcctctccccacctgaggcagaagtttccttgtgaaccattgctctttttagaat

SEQ ID NO: 17836 - RNA, 11775 nt, Homo sapiens
  source 1..11775: mol_type = other RNA
tcgaggagctcacagtctagtaagaaagagatgaatttgaaaatatatttgaaactgtaggcaaaataagtaccctcacagagaaattcaacatttggtttcaaatttgttatgcagtgaaaattagaaactacaaccaagatttttttaaaacattatgttcatataacgctgtagtatacctgaaaggcaagaacttaaacaagtgtgctgaaaaacaaattaggaatatttgaacaaaatatactttaaaaatgatcaacaacgtaaaatattcctgatttaaataaatctaagttattttatttagtttaagcaaaatatgtatccatatgaaaatgccagttctttcatttttggttaattcctttacacatattatttgctaagttcagaaatgctatatatacaaaaatttcaaaaataaataagtatcccaagatcacataacaatactttaagtacattcatgtgtaagaaggcaaaaaaagaaggttctatcttatattttaaaactttgacaggtattttaaatgtattattttatactttattttctttaaaaatgaaataatacagccatgatttaagtcatgtaaaaacaactgtttggatcatttaggtgtcaagcaaaactatcctctttatttcactatcatagtaaccatagttgatagaccatgtggcaatatgatcatttgttcagtggtcattaagatatctatagaataaacaagacaactacattttatttttttcacttaaaaatcacaaaaatacagcctaaaatataatttatattttaaaaataattctaaacattaacccctaaatctaatcccttaaaaaattcttgcaaaagttagctggatgtggctgttgccaaggaatgtcttttattagcaacaagtgactatctataacttttattccaacaatcttattttaaatatttgtttcaatttaatgctgggattagaaaaacatatttgttcaaagtatgtaagtagtaagtaaaacaatttcaaaaatctatcaaaaaaggagaattattcattctaggaaataattaacatactggtttaaaatatctgggagaagaacttttacataaaaagcttcaaatttagtcagttgtagcaagcacttgaaaagaccctgctctttcatctgcaatatcaggaattactatatctgactcatatttgattaagttacaatctcatttttgttgtcactacaaagaaggatccttatattagtaaatgcactcactgcaactactgaggcctgcctcctgtcagaatgacaatgcagtcttagcatacgggtgtcggtttggctgaatctaaccaaacacatcacgtactacagatgtttttagggcccacccaattcataaaagattttactgcgatacatgagtttacccaaatttttattaaaatgtgtttttagggtaaatatcttgatgaactaggcaaacaaatactgaatgcagattactgtttttacagttttaccgggaaaactcctaatagcaacccctcttccccttcaccacagatctttaatttaggtgtgatttttgtttgttctctacatgggaataaaggagaaagtttagaaagactgtatctagctagataagatgcagaggtagatggaatctctaacataaaagaagctctaattacactgttgccagacagctgttatggattttagtattgtttattaggtgaagaaaacattcataaaataagaaatttttgagatagaacttactctaataatttcattaacatatgttcaggttcttagatcaagaaatactgtagaggtgttctcctcaagactatgctatggcaataatttcttgcatacaatttaataatttaaacttgaactgtgtgttctgtgctctggcgttctacttcagaaaaaaatgaacactgcttctaaaataaaaaggaacataaaataaaaaaggaattaatgagatattgacatgttttctattaatacaatattgatgttttaaatgattttgatattgctataacaacatatattgtgcaaaataattaatctcactaaatattatttctgatttgccacgaattatctgccgtggcaatcaggaaatagtcttcaaagtaagtttgcaaacatgattttgcaaaccatgattggaaaaatatattcatttgggctataaactatcaagtagggttgttatatatatttctaggaaaatattttatttactctacaaagatcatcattatgaccttacggcttctgtagtgcaatggagaaaaaagtgtgttagaagttaaaagacctgaattctatctccaaccctgcatttattcagagtattggtataggtttaggcaaaatccttaatccagtctagttttatatggtaaaaatgtggatacctatcaaaactgagggttgagaggatgaaatgaattcattaaacatatcttctgagacataaatatatcaaaacaaatcaaaatacaattagatctaatgtttagaaataaatattttaattcatatttgctatttcactaaatctagaaatactaatgctttagttaaatatagaaagttgatgatagaaaaataaaatccatcgtaccattgaaaagcttgtcagaaatatgtactcttgagattcggaggatgagaaaaaaaatgtgtactctaacgaggaagctatataaactgagtctaactcaaaacatttattttagatgcatataagaattaaagtcttagtcaaaagaatgttttaaaatttcatcctaaatttatgtgagataaaatgccattcttttgtttttctgaacagaggagcttttatcaacttattctattttatttttatttttattattttattttattttatttattattattatactttaagttttagggtacatgtgcacaatgtgcaggttagttacatatgtatacatgtgccatgctggtgcgctgcacccactaactcgtcacctagcattaggtatatctcccaatgctatccctcccccctcccccgaccccaccacagtccccagagtgtgatgttccccttcctgtgtccatgtgttctcattgttcagttcccacctatgagtgagaatatgcggtgtttggttttttgttcttgcgatagtttactgagaatgatgatttctaatttcatccatgtccctacacgaacttattctattttaatagaatgttcagtatcagtgttttcacactgagattctctagcttattttgccatatttaaattaaaaagaaacaaaaaatcctgtttgatcatgtgaaaaatatttactgaaatgtgaataaatttatgatcattaattgcctactgaaatattcctgaatattgctcaccttattaacaagtatatatggagactgaaaaacatgtagatcatgcaaacaagtgtaactaactataccaaagaaacaaaagtccatactaaatatgtccataattaaataaaaaatgctaaacaagttttacctagatattataaaaacatagaaaggaaaacatttaggagatgatgaagaagcaggagattgggatgggagatgtaatttgatctaaattcccatatgcttctgtaaaatcaaaaattcattttgcaatattaattttgctcttaaggtagagacttttaaaatgaccattctcaatactacagcaattcttccctgatttgcacataaatgaattaaagtgaagaaaaagcagtagaggagagaagactaaaataaaccagattgtagcaccctgtaaagagctaaaatctccagtgtacaaacaactgataggaaagaagagaaaatcagaactataaaaaagtgacataagctcagaaaattactcatttttaattgtatcaacaaagataatttgtaattttgatcatgcaagcattataattactgataattgggcctttcagcttttaagtgccttctcaaacatgagttctgcatatggttgtgcagaaatcaaaatcttaaagagagatgagtaaagtcaagtttgtaatattaatcttatattctcaatatagatgctaattagtgctctgaatggttgtggttagaaatcttgttggtatgatgtatcagtgatgtcactgcattgatggagacagaataatacataatggtgcaatgtggtgatggtaagctttgttactcaatattgtcaggcactttaagaaaatcagaaacattcaggatagtgccaaagaagatcagtttttcaagactctaaaatcatattcaattatatgtgtatgtaattataaatatgtgcatcatggctgactttgagaagaatgcagcgccttgcaagtgcactatttgaatagagctaaggagaactatagtctaaggactgcaaaagtctagatggagaagacaaaagcaatgacacttgttttctctacagaacaaatagacaaagaggtgaatgacaacaaagatgttcagagaaacttgaaaaataagctacggtgtagggtaagttgtattaaatgatgaaaattaatatgtaactgtatgggtaaaccaaatcatttgtatcttataatcttttttttggtagctacggataatattataaatggaataatcactaaaattctaaatataatgttttctagtaagaacattttattttttttttaatagagacagattctcactctattgcctaggctggactgcaagtggggccattatagctcactgaagcctcaacttcctgggctcaaatgaccctctcgtctcagcctcccgagtagctgggactacaggtgcacatcaccacatccaggtaattattttactttttgaatcatgatatgtagcaaccaatctgggaattatttattcataaaagataacattttcctgctaactccaacctcagaaaaaatgtattatgcctgactcaaatatgtcattatttttatgagaaaaagagtcatattgaagtaattatgtctatatgtaataattatcattatttgagataatttgcattggggagaaaagcaggcaatcagaaattacatattcaaggctgggcgcagtggctcacgcctgtaatcccagcactttgggaggcagaggcgagtgaatcacctgaggtcagagttcaagaccagcctgaccaacaaggagaaaccccatctctactaaaacaaaacaaaacaaaacaaaacaaaaaaagccacaaaattagccgggcatggtggcacatgcctgtaattccagttactcgggaggctgaggcaggagaattgcttgaacctgggaggcagaggttgtagtaagccgagattgtgccactgcacgccagcctgggcgacaagaacgagactcagtctcaaaaaaaaaaaaaaagaaagaaagaaagaaattacatattcaggttctagcaaatgcagttctctaataaacactaaataaatcataatacaagttacagttaaacctaattgttttactatataggatgtatcttttttgtacctatattttatcttcctttgcttctctggcctctattgggaggcagcacggtagtgaacacctcggggatctttctggttacgtaaacctgagttttaattttggttcatactaccttttaactttgggtagtctgctgagcttgttttttgttttcactcatctgtcatatcaagctagtaataattctgccatggttttggttttcatattgaaaggcattacataagcaaaatgcataacatataaatattagttccctttccactatgcatccaatctccctattaaattaagcctaaaaataataatttttgttttattaaaagccttccacattctacatatgaaagggattttttaaaggtgttttagataaaaaatgtttcaaccaactgaccaagaatatctcttcatatttatgtcatctacataaaaacttacatttatatcatatatcttttagtcttcttttctatattcttgattgtcatgttgtacagccagaaaagaatgagtataaattatctagattttttaaagtgcacattcaaacatagaaaatctaattattttacttgtttcttagtattaggctgaggccaatgagtccatgagctaaagggttgaaacttggcaccaaaaaagtgattgtttatgagtcctgtagatttatactgagaaaacatcatgtcttccaatgtgaaatacactaaaacctgattttttgtctcttaaggtgtgctaggtgaatgcaaaaaggatcaggaaagggggtgaggataggtcaggaaaagtgcaaacacaatgttctattcataaattagtgatggcatatttaaggttaagtagtaaaaaatatggggggctcagttaacacgaatgaaaaaatagttaaagtagccatgaattatctggataccttgatttaatgacaccctttcttctgtacaatttcataatgtgggaatagagattagtggggattgtagtggtataccctgactttgcttcatgatatctcaaatgtttaaaacctattattccctagagaaagaaatatgttcatactaattgttgcagaggcagaagccaaatatatctcctcctccatttatgtgactatatagtaatgaaaatcctaggttgatacacttttctcaatcttggaaagattctgctaaagcagcaaatcttctaacaagttcaagagggtggggagagtgaacaagtagaataatttatattaccctggaacaattctgaatcctgtaggtatttatgtcactgtttcaattgtgttctggtttaactgtcaatatttatgcatagcagttaacgtgtgtgcatatttgtaactgtgcagtgctactgccaggtgtgactgtacaaatcatgtgctttgaatgtgcaagttttactttcttttctaacaatttaatacagtgttagaaataaataacgaatgaagacaaccaaagagcagccagacaaatgtgaactggttttgacgtgacgagaaactcatcagtaagtaaataaacctcctccctggagaaggccactgaaatgcacccaggaggatgtctctactagaaggtaataaaaaatatatataatgtagtctttgacctaaaacctcatgattattactttgccatttatttccccctggtatctgatgttcatattagtttaatgtgccttttcagagaattcaagacactttttggaaagtagaatttttttttgaaaatttatgattggagaggtactacacaatttagaggttacatttcttgacaaatctgagttgaataaaaaagaactaaaaatataaacatagctaattcaagaatcaagatcgggtgaaactaaattaaaaacagccataaagtcccacattttccctaatttatttacctatgatattggcacatcttgttttacttaacatttgaaaaatacaaatatctcttcatatgcaaaagagcaaatgttaaatgaaaaactgaattttatatagcttcctaaatatgagccacatgcttaagcagtgaattaactttatgaatcaaatgtttaatgttaactattacaaaagcctggtatccaggtgcaatctcaccagaaaaaaatagcacctgcctttattacaataaaaaaaatggctaattccctttgacatcttaagagtgacactactttgtcaagcactaaatactttttaaattaatcatgttaaacttcagatttatagatataaatattgtatttataactttagtcataatgtacaatttctttcttgtttaaaagtactttctcactcaaaatggtatttatagtttaaaaagaatatgcctctgtattcaggagtgattcaaattcccagatgttttcacatagttatgaaaatgggaaagtgctgaattaaactgggctgcaatatttcaagttttttgctatcaggttataaactatacctacgattgcaagtcatacagtgcctctatttctagaaggcttttaaagtttcctggcttagttatgtccaaaggcagcaggaagtctcatcagtagagggcagaattttcaagtgctgccattcttatcccaggaggcatttccagtggttgagcacaaggcctgtttgtagtttgcttttgctcttgcattttgtggaagggaaggaactgagagagcttagagggttcattaaaaccacccctcactctcttagtcgtagtcagatggagtattcataacagtaacctccaattaccactatgtgttgggaaaaattagaattcggtctacttacaatcctgccaactaggattttactttgatatttcagtataacagtgaatctggattgatgcctgattaaaataaaatccctgattattactttctggattacgaactaaaatccctgtaaaatcaatggatgtgactcattgttaagagtcatgcagacttttacatattaggtaagaattctaaaaattatttgagggttctattctctagcaccaggtactaatgctccctactcaaaaaaaatcatgtgcatggattaatcaagtctaacagtgctcagatttaatggtttaacattgattttcttttctttgtcaaacttatatatgcaaatatttttatagtagtcagatgttatttttgaataaggatcaccctcatttttacccatgtgcttatctttaaaaccaacattgtaaagtagcacgcagacatatgtttcttttatcttcatggattatttttaccttaaaaataaattatcatttttttttttgaatttgggttttattctccagatactctgtgtacatgtgggtaagtatgtgggagtatgtgtgtttgtgtgtaagaggggataattaattgtctctcaactctatctcatactttaatatcaaataaaaaatgaaatgtataaagggtcactttgtaggattaggcatcctccttctacctacttaaaccaggggtttgggattcagaattctccatataaccaagaccgaaagtcactggaagactttaaaattagtattttaaccaccacacccagagtcaggtatggaaataaacctatagcatggattctttctatgcataatctcaaaatttaactacccaaataagtaagtttttaaaaactaatttaaaatttgccattgaggaaaatatcacctccatccttaattgtgactcctcatttcagctaaaaccttttctaatactttaaaaaaacaaaatgaaaaacaaactcctagataaagtcataaacactgaaatcagagatgtgattcttgttaaatgttagtttctctttctgaggttacactctgtgcatttgaaactttgacgttaacatcttccgaatgtttagatttgctcaagggttcagattctctggtcttctgccttgcattttcctccttcctttcctttgcaagcaatctatagttgatagcattgccaatgagcagccacacgcttgctgctaccacaatagccccacaggacatgtacatgtatttatattctccagttaaatccaccaatttacctgcaagaggagggccaagaagaactgggccacactccacaattgtgacaagtccgacggcactggaaaatcttggtgcacccacgaggtccatgagagtttcaaagagaacactgctaacactcccaaatccaaggccaaaaaatacagcatataataccaggcttgtgtagtcctgtgccagtgggcacaagaggtgacacactccattgaacatgattgcaaaactgaagaagtactgaattcgaggtcgaatatatttggagtttgcaattaatcctacagaaggcctagcaaacatatcaacgaaagccataacagatagcagaaaagctgccgagtactcatcaattccttggtctttagcatatggagccaagaatataatgggggcaaaaaaacctaggaacataatgacatttccagacagatatatcagaaatcctctatgcttaaaaagggagaaatctaaatacttattaactttttcccaagttgatttcttcgttttgattttctttgggcttgaatcatcttctgttttgccagtcttatttttagacttagaagtggtttgattgggtccaaggggtctcatgagggaaccagccacacaggcattcaaaagtagacttcccaaaatcaggaagcttcctttccagccaaaagtattaaaaaggtactgattgaaaggagccaatgaacttaagaaaacaggacttcctgccatggccaatccatttgccatgggtcgcttcctatagaagtatttgccaattatggttaaggcgggttgcaggttgaaggctaaacctaaacctgtaatgaatcccatagtgaggtacagctgtaccacgctgctactaaaggaggccaacaccattccaagacagcataataagcctcctgctatcaccaccggccggctgccgtatttattcaccaaaacactacttacaggacttcactgaagtcctgagcctcttaaagtcacccatgaggattgaaataaacttcttccaaacttctgttaatgttggtattttgacctcctcccataacagtgaatgatcgtgatgttatctagaatagcaaatcctttccagaagattttccatctccttttcccagattcatcagaggagtcattatgtacggcagctgtaagcttcagtagaattgaagacagttagggccctgctctggattaggctctggcttagggaatgttgtgggtggtttgatcttgtatccaaacttctaaaactttcttcacttttcctttgcattcacaacttggctaaccttagtgctagacacctagctttcagcctgtgctttcagcacctttctcattaaggtgaatcatttctagcttttgatttcaaatgagagacttgcaactcttcctttcacttgaacacttagaagccactgtaggtttattaagtggcctaatttcaatactgttgtatctcagacagtagagaggccctaggcatgatcctgattgagtaaagctgcactgaatcctcaaggatgtgaagatcaaaaagctttcaaatattctacctcaagtagatggtgatctctttaaagggtgaatgatgcattccgcttctccttttttcctgggtgccatggagggcatgttgatggtgggaggcagacagattcctgggcagaaaggggtggatccttggtgaaaccccacctttaatccagagacagcctgaggcctgggggtcagactgtcagttctgggtagtctgtagaccaaagtgagaacttatggagctttttccaggcccacccatggctgcccacagaccaatcagcatgcacttcctcccttctgaccccttaaaaaccccagactctgccagactcacacagacgtcaggattaccagctgtgggaaggagatacccactttgggtctcctcagctagtcaggacgacctgcctgcagaaagaaggtgcccaccgtggctctcctaagagttgttttgttgctcagtgaagctcctctctgccttgctcgctctccggttgtccatgtgcttcattcttcc

SEQ ID NO: 17837 - RNA, 11830 nt, Homo sapiens
  source 1..11830: mol_type = other RNA
tcgaggagctcacagtctagtaagaaagagatgaatttgaaaatatatttgaaactgtaggcaaaataagtaccctcacagagaaattcaacatttggtttcaaatttgttatgcagtgaaaattagaaactacaaccaagatttttttaaaacattatgttcatataacgctgtagtatacctgaaaggcaagaacttaaacaagtgtgctgaaaaacaaattaggaatatttgaacaaaatatactttaaaaatgatcaacaacgtaaaatattcctgatttaaataaatctaagttattttatttagtttaagcaaaatatgtatccatatgaaaatgccagttctttcatttttggttaattcctttacacatattatttgctaagttcagaaatgctatatatacaaaaatttcaaaaataaataagtatcccaagatcacataacaatactttaagtacattcatgtgtaagaaggcaaaaaaagaaggttctatcttatattttaaaactttgacaggtattttaaatgtattattttatactttattttctttaaaaatgaaataatacagccatgatttaagtcatgtaaaaacaactgtttggatcatttaggtgtcaagcaaaactatcctctttatttcactatcatagtaaccatagttgatagaccatgtggcaatatgatcatttgttcagtggtcattaagatatctatagaataaacaagacaactacattttatttttttcacttaaaaatcacaaaaatacagcctaaaatataatttatattttaaaaataattctaaacattaacccctaaatctaatcccttaaaaaattcttgcaaaagttagctggatgtggctgttgccaaggaatgtcttttattagcaacaagtgactatctataacttttattccaacaatcttattttaaatatttgtttcaatttaatgctgggattagaaaaacatatttgttcaaagtatgtaagtagtaagtaaaacaatttcaaaaatctatcaaaaaaggagaattattcattctaggaaataattaacatactggtttaaaatatctgggagaagaacttttacataaaaagcttcaaatttagtcagttgtagcaagcacttgaaaagaccctgctctttcatctgcaatatcaggaattactatatctgactcatatttgattaagttacaatctcatttttgttgtcactacaaagaaggatccttatattagtaaatgcactcactgcaactactgaggcctgcctcctgtcagaatgacaatgcagtcttagcatacgggtgtcggtttggctgaatctaaccaaacacatcacgtactacagatgtttttagggcccacccaattcataaaagattttactgcgatacatgagtttacccaaatttttattaaaatgtgtttttagggtaaatatcttgatgaactaggcaaacaaatactgaatgcagattactgtttttacagttttaccgggaaaactcctaatagcaacccctcttccccttcaccacagatctttaatttaggtgtgatttttgtttgttctctacatgggaataaaggagaaagtttagaaagactgtatctagctagataagatgcagaggtagatggaatctctaacataaaagaagctctaattacactgttgccagacagctgttatggattttagtattgtttattaggtgaagaaaacattcataaaataagaaatttttgagatagaacttactctaataatttcattaacatatgttcaggttcttagatcaagaaatactgtagaggtgttctcctcaagactatgctatggcaataatttcttgcatacaatttaataatttaaacttgaactgtgtgttctgtgctctggcgttctacttcagaaaaaaatgaacactgcttctaaaataaaaaggaacataaaataaaaaaggaattaatgagatattgacatgttttctattaatacaatattgatgttttaaatgattttgatattgctataacaacatatattgtgcaaaataattaatctcactaaatattatttctgatttgccacgaattatctgccgtggcaatcaggaaatagtcttcaaagtaagtttgcaaacatgattttgcaaaccatgattggaaaaatatattcatttgggctataaactatcaagtagggttgttatatatatttctaggaaaatattttatttactctacaaagatcatcattatgaccttacggcttctgtagtgcaatggagaaaaaagtgtgttagaagttaaaagacctgaattctatctccaaccctgcatttattcagagtattggtataggtttaggcaaaatccttaatccagtctagttttatatggtaaaaatgtggatacctatcaaaactgagggttgagaggatgaaatgaattcattaaacatatcttctgagacataaatatatcaaaacaaatcaaaatacaattagatctaatgtttagaaataaatattttaattcatatttgctatttcactaaatctagaaatactaatgctttagttaaatatagaaagttgatgatagaaaaataaaatccatcgtaccattgaaaagcttgtcagaaatatgtactcttgagattcggaggatgagaaaaaaaatgtgtactctaacgaggaagctatataaactgagtctaactcaaaacatttattttagatgcatataagaattaaagtcttagtcaaaagaatgttttaaaatttcatcctaaatttatgtgagataaaatgccattcttttgtttttctgaacagaggagcttttatcaacttattctattttatttttatttttattattttattttattttatttattattattatactttaagttttagggtacatgtgcacaatgtgcaggttagttacatatgtatacatgtgccatgctggtgcgctgcacccactaactcgtcacctagcattaggtatatctcccaatgctatccctcccccctcccccgaccccaccacagtccccagagtgtgatgttccccttcctgtgtccatgtgttctcattgttcagttcccacctatgagtgagaatatgcggtgtttggttttttgttcttgcgatagtttactgagaatgatgatttctaatttcatccatgtccctacacgaacttattctattttaatagaatgttcagtatcagtgttttcacactgagattctctagcttattttgccatatttaaattaaaaagaaacaaaaaatcctgtttgatcatgtgaaaaatatttactgaaatgtgaataaatttatgatcattaattgcctactgaaatattcctgaatattgctcaccttattaacaagtatatatggagactgaaaaacatgtagatcatgcaaacaagtgtaactaactataccaaagaaacaaaagtccatactaaatatgtccataattaaataaaaaatgctaaacaagttttacctagatattataaaaacatagaaaggaaaacatttaggagatgatgaagaagcaggagattgggatgggagatgtaatttgatctaaattcccatatgcttctgtaaaatcaaaaattcattttgcaatattaattttgctcttaaggtagagacttttaaaatgaccattctcaatactacagcaattcttccctgatttgcacataaatgaattaaagtgaagaaaaagcagtagaggagagaagactaaaataaaccagattgtagcaccctgtaaagagctaaaatctccagtgtacaaacaactgataggaaagaagagaaaatcagaactataaaaaagtgacataagctcagaaaattactcatttttaattgtatcaacaaagataatttgtaattttgatcatgcaagcattataattactgataattgggcctttcagcttttaagtgccttctcaaacatgagttctgcatatggttgtgcagaaatcaaaatcttaaagagagatgagtaaagtcaagtttgtaatattaatcttatattctcaatatagatgctaattagtgctctgaatggttgtggttagaaatcttgttggtatgatgtatcagtgatgtcactgcattgatggagacagaataatacataatggtgcaatgtggtgatggtaagctttgttactcaatattgtcaggcactttaagaaaatcagaaacattcaggatagtgccaaagaagatcagtttttcaagactctaaaatcatattcaattatatgtgtatgtaattataaatatgtgcatcatggctgactttgagaagaatgcagcgccttgcaagtgcactatttgaatagagctaaggagaactatagtctaaggactgcaaaagtctagatggagaagacaaaagcaatgacacttgttttctctacagaacaaatagacaaagaggtgaatgacaacaaagatgttcagagaaacttgaaaaataagctacggtgtagggtaagttgtattaaatgatgaaaattaatatgtaactgtatgggtaaaccaaatcatttgtatcttataatcttttttttggtagctacggataatattataaatggaataatcactaaaattctaaatataatgttttctagtaagaacattttattttttttttaatagagacagattctcactctattgcctaggctggactgcaagtggggccattatagctcactgaagcctcaacttcctgggctcaaatgaccctctcgtctcagcctcccgagtagctgggactacaggtgcacatcaccacatccaggtaattattttactttttgaatcatgatatgtagcaaccaatctgggaattatttattcataaaagataacattttcctgctaactccaacctcagaaaaaatgtattatgcctgactcaaatatgtcattatttttatgagaaaaagagtcatattgaagtaattatgtctatatgtaataattatcattatttgagataatttgcattggggagaaaagcaggcaatcagaaattacatattcaaggctgggcgcagtggctcacgcctgtaatcccagcactttgggaggcagaggcgagtgaatcacctgaggtcagagttcaagaccagcctgaccaacaaggagaaaccccatctctactaaaacaaaacaaaacaaaacaaaacaaaaaaagccacaaaattagccgggcatggtggcacatgcctgtaattccagttactcgggaggctgaggcaggagaattgcttgaacctgggaggcagaggttgtagtaagccgagattgtgccactgcacgccagcctgggcgacaagaacgagactcagtctcaaaaaaaaaaaaaaagaaagaaagaaagaaattacatattcaggttctagcaaatgcagttctctaataaacactaaataaatcataatacaagttacagttaaacctaattgttttactatataggatgtatcttttttgtacctatattttatcttcctttgcttctctggcctctattgggaggcagcacggtagtgaacacctcggggatctttctggttacgtaaacctgagttttaattttggttcatactaccttttaactttgggtagtctgctgagcttgttttttgttttcactcatctgtcatatcaagctagtaataattctgccatggttttggttttcatattgaaaggcattacataagcaaaatgcataacatataaatattagttccctttccactatgcatccaatctccctattaaattaagcctaaaaataataatttttgttttattaaaagccttccacattctacatatgaaagggattttttaaaggtgttttagataaaaaatgtttcaaccaactgaccaagaatatctcttcatatttatgtcatctacataaaaacttacatttatatcatatatcttttagtcttcttttctatattcttgattgtcatgttgtacagccagaaaagaatgagtataaattatctagattttttaaagtgcacattcaaacatagaaaatctaattattttacttgtttcttagtattaggctgaggccaatgagtccatgagctaaagggttgaaacttggcaccaaaaaagtgattgtttatgagtcctgtagatttatactgagaaaacatcatgtcttccaatgtgaaatacactaaaacctgattttttgtctcttaaggtgtgctaggtgaatgcaaaaaggatcaggaaagggggtgaggataggtcaggaaaagtgcaaacacaatgttctattcataaattagtgatggcatatttaaggttaagtagtaaaaaatatggggggctcagttaacacgaatgaaaaaatagttaaagtagccatgaattatctggataccttgatttaatgacaccctttcttctgtacaatttcataatgtgggaatagagattagtggggattgtagtggtataccctgactttgcttcatgatatctcaaatgtttaaaacctattattccctagagaaagaaatatgttcatactaattgttgcagaggcagaagccaaatatatctcctcctccatttatgtgactatatagtaatgaaaatcctaggttgatacacttttctcaatcttggaaagattctgctaaagcagcaaatcttctaacaagttcaagagggtggggagagtgaacaagtagaataatttatattaccctggaacaattctgaatcctgtaggtatttatgtcactgtttcaattgtgttctggtttaactgtcaatatttatgcatagcagttaacgtgtgtgcatatttgtaactgtgcagtgctactgccaggtgtgactgtacaaatcatgtgctttgaatgtgcaagttttactttcttttctaacaatttaatacagtgttagaaataaataacgaatgaagacaaccaaagagcagccagacaaatgtgaactggttttgacgtgacgagaaactcatcagtaagtaaataaacctcctccctggagaaggccactgaaatgcacccaggaggatgtctctactagaaggtaataaaaaatatatataatgtagtctttgacctaaaacctcatgattattactttgccatttatttccccctggtatctgatgttcatattagtttaatgtgccttttcagagaattcaagacactttttggaaagtagaatttttttttgaaaatttatgattggagaggtactacacaatttagaggttacatttcttgacaaatctgagttgaataaaaaagaactaaaaatataaacatagctaattcaagaatcaagatcgggtgaaactaaattaaaaacagccataaagtcccacattttccctaatttatttacctatgatattggcacatcttgttttacttaacatttgaaaaatacaaatatctcttcatatgcaaaagagcaaatgttaaatgaaaaactgaattttatatagcttcctaaatatgagccacatgcttaagcagtgaattaactttatgaatcaaatgtttaatgttaactattacaaaagcctggtatccaggtgcaatctcaccagaaaaaaatagcacctgcctttattacaataaaaaaaatggctaattccctttgacatcttaagagtgacactactttgtcaagcactaaatactttttaaattaatcatgttaaacttcagatttatagatataaatattgtatttataactttagtcataatgtacaatttctttcttgtttaaaagtactttctcactcaaaatggtatttatagtttaaaaagaatatgcctctgtattcaggagtgattcaaattcccagatgttttcacatagttatgaaaatgggaaagtgctgaattaaactgggctgcaatatttcaagttttttgctatcaggttataaactatacctacgattgcaagtcatacagtgcctctatttctagaaggcttttaaagtttcctggcttagttatgtccaaaggcagcaggaagtctcatcagtagagggcagaattttcaagtgctgccattcttatcccaggaggcatttccagtggttgagcacaaggcctgtttgtagtttgcttttgctcttgcattttgtggaagggaaggaactgagagagcttagagggttcattaaaaccacccctcactctcttagtcgtagtcagatggagtattcataacagtaacctccaattaccactatgtgttgggaaaaattagaattcggtctacttacaatcctgccaactaggattttactttgatatttcagtataacagtgaatctggattgatgcctgattaaaataaaatccctgattattactttctggattacgaactaaaatccctgtaaaatcaatggatgtgactcattgttaagagtcatgcagacttttacatattaggtaagaattctaaaaattatttgagggttctattctctagcaccaggtactaatgctccctactcaaaaaaaatcatgtgcatggattaatcaagtctaacagtgctcagatttaatggtttaacattgattttcttttctttgtcaaacttatatatgcaaatatttttatagtagtcagatgttatttttgaataaggatcaccctcatttttacccatgtgcttatctttaaaaccaacattgtaaagtagcacgcagacatatgtttcttttatcttcatggattatttttaccttaaaaataaattatcatttttttttttgaatttgggttttattctccagatactctgtgtacatgtgggtaagtatgtgggagtatgtgtgtttgtgtgtaagaggggataattaattgtctctcaactctatctcatactttaatatcaaataaaaaatgaaatgtataaagggtcactttgtaggattaggcatcctccttctacctacttaaaccaggggtttgggattcagaattctccatataaccaagaccgaaagtcactggaagactttaaaattagtattttaaccaccacacccagagtcaggtatggaaataaacctatagcatggattctttctatgcataatctcaaaatttaactacccaaataagtaagtttttaaaaactaatttaaaatttgccattgaggaaaatatcacctccatccttaattgtgactcctcatttcagctaaaaccttttctaatactttaaaaaaacaaaatgaaaaacaaactcctagataaagtcataaacactgaaatcagagatgtgattcttgttaaatgttagtttctctttctgaggttacactctgtgcatttgaaactttgacgttaacatcttccgaatgtttagatttgctcaagggttcagattctctggtcttctgccttgcattttcctccttcctttcctttgcaagcaatctatagttgatagcattgccaatgagcagccacacgcttgctgctaccacaatagccccacaggacatgtacatgtatttatattctccagttaaatccaccaatttacctgcaagaggagggccaagaagaactgggccacactccacaattgtgacaagtccgacggcactggaaaatcttggtgcacccacgaggtccatgagagtttcaaagagaacactgctaacactcccaaatccaaggccaaaaaatacagcatataataccaggcttgtgtagtcctgtgccagtgggcacaagaggtgacacactccattgaacatgattgcaaaactgaagaagtactgaattcgaggtcgaatatatttggagtttgcaattaatcctacagaaggcctagcaaacatatcaacgaaagccataacagatagcagaaaagctgccgagtactcatcaattccttggtctttagcatatggagccaagaatataatgggggcaaaaaaacctaggaacataatgacatttccagacagatatatcagaaatcctctatgcttaaaaagggagaaatctaaatacttattaactttttcccaagttgatttcttcgttttgattttctttgggcttgaatcatcttctgttttgccagtcttatttttagacttagaagtggtttgattgggtccaaggggtctcatgagggaaccagccacacaggcattcaaaagtagacttcccaaaatcaggaagcttcctttccagccaaaagtattaaaaaggtactgattgaaaggagccaatgaacttaagaaaacaggacttcctgccatggccaatccatttgccatgggtcgcttcctatagaagtatttgccaattatggttaaggcgggttgcaggttgaaggctaaacctaaacctgtaatgaatcccatagtgaggtacagctgtaccacgctgctactaaaggaggccaacaccattccaagacagcataataagcctcctgctatcaccaccggccggctgccgtatttattcaccaaaacactacttacaggacttcactgaagtcctgagcctcttaaagtcacccatgaggattgaaataaacttcttccaaacttctgttaatgttggtattttgacctcctcccataacagtgaatgatcgtgatgttatctagaatagcaaatcctttccagaagattttccatctccttttcccagattcatcagaggagtcattatgtacggcagctgtaagcttcagtagaattgaagacagttagggccctgctctggattaggctctggcttagggaatgttgtgggtggtttgatcttgtatccaaacttctaaaactttcttcacttttcctttgcattcacaacttggctaaccttagtgctagacacctagctttcagcctgtgctttcagcacctttctcattaaggtgaatcatttctagcttttgatttcaaatgagagacttgcaactcttcctttcacttgaacacttagaagccactgtaggtttattaagtggcctaatttcaatactgttgtatctcagacagtagagaggccctaggcatgatcctgattgagtaaagctgcactgaatcctcaaggatgtgaagatcaaaaagctttcaaatattctacctcaagtagatggtgatctctttaaagggtgaatgatgcattccgcttctccttttttcctgggtgccatggagggcatgttgatggtgggaggcagacagattcctgggcagaaaggggtggatccttggtgaaaccccacctttaatccagagacagcctgaggcctgggggtcagactgtcagttctgggtagtctgtagaccaaagtgagaacttatggagctttttccaggcccacccatggctgcccacagaccaatcagcatgcacttcctcccttctgaccccttaaaaaccccagactctgccagactcacacagacgtcaggattaccagctgtgggaaggagatacccactttgggtctcctcagctagtcaggacgacctgcctgcagaaagaaggtgcccaccgtggctctcctaagagttgttttgttgctcagtgaagctcctctctgccttgctcgctctccggttgtccatgtgcttcattcttcctcctgcgtacataacagccagcataatggatgaaatccatgctatttcactgtag

SEQ ID NO: 17838 - RNA, 11781 nt, Homo sapiens
  source 1..11781: mol_type = other RNA
tcgaggagctcacagtctagtaagaaagagatgaatttgaaaatatatttgaaactgtaggcaaaataagtaccctcacagagaaattcaacatttggtttcaaatttgttatgcagtgaaaattagaaactacaaccaagatttttttaaaacattatgttcatataacgctgtagtatacctgaaaggcaagaacttaaacaagtgtgctgaaaaacaaattaggaatatttgaacaaaatatactttaaaaatgatcaacaacgtaaaatattcctgatttaaataaatctaagttattttatttagtttaagcaaaatatgtatccatatgaaaatgccagttctttcatttttggttaattcctttacacatattatttgctaagttcagaaatgctatatatacaaaaatttcaaaaataaataagtatcccaagatcacataacaatactttaagtacattcatgtgtaagaaggcaaaaaaagaaggttctatcttatattttaaaactttgacaggtattttaaatgtattattttatactttattttctttaaaaatgaaataatacagccatgatttaagtcatgtaaaaacaactgtttggatcatttaggtgtcaagcaaaactatcctctttatttcactatcatagtaaccatagttgatagaccatgtggcaatatgatcatttgttcagtggtcattaagatatctatagaataaacaagacaactacattttatttttttcacttaaaaatcacaaaaatacagcctaaaatataatttatattttaaaaataattctaaacattaacccctaaatctaatcccttaaaaaattcttgcaaaagttagctggatgtggctgttgccaaggaatgtcttttattagcaacaagtgactatctataacttttattccaacaatcttattttaaatatttgtttcaatttaatgctgggattagaaaaacatatttgttcaaagtatgtaagtagtaagtaaaacaatttcaaaaatctatcaaaaaaggagaattattcattctaggaaataattaacatactggtttaaaatatctgggagaagaacttttacataaaaagcttcaaatttagtcagttgtagcaagcacttgaaaagaccctgctctttcatctgcaatatcaggaattactatatctgactcatatttgattaagttacaatctcatttttgttgtcactacaaagaaggatccttatattagtaaatgcactcactgcaactactgaggcctgcctcctgtcagaatgacaatgcagtcttagcatacgggtgtcggtttggctgaatctaaccaaacacatcacgtactacagatgtttttagggcccacccaattcataaaagattttactgcgatacatgagtttacccaaatttttattaaaatgtgtttttagggtaaatatcttgatgaactaggcaaacaaatactgaatgcagattactgtttttacagttttaccgggaaaactcctaatagcaacccctcttccccttcaccacagatctttaatttaggtgtgatttttgtttgttctctacatgggaataaaggagaaagtttagaaagactgtatctagctagataagatgcagaggtagatggaatctctaacataaaagaagctctaattacactgttgccagacagctgttatggattttagtattgtttattaggtgaagaaaacattcataaaataagaaatttttgagatagaacttactctaataatttcattaacatatgttcaggttcttagatcaagaaatactgtagaggtgttctcctcaagactatgctatggcaataatttcttgcatacaatttaataatttaaacttgaactgtgtgttctgtgctctggcgttctacttcagaaaaaaatgaacactgcttctaaaataaaaaggaacataaaataaaaaaggaattaatgagatattgacatgttttctattaatacaatattgatgttttaaatgattttgatattgctataacaacatatattgtgcaaaataattaatctcactaaatattatttctgatttgccacgaattatctgccgtggcaatcaggaaatagtcttcaaagtaagtttgcaaacatgattttgcaaaccatgattggaaaaatatattcatttgggctataaactatcaagtagggttgttatatatatttctaggaaaatattttatttactctacaaagatcatcattatgaccttacggcttctgtagtgcaatggagaaaaaagtgtgttagaagttaaaagacctgaattctatctccaaccctgcatttattcagagtattggtataggtttaggcaaaatccttaatccagtctagttttatatggtaaaaatgtggatacctatcaaaactgagggttgagaggatgaaatgaattcattaaacatatcttctgagacataaatatatcaaaacaaatcaaaatacaattagatctaatgtttagaaataaatattttaattcatatttgctatttcactaaatctagaaatactaatgctttagttaaatatagaaagttgatgatagaaaaataaaatccatcgtaccattgaaaagcttgtcagaaatatgtactcttgagattcggaggatgagaaaaaaaatgtgtactctaacgaggaagctatataaactgagtctaactcaaaacatttattttagatgcatataagaattaaagtcttagtcaaaagaatgttttaaaatttcatcctaaatttatgtgagataaaatgccattcttttgtttttctgaacagaggagcttttatcaacttattctattttatttttatttttattattttattttattttatttattattattatactttaagttttagggtacatgtgcacaatgtgcaggttagttacatatgtatacatgtgccatgctggtgcgctgcacccactaactcgtcacctagcattaggtatatctcccaatgctatccctcccccctcccccgaccccaccacagtccccagagtgtgatgttccccttcctgtgtccatgtgttctcattgttcagttcccacctatgagtgagaatatgcggtgtttggttttttgttcttgcgatagtttactgagaatgatgatttctaatttcatccatgtccctacacgaacttattctattttaatagaatgttcagtatcagtgttttcacactgagattctctagcttattttgccatatttaaattaaaaagaaacaaaaaatcctgtttgatcatgtgaaaaatatttactgaaatgtgaataaatttatgatcattaattgcctactgaaatattcctgaatattgctcaccttattaacaagtatatatggagactgaaaaacatgtagatcatgcaaacaagtgtaactaactataccaaagaaacaaaagtccatactaaatatgtccataattaaataaaaaatgctaaacaagttttacctagatattataaaaacatagaaaggaaaacatttaggagatgatgaagaagcaggagattgggatgggagatgtaatttgatctaaattcccatatgcttctgtaaaatcaaaaattcattttgcaatattaattttgctcttaaggtagagacttttaaaatgaccattctcaatactacagcaattcttccctgatttgcacataaatgaattaaagtgaagaaaaagcagtagaggagagaagactaaaataaaccagattgtagcaccctgtaaagagctaaaatctccagtgtacaaacaactgataggaaagaagagaaaatcagaactataaaaaagtgacataagctcagaaaattactcatttttaattgtatcaacaaagataatttgtaattttgatcatgcaagcattataattactgataattgggcctttcagcttttaagtgccttctcaaacatgagttctgcatatggttgtgcagaaatcaaaatcttaaagagagatgagtaaagtcaagtttgtaatattaatcttatattctcaatatagatgctaattagtgctctgaatggttgtggttagaaatcttgttggtatgatgtatcagtgatgtcactgcattgatggagacagaataatacataatggtgcaatgtggtgatggtaagctttgttactcaatattgtcaggcactttaagaaaatcagaaacattcaggatagtgccaaagaagatcagtttttcaagactctaaaatcatattcaattatatgtgtatgtaattataaatatgtgcatcatggctgactttgagaagaatgcagcgccttgcaagtgcactatttgaatagagctaaggagaactatagtctaaggactgcaaaagtctagatggagaagacaaaagcaatgacacttgttttctctacagaacaaatagacaaagaggtgaatgacaacaaagatgttcagagaaacttgaaaaataagctacggtgtagggtaagttgtattaaatgatgaaaattaatatgtaactgtatgggtaaaccaaatcatttgtatcttataatcttttttttggtagctacggataatattataaatggaataatcactaaaattctaaatataatgttttctagtaagaacattttattttttttttaatagagacagattctcactctattgcctaggctggactgcaagtggggccattatagctcactgaagcctcaacttcctgggctcaaatgaccctctcgtctcagcctcccgagtagctgggactacaggtgcacatcaccacatccaggtaattattttactttttgaatcatgatatgtagcaaccaatctgggaattatttattcataaaagataacattttcctgctaactccaacctcagaaaaaatgtattatgcctgactcaaatatgtcattatttttatgagaaaaagagtcatattgaagtaattatgtctatatgtaataattatcattatttgagataatttgcattggggagaaaagcaggcaatcagaaattacatattcaaggctgggcgcagtggctcacgcctgtaatcccagcactttgggaggcagaggcgagtgaatcacctgaggtcagagttcaagaccagcctgaccaacaaggagaaaccccatctctactaaaacaaaacaaaacaaaacaaaacaaaaaaagccacaaaattagccgggcatggtggcacatgcctgtaattccagttactcgggaggctgaggcaggagaattgcttgaacctgggaggcagaggttgtagtaagccgagattgtgccactgcacgccagcctgggcgacaagaacgagactcagtctcaaaaaaaaaaaaaaagaaagaaagaaagaaattacatattcaggttctagcaaatgcagttctctaataaacactaaataaatcataatacaagttacagttaaacctaattgttttactatataggatgtatcttttttgtacctatattttatcttcctttgcttctctggcctctattgggaggcagcacggtagtgaacacctcggggatctttctggttacgtaaacctgagttttaattttggttcatactaccttttaactttgggtagtctgctgagcttgttttttgttttcactcatctgtcatatcaagctagtaataattctgccatggttttggttttcatattgaaaggcattacataagcaaaatgcataacatataaatattagttccctttccactatgcatccaatctccctattaaattaagcctaaaaataataatttttgttttattaaaagccttccacattctacatatgaaagggattttttaaaggtgttttagataaaaaatgtttcaaccaactgaccaagaatatctcttcatatttatgtcatctacataaaaacttacatttatatcatatatcttttagtcttcttttctatattcttgattgtcatgttgtacagccagaaaagaatgagtataaattatctagattttttaaagtgcacattcaaacatagaaaatctaattattttacttgtttcttagtattaggctgaggccaatgagtccatgagctaaagggttgaaacttggcaccaaaaaagtgattgtttatgagtcctgtagatttatactgagaaaacatcatgtcttccaatgtgaaatacactaaaacctgattttttgtctcttaaggtgtgctaggtgaatgcaaaaaggatcaggaaagggggtgaggataggtcaggaaaagtgcaaacacaatgttctattcataaattagtgatggcatatttaaggttaagtagtaaaaaatatggggggctcagttaacacgaatgaaaaaatagttaaagtagccatgaattatctggataccttgatttaatgacaccctttcttctgtacaatttcataatgtgggaatagagattagtggggattgtagtggtataccctgactttgcttcatgatatctcaaatgtttaaaacctattattccctagagaaagaaatatgttcatactaattgttgcagaggcagaagccaaatatatctcctcctccatttatgtgactatatagtaatgaaaatcctaggttgatacacttttctcaatcttggaaagattctgctaaagcagcaaatcttctaacaagttcaagagggtggggagagtgaacaagtagaataatttatattaccctggaacaattctgaatcctgtaggtatttatgtcactgtttcaattgtgttctggtttaactgtcaatatttatgcatagcagttaacgtgtgtgcatatttgtaactgtgcagtgctactgccaggtgtgactgtacaaatcatgtgctttgaatgtgcaagttttactttcttttctaacaatttaatacagtgttagaaataaataacgaatgaagacaaccaaagagcagccagacaaatgtgaactggttttgacgtgacgagaaactcatcagtaagtaaataaacctcctccctggagaaggccactgaaatgcacccaggaggatgtctctactagaaggtaataaaaaatatatataatgtagtctttgacctaaaacctcatgattattactttgccatttatttccccctggtatctgatgttcatattagtttaatgtgccttttcagagaattcaagacactttttggaaagtagaatttttttttgaaaatttatgattggagaggtactacacaatttagaggttacatttcttgacaaatctgagttgaataaaaaagaactaaaaatataaacatagctaattcaagaatcaagatcgggtgaaactaaattaaaaacagccataaagtcccacattttccctaatttatttacctatgatattggcacatcttgttttacttaacatttgaaaaatacaaatatctcttcatatgcaaaagagcaaatgttaaatgaaaaactgaattttatatagcttcctaaatatgagccacatgcttaagcagtgaattaactttatgaatcaaatgtttaatgttaactattacaaaagcctggtatccaggtgcaatctcaccagaaaaaaatagcacctgcctttattacaataaaaaaaatggctaattccctttgacatcttaagagtgacactactttgtcaagcactaaatactttttaaattaatcatgttaaacttcagatttatagatataaatattgtatttataactttagtcataatgtacaatttctttcttgtttaaaagtactttctcactcaaaatggtatttatagtttaaaaagaatatgcctctgtattcaggagtgattcaaattcccagatgttttcacatagttatgaaaatgggaaagtgctgaattaaactgggctgcaatatttcaagttttttgctatcaggttataaactatacctacgattgcaagtcatacagtgcctctatttctagaaggcttttaaagtttcctggcttagttatgtccaaaggcagcaggaagtctcatcagtagagggcagaattttcaagtgctgccattcttatcccaggaggcatttccagtggttgagcacaaggcctgtttgtagtttgcttttgctcttgcattttgtggaagggaaggaactgagagagcttagagggttcattaaaaccacccctcactctcttagtcgtagtcagatggagtattcataacagtaacctccaattaccactatgtgttgggaaaaattagaattcggtctacttacaatcctgccaactaggattttactttgatatttcagtataacagtgaatctggattgatgcctgattaaaataaaatccctgattattactttctggattacgaactaaaatccctgtaaaatcaatggatgtgactcattgttaagagtcatgcagacttttacatattaggtaagaattctaaaaattatttgagggttctattctctagcaccaggtactaatgctccctactcaaaaaaaatcatgtgcatggattaatcaagtctaacagtgctcagatttaatggtttaacattgattttcttttctttgtcaaacttatatatgcaaatatttttatagtagtcagatgttatttttgaataaggatcaccctcatttttacccatgtgcttatctttaaaaccaacattgtaaagtagcacgcagacatatgtttcttttatcttcatggattatttttaccttaaaaataaattatcatttttttttttgaatttgggttttattctccagatactctgtgtacatgtgggtaagtatgtgggagtatgtgtgtttgtgtgtaagaggggataattaattgtctctcaactctatctcatactttaatatcaaataaaaaatgaaatgtataaagggtcactttgtaggattaggcatcctccttctacctacttaaaccaggggtttgggattcagaattctccatataaccaagaccgaaagtcactggaagactttaaaattagtattttaaccaccacacccagagtcaggtatggaaataaacctatagcatggattctttctatgcataatctcaaaatttaactacccaaataagtaagtttttaaaaactaatttaaaatttgccattgaggaaaatatcacctccatccttaattgtgactcctcatttcagctaaaaccttttctaatactttaaaaaaacaaaatgaaaaacaaactcctagataaagtcataaacactgaaatcagagatgtgattcttgttaaatgttagtttctctttctgaggttacactctgtgcatttgaaactttgacgttaacatcttccgaatgtttagatttgctcaagggttcagattctctggtcttctgccttgcattttcctccttcctttcctttgcaagcaatctatagttgatagcattgccaatgagcagccacacgcttgctgctaccacaatagccccacaggacatgtacatgtatttatattctccagttaaatccaccaatttacctgcaagaggagggccaagaagaactgggccacactccacaattgtgacaagtccgacggcactggaaaatcttggtgcacccacgaggtccatgagagtttcaaagagaacactgctaacactcccaaatccaaggccaaaaaatacagcatataataccaggcttgtgtagtcctgtgccagtgggcacaagaggtgacacactccattgaacatgattgcaaaactgaagaagtactgaattcgaggtcgaatatatttggagtttgcaattaatcctacagaaggcctagcaaacatatcaacgaaagccataacagatagcagaaaagctgccgagtactcatcaattccttggtctttagcatatggagccaagaatataatgggggcaaaaaaacctaggaacataatgacatttccagacagatatatcagaaatcctctatgcttaaaaagggagaaatctaaatacttattaactttttcccaagttgatttcttcgttttgattttctttgggcttgaatcatcttctgttttgccagtcttatttttagacttagaagtggtttgattgggtccaaggggtctcatgagggaaccagccacacaggcattcaaaagtagacttcccaaaatcaggaagcttcctttccagccaaaagtattaaaaaggtactgattgaaaggagccaatgaacttaagaaaacaggacttcctgccatggccaatccatttgccatgggtcgcttcctatagaagtatttgccaattatggttaaggcgggttgcaggttgaaggctaaacctaaacctgtaatgaatcccatagtgaggtacagctgtaccacgctgctactaaaggaggccaacaccattccaagacagcataataagcctcctgctatcaccaccggccggctgccgtatttattcaccaaaacactacttacaggacttcactgaagtcctgagcctcttaaagtcacccatgaggattgaaataaacttcttccaaacttctgttaatgttggtattttgacctcctcccataacagtgaatgatcgtgatgttatctagaatagcaaatcctttccagaagattttccatctccttttcccagattcatcagaggagtcattatgtacggcagctgtaagcttcagtagaattgaagacagttagggccctgctctggattaggctctggcttagggaatgttgtgggtggtttgatcttgtatccaaacttctaaaactttcttcacttttcctttgcattcacaacttggctaaccttagtgctagacacctagctttcagcctgtgctttcagcacctttctcattaaggtgaatcatttctagcttttgatttcaaatgagagacttgcaactcttcctttcacttgaacacttagaagccactgtaggtttattaagtggcctaatttcaatactgttgtatctcagacagtagagaggccctaggcatgatcctgattgagtaaagctgcactgaatcctcaaggatgtgaagatcaaaaagctttcaaatattctacctcctgcgtacataacagccagcataatggatgaaatccatgctatttcactgtaggtagtgtggaatatttgctgaatttctttgaagaatacggtgacagctttggggaatgcataggaaaatccaatggagataaaagctgctccaaccacaatccaaccccatcctccatctggaggtggatgcacaggtggggcacttggcattggtggcatttctgctcctctagtggaaattcaagtaacctggcgacaggtgtttagaaacatggtcttccatttcaccaagacataagtttccctgatctatggactcctctccccacctgaggcagaagtttccttgtgaaccattgctctttttagaatcctgaacatacttagttccatctatctctttgtcactcaacactttgtcagctagtctcaggattctatgaccccttcccctagctcacttgagtaatcataatatgggaaaactaatctaaatgccaactctgagaag

SEQ ID NO: 17839 - RNA, 11694 nt, Homo sapiens
  source 1..11694: mol_type = other RNA
tcgaggagctcacagtctagtaagaaagagatgaatttgaaaatatatttgaaactgtaggcaaaataagtaccctcacagagaaattcaacatttggtttcaaatttgttatgcagtgaaaattagaaactacaaccaagatttttttaaaacattatgttcatataacgctgtagtatacctgaaaggcaagaacttaaacaagtgtgctgaaaaacaaattaggaatatttgaacaaaatatactttaaaaatgatcaacaacgtaaaatattcctgatttaaataaatctaagttattttatttagtttaagcaaaatatgtatccatatgaaaatgccagttctttcatttttggttaattcctttacacatattatttgctaagttcagaaatgctatatatacaaaaatttcaaaaataaataagtatcccaagatcacataacaatactttaagtacattcatgtgtaagaaggcaaaaaaagaaggttctatcttatattttaaaactttgacaggtattttaaatgtattattttatactttattttctttaaaaatgaaataatacagccatgatttaagtcatgtaaaaacaactgtttggatcatttaggtgtcaagcaaaactatcctctttatttcactatcatagtaaccatagttgatagaccatgtggcaatatgatcatttgttcagtggtcattaagatatctatagaataaacaagacaactacattttatttttttcacttaaaaatcacaaaaatacagcctaaaatataatttatattttaaaaataattctaaacattaacccctaaatctaatcccttaaaaaattcttgcaaaagttagctggatgtggctgttgccaaggaatgtcttttattagcaacaagtgactatctataacttttattccaacaatcttattttaaatatttgtttcaatttaatgctgggattagaaaaacatatttgttcaaagtatgtaagtagtaagtaaaacaatttcaaaaatctatcaaaaaaggagaattattcattctaggaaataattaacatactggtttaaaatatctgggagaagaacttttacataaaaagcttcaaatttagtcagttgtagcaagcacttgaaaagaccctgctctttcatctgcaatatcaggaattactatatctgactcatatttgattaagttacaatctcatttttgttgtcactacaaagaaggatccttatattagtaaatgcactcactgcaactactgaggcctgcctcctgtcagaatgacaatgcagtcttagcatacgggtgtcggtttggctgaatctaaccaaacacatcacgtactacagatgtttttagggcccacccaattcataaaagattttactgcgatacatgagtttacccaaatttttattaaaatgtgtttttagggtaaatatcttgatgaactaggcaaacaaatactgaatgcagattactgtttttacagttttaccgggaaaactcctaatagcaacccctcttccccttcaccacagatctttaatttaggtgtgatttttgtttgttctctacatgggaataaaggagaaagtttagaaagactgtatctagctagataagatgcagaggtagatggaatctctaacataaaagaagctctaattacactgttgccagacagctgttatggattttagtattgtttattaggtgaagaaaacattcataaaataagaaatttttgagatagaacttactctaataatttcattaacatatgttcaggttcttagatcaagaaatactgtagaggtgttctcctcaagactatgctatggcaataatttcttgcatacaatttaataatttaaacttgaactgtgtgttctgtgctctggcgttctacttcagaaaaaaatgaacactgcttctaaaataaaaaggaacataaaataaaaaaggaattaatgagatattgacatgttttctattaatacaatattgatgttttaaatgattttgatattgctataacaacatatattgtgcaaaataattaatctcactaaatattatttctgatttgccacgaattatctgccgtggcaatcaggaaatagtcttcaaagtaagtttgcaaacatgattttgcaaaccatgattggaaaaatatattcatttgggctataaactatcaagtagggttgttatatatatttctaggaaaatattttatttactctacaaagatcatcattatgaccttacggcttctgtagtgcaatggagaaaaaagtgtgttagaagttaaaagacctgaattctatctccaaccctgcatttattcagagtattggtataggtttaggcaaaatccttaatccagtctagttttatatggtaaaaatgtggatacctatcaaaactgagggttgagaggatgaaatgaattcattaaacatatcttctgagacataaatatatcaaaacaaatcaaaatacaattagatctaatgtttagaaataaatattttaattcatatttgctatttcactaaatctagaaatactaatgctttagttaaatatagaaagttgatgatagaaaaataaaatccatcgtaccattgaaaagcttgtcagaaatatgtactcttgagattcggaggatgagaaaaaaaatgtgtactctaacgaggaagctatataaactgagtctaactcaaaacatttattttagatgcatataagaattaaagtcttagtcaaaagaatgttttaaaatttcatcctaaatttatgtgagataaaatgccattcttttgtttttctgaacagaggagcttttatcaacttattctattttatttttatttttattattttattttattttatttattattattatactttaagttttagggtacatgtgcacaatgtgcaggttagttacatatgtatacatgtgccatgctggtgcgctgcacccactaactcgtcacctagcattaggtatatctcccaatgctatccctcccccctcccccgaccccaccacagtccccagagtgtgatgttccccttcctgtgtccatgtgttctcattgttcagttcccacctatgagtgagaatatgcggtgtttggttttttgttcttgcgatagtttactgagaatgatgatttctaatttcatccatgtccctacacgaacttattctattttaatagaatgttcagtatcagtgttttcacactgagattctctagcttattttgccatatttaaattaaaaagaaacaaaaaatcctgtttgatcatgtgaaaaatatttactgaaatgtgaataaatttatgatcattaattgcctactgaaatattcctgaatattgctcaccttattaacaagtatatatggagactgaaaaacatgtagatcatgcaaacaagtgtaactaactataccaaagaaacaaaagtccatactaaatatgtccataattaaataaaaaatgctaaacaagttttacctagatattataaaaacatagaaaggaaaacatttaggagatgatgaagaagcaggagattgggatgggagatgtaatttgatctaaattcccatatgcttctgtaaaatcaaaaattcattttgcaatattaattttgctcttaaggtagagacttttaaaatgaccattctcaatactacagcaattcttccctgatttgcacataaatgaattaaagtgaagaaaaagcagtagaggagagaagactaaaataaaccagattgtagcaccctgtaaagagctaaaatctccagtgtacaaacaactgataggaaagaagagaaaatcagaactataaaaaagtgacataagctcagaaaattactcatttttaattgtatcaacaaagataatttgtaattttgatcatgcaagcattataattactgataattgggcctttcagcttttaagtgccttctcaaacatgagttctgcatatggttgtgcagaaatcaaaatcttaaagagagatgagtaaagtcaagtttgtaatattaatcttatattctcaatatagatgctaattagtgctctgaatggttgtggttagaaatcttgttggtatgatgtatcagtgatgtcactgcattgatggagacagaataatacataatggtgcaatgtggtgatggtaagctttgttactcaatattgtcaggcactttaagaaaatcagaaacattcaggatagtgccaaagaagatcagtttttcaagactctaaaatcatattcaattatatgtgtatgtaattataaatatgtgcatcatggctgactttgagaagaatgcagcgccttgcaagtgcactatttgaatagagctaaggagaactatagtctaaggactgcaaaagtctagatggagaagacaaaagcaatgacacttgttttctctacagaacaaatagacaaagaggtgaatgacaacaaagatgttcagagaaacttgaaaaataagctacggtgtagggtaagttgtattaaatgatgaaaattaatatgtaactgtatgggtaaaccaaatcatttgtatcttataatcttttttttggtagctacggataatattataaatggaataatcactaaaattctaaatataatgttttctagtaagaacattttattttttttttaatagagacagattctcactctattgcctaggctggactgcaagtggggccattatagctcactgaagcctcaacttcctgggctcaaatgaccctctcgtctcagcctcccgagtagctgggactacaggtgcacatcaccacatccaggtaattattttactttttgaatcatgatatgtagcaaccaatctgggaattatttattcataaaagataacattttcctgctaactccaacctcagaaaaaatgtattatgcctgactcaaatatgtcattatttttatgagaaaaagagtcatattgaagtaattatgtctatatgtaataattatcattatttgagataatttgcattggggagaaaagcaggcaatcagaaattacatattcaaggctgggcgcagtggctcacgcctgtaatcccagcactttgggaggcagaggcgagtgaatcacctgaggtcagagttcaagaccagcctgaccaacaaggagaaaccccatctctactaaaacaaaacaaaacaaaacaaaacaaaaaaagccacaaaattagccgggcatggtggcacatgcctgtaattccagttactcgggaggctgaggcaggagaattgcttgaacctgggaggcagaggttgtagtaagccgagattgtgccactgcacgccagcctgggcgacaagaacgagactcagtctcaaaaaaaaaaaaaaagaaagaaagaaagaaattacatattcaggttctagcaaatgcagttctctaataaacactaaataaatcataatacaagttacagttaaacctaattgttttactatataggatgtatcttttttgtacctatattttatcttcctttgcttctctggcctctattgggaggcagcacggtagtgaacacctcggggatctttctggttacgtaaacctgagttttaattttggttcatactaccttttaactttgggtagtctgctgagcttgttttttgttttcactcatctgtcatatcaagctagtaataattctgccatggttttggttttcatattgaaaggcattacataagcaaaatgcataacatataaatattagttccctttccactatgcatccaatctccctattaaattaagcctaaaaataataatttttgttttattaaaagccttccacattctacatatgaaagggattttttaaaggtgttttagataaaaaatgtttcaaccaactgaccaagaatatctcttcatatttatgtcatctacataaaaacttacatttatatcatatatcttttagtcttcttttctatattcttgattgtcatgttgtacagccagaaaagaatgagtataaattatctagattttttaaagtgcacattcaaacatagaaaatctaattattttacttgtttcttagtattaggctgaggccaatgagtccatgagctaaagggttgaaacttggcaccaaaaaagtgattgtttatgagtcctgtagatttatactgagaaaacatcatgtcttccaatgtgaaatacactaaaacctgattttttgtctcttaaggtgtgctaggtgaatgcaaaaaggatcaggaaagggggtgaggataggtcaggaaaagtgcaaacacaatgttctattcataaattagtgatggcatatttaaggttaagtagtaaaaaatatggggggctcagttaacacgaatgaaaaaatagttaaagtagccatgaattatctggataccttgatttaatgacaccctttcttctgtacaatttcataatgtgggaatagagattagtggggattgtagtggtataccctgactttgcttcatgatatctcaaatgtttaaaacctattattccctagagaaagaaatatgttcatactaattgttgcagaggcagaagccaaatatatctcctcctccatttatgtgactatatagtaatgaaaatcctaggttgatacacttttctcaatcttggaaagattctgctaaagcagcaaatcttctaacaagttcaagagggtggggagagtgaacaagtagaataatttatattaccctggaacaattctgaatcctgtaggtatttatgtcactgtttcaattgtgttctggtttaactgtcaatatttatgcatagcagttaacgtgtgtgcatatttgtaactgtgcagtgctactgccaggtgtgactgtacaaatcatgtgctttgaatgtgcaagttttactttcttttctaacaatttaatacagtgttagaaataaataacgaatgaagacaaccaaagagcagccagacaaatgtgaactggttttgacgtgacgagaaactcatcagtaagtaaataaacctcctccctggagaaggccactgaaatgcacccaggaggatgtctctactagaaggtaataaaaaatatatataatgtagtctttgacctaaaacctcatgattattactttgccatttatttccccctggtatctgatgttcatattagtttaatgtgccttttcagagaattcaagacactttttggaaagtagaatttttttttgaaaatttatgattggagaggtactacacaatttagaggttacatttcttgacaaatctgagttgaataaaaaagaactaaaaatataaacatagctaattcaagaatcaagatcgggtgaaactaaattaaaaacagccataaagtcccacattttccctaatttatttacctatgatattggcacatcttgttttacttaacatttgaaaaatacaaatatctcttcatatgcaaaagagcaaatgttaaatgaaaaactgaattttatatagcttcctaaatatgagccacatgcttaagcagtgaattaactttatgaatcaaatgtttaatgttaactattacaaaagcctggtatccaggtgcaatctcaccagaaaaaaatagcacctgcctttattacaataaaaaaaatggctaattccctttgacatcttaagagtgacactactttgtcaagcactaaatactttttaaattaatcatgttaaacttcagatttatagatataaatattgtatttataactttagtcataatgtacaatttctttcttgtttaaaagtactttctcactcaaaatggtatttatagtttaaaaagaatatgcctctgtattcaggagtgattcaaattcccagatgttttcacatagttatgaaaatgggaaagtgctgaattaaactgggctgcaatatttcaagttttttgctatcaggttataaactatacctacgattgcaagtcatacagtgcctctatttctagaaggcttttaaagtttcctggcttagttatgtccaaaggcagcaggaagtctcatcagtagagggcagaattttcaagtgctgccattcttatcccaggaggcatttccagtggttgagcacaaggcctgtttgtagtttgcttttgctcttgcattttgtggaagggaaggaactgagagagcttagagggttcattaaaaccacccctcactctcttagtcgtagtcagatggagtattcataacagtaacctccaattaccactatgtgttgggaaaaattagaattcggtctacttacaatcctgccaactaggattttactttgatatttcagtataacagtgaatctggattgatgcctgattaaaataaaatccctgattattactttctggattacgaactaaaatccctgtaaaatcaatggatgtgactcattgttaagagtcatgcagacttttacatattaggtaagaattctaaaaattatttgagggttctattctctagcaccaggtactaatgctccctactcaaaaaaaatcatgtgcatggattaatcaagtctaacagtgctcagatttaatggtttaacattgattttcttttctttgtcaaacttatatatgcaaatatttttatagtagtcagatgttatttttgaataaggatcaccctcatttttacccatgtgcttatctttaaaaccaacattgtaaagtagcacgcagacatatgtttcttttatcttcatggattatttttaccttaaaaataaattatcatttttttttttgaatttgggttttattctccagatactctgtgtacatgtgggtaagtatgtgggagtatgtgtgtttgtgtgtaagaggggataattaattgtctctcaactctatctcatactttaatatcaaataaaaaatgaaatgtataaagggtcactttgtaggattaggcatcctccttctacctacttaaaccaggggtttgggattcagaattctccatataaccaagaccgaaagtcactggaagactttaaaattagtattttaaccaccacacccagagtcaggtatggaaataaacctatagcatggattctttctatgcataatctcaaaatttaactacccaaataagtaagtttttaaaaactaatttaaaatttgccattgaggaaaatatcacctccatccttaattgtgactcctcatttcagctaaaaccttttctaatactttaaaaaaacaaaatgaaaaacaaactcctagataaagtcataaacactgaaatcagagatgtgattcttgttaaatgttagtttctctttctgaggttacactctgtgcatttgaaactttgacgttaacatcttccgaatgtttagatttgctcaagggttcagattctctggtcttctgccttgcattttcctccttcctttcctttgcaagcaatctatagttgatagcattgccaatgagcagccacacgcttgctgctaccacaatagccccacaggacatgtacatgtatttatattctccagttaaatccaccaatttacctgcaagaggagggccaagaagaactgggccacactccacaattgtgacaagtccgacggcactggaaaatcttggtgcacccacgaggtccatgagagtttcaaagagaacactgctaacactcccaaatccaaggccaaaaaatacagcatataataccaggcttgtgtagtcctgtgccagtgggcacaagaggtgacacactccattgaacatgattgcaaaactgaagaagtactgaattcgaggtcgaatatatttggagtttgcaattaatcctacagaaggcctagcaaacatatcaacgaaagccataacagatagcagaaaagctgccgagtactcatcaattccttggtctttagcatatggagccaagaatataatgggggcaaaaaaacctaggaacataatgacatttccagacagatatatcagaaatcctctatgcttaaaaagggagaaatctaaatacttattaactttttcccaagttgatttcttcgttttgattttctttgggcttgaatcatcttctgttttgccagtcttatttttagacttagaagtggtttgattgggtccaaggggtctcatgagggaaccagccacacaggcattcaaaagtagacttcccaaaatcaggaagcttcctttccagccaaaagtattaaaaaggtactgattgaaaggagccaatgaacttaagaaaacaggacttcctgccatggccaatccatttgccatgggtcgcttcctatagaagtatttgccaattatggttaaggcgggttgcaggttgaaggctaaacctaaacctgtaatgaatcccatagtgaggtacagctgtaccacgctgctactaaaggaggccaacaccattccaagacagcataataagcctcctgctatcaccaccggccggctgccgtatttattcaccaaaacactacttacaggacttcactgaagtcctgagcctcttaaagtcacccatgaggattgaaataaacttcttccaaacttctgttaatgttggtattttgacctcctcccataacagtgaatgatcgtgatgttatctagaatagcaaatcctttccagaagattttccatctccttttcccagattcatcagaggagtcattatgtacggcagcttcagtagaattgaagacagttagggccctgctctggattaggctctggcttagggaatgttgtgggtggtttgatcttgtatccaaacttctaaaactttcttcacttttcctttgcattcacaacttggctaaccttagtgctagacacctagctttcagcctgtgctttcagcacctttctcattaaggtgaatcatttctagcttttgatttcaaatgagagacttgcaactcttcctttcacttgaacacttagaagccactgtaggtttattaagtggcctaatttcaatactgttgtatctcagacagtagagaggccctaggcatgatcctgattgagtaaagctgcactgaatcctcaaggatgtgaagatcaaaaagctttcaaatattctacctcaagtagatggtgatctctttaaagggtgaatgatgcattccgcttctccttttttcctcctgcgtacataacagccagcataatggatgaaatccatgctatttcactgtaggtagtgtggaatatttgctgaatttctttgaagaatacggtgacagctttggggaatgcataggaaaatccaatggagataaaagctgctccaaccacaatccaaccccatcctccatctggaggtggatgcacaggtggggcacttggcattggtggcatttctgctcctctagtggaaattcaagtaacctggcgacaggtgtttagaaacatggtcttccatttcaccaagacataagtttccctgatctatggactcctctccccacctgaggcagaagtttccttgtgaaccattgctctttttagaat

SEQ ID NO: 17840 - RNA, 1557 nt, Homo sapiens
  source 1..1557: mol_type = other RNA
tcgaggagctcacagtctagtaaggaagacatatggggaaccgattccccaaagatgcggggagtaggggaggcagtgcttagagtggggagccattgtcccacccaccccacgctccaaagtccaggctggctaggagaaagtgagtaggaagcttagcatcctctctctcaccttccccgtgacagctgacttctctcactctgtcctaacatcacaagaggacaagcggagagacaaggatgagaaggatacaggagctgtcctcaaaaagctagaacacccctggcagaatatatacaacggtattttatttcccaaagccgcaaaccagcgcagcagaagctggggatactggggaatgttggaaaaacaggggctgggccagcccagtccagtggtgggaacaggaagtgatgagaagaggggtacccagggccagagaagtaggtgagagggaaatttccaggtggagaagctcacagtaggacaccagcagccacggccaacagaagggctgccaatccagctgtgggagccacacagcctttattatggggctgctggggccccccttttgcaggatactgccctgaattgctgcggtcctggtggccagcggcgcctccagtcaacctgggctcctcatcccgggaggcctcgtgttctactccctgtctcggagtctgactggttggcgctggcatgggtttggtggtggatgtgggtctcactggggccgaggtagaagtggtgacagatgtggttgaggccacagtcgtgggctctggagggggcagccggacaaggggtgggattcgaggggagaagtaggtcttgttgcggaggtcagagttacagcgggacccctggcaacaggagccactgagcgtgaaccctgggcctgttactccatcccgagtgcagaattcatcctggacacagccccggacaggcaaggacacagtcacattagctgccgtcaaggtgacgttgccgtcgaagcagcccttgtagacatgatcgctggcgttgtagcagctcacgaccggcggcgatgtaccctggcacgcctcccggctcaggcccacacagctgtagcactccacgccgttgggcgggtatgcactctcattacctgccgggtcgagcgcccgcgaggtgaggttgagcttggcgttgcagcgatcctgagcgcattgctgcagctggatgaacgccagaagcccgtgaagatccaggccgcggtcattcttgccggggagtcccgaaccgcaaccccgcactgccagcgagaattgtccgtggatggtctccaccgcccccacggcctcggtgcagacgtccacgcccggcgcgcacttcactgtcttcatcttgttcggggagcatccgtcatctgctttctgcacgcagctgtagcactccagggcctgcgctcctccgcgaagcagcagcagcagcagccagcctgcagtccagatcatggcctgggcacctgctttcctggcggggtccatggctccgtcctgctcccttggcgtcccccctggatgt

SEQ ID NO: 17841 - RNA, 3228 nt, Homo sapiens
  source 1..3228: mol_type = other RNA
tcgaggagctcacagtctagtaaggaaggtaaacataaacaaatcattacaatacaacaggaaaagagctagagcgaagatatagaacaattgcacagaggaaagagtaactaattctgcctgaaggtaacaaggaagagatggcacttgattttgaagtttaaggatgagtgatattttagcacggcagagggcagagggggcacagggcattccaggcagagggaatagcatgtgcaaaggcactgaggtaaaaacatgagcatggttggttcagagaatggtgttgaagggtacacagaggcgggctgtaaagggtcttgtacaccacactaggaagtttgaattttatcctgtaggcaatgggaaggcttcaagcccacatctctccatctggttcacaaggatatcataagaggctctgttaaatgccttgctgaaatccagttacattatgtctatggcactttcctggtcttccagtctagtagcccttgtggcccaggagatgccaccttggggccagtgatctctaggtttgcttggtaacgatgtccattttctatctgacctgtttctacttttttcccaggagttttcttatgatctcctttgggtttctttacacgtttgacctggaatgtaatccattctgttgcttcatcatcttcacttctgcagtctccatagcaagagcttctggccactccatcctggggacctttcttcagcacccgtattccttgtaagtctagacgccgccctttcatctctagtgcacccccaaagccttccaaaggccatgcctgttgaaattcatccaccaaagccagtatttcttctgacattttggtttcatctgaattctccatctcatcagaaccattgctctcctcaaccaccgtaccactgcaaacagaagaagtgatgttgtacagaaaaggataaaactgcatacagcggatcaacttcaggctgttttcacactctggacatttggtggttaatttcaaggcctgtctaaaggcctcaagtgccccactgatattcttcagagcaaggtaagcatttcccaggctcaaaaaggtcagaggctcagagctattgatggccaaagcttgaagtagcagcttagtggcatcaagatgaaggccgtaatgaatcaaaaggttggccaagttgacaagaggaacatcttggtattgaagtggagctaaattcaaagccctctgaagacaggcaatagcaaaagtgctatttcctactgctctccagtatagtccagcttcattgagtatgagccagataggagcatttggcttattaatagcatgaaataagaaagacccaatttcttcttctgggatagtatagttattaatacgggaaagcaaaatttttcgtgcatggtcatctggcattttggctttcagatccatgcgaacctctaattctttgactaagtaggacagagtgtggctttttctgaagtcagttatggaacagtcaggggtttgggcctcttcttctgtagaataatcatcactgctgagttcgtggatcctgagtcctttgttttccggaggcagaaaatacgttggcaattccccaccaacagggactctagggtagctttctgtacaatctgctcttttaggccatagaatatgctgtttgtccctatatgcatcagagtccctgccccaaatccagagaatagaatgggctacgggagaagacttgaccgaatcattgatatcactctgatttgattgaacatcaaagttcacagacatcatactggaggttgatgaatcctcaccaaactgaacatagtccacattttcaaagatatctccacgatgatagcgtacaggctggtcccactggcaatgtaaactatgctgctggttgaccagtcggcatatctgatgatttcctaattgtgcctcttttgccatctgagtctcatgaatgatatttcttaagatttgctcctcctgaatcagtttatgtttttctaggatttcctgctgtctcaggtagtggtcatgctgcttttgatactcttttaactcattcagtgttcgctggagagatctatgctgagcctccaatttctgctccagtttttgctgacataggacagcatgcttcctctttatagcttgctcaaacccaggtctggcctgcaaagcgtggtcataacagagcactgagtggttatattccccaagcattgcatatatattccccaaagtgtaatagctggtgaagaagtcactgtcatccagagctgcatggaccacgacagcagcatcagcagagaagtgtgctctgtgtagaacgtttgccaggttgaccagggcaatgtctttattgtgcctggaagagaagtgaagtgctcgcatggcacattctactacctgatatggctcattcttaattctccagtaaaatgaagccatgttatacagtacccacgaggaagtgttcttctgtaggccttcatgaatgaggtgacctatgtcatctatactccttcctaaccgtttagataaatatgtgaagattgggtcttctttaggtagcagaggtgcagaaagattaactctctcctgtacacctctcaagtgctgaaaagcatgtatactatatggaagttctagaattttagtacaatcaggttgctctgggtctggagggacaggagattctgtgtctatataatcttcaggactgatgtctttgctctccaaagttatgtatgtgccatcatatagatccaggtcccctaagggcaccttggctttgatgcagtctgggtcttctttattatgtctctgttccagtcctgtgtctctgtcctcattctcttctatgtgaattttttgagcaactaattgtttctctaattctttgaggtagttaactgttgcttcttgtctcattaatatgactaggtcatgaggatgcttcaagttcattggtgaatccacctgctgctggattttcccgtcctccgtgacgacccagtgcgtggtggcgaaggcccctcgtgccgccacactcagcaaggcggaaaggctgaggagccagcctgggccggagcaaggcggcagctcgtaccggccacgaacccctactgccgccgccatcttgcccccccggccgggccgctcacaccggaagcggaagctagtctccggcgcccgccatcttgaagag

SEQ ID NO: 17842 - RNA, 3364 nt, Homo sapiens
  source 1..3364: mol_type = other RNA
tcgaggagctcacagtctagtaaggaaggtaaacataaacaaatcattacaatacaacaggaaaagagctagagcgaagatatagaacaattgcacagaggaaagagtaactaattctgcctgaaggtaacaaggaagagatggcacttgattttgaagtttaaggatgagtgatattttagcacggcagagggcagagggggcacagggcattccaggcagagggaatagcatgtgcaaaggcactgaggtaaaaacatgagcatggttggttcagagaatggtgttgaagggtacacagaggcgggctgtaaagggtcttgtacaccacactaggaagtttgaattttatcctgtaggcaatgggaaggcttcaagcccacatctctccatctggttcacaaggatatcataagaggctctgttaaatgccttgctgaaatccagttacattatgtctatggcactttcctggtcttccagtctagtagcccttgtggcccaggagatgccaccttggggccagtgatctctaggtttgcttggtaacgatgtccattttctatctgacctgtttctacttttttcccaggagttttcttatgatctcctttgggtttctttacacgtttgacctggaatgtaatccattctgttgcttcatcatcttcacttctgcagtctccatagcaagagcttctggccactccatcctggggacctttcttcagcacccgtattccttgtaagtctagacgccgccctttcatctctagtgcacccccaaagccttccaaaggccatgcctgttgaaattcatccaccaaagccagtatttcttctgacattttggtttcatctgaattctccatctcatcagaaccattgctctcctcaaccaccgtactttcaagtctaagggcatctgagtccctccctgaattctcaacagagaatacagggtcctcctctgttcctctctcagagggctcttcttcagcagcatccagtgactgtgagttgtcaaaatatttctgtttgtcatggctgttgtccagggttttctcatgacaattaccactgcaaacagaagaagtgatgttgtacagaaaaggataaaactgcatacagcggatcaacttcaggctgttttcacactctggacatttggtggttaatttcaaggcctgtctaaaggcctcaagtgccccactgatattcttcagagcaaggtaagcatttcccaggctcaaaaaggtcagaggctcagagctattgatggccaaagcttgaagtagcagcttagtggcatcaagatgaaggccgtaatgaatcaaaaggttggccaagttgacaagaggaacatcttggtattgaagtggagctaaattcaaagccctctgaagacaggcaatagcaaaagtgctatttcctactgctctccagtatagtccagcttcattgagtatgagccagataggagcatttggcttattaatagcatgaaataagaaagacccaatttcttcttctgggatagtatagttattaatacgggaaagcaaaatttttcgtgcatggtcatctggcattttggctttcagatccatgcgaacctctaattctttgactaagtaggacagagtgtggctttttctgaagtcagttatggaacagtcaggggtttgggcctcttcttctgtagaataatcatcactgctgagttcgtggatcctgagtcctttgttttccggaggcagaaaatacgttggcaattccccaccaacagggactctagggtagctttctgtacaatctgctcttttaggccatagaatatgctgtttgtccctatatgcatcagagtccctgccccaaatccagagaatagaatgggctacgggagaagacttgaccgaatcattgatatcactctgatttgattgaacatcaaagttcacagacatcatactggaggttgatgaatcctcaccaaactgaacatagtccacattttcaaagatatctccacgatgatagcgtacaggctggtcccactggcaatgtaaactatgctgctggttgaccagtcggcatatctgatgatttcctaattgtgcctcttttgccatctgagtctcatgaatgatatttcttaagatttgctcctcctgaatcagtttatgtttttctaggatttcctgctgtctcaggtagtggtcatgctgcttttgatactcttttaactcattcagtgttcgctggagagatctatgctgagcctccaatttctgctccagtttttgctgacataggacagcatgcttcctctttatagcttgctcaaacccaggtctggcctgcaaagcgtggtcataacagagcactgagtggttatattccccaagcattgcatatatattccccaaagtgtaatagctggtgaagaagtcactgtcatccagagctgcatggaccacgacagcagcatcagcagagaagtgtgctctgtgtagaacgtttgccaggttgaccagggcaatgtctttattgtgcctggaagagaagtgaagtgctcgcatggcacattctactacctgatatggctcattcttaattctccagtaaaatgaagccatgttatacagtacccacgaggaagtgttcttctgtaggccttcatgaatgaggtgacctatgtcatctatactccttcctaaccgtttagataaatatgtgaagattgggtcttctttaggtagcagaggtgcagaaagattaactctctcctgtacacctctcaagtgctgaaaagcatgtatactatatggaagttctagaattttagtacaatcaggttgctctgggtctggagggacaggagattctgtgtctatataatcttcaggactgatgtctttgctctccaaagttatgtatgtgccatcatatagatccaggtcccctaagggcaccttggctttgatgcagtctgggtcttctttattatgtctctgttccagtcctgtgtctctgtcctcattctcttctatgtgaattttttgagcaactaattgtttctctaattctttgaggtagttaactgttgcttcttgtctcattaatatgactaggtcatgaggatgcttcaagttcattggtgaatccacctgctgctggattttcccgtcctccgtgacgacccagtgcgtggtggcgaaggcccctcgtgccgccacactcagcaaggcggaaaggctgaggagccagcctgggccggagcaaggcggcagctcgtaccggccacgaacccctactgccgccgccatcttgcccccccggccgggccgctcacaccggaagc

SEQ ID NO: 17843 - RNA, 1113 nt, Homo sapiens
  source 1..1113: mol_type = other RNA
tcgaggagctcacagtctagtaatggagataagaaaattggagatttggtagtatatgatgatagttgtgataaaatattcataacctcagtgagtcaaaacagatttcacagggaacttaatgtctaacattaagtggagaggatcaccccagacaggtacagcctgctcggagaactgccaggacctccagtggggtgagcacggagctcaggggtcagggccaggaggtgactggaagcatctcacattttgttgtgtaaggactgagcatcctccgtgcagacaggggtgtggagtcagagtcctgttgcctgtttacatcagcgtttatcctttgctccatctcgtggcatgacagaacttttaacaactgaaaactgcactgccttgccacatgtatgtttatttgcacaatggctgtgagagcaagctggatctaccatgcaatggctgtgctctatctcctctgtgtgggaaatgcagggttctgaaatgaaaaagtcaggccggattctcaggctttctttgccacctgcttaagaaagtgcccgttttactgaacgcacaacacaaaagtttccatcttcttcctcatatggaaattttatgtgaaattttccctttttttttttttttttgttccttcacttccagaatcacaggctgcctgacaggattagcacgttccaggttccaactaaagccgtcttttgattgcaattgtggtgattgagtcatgaatgcagctttcaggactggaagttgctctggctgggtcagtgagcgagtggtgagtggatgtgaaagccttggacattactgtatgctactgcagactttacaagcactgtacacttagactcagcctcccaaagtgctgggattatagacgtgagccaccatgccaggccgaaacttgccatttttaaacatacacacttgtcctttatgtgatgttctcctggtgctgaatctgtctgccattcccagattgtggagttggggggtgaagttcctgaagtcatttctaggagggactcagtatcctatattcatcacaattgatgctgtaaccacagcatgagatgcacaggtatcctccaacatcat

SEQ ID NO: 17844 - RNA, 853 nt, Homo sapiens
  source 1..853: mol_type = other RNA
tcgaggagctcacagtctagtggaggagacagactgtgagcacttcaaagtgatttcagatgagggagcaattaactcaatatgggatttccaaattttgatatttgaacttgagggttcaggaagaggatgcacaagggcatggaagtgggaagaactggggggttcagggagcagccatggttctgtgtggctagggcaaaagagacatgggagatgctgagaggtcagcctggaaagcaggagggtgaggaagggagccccaacttgcttggcaagagactcccaccccaagcttcctcagtcattgttcaaattgtaatgggtacatttattaatgaaaacttttctttggtaatgaggtctgtgagttattcctcttctacatgaagaaggacttcctttgatttatcttatattgttcatttccatctctctatgcagcttgatgtagttgacacctcttaagttcctcattgcccttagtccagttacatgctcttttatgcttgagacactggcattgctgagttagcctgattctgtcttccccttgcccattccttgagatgcagtcctcggcagtaatcttttggccgtgacgtccaccgtgggttcccctgggccttccaaaggcactcatagcagttctcagccatgccctcaggatggcttggagttgcagtggtcacctcagatcttaaggtcactttggagatggaacccctgtgactgtcaggtctgctttgcctatatcacaggattgctgagctctcatcacagctcccgtgtggttgtaatcaccccagagggaaaaataatttcggttttttatggtttaattattggtgat

SEQ ID NO: 17845 - RNA, 4043 nt, Homo sapiens
  source 1..4043: mol_type = other RNA
tcgaggagctcacagtctagtgggggaaaaaagacacaagaataaataaatataatgtatttggagtttgcaaagggggccactatgggagacaaagaacagaggaacctaaatatcctatagttagcatccacaggaaagaaagacctggcaatgtacatttttgtaaagaatagataaggcagtggttctcaaagtgtggctggctaattacctacatcagaatcatttggagcacatattaacaagtagattcccagtaccttctgcacatattcttgatttagtacgtgtgtgggggggtggtgtacggttgaggcctgagaatctgcattttaaaagcactttaggtgatgctactgcatcttaaagtttcagaactgatgagataaagtttgttcttttaactggaataaagaatgatctacacatctgaaatgctaacttgtattagtctttaatgaggggcaagggaagtagagaaaaggatggtagttgatattttctactatagtgaagttaatttaattctcacaataatcctatgaggtagatattattatccctattttagatggaaaaaaaaccccaaaattagatagtttaagcaatttgttcaacagtatagagctaatgaatagcaacactaacatatgaacccagattcacttaactctaaagcctgtccactttctataacaccatgctagcaccaggggacaaatttactgattaaatggtacaattttctttgagttctttgccagatctttctaggtaaataaatataaagaacagctacgtggtactttagtcatgccccacacatttatccatggacacatcctacttggcagttggggactgaggacaaatccaggaggaatgattaaaacgaatggccacttcttactcctttttccatcatttcctcacccgctggtggaggtgtatcaatgtactatgtatggctaataactgggcccatctggaaagacaagcaaacataactggataccaataaaaacaaccccatctgatgtcaaaaattcttgggacccaaaacattcagaaggtcagaaggcatttaatgaaaatggcagggcagataagactcaagtttctcaaaagataaactgccaggaccagaagcaggtccagaatttacattagttaacagctcaacctttagagaaatagtgaaaggatagcagcttccccagtttaaaaaaatactatctgtctctctcaatacatagactcaaaggtgcaacaaaatagacacggctcagagaatagtgggatgtccaccctatttaaagagcttagggacaggcccaacctataaaaattcttctggaaggaagaaaacacacacacacaaactgcgaatactgcttaaattcccactcaccacattcagtgtcatataaccagatcttaggcaggagcagcagagtggagcatgttagatcaataaagaaatgtcaggccaggcacggtggctcacacctgtaatcccagcactttgggaggccaaggtggtggatcacttgaggccaggagttcgagaccagccagcctggccaacaaagtgaaaccctgtctctacaacaatacaaaaataagccaggtatggtggcatgcgcctgtaatcctagctcctcaggaggctgacgcagcagaatcacttgaaccagggaggtagaggttgcagcgagctgagatcacgctactgtactccagcctgggcaagacagagcaagacttcatctcaggaaaaaaagaaagagaaagaaatgccatggtaaaggcagctgacaacaatactgggggccttgggttcagaaggctggtgtgtaaccaccgtcctttcctatcactgagcttggagccacaacagtgacactacaaacgaaagatgggtttccagctctggagaacaactttcttatttctggcattccaaacaatttttcagtcccaagatgagttttgataaaatcagcccatagccctgacacaatggacagtacataactcagatttcattattttgtataacaaacattgtaagccagacttaaaaaaaaaattattgctatattttccccacatccaatctgggaacatttgctttcatccactttttcgtatcatgtttagagttgtttttaaaaaaatcatgcaaaccaggattaatcttctccttacaaaagaattttatttatactgcactgattcattccttcaaacacatagcttctaacaggtggagttagaaaagcgggtgccacaaactatggtttaatagtatgcaggccctgtacctgtttatctaactatacctgaaatttgctgataccccaagccagctacttacactaaaggcatctctggggggcatcatctagatgaagtctttaacctgatgggaatatctggttattctacagtttaaacaggatgtttggcttatgcttttgttcagctgactggtgcctgggaaggattaaagcccatatctaactacagcaggtcttcaagcttattatcctgtcatgagttcataaagatgacaaactcatcatttgggagctataaggtcaaagtggccagaatgcaactgcgctgttacactgtgcaaaatcaagtcaactgtcttgtaggtccttggctgtctcttgttataacctcgaacacttaaaaaaggaaacctcaagtatgctgagataattatcagaatgttcaggtacctttgttcctgaatatcaagtaatagggctcatctctgtgactgcttgcgacaagcacatagggcaactcattaccaactgctcattataaatgctgagctcttgagttcctgaggagggggtgggctctagactatcgagggctgagtcaactaggtgaagggccaacctgtacagttctaagtcttattttggttctgggcacatttcagttctgctccaagtccgctttgctccaattcagcgatgacagacatatatttgaactcatttggtctgaggttaaaggtctccactaacccgtaggtctctttccgatcagtagcgtagaagagctgaacttggttggcgatgcactgtgcctcagcaacattcagaaatgtggaatccatttctgcagtcatcagcactatgcccttttcttccttaagttcaggatagtgatataaaatcagctggctggctgcagcttcccctcgggtctgaatatttataagtgcagtgaagtggagttcagtacctgtccattgtcctacaaaaaactcataaccttcccttcttggcagagcacatagaaatgttggacaggactgagcccggttccagatcaaatcaaacttttctgcaggaataactgcgtagactgtatcttttgctgcaaaatattgctgccaaatctgttttatttcttctgcagttttttcttttaccatctcaatgttaaagattgaactgagagtcttgtccttagtgaatcctctgttcacagactgtttccccaaggcatctgtcttctgttccacacatttgataaaatcaccttgcctggaatgccccactggctgcttccgaaattcactgcgtttctccaggcgggactcaaaagcagctgggtctgacctgcgcagcagctggatcttgtcgcggtagcggtcgtagaaagggttggcctggagctcggcctcggccccgaccccgctgctgtcggcgcccccctcgggccggcccgagccggggcgcactgggaagacgcgcagctgcgcgggtgacacgagccccaggcccagggcgcggctgcgcaccgcgcacaggccccggtagagaccggccacctgcaggaccgccggtcccgcgccacccgcagccgccaccaccacagcagccatggccgcccccgcctcctcctcctcctcaggcgcgtcggcctcggcccgcggcccgcgcgcccgctccatcccgctccgagtgcgccgcgcccgcgctccggcaccgaggttccgcgcgccc

SEQ ID NO: 17846 - RNA, 1420 nt, Homo sapiens
  source 1..1420: mol_type = other RNA
tcgaggagctcacagtctagtgggggaaacagataggttgacattgattttaaaattataaaaattattaaacaactttataaacttcacttgcaatcaaacaaactttgggtgttatgaatggatggtaaaaagggatgatgtccaatgcagtgaaaaaccatctgcttcgatatcatgtgacttctgcgaaggcagtgatgtggttctgaatgcttgaattctctccaaagtaccatggacaagtaattatttagctattctggaattcctgtacagatgttaccttttccaaaggactttctactcgaggaatgctgatcattggcatctgtgccagattatccatgtgtatatgctcattttctgcttgtctccctttgaaattattcaccacgcacacaaccagaaatactgctatagatattccaaccagaaagcctgctataacatctgaccaatgatttcgatattctgctactctgttgagtccagtaagaaatgccaaacacattaagcccaagcatagaactggcttagcaagtctggttcccttggctttgattgtgttggtgatgtacatggtcagatacatagctgcatagacactgagagctgcttctttggatggaaaggtttttcgggctctcatgatgagatctgggttgccagtacaggcctcttccccactgatgaattgtgtatactgctgacatccaagtgctgtataattgggcttacacagggcaaggaaatgtggggccagatttcctgtgactacttgtccagcatttacaaagatatctgtagcaaacagtccaaatgtataaattccaagaaatcggacagttcggcgcaccagcgggtttatatagcaacagtctccagttaaaatagttttttcctggttttcaaaatcccttgtggctagttgtaggcaaaagacagcagtttctccaactattatcacgagcacggggaccccggcggccagcgagtagaggagcacggggggcacggcgctgctgtcctccgggcccgggtagggtttgcggtaggcgctgtcgtggcagaagaagccctgcacgttcacggtgaacgtgtccgtatactcgaagtagtacgccagcatcaccgtccctgccatgatcaccatctggaaatagagcatgctgctggtgagcgccgcgggcagcaggggcatgcacgcctcccgggccgggccgagccgagccgagcgggcggtcgacgcggtgggccccctccccggtccgccgaggcagccaccgggggcgcggcggcggaggcggcgggaggacgaggcacgggaggcgggatggagccgctggaggaagaggcggaggcaggtccgggcttcgaggcgccggcaggctgcagaggaggcggctacccccggacg

SEQ ID NO: 17847 - RNA, 1331 nt, Homo sapiens
  source 1..1331: mol_type = other RNA
tcgaggagctcacagtctagtgggggaaacagataggttgacattgattttaaaattataaaaattattaaacaactttataaacttcacttgcaatcaaacaaactttgggtgttatgaatggatggtaaaaagggatgatgtccaatgcagtgaaaaaccatctgcttcgatatcatgtgacttctgcgaaggcagtgatgtggttctgtacagatgttaccttttccaaaggactttctactcgaggaatgctgatcattggcatctgtgccagattatccatgtgtatatgctcattttctgcttgtctccctttgaaattattcaccacgcacacaaccagaaatactgctatagatattccaaccagaaagcctgctataacatctgaccaatgatttcgatattctgctactctgttgagtccagtaagaaatgccaaacacattaagcccaagcatagaactggcttagcaagtctggttcccttggctttgattgtgttggtgatgtacatggtcagatacatagctgcatagacactgagagctgcttctttggatggaaaggtttttcgggctctcatgatgagatctgggttgccagtacaggcctcttccccactgatgaattgtgtatactgctgacatccaagtgctgtataattgggcttacacagggcaaggaaatgtggggccagatttcctgtgactacttgtccagcatttacaaagatatctgtagcaaacagtccaaatgtataaattccaagaaatcggacagttcggcgcaccagcgggtttatatagcaacagtctccagttaaaatagttttttcctggttttcaaaatcccttgtggctagttgtaggcaaaagacagcagtttctccaactattatcacgagcacggggaccccggcggccagcgagtagaggagcacggggggcacggcgctgctgtcctccgggcccgggtagggtttgcggtaggcgctgtcgtggcagaagaagccctgcacgttcacggtgaacgtgtccgtatactcgaagtagtacgccagcatcaccgtccctgccatgatcaccatctggaaatagagcatgctgctggtgagcgccgcgggcagcaggggcatgcacgcctcccgggccgggccgagccgagccgagcgggcggtcgacgcggtgggccccctccccggtccgccgaggcagccaccgggggcgcggcggcggaggcggcgggaggacgaggcacgggaggcgggatggagccgctggaggaagaggcggaggcaggtccgggcttcgaggcgccggcaggct

SEQ ID NO: 17848 - RNA, 2118 nt, Homo sapiens
  source 1..2118: mol_type = other RNA
tcgaggagctcacagtctagtgggggaaacagataggttgacattgattttaaaattataaaaattattaaacaactttataaacttcacttgcaatcaaacaaactttgggtgttatgaatggatggtaaaaagggatgatgtccaatgcagtgaaaaaccatctgcttcgatatcatgtgacttctgcgaaggcagtgatgtggttctgtacagatgttaccttttccaaaggactttctactcgaggaatgctgatcattggcatctgtgccagattatccatgtgtatatgctcattttctgcttgtctccctttgaaattattcaccacgcacacaaccagaaatactgctatagatattccaaccagaaagcctgctataacatctgaccaatgatttcgatattctgctactctgttgagtccagtaagaaatgccaaacacattaagcccaagcatagaactggcttagcaagtctggttcccttggctttgattgtgttggtgatgtacatggtcagatacatagctgcatagacactgagagctgcttctttggatggaaaggtttttcgggctctcatgatgagatctgggttgccagtacaggcctcttccccactgatgaattgtgtatactgctgacatccaagtgctgtataattgggcttacacagggcaaggaaatgtggggccagatttcctgtgactacttgtccagcatttacaaagatatctgtagcaaacagtccaaatgtataaattccaagaaatcggacagttcggcgcaccagcgggtttatatagcaacagtctccagttaaaatagttttttcctggttttcaaaatcccttgtggctagttgtaggcaaaagacagcagtttctccaactattatcacgagcacggggaccccggcggccagcgagtagaggagcacggggggcacggcgctgctgtcctccgggcccgggtagggtttgcggtaggcgctgtcgtggcagaagaagccctgcacgttcacggtgaacgtgtccgtatactcgaagtagtacgccagcatcaccgtccctgccatgatcaccatctgtacccctcacagggcggacgctgtggggctggagaagctcctggcgggggtaaaatcaaaagggggggaggggaggcagtagagatggagcttccagaaactcttccgaggcaccagctgagaggtttaagaaacccgcacaacgcctgggaaaatggtgcgtggacgcgtcttccgagcgcaaagcccaccaaggcgcaaagtgccgatgcggcgcccagagtttcaaccggtgcgttcagcctgcatccctcgaattccttgacccagcccggggctggagcctggcggtggtttctaggcgctgttagaaaaatctcagcgaggtttctttgcctcctctgcagcttcctagggctttgtgtatatatatatgtatatacaaataataatagaaatcatagcccagtagctcccgaagcatcatctcttgtacagcggccccttcctggatccatgcattctcttgctcatcttttcagtctgtctttattagctgcttgtgagaggaggcattgcagattccaggcactgagcggtcccagccaccagggtaggaaaaaggactatttgcctcatctcgttctttattccctgaattccagggaactgcagggattcctcaggggtcgggataaaggagagggagaccaatgctggctcacagcacatgcatacaaaaattcatccgtccatggctatccacgcctatgcgtgggtatgtaactaactatggaactgcatatgtgcaaggagcccgttctgtcatgccatgtgggtccctgctgcaagcttagtcagcagactctcaaggggtctttctttgagcctcaggctgacactcctctactccagtgagcaggtgaggaagcatgaatacaagcaagaggaggaaaatatttttagagccctgccctgctcattaaaacctggaatcaccttagcagggttctagaatgttggttcattgtaataggctgtagcttgatgaattttagaggtgggcctttatcatcaggaaa

SEQ ID NO: 17849 - RNA, 1316 nt, Homo sapiens
  source 1..1316: mol_type = other RNA
tcgaggagctcacagtctagtgggggaaacagataggttgacattgattttaaaattataaaaattattaaacaactttataaacttcacttgcaatcaaacaaactttgggtgttatgaatggatggtaaaaagggatgatgtccaatgcagtgaaaaaccatctgcttcgatatcatgtgacttctgcgaaggcagtgatgtggttcttttccaaaggactttctactcgaggaatgctgatcattggcatctgtgccagattatccatgtgtatatgctcattttctgcttgtctccctttgaaattattcaccacgcacacaaccagaaatactgctatagatattccaaccagaaagcctgctataacatctgaccaatgatttcgatattctgctactctgttgagtccagtaagaaatgccaaacacattaagcccaagcatagaactggcttagcaagtctggttcccttggctttgattgtgttggtgatgtacatggtcagatacatagctgcatagacactgagagctgcttctttggatggaaaggtttttcgggctctcatgatgagatctgggttgccagtacaggcctcttccccactgatgaattgtgtatactgctgacatccaagtgctgtataattgggcttacacagggcaaggaaatgtggggccagatttcctgtgactacttgtccagcatttacaaagatatctgtagcaaacagtccaaatgtataaattccaagaaatcggacagttcggcgcaccagcgggtttatatagcaacagtctccagttaaaatagttttttcctggttttcaaaatcccttgtggctagttgtaggcaaaagacagcagtttctccaactattatcacgagcacggggaccccggcggccagcgagtagaggagcacggggggcacggcgctgctgtcctccgggcccgggtagggtttgcggtaggcgctgtcgtggcagaagaagccctgcacgttcacggtgaacgtgtccgtatactcgaagtagtacgccagcatcaccgtccctgccatgatcaccatctggaaatagagcatgctgctggtgagcgccgcgggcagcaggggcatgcacgcctcccgggccgggccgagccgagccgagcgggcggtcgacgcggtgggccccctccccggtccgccgaggcagccaccgggggcgcggcggcggaggcggcgggaggacgaggcacgggaggcgggatggagccgctggaggaagaggcggaggcaggtccgggcttcgaggcgccggcaggct

SEQ ID NO: 17850 - RNA, 5026 nt, Homo sapiens
  source 1..5026: mol_type = other RNA
tcgaggagctcacagtctagttggggcaatggactctgcacagatgggacagttaaggaacaatacccgacagacgcgatggaagtgtatgctgagaacctggagcgactcatttcagacagaggccttgactgggtcaggaaggcagccgtgctgattgggcatcagaaggccccgctgcatcctggcccggccacccaccagctgttggtgataatgatcacacaggcctggcagggggagatgggcagcctttgcctcggttccccgcctgcctcctggcactgcagtgctgcccgagttccaggcctcttctctgcagctgtccccaccaaatgctccagaaggagccctgtgatgctcctcaccaaaggtgcttgcattcaatagggtcatctgtaagctctccgtcatccataggggatgaaaggtggaatttcaggccatcgcaggcagcttgagactacagaacagggctggacagagtctattcagccagcaccctacaagcgaacacatcactcaggaaggtggacacacacgctgacgtacacggacattcatagaaacgaatgggtctcaatccagtctcacaggcagatatgtgagattgcacacacagacctgtgtttgcacacactcctgcccaacaatgtacccacggtggtacctagacacagacgggcacaaacacatacacacatatgcacgcatgcctaaagagtcattctagaaggggctgggccttctctctcccatggatggctaggtgggggctcaggtgatgtcaaggaggaaagatctagatcccatcatgtcaatctcaggtgcctaacccaggacccaaggacagggatccctttcacagctcccagagagtgaggggactggcacctgctccctccaccaatcccagctctataagcccctcctccttcactgcccctgggtggagaagggaactttcaactagacagtgctttttggcattttgccctgtacacaccctcctatccagggcaccctttcatgccaagtagataagaaatgaaggcccctctccacttccaaattcattgtctgatatgggggcaccaaatcacagaagcgggacgtctcttctgcctttctccaagtcaagcctcaccccagaaaatgggctggccaccgctcccccagctcctctgagacccagctgggggctgaggctaggagagaaccgtgttctcaggagtcccactgcttgtagggtggagtggggaagttatcagtcttcagactgcccaggcccaagaccctgtgctgggtcccttcaaagggtgcacactgaggagggaaatatggtgtcccagaaataggtcaaggaatctggggtgacctatggtctccaccatccagtgctcactctggacagaatcgtgtgcagcaggtgccctaccttccttgtctcctggacgtgggacagtcacagagctcgcaaagtcccacctgttcgtcctctgatccctgcctctcccatctcaggagtcccagagtctgaccaagggaggggctccatgtctgccccacttctggctcccttctggcaaagccaccaggctggagttcggccttgacttaggggacagggtaaagtcagaagcacaccacgagtgcagcaaggacaaggcctatgttgcgccgaggtccctgggttggcggatgccattcaggcaagtcccctgtctttgcagtaaagaaggtgctggcaggtcagatagaaacttgtgctttaatatatctctgtgtgtgtgagcatgagtgtgtgcgtgtgtgcaagtggaacagctgtctccagggcctcagtgcctggcctctgtccttgttctctgctcatccttgcagccaatgcaggccccctccctggcgggccggccctgcccctgggcaccccagctggcgggggtcagtctttggtacaatgtggacactttggtgtgccgggggcaaggttgggggggtggccacacagctctcatcatctctgcaacgccaagaggaagatggccatgggcccccacagctgtgggctggactggcagggggctccactgcccggcatcaccaccactccttcccgtcttgcacctttattgggatccgtctgcttccggggacactcccccttcttcagtgtgacgtcatctatggcaatatcccccaggtagcccgggcctcgaaccccctcaaaaataatctggaagggcccactggggctgatgggcacatgggcctgctgccacacattgcccttattgccactgagagaccaggcgtgcgtgtccagagcccctttgttccgggaccgcaccaggaggttgagggagccgatgtgtttcccgtacatgtggtagaagaaggagacacagtagaacttggcgctggcattgtagaggggactcactaaccttgcacggtcccccagctcccgaggcctcgatgtctcgatgaacatgtagtagccctcaggggtgccacttatgtcggtggggggaccagtgttgggggagcgtttggggttctgggtgagggcattctgccgcgtccagtcaaagttgtctgtcaggtcctgggtatagccacagatcttctcatcctcaaagtggcaggtgttgtctgaaaggttcggagagttgatgggctctgtgtagtggatgatgcgggaggccatgtcaccagccccgaaggtggtatagggtgtgaggcggacctcatagctgtggggcacacggagatcggtcaggatgtactccagcagctgccccttctccacacgccggaccgggatggccttgaccaccgcattgtgctggttcaactggcggatgctgagtctgtagttgagcacagggtcgacagcgtcgggctccctctgagtccactgcagcacgtaggagtagttcttggacagcttgtggctgcgggtggggttgggggtgtcgaagtaaaactccgggctgtaggctttggcggagacctggaagaggcaggcagccgagcccacatcgttggagacgctgcactcgtagctgccgctgctgtcgcgagttacggcgtcgaggcgcagctccgcgtgatccggcgcctcggcggcggcgggaacaacaggcggcggcggcagcagctgccctttgaaacgccacacagccgaggcgatgcgctgggggctgcctcgcagcagcgagcagcgcaggagcacgggccggcccagcgcctggcgcacgtcctgggaactgggctccacctccggcgggaactgcacgttcagctgcacctgggcctcacgggggcgcacgttgaagccattatagcgggccgtctggcagcggtaggtcccgctcatgtctcggctcactcgctccagccgcagcttcccgtccggagtctcctccaggggcagccccgagggcagcagtgcagcctccttgtccacgcgggaccagagcactggcggccgcggcttgccccgcacctcgcattgcagctcggcaggcgatccctcgcgcacggtcaccacggccctacccttgggcacactgatggtgggcggcactgtctcagaggagatgttgacctcgacgctgaggtcgggcacgggtgcccctgggaaagaagccatgcacaggtaggtgccatagtcactgaagtgcaggtcaatgagctctaggctgctggtgactgcgggcagctcaggatcattgcgggtcaccagcagccgcttggacatgcgtgccggcttgccattcttgaaccactggtaggtcaccttctcctggggcactgcatccacgtggcacgatagcttcaggtcctggcccagctggatgttctcactctctttgatcacgtcaggagtgatctggaatgtagcgttcttcatggatcgcaccagcaggttgacagtcttcttggcagggttgcccacattgttggtggctgtgcagttgtagtagccagagtcccgggcctgcactgaagggatgctgagggtgccaccctgggccagagcacccaggggcagtgggccaggcccatgggaccactgcagctgggggaggggatcaccgcctgtcagcagacactgcaccgtcacattctccccagggttcaccaccagagtttcgttcacagacagcttcagggctggtggtgccgtggtgttggtgagccggaaggtgatggccttgtctgggatgccgcacacgttacgcacagacacctggcaggtgtagctggcatagtcctggggccgcaggttcttcagcttcaggaccttggtctccccctgagtgtagaggggctcatagatgtcaaccccattgtcctggctgtgggatagggtatcggaaccccgcttccagatgaagcgggcaggcgggttggagttgacagtacagcgcaggaacaccgtcttctcctggtagaagttgcctcgcacatcgctcaccgtctggtgcaccgtcagcattggctcatccaggtactgcacgtccacgcggatggacttgatggccggcacccccacgccgttctcagccttgcagtagtagcggccgccctgcgtgcgtgcaatacgctcgatgcgcagcgtctcgttgaacaccgatgtctcctggaacttgtccgaggcgctacctgccgtcttggtccaccgtacctggggtcgagggtgccctgttacaaggcactgcagcatgagggtgtccccctcccggatggtgtagacacgctcgctgatattgtcctctttcaccacacatgcctggcccgcatgcacgatctgcgcctgggctggagcgtagactccttgtccccggcagtggaaggggatcagcgccagaagtagaaggcaggtcacctccatcttcacggccggtgcttcatccccgcgaggcggcgcagcccgagaggcggcggggggcgcattcgccggggccccgcgacgcccctatgtccccccctttccctgagaggtgagagagagagc

SEQ ID NO: 17851 - RNA, 5957 nt, Homo sapiens
  source 1..5957: mol_type = other RNA
tcgaggagctcacagtctagttggggcaatggactctgcacagatgggacagttaaggaacaatacccgacagacgcgatggaagtgtatgctgagaacctggagcgactcatttcagacagaggccttgactgggtcaggaaggcagccgtgctgattgggcatcagaaggccccgctgcatcctggcccggccacccaccagctgttggtgataatgatcacacaggcctggcagggggagatgggcagcctttgcctcggttccccgcctgcctcctggcactgcagtgctgcccgagttccaggcctcttctctgcagctgtccccaccaaatgctccagaaggagccctgtgatgctcctcaccaaaggtgcttgcattcaatagggtcatctgtaagctctccgtcatccataggggatgaaaggtggaatttcaggccatcgcaggcagcttgagactacagaacagggctggacagagtctattcagccagcaccctacaagcgaacacatcactcaggaaggtggacacacacgctgacgtacacggacattcatagaaacgaatgggtctcaatccagtctcacaggcagatatgtgagattgcacacacagacctgtgtttgcacacactcctgcccaacaatgtacccacggtggtacctagacacagacgggcacaaacacatacacacatatgcacgcatgcctaaagagtcattctagaaggggctgggccttctctctcccatggatggctaggtgggggctcaggtgatgtcaaggaggaaagatctagatcccatcatgtcaatctcaggtgcctaacccaggacccaaggacagggatccctttcacagctcccagagagtgaggggactggcacctgctccctccaccaatcccagctctataagcccctcctccttcactgcccctgggtggagaagggaactttcaactagacagtgctttttggcattttgccctgtacacaccctcctatccagggcaccctttcatgccaagtagataagaaatgaaggcccctctccacttccaaattcattgtctgatatgggggcaccaaatcacagaagcgggacgtctcttctgcctttctccaagtcaagcctcaccccagaaaatgggctggccaccgctcccccagctcctctgagacccagctgggggctgaggctaggagagaaccgtgttctcaggagtcccactgcttgtagggtggagtggggaagttatcagtcttcagactgcccaggcccaagaccctgtgctgggtcccttcaaagggtgcacactgaggagggaaatatggtgtcccagaaataggtcaaggaatctggggtgacctatggtctccaccatccagtgctcactctggacagaatcgtgtgcagcaggtgccctaccttccttgtctcctggacgtgggacagtcacagagctcgcaaagtcccacctgttcgtcctctgatccctgcctctcccatctcaggagtcccagagtctgaccaagggaggggctccatgtctgccccacttctggctcccttctggcaaagccaccaggctggagttcggccttgacttaggggacagggtaaagtcagaagcacaccacgagtgcagcaaggacaaggcctatgttgcgccgaggtccctgggttggcggatgccattcaggcaagtcccctgtctttgcagtaaagaaggtgctggcaggtcagatagaaacttgtgctttaatatatctctgtgtgtgtgagcatgagtgtgtgcgtgtgtgcaagtggaacagctgtctccagggcctcagtgcctggcctctgtccttgttctctgctcatccttgcagccaatgcaggccccctccctggcgggccggccctgcccctgggcaccccagctggcgggggtcagtctttggtacaatgtggacactttggtgtgccgggggcaaggttgggggggtggccacacagctctcatcatctctgcaacgccaagaggaagatggccatgggcccccacagctgtgggctggactggcagggggctccactgcccggcatcaccaccactttattgggatccgtctgcttccggggacactcccccttcttcagtgtgacgtcatctatggcaatatcccccaggtagcccgggcctcgaaccccctcaaaaataatctggaagggcccactggggctgatgggcacatgggcctgctgccacacattgcccttattgccactgagagaccaggcgtgcgtgtccagagcccctttgttccgggaccgcaccaggaggttgagggagccgatgtgtttcccgtacatgtggtagaagaaggagacacagtagaacttggcgctggcattgtagaggggactcactaaccttgcacggtcccccagctcccgaggcctcgatgtctcgatgaacatgtagtagccctcaggggtgccacttatgtcggtggggggaccagtgttgggggagcgtttggggttctgggtgagggcattctgccgcgtccagtcaaagttgtctgtcaggtcctgggtatagccacagatcttctcatcctcaaagtggcaggtgttgtctgaaaggttcggagagttgatgggctctgtgtagtggatgatgcgggaggccatgtcaccagccccgaaggtggtatagggtgtgaggcggacctcatagctgtggggcacacggagatcggtcaggatgtactccagcagctgccccttctccacacgccggaccgggatggccttgaccaccgcattgtgctggttcaactggcggatgctgagtctgtagttgagcacagggtcgacagcgtcgggctccctctgagtccactgcagcacgtaggagtagttcttggacagcttgtggctgcgggtggggttgggggtgtcgaagtaaaactccgggctgtaggctttggcggagacctggaagaggcaggcagccgagcccacatcgttggagacgctgcactcgtagctgccgctgctgtcgcgagttacggcgtcgaggcgcagctccgcgtgatccggcgcctcggcggcggcgggaacaacaggcggcggcggcagcagctgccctttgaaacgccacacagccgaggcgatgcgctgggggctgcctcgcagcagcgagcagcgcaggagcacgggccggcccagcgcctggcgcacgtcctgggaactgggctccacctccggcgggaactgcacgttcagctgcacctgggcctcacgggggcgcacgttgaagccattatagcgggccgtctggcagcggtaggtcccgctcatgtctcggctcactcgctccagccgcagcttcccgtccggagtctcctccaggggcagccccgagggcagcagtgcagcctccttgtccacgcgggaccagagcactggcggccgcggcttgccccgcacctcgcattgcagctcggcaggcgatccctcgcgcacggtcaccacggccctacccttgggcacactgatggtgggcggcactgtctcagaggagatgttgacctcgacgctgaggtcgggcacgggtgcccctgggaaagaagccatgcacaggtaggtgccatagtcactgaagtgcaggtcaatgagctctaggctgctggtgactgcgggcagctcaggatcattgcgggtcaccagcagccgcttggacatgcgtgccggcttgccattcttgaaccactggtaggtcaccttctcctggggcactgcatccacgtggcacgatagcttcaggtcctggcccagctggatgttctcactctctttgatcacgtcaggagtgatctggaatgtagcgttcttcatggatcgcaccagcaggttgacagtcttcttggcagggttgcccacattgttggtggctgtgcagttgtagtagccagagtcccgggcctgcactgaagggatgctgagggtgccaccctgggccagagcacccaggggcagtgggccaggcccatgggaccactgcagctgggggaggggatcaccgcctgtcagcagacactgcaccgtcacattctccccagggttcaccaccagagtttcgttcacagacagcttcagggctggtggtgccgtggtgttggtgagccggaaggtgatggccttgtctgggatgccgcacacgttacgcacagacacctggcaggtgtagctggcatagtcctggggccgcaggttcttcagcttcaggaccttggtctccccctgagtgtagaggggctcatagatgtcaaccccattgtcctggctgtgggatagggtatcggaaccccgcttccagatgaagcgggcaggcgggttggagttgacagtacagcgcaggaacaccgtcttctcctggtagaagttgcctcgcacatcgctcaccgtctggtgcaccgtcagcattggctcatccaggtactgcacgtccacgcggatggacttgatggccggcacccccacgccgttctcagccttgcagtagtagcggccgccctgcgtgcgtgcaatacgctcgatgcgcagcgtctcgttgaacaccgatgtctcctggaacttgtccgaggcgctacctgccgtcttggtccaccgtacctggggtcgagggtgccctgttacaaggcactgcagcatgagggtgtccccctcccggatggtgtagacacgctcgctgatattgtcctctttcaccacacatgcctggcccgcatgcacgatctgcgcctgggctggagcgtagactccttgtccccggcagtggaaggggatcagcgccagaagtagaaggcaggtcacctccatcttcacggccggtgcttcatccccgcgaggcggcgcagcccgagaggcggcggggggcgcattcgccggggccccgcgacgcccctatgtccccccctttccctgagaggtgagagagagagcggcgacgaagaccaggagactgaagaggcggaggtggcggcgacccgtgtttctcctccggcggggccgctgcccgcgtggggacgcagggggcgctggcccagccccgggtgcctcggcgcgcccggcacagcagccagcgccccgacccgaggagcccggccgccgagccgccccgggtacccagggccgtccgcgcgggatgctaggcgccggggacctctcggcggcggaggcggcgcttcgatccaacaggccacggacgactgacaaacttgtcgtttccccgcactggggccgcccctcagcggagcggagtcggggaggccggggctccgctcgagttaatcaatctgctgtttccagtcctgcggccgctgccgtgggctcagcggcccgactccagggggccgggctgaaagcactcgcggcggcgaagcagccccgggcccggccctcctgatccggggagcagcgcgggctgggttcggccgagggacgagcgccgcgggtccccgggtccgtgaagttagccgagccgccgataaacccgggggaagaatagcagcccggcgccccgcgggaatctggagagcaattccaggcaagaagggccccagaaaacggggaaaggaggaaagtttgagtcttttgaaaaatattcgcgctctcgcccaggccggggctgcggcgcgggcgccgctcgccgcctccgctcgccgcgctcctctcccgccgtctggccgcggccgtagccctcccgggctccgagctctcgggagagcggggctacgccgcgccccaagttggtcgtccccgcccccgcccggcggccttggcctgcgggggcccagagcgggcggggccgggccgggctccggggcgcggcggccgctcggctccgggccgcgggagcgctccgctcgctcagcaacttgggctttgctgt

SEQ ID NO: 17852 - RNA, 79 nt, Homo sapiens
  source 1..79: mol_type = other RNA
tcgaggagctcacagtctagttgtgttcatgtgcaagtcatttacccccagctagattgtaagctccttgagggcagtt

SEQ ID NO: 17853 - RNA, 3690 nt, Homo sapiens
  source 1..3690: mol_type = other RNA
tcgaggagctcacagtctccagatgttagtagccaaggatatggttttctatttagaagaggactccaaattaaccttataatagtaactttccatttaaaaagaaacaagagtaataaaactgtcaatgcttttttataaatgaaaactgactaatcagtgttatccggtaacagtcacatttctgtgtcccgtcaatgctgtgtggaccttcagacggcagctctgagcacgcaagtgaaaagcgcgtatttcagggcaagaatagagatgtgggtctgttttccgaggatgagccagctatccttcctcagccacaggagtggtgagcgtgagcaccctgggctgggtggtgaggactgcgtactgtggggcggcccttcccaactcttggctgtgcccagcagcacctctggggcacaagggcaggccctctttagagagaaccagggaatccaacctgagatgtcggggcttctttgttagggtttgacagaatatttgagacctaagattgtgaataaaggaacatgacagcatcgattctctgccgagcagaggtaaaaaggaccctacagaagtacctttctaactcatcttatgtaaatccaagtgctgggccagtgcctgggcggcaaagtgaggcctgtgagcatttctgtgttcagcacaacctgaacctgactgtccattcagacacgctgatccagaggaaagcaacactgaatcttaacatgaatgtgaagatagaagatgtacatttattttcatgaattacaaatgcatttctgttcatattagcaggcagtctttatataacccattctccattgctgtcaaaaatcaaacaagaaaaaaggacagctgagaaatgaaaagctaaaaatagaattatttttcctaaatgatctgctggatagcattttccgtggaacacaactcagaggtaacaatagagttttcatttcaatcgtaggcatgtggcacttggacagtcatctctgcacagaaagctgtaacagtcatgcgagggtacagtaattattgaacaaggcaaatttctcaccacagagagcagtggggaagtcaagaggaggcaccgcactgggacagaacaccgagtcaactccacagtacacagtggcaggaacaaatacttaaagagatcagtaaaatatggatagagctccaaacacgagttagtgctagctttttctgacagtctgactcagcagtatcagaaatatttgagtacttgaggacagaacagtgcttcacgtcatgagctcctggaggctttattacaaattgttatactgtaggttgaaaaatgaacttgagatgctgacatgctgtagaaggaaaaagaattgtatactttctcatttaaagacgcagtgttcctctctgctaaatcctcaggcatggaacgtggttactgaaacacccacatttgaagtagctcaagggcgtatatgcaccagcatgtggagttccaccctgggacatccccagaaaccgcccacagctcagcactgcaacctttgtacttctctcaccaaatgtcgagtgaagctgccactttaaatctttttttgtaagtcttacaaacattaagtactgcacataacgcttcttgacaagtgttacacctctatatggtacaagtgaccacagtaactacagagtgacactgctgggtgcagtacttcctttttatttagaaaaatgactgcattttctaaaagctgggccaatagcacataccttatatatgttagtgactaccatgatatgagaaaagacgtggacaagtgctccccaaggattccggagacggaagcacttgctgcaggctgcaacatcagccaaggtatttccacaagctcctgctctggggaaacagttatggtcaaaaggtgaagtgcaaataaggggctgtcactgacttaaagtgccctaggtagtagccttccctatcataaagtgagatgccagtgactagagccaattggggaagaatctctctctggtgcggctgcatggtcagcagggcatcatgtagaaaaggattcaggagagggaggaaccactgcatctttcaaaccagaaagcaattagtgactaaagcaacagtaagcagtaggtgcactgaagtacatactgccgcaggtcaccaatgggtgacacacacagggctgccaggaggaattctctggactgaagaaattctttgaaagcataaaagccacaactaccagaaaccgcccctccaaacggctcaaaggagtcaaagtggataagccaagacgggctggagacaggaccaggggtcaagaactgggaagaagaacaccgatgtctgagcacgtccagtcctctgagcccttgtcctgacaaatttaagatctgtatcctggctggaatctagcagtctcttcaaaaattagttctttgagcttttccttaggcaagtcatccaattccatgtcgaacttgaatggtgcttcggcgatgggctcgtcactcgggtcgtaatactgctccagatatgggtgggccagagcctgttctacttcaatcctcttgtgtgggttgaatgtcaacattttgtccaataagtccagagctttggagtcagcatttgggaacagcctgttccatggcaccttatttttgtgtggaagagaaagcaaatagttcctagcttttaaatttattatacaattcaggtcttcttgtgatggggatccaagaatacccaaaatgtggttcagctggtcaagataatgcttccctggaaagatgggcctgttagaaagcatttctgccagaatgcagcctacagaccaaatatcaatggacttggtgtagcccttggaattcaacataatttctggagccctgtaccaacgtgtggccacatattctgtcaggaaccctgtgtgatcatggtctggatctgcaacacgggccaggccaaagtcacagatcttgagatcacaggtggtgttgagcagcaggttggaaggcttgaggtcacggtgcagaacgttagctgaatggatatattttaaccctctgaggatctggtagagaaaatagcagatatggtcattgctgaggtgttgtgtcttcaagagcttgtaaagatctgtttccatgaggtcctgtactatatatacatctttcatttgctcgatggttggtgctcgaataatgtcattgattccaatgatgttctcatgtctgaagcgcagtaagatttttatctccctcagggttctctggcagtaggtctggtgctcaaaggggctgattttcttgatagctactcgaactttgttgacattatcataagcagagcacaccatgccgtaggcgccctcgccgatgtacgagaggttggtgtagcgcggccccacgtcgaacacctgcccgcggaccatctccgggcccgcgcccgccgccgccgccgccgccatgttggctgccgggccgccgccgcctccgccgcgctgagctcgacgctcggcggccgccgctcagctcttgtcgcccctcccgcagggactgcgccgccgccggtgcagccgccgacgctgaccgggaggaggaaggaagacgccgagcgggagagctgaagagccgacagccactcggaccgattgcctgcctgcctgccagact

SEQ ID NO: 17854 - RNA, 3462 nt, Homo sapiens
  source 1..3462: mol_type = other RNA
tcgaggagctcacagtctggggggacagacatgtaaacacatgagttacaacgcgctgcgtgaagtgtgtggcagaggtataacaaagtgctgtggggcacaacagagcgaccagtgaactcttcctgggcaggggtcagggaagccttcacagatcagtcaataaatacggtgccatgggagtgccttgcacaccacgggcactcacatcttgaatgctggtccactggaggcccttgggttgggcgggagcaaggcctacttctgcttcctcaggacaacttccccacctctgtcctgggaccacctgcccgcctgggcctgcagtgactaaggacgctgctcccactccaggggccagtgacagagagcagctatacagagggcccaccccgcaggatccttgacaggagctgagacagaacaaactgctgcttgtctccctaccctgggggctgtgatattcttggtaacatctctgagctggtctgtgaggtcacttcctcttttaacactgttgaggagactccaaaccctgtcttttcctcgtcttctcatgtcgattgggcaccagccattctcaggcaccagagcacagccccacacgggtgccccatcagacagggctgcccacagcagcctcctacacctgaactgggtttctctgcacactcacagccgtctcaccagctcaatgagctgctggatgtttttgttttggttcgacaagccgttcctgatgttttcgagtaggcatctcttcaattcaaatatggcttcactgtaggccaagctcactgcggccatgggaggtgctccgtgccacaggcctgggatgtgccagatgtgctgcttctcagggtcgcagaaggccaggcctgccagtgcccggaagccgtcgccctgtttctccatctgggctgcagccctgctcaggtcaccaggtggatccaggagctgtctcttgtctctgggcctagggccgggaacagatacatcatgaaggttctggtatacaaactggtagttgggcatgtgccccgttttttctaacctcagaaatgcatgcagaatagctgctggaatgtccttggtttcagctagactgatcacggtgacattgctcagtcccatgagcagagtggccaaggaagcctccagctcaaatctgtccccagctgacgtcaaggccccacctatcaagcccccggagtctatcaccaggatgtggtcacagcccaggtcctggctgaagccctcagccactgtgatgagctgcatgaaggcccctcgaggaccgcagctcttccctgtggcaaaccgcagcccaaacatggtgttgaggagtgtggacttgcccgtgcctggcaccccgacggttgacagaaccaccagccttgaccgtctctccagtcggacgtgcagctccttcaggagccctgtgacccagcggacgggcatgctcagcgtgctcccatcgattagctccagaggcagccctgtcagcagcagctccgaggccaagcctgggaagtgggcaaaacgcctctggcctgccggcagcctccctgcctccacaagacagctctcagcctcataaaactgtcccatctcccgcaagaagtgttccacccctaggggctcaggccagagcggctcccccacgtctgtggtgcccccatgctttggtctcagggtgagaagcgtctccggaggctgtctcagtcgcggctgggccacccgtgccaggccccactccatccacctcaggaagtactgcttctcactcaaggaggggctgctgatccccgagatgaactcctgcacccccgaggagggatcatggccgttctgctgcattcgaagttctagcagccgccgcctcagctcagccctgtgcttctcaggggggtccacggcccactggagctggcagaactccttctccacttgggctgcctttctccaggggtccccctgcagcctcagctcgtcccttctgtaggcatccgagtctttgattttcctggtaatcctctccatccggtctttcgctttctgacactcctcacagtcctcgtcgacctttaggcccagtttgcgggctgcgtgcgccatgtcctccacagatacccgcctgcagggtgcccgcagcacattcccaacgatggcccggatcctcttcacgaagctgtcgctgtcagtgctgctgacctttaccaggacatgtgagtggtctattttcagcacaggaattaacttattcagaaatctcaggtttgtgttgcgcttcccacggtagggactcaggatgaagtagtattttgtggttgactccttcatggagtacagcaatttgtattccttcttactgatattgtcagtcaatataaacacagcggaggagatttctgtcaagagcttaaactgcagccagtgagacccgatgtcacctctcaggttcagaaaggccacaggttctgggaaaatgtccaagtcctcccttccgctgggaaaaaaccaggaaatttctaccaacccatccgaaatctcccgggcattggtgcccaagttgaggtcccgatgccagaagcagtcccactgcctgtggcccgggctgaggacggcgttgagaagctgggacttggagttgctactgacgtccatgcgcacgaaggcgaaggcgggcgccctggacaagaccacgctgtcttcccggaagctccccatgccccttgggggctgggaccaccatgtcctcacaatgccccgcatggcccacagcagaaatgtatggtagtggttctccgagtcaggcaacacgagtgggagtgcaaactggcagagggccattttcaacgctatttcttgttgcaggaaactgtctgaggagagcagcagggcacagagaaggtctaaggggttcactggcgtatcaggggtgggcagctcagaaaaggaataaatgtcggcagcaaggtcatcagctgggtcccagtagatgatctcctcttccatctggctctccttctccacaggcctggcgtctgggagcacgtccagcaccatagtggtattcctggcatcagcattgagggcctgcaacttcctgaggaaattccagggcaagtctttgggaacctgaggggcccagttcttcatactgtcaaaactgatctgcagagagtcctggaggctgagtttctggacctggtacgtctctaggcccaaaagtgacagcatttcttgaagcctgcttctctccactgttggaaaatcattgtcctgagcctcatttgtaccatctccataacggaactcgcaatcatctccttccatttctctccattccaaatctgcaatggccacagctgttcgtctctctgatgcttttatttctggggctacttctcccaaatctgaatgcccgggcgacgccatgagcgcagcgaggtctccgct

SEQ ID NO: 17855 - RNA, 3484 nt, Homo sapiens
  source 1..3484: mol_type = other RNA
tcgaggagctcacagtctggggggacagacatgtaaacacatgagttacaacgcgctgcgtgaagtgtgtggcagaggtataacaaagtgctgtggggcacaacagagcgaccagtgaactcttcctgggcaggggtcagggaagccttcacagatcagtcaataaatacggtgccatgggagtgccttgcacaccacgggcactcacatcttgaatgctggtccactggaggcccttgggttgggcgggagcaaggcctacttctgcttcctcaggacaacttccccacctctgtcctgggaccacctgcccgcctgggcctgcagtgactaaggacgctgctcccactccaggggccagtgacagagagcagctatacagagggcccaccccgcaggatccttgacaggagctgagacagaacaaactgctgcttgtctccctaccctgggggctgtgatattcttggtaacatctctgagctggtctgtgaggtcacttcctcttttaacactgttgaggagactccaaaccctgtcttttcctcgtcttctcatgtcgattgggcaccagccattctcaggcaccagagcacagccccacacgggtgccccatcagacagggctgcccacagcagcctcctacacctgaactgggtttctctgcacactcacagccgtctcaccagctcaatgagctgctggatgtttttgttttggttcgacaagccgttcctgatgttttcgagtaggcatctcttcaattcaaatatggcttcactgtaggccaagctcactgcggccatgggaggtgctccgtgccacaggcctgggatgtgccagatgtgctgcttctcagggtcgcagaaggccaggcctgccagtgcccggaagccgtcgccctgtttctccatctgggctgcagccctgctcaggtcaccaggtggatccaggagctgtctcttgtctctgggcctagggccgggaacagatacatcatgaaggttctggtatacaaactggtagttgggcatgtgccccgttttttctaacctcagaaatgcatgcagaatagctgctggaatgtccttggtttcagctagactgatcacggtgacattgctcagtcccatgagcagagtggccaaggaagcctccagctcaaatctgtccccagctgacgtcaaggccccacctatcaagcccccggagtctatcaccaggatgtggtcacagcccaggtcctggctgaagccctcagccactgtgatgagctgcatgaaggcccctcgaggaccgcagctcttccctgtggcaaaccgcagcccaaacatggtgttgaggagtgtggacttgcccgtgcctggcaccccgacggttgacagaaccaccagccttgaccgtctctccagtcggacgtgcagctccttcaggagccctgtgacccagcggacgggcatgctcagcgtgctcccatcgattagctccagaggcagccctgtcagcagcagctccgaggccaagcctgggaagtgggcaaaacgcctctggcctgccggcagcctccctgcctccacaagacagctctcagcctcataaaactgtcccatctcccgcaagaagtgttccacccctaggggctcaggccagagcggctcccccacgtctgtggtgcccccatgctttggtctcagggtgagaagcgtctccggaggctgtctcagtcgcggctgggccacccgtgccaggccccactccatccacctcaggaagtactgcttctcactcaaggaggggctgctgatccccgagatgaactcctgcacccccgaggagggatcatggccgttctgctgcattcgaagttctagcagccgccgcctcagctcagccctgtgcttctcaggggggtccacggcccactggagctggcagaactccttctccacttgggctgcctttctccaggggtccccctgcagcctcagctcgtcccttctgtaggcatccgagtctttgattttcctggtaatcctctccatccggtctttcgctttctgacactcctcacagtcctcgtcgacctttaggcccagtttgcgggctgcgtgcgccatgtcctccacagatacccgcctgcagggtgcccgcagcacattcccaacgatggcccggatcctcttcacgaagctgtcgctgtcagtgctgctgacctttaccaggacatgtgagtggtctattttcagcacaggaattaacttattcagaaatctcaggtttgtgttgcgcttcccacggtagggactcaggatgaagtagtattttgtggttgactccttcatggagtacagcaatttgtattccttcttactgatattgtcagtcaatataaacacagcggaggagatttctgtcaagagcttaaactgcagccagtgagacccgatgtcacctctcaggttcagaaaggccacaggttctgggaaaatgtccaagtcctcccttccgctgggaaaaaaccaggaaatttctaccaacccatccgaaatctcccgggcattggtgcccaagttgaggtcccgatgccagaagcagtcccactgcctgtggcccgggctgaggacggcgttgagaagctgggacttggagttgctactgacgtccatgcgcacgaaggcgaaggcgggcgccctggacaagaccacgctgtcttcccggaagctccccatgccccttgggggctgggaccaccatgtcctcacaatgccccgcatggcccacagcagaaatgtatggtagtggttctccgagtcaggcaacacgagtgggagtgcaaactggcagagggccattttcaacgctatttcttgttgcaggaaactgtctgaggagagcagcagggcacagagaaggtctaaggggttcactggcgtatcaggggtgggcagctcagaaaaggaataaatgtcggcagcaaggtcatcagctgggtcccagtagatgatctcctcttccatctggctctccttctccacaggcctggcgtctgggagcacgtccagcaccatagtggtattcctggcatcagcattgagggcctgcaacttcctgaggaaattccagggcaagtctttgggaacctgaggggcccagttcttcatactgtcaaaactgatctgcagagagtcctggaggctgagtttctggacctggtacgtctctaggcccaaaagtgacagcatttcttgaagcctgcttctctccactgttggaaaatcattgtcctgagcctcatttgtaccatctccataacggaactcgcaatcatctccttccatttctctccattccaaatctgcaatggccacagctgttcgtctctctgatgcttttatttctggggctacttctcccaaatctgaatgccctttgcccagtaattccacttccgggcgacgccatgagcgcagcgaggtctccgct

SEQ ID NO: 17856 - RNA, 4049 nt, Homo sapiens
  source 1..4049: mol_type = other RNA
tcgaggagctcacagtctggggggacagacatgtaaacacatgagttacaacgcgctgcgtgaagtgtgtggcagaggtataacaaagtgctgtggggcacaacagagcgaccagtgaactcttcctgggcaggggtcagggaagccttcacagatcagtcaataaatacggtgccatgggagtgccttgcacaccacgggcactcacatcttgaatgctggtccactggaggcccttgggttgggcgggagcaaggcctacttctgcttcctcaggacaacttccccacctctgtcctgggaccacctgcccgcctgggcctgcagtgactaaggacgctgctcccactccaggggccagtgacagagagcagctatacagagggcccaccccgcaggatccttgacaggagctgagacagaacaaactgctgcttgtctccctaccctgggggctgtgatattcttggtaacatctctgagctggtctgtgaggtcacttcctcttttaacactgttgaggagactccaaaccctgtcttttcctcgtcttctcatgtcgattgggcaccagccattctcaggcaccagagcacagccccacacgggtgccccatcagacagggctgcccacagcagcctcctacacctgaactgggtttctctgcacactcacagccgtctcaccagctcaatgagctgctggatgtttttgttttggttcgacaagccgttcctgatgttttcgagtaggcatctcttcaattcaaatatggcttcactgtaggccaagctcactgcggccatgggaggtgctccgtgccacaggcctgggatgtgccagatgtgctgcttctcagggtcgcagaaggccaggcctgccagtgcccggaagccgtcgccctgtttctccatctgggctgcagccctgctcaggtcaccaggtggatccaggagctgtctcttgtctctgggcctagggccgggaacagatacatcatgaaggttctggtatacaaactggtagttgggcatgtgccccgttttttctaacctcagaaatgcatgcagaatagctgctggaatgtccttggtttcagctagactgatcacggtgacattgctcagtcccatgagcagagtggccaaggaagcctccagctcaaatctgtccccagctgacgtcaaggccccacctatcaagcccccggagtctatcaccaggatgtggtcacagcccaggtcctggctgaagccctcagccactgtgatgagctgcatgaaggcccctcgaggaccgcagctcttccctgtggcaaaccgcagcccaaacatggtgttgaggagtgtggacttgcccgtgcctggcaccccgacggttgacagaaccaccagccttgaccgtctctccagtcggacgtgcagctccttcaggagccctgtgacccagcggacgggcatgctcagcgtgctcccatcgattagctccagaggcagccctgtcagcagcagctccgaggccaagcctgggaagtgggcaaaacgcctctggcctgccggcagcctccctgcctccacaagacagctctcagcctcataaaactgtcccatctcccgcaagaagtgttccacccctaggggctcaggccagagcggctcccccacgtctgtggtgcccccatgctttggtctcagggtgagaagcgtctccggaggctgtctcagtcgcggctgggccacccgtgccaggccccactccatccacctcaggaagtactgcttctcactcaaggaggggctgctgatccccgagatgaactcctgcacccccgaggagggatcatggccgttctgctgcattcgaagttctagcagccgccgcctcagctcagccctgtgcttctcaggggggtccacggcccactggagctggcagaactccttctccacttgggctgcctttctccaggggtccccctgcagcctcagctcgtcccttctgtaggcatccgagtctttgattttcctggtaatcctctccatccggtctttcgctttctgacactcctcacagtcctcgtcgacctttaggcccagtttgcgggctgcgtgcgccatgtcctccacagatacccgcctgcagggtgcccgcagcacattcccaacgatggcccggatcctcttcacgaagctgtcgctgtcagtgctgctgacctttaccaggacatgtgagtggtctattttcagcacaggaattaacttattcagaaatctcaggtttgtgttgcgcttcccacggtagggactcaggatgaagtagtattttgtggttgactccttcatggagtacagcaatttgtattccttcttactgatattgtcagtcaatataaacacagcggaggagatttctgtcaagagcttaaactgcagccagtgagacccgatgtcacctctcaggttcagaaaggccacaggttctgggaaaatgtccaagtcctcccttccgctgggaaaaaaccaggaaatttctaccaacccatccgaaatctcccgggcattggtgcccaagttgaggtcccgatgccagaagcagtcccactgcctgtggcccgggctgaggacggcgttgagaagctgggacttggagttgctactgacgtccatgcgcacgaaggcgaaggcgggcgccctggacaagaccacgctgtcttcccggaagctccccatgccccttgggggctgggaccaccatgtcctcacaatgccccgcatggcccacagcagaaatgtatggtagtggttctccgagtcaggcaacacgagtgggagtgcaaactggcagagggccattttcaacgctatttcttgttgcaggaaactgtctgaggagagcagcagggcacagagaaggtctaaggggttcactggcgtatcaggggtgggcagctcagaaaaggaataaatgtcggcagcaaggtcatcagctgggtcccagtagatgatctcctcttccatctggctctccttctccacaggcctggcgtctgggagcacgtccagcaccatagtggtattcctggcatcagcattgagggcctgcaacttcctgaggaaattccagggcaagtctttgggaacctgaggggcccagttcttcatactgtcaaaactgatctgcagagagtcctggaggctgagtttctggacctggtacgtctctaggcccaaaagtgacagcatttcttgaagcctgcttctctccactgttggaaaatcattgtcctgagcctcatttgtaccatctccataacggaactcgcaatcatctccttccatttctctccattccaaatctgcaatggccacagctgttcgtctctctgatgcttttatttctggggctacttctcccaaatctgaatgccctttgcccagtaattccacttctatcagagttaagaaccactattctcaggagttatatgacagcctgggaagacgcccaggatgtaggaacagggagcaggcgagcgtgtggcaccttgagggtgctccgcgcgtctccgtaaagccaacgagcccctcctcttcgctggcctctccggggccttgctgactagtggtcgaagccacaggaccaggtgcgggtggccagcgtaacccgggcagccccgctgcttcccctcggccgcgccaggacgctcggcacgcggcgacgacggccccacagtgccccgcgcgcgcaagcgcaggctgcggctcccggcgtgcagcttggtggcggctgagccggcagcgggccgcctcaggcagccccggccgggccgcccgggtccccggcagcggggtaggatggcgctaaagcggatccagaaggtacgcactttcccaccctccaactctttgggtgtccgaagcgtcgaggtgtgggcggggcgccgctgccgtgaagtgaaaggtgacggaggctccgcgagtcgcggatacacctgcctgggaaggaggcagaacagcctcccgcgcagcctgaaaagcgaacgcagcct

SEQ ID NO: 17857 - RNA, 3489 nt, Homo sapiens
  source 1..3489: mol_type = other RNA
tcgaggagctcacagtctggggggacagacatgtaaacacatgagttacaacgcgctgcgtgaagtgtgtggcagaggtataacaaagtgctgtggggcacaacagagcgaccagtgaactcttcctgggcaggggtcagggaagccttcacagatcagtcaataaatacggtgccatgggagtgccttgcacaccacgggcactcacatcttgaatgctggtccactggaggcccttgggttgggcgggagcaaggcctacttctgcttcctcaggacaacttccccacctctgtcctgggaccacctgcccgcctgggcctgcagtgactaaggacgctgctcccactccaggggccagtgacagagagcagctatacagagggcccaccccgcaggatccttgacaggagctgagacagaacaaactgctgcttgtctccctaccctgggggctgtgatattcttggtaacatctctgagctggtctgtgaggtcacttcctcttttaacactgttgaggagactccaaaccctgtcttttcctcgtcttctcatgtcgattgggcaccagccattctcaggcaccagagcacagccccacacgggtgccccatcagacagggctgcccacagcagcctcctacacctgaactgggtttctctgcacactcacagccgtctcaccagctcaatgagctgctggatgtttttgttttggttcgacaagccgttcctgatgttttcgagtaggcatctcttcaattcaaatatggcttcactgtaggccaagctcactgcggccatgggaggtgctccgtgccacaggcctgggatgtgccagatgtgctgcttctcagggtcgcagaaggccaggcctgccagtgcccggaagccgtcgccctgtttctccatctgggctgcagccctgctcaggtcaccaggtggatccaggagctgtctcttgtctctgggcctagggccgggaacagatacatcatgaaggttctggtatacaaactggtagttgggcatgtgccccgttttttctaacctcagaaatgcatgcagaatagctgctggaatgtccttggtttcagctagactgatcacggtgacattgctcagtcccatgagcagagtggccaaggaagcctccagctcaaatctgtccccagctgacgtcaaggccccacctatcaagcccccggagtctatcaccaggatgtggtcacagcccaggtcctggctgaagccctcagccactgtgatgagctgcatgaaggcccctcgaggaccgcagctcttccctgtggcaaaccgcagcccaaacatggtgttgaggagtgtggacttgcccgtgcctggcaccccgacggttgacagaaccaccagccttgaccgtctctccagtcggacgtgcagctccttcaggagccctgtgacccagcggacgggcatgctcagcgtgctcccatcgattagctccagaggcagccctgtcagcagcagctccgaggccaagcctgggaagtgggcaaaacgcctctggcctgccggcagcctccctgcctccacaagacagctctcagcctcataaaactgtcccatctcccgcaagaagtgttccacccctaggggctcaggccagagcggctcccccacgtctgtggtgcccccatgctttggtctcagggtgagaagcgtctccggaggctgtctcagtcgcggctgggccacccgtgccaggccccactccatccacctcaggaagtactgcttctcactcaaggaggggctgctgatccccgagatgaactcctgcacccccgaggagggatcatggccgttctgctgcattcgaagttctagcagccgccgcctcagctcagccctgtgcttctcaggggggtccacggcccactggagctggcagaactccttctccacttgggctgcctttctccaggggtccccctgcagcctcagctcgtcccttctgtaggcatccgagtctttgattttcctggtaatcctctccatccggtctttcgctttctgacactcctcacagtcctcgtcgacctttaggcccagtttgcgggctgcgtgcgccatgtcctccacagatacccgcctgcagggtgcccgcagcacattcccaacgatggcccggatcctcttcacgaagctgtcgctgtcagtgctgctgacctttaccaggacatgtgagtggtctattttcagcacaggaattaacttattcagaaatctcaggtttgtgttgcgcttcccacggtagggactcaggatgaagtagtattttgtggttgactccttcatggagtacagcaatttgtattccttcttactgatattgtcagtcaatataaacacagcggaggagatttctgtcaagagcttaaactgcagccagtgagacccgatgtcacctctcaggttcagaaaggccacaggttctgggaaaatgtccaagtcctcccttccgctgggaaaaaaccaggaaatttctaccaacccatccgaaatctcccgggcattggtgcccaagttgaggtcccgatgccagaagcagtcccactgcctgtggcccgggctgaggacggcgttgagaagctgggacttggagttgctactgacgtccatgcgcacgaaggcgaaggcgggcgccctggacaagaccacgctgtcttcccggaagctccccatgccccttgggggctgggaccaccatgtcctcacaatgccccgcatggcccacagcagaaatgtatggtagtggttctccgagtcaggcaacacgagtgggagtgcaaactggcagagggccattttcaacgctatttcttgttgcaggaaactgtctgaggagagcagcagggcacagagaaggtctaaggggttcactggcgtatcaggggtgggcagctcagaaaaggaataaatgtcggcagcaaggtcatcagctgggtcccagtagatgatctcctcttccatctggctctccttctccacaggcctggcgtctgggagcacgtccagcaccatagtggtattcctggcatcagcattgagggcctgcaacttcctgaggaaattccagggcaagtctttgggaacctgaggggcccagttcttcatactgtcaaaactgatctgcagagagtcctggaggctgagtttctggacctggtacgtctctaggcccaaaagtgacagcatttcttgaagcctgcttctctccactgttggaaaatcattgtcctgagcctcatttgtaccatctccataacggaactcgcaatcatctccttccatttctctccattccaaatctgcaatggccacagctgttcgtctctctgatgcttttatttctggggctacttctcccaaatctgaatgccctttgcccagtaattccacttctatcccgggcgacgccatgagcgcagcgaggtctccgct

SEQ ID NO: 17858 - RNA, 4171 nt, Homo sapiens
  source 1..4171: mol_type = other RNA
tcgaggagctcacagtctggggggacagacatgtaaacacatgagttacaacgcgctgcgtgaagtgtgtggcagaggtataacaaagtgctgtggggcacaacagagcgaccagtgaactcttcctgggcaggggtcagggaagccttcacagatcagtcaataaatacggtgccatgggagtgccttgcacaccacgggcactcacatcttgaatgctggtccactggaggcccttgggttgggcgggagcaaggcctacttctgcttcctcaggacaacttccccacctctgtcctgggaccacctgcccgcctgggcctgcagtgactaaggacgctgctcccactccaggggccagtgacagagagcagctatacagagggcccaccccgcaggatccttgacaggagctgagacagaacaaactgctgcttgtctccctaccctgggggctgtgatattcttggtaacatctctgagctggtctgtgaggtcacttcctcttttaacactgttgaggagactccaaaccctgtcttttcctcgtcttctcatgtcgattgggcaccagccattctcaggcaccagagcacagccccacacgggtgccccatcagacagggctgcccacagcagcctcctacacctgaactgggtttctctgcacactcacagccgtctcaccagctcaatgagctgctggatgtttttgttttggttcgacaagccgttcctgatgttttcgagtaggcatctcttcaattcaaatatggcttcactgtaggccaagctcactgcggccatgggaggtgctccgtgccacaggcctgggatgtgccagatgtgctgcttctcagggtcgcagaaggccaggcctgccagtgcccggaagccgtcgccctgtttctccatctgggctgcagccctgctcaggtcaccaggtggatccaggagctgtctcttgtctctgggcctagggccgggaacagatacatcatgaaggttctggtatacaaactggtagttgggcatgtgccccgttttttctaacctcagaaatgcatgcagaatagctgctggaatgtccttggtttcagctagactgatcacggtgacattgctcagtcccatgagcagagtggccaaggaagcctccagctcaaatctgtccccagctgacgtcaaggccccacctatcaagcccccggagtctatcaccaggatgtggtcacagcccaggtcctggctgaagccctcagccactgtgatgagctgcatgaaggcccctcgaggaccgcagctcttccctgtggcaaaccgcagcccaaacatggtgttgaggagtgtggacttgcccgtgcctggcaccccgacggttgacagaaccaccagccttgaccgtctctccagtcggacgtgcagctccttcaggagccctgtgacccagcggacgggcatgctcagcgtgctcccatcgattagctccagaggcagccctgtcagcagcagctccgaggccaagcctgggaagtgggcaaaacgcctctggcctgccggcagcctccctgcctccacaagacagctctcagcctcataaaactgtcccatctcccgcaagaagtgttccacccctaggggctcaggccagagcggctcccccacgtctgtggtgcccccatgctttggtctcagggtgagaagcgtctccggaggctgtctcagtcgcggctgggccacccgtgccaggccccactccatccacctcaggaagtactgcttctcactcaaggaggggctgctgatccccgagatgaactcctgcacccccgaggagggatcatggccgttctgctgcattcgaagttctagcagccgccgcctcagctcagccctgtgcttctcaggggggtccacggcccactggagctggcagaactccttctccacttgggctgcctttctccaggggtccccctgcagcctcagctcgtcccttctgtaggcatccgagtctttgattttcctggtaatcctctccatccggtctttcgctttctgacactcctcacagtcctcgtcgacctttaggcccagtttgcgggctgcgtgcgccatgtcctccacagatacccgcctgcagggtgcccgcagcacattcccaacgatggcccggatcctcttcacgaagctgtcgctgtcagtgctgctgacctttaccaggacatgtgagtggtctattttcagcacaggaattaacttattcagaaatctcaggtttgtgttgcgcttcccacggtagggactcaggatgaagtagtattttgtggttgactccttcatggagtacagcaatttgtattccttcttactgatattgtcagtcaatataaacacagcggaggagatttctgtcaagagcttaaactgcagccagtgagacccgatgtcacctctcaggttcagaaaggccacaggttctgggaaaatgtccaagtcctcccttccgctgggaaaaaaccaggaaatttctaccaacccatccgaaatctcccgggcattggtgcccaagttgaggtcccgatgccagaagcagtcccactgcctgtggcccgggctgaggacggcgttgagaagctgggacttggagttgctactgacgtccatgcgcacgaaggcgaaggcgggcgccctggacaagaccacgctgtcttcccggaagctccccatgccccttgggggctgggaccaccatgtcctcacaatgccccgcatggcccacagcagaaatgtatggtagtggttctccgagtcaggcaacacgagtgggagtgcaaactggcagagggccattttcaacgctatttcttgttgcaggaaactgtctgaggagagcagcagggcacagagaaggtctaaggggttcactggcgtatcaggggtgggcagctcagaaaaggaataaatgtcggcagcaaggtcatcagctgggtcccagtagatgatctcctcttccatctggctctccttctccacaggcctggcgtctgggagcacgtccagcaccatagtggtattcctggcatcagcattgagggcctgcaacttcctgaggaaattccagggcaagtctttgggaacctgaggggcccagttcttcatactgtcaaaactgatctgcagagagtcctggaggctgagtttctggacctggtacgtctctaggcccaaaagtgacagcatttcttgaagcctgcttctctccactgttggaaaatcattgtcctgagcctcatttgtaccatctccataacggaactcgcaatcatctccttccatttctctccattccaaatctgcaatggccacagctgttcgtctctctgatgcttttatttctggggctacttctcccaaatctgaatgccctttgcccagtaattccacttctatcctgtagtcccagctactcaggaggctgagatggtaggatctcttgagcctgggaggctgaagccacagtgagccaagatttcaccactgcactccagcctgggtgacacagcaagactctttagagttaagaaccactattctcaggagttatatgacagcctgggaagacgcccaggatgtaggaacagggagcaggcgagcgtgtggcaccttgagggtgctccgcgcgtctccgtaaagccaacgagcccctcctcttcgctggcctctccggggccttgctgactagtggtcgaagccacaggaccaggtgcgggtggccagcgtaacccgggcagccccgctgcttcccctcggccgcgccaggacgctcggcacgcggcgacgacggccccacagtgccccgcgcgcgcaagcgcaggctgcggctcccggcgtgcagcttggtggcggctgagccggcagcgggccgcctcaggcagccccggccgggccgcccgggtccccggcagcggggtaggatggcgctaaagcggatccagaaggtacgcactttcccaccctccaactctttgggtgtccgaagcgtcgaggtgtgggcggggcgccgctgccgtgaagtgaaaggtgacggaggctccgcgagtcgcggatacacctgcctgggaaggaggcagaacagcctcccgcgcagcctgaaaagcgaacgcagcct

SEQ ID NO: 17859 - RNA, 5773 nt, Homo sapiens
  source 1..5773: mol_type = other RNA
tcgaggagctcacagtcttaataggaagagaaatgtgcacacattttttgaggacagaaagaacagactaggagaagggttcaatggttctcaacccttgtgacatattagaatcatttggattttttttaagagatagagtcttgctctgtaacccaggctggagtgcagtggagtaatcataggtcactgtagcctcaaactcctgggctcaagtgatcctcccaccttggcctctggagtagctaggattaaaagcatgcaccaccatgcccaactaagtttttaaaaaaattttttttgtagagatggggtcttgttatgttgcccaggctggtctccaactcctggcttcaagtgattcccccagacctcagcctctcaaagttctggtattacaggcaccagccactgcaccctgcctggacaacatttaataaataccgatgcccgagcctgtgttcagacacactgaggttaattagtctggtgtctggcctgatcactgattttttttaagtcgcccaggaaattataatgagcatccagggttgagaatcactgagttagttattctactttcatcctgattgaattgtttcactagactaagaactgacaaagactctcaaattcaatatttaaaacaattctttacaaatcaattcttttattaaaaattatatgatgcatgcatatattttaaaaagtcaaatggtactaaggcttatgactaaaatatagcaattccttgtcccactcatactccttcatactctgttgactttgactgtttaaattatttttatagaattcatacatctccctacatcagaatgtcaatgcactggcatcttttgcaaaaccgattgctgaacttcatttcctcctatccaaaactaccctaaagcccccaaggaaaggtaaaaaggaagaaacaccaggtaattagagcagtaggaagcaagggagaggtttttcttttcaacccgtgcctaggtacagactagcccttctaatgggcctaagcaattcagaaaggcagctaagagagcttctcgaaaccctgcctgctcttccacctcttggaaggctgaggggctttatctaaaatcataaccaaaatttccacatgtctcctggattcaagcctccccagagtcaatcaagttatcctaaacttttctagaagttaaaaacagtttggaaatatgaatacttccaaagcaatttaaaaatccttgcaaaagcaagagtaatttgaagagtacagaattggctcagccatttggggaactgactagaaaaggggaactttgatttcatttctaatatgtatcatatacattggaaagtttcacttagggagataataaaagtttaattgaggtagtaggcatttgaaaaaggatgtgattgccaagtaaggatttcaaaggtggaggggacagaaaagggtttaaagactgagaaaatggcacaggcacagaccaggagtcggggatgtgtgtgggtggtgttggtggtaaagttgccaccaaggatccccataaactctgagagttggatttaaaaattagcaccaagtcataatggaagaaatcagagatgtgcaaaggccccttgtaggaagactactttccaggccagcggcagagtataaggcatttctagcctacatgaatgtattcacatacatagaggataaatgtaggcaaaatttgtatatgttgggggcagtaaggagagggttggtggtgaacctggaaattttagaaaccaagacagagaaaaaaaaattcatctgagggcaaagaataatgaaaaactagtcatccttagcattctaaatttgctttagcttgtaaactgtaaactaatttgtctagtccttgtgatagaaatatctttattttagaaattattgcaatcttattttatattaagttggtgcaaaagtaattgtggcttttgcacttttgcaccaacctaatagatattgcaatagtctaatataatctgaagatttttaagatttgaatcaaattaccagcttcccttactgtaaggctatgttcatataatttggcttcctatattactgttgagggcactgattagcaaaagcatttgacccacttatgactatggtcctcactataaattaacagagtaacattttgatgtatgcattggtcctttgtgagcttgattagcataaagcatccccaagagactgatctagacttggtacaaaaaggcaatcaagttctggacctggaaagcttgagacccatagccagtatgaggtgccagtcaattggctacttttgagacctatgcagtcaaagtaaccagcctggagggcaccataccaccacccaaaaattatgccaggtgggctggggtgcatgagaaacatggggagatggagatacaataaaggatgtggttgggagagcaagtcagggcatattaatgaaagccttgaaaattggttaggtttgaaggctgtggggactcattgaagatatgttagcaaggtattacataaaatcagttctctatttgaggaaaaattctctgatggatgacagctggattgagtgggaaagctggagacaggggactaatgaagtctattgtaattgtataggtaggaggtgaaggaaattgtgaaaaggccagtggcattgaaatagagtggaaggctcagctccaagagacatttctgtggctccaggccatactgatgtgccttgatttcctcacttgtaatattaaaatggagtcactgctacctgtctaggagaaaggactctgctcttcctgtcttcctctattatttgtaataattttcagtaggctgccctcttttcataaagcaggtagaggtgtttaatggctcttgaagcaaagcagagcttatgaaattcctctgactggtcacattctggactaagcccaaacacgacagtcctctccaggcctgaaaattgctgaatactgtctaaaacaatgtgacttccccaaacaccggtggccgggctaaacacaacctctgatggtctgtgggtctcaattaattccattgctttgagtagtgcaagcctatagcgtcctctgtcctcccctctcctgcacagaattgctatatctttgggcagatagccacactggaacaggctgtgacattttcttgccacatagttagctatttgttctgttgtcagattagtctttgtctcacacaccccaggcagagcctgggcacacgttgcttcctcataggcagtctcgctgaacaatgctaatgtgtctggagacatgttggagggaggattttctttgatcctcttcatttcttctttcataaccttcgctatttccagagcacagtggatcccactggtgattgtttttcgaggaaactgagcagatggagggggaaggccattgacatctgcgtgatggatttgaaaagggtcaagaaaaagccagagaatcccatggtgaaggttttcacttccagtccccttcgcctttggatgggtgatgttcttagccttcatgtaccaattgccatatttgctgcagaaattctcagtctcatccatcactatgtgtttaatctttagaaactccccttgcatgaaagttttcctggtcacagcttggcaggtggtttgttgggtcacaaaatcctttagggagtcgctttcacaaacatagaggatctcttttggtttgcagtgaaacaagtccttaattttctccatgatctttatggctagggctgtcttcctgactcctggaaagcagtagatgaataattcacgtgtcttctgaagactctcagaaagcaactggctctgctccattatgagcaagttgaaaaattcacagcccatctggtcactcagaagagatctggaggacagggagaccaccaccagagcctgcagcaagtcttccatttcctcctcatcagcaagcctgtaggacctggggtaacgcagggggatctcaccaggtctactctgtgtgctgctcaggtgtatcagccttggaatgatgcacactttccctgtgtaaccaccaacagtttgcagtttctgctttaactgatgagctgtgtttcgggcatattcaagtcctccaggccaattggggtctattaagattgtatagagtaccacggggctgttaactgctatcaggagagcatcacacaggacattctgttctttcctgaagccaacatcaccagcccagcttctagaaaatatcacaatcccctgagaacaaggatgtatcagggtcttcattaaaccctccagttctttatgatctgagaacagcttcttacagagggattctggtttaaattgtacctcttcctgtgtcactggaaacaaatgtcgttgcagagcctccttaaatttgtggacttttatgggatatccgggactttttcgtgcagatgaagctgatgaaatcaggcaagagttgtagtctgtgaccaaactgggaggagctgactgagtatccagcatcatgaccacccactgctcagctgtcagccgtgtgacagaattgtctttcatgatccaggaatctggggcctctgcaaacaccacgcaacagaagggctccacttgaatcacacagacataaccatccaggacatctttttggtacacattcaggatttttgtagtgaaatttacctttggcttctcacagcagaagtggaatgtaggcaatttttctatgcagttttcgatttctttttttagtaagtcaggattcactttttcccacttacatccaaccacttctttgctcttatcatccaccccaatgaggacatatcccccttgagtgttggcaaatgcagaaacataatgaggcagcatttccttaatccgaggtatgacttttttggtggtgaaccttttaaattcaacatgtgttgactcagtaaagttgagtttctccttatacatgagtttgtcctttttaaaaaattctgaggccaatatcctcatatcttcctcttcctgaatgcatctattgagaacctgctgaggatgcaacttcttcacccttggtcttcctctttgggctctaaaccccttctctctgagaagctccagggcactgctagcactcaagttgatagcagaagtcacatctctccgatacaaattggagcgcaagctgcaaatccttagtggaaggctgaaaacatctgggctccatgacttcacaaaaatcaggagattgtgcccctgctgcatgtagtcaaggtatttctgtgaacctgaaggaaggagcttttgaaaagaagtttccaaatcctgtcccagcccatggcattggtaactataggttttatcatcaatctctgctttgatcacaccacctccagaatttaacagtgcacatatagcccggataattctagaattctcagatcttttcaaacagctgttggtcatcttcttcctgttttcttctccaaaaatcactctgcccacatctactattacctcaggatacggcatttcagtatcagtcttgagactctccatttcagcagcccctctgtgctccaaacaataaaagaaaggagttccaagaggaagaaagcaggcatccggcaagacatgtgcactcccctgatatcaatttgttcttggttgccttctcacttcctatgctcctgtgtttcctcttgctgcttcagtttcacatctggctgtagtct

SEQ ID NO: 17860 - RNA, 1020 nt, Homo sapiens
  source 1..1020: mol_type = other RNA
tcgcctcctcctctcccacctgaagtcaagtgggctcagtgaagtttcacctgcagggtagctggggatgcagggagtctccaagtcctaggctggagtcccgaccccgtttgctctcaggaagatgacaaggaccatggttcctagcacggagtagtgtcctcctgtctcccaccttcagtgtgacctggcagtaagacaccactcccacttctatcaggaggtgaccctgacactcagagacacctgcggacccgatgatgtctggccaccagtggacaggcgctctcagccctcctgcaaacggctggcacacctacctgagagaccaaacatttccccaaagcacattatacaacaagaacaatttcaatttgcaaaaaaaacgagtgacacagtagagctttcttttcaggccctacaattcaccagtgctggcaatatgtgtaacggaatgtggctcacaacagtaaggcaagctccttcgcaggaccccaagttccctgagatgacagaagtgtgttcaaacccatcgaggcactccttctacaatgaggtagaccatgtgtttaaaagagagactatcgtgcctggaaaactcggaaccggtacaaatacgaagcgagttctcctccacggagaggcccgtccgtatggggcctggctccctggggtcgcctctgccggggactgcctcccgccgctcagcctggaacctacccttggccaacgcctcctggtacttctcctcggtgacgttcaggttgttcacgtaggccgcgtggtgcttgctgtggtgcagctgcatgatctgcgcgttgatgtgaggttccagggcgccgtagtcgtagggcaggtcggggaggctgtgcttctgcctggagcccagataccccaaaaccggagccagctgcctgctggtgccgcacactgcccggctcaacatgctgctagtgctggtgctaccgctgatgccgccgatctgctgaagccgctgccgaagccaccacagccacgagt

SEQ ID NO: 17861 - RNA, 2579 nt, Homo sapiens
  source 1..2579: mol_type = other RNA
tcgcctcctcctctcccattttgggaggattctcaaggttctcagaagcaccaatgccacctcggctctgcaccggggccgccgagcttgggttccgtgactgctgcccggacatcgcctcttctggaggctgaacaacaggtggctgaggttttgcacacacataaagcgccggggctgcaggggccagaaggacgttgcctccaaaatctggcagctcactttgcgcccacagagtcgttgctgggctctcacacttcacgggcccctgggtcctggctgaaggcctcttctcgggtgctggatacacagtatccaagggcggtgcccctgcgtgcggaagcatgtgcacagcttccgtggtggagttaagaggcaggggacagacctggggtgcacagagggtctccatgttgtctggtggctgctccaggttgccaggggaagcatcgggcagggcggcagctggtctgcactgcttctggcggacacaggtctcccttacttcaccaaccacgttggcgcgatctgcctcaaatggttttaccccaactaagtgagattttaccggttcgaaagaactatttgcacttgtctgaaatattcctgtaggtttcggggggctcggggttgagggctgggacacgctgccacggtaattctggctcacagtggtctcgtctgtttcacctcctacgggagaagaatcgatttgcttaaaaaaactacctgaagcttcatcctcgggttttccaacttcttgctgaatgaatgtgccaaccagctcctggggcctggctgagcctgagagccttccgtggcttctgctgctatagctggatgacacgctgtcagggtgcactgtatgcagtgtggcatcaggggctccggtgtggcacacagcaccatgcctgggcacagctggcccaggaaggggcccatatctgaactggtcactcggggaggaagggtccaaattgaggggctcacttggcagaacttcttgattctgaacaaattctaagttctcaacattctcatactgcgagccgctggcatccggcacccctgtgctcgctgtgtcaccccacacatcaccagcagcctcattgctggggcctgggagaagggcctggcagaggctgcctgcccccacgtgtgtaggtgcgggcggacggcctagcccagggctggagcagaaatcgtcaaagtccgcttgaccagataagcctgctttttcagatgagagattctcctcattttctgtctctcccccttggaaaaacatcgccagagctcctgaagctcctgagtctgcttctagcggggcacagccagacccggccccagcccccagtgggtggtgcgtacggttttctgggctatctccccgggcgagggggttcacaagagcagaggcgggccggtgctcattcttcactcctggattctgcctgagctctgggcttgcccagtgattcacaattctgggattttgcctgaatgtactttcaggatcagagttattggccaggtggcttccactttgcaagtggctcacctcgtctcttccgtcactgggcaaggctgctgggggagccaccagagggctgtgttgctcatgaccagggccctgatgtaggatggacggggtggggaaatgaggaacgctggtggcacagggcaccccgctgggaacaggtccttcagggcagggtgaacgatgttgccccgagggctgtgggcctccctgcactggcccccactgtcctggcatctgcagaccaggctgagggagggaaggggatgctgctggggtgaccacaccgtcatgtgggttttgcctgctcaggggtcggtcgagcccaggcatgttcccatgagggtggcccccatgagacgtttcaggatccactcctggaatgtagtgaggaagatatggcagagtctgaacttcaggctctgaactgggaccgacctctgcactcctgttcatctcaggcccaggaggtgctgaaggtgtcaatgcaccagaaaacggactggcatgtgctctgggctgtgtcagaggtccaggcaggggctcacagggtccctgagagctatctctggcatgtgtgtgaggaacaagcaaaccggggtgctgagaaaaccctgcgggggctgggccttgcaagacaggtggactgcttttggacgaactgcccagtggtgtactttggagcgcctgtctactaaaagcaaatggatccgtgaccggctgcaacgggcaagttgtcggagccactgctgcattattattagcccgtctcctgtaagggctgctagcccagaacacgctccgaggattcccggctggaggtggcccagccatgccagacgggaccgtctggggcggtggctgcatgactgaacccttgcacaagtcgatgctgcttacagaaggaagcaggatatagctgttccttaattggagccgcgcggctgagaccgatccctcaggagccgcgggcgaaagcccacccgacgctggcgacgagcacagacacctcagccgccgcagccatcttggcacatcc

SEQ ID NO: 17862 - RNA, 2556 nt, Homo sapiens
  source 1..2556: mol_type = other RNA
tcgcctcctcctctcccattttgggaggattctcaaggttctcagaagcaccaatgccacctcggctctgcaccggggccgccgagcttgggttccgtgactgctgcccggacatcgcctcttctggaggctgaacaacaggtggctgaggttttgcacacacataaagcgccggggctgcaggggccagaaggacgttgcctccaaaatctggcagctcactttgcgcccacagagtcgttgctgggctctcacacttcacgggcccctgggtcctggctgaaggcctcttctcgggtgctggatacacagtatccaagggcggtgcccctgcgtgcggaagcatgtgcacagcttccgtggtggagttaagaggcaggggacagacctggggtgcacagagggtctccatgttgtctggtggctgctccaggttgccaggggaagcatcgggcagggcggcagctggtctgcactgcttctggcggacacaggtctcccttacttcaccaaccacgttggcgcgatctgcctcaaatggttttaccccaactaagtgagattttaccggttcgaaagaactatttgcacttgtctgaaatattcctgtaggtttcggggggctcggggttgagggctgggacacgctgccacggtaattctggctcacagtggtctcgtctgtttcacctcctacgggagaagaatcgatttgcttaaaaaaactacctgaagcttcatcctcgggttttccaacttcttgctgaatgaatgtgccaaccagctcctggggcctggctgagcctgagagccttccgtggcttctgctgctatagctggatgacacgctgtcagggtgcactgtatgcagtgtggcatcaggggctccggtgtggcacacagcaccatgcctgggcacagctggcccaggaaggggcccatatctgaactggtcactcggggaggaagggtccaaattgaggggctcacttggcagaacttcttgattctgaacaaattctaagttctcaacattctcatactgcgagccgctggcatccggcacccctgtgctcgctgtgtcaccccacacatcaccagcagcctcattgctggggcctgggagaagggcctggcagaggctgcctgcccccacgtgtgtaggtgcgggcggacggcctagcccagggctggagcagaaatcgtcaaagtccgcttgaccagataagcctgctttttcagatgagagattctcctcattttctgtctctcccccttggaaaaacatcgccagagctcctgaagctcctgagtctgcttctagcggggcacagccagacccggccccagcccccagtgggtggtgcgtacggttttctgggctatctccccgggcgagggggttcacaagagcagaggcgggccggtgctcattcttcactcctggattctgcctgagctctgggcttgcccagtgattcacaattctgggattttgcctgaatgtactttcaggatcagagttattggccaggtggcttccactttgcaagtggctcacctcgtctcttccgtcactgggcaaggctgctgggggagccaccagagggctgtgttgctcatgaccagggccctgatgtaggatggacggggtggggaaatgaggaacgctggtggcacagggcaccccgctgggaacaggtccttcagggcagggtgaacgatgttgccccgagggctgtgggcctccctgcactggcccccactgtcctggcatctgcagaccaggctgagggagggaaggggatgctgctggggtgaccacaccgtcatgtgggttttgcctgctcaggggtcggtcgagcccaggcatgttcccatgagggtggcccccatgagacgtttcaggatccactcctggaatgtagtgaggaagatatggcagagtctgaacttcaggctctgaactgggaccgacctctgcactcctgttcatctcaggcccaggaggtgctgaaggtgtcaatgcaccagaaaacggactggcatgtgctctgggctgtgtcagaggtccaggcaggggctcacagggtccctgagagctatctctggcatgtgtgtgaggaacaagcaaaccggggtgctgagaaaaccctgcgggggctgggccttgcaagacaggtggactgcttttggacgaactgcccagtggtgtactttggagcgcctgtctactaaaagcaaatggatccgtgaccggctgcaacgggcaagttgtcggagccactgctgcattattattagcccgtctcctgtaagggctgctagcccagaacacgctccgaggattcccggctggaggtggcccagccatgccagacgggaccgtctggggcggtggctgcatgactgaacccttgcacaagtcgatgctgcttacagaaggaagcaggatatagctgttccttaattggagcgagaacggctactccgcccagctgagaagcgcggggccctgacgcgggcgcgctcctcgcattcttccgttgggctggg

SEQ ID NO: 17863 - RNA, 2650 nt, Homo sapiens
  source 1..2650: mol_type = other RNA
tcgcctcctcctctcccattttgggaggattctcaaggttctcagaagcaccaatgccacctcggctctgcaccggggccgccgagcttgggttccgtgactgctgcccggacatcgcctcttctggaggctgaacaacaggtggctgaggttttgcacacacataaagcgccggggctgcaggggccagaaggacgttgcctccaaaatctggcagctcactttgcgcccacagagtcgttgctgggctctcacacttcacgggcccctgggtcctggctgaaggcctcttctcgggtgctggatacacagtatccaagggcggtgcccctgcgtgcggaagcatgtgcacagcttccgtggtggagttaagaggcaggggacagacctggggtgcacagagggtctccatgttgtctggtggctgctccaggttgccaggggaagcatcgggcagggcggcagctggtctgcactgcttctggcggacacaggtctcccttacttcaccaaccacgttggcgcgatctgcctcaaatggttttaccccaactaagtgagattttaccggttcgaaagaactatttgcacttgtctgaaatattcctgtaggtttcggggggctcggggttgagggctgggacacgctgccacggtaattctggctcacagtggtctcgtctgtttcacctcctacgggagaagaatcgatttgcttaaaaaaactacctgaagcttcatcctcgggttttccaacttcttgctgaatgaatgtgccaaccagctcctggggcctggctgagcctgagagccttccgtggcttctgctgctatagctggatgacacgctgtcagggtgcactgtatgcagtgtggcatcaggggctccggtgtggcacacagcaccatgcctgggcacagctggcccaggaaggggcccatatctgaactggtcactcggggaggaagggtccaaattgaggggctcacttggcagaacttcttgattctgaacaaattctaagttctcaacattctcatactgcgagccgctggcatccggcacccctgtgctcgctgtgtcaccccacacatcaccagcagcctcattgctggggcctgggagaagggcctggcagaggctgcctgcccccacgtgtgtaggtgcgggcggacggcctagcccagggctggagcagaaatcgtcaaagtccgcttgaccagataagcctgctttttcagatgagagattctcctcattttctgtctctcccccttggaaaaacatcgccagagctcctgaagctcctgagtctgcttctagcggggcacagccagacccggccccagcccccagtgggtggtgcgtacggttttctgggctatctccccgggcgagggggttcacaagagcagaggcgggccggtgctcattcttcactcctggattctgcctgagctctgggcttgcccagtgattcacaattctgggattttgcctgaatgtactttcaggatcagagttattggccaggtggcttccactttgcaagtggctcacctcgtctcttccgtcactgggcaaggctgctgggggagccaccagagggctgtgttgctcatgaccagggccctgatgtaggatggacggggtggggaaatgaggaacgctggtggcacagggcaccccgctgggaacaggtccttcagggcagggtgaacgatgttgccccgagggctgtgggcctccctgcactggcccccactgtcctggcatctgcagaccaggctgagggagggaaggggatgctgctggggtgaccacaccgtcatgtgggttttgcctgctcaggggtcggtcgagcccaggcatgttcccatgagggtggcccccatgagacgtttcaggatccactcctggaatgtagtgaggaagatatggcagagtctgaacttcaggctctgaactgggaccgacctctgcactcctgttcatctcaggcccaggaggtgctgaaggtgtcaatgcaccagaaaacggactggcatgtgctctgggctgtgtcagaggtccaggcaggggctcacagggtccctgagagctatctctggcatgtgtgtgaggaacaagcaaaccggggtgctgagaaaaccctgcgggggctgggccttgcaagacaggtggactgcttttggacgaactgcccagtggtgtactttggagcgcctgtctactaaaagcaaatggatccgtgaccggctgcaacgggcaagttgtcggagccactgctgcattattattagcccgtctcctgtaagggctgctagcccagaacacgctccgaggattcccggctggaggtggcccagccatgccagacgggaccgtctggggcggtggctgcatgactgaacccttgcacaagtcgatgctgcttacagaaggaagcaggatatagctgttccttaattggagcgcttggccccgcccctcgccacctgcccggccaggcgcgccggggccgtcccagtacgtcgccctgtttacgctggctctttctcccagtcttttttcgttttaagatgtgagaagagatgggattcttcaatcaaggccacaagcgggaaatcagtctgcaggaccgatgcc

SEQ ID NO: 17864 - RNA, 2750 nt, Homo sapiens
  source 1..2750: mol_type = other RNA
tcgcctcctcctctcccattttgggaggattctcaaggttctcagaagcaccaatgccacctcggctctgcaccggggccgccgagcttgggttccgtgactgctgcccggacatcgcctcttctggaggctgaacaacaggtggctgaggttttgcacacacataaagcgccggggctgcaggggccagaaggacgttgcctccaaaatctggcagctcactttgcgcccacagagtcgttgctgggctctcacacttcacgggcccctgggtcctggctgaaggcctcttctcgggtgctggatacacagtatccaagggcggtgcccctgcgtgcggaagcatgtgcacagcttccgtggtggagttaagaggcaggggacagacctggggtgcacagagggtctccatgttgtctggtggctgctccaggttgccaggggaagcatcgggcagggcggcagctggtctgcactgcttctggcggacacaggtctcccttacttcaccaaccacgttggcgcgatctgcctcaaatggttttaccccaactaagtgagattttaccggttcgaaagaactatttgcacttgtctgaaatattcctgtaggtttcggggggctcggggttgagggctgggacacgctgccacggtaattctggctcacagtggtctcgtctgtttcacctcctacgggagaagaatcgatttgcttaaaaaaactacctgaagcttcatcctcgggttttccaacttcttgctgaatgaatgtgccaaccagctcctggggcctggctgagcctgagagccttccgtggcttctgctgctatagctggatgacacgctgtcagggtgcactgtatgcagtgtggcatcaggggctccggtgtggcacacagcaccatgcctgggcacagctggcccaggaaggggcccatatctgaactggtcactcggggaggaagggtccaaattgaggggctcacttggcagaacttcttgattctgaacaaattctaagttctcaacattctcatactgcgagccgctggcatccggcacccctgtgctcgctgtgtcaccccacacatcaccagcagcctcattgctggggcctgggagaagggcctggcagaggctgcctgcccccacgtgtgtaggtgcgggcggacggcctagcccagggctggagcagaaatcgtcaaagtccgcttgaccagataagcctgctttttcagatgagagattctcctcattttctgtctctcccccttggaaaaacatcgccagagctcctgaagctcctgagtctgcttctagcggggcacagccagacccggccccagcccccagtgggtggtgcgtacggttttctgggctatctccccgggcgagggggttcacaagagcagaggcgggccggtgctcattcttcactcctggattctgcctgagctctgggcttgcccagtgattcacaattctgggattttgcctgaatgtactttcaggatcagagttattggccaggtggcttccactttgcaagtggctcacctcgtctcttccgtcactgggcaaggctgctgggggagccaccagagggctgtgttgctcatgaccagggccctgatgtaggatggacggggtggggaaatgaggaacgctggtggcacagggcaccccgctgggaacaggtccttcagggcagggtgaacgatgttgccccgagggctgtgggcctccctgcactggcccccactgtcctggcatctgcagaccaggctgagggagggaaggggatgctgctggggtgaccacaccgtcatgtgggttttgcctgctcaggggtcggtcgagcccaggcatgttcccatgagggtggcccccatgagacgtttcaggatccactcctggaatgtagtgaggaagatatggcagagtctgaacttcaggctctgaactgggaccgacctctgcactcctgttcatctcaggcccaggaggtgctgaaggtgtcaatgcaccagaaaacggactggcatgtgctctgggctgtgtcagaggtccaggcaggggctcacagggtccctgagagctatctctggcatgtgtgtgaggaacaagcaaaccggggtgctgagaaaaccctgcgggggctgggccttgcaagacaggtggactgcttttggacgaactgcccagtggtgtactttggagcgcctgtctactaaaagcaaatggatccgtgaccggctgcaacgggcaagttgtcggagccactgctgcattattattagcccgtctcctgtaagggctgctagcccagaacacgctccgaggattcccggctggaggtggcccagccatgccagacgggaccgtctggggcggtggctgcatgactgaacccttgcacaagtcgatgctgcttacagaaggaagcaggatatagctgttccttaattggagcgcttggccccgcccctcgccacctgcccggccaggcgcgccggggccgtcccagtacgtcgccctgtttacgctggctctttctcccagtcttttttcgttttaagatgtgagaagagatgggattcttcaatcaaggccacaagcgggaaatcagtctgcaggaccgatgccagcaggctcacgcaccgagaacggctactccgcccagctgagaagcgcggggccctgacgcgggcgcgctcctcgcattcttccgttgggctgggaggct

SEQ ID NO: 17865 - RNA, 2563 nt, Homo sapiens
  source 1..2563: mol_type = other RNA
tcgcctcctcctctcccattttgggaggattctcaaggttctcagaagcaccaatgccacctcggctctgcaccggggccgccgagcttgggttccgtgactgctgcccggacatcgcctcttctggaggctgaacaacaggtggctgaggttttgcacacacataaagcgccggggctgcaggggccagaaggacgttgcctccaaaatctggcagctcactttgcgcccacagagtcgttgctgggctctcacacttcacgggcccctgggtcctggctgaaggcctcttctcgggtgctggatacacagtatccaagggcggtgcccctgcgtgcggaagcatgtgcacagcttccgtggtggagttaagaggcaggggacagacctggggtgcacagagggtctccatgttgtctggtggctgctccaggttgccaggggaagcatcgggcagggcggcagctggtctgcactgcttctggcggacacaggtctcccttacttcaccaaccacgttggcgcgatctgcctcaaatggttttaccccaactaagtgagattttaccggttcgaaagaactatttgcacttgtctgaaatattcctgtaggtttcggggggctcggggttgagggctgggacacgctgccacggtaattctggctcacagtggtctcgtctgtttcacctcctacgggagaagaatcgatttgcttaaaaaaactacctgaagcttcatcctcgggttttccaacttcttgctgaatgaatgtgccaaccagctcctggggcctggctgagcctgagagccttccgtggcttctgctgctatagctggatgacacgctgtcagggtgcactgtatgcagtgtggcatcaggggctccggtgtggcacacagcaccatgcctgggcacagctggcccaggaaggggcccatatctgaactggtcactcggggaggaagggtccaaattgaggggctcacttggcagaacttcttgattctgaacaaattctaagttctcaacattctcatactgcgagccgctggcatccggcacccctgtgctcgctgtgtcaccccacacatcaccagcagcctcattgctggggcctgggagaagggcctggcagaggctgcctgcccccacgtgtgtaggtgcgggcggacggcctagcccagggctggagcagaaatcgtcaaagtccgcttgaccagataagcctgctttttcagatgagagattctcctcattttctgtctctcccccttggaaaaacatcgccagagctcctgaagctcctgagtctgcttctagcggggcacagccagacccggccccagcccccagtgggtggtgcgtacggttttctgggctatctccccgggcgagggggttcacaagagcagaggcgggccggtgctcattcttcactcctggattctgcctgagctctgggcttgcccagtgattcacaattctgggattttgcctgaatgtactttcaggatcagagttattggccaggtggcttccactttgcaagtggctcacctcgtctcttccgtcactgggcaaggctgctgggggagccaccagagggctgtgttgctcatgaccagggccctgatgtaggatggacggggtggggaaatgaggaacgctggtggcacagggcaccccgctgggaacaggtccttcagggcagggtgaacgatgttgccccgagggctgtgggcctccctgcactggcccccactgtcctggcatctgcagaccaggctgagggagggaaggggatgctgctggggtgaccacaccgtcatgtgggttttgcctgctcaggggtcggtcgagcccaggcatgttcccatgagggtggcccccatgagacgtttcaggatccactcctggaatgtagtgaggaagatatggcagagtctgaacttcaggctctgaactgggaccgacctctgcactcctgttcatctcaggcccaggaggtgctgaaggtgtcaatgcaccagaaaacggactggcatgtgctctgggctgtgtcagaggtccaggcaggggctcacagggtccctgagagctatctctggcatgtgtgtgaggaacaagcaaaccggggtgctgagaaaaccctgcgggggctgggccttgcaagacaggtggactgcttttggacgaactgcccagtggtgtactttggagcgcctgtctactaaaagcaaatggatccgtgaccggctgcaacgggcaagttgtcggagccactgctgcattattattagcccgtctcctgtaagggctgctagcccagaacacgctccgaggattcccggctggaggtggcccagccatgccagacgggaccgtctggggcggtggctgcatgactgaacccttgcacaagtcgatgctgcttacagaaggaagcaggatatagctgttccttaattggagctgcacacctgcctggcaagggcagggaagagccgcggccttcctctgctgctccttccagagggcaggcgccgtggtgggggtgcc

SEQ ID NO: 17866 - RNA, 2701 nt, Homo sapiens
  source 1..2701: mol_type = other RNA
tcgcctcctcctctcccattttgggaggattctcaaggttctcagaagcaccaatgccacctcggctctgcaccggggccgccgagcttgggttccgtgactgctgcccggacatcgcctcttctggaggctgaacaacaggtggctgaggttttgcacacacataaagcgccggggctgcaggggccagaaggacgttgcctccaaaatctggcagctcactttgcgcccacagagtcgttgctgggctctcacacttcacgggcccctgggtcctggctgaaggcctcttctcgggtgctggatacacagtatccaagggcggtgcccctgcgtgcggaagcatgtgcacagcttccgtggtggagttaagaggcaggggacagacctggggtgcacagagggtctccatgttgtctggtggctgctccaggttgccaggggaagcatcgggcagggcggcagctggtctgcactgcttctggcggacacaggtctcccttacttcaccaaccacgttggcgcgatctgcctcaaatggttttaccccaactaagtgagattttaccggttcgaaagaactatttgcacttgtctgaaatattcctgtaggtttcggggggctcggggttgagggctgggacacgctgccacggtaattctggctcacagtggtctcgtctgtttcacctcctacgggagaagaatcgatttgcttaaaaaaactacctgaagcttcatcctcgggttttccaacttcttgctgaatgaatgtgccaaccagctcctggggcctggctgagcctgagagccttccgtggcttctgctgctatagctggatgacacgctgtcagggtgcactgtatgcagtgtggcatcaggggctccggtgtggcacacagcaccatgcctgggcacagctggcccaggaaggggcccatatctgaactggtcactcggggaggaagggtccaaattgaggggctcacttggcagaacttcttgattctgaacaaattctaagttctcaacattctcatactgcgagccgctggcatccggcacccctgtgctcgctgtgtcaccccacacatcaccagcagcctcattgctggggcctgggagaagggcctggcagaggctgcctgcccccacgtgtgtaggtgcgggcggacggcctagcccagggctggagcagaaatcgtcaaagtccgcttgaccagataagcctgctttttcagatgagagattctcctcattttctgtctctcccccttggaaaaacatcgccagagctcctgaagctcctgagtctgcttctagcggggcacagccagacccggccccagcccccagtgggtggtgcgtacggttttctgggctatctccccgggcgagggggttcacaagagcagaggcgggccggtgctcattcttcactcctggattctgcctgagctctgggcttgcccagtgattcacaattctgggattttgcctgaatgtactttcaggatcagagttattggccaggtggcttccactttgcaagtggctcacctcgtctcttccgtcactgggcaaggctgctgggggagccaccagagggctgtgttgctcatgaccagggccctgatgtaggatggacggggtggggaaatgaggaacgctggtggcacagggcaccccgctgggaacaggtccttcagggcagggtgaacgatgttgccccgagggctgtgggcctccctgcactggcccccactgtcctggcatctgcagaccaggctgagggagggaaggggatgctgctggggtgaccacaccgtcatgtgggttttgcctgctcaggggtcggtcgagcccaggcatgttcccatgagggtggcccccatgagacgtttcaggatccactcctggaatgtagtgaggaagatatggcagagtctgaacttcaggctctgaactgggaccgacctctgcactcctgttcatctcaggcccaggaggtgctgaaggtgtcaatgcaccagaaaacggactggcatgtgctctgggctgtgtcagaggtccaggcaggggctcacagggtccctgagagctatctctggcatgtgtgtgaggaacaagcaaaccggggtgctgagaaaaccctgcgggggctgggccttgcaagacaggtggactgcttttggacgaactgcccagtggtgtactttggagcgcctgtctactaaaagcaaatggatccgtgaccggctgcaacgggcaagttgtcggagccactgctgcattattattagcccgtctcctgtaagggctgctagcccagaacacgctccgaggattcccggctggaggtggcccagccatgccagacgggaccgtctggggcggtggctgcatgactgaacccttgcacaagtcgatgctgcttacagaaggaagcaggatatagctgttccttaattggagctgtagtcccagggactcagggggttaaggaaggaagatcacttgtgtccatgagttcgaggctgcagtgagctatgattataccaccgcggtccagcctgggcaacagagcaagacggtctccgcgcggctgagaccgatccctcaggagccgcgggcgaaagcccacccgacgctggcgacgagcacagacacctcagccgccgcagccatcttggcacatcc

SEQ ID NO: 17867 - RNA, 2725 nt, Homo sapiens
  source 1..2725: mol_type = other RNA
tcgcctcctcctctcccattttgggaggattctcaaggttctcagaagcaccaatgccacctcggctctgcaccggggccgccgagcttgggttccgtgactgctgcccggacatcgcctcttctggaggctgaacaacaggtggctgaggttttgcacacacataaagcgccggggctgcaggggccagaaggacgttgcctccaaaatctggcagctcactttgcgcccacagagtcgttgctgggctctcacacttcacgggcccctgggtcctggctgaaggcctcttctcgggtgctggatacacagtatccaagggcggtgcccctgcgtgcggaagcatgtgcacagcttccgtggtggagttaagaggcaggggacagacctggggtgcacagagggtctccatgttgtctggtggctgctccaggttgccaggggaagcatcgggcagggcggcagctggtctgcactgcttctggcggacacaggtctcccttacttcaccaaccacgttggcgcgatctgcctcaaatggttttaccccaactaagtgagattttaccggttcgaaagaactatttgcacttgtctgaaatattcctgtaggtttcggggggctcggggttgagggctgggacacgctgccacggtaattctggctcacagtggtctcgtctgtttcacctcctacgggagaagaatcgatttgcttaaaaaaactacctgaagcttcatcctcgggttttccaacttcttgctgaatgaatgtgccaaccagctcctggggcctggctgagcctgagagccttccgtggcttctgctgctatagctggatgacacgctgtcagggtgcactgtatgcagtgtggcatcaggggctccggtgtggcacacagcaccatgcctgggcacagctggcccaggaaggggcccatatctgaactggtcactcggggaggaagggtccaaattgaggggctcacttggcagaacttcttgattctgaacaaattctaagttctcaacattctcatactgcgagccgctggcatccggcacccctgtgctcgctgtgtcaccccacacatcaccagcagcctcattgctggggcctgggagaagggcctggcagaggctgcctgcccccacgtgtgtaggtgcgggcggacggcctagcccagggctggagcagaaatcgtcaaagtccgcttgaccagataagcctgctttttcagatgagagattctcctcattttctgtctctcccccttggaaaaacatcgccagagctcctgaagctcctgagtctgcttctagcggggcacagccagacccggccccagcccccagtgggtggtgcgtacggttttctgggctatctccccgggcgagggggttcacaagagcagaggcgggccggtgctcattcttcactcctggattctgcctgagctctgggcttgcccagtgattcacaattctgggattttgcctgaatgtactttcaggatcagagttattggccaggtggcttccactttgcaagtggctcacctcgtctcttccgtcactgggcaaggctgctgggggagccaccagagggctgtgttgctcatgaccagggccctgatgtaggatggacggggtggggaaatgaggaacgctggtggcacagggcaccccgctgggaacaggtccttcagggcagggtgaacgatgttgccccgagggctgtgggcctccctgcactggcccccactgtcctggcatctgcagaccaggctgagggagggaaggggatgctgctggggtgaccacaccgtcatgtgggttttgcctgctcaggggtcggtcgagcccaggcatgttcccatgagggtggcccccatgagacgtttcaggatccactcctggaatgtagtgaggaagatatggcagagtctgaacttcaggctctgaactgggaccgacctctgcactcctgttcatctcaggcccaggaggtgctgaaggtgtcaatgcaccagaaaacggactggcatgtgctctgggctgtgtcagaggtccaggcaggggctcacagggtccctgagagctatctctggcatgtgtgtgaggaacaagcaaaccggggtgctgagaaaaccctgcgggggctgggccttgcaagacaggtggactgcttttggacgaactgcccagtggtgtactttggagcgcctgtctactaaaagcaaatggatccgtgaccggctgcaacgggcaagttgtcggagccactgctgcattattattagcccgtctcctgtaagggctgctagcccagaacacgctccgaggattcccggctggaggtggcccagccatgccagacgggaccgtctggggcggtggctgcatgactgaacccttgcacaagtcgatgctgcttacagaaggaagcaggatatagctgttccttaattggagctgtagtcccagggactcagggggttaaggaaggaagatcacttgtgtccatgagttcgaggctgcagtgagctatgattataccaccgcggtccagcctgggcaacagagcaagacggtctccgcgcggctgagaccgatccctcaggagccgcgggcgaaagcccacccgacgctggcgacgagcacagacacctcagccgccgcagccatcttggcacatccggctcgggtctccgcggccgccgc

SEQ ID NO: 17868 - RNA, 412 nt, Homo sapiens
  source 1..412: mol_type = other RNA
tcgcctcctcctctccccatggtgcgggaaaacccgacgggaaagtgggggaggcgcagagaaaggaggtgtagggaggtgaagcgggtactatcttcccactcggagcgccccttcggcagcacagctgcccggtcctccctctgctaagccctgactgctgcaggggagcaggaggagccggcacctcccagaaagcagaccctctctctggatcccgtttgcctgcaattcaatgcccctgggtgggtgtgaggtttcagggaggtcacaagtcatatcaagatgaggcgagctcacagctggagagtctccatcctgctgcccatctctgaacagatcagagatcttaaaaggcggcccttttaagaggccagctcggacccaggcaggggtcccggtgcccacgacc

SEQ ID NO: 17869 - RNA, 415 nt, Homo sapiens
  source 1..415: mol_type = other RNA
tcgcctcctcctctccccatggtgcgggaaaacccgacgggaaagtgggggaggcgcagagaaaggaggtgtagggaggtgaagcgggtactatcttcccactcggagcgccccttcggcagcacagctgcccggtcctccctctgctaagccctgactgctgcaggggagcaggaggagccggcacctcccagaaagcagaccctctctctggatcccgtttgcctgcaattcaatgcccctgggtgggtgtgaggtttcagggaggtcacaagtcatatcaagatgaggcgagctcacagctggagagtctccatcctgctgcccatctctgaacagatcagagatcttaaaaggcggcccttttaagaggccagctcggacccaggcaggggtcccggtgcccacgacctcc

SEQ ID NO: 17870 - RNA, 5130 nt, Homo sapiens
  source 1..5130: mol_type = other RNA
tcgcctcctcctctccccctccaaagcaacccattcaaaaaaaacactagggggaaagaggaaaatttccattttctgtcaaaatttatataaggtatggacttcctatctgttcagtttttaaaatattttaattgtaataaaagctttgccctgttttgtataagcaggagttaatttagacaggaggtattacacaaaggagaagcaatgaaaatgagctcatctatattatgtgaggtagttaagtgctgttttccaaattaatacaccaggaactagaggagagacaggatttgcccaagacatctttagatttcagaagcaatcagggaacctcagtccagcaatcaagaaacaaaatatattctcagcactggggtcttgacccgacactcactccctccctgcccatgtgattaaatttgtctttagattaatgggaatcttctaaactttatatatatatatatatatatatatatatatatatatatatatatatatatatatgcattcatcctgaaaactaagaaaaaaaggatattaacatagttaacataacaataacatggtcttgattaatatgctcaggaaatgcaagacactgatagaagcataaaaatacaacccgaattctatcctgcagcaaaaaagtttgctttttctttagcagtttgatcaaaaaaaagaaagaattttatttagatgaatgcctgattataaactatccattaagactatttcaaaggtttccccttctacccaacaataacaaatatgctccaaaatattcccttactaagccagacttctccatggaagagtctcaccttattttcctattgaaaaacccgaggcacagttcttaggagacacccccagtgattcagaagcagacagcaactgcagccctaaatcctaggtccagctttttcttatagaatactttccagagtttacgtagttttcaatttatttaaacacagcattcagtctttatagaaataaaaatggtaacatctcttactacattctgaaaacttaagctgaaaaaaaaacagtgtgccctatatttaattttttcatagaaaactcttcttccaacagtgtttaaaatccaggttaattatatgacataagtaacaagtaatctccatcttctccaggcttctaatcagtttcagaacaggagttttggttaaacctcttccacttgttgctctctcacaaaagctgcaaactcaggatcattggcatacagttccaaaactctcattctctcttgaatttcctctctggaaagctcactgctctcatacatctgtctgatttcttctctgctcagcccaccaatcacgtctccgctagcagagctgtagaagggatgctgaggatagggtccctcatacttctcacatccagccctgtgactttcatacacggggttgtacttcacagcattctcaatagatgagaggctgtcaggctgcctgctggagccactgaagggactctctctttcactcctgtcatggtgtgcttggagagtcctgatgaagaagtagatgatagcagaaaagatgacaagaagtccaaccacggaggcaatagtgatgcctatgatcacgggctcagacacaaattcctcacagtgcttgcctcggtaccaccagttctcacccacccggcacctacaaatggccccgtgcccaggcataatgtcacactttccatcattcaagcagaagtcaggctgtaggtcacagagactctgacagggccgttcttccacactcaggtatccagggaagcatctgcactttgcttctccactccaggggttgaccagacactctgaaaattcattacaggcctgaaacttgcaagggttggcttcatcacctgattccacatcaagagagtatttatcaatagccaagttcatggtattgtaggcagtggtacaaaagtcttccagaatcatgtacaccgcattgttgacgttaggagggacagaattggcaaacttcattcgactgttcaccacaatgctgccatttctgaagttgaggatttctaagttctggaaccccgtgagatttgactggagatagggaaccagcaattctaagaatctttgctccagggctttatactccaaggagtttttattaaacagatcttctgaaaacatcatgttagtcactcggaggctgaagaaaaccaccaaagctcctgaagtctgggtataactcaagtcatctcctccttctgtgggccaagccacactaaccatctctgtggagtgaacacttgttgacatttccacataactaccaaccttgccattttgctcttggacttgctcaggctgatagtaatctgtgcctatccggtccagttctaacgaaatatcctgtacacccataattacttcatcctctagcagggtggagattgtggttggaggcaatttggtagactgtgtcacagataaccagagcctgtcagcactctgtggtgtacttgccaatatgtctctggacaatttctctagggaagaagttcttgtccaaactctctctgattctggcaatatagtccacaaagtttgcatatctggctttaccattgaaacctcactgtcaaaccattcatagttggatgactcagtaatttgttccatatcctcccttaggatggcatctgcctgatctgatttatcagtagaggcagagattgctacagatgtcagtataagaggtgctttggtaactgagtaatcatcaacaccaggtacttctgatatgtgcttggggagggttagagacgcagattcagctgcagtatctgcgaagatgggcacagcaggcccactaagaggctcttcctctggaaagtgtgtggatctgtcatcatgttcatattttgagtgcttactaatttggtctgtggaatccattttgtcaactaaaactagtttcttgtcttcaatctcagctggcaaaagtgaatcatcatcttcaagccacggcttggacagtggttcagcgctcttctctgatgaagtctcactccatggccaagtaatcagatctaccttttgcccagaccctgaacctaaaccaccgtcaaatattaactctttttccatggatgcatctggcaggaaagggctcacttttaattggtctttgactttggaggtcaaggagtccaagccaaaaggtatagaagaggtcagatatggtgaagatgttaaggacacatcagagtcttccatggatggtattgtttcttttggcacaggttgagtgaatgaacttgaaggcaatgaatcaatagaaagaaaatcttctgactcttcaacattggctaatccatcttctaccaagtgagatccagaagtcctttcctcagaagccacaggcaagccagtctgaagcactgccggggtgacagaatgaagagtcaagctgctaacctctaaaacctctggggaagagctgaggcccatcttcgagggaaaggctaatttgtgtgtagacactaaatcacccaaaggactttctgaccagagttccctgccagtggctgagggaggaccagagctgaaatcaagtggtggaatactgctggtgatggattcatctgctgagggccatgcagcttgaaaggtattatccagaatagatgacggcgttgcctgaagacttgaactttgggtgttccaaactagatcttcagtttggtgacgcaaaactcctctcacattgataagctgcagggaatcaggatctggattcaaggaagagttccccagcaaaaaattctgctgcaatgtctcagcaatataatctctgaagttactgattgtataaacaacagtgggtttatcatccagttccacaaggccatggttttccaccttgttggagtgaaggctaatgaggtcccaggtggtattgctgatggcctcaccattgaaggtaactgcatagtaaacatctacgccactgtcattttccttgggggacctaaattcaagtacacgaatttccttgtagcctggtaacccagtaaatgcattttcaacctctgaaataaattcttcttcaaggtgctggtggtgaaagctggaggaatcctgtagttcttccctgtactgcttccccaaaaggtggatactgaattctgcaatctgttcacctgctggttttgtggcttcttctatcacattctcaatttcattgctaatactctcctctggcctttccaagctgctctctgaggcaccttcataggcgtccacctctggatgtggaacactgagagtagtgtctcccaatgttgaagtatcaccaacaggaactggagaagacagttcagagctgcttacagtttcctttgcataagtcagtttcttcatgattaagcttctatgttccacagattcactaaaatttgtgcccatttcaaatatacttgtgactccatcctcacacaaattcatccagtaatgatattcctcacgcccaggaagtcgatcccaaaaagtcctgaaggcttcccagacagcttcctgacacactcggactttaaaatacttcacatgatttgccacagcctctgcaacactttcatctgggcagattttcactccattaggaaacagaatagatctccgccttctgattaaccactgtctttcagtttctctgcggtccagaggctgtttctttttggtagctagagaaaggtctgttgattcttcaggcaggagaaaagaaactgcactcttgggttcttggatctcctctatagataagtaggtttgtgctgttaatgatggaaagtctccttctatcaggacaaatatcaaaatacccagagaaatcttcccaaaaagaggaaacataatcatttgggccaaaaccaaaggaatgaggagaggacagaatccttaattgagtgtccaaatccttgaaacttccaataacaaagagttataggaaagacctaacatttaaaagtctatgtttgagaatgaacaaccacttcaaaaccattataaattagcggaaagaaaaatggttgtcctttcaaagtagctctcacttcttttct

SEQ ID NO: 17871 - RNA, 1296 nt, Homo sapiens
  source 1..1296: mol_type = other RNA
tcgcctcctcctctcccggcccagaccagccccttctgcttatcttcacggatcataatcacgtcttccaggaaggcagtgaggctctattctccccagaagcaccccatggaaaactgcaccgtcattgcagtgagccatctaatacaacagaggatgagtctggggatgataccctgagagaagggatgcaaatcaatactgcactttgggtgccaaggaggcagagggctgtgccatggtgcatgtcagccagctcagtttctctctgagggcctactcagtactgctttgagaaggactttcccaatttatgaaaaaaaattcatcttgacccacaaaggcagtgtcaacagaacctcccaccatccgcccacacttaggaccaacctcgctgcctactgggactgggtttatttgatctcatcatttggatgagagaacagaaatttctgtgtgaagccaattttagttcctctcccacctttctccaggaaatgtgattctcaggactgccaagagcaactgaaaggaaaagtacagagggaaagagacacagaaagacagagacatggaaagggagacagaaaaaggaacacaaatagagagacagagagagatagagacagaagaaagagaaacagaggcaaagggttagtgagagagacagaaacatgcagaggtcactgccttcctttacagcctgttgggctctgcgcttgtgggttcattcttgctgtagccagcatcacagagtggccctcggtgcctcgctgggtggggcagagccaggcccgagcaccacatccctcaccactgaggcccccaggcgtgcttttcaggtcggaagagtcgtcgtcaaataagtgcctcctgatcatgcagatcttcagggccaggaagccagcagatatggcgacacccacagcagtcccgatgagggcgtacttgaaatcaatttcagccccaggggtcttgcctgttgccagcacttgagctcctcctacatccaggaggaagaggatcctcagcatgctgacccccaagttcatgctggcgctctgctcttggctcctggctcctggctgctggcagcgcaggcacaatgagccatgtgacccaaggctctggggacaggacaagacccacgtgactgatggggaaggaaaccactgtcacagccaggaggctgttcagttcctctcagcctctctgaagacagggctgaaggaagcccctgtcattctggactccaccagaagctggctgtgattagacccattgtacatgctgggg

SEQ ID NO: 17872 - RNA, 522 nt, Homo sapiens
  source 1..522: mol_type = other RNA
tcgcctcctcctctcccggtccccagagaacaacgcgagacagaaagtggcccctcagcatcagcgaaaccgtgcgcacagacacggggcccagccgggacgccccagacccctcggtcgcggcagacgggctgcccgcggcccccgaaagtctctcggataacacaggcgcctaggcgccgcctttgttcctccccagcgctctgctgcgccctgggcgcagtactggcccggttcctgcacccgcactgcggcggcggcggggcttgaggatttggggctaagctaaacctcacaaaacataccaccaccctcgcccagagagcttacgaaagaaaagagcttaaaggttttccaagtagagcctgggggcgctgactccacccaacggccacaaagagccgaagccgattctcaccatggttgctgcttcgcgactgccgagctgatggcggagacgaagaggagaggttgttgcttcttacagcgcgactcttaggcggtcgatgtaagagaacctgc

SEQ ID NO: 17873 - RNA, 2311 nt, Homo sapiens
  source 1..2311: mol_type = other RNA
tcgcctcctcctctcccttctctctcctgtctgctcaggttctcttctgtgctgcagtggacatgccaggctcctttgaccctcctgatgaatgcacacactgttgtcttcgcctgaatgctcctctccttgctcaccctcatccacctgccaacattttatttcaggtgtaactctactgctgcctcctggaaggttcctcttcctcagacttatctcttgtgtagatactctagggtgcacccatggctttaggatattccctaagtactttttgcctctcagattacgctcgattataattgattatttgcatttcagattccaccgctctactgtgaacatctcaaaaactagaattatgactcatccactttcctatgcccaaggcaccagcatatagtaggtgttcaataatatttgtaaaataaatgaagtctcagttctgccatttactagctattactttgagcaactcccttaacctcttaagcttcattttcttcctctgtaagtggacagaaactaatggttatcgagtacttctatgcatcgggccctatattgtatgtctttacatatgttatttaattttcaccacaaacctcggaaatagaaatgattcctcatcctataggtaagaaaagggagagaaatgaagcaaattgtccatggtttggtagtcagaggcagaatctgaacttaagtctgtctgattccacagctctttccactacaccaagctgccaataaaatggagaagaagactatcgacctcactgggattaaatgtgataatgtatgtgaaagcactttgtaaactgttaaacgccatcaaaatgtgagatgatgttattgtcattaagatctgccatggtctgcatatcatggtcagaattttcagtaactgatatcggaaatcattcagttgtagctggctgcaagggcctatgggaatcagacacctctctggggctatttccgcagcatacttgctcccctgcttgtagatgcaaataaatagcaatgcaacaggaggcccagtggagcgcaaggatgcagcatgcccaaggagaaatgatgatgagtatgcttgtcagttacaggttacagcaccctgtgaatgtcctggtgacaccattatgttttagaatcttcaggctgctttgttgtcgcaacatcccatttagaatcttggcgtgtgctgagggtcgcgaactgcactgcttttagctgctgccaccagtttgtgaatcatcctgtttacaatctttcagatgctatctgggtggcgcgcctgatgctcttgactctctgttccagcactctacactggtccaagctgtttccaaacacactggagacagtaaacatttagggttctctggtcttcttgcctccatctttgatcatttctgttgttttggagagctgaaggcatctctgtgatcctacacatgtttctccacctccctgggcctcccttttctcatctgtagaatctgggagttgggttaataatctccaaaaggctagaattagaagtctatttcttcggggttgttcactccacaatttcacagattgtttccaatcatgcgggcgcagcccgagttgcagagcgttgtggttactgttccttccaccctagtgaggtgggagtcgagaagtccggtgactcaccacaggctaccagccatgtgatggcgcttcatcacgttgtccttctgtgtgcccagcactttgctggtaggtgctcaaataaatgtggatgtccctttcagggggccatctcttctttttcaccttctggccactctttatccatttcctgccgatcatgaacataatgaggggcagtgtgcaggtccgagatgaggcccggcatgcttcattccttcgttgtgagtcagacacattctcccatgcctaaccctgcctatgttctctcccagaactctggacagagagatacaattcagccaattagagcactgcttaattgctagcattttgcaaaccactgccttattggctagaagggcaataatatcaaaaagacctcctggtgacttcacagttgggaaaaatagatgctcctaagtcatcccttctaccctcctctaagtaacaaacacctttctcccctggggaaatttcttctttcatttgctgtaaagtgacttctgctgaagtgtgtgtttttgaagtggaaaattgaaagcacatgattcattccaaaagcaaactgttagttcacagctgagaaatcactttgctattggtccaaagagttgcttctcaggtttga

SEQ ID NO: 17874 - RNA, 556 nt, Homo sapiens
  source 1..556: mol_type = other RNA
tcgcggtttgtgccagatgacgtatctttgctagagcaggttaatgctgcctcaggacattaaatgtgtccactgatcttgcgaatacattcttttccatttctggaagtacctggaaaggtgcaagcaaggtatcccatcatttttctgtcccctttttaacacagtctcttcatcctatgagtatgtcttttacgggttccatctccttaatctgtctccaatcaatctcttcctattgttaggacattcaacttcgattctgagaactgatttagtatcctaatttgtttccagtgctccaggcttgatccccaaccaaaccaattttcacaccagaatgatcttcattttctgctccagccacactccatgctgtctctttcctctggggtttggtgctctctattttgttttcctggtaaatattcttattctctttatctccctactttccgccaacttctctaacagcttatttctattcattcttcagggtttggtatagacatctactcctacgaaaagccttccctgatgcctatgactcagattc

SEQ ID NO: 17875 - RNA, 2116 nt, Homo sapiens
  source 1..2116: mol_type = other RNA
tcggatccgtctgagcttggctggtcggaagtctcatcatctgcttccttcgggttaaacacgtcggccaggtctgagtatgggtgtggcagtccgggtagcaggctcatgccgtgcctctctagggcaatgcatggcgggggcgggcggaagcagttcttcaggcagtagggagagtggaaggtgcagcggcctttgatccagtcgacttcgggggcgtggactcggagccagcggatgcctaggaccacagagaagttcggtgaaggtacgatgtcaaattcgatggactcctggtggttctggtggatacacaccaggggctccgtgtagagccagacaggctcgttgccaatcagcgagccgtccacggattggaccggctgtgggtacggcttctcgtagagctcgacgtagtgctcttgggcgaacttctcatccatgaagttgccgtcagctcccgaatccaccagggcctggaccgcgacgctgtggtaggggttcactctcaccatgagcagcaggaagaggtgggcgcgattgatgtccggatggacttcgctgggcaaccagctgctgaccatccacctctctggagcaggtgagtcgatccaggtcaggttccgggggcgggcctcggggggcagcctgagcatagctcttctctctgccagcttctcttctatttgcaggatgagcacaatcagactgtctagggaatccggctgagggacccggaatagatagtgcctgatctcctcgttgagcccctggcacaagtgggcctgcaggacttcatctggccagcccaagatgggtaccaggctctggaactcatcgatgtactcagtggcagagcggccgccctgcctgatggtgaacatggcctcttctgccacacgcagtgcctggcggtactcaaacacttcggacatggcctccaggaaggctgggaagtctccgatcagggggctgttttcctgcagtagagctttggcccattctaatgccaagccggacaggtgattgatgacatagccaactctcagacggtcgttatagaacattcttgggtagctctgtaaggtcagttggcagagtacgatgaactcgtggaattctctgcgatcgccagagaagtgctttggggcgggcagttggcctgcattgatccctttgatcaagatctcttctgctactctctgttgctctttgaggtcttgcattcggaagtacagcgagatgatggacctcaccatggccataagttctgcggttgagtgctcggtctggttttgctcttgaggagtctcctcccttcccgattccttcaggtcagtgtgagcctcttgttcttctcgggctcccgatgggttgactgatgcttctttcatcctatcagatgctccactgagtggatccccccttgcctggtgtgaaccgttgcatgactcctccaggtcttggagtaggtcattgggtggatcctctatttccttacgtgggccactggatggctcctccatgtcttggagtagatcagtgggcagctcttccatttcctggagtgggccactggggggctccttcttttcctgggctgggccgctggctggccctgcctctccccgcactccactgcccgacgtcgcctcggtggtgttggatgagccctcggaggactccatttgttttgatgatggattcttatgctccatcatcgtctcaaatgagtcttcagagggttctatcatttcgtcggatggaaaggagtgtattctgaagattggtaaggttgtgatggcgtccagtcagtagctgggaccgtggagatcagaaccttggctgcaagcgttcaagtggatctcctcccgtcctgtgccactcgatcctcgctgcttgcttccccgggcccagtcccaagcgtgaggctggggatgaagtgatgccggtggcttagtgatgccggtggcttcctgtcctcgaagctcagtcggtcgtctctcagctggtgtgaggctgggccaggatggaaccccagactctccgaggctccccaccacaccctgctgctgaaggctgctcagcgaggctgtgccgagtgctgggggggtgt

SEQ ID NO: 17876 - RNA, 11498 nt, Homo sapiens
  source 1..11498: mol_type = other RNA
tcggcctggggaggaggaaggggagggaggatggaaacataccgtacacaaaatactcaattcctagttttctctttaaaaatggctagaaaaaattcatcaaaatgcagcactttaatcaattatttacaatttctatgttacaatgaaaaaatgtacatcttatagaacatatttcataaaactgctccactggaaacaactagatcaaaacagcaaaccttccatttaatatccacaaagttggattatttttcctttttgaagtagattcgccacaatcaaatttgaatacagagaattttgaagtttaagcatcaaacaacaaagtaaaagtccccaagatacaacaaagatctaggcaagtcttgttcctgtcccactcccaccccacccctaatgaaacttaaaaggtattcccatttcaattatggcctgtatcattcttggcagtttgggaagagaacttttggcttccattggtaactcaacataaatgttgcatagaatttatatatttcaaaattggcctaactgtagaaaaggcaaaatggaagcatttccgatagagccctaaatgagtacaaagtcactttgtaaaaggtgagtgacactaaagtaaaaatatgaccaaaataagaaatgtgcatattagacaaccctgcttcccgaaactttaggaaggacacggagttgtgagtcacacaagggctatgctacttgaagtcaatgttcaccaatcaggcagcactaggtacagaagtcttggttctgaacctggacccaggagggaagtctgtgggaaaggggagaagagaatgacaagagaggatgtcatattaaaaaaaggtttcaaacaatattggcaggtgtctactcacaaggtgattggaaaactgcccacgaggagaagtcaactttacctcctcccaaattcacagtacgcgagtgtagtagggtcattgctgggagataaattgtctgaggagggccacccttcaggtttaccagaaatcttagggtttggcccccctggtcacaggctaaatatatggtttaaaagttttattaaaaagaaaaacagaacaagacacactcacacccagatgactaatgaaggctaagcagaatagtctgagtttgctgagactaaagcagggatagtgttgaaaagttttcctttcactagtgggacacattccccttttcttttcaaagaggaagaacatggtgtcatccaatgtgaagtgagcagtttcgggtcaaactcttatggtaagaaactaaaaaaagatgccaagagacaaaccttcagaaatagaagaaatgcaaaagatggaataaaaaccctgatcattaaaacagagacaccttcactggtgtccaataaggattctctttacaaaacagaaacaaacaactcaaaaatttaccatactttgtaatgaaaataccagtatgttgaagacacagcagactgggtttctattagaacaagtatcagcaaggtcatgtagacttgtagaaacttttgccttctcctgcaccagacagatcattgtccagttgggttgtcagctggagaccgaaaagaacctaaaaaatggatctttttttttttctttttcccatggtcacgcatccacacaaatgagtcttttggatgagaaaagtcacagcaacttgagttctcctaatgaacagatgactttttagccctgtttgtttcaatggggaaaacaatgacaaaaaaaacaaaccccaggcaggcacgacacttatgtaaaatgaacacagttagtacaaaaccagtaaggcatcactttgggaaggtcagcaccgaagaggtcaggcaaggctcgtccagacggggcttctgggagggagtgaccctcacccttattgagctgcgtcatgttggttctgaggaaagtgcaagtcttttgcagggtgaccgcatcaccccaccggaagctggggcggggacgctggaggtgttggtgtgtgttctaaaccctcaaggacgagaagggaaggcaaggtccatggctcacccacatgtcgaggaccaggtcctcatccattttaaaggacacagatacccccagccctagcaggaggaggcgagtgtgtaggactgtgaggatggacaactaaaaaccaaaactgagcaggaccaaaccaaaactcaactcctgcggttcttactttcaccaaaggattgattctgaccaagaggggaagggggaaaaaaaaatcttcaaaaatcaatgcatcagaaaggaagaaactcaacctcattttcaaaaggtaacctgttctccaaagtagaacaagtctcactatacacagtgtttgcagaaaaaaaaaaaaaaaaacctgattcattcatatatcagaaggaaagagacacatgctgttctgcactgacagccacatccactcgctcacactctcactccgtcactcactctcacggatattaatcagaggctgatggacctgaatggggtggtttgattggaacaggcaaaatacctctcgggtaaggaaagcaccatttaaaaaacatgaaagcacggtttatttgctcctaaggtttccctgtgtcgtagctctgtagtgcgttgaacgtgaccaaagcaagcaccctggttagcaccagttctccctgtggccggctgtgtgggagggtgggtggcacggctctgagacccagtctggagggtctgtgctgaggggaagccgtgcttctctgtgtttccgactttgctccagtctcttctgtctctgggaagctcatggcaggatgctgtttggtttcagagcttcatgtgggttctctttttttttttctctctgtctctcttttcatttcaacggcgatgatcctttcccgagaagtatcttcagtgtcttagggaggtcacagcaacaaggcaaaacaataattaaagtacaacagaaggtagtgcagttctcgctgtggaaggaagcggtccgcaggcagctggcccgggatgcctgcacccaggtcgaggctgaaggacggggggtctcggtgttcccgcagctctaaggctgtggctgggggctggctcaggaagtcatcttcagggtgatgtgggggatgcaggtggaatgcggtgaggagaagaggagggcgctgggctccgggcccctgtcacagagtggactccaaagaggagtccaagatgtcatcgtgatggctgttgctgttggagtcgctgtcatagctctgggggctggagtagttggctgcctcctgcagcctcatcagcatgttcatcagcgggtcaccttcagcatcactggggggcatctgcttgcttgtcgatccctcccgaggcatggagtagccgtcgaagccgacatcctcaggccgtaactgcagcaggggaggccactcgtgctgttgtgggctggctgcccatggatatgtgtccatcacccacttggcaggatcctcccagggggcgcgccttccatagagctggagtccttctctgacggcttccaggagataggggataatggaatagttccacaagtcggtgaaccacactctcgagccgtccacatcgatggggcatgacaggaagagccgggggccgatggtgacgtccgaggaactgtgagcctccaggaagcggttgaggtgatgccagaccttgggaatccagtcaatgatttttaccagctccatattgcgcacccgcccactgatctctgtttccatgagcttcctcctcaggaatcggccaaggaaacccttcacaggctccgtgtggttggcacaaagcacccatctgaagttatggtgaagctgcaggttgggagtcgaagaggtagcctggttcattgtgccaattatgtaagggcatttgtggtacttgcagttgagcagcccattgaagatctctcccagagagctcacgtggtgtaggttgtccaggatgatgacgaggggcatgtccacagcattgttctcactgttgcactggtcagcaaggttggacaggtactggcgcaattccttgctggacttatggtccacgttaaaggtggcgataaccccgtctgtcaactcccgtccctctcgaagcactatatactcagacagccggttggccaggtaggttttcccagtgccgctggggccagagagaatgatccgacggtgctctatcaggagggagacgtagcgctgcaggatgggcttgggaatcaaggactcaaacaccagtgagtccaggctgttttctgcgagccctttcacagtcactgagatggtcgtgttctctccaaccagatagccacaaggaagcagctccggtgtttcggaagtgttgctgcgcttgatttctccaatgctgtagccaagaacgctgtctgaattcagccctagctgactcactgggtcgacatgaatgatgtattctttgaacagccgtctaaccaccccatcgagcacatcccacttcgtcttgccactaactccaatgcagccaataagaaagagatgtggtctggaatcctccttccacttcatttcctcctgaaagctgacaactatcttaacatgcctgcctccttccttccgagccgagcattcaccagtgtcatccagcaacatgtccaggctggttgactcagtgaggttcaagctgtgctgggagaggcccatggactgcctcggggaggcagagatggacacttgggaaggagcccggctgcagccactgccttgagactctgacttcagccgatcattctcagctttcagcttctctatttcactctgcatcctgttcatggcctcccggagctggtccagctggtgggcagaactgagagcttctaagcggatatccgtcagcttcatctccttgtctcttaactcatttcggagctgcatgacggtctcagcttcactatccatgcattctgaaattagagagttggagtgagaattcctcagcagtggggtggaacctgtggacccattgtgcggtaactttggtgaggaaggcaaagaagaatccgtcatctcctcaatatctgaatgagaggacgcagattttggggacttcttcttcccgaaagcttgcttgaaggagctgcgtaaccagttcttccgcttcttcttctttgagtcactctctatgttgctgcccacgctggagtggctggtggcactgttgatgctggagacgctgtctgaggagtgctgcctgcggatgcggaggtctgcagactgggcagtgccgtttcctttgcagttgagctcaggtgtgttaattactccattaatggcagcctgggcagctgcgttctgtttctttagcagctcaatggtttttcttaactcattcagttctgagtccttctgctcagctgtcatggtcagactctggagcctgattgtcatgttaccaagactctgttcaaaggctgccacaaggtgagcatttgctgtcagctgggtggtcaaagctgaaactttctcctgggaggcatccagttcccgccgcagcttgcgaatctctgactggcatttttcttctggtgtagaataaactgacgatgtgctggaaaccaaggagagtgaggatccatgaactaactcataccttgcgtgatggaacaaaggaagagagaaatgaagtgagctgtgaagacggctgacaaagttgtccacagaacttttctcccatgattcttcttcaaacccatcccggaatgagcctgaacggctcatggttctgctcttctcatccagggacatggagctattccggaagcggctgtcagtgtatggatcatactgcccatcagcattggagaggctgtgagtcctcagcatggtcgggttggacaagctcatctgggtgacagtggtgggactcgcaagctgggaaaagttgaatcttgttccggagggagaagtcacgctggagccagaggaaaagggggaattggcagcggtgtcctgaaggcctcctgcagaatgggaccgtaaccattcttttgcatcttcttgcgtgcgaagctgggaggtgggagtatacctgagtcctttcttaggcaaagtgttcctatcaaggtgcgggtcactgtcctgtttcctgggcagagtacttctgcagaacttagggctagcagcaggggaagagagagggctttctgacagtgtggtcttcacactgttagttctgacaaagggagtcaaggagtcgtccttggaggaggcgatgaggccagtggaagaattgtggctggggacccctccactgctgagggagatgtcgatggactcacagctggtgtggaggctgctgacagactgaaagcccaggccatccttgctaactgcggaggagctgctggcgttggtgccccaggtgaggctgttggaaggggccgagtgggctgagctggggctggaggctagcggagactggttgaggtccacattcttgctgtagagaggactgctgctcccactgctcaggacgccactgcctgacggggagtctaggttaccttgctgagtcatggtggcatgaggattggagatgaccaccgaatttttcatgttttcagctgtggcgatgggcacttgcttggtaggcttcccaccaaagagtctgcggagtgtgggagaggccacatctgggtacttggctccaggctggagactggtctgagccggactggacacaggctgggctgccggattcactttcaccgagttacaggaagccacactctcgttgtctgatgagatgcctttctccttgtctgtttggttgaccagacctggtagagagctgcctagggctgttttggaaggctccctcagtttgggcactggcaggcctgcggacttgctgctaatgttggaatctatgctgctggtgctagacctgttcccagccccgttccggctgttggacttactgggcctcggcaaactccggtactgaaggtttgtccgggagcttagggctagatacccgtcatcctgattctgagccccatccatacttgacttccgaccagcagaccgactgacgagtgcagatgactttgggattttgcccagtgtggctgacctgctggtgacagtcaccccgctggctgtgatcatggccaggccggcggcggaaccactctgcttcttgaacccaaagctgttggcattggcagtaggtgtcctagagctgctggggaggggctttttggattcgtcaccactgctccggcctgcatctgatggggagcgcttcacctgggaggctttaggagaaagccttcctttctcagacacctttgcgtcgtctgtttttccagttcctggggtcttcagtgcgcctgccggggctgaaggcttcgtccttggcatggtgatgcccacctgagctgtcatgcctcgccgccatgagcctgtctgggagatgacaggattcttcttgcccgacgtgcttttgtcggactcgtcagacacatcagaaggattccgcctccacttggaacctggctccatttttatgccgctgtctgagcctccgtctgatttcttgacatcatcaccagaccacagggaattcctctccacctgtgagtgcttctcagcatcagtctgcacatccaggttttttcgagaggaggcaggtgtgttggcataagagctgatggaggagctggtgttgatgtcatcagtgctgaggttgtctatggtgtcgctgatgccgctgctgacggagctgctgtcgtcccagctgtcagcgtctccgaggcccagggaggtatttcgttgcagggtctcccgtaccacagccatcccatcagggagccggttcaggcgacgggtatagaggccaagtccaccatcagtcatgtatccgcttgtaatgtcatcggtccggatgttcttgctcagaacatccccgtcgctcatgtagccgggggcatccatgctgatgccttccaggtccatctcatctcctgccttgtctgagacgtccacatggcagacactactgccccgggaggccagctgccttctcagaggggcggagtacacatagcgacctgactcagtgttgatgaacctgctggcgttggctcgagggggatacccattgcccattgagggggcgtctcctgcttggagccgagggctggactggcccagtctccaggacagaggtgtgggcctccctgtcaagctgagtatgctacggccactcatctccgtggtgacattggtgtcaaacgtggtttccaatgtgctgtgtgtaacctgagttccccttaaactggacatggtttcctccaaattctgccgcagatcagcgatgttcttcactgtccgcagccgccgagcctcaggatcttccccagtgagttcttccagagcaggctgtccagtcttggtgaagtggctgggctccacgctcacacctgttgagcttgactcggcagtaacattcccttcagtgtccgtctgagacctgtacaggaaaggtgcaaccgtggcagtgttgggatggttgtattgctgctggggctgaggtagctgaacactgacggtattgcttcctgtggtctgggtggtcccgacagacccactgacagtctggctgctgatgctgtggttcagggtggtccctcctgggccttttccttctgaggacgccaggctggaagaggaactggagtgtctgccgtccagctggggcttctgctgggggagtcctgagctcagcttcccactccggctccgctccccttccttggaaggcgctggggcacttggggatttcccgggcatgcttttcattcctggttttggtattccactgtgggaaggggccatgggctccttcttggcactgttgagcttcccccctttggggatgaagctggcaatcttggaggacttttttggcatctcgggcacagctgctccactggggtcttcttttggctcctccttgaggtccagcctctccgtcacagaggctctcttggcaaggtccttgcttttctccttatccttctcccgctgttgtttctccttctctttctcattgcctttcagagaactcttcttgttggtcagtgcccggctaaaagtcctctgggcaatgcccttgagtgcaatcttggggctgctggaagcagggcccacggtggtgagcatgcgactggcggcctccagctcctcgctctcttcgaagctgggcagagtctccagccgctcacagcttgtgtcccgggaccccggcccctcacctgcctttgagccccctttactgttgaaaagtttcagcttttccagcatggacttctgattgttgggggccggcttcatggcttcaggtgtgggcctgggggcctcaggcccaggaggcttgaccgagagcatggataccgtggcactgtgcttcacgctgagggatttgctgcgccaaggcttggtggctgcaccgggctgcgggatggccgaggaggtactgcaattagtaggggtggagctgctgccgctctccaaggaagcaggtgcattgtcactcattccggggtgggaggaggctgaacttgccaaaggctctttctcgtggctgcttggcggtgggggtggggaggtgactggtttggatttatcatagttgttaaagctctggctgcgtcggttgttagcagtagttgaccctccgcgtgttttggcctcgctgcctgcagcggataccctcgcggtaggacctggaagtctagagatctttttctgacccagagtgaagcggatgattttgctttgagatgagtccttggatgatgcactggactgcatttcagcttgtgcttttgactgctgatgtggcgctggctggtgaggctggcacggggcttggggagtgactggcacctgctgctgaggggtgccagcctggcactgggagggggccccggccacctgggatacggcgggcggcagaggtgaggagaggtgctgcttctggggctgctgctgctgctgcttgtatcgggagaggctgaagaagaggcctagaatggccttgaggtttccattcctgatctcttctgcagacagcccctggatgtttattcccttagctgccaggaaattcaagcaggcatctatgttttcaatcatttgggatctgttcttcggacagccattgatgtcttcaatcttttcatttgccacaacctggataatctgggccaggaggacgccatctgtcacatcttgctggagatccctgatgagacgcttgtggccggatttggctaggtaatgattggcccagtctgtgtagatctgggtatcgaacccgttttccaccgagccgctcttccgcagcgggagcccctcccccgctggctcctgcagcccctgcagcacctgcgatttcagggggatctggctaggataggtggtcttgctcacctccaccttgcttcccaacttcaggtagcagggctgggggcccgcccgggccgggggcacgtgcaggatgggcgcggcgctgtgcacgggtttgggcagtcccgacttcattttggaggcgaccaggatggccggcatcttctcccggggcttgggctttcccagcacgtccctggcagcggcggcgggggcgaccgctaaaggcagcgcgggtagcagagcaggcgccgggccttagcccacgaggcgcccaccaccagcggctaaaaaaaaaatccccaggtcggggaactcgaagcaatcgggcgagcgcgcctttggggtgccgggatgggaatgggggactggccacggcgctcagcgggtcccacctggacggatgctgccgccgggtctcacacctctcctgggtggcctttcaagagctctgggcgctcaggggctgccgcctcttgcaaatttcctcctgggaaacagaggcttggacgcccatattaacttgtcactgcatctccgaagtgaggaggcccctttggaagagacagaggcggcggcgacccacgagtcccgttccggaggctacgggtctgagccggcgagagaaagagcgagcagccaaggaaggaaaggagacagcagcgaaggaaggagagaagaagggcgcaagggtcccaagacgtctccaccgagaggcagctgccaccctgctcgcgagcaccgcagtgtcacccgcgacgcagcagaggtgcggcaagagcccccgaaaggtctctcttggggtgacagtcaccgctgcccagaaggcccccggactgagagcaccttagcgcctgcgggtctgcacatgctccgtgagctagatagaggcaaggctgtggccgtggggcgcgggcgccgggacgcgcggctggcgggccgggcagggctgcgctcgggagcggccgccgcgcttcccgggaaggctgcgctggctgcggggctcagcgcaggggag

SEQ ID NO: 17877 - RNA, 11399 nt, Homo sapiens
  source 1..11399: mol_type = other RNA
tcggcctggggaggaggaaggggagggaggatggaaacataccgtacacaaaatactcaattcctagttttctctttaaaaatggctagaaaaaattcatcaaaatgcagcactttaatcaattatttacaatttctatgttacaatgaaaaaatgtacatcttatagaacatatttcataaaactgctccactggaaacaactagatcaaaacagcaaaccttccatttaatatccacaaagttggattatttttcctttttgaagtagattcgccacaatcaaatttgaatacagagaattttgaagtttaagcatcaaacaacaaagtaaaagtccccaagatacaacaaagatctaggcaagtcttgttcctgtcccactcccaccccacccctaatgaaacttaaaaggtattcccatttcaattatggcctgtatcattcttggcagtttgggaagagaacttttggcttccattggtaactcaacataaatgttgcatagaatttatatatttcaaaattggcctaactgtagaaaaggcaaaatggaagcatttccgatagagccctaaatgagtacaaagtcactttgtaaaaggtgagtgacactaaagtaaaaatatgaccaaaataagaaatgtgcatattagacaaccctgcttcccgaaactttaggaaggacacggagttgtgagtcacacaagggctatgctacttgaagtcaatgttcaccaatcaggcagcactaggtacagaagtcttggttctgaacctggacccaggagggaagtctgtgggaaaggggagaagagaatgacaagagaggatgtcatattaaaaaaaggtttcaaacaatattggcaggtgtctactcacaaggtgattggaaaactgcccacgaggagaagtcaactttacctcctcccaaattcacagtacgcgagtgtagtagggtcattgctgggagataaattgtctgaggagggccacccttcaggtttaccagaaatcttagggtttggcccccctggtcacaggctaaatatatggtttaaaagttttattaaaaagaaaaacagaacaagacacactcacacccagatgactaatgaaggctaagcagaatagtctgagtttgctgagactaaagcagggatagtgttgaaaagttttcctttcactagtgggacacattccccttttcttttcaaagaggaagaacatggtgtcatccaatgtgaagtgagcagtttcgggtcaaactcttatggtaagaaactaaaaaaagatgccaagagacaaaccttcagaaatagaagaaatgcaaaagatggaataaaaaccctgatcattaaaacagagacaccttcactggtgtccaataaggattctctttacaaaacagaaacaaacaactcaaaaatttaccatactttgtaatgaaaataccagtatgttgaagacacagcagactgggtttctattagaacaagtatcagcaaggtcatgtagacttgtagaaacttttgccttctcctgcaccagacagatcattgtccagttgggttgtcagctggagaccgaaaagaacctaaaaaatggatctttttttttttctttttcccatggtcacgcatccacacaaatgagtcttttggatgagaaaagtcacagcaacttgagttctcctaatgaacagatgactttttagccctgtttgtttcaatggggaaaacaatgacaaaaaaaacaaaccccaggcaggcacgacacttatgtaaaatgaacacagttagtacaaaaccagtaaggcatcactttgggaaggtcagcaccgaagaggtcaggcaaggctcgtccagacggggcttctgggagggagtgaccctcacccttattgagctgcgtcatgttggttctgaggaaagtgcaagtcttttgcagggtgaccgcatcaccccaccggaagctggggcggggacgctggaggtgttggtgtgtgttctaaaccctcaaggacgagaagggaaggcaaggtccatggctcacccacatgtcgaggaccaggtcctcatccattttaaaggacacagatacccccagccctagcaggaggaggcgagtgtgtaggactgtgaggatggacaactaaaaaccaaaactgagcaggaccaaaccaaaactcaactcctgcggttcttactttcaccaaaggattgattctgaccaagaggggaagggggaaaaaaaaatcttcaaaaatcaatgcatcagaaaggaagaaactcaacctcattttcaaaaggtaacctgttctccaaagtagaacaagtctcactatacacagtgtttgcagaaaaaaaaaaaaaaaaacctgattcattcatatatcagaaggaaagagacacatgctgttctgcactgacagccacatccactcgctcacactctcactccgtcactcactctcacggatattaatcagaggctgatggacctgaatggggtggtttgattggaacaggcaaaatacctctcgggtaaggaaagcaccatttaaaaaacatgaaagcacggtttatttgctcctaaggtttccctgtgtcgtagctctgtagtgcgttgaacgtgaccaaagcaagcaccctggttagcaccagttctccctgtggccggctgtgtgggagggtgggtggcacggctctgagacccagtctggagggtctgtgctgaggggaagccgtgcttctctgtgtttccgactttgctccagtctcttctgtctctgggaagctcatggcaggatgctgtttggtttcagagcttcatgtgggttctctttttttttttctctctgtctctcttttcatttcaacggcgatgatcctttcccgagaagtatcttcagtgtcttagggaggtcacagcaacaaggcaaaacaataattaaagtacaacagaaggtagtgcagttctcgctgtggaaggaagcggtccgcaggcagctggcccgggatgcctgcacccaggtcgaggctgaaggacggggggtctcggtgttcccgcagctctaaggctgtggctgggggctggctcaggaagtcatcttcagggtgatgtgggggatgcaggtggaatgcggtgaggagaagaggagggcgctgggctccgggcccctgtcacagagtggactccaaagaggagtccaagatgtcatcgtgatggctgttgctgttggagtcgctgtcatagctctgggggctggagtagttggctgcctcctgcagcctcatcagcatgttcatcagcgggtcaccttcagcatcactggggggcatctgcttgcttgtcgatccctcccgaggcatggagtagccgtcgaagccgacatcctcaggccgtaactgcagcaggggaggccactcgtgctgttgtgggctggctgcccatggatatgtgtccatcacccacttggcaggatcctcccagggggcgcgccttccatagagctggagtccttctctgacggcttccaggagataggggataatggaatagttccacaagtcggtgaaccacactctcgagccgtccacatcgatggggcatgacaggaagagccgggggccgatggtgacgtccgaggaactgtgagcctccaggaagcggttgaggtgatgccagaccttgggaatccagtcaatgatttttaccagctccatattgcgcacccgcccactgatctctgtttccatgagcttcctcctcaggaatcggccaaggaaacccttcacaggctccgtgtggttggcacaaagcacccatctgaagttatggtgaagctgcaggttgggagtcgaagaggtagcctggttcattgtgccaattatgtaagggcatttgtggtacttgcagttgagcagcccattgaagatctctcccagagagctcacgtggtgtaggttgtccaggatgatgacgaggggcatgtccacagcattgttctcactgttgcactggtcagcaaggttggacaggtactggcgcaattccttgctggacttatggtccacgttaaaggtggcgataaccccgtctgtcaactcccgtccctctcgaagcactatatactcagacagccggttggccaggtaggttttcccagtgccgctggggccagagagaatgatccgacggtgctctatcaggagggagacgtagcgctgcaggatgggcttgggaatcaaggactcaaacaccagtgagtccaggctgttttctgcgagccctttcacagtcactgagatggtcgtgttctctccaaccagatagccacaaggaagcagctccggtgtttcggaagtgttgctgcgcttgatttctccaatgctgtagccaagaacgctgtctgaattcagccctagctgactcactgggtcgacatgaatgatgtattctttgaacagccgtctaaccaccccatcgagcacatcccacttcgtcttgccactaactccaatgcagccaataagaaagagatgtggtctggaatcctccttccacttcatttcctcctgaaagctgacaactatcttaacatgcctgcctccttccttccgagccgagcattcaccagtgtcatccagcaacatgtccaggctggttgactcagtgaggttcaagctgtgctgggagaggcccatggactgcctcggggaggcagagatggacacttgggaaggagcccggctgcagccactgccttgagactctgacttcagccgatcattctcagctttcagcttctctatttcactctgcatcctgttcatggcctcccggagctggtccagctggtgggcagaactgagagcttctaagcggatatccgtcagcttcatctccttgtctcttaactcatttcggagctgcatgacggtctcagcttcactatccatgcattctgaaattagagagttggagtgagaattcctcagcagtggggtggaacctgtggacccattgtgcggtaactttggtgaggaaggcaaagaagaatccgtcatctcctcaatatctgaatgagaggacgcagattttggggacttcttcttcccgaaagcttgcttgaaggagctgcgtaaccagttcttccgcttcttcttctttgagtcactctctatgttgctgcccacgctggagtggctggtggcactgttgatgctggagacgctgtctgaggagtgctgcctgcggatgcggaggtctgcagactgggcagtgccgtttcctttgcagttgagctcaggtgtgttaattactccattaatggcagcctgggcagctgcgttctgtttctttagcagctcaatggtttttcttaactcattcagttctgagtccttctgctcagctgtcatggtcagactctggagcctgattgtcatgttaccaagactctgttcaaaggctgccacaaggtgagcatttgctgtcagctgggtggtcaaagctgaaactttctcctgggaggcatccagttcccgccgcagcttgcgaatctctgactggcatttttcttctggtgtagaataaactgacgatgtgctggaaaccaaggagagtgaggatccatgaacttcttcaaacccatcccggaatgagcctgaacggctcatggttctgctcttctcatccagggacatggagctattccggaagcggctgtcagtgtatggatcatactgcccatcagcattggagaggctgtgagtcctcagcatggtcgggttggacaagctcatctgggtgacagtggtgggactcgcaagctgggaaaagttgaatcttgttccggagggagaagtcacgctggagccagaggaaaagggggaattggcagcggtgtcctgaaggcctcctgcagaatgggaccgtaaccattcttttgcatcttcttgcgtgcgaagctgggaggtgggagtatacctgagtcctttcttaggcaaagtgttcctatcaaggtgcgggtcactgtcctgtttcctgggcagagtacttctgcagaacttagggctagcagcaggggaagagagagggctttctgacagtgtggtcttcacactgttagttctgacaaagggagtcaaggagtcgtccttggaggaggcgatgaggccagtggaagaattgtggctggggacccctccactgctgagggagatgtcgatggactcacagctggtgtggaggctgctgacagactgaaagcccaggccatccttgctaactgcggaggagctgctggcgttggtgccccaggtgaggctgttggaaggggccgagtgggctgagctggggctggaggctagcggagactggttgaggtccacattcttgctgtagagaggactgctgctcccactgctcaggacgccactgcctgacggggagtctaggttaccttgctgagtcatggtggcatgaggattggagatgaccaccgaatttttcatgttttcagctgtggcgatgggcacttgcttggtaggcttcccaccaaagagtctgcggagtgtgggagaggccacatctgggtacttggctccaggctggagactggtctgagccggactggacacaggctgggctgccggattcactttcaccgagttacaggaagccacactctcgttgtctgatgagatgcctttctccttgtctgtttggttgaccagacctggtagagagctgcctagggctgttttggaaggctccctcagtttgggcactggcaggcctgcggacttgctgctaatgttggaatctatgctgctggtgctagacctgttcccagccccgttccggctgttggacttactgggcctcggcaaactccggtactgaaggtttgtccgggagcttagggctagatacccgtcatcctgattctgagccccatccatacttgacttccgaccagcagaccgactgacgagtgcagatgactttgggattttgcccagtgtggctgacctgctggtgacagtcaccccgctggctgtgatcatggccaggccggcggcggaaccactctgcttcttgaacccaaagctgttggcattggcagtaggtgtcctagagctgctggggaggggctttttggattcgtcaccactgctccggcctgcatctgatggggagcgcttcacctgggaggctttaggagaaagccttcctttctcagacacctttgcgtcgtctgtttttccagttcctggggtcttcagtgcgcctgccggggctgaaggcttcgtccttggcatggtgatgcccacctgagctgtcatgcctcgccgccatgagcctgtctgggagatgacaggattcttcttgcccgacgtgcttttgtcggactcgtcagacacatcagaaggattccgcctccacttggaacctggctccatttttatgccgctgtctgagcctccgtctgatttcttgacatcatcaccagaccacagggaattcctctccacctgtgagtgcttctcagcatcagtctgcacatccaggttttttcgagaggaggcaggtgtgttggcataagagctgatggaggagctggtgttgatgtcatcagtgctgaggttgtctatggtgtcgctgatgccgctgctgacggagctgctgtcgtcccagctgtcagcgtctccgaggcccagggaggtatttcgttgcagggtctcccgtaccacagccatcccatcagggagccggttcaggcgacgggtatagaggccaagtccaccatcagtcatgtatccgcttgtaatgtcatcggtccggatgttcttgctcagaacatccccgtcgctcatgtagccgggggcatccatgctgatgccttccaggtccatctcatctcctgccttgtctgagacgtccacatggcagacactactgccccgggaggccagctgccttctcagaggggcggagtacacatagcgacctgactcagtgttgatgaacctgctggcgttggctcgagggggatacccattgcccattgagggggcgtctcctgcttggagccgagggctggactggcccagtctccaggacagaggtgtgggcctccctgtcaagctgagtatgctacggccactcatctccgtggtgacattggtgtcaaacgtggtttccaatgtgctgtgtgtaacctgagttccccttaaactggacatggtttcctccaaattctgccgcagatcagcgatgttcttcactgtccgcagccgccgagcctcaggatcttccccagtgagttcttccagagcaggctgtccagtcttggtgaagtggctgggctccacgctcacacctgttgagcttgactcggcagtaacattcccttcagtgtccgtctgagacctgtacaggaaaggtgcaaccgtggcagtgttgggatggttgtattgctgctggggctgaggtagctgaacactgacggtattgcttcctgtggtctgggtggtcccgacagacccactgacagtctggctgctgatgctgtggttcagggtggtccctcctgggccttttccttctgaggacgccaggctggaagaggaactggagtgtctgccgtccagctggggcttctgctgggggagtcctgagctcagcttcccactccggctccgctccccttccttggaaggcgctggggcacttggggatttcccgggcatgcttttcattcctggttttggtattccactgtgggaaggggccatgggctccttcttggcactgttgagcttcccccctttggggatgaagctggcaatcttggaggacttttttggcatctcgggcacagctgctccactggggtcttcttttggctcctccttgaggtccagcctctccgtcacagaggctctcttggcaaggtccttgcttttctccttatccttctcccgctgttgtttctccttctctttctcattgcctttcagagaactcttcttgttggtcagtgcccggctaaaagtcctctgggcaatgcccttgagtgcaatcttggggctgctggaagcagggcccacggtggtgagcatgcgactggcggcctccagctcctcgctctcttcgaagctgggcagagtctccagccgctcacagcttgtgtcccgggaccccggcccctcacctgcctttgagccccctttactgttgaaaagtttcagcttttccagcatggacttctgattgttgggggccggcttcatggcttcaggtgtgggcctgggggcctcaggcccaggaggcttgaccgagagcatggataccgtggcactgtgcttcacgctgagggatttgctgcgccaaggcttggtggctgcaccgggctgcgggatggccgaggaggtactgcaattagtaggggtggagctgctgccgctctccaaggaagcaggtgcattgtcactcattccggggtgggaggaggctgaacttgccaaaggctctttctcgtggctgcttggcggtgggggtggggaggtgactggtttggatttatcatagttgttaaagctctggctgcgtcggttgttagcagtagttgaccctccgcgtgttttggcctcgctgcctgcagcggataccctcgcggtaggacctggaagtctagagatctttttctgacccagagtgaagcggatgattttgctttgagatgagtccttggatgatgcactggactgcatttcagcttgtgcttttgactgctgatgtggcgctggctggtgaggctggcacggggcttggggagtgactggcacctgctgctgaggggtgccagcctggcactgggagggggccccggccacctgggatacggcgggcggcagaggtgaggagaggtgctgcttctggggctgctgctgctgctgcttgtatcgggagaggctgaagaagaggcctagaatggccttgaggtttccattcctgatctcttctgcagacagcccctggatgtttattcccttagctgccaggaaattcaagcaggcatctatgttttcaatcatttgggatctgttcttcggacagccattgatgtcttcaatcttttcatttgccacaacctggataatctgggccaggaggacgccatctgtcacatcttgctggagatccctgatgagacgcttgtggccggatttggctaggtaatgattggcccagtctgtgtagatctgggtatcgaacccgttttccaccgagccgctcttccgcagcgggagcccctcccccgctggctcctgcagcccctgcagcacctgcgatttcagggggatctggctaggataggtggtcttgctcacctccaccttgcttcccaacttcaggtagcagggctgggggcccgcccgggccgggggcacgtgcaggatgggcgcggcgctgtgcacgggtttgggcagtcccgacttcattttggaggcgaccaggatggccggcatcttctcccggggcttgggctttcccagcacgtccctggcagcggcggcgggggcgaccgctaaaggcagcgcgggtagcagagcaggcgccgggccttagcccacgaggcgcccaccaccagcggctaaaaaaaaaatccccaggtcggggaactcgaagcaatcgggcgagcgcgcctttggggtgccgggatgggaatgggggactggccacggcgctcagcgggtcccacctggacggatgctgccgccgggtctcacacctctcctgggtggcctttcaagagctctgggcgctcaggggctgccgcctcttgcaaatttcctcctgggaaacagaggcttggacgcccatattaacttgtcactgcatctccgaagtgaggaggcccctttggaagagacagaggcggcggcgacccacgagtcccgttccggaggctacgggtctgagccggcgagagaaagagcgagcagccaaggaaggaaaggagacagcagcgaaggaaggagagaagaagggcgcaagggtcccaagacgtctccaccgagaggcagctgccaccctgctcgcgagcaccgcagtgtcacccgcgacgcagcagaggtgcggcaagagcccccgaaaggtctctcttggggtgacagtcaccgctgcccagaaggcccccggactgagagcaccttagcgcctgcgggtctgcacatgctccgtgagctagatagaggcaaggctgtggccgtggggcgcgggcgccgggacgcgcggctggcgggccgggcagggctgcgctcgggagcggccgccgcgcttcccgggaaggctgcgctggctgcggggctcagcgcaggggag

SEQ ID NO: 17878 - RNA, 10938 nt, Homo sapiens
  source 1..10938: mol_type = other RNA
tcggcctggggaggaggaaggggagggaggatggaaacataccgtacacaaaatactcaattcctagttttctctttaaaaatggctagaaaaaattcatcaaaatgcagcactttaatcaattatttacaatttctatgttacaatgaaaaaatgtacatcttatagaacatatttcataaaactgctccactggaaacaactagatcaaaacagcaaaccttccatttaatatccacaaagttggattatttttcctttttgaagtagattcgccacaatcaaatttgaatacagagaattttgaagtttaagcatcaaacaacaaagtaaaagtccccaagatacaacaaagatctaggcaagtcttgttcctgtcccactcccaccccacccctaatgaaacttaaaaggtattcccatttcaattatggcctgtatcattcttggcagtttgggaagagaacttttggcttccattggtaactcaacataaatgttgcatagaatttatatatttcaaaattggcctaactgtagaaaaggcaaaatggaagcatttccgatagagccctaaatgagtacaaagtcactttgtaaaaggtgagtgacactaaagtaaaaatatgaccaaaataagaaatgtgcatattagacaaccctgcttcccgaaactttaggaaggacacggagttgtgagtcacacaagggctatgctacttgaagtcaatgttcaccaatcaggcagcactaggtacagaagtcttggttctgaacctggacccaggagggaagtctgtgggaaaggggagaagagaatgacaagagaggatgtcatattaaaaaaaggtttcaaacaatattggcaggtgtctactcacaaggtgattggaaaactgcccacgaggagaagtcaactttacctcctcccaaattcacagtacgcgagtgtagtagggtcattgctgggagataaattgtctgaggagggccacccttcaggtttaccagaaatcttagggtttggcccccctggtcacaggctaaatatatggtttaaaagttttattaaaaagaaaaacagaacaagacacactcacacccagatgactaatgaaggctaagcagaatagtctgagtttgctgagactaaagcagggatagtgttgaaaagttttcctttcactagtgggacacattccccttttcttttcaaagaggaagaacatggtgtcatccaatgtgaagtgagcagtttcgggtcaaactcttatggtaagaaactaaaaaaagatgccaagagacaaaccttcagaaatagaagaaatgcaaaagatggaataaaaaccctgatcattaaaacagagacaccttcactggtgtccaataaggattctctttacaaaacagaaacaaacaactcaaaaatttaccatactttgtaatgaaaataccagtatgttgaagacacagcagactgggtttctattagaacaagtatcagcaaggtcatgtagacttgtagaaacttttgccttctcctgcaccagacagatcattgtccagttgggttgtcagctggagaccgaaaagaacctaaaaaatggatctttttttttttctttttcccatggtcacgcatccacacaaatgagtcttttggatgagaaaagtcacagcaacttgagttctcctaatgaacagatgactttttagccctgtttgtttcaatggggaaaacaatgacaaaaaaaacaaaccccaggcaggcacgacacttatgtaaaatgaacacagttagtacaaaaccagtaaggcatcactttgggaaggtcagcaccgaagaggtcaggcaaggctcgtccagacggggcttctgggagggagtgaccctcacccttattgagctgcgtcatgttggttctgaggaaagtgcaagtcttttgcagggtgaccgcatcaccccaccggaagctggggcggggacgctggaggtgttggtgtgtgttctaaaccctcaaggacgagaagggaaggcaaggtccatggctcacccacatgtcgaggaccaggtcctcatccattttaaaggacacagatacccccagccctagcaggaggaggcgagtgtgtaggactgtgaggatggacaactaaaaaccaaaactgagcaggaccaaaccaaaactcaactcctgcggttcttactttcaccaaaggattgattctgaccaagaggggaagggggaaaaaaaaatcttcaaaaatcaatgcatcagaaaggaagaaactcaacctcattttcaaaaggtaacctgttctccaaagtagaacaagtctcactatacacagtgtttgcagaaaaaaaaaaaaaaaaacctgattcattcatatatcagaaggaaagagacacatgctgttctgcactgacagccacatccactcgctcacactctcactccgtcactcactctcacggatattaatcagaggctgatggacctgaatggggtggtttgattggaacaggcaaaatacctctcgggtaaggaaagcaccatttaaaaaacatgaaagcacggtttatttgctcctaaggtttccctgtgtcgtagctctgtagtgcgttgaacgtgaccaaagcaagcaccctggttagcaccagttctccctgtggccggctgtgtgggagggtgggtggcacggctctgagacccagtctggagggtctgtgctgaggggaagccgtgcttctctgtgtttccgactttgctccagtctcttctgtctctgggaagctcatggcaggatgctgtttggtttcagagcttcatgtgggttctctttttttttttctctctgtctctcttttcatttcaacggcgatgatcctttcccgagaagtatcttcagtgtcttagggaggtcacagcaacaaggcaaaacaataattaaagtacaacagaaggtagtgcagttctcgctgtggaaggaagcggtccgcaggcagctggcccgggatgcctgcacccaggtcgaggctgaaggacggggggtctcggtgttcccgcagctctaaggctgtggctgggggctggctcaggaagtcatcttcagggtgatgtgggggatgcaggtggaatgcggtgaggagaagaggagggcgctgggctccgggcccctgtcacagagtggactccaaagaggagtccaagatgtcatcgtgatggctgttgctgttggagtcgctgtcatagctctgggggctggagtagttggctgcctcctgcagcctcatcagcatgttcatcagcgggtcaccttcagcatcactggggggcatctgcttgcttgtcgatccctcccgaggcatggagtagccgtcgaagccgacatcctcaggccgtaactgcagcaggggaggccactcgtgctgttgtgggctggctgcccatggatatgtgtccatcacccacttggcaggatcctcccagggggcgcgccttccatagagctggagtccttctctgacggcttccaggagataggggataatggaatagttccacaagtcggtgaaccacactctcgagccgtccacatcgatggggcatgacaggaagagccgggggccgatggtgacgtccgaggaactgtgagcctccaggaagcggttgaggtgatgccagaccttgggaatccagtcaatgatttttaccagctccatattgcgcacccgcccactgatctctgtttccatgagcttcctcctcaggaatcggccaaggaaacccttcacaggctccgtgtggttggcacaaagcacccatctgaagttatggtgaagctgcaggttgggagtcgaagaggtagcctggttcattgtgccaattatgtaagggcatttgtggtacttgcagttgagcagcccattgaagatctctcccagagagctcacgtggtgtaggttgtccaggatgatgacgaggggcatgtccacagcattgttctcactgttgcactggtcagcaaggttggacaggtactggcgcaattccttgctggacttatggtccacgttaaaggtggcgataaccccgtctgtcaactcccgtccctctcgaagcactatatactcagacagccggttggccaggtaggttttcccagtgccgctggggccagagagaatgatccgacggtgctctatcaggagggagacgtagcgctgcaggatgggcttgggaatcaaggactcaaacaccagtgagtccaggctgttttctgcgagccctttcacagtcactgagatggtcgtgttctctccaaccagatagccacaaggaagcagctccggtgtttcggaagtgttgctgcgcttgatttctccaatgctgtagccaagaacgctgtctgaattcagccctagctgactcactgggtcgacatgaatgatgtattctttgaacagccgtctaaccaccccatcgagcacatcccacttcgtcttgccactaactccaatgcagccaataagaaagagatgtggtctggaatcctccttccacttcatttcctcctgaaagctgacaactatcttaacatgcctgcctccttccttccgagccgagcattcaccagtgtcatccagcaacatgtccaggctggttgactcagtgaggttcaagctgtgctgggagaggcccatggactgcctcggggaggcagagatggacacttgggaaggagcccggctgcagccactgccttgagactctgacttcagccgatcattctcagctttcagcttctctatttcactctgcatcctgttcatggcctcccggagctggtccagctggtgggcagaactgagagcttctaagcggatatccgtcagcttcatctccttgtctcttaactcatttcggagctgcatgacggtctcagcttcactatccatgcattctgaaattagagagttggagtgagaattcctcagcagtggggtggaacctgtggacccattgtgcggtaactttggtgaggaaggcaaagaagaatccgtcatctcctcaatatctgaatgagaggacgcagattttggggacttcttcttcccgaaagcttgcttgaaggagctgcgtaaccagttcttccgcttcttcttctttgagtcactctctatgttgctgcccacgctggagtggctggtggcactgttgatgctggagacgctgtctgaggagtgctgcctgcggatgcggaggtctgcagactgggcagtgccgtttcctttgcagttgagctcaggtgtgttaattactccattaatggcagcctgggcagctgcgttctgtttctttagcagctcaatggtttttcttaactcattcagttctgagtccttctgctcagctgtcatggtcagactctggagcctgattgtcatgttaccaagactctgttcaaaggctgccacaaggtgagcatttgctgtcagctgggtggtcaaagctgaaactttctcctgggaggcatccagttcccgccgcagcttgcgaatctctgactggcatttttcttctggtgtagaataaactgacgatgtgctggaaaccaaggagagtgaggatccatgaacttcttcaaacccatcccggaatgagcctgaacggctcatggttctgctcttctcatccagggacatggagctattccggaagcggctgtcagtgtatggatcatactgcccatcagcattggagaggctgtgagtcctcagcatggtcgggttggacaagctcatctgggtgacagtggtgggactcgcaagctgggaaaagttgaatcttgttccggagggagaagtcacgctggagccagaggaaaagggggaattggcagcggtgtcctgaaggcctcctgcagaatgggaccgtaaccattcttttgcatcttcttgcgtgcgaagctgggaggtgggagtatacctgagtcctttcttaggcaaagtgttcctatcaaggtgcgggtcactgtcctgtttcctgggcagagtacttctgcagaacttagggctagcagcaggggaagagagagggctttctgacagtgtggtcttcacactgttagttctgacaaagggagtcaaggagtcgtccttggaggaggcgatgaggccagtggaagaattgtggctggggacccctccactgctgagggagatgtcgatggactcacagctggtgtggaggctgctgacagactgaaagcccaggccatccttgctaactgcggaggagctgctggcgttggtgccccaggtgaggctgttggaaggggccgagtgggctgagctggggctggaggctagcggagactggttgaggtccacattcttgctgtagagaggactgctgctcccactgctcaggacgccactgcctgacggggagtctaggttaccttgctgagtcatggtggcatgaggattggagatgaccaccgaatttttcatgttttcagctgtggcgatgggcacttgcttggtaggcttcccaccaaagagtctgcggagtgtgggagaggccacatctgggtacttggctccaggctggagactggtctgagccggactggacacaggctgggctgccggattcactttcaccgagttacaggaagccacactctcgttgtctgatgagatgcctttctccttgtctgtttggttgaccagacctggtagagagctgcctagggctgttttggaaggctccctcagtttgggcactggcaggcctgcggacttgctgctaatgttggaatctatgctgctggtgctagacctgttcccagccccgttccggctgttggacttactgggcctcggcaaactccggtactgaaggtttgtccgggagcttagggctagatacccgtcatcctgattctgagccccatccatacttgacttccgaccagcagaccgactgacgagtgcagatgactttgggattttgcccagtgtggctgacctgctggtgacagtcaccccgctggctgtgatcatggccaggccggcggcggaaccactctgcttcttgaacccaaagctgttggcattggcagtaggtgtcctagagctgctggggaggggctttttggattcgtcaccactgctccggcctgcatctgatggggagcgcttcacctgggaggctttaggagaaagccttcctttctcagacacctttgcgtcgtctgtttttccagttcctggggtcttcagtgcgcctgccggggctgaaggcttcgtccttggcatggtgatgcccacctgagctgtcatgcctcgccgccatgagcctgtctgggagatgacaggattcttcttgcccgacgtgcttttgtcggactcgtcagacacatcagaaggattccgcctccacttggaacctggctccatttttatgccgctgtctgagcctccgtctgatttcttgacatcatcaccagaccacagggaattcctctccacctgtgagtgcttctcagcatcagtctgcacatccaggttttttcgagaggaggcaggtgtgttggcataagagctgatggaggagctggtgttgatgtcatcagtgctgaggttgtctatggtgtcgctgatgccgctgctgacggagctgctgtcgtcccagctgtcagcgtctccgaggcccagggaggtatttcgttgcagggtctcccgtaccacagccatcccatcagggagccggttcaggcgacgggtatagaggccaagtccaccatcagtcatgtatccgcttgtaatgtcatcggtccggatgttcttgctcagaacatccccgtcgctcatgtagccgggggcatccatgctgatgccttccaggtccatctcatctcctgccttgtctgagacgtccacatggcagacactactgccccgggaggccagctgccttctcagaggggcggagtacacatagcgacctgactcagtgttgatgaacctgctggcgttggctcgagggggatacccattgcccattgagggggcgtctcctgcttggagccgagggctggactggcccagtctccaggacagaggtgtgggcctccctgtcaagctgagtatgctacggccactcatctccgtggtgacattggtgtcaaacgtggtttccaatgtgctgtgtgtaacctgagttccccttaaactggacatggtttcctccaaattctgccgcagatcagcgatgttcttcactgtccgcagccgccgagcctcaggatcttccccagtgagttcttccagagcaggctgtccagtcttggtgaagtggctgggctccacgctcacacctgttgagcttgactcggcagtaacattcccttcagtgtccgtctgagacctgtacaggaaaggtgcaaccgtggcagtgttgggatggttgtattgctgctggggctgaggtagctgaacactgacggtattgcttcctgtggtctgggtggtcccgacagacccactgacagtctggctgctgatgctgtggttcagggtggtccctcctgggccttttccttctgaggacgccaggctggaagaggaactggagtgtctgccgtccagctggggcttctgctgggggagtcctgagctcagcttcccactccggctccgctccccttccttggaaggcgctggggcacttggggatttcccgggcatgcttttcattcctggttttggtattccactgtgggaaggggccatgggctccttcttggcactgttgagcttcccccctttggggatgaagctggcaatcttggaggacttttttggcatctcgggcacagctgctccactggggtcttcttttggctcctccttgaggtccagcctctccgtcacagaggctctcttggcaaggtccttgcttttctccttatccttctcccgctgttgtttctccttctctttctcattgcctttcagagaactcttcttgttggtcagtgcccggctaaaagtcctctgggcaatgcccttgagtgcaatcttggggctgctggaagcagggcccacggtggtgagcatgcgactggcggcctccagctcctcgctctcttcgaagctgggcagagtctccagccgctcacagcttgtgtcccgggaccccggcccctcacctgcctttgagccccctttactgttgaaaagtttcagcttttccagcatggacttctgattgttgggggccggcttcatggcttcaggtgtgggcctgggggcctcaggcccaggaggcttgaccgagagcatggataccgtggcactgtgcttcacgctgagggatttgctgcgccaaggcttggtggctgcaccgggctgcgggatggccgaggaggtactgcaattagtaggggtggagctgctgccgctctccaaggaagcaggtgcattgtcactcattccggggtgggaggaggctgaacttgccaaaggctctttctcgtggctgcttggcggtgggggtggggaggtgactggtttggatttatcatagttgttaaagctctggctgcgtcggttgttagcagtagttgaccctccgcgtgttttggcctcgctgcctgcagcggataccctcgcggtaggacctggaagtctggactgcatttcagcttgtgcttttgactgctgatgtggcgctggctggtgaggctggcacggggcttggggagtgactggcacctgctgctgaggggtgccagcctggcactgggagggggccccggccacctgggatacggcgggcggcagaggtgaggagaggtgctgcttctggggctgctgctgctgctgcttgtatcgggagaggctgaagaagaggcctagaatggccttgaggtttccattcctgatctcttctgcagacagcccctggatgtttattcccttagctgccaggaaattcaagcaggcatctatgttttcaatcatttgggatctgttcttcggacagccattgatgtcttcaatcttttcatttgccacaacctggataatctgggccaggaggacgccatctgtcacatcttgctggagatccctgatgagacgcttgtggccggatttggctaggtaatgattggcccagtctgtgtagatcctcttttgatcttccagtccgtggataactggctttctcttctgctgttggctggactcagaaaccgattccatttcccagaaataaaatcctctctctccttcagcgatgcttccaaatccacagaggaacaaaataacccacacaaaagtgatgcatgcaacagccagacagagttcccgccagccaaggaaatcagcaccacctcttcaaaggtcttcctgtcttcttaaaatccactcgggaacctcactcggcaccactgcctttgcaatgagggtgactgctgccggcatcatgagagctaagtcttggggttttactttaggtctgagactcgcttcatgagagcccagaggacaaatctgggcaaagacaagtccatatcctgaggcacataccacattactgccccagaaaccctttccttcactgtctccttggcacagataatttatatgtcaataacaatgtaaatgggcatttaatccaccaagctgctaacatccacatccctctctggcagcccctgactcccataaatcactgcaaacactgcgcggaaagccgcccctcatggctcctgcaagcgttcatcacagcggtggctcccctcctgggctgtcatcttccttcatggtgtaagacccatacctgcgcccacaccggcttcgcggagccgcctcctccagccggtctcgcactgcactccggcccgcgcttctcagcc

SEQ ID NO: 17879 - RNA, 11333 nt, Homo sapiens
  source 1..11333: mol_type = other RNA
tcggcctggggaggaggaaggggagggaggatggaaacataccgtacacaaaatactcaattcctagttttctctttaaaaatggctagaaaaaattcatcaaaatgcagcactttaatcaattatttacaatttctatgttacaatgaaaaaatgtacatcttatagaacatatttcataaaactgctccactggaaacaactagatcaaaacagcaaaccttccatttaatatccacaaagttggattatttttcctttttgaagtagattcgccacaatcaaatttgaatacagagaattttgaagtttaagcatcaaacaacaaagtaaaagtccccaagatacaacaaagatctaggcaagtcttgttcctgtcccactcccaccccacccctaatgaaacttaaaaggtattcccatttcaattatggcctgtatcattcttggcagtttgggaagagaacttttggcttccattggtaactcaacataaatgttgcatagaatttatatatttcaaaattggcctaactgtagaaaaggcaaaatggaagcatttccgatagagccctaaatgagtacaaagtcactttgtaaaaggtgagtgacactaaagtaaaaatatgaccaaaataagaaatgtgcatattagacaaccctgcttcccgaaactttaggaaggacacggagttgtgagtcacacaagggctatgctacttgaagtcaatgttcaccaatcaggcagcactaggtacagaagtcttggttctgaacctggacccaggagggaagtctgtgggaaaggggagaagagaatgacaagagaggatgtcatattaaaaaaaggtttcaaacaatattggcaggtgtctactcacaaggtgattggaaaactgcccacgaggagaagtcaactttacctcctcccaaattcacagtacgcgagtgtagtagggtcattgctgggagataaattgtctgaggagggccacccttcaggtttaccagaaatcttagggtttggcccccctggtcacaggctaaatatatggtttaaaagttttattaaaaagaaaaacagaacaagacacactcacacccagatgactaatgaaggctaagcagaatagtctgagtttgctgagactaaagcagggatagtgttgaaaagttttcctttcactagtgggacacattccccttttcttttcaaagaggaagaacatggtgtcatccaatgtgaagtgagcagtttcgggtcaaactcttatggtaagaaactaaaaaaagatgccaagagacaaaccttcagaaatagaagaaatgcaaaagatggaataaaaaccctgatcattaaaacagagacaccttcactggtgtccaataaggattctctttacaaaacagaaacaaacaactcaaaaatttaccatactttgtaatgaaaataccagtatgttgaagacacagcagactgggtttctattagaacaagtatcagcaaggtcatgtagacttgtagaaacttttgccttctcctgcaccagacagatcattgtccagttgggttgtcagctggagaccgaaaagaacctaaaaaatggatctttttttttttctttttcccatggtcacgcatccacacaaatgagtcttttggatgagaaaagtcacagcaacttgagttctcctaatgaacagatgactttttagccctgtttgtttcaatggggaaaacaatgacaaaaaaaacaaaccccaggcaggcacgacacttatgtaaaatgaacacagttagtacaaaaccagtaaggcatcactttgggaaggtcagcaccgaagaggtcaggcaaggctcgtccagacggggcttctgggagggagtgaccctcacccttattgagctgcgtcatgttggttctgaggaaagtgcaagtcttttgcagggtgaccgcatcaccccaccggaagctggggcggggacgctggaggtgttggtgtgtgttctaaaccctcaaggacgagaagggaaggcaaggtccatggctcacccacatgtcgaggaccaggtcctcatccattttaaaggacacagatacccccagccctagcaggaggaggcgagtgtgtaggactgtgaggatggacaactaaaaaccaaaactgagcaggaccaaaccaaaactcaactcctgcggttcttactttcaccaaaggattgattctgaccaagaggggaagggggaaaaaaaaatcttcaaaaatcaatgcatcagaaaggaagaaactcaacctcattttcaaaaggtaacctgttctccaaagtagaacaagtctcactatacacagtgtttgcagaaaaaaaaaaaaaaaaacctgattcattcatatatcagaaggaaagagacacatgctgttctgcactgacagccacatccactcgctcacactctcactccgtcactcactctcacggatattaatcagaggctgatggacctgaatggggtggtttgattggaacaggcaaaatacctctcgggtaaggaaagcaccatttaaaaaacatgaaagcacggtttatttgctcctaaggtttccctgtgtcgtagctctgtagtgcgttgaacgtgaccaaagcaagcaccctggttagcaccagttctccctgtggccggctgtgtgggagggtgggtggcacggctctgagacccagtctggagggtctgtgctgaggggaagccgtgcttctctgtgtttccgactttgctccagtctcttctgtctctgggaagctcatggcaggatgctgtttggtttcagagcttcatgtgggttctctttttttttttctctctgtctctcttttcatttcaacggcgatgatcctttcccgagaagtatcttcagtgtcttagggaggtcacagcaacaaggcaaaacaataattaaagtacaacagaaggtagtgcagttctcgctgtggaaggaagcggtccgcaggcagctggcccgggatgcctgcacccaggtcgaggctgaaggacggggggtctcggtgttcccgcagctctaaggctgtggctgggggctggctcaggaagtcatcttcagggtgatgtgggggatgcaggtggaatgcggtgaggagaagaggagggcgctgggctccgggcccctgtcacagagtggactccaaagaggagtccaagatgtcatcgtgatggctgttgctgttggagtcgctgtcatagctctgggggctggagtagttggctgcctcctgcagcctcatcagcatgttcatcagcgggtcaccttcagcatcactggggggcatctgcttgcttgtcgatccctcccgaggcatggagtagccgtcgaagccgacatcctcaggccgtaactgcagcaggggaggccactcgtgctgttgtgggctggctgcccatggatatgtgtccatcacccacttggcaggatcctcccagggggcgcgccttccatagagctggagtccttctctgacggcttccaggagataggggataatggaatagttccacaagtcggtgaaccacactctcgagccgtccacatcgatggggcatgacaggaagagccgggggccgatggtgacgtccgaggaactgtgagcctccaggaagcggttgaggtgatgccagaccttgggaatccagtcaatgatttttaccagctccatattgcgcacccgcccactgatctctgtttccatgagcttcctcctcaggaatcggccaaggaaacccttcacaggctccgtgtggttggcacaaagcacccatctgaagttatggtgaagctgcaggttgggagtcgaagaggtagcctggttcattgtgccaattatgtaagggcatttgtggtacttgcagttgagcagcccattgaagatctctcccagagagctcacgtggtgtaggttgtccaggatgatgacgaggggcatgtccacagcattgttctcactgttgcactggtcagcaaggttggacaggtactggcgcaattccttgctggacttatggtccacgttaaaggtggcgataaccccgtctgtcaactcccgtccctctcgaagcactatatactcagacagccggttggccaggtaggttttcccagtgccgctggggccagagagaatgatccgacggtgctctatcaggagggagacgtagcgctgcaggatgggcttgggaatcaaggactcaaacaccagtgagtccaggctgttttctgcgagccctttcacagtcactgagatggtcgtgttctctccaaccagatagccacaaggaagcagctccggtgtttcggaagtgttgctgcgcttgatttctccaatgctgtagccaagaacgctgtctgaattcagccctagctgactcactgggtcgacatgaatgatgtattctttgaacagccgtctaaccaccccatcgagcacatcccacttcgtcttgccactaactccaatgcagccaataagaaagagatgtggtctggaatcctccttccacttcatttcctcctgaaagctgacaactatcttaacatgcctgcctccttccttccgagccgagcattcaccagtgtcatccagcaacatgtccaggctggttgactcagtgaggttcaagctgtgctgggagaggcccatggactgcctcggggaggcagagatggacacttgggaaggagcccggctgcagccactgccttgagactctgacttcagccgatcattctcagctttcagcttctctatttcactctgcatcctgttcatggcctcccggagctggtccagctggtgggcagaactgagagcttctaagcggatatccgtcagcttcatctccttgtctcttaactcatttcggagctgcatgacggtctcagcttcactatccatgcattctgaaattagagagttggagtgagaattcctcagcagtggggtggaacctgtggacccattgtgcggtaactttggtgaggaaggcaaagaagaatccgtcatctcctcaatatctgaatgagaggacgcagattttggggacttcttcttcccgaaagcttgcttgaaggagctgcgtaaccagttcttccgcttcttcttctttgagtcactctctatgttgctgcccacgctggagtggctggtggcactgttgatgctggagacgctgtctgaggagtgctgcctgcggatgcggaggtctgcagactgggcagtgccgtttcctttgcagttgagctcaggtgtgttaattactccattaatggcagcctgggcagctgcgttctgtttctttagcagctcaatggtttttcttaactcattcagttctgagtccttctgctcagctgtcatggtcagactctggagcctgattgtcatgttaccaagactctgttcaaaggctgccacaaggtgagcatttgctgtcagctgggtggtcaaagctgaaactttctcctgggaggcatccagttcccgccgcagcttgcgaatctctgactggcatttttcttctggtgtagaataaactgacgatgtgctggaaaccaaggagagtgaggatccatgaacttcttcaaacccatcccggaatgagcctgaacggctcatggttctgctcttctcatccagggacatggagctattccggaagcggctgtcagtgtatggatcatactgcccatcagcattggagaggctgtgagtcctcagcatggtcgggttggacaagctcatctgggtgacagtggtgggactcgcaagctgggaaaagttgaatcttgttccggagggagaagtcacgctggagccagaggaaaagggggaattggcagcggtgtcctgaaggcctcctgcagaatgggaccgtaaccattcttttgcatcttcttgcgtgcgaagctgggaggtgggagtatacctgagtcctttcttaggcaaagtgttcctatcaaggtgcgggtcactgtcctgtttcctgggcagagtacttctgcagaacttagggctagcagcaggggaagagagagggctttctgacagtgtggtcttcacactgttagttctgacaaagggagtcaaggagtcgtccttggaggaggcgatgaggccagtggaagaattgtggctggggacccctccactgctgagggagatgtcgatggactcacagctggtgtggaggctgctgacagactgaaagcccaggccatccttgctaactgcggaggagctgctggcgttggtgccccaggtgaggctgttggaaggggccgagtgggctgagctggggctggaggctagcggagactggttgaggtccacattcttgctgtagagaggactgctgctcccactgctcaggacgccactgcctgacggggagtctaggttaccttgctgagtcatggtggcatgaggattggagatgaccaccgaatttttcatgttttcagctgtggcgatgggcacttgcttggtaggcttcccaccaaagagtctgcggagtgtgggagaggccacatctgggtacttggctccaggctggagactggtctgagccggactggacacaggctgggctgccggattcactttcaccgagttacaggaagccacactctcgttgtctgatgagatgcctttctccttgtctgtttggttgaccagacctggtagagagctgcctagggctgttttggaaggctccctcagtttgggcactggcaggcctgcggacttgctgctaatgttggaatctatgctgctggtgctagacctgttcccagccccgttccggctgttggacttactgggcctcggcaaactccggtactgaaggtttgtccgggagcttagggctagatacccgtcatcctgattctgagccccatccatacttgacttccgaccagcagaccgactgacgagtgcagatgactttgggattttgcccagtgtggctgacctgctggtgacagtcaccccgctggctgtgatcatggccaggccggcggcggaaccactctgcttcttgaacccaaagctgttggcattggcagtaggtgtcctagagctgctggggaggggctttttggattcgtcaccactgctccggcctgcatctgatggggagcgcttcacctgggaggctttaggagaaagccttcctttctcagacacctttgcgtcgtctgtttttccagttcctggggtcttcagtgcgcctgccggggctgaaggcttcgtccttggcatggtgatgcccacctgagctgtcatgcctcgccgccatgagcctgtctgggagatgacaggattcttcttgcccgacgtgcttttgtcggactcgtcagacacatcagaaggattccgcctccacttggaacctggctccatttttatgccgctgtctgagcctccgtctgatttcttgacatcatcaccagaccacagggaattcctctccacctgtgagtgcttctcagcatcagtctgcacatccaggttttttcgagaggaggcaggtgtgttggcataagagctgatggaggagctggtgttgatgtcatcagtgctgaggttgtctatggtgtcgctgatgccgctgctgacggagctgctgtcgtcccagctgtcagcgtctccgaggcccagggaggtatttcgttgcagggtctcccgtaccacagccatcccatcagggagccggttcaggcgacgggtatagaggccaagtccaccatcagtcatgtatccgcttgtaatgtcatcggtccggatgttcttgctcagaacatccccgtcgctcatgtagccgggggcatccatgctgatgccttccaggtccatctcatctcctgccttgtctgagacgtccacatggcagacactactgccccgggaggccagctgccttctcagaggggcggagtacacatagcgacctgactcagtgttgatgaacctgctggcgttggctcgagggggatacccattgcccattgagggggcgtctcctgcttggagccgagggctggactggcccagtctccaggacagaggtgtgggcctccctgtcaagctgagtatgctacggccactcatctccgtggtgacattggtgtcaaacgtggtttccaatgtgctgtgtgtaacctgagttccccttaaactggacatggtttcctccaaattctgccgcagatcagcgatgttcttcactgtccgcagccgccgagcctcaggatcttccccagtgagttcttccagagcaggctgtccagtcttggtgaagtggctgggctccacgctcacacctgttgagcttgactcggcagtaacattcccttcagtgtccgtctgagacctgtacaggaaaggtgcaaccgtggcagtgttgggatggttgtattgctgctggggctgaggtagctgaacactgacggtattgcttcctgtggtctgggtggtcccgacagacccactgacagtctggctgctgatgctgtggttcagggtggtccctcctgggccttttccttctgaggacgccaggctggaagaggaactggagtgtctgccgtccagctggggcttctgctgggggagtcctgagctcagcttcccactccggctccgctccccttccttggaaggcgctggggcacttggggatttcccgggcatgcttttcattcctggttttggtattccactgtgggaaggggccatgggctccttcttggcactgttgagcttcccccctttggggatgaagctggcaatcttggaggacttttttggcatctcgggcacagctgctccactggggtcttcttttggctcctccttgaggtccagcctctccgtcacagaggctctcttggcaaggtccttgcttttctccttatccttctcccgctgttgtttctccttctctttctcattgcctttcagagaactcttcttgttggtcagtgcccggctaaaagtcctctgggcaatgcccttgagtgcaatcttggggctgctggaagcagggcccacggtggtgagcatgcgactggcggcctccagctcctcgctctcttcgaagctgggcagagtctccagccgctcacagcttgtgtcccgggaccccggcccctcacctgcctttgagccccctttactgttgaaaagtttcagcttttccagcatggacttctgattgttgggggccggcttcatggcttcaggtgtgggcctgggggcctcaggcccaggaggcttgaccgagagcatggataccgtggcactgtgcttcacgctgagggatttgctgcgccaaggcttggtggctgcaccgggctgcgggatggccgaggaggtactgcaattagtaggggtggagctgctgccgctctccaaggaagcaggtgcattgtcactcattccggggtgggaggaggctgaacttgccaaaggctctttctcgtggctgcttggcggtgggggtggggaggtgactggtttggatttatcatagttgttaaagctctggctgcgtcggttgttagcagtagttgaccctccgcgtgttttggcctcgctgcctgcagcggataccctcgcggtaggacctggaagtctggactgcatttcagcttgtgcttttgactgctgatgtggcgctggctggtgaggctggcacggggcttggggagtgactggcacctgctgctgaggggtgccagcctggcactgggagggggccccggccacctgggatacggcgggcggcagaggtgaggagaggtgctgcttctggggctgctgctgctgctgcttgtatcgggagaggctgaagaagaggcctagaatggccttgaggtttccattcctgatctcttctgcagacagcccctggatgtttattcccttagctgccaggaaattcaagcaggcatctatgttttcaatcatttgggatctgttcttcggacagccattgatgtcttcaatcttttcatttgccacaacctggataatctgggccaggaggacgccatctgtcacatcttgctggagatccctgatgagacgcttgtggccggatttggctaggtaatgattggcccagtctgtgtagatctgggtatcgaacccgttttccaccgagccgctcttccgcagcgggagcccctcccccgctggctcctgcagcccctgcagcacctgcgatttcagggggatctggctaggataggtggtcttgctcacctccaccttgcttcccaacttcaggtagcagggctgggggcccgcccgggccgggggcacgtgcaggatgggcgcggcgctgtgcacgggtttgggcagtcccgacttcattttggaggcgaccaggatggccggcatcttctcccggggcttgggctttcccagcacgtccctggcagcggcggcgggggcgaccgctaaaggcagcgcgggtagcagagcaggcgccgggccttagcccacgaggcgcccaccaccagcggctaaaaaaaaaatccccaggtcggggaactcgaagcaatcgggcgagcgcgcctttggggtgccgggatgggaatgggggactggccacggcgctcagcgggtcccacctggacggatgctgccgccgggtctcacacctctcctgggtggcctttcaagagctctgggcgctcaggggctgccgcctcttgcaaatttcctcctgggaaacagaggcttggacgcccatattaacttgtcactgcatctccgaagtgaggaggcccctttggaagagacagaggcggcggcgacccacgagtcccgttccggaggctacgggtctgagccggcgagagaaagagcgagcagccaaggaaggaaaggagacagcagcgaaggaaggagagaagaagggcgcaagggtcccaagacgtctccaccgagaggcagctgccaccctgctcgcgagcaccgcagtgtcacccgcgacgcagcagaggtgcggcaagagcccccgaaaggtctctcttggggtgacagtcaccgctgcccagaaggcccccggactgagagcaccttagcgcctgcgggtctgcacatgctccgtgagctagatagaggcaaggctgtggccgtggggcgcgggcgccgggacgcgcggctggcgggccgggcagggctgcgctcgggagcggccgccgcgcttcccgggaaggctgcgctggctgcggggctcagcgcaggggaggac

SEQ ID NO: 17880 - RNA, 11333 nt, Homo sapiens
  source 1..11333: mol_type = other RNA
tcggcctggggaggaggaaggggagggaggatggaaacataccgtacacaaaatactcaattcctagttttctctttaaaaatggctagaaaaaattcatcaaaatgcagcactttaatcaattatttacaatttctatgttacaatgaaaaaatgtacatcttatagaacatatttcataaaactgctccactggaaacaactagatcaaaacagcaaaccttccatttaatatccacaaagttggattatttttcctttttgaagtagattcgccacaatcaaatttgaatacagagaattttgaagtttaagcatcaaacaacaaagtaaaagtccccaagatacaacaaagatctaggcaagtcttgttcctgtcccactcccaccccacccctaatgaaacttaaaaggtattcccatttcaattatggcctgtatcattcttggcagtttgggaagagaacttttggcttccattggtaactcaacataaatgttgcatagaatttatatatttcaaaattggcctaactgtagaaaaggcaaaatggaagcatttccgatagagccctaaatgagtacaaagtcactttgtaaaaggtgagtgacactaaagtaaaaatatgaccaaaataagaaatgtgcatattagacaaccctgcttcccgaaactttaggaaggacacggagttgtgagtcacacaagggctatgctacttgaagtcaatgttcaccaatcaggcagcactaggtacagaagtcttggttctgaacctggacccaggagggaagtctgtgggaaaggggagaagagaatgacaagagaggatgtcatattaaaaaaaggtttcaaacaatattggcaggtgtctactcacaaggtgattggaaaactgcccacgaggagaagtcaactttacctcctcccaaattcacagtacgcgagtgtagtagggtcattgctgggagataaattgtctgaggagggccacccttcaggtttaccagaaatcttagggtttggcccccctggtcacaggctaaatatatggtttaaaagttttattaaaaagaaaaacagaacaagacacactcacacccagatgactaatgaaggctaagcagaatagtctgagtttgctgagactaaagcagggatagtgttgaaaagttttcctttcactagtgggacacattccccttttcttttcaaagaggaagaacatggtgtcatccaatgtgaagtgagcagtttcgggtcaaactcttatggtaagaaactaaaaaaagatgccaagagacaaaccttcagaaatagaagaaatgcaaaagatggaataaaaaccctgatcattaaaacagagacaccttcactggtgtccaataaggattctctttacaaaacagaaacaaacaactcaaaaatttaccatactttgtaatgaaaataccagtatgttgaagacacagcagactgggtttctattagaacaagtatcagcaaggtcatgtagacttgtagaaacttttgccttctcctgcaccagacagatcattgtccagttgggttgtcagctggagaccgaaaagaacctaaaaaatggatctttttttttttctttttcccatggtcacgcatccacacaaatgagtcttttggatgagaaaagtcacagcaacttgagttctcctaatgaacagatgactttttagccctgtttgtttcaatggggaaaacaatgacaaaaaaaacaaaccccaggcaggcacgacacttatgtaaaatgaacacagttagtacaaaaccagtaaggcatcactttgggaaggtcagcaccgaagaggtcaggcaaggctcgtccagacggggcttctgggagggagtgaccctcacccttattgagctgcgtcatgttggttctgaggaaagtgcaagtcttttgcagggtgaccgcatcaccccaccggaagctggggcggggacgctggaggtgttggtgtgtgttctaaaccctcaaggacgagaagggaaggcaaggtccatggctcacccacatgtcgaggaccaggtcctcatccattttaaaggacacagatacccccagccctagcaggaggaggcgagtgtgtaggactgtgaggatggacaactaaaaaccaaaactgagcaggaccaaaccaaaactcaactcctgcggttcttactttcaccaaaggattgattctgaccaagaggggaagggggaaaaaaaaatcttcaaaaatcaatgcatcagaaaggaagaaactcaacctcattttcaaaaggtaacctgttctccaaagtagaacaagtctcactatacacagtgtttgcagaaaaaaaaaaaaaaaaacctgattcattcatatatcagaaggaaagagacacatgctgttctgcactgacagccacatccactcgctcacactctcactccgtcactcactctcacggatattaatcagaggctgatggacctgaatggggtggtttgattggaacaggcaaaatacctctcgggtaaggaaagcaccatttaaaaaacatgaaagcacggtttatttgctcctaaggtttccctgtgtcgtagctctgtagtgcgttgaacgtgaccaaagcaagcaccctggttagcaccagttctccctgtggccggctgtgtgggagggtgggtggcacggctctgagacccagtctggagggtctgtgctgaggggaagccgtgcttctctgtgtttccgactttgctccagtctcttctgtctctgggaagctcatggcaggatgctgtttggtttcagagcttcatgtgggttctctttttttttttctctctgtctctcttttcatttcaacggcgatgatcctttcccgagaagtatcttcagtgtcttagggaggtcacagcaacaaggcaaaacaataattaaagtacaacagaaggtagtgcagttctcgctgtggaaggaagcggtccgcaggcagctggcccgggatgcctgcacccaggtcgaggctgaaggacggggggtctcggtgttcccgcagctctaaggctgtggctgggggctggctcaggaagtcatcttcagggtgatgtgggggatgcaggtggaatgcggtgaggagaagaggagggcgctgggctccgggcccctgtcacagagtggactccaaagaggagtccaagatgtcatcgtgatggctgttgctgttggagtcgctgtcatagctctgggggctggagtagttggctgcctcctgcagcctcatcagcatgttcatcagcgggtcaccttcagcatcactggggggcatctgcttgcttgtcgatccctcccgaggcatggagtagccgtcgaagccgacatcctcaggccgtaactgcagcaggggaggccactcgtgctgttgtgggctggctgcccatggatatgtgtccatcacccacttggcaggatcctcccagggggcgcgccttccatagagctggagtccttctctgacggcttccaggagataggggataatggaatagttccacaagtcggtgaaccacactctcgagccgtccacatcgatggggcatgacaggaagagccgggggccgatggtgacgtccgaggaactgtgagcctccaggaagcggttgaggtgatgccagaccttgggaatccagtcaatgatttttaccagctccatattgcgcacccgcccactgatctctgtttccatgagcttcctcctcaggaatcggccaaggaaacccttcacaggctccgtgtggttggcacaaagcacccatctgaagttatggtgaagctgcaggttgggagtcgaagaggtagcctggttcattgtgccaattatgtaagggcatttgtggtacttgcagttgagcagcccattgaagatctctcccagagagctcacgtggtgtaggttgtccaggatgatgacgaggggcatgtccacagcattgttctcactgttgcactggtcagcaaggttggacaggtactggcgcaattccttgctggacttatggtccacgttaaaggtggcgataaccccgtctgtcaactcccgtccctctcgaagcactatatactcagacagccggttggccaggtaggttttcccagtgccgctggggccagagagaatgatccgacggtgctctatcaggagggagacgtagcgctgcaggatgggcttgggaatcaaggactcaaacaccagtgagtccaggctgttttctgcgagccctttcacagtcactgagatggtcgtgttctctccaaccagatagccacaaggaagcagctccggtgtttcggaagtgttgctgcgcttgatttctccaatgctgtagccaagaacgctgtctgaattcagccctagctgactcactgggtcgacatgaatgatgtattctttgaacagccgtctaaccaccccatcgagcacatcccacttcgtcttgccactaactccaatgcagccaataagaaagagatgtggtctggaatcctccttccacttcatttcctcctgaaagctgacaactatcttaacatgcctgcctccttccttccgagccgagcattcaccagtgtcatccagcaacatgtccaggctggttgactcagtgaggttcaagctgtgctgggagaggcccatggactgcctcggggaggcagagatggacacttgggaaggagcccggctgcagccactgccttgagactctgacttcagccgatcattctcagctttcagcttctctatttcactctgcatcctgttcatggcctcccggagctggtccagctggtgggcagaactgagagcttctaagcggatatccgtcagcttcatctccttgtctcttaactcatttcggagctgcatgacggtctcagcttcactatccatgcattctgaaattagagagttggagtgagaattcctcagcagtggggtggaacctgtggacccattgtgcggtaactttggtgaggaaggcaaagaagaatccgtcatctcctcaatatctgaatgagaggacgcagattttggggacttcttcttcccgaaagcttgcttgaaggagctgcgtaaccagttcttccgcttcttcttctttgagtcactctctatgttgctgcccacgctggagtggctggtggcactgttgatgctggagacgctgtctgaggagtgctgcctgcggatgcggaggtctgcagactgggcagtgccgtttcctttgcagttgagctcaggtgtgttaattactccattaatggcagcctgggcagctgcgttctgtttctttagcagctcaatggtttttcttaactcattcagttctgagtccttctgctcagctgtcatggtcagactctggagcctgattgtcatgttaccaagactctgttcaaaggctgccacaaggtgagcatttgctgtcagctgggtggtcaaagctgaaactttctcctgggaggcatccagttcccgccgcagcttgcgaatctctgactggcatttttcttctggtgtagaataaactgacgatgtgctggaaaccaaggagagtgaggatccatgaacttcttcaaacccatcccggaatgagcctgaacggctcatggttctgctcttctcatccagggacatggagctattccggaagcggctgtcagtgtatggatcatactgcccatcagcattggagaggctgtgagtcctcagcatggtcgggttggacaagctcatctgggtgacagtggtgggactcgcaagctgggaaaagttgaatcttgttccggagggagaagtcacgctggagccagaggaaaagggggaattggcagcggtgtcctgaaggcctcctgcagaatgggaccgtaaccattcttttgcatcttcttgcgtgcgaagctgggaggtgggagtatacctgagtcctttcttaggcaaagtgttcctatcaaggtgcgggtcactttctgacagtgtggtcttcacactgttagttctgacaaagggagtcaaggagtcgtccttggaggaggcgatgaggccagtggaagaattgtggctggggacccctccactgctgagggagatgtcgatggactcacagctggtgtggaggctgctgacagactgaaagcccaggccatccttgctaactgcggaggagctgctggcgttggtgccccaggtgaggctgttggaaggggccgagtgggctgagctggggctggaggctagcggagactggttgaggtccacattcttgctgtagagaggactgctgctcccactgctcaggacgccactgcctgacggggagtctaggttaccttgctgagtcatggtggcatgaggattggagatgaccaccgaatttttcatgttttcagctgtggcgatgggcacttgcttggtaggcttcccaccaaagagtctgcggagtgtgggagaggccacatctgggtacttggctccaggctggagactggtctgagccggactggacacaggctgggctgccggattcactttcaccgagttacaggaagccacactctcgttgtctgatgagatgcctttctccttgtctgtttggttgaccagacctggtagagagctgcctagggctgttttggaaggctccctcagtttgggcactggcaggcctgcggacttgctgctaatgttggaatctatgctgctggtgctagacctgttcccagccccgttccggctgttggacttactgggcctcggcaaactccggtactgaaggtttgtccgggagcttagggctagatacccgtcatcctgattctgagccccatccatacttgacttccgaccagcagaccgactgacgagtgcagatgactttgggattttgcccagtgtggctgacctgctggtgacagtcaccccgctggctgtgatcatggccaggccggcggcggaaccactctgcttcttgaacccaaagctgttggcattggcagtaggtgtcctagagctgctggggaggggctttttggattcgtcaccactgctccggcctgcatctgatggggagcgcttcacctgggaggctttaggagaaagccttcctttctcagacacctttgcgtcgtctgtttttccagttcctggggtcttcagtgcgcctgccggggctgaaggcttcgtccttggcatggtgatgcccacctgagctgtcatgcctcgccgccatgagcctgtctgggagatgacaggattcttcttgcccgacgtgcttttgtcggactcgtcagacacatcagaaggattccgcctccacttggaacctggctccatttttatgccgctgtctgagcctccgtctgatttcttgacatcatcaccagaccacagggaattcctctccacctgtgagtgcttctcagcatcagtctgcacatccaggttttttcgagaggaggcaggtgtgttggcataagagctgatggaggagctggtgttgatgtcatcagtgctgaggttgtctatggtgtcgctgatgccgctgctgacggagctgctgtcgtcccagctgtcagcgtctccgaggcccagggaggtatttcgttgcagggtctcccgtaccacagccatcccatcagggagccggttcaggcgacgggtatagaggccaagtccaccatcagtcatgtatccgcttgtaatgtcatcggtccggatgttcttgctcagaacatccccgtcgctcatgtagccgggggcatccatgctgatgccttccaggtccatctcatctcctgccttgtctgagacgtccacatggcagacactactgccccgggaggccagctgccttctcagaggggcggagtacacatagcgacctgactcagtgttgatgaacctgctggcgttggctcgagggggatacccattgcccattgagggggcgtctcctgcttggagccgagggctggactggcccagtctccaggacagaggtgtgggcctccctgtcaagctgagtatgctacggccactcatctccgtggtgacattggtgtcaaacgtggtttccaatgtgctgtgtgtaacctgagttccccttaaactggacatggtttcctccaaattctgccgcagatcagcgatgttcttcactgtccgcagccgccgagcctcaggatcttccccagtgagttcttccagagcaggctgtccagtcttggtgaagtggctgggctccacgctcacacctgttgagcttgactcggcagtaacattcccttcagtgtccgtctgagacctgtacaggaaaggtgcaaccgtggcagtgttgggatggttgtattgctgctggggctgaggtagctgaacactgacggtattgcttcctgtggtctgggtggtcccgacagacccactgacagtctggctgctgatgctgtggttcagggtggtccctcctgggccttttccttctgaggacgccaggctggaagaggaactggagtgtctgccgtccagctggggcttctgctgggggagtcctgagctcagcttcccactccggctccgctccccttccttggaaggcgctggggcacttggggatttcccgggcatgcttttcattcctggttttggtattccactgtgggaaggggccatgggctccttcttggcactgttgagcttcccccctttggggatgaagctggcaatcttggaggacttttttggcatctcgggcacagctgctccactggggtcttcttttggctcctccttgaggtccagcctctccgtcacagaggctctcttggcaaggtccttgcttttctccttatccttctcccgctgttgtttctccttctctttctcattgcctttcagagaactcttcttgttggtcagtgcccggctaaaagtcctctgggcaatgcccttgagtgcaatcttggggctgctggaagcagggcccacggtggtgagcatgcgactggcggcctccagctcctcgctctcttcgaagctgggcagagtctccagccgctcacagcttgtgtcccgggaccccggcccctcacctgcctttgagccccctttactgttgaaaagtttcagcttttccagcatggacttctgattgttgggggccggcttcatggcttcaggtgtgggcctgggggcctcaggcccaggaggcttgaccgagagcatggataccgtggcactgtgcttcacgctgagggatttgctgcgccaaggcttggtggctgcaccgggctgcgggatggccgaggaggtactgcaattagtaggggtggagctgctgccgctctccaaggaagcaggtgcattgtcactcattccggggtgggaggaggctgaacttgccaaaggctctttctcgtggctgcttggcggtgggggtggggaggtgactggtttggatttatcatagttgttaaagctctggctgcgtcggttgttagcagtagttgaccctccgcgtgttttggcctcgctgcctgcagcggataccctcgcggtaggacctggaagtctagagatctttttctgacccagagtgaagcggatgattttgctttgagatgagtccttggatgatgcactggactgcatttcagcttgtgcttttgactgctgatgtggcgctggctggtgaggctggcacggggcttggggagtgactggcacctgctgctgaggggtgccagcctggcactgggagggggccccggccacctgggatacggcgggcggcagaggtgaggagaggtgctgcttctggggctgctgctgctgctgcttgtatcgggagaggctgaagaagaggcctagaatggccttgaggtttccattcctgatctcttctgcagacagcccctggatgtttattcccttagctgccaggaaattcaagcaggcatctatgttttcaatcatttgggatctgttcttcggacagccattgatgtcttcaatcttttcatttgccacaacctggataatctgggccaggaggacgccatctgtcacatcttgctggagatccctgatgagacgcttgtggccggatttggctaggtaatgattggcccagtctgtgtagatctgggtatcgaacccgttttccaccgagccgctcttccgcagcgggagcccctcccccgctggctcctgcagcccctgcagcacctgcgatttcagggggatctggctaggataggtggtcttgctcacctccaccttgcttcccaacttcaggtagcagggctgggggcccgcccgggccgggggcacgtgcaggatgggcgcggcgctgtgcacgggtttgggcagtcccgacttcattttggaggcgaccaggatggccggcatcttctcccggggcttgggctttcccagcacgtccctggcagcggcggcgggggcgaccgctaaaggcagcgcgggtagcagagcaggcgccgggccttagcccacgaggcgcccaccaccagcggctaaaaaaaaaatccccaggtcggggaactcgaagcaatcgggcgagcgcgcctttggggtgccgggatgggaatgggggactggccacggcgctcagcgggtcccacctggacggatgctgccgccgggtctcacacctctcctgggtggcctttcaagagctctgggcgctcaggggctgccgcctcttgcaaatttcctcctgggaaacagaggcttggacgcccatattaacttgtcactgcatctccgaagtgaggaggcccctttggaagagacagaggcggcggcgacccacgagtcccgttccggaggctacgggtctgagccggcgagagaaagagcgagcagccaaggaaggaaaggagacagcagcgaaggaaggagagaagaagggcgcaagggtcccaagacgtctccaccgagaggcagctgccaccctgctcgcgagcaccgcagtgtcacccgcgacgcagcagaggtgcggcaagagcccccgaaaggtctctcttggggtgacagtcaccgctgcccagaaggcccccggactgagagcaccttagcgcctgcgggtctgcacatgctccgtgagctagatagaggcaaggctgtggccgtggggcgcgggcgccgggacgcgcggctggcgggccgggcagggctgcgctcgggagcggccgccgcgcttcccgggaaggctgcgctggctgcggggctcagcgcaggggag

SEQ ID NO: 17881 - RNA, 7923 nt, Homo sapiens
  source 1..7923: mol_type = other RNA
tcggcctggggaggaggaaggggagggaggatggaaacataccgtacacaaaatactcaattcctagttttctctttaaaaatggctagaaaaaattcatcaaaatgcagcactttaatcaattatttacaatttctatgttacaatgaaaaaatgtacatcttatagaacatatttcataaaactgctccactggaaacaactagatcaaaacagcaaaccttccatttaatatccacaaagttggattatttttcctttttgaagtagattcgccacaatcaaatttgaatacagagaattttgaagtttaagcatcaaacaacaaagtaaaagtccccaagatacaacaaagatctaggcaagtcttgttcctgtcccactcccaccccacccctaatgaaacttaaaaggtattcccatttcaattatggcctgtatcattcttggcagtttgggaagagaacttttggcttccattggtaactcaacataaatgttgcatagaatttatatatttcaaaattggcctaactgtagaaaaggcaaaatggaagcatttccgatagagccctaaatgagtacaaagtcactttgtaaaaggtgagtgacactaaagtaaaaatatgaccaaaataagaaatgtgcatattagacaaccctgcttcccgaaactttaggaaggacacggagttgtgagtcacacaagggctatgctacttgaagtcaatgttcaccaatcaggcagcactaggtacagaagtcttggttctgaacctggacccaggagggaagtctgtgggaaaggggagaagagaatgacaagagaggatgtcatattaaaaaaaggtttcaaacaatattggcaggtgtctactcacaaggtgattggaaaactgcccacgaggagaagtcaactttacctcctcccaaattcacagtacgcgagtgtagtagggtcattgctgggagataaattgtctgaggagggccacccttcaggtttaccagaaatcttagggtttggcccccctggtcacaggctaaatatatggtttaaaagttttattaaaaagaaaaacagaacaagacacactcacacccagatgactaatgaaggctaagcagaatagtctgagtttgctgagactaaagcagggatagtgttgaaaagttttcctttcactagtgggacacattccccttttcttttcaaagaggaagaacatggtgtcatccaatgtgaagtgagcagtttcgggtcaaactcttatggtaagaaactaaaaaaagatgccaagagacaaaccttcagaaatagaagaaatgcaaaagatggaataaaaaccctgatcattaaaacagagacaccttcactggtgtccaataaggattctctttacaaaacagaaacaaacaactcaaaaatttaccatactttgtaatgaaaataccagtatgttgaagacacagcagactgggtttctattagaacaagtatcagcaaggtcatgtagacttgtagaaacttttgccttctcctgcaccagacagatcattgtccagttgggttgtcagctggagaccgaaaagaacctaaaaaatggatctttttttttttctttttcccatggtcacgcatccacacaaatgagtcttttggatgagaaaagtcacagcaacttgagttctcctaatgaacagatgactttttagccctgtttgtttcaatggggaaaacaatgacaaaaaaaacaaaccccaggcaggcacgacacttatgtaaaatgaacacagttagtacaaaaccagtaaggcatcactttgggaaggtcagcaccgaagaggtcaggcaaggctcgtccagacggggcttctgggagggagtgaccctcacccttattgagctgcgtcatgttggttctgaggaaagtgcaagtcttttgcagggtgaccgcatcaccccaccggaagctggggcggggacgctggaggtgttggtgtgtgttctaaaccctcaaggacgagaagggaaggcaaggtccatggctcacccacatgtcgaggaccaggtcctcatccattttaaaggacacagatacccccagccctagcaggaggaggcgagtgtgtaggactgtgaggatggacaactaaaaaccaaaactgagcaggaccaaaccaaaactcaactcctgcggttcttactttcaccaaaggattgattctgaccaagaggggaagggggaaaaaaaaatcttcaaaaatcaatgcatcagaaaggaagaaactcaacctcattttcaaaaggtaacctgttctccaaagtagaacaagtctcactatacacagtgtttgcagaaaaaaaaaaaaaaaaacctgattcattcatatatcagaaggaaagagacacatgctgttctgcactgacagccacatccactcgctcacactctcactccgtcactcactctcacggatattaatcagaggctgatggacctgaatggggtggtttgattggaacaggcaaaatacctctcgggtaaggaaagcaccatttaaaaaacatgaaagcacggtttatttgctcctaaggtttccctgtgtcgtagctctgtagtgcgttgaacgtgaccaaagcaagcaccctggttagcaccagttctccctgtggccggctgtgtgggagggtgggtggcacggctctgagacccagtctggagggtctgtgctgaggggaagccgtgcttctctgtgtttccgactttgctccagtctcttctgtctctgggaagctcatggcaggatgctgtttggtttcagagcttcatgtgggttctctttttttttttctctctgtctctcttttcatttcaacggcgatgatcctttcccgagaagtatcttcagtgtcttagggaggtcacagcaacaaggcaaaacaataattaaagtacaacagaaggtagtgcagttctcgctgtggaaggaagcggtccgcaggcagctggcccgggatgcctgcacccaggtcgaggctgaaggacggggggtctcggtgttcccgcagctctaaggctgtggctgggggctggctcaggaagtcatcttcagggtgatgtgggggatgcaggtggaatgcggtgaggagaagaggagggcgctgggctccgggcccctgtcacagagtggactccaaagaggagtccaagatgtcatcgtgatggctgttgctgttggagtcgctgtcatagctctgggggctggagtagttggctgcctcctgcagcctcatcagcatgttcatcagcgggtcaccttcagcatcactggggggcatctgcttgcttgtcgatccctcccgaggcatggagtagccgtcgaagccgacatcctcaggccgtaactgcagcaggggaggccactcgtgctgttgtgggctggctgcccatggatatgtgtccatcacccacttggcaggatcctcccagggggcgcgccttccatagagctggagtccttctctgacggcttccaggagataggggataatggaatagttccacaagtcggtgaaccacactctcgagccgtccacatcgatggggcatgacaggaagagccgggggccgatggtgacgtccgaggaactgtgagcctccaggaagcggttgaggtgatgccagaccttgggaatccagtcaatgatttttaccagctccatattgcgcacccgcccactgatctctgtttccatgagcttcctcctcaggaatcggccaaggaaacccttcacaggctccgtgtggttggcacaaagcacccatctgaagttatggtgaagctgcaggttgggagtcgaagaggtagcctggttcattgtgccaattatgtaagggcatttgtggtacttgcagttgagcagcccattgaagatctctcccagagagctcacgtggtgtaggttgtccaggatgatgacgaggggcatgtccacagcattgttctcactgttgcactggtcagcaaggttggacaggtactggcgcaattccttgctggacttatggtccacgttaaaggtggcgataaccccgtctgtcaactcccgtccctctcgaagcactatatactcagacagccggttggccaggtaggttttcccagtgccgctggggccagagagaatgatccgacggtgctctatcaggagggagacgtagcgctgcaggatgggcttgggaatcaaggactcaaacaccagtgagtccaggctgttttctgcgagccctttcacagtcactgagatggtcgtgttctctccaaccagatagccacaaggaagcagctccggtgtttcggaagtgttgctgcgcttgatttctccaatgctgtagccaagaacgctgtctgaattcagccctagctgactcactgggtcgacatgaatgatgtattctttgaacagccgtctaaccaccccatcgagcacatcccacttcgtcttgccactaactccaatgcagccaataagaaagagatgtggtctggaatcctccttccacttcatttcctcctgaaagctgacaactatcttaacatgcctgcctccttccttccgagccgagcattcaccagtgtcatccagcaacatgtccaggctggttgactcagtgaggttcaagctgtgctgggagaggcccatggactgcctcggggaggcagagatggacacttgggaaggagcccggctgcagccactgccttgagactctgacttcagccgatcattctcagctttcagcttctctatttcactctgcatcctgttcatggcctcccggagctggtccagctggtgggcagaactgagagcttctaagcggatatccgtcagcttcatctccttgtctcttaactcatttcggagctgcatgacggtctcagcttcactatccatgcattctgaaattagagagttggagtgagaattcctcagcagtggggtggaacctgtggacccattgtgcggtaactttggtgaggaaggcaaagaagaatccgtcatctcctcaatatctgaatgagaggacgcagattttggggacttcttcttcccgaaagcttgcttgaaggagctgcgtaaccagttcttccgcttcttcttctttgagtcactctctatgttgctgcccacgctggagtggctggtggcactgttgatgctggagacgctgtctgaggagtgctgcctgcggatgcggaggtctgcagactgggcagtgccgtttcctttgcagttgagctcaggtgtgttaattactccattaatggcagcctgggcagctgcgttctgtttctttagcagctcaatggtttttcttaactcattcagttctgagtccttctgctcagctgtcatggtcagactctggagcctgattgtcatgttaccaagactctgttcaaaggctgccacaaggtgagcatttgctgtcagctgggtggtcaaagctgaaactttctcctgggaggcatccagttcccgccgcagcttgcgaatctctgactggcatttttcttctggtgtagaataaactgacgatgtgctggaaaccaaggagagtgaggatccatgaacttcttcaaacccatcccggaatgagcctgaacggctcatggttctgctcttctcatccagggacatggagctattccggaagcggctgtcagtgtatggatcatactgcccatcagcattggagaggctgtgagtcctcagcatggtcgggttggacaagctcatctgggtgacagtggtgggactcgcaagctgggaaaagttgaatcttgttccggagggagaagtcacgctggagccagaggaaaagggggaattggcagcggtgtcctgaaggcctcctgcagaatgggaccgtaaccattcttttgcatcttcttgcgtgcgaagctgggaggtgggagtatacctgagtcctttcttaggcaaagtgttcctatcaaggtgcgggtcactttctgacagtgtggtcttcacactgttagttctgacaaagggagtcaaggagtcgtccttggaggaggcgatgaggccagtggaagaattgtggctggggacccctccactgctgagggagatgtcgatggactcacagctggtgtggaggctgctgacagactgaaagcccaggccatccttgctaactgcggaggagctgctggcgttggtgccccaggtgaggctgttggaaggggccgagtgggctgagctggggctggaggctagcggagactggttgaggtccacattcttgctgtagagaggactgctgctcccactgctcaggacgccactgcctgacggggagtctaggttaccttgctgagtcatggtggcatgaggattggagatgaccaccgaatttttcatgttttcagctgtggcgatgggcacttgcttggtaggcttcccaccaaagagtctgcggagtgtgggagaggccacatctgggtacttggctccaggctggagactggtctgagccggactggacacaggctgggctgccggattcactttcaccgagttacaggaagccacactctcgttgtctgatgagatgcctttctccttgtctgtttggttgaccagacctggtagagagctgcctagggctgttttggaaggctccctcagtttgggcactggcaggcctgcggacttgctgctaatgttggaatctatgctgctggtgctagacctgttcccagccccgttccggctgttggacttactgggcctcggcaaactccggtactgaaggtttgtccgggagcttagggctagatacccgtcatcctgattctgagccccatccatacttgacttccgaccagcagaccgactgacgagtgcagatgactttgggattttgcccagtgtggctgacctgctggtgacagtcaccccgctggctgtgatcatggccaggccggcggcggaaccactctgcttcttgaacccaaagctgttggcattggcagtaggtgtcctagagctgctggggaggggctttttggattcgtcaccactgctccggcctgcatctgatggggagcgcttcacctgggaggctttaggagaaagccttcctttctcagacacctttgcgtcgtctgtttttccagttcctggggtcttcagtgcgcctgccggggctgaaggcttcgtccttggcatggtgatgcccacctgagctgtcatgcctcgccgccatgagcctgtctgggagatgacaggattcttcttgcccgacgtgcttttgtcggactcgtcagacacatcagaaggattccgcctccacttggaacctggctccatttttatgccgctgtctgagcctccgtctgatttcttgacatcatcaccagaccacagggaattcctctccacctgtgagtgcttctcagcatcagtctgcacatccaggttttttcgagaggaggcaggtgtgttggcataagagctgatggaggagctggtgttgatgtcatcagtgctgaggttgtctatggtgtcgctgatgccgctgctgacggagctgctgtcgtcccagcttgtaaggttcctaggccagagcatttcactacattgcggcccgtaaagcactgaatggaagggccctccatgtggtcccaggggagtttgcaacagcgggtcaaattgaagaaaatctaagaatgaaaaactactttaaatcctcacagactgcacagaaacattgcagaaagtctttccagccctaagtgctacttttaatgatgcaaaaatcattgactataacatttcttagctcattccattgacgtctgaaggcaaagcattcgattgaaaagatt

SEQ ID NO: 17882 - RNA, 12355 nt, Homo sapiens
  source 1..12355: mol_type = other RNA
tcggcctggggaggaggaaggggagggaggatggaaacataccgtacacaaaatactcaattcctagttttctctttaaaaatggctagaaaaaattcatcaaaatgcagcactttaatcaattatttacaatttctatgttacaatgaaaaaatgtacatcttatagaacatatttcataaaactgctccactggaaacaactagatcaaaacagcaaaccttccatttaatatccacaaagttggattatttttcctttttgaagtagattcgccacaatcaaatttgaatacagagaattttgaagtttaagcatcaaacaacaaagtaaaagtccccaagatacaacaaagatctaggcaagtcttgttcctgtcccactcccaccccacccctaatgaaacttaaaaggtattcccatttcaattatggcctgtatcattcttggcagtttgggaagagaacttttggcttccattggtaactcaacataaatgttgcatagaatttatatatttcaaaattggcctaactgtagaaaaggcaaaatggaagcatttccgatagagccctaaatgagtacaaagtcactttgtaaaaggtgagtgacactaaagtaaaaatatgaccaaaataagaaatgtgcatattagacaaccctgcttcccgaaactttaggaaggacacggagttgtgagtcacacaagggctatgctacttgaagtcaatgttcaccaatcaggcagcactaggtacagaagtcttggttctgaacctggacccaggagggaagtctgtgggaaaggggagaagagaatgacaagagaggatgtcatattaaaaaaaggtttcaaacaatattggcaggtgtctactcacaaggtgattggaaaactgcccacgaggagaagtcaactttacctcctcccaaattcacagtacgcgagtgtagtagggtcattgctgggagataaattgtctgaggagggccacccttcaggtttaccagaaatcttagggtttggcccccctggtcacaggctaaatatatggtttaaaagttttattaaaaagaaaaacagaacaagacacactcacacccagatgactaatgaaggctaagcagaatagtctgagtttgctgagactaaagcagggatagtgttgaaaagttttcctttcactagtgggacacattccccttttcttttcaaagaggaagaacatggtgtcatccaatgtgaagtgagcagtttcgggtcaaactcttatggtaagaaactaaaaaaagatgccaagagacaaaccttcagaaatagaagaaatgcaaaagatggaataaaaaccctgatcattaaaacagagacaccttcactggtgtccaataaggattctctttacaaaacagaaacaaacaactcaaaaatttaccatactttgtaatgaaaataccagtatgttgaagacacagcagactgggtttctattagaacaagtatcagcaaggtcatgtagacttgtagaaacttttgccttctcctgcaccagacagatcattgtccagttgggttgtcagctggagaccgaaaagaacctaaaaaatggatctttttttttttctttttcccatggtcacgcatccacacaaatgagtcttttggatgagaaaagtcacagcaacttgagttctcctaatgaacagatgactttttagccctgtttgtttcaatggggaaaacaatgacaaaaaaaacaaaccccaggcaggcacgacacttatgtaaaatgaacacagttagtacaaaaccagtaaggcatcactttgggaaggtcagcaccgaagaggtcaggcaaggctcgtccagacggggcttctgggagggagtgaccctcacccttattgagctgcgtcatgttggttctgaggaaagtgcaagtcttttgcagggtgaccgcatcaccccaccggaagctggggcggggacgctggaggtgttggtgtgtgttctaaaccctcaaggacgagaagggaaggcaaggtccatggctcacccacatgtcgaggaccaggtcctcatccattttaaaggacacagatacccccagccctagcaggaggaggcgagtgtgtaggactgtgaggatggacaactaaaaaccaaaactgagcaggaccaaaccaaaactcaactcctgcggttcttactttcaccaaaggattgattctgaccaagaggggaagggggaaaaaaaaatcttcaaaaatcaatgcatcagaaaggaagaaactcaacctcattttcaaaaggtaacctgttctccaaagtagaacaagtctcactatacacagtgtttgcagaaaaaaaaaaaaaaaaacctgattcattcatatatcagaaggaaagagacacatgctgttctgcactgacagccacatccactcgctcacactctcactccgtcactcactctcacggatattaatcagaggctgatggacctgaatggggtggtttgattggaacaggcaaaatacctctcgggtaaggaaagcaccatttaaaaaacatgaaagcacggtttatttgctcctaaggtttccctgtgtcgtagctctgtagtgcgttgaacgtgaccaaagcaagcaccctggttagcaccagttctccctgtggccggctgtgtgggagggtgggtggcacggctctgagacccagtctggagggtctgtgctgaggggaagccgtgcttctctgtgtttccgactttgctccagtctcttctgtctctgggaagctcatggcaggatgctgtttggtttcagagcttcatgtgggttctctttttttttttctctctgtctctcttttcatttcaacggcgatgatcctttcccgagaagtatcttcagtgtcttagggaggtcacagcaacaaggcaaaacaataattaaagtacaacagaaggtagtgcagttctcgctgtggaaggaagcggtccgcaggcagctggcccgggatgcctgcacccaggtcgaggctgaaggacggggggtctcggtgttcccgcagctctaaggctgtggctgggggctggctcaggaagtcatcttcagggtgatgtgggggatgcaggtggaatgcggtgaggagaagaggagggcgctgggctccgggcccctgtcacagagtggactccaaagaggagtccaagatgtcatcgtgatggctgttgctgttggagtcgctgtcatagctctgggggctggagtagttggctgcctcctgcagcctcatcagcatgttcatcagcgggtcaccttcagcatcactggggggcatctgcttgcttgtcgatccctcccgaggcatggagtagccgtcgaagccgacatcctcaggccgtaactgcagcaggggaggccactcgtgctgttgtgggctggctgcccatggatatgtgtccatcacccacttggcaggatcctcccagggggcgcgccttccatagagctggagtccttctctgacggcttccaggagataggggataatggaatagttccacaagtcggtgaaccacactctcgagccgtccacatcgatggggcatgacaggaagagccgggggccgatggtgacgtccgaggaactgtgagcctccaggaagcggttgaggtgatgccagaccttgggaatccagtcaatgatttttaccagctccatattgcgcacccgcccactgatctctgtttccatgagcttcctcctcaggaatcggccaaggaaacccttcacaggctccgtgtggttggcacaaagcacccatctgaagttatggtgaagctgcaggttgggagtcgaagaggtagcctggttcattgtgccaattatgtaagggcatttgtggtacttgcagttgagcagcccattgaagatctctcccagagagctcacgtggtgtaggttgtccaggatgatgacgaggggcatgtccacagcattgttctcactgttgcactggtcagcaaggttggacaggtactggcgcaattccttgctggacttatggtccacgttaaaggtggcgataaccccgtctgtcaactcccgtccctctcgaagcactatatactcagacagccggttggccaggtaggttttcccagtgccgctggggccagagagaatgatccgacggtgctctatcaggagggagacgtagcgctgcaggatgggcttgggaatcaaggactcaaacaccagtgagtccaggctgttttctgcgagccctttcacagtcactgagatggtcgtgttctctccaaccagatagccacaaggaagcagctccggtgtttcggaagtgttgctgcgcttgatttctccaatgctgtagccaagaacgctgtctgaattcagccctagctgactcactgggtcgacatgaatgatgtattctttgaacagccgtctaaccaccccatcgagcacatcccacttcgtcttgccactaactccaatgcagccaataagaaagagatgtggtctggaatcctccttccacttcatttcctcctgaaagctgacaactatcttaacatgcctgcctccttccttccgagccgagcattcaccagtgtcatccagcaacatgtccaggctggttgactcagtgaggttcaagctgtgctgggagaggcccatggactgcctcggggaggcagagatggacacttgggaaggagcccggctgcagccactgccttgagactctgacttcagccgatcattctcagctttcagcttctctatttcactctgcatcctgttcatggcctcccggagctggtccagctggtgggcagaactgagagcttctaagcggatatccgtcagcttcatctccttgtctcttaactcatttcggagctgcatgacggtctcagcttcactatccatgcattctgaaattagagagttggagtgagaattcctcagcagtggggtggaacctgtggacccattgtgcggtaactttggtgaggaaggcaaagaagaatccgtcatctcctcaatatctgaatgagaggacgcagattttggggacttcttcttcccgaaagcttgcttgaaggagctgcgtaaccagttcttccgcttcttcttctttgagtcactctctatgttgctgcccacgctggagtggctggtggcactgttgatgctggagacgctgtctgaggagtgctgcctgcggatgcggaggtctgcagactgggcagtgccgtttcctttgcagttgagctcaggtgtgttaattactccattaatggcagcctgggcagctgcgttctgtttctttagcagctcaatggtttttcttaactcattcagttctgagtccttctgctcagctgtcatggtcagactctggagcctgattgtcatgttaccaagactctgttcaaaggctgccacaaggtgagcatttgctgtcagctgggtggtcaaagctgaaactttctcctgggaggcatccagttcccgccgcagcttgcgaatctctgactggcatttttcttctggtgtagaataaactgacgatgtgctggaaaccaaggagagtgaggatccatgaacttcttcaaacccatcccggaatgagcctgaacggctcatggttctgctcttctcatccagggacatggagctattccggaagcggctgtcagtgtatggatcatactgcccatcagcattggagaggctgtgagtcctcagcatggtcgggttggacaagctcatctgggtgacagtggtgggactcgcaagctgggaaaagttgaatcttgttccggagggagaagtcacgctggagccagaggaaaagggggaattggcagcggtgtcctgaaggcctcctgcagaatgggaccgtaaccattcttttgcatcttcttgcgtgcgaagctgggaggtgggagtatacctgagtcctttcttaggcaaagtgttcctatcaaggtgcgggtcactttctgacagtgtggtcttcacactgttagttctgacaaagggagtcaaggagtcgtccttggaggaggcgatgaggccagtggaagaattgtggctggggacccctccactgctgagggagatgtcgatggactcacagctggtgtggaggctgctgacagactgaaagcccaggccatccttgctaactgcggaggagctgctggcgttggtgccccaggtgaggctgttggaaggggccgagtgggctgagctggggctggaggctagcggagactggttgaggtccacattcttgctgtagagaggactgctgctcccactgctcaggacgccactgcctgacggggagtctaggttaccttgctgagtcatggtggcatgaggattggagatgaccaccgaatttttcatgttttcagctgtggcgatgggcacttgcttggtaggcttcccaccaaagagtctgcggagtgtgggagaggccacatctgggtacttggctccaggctggagactggtctgagccggactggacacaggctgggctgccggattcactttcaccgagttacaggaagccacactctcgttgtctgatgagatgcctttctccttgtctgtttggttgaccagacctggtagagagctgcctagggctgttttggaaggctccctcagtttgggcactggcaggcctgcggacttgctgctaatgttggaatctatgctgctggtgctagacctgttcccagccccgttccggctgttggacttactgggcctcggcaaactccggtactgaaggtttgtccgggagcttagggctagatacccgtcatcctgattctgagccccatccatacttgacttccgaccagcagaccgactgacgagtgcagatgactttgggattttgcccagtgtggctgacctgctggtgacagtcaccccgctggctgtgatcatggccaggccggcggcggaaccactctgcttcttgaacccaaagctgttggcattggcagtaggtgtcctagagctgctggggaggggctttttggattcgtcaccactgctccggcctgcatctgatggggagcgcttcacctgggaggctttaggagaaagccttcctttctcagacacctttgcgtcgtctgtttttccagttcctggggtcttcagtgcgcctgccggggctgaaggcttcgtccttggcatggtgatgcccacctgagctgtcatgcctcgccgccatgagcctgtctgggagatgacaggattcttcttgcccgacgtgcttttgtcggactcgtcagacacatcagaaggattccgcctccacttggaacctggctccatttttatgccgctgtctgagcctccgtctgatttcttgacatcatcaccagaccacagggaattcctctccacctgtgagtgcttctcagcatcagtctgcacatccaggttttttcgagaggaggcaggtgtgttggcataagagctgatggaggagctggtgttgatgtcatcagtgctgaggttgtctatggtgtcgctgatgccgctgctgacggagctgctgtcgtcccagcttgtaaggttcctaggccagagcatttcactacattgcggcccttggagaacagcggacaaagaagctgaatgaatctcacaggatggcaagtcctttagccagctgagccagcccacactgggccagggaatcccaggcacccagcaactctgtaactaaaggactagctagcagggatcaccattccccaggccaggaaagaaatccgatcccccaacaaaattaacctctgaagtgctgaaggatcgagaggtcaggcctcagtgctggtatcaagtcagctgtgaaaagtttcagcaaagcaaaagctaacaccaaactctgaaaccattaccgtaaagcactgaatggaagggccctccatgtggtcccaggggagtttgcaacagcgggtcaaattgaagaaaatctaagaatgaaaaactactttaaatcctcacagactgcacagaaacattgcagaaagtctttccagccctaagtgctacttttaatgatgcaaaaatcattgactataacatttcttagctcattccattgacgtctgaaggcaaagcattcgattgaaaagattagcctacagagagaatttctgaacctaaaaaggaaatgatacctgtttgtacagttaacaacgacacacatacattatttccggtgatgtcaattttgatgcagtgccaacaaaaatatgcattaattccgcaggctacttatttcaaaagaaaaagaatctcagtctaggcatggctacattaaacattatggtacagaggctggaaggggaggtgggtgggagagagtcccagctctgggatgggaaggggttgcatggactaatccctattaaaacctgtaatcaaggcactcagaaagaactatgtaaacagatgctatgaacaatgaacaactgtattactactgagaactcaaaagcaaacttatgttatagccacaagctttatttgaaaacgaaggattaagatgttctccaaaaccctgactccctctccaaaaatcctaccagttggttcctggtagctttcaaagactttccccaagaaaggctctccccctggccagggtggcctctccagtggaagcagggagcgggggttgtggccctgggggatggttagggaaggaagcagtaactggctccaagcgaggtctctgtgtggtcagcatttgctcagcaaacagaagctttcaaaggggaatgaagagccattcctctcccactgaaaagggagggaataaaagatctgctcaaagaggagaggagggtctggtggtgattcccaggtgaatgaaaaaaagattgtaatctcgaaggagtcccaaccaaagttaatcattcacatctcatccttcagggccctcgtccacttgaaatactgctgaggcatctgccgtggggagtgggaagcagaggtgggggtgggcagtgggtgagtttgagggaaggagtagtgtccagatatattaagacaaaaaagttgggacagacccaagttctggctgacaaggatgcttcaaaccaccccttaccttctatgctgtccctggaactgactgtatctttacgatattacttctttgagaatctgtccaacatccgagttaacttgggaatgggatggtgattgtgtgtatggagacacacaggcacatgggcacagatgcacacacacgctctaaaaagtttccattgtttcctcgctctaggcaaacataataggtaaacattctgatttgtcatcaaggtaagctaggaaatgttgatgtattcatttattcattcatcaactaccatatttataaagcatctgcaatgtggcaagtgctgttctaagtgcagaagatacaagcagtcaacaaaatagaccaaaaatctcaactctaatggaacttagcttcagtggtagaactataaaataaatgagacaaaatgtaaattttacagtacattagcaataaatgctcgggagaacaacgtattgtaaagaagaagatgtgatttgtcaaggtggggtgtgggaaattttacatgggctggctatggcaggtctgctgagggcatggtttttattacaaatctaaaagaagtatgggagctgggtatctgaatacctggggataagggactttcaagagaggaaatggtcagtgcaaaggccctgagatagtatacgacttgcaatgcattccaagaatgagtggctggagcagtgagcggtgaaccaaagtggggtgaggagggggtcaggccagagagtccaagggtacagcgagagaggagagtgcctaaatggggccctgcaagtcagcgtaagcagcttgtcttttactctgagggagagaggatacattggaggtttaatagatggagtttcttctttttataaaagttcatgtaaatgtacaacactaaacatatcgttttgattacacatgatttttacaggggtgagtttattgtaggagacatagtgctttaaggaggtcttagttttctttctatggttaaaagaatcacacctttcatgttagaggctctgaattatttgcagctacaggttctaattgagtcagggttttctcatggtttgaaagataataattagtagggataagggagacccaggcaacgagagaggaaaagggaaagtaaaccaactccatgagggcagatgccctttggcgcttttcaagagccaggattgctctgtcatttttgacgcttgcttctaaacaggccaaattccaaagggctcccagaactcataacacttttctccacagaaacaatgttatcagtgatgttaaggtttccaggttactcacagagccatctataaaaccaagatgtagttgatgaactctactcaggtatcaaagagtagaagaaaactttattcttggaatacagtacataattagacaaaacagaaaaccacaaatctaaaaagatgttcacttatttctaatgagtattttatgaaaacaatgctagtgaagacacttcgttccttttcttccaacatattcaaccctctttcctggcttttccctgcaggctgaaaaatatatcactaatctcatcaaatcaaacaaaaacttttttttttttttacctcatgcccatattctcctccactcctttgaggtgttttcctgtacttctcatgttccgtgatccttcaacccaccaggcaagatgtttgttcccactactccactgagaccactttctcttttccctgagaacatcaatggcttcctccttgccaaagccaatggtcaactctctgtccttaccctacttgagttttcagcagcaggtagcatcgacagattctcccttcttgagtgggcctcatcccgggtttccatactgtcatctgtacctggttcctacctccctaactgcgcttctcaatctcctaggctcaccctcctcttcacctctccagaactccagggcctccatccctggacccctcctcttctctaactataacttctcactaacttctaactaagttataactaccacttctaactaacttcttttcctgggtgatctcatccatggcttcaaatactaggtgaaggcagacaactctaaagtctgtaatctctagcctggcccctttgtgtacccaacacatctgaaatcaaatttaccttactcaaaactattgctcccaacttccaatgtgtccgcacccccactcccaaagtcttctgtatctcagaatatgactctacattaacagtcctaattctctccctccttcttgcctccgatgtaatccattaagaaggccttttgcctagagtccccaaatataccttgaacccaatcactactgaacatctgcaataagataaccttggaccaagatgccatcatctctttcctgcaacagacacctcccgggtcgctcagccttccctcatgccttgctaggctccatcctgcacaccccaggggcagcaatctttctccagtgtacagcagattctgtcacattcctgcttaaagcccactgatagcttcccagggaacttagaataaaattcaaatttgttcccttggcctagaagccctgatgtgatctggcttctcctcttcattacgtccaaagacaggacccacaaatgcaccaagcttcttcccacttcctaggccctcgcactgtgcctcctttctggaatgctcctccccatgtctcccactggcggcccacttctcacgggtcagatgttggttggaatggcacctcctcagggatttcctcttagactctggcccaattacattccaccatatgattttcttcatggcatcaaccagtcaacacattgtctttcaacagtctgtctttccctcaacacagggagctcctcgagcacaggtgtactgtttgcctttgttctgagccatatcctcccagtgcctaaatcactgctgatgtggtcctggatcaaccaagcataggaggacaaaatggaactgattattccatgcagtctcctggggactgtgtagtacttccaaggactttagttcaatggttttatttggtcacagacccacttaggggcccgtctctccataagaaaaaagatacacaaacaatattttacacagaatttccagggactcactgatcccctgaatcctgtccataaagcccaggtta

SEQ ID NO: 17883 - RNA, 11288 nt, Homo sapiens
  source 1..11288: mol_type = other RNA
tcggcctggggaggaggaaggggagggaggatggaaacataccgtacacaaaatactcaattcctagttttctctttaaaaatggctagaaaaaattcatcaaaatgcagcactttaatcaattatttacaatttctatgttacaatgaaaaaatgtacatcttatagaacatatttcataaaactgctccactggaaacaactagatcaaaacagcaaaccttccatttaatatccacaaagttggattatttttcctttttgaagtagattcgccacaatcaaatttgaatacagagaattttgaagtttaagcatcaaacaacaaagtaaaagtccccaagatacaacaaagatctaggcaagtcttgttcctgtcccactcccaccccacccctaatgaaacttaaaaggtattcccatttcaattatggcctgtatcattcttggcagtttgggaagagaacttttggcttccattggtaactcaacataaatgttgcatagaatttatatatttcaaaattggcctaactgtagaaaaggcaaaatggaagcatttccgatagagccctaaatgagtacaaagtcactttgtaaaaggtgagtgacactaaagtaaaaatatgaccaaaataagaaatgtgcatattagacaaccctgcttcccgaaactttaggaaggacacggagttgtgagtcacacaagggctatgctacttgaagtcaatgttcaccaatcaggcagcactaggtacagaagtcttggttctgaacctggacccaggagggaagtctgtgggaaaggggagaagagaatgacaagagaggatgtcatattaaaaaaaggtttcaaacaatattggcaggtgtctactcacaaggtgattggaaaactgcccacgaggagaagtcaactttacctcctcccaaattcacagtacgcgagtgtagtagggtcattgctgggagataaattgtctgaggagggccacccttcaggtttaccagaaatcttagggtttggcccccctggtcacaggctaaatatatggtttaaaagttttattaaaaagaaaaacagaacaagacacactcacacccagatgactaatgaaggctaagcagaatagtctgagtttgctgagactaaagcagggatagtgttgaaaagttttcctttcactagtgggacacattccccttttcttttcaaagaggaagaacatggtgtcatccaatgtgaagtgagcagtttcgggtcaaactcttatggtaagaaactaaaaaaagatgccaagagacaaaccttcagaaatagaagaaatgcaaaagatggaataaaaaccctgatcattaaaacagagacaccttcactggtgtccaataaggattctctttacaaaacagaaacaaacaactcaaaaatttaccatactttgtaatgaaaataccagtatgttgaagacacagcagactgggtttctattagaacaagtatcagcaaggtcatgtagacttgtagaaacttttgccttctcctgcaccagacagatcattgtccagttgggttgtcagctggagaccgaaaagaacctaaaaaatggatctttttttttttctttttcccatggtcacgcatccacacaaatgagtcttttggatgagaaaagtcacagcaacttgagttctcctaatgaacagatgactttttagccctgtttgtttcaatggggaaaacaatgacaaaaaaaacaaaccccaggcaggcacgacacttatgtaaaatgaacacagttagtacaaaaccagtaaggcatcactttgggaaggtcagcaccgaagaggtcaggcaaggctcgtccagacggggcttctgggagggagtgaccctcacccttattgagctgcgtcatgttggttctgaggaaagtgcaagtcttttgcagggtgaccgcatcaccccaccggaagctggggcggggacgctggaggtgttggtgtgtgttctaaaccctcaaggacgagaagggaaggcaaggtccatggctcacccacatgtcgaggaccaggtcctcatccattttaaaggacacagatacccccagccctagcaggaggaggcgagtgtgtaggactgtgaggatggacaactaaaaaccaaaactgagcaggaccaaaccaaaactcaactcctgcggttcttactttcaccaaaggattgattctgaccaagaggggaagggggaaaaaaaaatcttcaaaaatcaatgcatcagaaaggaagaaactcaacctcattttcaaaaggtaacctgttctccaaagtagaacaagtctcactatacacagtgtttgcagaaaaaaaaaaaaaaaaacctgattcattcatatatcagaaggaaagagacacatgctgttctgcactgacagccacatccactcgctcacactctcactccgtcactcactctcacggatattaatcagaggctgatggacctgaatggggtggtttgattggaacaggcaaaatacctctcgggtaaggaaagcaccatttaaaaaacatgaaagcacggtttatttgctcctaaggtttccctgtgtcgtagctctgtagtgcgttgaacgtgaccaaagcaagcaccctggttagcaccagttctccctgtggccggctgtgtgggagggtgggtggcacggctctgagacccagtctggagggtctgtgctgaggggaagccgtgcttctctgtgtttccgactttgctccagtctcttctgtctctgggaagctcatggcaggatgctgtttggtttcagagcttcatgtgggttctctttttttttttctctctgtctctcttttcatttcaacggcgatgatcctttcccgagaagtatcttcagtgtcttagggaggtcacagcaacaaggcaaaacaataattaaagtacaacagaaggtagtgcagttctcgctgtggaaggaagcggtccgcaggcagctggcccgggatgcctgcacccaggtcgaggctgaaggacggggggtctcggtgttcccgcagctctaaggctgtggctgggggctggctcaggaagtcatcttcagggtgatgtgggggatgcaggtggaatgcggtgaggagaagaggagggcgctgggctccgggcccctgtcacagagtggactccaaagaggagtccaagatgtcatcgtgatggctgttgctgttggagtcgctgtcatagctctgggggctggagtagttggctgcctcctgcagcctcatcagcatgttcatcagcgggtcaccttcagcatcactggggggcatctgcttgcttgtcgatccctcccgaggcatggagtagccgtcgaagccgacatcctcaggccgtaactgcagcaggggaggccactcgtgctgttgtgggctggctgcccatggatatgtgtccatcacccacttggcaggatcctcccagggggcgcgccttccatagagctggagtccttctctgacggcttccaggagataggggataatggaatagttccacaagtcggtgaaccacactctcgagccgtccacatcgatggggcatgacaggaagagccgggggccgatggtgacgtccgaggaactgtgagcctccaggaagcggttgaggtgatgccagaccttgggaatccagtcaatgatttttaccagctccatattgcgcacccgcccactgatctctgtttccatgagcttcctcctcaggaatcggccaaggaaacccttcacaggctccgtgtggttggcacaaagcacccatctgaagttatggtgaagctgcaggttgggagtcgaagaggtagcctggttcattgtgccaattatgtaagggcatttgtggtacttgcagttgagcagcccattgaagatctctcccagagagctcacgtggtgtaggttgtccaggatgatgacgaggggcatgtccacagcattgttctcactgttgcactggtcagcaaggttggacaggtactggcgcaattccttgctggacttatggtccacgttaaaggtggcgataaccccgtctgtcaactcccgtccctctcgaagcactatatactcagacagccggttggccaggtaggttttcccagtgccgctggggccagagagaatgatccgacggtgctctatcaggagggagacgtagcgctgcaggatgggcttgggaatcaaggactcaaacaccagtgagtccaggctgttttctgcgagccctttcacagtcactgagatggtcgtgttctctccaaccagatagccacaaggaagcagctccggtgtttcggaagtgttgctgcgcttgatttctccaatgctgtagccaagaacgctgtctgaattcagccctagctgactcactgggtcgacatgaatgatgtattctttgaacagccgtctaaccaccccatcgagcacatcccacttcgtcttgccactaactccaatgcagccaataagaaagagatgtggtctggaatcctccttccacttcatttcctcctgaaagctgacaactatcttaacatgcctgcctccttccttccgagccgagcattcaccagtgtcatccagcaacatgtccaggctggttgactcagtgaggttcaagctgtgctgggagaggcccatggactgcctcggggaggcagagatggacacttgggaaggagcccggctgcagccactgccttgagactctgacttcagccgatcattctcagctttcagcttctctatttcactctgcatcctgttcatggcctcccggagctggtccagctggtgggcagaactgagagcttctaagcggatatccgtcagcttcatctccttgtctcttaactcatttcggagctgcatgacggtctcagcttcactatccatgcattctgaaattagagagttggagtgagaattcctcagcagtggggtggaacctgtggacccattgtgcggtaactttggtgaggaaggcaaagaagaatccgtcatctcctcaatatctgaatgagaggacgcagattttggggacttcttcttcccgaaagcttgcttgaaggagctgcgtaaccagttcttccgcttcttcttctttgagtcactctctatgttgctgcccacgctggagtggctggtggcactgttgatgctggagacgctgtctgaggagtgctgcctgcggatgcggaggtctgcagactgggcagtgccgtttcctttgcagttgagctcaggtgtgttaattactccattaatggcagcctgggcagctgcgttctgtttctttagcagctcaatggtttttcttaactcattcagttctgagtccttctgctcagctgtcatggtcagactctggagcctgattgtcatgttaccaagactctgttcaaaggctgccacaaggtgagcatttgctgtcagctgggtggtcaaagctgaaactttctcctgggaggcatccagttcccgccgcagcttgcgaatctctgactggcatttttcttctggtgtagaataaactgacgatgtgctggaaaccaaggagagtgaggatccatgaacttcttcaaacccatcccggaatgagcctgaacggctcatggttctgctcttctcatccagggacatggagctattccggaagcggctgtcagtgtatggatcatactgcccatcagcattggagaggctgtgagtcctcagcatggtcgggttggacaagctcatctgggtgacagtggtgggactcgcaagctgggaaaagttgaatcttgttccggagggagaagtcacgctggagccagaggaaaagggggaattggcagcggtgtcctgaaggcctcctgcagaatgggaccgtaaccattcttttgcatcttcttgcgtgcgaagctgggaggtgggagtatacctttctgacagtgtggtcttcacactgttagttctgacaaagggagtcaaggagtcgtccttggaggaggcgatgaggccagtggaagaattgtggctggggacccctccactgctgagggagatgtcgatggactcacagctggtgtggaggctgctgacagactgaaagcccaggccatccttgctaactgcggaggagctgctggcgttggtgccccaggtgaggctgttggaaggggccgagtgggctgagctggggctggaggctagcggagactggttgaggtccacattcttgctgtagagaggactgctgctcccactgctcaggacgccactgcctgacggggagtctaggttaccttgctgagtcatggtggcatgaggattggagatgaccaccgaatttttcatgttttcagctgtggcgatgggcacttgcttggtaggcttcccaccaaagagtctgcggagtgtgggagaggccacatctgggtacttggctccaggctggagactggtctgagccggactggacacaggctgggctgccggattcactttcaccgagttacaggaagccacactctcgttgtctgatgagatgcctttctccttgtctgtttggttgaccagacctggtagagagctgcctagggctgttttggaaggctccctcagtttgggcactggcaggcctgcggacttgctgctaatgttggaatctatgctgctggtgctagacctgttcccagccccgttccggctgttggacttactgggcctcggcaaactccggtactgaaggtttgtccgggagcttagggctagatacccgtcatcctgattctgagccccatccatacttgacttccgaccagcagaccgactgacgagtgcagatgactttgggattttgcccagtgtggctgacctgctggtgacagtcaccccgctggctgtgatcatggccaggccggcggcggaaccactctgcttcttgaacccaaagctgttggcattggcagtaggtgtcctagagctgctggggaggggctttttggattcgtcaccactgctccggcctgcatctgatggggagcgcttcacctgggaggctttaggagaaagccttcctttctcagacacctttgcgtcgtctgtttttccagttcctggggtcttcagtgcgcctgccggggctgaaggcttcgtccttggcatggtgatgcccacctgagctgtcatgcctcgccgccatgagcctgtctgggagatgacaggattcttcttgcccgacgtgcttttgtcggactcgtcagacacatcagaaggattccgcctccacttggaacctggctccatttttatgccgctgtctgagcctccgtctgatttcttgacatcatcaccagaccacagggaattcctctccacctgtgagtgcttctcagcatcagtctgcacatccaggttttttcgagaggaggcaggtgtgttggcataagagctgatggaggagctggtgttgatgtcatcagtgctgaggttgtctatggtgtcgctgatgccgctgctgacggagctgctgtcgtcccagctgtcagcgtctccgaggcccagggaggtatttcgttgcagggtctcccgtaccacagccatcccatcagggagccggttcaggcgacgggtatagaggccaagtccaccatcagtcatgtatccgcttgtaatgtcatcggtccggatgttcttgctcagaacatccccgtcgctcatgtagccgggggcatccatgctgatgccttccaggtccatctcatctcctgccttgtctgagacgtccacatggcagacactactgccccgggaggccagctgccttctcagaggggcggagtacacatagcgacctgactcagtgttgatgaacctgctggcgttggctcgagggggatacccattgcccattgagggggcgtctcctgcttggagccgagggctggactggcccagtctccaggacagaggtgtgggcctccctgtcaagctgagtatgctacggccactcatctccgtggtgacattggtgtcaaacgtggtttccaatgtgctgtgtgtaacctgagttccccttaaactggacatggtttcctccaaattctgccgcagatcagcgatgttcttcactgtccgcagccgccgagcctcaggatcttccccagtgagttcttccagagcaggctgtccagtcttggtgaagtggctgggctccacgctcacacctgttgagcttgactcggcagtaacattcccttcagtgtccgtctgagacctgtacaggaaaggtgcaaccgtggcagtgttgggatggttgtattgctgctggggctgaggtagctgaacactgacggtattgcttcctgtggtctgggtggtcccgacagacccactgacagtctggctgctgatgctgtggttcagggtggtccctcctgggccttttccttctgaggacgccaggctggaagaggaactggagtgtctgccgtccagctggggcttctgctgggggagtcctgagctcagcttcccactccggctccgctccccttccttggaaggcgctggggcacttggggatttcccgggcatgcttttcattcctggttttggtattccactgtgggaaggggccatgggctccttcttggcactgttgagcttcccccctttggggatgaagctggcaatcttggaggacttttttggcatctcgggcacagctgctccactggggtcttcttttggctcctccttgaggtccagcctctccgtcacagaggctctcttggcaaggtccttgcttttctccttatccttctcccgctgttgtttctccttctctttctcattgcctttcagagaactcttcttgttggtcagtgcccggctaaaagtcctctgggcaatgcccttgagtgcaatcttggggctgctggaagcagggcccacggtggtgagcatgcgactggcggcctccagctcctcgctctcttcgaagctgggcagagtctccagccgctcacagcttgtgtcccgggaccccggcccctcacctgcctttgagccccctttactgttgaaaagtttcagcttttccagcatggacttctgattgttgggggccggcttcatggcttcaggtgtgggcctgggggcctcaggcccaggaggcttgaccgagagcatggataccgtggcactgtgcttcacgctgagggatttgctgcgccaaggcttggtggctgcaccgggctgcgggatggccgaggaggtactgcaattagtaggggtggagctgctgccgctctccaaggaagcaggtgcattgtcactcattccggggtgggaggaggctgaacttgccaaaggctctttctcgtggctgcttggcggtgggggtggggaggtgactggtttggatttatcatagttgttaaagctctggctgcgtcggttgttagcagtagttgaccctccgcgtgttttggcctcgctgcctgcagcggataccctcgcggtaggacctggaagtctagagatctttttctgacccagagtgaagcggatgattttgctttgagatgagtccttggatgatgcactggactgcatttcagcttgtgcttttgactgctgatgtggcgctggctggtgaggctggcacggggcttggggagtgactggcacctgctgctgaggggtgccagcctggcactgggagggggccccggccacctgggatacggcgggcggcagaggtgaggagaggtgctgcttctggggctgctgctgctgctgcttgtatcgggagaggctgaagaagaggcctagaatggccttgaggtttccattcctgatctcttctgcagacagcccctggatgtttattcccttagctgccaggaaattcaagcaggcatctatgttttcaatcatttgggatctgttcttcggacagccattgatgtcttcaatcttttcatttgccacaacctggataatctgggccaggaggacgccatctgtcacatcttgctggagatccctgatgagacgcttgtggccggatttggctaggtaatgattggcccagtctgtgtagatctgggtatcgaacccgttttccaccgagccgctcttccgcagcgggagcccctcccccgctggctcctgcagcccctgcagcacctgcgatttcagggggatctggctaggataggtggtcttgctcacctccaccttgcttcccaacttcaggtagcagggctgggggcccgcccgggccgggggcacgtgcaggatgggcgcggcgctgtgcacgggtttgggcagtcccgacttcattttggaggcgaccaggatggccggcatcttctcccggggcttgggctttcccagcacgtccctggcagcggcggcgggggcgaccgctaaaggcagcgcgggtagcagagcaggcgccgggccttagcccacgaggcgcccaccaccagcggctaaaaaaaaaatccccaggtcggggaactcgaagcaatcgggcgagcgcgcctttggggtgccgggatgggaatgggggactggccacggcgctcagcgggtcccacctggacggatgctgccgccgggtctcacacctctcctgggtggcctttcaagagctctgggcgctcaggggctgccgcctcttgcaaatttcctcctgggaaacagaggcttggacgcccatattaacttgtcactgcatctccgaagtgaggaggcccctttggaagagacagaggcggcggcgacccacgagtcccgttccggaggctacgggtctgagccggcgagagaaagagcgagcagccaaggaaggaaaggagacagcagcgaaggaaggagagaagaagggcgcaagggtcccaagacgtctccaccgagaggcagctgccaccctgctcgcgagcaccgcagtgtcacccgcgacgcagcagaggtgcggcaagagcccccgaaaggtctctcttggggtgacagtcaccgctgcccagaaggcccccggactgagagcaccttagcgcctgcgggtctgcacatgctccgtgagctagatagaggcaaggctgtggccgtggggcgcgggcgccgggacgcgcggctggcgggccgggcagggctgcgctcgggagcggccgccgcgcttcccgggaaggctgcgctggctgcggggctcagcgcaggggag

SEQ ID NO: 17884 - RNA, 8027 nt, Homo sapiens
  source 1..8027: mol_type = other RNA
tcggcctggggaggaggaaggggagggaggatggaaacataccgtacacaaaatactcaattcctagttttctctttaaaaatggctagaaaaaattcatcaaaatgcagcactttaatcaattatttacaatttctatgttacaatgaaaaaatgtacatcttatagaacatatttcataaaactgctccactggaaacaactagatcaaaacagcaaaccttccatttaatatccacaaagttggattatttttcctttttgaagtagattcgccacaatcaaatttgaatacagagaattttgaagtttaagcatcaaacaacaaagtaaaagtccccaagatacaacaaagatctaggcaagtcttgttcctgtcccactcccaccccacccctaatgaaacttaaaaggtattcccatttcaattatggcctgtatcattcttggcagtttgggaagagaacttttggcttccattggtaactcaacataaatgttgcatagaatttatatatttcaaaattggcctaactgtagaaaaggcaaaatggaagcatttccgatagagccctaaatgagtacaaagtcactttgtaaaaggtgagtgacactaaagtaaaaatatgaccaaaataagaaatgtgcatattagacaaccctgcttcccgaaactttaggaaggacacggagttgtgagtcacacaagggctatgctacttgaagtcaatgttcaccaatcaggcagcactaggtacagaagtcttggttctgaacctggacccaggagggaagtctgtgggaaaggggagaagagaatgacaagagaggatgtcatattaaaaaaaggtttcaaacaatattggcaggtgtctactcacaaggtgattggaaaactgcccacgaggagaagtcaactttacctcctcccaaattcacagtacgcgagtgtagtagggtcattgctgggagataaattgtctgaggagggccacccttcaggtttaccagaaatcttagggtttggcccccctggtcacaggctaaatatatggtttaaaagttttattaaaaagaaaaacagaacaagacacactcacacccagatgactaatgaaggctaagcagaatagtctgagtttgctgagactaaagcagggatagtgttgaaaagttttcctttcactagtgggacacattccccttttcttttcaaagaggaagaacatggtgtcatccaatgtgaagtgagcagtttcgggtcaaactcttatggtaagaaactaaaaaaagatgccaagagacaaaccttcagaaatagaagaaatgcaaaagatggaataaaaaccctgatcattaaaacagagacaccttcactggtgtccaataaggattctctttacaaaacagaaacaaacaactcaaaaatttaccatactttgtaatgaaaataccagtatgttgaagacacagcagactgggtttctattagaacaagtatcagcaaggtcatgtagacttgtagaaacttttgccttctcctgcaccagacagatcattgtccagttgggttgtcagctggagaccgaaaagaacctaaaaaatggatctttttttttttctttttcccatggtcacgcatccacacaaatgagtcttttggatgagaaaagtcacagcaacttgagttctcctaatgaacagatgactttttagccctgtttgtttcaatggggaaaacaatgacaaaaaaaacaaaccccaggcaggcacgacacttatgtaaaatgaacacagttagtacaaaaccagtaaggcatcactttgggaaggtcagcaccgaagaggtcaggcaaggctcgtccagacggggcttctgggagggagtgaccctcacccttattgagctgcgtcatgttggttctgaggaaagtgcaagtcttttgcagggtgaccgcatcaccccaccggaagctggggcggggacgctggaggtgttggtgtgtgttctaaaccctcaaggacgagaagggaaggcaaggtccatggctcacccacatgtcgaggaccaggtcctcatccattttaaaggacacagatacccccagccctagcaggaggaggcgagtgtgtaggactgtgaggatggacaactaaaaaccaaaactgagcaggaccaaaccaaaactcaactcctgcggttcttactttcaccaaaggattgattctgaccaagaggggaagggggaaaaaaaaatcttcaaaaatcaatgcatcagaaaggaagaaactcaacctcattttcaaaaggtaacctgttctccaaagtagaacaagtctcactatacacagtgtttgcagaaaaaaaaaaaaaaaaacctgattcattcatatatcagaaggaaagagacacatgctgttctgcactgacagccacatccactcgctcacactctcactccgtcactcactctcacggatattaatcagaggctgatggacctgaatggggtggtttgattggaacaggcaaaatacctctcgggtaaggaaagcaccatttaaaaaacatgaaagcacggtttatttgctcctaaggtttccctgtgtcgtagctctgtagtgcgttgaacgtgaccaaagcaagcaccctggttagcaccagttctccctgtggccggctgtgtgggagggtgggtggcacggctctgagacccagtctggagggtctgtgctgaggggaagccgtgcttctctgtgtttccgactttgctccagtctcttctgtctctgggaagctcatggcaggatgctgtttggtttcagagcttcatgtgggttctctttttttttttctctctgtctctcttttcatttcaacggcgatgatcctttcccgagaagtatcttcagtgtcttagggaggtcacagcaacaaggcaaaacaataattaaagtacaacagaaggtagtgcagttctcgctgtggaaggaagcggtccgcaggcagctggcccgggatgcctgcacccaggtcgaggctgaaggacggggggtctcggtgttcccgcagctctaaggctgtggctgggggctggctcaggaagtcatcttcagggtgatgtgggggatgcaggtggaatgcggtgaggagaagaggagggcgctgggctccgggcccctgtcacagagtggactccaaagaggagtccaagatgtcatcgtgatggctgttgctgttggagtcgctgtcatagctctgggggctggagtagttggctgcctcctgcagcctcatcagcatgttcatcagcgggtcaccttcagcatcactggggggcatctgcttgcttgtcgatccctcccgaggcatggagtagccgtcgaagccgacatcctcaggccgtaactgcagcaggggaggccactcgtgctgttgtgggctggctgcccatggatatgtgtccatcacccacttggcaggatcctcccagggggcgcgccttccatagagctggagtccttctctgacggcttccaggagataggggataatggaatagttccacaagtcggtgaaccacactctcgagccgtccacatcgatggggcatgacaggaagagccgggggccgatggtgacgtccgaggaactgtgagcctccaggaagcggttgaggtgatgccagaccttgggaatccagtcaatgatttttaccagctccatattgcgcacccgcccactgatctctgtttccatgagcttcctcctcaggaatcggccaaggaaacccttcacaggctccgtgtggttggcacaaagcacccatctgaagttatggtgaagctgcaggttgggagtcgaagaggtagcctggttcattgtgccaattatgtaagggcatttgtggtacttgcagttgagcagcccattgaagatctctcccagagagctcacgtggtgtaggttgtccaggatgatgacgaggggcatgtccacagcattgttctcactgttgcactggtcagcaaggttggacaggtactggcgcaattccttgctggacttatggtccacgttaaaggtggcgataaccccgtctgtcaactcccgtccctctcgaagcactatatactcagacagccggttggccaggtaggttttcccagtgccgctggggccagagagaatgatccgacggtgctctatcaggagggagacgtagcgctgcaggatgggcttgggaatcaaggactcaaacaccagtgagtccaggctgttttctgcgagccctttcacagtcactgagatggtcgtgttctctccaaccagatagccacaaggaagcagctccggtgtttcggaagtgttgctgcgcttgatttctccaatgctgtagccaagaacgctgtctgaattcagccctagctgactcactgggtcgacatgaatgatgtattctttgaacagccgtctaaccaccccatcgagcacatcccacttcgtcttgccactaactccaatgcagccaataagaaagagatgtggtctggaatcctccttccacttcatttcctcctgaaagctgacaactatcttaacatgcctgcctccttccttccgagccgagcattcaccagtgtcatccagcaacatgtccaggctggttgactcagtgaggttcaagctgtgctgggagaggcccatggactgcctcggggaggcagagatggacacttgggaaggagcccggctgcagccactgccttgagactctgacttcagccgatcattctcagctttcagcttctctatttcactctgcatcctgttcatggcctcccggagctggtccagctggtgggcagaactgagagcttctaagcggatatccgtcagcttcatctccttgtctcttaactcatttcggagctgcatgacggtctcagcttcactatccatgcattctgaaattagagagttggagtgagaattcctcagcagtggggtggaacctgtggacccattgtgcggtaactttggtgaggaaggcaaagaagaatccgtcatctcctcaatatctgaatgagaggacgcagattttggggacttcttcttcccgaaagcttgcttgaaggagctgcgtaactcattgacccagttcttccgcttcttcttctttgagtcactctctatgttgctgcccacgctggagtggctggtggcactgttgatgctggagacgctgtctgaggagtgctgcctgcggatgcggaggtctgcagactgggcagtgccgtttcctttgcagttgagctcaggtgtgttaattactccattaatggcagcctgggcagctgcgttctgtttctttagcagctcaatggtttttcttaactcattcagttctgagtccttctgctcagctgtcatggtcagactctggagcctgattgtcatgttaccaagactctgttcaaaggctgccacaaggtgagcatttgctgtcagctgggtggtcaaagctgaaactttctcctgggaggcatccagttcccgccgcagcttgcgaatctctgactggcatttttcttctggtgtagaataaactgacgatgtgctggaaaccaaggagagtgaggatccatgaactaactcataccttgcgtgatggaacaaaggaagagagaaatgaagtgagctgtgaagacggctgacaaagttgtccacagaacttttctcccatgattcttcttcaaacccatcccggaatgagcctgaacggctcatggttctgctcttctcatccagggacatggagctattccggaagcggctgtcagtgtatggatcatactgcccatcagcattggagaggctgtgagtcctcagcatggtcgggttggacaagctcatctgggtgacagtggtgggactcgcaagctgggaaaagttgaatcttgttccggagggagaagtcacgctggagccagaggaaaagggggaattggcagcggtgtcctgaaggcctcctgcagaatgggaccgtaaccattcttttgcatcttcttgcgtgcgaagctgggaggtgggagtatacctgagtcctttcttaggcaaagtgttcctatcaaggtgcgggtcactgtcctgtttcctgggcagagtacttctgcagaacttagggctagcagcaggggaagagagagggctttctgacagtgtggtcttcacactgttagttctgacaaagggagtcaaggagtcgtccttggaggaggcgatgaggccagtggaagaattgtggctggggacccctccactgctgagggagatgtcgatggactcacagctggtgtggaggctgctgacagactgaaagcccaggccatccttgctaactgcggaggagctgctggcgttggtgccccaggtgaggctgttggaaggggccgagtgggctgagctggggctggaggctagcggagactggttgaggtccacattcttgctgtagagaggactgctgctcccactgctcaggacgccactgcctgacggggagtctaggttaccttgctgagtcatggtggcatgaggattggagatgaccaccgaatttttcatgttttcagctgtggcgatgggcacttgcttggtaggcttcccaccaaagagtctgcggagtgtgggagaggccacatctgggtacttggctccaggctggagactggtctgagccggactggacacaggctgggctgccggattcactttcaccgagttacaggaagccacactctcgttgtctgatgagatgcctttctccttgtctgtttggttgaccagacctggtagagagctgcctagggctgttttggaaggctccctcagtttgggcactggcaggcctgcggacttgctgctaatgttggaatctatgctgctggtgctagacctgttcccagccccgttccggctgttggacttactgggcctcggcaaactccggtactgaaggtttgtccgggagcttagggctagatacccgtcatcctgattctgagccccatccatacttgacttccgaccagcagaccgactgacgagtgcagatgactttgggattttgcccagtgtggctgacctgctggtgacagtcaccccgctggctgtgatcatggccaggccggcggcggaaccactctgcttcttgaacccaaagctgttggcattggcagtaggtgtcctagagctgctggggaggggctttttggattcgtcaccactgctccggcctgcatctgatggggagcgcttcacctgggaggctttaggagaaagccttcctttctcagacacctttgcgtcgtctgtttttccagttcctggggtcttcagtgcgcctgccggggctgaaggcttcgtccttggcatggtgatgcccacctgagctgtcatgcctcgccgccatgagcctgtctgggagatgacaggattcttcttgcccgacgtgcttttgtcggactcgtcagacacatcagaaggattccgcctccacttggaacctggctccatttttatgccgctgtctgagcctccgtctgatttcttgacatcatcaccagaccacagggaattcctctccacctgtgagtgcttctcagcatcagtctgcacatccaggttttttcgagaggaggcaggtgtgttggcataagagctgatggaggagctggtgttgatgtcatcagtgctgaggttgtctatggtgtcgctgatgccgctgctgacggagctgctgtcgtcccagctgctcaattttccagttctgctccagaatcaaggcacagcccatttacagggctggcccatgccccccgccagacagctgcattcagttgcaaaaaagtccagactggtggaactcgttttctggctattgttcaaggcaattgttcccgtgaaaccccggggcccgagcggaacgagatcctttggtgtggatgagtgagcaagcctaact

SEQ ID NO: 17885 - RNA, 9677 nt, Homo sapiens
  source 1..9677: mol_type = other RNA
tcggcctggggaggaggaaggggagggaggatggaaacataccgtacacaaaatactcaattcctagttttctctttaaaaatggctagaaaaaattcatcaaaatgcagcactttaatcaattatttacaatttctatgttacaatgaaaaaatgtacatcttatagaacatatttcataaaactgctccactggaaacaactagatcaaaacagcaaaccttccatttaatatccacaaagttggattatttttcctttttgaagtagattcgccacaatcaaatttgaatacagagaattttgaagtttaagcatcaaacaacaaagtaaaagtccccaagatacaacaaagatctaggcaagtcttgttcctgtcccactcccaccccacccctaatgaaacttaaaaggtattcccatttcaattatggcctgtatcattcttggcagtttgggaagagaacttttggcttccattggtaactcaacataaatgttgcatagaatttatatatttcaaaattggcctaactgtagaaaaggcaaaatggaagcatttccgatagagccctaaatgagtacaaagtcactttgtaaaaggtgagtgacactaaagtaaaaatatgaccaaaataagaaatgtgcatattagacaaccctgcttcccgaaactttaggaaggacacggagttgtgagtcacacaagggctatgctacttgaagtcaatgttcaccaatcaggcagcactaggtacagaagtcttggttctgaacctggacccaggagggaagtctgtgggaaaggggagaagagaatgacaagagaggatgtcatattaaaaaaaggtttcaaacaatattggcaggtgtctactcacaaggtgattggaaaactgcccacgaggagaagtcaactttacctcctcccaaattcacagtacgcgagtgtagtagggtcattgctgggagataaattgtctgaggagggccacccttcaggtttaccagaaatcttagggtttggcccccctggtcacaggctaaatatatggtttaaaagttttattaaaaagaaaaacagaacaagacacactcacacccagatgactaatgaaggctaagcagaatagtctgagtttgctgagactaaagcagggatagtgttgaaaagttttcctttcactagtgggacacattccccttttcttttcaaagaggaagaacatggtgtcatccaatgtgaagtgagcagtttcgggtcaaactcttatggtaagaaactaaaaaaagatgccaagagacaaaccttcagaaatagaagaaatgcaaaagatggaataaaaaccctgatcattaaaacagagacaccttcactggtgtccaataaggattctctttacaaaacagaaacaaacaactcaaaaatttaccatactttgtaatgaaaataccagtatgttgaagacacagcagactgggtttctattagaacaagtatcagcaaggtcatgtagacttgtagaaacttttgccttctcctgcaccagacagatcattgtccagttgggttgtcagctggagaccgaaaagaacctaaaaaatggatctttttttttttctttttcccatggtcacgcatccacacaaatgagtcttttggatgagaaaagtcacagcaacttgagttctcctaatgaacagatgactttttagccctgtttgtttcaatggggaaaacaatgacaaaaaaaacaaaccccaggcaggcacgacacttatgtaaaatgaacacagttagtacaaaaccagtaaggcatcactttgggaaggtcagcaccgaagaggtcaggcaaggctcgtccagacggggcttctgggagggagtgaccctcacccttattgagctgcgtcatgttggttctgaggaaagtgcaagtcttttgcagggtgaccgcatcaccccaccggaagctggggcggggacgctggaggtgttggtgtgtgttctaaaccctcaaggacgagaagggaaggcaaggtccatggctcacccacatgtcgaggaccaggtcctcatccattttaaaggacacagatacccccagccctagcaggaggaggcgagtgtgtaggactgtgaggatggacaactaaaaaccaaaactgagcaggaccaaaccaaaactcaactcctgcggttcttactttcaccaaaggattgattctgaccaagaggggaagggggaaaaaaaaatcttcaaaaatcaatgcatcagaaaggaagaaactcaacctcattttcaaaaggtaacctgttctccaaagtagaacaagtctcactatacacagtgtttgcagaaaaaaaaaaaaaaaaacctgattcattcatatatcagaaggaaagagacacatgctgttctgcactgacagccacatccactcgctcacactctcactccgtcactcactctcacggatattaatcagaggctgatggacctgaatggggtggtttgattggaacaggcaaaatacctctcgggtaaggaaagcaccatttaaaaaacatgaaagcacggtttatttgctcctaaggtttccctgtgtcgtagctctgtagtgcgttgaacgtgaccaaagcaagcaccctggttagcaccagttctccctgtggccggctgtgtgggagggtgggtggcacggctctgagacccagtctggagggtctgtgctgaggggaagccgtgcttctctgtgtttccgactttgctccagtctcttctgtctctgggaagctcatggcaggatgctgtttggtttcagagcttcatgtgggttctctttttttttttctctctgtctctcttttcatttcaacggcgatgatcctttcccgagaagtatcttcagtgtcttagggaggtcacagcaacaaggcaaaacaataattaaagtacaacagaaggtagtgcagttctcgctgtggaaggaagcggtccgcaggcagctggcccgggatgcctgcacccaggtcgaggctgaaggacggggggtctcggtgttcccgcagctctaaggctgtggctgggggctggctcaggaagtcatcttcagggtgatgtgggggatgcaggtggaatgcggtgaggagaagaggagggcgctgggctccgggcccctgtcacagagtggactccaaagaggagtccaagatgtcatcgtgatggctgttgctgttggagtcgctgtcatagctctgggggctggagtagttggctgcctcctgcagcctcatcagcatgttcatcagcgggtcaccttcagcatcactggggggcatctgcttgcttgtcgatccctcccgaggcatggagtagccgtcgaagccgacatcctcaggccgtaactgcagcaggggaggccactcgtgctgttgtgggctggctgcccatggatatgtgtccatcacccacttggcaggatcctcccagggggcgcgccttccatagagctggagtccttctctgacggcttccaggagataggggataatggaatagttccacaagtcggtgaaccacactctcgagccgtccacatcgatggggcatgacaggaagagccgggggccgatggtgacgtccgaggaactgtgagcctccaggaagcggttgaggtgatgccagaccttgggaatccagtcaatgatttttaccagctccatattgcgcacccgcccactgatctctgtttccatgagcttcctcctcaggaatcggccaaggaaacccttcacaggctccgtgtggttggcacaaagcacccatctgaagttatggtgaagctgcaggttgggagtcgaagaggtagcctggttcattgtgccaattatgtaagggcatttgtggtacttgcagttgagcagcccattgaagatctctcccagagagctcacgtggtgtaggttgtccaggatgatgacgaggggcatgtccacagcattgttctcactgttgcactggtcagcaaggttggacaggtactggcgcaattccttgctggacttatggtccacgttaaaggtggcgataaccccgtctgtcaactcccgtccctctcgaagcactatatactcagacagccggttggccaggtaggttttcccagtgccgctggggccagagagaatgatccgacggtgctctatcaggagggagacgtagcgctgcaggatgggcttgggaatcaaggactcaaacaccagtgagtccaggctgttttctgcgagccctttcacagtcactgagatggtcgtgttctctccaaccagatagccacaaggaagcagctccggtgtttcggaagtgttgctgcgcttgatttctccaatgctgtagccaagaacgctgtctgaattcagccctagctgactcactgggtcgacatgaatgatgtattctttgaacagccgtctaaccaccccatcgagcacatcccacttcgtcttgccactaactccaatgcagccaataagaaagagatgtggtctggaatcctccttccacttcatttcctcctgaaagctgacaactatcttaacatgcctgcctccttccttccgagccgagcattcaccagtgtcatccagcaacatgtccaggctggttgactcagtgaggttcaagctgtgctgggagaggcccatggactgcctcggggaggcagagatggacacttgggaaggagcccggctgcagccactgccttgagactctgacttcagccgatcattctcagctttcagcttctctatttcactctgcatcctgttcatggcctcccggagctggtccagctggtgggcagaactgagagcttctaagcggatatccgtcagcttcatctccttgtctcttaactcatttcggagctgcatgacggtctcagcttcactatccatgcattctgaaattagagagttggagtgagaattcctcagcagtggggtggaacctgtggacccattgtgcggtaactttggtgaggaaggcaaagaagaatccgtcatctcctcaatatctgaatgagaggacgcagattttggggacttcttcttcccgaaagcttgcttgaaggagctgcgtaactcattgacccagttcttccgcttcttcttctttgagtcactctctatgttgctgcccacgctggagtggctggtggcactgttgatgctggagacgctgtctgaggagtgctgcctgcggatgcggaggtctgcagactgggcagtgccgtttcctttgcagttgagctcaggtgtgttaattactccattaatggcagcctgggcagctgcgttctgtttctttagcagctcaatggtttttcttaactcattcagttctgagtccttctgctcagctgtcatggtcagactctggagcctgattgtcatgttaccaagactctgttcaaaggctgccacaaggtgagcatttgctgtcagctgggtggtcaaagctgaaactttctcctgggaggcatccagttcccgccgcagcttgcgaatctctgactggcatttttcttctggtgtagaataaactgacgatgtgctggaaaccaaggagagtgaggatccatgaactaactcataccttgcgtgatggaacaaaggaagagagaaatgaagtgagctgtgaagacggctgacaaagttgtccacagaacttttctcccatgattcttcttcaaacccatcccggaatgagcctgaacggctcatggttctgctcttctcatccagggacatggagctattccggaagcggctgtcagtgtatggatcatactgcccatcagcattggagaggctgtgagtcctcagcatggtcgggttggacaagctcatctgggtgacagtggtgggactcgcaagctgggaaaagttgaatcttgttccggagggagaagtcacgctggagccagaggaaaagggggaattggcagcggtgtcctgaaggcctcctgcagaatgggaccgtaaccattcttttgcatcttcttgcgtgcgaagctgggaggtgggagtatacctgagtcctttcttaggcaaagtgttcctatcaaggtgcgggtcactgtcctgtttcctgggcagagtacttctgcagaacttagggctagcagcaggggaagagagagggctttctgacagtgtggtcttcacactgttagttctgacaaagggagtcaaggagtcgtccttggaggaggcgatgaggccagtggaagaattgtggctggggacccctccactgctgagggagatgtcgatggactcacagctggtgtggaggctgctgacagactgaaagcccaggccatccttgctaactgcggaggagctgctggcgttggtgccccaggtgaggctgttggaaggggccgagtgggctgagctggggctggaggctagcggagactggttgaggtccacattcttgctgtagagaggactgctgctcccactgctcaggacgccactgcctgacggggagtctaggttaccttgctgagtcatggtggcatgaggattggagatgaccaccgaatttttcatgttttcagctgtggcgatgggcacttgcttggtaggcttcccaccaaagagtctgcggagtgtgggagaggccacatctgggtacttggctccaggctggagactggtctgagccggactggacacaggctgggctgccggattcactttcaccgagttacaggaagccacactctcgttgtctgatgagatgcctttctccttgtctgtttggttgaccagacctggtagagagctgcctagggctgttttggaaggctccctcagtttgggcactggcaggcctgcggacttgctgctaatgttggaatctatgctgctggtgctagacctgttcccagccccgttccggctgttggacttactgggcctcggcaaactccggtactgaaggtttgtccgggagcttagggctagatacccgtcatcctgattctgagccccatccatacttgacttccgaccagcagaccgactgacgagtgcagatgactttgggattttgcccagtgtggctgacctgctggtgacagtcaccccgctggctgtgatcatggccaggccggcggcggaaccactctgcttcttgaacccaaagctgttggcattggcagtaggtgtcctagagctgctggggaggggctttttggattcgtcaccactgctccggcctgcatctgatggggagcgcttcacctgggaggctttaggagaaagccttcctttctcagacacctttgcgtcgtctgtttttccagttcctggggtcttcagtgcgcctgccggggctgaaggcttcgtccttggcatggtgatgcccacctgagctgtcatgcctcgccgccatgagcctgtctgggagatgacaggattcttcttgcccgacgtgcttttgtcggactcgtcagacacatcagaaggattccgcctccacttggaacctggctccatttttatgccgctgtctgagcctccgtctgatttcttgacatcatcaccagaccacagggaattcctctccacctgtgagtgcttctcagcatcagtctgcacatccaggttttttcgagaggaggcaggtgtgttggcataagagctgatggaggagctggtgttgatgtcatcagtgctgaggttgtctatggtgtcgctgatgccgctgctgacggagctgctgtcgtcccagctgtcagcgtctccgaggcccagggaggtatttcgttgcagggtctcccgtaccacagccatcccatcagggagccggttcaggcgacgggtatagaggccaagtccaccatcagtcatgtatccgcttgtaatgtcatcggtccggatgttcttgctcagaacatccccgtcgctcatgtagccgggggcatccatgctgatgccttccaggtccatctcatctcctgccttgtctgagacgtccacatggcagacactactgccccgggaggccagctgccttctcagaggggcggagtacacatagcgacctgactcagtgttgatgaacctgctggcgttggctcgagggggatacccattgcccattgagggggcgtctcctgcttggagccgagggctggactggcccagtctccaggacagaggtgtgggcctccctgtcaagctgagtatgctacggccactcatctccgtggtgacattggtgtcaaacgtggtttccaatgtgctgtgtgtaacctgagttccccttaaactggacatggtttcctccaaattctgccgcagatcagcgatgttcttcactgtccgcagccgccgagcctcaggatcttccccagtgagttcttccagagcaggctgtccagtcttggtgaagtggctgggctccacgctcacacctgttgagcttgactcggcagtaacattcccttcagtgtccgtctgagacctgtacaggaaaggtgcaaccgtggcagtgttgggatggttgtattgctgctggggctgaggtagctgaacactgacggtattgcttcctgtggtctgggtggtcccgacagacccactgacagtctggctgctgatgctgtggttcagggtggtccctcctgggccttttccttctgaggacgccaggctggaagaggaactggagtgtctgccgtccagctggggcttctgctgggggagtcctgagctcagcttcccactccggctccgctccccttccttggaaggcgctggggcacttggggatttcccgggcatgcttttcattcctggttttggtattccactgtgggaaggggccatgggctccttcttggcactgttgagcttcccccctttggggatgaagctggcaatcttggaggacttttttggcatctcgggcacagctgctccactggggtcttcttttggctcctccttgaggtccagcctctccgtcacagaggctctcttggcaaggtccttgcttttctccttatccttctcccgctgttgtttctccttctctttctcattgcctttcagagaactcttcttgttggtcagtgcccggctaaaagtcctctgggcaatgcccttgagtgcaatcttggggctgctggaagcagggcccacggtggtgagcatgcgactggcggcctccagctcctcgctctcttcgaagctgggcagagtctccagccgctcacagcttgtgtcccgggaccccggcccctcacctgcctttgagccccctttactgttgaaaagtttcagcttttccagcatggacttctgattgttgggggccggcttcatggcttcaggtgtgggcctgggggcctcaggcccaggaggcttgaccgagagcatggataccgtggcactgtgcttcacgctgagggatttgctgcgccaaggcttggtggctgcaccgggctgcgggatggccgaggaggtactgcaattagtaggggtggagctgctgccgctctccaaggaagcaggtgcattgtcactcattccggggtgggaggaggctgaacttgccaaaggctctagcagcagccactttctcctgcaa

SEQ ID NO: 17886 - RNA, 10792 nt, Homo sapiens
  source 1..10792: mol_type = other RNA
tcggcctggggaggaggaaggggagggaggatggaaacataccgtacacaaaatactcaattcctagttttctctttaaaaatggctagaaaaaattcatcaaaatgcagcactttaatcaattatttacaatttctatgttacaatgaaaaaatgtacatcttatagaacatatttcataaaactgctccactggaaacaactagatcaaaacagcaaaccttccatttaatatccacaaagttggattatttttcctttttgaagtagattcgccacaatcaaatttgaatacagagaattttgaagtttaagcatcaaacaacaaagtaaaagtccccaagatacaacaaagatctaggcaagtcttgttcctgtcccactcccaccccacccctaatgaaacttaaaaggtattcccatttcaattatggcctgtatcattcttggcagtttgggaagagaacttttggcttccattggtaactcaacataaatgttgcatagaatttatatatttcaaaattggcctaactgtagaaaaggcaaaatggaagcatttccgatagagccctaaatgagtacaaagtcactttgtaaaaggtgagtgacactaaagtaaaaatatgaccaaaataagaaatgtgcatattagacaaccctgcttcccgaaactttaggaaggacacggagttgtgagtcacacaagggctatgctacttgaagtcaatgttcaccaatcaggcagcactaggtacagaagtcttggttctgaacctggacccaggagggaagtctgtgggaaaggggagaagagaatgacaagagaggatgtcatattaaaaaaaggtttcaaacaatattggcaggtgtctactcacaaggtgattggaaaactgcccacgaggagaagtcaactttacctcctcccaaattcacagtacgcgagtgtagtagggtcattgctgggagataaattgtctgaggagggccacccttcaggtttaccagaaatcttagggtttggcccccctggtcacaggctaaatatatggtttaaaagttttattaaaaagaaaaacagaacaagacacactcacacccagatgactaatgaaggctaagcagaatagtctgagtttgctgagactaaagcagggatagtgttgaaaagttttcctttcactagtgggacacattccccttttcttttcaaagaggaagaacatggtgtcatccaatgtgaagtgagcagtttcgggtcaaactcttatggtaagaaactaaaaaaagatgccaagagacaaaccttcagaaatagaagaaatgcaaaagatggaataaaaaccctgatcattaaaacagagacaccttcactggtgtccaataaggattctctttacaaaacagaaacaaacaactcaaaaatttaccatactttgtaatgaaaataccagtatgttgaagacacagcagactgggtttctattagaacaagtatcagcaaggtcatgtagacttgtagaaacttttgccttctcctgcaccagacagatcattgtccagttgggttgtcagctggagaccgaaaagaacctaaaaaatggatctttttttttttctttttcccatggtcacgcatccacacaaatgagtcttttggatgagaaaagtcacagcaacttgagttctcctaatgaacagatgactttttagccctgtttgtttcaatggggaaaacaatgacaaaaaaaacaaaccccaggcaggcacgacacttatgtaaaatgaacacagttagtacaaaaccagtaaggcatcactttgggaaggtcagcaccgaagaggtcaggcaaggctcgtccagacggggcttctgggagggagtgaccctcacccttattgagctgcgtcatgttggttctgaggaaagtgcaagtcttttgcagggtgaccgcatcaccccaccggaagctggggcggggacgctggaggtgttggtgtgtgttctaaaccctcaaggacgagaagggaaggcaaggtccatggctcacccacatgtcgaggaccaggtcctcatccattttaaaggacacagatacccccagccctagcaggaggaggcgagtgtgtaggactgtgaggatggacaactaaaaaccaaaactgagcaggaccaaaccaaaactcaactcctgcggttcttactttcaccaaaggattgattctgaccaagaggggaagggggaaaaaaaaatcttcaaaaatcaatgcatcagaaaggaagaaactcaacctcattttcaaaaggtaacctgttctccaaagtagaacaagtctcactatacacagtgtttgcagaaaaaaaaaaaaaaaaacctgattcattcatatatcagaaggaaagagacacatgctgttctgcactgacagccacatccactcgctcacactctcactccgtcactcactctcacggatattaatcagaggctgatggacctgaatggggtggtttgattggaacaggcaaaatacctctcgggtaaggaaagcaccatttaaaaaacatgaaagcacggtttatttgctcctaaggtttccctgtgtcgtagctctgtagtgcgttgaacgtgaccaaagcaagcaccctggttagcaccagttctccctgtggccggctgtgtgggagggtgggtggcacggctctgagacccagtctggagggtctgtgctgaggggaagccgtgcttctctgtgtttccgactttgctccagtctcttctgtctctgggaagctcatggcaggatgctgtttggtttcagagcttcatgtgggttctctttttttttttctctctgtctctcttttcatttcaacggcgatgatcctttcccgagaagtatcttcagtgtcttagggaggtcacagcaacaaggcaaaacaataattaaagtacaacagaaggtagtgcagttctcgctgtggaaggaagcggtccgcaggcagctggcccgggatgcctgcacccaggtcgaggctgaaggacggggggtctcggtgttcccgcagctctaaggctgtggctgggggctggctcaggaagtcatcttcagggtgatgtgggggatgcaggtggaatgcggtgaggagaagaggagggcgctgggctccgggcccctgtcacagagtggactccaaagaggagtccaagatgtcatcgtgatggctgttgctgttggagtcgctgtcatagctctgggggctggagtagttggctgcctcctgcagcctcatcagcatgttcatcagcgggtcaccttcagcatcactggggggcatctgcttgcttgtcgatccctcccgaggcatggagtagccgtcgaagccgacatcctcaggccgtaactgcagcaggggaggccactcgtgctgttgtgggctggctgcccatggatatgtgtccatcacccacttggcaggatcctcccagggggcgcgccttccatagagctggagtccttctctgacggcttccaggagataggggataatggaatagttccacaagtcggtgaaccacactctcgagccgtccacatcgatggggcatgacaggaagagccgggggccgatggtgacgtccgaggaactgtgagcctccaggaagcggttgaggtgatgccagaccttgggaatccagtcaatgatttttaccagctccatattgcgcacccgcccactgatctctgtttccatgagcttcctcctcaggaatcggccaaggaaacccttcacaggctccgtgtggttggcacaaagcacccatctgaagttatggtgaagctgcaggttgggagtcgaagaggtagcctggttcattgtgccaattatgtaagggcatttgtggtacttgcagttgagcagcccattgaagatctctcccagagagctcacgtggtgtaggttgtccaggatgatgacgaggggcatgtccacagcattgttctcactgttgcactggtcagcaaggttggacaggtactggcgcaattccttgctggacttatggtccacgttaaaggtggcgataaccccgtctgtcaactcccgtccctctcgaagcactatatactcagacagccggttggccaggtaggttttcccagtgccgctggggccagagagaatgatccgacggtgctctatcaggagggagacgtagcgctgcaggatgggcttgggaatcaaggactcaaacaccagtgagtccaggctgttttctgcgagccctttcacagtcactgagatggtcgtgttctctccaaccagatagccacaaggaagcagctccggtgtttcggaagtgttgctgcgcttgatttctccaatgctgtagccaagaacgctgtctgaattcagccctagctgactcactgggtcgacatgaatgatgtattctttgaacagccgtctaaccaccccatcgagcacatcccacttcgtcttgccactaactccaatgcagccaataagaaagagatgtggtctggaatcctccttccacttcatttcctcctgaaagctgacaactatcttaacatgcctgcctccttccttccgagccgagcattcaccagtgtcatccagcaacatgtccaggctggttgactcagtgaggttcaagctgtgctgggagaggcccatggactgcctcggggaggcagagatggacacttgggaaggagcccggctgcagccactgccttgagactctgacttcagccgatcattctcagctttcagcttctctatttcactctgcatcctgttcatggcctcccggagctggtccagctggtgggcagaactgagagcttctaagcggatatccgtcagcttcatctccttgtctcttaactcatttcggagctgcatgacggtctcagcttcactatccatgcattctgaaattagagagttggagtgagaattcctcagcagtggggtggaacctgtggacccattgtgcggtaactttggtgaggaaggcaaagaagaatccgtcatctcctcaatatctgaatgagaggacgcagattttggggacttcttcttcccgaaagcttgcttgaaggagctgcgtaactcattgacccagttcttccgcttcttcttctttgagtcactctctatgttgctgcccacgctggagtggctggtggcactgttgatgctggagacgctgtctgaggagtgctgcctgcggatgcggaggtctgcagactgggcagtgccgtttcctttgcagttgagctcaggtgtgttaattactccattaatggcagcctgggcagctgcgttctgtttctttagcagctcaatggtttttcttaactcattcagttctgagtccttctgctcagctgtcatggtcagactctggagcctgattgtcatgttaccaagactctgttcaaaggctgccacaaggtgagcatttgctgtcagctgggtggtcaaagctgaaactttctcctgggaggcatccagttcccgccgcagcttgcgaatctctgactggcatttttcttctggtgtagaataaactgacgatgtgctggaaaccaaggagagtgaggatccatgaactaactcataccttgcgtgatggaacaaaggaagagagaaatgaagtgagctgtgaagacggctgacaaagttgtccacagaacttttctcccatgattcttcttcaaacccatcccggaatgagcctgaacggctcatggttctgctcttctcatccagggacatggagctattccggaagcggctgtcagtgtatggatcatactgcccatcagcattggagaggctgtgagtcctcagcatggtcgggttggacaagctcatctgggtgacagtggtgggactcgcaagctgggaaaagttgaatcttgttccggagggagaagtcacgctggagccagaggaaaagggggaattggcagcggtgtcctgaaggcctcctgcagaatgggaccgtaaccattcttttgcatcttcttgcgtgcgaagctgggaggtgggagtatacctgagtcctttcttaggcaaagtgttcctatcaaggtgcgggtcactgtcctgtttcctgggcagagtacttctgcagaacttagggctagcagcaggggaagagagagggctttctgacagtgtggtcttcacactgttagttctgacaaagggagtcaaggagtcgtccttggaggaggcgatgaggccagtggaagaattgtggctggggacccctccactgctgagggagatgtcgatggactcacagctggtgtggaggctgctgacagactgaaagcccaggccatccttgctaactgcggaggagctgctggcgttggtgccccaggtgaggctgttggaaggggccgagtgggctgagctggggctggaggctagcggagactggttgaggtccacattcttgctgtagagaggactgctgctcccactgctcaggacgccactgcctgacggggagtctaggttaccttgctgagtcatggtggcatgaggattggagatgaccaccgaatttttcatgttttcagctgtggcgatgggcacttgcttggtaggcttcccaccaaagagtctgcggagtgtgggagaggccacatctgggtacttggctccaggctggagactggtctgagccggactggacacaggctgggctgccggattcactttcaccgagttacaggaagccacactctcgttgtctgatgagatgcctttctccttgtctgtttggttgaccagacctggtagagagctgcctagggctgttttggaaggctccctcagtttgggcactggcaggcctgcggacttgctgctaatgttggaatctatgctgctggtgctagacctgttcccagccccgttccggctgttggacttactgggcctcggcaaactccggtactgaaggtttgtccgggagcttagggctagatacccgtcatcctgattctgagccccatccatacttgacttccgaccagcagaccgactgacgagtgcagatgactttgggattttgcccagtgtggctgacctgctggtgacagtcaccccgctggctgtgatcatggccaggccggcggcggaaccactctgcttcttgaacccaaagctgttggcattggcagtaggtgtcctagagctgctggggaggggctttttggattcgtcaccactgctccggcctgcatctgatggggagcgcttcacctgggaggctttaggagaaagccttcctttctcagacacctttgcgtcgtctgtttttccagttcctggggtcttcagtgcgcctgccggggctgaaggcttcgtccttggcatggtgatgcccacctgagctgtcatgcctcgccgccatgagcctgtctgggagatgacaggattcttcttgcccgacgtgcttttgtcggactcgtcagacacatcagaaggattccgcctccacttggaacctggctccatttttatgccgctgtctgagcctccgtctgatttcttgacatcatcaccagaccacagggaattcctctccacctgtgagtgcttctcagcatcagtctgcacatccaggttttttcgagaggaggcaggtgtgttggcataagagctgatggaggagctggtgttgatgtcatcagtgctgaggttgtctatggtgtcgctgatgccgctgctgacggagctgctgtcgtcccagctgtcagcgtctccgaggcccagggaggtatttcgttgcagggtctcccgtaccacagccatcccatcagggagccggttcaggcgacgggtatagaggccaagtccaccatcagtcatgtatccgcttgtaatgtcatcggtccggatgttcttgctcagaacatccccgtcgctcatgtagccgggggcatccatgctgatgccttccaggtccatctcatctcctgccttgtctgagacgtccacatggcagacactactgccccgggaggccagctgccttctcagaggggcggagtacacatagcgacctgactcagtgttgatgaacctgctggcgttggctcgagggggatacccattgcccattgagggggcgtctcctgcttggagccgagggctggactggcccagtctccaggacagaggtgtgggcctccctgtcaagctgagtatgctacggccactcatctccgtggtgacattggtgtcaaacgtggtttccaatgtgctgtgtgtaacctgagttccccttaaactggacatggtttcctccaaattctgccgcagatcagcgatgttcttcactgtccgcagccgccgagcctcaggatcttccccagtgagttcttccagagcaggctgtccagtcttggtgaagtggctgggctccacgctcacacctgttgagcttgactcggcagtaacattcccttcagtgtccgtctgagacctgtacaggaaaggtgcaaccgtggcagtgttgggatggttgtattgctgctggggctgaggtagctgaacactgacggtattgcttcctgtggtctgggtggtcccgacagacccactgacagtctggctgctgatgctgtggttcagggtggtccctcctgggccttttccttctgaggacgccaggctggaagaggaactggagtgtctgccgtccagctggggcttctgctgggggagtcctgagctcagcttcccactccggctccgctccccttccttggaaggcgctggggcacttggggatttcccgggcatgcttttcattcctggttttggtattccactgtgggaaggggccatgggctccttcttggcactgttgagcttcccccctttggggatgaagctggcaatcttggaggacttttttggcatctcgggcacagctgctccactggggtcttcttttggctcctccttgaggtccagcctctccgtcacagaggctctcttggcaaggtccttgcttttctccttatccttctcccgctgttgtttctccttctctttctcattgcctttcagagaactcttcttgttggtcagtgcccggctaaaagtcctctgggcaatgcccttgagtgcaatcttggggctgctggaagcagggcccacggtggtgagcatgcgactggcggcctccagctcctcgctctcttcgaagctgggcagagtctccagccgctcacagcttgtgtcccgggaccccggcccctcacctgcctttgagccccctttactgttgaaaagtttcagcttttccagcatggacttctgattgttgggggccggcttcatggcttcaggtgtgggcctgggggcctcaggcccaggaggcttgaccgagagcatggataccgtggcactgtgcttcacgctgagggatttgctgcgccaaggcttggtggctgcaccgggctgcgggatggccgaggaggtactgcaattagtaggggtggagctgctgccgctctccaaggaagcaggtgcattgtcactcattccggggtgggaggaggctgaacttgccaaaggctctttctcgtggctgcttggcggtgggggtggggaggtgactggtttggatttatcatagttgttaaagctctggctgcgtcggttgttagcagtagttgaccctccgcgtgttttggcctcgctgcctgcagcggataccctcgcggtaggacctggaagtctagagatctttttctgacccagagtgaagcggatgattttgctttgagatgagtccttggatgatgcactggactgcatttcagcttgtgcttttgactgctgatgtggcgctggctggtgaggctggcacggggcttggggagtgactggcacctgctgctgaggggtgccagcctggcactgggagggggccccggccacctgggatacggcgggcggcagaggtgaggagaggtgctgcttctggggctgctgctgctgctgcttgtatcgggagaggctgaagaagaggcctagaatggccttgaggtttccattcctgatctcttctgcagacagcccctggatgtttattcccttagctgccaggaaattcaagcaggcatctatgttttcaatcatttgggatctgttcttcggacagccattgatgtcttcaatcttttcatttgccacaacctggataatctgggccaggaggacgccatctgtcacatcttgctggagatccctgatgagacgcttgtggccggatttggctaggtaatgattggcccagtctgtgtagatcagcttcatggtggtgttattctgttcccagcgccacagcatcacgctcatcttacttcagggcgaggaaggaaggggcagaggaaaaaggaggaggggaaaaaaaaaaaaagccgaagcacctgcccgcgcgcccggcaggtctggccgtccagtcccgggtctcctctcggccgcggcccctccaggcatccccggcgcccgcggtcgcctcgcccccgccccggggccgctgctgcgcgcggggaccctaccctggagaccggcgcccgcgctgcccagctctcgtgcctccctcgctcgctccccgccggcctccccgcctccgccaaatcaaacaactcgccctgtgtccaagcgcccgctcctcgcagcgcggaggccgctggggccgcggcggccgagggc

SEQ ID NO: 17887 - RNA, 12011 nt, Homo sapiens
  source 1..12011: mol_type = other RNA
tcggcctggggaggaggaaggggagggaggatggaaacataccgtacacaaaatactcaattcctagttttctctttaaaaatggctagaaaaaattcatcaaaatgcagcactttaatcaattatttacaatttctatgttacaatgaaaaaatgtacatcttatagaacatatttcataaaactgctccactggaaacaactagatcaaaacagcaaaccttccatttaatatccacaaagttggattatttttcctttttgaagtagattcgccacaatcaaatttgaatacagagaattttgaagtttaagcatcaaacaacaaagtaaaagtccccaagatacaacaaagatctaggcaagtcttgttcctgtcccactcccaccccacccctaatgaaacttaaaaggtattcccatttcaattatggcctgtatcattcttggcagtttgggaagagaacttttggcttccattggtaactcaacataaatgttgcatagaatttatatatttcaaaattggcctaactgtagaaaaggcaaaatggaagcatttccgatagagccctaaatgagtacaaagtcactttgtaaaaggtgagtgacactaaagtaaaaatatgaccaaaataagaaatgtgcatattagacaaccctgcttcccgaaactttaggaaggacacggagttgtgagtcacacaagggctatgctacttgaagtcaatgttcaccaatcaggcagcactaggtacagaagtcttggttctgaacctggacccaggagggaagtctgtgggaaaggggagaagagaatgacaagagaggatgtcatattaaaaaaaggtttcaaacaatattggcaggtgtctactcacaaggtgattggaaaactgcccacgaggagaagtcaactttacctcctcccaaattcacagtacgcgagtgtagtagggtcattgctgggagataaattgtctgaggagggccacccttcaggtttaccagaaatcttagggtttggcccccctggtcacaggctaaatatatggtttaaaagttttattaaaaagaaaaacagaacaagacacactcacacccagatgactaatgaaggctaagcagaatagtctgagtttgctgagactaaagcagggatagtgttgaaaagttttcctttcactagtgggacacattccccttttcttttcaaagaggaagaacatggtgtcatccaatgtgaagtgagcagtttcgggtcaaactcttatggtaagaaactaaaaaaagatgccaagagacaaaccttcagaaatagaagaaatgcaaaagatggaataaaaaccctgatcattaaaacagagacaccttcactggtgtccaataaggattctctttacaaaacagaaacaaacaactcaaaaatttaccatactttgtaatgaaaataccagtatgttgaagacacagcagactgggtttctattagaacaagtatcagcaaggtcatgtagacttgtagaaacttttgccttctcctgcaccagacagatcattgtccagttgggttgtcagctggagaccgaaaagaacctaaaaaatggatctttttttttttctttttcccatggtcacgcatccacacaaatgagtcttttggatgagaaaagtcacagcaacttgagttctcctaatgaacagatgactttttagccctgtttgtttcaatggggaaaacaatgacaaaaaaaacaaaccccaggcaggcacgacacttatgtaaaatgaacacagttagtacaaaaccagtaaggcatcactttgggaaggtcagcaccgaagaggtcaggcaaggctcgtccagacggggcttctgggagggagtgaccctcacccttattgagctgcgtcatgttggttctgaggaaagtgcaagtcttttgcagggtgaccgcatcaccccaccggaagctggggcggggacgctggaggtgttggtgtgtgttctaaaccctcaaggacgagaagggaaggcaaggtccatggctcacccacatgtcgaggaccaggtcctcatccattttaaaggacacagatacccccagccctagcaggaggaggcgagtgtgtaggactgtgaggatggacaactaaaaaccaaaactgagcaggaccaaaccaaaactcaactcctgcggttcttactttcaccaaaggattgattctgaccaagaggggaagggggaaaaaaaaatcttcaaaaatcaatgcatcagaaaggaagaaactcaacctcattttcaaaaggtaacctgttctccaaagtagaacaagtctcactatacacagtgtttgcagaaaaaaaaaaaaaaaaacctgattcattcatatatcagaaggaaagagacacatgctgttctgcactgacagccacatccactcgctcacactctcactccgtcactcactctcacggatattaatcagaggctgatggacctgaatggggtggtttgattggaacaggcaaaatacctctcgggtaaggaaagcaccatttaaaaaacatgaaagcacggtttatttgctcctaaggtttccctgtgtcgtagctctgtagtgcgttgaacgtgaccaaagcaagcaccctggttagcaccagttctccctgtggccggctgtgtgggagggtgggtggcacggctctgagacccagtctggagggtctgtgctgaggggaagccgtgcttctctgtgtttccgactttgctccagtctcttctgtctctgggaagctcatggcaggatgctgtttggtttcagagcttcatgtgggttctctttttttttttctctctgtctctcttttcatttcaacggcgatgatcctttcccgagaagtatcttcagtgtcttagggaggtcacagcaacaaggcaaaacaataattaaagtacaacagaaggtagtgcagttctcgctgtggaaggaagcggtccgcaggcagctggcccgggatgcctgcacccaggtcgaggctgaaggacggggggtctcggtgttcccgcagctctaaggctgtggctgggggctggctcaggaagtcatcttcagggtgatgtgggggatgcaggtggaatgcggtgaggagaagaggagggcgctgggctccgggcccctgtcacagagtggactccaaagaggagtccaagatgtcatcgtgatggctgttgctgttggagtcgctgtcatagctctgggggctggagtagttggctgcctcctgcagcctcatcagcatgttcatcagcgggtcaccttcagcatcactggggggcatctgcttgcttgtcgatccctcccgaggcatggagtagccgtcgaagccgacatcctcaggccgtaactgcagcaggggaggccactcgtgctgttgtgggctggctgcccatggatatgtgtccatcacccacttggcaggatcctcccagggggcgcgccttccatagagctggagtccttctctgacggcttccaggagataggggataatggaatagttccacaagtcggtgaaccacactctcgagccgtccacatcgatggggcatgacaggaagagccgggggccgatggtgacgtccgaggaactgtgagcctccaggaagcggttgaggtgatgccagaccttgggaatccagtcaatgatttttaccagctccatattgcgcacccgcccactgatctctgtttccatgagcttcctcctcaggaatcggccaaggaaacccttcacaggctccgtgtggttggcacaaagcacccatctgaagttatggtgaagctgcaggttgggagtcgaagaggtagcctggttcattgtgccaattatgtaagggcatttgtggtacttgcagttgagcagcccattgaagatctctcccagagagctcacgtggtgtaggttgtccaggatgatgacgaggggcatgtccacagcattgttctcactgttgcactggtcagcaaggttggacaggtactggcgcaattccttgctggacttatggtccacgttaaaggtggcgataaccccgtctgtcaactcccgtccctctcgaagcactatatactcagacagccggttggccaggtaggttttcccagtgccgctggggccagagagaatgatccgacggtgctctatcaggagggagacgtagcgctgcaggatgggcttgggaatcaaggactcaaacaccagtgagtccaggctgttttctgcgagccctttcacagtcactgagatggtcgtgttctctccaaccagatagccacaaggaagcagctccggtgtttcggaagtgttgctgcgcttgatttctccaatgctgtagccaagaacgctgtctgaattcagccctagctgactcactgggtcgacatgaatgatgtattctttgaacagccgtctaaccaccccatcgagcacatcccacttcgtcttgccactaactccaatgcagccaataagaaagagatgtggtctggaatcctccttccacttcatttcctcctgaaagctgacaactatcttaacatgcctgcctccttccttccgagccgagcattcaccagtgtcatccagcaacatgtccaggctggttgactcagtgaggttcaagctgtgctgggagaggcccatggactgcctcggggaggcagagatggacacttgggaaggagcccggctgcagccactgccttgagactctgacttcagccgatcattctcagctttcagcttctctatttcactctgcatcctgttcatggcctcccggagctggtccagctggtgggcagaactgagagcttctaagcggatatccgtcagcttcatctccttgtctcttaactcatttcggagctgcatgacggtctcagcttcactatccatgcattctgaaattagagagttggagtgagaattcctcagcagtggggtggaacctgtggacccattgtgcggtaactttggtgaggaaggcaaagaagaatccgtcatctcctcaatatctgaatgagaggacgcagattttggggacttcttcttcccgaaagcttgcttgaaggagctgcgtaactcattgacccagttcttccgcttcttcttctttgagtcactctctatgttgctgcccacgctggagtggctggtggcactgttgatgctggagacgctgtctgaggagtgctgcctgcggatgcggaggtctgcagactgggcagtgccgtttcctttgcagttgagctcaggtgtgttaattactccattaatggcagcctgggcagctgcgttctgtttctttagcagctcaatggtttttcttaactcattcagttctgagtccttctgctcagctgtcatggtcagactctggagcctgattgtcatgttaccaagactctgttcaaaggctgccacaaggtgagcatttgctgtcagctgggtggtcaaagctgaaactttctcctgggaggcatccagttcccgccgcagcttgcgaatctctgactggcatttttcttctggtgtagaataaactgacgatgtgctggaaaccaaggagagtgaggatccatgaactaactcataccttgcgtgatggaacaaaggaagagagaaatgaagtgagctgtgaagacggctgacaaagttgtccacagaacttttctcccatgattcttcttcaaacccatcccggaatgagcctgaacggctcatggttctgctcttctcatccagggacatggagctattccggaagcggctgtcagtgtatggatcatactgcccatcagcattggagaggctgtgagtcctcagcatggtcgggttggacaagctcatctgggtgacagtggtgggactcgcaagctgggaaaagttgaatcttgttccggagggagaagtcacgctggagccagaggaaaagggggaattggcagcggtgtcctgaaggcctcctgcagaatgggaccgtaaccattcttttgcatcttcttgcgtgcgaagctgggaggtgggagtatacctgagtcctttcttaggcaaagtgttcctatcaaggtgcgggtcactgtcctgtttcctgggcagagtacttctgcagaacttagggctagcagcaggggaagagagagggctttctgacagtgtggtcttcacactgttagttctgacaaagggagtcaaggagtcgtccttggaggaggcgatgaggccagtggaagaattgtggctggggacccctccactgctgagggagatgtcgatggactcacagctggtgtggaggctgctgacagactgaaagcccaggccatccttgctaactgcggaggagctgctggcgttggtgccccaggtgaggctgttggaaggggccgagtgggctgagctggggctggaggctagcggagactggttgaggtccacattcttgctgtagagaggactgctgctcccactgctcaggacgccactgcctgacggggagtctaggttaccttgctgagtcatggtggcatgaggattggagatgaccaccgaatttttcatgttttcagctgtggcgatgggcacttgcttggtaggcttcccaccaaagagtctgcggagtgtgggagaggccacatctgggtacttggctccaggctggagactggtctgagccggactggacacaggctgggctgccggattcactttcaccgagttacaggaagccacactctcgttgtctgatgagatgcctttctccttgtctgtttggttgaccagacctggtagagagctgcctagggctgttttggaaggctccctcagtttgggcactggcaggcctgcggacttgctgctaatgttggaatctatgctgctggtgctagacctgttcccagccccgttccggctgttggacttactgggcctcggcaaactccggtactgaaggtttgtccgggagcttagggctagatacccgtcatcctgattctgagccccatccatacttgacttccgaccagcagaccgactgacgagtgcagatgactttgggattttgcccagtgtggctgacctgctggtgacagtcaccccgctggctgtgatcatggccaggccggcggcggaaccactctgcttcttgaacccaaagctgttggcattggcagtaggtgtcctagagctgctggggaggggctttttggattcgtcaccactgctccggcctgcatctgatggggagcgcttcacctgggaggctttaggagaaagccttcctttctcagacacctttgcgtcgtctgtttttccagttcctggggtcttcagtgcgcctgccggggctgaaggcttcgtccttggcatggtgatgcccacctgagctgtcatgcctcgccgccatgagcctgtctgggagatgacaggattcttcttgcccgacgtgcttttgtcggactcgtcagacacatcagaaggattccgcctccacttggaacctggctccatttttatgccgctgtctgagcctccgtctgatttcttgacatcatcaccagaccacagggaattcctctccacctgtgagtgcttctcagcatcagtctgcacatccaggttttttcgagaggaggcaggtgtgttggcataagagctgatggaggagctggtgttgatgtcatcagtgctgaggttgtctatggtgtcgctgatgccgctgctgacggagctgctgtcgtcccagctgtcagcgtctccgaggcccagggaggtatttcgttgcagggtctcccgtaccacagccatcccatcagggagccggttcaggcgacgggtatagaggccaagtccaccatcagtcatgtatccgcttgtaatgtcatcggtccggatgttcttgctcagaacatccccgtcgctcatgtagccgggggcatccatgctgatgccttccaggtccatctcatctcctgccttgtctgagacgtccacatggcagacactactgccccgggaggccagctgccttctcagaggggcggagtacacatagcgacctgactcagtgttgatgaacctgctggcgttggctcgagggggatacccattgcccattgagggggcgtctcctgcttggagccgagggctggactggcccagtctccaggacagaggtgtgggcctccctgtcaagctgagtatgctacggccactcatctccgtggtgacattggtgtcaaacgtggtttccaatgtgctgtgtgtaacctgagttccccttaaactggacatggtttcctccaaattctgccgcagatcagcgatgttcttcactgtccgcagccgccgagcctcaggatcttccccagtgagttcttccagagcaggctgtccagtcttggtgaagtggctgggctccacgctcacacctgttgagcttgactcggcagtaacattcccttcagtgtccgtctgagacctgtacaggaaaggtgcaaccgtggcagtgttgggatggttgtattgctgctggggctgaggtagctgaacactgacggtattgcttcctgtggtctgggtggtcccgacagacccactgacagtctggctgctgatgctgtggttcagggtggtccctcctgggccttttccttctgaggacgccaggctggaagaggaactggagtgtctgccgtccagctggggcttctgctgggggagtcctgagctcagcttcccactccggctccgctccccttccttggaaggcgctggggcacttggggatttcccgggcatgcttttcattcctggttttggtattccactgtgggaaggggccatgggctccttcttggcactgttgagcttcccccctttggggatgaagctggcaatcttggaggacttttttggcatctcgggcacagctgctccactggggtcttcttttggctcctccttgaggtccagcctctccgtcacagaggctctcttggcaaggtccttgcttttctccttatccttctcccgctgttgtttctccttctctttctcattgcctttcagagaactcttcttgttggtcagtgcccggctaaaagtcctctgggcaatgcccttgagtgcaatcttggggctgctggaagcagggcccacggtggtgagcatgcgactggcggcctccagctcctcgctctcttcgaagctgggcagagtctccagccgctcacagcttgtgtcccgggaccccggcccctcacctgcctttgagccccctttactgttgaaaagtttcagcttttccagcatggacttctgattgttgggggccggcttcatggcttcaggtgtgggcctgggggcctcaggcccaggaggcttgaccgagagcatggataccgtggcactgtgcttcacgctgagggatttgctgcgccaaggcttggtggctgcaccgggctgcgggatggccgaggaggtactgcaattagtaggggtggagctgctgccgctctccaaggaagcaggtgcattgtcactcattccggggtgggaggaggctgaacttgccaaaggctctttctcgtggctgcttggcggtgggggtggggaggtgactggtttggatttatcatagttgttaaagctctggctgcgtcggttgttagcagtagttgaccctccgcgtgttttggcctcgctgcctgcagcggataccctcgcggtaggacctggaagtctagagatctttttctgacccagagtgaagcggatgattttgctttgagatgagtccttggatgatgcactggactgcatttcagcttgtgcttttgactgctgatgtggcgctggctggtgaggctggcacggggcttggggagtgactggcacctgctgctgaggggtgccagcctggcactgggagggggccccggccacctgggatacggcgggcggcagaggtgaggagaggtgctgcttctggggctgctgctgctgctgcttgtatcgggagaggctgaagaagaggcctagaatggccttgaggtttccattcctgatctcttctgcagacagcccctggatgtttattcccttagctgccaggaaattcaagcaggcatctatgttttcaatcatttgggatctgttcttcggacagccattgatgtcttcaatcttttcatttgccacaacctggataatctgggccaggaggacgccatctgtcacatcttgctggagatccctgatgagacgcttgtggccggatttggctaggtaatgattggcccagtctgtgtagatccatctctgcactcctggtagtgcgtcacaggggctggcccaccgcaggaggctggtaagtggtcgccaggtagagctgaatatggagaaaaagggcaaatcttgggaaactgattacacttgagacttacatgatgtgggctctcagcaaatcctccaatcagaatctctttattgattaaaaagagcagggagcagggaaaataaatcactccatagctcaggctcattaatcagaaaccatttcacaaggatcattaattatctggagtttcctctcccttccctccctgtccccagctctcaactttttgaagtgaatcaagaaaacacctagatttattttttaagtcagtgttcatgggccatgctaatcatggacataaattcagccccatctccttcacttgctgtttcattagctcatgcaaggaaaatcattcttccaaggggtacccttgaaaaataaacttataatttctttagtcatcaaagatagatttcatcaggtccagcaattcagcaaaaacggagcaatgtgcgttttgagtaagggctcaagattttgagtaagggcttaaagcaagcaggcttcctgtctgagcctcagctatccagaattgttttctccaaaggctttcattccctaaaatgatggaaaattgagggctgctgttgctttttccccaggagcccattgattcttcatcctggtttgcccccaggtggatagctgtgaagtttcagtagaaactgattggacaaagaacagcaggaaagaccaaaaccaccatcccatccccaattccaattctaaatcatcaagtcatttcacgagaaagtctctaggatcctttgacactagtacccaagaatgagtccagccatcctcttgctccaatcactccatcttgcagaggtacccctctgcccatcccttctaaccaaaaactcagtgctccagaactgctctgtgagggagagaagctgctgtcaaaggcttgacaagataaaaggggaaggaaagctaagacagctaaacagtgaattcattttgattcactttattacccctgacagaattttaaggagtgcatcatttgtttgcttataactccacatcattccacatcaaacaggctgaaatccaaaagagaacattttgacagatcaattcaagtaaagaacctaatcattagttgtaataacaaaaactgataataattgtaccatgttaaaccaaaggggataataacactgctaagtttatactgcaattagccctcaaatgaagccgggtagcactaaagaacccaagaaaaattctgcaaaacaactgcactgaaagtgctagaatggagccttagctaccaaactataaatgcagatggatatgccaggcagcctgatggatccagaggcagatggcatcaggttagcagctccaggagaaacagagcaaactgtatttcttagaaggaaatgccagtgtggagactaatgtttaaagtaaaccagtcgtttagcatctgaggcatttccagtggattgattgtaaggggaatgctactgtttggccccaattcaggaagcctcactctagactttggtaatgtcatcatataat

SEQ ID NO: 17888 - RNA, 11212 nt, Homo sapiens
  source 1..11212: mol_type = other RNA
tcggcctggggaggaggaaggggagggaggatggaaacataccgtacacaaaatactcaattcctagttttctctttaaaaatggctagaaaaaattcatcaaaatgcagcactttaatcaattatttacaatttctatgttacaatgaaaaaatgtacatcttatagaacatatttcataaaactgctccactggaaacaactagatcaaaacagcaaaccttccatttaatatccacaaagttggattatttttcctttttgaagtagattcgccacaatcaaatttgaatacagagaattttgaagtttaagcatcaaacaacaaagtaaaagtccccaagatacaacaaagatctaggcaagtcttgttcctgtcccactcccaccccacccctaatgaaacttaaaaggtattcccatttcaattatggcctgtatcattcttggcagtttgggaagagaacttttggcttccattggtaactcaacataaatgttgcatagaatttatatatttcaaaattggcctaactgtagaaaaggcaaaatggaagcatttccgatagagccctaaatgagtacaaagtcactttgtaaaaggtgagtgacactaaagtaaaaatatgaccaaaataagaaatgtgcatattagacaaccctgcttcccgaaactttaggaaggacacggagttgtgagtcacacaagggctatgctacttgaagtcaatgttcaccaatcaggcagcactaggtacagaagtcttggttctgaacctggacccaggagggaagtctgtgggaaaggggagaagagaatgacaagagaggatgtcatattaaaaaaaggtttcaaacaatattggcaggtgtctactcacaaggtgattggaaaactgcccacgaggagaagtcaactttacctcctcccaaattcacagtacgcgagtgtagtagggtcattgctgggagataaattgtctgaggagggccacccttcaggtttaccagaaatcttagggtttggcccccctggtcacaggctaaatatatggtttaaaagttttattaaaaagaaaaacagaacaagacacactcacacccagatgactaatgaaggctaagcagaatagtctgagtttgctgagactaaagcagggatagtgttgaaaagttttcctttcactagtgggacacattccccttttcttttcaaagaggaagaacatggtgtcatccaatgtgaagtgagcagtttcgggtcaaactcttatggtaagaaactaaaaaaagatgccaagagacaaaccttcagaaatagaagaaatgcaaaagatggaataaaaaccctgatcattaaaacagagacaccttcactggtgtccaataaggattctctttacaaaacagaaacaaacaactcaaaaatttaccatactttgtaatgaaaataccagtatgttgaagacacagcagactgggtttctattagaacaagtatcagcaaggtcatgtagacttgtagaaacttttgccttctcctgcaccagacagatcattgtccagttgggttgtcagctggagaccgaaaagaacctaaaaaatggatctttttttttttctttttcccatggtcacgcatccacacaaatgagtcttttggatgagaaaagtcacagcaacttgagttctcctaatgaacagatgactttttagccctgtttgtttcaatggggaaaacaatgacaaaaaaaacaaaccccaggcaggcacgacacttatgtaaaatgaacacagttagtacaaaaccagtaaggcatcactttgggaaggtcagcaccgaagaggtcaggcaaggctcgtccagacggggcttctgggagggagtgaccctcacccttattgagctgcgtcatgttggttctgaggaaagtgcaagtcttttgcagggtgaccgcatcaccccaccggaagctggggcggggacgctggaggtgttggtgtgtgttctaaaccctcaaggacgagaagggaaggcaaggtccatggctcacccacatgtcgaggaccaggtcctcatccattttaaaggacacagatacccccagccctagcaggaggaggcgagtgtgtaggactgtgaggatggacaactaaaaaccaaaactgagcaggaccaaaccaaaactcaactcctgcggttcttactttcaccaaaggattgattctgaccaagaggggaagggggaaaaaaaaatcttcaaaaatcaatgcatcagaaaggaagaaactcaacctcattttcaaaaggtaacctgttctccaaagtagaacaagtctcactatacacagtgtttgcagaaaaaaaaaaaaaaaaacctgattcattcatatatcagaaggaaagagacacatgctgttctgcactgacagccacatccactcgctcacactctcactccgtcactcactctcacggatattaatcagaggctgatggacctgaatggggtggtttgattggaacaggcaaaatacctctcgggtaaggaaagcaccatttaaaaaacatgaaagcacggtttatttgctcctaaggtttccctgtgtcgtagctctgtagtgcgttgaacgtgaccaaagcaagcaccctggttagcaccagttctccctgtggccggctgtgtgggagggtgggtggcacggctctgagacccagtctggagggtctgtgctgaggggaagccgtgcttctctgtgtttccgactttgctccagtctcttctgtctctgggaagctcatggcaggatgctgtttggtttcagagcttcatgtgggttctctttttttttttctctctgtctctcttttcatttcaacggcgatgatcctttcccgagaagtatcttcagtgtcttagggaggtcacagcaacaaggcaaaacaataattaaagtacaacagaaggtagtgcagttctcgctgtggaaggaagcggtccgcaggcagctggcccgggatgcctgcacccaggtcgaggctgaaggacggggggtctcggtgttcccgcagctctaaggctgtggctgggggctggctcaggaagtcatcttcagggtgatgtgggggatgcaggtggaatgcggtgaggagaagaggagggcgctgggctccgggcccctgtcacagagtggactccaaagaggagtccaagatgtcatcgtgatggctgttgctgttggagtcgctgtcatagctctgggggctggagtagttggctgcctcctgcagcctcatcagcatgttcatcagcgggtcaccttcagcatcactggggggcatctgcttgcttgtcgatccctcccgaggcatggagtagccgtcgaagccgacatcctcaggccgtaactgcagcaggggaggccactcgtgctgttgtgggctggctgcccatggatatgtgtccatcacccacttggcaggatcctcccagggggcgcgccttccatagagctggagtccttctctgacggcttccaggagataggggataatggaatagttccacaagtcggtgaaccacactctcgagccgtccacatcgatggggcatgacaggaagagccgggggccgatggtgacgtccgaggaactgtgagcctccaggaagcggttgaggtgatgccagaccttgggaatccagtcaatgatttttaccagctccatattgcgcacccgcccactgatctctgtttccatgagcttcctcctcaggaatcggccaaggaaacccttcacaggctccgtgtggttggcacaaagcacccatctgaagttatggtgaagctgcaggttgggagtcgaagaggtagcctggttcattgtgccaattatgtaagggcatttgtggtacttgcagttgagcagcccattgaagatctctcccagagagctcacgtggtgtaggttgtccaggatgatgacgaggggcatgtccacagcattgttctcactgttgcactggtcagcaaggttggacaggtactggcgcaattccttgctggacttatggtccacgttaaaggtggcgataaccccgtctgtcaactcccgtccctctcgaagcactatatactcagacagccggttggccaggtaggttttcccagtgccgctggggccagagagaatgatccgacggtgctctatcaggagggagacgtagcgctgcaggatgggcttgggaatcaaggactcaaacaccagtgagtccaggctgttttctgcgagccctttcacagtcactgagatggtcgtgttctctccaaccagatagccacaaggaagcagctccggtgtttcggaagtgttgctgcgcttgatttctccaatgctgtagccaagaacgctgtctgaattcagccctagctgactcactgggtcgacatgaatgatgtattctttgaacagccgtctaaccaccccatcgagcacatcccacttcgtcttgccactaactccaatgcagccaataagaaagagatgtggtctggaatcctccttccacttcatttcctcctgaaagctgacaactatcttaacatgcctgcctccttccttccgagccgagcattcaccagtgtcatccagcaacatgtccaggctggttgactcagtgaggttcaagctgtgctgggagaggcccatggactgcctcggggaggcagagatggacacttgggaaggagcccggctgcagccactgccttgagactctgacttcagccgatcattctcagctttcagcttctctatttcactctgcatcctgttcatggcctcccggagctggtccagctggtgggcagaactgagagcttctaagcggatatccgtcagcttcatctccttgtctcttaactcatttcggagctgcatgacggtctcagcttcactatccatgcattctgaaattagagagttggagtgagaattcctcagcagtggggtggaacctgtggacccattgtgcggtaactttggtgaggaaggcaaagaagaatccgtcatctcctcaatatctgaatgagaggacgcagattttggggacttcttcttcccgaaagcttgcttgaaggagctgcgtaactcattgacccagttcttccgcttcttcttctttgagtcactctctatgttgctgcccacgctggagtggctggtggcactgttgatgctggagacgctgtctgaggagtgctgcctgcggatgcggaggtctgcagactgggcagtgccgtttcctttgcagttgagctcaggtgtgttaattactccattaatggcagcctgggcagctgcgttctgtttctttagcagctcaatggtttttcttaactcattcagttctgagtccttctgctcagctgtcatggtcagactctggagcctgattgtcatgttaccaagactctgttcaaaggctgccacaaggtgagcatttgctgtcagctgggtggtcaaagctgaaactttctcctgggaggcatccagttcccgccgcagcttgcgaatctctgactggcatttttcttctggtgtagaataaactgacgatgtgctggaaaccaaggagagtgaggatccatgaactaactcataccttgcgtgatggaacaaaggaagagagaaatgaagtgagctgtgaagacggctgacaaagttgtccacagaacttttctcccatgattcttcttcaaacccatcccggaatgagcctgaacggctcatggttctgctcttctcatccagggacatggagctattccggaagcggctgtcagtgtatggatcatactgcccatcagcattggagaggctgtgagtcctcagcatggtcgggttggacaagctcatctgggtgacagtggtgggactcgcaagctgggaaaagttgaatcttgttccggagggagaagtcacgctggagccagaggaaaagggggaattggcagcggtgtcctgaaggcctcctgcagaatgggaccgtaaccattcttttgcatcttcttgcgtgcgaagctgggaggtgggagtatacctgagtcctttcttaggcaaagtgttcctatcaaggtgcgggtcactgtcctgtttcctgggcagagtacttctgcagaacttagggctagcagcaggggaagagagagggctttctgacagtgtggtcttcacactgttagttctgacaaagggagtcaaggagtcgtccttggaggaggcgatgaggccagtggaagaattgtggctggggacccctccactgctgagggagatgtcgatggactcacagctggtgtggaggctgctgacagactgaaagcccaggccatccttgctaactgcggaggagctgctggcgttggtgccccaggtgaggctgttggaaggggccgagtgggctgagctggggctggaggctagcggagactggttgaggtccacattcttgctgtagagaggactgctgctcccactgctcaggacgccactgcctgacggggagtctaggttaccttgctgagtcatggtggcatgaggattggagatgaccaccgaatttttcatgttttcagctgtggcgatgggcacttgcttggtaggcttcccaccaaagagtctgcggagtgtgggagaggccacatctgggtacttggctccaggctggagactggtctgagccggactggacacaggctgggctgccggattcactttcaccgagttacaggaagccacactctcgttgtctgatgagatgcctttctccttgtctgtttggttgaccagacctggtagagagctgcctagggctgttttggaaggctccctcagtttgggcactggcaggcctgcggacttgctgctaatgttggaatctatgctgctggtgctagacctgttcccagccccgttccggctgttggacttactgggcctcggcaaactccggtactgaaggtttgtccgggagcttagggctagatacccgtcatcctgattctgagccccatccatacttgacttccgaccagcagaccgactgacgagtgcagatgactttgggattttgcccagtgtggctgacctgctggtgacagtcaccccgctggctgtgatcatggccaggccggcggcggaaccactctgcttcttgaacccaaagctgttggcattggcagtaggtgtcctagagctgctggggaggggctttttggattcgtcaccactgctccggcctgcatctgatggggagcgcttcacctgggaggctttaggagaaagccttcctttctcagacacctttgcgtcgtctgtttttccagttcctggggtcttcagtgcgcctgccggggctgaaggcttcgtccttggcatggtgatgcccacctgagctgtcatgcctcgccgccatgagcctgtctgggagatgacaggattcttcttgcccgacgtgcttttgtcggactcgtcagacacatcagaaggattccgcctccacttggaacctggctccatttttatgccgctgtctgagcctccgtctgatttcttgacatcatcaccagaccacagggaattcctctccacctgtgagtgcttctcagcatcagtctgcacatccaggttttttcgagaggaggcaggtgtgttggcataagagctgatggaggagctggtgttgatgtcatcagtgctgaggttgtctatggtgtcgctgatgccgctgctgacggagctgctgtcgtcccagctgtcagcgtctccgaggcccagggaggtatttcgttgcagggtctcccgtaccacagccatcccatcagggagccggttcaggcgacgggtatagaggccaagtccaccatcagtcatgtatccgcttgtaatgtcatcggtccggatgttcttgctcagaacatccccgtcgctcatgtagccgggggcatccatgctgatgccttccaggtccatctcatctcctgccttgtctgagacgtccacatggcagacactactgccccgggaggccagctgccttctcagaggggcggagtacacatagcgacctgactcagtgttgatgaacctgctggcgttggctcgagggggatacccattgcccattgagggggcgtctcctgcttggagccgagggctggactggcccagtctccaggacagaggtgtgggcctccctgtcaagctgagtatgctacggccactcatctccgtggtgacattggtgtcaaacgtggtttccaatgtgctgtgtgtaacctgagttccccttaaactggacatggtttcctccaaattctgccgcagatcagcgatgttcttcactgtccgcagccgccgagcctcaggatcttccccagtgagttcttccagagcaggctgtccagtcttggtgaagtggctgggctccacgctcacacctgttgagcttgactcggcagtaacattcccttcagtgtccgtctgagacctgtacaggaaaggtgcaaccgtggcagtgttgggatggttgtattgctgctggggctgaggtagctgaacactgacggtattgcttcctgtggtctgggtggtcccgacagacccactgacagtctggctgctgatgctgtggttcagggtggtccctcctgggccttttccttctgaggacgccaggctggaagaggaactggagtgtctgccgtccagctggggcttctgctgggggagtcctgagctcagcttcccactccggctccgctccccttccttggaaggcgctggggcacttggggatttcccgggcatgcttttcattcctggttttggtattccactgtgggaaggggccatgggctccttcttggcactgttgagcttcccccctttggggatgaagctggcaatcttggaggacttttttggcatctcgggcacagctgctccactggggtcttcttttggctcctccttgaggtccagcctctccgtcacagaggctctcttggcaaggtccttgcttttctccttatccttctcccgctgttgtttctccttctctttctcattgcctttcagagaactcttcttgttggtcagtgcccggctaaaagtcctctgggcaatgcccttgagtgcaatcttggggctgctggaagcagggcccacggtggtgagcatgcgactggcggcctccagctcctcgctctcttcgaagctgggcagagtctccagccgctcacagcttgtgtcccgggaccccggcccctcacctgcctttgagccccctttactgttgaaaagtttcagcttttccagcatggacttctgattgttgggggccggcttcatggcttcaggtgtgggcctgggggcctcaggcccaggaggcttgaccgagagcatggataccgtggcactgtgcttcacgctgagggatttgctgcgccaaggcttggtggctgcaccgggctgcgggatggccgaggaggtactgcaattagtaggggtggagctgctgccgctctccaaggaagcaggtgcattgtcactcattccggggtgggaggaggctgaacttgccaaaggctctttctcgtggctgcttggcggtgggggtggggaggtgactggtttggatttatcatagttgttaaagctctggctgcgtcggttgttagcagtagttgaccctccgcgtgttttggcctcgctgcctgcagcggataccctcgcggtaggacctggaagtctagagatctttttctgacccagagtgaagcggatgattttgctttgagatgagtccttggatgatgcactggactgcatttcagcttgtgcttttgactgctgatgtggcgctggctggtgaggctggcacggggcttggggagtgactggcacctgctgctgaggggtgccagcctggcactgggagggggccccggccacctgggatacggcgggcggcagaggtgaggagaggtgctgcttctggggctgctgctgctgctgcttgtatcgggagaggctgaagaagaggcctagaatggccttgaggtttccattcctgatctcttctgcagacagcccctggatgtttattcccttagctgccaggaaattcaagcaggcatctatgttttcaatcatttgggatctgttcttcggacagccattgatgtcttcaatcttttcatttgccacaacctggataatctgggccaggaggacgccatctgtcacatcttgctggagatccctgatgagacgcttgtggccggatttggctaggtaatgattggcccagtctgtgtagatcctcttttgatcttccagtccgtggataactggctttctcttctgctgttggctggactcagaaaccgattccatttcccagaaataaaatcctctctctccttcagcgatgcttccaaatccacagaggaacaaaataacccacacaaaagtgatgcatgcaacagccagacagagttcccgccagccaaggaaatcagcaccacctcttcaaaggtcttcctgtcttcttaaaatccactcgggaacctcactcggcaccactgcctttgcaatgagggtgactgctgccggcatcatgagagctaagtcttggggttttactttaggtctgagactcgcttcatgagagcccagaggacaaatctgggcaaagacaagtccatatcctgaggcacataccacattactgccccagaaaccctttccttcactgtctccttggcacagataatttatatgtcaataacaatgtaaatgggcatttaatccaccaagctgctaacatccacatccctctctggcagcccctgactcccataaatcactgcaaacactgcgcggaaagccgcccctcatggctcctgcaagcgttcatcacagcggtggctcccctcctgggctgtcatcttccttcatggtgtaagacccatacctgaggagaaaacgttcaacagtcagatttgtcttttgtagaaaagtacagatttgagctgtctttcccaccatctggagccacatagtgaggcctgaaccaagcagcagccgatgatcgttttccaagctcctctgagcacatccatggacaaggaaactccaggggcctca

SEQ ID NO: 17889 - RNA, 11140 nt, Homo sapiens
  source 1..11140: mol_type = other RNA
tcggcctggggaggaggaaggggagggaggatggaaacataccgtacacaaaatactcaattcctagttttctctttaaaaatggctagaaaaaattcatcaaaatgcagcactttaatcaattatttacaatttctatgttacaatgaaaaaatgtacatcttatagaacatatttcataaaactgctccactggaaacaactagatcaaaacagcaaaccttccatttaatatccacaaagttggattatttttcctttttgaagtagattcgccacaatcaaatttgaatacagagaattttgaagtttaagcatcaaacaacaaagtaaaagtccccaagatacaacaaagatctaggcaagtcttgttcctgtcccactcccaccccacccctaatgaaacttaaaaggtattcccatttcaattatggcctgtatcattcttggcagtttgggaagagaacttttggcttccattggtaactcaacataaatgttgcatagaatttatatatttcaaaattggcctaactgtagaaaaggcaaaatggaagcatttccgatagagccctaaatgagtacaaagtcactttgtaaaaggtgagtgacactaaagtaaaaatatgaccaaaataagaaatgtgcatattagacaaccctgcttcccgaaactttaggaaggacacggagttgtgagtcacacaagggctatgctacttgaagtcaatgttcaccaatcaggcagcactaggtacagaagtcttggttctgaacctggacccaggagggaagtctgtgggaaaggggagaagagaatgacaagagaggatgtcatattaaaaaaaggtttcaaacaatattggcaggtgtctactcacaaggtgattggaaaactgcccacgaggagaagtcaactttacctcctcccaaattcacagtacgcgagtgtagtagggtcattgctgggagataaattgtctgaggagggccacccttcaggtttaccagaaatcttagggtttggcccccctggtcacaggctaaatatatggtttaaaagttttattaaaaagaaaaacagaacaagacacactcacacccagatgactaatgaaggctaagcagaatagtctgagtttgctgagactaaagcagggatagtgttgaaaagttttcctttcactagtgggacacattccccttttcttttcaaagaggaagaacatggtgtcatccaatgtgaagtgagcagtttcgggtcaaactcttatggtaagaaactaaaaaaagatgccaagagacaaaccttcagaaatagaagaaatgcaaaagatggaataaaaaccctgatcattaaaacagagacaccttcactggtgtccaataaggattctctttacaaaacagaaacaaacaactcaaaaatttaccatactttgtaatgaaaataccagtatgttgaagacacagcagactgggtttctattagaacaagtatcagcaaggtcatgtagacttgtagaaacttttgccttctcctgcaccagacagatcattgtccagttgggttgtcagctggagaccgaaaagaacctaaaaaatggatctttttttttttctttttcccatggtcacgcatccacacaaatgagtcttttggatgagaaaagtcacagcaacttgagttctcctaatgaacagatgactttttagccctgtttgtttcaatggggaaaacaatgacaaaaaaaacaaaccccaggcaggcacgacacttatgtaaaatgaacacagttagtacaaaaccagtaaggcatcactttgggaaggtcagcaccgaagaggtcaggcaaggctcgtccagacggggcttctgggagggagtgaccctcacccttattgagctgcgtcatgttggttctgaggaaagtgcaagtcttttgcagggtgaccgcatcaccccaccggaagctggggcggggacgctggaggtgttggtgtgtgttctaaaccctcaaggacgagaagggaaggcaaggtccatggctcacccacatgtcgaggaccaggtcctcatccattttaaaggacacagatacccccagccctagcaggaggaggcgagtgtgtaggactgtgaggatggacaactaaaaaccaaaactgagcaggaccaaaccaaaactcaactcctgcggttcttactttcaccaaaggattgattctgaccaagaggggaagggggaaaaaaaaatcttcaaaaatcaatgcatcagaaaggaagaaactcaacctcattttcaaaaggtaacctgttctccaaagtagaacaagtctcactatacacagtgtttgcagaaaaaaaaaaaaaaaaacctgattcattcatatatcagaaggaaagagacacatgctgttctgcactgacagccacatccactcgctcacactctcactccgtcactcactctcacggatattaatcagaggctgatggacctgaatggggtggtttgattggaacaggcaaaatacctctcgggtaaggaaagcaccatttaaaaaacatgaaagcacggtttatttgctcctaaggtttccctgtgtcgtagctctgtagtgcgttgaacgtgaccaaagcaagcaccctggttagcaccagttctccctgtggccggctgtgtgggagggtgggtggcacggctctgagacccagtctggagggtctgtgctgaggggaagccgtgcttctctgtgtttccgactttgctccagtctcttctgtctctgggaagctcatggcaggatgctgtttggtttcagagcttcatgtgggttctctttttttttttctctctgtctctcttttcatttcaacggcgatgatcctttcccgagaagtatcttcagtgtcttagggaggtcacagcaacaaggcaaaacaataattaaagtacaacagaaggtagtgcagttctcgctgtggaaggaagcggtccgcaggcagctggcccgggatgcctgcacccaggtcgaggctgaaggacggggggtctcggtgttcccgcagctctaaggctgtggctgggggctggctcaggaagtcatcttcagggtgatgtgggggatgcaggtggaatgcggtgaggagaagaggagggcgctgggctccgggcccctgtcacagagtggactccaaagaggagtccaagatgtcatcgtgatggctgttgctgttggagtcgctgtcatagctctgggggctggagtagttggctgcctcctgcagcctcatcagcatgttcatcagcgggtcaccttcagcatcactggggggcatctgcttgcttgtcgatccctcccgaggcatggagtagccgtcgaagccgacatcctcaggccgtaactgcagcaggggaggccactcgtgctgttgtgggctggctgcccatggatatgtgtccatcacccacttggcaggatcctcccagggggcgcgccttccatagagctggagtccttctctgacggcttccaggagataggggataatggaatagttccacaagtcggtgaaccacactctcgagccgtccacatcgatggggcatgacaggaagagccgggggccgatggtgacgtccgaggaactgtgagcctccaggaagcggttgaggtgatgccagaccttgggaatccagtcaatgatttttaccagctccatattgcgcacccgcccactgatctctgtttccatgagcttcctcctcaggaatcggccaaggaaacccttcacaggctccgtgtggttggcacaaagcacccatctgaagttatggtgaagctgcaggttgggagtcgaagaggtagcctggttcattgtgccaattatgtaagggcatttgtggtacttgcagttgagcagcccattgaagatctctcccagagagctcacgtggtgtaggttgtccaggatgatgacgaggggcatgtccacagcattgttctcactgttgcactggtcagcaaggttggacaggtactggcgcaattccttgctggacttatggtccacgttaaaggtggcgataaccccgtctgtcaactcccgtccctctcgaagcactatatactcagacagccggttggccaggtaggttttcccagtgccgctggggccagagagaatgatccgacggtgctctatcaggagggagacgtagcgctgcaggatgggcttgggaatcaaggactcaaacaccagtgagtccaggctgttttctgcgagccctttcacagtcactgagatggtcgtgttctctccaaccagatagccacaaggaagcagctccggtgtttcggaagtgttgctgcgcttgatttctccaatgctgtagccaagaacgctgtctgaattcagccctagctgactcactgggtcgacatgaatgatgtattctttgaacagccgtctaaccaccccatcgagcacatcccacttcgtcttgccactaactccaatgcagccaataagaaagagatgtggtctggaatcctccttccacttcatttcctcctgaaagctgacaactatcttaacatgcctgcctccttccttccgagccgagcattcaccagtgtcatccagcaacatgtccaggctggttgactcagtgaggttcaagctgtgctgggagaggcccatggactgcctcggggaggcagagatggacacttgggaaggagcccggctgcagccactgccttgagactctgacttcagccgatcattctcagctttcagcttctctatttcactctgcatcctgttcatggcctcccggagctggtccagctggtgggcagaactgagagcttctaagcggatatccgtcagcttcatctccttgtctcttaactcatttcggagctgcatgacggtctcagcttcactatccatgcattctgaaattagagagttggagtgagaattcctcagcagtggggtggaacctgtggacccattgtgcggtaactttggtgaggaaggcaaagaagaatccgtcatctcctcaatatctgaatgagaggacgcagattttggggacttcttcttcccgaaagcttgcttgaaggagctgcgtaactcattgacccagttcttccgcttcttcttctttgagtcactctctatgttgctgcccacgctggagtggctggtggcactgttgatgctggagacgctgtctgaggagtgctgcctgcggatgcggaggtctgcagactgggcagtgccgtttcctttgcagttgagctcaggtgtgttaattactccattaatggcagcctgggcagctgcgttctgtttctttagcagctcaatggtttttcttaactcattcagttctgagtccttctgctcagctgtcatggtcagactctggagcctgattgtcatgttaccaagactctgttcaaaggctgccacaaggtgagcatttgctgtcagctgggtggtcaaagctgaaactttctcctgggaggcatccagttcccgccgcagcttgcgaatctctgactggcatttttcttctggtgtagaataaactgacgatgtgctggaaaccaaggagagtgaggatccatgaactaactcataccttgcgtgatggaacaaaggaagagagaaatgaagtgagctgtgaagacggctgacaaagttgtccacagaacttttctcccatgattcttcttcaaacccatcccggaatgagcctgaacggctcatggttctgctcttctcatccagggacatggagctattccggaagcggctgtcagtgtatggatcatactgcccatcagcattggagaggctgtgagtcctcagcatggtcgggttggacaagctcatctgggtgacagtggtgggactcgcaagctgggaaaagttgaatcttgttccggagggagaagtcacgctggagccagaggaaaagggggaattggcagcggtgtcctgaaggcctcctgcagaatgggaccgtaaccattcttttgcatcttcttgcgtgcgaagctgggaggtgggagtatacctgagtcctttcttaggcaaagtgttcctatcaaggtgcgggtcactgtcctgtttcctgggcagagtacttctgcagaacttagggctagcagcaggggaagagagagggctttctgacagtgtggtcttcacactgttagttctgacaaagggagtcaaggagtcgtccttggaggaggcgatgaggccagtggaagaattgtggctggggacccctccactgctgagggagatgtcgatggactcacagctggtgtggaggctgctgacagactgaaagcccaggccatccttgctaactgcggaggagctgctggcgttggtgccccaggtgaggctgttggaaggggccgagtgggctgagctggggctggaggctagcggagactggttgaggtccacattcttgctgtagagaggactgctgctcccactgctcaggacgccactgcctgacggggagtctaggttaccttgctgagtcatggtggcatgaggattggagatgaccaccgaatttttcatgttttcagctgtggcgatgggcacttgcttggtaggcttcccaccaaagagtctgcggagtgtgggagaggccacatctgggtacttggctccaggctggagactggtctgagccggactggacacaggctgggctgccggattcactttcaccgagttacaggaagccacactctcgttgtctgatgagatgcctttctccttgtctgtttggttgaccagacctggtagagagctgcctagggctgttttggaaggctccctcagtttgggcactggcaggcctgcggacttgctgctaatgttggaatctatgctgctggtgctagacctgttcccagccccgttccggctgttggacttactgggcctcggcaaactccggtactgaaggtttgtccgggagcttagggctagatacccgtcatcctgattctgagccccatccatacttgacttccgaccagcagaccgactgacgagtgcagatgactttgggattttgcccagtgtggctgacctgctggtgacagtcaccccgctggctgtgatcatggccaggccggcggcggaaccactctgcttcttgaacccaaagctgttggcattggcagtaggtgtcctagagctgctggggaggggctttttggattcgtcaccactgctccggcctgcatctgatggggagcgcttcacctgggaggctttaggagaaagccttcctttctcagacacctttgcgtcgtctgtttttccagttcctggggtcttcagtgcgcctgccggggctgaaggcttcgtccttggcatggtgatgcccacctgagctgtcatgcctcgccgccatgagcctgtctgggagatgacaggattcttcttgcccgacgtgcttttgtcggactcgtcagacacatcagaaggattccgcctccacttggaacctggctccatttttatgccgctgtctgagcctccgtctgatttcttgacatcatcaccagaccacagggaattcctctccacctgtgagtgcttctcagcatcagtctgcacatccaggttttttcgagaggaggcaggtgtgttggcataagagctgatggaggagctggtgttgatgtcatcagtgctgaggttgtctatggtgtcgctgatgccgctgctgacggagctgctgtcgtcccagctgtcagcgtctccgaggcccagggaggtatttcgttgcagggtctcccgtaccacagccatcccatcagggagccggttcaggcgacgggtatagaggccaagtccaccatcagtcatgtatccgcttgtaatgtcatcggtccggatgttcttgctcagaacatccccgtcgctcatgtagccgggggcatccatgctgatgccttccaggtccatctcatctcctgccttgtctgagacgtccacatggcagacactactgccccgggaggccagctgccttctcagaggggcggagtacacatagcgacctgactcagtgttgatgaacctgctggcgttggctcgagggggatacccattgcccattgagggggcgtctcctgcttggagccgagggctggactggcccagtctccaggacagaggtgtgggcctccctgtcaagctgagtatgctacggccactcatctccgtggtgacattggtgtcaaacgtggtttccaatgtgctgtgtgtaacctgagttccccttaaactggacatggtttcctccaaattctgccgcagatcagcgatgttcttcactgtccgcagccgccgagcctcaggatcttccccagtgagttcttccagagcaggctgtccagtcttggtgaagtggctgggctccacgctcacacctgttgagcttgactcggcagtaacattcccttcagtgtccgtctgagacctgtacaggaaaggtgcaaccgtggcagtgttgggatggttgtattgctgctggggctgaggtagctgaacactgacggtattgcttcctgtggtctgggtggtcccgacagacccactgacagtctggctgctgatgctgtggttcagggtggtccctcctgggccttttccttctgaggacgccaggctggaagaggaactggagtgtctgccgtccagctggggcttctgctgggggagtcctgagctcagcttcccactccggctccgctccccttccttggaaggcgctggggcacttggggatttcccgggcatgcttttcattcctggttttggtattccactgtgggaaggggccatgggctccttcttggcactgttgagcttcccccctttggggatgaagctggcaatcttggaggacttttttggcatctcgggcacagctgctccactggggtcttcttttggctcctccttgaggtccagcctctccgtcacagaggctctcttggcaaggtccttgcttttctccttatccttctcccgctgttgtttctccttctctttctcattgcctttcagagaactcttcttgttggtcagtgcccggctaaaagtcctctgggcaatgcccttgagtgcaatcttggggctgctggaagcagggcccacggtggtgagcatgcgactggcggcctccagctcctcgctctcttcgaagctgggcagagtctccagccgctcacagcttgtgtcccgggaccccggcccctcacctgcctttgagccccctttactgttgaaaagtttcagcttttccagcatggacttctgattgttgggggccggcttcatggcttcaggtgtgggcctgggggcctcaggcccaggaggcttgaccgagagcatggataccgtggcactgtgcttcacgctgagggatttgctgcgccaaggcttggtggctgcaccgggctgcgggatggccgaggaggtactgcaattagtaggggtggagctgctgccgctctccaaggaagcaggtgcattgtcactcattccggggtgggaggaggctgaacttgccaaaggctctttctcgtggctgcttggcggtgggggtggggaggtgactggtttggatttatcatagttgttaaagctctggctgcgtcggttgttagcagtagttgaccctccgcgtgttttggcctcgctgcctgcagcggataccctcgcggtaggacctggaagtctagagatctttttctgacccagagtgaagcggatgattttgctttgagatgagtccttggatgatgcactggactgcatttcagcttgtgcttttgactgctgatgtggcgctggctggtgaggctggcacggggcttggggagtgactggcacctgctgctgaggggtgccagcctggcactgggagggggccccggccacctgggatacggcgggcggcagaggtgaggagaggtgctgcttctggggctgctgctgctgctgcttgtatcgggagaggctgaagaagaggcctagaatggccttgaggtttccattcctgatctcttctgcagacagcccctggatgtttattcccttagctgccaggaaattcaagcaggcatctatgttttcaatcatttgggatctgttcttcggacagccattgatgtcttcaatcttttcatttgccacaacctggataatctgggccaggaggacgccatctgtcacatcttgctggagatccctgatgagacgcttgtggccggatttggctaggtaatgattggcccagtctgtgtagatcctcttttgatcttccagtccgtggataactggctttctcttctgctgttggctggactcagaaaccgattccatttcccagaaataaaatcctctctctccttcagcgatgcttccaaatccacagaggaacaaaataacccacacaaaagtgatgcatgcaacagccagacagagttcccgccagccaaggaaatcagcaccacctcttcaaaggtcttcctgtcttcttaaaatccactcgggaacctcactcggcaccactgcctttgcaatgagggtgactgctgccggcatcatgagagctaagtcttggggttttactttaggtctgagactcgcttcatgagagcccagaggacaaatctgggcaaagacaagtccatatcctgaggcacataccacattactgccccagaaaccctttccttcactgtctccttggcacagataatttatatgtcaataacaatgtaaatgggcatttaatccaccaagctgctaacatccacatccctctctggcagcccctgactcccataaatcactgcaaacactgcgcggaaagccgcccctcatggctcctgcaagcgttcatcacagcggtggctcccctcctgggctgtcatcttccttcatggtgtaagacccatacctgcgcccacaccggcttcgcggagccgcctcctccagccggtctcgcactgcactccggcccgcgcttctcagccgcggccgctgccgctgcagccgctc

SEQ ID NO: 17890 - RNA, 11378 nt, Homo sapiens
  source 1..11378: mol_type = other RNA
tcggcctggggaggaggaaggggagggaggatggaaacataccgtacacaaaatactcaattcctagttttctctttaaaaatggctagaaaaaattcatcaaaatgcagcactttaatcaattatttacaatttctatgttacaatgaaaaaatgtacatcttatagaacatatttcataaaactgctccactggaaacaactagatcaaaacagcaaaccttccatttaatatccacaaagttggattatttttcctttttgaagtagattcgccacaatcaaatttgaatacagagaattttgaagtttaagcatcaaacaacaaagtaaaagtccccaagatacaacaaagatctaggcaagtcttgttcctgtcccactcccaccccacccctaatgaaacttaaaaggtattcccatttcaattatggcctgtatcattcttggcagtttgggaagagaacttttggcttccattggtaactcaacataaatgttgcatagaatttatatatttcaaaattggcctaactgtagaaaaggcaaaatggaagcatttccgatagagccctaaatgagtacaaagtcactttgtaaaaggtgagtgacactaaagtaaaaatatgaccaaaataagaaatgtgcatattagacaaccctgcttcccgaaactttaggaaggacacggagttgtgagtcacacaagggctatgctacttgaagtcaatgttcaccaatcaggcagcactaggtacagaagtcttggttctgaacctggacccaggagggaagtctgtgggaaaggggagaagagaatgacaagagaggatgtcatattaaaaaaaggtttcaaacaatattggcaggtgtctactcacaaggtgattggaaaactgcccacgaggagaagtcaactttacctcctcccaaattcacagtacgcgagtgtagtagggtcattgctgggagataaattgtctgaggagggccacccttcaggtttaccagaaatcttagggtttggcccccctggtcacaggctaaatatatggtttaaaagttttattaaaaagaaaaacagaacaagacacactcacacccagatgactaatgaaggctaagcagaatagtctgagtttgctgagactaaagcagggatagtgttgaaaagttttcctttcactagtgggacacattccccttttcttttcaaagaggaagaacatggtgtcatccaatgtgaagtgagcagtttcgggtcaaactcttatggtaagaaactaaaaaaagatgccaagagacaaaccttcagaaatagaagaaatgcaaaagatggaataaaaaccctgatcattaaaacagagacaccttcactggtgtccaataaggattctctttacaaaacagaaacaaacaactcaaaaatttaccatactttgtaatgaaaataccagtatgttgaagacacagcagactgggtttctattagaacaagtatcagcaaggtcatgtagacttgtagaaacttttgccttctcctgcaccagacagatcattgtccagttgggttgtcagctggagaccgaaaagaacctaaaaaatggatctttttttttttctttttcccatggtcacgcatccacacaaatgagtcttttggatgagaaaagtcacagcaacttgagttctcctaatgaacagatgactttttagccctgtttgtttcaatggggaaaacaatgacaaaaaaaacaaaccccaggcaggcacgacacttatgtaaaatgaacacagttagtacaaaaccagtaaggcatcactttgggaaggtcagcaccgaagaggtcaggcaaggctcgtccagacggggcttctgggagggagtgaccctcacccttattgagctgcgtcatgttggttctgaggaaagtgcaagtcttttgcagggtgaccgcatcaccccaccggaagctggggcggggacgctggaggtgttggtgtgtgttctaaaccctcaaggacgagaagggaaggcaaggtccatggctcacccacatgtcgaggaccaggtcctcatccattttaaaggacacagatacccccagccctagcaggaggaggcgagtgtgtaggactgtgaggatggacaactaaaaaccaaaactgagcaggaccaaaccaaaactcaactcctgcggttcttactttcaccaaaggattgattctgaccaagaggggaagggggaaaaaaaaatcttcaaaaatcaatgcatcagaaaggaagaaactcaacctcattttcaaaaggtaacctgttctccaaagtagaacaagtctcactatacacagtgtttgcagaaaaaaaaaaaaaaaaacctgattcattcatatatcagaaggaaagagacacatgctgttctgcactgacagccacatccactcgctcacactctcactccgtcactcactctcacggatattaatcagaggctgatggacctgaatggggtggtttgattggaacaggcaaaatacctctcgggtaaggaaagcaccatttaaaaaacatgaaagcacggtttatttgctcctaaggtttccctgtgtcgtagctctgtagtgcgttgaacgtgaccaaagcaagcaccctggttagcaccagttctccctgtggccggctgtgtgggagggtgggtggcacggctctgagacccagtctggagggtctgtgctgaggggaagccgtgcttctctgtgtttccgactttgctccagtctcttctgtctctgggaagctcatggcaggatgctgtttggtttcagagcttcatgtgggttctctttttttttttctctctgtctctcttttcatttcaacggcgatgatcctttcccgagaagtatcttcagtgtcttagggaggtcacagcaacaaggcaaaacaataattaaagtacaacagaaggtagtgcagttctcgctgtggaaggaagcggtccgcaggcagctggcccgggatgcctgcacccaggtcgaggctgaaggacggggggtctcggtgttcccgcagctctaaggctgtggctgggggctggctcaggaagtcatcttcagggtgatgtgggggatgcaggtggaatgcggtgaggagaagaggagggcgctgggctccgggcccctgtcacagagtggactccaaagaggagtccaagatgtcatcgtgatggctgttgctgttggagtcgctgtcatagctctgggggctggagtagttggctgcctcctgcagcctcatcagcatgttcatcagcgggtcaccttcagcatcactggggggcatctgcttgcttgtcgatccctcccgaggcatggagtagccgtcgaagccgacatcctcaggccgtaactgcagcaggggaggccactcgtgctgttgtgggctggctgcccatggatatgtgtccatcacccacttggcaggatcctcccagggggcgcgccttccatagagctggagtccttctctgacggcttccaggagataggggataatggaatagttccacaagtcggtgaaccacactctcgagccgtccacatcgatggggcatgacaggaagagccgggggccgatggtgacgtccgaggaactgtgagcctccaggaagcggttgaggtgatgccagaccttgggaatccagtcaatgatttttaccagctccatattgcgcacccgcccactgatctctgtttccatgagcttcctcctcaggaatcggccaaggaaacccttcacaggctccgtgtggttggcacaaagcacccatctgaagttatggtgaagctgcaggttgggagtcgaagaggtagcctggttcattgtgccaattatgtaagggcatttgtggtacttgcagttgagcagcccattgaagatctctcccagagagctcacgtggtgtaggttgtccaggatgatgacgaggggcatgtccacagcattgttctcactgttgcactggtcagcaaggttggacaggtactggcgcaattccttgctggacttatggtccacgttaaaggtggcgataaccccgtctgtcaactcccgtccctctcgaagcactatatactcagacagccggttggccaggtaggttttcccagtgccgctggggccagagagaatgatccgacggtgctctatcaggagggagacgtagcgctgcaggatgggcttgggaatcaaggactcaaacaccagtgagtccaggctgttttctgcgagccctttcacagtcactgagatggtcgtgttctctccaaccagatagccacaaggaagcagctccggtgtttcggaagtgttgctgcgcttgatttctccaatgctgtagccaagaacgctgtctgaattcagccctagctgactcactgggtcgacatgaatgatgtattctttgaacagccgtctaaccaccccatcgagcacatcccacttcgtcttgccactaactccaatgcagccaataagaaagagatgtggtctggaatcctccttccacttcatttcctcctgaaagctgacaactatcttaacatgcctgcctccttccttccgagccgagcattcaccagtgtcatccagcaacatgtccaggctggttgactcagtgaggttcaagctgtgctgggagaggcccatggactgcctcggggaggcagagatggacacttgggaaggagcccggctgcagccactgccttgagactctgacttcagccgatcattctcagctttcagcttctctatttcactctgcatcctgttcatggcctcccggagctggtccagctggtgggcagaactgagagcttctaagcggatatccgtcagcttcatctccttgtctcttaactcatttcggagctgcatgacggtctcagcttcactatccatgcattctgaaattagagagttggagtgagaattcctcagcagtggggtggaacctgtggacccattgtgcggtaactttggtgaggaaggcaaagaagaatccgtcatctcctcaatatctgaatgagaggacgcagattttggggacttcttcttcccgaaagcttgcttgaaggagctgcgtaactcattgacccagttcttccgcttcttcttctttgagtcactctctatgttgctgcccacgctggagtggctggtggcactgttgatgctggagacgctgtctgaggagtgctgcctgcggatgcggaggtctgcagactgggcagtgccgtttcctttgcagttgagctcaggtgtgttaattactccattaatggcagcctgggcagctgcgttctgtttctttagcagctcaatggtttttcttaactcattcagttctgagtccttctgctcagctgtcatggtcagactctggagcctgattgtcatgttaccaagactctgttcaaaggctgccacaaggtgagcatttgctgtcagctgggtggtcaaagctgaaactttctcctgggaggcatccagttcccgccgcagcttgcgaatctctgactggcatttttcttctggtgtagaataaactgacgatgtgctggaaaccaaggagagtgaggatccatgaactaactcataccttgcgtgatggaacaaaggaagagagaaatgaagtgagctgtgaagacggctgacaaagttgtccacagaacttttctcccatgattcttcttcaaacccatcccggaatgagcctgaacggctcatggttctgctcttctcatccagggacatggagctattccggaagcggctgtcagtgtatggatcatactgcccatcagcattggagaggctgtgagtcctcagcatggtcgggttggacaagctcatctgggtgacagtggtgggactcgcaagctgggaaaagttgaatcttgttccggagggagaagtcacgctggagccagaggaaaagggggaattggcagcggtgtcctgaaggcctcctgcagaatgggaccgtaaccattcttttgcatcttcttgcgtgcgaagctgggaggtgggagtatacctgagtcctttcttaggcaaagtgttcctatcaaggtgcgggtcactgtcctgtttcctgggcagagtacttctgcagaacttagggctagcagcaggggaagagagagggctttctgacagtgtggtcttcacactgttagttctgacaaagggagtcaaggagtcgtccttggaggaggcgatgaggccagtggaagaattgtggctggggacccctccactgctgagggagatgtcgatggactcacagctggtgtggaggctgctgacagactgaaagcccaggccatccttgctaactgcggaggagctgctggcgttggtgccccaggtgaggctgttggaaggggccgagtgggctgagctggggctggaggctagcggagactggttgaggtccacattcttgctgtagagaggactgctgctcccactgctcaggacgccactgcctgacggggagtctaggttaccttgctgagtcatggtggcatgaggattggagatgaccaccgaatttttcatgttttcagctgtggcgatgggcacttgcttggtaggcttcccaccaaagagtctgcggagtgtgggagaggccacatctgggtacttggctccaggctggagactggtctgagccggactggacacaggctgggctgccggattcactttcaccgagttacaggaagccacactctcgttgtctgatgagatgcctttctccttgtctgtttggttgaccagacctggtagagagctgcctagggctgttttggaaggctccctcagtttgggcactggcaggcctgcggacttgctgctaatgttggaatctatgctgctggtgctagacctgttcccagccccgttccggctgttggacttactgggcctcggcaaactccggtactgaaggtttgtccgggagcttagggctagatacccgtcatcctgattctgagccccatccatacttgacttccgaccagcagaccgactgacgagtgcagatgactttgggattttgcccagtgtggctgacctgctggtgacagtcaccccgctggctgtgatcatggccaggccggcggcggaaccactctgcttcttgaacccaaagctgttggcattggcagtaggtgtcctagagctgctggggaggggctttttggattcgtcaccactgctccggcctgcatctgatggggagcgcttcacctgggaggctttaggagaaagccttcctttctcagacacctttgcgtcgtctgtttttccagttcctggggtcttcagtgcgcctgccggggctgaaggcttcgtccttggcatggtgatgcccacctgagctgtcatgcctcgccgccatgagcctgtctgggagatgacaggattcttcttgcccgacgtgcttttgtcggactcgtcagacacatcagaaggattccgcctccacttggaacctggctccatttttatgccgctgtctgagcctccgtctgatttcttgacatcatcaccagaccacagggaattcctctccacctgtgagtgcttctcagcatcagtctgcacatccaggttttttcgagaggaggcaggtgtgttggcataagagctgatggaggagctggtgttgatgtcatcagtgctgaggttgtctatggtgtcgctgatgccgctgctgacggagctgctgtcgtcccagctgtcagcgtctccgaggcccagggaggtatttcgttgcagggtctcccgtaccacagccatcccatcagggagccggttcaggcgacgggtatagaggccaagtccaccatcagtcatgtatccgcttgtaatgtcatcggtccggatgttcttgctcagaacatccccgtcgctcatgtagccgggggcatccatgctgatgccttccaggtccatctcatctcctgccttgtctgagacgtccacatggcagacactactgccccgggaggccagctgccttctcagaggggcggagtacacatagcgacctgactcagtgttgatgaacctgctggcgttggctcgagggggatacccattgcccattgagggggcgtctcctgcttggagccgagggctggactggcccagtctccaggacagaggtgtgggcctccctgtcaagctgagtatgctacggccactcatctccgtggtgacattggtgtcaaacgtggtttccaatgtgctgtgtgtaacctgagttccccttaaactggacatggtttcctccaaattctgccgcagatcagcgatgttcttcactgtccgcagccgccgagcctcaggatcttccccagtgagttcttccagagcaggctgtccagtcttggtgaagtggctgggctccacgctcacacctgttgagcttgactcggcagtaacattcccttcagtgtccgtctgagacctgtacaggaaaggtgcaaccgtggcagtgttgggatggttgtattgctgctggggctgaggtagctgaacactgacggtattgcttcctgtggtctgggtggtcccgacagacccactgacagtctggctgctgatgctgtggttcagggtggtccctcctgggccttttccttctgaggacgccaggctggaagaggaactggagtgtctgccgtccagctggggcttctgctgggggagtcctgagctcagcttcccactccggctccgctccccttccttggaaggcgctggggcacttggggatttcccgggcatgcttttcattcctggttttggtattccactgtgggaaggggccatgggctccttcttggcactgttgagcttcccccctttggggatgaagctggcaatcttggaggacttttttggcatctcgggcacagctgctccactggggtcttcttttggctcctccttgaggtccagcctctccgtcacagaggctctcttggcaaggtccttgcttttctccttatccttctcccgctgttgtttctccttctctttctcattgcctttcagagaactcttcttgttggtcagtgcccggctaaaagtcctctgggcaatgcccttgagtgcaatcttggggctgctggaagcagggcccacggtggtgagcatgcgactggcggcctccagctcctcgctctcttcgaagctgggcagagtctccagccgctcacagcttgtgtcccgggaccccggcccctcacctgcctttgagccccctttactgttgaaaagtttcagcttttccagcatggacttctgattgttgggggccggcttcatggcttcaggtgtgggcctgggggcctcaggcccaggaggcttgaccgagagcatggataccgtggcactgtgcttcacgctgagggatttgctgcgccaaggcttggtggctgcaccgggctgcgggatggccgaggaggtactgcaattagtaggggtggagctgctgccgctctccaaggaagcaggtgcattgtcactcattccggggtgggaggaggctgaacttgccaaaggctctttctcgtggctgcttggcggtgggggtggggaggtgactggtttggatttatcatagttgttaaagctctggctgcgtcggttgttagcagtagttgaccctccgcgtgttttggcctcgctgcctgcagcggataccctcgcggtaggacctggaagtctagagatctttttctgacccagagtgaagcggatgattttgctttgagatgagtccttggatgatgcactggactgcatttcagcttgtgcttttgactgctgatgtggcgctggctggtgaggctggcacggggcttggggagtgactggcacctgctgctgaggggtgccagcctggcactgggagggggccccggccacctgggatacggcgggcggcagaggtgaggagaggtgctgcttctggggctgctgctgctgctgcttgtatcgggagaggctgaagaagaggcctagaatggccttgaggtttccattcctgatctcttctgcagacagcccctggatgtttattcccttagctgccaggaaattcaagcaggcatctatgttttcaatcatttgggatctgttcttcggacagccattgatgtcttcaatcttttcatttgccacaacctggataatctgggccaggaggacgccatctgtcacatcttgctggagatccctgatgagacgcttgtggccggatttggctaggtaatgattggcccagtctgtgtagatctccaccttgcttcccaacttcaggtagcagggctgggggcccgcccgggccgggggcacgtgcaggatgggcgcggcgctgtgcacgggtttgggcagtcccgacttcattttggaggcgaccaggatggccggcatcttctcccggggcttgggctttcccagcacgtccctggcagcggcggcgggggcgaccgctaaaggcagcgcgggtagcagagcaggcgccgggccttagcccacgaggcgcccaccaccagcggctaaaaaaaaaatccccaggtcggggaactcgaagcaatcgggcgagcgcgcctttggggtgccgggatgggaatgggggactggccacggcgctcagcgggtcccacctggacggatgctgccgccgggtctcacacctctcctgggtggcctttcaagagctctgggcgctcaggggctgccgcctcttgcaaatttcctcctgggaaacagaggcttggacgcccatattaacttgtcactgcatctccgaagtgaggaggcccctttggaagagacagaggcggcggcgacccacgagtcccgttccggaggctacgggtctgagccggcgagagaaagagcgagcagccaaggaaggaaaggagacagcagcgaaggaaggagagaagaagggcgcaagggtcccaagacgtctccaccgagaggcagctgccaccctgctcgcgagcaccgcagtgtcacccgcgacgcagcagaggtgcggcaagagcccccgaaaggtctctcttggggtgacagtcaccgctgcccagaaggcccccggactgagagcaccttagcgcctgcgggtctgcacatgctccgtgagctagatagaggcaaggctgtggccgtggggcgcgggcgccgggacgcgcggctggcgggccgggcagggctgcgctcgggagcggccgccgcgcttcccgggaaggctgcgctggctgcggggctcagcgcaggggag

SEQ ID NO: 17891 - RNA, 11007 nt, Homo sapiens
  source 1..11007: mol_type = other RNA
tcggcctggggaggaggaaggggagggaggatggaaacataccgtacacaaaatactcaattcctagttttctctttaaaaatggctagaaaaaattcatcaaaatgcagcactttaatcaattatttacaatttctatgttacaatgaaaaaatgtacatcttatagaacatatttcataaaactgctccactggaaacaactagatcaaaacagcaaaccttccatttaatatccacaaagttggattatttttcctttttgaagtagattcgccacaatcaaatttgaatacagagaattttgaagtttaagcatcaaacaacaaagtaaaagtccccaagatacaacaaagatctaggcaagtcttgttcctgtcccactcccaccccacccctaatgaaacttaaaaggtattcccatttcaattatggcctgtatcattcttggcagtttgggaagagaacttttggcttccattggtaactcaacataaatgttgcatagaatttatatatttcaaaattggcctaactgtagaaaaggcaaaatggaagcatttccgatagagccctaaatgagtacaaagtcactttgtaaaaggtgagtgacactaaagtaaaaatatgaccaaaataagaaatgtgcatattagacaaccctgcttcccgaaactttaggaaggacacggagttgtgagtcacacaagggctatgctacttgaagtcaatgttcaccaatcaggcagcactaggtacagaagtcttggttctgaacctggacccaggagggaagtctgtgggaaaggggagaagagaatgacaagagaggatgtcatattaaaaaaaggtttcaaacaatattggcaggtgtctactcacaaggtgattggaaaactgcccacgaggagaagtcaactttacctcctcccaaattcacagtacgcgagtgtagtagggtcattgctgggagataaattgtctgaggagggccacccttcaggtttaccagaaatcttagggtttggcccccctggtcacaggctaaatatatggtttaaaagttttattaaaaagaaaaacagaacaagacacactcacacccagatgactaatgaaggctaagcagaatagtctgagtttgctgagactaaagcagggatagtgttgaaaagttttcctttcactagtgggacacattccccttttcttttcaaagaggaagaacatggtgtcatccaatgtgaagtgagcagtttcgggtcaaactcttatggtaagaaactaaaaaaagatgccaagagacaaaccttcagaaatagaagaaatgcaaaagatggaataaaaaccctgatcattaaaacagagacaccttcactggtgtccaataaggattctctttacaaaacagaaacaaacaactcaaaaatttaccatactttgtaatgaaaataccagtatgttgaagacacagcagactgggtttctattagaacaagtatcagcaaggtcatgtagacttgtagaaacttttgccttctcctgcaccagacagatcattgtccagttgggttgtcagctggagaccgaaaagaacctaaaaaatggatctttttttttttctttttcccatggtcacgcatccacacaaatgagtcttttggatgagaaaagtcacagcaacttgagttctcctaatgaacagatgactttttagccctgtttgtttcaatggggaaaacaatgacaaaaaaaacaaaccccaggcaggcacgacacttatgtaaaatgaacacagttagtacaaaaccagtaaggcatcactttgggaaggtcagcaccgaagaggtcaggcaaggctcgtccagacggggcttctgggagggagtgaccctcacccttattgagctgcgtcatgttggttctgaggaaagtgcaagtcttttgcagggtgaccgcatcaccccaccggaagctggggcggggacgctggaggtgttggtgtgtgttctaaaccctcaaggacgagaagggaaggcaaggtccatggctcacccacatgtcgaggaccaggtcctcatccattttaaaggacacagatacccccagccctagcaggaggaggcgagtgtgtaggactgtgaggatggacaactaaaaaccaaaactgagcaggaccaaaccaaaactcaactcctgcggttcttactttcaccaaaggattgattctgaccaagaggggaagggggaaaaaaaaatcttcaaaaatcaatgcatcagaaaggaagaaactcaacctcattttcaaaaggtaacctgttctccaaagtagaacaagtctcactatacacagtgtttgcagaaaaaaaaaaaaaaaaacctgattcattcatatatcagaaggaaagagacacatgctgttctgcactgacagccacatccactcgctcacactctcactccgtcactcactctcacggatattaatcagaggctgatggacctgaatggggtggtttgattggaacaggcaaaatacctctcgggtaaggaaagcaccatttaaaaaacatgaaagcacggtttatttgctcctaaggtttccctgtgtcgtagctctgtagtgcgttgaacgtgaccaaagcaagcaccctggttagcaccagttctccctgtggccggctgtgtgggagggtgggtggcacggctctgagacccagtctggagggtctgtgctgaggggaagccgtgcttctctgtgtttccgactttgctccagtctcttctgtctctgggaagctcatggcaggatgctgtttggtttcagagcttcatgtgggttctctttttttttttctctctgtctctcttttcatttcaacggcgatgatcctttcccgagaagtatcttcagtgtcttagggaggtcacagcaacaaggcaaaacaataattaaagtacaacagaaggtagtgcagttctcgctgtggaaggaagcggtccgcaggcagctggcccgggatgcctgcacccaggtcgaggctgaaggacggggggtctcggtgttcccgcagctctaaggctgtggctgggggctggctcaggaagtcatcttcagggtgatgtgggggatgcaggtggaatgcggtgaggagaagaggagggcgctgggctccgggcccctgtcacagagtggactccaaagaggagtccaagatgtcatcgtgatggctgttgctgttggagtcgctgtcatagctctgggggctggagtagttggctgcctcctgcagcctcatcagcatgttcatcagcgggtcaccttcagcatcactggggggcatctgcttgcttgtcgatccctcccgaggcatggagtagccgtcgaagccgacatcctcaggccgtaactgcagcaggggaggccactcgtgctgttgtgggctggctgcccatggatatgtgtccatcacccacttggcaggatcctcccagggggcgcgccttccatagagctggagtccttctctgacggcttccaggagataggggataatggaatagttccacaagtcggtgaaccacactctcgagccgtccacatcgatggggcatgacaggaagagccgggggccgatggtgacgtccgaggaactgtgagcctccaggaagcggttgaggtgatgccagaccttgggaatccagtcaatgatttttaccagctccatattgcgcacccgcccactgatctctgtttccatgagcttcctcctcaggaatcggccaaggaaacccttcacaggctccgtgtggttggcacaaagcacccatctgaagttatggtgaagctgcaggttgggagtcgaagaggtagcctggttcattgtgccaattatgtaagggcatttgtggtacttgcagttgagcagcccattgaagatctctcccagagagctcacgtggtgtaggttgtccaggatgatgacgaggggcatgtccacagcattgttctcactgttgcactggtcagcaaggttggacaggtactggcgcaattccttgctggacttatggtccacgttaaaggtggcgataaccccgtctgtcaactcccgtccctctcgaagcactatatactcagacagccggttggccaggtaggttttcccagtgccgctggggccagagagaatgatccgacggtgctctatcaggagggagacgtagcgctgcaggatgggcttgggaatcaaggactcaaacaccagtgagtccaggctgttttctgcgagccctttcacagtcactgagatggtcgtgttctctccaaccagatagccacaaggaagcagctccggtgtttcggaagtgttgctgcgcttgatttctccaatgctgtagccaagaacgctgtctgaattcagccctagctgactcactgggtcgacatgaatgatgtattctttgaacagccgtctaaccaccccatcgagcacatcccacttcgtcttgccactaactccaatgcagccaataagaaagagatgtggtctggaatcctccttccacttcatttcctcctgaaagctgacaactatcttaacatgcctgcctccttccttccgagccgagcattcaccagtgtcatccagcaacatgtccaggctggttgactcagtgaggttcaagctgtgctgggagaggcccatggactgcctcggggaggcagagatggacacttgggaaggagcccggctgcagccactgccttgagactctgacttcagccgatcattctcagctttcagcttctctatttcactctgcatcctgttcatggcctcccggagctggtccagctggtgggcagaactgagagcttctaagcggatatccgtcagcttcatctccttgtctcttaactcatttcggagctgcatgacggtctcagcttcactatccatgcattctgaaattagagagttggagtgagaattcctcagcagtggggtggaacctgtggacccattgtgcggtaactttggtgaggaaggcaaagaagaatccgtcatctcctcaatatctgaatgagaggacgcagattttggggacttcttcttcccgaaagcttgcttgaaggagctgcgtaactcattgacccagttcttccgcttcttcttctttgagtcactctctatgttgctgcccacgctggagtggctggtggcactgttgatgctggagacgctgtctgaggagtgctgcctgcggatgcggaggtctgcagactgggcagtgccgtttcctttgcagttgagctcaggtgtgttaattactccattaatggcagcctgggcagctgcgttctgtttctttagcagctcaatggtttttcttaactcattcagttctgagtccttctgctcagctgtcatggtcagactctggagcctgattgtcatgttaccaagactctgttcaaaggctgccacaaggtgagcatttgctgtcagctgggtggtcaaagctgaaactttctcctgggaggcatccagttcccgccgcagcttgcgaatctctgactggcatttttcttctggtgtagaataaactgacgatgtgctggaaaccaaggagagtgaggatccatgaactaactcataccttgcgtgatggaacaaaggaagagagaaatgaagtgagctgtgaagacggctgacaaagttgtccacagaacttttctcccatgattcttcttcaaacccatcccggaatgagcctgaacggctcatggttctgctcttctcatccagggacatggagctattccggaagcggctgtcagtgtatggatcatactgcccatcagcattggagaggctgtgagtcctcagcatggtcgggttggacaagctcatctgggtgacagtggtgggactcgcaagctgggaaaagttgaatcttgttccggagggagaagtcacgctggagccagaggaaaagggggaattggcagcggtgtcctgaaggcctcctgcagaatgggaccgtaaccattcttttgcatcttcttgcgtgcgaagctgggaggtgggagtatacctgagtcctttcttaggcaaagtgttcctatcaaggtgcgggtcactgtcctgtttcctgggcagagtacttctgcagaacttagggctagcagcaggggaagagagagggctttctgacagtgtggtcttcacactgttagttctgacaaagggagtcaaggagtcgtccttggaggaggcgatgaggccagtggaagaattgtggctggggacccctccactgctgagggagatgtcgatggactcacagctggtgtggaggctgctgacagactgaaagcccaggccatccttgctaactgcggaggagctgctggcgttggtgccccaggtgaggctgttggaaggggccgagtgggctgagctggggctggaggctagcggagactggttgaggtccacattcttgctgtagagaggactgctgctcccactgctcaggacgccactgcctgacggggagtctaggttaccttgctgagtcatggtggcatgaggattggagatgaccaccgaatttttcatgttttcagctgtggcgatgggcacttgcttggtaggcttcccaccaaagagtctgcggagtgtgggagaggccacatctgggtacttggctccaggctggagactggtctgagccggactggacacaggctgggctgccggattcactttcaccgagttacaggaagccacactctcgttgtctgatgagatgcctttctccttgtctgtttggttgaccagacctggtagagagctgcctagggctgttttggaaggctccctcagtttgggcactggcaggcctgcggacttgctgctaatgttggaatctatgctgctggtgctagacctgttcccagccccgttccggctgttggacttactgggcctcggcaaactccggtactgaaggtttgtccgggagcttagggctagatacccgtcatcctgattctgagccccatccatacttgacttccgaccagcagaccgactgacgagtgcagatgactttgggattttgcccagtgtggctgacctgctggtgacagtcaccccgctggctgtgatcatggccaggccggcggcggaaccactctgcttcttgaacccaaagctgttggcattggcagtaggtgtcctagagctgctggggaggggctttttggattcgtcaccactgctccggcctgcatctgatggggagcgcttcacctgggaggctttaggagaaagccttcctttctcagacacctttgcgtcgtctgtttttccagttcctggggtcttcagtgcgcctgccggggctgaaggcttcgtccttggcatggtgatgcccacctgagctgtcatgcctcgccgccatgagcctgtctgggagatgacaggattcttcttgcccgacgtgcttttgtcggactcgtcagacacatcagaaggattccgcctccacttggaacctggctccatttttatgccgctgtctgagcctccgtctgatttcttgacatcatcaccagaccacagggaattcctctccacctgtgagtgcttctcagcatcagtctgcacatccaggttttttcgagaggaggcaggtgtgttggcataagagctgatggaggagctggtgttgatgtcatcagtgctgaggttgtctatggtgtcgctgatgccgctgctgacggagctgctgtcgtcccagctgtcagcgtctccgaggcccagggaggtatttcgttgcagggtctcccgtaccacagccatcccatcagggagccggttcaggcgacgggtatagaggccaagtccaccatcagtcatgtatccgcttgtaatgtcatcggtccggatgttcttgctcagaacatccccgtcgctcatgtagccgggggcatccatgctgatgccttccaggtccatctcatctcctgccttgtctgagacgtccacatggcagacactactgccccgggaggccagctgccttctcagaggggcggagtacacatagcgacctgactcagtgttgatgaacctgctggcgttggctcgagggggatacccattgcccattgagggggcgtctcctgcttggagccgagggctggactggcccagtctccaggacagaggtgtgggcctccctgtcaagctgagtatgctacggccactcatctccgtggtgacattggtgtcaaacgtggtttccaatgtgctgtgtgtaacctgagttccccttaaactggacatggtttcctccaaattctgccgcagatcagcgatgttcttcactgtccgcagccgccgagcctcaggatcttccccagtgagttcttccagagcaggctgtccagtcttggtgaagtggctgggctccacgctcacacctgttgagcttgactcggcagtaacattcccttcagtgtccgtctgagacctgtacaggaaaggtgcaaccgtggcagtgttgggatggttgtattgctgctggggctgaggtagctgaacactgacggtattgcttcctgtggtctgggtggtcccgacagacccactgacagtctggctgctgatgctgtggttcagggtggtccctcctgggccttttccttctgaggacgccaggctggaagaggaactggagtgtctgccgtccagctggggcttctgctgggggagtcctgagctcagcttcccactccggctccgctccccttccttggaaggcgctggggcacttggggatttcccgggcatgcttttcattcctggttttggtattccactgtgggaaggggccatgggctccttcttggcactgttgagcttcccccctttggggatgaagctggcaatcttggaggacttttttggcatctcgggcacagctgctccactggggtcttcttttggctcctccttgaggtccagcctctccgtcacagaggctctcttggcaaggtccttgcttttctccttatccttctcccgctgttgtttctccttctctttctcattgcctttcagagaactcttcttgttggtcagtgcccggctaaaagtcctctgggcaatgcccttgagtgcaatcttggggctgctggaagcagggcccacggtggtgagcatgcgactggcggcctccagctcctcgctctcttcgaagctgggcagagtctccagccgctcacagcttgtgtcccgggaccccggcccctcacctgcctttgagccccctttactgttgaaaagtttcagcttttccagcatggacttctgattgttgggggccggcttcatggcttcaggtgtgggcctgggggcctcaggcccaggaggcttgaccgagagcatggataccgtggcactgtgcttcacgctgagggatttgctgcgccaaggcttggtggctgcaccgggctgcgggatggccgaggaggtactgcaattagtaggggtggagctgctgccgctctccaaggaagcaggtgcattgtcactcattccggggtgggaggaggctgaacttgccaaaggctctttctcgtggctgcttggcggtgggggtggggaggtgactggtttggatttatcatagttgttaaagctctggctgcgtcggttgttagcagtagttgaccctccgcgtgttttggcctcgctgcctgcagcggataccctcgcggtaggacctggaagtctagagatctttttctgacccagagtgaagcggatgattttgctttgagatgagtccttggatgatgcactggactgcatttcagcttgtgcttttgactgctgatgtggcgctggctggtgaggctggcacggggcttggggagtgactggcacctgctgctgaggggtgccagcctggcactgggagggggccccggccacctgggatacggcgggcggcagaggtgaggagaggtgctgcttctggggctgctgctgctgctgcttgtatcgggagaggctgaagaagaggcctagaatggccttgaggtttccattcctgatctcttctgcagacagcccctggatgtttattcccttagctgccaggaaattcaagcaggcatctatgttttcaatcatttgggatctgttcttcggacagccattgatgtcttcaatcttttcatttgccacaacctggataatctgggccaggaggacgccatctgtcacatcttgctggagatccctgatgagacgcttgtggccggatttggctaggtaatgattggcccagtctgtgtagatctggacggatgctgccgccgggtctcacacctctcctgggtggcctttcaagagctctgggcgctcaggggctgccgcctcttgcaaatttcctcctgggaaacagaggcttggacgcccatattaacttgtcactgcatctccgaagtgaggaggcccctttggaagagacagaggcggcggcgacccacgagtcccgttccggaggctacgggtctgagccggcgagagaaagagcgagcagccaaggaaggaaaggagacagcagcgaaggaaggagagaagaagggcgcaagggtcccaagacgtctccaccgagaggcagctgccaccctgctcgcgagcaccgcagtgtcacccgcgacgcagcagaggtgcggcaagagcccccgaaaggtctctcttggggtgacagtcaccgctgcccagaaggcccccggactgagagcaccttagcgcctgcgggtctgcacatgctccgtgagctagatagaggcaaggctgtggccgtggggcgcgggcgccgggacgcgcggctggcgggccgggcagggctgcgctcgggagcggccgccgcgcttcccgggaaggctgcgctggctgcggggctcagcgcaggggag

SEQ ID NO: 17892 - RNA, 11510 nt, Homo sapiens
  source 1..11510: mol_type = other RNA
tcggcctggggaggaggaaggggagggaggatggaaacataccgtacacaaaatactcaattcctagttttctctttaaaaatggctagaaaaaattcatcaaaatgcagcactttaatcaattatttacaatttctatgttacaatgaaaaaatgtacatcttatagaacatatttcataaaactgctccactggaaacaactagatcaaaacagcaaaccttccatttaatatccacaaagttggattatttttcctttttgaagtagattcgccacaatcaaatttgaatacagagaattttgaagtttaagcatcaaacaacaaagtaaaagtccccaagatacaacaaagatctaggcaagtcttgttcctgtcccactcccaccccacccctaatgaaacttaaaaggtattcccatttcaattatggcctgtatcattcttggcagtttgggaagagaacttttggcttccattggtaactcaacataaatgttgcatagaatttatatatttcaaaattggcctaactgtagaaaaggcaaaatggaagcatttccgatagagccctaaatgagtacaaagtcactttgtaaaaggtgagtgacactaaagtaaaaatatgaccaaaataagaaatgtgcatattagacaaccctgcttcccgaaactttaggaaggacacggagttgtgagtcacacaagggctatgctacttgaagtcaatgttcaccaatcaggcagcactaggtacagaagtcttggttctgaacctggacccaggagggaagtctgtgggaaaggggagaagagaatgacaagagaggatgtcatattaaaaaaaggtttcaaacaatattggcaggtgtctactcacaaggtgattggaaaactgcccacgaggagaagtcaactttacctcctcccaaattcacagtacgcgagtgtagtagggtcattgctgggagataaattgtctgaggagggccacccttcaggtttaccagaaatcttagggtttggcccccctggtcacaggctaaatatatggtttaaaagttttattaaaaagaaaaacagaacaagacacactcacacccagatgactaatgaaggctaagcagaatagtctgagtttgctgagactaaagcagggatagtgttgaaaagttttcctttcactagtgggacacattccccttttcttttcaaagaggaagaacatggtgtcatccaatgtgaagtgagcagtttcgggtcaaactcttatggtaagaaactaaaaaaagatgccaagagacaaaccttcagaaatagaagaaatgcaaaagatggaataaaaaccctgatcattaaaacagagacaccttcactggtgtccaataaggattctctttacaaaacagaaacaaacaactcaaaaatttaccatactttgtaatgaaaataccagtatgttgaagacacagcagactgggtttctattagaacaagtatcagcaaggtcatgtagacttgtagaaacttttgccttctcctgcaccagacagatcattgtccagttgggttgtcagctggagaccgaaaagaacctaaaaaatggatctttttttttttctttttcccatggtcacgcatccacacaaatgagtcttttggatgagaaaagtcacagcaacttgagttctcctaatgaacagatgactttttagccctgtttgtttcaatggggaaaacaatgacaaaaaaaacaaaccccaggcaggcacgacacttatgtaaaatgaacacagttagtacaaaaccagtaaggcatcactttgggaaggtcagcaccgaagaggtcaggcaaggctcgtccagacggggcttctgggagggagtgaccctcacccttattgagctgcgtcatgttggttctgaggaaagtgcaagtcttttgcagggtgaccgcatcaccccaccggaagctggggcggggacgctggaggtgttggtgtgtgttctaaaccctcaaggacgagaagggaaggcaaggtccatggctcacccacatgtcgaggaccaggtcctcatccattttaaaggacacagatacccccagccctagcaggaggaggcgagtgtgtaggactgtgaggatggacaactaaaaaccaaaactgagcaggaccaaaccaaaactcaactcctgcggttcttactttcaccaaaggattgattctgaccaagaggggaagggggaaaaaaaaatcttcaaaaatcaatgcatcagaaaggaagaaactcaacctcattttcaaaaggtaacctgttctccaaagtagaacaagtctcactatacacagtgtttgcagaaaaaaaaaaaaaaaaacctgattcattcatatatcagaaggaaagagacacatgctgttctgcactgacagccacatccactcgctcacactctcactccgtcactcactctcacggatattaatcagaggctgatggacctgaatggggtggtttgattggaacaggcaaaatacctctcgggtaaggaaagcaccatttaaaaaacatgaaagcacggtttatttgctcctaaggtttccctgtgtcgtagctctgtagtgcgttgaacgtgaccaaagcaagcaccctggttagcaccagttctccctgtggccggctgtgtgggagggtgggtggcacggctctgagacccagtctggagggtctgtgctgaggggaagccgtgcttctctgtgtttccgactttgctccagtctcttctgtctctgggaagctcatggcaggatgctgtttggtttcagagcttcatgtgggttctctttttttttttctctctgtctctcttttcatttcaacggcgatgatcctttcccgagaagtatcttcagtgtcttagggaggtcacagcaacaaggcaaaacaataattaaagtacaacagaaggtagtgcagttctcgctgtggaaggaagcggtccgcaggcagctggcccgggatgcctgcacccaggtcgaggctgaaggacggggggtctcggtgttcccgcagctctaaggctgtggctgggggctggctcaggaagtcatcttcagggtgatgtgggggatgcaggtggaatgcggtgaggagaagaggagggcgctgggctccgggcccctgtcacagagtggactccaaagaggagtccaagatgtcatcgtgatggctgttgctgttggagtcgctgtcatagctctgggggctggagtagttggctgcctcctgcagcctcatcagcatgttcatcagcgggtcaccttcagcatcactggggggcatctgcttgcttgtcgatccctcccgaggcatggagtagccgtcgaagccgacatcctcaggccgtaactgcagcaggggaggccactcgtgctgttgtgggctggctgcccatggatatgtgtccatcacccacttggcaggatcctcccagggggcgcgccttccatagagctggagtccttctctgacggcttccaggagataggggataatggaatagttccacaagtcggtgaaccacactctcgagccgtccacatcgatggggcatgacaggaagagccgggggccgatggtgacgtccgaggaactgtgagcctccaggaagcggttgaggtgatgccagaccttgggaatccagtcaatgatttttaccagctccatattgcgcacccgcccactgatctctgtttccatgagcttcctcctcaggaatcggccaaggaaacccttcacaggctccgtgtggttggcacaaagcacccatctgaagttatggtgaagctgcaggttgggagtcgaagaggtagcctggttcattgtgccaattatgtaagggcatttgtggtacttgcagttgagcagcccattgaagatctctcccagagagctcacgtggtgtaggttgtccaggatgatgacgaggggcatgtccacagcattgttctcactgttgcactggtcagcaaggttggacaggtactggcgcaattccttgctggacttatggtccacgttaaaggtggcgataaccccgtctgtcaactcccgtccctctcgaagcactatatactcagacagccggttggccaggtaggttttcccagtgccgctggggccagagagaatgatccgacggtgctctatcaggagggagacgtagcgctgcaggatgggcttgggaatcaaggactcaaacaccagtgagtccaggctgttttctgcgagccctttcacagtcactgagatggtcgtgttctctccaaccagatagccacaaggaagcagctccggtgtttcggaagtgttgctgcgcttgatttctccaatgctgtagccaagaacgctgtctgaattcagccctagctgactcactgggtcgacatgaatgatgtattctttgaacagccgtctaaccaccccatcgagcacatcccacttcgtcttgccactaactccaatgcagccaataagaaagagatgtggtctggaatcctccttccacttcatttcctcctgaaagctgacaactatcttaacatgcctgcctccttccttccgagccgagcattcaccagtgtcatccagcaacatgtccaggctggttgactcagtgaggttcaagctgtgctgggagaggcccatggactgcctcggggaggcagagatggacacttgggaaggagcccggctgcagccactgccttgagactctgacttcagccgatcattctcagctttcagcttctctatttcactctgcatcctgttcatggcctcccggagctggtccagctggtgggcagaactgagagcttctaagcggatatccgtcagcttcatctccttgtctcttaactcatttcggagctgcatgacggtctcagcttcactatccatgcattctgaaattagagagttggagtgagaattcctcagcagtggggtggaacctgtggacccattgtgcggtaactttggtgaggaaggcaaagaagaatccgtcatctcctcaatatctgaatgagaggacgcagattttggggacttcttcttcccgaaagcttgcttgaaggagctgcgtaactcattgacccagttcttccgcttcttcttctttgagtcactctctatgttgctgcccacgctggagtggctggtggcactgttgatgctggagacgctgtctgaggagtgctgcctgcggatgcggaggtctgcagactgggcagtgccgtttcctttgcagttgagctcaggtgtgttaattactccattaatggcagcctgggcagctgcgttctgtttctttagcagctcaatggtttttcttaactcattcagttctgagtccttctgctcagctgtcatggtcagactctggagcctgattgtcatgttaccaagactctgttcaaaggctgccacaaggtgagcatttgctgtcagctgggtggtcaaagctgaaactttctcctgggaggcatccagttcccgccgcagcttgcgaatctctgactggcatttttcttctggtgtagaataaactgacgatgtgctggaaaccaaggagagtgaggatccatgaactaactcataccttgcgtgatggaacaaaggaagagagaaatgaagtgagctgtgaagacggctgacaaagttgtccacagaacttttctcccatgattcttcttcaaacccatcccggaatgagcctgaacggctcatggttctgctcttctcatccagggacatggagctattccggaagcggctgtcagtgtatggatcatactgcccatcagcattggagaggctgtgagtcctcagcatggtcgggttggacaagctcatctgggtgacagtggtgggactcgcaagctgggaaaagttgaatcttgttccggagggagaagtcacgctggagccagaggaaaagggggaattggcagcggtgtcctgaaggcctcctgcagaatgggaccgtaaccattcttttgcatcttcttgcgtgcgaagctgggaggtgggagtatacctgagtcctttcttaggcaaagtgttcctatcaaggtgcgggtcactgtcctgtttcctgggcagagtacttctgcagaacttagggctagcagcaggggaagagagagggctttctgacagtgtggtcttcacactgttagttctgacaaagggagtcaaggagtcgtccttggaggaggcgatgaggccagtggaagaattgtggctggggacccctccactgctgagggagatgtcgatggactcacagctggtgtggaggctgctgacagactgaaagcccaggccatccttgctaactgcggaggagctgctggcgttggtgccccaggtgaggctgttggaaggggccgagtgggctgagctggggctggaggctagcggagactggttgaggtccacattcttgctgtagagaggactgctgctcccactgctcaggacgccactgcctgacggggagtctaggttaccttgctgagtcatggtggcatgaggattggagatgaccaccgaatttttcatgttttcagctgtggcgatgggcacttgcttggtaggcttcccaccaaagagtctgcggagtgtgggagaggccacatctgggtacttggctccaggctggagactggtctgagccggactggacacaggctgggctgccggattcactttcaccgagttacaggaagccacactctcgttgtctgatgagatgcctttctccttgtctgtttggttgaccagacctggtagagagctgcctagggctgttttggaaggctccctcagtttgggcactggcaggcctgcggacttgctgctaatgttggaatctatgctgctggtgctagacctgttcccagccccgttccggctgttggacttactgggcctcggcaaactccggtactgaaggtttgtccgggagcttagggctagatacccgtcatcctgattctgagccccatccatacttgacttccgaccagcagaccgactgacgagtgcagatgactttgggattttgcccagtgtggctgacctgctggtgacagtcaccccgctggctgtgatcatggccaggccggcggcggaaccactctgcttcttgaacccaaagctgttggcattggcagtaggtgtcctagagctgctggggaggggctttttggattcgtcaccactgctccggcctgcatctgatggggagcgcttcacctgggaggctttaggagaaagccttcctttctcagacacctttgcgtcgtctgtttttccagttcctggggtcttcagtgcgcctgccggggctgaaggcttcgtccttggcatggtgatgcccacctgagctgtcatgcctcgccgccatgagcctgtctgggagatgacaggattcttcttgcccgacgtgcttttgtcggactcgtcagacacatcagaaggattccgcctccacttggaacctggctccatttttatgccgctgtctgagcctccgtctgatttcttgacatcatcaccagaccacagggaattcctctccacctgtgagtgcttctcagcatcagtctgcacatccaggttttttcgagaggaggcaggtgtgttggcataagagctgatggaggagctggtgttgatgtcatcagtgctgaggttgtctatggtgtcgctgatgccgctgctgacggagctgctgtcgtcccagctgtcagcgtctccgaggcccagggaggtatttcgttgcagggtctcccgtaccacagccatcccatcagggagccggttcaggcgacgggtatagaggccaagtccaccatcagtcatgtatccgcttgtaatgtcatcggtccggatgttcttgctcagaacatccccgtcgctcatgtagccgggggcatccatgctgatgccttccaggtccatctcatctcctgccttgtctgagacgtccacatggcagacactactgccccgggaggccagctgccttctcagaggggcggagtacacatagcgacctgactcagtgttgatgaacctgctggcgttggctcgagggggatacccattgcccattgagggggcgtctcctgcttggagccgagggctggactggcccagtctccaggacagaggtgtgggcctccctgtcaagctgagtatgctacggccactcatctccgtggtgacattggtgtcaaacgtggtttccaatgtgctgtgtgtaacctgagttccccttaaactggacatggtttcctccaaattctgccgcagatcagcgatgttcttcactgtccgcagccgccgagcctcaggatcttccccagtgagttcttccagagcaggctgtccagtcttggtgaagtggctgggctccacgctcacacctgttgagcttgactcggcagtaacattcccttcagtgtccgtctgagacctgtacaggaaaggtgcaaccgtggcagtgttgggatggttgtattgctgctggggctgaggtagctgaacactgacggtattgcttcctgtggtctgggtggtcccgacagacccactgacagtctggctgctgatgctgtggttcagggtggtccctcctgggccttttccttctgaggacgccaggctggaagaggaactggagtgtctgccgtccagctggggcttctgctgggggagtcctgagctcagcttcccactccggctccgctccccttccttggaaggcgctggggcacttggggatttcccgggcatgcttttcattcctggttttggtattccactgtgggaaggggccatgggctccttcttggcactgttgagcttcccccctttggggatgaagctggcaatcttggaggacttttttggcatctcgggcacagctgctccactggggtcttcttttggctcctccttgaggtccagcctctccgtcacagaggctctcttggcaaggtccttgcttttctccttatccttctcccgctgttgtttctccttctctttctcattgcctttcagagaactcttcttgttggtcagtgcccggctaaaagtcctctgggcaatgcccttgagtgcaatcttggggctgctggaagcagggcccacggtggtgagcatgcgactggcggcctccagctcctcgctctcttcgaagctgggcagagtctccagccgctcacagcttgtgtcccgggaccccggcccctcacctgcctttgagccccctttactgttgaaaagtttcagcttttccagcatggacttctgattgttgggggccggcttcatggcttcaggtgtgggcctgggggcctcaggcccaggaggcttgaccgagagcatggataccgtggcactgtgcttcacgctgagggatttgctgcgccaaggcttggtggctgcaccgggctgcgggatggccgaggaggtactgcaattagtaggggtggagctgctgccgctctccaaggaagcaggtgcattgtcactcattccggggtgggaggaggctgaacttgccaaaggctctttctcgtggctgcttggcggtgggggtggggaggtgactggtttggatttatcatagttgttaaagctctggctgcgtcggttgttagcagtagttgaccctccgcgtgttttggcctcgctgcctgcagcggataccctcgcggtaggacctggaagtctagagatctttttctgacccagagtgaagcggatgattttgctttgagatgagtccttggatgatgcactggactgcatttcagcttgtgcttttgactgctgatgtggcgctggctggtgaggctggcacggggcttggggagtgactggcacctgctgctgaggggtgccagcctggcactgggagggggccccggccacctgggatacggcgggcggcagaggtgaggagaggtgctgcttctggggctgctgctgctgctgcttgtatcgggagaggctgaagaagaggcctagaatggccttgaggtttccattcctgatctcttctgcagacagcccctggatgtttattcccttagctgccaggaaattcaagcaggcatctatgttttcaatcatttgggatctgttcttcggacagccattgatgtcttcaatcttttcatttgccacaacctggataatctgggccaggaggacgccatctgtcacatcttgctggagatccctgatgagacgcttgtggccggatttggctaggtaatgattggcccagtctgtgtagatctgggtatcgaacccgttttccaccgagccgctcttccgcagcgggagcccctcccccgctggctcctgcagcccctgcagcacctgcgatttcagggggatctggctaggataggtggtcttgctcacctccaccttgcttcccaacttcaggtagcagggctgggggcccgcccgggccgggggcacgtgcaggatgggcgcggcgctgtgcacgggtttgggcagtcccgacttcattttggaggcgaccaggatggccggcatcttctcccggggcttgggctttcccagcacgtccctggcagcggcggcgggggcgaccgctaaaggcagcgcgggtagcagagcaggcgccgggccttagcccacgaggcgcccaccaccagcggctaaaaaaaaaatccccaggtcggggaactcgaagcaatcgggcgagcgcgcctttggggtgccgggatgggaatgggggactggccacggcgctcagcgggtcccacctggacggatgctgccgccgggtctcacacctctcctgggtggcctttcaagagctctgggcgctcaggggctgccgcctcttgcaaatttcctcctgggaaacagaggcttggacgcccatattaacttgtcactgcatctccgaagtgaggaggcccctttggaagagacagaggcggcggcgacccacgagtcccgttccggaggctacgggtctgagccggcgagagaaagagcgagcagccaaggaaggaaaggagacagcagcgaaggaaggagagaagaagggcgcaagggtcccaagacgtctccaccgagaggcagctgccaccctgctcgcgagcaccgcagtgtcacccgcgacgcagcagaggtgcggcaagagcccccgaaaggtctctcttggggtgacagtcaccgctgcccagaaggcccccggactgagagcaccttagcgcctgcgggtctgcacatgctccgtgagctagatagaggcaaggctgtggccgtggggcgcgggcgccgggacgcgcggctggcgggccgggcagggctgcgctcgggagcggccgccgcgcttcccgggaaggctgcgctggctgcggggctcagcgcaggggaggac

SEQ ID NO: 17893 - RNA, 11082 nt, Homo sapiens
  source 1..11082: mol_type = other RNA
tcggcctggggaggaggaaggggagggaggatggaaacataccgtacacaaaatactcaattcctagttttctctttaaaaatggctagaaaaaattcatcaaaatgcagcactttaatcaattatttacaatttctatgttacaatgaaaaaatgtacatcttatagaacatatttcataaaactgctccactggaaacaactagatcaaaacagcaaaccttccatttaatatccacaaagttggattatttttcctttttgaagtagattcgccacaatcaaatttgaatacagagaattttgaagtttaagcatcaaacaacaaagtaaaagtccccaagatacaacaaagatctaggcaagtcttgttcctgtcccactcccaccccacccctaatgaaacttaaaaggtattcccatttcaattatggcctgtatcattcttggcagtttgggaagagaacttttggcttccattggtaactcaacataaatgttgcatagaatttatatatttcaaaattggcctaactgtagaaaaggcaaaatggaagcatttccgatagagccctaaatgagtacaaagtcactttgtaaaaggtgagtgacactaaagtaaaaatatgaccaaaataagaaatgtgcatattagacaaccctgcttcccgaaactttaggaaggacacggagttgtgagtcacacaagggctatgctacttgaagtcaatgttcaccaatcaggcagcactaggtacagaagtcttggttctgaacctggacccaggagggaagtctgtgggaaaggggagaagagaatgacaagagaggatgtcatattaaaaaaaggtttcaaacaatattggcaggtgtctactcacaaggtgattggaaaactgcccacgaggagaagtcaactttacctcctcccaaattcacagtacgcgagtgtagtagggtcattgctgggagataaattgtctgaggagggccacccttcaggtttaccagaaatcttagggtttggcccccctggtcacaggctaaatatatggtttaaaagttttattaaaaagaaaaacagaacaagacacactcacacccagatgactaatgaaggctaagcagaatagtctgagtttgctgagactaaagcagggatagtgttgaaaagttttcctttcactagtgggacacattccccttttcttttcaaagaggaagaacatggtgtcatccaatgtgaagtgagcagtttcgggtcaaactcttatggtaagaaactaaaaaaagatgccaagagacaaaccttcagaaatagaagaaatgcaaaagatggaataaaaaccctgatcattaaaacagagacaccttcactggtgtccaataaggattctctttacaaaacagaaacaaacaactcaaaaatttaccatactttgtaatgaaaataccagtatgttgaagacacagcagactgggtttctattagaacaagtatcagcaaggtcatgtagacttgtagaaacttttgccttctcctgcaccagacagatcattgtccagttgggttgtcagctggagaccgaaaagaacctaaaaaatggatctttttttttttctttttcccatggtcacgcatccacacaaatgagtcttttggatgagaaaagtcacagcaacttgagttctcctaatgaacagatgactttttagccctgtttgtttcaatggggaaaacaatgacaaaaaaaacaaaccccaggcaggcacgacacttatgtaaaatgaacacagttagtacaaaaccagtaaggcatcactttgggaaggtcagcaccgaagaggtcaggcaaggctcgtccagacggggcttctgggagggagtgaccctcacccttattgagctgcgtcatgttggttctgaggaaagtgcaagtcttttgcagggtgaccgcatcaccccaccggaagctggggcggggacgctggaggtgttggtgtgtgttctaaaccctcaaggacgagaagggaaggcaaggtccatggctcacccacatgtcgaggaccaggtcctcatccattttaaaggacacagatacccccagccctagcaggaggaggcgagtgtgtaggactgtgaggatggacaactaaaaaccaaaactgagcaggaccaaaccaaaactcaactcctgcggttcttactttcaccaaaggattgattctgaccaagaggggaagggggaaaaaaaaatcttcaaaaatcaatgcatcagaaaggaagaaactcaacctcattttcaaaaggtaacctgttctccaaagtagaacaagtctcactatacacagtgtttgcagaaaaaaaaaaaaaaaaacctgattcattcatatatcagaaggaaagagacacatgctgttctgcactgacagccacatccactcgctcacactctcactccgtcactcactctcacggatattaatcagaggctgatggacctgaatggggtggtttgattggaacaggcaaaatacctctcgggtaaggaaagcaccatttaaaaaacatgaaagcacggtttatttgctcctaaggtttccctgtgtcgtagctctgtagtgcgttgaacgtgaccaaagcaagcaccctggttagcaccagttctccctgtggccggctgtgtgggagggtgggtggcacggctctgagacccagtctggagggtctgtgctgaggggaagccgtgcttctctgtgtttccgactttgctccagtctcttctgtctctgggaagctcatggcaggatgctgtttggtttcagagcttcatgtgggttctctttttttttttctctctgtctctcttttcatttcaacggcgatgatcctttcccgagaagtatcttcagtgtcttagggaggtcacagcaacaaggcaaaacaataattaaagtacaacagaaggtagtgcagttctcgctgtggaaggaagcggtccgcaggcagctggcccgggatgcctgcacccaggtcgaggctgaaggacggggggtctcggtgttcccgcagctctaaggctgtggctgggggctggctcaggaagtcatcttcagggtgatgtgggggatgcaggtggaatgcggtgaggagaagaggagggcgctgggctccgggcccctgtcacagagtggactccaaagaggagtccaagatgtcatcgtgatggctgttgctgttggagtcgctgtcatagctctgggggctggagtagttggctgcctcctgcagcctcatcagcatgttcatcagcgggtcaccttcagcatcactggggggcatctgcttgcttgtcgatccctcccgaggcatggagtagccgtcgaagccgacatcctcaggccgtaactgcagcaggggaggccactcgtgctgttgtgggctggctgcccatggatatgtgtccatcacccacttggcaggatcctcccagggggcgcgccttccatagagctggagtccttctctgacggcttccaggagataggggataatggaatagttccacaagtcggtgaaccacactctcgagccgtccacatcgatggggcatgacaggaagagccgggggccgatggtgacgtccgaggaactgtgagcctccaggaagcggttgaggtgatgccagaccttgggaatccagtcaatgatttttaccagctccatattgcgcacccgcccactgatctctgtttccatgagcttcctcctcaggaatcggccaaggaaacccttcacaggctccgtgtggttggcacaaagcacccatctgaagttatggtgaagctgcaggttgggagtcgaagaggtagcctggttcattgtgccaattatgtaagggcatttgtggtacttgcagttgagcagcccattgaagatctctcccagagagctcacgtggtgtaggttgtccaggatgatgacgaggggcatgtccacagcattgttctcactgttgcactggtcagcaaggttggacaggtactggcgcaattccttgctggacttatggtccacgttaaaggtggcgataaccccgtctgtcaactcccgtccctctcgaagcactatatactcagacagccggttggccaggtaggttttcccagtgccgctggggccagagagaatgatccgacggtgctctatcaggagggagacgtagcgctgcaggatgggcttgggaatcaaggactcaaacaccagtgagtccaggctgttttctgcgagccctttcacagtcactgagatggtcgtgttctctccaaccagatagccacaaggaagcagctccggtgtttcggaagtgttgctgcgcttgatttctccaatgctgtagccaagaacgctgtctgaattcagccctagctgactcactgggtcgacatgaatgatgtattctttgaacagccgtctaaccaccccatcgagcacatcccacttcgtcttgccactaactccaatgcagccaataagaaagagatgtggtctggaatcctccttccacttcatttcctcctgaaagctgacaactatcttaacatgcctgcctccttccttccgagccgagcattcaccagtgtcatccagcaacatgtccaggctggttgactcagtgaggttcaagctgtgctgggagaggcccatggactgcctcggggaggcagagatggacacttgggaaggagcccggctgcagccactgccttgagactctgacttcagccgatcattctcagctttcagcttctctatttcactctgcatcctgttcatggcctcccggagctggtccagctggtgggcagaactgagagcttctaagcggatatccgtcagcttcatctccttgtctcttaactcatttcggagctgcatgacggtctcagcttcactatccatgcattctgaaattagagagttggagtgagaattcctcagcagtggggtggaacctgtggacccattgtgcggtaactttggtgaggaaggcaaagaagaatccgtcatctcctcaatatctgaatgagaggacgcagattttggggacttcttcttcccgaaagcttgcttgaaggagctgcgtaactcattgacccagttcttccgcttcttcttctttgagtcactctctatgttgctgcccacgctggagtggctggtggcactgttgatgctggagacgctgtctgaggagtgctgcctgcggatgcggaggtctgcagactgggcagtgccgtttcctttgcagttgagctcaggtgtgttaattactccattaatggcagcctgggcagctgcgttctgtttctttagcagctcaatggtttttcttaactcattcagttctgagtccttctgctcagctgtcatggtcagactctggagcctgattgtcatgttaccaagactctgttcaaaggctgccacaaggtgagcatttgctgtcagctgggtggtcaaagctgaaactttctcctgggaggcatccagttcccgccgcagcttgcgaatctctgactggcatttttcttctggtgtagaataaactgacgatgtgctggaaaccaaggagagtgaggatccatgaactaactcataccttgcgtgatggaacaaaggaagagagaaatgaagtgagctgtgaagacggctgacaaagttgtccacagaacttttctcccatgattcttcttcaaacccatcccggaatgagcctgaacggctcatggttctgctcttctcatccagggacatggagctattccggaagcggctgtcagtgtatggatcatactgcccatcagcattggagaggctgtgagtcctcagcatggtcgggttggacaagctcatctgggtgacagtggtgggactcgcaagctgggaaaagttgaatcttgttccggagggagaagtcacgctggagccagaggaaaagggggaattggcagcggtgtcctgaaggcctcctgcagaatgggaccgtaaccattcttttgcatcttcttgcgtgcgaagctgggaggtgggagtatacctgagtcctttcttaggcaaagtgttcctatcaaggtgcgggtcactgtcctgtttcctgggcagagtacttctgcagaacttagggctagcagcaggggaagagagagggctttctgacagtgtggtcttcacactgttagttctgacaaagggagtcaaggagtcgtccttggaggaggcgatgaggccagtggaagaattgtggctggggacccctccactgctgagggagatgtcgatggactcacagctggtgtggaggctgctgacagactgaaagcccaggccatccttgctaactgcggaggagctgctggcgttggtgccccaggtgaggctgttggaaggggccgagtgggctgagctggggctggaggctagcggagactggttgaggtccacattcttgctgtagagaggactgctgctcccactgctcaggacgccactgcctgacggggagtctaggttaccttgctgagtcatggtggcatgaggattggagatgaccaccgaatttttcatgttttcagctgtggcgatgggcacttgcttggtaggcttcccaccaaagagtctgcggagtgtgggagaggccacatctgggtacttggctccaggctggagactggtctgagccggactggacacaggctgggctgccggattcactttcaccgagttacaggaagccacactctcgttgtctgatgagatgcctttctccttgtctgtttggttgaccagacctggtagagagctgcctagggctgttttggaaggctccctcagtttgggcactggcaggcctgcggacttgctgctaatgttggaatctatgctgctggtgctagacctgttcccagccccgttccggctgttggacttactgggcctcggcaaactccggtactgaaggtttgtccgggagcttagggctagatacccgtcatcctgattctgagccccatccatacttgacttccgaccagcagaccgactgacgagtgcagatgactttgggattttgcccagtgtggctgacctgctggtgacagtcaccccgctggctgtgatcatggccaggccggcggcggaaccactctgcttcttgaacccaaagctgttggcattggcagtaggtgtcctagagctgctggggaggggctttttggattcgtcaccactgctccggcctgcatctgatggggagcgcttcacctgggaggctttaggagaaagccttcctttctcagacacctttgcgtcgtctgtttttccagttcctggggtcttcagtgcgcctgccggggctgaaggcttcgtccttggcatggtgatgcccacctgagctgtcatgcctcgccgccatgagcctgtctgggagatgacaggattcttcttgcccgacgtgcttttgtcggactcgtcagacacatcagaaggattccgcctccacttggaacctggctccatttttatgccgctgtctgagcctccgtctgatttcttgacatcatcaccagaccacagggaattcctctccacctgtgagtgcttctcagcatcagtctgcacatccaggttttttcgagaggaggcaggtgtgttggcataagagctgatggaggagctggtgttgatgtcatcagtgctgaggttgtctatggtgtcgctgatgccgctgctgacggagctgctgtcgtcccagctgtcagcgtctccgaggcccagggaggtatttcgttgcagggtctcccgtaccacagccatcccatcagggagccggttcaggcgacgggtatagaggccaagtccaccatcagtcatgtatccgcttgtaatgtcatcggtccggatgttcttgctcagaacatccccgtcgctcatgtagccgggggcatccatgctgatgccttccaggtccatctcatctcctgccttgtctgagacgtccacatggcagacactactgccccgggaggccagctgccttctcagaggggcggagtacacatagcgacctgactcagtgttgatgaacctgctggcgttggctcgagggggatacccattgcccattgagggggcgtctcctgcttggagccgagggctggactggcccagtctccaggacagaggtgtgggcctccctgtcaagctgagtatgctacggccactcatctccgtggtgacattggtgtcaaacgtggtttccaatgtgctgtgtgtaacctgagttccccttaaactggacatggtttcctccaaattctgccgcagatcagcgatgttcttcactgtccgcagccgccgagcctcaggatcttccccagtgagttcttccagagcaggctgtccagtcttggtgaagtggctgggctccacgctcacacctgttgagcttgactcggcagtaacattcccttcagtgtccgtctgagacctgtacaggaaaggtgcaaccgtggcagtgttgggatggttgtattgctgctggggctgaggtagctgaacactgacggtattgcttcctgtggtctgggtggtcccgacagacccactgacagtctggctgctgatgctgtggttcagggtggtccctcctgggccttttccttctgaggacgccaggctggaagaggaactggagtgtctgccgtccagctggggcttctgctgggggagtcctgagctcagcttcccactccggctccgctccccttccttggaaggcgctggggcacttggggatttcccgggcatgcttttcattcctggttttggtattccactgtgggaaggggccatgggctccttcttggcactgttgagcttcccccctttggggatgaagctggcaatcttggaggacttttttggcatctcgggcacagctgctccactggggtcttcttttggctcctccttgaggtccagcctctccgtcacagaggctctcttggcaaggtccttgcttttctccttatccttctcccgctgttgtttctccttctctttctcattgcctttcagagaactcttcttgttggtcagtgcccggctaaaagtcctctgggcaatgcccttgagtgcaatcttggggctgctggaagcagggcccacggtggtgagcatgcgactggcggcctccagctcctcgctctcttcgaagctgggcagagtctccagccgctcacagcttgtgtcccgggaccccggcccctcacctgcctttgagccccctttactgttgaaaagtttcagcttttccagcatggacttctgattgttgggggccggcttcatggcttcaggtgtgggcctgggggcctcaggcccaggaggcttgaccgagagcatggataccgtggcactgtgcttcacgctgagggatttgctgcgccaaggcttggtggctgcaccgggctgcgggatggccgaggaggtactgcaattagtaggggtggagctgctgccgctctccaaggaagcaggtgcattgtcactcattccggggtgggaggaggctgaacttgccaaaggctctttctcgtggctgcttggcggtgggggtggggaggtgactggtttggatttatcatagttgttaaagctctggctgcgtcggttgttagcagtagttgaccctccgcgtgttttggcctcgctgcctgcagcggataccctcgcggtaggacctggaagtctggactgcatttcagcttgtgcttttgactgctgatgtggcgctggctggtgaggctggcacggggcttggggagtgactggcacctgctgctgaggggtgccagcctggcactgggagggggccccggccacctgggatacggcgggcggcagaggtgaggagaggtgctgcttctggggctgctgctgctgctgcttgtatcgggagaggctgaagaagaggcctagaatggccttgaggtttccattcctgatctcttctgcagacagcccctggatgtttattcccttagctgccaggaaattcaagcaggcatctatgttttcaatcatttgggatctgttcttcggacagccattgatgtcttcaatcttttcatttgccacaacctggataatctgggccaggaggacgccatctgtcacatcttgctggagatccctgatgagacgcttgtggccggatttggctaggtaatgattggcccagtctgtgtagatcctcttttgatcttccagtccgtggataactggctttctcttctgctgttggctggactcagaaaccgattccatttcccagaaataaaatcctctctctccttcagcgatgcttccaaatccacagaggaacaaaataacccacacaaaagtgatgcatgcaacagccagacagagttcccgccagccaaggaaatcagcaccacctcttcaaaggtcttcctgtcttcttaaaatccactcgggaacctcactcggcaccactgcctttgcaatgagggtgactgctgccggcatcatgagagctaagtcttggggttttactttaggtctgagactcgcttcatgagagcccagaggacaaatctgggcaaagacaagtccatatcctgaggcacataccacattactgccccagaaaccctttccttcactgtctccttggcacagataatttatatgtcaataacaatgtaaatgggcatttaatccaccaagctgctaacatccacatccctctctggcagcccctgactcccataaatcactgcaaacactgcgcggaaagccgcccctcatggctcctgcaagcgttcatcacagcggtggctcccctcctgggctgtcatcttccttcatggtgtaagacccatacctgcgcccacaccggcttcgcggagccgcctcctccagccggtctcgcactgcactccggcccgcgcttctcagccgcggccgctgccgctgcagccgctccttgccctccc

SEQ ID NO: 17894 - RNA, 11438 nt, Homo sapiens
  source 1..11438: mol_type = other RNA
tcggcctggggaggaggaaggggagggaggatggaaacataccgtacacaaaatactcaattcctagttttctctttaaaaatggctagaaaaaattcatcaaaatgcagcactttaatcaattatttacaatttctatgttacaatgaaaaaatgtacatcttatagaacatatttcataaaactgctccactggaaacaactagatcaaaacagcaaaccttccatttaatatccacaaagttggattatttttcctttttgaagtagattcgccacaatcaaatttgaatacagagaattttgaagtttaagcatcaaacaacaaagtaaaagtccccaagatacaacaaagatctaggcaagtcttgttcctgtcccactcccaccccacccctaatgaaacttaaaaggtattcccatttcaattatggcctgtatcattcttggcagtttgggaagagaacttttggcttccattggtaactcaacataaatgttgcatagaatttatatatttcaaaattggcctaactgtagaaaaggcaaaatggaagcatttccgatagagccctaaatgagtacaaagtcactttgtaaaaggtgagtgacactaaagtaaaaatatgaccaaaataagaaatgtgcatattagacaaccctgcttcccgaaactttaggaaggacacggagttgtgagtcacacaagggctatgctacttgaagtcaatgttcaccaatcaggcagcactaggtacagaagtcttggttctgaacctggacccaggagggaagtctgtgggaaaggggagaagagaatgacaagagaggatgtcatattaaaaaaaggtttcaaacaatattggcaggtgtctactcacaaggtgattggaaaactgcccacgaggagaagtcaactttacctcctcccaaattcacagtacgcgagtgtagtagggtcattgctgggagataaattgtctgaggagggccacccttcaggtttaccagaaatcttagggtttggcccccctggtcacaggctaaatatatggtttaaaagttttattaaaaagaaaaacagaacaagacacactcacacccagatgactaatgaaggctaagcagaatagtctgagtttgctgagactaaagcagggatagtgttgaaaagttttcctttcactagtgggacacattccccttttcttttcaaagaggaagaacatggtgtcatccaatgtgaagtgagcagtttcgggtcaaactcttatggtaagaaactaaaaaaagatgccaagagacaaaccttcagaaatagaagaaatgcaaaagatggaataaaaaccctgatcattaaaacagagacaccttcactggtgtccaataaggattctctttacaaaacagaaacaaacaactcaaaaatttaccatactttgtaatgaaaataccagtatgttgaagacacagcagactgggtttctattagaacaagtatcagcaaggtcatgtagacttgtagaaacttttgccttctcctgcaccagacagatcattgtccagttgggttgtcagctggagaccgaaaagaacctaaaaaatggatctttttttttttctttttcccatggtcacgcatccacacaaatgagtcttttggatgagaaaagtcacagcaacttgagttctcctaatgaacagatgactttttagccctgtttgtttcaatggggaaaacaatgacaaaaaaaacaaaccccaggcaggcacgacacttatgtaaaatgaacacagttagtacaaaaccagtaaggcatcactttgggaaggtcagcaccgaagaggtcaggcaaggctcgtccagacggggcttctgggagggagtgaccctcacccttattgagctgcgtcatgttggttctgaggaaagtgcaagtcttttgcagggtgaccgcatcaccccaccggaagctggggcggggacgctggaggtgttggtgtgtgttctaaaccctcaaggacgagaagggaaggcaaggtccatggctcacccacatgtcgaggaccaggtcctcatccattttaaaggacacagatacccccagccctagcaggaggaggcgagtgtgtaggactgtgaggatggacaactaaaaaccaaaactgagcaggaccaaaccaaaactcaactcctgcggttcttactttcaccaaaggattgattctgaccaagaggggaagggggaaaaaaaaatcttcaaaaatcaatgcatcagaaaggaagaaactcaacctcattttcaaaaggtaacctgttctccaaagtagaacaagtctcactatacacagtgtttgcagaaaaaaaaaaaaaaaaacctgattcattcatatatcagaaggaaagagacacatgctgttctgcactgacagccacatccactcgctcacactctcactccgtcactcactctcacggatattaatcagaggctgatggacctgaatggggtggtttgattggaacaggcaaaatacctctcgggtaaggaaagcaccatttaaaaaacatgaaagcacggtttatttgctcctaaggtttccctgtgtcgtagctctgtagtgcgttgaacgtgaccaaagcaagcaccctggttagcaccagttctccctgtggccggctgtgtgggagggtgggtggcacggctctgagacccagtctggagggtctgtgctgaggggaagccgtgcttctctgtgtttccgactttgctccagtctcttctgtctctgggaagctcatggcaggatgctgtttggtttcagagcttcatgtgggttctctttttttttttctctctgtctctcttttcatttcaacggcgatgatcctttcccgagaagtatcttcagtgtcttagggaggtcacagcaacaaggcaaaacaataattaaagtacaacagaaggtagtgcagttctcgctgtggaaggaagcggtccgcaggcagctggcccgggatgcctgcacccaggtcgaggctgaaggacggggggtctcggtgttcccgcagctctaaggctgtggctgggggctggctcaggaagtcatcttcagggtgatgtgggggatgcaggtggaatgcggtgaggagaagaggagggcgctgggctccgggcccctgtcacagagtggactccaaagaggagtccaagatgtcatcgtgatggctgttgctgttggagtcgctgtcatagctctgggggctggagtagttggctgcctcctgcagcctcatcagcatgttcatcagcgggtcaccttcagcatcactggggggcatctgcttgcttgtcgatccctcccgaggcatggagtagccgtcgaagccgacatcctcaggccgtaactgcagcaggggaggccactcgtgctgttgtgggctggctgcccatggatatgtgtccatcacccacttggcaggatcctcccagggggcgcgccttccatagagctggagtccttctctgacggcttccaggagataggggataatggaatagttccacaagtcggtgaaccacactctcgagccgtccacatcgatggggcatgacaggaagagccgggggccgatggtgacgtccgaggaactgtgagcctccaggaagcggttgaggtgatgccagaccttgggaatccagtcaatgatttttaccagctccatattgcgcacccgcccactgatctctgtttccatgagcttcctcctcaggaatcggccaaggaaacccttcacaggctccgtgtggttggcacaaagcacccatctgaagttatggtgaagctgcaggttgggagtcgaagaggtagcctggttcattgtgccaattatgtaagggcatttgtggtacttgcagttgagcagcccattgaagatctctcccagagagctcacgtggtgtaggttgtccaggatgatgacgaggggcatgtccacagcattgttctcactgttgcactggtcagcaaggttggacaggtactggcgcaattccttgctggacttatggtccacgttaaaggtggcgataaccccgtctgtcaactcccgtccctctcgaagcactatatactcagacagccggttggccaggtaggttttcccagtgccgctggggccagagagaatgatccgacggtgctctatcaggagggagacgtagcgctgcaggatgggcttgggaatcaaggactcaaacaccagtgagtccaggctgttttctgcgagccctttcacagtcactgagatggtcgtgttctctccaaccagatagccacaaggaagcagctccggtgtttcggaagtgttgctgcgcttgatttctccaatgctgtagccaagaacgctgtctgaattcagccctagctgactcactgggtcgacatgaatgatgtattctttgaacagccgtctaaccaccccatcgagcacatcccacttcgtcttgccactaactccaatgcagccaataagaaagagatgtggtctggaatcctccttccacttcatttcctcctgaaagctgacaactatcttaacatgcctgcctccttccttccgagccgagcattcaccagtgtcatccagcaacatgtccaggctggttgactcagtgaggttcaagctgtgctgggagaggcccatggactgcctcggggaggcagagatggacacttgggaaggagcccggctgcagccactgccttgagactctgacttcagccgatcattctcagctttcagcttctctatttcactctgcatcctgttcatggcctcccggagctggtccagctggtgggcagaactgagagcttctaagcggatatccgtcagcttcatctccttgtctcttaactcatttcggagctgcatgacggtctcagcttcactatccatgcattctgaaattagagagttggagtgagaattcctcagcagtggggtggaacctgtggacccattgtgcggtaactttggtgaggaaggcaaagaagaatccgtcatctcctcaatatctgaatgagaggacgcagattttggggacttcttcttcccgaaagcttgcttgaaggagctgcgtaactcattgacccagttcttccgcttcttcttctttgagtcactctctatgttgctgcccacgctggagtggctggtggcactgttgatgctggagacgctgtctgaggagtgctgcctgcggatgcggaggtctgcagactgggcagtgccgtttcctttgcagttgagctcaggtgtgttaattactccattaatggcagcctgggcagctgcgttctgtttctttagcagctcaatggtttttcttaactcattcagttctgagtccttctgctcagctgtcatggtcagactctggagcctgattgtcatgttaccaagactctgttcaaaggctgccacaaggtgagcatttgctgtcagctgggtggtcaaagctgaaactttctcctgggaggcatccagttcccgccgcagcttgcgaatctctgactggcatttttcttctggtgtagaataaactgacgatgtgctggaaaccaaggagagtgaggatccatgaactaactcataccttgcgtgatggaacaaaggaagagagaaatgaagtgagctgtgaagacggctgacaaagttgtccacagaacttttctcccatgattcttcttcaaacccatcccggaatgagcctgaacggctcatggttctgctcttctcatccagggacatggagctattccggaagcggctgtcagtgtatggatcatactgcccatcagcattggagaggctgtgagtcctcagcatggtcgggttggacaagctcatctgggtgacagtggtgggactcgcaagctgggaaaagttgaatcttgttccggagggagaagtcacgctggagccagaggaaaagggggaattggcagcggtgtcctgaaggcctcctgcagaatgggaccgtaaccattcttttgcatcttcttgcgtgcgaagctgggaggtgggagtatacctgagtcctttcttaggcaaagtgttcctatcaaggtgcgggtcactgtcctgtttcctgggcagagtacttctgcagaacttagggctagcagcaggggaagagagagggctttctgacagtgtggtcttcacactgttagttctgacaaagggagtcaaggagtcgtccttggaggaggcgatgaggccagtggaagaattgtggctggggacccctccactgctgagggagatgtcgatggactcacagctggtgtggaggctgctgacagactgaaagcccaggccatccttgctaactgcggaggagctgctggcgttggtgccccaggtgaggctgttggaaggggccgagtgggctgagctggggctggaggctagcggagactggttgaggtccacattcttgctgtagagaggactgctgctcccactgctcaggacgccactgcctgacggggagtctaggttaccttgctgagtcatggtggcatgaggattggagatgaccaccgaatttttcatgttttcagctgtggcgatgggcacttgcttggtaggcttcccaccaaagagtctgcggagtgtgggagaggccacatctgggtacttggctccaggctggagactggtctgagccggactggacacaggctgggctgccggattcactttcaccgagttacaggaagccacactctcgttgtctgatgagatgcctttctccttgtctgtttggttgaccagacctggtagagagctgcctagggctgttttggaaggctccctcagtttgggcactggcaggcctgcggacttgctgctaatgttggaatctatgctgctggtgctagacctgttcccagccccgttccggctgttggacttactgggcctcggcaaactccggtactgaaggtttgtccgggagcttagggctagatacccgtcatcctgattctgagccccatccatacttgacttccgaccagcagaccgactgacgagtgcagatgactttgggattttgcccagtgtggctgacctgctggtgacagtcaccccgctggctgtgatcatggccaggccggcggcggaaccactctgcttcttgaacccaaagctgttggcattggcagtaggtgtcctagagctgctggggaggggctttttggattcgtcaccactgctccggcctgcatctgatggggagcgcttcacctgggaggctttaggagaaagccttcctttctcagacacctttgcgtcgtctgtttttccagttcctggggtcttcagtgcgcctgccggggctgaaggcttcgtccttggcatggtgatgcccacctgagctgtcatgcctcgccgccatgagcctgtctgggagatgacaggattcttcttgcccgacgtgcttttgtcggactcgtcagacacatcagaaggattccgcctccacttggaacctggctccatttttatgccgctgtctgagcctccgtctgatttcttgacatcatcaccagaccacagggaattcctctccacctgtgagtgcttctcagcatcagtctgcacatccaggttttttcgagaggaggcaggtgtgttggcataagagctgatggaggagctggtgttgatgtcatcagtgctgaggttgtctatggtgtcgctgatgccgctgctgacggagctgctgtcgtcccagctgtcagcgtctccgaggcccagggaggtatttcgttgcagggtctcccgtaccacagccatcccatcagggagccggttcaggcgacgggtatagaggccaagtccaccatcagtcatgtatccgcttgtaatgtcatcggtccggatgttcttgctcagaacatccccgtcgctcatgtagccgggggcatccatgctgatgccttccaggtccatctcatctcctgccttgtctgagacgtccacatggcagacactactgccccgggaggccagctgccttctcagaggggcggagtacacatagcgacctgactcagtgttgatgaacctgctggcgttggctcgagggggatacccattgcccattgagggggcgtctcctgcttggagccgagggctggactggcccagtctccaggacagaggtgtgggcctccctgtcaagctgagtatgctacggccactcatctccgtggtgacattggtgtcaaacgtggtttccaatgtgctgtgtgtaacctgagttccccttaaactggacatggtttcctccaaattctgccgcagatcagcgatgttcttcactgtccgcagccgccgagcctcaggatcttccccagtgagttcttccagagcaggctgtccagtcttggtgaagtggctgggctccacgctcacacctgttgagcttgactcggcagtaacattcccttcagtgtccgtctgagacctgtacaggaaaggtgcaaccgtggcagtgttgggatggttgtattgctgctggggctgaggtagctgaacactgacggtattgcttcctgtggtctgggtggtcccgacagacccactgacagtctggctgctgatgctgtggttcagggtggtccctcctgggccttttccttctgaggacgccaggctggaagaggaactggagtgtctgccgtccagctggggcttctgctgggggagtcctgagctcagcttcccactccggctccgctccccttccttggaaggcgctggggcacttggggatttcccgggcatgcttttcattcctggttttggtattccactgtgggaaggggccatgggctccttcttggcactgttgagcttcccccctttggggatgaagctggcaatcttggaggacttttttggcatctcgggcacagctgctccactggggtcttcttttggctcctccttgaggtccagcctctccgtcacagaggctctcttggcaaggtccttgcttttctccttatccttctcccgctgttgtttctccttctctttctcattgcctttcagagaactcttcttgttggtcagtgcccggctaaaagtcctctgggcaatgcccttgagtgcaatcttggggctgctggaagcagggcccacggtggtgagcatgcgactggcggcctccagctcctcgctctcttcgaagctgggcagagtctccagccgctcacagcttgtgtcccgggaccccggcccctcacctgcctttgagccccctttactgttgaaaagtttcagcttttccagcatggacttctgattgttgggggccggcttcatggcttcaggtgtgggcctgggggcctcaggcccaggaggcttgaccgagagcatggataccgtggcactgtgcttcacgctgagggatttgctgcgccaaggcttggtggctgcaccgggctgcgggatggccgaggaggtactgcaattagtaggggtggagctgctgccgctctccaaggaagcaggtgcattgtcactcattccggggtgggaggaggctgaacttgccaaaggctctttctcgtggctgcttggcggtgggggtggggaggtgactggtttggatttatcatagttgttaaagctctggctgcgtcggttgttagcagtagttgaccctccgcgtgttttggcctcgctgcctgcagcggataccctcgcggtaggacctggaagtctggactgcatttcagcttgtgcttttgactgctgatgtggcgctggctggtgaggctggcacggggcttggggagtgactggcacctgctgctgaggggtgccagcctggcactgggagggggccccggccacctgggatacggcgggcggcagaggtgaggagaggtgctgcttctggggctgctgctgctgctgcttgtatcgggagaggctgaagaagaggcctagaatggccttgaggtttccattcctgatctcttctgcagacagcccctggatgtttattcccttagctgccaggaaattcaagcaggcatctatgttttcaatcatttgggatctgttcttcggacagccattgatgtcttcaatcttttcatttgccacaacctggataatctgggccaggaggacgccatctgtcacatcttgctggagatccctgatgagacgcttgtggccggatttggctaggtaatgattggcccagtctgtgtagatctgggtatcgaacccgttttccaccgagccgctcttccgcagcgggagcccctcccccgctggctcctgcagcccctgcagcacctgcgatttcagggggatctggctaggataggtggtcttgctcacctccaccttgcttcccaacttcaggtagcagggctgggggcccgcccgggccgggggcacgtgcaggatgggcgcggcgctgtgcacgggtttgggcagtcccgacttcattttggaggcgaccaggatggccggcatcttctcccggggcttgggctttcccagcacgtccctggcagcggcggcgggggcgaccgctaaaggcagcgcgggtagcagagcaggcgccgggccttagcccacgaggcgcccaccaccagcggctaaaaaaaaaatccccaggtcggggaactcgaagcaatcgggcgagcgcgcctttggggtgccgggatgggaatgggggactggccacggcgctcagcgggtcccacctggacggatgctgccgccgggtctcacacctctcctgggtggcctttcaagagctctgggcgctcaggggctgccgcctcttgcaaatttcctcctgggaaacagaggcttggacgcccatattaacttgtcactgcatctccgaagtgaggaggcccctttggaagagacagaggcggcggcgacccacgagtcccgttccggaggctacgggtctgagccggcgagagaaagagcgagcagccaaggaaggaaaggagacagcagcgaaggaaggagagaagaagggcgcaagggtcccaagacgtctccaccgagaggcagctgccaccctgctcgcgagcaccgcagtgtcacccgcgacgcagcagaggtgcggcaagagcccccgaaaggtctctcttggggtgacagtcaccgctgcccagaaggcccccggactgagagcaccttagcgcctgcgggtctgcacatgctccgtgagctagatagaggcaaggctgtggccgtggggcgcgggcgccgggacgcgcggctggcgggccgggcagggctgcgctcgggagcggccgccgcgcttcccgggaaggctgcgctggctgcggggctcagcgcaggggag

SEQ ID NO: 17895 - RNA, 10712 nt, Homo sapiens
  source 1..10712: mol_type = other RNA
tcggcctggggaggaggaaggggagggaggatggaaacataccgtacacaaaatactcaattcctagttttctctttaaaaatggctagaaaaaattcatcaaaatgcagcactttaatcaattatttacaatttctatgttacaatgaaaaaatgtacatcttatagaacatatttcataaaactgctccactggaaacaactagatcaaaacagcaaaccttccatttaatatccacaaagttggattatttttcctttttgaagtagattcgccacaatcaaatttgaatacagagaattttgaagtttaagcatcaaacaacaaagtaaaagtccccaagatacaacaaagatctaggcaagtcttgttcctgtcccactcccaccccacccctaatgaaacttaaaaggtattcccatttcaattatggcctgtatcattcttggcagtttgggaagagaacttttggcttccattggtaactcaacataaatgttgcatagaatttatatatttcaaaattggcctaactgtagaaaaggcaaaatggaagcatttccgatagagccctaaatgagtacaaagtcactttgtaaaaggtgagtgacactaaagtaaaaatatgaccaaaataagaaatgtgcatattagacaaccctgcttcccgaaactttaggaaggacacggagttgtgagtcacacaagggctatgctacttgaagtcaatgttcaccaatcaggcagcactaggtacagaagtcttggttctgaacctggacccaggagggaagtctgtgggaaaggggagaagagaatgacaagagaggatgtcatattaaaaaaaggtttcaaacaatattggcaggtgtctactcacaaggtgattggaaaactgcccacgaggagaagtcaactttacctcctcccaaattcacagtacgcgagtgtagtagggtcattgctgggagataaattgtctgaggagggccacccttcaggtttaccagaaatcttagggtttggcccccctggtcacaggctaaatatatggtttaaaagttttattaaaaagaaaaacagaacaagacacactcacacccagatgactaatgaaggctaagcagaatagtctgagtttgctgagactaaagcagggatagtgttgaaaagttttcctttcactagtgggacacattccccttttcttttcaaagaggaagaacatggtgtcatccaatgtgaagtgagcagtttcgggtcaaactcttatggtaagaaactaaaaaaagatgccaagagacaaaccttcagaaatagaagaaatgcaaaagatggaataaaaaccctgatcattaaaacagagacaccttcactggtgtccaataaggattctctttacaaaacagaaacaaacaactcaaaaatttaccatactttgtaatgaaaataccagtatgttgaagacacagcagactgggtttctattagaacaagtatcagcaaggtcatgtagacttgtagaaacttttgccttctcctgcaccagacagatcattgtccagttgggttgtcagctggagaccgaaaagaacctaaaaaatggatctttttttttttctttttcccatggtcacgcatccacacaaatgagtcttttggatgagaaaagtcacagcaacttgagttctcctaatgaacagatgactttttagccctgtttgtttcaatggggaaaacaatgacaaaaaaaacaaaccccaggcaggcacgacacttatgtaaaatgaacacagttagtacaaaaccagtaaggcatcactttgggaaggtcagcaccgaagaggtcaggcaaggctcgtccagacggggcttctgggagggagtgaccctcacccttattgagctgcgtcatgttggttctgaggaaagtgcaagtcttttgcagggtgaccgcatcaccccaccggaagctggggcggggacgctggaggtgttggtgtgtgttctaaaccctcaaggacgagaagggaaggcaaggtccatggctcacccacatgtcgaggaccaggtcctcatccattttaaaggacacagatacccccagccctagcaggaggaggcgagtgtgtaggactgtgaggatggacaactaaaaaccaaaactgagcaggaccaaaccaaaactcaactcctgcggttcttactttcaccaaaggattgattctgaccaagaggggaagggggaaaaaaaaatcttcaaaaatcaatgcatcagaaaggaagaaactcaacctcattttcaaaaggtaacctgttctccaaagtagaacaagtctcactatacacagtgtttgcagaaaaaaaaaaaaaaaaacctgattcattcatatatcagaaggaaagagacacatgctgttctgcactgacagccacatccactcgctcacactctcactccgtcactcactctcacggatattaatcagaggctgatggacctgaatggggtggtttgattggaacaggcaaaatacctctcgggtaaggaaagcaccatttaaaaaacatgaaagcacggtttatttgctcctaaggtttccctgtgtcgtagctctgtagtgcgttgaacgtgaccaaagcaagcaccctggttagcaccagttctccctgtggccggctgtgtgggagggtgggtggcacggctctgagacccagtctggagggtctgtgctgaggggaagccgtgcttctctgtgtttccgactttgctccagtctcttctgtctctgggaagctcatggcaggatgctgtttggtttcagagcttcatgtgggttctctttttttttttctctctgtctctcttttcatttcaacggcgatgatcctttcccgagaagtatcttcagtgtcttagggaggtcacagcaacaaggcaaaacaataattaaagtacaacagaaggtagtgcagttctcgctgtggaaggaagcggtccgcaggcagctggcccgggatgcctgcacccaggtcgaggctgaaggacggggggtctcggtgttcccgcagctctaaggctgtggctgggggctggctcaggaagtcatcttcagggtgatgtgggggatgcaggtggaatgcggtgaggagaagaggagggcgctgggctccgggcccctgtcacagagtggactccaaagaggagtccaagatgtcatcgtgatggctgttgctgttggagtcgctgtcatagctctgggggctggagtagttggctgcctcctgcagcctcatcagcatgttcatcagcgggtcaccttcagcatcactggggggcatctgcttgcttgtcgatccctcccgaggcatggagtagccgtcgaagccgacatcctcaggccgtaactgcagcaggggaggccactcgtgctgttgtgggctggctgcccatggatatgtgtccatcacccacttggcaggatcctcccagggggcgcgccttccatagagctggagtccttctctgacggcttccaggagataggggataatggaatagttccacaagtcggtgaaccacactctcgagccgtccacatcgatggggcatgacaggaagagccgggggccgatggtgacgtccgaggaactgtgagcctccaggaagcggttgaggtgatgccagaccttgggaatccagtcaatgatttttaccagctccatattgcgcacccgcccactgatctctgtttccatgagcttcctcctcaggaatcggccaaggaaacccttcacaggctccgtgtggttggcacaaagcacccatctgaagttatggtgaagctgcaggttgggagtcgaagaggtagcctggttcattgtgccaattatgtaagggcatttgtggtacttgcagttgagcagcccattgaagatctctcccagagagctcacgtggtgtaggttgtccaggatgatgacgaggggcatgtccacagcattgttctcactgttgcactggtcagcaaggttggacaggtactggcgcaattccttgctggacttatggtccacgttaaaggtggcgataaccccgtctgtcaactcccgtccctctcgaagcactatatactcagacagccggttggccaggtaggttttcccagtgccgctggggccagagagaatgatccgacggtgctctatcaggagggagacgtagcgctgcaggatgggcttgggaatcaaggactcaaacaccagtgagtccaggctgttttctgcgagccctttcacagtcactgagatggtcgtgttctctccaaccagatagccacaaggaagcagctccggtgtttcggaagtgttgctgcgcttgatttctccaatgctgtagccaagaacgctgtctgaattcagccctagctgactcactgggtcgacatgaatgatgtattctttgaacagccgtctaaccaccccatcgagcacatcccacttcgtcttgccactaactccaatgcagccaataagaaagagatgtggtctggaatcctccttccacttcatttcctcctgaaagctgacaactatcttaacatgcctgcctccttccttccgagccgagcattcaccagtgtcatccagcaacatgtccaggctggttgactcagtgaggttcaagctgtgctgggagaggcccatggactgcctcggggaggcagagatggacacttgggaaggagcccggctgcagccactgccttgagactctgacttcagccgatcattctcagctttcagcttctctatttcactctgcatcctgttcatggcctcccggagctggtccagctggtgggcagaactgagagcttctaagcggatatccgtcagcttcatctccttgtctcttaactcatttcggagctgcatgacggtctcagcttcactatccatgcattctgaaattagagagttggagtgagaattcctcagcagtggggtggaacctgtggacccattgtgcggtaactttggtgaggaaggcaaagaagaatccgtcatctcctcaatatctgaatgagaggacgcagattttggggacttcttcttcccgaaagcttgcttgaaggagctgcgtaactcattgacccagttcttccgcttcttcttctttgagtcactctctatgttgctgcccacgctggagtggctggtggcactgttgatgctggagacgctgtctgaggagtgctgcctgcggatgcggaggtctgcagactgggcagtgccgtttcctttgcagttgagctcaggtgtgttaattactccattaatggcagcctgggcagctgcgttctgtttctttagcagctcaatggtttttcttaactcattcagttctgagtccttctgctcagctgtcatggtcagactctggagcctgattgtcatgttaccaagactctgttcaaaggctgccacaaggtgagcatttgctgtcagctgggtggtcaaagctgaaactttctcctgggaggcatccagttcccgccgcagcttgcgaatctctgactggcatttttcttctggtgtagaataaactgacgatgtgctggaaaccaaggagagtgaggatccatgaactaactcataccttgcgtgatggaacaaaggaagagagaaatgaagtgagctgtgaagacggctgacaaagttgtccacagaacttttctcccatgattcttcttcaaacccatcccggaatgagcctgaacggctcatggttctgctcttctcatccagggacatggagctattccggaagcggctgtcagtgtatggatcatactgcccatcagcattggagaggctgtgagtcctcagcatggtcgggttggacaagctcatctgggtgacagtggtgggactcgcaagctgggaaaagttgaatcttgttccggagggagaagtcacgctggagccagaggaaaagggggaattggcagcggtgtcctgaaggcctcctgcagaatgggaccgtaaccattcttttgcatcttcttgcgtgcgaagctgggaggtgggagtatacctgagtcctttcttaggcaaagtgttcctatcaaggtgcgggtcactgtcctgtttcctgggcagagtacttctgcagaacttagggctagcagcaggggaagagagagggctttctgacagtgtggtcttcacactgttagttctgacaaagggagtcaaggagtcgtccttggaggaggcgatgaggccagtggaagaattgtggctggggacccctccactgctgagggagatgtcgatggactcacagctggtgtggaggctgctgacagactgaaagcccaggccatccttgctaactgcggaggagctgctggcgttggtgccccaggtgaggctgttggaaggggccgagtgggctgagctggggctggaggctagcggagactggttgaggtccacattcttgctgtagagaggactgctgctcccactgctcaggacgccactgcctgacggggagtctaggttaccttgctgagtcatggtggcatgaggattggagatgaccaccgaatttttcatgttttcagctgtggcgatgggcacttgcttggtaggcttcccaccaaagagtctgcggagtgtgggagaggccacatctgggtacttggctccaggctggagactggtctgagccggactggacacaggctgggctgccggattcactttcaccgagttacaggaagccacactctcgttgtctgatgagatgcctttctccttgtctgtttggttgaccagacctggtagagagctgcctagggctgttttggaaggctccctcagtttgggcactggcaggcctgcggacttgctgctaatgttggaatctatgctgctggtgctagacctgttcccagccccgttccggctgttggacttactgggcctcggcaaactccggtactgaaggtttgtccgggagcttagggctagatacccgtcatcctgattctgagccccatccatacttgacttccgaccagcagaccgactgacgagtgcagatgactttgggattttgcccagtgtggctgacctgctggtgacagtcaccccgctggctgtgatcatggccaggccggcggcggaaccactctgcttcttgaacccaaagctgttggcattggcagtaggtgtcctagagctgctggggaggggctttttggattcgtcaccactgctccggcctgcatctgatggggagcgcttcacctgggaggctttaggagaaagccttcctttctcagacacctttgcgtcgtctgtttttccagttcctggggtcttcagtgcgcctgccggggctgaaggcttcgtccttggcatggtgatgcccacctgagctgtcatgcctcgccgccatgagcctgtctgggagatgacaggattcttcttgcccgacgtgcttttgtcggactcgtcagacacatcagaaggattccgcctccacttggaacctggctccatttttatgccgctgtctgagcctccgtctgatttcttgacatcatcaccagaccacagggaattcctctccacctgtgagtgcttctcagcatcagtctgcacatccaggttttttcgagaggaggcaggtgtgttggcataagagctgatggaggagctggtgttgatgtcatcagtgctgaggttgtctatggtgtcgctgatgccgctgctgacggagctgctgtcgtcccagctgtcagcgtctccgaggcccagggaggtatttcgttgcagggtctcccgtaccacagccatcccatcagggagccggttcaggcgacgggtatagaggccaagtccaccatcagtcatgtatccgcttgtaatgtcatcggtccggatgttcttgctcagaacatccccgtcgctcatgtagccgggggcatccatgctgatgccttccaggtccatctcatctcctgccttgtctgagacgtccacatggcagacactactgccccgggaggccagctgccttctcagaggggcggagtacacatagcgacctgactcagtgttgatgaacctgctggcgttggctcgagggggatacccattgcccattgagggggcgtctcctgcttggagccgagggctggactggcccagtctccaggacagaggtgtgggcctccctgtcaagctgagtatgctacggccactcatctccgtggtgacattggtgtcaaacgtggtttccaatgtgctgtgtgtaacctgagttccccttaaactggacatggtttcctccaaattctgccgcagatcagcgatgttcttcactgtccgcagccgccgagcctcaggatcttccccagtgagttcttccagagcaggctgtccagtcttggtgaagtggctgggctccacgctcacacctgttgagcttgactcggcagtaacattcccttcagtgtccgtctgagacctgtacaggaaaggtgcaaccgtggcagtgttgggatggttgtattgctgctggggctgaggtagctgaacactgacggtattgcttcctgtggtctgggtggtcccgacagacccactgacagtctggctgctgatgctgtggttcagggtggtccctcctgggccttttccttctgaggacgccaggctggaagaggaactggagtgtctgccgtccagctggggcttctgctgggggagtcctgagctcagcttcccactccggctccgctccccttccttggaaggcgctggggcacttggggatttcccgggcatgcttttcattcctggttttggtattccactgtgggaaggggccatgggctccttcttggcactgttgagcttcccccctttggggatgaagctggcaatcttggaggacttttttggcatctcgggcacagctgctccactggggtcttcttttggctcctccttgaggtccagcctctccgtcacagaggctctcttggcaaggtccttgcttttctccttatccttctcccgctgttgtttctccttctctttctcattgcctttcagagaactcttcttgttggtcagtgcccggctaaaagtcctctgggcaatgcccttgagtgcaatcttggggctgctggaagcagggcccacggtggtgagcatgcgactggcggcctccagctcctcgctctcttcgaagctgggcagagtctccagccgctcacagcttgtgtcccgggaccccggcccctcacctgcctttgagccccctttactgttgaaaagtttcagcttttccagcatggacttctgattgttgggggccggcttcatggcttcaggtgtgggcctgggggcctcaggcccaggaggcttgaccgagagcatggataccgtggcactgtgcttcacgctgagggatttgctgcgccaaggcttggtggctgcaccgggctgcgggatggccgaggaggtactgcaattagtaggggtggagctgctgccgctctccaaggaagcaggtgcattgtcactcattccggggtgggaggaggctgaacttgccaaaggctctttctcgtggctgcttggcggtgggggtggggaggtgactggtttggatttatcatagttgttaaagctctggctgcgtcggttgttagcagtagttgaccctccgcgtgttttggcctcgctgcctgcagcggataccctcgcggtaggacctggaagtctggactgcatttcagcttgtgcttttgactgctgatgtggcgctggctggtgaggctggcacggggcttggggagtgactggcacctgctgctgaggggtgccagcctggcactgggagggggccccggccacctgggatacggcgggcggcagaggtgaggagaggtgctgcttctggggctgctgctgctgctgcttgtatcgggagaggctgaagaagaggcctagaatggccttgaggtttccattcctgatctcttctgcagacagcccctggatgtttattcccttagctgccaggaaattcaagcaggcatctatgttttcaatcatttgggatctgttcttcggacagccattgatgtcttcaatcttttcatttgccacaacctggataatctgggccaggaggacgccatctgtcacatcttgctggagatccctgatgagacgcttgtggccggatttggctaggtaatgattggcccagtctgtgtagattcggggctcatgtattccccacagacaagccaaaccgcagtagagatcaatagccatgtgcaccccaaagtatcaagacacaatgggggctcgggggacgcggaccacgctgtcccgggacaggctgtgagggcgcagacatgctcgtaggagacaatcccagcgtgtgcaatccaagagagctccaggaattcgtaggtggaagggacggagagataatgcagcccagtcccaccccccttcaatgactcacaaccagagacatacacacatcgactttcctggtttaaacacacacacctcccctgagatctagcttcaaaacaataagggaaataccaagtgcggaatgcatttcaggggctttccaccacccgggccagttcctaaaggggat

SEQ ID NO: 17896 - RNA, 10313 nt, Homo sapiens
  source 1..10313: mol_type = other RNA
tcggcctggggaggaggaaggggagggaggatggaaacataccgtacacaaaatactcaattcctagttttctctttaaaaatggctagaaaaaattcatcaaaatgcagcactttaatcaattatttacaatttctatgttacaatgaaaaaatgtacatcttatagaacatatttcataaaactgctccactggaaacaactagatcaaaacagcaaaccttccatttaatatccacaaagttggattatttttcctttttgaagtagattcgccacaatcaaatttgaatacagagaattttgaagtttaagcatcaaacaacaaagtaaaagtccccaagatacaacaaagatctaggcaagtcttgttcctgtcccactcccaccccacccctaatgaaacttaaaaggtattcccatttcaattatggcctgtatcattcttggcagtttgggaagagaacttttggcttccattggtaactcaacataaatgttgcatagaatttatatatttcaaaattggcctaactgtagaaaaggcaaaatggaagcatttccgatagagccctaaatgagtacaaagtcactttgtaaaaggtgagtgacactaaagtaaaaatatgaccaaaataagaaatgtgcatattagacaaccctgcttcccgaaactttaggaaggacacggagttgtgagtcacacaagggctatgctacttgaagtcaatgttcaccaatcaggcagcactaggtacagaagtcttggttctgaacctggacccaggagggaagtctgtgggaaaggggagaagagaatgacaagagaggatgtcatattaaaaaaaggtttcaaacaatattggcaggtgtctactcacaaggtgattggaaaactgcccacgaggagaagtcaactttacctcctcccaaattcacagtacgcgagtgtagtagggtcattgctgggagataaattgtctgaggagggccacccttcaggtttaccagaaatcttagggtttggcccccctggtcacaggctaaatatatggtttaaaagttttattaaaaagaaaaacagaacaagacacactcacacccagatgactaatgaaggctaagcagaatagtctgagtttgctgagactaaagcagggatagtgttgaaaagttttcctttcactagtgggacacattccccttttcttttcaaagaggaagaacatggtgtcatccaatgtgaagtgagcagtttcgggtcaaactcttatggtaagaaactaaaaaaagatgccaagagacaaaccttcagaaatagaagaaatgcaaaagatggaataaaaaccctgatcattaaaacagagacaccttcactggtgtccaataaggattctctttacaaaacagaaacaaacaactcaaaaatttaccatactttgtaatgaaaataccagtatgttgaagacacagcagactgggtttctattagaacaagtatcagcaaggtcatgtagacttgtagaaacttttgccttctcctgcaccagacagatcattgtccagttgggttgtcagctggagaccgaaaagaacctaaaaaatggatctttttttttttctttttcccatggtcacgcatccacacaaatgagtcttttggatgagaaaagtcacagcaacttgagttctcctaatgaacagatgactttttagccctgtttgtttcaatggggaaaacaatgacaaaaaaaacaaaccccaggcaggcacgacacttatgtaaaatgaacacagttagtacaaaaccagtaaggcatcactttgggaaggtcagcaccgaagaggtcaggcaaggctcgtccagacggggcttctgggagggagtgaccctcacccttattgagctgcgtcatgttggttctgaggaaagtgcaagtcttttgcagggtgaccgcatcaccccaccggaagctggggcggggacgctggaggtgttggtgtgtgttctaaaccctcaaggacgagaagggaaggcaaggtccatggctcacccacatgtcgaggaccaggtcctcatccattttaaaggacacagatacccccagccctagcaggaggaggcgagtgtgtaggactgtgaggatggacaactaaaaaccaaaactgagcaggaccaaaccaaaactcaactcctgcggttcttactttcaccaaaggattgattctgaccaagaggggaagggggaaaaaaaaatcttcaaaaatcaatgcatcagaaaggaagaaactcaacctcattttcaaaaggtaacctgttctccaaagtagaacaagtctcactatacacagtgtttgcagaaaaaaaaaaaaaaaaacctgattcattcatatatcagaaggaaagagacacatgctgttctgcactgacagccacatccactcgctcacactctcactccgtcactcactctcacggatattaatcagaggctgatggacctgaatggggtggtttgattggaacaggcaaaatacctctcgggtaaggaaagcaccatttaaaaaacatgaaagcacggtttatttgctcctaaggtttccctgtgtcgtagctctgtagtgcgttgaacgtgaccaaagcaagcaccctggttagcaccagttctccctgtggccggctgtgtgggagggtgggtggcacggctctgagacccagtctggagggtctgtgctgaggggaagccgtgcttctctgtgtttccgactttgctccagtctcttctgtctctgggaagctcatggcaggatgctgtttggtttcagagcttcatgtgggttctctttttttttttctctctgtctctcttttcatttcaacggcgatgatcctttcccgagaagtatcttcagtgtcttagggaggtcacagcaacaaggcaaaacaataattaaagtacaacagaaggtagtgcagttctcgctgtggaaggaagcggtccgcaggcagctggcccgggatgcctgcacccaggtcgaggctgaaggacggggggtctcggtgttcccgcagctctaaggctgtggctgggggctggctcaggaagtcatcttcagggtgatgtgggggatgcaggtggaatgcggtgaggagaagaggagggcgctgggctccgggcccctgtcacagagtggactccaaagaggagtccaagatgtcatcgtgatggctgttgctgttggagtcgctgtcatagctctgggggctggagtagttggctgcctcctgcagcctcatcagcatgttcatcagcgggtcaccttcagcatcactggggggcatctgcttgcttgtcgatccctcccgaggcatggagtagccgtcgaagccgacatcctcaggccgtaactgcagcaggggaggccactcgtgctgttgtgggctggctgcccatggatatgtgtccatcacccacttggcaggatcctcccagggggcgcgccttccatagagctggagtccttctctgacggcttccaggagataggggataatggaatagttccacaagtcggtgaaccacactctcgagccgtccacatcgatggggcatgacaggaagagccgggggccgatggtgacgtccgaggaactgtgagcctccaggaagcggttgaggtgatgccagaccttgggaatccagtcaatgatttttaccagctccatattgcgcacccgcccactgatctctgtttccatgagcttcctcctcaggaatcggccaaggaaacccttcacaggctccgtgtggttggcacaaagcacccatctgaagttatggtgaagctgcaggttgggagtcgaagaggtagcctggttcattgtgccaattatgtaagggcatttgtggtacttgcagttgagcagcccattgaagatctctcccagagagctcacgtggtgtaggttgtccaggatgatgacgaggggcatgtccacagcattgttctcactgttgcactggtcagcaaggttggacaggtactggcgcaattccttgctggacttatggtccacgttaaaggtggcgataaccccgtctgtcaactcccgtccctctcgaagcactatatactcagacagccggttggccaggtaggttttcccagtgccgctggggccagagagaatgatccgacggtgctctatcaggagggagacgtagcgctgcaggatgggcttgggaatcaaggactcaaacaccagtgagtccaggctgttttctgcgagccctttcacagtcactgagatggtcgtgttctctccaaccagatagccacaaggaagcagctccggtgtttcggaagtgttgctgcgcttgatttctccaatgctgtagccaagaacgctgtctgaattcagccctagctgactcactgggtcgacatgaatgatgtattctttgaacagccgtctaaccaccccatcgagcacatcccacttcgtcttgccactaactccaatgcagccaataagaaagagatgtggtctggaatcctccttccacttcatttcctcctgaaagctgacaactatcttaacatgcctgcctccttccttccgagccgagcattcaccagtgtcatccagcaacatgtccaggctggttgactcagtgaggttcaagctgtgctgggagaggcccatggactgcctcggggaggcagagatggacacttgggaaggagcccggctgcagccactgccttgagactctgacttcagccgatcattctcagctttcagcttctctatttcactctgcatcctgttcatggcctcccggagctggtccagctggtgggcagaactgagagcttctaagcggatatccgtcagcttcatctccttgtctcttaactcatttcggagctgcatgacggtctcagcttcactatccatgcattctgaaattagagagttggagtgagaattcctcagcagtggggtggaacctgtggacccattgtgcggtaactttggtgaggaaggcaaagaagaatccgtcatctcctcaatatctgaatgagaggacgcagattttggggacttcttcttcccgaaagcttgcttgaaggagctgcgtaactcattgacccagttcttccgcttcttcttctttgagtcactctctatgttgctgcccacgctggagtggctggtggcactgttgatgctggagacgctgtctgaggagtgctgcctgcggatgcggaggtctgcagactgggcagtgccgtttcctttgcagttgagctcaggtgtgttaattactccattaatggcagcctgggcagctgcgttctgtttctttagcagctcaatggtttttcttaactcattcagttctgagtccttctgctcagctgtcatggtcagactctggagcctgattgtcatgttaccaagactctgttcaaaggctgccacaaggtgagcatttgctgtcagctgggtggtcaaagctgaaactttctcctgggaggcatccagttcccgccgcagcttgcgaatctctgactggcatttttcttctggtgtagaataaactgacgatgtgctggaaaccaaggagagtgaggatccatgaactaactcataccttgcgtgatggaacaaaggaagagagaaatgaagtgagctgtgaagacggctgacaaagttgtccacagaacttttctcccatgattcttcttcaaacccatcccggaatgagcctgaacggctcatggttctgctcttctcatccagggacatggagctattccggaagcggctgtcagtgtatggatcatactgcccatcagcattggagaggctgtgagtcctcagcatggtcgggttggacaagctcatctgggtgacagtggtgggactcgcaagctgggaaaagttgaatcttgttccggagggagaagtcacgctggagccagaggaaaagggggaattggcagcggtgtcctgaaggcctcctgcagaatgggaccgtaaccattcttttgcatcttcttgcgtgcgaagctgggaggtgggagtatacctgagtcctttcttaggcaaagtgttcctatcaaggtgcgggtcactgtcctgtttcctgggcagagtacttctgcagaacttagggctagcagcaggggaagagagagggctttctgacagtgtggtcttcacactgttagttctgacaaagggagtcaaggagtcgtccttggaggaggcgatgaggccagtggaagaattgtggctggggacccctccactgctgagggagatgtcgatggactcacagctggtgtggaggctgctgacagactgaaagcccaggccatccttgctaactgcggaggagctgctggcgttggtgccccaggtgaggctgttggaaggggccgagtgggctgagctggggctggaggctagcggagactggttgaggtccacattcttgctgtagagaggactgctgctcccactgctcaggacgccactgcctgacggggagtctaggttaccttgctgagtcatggtggcatgaggattggagatgaccaccgaatttttcatgttttcagctgtggcgatgggcacttgcttggtaggcttcccaccaaagagtctgcggagtgtgggagaggccacatctgggtacttggctccaggctggagactggtctgagccggactggacacaggctgggctgccggattcactttcaccgagttacaggaagccacactctcgttgtctgatgagatgcctttctccttgtctgtttggttgaccagacctggtagagagctgcctagggctgttttggaaggctccctcagtttgggcactggcaggcctgcggacttgctgctaatgttggaatctatgctgctggtgctagacctgttcccagccccgttccggctgttggacttactgggcctcggcaaactccggtactgaaggtttgtccgggagcttagggctagatacccgtcatcctgattctgagccccatccatacttgacttccgaccagcagaccgactgacgagtgcagatgactttgggattttgcccagtgtggctgacctgctggtgacagtcaccccgctggctgtgatcatggccaggccggcggcggaaccactctgcttcttgaacccaaagctgttggcattggcagtaggtgtcctagagctgctggggaggggctttttggattcgtcaccactgctccggcctgcatctgatggggagcgcttcacctgggaggctttaggagaaagccttcctttctcagacacctttgcgtcgtctgtttttccagttcctggggtcttcagtgcgcctgccggggctgaaggcttcgtccttggcatggtgatgcccacctgagctgtcatgcctcgccgccatgagcctgtctgggagatgacaggattcttcttgcccgacgtgcttttgtcggactcgtcagacacatcagaaggattccgcctccacttggaacctggctccatttttatgccgctgtctgagcctccgtctgatttcttgacatcatcaccagaccacagggaattcctctccacctgtgagtgcttctcagcatcagtctgcacatccaggttttttcgagaggaggcaggtgtgttggcataagagctgatggaggagctggtgttgatgtcatcagtgctgaggttgtctatggtgtcgctgatgccgctgctgacggagctgctgtcgtcccagctgtcagcgtctccgaggcccagggaggtatttcgttgcagggtctcccgtaccacagccatcccatcagggagccggttcaggcgacgggtatagaggccaagtccaccatcagtcatgtatctttctgcttgatgcaaaattggggcaccctttatgcgatttcctactgtcctccaggactgtcagctcttcaggatgtcaccaagttgatagcgacttgttctttttaggaggatttgggagttcaatgtacatcgtgagtaaaatcttcccttatgtcactcaagcctggaacagtctcctgtggccacaacacacaccaccttggttcagagcataggatgacgtgaccatggcatatagactgcactgctgcaaagtttcttcaatggccacgagccatcccccaggagaacacacagttgaaggggcaccagcccctgcttctctgctgcaaagtgagccagataaccaggaaaacccagataaatcctctggtcaaggtacagcaggaagtcaaggctgctgcagaagtgaactcactcaggagttctggagctgactctggctagtcccagtcaacagagcacacctcactggggagtactgcaaagatgttgctaagctaatcaaacaagggctcagatctagcaggccatggggacagaggcagcagcaggaaaaggtgggcctgagttaaagaggagtcaaaaggtcccaggggccccctgccagcctcgccagggaaaactggtgtcacagacttttgccatttctacttcctaaagccagtgctgaggactgcttgaaagagagagagacagaagagatagcgtgggagtcgctgtctgcagctcaactcaacacacgcctctccatctacctgctgcttgaaatacgggccatggagcagtagtttcaacatcacctggaagctgtcttaaaaagcaatatccgagaccttctaaatcagactcaacatttccataaaccccccaggtgatttgtgtgcacactaaagaaaaagaagcactggacccgggcagtggtctctgtagaggggagcacagatgatccaggagtgaaaacgcaagtgcttctacgtatatttatttctcatcaagatctttctgattcctatgtttttgcacgctatagagtatatgcaatatttcaatagcatggcacatatatattttaaaaacaactacaaccaaatccagtttacagaccattatcgaaatcagaaattcctaaactttcttattaacctctttggagaaacgagtgaaagctagggacctcatctcacatatgtgcaaaattcacatccagcatgagttggctcacagacctcgaggccccaccttagcagtgactttgctaaaacagggcagaagtagatcctggctgagcagatgcttcaacacactctacaatgatttctacattgcaagacttgtctgtttgctataaaccaattccgcagtggctcatggcattgctacaattcacgttaccctgagttttagcacacaggctcaatctcaccactgcttgggtcttgctttcaccaaactcctagcagagagattgatcacgtggagaatttctgtgtggtggtgaaacaggctaccaaggtttgtgtgtcttttgcaaaatgcaatgtgactttccacaagtttaataaaattccatctaatactaatttccagagcattttggttgaaaaagatctatacgtatataaagtccaggagcattttaatttgaaaggcctataatagccctaataaaatacatactccgatgcacaaagagccaaggattataacaatagtgtacttatcacccttaaaccaatagagatatgtaaaattttaattataatccatggctacgcttgtttgaaatggacgcaggcagggcacacttctgaagaaaggctgcacacgttcgaaaattgacagttcctgtgtctgaaactggtcttgcctgaattgtctttactgtggttcaactgtcagtgtggaattgcagcaaatatttctagcattagcaggaagctttttgtccaccttctgaaagatgaaacacatcctaacacacaagagacagttctctagacaaagcccctttaagctctttcttagaatgaaacagatggtgaaaggagatggactgatatccaggaattctcaaacctcagaatacaggcagatcctctggagagcctgaccaaaatgcttattccaaggcctcagcttcatacacgcaagatgtatttagtgaggcccaaatcttgcatatttttaaaaaacagactttactttttaagagattatttctctaacactgtacagaaattacagagttcctttatatcccctcttccccccaacactttgctctattattatgtacacttttttcttagaaacagggtcttgctttgtcacccaaggtagactgtacactgctgtcctaaactcctgg

SEQ ID NO: 17897 - RNA, 12532 nt, Homo sapiens
  source 1..12532: mol_type = other RNA
tcggcctggggaggaggaaggggagggaggatggaaacataccgtacacaaaatactcaattcctagttttctctttaaaaatggctagaaaaaattcatcaaaatgcagcactttaatcaattatttacaatttctatgttacaatgaaaaaatgtacatcttatagaacatatttcataaaactgctccactggaaacaactagatcaaaacagcaaaccttccatttaatatccacaaagttggattatttttcctttttgaagtagattcgccacaatcaaatttgaatacagagaattttgaagtttaagcatcaaacaacaaagtaaaagtccccaagatacaacaaagatctaggcaagtcttgttcctgtcccactcccaccccacccctaatgaaacttaaaaggtattcccatttcaattatggcctgtatcattcttggcagtttgggaagagaacttttggcttccattggtaactcaacataaatgttgcatagaatttatatatttcaaaattggcctaactgtagaaaaggcaaaatggaagcatttccgatagagccctaaatgagtacaaagtcactttgtaaaaggtgagtgacactaaagtaaaaatatgaccaaaataagaaatgtgcatattagacaaccctgcttcccgaaactttaggaaggacacggagttgtgagtcacacaagggctatgctacttgaagtcaatgttcaccaatcaggcagcactaggtacagaagtcttggttctgaacctggacccaggagggaagtctgtgggaaaggggagaagagaatgacaagagaggatgtcatattaaaaaaaggtttcaaacaatattggcaggtgtctactcacaaggtgattggaaaactgcccacgaggagaagtcaactttacctcctcccaaattcacagtacgcgagtgtagtagggtcattgctgggagataaattgtctgaggagggccacccttcaggtttaccagaaatcttagggtttggcccccctggtcacaggctaaatatatggtttaaaagttttattaaaaagaaaaacagaacaagacacactcacacccagatgactaatgaaggctaagcagaatagtctgagtttgctgagactaaagcagggatagtgttgaaaagttttcctttcactagtgggacacattccccttttcttttcaaagaggaagaacatggtgtcatccaatgtgaagtgagcagtttcgggtcaaactcttatggtaagaaactaaaaaaagatgccaagagacaaaccttcagaaatagaagaaatgcaaaagatggaataaaaaccctgatcattaaaacagagacaccttcactggtgtccaataaggattctctttacaaaacagaaacaaacaactcaaaaatttaccatactttgtaatgaaaataccagtatgttgaagacacagcagactgggtttctattagaacaagtatcagcaaggtcatgtagacttgtagaaacttttgccttctcctgcaccagacagatcattgtccagttgggttgtcagctggagaccgaaaagaacctaaaaaatggatctttttttttttctttttcccatggtcacgcatccacacaaatgagtcttttggatgagaaaagtcacagcaacttgagttctcctaatgaacagatgactttttagccctgtttgtttcaatggggaaaacaatgacaaaaaaaacaaaccccaggcaggcacgacacttatgtaaaatgaacacagttagtacaaaaccagtaaggcatcactttgggaaggtcagcaccgaagaggtcaggcaaggctcgtccagacggggcttctgggagggagtgaccctcacccttattgagctgcgtcatgttggttctgaggaaagtgcaagtcttttgcagggtgaccgcatcaccccaccggaagctggggcggggacgctggaggtgttggtgtgtgttctaaaccctcaaggacgagaagggaaggcaaggtccatggctcacccacatgtcgaggaccaggtcctcatccattttaaaggacacagatacccccagccctagcaggaggaggcgagtgtgtaggactgtgaggatggacaactaaaaaccaaaactgagcaggaccaaaccaaaactcaactcctgcggttcttactttcaccaaaggattgattctgaccaagaggggaagggggaaaaaaaaatcttcaaaaatcaatgcatcagaaaggaagaaactcaacctcattttcaaaaggtaacctgttctccaaagtagaacaagtctcactatacacagtgtttgcagaaaaaaaaaaaaaaaaacctgattcattcatatatcagaaggaaagagacacatgctgttctgcactgacagccacatccactcgctcacactctcactccgtcactcactctcacggatattaatcagaggctgatggacctgaatggggtggtttgattggaacaggcaaaatacctctcgggtaaggaaagcaccatttaaaaaacatgaaagcacggtttatttgctcctaaggtttccctgtgtcgtagctctgtagtgcgttgaacgtgaccaaagcaagcaccctggttagcaccagttctccctgtggccggctgtgtgggagggtgggtggcacggctctgagacccagtctggagggtctgtgctgaggggaagccgtgcttctctgtgtttccgactttgctccagtctcttctgtctctgggaagctcatggcaggatgctgtttggtttcagagcttcatgtgggttctctttttttttttctctctgtctctcttttcatttcaacggcgatgatcctttcccgagaagtatcttcagtgtcttagggaggtcacagcaacaaggcaaaacaataattaaagtacaacagaaggtagtgcagttctcgctgtggaaggaagcggtccgcaggcagctggcccgggatgcctgcacccaggtcgaggctgaaggacggggggtctcggtgttcccgcagctctaaggctgtggctgggggctggctcaggaagtcatcttcagggtgatgtgggggatgcaggtggaatgcggtgaggagaagaggagggcgctgggctccgggcccctgtcacagagtggactccaaagaggagtccaagatgtcatcgtgatggctgttgctgttggagtcgctgtcatagctctgggggctggagtagttggctgcctcctgcagcctcatcagcatgttcatcagcgggtcaccttcagcatcactggggggcatctgcttgcttgtcgatccctcccgaggcatggagtagccgtcgaagccgacatcctcaggccgtaactgcagcaggggaggccactcgtgctgttgtgggctggctgcccatggatatgtgtccatcacccacttggcaggatcctcccagggggcgcgccttccatagagctggagtccttctctgacggcttccaggagataggggataatggaatagttccacaagtcggtgaaccacactctcgagccgtccacatcgatggggcatgacaggaagagccgggggccgatggtgacgtccgaggaactgtgagcctccaggaagcggttgaggtgatgccagaccttgggaatccagtcaatgatttttaccagctccatattgcgcacccgcccactgatctctgtttccatgagcttcctcctcaggaatcggccaaggaaacccttcacaggctccgtgtggttggcacaaagcacccatctgaagttatggtgaagctgcaggttgggagtcgaagaggtagcctggttcattgtgccaattatgtaagggcatttgtggtacttgcagttgagcagcccattgaagatctctcccagagagctcacgtggtgtaggttgtccaggatgatgacgaggggcatgtccacagcattgttctcactgttgcactggtcagcaaggttggacaggtactggcgcaattccttgctggacttatggtccacgttaaaggtggcgataaccccgtctgtcaactcccgtccctctcgaagcactatatactcagacagccggttggccaggtaggttttcccagtgccgctggggccagagagaatgatccgacggtgctctatcaggagggagacgtagcgctgcaggatgggcttgggaatcaaggactcaaacaccagtgagtccaggctgttttctgcgagccctttcacagtcactgagatggtcgtgttctctccaaccagatagccacaaggaagcagctccggtgtttcggaagtgttgctgcgcttgatttctccaatgctgtagccaagaacgctgtctgaattcagccctagctgactcactgggtcgacatgaatgatgtattctttgaacagccgtctaaccaccccatcgagcacatcccacttcgtcttgccactaactccaatgcagccaataagaaagagatgtggtctggaatcctccttccacttcatttcctcctgaaagctgacaactatcttaacatgcctgcctccttccttccgagccgagcattcaccagtgtcatccagcaacatgtccaggctggttgactcagtgaggttcaagctgtgctgggagaggcccatggactgcctcggggaggcagagatggacacttgggaaggagcccggctgcagccactgccttgagactctgacttcagccgatcattctcagctttcagcttctctatttcactctgcatcctgttcatggcctcccggagctggtccagctggtgggcagaactgagagcttctaagcggatatccgtcagcttcatctccttgtctcttaactcatttcggagctgcatgacggtctcagcttcactatccatgcattctgaaattagagagttggagtgagaattcctcagcagtggggtggaacctgtggacccattgtgcggtaactttggtgaggaaggcaaagaagaatccgtcatctcctcaatatctgaatgagaggacgcagattttggggacttcttcttcccgaaagcttgcttgaaggagctgcgtaactcattgacccagttcttccgcttcttcttctttgagtcactctctatgttgctgcccacgctggagtggctggtggcactgttgatgctggagacgctgtctgaggagtgctgcctgcggatgcggaggtctgcagactgggcagtgccgtttcctttgcagttgagctcaggtgtgttaattactccattaatggcagcctgggcagctgcgttctgtttctttagcagctcaatggtttttcttaactcattcagttctgagtccttctgctcagctgtcatggtcagactctggagcctgattgtcatgttaccaagactctgttcaaaggctgccacaaggtgagcatttgctgtcagctgggtggtcaaagctgaaactttctcctgggaggcatccagttcccgccgcagcttgcgaatctctgactggcatttttcttctggtgtagaataaactgacgatgtgctggaaaccaaggagagtgaggatccatgaactaactcataccttgcgtgatggaacaaaggaagagagaaatgaagtgagctgtgaagacggctgacaaagttgtccacagaacttttctcccatgattcttcttcaaacccatcccggaatgagcctgaacggctcatggttctgctcttctcatccagggacatggagctattccggaagcggctgtcagtgtatggatcatactgcccatcagcattggagaggctgtgagtcctcagcatggtcgggttggacaagctcatctgggtgacagtggtgggactcgcaagctgggaaaagttgaatcttgttccggagggagaagtcacgctggagccagaggaaaagggggaattggcagcggtgtcctgaaggcctcctgcagaatgggaccgtaaccattcttttgcatcttcttgcgtgcgaagctgggaggtgggagtatacctgagtcctttcttaggcaaagtgttcctatcaaggtgcgggtcactgtcctgtttcctgggcagagtacttctgcagaacttagggctagcagcaggggaagagagagggctttctgacagtgtggtcttcacactgttagttctgacaaagggagtcaaggagtcgtccttggaggaggcgatgaggccagtggaagaattgtggctggggacccctccactgctgagggagatgtcgatggactcacagctggtgtggaggctgctgacagactgaaagcccaggccatccttgctaactgcggaggagctgctggcgttggtgccccaggtgaggctgttggaaggggccgagtgggctgagctggggctggaggctagcggagactggttgaggtccacattcttgctgtagagaggactgctgctcccactgctcaggacgccactgcctgacggggagtctaggttaccttgctgagtcatggtggcatgaggattggagatgaccaccgaatttttcatgttttcagctgtggcgatgggcacttgcttggtaggcttcccaccaaagagtctgcggagtgtgggagaggccacatctgggtacttggctccaggctggagactggtctgagccggactggacacaggctgggctgccggattcactttcaccgagttacaggaagccacactctcgttgtctgatgagatgcctttctccttgtctgtttggttgaccagacctggtagagagctgcctagggctgttttggaaggctccctcagtttgggcactggcaggcctgcggacttgctgctaatgttggaatctatgctgctggtgctagacctgttcccagccccgttccggctgttggacttactgggcctcggcaaactccggtactgaaggtttgtccgggagcttagggctagatacccgtcatcctgattctgagccccatccatacttgacttccgaccagcagaccgactgacgagtgcagatgactttgggattttgcccagtgtggctgacctgctggtgacagtcaccccgctggctgtgatcatggccaggccggcggcggaaccactctgcttcttgaacccaaagctgttggcattggcagtaggtgtcctagagctgctggggaggggctttttggattcgtcaccactgctccggcctgcatctgatggggagcgcttcacctgggaggctttaggagaaagccttcctttctcagacacctttgcgtcgtctgtttttccagttcctggggtcttcagtgcgcctgccggggctgaaggcttcgtccttggcatggtgatgcccacctgagctgtcatgcctcgccgccatgagcctgtctgggagatgacaggattcttcttgcccgacgtgcttttgtcggactcgtcagacacatcagaaggattccgcctccacttggaacctggctccatttttatgccgctgtctgagcctccgtctgatttcttgacatcatcaccagaccacagggaattcctctccacctgtgagtgcttctcagcatcagtctgcacatccaggttttttcgagaggaggcaggtgtgttggcataagagctgatggaggagctggtgttgatgtcatcagtgctgaggttgtctatggtgtcgctgatgccgctgctgacggagctgctgtcgtcccagcttgtaaggttcctaggccagagcatttcactacattgcggcccttggagaacagcggacaaagaagctgaatgaatctcacaggatggcaagtcctttagccagctgagccagcccacactgggccagggaatcccaggcacccagcaactctgtaactaaaggactagctagcagggatcaccattccccaggccaggaaagaaatccgatcccccaacaaaattaacctctgaagtgctgaaggatcgagaggtcaggcctcagtgctggtatcaagtcagctgtgaaaagtttcagcaaagcaaaagctaacaccaaactctgaaaccattaccgtaaagcactgaatggaagggccctccatgtggtcccaggggagtttgcaacagcgggtcaaattgaagaaaatctaagaatgaaaaactactttaaatcctcacagactgcacagaaacattgcagaaagtctttccagccctaagtgctacttttaatgatgcaaaaatcattgactataacatttcttagctcattccattgacgtctgaaggcaaagcattcgattgaaaagattagcctacagagagaatttctgaacctaaaaaggaaatgatacctgtttgtacagttaacaacgacacacatacattatttccggtgatgtcaattttgatgcagtgccaacaaaaatatgcattaattccgcaggctacttatttcaaaagaaaaagaatctcagtctaggcatggctacattaaacattatggtacagaggctggaaggggaggtgggtgggagagagtcccagctctgggatgggaaggggttgcatggactaatccctattaaaacctgtaatcaaggcactcagaaagaactatgtaaacagatgctatgaacaatgaacaactgtattactactgagaactcaaaagcaaacttatgttatagccacaagctttatttgaaaacgaaggattaagatgttctccaaaaccctgactccctctccaaaaatcctaccagttggttcctggtagctttcaaagactttccccaagaaaggctctccccctggccagggtggcctctccagtggaagcagggagcgggggttgtggccctgggggatggttagggaaggaagcagtaactggctccaagcgaggtctctgtgtggtcagcatttgctcagcaaacagaagctttcaaaggggaatgaagagccattcctctcccactgaaaagggagggaataaaagatctgctcaaagaggagaggagggtctggtggtgattcccaggtgaatgaaaaaaagattgtaatctcgaaggagtcccaaccaaagttaatcattcacatctcatccttcagggccctcgtccacttgaaatactgctgaggcatctgccgtggggagtgggaagcagaggtgggggtgggcagtgggtgagtttgagggaaggagtagtgtccagatatattaagacaaaaaagttgggacagacccaagttctggctgacaaggatgcttcaaaccaccccttaccttctatgctgtccctggaactgactgtatctttacgatattacttctttgagaatctgtccaacatccgagttaacttgggaatgggatggtgattgtgtgtatggagacacacaggcacatgggcacagatgcacacacacgctctaaaaagtttccattgtttcctcgctctaggcaaacataataggtaaacattctgatttgtcatcaaggtaagctaggaaatgttgatgtattcatttattcattcatcaactaccatatttataaagcatctgcaatgtggcaagtgctgttctaagtgcagaagatacaagcagtcaacaaaatagaccaaaaatctcaactctaatggaacttagcttcagtggtagaactataaaataaatgagacaaaatgtaaattttacagtacattagcaataaatgctcgggagaacaacgtattgtaaagaagaagatgtgatttgtcaaggtggggtgtgggaaattttacatgggctggctatggcaggtctgctgagggcatggtttttattacaaatctaaaagaagtatgggagctgggtatctgaatacctggggataagggactttcaagagaggaaatggtcagtgcaaaggccctgagatagtatacgacttgcaatgcattccaagaatgagtggctggagcagtgagcggtgaaccaaagtggggtgaggagggggtcaggccagagagtccaagggtacagcgagagaggagagtgcctaaatggggccctgcaagtcagcgtaagcagcttgtcttttactctgagggagagaggatacattggaggtttaatagatggagtttcttctttttataaaagttcatgtaaatgtacaacactaaacatatcgttttgattacacatgatttttacaggggtgagtttattgtaggagacatagtgctttaaggaggtcttagttttctttctatggttaaaagaatcacacctttcatgttagaggctctgaattatttgcagctacaggttctaattgagtcagggttttctcatggtttgaaagataataattagtagggataagggagacccaggcaacgagagaggaaaagggaaagtaaaccaactccatgagggcagatgccctttggcgcttttcaagagccaggattgctctgtcatttttgacgcttgcttctaaacaggccaaattccaaagggctcccagaactcataacacttttctccacagaaacaatgttatcagtgatgttaaggtttccaggttactcacagagccatctataaaaccaagatgtagttgatgaactctactcaggtatcaaagagtagaagaaaactttattcttggaatacagtacataattagacaaaacagaaaaccacaaatctaaaaagatgttcacttatttctaatgagtattttatgaaaacaatgctagtgaagacacttcgttccttttcttccaacatattcaaccctctttcctggcttttccctgcaggctgaaaaatatatcactaatctcatcaaatcaaacaaaaacttttttttttttttacctcatgcccatattctcctccactcctttgaggtgttttcctgtacttctcatgttccgtgatccttcaacccaccaggcaagatgtttgttcccactactccactgagaccactttctcttttccctgagaacatcaatggcttcctccttgccaaagccaatggtcaactctctgtccttaccctacttgagttttcagcagcaggtagcatcgacagattctcccttcttgagtgggcctcatcccgggtttccatactgtcatctgtacctggttcctacctccctaactgcgcttctcaatctcctaggctcaccctcctcttcacctctccagaactccagggcctccatccctggacccctcctcttctctaactataacttctcactaacttctaactaagttataactaccacttctaactaacttcttttcctgggtgatctcatccatggcttcaaatactaggtgaaggcagacaactctaaagtctgtaatctctagcctggcccctttgtgtacccaacacatctgaaatcaaatttaccttactcaaaactattgctcccaacttccaatgtgtccgcacccccactcccaaagtcttctgtatctcagaatatgactctacattaacagtcctaattctctccctccttcttgcctccgatgtaatccattaagaaggccttttgcctagagtccccaaatataccttgaacccaatcactactgaacatctgcaataagataaccttggaccaagatgccatcatctctttcctgcaacagacacctcccgggtcgctcagccttccctcatgccttgctaggctccatcctgcacaccccaggggcagcaatctttctccagtgtacagcagattctgtcacattcctgcttaaagcccactgatagcttcccagggaacttagaataaaattcaaatttgttcccttggcctagaagccctgatgtgatctggcttctcctcttcattacgtccaaagacaggacccacaaatgcaccaagcttcttcccacttcctaggccctcgcactgtgcctcctttctggaatgctcctccccatgtctcccactggcggcccacttctcacgggtcagatgttggttggaatggcacctcctcagggatttcctcttagactctggcccaattacattccaccatatgattttcttcatggcatcaaccagtcaacacattgtctttcaacagtctgtctttccctcaacacagggagctcctcgagcacaggtgtactgtttgcctttgttctgagccatatcctcccagtgcctaaatcactgctgatgtggtcctggatcaaccaagcataggaggacaaaatggaactgattattccatgcagtctcctggggactgtgtagtacttccaaggactttagttcaatggttttatttggtcacagacccacttaggggcccgtctctccataagaaaaaagatacacaaacaatattttacacagaatttccagggactcactgatcccctgaatcctgtccataaagcccaggttaagc

SEQ ID NO: 17898 - RNA, 7962 nt, Homo sapiens
  source 1..7962: mol_type = other RNA
tcggcctggggaggaggaaggggagggaggatggaaacataccgtacacaaaatactcaattcctagttttctctttaaaaatggctagaaaaaattcatcaaaatgcagcactttaatcaattatttacaatttctatgttacaatgaaaaaatgtacatcttatagaacatatttcataaaactgctccactggaaacaactagatcaaaacagcaaaccttccatttaatatccacaaagttggattatttttcctttttgaagtagattcgccacaatcaaatttgaatacagagaattttgaagtttaagcatcaaacaacaaagtaaaagtccccaagatacaacaaagatctaggcaagtcttgttcctgtcccactcccaccccacccctaatgaaacttaaaaggtattcccatttcaattatggcctgtatcattcttggcagtttgggaagagaacttttggcttccattggtaactcaacataaatgttgcatagaatttatatatttcaaaattggcctaactgtagaaaaggcaaaatggaagcatttccgatagagccctaaatgagtacaaagtcactttgtaaaaggtgagtgacactaaagtaaaaatatgaccaaaataagaaatgtgcatattagacaaccctgcttcccgaaactttaggaaggacacggagttgtgagtcacacaagggctatgctacttgaagtcaatgttcaccaatcaggcagcactaggtacagaagtcttggttctgaacctggacccaggagggaagtctgtgggaaaggggagaagagaatgacaagagaggatgtcatattaaaaaaaggtttcaaacaatattggcaggtgtctactcacaaggtgattggaaaactgcccacgaggagaagtcaactttacctcctcccaaattcacagtacgcgagtgtagtagggtcattgctgggagataaattgtctgaggagggccacccttcaggtttaccagaaatcttagggtttggcccccctggtcacaggctaaatatatggtttaaaagttttattaaaaagaaaaacagaacaagacacactcacacccagatgactaatgaaggctaagcagaatagtctgagtttgctgagactaaagcagggatagtgttgaaaagttttcctttcactagtgggacacattccccttttcttttcaaagaggaagaacatggtgtcatccaatgtgaagtgagcagtttcgggtcaaactcttatggtaagaaactaaaaaaagatgccaagagacaaaccttcagaaatagaagaaatgcaaaagatggaataaaaaccctgatcattaaaacagagacaccttcactggtgtccaataaggattctctttacaaaacagaaacaaacaactcaaaaatttaccatactttgtaatgaaaataccagtatgttgaagacacagcagactgggtttctattagaacaagtatcagcaaggtcatgtagacttgtagaaacttttgccttctcctgcaccagacagatcattgtccagttgggttgtcagctggagaccgaaaagaacctaaaaaatggatctttttttttttctttttcccatggtcacgcatccacacaaatgagtcttttggatgagaaaagtcacagcaacttgagttctcctaatgaacagatgactttttagccctgtttgtttcaatggggaaaacaatgacaaaaaaaacaaaccccaggcaggcacgacacttatgtaaaatgaacacagttagtacaaaaccagtaaggcatcactttgggaaggtcagcaccgaagaggtcaggcaaggctcgtccagacggggcttctgggagggagtgaccctcacccttattgagctgcgtcatgttggttctgaggaaagtgcaagtcttttgcagggtgaccgcatcaccccaccggaagctggggcggggacgctggaggtgttggtgtgtgttctaaaccctcaaggacgagaagggaaggcaaggtccatggctcacccacatgtcgaggaccaggtcctcatccattttaaaggacacagatacccccagccctagcaggaggaggcgagtgtgtaggactgtgaggatggacaactaaaaaccaaaactgagcaggaccaaaccaaaactcaactcctgcggttcttactttcaccaaaggattgattctgaccaagaggggaagggggaaaaaaaaatcttcaaaaatcaatgcatcagaaaggaagaaactcaacctcattttcaaaaggtaacctgttctccaaagtagaacaagtctcactatacacagtgtttgcagaaaaaaaaaaaaaaaaacctgattcattcatatatcagaaggaaagagacacatgctgttctgcactgacagccacatccactcgctcacactctcactccgtcactcactctcacggatattaatcagaggctgatggacctgaatggggtggtttgattggaacaggcaaaatacctctcgggtaaggaaagcaccatttaaaaaacatgaaagcacggtttatttgctcctaaggtttccctgtgtcgtagctctgtagtgcgttgaacgtgaccaaagcaagcaccctggttagcaccagttctccctgtggccggctgtgtgggagggtgggtggcacggctctgagacccagtctggagggtctgtgctgaggggaagccgtgcttctctgtgtttccgactttgctccagtctcttctgtctctgggaagctcatggcaggatgctgtttggtttcagagcttcatgtgggttctctttttttttttctctctgtctctcttttcatttcaacggcgatgatcctttcccgagaagtatcttcagtgtcttagggaggtcacagcaacaaggcaaaacaataattaaagtacaacagaaggtagtgcagttctcgctgtggaaggaagcggtccgcaggcagctggcccgggatgcctgcacccaggtcgaggctgaaggacggggggtctcggtgttcccgcagctctaaggctgtggctgggggctggctcaggaagtcatcttcagggtgatgtgggggatgcaggtggaatgcggtgaggagaagaggagggcgctgggctccgggcccctgtcacagagtggactccaaagaggagtccaagatgtcatcgtgatggctgttgctgttggagtcgctgtcatagctctgggggctggagtagttggctgcctcctgcagcctcatcagcatgttcatcagcgggtcaccttcagcatcactggggggcatctgcttgcttgtcgatccctcccgaggcatggagtagccgtcgaagccgacatcctcaggccgtaactgcagcaggggaggccactcgtgctgttgtgggctggctgcccatggatatgtgtccatcacccacttggcaggatcctcccagggggcgcgccttccatagagctggagtccttctctgacggcttccaggagataggggataatggaatagttccacaagtcggtgaaccacactctcgagccgtccacatcgatggggcatgacaggaagagccgggggccgatggtgacgtccgaggaactgtgagcctccaggaagcggttgaggtgatgccagaccttgggaatccagtcaatgatttttaccagctccatattgcgcacccgcccactgatctctgtttccatgagcttcctcctcaggaatcggccaaggaaacccttcacaggctccgtgtggttggcacaaagcacccatctgaagttatggtgaagctgcaggttgggagtcgaagaggtagcctggttcattgtgccaattatgtaagggcatttgtggtacttgcagttgagcagcccattgaagatctctcccagagagctcacgtggtgtaggttgtccaggatgatgacgaggggcatgtccacagcattgttctcactgttgcactggtcagcaaggttggacaggtactggcgcaattccttgctggacttatggtccacgttaaaggtggcgataaccccgtctgtcaactcccgtccctctcgaagcactatatactcagacagccggttggccaggtaggttttcccagtgccgctggggccagagagaatgatccgacggtgctctatcaggagggagacgtagcgctgcaggatgggcttgggaatcaaggactcaaacaccagtgagtccaggctgttttctgcgagccctttcacagtcactgagatggtcgtgttctctccaaccagatagccacaaggaagcagctccggtgtttcggaagtgttgctgcgcttgatttctccaatgctgtagccaagaacgctgtctgaattcagccctagctgactcactgggtcgacatgaatgatgtattctttgaacagccgtctaaccaccccatcgagcacatcccacttcgtcttgccactaactccaatgcagccaataagaaagagatgtggtctggaatcctccttccacttcatttcctcctgaaagctgacaactatcttaacatgcctgcctccttccttccgagccgagcattcaccagtgtcatccagcaacatgtccaggctggttgactcagtgaggttcaagctgtgctgggagaggcccatggactgcctcggggaggcagagatggacacttgggaaggagcccggctgcagccactgccttgagactctgacttcagccgatcattctcagctttcagcttctctatttcactctgcatcctgttcatggcctcccggagctggtccagctggtgggcagaactgagagcttctaagcggatatccgtcagcttcatctccttgtctcttaactcatttcggagctgcatgacggtctcagcttcactatccatgcattctgaaattagagagttggagtgagaattcctcagcagtggggtggaacctgtggacccattgtgcggtaactttggtgaggaaggcaaagaagaatccgtcatctcctcaatatctgaatgagaggacgcagattttggggacttcttcttcccgaaagcttgcttgaaggagctgcgtaactcattgacccagttcttccgcttcttcttctttgagtcactctctatgttgctgcccacgctggagtggctggtggcactgttgatgctggagacgctgtctgaggagtgctgcctgcggatgcggaggtctgcagactgggcagtgccgtttcctttgcagttgagctcaggtgtgttaattactccattaatggcagcctgggcagctgcgttctgtttctttagcagctcaatggtttttcttaactcattcagttctgagtccttctgctcagctgtcatggtcagactctggagcctgattgtcatgttaccaagactctgttcaaaggctgccacaaggtgagcatttgctgtcagctgggtggtcaaagctgaaactttctcctgggaggcatccagttcccgccgcagcttgcgaatctctgactggcatttttcttctggtgtagaataaactgacgatgtgctggaaaccaaggagagtgaggatccatgaactaactcataccttgcgtgatggaacaaaggaagagagaaatgaagtgagctgtgaagacggctgacaaagttgtccacagaacttttctcccatgattcttcttcaaacccatcccggaatgagcctgaacggctcatggttctgctcttctcatccagggacatggagctattccggaagcggctgtcagtgtatggatcatactgcccatcagcattggagaggctgtgagtcctcagcatggtcgggttggacaagctcatctgggtgacagtggtgggactcgcaagctgggaaaagttgaatcttgttccggagggagaagtcacgctggagccagaggaaaagggggaattggcagcggtgtcctgaaggcctcctgcagaatgggaccgtaaccattcttttgcatcttcttgcgtgcgaagctgggaggtgggagtatacctgagtcctttcttaggcaaagtgttcctatcaaggtgcgggtcactgtcctgtttcctgggcagagtacttctgcagaacttagggctagcagcaggggaagagagagggctttctgacagtgtggtcttcacactgttagttctgacaaagggagtcaaggagtcgtccttggaggaggcgatgaggccagtggaagaattgtggctggggacccctccactgctgagggagatgtcgatggactcacagctggtgtggaggctgctgacagactgaaagcccaggccatccttgctaactgcggaggagctgctggcgttggtgccccaggtgaggctgttggaaggggccgagtgggctgagctggggctggaggctagcggagactggttgaggtccacattcttgctgtagagaggactgctgctcccactgctcaggacgccactgcctgacggggagtctaggttaccttgctgagtcatggtggcatgaggattggagatgaccaccgaatttttcatgttttcagctgtggcgatgggcacttgcttggtaggcttcccaccaaagagtctgcggagtgtgggagaggccacatctgggtacttggctccaggctggagactggtctgagccggactggacacaggctgggctgccggattcactttcaccgagttacaggaagccacactctcgttgtctgatgagatgcctttctccttgtctgtttggttgaccagacctggtagagagctgcctagggctgttttggaaggctccctcagtttgggcactggcaggcctgcggacttgctgctaatgttggaatctatgctgctggtgctagacctgttcccagccccgttccggctgttggacttactgggcctcggcaaactccggtactgaaggtttgtccgggagcttagggctagatacccgtcatcctgattctgagccccatccatacttgacttccgaccagcagaccgactgacgagtgcagatgactttgggattttgcccagtgtggctgacctgctggtgacagtcaccccgctggctgtgatcatggccaggccggcggcggaaccactctgcttcttgaacccaaagctgttggcattggcagtaggtgtcctagagctgctggggaggggctttttggattcgtcaccactgctccggcctgcatctgatggggagcgcttcacctgggaggctttaggagaaagccttcctttctcagacacctttgcgtcgtctgtttttccagttcctggggtcttcagtgcgcctgccggggctgaaggcttcgtccttggcatggtgatgcccacctgagctgtcatgcctcgccgccatgagcctgtctgggagatgacaggattcttcttgcccgacgtgcttttgtcggactcgtcagacacatcagaaggattccgcctccacttggaacctggctccatttttatgccgctgtctgagcctccgtctgatttcttgacatcatcaccagaccacagggaattcctctccacctgtgagtgcttctcagcatcagtctgcacatccaggttttttcgagaggaggcaggtgtgttggcataagagctgatggaggagctggtgttgatgtcatcagtgctgaggttgtctatggtgtcgctgatgccgctgctgacggagctgctgtcgtcccagtaataaaaccacagccggtgagcagagatgaggttctctaactacggttctgaaaagcagtcttcacaaagcaaggatcctaatcctccccaaactccaaaggctgggtctgcttccaggaggcccttactgtccttggaaacagtct

SEQ ID NO: 17899 - RNA, 11441 nt, Homo sapiens
  source 1..11441: mol_type = other RNA
tcggcctggggaggaggaaggggagggaggatggaaacataccgtacacaaaatactcaattcctagttttctctttaaaaatggctagaaaaaattcatcaaaatgcagcactttaatcaattatttacaatttctatgttacaatgaaaaaatgtacatcttatagaacatatttcataaaactgctccactggaaacaactagatcaaaacagcaaaccttccatttaatatccacaaagttggattatttttcctttttgaagtagattcgccacaatcaaatttgaatacagagaattttgaagtttaagcatcaaacaacaaagtaaaagtccccaagatacaacaaagatctaggcaagtcttgttcctgtcccactcccaccccacccctaatgaaacttaaaaggtattcccatttcaattatggcctgtatcattcttggcagtttgggaagagaacttttggcttccattggtaactcaacataaatgttgcatagaatttatatatttcaaaattggcctaactgtagaaaaggcaaaatggaagcatttccgatagagccctaaatgagtacaaagtcactttgtaaaaggtgagtgacactaaagtaaaaatatgaccaaaataagaaatgtgcatattagacaaccctgcttcccgaaactttaggaaggacacggagttgtgagtcacacaagggctatgctacttgaagtcaatgttcaccaatcaggcagcactaggtacagaagtcttggttctgaacctggacccaggagggaagtctgtgggaaaggggagaagagaatgacaagagaggatgtcatattaaaaaaaggtttcaaacaatattggcaggtgtctactcacaaggtgattggaaaactgcccacgaggagaagtcaactttacctcctcccaaattcacagtacgcgagtgtagtagggtcattgctgggagataaattgtctgaggagggccacccttcaggtttaccagaaatcttagggtttggcccccctggtcacaggctaaatatatggtttaaaagttttattaaaaagaaaaacagaacaagacacactcacacccagatgactaatgaaggctaagcagaatagtctgagtttgctgagactaaagcagggatagtgttgaaaagttttcctttcactagtgggacacattccccttttcttttcaaagaggaagaacatggtgtcatccaatgtgaagtgagcagtttcgggtcaaactcttatggtaagaaactaaaaaaagatgccaagagacaaaccttcagaaatagaagaaatgcaaaagatggaataaaaaccctgatcattaaaacagagacaccttcactggtgtccaataaggattctctttacaaaacagaaacaaacaactcaaaaatttaccatactttgtaatgaaaataccagtatgttgaagacacagcagactgggtttctattagaacaagtatcagcaaggtcatgtagacttgtagaaacttttgccttctcctgcaccagacagatcattgtccagttgggttgtcagctggagaccgaaaagaacctaaaaaatggatctttttttttttctttttcccatggtcacgcatccacacaaatgagtcttttggatgagaaaagtcacagcaacttgagttctcctaatgaacagatgactttttagccctgtttgtttcaatggggaaaacaatgacaaaaaaaacaaaccccaggcaggcacgacacttatgtaaaatgaacacagttagtacaaaaccagtaaggcatcactttgggaaggtcagcaccgaagaggtcaggcaaggctcgtccagacggggcttctgggagggagtgaccctcacccttattgagctgcgtcatgttggttctgaggaaagtgcaagtcttttgcagggtgaccgcatcaccccaccggaagctggggcggggacgctggaggtgttggtgtgtgttctaaaccctcaaggacgagaagggaaggcaaggtccatggctcacccacatgtcgaggaccaggtcctcatccattttaaaggacacagatacccccagccctagcaggaggaggcgagtgtgtaggactgtgaggatggacaactaaaaaccaaaactgagcaggaccaaaccaaaactcaactcctgcggttcttactttcaccaaaggattgattctgaccaagaggggaagggggaaaaaaaaatcttcaaaaatcaatgcatcagaaaggaagaaactcaacctcattttcaaaaggtaacctgttctccaaagtagaacaagtctcactatacacagtgtttgcagaaaaaaaaaaaaaaaaacctgattcattcatatatcagaaggaaagagacacatgctgttctgcactgacagccacatccactcgctcacactctcactccgtcactcactctcacggatattaatcagaggctgatggacctgaatggggtggtttgattggaacaggcaaaatacctctcgggtaaggaaagcaccatttaaaaaacatgaaagcacggtttatttgctcctaaggtttccctgtgtcgtagctctgtagtgcgttgaacgtgaccaaagcaagcaccctggttagcaccagttctccctgtggccggctgtgtgggagggtgggtggcacggctctgagacccagtctggagggtctgtgctgaggggaagccgtgcttctctgtgtttccgactttgctccagtctcttctgtctctgggaagctcatggcaggatgctgtttggtttcagagcttcatgtgggttctctttttttttttctctctgtctctcttttcatttcaacggcgatgatcctttcccgagaagtatcttcagtgtcttagggaggtcacagcaacaaggcaaaacaataattaaagtacaacagaaggtagtgcagttctcgctgtggaaggaagcggtccgcaggcagctggcccgggatgcctgcacccaggtcgaggctgaaggacggggggtctcggtgttcccgcagctctaaggctgtggctgggggctggctcaggaagtcatcttcagggtgatgtgggggatgcaggtggaatgcggtgaggagaagaggagggcgctgggctccgggcccctgtcacagagtggactccaaagaggagtccaagatgtcatcgtgatggctgttgctgttggagtcgctgtcatagctctgggggctggagtagttggctgcctcctgcagcctcatcagcatgttcatcagcgggtcaccttcagcatcactggggggcatctgcttgcttgtcgatccctcccgaggcatggagtagccgtcgaagccgacatcctcaggccgtaactgcagcaggggaggccactcgtgctgttgtgggctggctgcccatggatatgtgtccatcacccacttggcaggatcctcccagggggcgcgccttccatagagctggagtccttctctgacggcttccaggagataggggataatggaatagttccacaagtcggtgaaccacactctcgagccgtccacatcgatggggcatgacaggaagagccgggggccgatggtgacgtccgaggaactgtgagcctccaggaagcggttgaggtgatgccagaccttgggaatccagtcaatgatttttaccagctccatattgcgcacccgcccactgatctctgtttccatgagcttcctcctcaggaatcggccaaggaaacccttcacaggctccgtgtggttggcacaaagcacccatctgaagttatggtgaagctgcaggttgggagtcgaagaggtagcctggttcattgtgccaattatgtaagggcatttgtggtacttgcagttgagcagcccattgaagatctctcccagagagctcacgtggtgtaggttgtccaggatgatgacgaggggcatgtccacagcattgttctcactgttgcactggtcagcaaggttggacaggtactggcgcaattccttgctggacttatggtccacgttaaaggtggcgataaccccgtctgtcaactcccgtccctctcgaagcactatatactcagacagccggttggccaggtaggttttcccagtgccgctggggccagagagaatgatccgacggtgctctatcaggagggagacgtagcgctgcaggatgggcttgggaatcaaggactcaaacaccagtgagtccaggctgttttctgcgagccctttcacagtcactgagatggtcgtgttctctccaaccagatagccacaaggaagcagctccggtgtttcggaagtgttgctgcgcttgatttctccaatgctgtagccaagaacgctgtctgaattcagccctagctgactcactgggtcgacatgaatgatgtattctttgaacagccgtctaaccaccccatcgagcacatcccacttcgtcttgccactaactccaatgcagccaataagaaagagatgtggtctggaatcctccttccacttcatttcctcctgaaagctgacaactatcttaacatgcctgcctccttccttccgagccgagcattcaccagtgtcatccagcaacatgtccaggctggttgactcagtgaggttcaagctgtgctgggagaggcccatggactgcctcggggaggcagagatggacacttgggaaggagcccggctgcagccactgccttgagactctgacttcagccgatcattctcagctttcagcttctctatttcactctgcatcctgttcatggcctcccggagctggtccagctggtgggcagaactgagagcttctaagcggatatccgtcagcttcatctccttgtctcttaactcatttcggagctgcatgacggtctcagcttcactatccatgcattctgaaattagagagttggagtgagaattcctcagcagtggggtggaacctgtggacccattgtgcggtaactttggtgaggaaggcaaagaagaatccgtcatctcctcaatatctgaatgagaggacgcagattttggggacttcttcttcccgaaagcttgcttgaaggagctgcgtaactcattgacccagttcttccgcttcttcttctttgagtcactctctatgttgctgcccacgctggagtggctggtggcactgttgatgctggagacgctgtctgaggagtgctgcctgcggatgcggaggtctgcagactgggcagtgccgtttcctttgcagttgagctcaggtgtgttaattactccattaatggcagcctgggcagctgcgttctgtttctttagcagctcaatggtttttcttaactcattcagttctgagtccttctgctcagctgtcatggtcagactctggagcctgattgtcatgttaccaagactctgttcaaaggctgccacaaggtgagcatttgctgtcagctgggtggtcaaagctgaaactttctcctgggaggcatccagttcccgccgcagcttgcgaatctctgactggcatttttcttctggtgtagaataaactgacgatgtgctggaaaccaaggagagtgaggatccatgaactaactcataccttgcgtgatggaacaaaggaagagagaaatgaagtgagctgtgaagacggctgacaaagttgtccacagaacttttctcccatgattcttcttcaaacccatcccggaatgagcctgaacggctcatggttctgctcttctcatccagggacatggagctattccggaagcggctgtcagtgtatggatcatactgcccatcagcattggagaggctgtgagtcctcagcatggtcgggttggacaagctcatctgggtgacagtggtgggactcgcaagctgggaaaagttgaatcttgttccggagggagaagtcacgctggagccagaggaaaagggggaattggcagcggtgtcctgaaggcctcctgcagaatgggaccgtaaccattcttttgcatcttcttgcgtgcgaagctgggaggtgggagtatacctgagtcctttcttaggcaaagtgttcctatcaaggtgcgggtcactttctgacagtgtggtcttcacactgttagttctgacaaagggagtcaaggagtcgtccttggaggaggcgatgaggccagtggaagaattgtggctggggacccctccactgctgagggagatgtcgatggactcacagctggtgtggaggctgctgacagactgaaagcccaggccatccttgctaactgcggaggagctgctggcgttggtgccccaggtgaggctgttggaaggggccgagtgggctgagctggggctggaggctagcggagactggttgaggtccacattcttgctgtagagaggactgctgctcccactgctcaggacgccactgcctgacggggagtctaggttaccttgctgagtcatggtggcatgaggattggagatgaccaccgaatttttcatgttttcagctgtggcgatgggcacttgcttggtaggcttcccaccaaagagtctgcggagtgtgggagaggccacatctgggtacttggctccaggctggagactggtctgagccggactggacacaggctgggctgccggattcactttcaccgagttacaggaagccacactctcgttgtctgatgagatgcctttctccttgtctgtttggttgaccagacctggtagagagctgcctagggctgttttggaaggctccctcagtttgggcactggcaggcctgcggacttgctgctaatgttggaatctatgctgctggtgctagacctgttcccagccccgttccggctgttggacttactgggcctcggcaaactccggtactgaaggtttgtccgggagcttagggctagatacccgtcatcctgattctgagccccatccatacttgacttccgaccagcagaccgactgacgagtgcagatgactttgggattttgcccagtgtggctgacctgctggtgacagtcaccccgctggctgtgatcatggccaggccggcggcggaaccactctgcttcttgaacccaaagctgttggcattggcagtaggtgtcctagagctgctggggaggggctttttggattcgtcaccactgctccggcctgcatctgatggggagcgcttcacctgggaggctttaggagaaagccttcctttctcagacacctttgcgtcgtctgtttttccagttcctggggtcttcagtgcgcctgccggggctgaaggcttcgtccttggcatggtgatgcccacctgagctgtcatgcctcgccgccatgagcctgtctgggagatgacaggattcttcttgcccgacgtgcttttgtcggactcgtcagacacatcagaaggattccgcctccacttggaacctggctccatttttatgccgctgtctgagcctccgtctgatttcttgacatcatcaccagaccacagggaattcctctccacctgtgagtgcttctcagcatcagtctgcacatccaggttttttcgagaggaggcaggtgtgttggcataagagctgatggaggagctggtgttgatgtcatcagtgctgaggttgtctatggtgtcgctgatgccgctgctgacggagctgctgtcgtcccagctgtcagcgtctccgaggcccagggaggtatttcgttgcagggtctcccgtaccacagccatcccatcagggagccggttcaggcgacgggtatagaggccaagtccaccatcagtcatgtatccgcttgtaatgtcatcggtccggatgttcttgctcagaacatccccgtcgctcatgtagccgggggcatccatgctgatgccttccaggtccatctcatctcctgccttgtctgagacgtccacatggcagacactactgccccgggaggccagctgccttctcagaggggcggagtacacatagcgacctgactcagtgttgatgaacctgctggcgttggctcgagggggatacccattgcccattgagggggcgtctcctgcttggagccgagggctggactggcccagtctccaggacagaggtgtgggcctccctgtcaagctgagtatgctacggccactcatctccgtggtgacattggtgtcaaacgtggtttccaatgtgctgtgtgtaacctgagttccccttaaactggacatggtttcctccaaattctgccgcagatcagcgatgttcttcactgtccgcagccgccgagcctcaggatcttccccagtgagttcttccagagcaggctgtccagtcttggtgaagtggctgggctccacgctcacacctgttgagcttgactcggcagtaacattcccttcagtgtccgtctgagacctgtacaggaaaggtgcaaccgtggcagtgttgggatggttgtattgctgctggggctgaggtagctgaacactgacggtattgcttcctgtggtctgggtggtcccgacagacccactgacagtctggctgctgatgctgtggttcagggtggtccctcctgggccttttccttctgaggacgccaggctggaagaggaactggagtgtctgccgtccagctggggcttctgctgggggagtcctgagctcagcttcccactccggctccgctccccttccttggaaggcgctggggcacttggggatttcccgggcatgcttttcattcctggttttggtattccactgtgggaaggggccatgggctccttcttggcactgttgagcttcccccctttggggatgaagctggcaatcttggaggacttttttggcatctcgggcacagctgctccactggggtcttcttttggctcctccttgaggtccagcctctccgtcacagaggctctcttggcaaggtccttgcttttctccttatccttctcccgctgttgtttctccttctctttctcattgcctttcagagaactcttcttgttggtcagtgcccggctaaaagtcctctgggcaatgcccttgagtgcaatcttggggctgctggaagcagggcccacggtggtgagcatgcgactggcggcctccagctcctcgctctcttcgaagctgggcagagtctccagccgctcacagcttgtgtcccgggaccccggcccctcacctgcctttgagccccctttactgttgaaaagtttcagcttttccagcatggacttctgattgttgggggccggcttcatggcttcaggtgtgggcctgggggcctcaggcccaggaggcttgaccgagagcatggataccgtggcactgtgcttcacgctgagggatttgctgcgccaaggcttggtggctgcaccgggctgcgggatggccgaggaggtactgcaattagtaggggtggagctgctgccgctctccaaggaagcaggtgcattgtcactcattccggggtgggaggaggctgaacttgccaaaggctctttctcgtggctgcttggcggtgggggtggggaggtgactggtttggatttatcatagttgttaaagctctggctgcgtcggttgttagcagtagttgaccctccgcgtgttttggcctcgctgcctgcagcggataccctcgcggtaggacctggaagtctagagatctttttctgacccagagtgaagcggatgattttgctttgagatgagtccttggatgatgcactggactgcatttcagcttgtgcttttgactgctgatgtggcgctggctggtgaggctggcacggggcttggggagtgactggcacctgctgctgaggggtgccagcctggcactgggagggggccccggccacctgggatacggcgggcggcagaggtgaggagaggtgctgcttctggggctgctgctgctgctgcttgtatcgggagaggctgaagaagaggcctagaatggccttgaggtttccattcctgatctcttctgcagacagcccctggatgtttattcccttagctgccaggaaattcaagcaggcatctatgttttcaatcatttgggatctgttcttcggacagccattgatgtcttcaatcttttcatttgccacaacctggataatctgggccaggaggacgccatctgtcacatcttgctggagatccctgatgagacgcttgtggccggatttggctaggtaatgattggcccagtctgtgtagatctgggtatcgaacccgttttccaccgagccgctcttccgcagcgggagcccctcccccgctggctcctgcagcccctgcagcacctgcgatttcagggggatctggctaggataggtggtcttgctcacctccaccttgcttcccaacttcaggtagcagggctgggggcccgcccgggccgggggcacgtgcaggatgggcgcggcgctgtgcacgggtttgggcagtcccgacttcattttggaggcgaccaggatggccggcatcttctcccggggcttgggctttcccagcacgtccctggcagcggcggcgggggcgaccgctaaaggcagcgcgggtagcagagcaggcgccgggccttagcccacgaggcgcccaccaccagcggctaaaaaaaaaatccccaggtcggggaactcgaagcaatcgggcgagcgcgcctttggggtgccgggatgggaatgggggactggccacggcgctcagcgggtcccacctggacggatgctgccgccgggtctcacacctctcctgggtggcctttcaagagctctgggcgctcaggggctgccgcctcttgcaaatttcctcctgggaaacagaggcttggacgcccatattaacttgtcactgcatctccgaagtgaggaggcccctttggaagagacagaggcggcggcgacccacgagtcccgttccggaggctacgggtctgagccggcgagagaaagagcgagcagccaaggaaggaaaggagacagcagcgaaggaaggagagaagaagggcgcaagggtcccaagacgtctccaccgagaggcagctgccaccctgctcgcgagcaccgcagtgtcacccgcgacgcagcagaggtgcggcaagagcccccgaaaggtctctcttggggtgacagtcaccgctgcccagaaggcccccggactgagagcaccttagcgcctgcgggtctgcacatgctccgtgagctagatagaggcaaggctgtggccgtggggcgcgggcgccgggacgcgcggctggcgggccgggcagggctgcgctcgggagcggccgccgcgcttcccgggaaggctgcgctggctgcggggctcagcgcaggggag

SEQ ID NO: 17900 - RNA, 11396 nt, Homo sapiens
  source 1..11396: mol_type = other RNA
tcggcctggggaggaggaaggggagggaggatggaaacataccgtacacaaaatactcaattcctagttttctctttaaaaatggctagaaaaaattcatcaaaatgcagcactttaatcaattatttacaatttctatgttacaatgaaaaaatgtacatcttatagaacatatttcataaaactgctccactggaaacaactagatcaaaacagcaaaccttccatttaatatccacaaagttggattatttttcctttttgaagtagattcgccacaatcaaatttgaatacagagaattttgaagtttaagcatcaaacaacaaagtaaaagtccccaagatacaacaaagatctaggcaagtcttgttcctgtcccactcccaccccacccctaatgaaacttaaaaggtattcccatttcaattatggcctgtatcattcttggcagtttgggaagagaacttttggcttccattggtaactcaacataaatgttgcatagaatttatatatttcaaaattggcctaactgtagaaaaggcaaaatggaagcatttccgatagagccctaaatgagtacaaagtcactttgtaaaaggtgagtgacactaaagtaaaaatatgaccaaaataagaaatgtgcatattagacaaccctgcttcccgaaactttaggaaggacacggagttgtgagtcacacaagggctatgctacttgaagtcaatgttcaccaatcaggcagcactaggtacagaagtcttggttctgaacctggacccaggagggaagtctgtgggaaaggggagaagagaatgacaagagaggatgtcatattaaaaaaaggtttcaaacaatattggcaggtgtctactcacaaggtgattggaaaactgcccacgaggagaagtcaactttacctcctcccaaattcacagtacgcgagtgtagtagggtcattgctgggagataaattgtctgaggagggccacccttcaggtttaccagaaatcttagggtttggcccccctggtcacaggctaaatatatggtttaaaagttttattaaaaagaaaaacagaacaagacacactcacacccagatgactaatgaaggctaagcagaatagtctgagtttgctgagactaaagcagggatagtgttgaaaagttttcctttcactagtgggacacattccccttttcttttcaaagaggaagaacatggtgtcatccaatgtgaagtgagcagtttcgggtcaaactcttatggtaagaaactaaaaaaagatgccaagagacaaaccttcagaaatagaagaaatgcaaaagatggaataaaaaccctgatcattaaaacagagacaccttcactggtgtccaataaggattctctttacaaaacagaaacaaacaactcaaaaatttaccatactttgtaatgaaaataccagtatgttgaagacacagcagactgggtttctattagaacaagtatcagcaaggtcatgtagacttgtagaaacttttgccttctcctgcaccagacagatcattgtccagttgggttgtcagctggagaccgaaaagaacctaaaaaatggatctttttttttttctttttcccatggtcacgcatccacacaaatgagtcttttggatgagaaaagtcacagcaacttgagttctcctaatgaacagatgactttttagccctgtttgtttcaatggggaaaacaatgacaaaaaaaacaaaccccaggcaggcacgacacttatgtaaaatgaacacagttagtacaaaaccagtaaggcatcactttgggaaggtcagcaccgaagaggtcaggcaaggctcgtccagacggggcttctgggagggagtgaccctcacccttattgagctgcgtcatgttggttctgaggaaagtgcaagtcttttgcagggtgaccgcatcaccccaccggaagctggggcggggacgctggaggtgttggtgtgtgttctaaaccctcaaggacgagaagggaaggcaaggtccatggctcacccacatgtcgaggaccaggtcctcatccattttaaaggacacagatacccccagccctagcaggaggaggcgagtgtgtaggactgtgaggatggacaactaaaaaccaaaactgagcaggaccaaaccaaaactcaactcctgcggttcttactttcaccaaaggattgattctgaccaagaggggaagggggaaaaaaaaatcttcaaaaatcaatgcatcagaaaggaagaaactcaacctcattttcaaaaggtaacctgttctccaaagtagaacaagtctcactatacacagtgtttgcagaaaaaaaaaaaaaaaaacctgattcattcatatatcagaaggaaagagacacatgctgttctgcactgacagccacatccactcgctcacactctcactccgtcactcactctcacggatattaatcagaggctgatggacctgaatggggtggtttgattggaacaggcaaaatacctctcgggtaaggaaagcaccatttaaaaaacatgaaagcacggtttatttgctcctaaggtttccctgtgtcgtagctctgtagtgcgttgaacgtgaccaaagcaagcaccctggttagcaccagttctccctgtggccggctgtgtgggagggtgggtggcacggctctgagacccagtctggagggtctgtgctgaggggaagccgtgcttctctgtgtttccgactttgctccagtctcttctgtctctgggaagctcatggcaggatgctgtttggtttcagagcttcatgtgggttctctttttttttttctctctgtctctcttttcatttcaacggcgatgatcctttcccgagaagtatcttcagtgtcttagggaggtcacagcaacaaggcaaaacaataattaaagtacaacagaaggtagtgcagttctcgctgtggaaggaagcggtccgcaggcagctggcccgggatgcctgcacccaggtcgaggctgaaggacggggggtctcggtgttcccgcagctctaaggctgtggctgggggctggctcaggaagtcatcttcagggtgatgtgggggatgcaggtggaatgcggtgaggagaagaggagggcgctgggctccgggcccctgtcacagagtggactccaaagaggagtccaagatgtcatcgtgatggctgttgctgttggagtcgctgtcatagctctgggggctggagtagttggctgcctcctgcagcctcatcagcatgttcatcagcgggtcaccttcagcatcactggggggcatctgcttgcttgtcgatccctcccgaggcatggagtagccgtcgaagccgacatcctcaggccgtaactgcagcaggggaggccactcgtgctgttgtgggctggctgcccatggatatgtgtccatcacccacttggcaggatcctcccagggggcgcgccttccatagagctggagtccttctctgacggcttccaggagataggggataatggaatagttccacaagtcggtgaaccacactctcgagccgtccacatcgatggggcatgacaggaagagccgggggccgatggtgacgtccgaggaactgtgagcctccaggaagcggttgaggtgatgccagaccttgggaatccagtcaatgatttttaccagctccatattgcgcacccgcccactgatctctgtttccatgagcttcctcctcaggaatcggccaaggaaacccttcacaggctccgtgtggttggcacaaagcacccatctgaagttatggtgaagctgcaggttgggagtcgaagaggtagcctggttcattgtgccaattatgtaagggcatttgtggtacttgcagttgagcagcccattgaagatctctcccagagagctcacgtggtgtaggttgtccaggatgatgacgaggggcatgtccacagcattgttctcactgttgcactggtcagcaaggttggacaggtactggcgcaattccttgctggacttatggtccacgttaaaggtggcgataaccccgtctgtcaactcccgtccctctcgaagcactatatactcagacagccggttggccaggtaggttttcccagtgccgctggggccagagagaatgatccgacggtgctctatcaggagggagacgtagcgctgcaggatgggcttgggaatcaaggactcaaacaccagtgagtccaggctgttttctgcgagccctttcacagtcactgagatggtcgtgttctctccaaccagatagccacaaggaagcagctccggtgtttcggaagtgttgctgcgcttgatttctccaatgctgtagccaagaacgctgtctgaattcagccctagctgactcactgggtcgacatgaatgatgtattctttgaacagccgtctaaccaccccatcgagcacatcccacttcgtcttgccactaactccaatgcagccaataagaaagagatgtggtctggaatcctccttccacttcatttcctcctgaaagctgacaactatcttaacatgcctgcctccttccttccgagccgagcattcaccagtgtcatccagcaacatgtccaggctggttgactcagtgaggttcaagctgtgctgggagaggcccatggactgcctcggggaggcagagatggacacttgggaaggagcccggctgcagccactgccttgagactctgacttcagccgatcattctcagctttcagcttctctatttcactctgcatcctgttcatggcctcccggagctggtccagctggtgggcagaactgagagcttctaagcggatatccgtcagcttcatctccttgtctcttaactcatttcggagctgcatgacggtctcagcttcactatccatgcattctgaaattagagagttggagtgagaattcctcagcagtggggtggaacctgtggacccattgtgcggtaactttggtgaggaaggcaaagaagaatccgtcatctcctcaatatctgaatgagaggacgcagattttggggacttcttcttcccgaaagcttgcttgaaggagctgcgtaactcattgacccagttcttccgcttcttcttctttgagtcactctctatgttgctgcccacgctggagtggctggtggcactgttgatgctggagacgctgtctgaggagtgctgcctgcggatgcggaggtctgcagactgggcagtgccgtttcctttgcagttgagctcaggtgtgttaattactccattaatggcagcctgggcagctgcgttctgtttctttagcagctcaatggtttttcttaactcattcagttctgagtccttctgctcagctgtcatggtcagactctggagcctgattgtcatgttaccaagactctgttcaaaggctgccacaaggtgagcatttgctgtcagctgggtggtcaaagctgaaactttctcctgggaggcatccagttcccgccgcagcttgcgaatctctgactggcatttttcttctggtgtagaataaactgacgatgtgctggaaaccaaggagagtgaggatccatgaactaactcataccttgcgtgatggaacaaaggaagagagaaatgaagtgagctgtgaagacggctgacaaagttgtccacagaacttttctcccatgattcttcttcaaacccatcccggaatgagcctgaacggctcatggttctgctcttctcatccagggacatggagctattccggaagcggctgtcagtgtatggatcatactgcccatcagcattggagaggctgtgagtcctcagcatggtcgggttggacaagctcatctgggtgacagtggtgggactcgcaagctgggaaaagttgaatcttgttccggagggagaagtcacgctggagccagaggaaaagggggaattggcagcggtgtcctgaaggcctcctgcagaatgggaccgtaaccattcttttgcatcttcttgcgtgcgaagctgggaggtgggagtatacctttctgacagtgtggtcttcacactgttagttctgacaaagggagtcaaggagtcgtccttggaggaggcgatgaggccagtggaagaattgtggctggggacccctccactgctgagggagatgtcgatggactcacagctggtgtggaggctgctgacagactgaaagcccaggccatccttgctaactgcggaggagctgctggcgttggtgccccaggtgaggctgttggaaggggccgagtgggctgagctggggctggaggctagcggagactggttgaggtccacattcttgctgtagagaggactgctgctcccactgctcaggacgccactgcctgacggggagtctaggttaccttgctgagtcatggtggcatgaggattggagatgaccaccgaatttttcatgttttcagctgtggcgatgggcacttgcttggtaggcttcccaccaaagagtctgcggagtgtgggagaggccacatctgggtacttggctccaggctggagactggtctgagccggactggacacaggctgggctgccggattcactttcaccgagttacaggaagccacactctcgttgtctgatgagatgcctttctccttgtctgtttggttgaccagacctggtagagagctgcctagggctgttttggaaggctccctcagtttgggcactggcaggcctgcggacttgctgctaatgttggaatctatgctgctggtgctagacctgttcccagccccgttccggctgttggacttactgggcctcggcaaactccggtactgaaggtttgtccgggagcttagggctagatacccgtcatcctgattctgagccccatccatacttgacttccgaccagcagaccgactgacgagtgcagatgactttgggattttgcccagtgtggctgacctgctggtgacagtcaccccgctggctgtgatcatggccaggccggcggcggaaccactctgcttcttgaacccaaagctgttggcattggcagtaggtgtcctagagctgctggggaggggctttttggattcgtcaccactgctccggcctgcatctgatggggagcgcttcacctgggaggctttaggagaaagccttcctttctcagacacctttgcgtcgtctgtttttccagttcctggggtcttcagtgcgcctgccggggctgaaggcttcgtccttggcatggtgatgcccacctgagctgtcatgcctcgccgccatgagcctgtctgggagatgacaggattcttcttgcccgacgtgcttttgtcggactcgtcagacacatcagaaggattccgcctccacttggaacctggctccatttttatgccgctgtctgagcctccgtctgatttcttgacatcatcaccagaccacagggaattcctctccacctgtgagtgcttctcagcatcagtctgcacatccaggttttttcgagaggaggcaggtgtgttggcataagagctgatggaggagctggtgttgatgtcatcagtgctgaggttgtctatggtgtcgctgatgccgctgctgacggagctgctgtcgtcccagctgtcagcgtctccgaggcccagggaggtatttcgttgcagggtctcccgtaccacagccatcccatcagggagccggttcaggcgacgggtatagaggccaagtccaccatcagtcatgtatccgcttgtaatgtcatcggtccggatgttcttgctcagaacatccccgtcgctcatgtagccgggggcatccatgctgatgccttccaggtccatctcatctcctgccttgtctgagacgtccacatggcagacactactgccccgggaggccagctgccttctcagaggggcggagtacacatagcgacctgactcagtgttgatgaacctgctggcgttggctcgagggggatacccattgcccattgagggggcgtctcctgcttggagccgagggctggactggcccagtctccaggacagaggtgtgggcctccctgtcaagctgagtatgctacggccactcatctccgtggtgacattggtgtcaaacgtggtttccaatgtgctgtgtgtaacctgagttccccttaaactggacatggtttcctccaaattctgccgcagatcagcgatgttcttcactgtccgcagccgccgagcctcaggatcttccccagtgagttcttccagagcaggctgtccagtcttggtgaagtggctgggctccacgctcacacctgttgagcttgactcggcagtaacattcccttcagtgtccgtctgagacctgtacaggaaaggtgcaaccgtggcagtgttgggatggttgtattgctgctggggctgaggtagctgaacactgacggtattgcttcctgtggtctgggtggtcccgacagacccactgacagtctggctgctgatgctgtggttcagggtggtccctcctgggccttttccttctgaggacgccaggctggaagaggaactggagtgtctgccgtccagctggggcttctgctgggggagtcctgagctcagcttcccactccggctccgctccccttccttggaaggcgctggggcacttggggatttcccgggcatgcttttcattcctggttttggtattccactgtgggaaggggccatgggctccttcttggcactgttgagcttcccccctttggggatgaagctggcaatcttggaggacttttttggcatctcgggcacagctgctccactggggtcttcttttggctcctccttgaggtccagcctctccgtcacagaggctctcttggcaaggtccttgcttttctccttatccttctcccgctgttgtttctccttctctttctcattgcctttcagagaactcttcttgttggtcagtgcccggctaaaagtcctctgggcaatgcccttgagtgcaatcttggggctgctggaagcagggcccacggtggtgagcatgcgactggcggcctccagctcctcgctctcttcgaagctgggcagagtctccagccgctcacagcttgtgtcccgggaccccggcccctcacctgcctttgagccccctttactgttgaaaagtttcagcttttccagcatggacttctgattgttgggggccggcttcatggcttcaggtgtgggcctgggggcctcaggcccaggaggcttgaccgagagcatggataccgtggcactgtgcttcacgctgagggatttgctgcgccaaggcttggtggctgcaccgggctgcgggatggccgaggaggtactgcaattagtaggggtggagctgctgccgctctccaaggaagcaggtgcattgtcactcattccggggtgggaggaggctgaacttgccaaaggctctttctcgtggctgcttggcggtgggggtggggaggtgactggtttggatttatcatagttgttaaagctctggctgcgtcggttgttagcagtagttgaccctccgcgtgttttggcctcgctgcctgcagcggataccctcgcggtaggacctggaagtctagagatctttttctgacccagagtgaagcggatgattttgctttgagatgagtccttggatgatgcactggactgcatttcagcttgtgcttttgactgctgatgtggcgctggctggtgaggctggcacggggcttggggagtgactggcacctgctgctgaggggtgccagcctggcactgggagggggccccggccacctgggatacggcgggcggcagaggtgaggagaggtgctgcttctggggctgctgctgctgctgcttgtatcgggagaggctgaagaagaggcctagaatggccttgaggtttccattcctgatctcttctgcagacagcccctggatgtttattcccttagctgccaggaaattcaagcaggcatctatgttttcaatcatttgggatctgttcttcggacagccattgatgtcttcaatcttttcatttgccacaacctggataatctgggccaggaggacgccatctgtcacatcttgctggagatccctgatgagacgcttgtggccggatttggctaggtaatgattggcccagtctgtgtagatctgggtatcgaacccgttttccaccgagccgctcttccgcagcgggagcccctcccccgctggctcctgcagcccctgcagcacctgcgatttcagggggatctggctaggataggtggtcttgctcacctccaccttgcttcccaacttcaggtagcagggctgggggcccgcccgggccgggggcacgtgcaggatgggcgcggcgctgtgcacgggtttgggcagtcccgacttcattttggaggcgaccaggatggccggcatcttctcccggggcttgggctttcccagcacgtccctggcagcggcggcgggggcgaccgctaaaggcagcgcgggtagcagagcaggcgccgggccttagcccacgaggcgcccaccaccagcggctaaaaaaaaaatccccaggtcggggaactcgaagcaatcgggcgagcgcgcctttggggtgccgggatgggaatgggggactggccacggcgctcagcgggtcccacctggacggatgctgccgccgggtctcacacctctcctgggtggcctttcaagagctctgggcgctcaggggctgccgcctcttgcaaatttcctcctgggaaacagaggcttggacgcccatattaacttgtcactgcatctccgaagtgaggaggcccctttggaagagacagaggcggcggcgacccacgagtcccgttccggaggctacgggtctgagccggcgagagaaagagcgagcagccaaggaaggaaaggagacagcagcgaaggaaggagagaagaagggcgcaagggtcccaagacgtctccaccgagaggcagctgccaccctgctcgcgagcaccgcagtgtcacccgcgacgcagcagaggtgcggcaagagcccccgaaaggtctctcttggggtgacagtcaccgctgcccagaaggcccccggactgagagcaccttagcgcctgcgggtctgcacatgctccgtgagctagatagaggcaaggctgtggccgtggggcgcgggcgccgggacgcgcggctggcgggccgggcagggctgcgctcgggagcggccgccgcgcttcccgggaaggctgcgctggctgcggggctcagcgcaggggag

SEQ ID NO: 17901 - RNA, 11408 nt, Homo sapiens
  source 1..11408: mol_type = other RNA
tcggcctggggaggaggaaggggagggaggatggaaacataccgtacacaaaatactcaattcctagttttctctttaaaaatggctagaaaaaattcatcaaaatgcagcactttaatcaattatttacaatttctatgttacaatgaaaaaatgtacatcttatagaacatatttcataaaactgctccactggaaacaactagatcaaaacagcaaaccttccatttaatatccacaaagttggattatttttcctttttgaagtagattcgccacaatcaaatttgaatacagagaattttgaagtttaagcatcaaacaacaaagtaaaagtccccaagatacaacaaagatctaggcaagtcttgttcctgtcccactcccaccccacccctaatgaaacttaaaaggtattcccatttcaattatggcctgtatcattcttggcagtttgggaagagaacttttggcttccattggtaactcaacataaatgttgcatagaatttatatatttcaaaattggcctaactgtagaaaaggcaaaatggaagcatttccgatagagccctaaatgagtacaaagtcactttgtaaaaggtgagtgacactaaagtaaaaatatgaccaaaataagaaatgtgcatattagacaaccctgcttcccgaaactttaggaaggacacggagttgtgagtcacacaagggctatgctacttgaagtcaatgttcaccaatcaggcagcactaggtacagaagtcttggttctgaacctggacccaggagggaagtctgtgggaaaggggagaagagaatgacaagagaggatgtcatattaaaaaaaggtttcaaacaatattggcaggtgtctactcacaaggtgattggaaaactgcccacgaggagaagtcaactttacctcctcccaaattcacagtacgcgagtgtagtagggtcattgctgggagataaattgtctgaggagggccacccttcaggtttaccagaaatcttagggtttggcccccctggtcacaggctaaatatatggtttaaaagttttattaaaaagaaaaacagaacaagacacactcacacccagatgactaatgaaggctaagcagaatagtctgagtttgctgagactaaagcagggatagtgttgaaaagttttcctttcactagtgggacacattccccttttcttttcaaagaggaagaacatggtgtcatccaatgtgaagtgagcagtttcgggtcaaactcttatggtaagaaactaaaaaaagatgccaagagacaaaccttcagaaatagaagaaatgcaaaagatggaataaaaaccctgatcattaaaacagagacaccttcactggtgtccaataaggattctctttacaaaacagaaacaaacaactcaaaaatttaccatactttgtaatgaaaataccagtatgttgaagacacagcagactgggtttctattagaacaagtatcagcaaggtcatgtagacttgtagaaacttttgccttctcctgcaccagacagatcattgtccagttgggttgtcagctggagaccgaaaagaacctaaaaaatggatctttttttttttctttttcccatggtcacgcatccacacaaatgagtcttttggatgagaaaagtcacagcaacttgagttctcctaatgaacagatgactttttagccctgtttgtttcaatggggaaaacaatgacaaaaaaaacaaaccccaggcaggcacgacacttatgtaaaatgaacacagttagtacaaaaccagtaaggcatcactttgggaaggtcagcaccgaagaggtcaggcaaggctcgtccagacggggcttctgggagggagtgaccctcacccttattgagctgcgtcatgttggttctgaggaaagtgcaagtcttttgcagggtgaccgcatcaccccaccggaagctggggcggggacgctggaggtgttggtgtgtgttctaaaccctcaaggacgagaagggaaggcaaggtccatggctcacccacatgtcgaggaccaggtcctcatccattttaaaggacacagatacccccagccctagcaggaggaggcgagtgtgtaggactgtgaggatggacaactaaaaaccaaaactgagcaggaccaaaccaaaactcaactcctgcggttcttactttcaccaaaggattgattctgaccaagaggggaagggggaaaaaaaaatcttcaaaaatcaatgcatcagaaaggaagaaactcaacctcattttcaaaaggtaacctgttctccaaagtagaacaagtctcactatacacagtgtttgcagaaaaaaaaaaaaaaaaacctgattcattcatatatcagaaggaaagagacacatgctgttctgcactgacagccacatccactcgctcacactctcactccgtcactcactctcacggatattaatcagaggctgatggacctgaatggggtggtttgattggaacaggcaaaatacctctcgggtaaggaaagcaccatttaaaaaacatgaaagcacggtttatttgctcctaaggtttccctgtgtcgtagctctgtagtgcgttgaacgtgaccaaagcaagcaccctggttagcaccagttctccctgtggccggctgtgtgggagggtgggtggcacggctctgagacccagtctggagggtctgtgctgaggggaagccgtgcttctctgtgtttccgactttgctccagtctcttctgtctctgggaagctcatggcaggatgctgtttggtttcagagcttcatgtgggttctctttttttttttctctctgtctctcttttcatttcaacggcgatgatcctttcccgagaagtatcttcagtgtcttagggaggtcacagcaacaaggcaaaacaataattaaagtacaacagaaggtagtgcagttctcgctgtggaaggaagcggtccgcaggcagctggcccgggatgcctgcacccaggtcgaggctgaaggacggggggtctcggtgttcccgcagctctaaggctgtggctgggggctggctcaggaagtcatcttcagggtgatgtgggggatgcaggtggaatgcggtgaggagaagaggagggcgctgggctccgggcccctgtcacagagtggactccaaagaggagtccaagatgtcatcgtgatggctgttgctgttggagtcgctgtcatagctctgggggctggagtagttggctgcctcctgcagcctcatcagcatgttcatcagcgggtcaccttcagcatcactggggggcatctgcttgcttgtcgatccctcccgaggcatggagtagccgtcgaagccgacatcctcaggccgtaactgcagcaggggaggccactcgtgctgttgtgggctggctgcccatggatatgtgtccatcacccacttggcaggatcctcccagggggcgcgccttccatagagctggagtccttctctgacggcttccaggagataggggataatggaatagttccacaagtcggtgaaccacactctcgagccgtccacatcgatggggcatgacaggaagagccgggggccgatggtgacgtccgaggaactgtgagcctccaggaagcggttgaggtgatgccagaccttgggaatccagtcaatgatttttaccagctccatattgcgcacccgcccactgatctctgtttccatgagcttcctcctcaggaatcggccaaggaaacccttcacaggctccgtgtggttggcacaaagcacccatctgaagttatggtgaagctgcaggttgggagtcgaagaggtagcctggttcattgtgccaattatgtaagggcatttgtggtacttgcagttgagcagcccattgaagatctctcccagagagctcacgtggtgtaggttgtccaggatgatgacgaggggcatgtccacagcattgttctcactgttgcactggtcagcaaggttggacaggtactggcgcaattccttgctggacttatggtccacgttaaaggtggcgataaccccgtctgtcaactcccgtccctctcgaagcactatatactcagacagccggttggccaggtaggttttcccagtgccgctggggccagagagaatgatccgacggtgctctatcaggagggagacgtagcgctgcaggatgggcttgggaatcaaggactcaaacaccagtgagtccaggctgttttctgcgagccctttcacagtcactgagatggtcgtgttctctccaaccagatagccacaaggaagcagctccggtgtttcggaagtgttgctgcgcttgatttctccaatgctgtagccaagaacgctgtctgaattcagccctagctgactcactgggtcgacatgaatgatgtattctttgaacagccgtctaaccaccccatcgagcacatcccacttcgtcttgccactaactccaatgcagccaataagaaagagatgtggtctggaatcctccttccacttcatttcctcctgaaagctgacaactatcttaacatgcctgcctccttccttccgagccgagcattcaccagtgtcatccagcaacatgtccaggctggttgactcagtgaggttcaagctgtgctgggagaggcccatggactgcctcggggaggcagagatggacacttgggaaggagcccggctgcagccactgccttgagactctgacttcagccgatcattctcagctttcagcttctctatttcactctgcatcctgttcatggcctcccggagctggtccagctggtgggcagaactgagagcttctaagcggatatccgtcagcttcatctccttgtctcttaactcatttcggagctgcatgacggtctcagcttcactatccatgcattctgaaattagagagttggagtgagaattcctcagcagtggggtggaacctgtggacccattgtgcggtaactttggtgaggaaggcaaagaagaatccgtcatctcctcaatatctgaatgagaggacgcagattttggggacttcttcttcccgaaagcttgcttgaaggagctgcgtaactcattgacccagttcttccgcttcttcttctttgagtcactctctatgttgctgcccacgctggagtggctggtggcactgttgatgctggagacgctgtctgaggagtgctgcctgcggatgcggaggtctgcagactgggcagtgccgtttcctttgcagttgagctcaggtgtgttaattactccattaatggcagcctgggcagctgcgttctgtttctttagcagctcaatggtttttcttaactcattcagttctgagtccttctgctcagctgtcatggtcagactctggagcctgattgtcatgttaccaagactctgttcaaaggctgccacaaggtgagcatttgctgtcagctgggtggtcaaagctgaaactttctcctgggaggcatccagttcccgccgcagcttgcgaatctctgactggcatttttcttctggtgtagaataaactgacgatgtgctggaaaccaaggagagtgaggatccatgaacttcttcaaacccatcccggaatgagcctgaacggctcatggttctgctcttctcatccagggacatggagctattccggaagcggctgtcagtgtatggatcatactgcccatcagcattggagaggctgtgagtcctcagcatggtcgggttggacaagctcatctgggtgacagtggtgggactcgcaagctgggaaaagttgaatcttgttccggagggagaagtcacgctggagccagaggaaaagggggaattggcagcggtgtcctgaaggcctcctgcagaatgggaccgtaaccattcttttgcatcttcttgcgtgcgaagctgggaggtgggagtatacctgagtcctttcttaggcaaagtgttcctatcaaggtgcgggtcactgtcctgtttcctgggcagagtacttctgcagaacttagggctagcagcaggggaagagagagggctttctgacagtgtggtcttcacactgttagttctgacaaagggagtcaaggagtcgtccttggaggaggcgatgaggccagtggaagaattgtggctggggacccctccactgctgagggagatgtcgatggactcacagctggtgtggaggctgctgacagactgaaagcccaggccatccttgctaactgcggaggagctgctggcgttggtgccccaggtgaggctgttggaaggggccgagtgggctgagctggggctggaggctagcggagactggttgaggtccacattcttgctgtagagaggactgctgctcccactgctcaggacgccactgcctgacggggagtctaggttaccttgctgagtcatggtggcatgaggattggagatgaccaccgaatttttcatgttttcagctgtggcgatgggcacttgcttggtaggcttcccaccaaagagtctgcggagtgtgggagaggccacatctgggtacttggctccaggctggagactggtctgagccggactggacacaggctgggctgccggattcactttcaccgagttacaggaagccacactctcgttgtctgatgagatgcctttctccttgtctgtttggttgaccagacctggtagagagctgcctagggctgttttggaaggctccctcagtttgggcactggcaggcctgcggacttgctgctaatgttggaatctatgctgctggtgctagacctgttcccagccccgttccggctgttggacttactgggcctcggcaaactccggtactgaaggtttgtccgggagcttagggctagatacccgtcatcctgattctgagccccatccatacttgacttccgaccagcagaccgactgacgagtgcagatgactttgggattttgcccagtgtggctgacctgctggtgacagtcaccccgctggctgtgatcatggccaggccggcggcggaaccactctgcttcttgaacccaaagctgttggcattggcagtaggtgtcctagagctgctggggaggggctttttggattcgtcaccactgctccggcctgcatctgatggggagcgcttcacctgggaggctttaggagaaagccttcctttctcagacacctttgcgtcgtctgtttttccagttcctggggtcttcagtgcgcctgccggggctgaaggcttcgtccttggcatggtgatgcccacctgagctgtcatgcctcgccgccatgagcctgtctgggagatgacaggattcttcttgcccgacgtgcttttgtcggactcgtcagacacatcagaaggattccgcctccacttggaacctggctccatttttatgccgctgtctgagcctccgtctgatttcttgacatcatcaccagaccacagggaattcctctccacctgtgagtgcttctcagcatcagtctgcacatccaggttttttcgagaggaggcaggtgtgttggcataagagctgatggaggagctggtgttgatgtcatcagtgctgaggttgtctatggtgtcgctgatgccgctgctgacggagctgctgtcgtcccagctgtcagcgtctccgaggcccagggaggtatttcgttgcagggtctcccgtaccacagccatcccatcagggagccggttcaggcgacgggtatagaggccaagtccaccatcagtcatgtatccgcttgtaatgtcatcggtccggatgttcttgctcagaacatccccgtcgctcatgtagccgggggcatccatgctgatgccttccaggtccatctcatctcctgccttgtctgagacgtccacatggcagacactactgccccgggaggccagctgccttctcagaggggcggagtacacatagcgacctgactcagtgttgatgaacctgctggcgttggctcgagggggatacccattgcccattgagggggcgtctcctgcttggagccgagggctggactggcccagtctccaggacagaggtgtgggcctccctgtcaagctgagtatgctacggccactcatctccgtggtgacattggtgtcaaacgtggtttccaatgtgctgtgtgtaacctgagttccccttaaactggacatggtttcctccaaattctgccgcagatcagcgatgttcttcactgtccgcagccgccgagcctcaggatcttccccagtgagttcttccagagcaggctgtccagtcttggtgaagtggctgggctccacgctcacacctgttgagcttgactcggcagtaacattcccttcagtgtccgtctgagacctgtacaggaaaggtgcaaccgtggcagtgttgggatggttgtattgctgctggggctgaggtagctgaacactgacggtattgcttcctgtggtctgggtggtcccgacagacccactgacagtctggctgctgatgctgtggttcagggtggtccctcctgggccttttccttctgaggacgccaggctggaagaggaactggagtgtctgccgtccagctggggcttctgctgggggagtcctgagctcagcttcccactccggctccgctccccttccttggaaggcgctggggcacttggggatttcccgggcatgcttttcattcctggttttggtattccactgtgggaaggggccatgggctccttcttggcactgttgagcttcccccctttggggatgaagctggcaatcttggaggacttttttggcatctcgggcacagctgctccactggggtcttcttttggctcctccttgaggtccagcctctccgtcacagaggctctcttggcaaggtccttgcttttctccttatccttctcccgctgttgtttctccttctctttctcattgcctttcagagaactcttcttgttggtcagtgcccggctaaaagtcctctgggcaatgcccttgagtgcaatcttggggctgctggaagcagggcccacggtggtgagcatgcgactggcggcctccagctcctcgctctcttcgaagctgggcagagtctccagccgctcacagcttgtgtcccgggaccccggcccctcacctgcctttgagccccctttactgttgaaaagtttcagcttttccagcatggacttctgattgttgggggccggcttcatggcttcaggtgtgggcctgggggcctcaggcccaggaggcttgaccgagagcatggataccgtggcactgtgcttcacgctgagggatttgctgcgccaaggcttggtggctgcaccgggctgcgggatggccgaggaggtactgcaattagtaggggtggagctgctgccgctctccaaggaagcaggtgcattgtcactcattccggggtgggaggaggctgaacttgccaaaggctctttctcgtggctgcttggcggtgggggtggggaggtgactggtttggatttatcatagttgttaaagctctggctgcgtcggttgttagcagtagttgaccctccgcgtgttttggcctcgctgcctgcagcggataccctcgcggtaggacctggaagtctagagatctttttctgacccagagtgaagcggatgattttgctttgagatgagtccttggatgatgcactggactgcatttcagcttgtgcttttgactgctgatgtggcgctggctggtgaggctggcacggggcttggggagtgactggcacctgctgctgaggggtgccagcctggcactgggagggggccccggccacctgggatacggcgggcggcagaggtgaggagaggtgctgcttctggggctgctgctgctgctgcttgtatcgggagaggctgaagaagaggcctagaatggccttgaggtttccattcctgatctcttctgcagacagcccctggatgtttattcccttagctgccaggaaattcaagcaggcatctatgttttcaatcatttgggatctgttcttcggacagccattgatgtcttcaatcttttcatttgccacaacctggataatctgggccaggaggacgccatctgtcacatcttgctggagatccctgatgagacgcttgtggccggatttggctaggtaatgattggcccagtctgtgtagatctgggtatcgaacccgttttccaccgagccgctcttccgcagcgggagcccctcccccgctggctcctgcagcccctgcagcacctgcgatttcagggggatctggctaggataggtggtcttgctcacctccaccttgcttcccaacttcaggtagcagggctgggggcccgcccgggccgggggcacgtgcaggatgggcgcggcgctgtgcacgggtttgggcagtcccgacttcattttggaggcgaccaggatggccggcatcttctcccggggcttgggctttcccagcacgtccctggcagcggcggcgggggcgaccgctaaaggcagcgcgggtagcagagcaggcgccgggccttagcccacgaggcgcccaccaccagcggctaaaaaaaaaatccccaggtcggggaactcgaagcaatcgggcgagcgcgcctttggggtgccgggatgggaatgggggactggccacggcgctcagcgggtcccacctggacggatgctgccgccgggtctcacacctctcctgggtggcctttcaagagctctgggcgctcaggggctgccgcctcttgcaaatttcctcctgggaaacagaggcttggacgcccatattaacttgtcactgcatctccgaagtgaggaggcccctttggaagagacagaggcggcggcgacccacgagtcccgttccggaggctacgggtctgagccggcgagagaaagagcgagcagccaaggaaggaaaggagacagcagcgaaggaaggagagaagaagggcgcaagggtcccaagacgtctccaccgagaggcagctgccaccctgctcgcgagcaccgcagtgtcacccgcgacgcagcagaggtgcggcaagagcccccgaaaggtctctcttggggtgacagtcaccgctgcccagaaggcccccggactgagagcaccttagcgcctgcgggtctgcacatgctccgtgagctagatagaggcaaggctgtggccgtggggcgcgggcgccgggacgcgcggctggcgggccgggcagggctgcgctcgggagcggccgccgcgcttcccgggaaggctgcgctggctgcggggctcagcgcaggggag

SEQ ID NO: 17902 - RNA, 11342 nt, Homo sapiens
  source 1..11342: mol_type = other RNA
tcggcctggggaggaggaaggggagggaggatggaaacataccgtacacaaaatactcaattcctagttttctctttaaaaatggctagaaaaaattcatcaaaatgcagcactttaatcaattatttacaatttctatgttacaatgaaaaaatgtacatcttatagaacatatttcataaaactgctccactggaaacaactagatcaaaacagcaaaccttccatttaatatccacaaagttggattatttttcctttttgaagtagattcgccacaatcaaatttgaatacagagaattttgaagtttaagcatcaaacaacaaagtaaaagtccccaagatacaacaaagatctaggcaagtcttgttcctgtcccactcccaccccacccctaatgaaacttaaaaggtattcccatttcaattatggcctgtatcattcttggcagtttgggaagagaacttttggcttccattggtaactcaacataaatgttgcatagaatttatatatttcaaaattggcctaactgtagaaaaggcaaaatggaagcatttccgatagagccctaaatgagtacaaagtcactttgtaaaaggtgagtgacactaaagtaaaaatatgaccaaaataagaaatgtgcatattagacaaccctgcttcccgaaactttaggaaggacacggagttgtgagtcacacaagggctatgctacttgaagtcaatgttcaccaatcaggcagcactaggtacagaagtcttggttctgaacctggacccaggagggaagtctgtgggaaaggggagaagagaatgacaagagaggatgtcatattaaaaaaaggtttcaaacaatattggcaggtgtctactcacaaggtgattggaaaactgcccacgaggagaagtcaactttacctcctcccaaattcacagtacgcgagtgtagtagggtcattgctgggagataaattgtctgaggagggccacccttcaggtttaccagaaatcttagggtttggcccccctggtcacaggctaaatatatggtttaaaagttttattaaaaagaaaaacagaacaagacacactcacacccagatgactaatgaaggctaagcagaatagtctgagtttgctgagactaaagcagggatagtgttgaaaagttttcctttcactagtgggacacattccccttttcttttcaaagaggaagaacatggtgtcatccaatgtgaagtgagcagtttcgggtcaaactcttatggtaagaaactaaaaaaagatgccaagagacaaaccttcagaaatagaagaaatgcaaaagatggaataaaaaccctgatcattaaaacagagacaccttcactggtgtccaataaggattctctttacaaaacagaaacaaacaactcaaaaatttaccatactttgtaatgaaaataccagtatgttgaagacacagcagactgggtttctattagaacaagtatcagcaaggtcatgtagacttgtagaaacttttgccttctcctgcaccagacagatcattgtccagttgggttgtcagctggagaccgaaaagaacctaaaaaatggatctttttttttttctttttcccatggtcacgcatccacacaaatgagtcttttggatgagaaaagtcacagcaacttgagttctcctaatgaacagatgactttttagccctgtttgtttcaatggggaaaacaatgacaaaaaaaacaaaccccaggcaggcacgacacttatgtaaaatgaacacagttagtacaaaaccagtaaggcatcactttgggaaggtcagcaccgaagaggtcaggcaaggctcgtccagacggggcttctgggagggagtgaccctcacccttattgagctgcgtcatgttggttctgaggaaagtgcaagtcttttgcagggtgaccgcatcaccccaccggaagctggggcggggacgctggaggtgttggtgtgtgttctaaaccctcaaggacgagaagggaaggcaaggtccatggctcacccacatgtcgaggaccaggtcctcatccattttaaaggacacagatacccccagccctagcaggaggaggcgagtgtgtaggactgtgaggatggacaactaaaaaccaaaactgagcaggaccaaaccaaaactcaactcctgcggttcttactttcaccaaaggattgattctgaccaagaggggaagggggaaaaaaaaatcttcaaaaatcaatgcatcagaaaggaagaaactcaacctcattttcaaaaggtaacctgttctccaaagtagaacaagtctcactatacacagtgtttgcagaaaaaaaaaaaaaaaaacctgattcattcatatatcagaaggaaagagacacatgctgttctgcactgacagccacatccactcgctcacactctcactccgtcactcactctcacggatattaatcagaggctgatggacctgaatggggtggtttgattggaacaggcaaaatacctctcgggtaaggaaagcaccatttaaaaaacatgaaagcacggtttatttgctcctaaggtttccctgtgtcgtagctctgtagtgcgttgaacgtgaccaaagcaagcaccctggttagcaccagttctccctgtggccggctgtgtgggagggtgggtggcacggctctgagacccagtctggagggtctgtgctgaggggaagccgtgcttctctgtgtttccgactttgctccagtctcttctgtctctgggaagctcatggcaggatgctgtttggtttcagagcttcatgtgggttctctttttttttttctctctgtctctcttttcatttcaacggcgatgatcctttcccgagaagtatcttcagtgtcttagggaggtcacagcaacaaggcaaaacaataattaaagtacaacagaaggtagtgcagttctcgctgtggaaggaagcggtccgcaggcagctggcccgggatgcctgcacccaggtcgaggctgaaggacggggggtctcggtgttcccgcagctctaaggctgtggctgggggctggctcaggaagtcatcttcagggtgatgtgggggatgcaggtggaatgcggtgaggagaagaggagggcgctgggctccgggcccctgtcacagagtggactccaaagaggagtccaagatgtcatcgtgatggctgttgctgttggagtcgctgtcatagctctgggggctggagtagttggctgcctcctgcagcctcatcagcatgttcatcagcgggtcaccttcagcatcactggggggcatctgcttgcttgtcgatccctcccgaggcatggagtagccgtcgaagccgacatcctcaggccgtaactgcagcaggggaggccactcgtgctgttgtgggctggctgcccatggatatgtgtccatcacccacttggcaggatcctcccagggggcgcgccttccatagagctggagtccttctctgacggcttccaggagataggggataatggaatagttccacaagtcggtgaaccacactctcgagccgtccacatcgatggggcatgacaggaagagccgggggccgatggtgacgtccgaggaactgtgagcctccaggaagcggttgaggtgatgccagaccttgggaatccagtcaatgatttttaccagctccatattgcgcacccgcccactgatctctgtttccatgagcttcctcctcaggaatcggccaaggaaacccttcacaggctccgtgtggttggcacaaagcacccatctgaagttatggtgaagctgcaggttgggagtcgaagaggtagcctggttcattgtgccaattatgtaagggcatttgtggtacttgcagttgagcagcccattgaagatctctcccagagagctcacgtggtgtaggttgtccaggatgatgacgaggggcatgtccacagcattgttctcactgttgcactggtcagcaaggttggacaggtactggcgcaattccttgctggacttatggtccacgttaaaggtggcgataaccccgtctgtcaactcccgtccctctcgaagcactatatactcagacagccggttggccaggtaggttttcccagtgccgctggggccagagagaatgatccgacggtgctctatcaggagggagacgtagcgctgcaggatgggcttgggaatcaaggactcaaacaccagtgagtccaggctgttttctgcgagccctttcacagtcactgagatggtcgtgttctctccaaccagatagccacaaggaagcagctccggtgtttcggaagtgttgctgcgcttgatttctccaatgctgtagccaagaacgctgtctgaattcagccctagctgactcactgggtcgacatgaatgatgtattctttgaacagccgtctaaccaccccatcgagcacatcccacttcgtcttgccactaactccaatgcagccaataagaaagagatgtggtctggaatcctccttccacttcatttcctcctgaaagctgacaactatcttaacatgcctgcctccttccttccgagccgagcattcaccagtgtcatccagcaacatgtccaggctggttgactcagtgaggttcaagctgtgctgggagaggcccatggactgcctcggggaggcagagatggacacttgggaaggagcccggctgcagccactgccttgagactctgacttcagccgatcattctcagctttcagcttctctatttcactctgcatcctgttcatggcctcccggagctggtccagctggtgggcagaactgagagcttctaagcggatatccgtcagcttcatctccttgtctcttaactcatttcggagctgcatgacggtctcagcttcactatccatgcattctgaaattagagagttggagtgagaattcctcagcagtggggtggaacctgtggacccattgtgcggtaactttggtgaggaaggcaaagaagaatccgtcatctcctcaatatctgaatgagaggacgcagattttggggacttcttcttcccgaaagcttgcttgaaggagctgcgtaactcattgacccagttcttccgcttcttcttctttgagtcactctctatgttgctgcccacgctggagtggctggtggcactgttgatgctggagacgctgtctgaggagtgctgcctgcggatgcggaggtctgcagactgggcagtgccgtttcctttgcagttgagctcaggtgtgttaattactccattaatggcagcctgggcagctgcgttctgtttctttagcagctcaatggtttttcttaactcattcagttctgagtccttctgctcagctgtcatggtcagactctggagcctgattgtcatgttaccaagactctgttcaaaggctgccacaaggtgagcatttgctgtcagctgggtggtcaaagctgaaactttctcctgggaggcatccagttcccgccgcagcttgcgaatctctgactggcatttttcttctggtgtagaataaactgacgatgtgctggaaaccaaggagagtgaggatccatgaacttcttcaaacccatcccggaatgagcctgaacggctcatggttctgctcttctcatccagggacatggagctattccggaagcggctgtcagtgtatggatcatactgcccatcagcattggagaggctgtgagtcctcagcatggtcgggttggacaagctcatctgggtgacagtggtgggactcgcaagctgggaaaagttgaatcttgttccggagggagaagtcacgctggagccagaggaaaagggggaattggcagcggtgtcctgaaggcctcctgcagaatgggaccgtaaccattcttttgcatcttcttgcgtgcgaagctgggaggtgggagtatacctgagtcctttcttaggcaaagtgttcctatcaaggtgcgggtcactgtcctgtttcctgggcagagtacttctgcagaacttagggctagcagcaggggaagagagagggctttctgacagtgtggtcttcacactgttagttctgacaaagggagtcaaggagtcgtccttggaggaggcgatgaggccagtggaagaattgtggctggggacccctccactgctgagggagatgtcgatggactcacagctggtgtggaggctgctgacagactgaaagcccaggccatccttgctaactgcggaggagctgctggcgttggtgccccaggtgaggctgttggaaggggccgagtgggctgagctggggctggaggctagcggagactggttgaggtccacattcttgctgtagagaggactgctgctcccactgctcaggacgccactgcctgacggggagtctaggttaccttgctgagtcatggtggcatgaggattggagatgaccaccgaatttttcatgttttcagctgtggcgatgggcacttgcttggtaggcttcccaccaaagagtctgcggagtgtgggagaggccacatctgggtacttggctccaggctggagactggtctgagccggactggacacaggctgggctgccggattcactttcaccgagttacaggaagccacactctcgttgtctgatgagatgcctttctccttgtctgtttggttgaccagacctggtagagagctgcctagggctgttttggaaggctccctcagtttgggcactggcaggcctgcggacttgctgctaatgttggaatctatgctgctggtgctagacctgttcccagccccgttccggctgttggacttactgggcctcggcaaactccggtactgaaggtttgtccgggagcttagggctagatacccgtcatcctgattctgagccccatccatacttgacttccgaccagcagaccgactgacgagtgcagatgactttgggattttgcccagtgtggctgacctgctggtgacagtcaccccgctggctgtgatcatggccaggccggcggcggaaccactctgcttcttgaacccaaagctgttggcattggcagtaggtgtcctagagctgctggggaggggctttttggattcgtcaccactgctccggcctgcatctgatggggagcgcttcacctgggaggctttaggagaaagccttcctttctcagacacctttgcgtcgtctgtttttccagttcctggggtcttcagtgcgcctgccggggctgaaggcttcgtccttggcatggtgatgcccacctgagctgtcatgcctcgccgccatgagcctgtctgggagatgacaggattcttcttgcccgacgtgcttttgtcggactcgtcagacacatcagaaggattccgcctccacttggaacctggctccatttttatgccgctgtctgagcctccgtctgatttcttgacatcatcaccagaccacagggaattcctctccacctgtgagtgcttctcagcatcagtctgcacatccaggttttttcgagaggaggcaggtgtgttggcataagagctgatggaggagctggtgttgatgtcatcagtgctgaggttgtctatggtgtcgctgatgccgctgctgacggagctgctgtcgtcccagctgtcagcgtctccgaggcccagggaggtatttcgttgcagggtctcccgtaccacagccatcccatcagggagccggttcaggcgacgggtatagaggccaagtccaccatcagtcatgtatccgcttgtaatgtcatcggtccggatgttcttgctcagaacatccccgtcgctcatgtagccgggggcatccatgctgatgccttccaggtccatctcatctcctgccttgtctgagacgtccacatggcagacactactgccccgggaggccagctgccttctcagaggggcggagtacacatagcgacctgactcagtgttgatgaacctgctggcgttggctcgagggggatacccattgcccattgagggggcgtctcctgcttggagccgagggctggactggcccagtctccaggacagaggtgtgggcctccctgtcaagctgagtatgctacggccactcatctccgtggtgacattggtgtcaaacgtggtttccaatgtgctgtgtgtaacctgagttccccttaaactggacatggtttcctccaaattctgccgcagatcagcgatgttcttcactgtccgcagccgccgagcctcaggatcttccccagtgagttcttccagagcaggctgtccagtcttggtgaagtggctgggctccacgctcacacctgttgagcttgactcggcagtaacattcccttcagtgtccgtctgagacctgtacaggaaaggtgcaaccgtggcagtgttgggatggttgtattgctgctggggctgaggtagctgaacactgacggtattgcttcctgtggtctgggtggtcccgacagacccactgacagtctggctgctgatgctgtggttcagggtggtccctcctgggccttttccttctgaggacgccaggctggaagaggaactggagtgtctgccgtccagctggggcttctgctgggggagtcctgagctcagcttcccactccggctccgctccccttccttggaaggcgctggggcacttggggatttcccgggcatgcttttcattcctggttttggtattccactgtgggaaggggccatgggctccttcttggcactgttgagcttcccccctttggggatgaagctggcaatcttggaggacttttttggcatctcgggcacagctgctccactggggtcttcttttggctcctccttgaggtccagcctctccgtcacagaggctctcttggcaaggtccttgcttttctccttatccttctcccgctgttgtttctccttctctttctcattgcctttcagagaactcttcttgttggtcagtgcccggctaaaagtcctctgggcaatgcccttgagtgcaatcttggggctgctggaagcagggcccacggtggtgagcatgcgactggcggcctccagctcctcgctctcttcgaagctgggcagagtctccagccgctcacagcttgtgtcccgggaccccggcccctcacctgcctttgagccccctttactgttgaaaagtttcagcttttccagcatggacttctgattgttgggggccggcttcatggcttcaggtgtgggcctgggggcctcaggcccaggaggcttgaccgagagcatggataccgtggcactgtgcttcacgctgagggatttgctgcgccaaggcttggtggctgcaccgggctgcgggatggccgaggaggtactgcaattagtaggggtggagctgctgccgctctccaaggaagcaggtgcattgtcactcattccggggtgggaggaggctgaacttgccaaaggctctttctcgtggctgcttggcggtgggggtggggaggtgactggtttggatttatcatagttgttaaagctctggctgcgtcggttgttagcagtagttgaccctccgcgtgttttggcctcgctgcctgcagcggataccctcgcggtaggacctggaagtctggactgcatttcagcttgtgcttttgactgctgatgtggcgctggctggtgaggctggcacggggcttggggagtgactggcacctgctgctgaggggtgccagcctggcactgggagggggccccggccacctgggatacggcgggcggcagaggtgaggagaggtgctgcttctggggctgctgctgctgctgcttgtatcgggagaggctgaagaagaggcctagaatggccttgaggtttccattcctgatctcttctgcagacagcccctggatgtttattcccttagctgccaggaaattcaagcaggcatctatgttttcaatcatttgggatctgttcttcggacagccattgatgtcttcaatcttttcatttgccacaacctggataatctgggccaggaggacgccatctgtcacatcttgctggagatccctgatgagacgcttgtggccggatttggctaggtaatgattggcccagtctgtgtagatctgggtatcgaacccgttttccaccgagccgctcttccgcagcgggagcccctcccccgctggctcctgcagcccctgcagcacctgcgatttcagggggatctggctaggataggtggtcttgctcacctccaccttgcttcccaacttcaggtagcagggctgggggcccgcccgggccgggggcacgtgcaggatgggcgcggcgctgtgcacgggtttgggcagtcccgacttcattttggaggcgaccaggatggccggcatcttctcccggggcttgggctttcccagcacgtccctggcagcggcggcgggggcgaccgctaaaggcagcgcgggtagcagagcaggcgccgggccttagcccacgaggcgcccaccaccagcggctaaaaaaaaaatccccaggtcggggaactcgaagcaatcgggcgagcgcgcctttggggtgccgggatgggaatgggggactggccacggcgctcagcgggtcccacctggacggatgctgccgccgggtctcacacctctcctgggtggcctttcaagagctctgggcgctcaggggctgccgcctcttgcaaatttcctcctgggaaacagaggcttggacgcccatattaacttgtcactgcatctccgaagtgaggaggcccctttggaagagacagaggcggcggcgacccacgagtcccgttccggaggctacgggtctgagccggcgagagaaagagcgagcagccaaggaaggaaaggagacagcagcgaaggaaggagagaagaagggcgcaagggtcccaagacgtctccaccgagaggcagctgccaccctgctcgcgagcaccgcagtgtcacccgcgacgcagcagaggtgcggcaagagcccccgaaaggtctctcttggggtgacagtcaccgctgcccagaaggcccccggactgagagcaccttagcgcctgcgggtctgcacatgctccgtgagctagatagaggcaaggctgtggccgtggggcgcgggcgccgggacgcgcggctggcgggccgggcagggctgcgctcgggagcggccgccgcgcttcccgggaaggctgcgctggctgcggggctcagcgcaggggaggac

SEQ ID NO: 17903 - RNA, 11297 nt, Homo sapiens
  source 1..11297: mol_type = other RNA
tcggcctggggaggaggaaggggagggaggatggaaacataccgtacacaaaatactcaattcctagttttctctttaaaaatggctagaaaaaattcatcaaaatgcagcactttaatcaattatttacaatttctatgttacaatgaaaaaatgtacatcttatagaacatatttcataaaactgctccactggaaacaactagatcaaaacagcaaaccttccatttaatatccacaaagttggattatttttcctttttgaagtagattcgccacaatcaaatttgaatacagagaattttgaagtttaagcatcaaacaacaaagtaaaagtccccaagatacaacaaagatctaggcaagtcttgttcctgtcccactcccaccccacccctaatgaaacttaaaaggtattcccatttcaattatggcctgtatcattcttggcagtttgggaagagaacttttggcttccattggtaactcaacataaatgttgcatagaatttatatatttcaaaattggcctaactgtagaaaaggcaaaatggaagcatttccgatagagccctaaatgagtacaaagtcactttgtaaaaggtgagtgacactaaagtaaaaatatgaccaaaataagaaatgtgcatattagacaaccctgcttcccgaaactttaggaaggacacggagttgtgagtcacacaagggctatgctacttgaagtcaatgttcaccaatcaggcagcactaggtacagaagtcttggttctgaacctggacccaggagggaagtctgtgggaaaggggagaagagaatgacaagagaggatgtcatattaaaaaaaggtttcaaacaatattggcaggtgtctactcacaaggtgattggaaaactgcccacgaggagaagtcaactttacctcctcccaaattcacagtacgcgagtgtagtagggtcattgctgggagataaattgtctgaggagggccacccttcaggtttaccagaaatcttagggtttggcccccctggtcacaggctaaatatatggtttaaaagttttattaaaaagaaaaacagaacaagacacactcacacccagatgactaatgaaggctaagcagaatagtctgagtttgctgagactaaagcagggatagtgttgaaaagttttcctttcactagtgggacacattccccttttcttttcaaagaggaagaacatggtgtcatccaatgtgaagtgagcagtttcgggtcaaactcttatggtaagaaactaaaaaaagatgccaagagacaaaccttcagaaatagaagaaatgcaaaagatggaataaaaaccctgatcattaaaacagagacaccttcactggtgtccaataaggattctctttacaaaacagaaacaaacaactcaaaaatttaccatactttgtaatgaaaataccagtatgttgaagacacagcagactgggtttctattagaacaagtatcagcaaggtcatgtagacttgtagaaacttttgccttctcctgcaccagacagatcattgtccagttgggttgtcagctggagaccgaaaagaacctaaaaaatggatctttttttttttctttttcccatggtcacgcatccacacaaatgagtcttttggatgagaaaagtcacagcaacttgagttctcctaatgaacagatgactttttagccctgtttgtttcaatggggaaaacaatgacaaaaaaaacaaaccccaggcaggcacgacacttatgtaaaatgaacacagttagtacaaaaccagtaaggcatcactttgggaaggtcagcaccgaagaggtcaggcaaggctcgtccagacggggcttctgggagggagtgaccctcacccttattgagctgcgtcatgttggttctgaggaaagtgcaagtcttttgcagggtgaccgcatcaccccaccggaagctggggcggggacgctggaggtgttggtgtgtgttctaaaccctcaaggacgagaagggaaggcaaggtccatggctcacccacatgtcgaggaccaggtcctcatccattttaaaggacacagatacccccagccctagcaggaggaggcgagtgtgtaggactgtgaggatggacaactaaaaaccaaaactgagcaggaccaaaccaaaactcaactcctgcggttcttactttcaccaaaggattgattctgaccaagaggggaagggggaaaaaaaaatcttcaaaaatcaatgcatcagaaaggaagaaactcaacctcattttcaaaaggtaacctgttctccaaagtagaacaagtctcactatacacagtgtttgcagaaaaaaaaaaaaaaaaacctgattcattcatatatcagaaggaaagagacacatgctgttctgcactgacagccacatccactcgctcacactctcactccgtcactcactctcacggatattaatcagaggctgatggacctgaatggggtggtttgattggaacaggcaaaatacctctcgggtaaggaaagcaccatttaaaaaacatgaaagcacggtttatttgctcctaaggtttccctgtgtcgtagctctgtagtgcgttgaacgtgaccaaagcaagcaccctggttagcaccagttctccctgtggccggctgtgtgggagggtgggtggcacggctctgagacccagtctggagggtctgtgctgaggggaagccgtgcttctctgtgtttccgactttgctccagtctcttctgtctctgggaagctcatggcaggatgctgtttggtttcagagcttcatgtgggttctctttttttttttctctctgtctctcttttcatttcaacggcgatgatcctttcccgagaagtatcttcagtgtcttagggaggtcacagcaacaaggcaaaacaataattaaagtacaacagaaggtagtgcagttctcgctgtggaaggaagcggtccgcaggcagctggcccgggatgcctgcacccaggtcgaggctgaaggacggggggtctcggtgttcccgcagctctaaggctgtggctgggggctggctcaggaagtcatcttcagggtgatgtgggggatgcaggtggaatgcggtgaggagaagaggagggcgctgggctccgggcccctgtcacagagtggactccaaagaggagtccaagatgtcatcgtgatggctgttgctgttggagtcgctgtcatagctctgggggctggagtagttggctgcctcctgcagcctcatcagcatgttcatcagcgggtcaccttcagcatcactggggggcatctgcttgcttgtcgatccctcccgaggcatggagtagccgtcgaagccgacatcctcaggccgtaactgcagcaggggaggccactcgtgctgttgtgggctggctgcccatggatatgtgtccatcacccacttggcaggatcctcccagggggcgcgccttccatagagctggagtccttctctgacggcttccaggagataggggataatggaatagttccacaagtcggtgaaccacactctcgagccgtccacatcgatggggcatgacaggaagagccgggggccgatggtgacgtccgaggaactgtgagcctccaggaagcggttgaggtgatgccagaccttgggaatccagtcaatgatttttaccagctccatattgcgcacccgcccactgatctctgtttccatgagcttcctcctcaggaatcggccaaggaaacccttcacaggctccgtgtggttggcacaaagcacccatctgaagttatggtgaagctgcaggttgggagtcgaagaggtagcctggttcattgtgccaattatgtaagggcatttgtggtacttgcagttgagcagcccattgaagatctctcccagagagctcacgtggtgtaggttgtccaggatgatgacgaggggcatgtccacagcattgttctcactgttgcactggtcagcaaggttggacaggtactggcgcaattccttgctggacttatggtccacgttaaaggtggcgataaccccgtctgtcaactcccgtccctctcgaagcactatatactcagacagccggttggccaggtaggttttcccagtgccgctggggccagagagaatgatccgacggtgctctatcaggagggagacgtagcgctgcaggatgggcttgggaatcaaggactcaaacaccagtgagtccaggctgttttctgcgagccctttcacagtcactgagatggtcgtgttctctccaaccagatagccacaaggaagcagctccggtgtttcggaagtgttgctgcgcttgatttctccaatgctgtagccaagaacgctgtctgaattcagccctagctgactcactgggtcgacatgaatgatgtattctttgaacagccgtctaaccaccccatcgagcacatcccacttcgtcttgccactaactccaatgcagccaataagaaagagatgtggtctggaatcctccttccacttcatttcctcctgaaagctgacaactatcttaacatgcctgcctccttccttccgagccgagcattcaccagtgtcatccagcaacatgtccaggctggttgactcagtgaggttcaagctgtgctgggagaggcccatggactgcctcggggaggcagagatggacacttgggaaggagcccggctgcagccactgccttgagactctgacttcagccgatcattctcagctttcagcttctctatttcactctgcatcctgttcatggcctcccggagctggtccagctggtgggcagaactgagagcttctaagcggatatccgtcagcttcatctccttgtctcttaactcatttcggagctgcatgacggtctcagcttcactatccatgcattctgaaattagagagttggagtgagaattcctcagcagtggggtggaacctgtggacccattgtgcggtaactttggtgaggaaggcaaagaagaatccgtcatctcctcaatatctgaatgagaggacgcagattttggggacttcttcttcccgaaagcttgcttgaaggagctgcgtaactcattgacccagttcttccgcttcttcttctttgagtcactctctatgttgctgcccacgctggagtggctggtggcactgttgatgctggagacgctgtctgaggagtgctgcctgcggatgcggaggtctgcagactgggcagtgccgtttcctttgcagttgagctcaggtgtgttaattactccattaatggcagcctgggcagctgcgttctgtttctttagcagctcaatggtttttcttaactcattcagttctgagtccttctgctcagctgtcatggtcagactctggagcctgattgtcatgttaccaagactctgttcaaaggctgccacaaggtgagcatttgctgtcagctgggtggtcaaagctgaaactttctcctgggaggcatccagttcccgccgcagcttgcgaatctctgactggcatttttcttctggtgtagaataaactgacgatgtgctggaaaccaaggagagtgaggatccatgaacttcttcaaacccatcccggaatgagcctgaacggctcatggttctgctcttctcatccagggacatggagctattccggaagcggctgtcagtgtatggatcatactgcccatcagcattggagaggctgtgagtcctcagcatggtcgggttggacaagctcatctgggtgacagtggtgggactcgcaagctgggaaaagttgaatcttgttccggagggagaagtcacgctggagccagaggaaaagggggaattggcagcggtgtcctgaaggcctcctgcagaatgggaccgtaaccattcttttgcatcttcttgcgtgcgaagctgggaggtgggagtatacctttctgacagtgtggtcttcacactgttagttctgacaaagggagtcaaggagtcgtccttggaggaggcgatgaggccagtggaagaattgtggctggggacccctccactgctgagggagatgtcgatggactcacagctggtgtggaggctgctgacagactgaaagcccaggccatccttgctaactgcggaggagctgctggcgttggtgccccaggtgaggctgttggaaggggccgagtgggctgagctggggctggaggctagcggagactggttgaggtccacattcttgctgtagagaggactgctgctcccactgctcaggacgccactgcctgacggggagtctaggttaccttgctgagtcatggtggcatgaggattggagatgaccaccgaatttttcatgttttcagctgtggcgatgggcacttgcttggtaggcttcccaccaaagagtctgcggagtgtgggagaggccacatctgggtacttggctccaggctggagactggtctgagccggactggacacaggctgggctgccggattcactttcaccgagttacaggaagccacactctcgttgtctgatgagatgcctttctccttgtctgtttggttgaccagacctggtagagagctgcctagggctgttttggaaggctccctcagtttgggcactggcaggcctgcggacttgctgctaatgttggaatctatgctgctggtgctagacctgttcccagccccgttccggctgttggacttactgggcctcggcaaactccggtactgaaggtttgtccgggagcttagggctagatacccgtcatcctgattctgagccccatccatacttgacttccgaccagcagaccgactgacgagtgcagatgactttgggattttgcccagtgtggctgacctgctggtgacagtcaccccgctggctgtgatcatggccaggccggcggcggaaccactctgcttcttgaacccaaagctgttggcattggcagtaggtgtcctagagctgctggggaggggctttttggattcgtcaccactgctccggcctgcatctgatggggagcgcttcacctgggaggctttaggagaaagccttcctttctcagacacctttgcgtcgtctgtttttccagttcctggggtcttcagtgcgcctgccggggctgaaggcttcgtccttggcatggtgatgcccacctgagctgtcatgcctcgccgccatgagcctgtctgggagatgacaggattcttcttgcccgacgtgcttttgtcggactcgtcagacacatcagaaggattccgcctccacttggaacctggctccatttttatgccgctgtctgagcctccgtctgatttcttgacatcatcaccagaccacagggaattcctctccacctgtgagtgcttctcagcatcagtctgcacatccaggttttttcgagaggaggcaggtgtgttggcataagagctgatggaggagctggtgttgatgtcatcagtgctgaggttgtctatggtgtcgctgatgccgctgctgacggagctgctgtcgtcccagctgtcagcgtctccgaggcccagggaggtatttcgttgcagggtctcccgtaccacagccatcccatcagggagccggttcaggcgacgggtatagaggccaagtccaccatcagtcatgtatccgcttgtaatgtcatcggtccggatgttcttgctcagaacatccccgtcgctcatgtagccgggggcatccatgctgatgccttccaggtccatctcatctcctgccttgtctgagacgtccacatggcagacactactgccccgggaggccagctgccttctcagaggggcggagtacacatagcgacctgactcagtgttgatgaacctgctggcgttggctcgagggggatacccattgcccattgagggggcgtctcctgcttggagccgagggctggactggcccagtctccaggacagaggtgtgggcctccctgtcaagctgagtatgctacggccactcatctccgtggtgacattggtgtcaaacgtggtttccaatgtgctgtgtgtaacctgagttccccttaaactggacatggtttcctccaaattctgccgcagatcagcgatgttcttcactgtccgcagccgccgagcctcaggatcttccccagtgagttcttccagagcaggctgtccagtcttggtgaagtggctgggctccacgctcacacctgttgagcttgactcggcagtaacattcccttcagtgtccgtctgagacctgtacaggaaaggtgcaaccgtggcagtgttgggatggttgtattgctgctggggctgaggtagctgaacactgacggtattgcttcctgtggtctgggtggtcccgacagacccactgacagtctggctgctgatgctgtggttcagggtggtccctcctgggccttttccttctgaggacgccaggctggaagaggaactggagtgtctgccgtccagctggggcttctgctgggggagtcctgagctcagcttcccactccggctccgctccccttccttggaaggcgctggggcacttggggatttcccgggcatgcttttcattcctggttttggtattccactgtgggaaggggccatgggctccttcttggcactgttgagcttcccccctttggggatgaagctggcaatcttggaggacttttttggcatctcgggcacagctgctccactggggtcttcttttggctcctccttgaggtccagcctctccgtcacagaggctctcttggcaaggtccttgcttttctccttatccttctcccgctgttgtttctccttctctttctcattgcctttcagagaactcttcttgttggtcagtgcccggctaaaagtcctctgggcaatgcccttgagtgcaatcttggggctgctggaagcagggcccacggtggtgagcatgcgactggcggcctccagctcctcgctctcttcgaagctgggcagagtctccagccgctcacagcttgtgtcccgggaccccggcccctcacctgcctttgagccccctttactgttgaaaagtttcagcttttccagcatggacttctgattgttgggggccggcttcatggcttcaggtgtgggcctgggggcctcaggcccaggaggcttgaccgagagcatggataccgtggcactgtgcttcacgctgagggatttgctgcgccaaggcttggtggctgcaccgggctgcgggatggccgaggaggtactgcaattagtaggggtggagctgctgccgctctccaaggaagcaggtgcattgtcactcattccggggtgggaggaggctgaacttgccaaaggctctttctcgtggctgcttggcggtgggggtggggaggtgactggtttggatttatcatagttgttaaagctctggctgcgtcggttgttagcagtagttgaccctccgcgtgttttggcctcgctgcctgcagcggataccctcgcggtaggacctggaagtctagagatctttttctgacccagagtgaagcggatgattttgctttgagatgagtccttggatgatgcactggactgcatttcagcttgtgcttttgactgctgatgtggcgctggctggtgaggctggcacggggcttggggagtgactggcacctgctgctgaggggtgccagcctggcactgggagggggccccggccacctgggatacggcgggcggcagaggtgaggagaggtgctgcttctggggctgctgctgctgctgcttgtatcgggagaggctgaagaagaggcctagaatggccttgaggtttccattcctgatctcttctgcagacagcccctggatgtttattcccttagctgccaggaaattcaagcaggcatctatgttttcaatcatttgggatctgttcttcggacagccattgatgtcttcaatcttttcatttgccacaacctggataatctgggccaggaggacgccatctgtcacatcttgctggagatccctgatgagacgcttgtggccggatttggctaggtaatgattggcccagtctgtgtagatctgggtatcgaacccgttttccaccgagccgctcttccgcagcgggagcccctcccccgctggctcctgcagcccctgcagcacctgcgatttcagggggatctggctaggataggtggtcttgctcacctccaccttgcttcccaacttcaggtagcagggctgggggcccgcccgggccgggggcacgtgcaggatgggcgcggcgctgtgcacgggtttgggcagtcccgacttcattttggaggcgaccaggatggccggcatcttctcccggggcttgggctttcccagcacgtccctggcagcggcggcgggggcgaccgctaaaggcagcgcgggtagcagagcaggcgccgggccttagcccacgaggcgcccaccaccagcggctaaaaaaaaaatccccaggtcggggaactcgaagcaatcgggcgagcgcgcctttggggtgccgggatgggaatgggggactggccacggcgctcagcgggtcccacctggacggatgctgccgccgggtctcacacctctcctgggtggcctttcaagagctctgggcgctcaggggctgccgcctcttgcaaatttcctcctgggaaacagaggcttggacgcccatattaacttgtcactgcatctccgaagtgaggaggcccctttggaagagacagaggcggcggcgacccacgagtcccgttccggaggctacgggtctgagccggcgagagaaagagcgagcagccaaggaaggaaaggagacagcagcgaaggaaggagagaagaagggcgcaagggtcccaagacgtctccaccgagaggcagctgccaccctgctcgcgagcaccgcagtgtcacccgcgacgcagcagaggtgcggcaagagcccccgaaaggtctctcttggggtgacagtcaccgctgcccagaaggcccccggactgagagcaccttagcgcctgcgggtctgcacatgctccgtgagctagatagaggcaaggctgtggccgtggggcgcgggcgccgggacgcgcggctggcgggccgggcagggctgcgctcgggagcggccgccgcgcttcccgggaaggctgcgctggctgcggggctcagcgcaggggag

SEQ ID NO: 17904 - RNA, 12319 nt, Homo sapiens
  source 1..12319: mol_type = other RNA
tcggcctggggaggaggaaggggagggaggatggaaacataccgtacacaaaatactcaattcctagttttctctttaaaaatggctagaaaaaattcatcaaaatgcagcactttaatcaattatttacaatttctatgttacaatgaaaaaatgtacatcttatagaacatatttcataaaactgctccactggaaacaactagatcaaaacagcaaaccttccatttaatatccacaaagttggattatttttcctttttgaagtagattcgccacaatcaaatttgaatacagagaattttgaagtttaagcatcaaacaacaaagtaaaagtccccaagatacaacaaagatctaggcaagtcttgttcctgtcccactcccaccccacccctaatgaaacttaaaaggtattcccatttcaattatggcctgtatcattcttggcagtttgggaagagaacttttggcttccattggtaactcaacataaatgttgcatagaatttatatatttcaaaattggcctaactgtagaaaaggcaaaatggaagcatttccgatagagccctaaatgagtacaaagtcactttgtaaaaggtgagtgacactaaagtaaaaatatgaccaaaataagaaatgtgcatattagacaaccctgcttcccgaaactttaggaaggacacggagttgtgagtcacacaagggctatgctacttgaagtcaatgttcaccaatcaggcagcactaggtacagaagtcttggttctgaacctggacccaggagggaagtctgtgggaaaggggagaagagaatgacaagagaggatgtcatattaaaaaaaggtttcaaacaatattggcaggtgtctactcacaaggtgattggaaaactgcccacgaggagaagtcaactttacctcctcccaaattcacagtacgcgagtgtagtagggtcattgctgggagataaattgtctgaggagggccacccttcaggtttaccagaaatcttagggtttggcccccctggtcacaggctaaatatatggtttaaaagttttattaaaaagaaaaacagaacaagacacactcacacccagatgactaatgaaggctaagcagaatagtctgagtttgctgagactaaagcagggatagtgttgaaaagttttcctttcactagtgggacacattccccttttcttttcaaagaggaagaacatggtgtcatccaatgtgaagtgagcagtttcgggtcaaactcttatggtaagaaactaaaaaaagatgccaagagacaaaccttcagaaatagaagaaatgcaaaagatggaataaaaaccctgatcattaaaacagagacaccttcactggtgtccaataaggattctctttacaaaacagaaacaaacaactcaaaaatttaccatactttgtaatgaaaataccagtatgttgaagacacagcagactgggtttctattagaacaagtatcagcaaggtcatgtagacttgtagaaacttttgccttctcctgcaccagacagatcattgtccagttgggttgtcagctggagaccgaaaagaacctaaaaaatggatctttttttttttctttttcccatggtcacgcatccacacaaatgagtcttttggatgagaaaagtcacagcaacttgagttctcctaatgaacagatgactttttagccctgtttgtttcaatggggaaaacaatgacaaaaaaaacaaaccccaggcaggcacgacacttatgtaaaatgaacacagttagtacaaaaccagtaaggcatcactttgggaaggtcagcaccgaagaggtcaggcaaggctcgtccagacggggcttctgggagggagtgaccctcacccttattgagctgcgtcatgttggttctgaggaaagtgcaagtcttttgcagggtgaccgcatcaccccaccggaagctggggcggggacgctggaggtgttggtgtgtgttctaaaccctcaaggacgagaagggaaggcaaggtccatggctcacccacatgtcgaggaccaggtcctcatccattttaaaggacacagatacccccagccctagcaggaggaggcgagtgtgtaggactgtgaggatggacaactaaaaaccaaaactgagcaggaccaaaccaaaactcaactcctgcggttcttactttcaccaaaggattgattctgaccaagaggggaagggggaaaaaaaaatcttcaaaaatcaatgcatcagaaaggaagaaactcaacctcattttcaaaaggtaacctgttctccaaagtagaacaagtctcactatacacagtgtttgcagaaaaaaaaaaaaaaaaacctgattcattcatatatcagaaggaaagagacacatgctgttctgcactgacagccacatccactcgctcacactctcactccgtcactcactctcacggatattaatcagaggctgatggacctgaatggggtggtttgattggaacaggcaaaatacctctcgggtaaggaaagcaccatttaaaaaacatgaaagcacggtttatttgctcctaaggtttccctgtgtcgtagctctgtagtgcgttgaacgtgaccaaagcaagcaccctggttagcaccagttctccctgtggccggctgtgtgggagggtgggtggcacggctctgagacccagtctggagggtctgtgctgaggggaagccgtgcttctctgtgtttccgactttgctccagtctcttctgtctctgggaagctcatggcaggatgctgtttggtttcagagcttcatgtgggttctctttttttttttctctctgtctctcttttcatttcaacggcgatgatcctttcccgagaagtatcttcagtgtcttagggaggtcacagcaacaaggcaaaacaataattaaagtacaacagaaggtagtgcagttctcgctgtggaaggaagcggtccgcaggcagctggcccgggatgcctgcacccaggtcgaggctgaaggacggggggtctcggtgttcccgcagctctaaggctgtggctgggggctggctcaggaagtcatcttcagggtgatgtgggggatgcaggtggaatgcggtgaggagaagaggagggcgctgggctccgggcccctgtcacagagtggactccaaagaggagtccaagatgtcatcgtgatggctgttgctgttggagtcgctgtcatagctctgggggctggagtagttggctgcctcctgcagcctcatcagcatgttcatcagcgggtcaccttcagcatcactggggggcatctgcttgcttgtcgatccctcccgaggcatggagtagccgtcgaagccgacatcctcaggccgtaactgcagcaggggaggccactcgtgctgttgtgggctggctgcccatggatatgtgtccatcacccacttggcaggatcctcccagggggcgcgccttccatagagctggagtccttctctgacggcttccaggagataggggataatggaatagttccacaagtcggtgaaccacactctcgagccgtccacatcgatggggcatgacaggaagagccgggggccgatggtgacgtccgaggaactgtgagcctccaggaagcggttgaggtgatgccagaccttgggaatccagtcaatgatttttaccagctccatattgcgcacccgcccactgatctctgtttccatgagcttcctcctcaggaatcggccaaggaaacccttcacaggctccgtgtggttggcacaaagcacccatctgaagttatggtgaagctgcaggttgggagtcgaagaggtagcctggttcattgtgccaattatgtaagggcatttgtggtacttgcagttgagcagcccattgaagatctctcccagagagctcacgtggtgtaggttgtccaggatgatgacgaggggcatgtccacagcattgttctcactgttgcactggtcagcaaggttggacaggtactggcgcaattccttgctggacttatggtccacgttaaaggtggcgataaccccgtctgtcaactcccgtccctctcgaagcactatatactcagacagccggttggccaggtaggttttcccagtgccgctggggccagagagaatgatccgacggtgctctatcaggagggagacgtagcgctgcaggatgggcttgggaatcaaggactcaaacaccagtgagtccaggctgttttctgcgagccctttcacagtcactgagatggtcgtgttctctccaaccagatagccacaaggaagcagctccggtgtttcggaagtgttgctgcgcttgatttctccaatgctgtagccaagaacgctgtctgaattcagccctagctgactcactgggtcgacatgaatgatgtattctttgaacagccgtctaaccaccccatcgagcacatcccacttcgtcttgccactaactccaatgcagccaataagaaagagatgtggtctggaatcctccttccacttcatttcctcctgaaagctgacaactatcttaacatgcctgcctccttccttccgagccgagcattcaccagtgtcatccagcaacatgtccaggctggttgactcagtgaggttcaagctgtgctgggagaggcccatggactgcctcggggaggcagagatggacacttgggaaggagcccggctgcagccactgccttgagactctgacttcagccgatcattctcagctttcagcttctctatttcactctgcatcctgttcatggcctcccggagctggtccagctggtgggcagaactgagagcttctaagcggatatccgtcagcttcatctccttgtctcttaactcatttcggagctgcatgacggtctcagcttcactatccatgcattctgaaattagagagttggagtgagaattcctcagcagtggggtggaacctgtggacccattgtgcggtaactttggtgaggaaggcaaagaagaatccgtcatctcctcaatatctgaatgagaggacgcagattttggggacttcttcttcccgaaagcttgcttgaaggagctgcgtaactcattgacccagttcttccgcttcttcttctttgagtcactctctatgttgctgcccacgctggagtggctggtggcactgttgatgctggagacgctgtctgaggagtgctgcctgcggatgcggaggtctgcagactgggcagtgccgtttcctttgcagttgagctcaggtgtgttaattactccattaatggcagcctgggcagctgcgttctgtttctttagcagctcaatggtttttcttaactcattcagttctgagtccttctgctcagctgtcatggtcagactctggagcctgattgtcatgttaccaagactctgttcaaaggctgccacaaggtgagcatttgctgtcagctgggtggtcaaagctgaaactttctcctgggaggcatccagttcccgccgcagcttgcgaatctctgactggcatttttcttctggtgtagaataaactgacgatgtgctggaaaccaaggagagtgaggatccatgaacttcttcaaacccatcccggaatgagcctgaacggctcatggttctgctcttctcatccagggacatggagctattccggaagcggctgtcagtgtatggatcatactgcccatcagcattggagaggctgtgagtcctcagcatggtcgggttggacaagctcatctgggtgacagtggtgggactcgcaagctgggaaaagttgaatcttgttccggagggagaagtcacgctggagccagaggaaaagggggaattggcagcggtgtcctgaaggcctcctgcagaatgggaccgtaaccattcttttgcatcttcttgcgtgcgaagctgggaggtgggagtatacctttctgacagtgtggtcttcacactgttagttctgacaaagggagtcaaggagtcgtccttggaggaggcgatgaggccagtggaagaattgtggctggggacccctccactgctgagggagatgtcgatggactcacagctggtgtggaggctgctgacagactgaaagcccaggccatccttgctaactgcggaggagctgctggcgttggtgccccaggtgaggctgttggaaggggccgagtgggctgagctggggctggaggctagcggagactggttgaggtccacattcttgctgtagagaggactgctgctcccactgctcaggacgccactgcctgacggggagtctaggttaccttgctgagtcatggtggcatgaggattggagatgaccaccgaatttttcatgttttcagctgtggcgatgggcacttgcttggtaggcttcccaccaaagagtctgcggagtgtgggagaggccacatctgggtacttggctccaggctggagactggtctgagccggactggacacaggctgggctgccggattcactttcaccgagttacaggaagccacactctcgttgtctgatgagatgcctttctccttgtctgtttggttgaccagacctggtagagagctgcctagggctgttttggaaggctccctcagtttgggcactggcaggcctgcggacttgctgctaatgttggaatctatgctgctggtgctagacctgttcccagccccgttccggctgttggacttactgggcctcggcaaactccggtactgaaggtttgtccgggagcttagggctagatacccgtcatcctgattctgagccccatccatacttgacttccgaccagcagaccgactgacgagtgcagatgactttgggattttgcccagtgtggctgacctgctggtgacagtcaccccgctggctgtgatcatggccaggccggcggcggaaccactctgcttcttgaacccaaagctgttggcattggcagtaggtgtcctagagctgctggggaggggctttttggattcgtcaccactgctccggcctgcatctgatggggagcgcttcacctgggaggctttaggagaaagccttcctttctcagacacctttgcgtcgtctgtttttccagttcctggggtcttcagtgcgcctgccggggctgaaggcttcgtccttggcatggtgatgcccacctgagctgtcatgcctcgccgccatgagcctgtctgggagatgacaggattcttcttgcccgacgtgcttttgtcggactcgtcagacacatcagaaggattccgcctccacttggaacctggctccatttttatgccgctgtctgagcctccgtctgatttcttgacatcatcaccagaccacagggaattcctctccacctgtgagtgcttctcagcatcagtctgcacatccaggttttttcgagaggaggcaggtgtgttggcataagagctgatggaggagctggtgttgatgtcatcagtgctgaggttgtctatggtgtcgctgatgccgctgctgacggagctgctgtcgtcccagcttgtaaggttcctaggccagagcatttcactacattgcggcccttggagaacagcggacaaagaagctgaatgaatctcacaggatggcaagtcctttagccagctgagccagcccacactgggccagggaatcccaggcacccagcaactctgtaactaaaggactagctagcagggatcaccattccccaggccaggaaagaaatccgatcccccaacaaaattaacctctgaagtgctgaaggatcgagaggtcaggcctcagtgctggtatcaagtcagctgtgaaaagtttcagcaaagcaaaagctaacaccaaactctgaaaccattaccgtaaagcactgaatggaagggccctccatgtggtcccaggggagtttgcaacagcgggtcaaattgaagaaaatctaagaatgaaaaactactttaaatcctcacagactgcacagaaacattgcagaaagtctttccagccctaagtgctacttttaatgatgcaaaaatcattgactataacatttcttagctcattccattgacgtctgaaggcaaagcattcgattgaaaagattagcctacagagagaatttctgaacctaaaaaggaaatgatacctgtttgtacagttaacaacgacacacatacattatttccggtgatgtcaattttgatgcagtgccaacaaaaatatgcattaattccgcaggctacttatttcaaaagaaaaagaatctcagtctaggcatggctacattaaacattatggtacagaggctggaaggggaggtgggtgggagagagtcccagctctgggatgggaaggggttgcatggactaatccctattaaaacctgtaatcaaggcactcagaaagaactatgtaaacagatgctatgaacaatgaacaactgtattactactgagaactcaaaagcaaacttatgttatagccacaagctttatttgaaaacgaaggattaagatgttctccaaaaccctgactccctctccaaaaatcctaccagttggttcctggtagctttcaaagactttccccaagaaaggctctccccctggccagggtggcctctccagtggaagcagggagcgggggttgtggccctgggggatggttagggaaggaagcagtaactggctccaagcgaggtctctgtgtggtcagcatttgctcagcaaacagaagctttcaaaggggaatgaagagccattcctctcccactgaaaagggagggaataaaagatctgctcaaagaggagaggagggtctggtggtgattcccaggtgaatgaaaaaaagattgtaatctcgaaggagtcccaaccaaagttaatcattcacatctcatccttcagggccctcgtccacttgaaatactgctgaggcatctgccgtggggagtgggaagcagaggtgggggtgggcagtgggtgagtttgagggaaggagtagtgtccagatatattaagacaaaaaagttgggacagacccaagttctggctgacaaggatgcttcaaaccaccccttaccttctatgctgtccctggaactgactgtatctttacgatattacttctttgagaatctgtccaacatccgagttaacttgggaatgggatggtgattgtgtgtatggagacacacaggcacatgggcacagatgcacacacacgctctaaaaagtttccattgtttcctcgctctaggcaaacataataggtaaacattctgatttgtcatcaaggtaagctaggaaatgttgatgtattcatttattcattcatcaactaccatatttataaagcatctgcaatgtggcaagtgctgttctaagtgcagaagatacaagcagtcaacaaaatagaccaaaaatctcaactctaatggaacttagcttcagtggtagaactataaaataaatgagacaaaatgtaaattttacagtacattagcaataaatgctcgggagaacaacgtattgtaaagaagaagatgtgatttgtcaaggtggggtgtgggaaattttacatgggctggctatggcaggtctgctgagggcatggtttttattacaaatctaaaagaagtatgggagctgggtatctgaatacctggggataagggactttcaagagaggaaatggtcagtgcaaaggccctgagatagtatacgacttgcaatgcattccaagaatgagtggctggagcagtgagcggtgaaccaaagtggggtgaggagggggtcaggccagagagtccaagggtacagcgagagaggagagtgcctaaatggggccctgcaagtcagcgtaagcagcttgtcttttactctgagggagagaggatacattggaggtttaatagatggagtttcttctttttataaaagttcatgtaaatgtacaacactaaacatatcgttttgattacacatgatttttacaggggtgagtttattgtaggagacatagtgctttaaggaggtcttagttttctttctatggttaaaagaatcacacctttcatgttagaggctctgaattatttgcagctacaggttctaattgagtcagggttttctcatggtttgaaagataataattagtagggataagggagacccaggcaacgagagaggaaaagggaaagtaaaccaactccatgagggcagatgccctttggcgcttttcaagagccaggattgctctgtcatttttgacgcttgcttctaaacaggccaaattccaaagggctcccagaactcataacacttttctccacagaaacaatgttatcagtgatgttaaggtttccaggttactcacagagccatctataaaaccaagatgtagttgatgaactctactcaggtatcaaagagtagaagaaaactttattcttggaatacagtacataattagacaaaacagaaaaccacaaatctaaaaagatgttcacttatttctaatgagtattttatgaaaacaatgctagtgaagacacttcgttccttttcttccaacatattcaaccctctttcctggcttttccctgcaggctgaaaaatatatcactaatctcatcaaatcaaacaaaaacttttttttttttttacctcatgcccatattctcctccactcctttgaggtgttttcctgtacttctcatgttccgtgatccttcaacccaccaggcaagatgtttgttcccactactccactgagaccactttctcttttccctgagaacatcaatggcttcctccttgccaaagccaatggtcaactctctgtccttaccctacttgagttttcagcagcaggtagcatcgacagattctcccttcttgagtgggcctcatcccgggtttccatactgtcatctgtacctggttcctacctccctaactgcgcttctcaatctcctaggctcaccctcctcttcacctctccagaactccagggcctccatccctggacccctcctcttctctaactataacttctcactaacttctaactaagttataactaccacttctaactaacttcttttcctgggtgatctcatccatggcttcaaatactaggtgaaggcagacaactctaaagtctgtaatctctagcctggcccctttgtgtacccaacacatctgaaatcaaatttaccttactcaaaactattgctcccaacttccaatgtgtccgcacccccactcccaaagtcttctgtatctcagaatatgactctacattaacagtcctaattctctccctccttcttgcctccgatgtaatccattaagaaggccttttgcctagagtccccaaatataccttgaacccaatcactactgaacatctgcaataagataaccttggaccaagatgccatcatctctttcctgcaacagacacctcccgggtcgctcagccttccctcatgccttgctaggctccatcctgcacaccccaggggcagcaatctttctccagtgtacagcagattctgtcacattcctgcttaaagcccactgatagcttcccagggaacttagaataaaattcaaatttgttcccttggcctagaagccctgatgtgatctggcttctcctcttcattacgtccaaagacaggacccacaaatgcaccaagcttcttcccacttcctaggccctcgcactgtgcctcctttctggaatgctcctccccatgtctcccactggcggcccacttctcacgggtcagatgttggttggaatggcacctcctcagggatttcctcttagactctggcccaattacattccaccatatgattttcttcatggcatcaaccagtcaacacattgtctttcaacagtctgtctttccctcaacacagggagctcctcgagcacaggtgtactgtttgcctttgttctgagccatatcctcccagtgcctaaatcactgctgatgtggtcctggatcaaccaagcataggaggacaaaatggaactgattattccatgcagtctcctggggactgtgtagtacttccaaggactttagttcaatggttttatttggtcacagacccacttaggggcccgtctctccataagaaaaaagatacacaaacaatattttacacagaatttccagggactcactgatcccctgaatcctgtccataaagcccaggtta

SEQ ID NO: 17905 - RNA, 7752 nt, Homo sapiens
  source 1..7752: mol_type = other RNA
tcggcctggggaggaggaaggggagggaggatggaaacataccgtacacaaaatactcaattcctagttttctctttaaaaatggctagaaaaaattcatcaaaatgcagcactttaatcaattatttacaatttctatgttacaatgaaaaaatgtacatcttatagaacatatttcataaaactgctccactggaaacaactagatcaaaacagcaaaccttccatttaatatccacaaagttggattatttttcctttttgaagtagattcgccacaatcaaatttgaatacagagaattttgaagtttaagcatcaaacaacaaagtaaaagtccccaagatacaacaaagatctaggcaagtcttgttcctgtcccactcccaccccacccctaatgaaacttaaaaggtattcccatttcaattatggcctgtatcattcttggcagtttgggaagagaacttttggcttccattggtaactcaacataaatgttgcatagaatttatatatttcaaaattggcctaactgtagaaaaggcaaaatggaagcatttccgatagagccctaaatgagtacaaagtcactttgtaaaaggtgagtgacactaaagtaaaaatatgaccaaaataagaaatgtgcatattagacaaccctgcttcccgaaactttaggaaggacacggagttgtgagtcacacaagggctatgctacttgaagtcaatgttcaccaatcaggcagcactaggtacagaagtcttggttctgaacctggacccaggagggaagtctgtgggaaaggggagaagagaatgacaagagaggatgtcatattaaaaaaaggtttcaaacaatattggcaggtgtctactcacaaggtgattggaaaactgcccacgaggagaagtcaactttacctcctcccaaattcacagtacgcgagtgtagtagggtcattgctgggagataaattgtctgaggagggccacccttcaggtttaccagaaatcttagggtttggcccccctggtcacaggctaaatatatggtttaaaagttttattaaaaagaaaaacagaacaagacacactcacacccagatgactaatgaaggctaagcagaatagtctgagtttgctgagactaaagcagggatagtgttgaaaagttttcctttcactagtgggacacattccccttttcttttcaaagaggaagaacatggtgtcatccaatgtgaagtgagcagtttcgggtcaaactcttatggtaagaaactaaaaaaagatgccaagagacaaaccttcagaaatagaagaaatgcaaaagatggaataaaaaccctgatcattaaaacagagacaccttcactggtgtccaataaggattctctttacaaaacagaaacaaacaactcaaaaatttaccatactttgtaatgaaaataccagtatgttgaagacacagcagactgggtttctattagaacaagtatcagcaaggtcatgtagacttgtagaaacttttgccttctcctgcaccagacagatcattgtccagttgggttgtcagctggagaccgaaaagaacctaaaaaatggatctttttttttttctttttcccatggtcacgcatccacacaaatgagtcttttggatgagaaaagtcacagcaacttgagttctcctaatgaacagatgactttttagccctgtttgtttcaatggggaaaacaatgacaaaaaaaacaaaccccaggcaggcacgacacttatgtaaaatgaacacagttagtacaaaaccagtaaggcatcactttgggaaggtcagcaccgaagaggtcaggcaaggctcgtccagacggggcttctgggagggagtgaccctcacccttattgagctgcgtcatgttggttctgaggaaagtgcaagtcttttgcagggtgaccgcatcaccccaccggaagctggggcggggacgctggaggtgttggtgtgtgttctaaaccctcaaggacgagaagggaaggcaaggtccatggctcacccacatgtcgaggaccaggtcctcatccattttaaaggacacagatacccccagccctagcaggaggaggcgagtgtgtaggactgtgaggatggacaactaaaaaccaaaactgagcaggaccaaaccaaaactcaactcctgcggttcttactttcaccaaaggattgattctgaccaagaggggaagggggaaaaaaaaatcttcaaaaatcaatgcatcagaaaggaagaaactcaacctcattttcaaaaggtaacctgttctccaaagtagaacaagtctcactatacacagtgtttgcagaaaaaaaaaaaaaaaaacctgattcattcatatatcagaaggaaagagacacatgctgttctgcactgacagccacatccactcgctcacactctcactccgtcactcactctcacggatattaatcagaggctgatggacctgaatggggtggtttgattggaacaggcaaaatacctctcgggtaaggaaagcaccatttaaaaaacatgaaagcacggtttatttgctcctaaggtttccctgtgtcgtagctctgtagtgcgttgaacgtgaccaaagcaagcaccctggttagcaccagttctccctgtggccggctgtgtgggagggtgggtggcacggctctgagacccagtctggagggtctgtgctgaggggaagccgtgcttctctgtgtttccgactttgctccagtctcttctgtctctgggaagctcatggcaggatgctgtttggtttcagagcttcatgtgggttctctttttttttttctctctgtctctcttttcatttcaacggcgatgatcctttcccgagaagtatcttcagtgtcttagggaggtcacagcaacaaggcaaaacaataattaaagtacaacagaaggtagtgcagttctcgctgtggaaggaagcggtccgcaggcagctggcccgggatgcctgcacccaggtcgaggctgaaggacggggggtctcggtgttcccgcagctctaaggctgtggctgggggctggctcaggaagtcatcttcagggtgatgtgggggatgcaggtggaatgcggtgaggagaagaggagggcgctgggctccgggcccctgtcacagagtggactccaaagaggagtccaagatgtcatcgtgatggctgttgctgttggagtcgctgtcatagctctgggggctggagtagttggctgcctcctgcagcctcatcagcatgttcatcagcgggtcaccttcagcatcactggggggcatctgcttgcttgtcgatccctcccgaggcatggagtagccgtcgaagccgacatcctcaggccgtaactgcagcaggggaggccactcgtgctgttgtgggctggctgcccatggatatgtgtccatcacccacttggcaggatcctcccagggggcgcgccttccatagagctggagtccttctctgacggcttccaggagataggggataatggaatagttccacaagtcggtgaaccacactctcgagccgtccacatcgatggggcatgacaggaagagccgggggccgatggtgacgtccgaggaactgtgagcctccaggaagcggttgaggtgatgccagaccttgggaatccagtcaatgatttttaccagctccatattgcgcacccgcccactgatctctgtttccatgagcttcctcctcaggaatcggccaaggaaacccttcacaggctccgtgtggttggcacaaagcacccatctgaagttatggtgaagctgcaggttgggagtcgaagaggtagcctggttcattgtgccaattatgtaagggcatttgtggtacttgcagttgagcagcccattgaagatctctcccagagagctcacgtggtgtaggttgtccaggatgatgacgaggggcatgtccacagcattgttctcactgttgcactggtcagcaaggttggacaggtactggcgcaattccttgctggacttatggtccacgttaaaggtggcgataaccccgtctgtcaactcccgtccctctcgaagcactatatactcagacagccggttggccaggtaggttttcccagtgccgctggggccagagagaatgatccgacggtgctctatcaggagggagacgtagcgctgcaggatgggcttgggaatcaaggactcaaacaccagtgagtccaggctgttttctgcgagccctttcacagtcactgagatggtcgtgttctctccaaccagatagccacaaggaagcagctccggtgtttcggaagtgttgctgcgcttgatttctccaatgctgtagccaagaacgctgtctgaattcagccctagctgactcactgggtcgacatgaatgatgtattctttgaacagccgtctaaccaccccatcgagcacatcccacttcgtcttgccactaactccaatgcagccaataagaaagagatgtggtctggaatcctccttccacttcatttcctcctgaaagctgacaactatcttaacatgcctgcctccttccttccgagccgagcattcaccagtgtcatccagcaacatgtccaggctggttgactcagtgaggttcaagctgtgctgggagaggcccatggactgcctcggggaggcagagatggacacttgggaaggagcccggctgcagccactgccttgagactctgacttcagccgatcattctcagctttcagcttctctatttcactctgcatcctgttcatggcctcccggagctggtccagctggtgggcagaactgagagcttctaagcggatatccgtcagcttcatctccttgtctcttaactcatttcggagctgcatgacggtctcagcttcactatccatgcattctgaaattagagagttggagtgagaattcctcagcagtggggtggaacctgtggacccattgtgcggtaactttggtgaggaaggcaaagaagaatccgtcatctcctcaatatctgaatgagaggacgcagattttggggacttcttcttcccgaaagcttgcttgaaggagctgcgtaactcattgacccagttcttccgcttcttcttctttgagtcactctctatgttgctgcccacgctggagtggctggtggcactgttgatgctggagacgctgtctgaggagtgctgcctgcggatgcggaggtctgcagactgggcagtgccgtttcctttgcagttgagctcaggtgtgttaattactccattaatggcagcctgggcagctgcgttctgtttctttagcagctcaatggtttttcttaactcattcagttctgagtccttctgctcagctgtcatggtcagactctggagcctgattgtcatgttaccaagactctgttcaaaggctgccacaaggtgagcatttgctgtcagctgggtggtcaaagctgaaactttctcctgggaggcatccagttcccgccgcagcttgcgaatctctgactggcatttttcttctggtgtagaataaactgacgatgtgctggaaaccaaggagagtgaggatccatgaacttcttcaaacccatcccggaatgagcctgaacggctcatggttctgctcttctcatccagggacatggagctattccggaagcggctgtcagtgtatggatcatactgcccatcagcattggagaggctgtgagtcctcagcatggtcgggttggacaagctcatctgggtgacagtggtgggactcgcaagctgggaaaagttgaatcttgttccggagggagaagtcacgctggagccagaggaaaagggggaattggcagcggtgtcctgaaggcctcctgcagaatgggaccgtaaccattcttttgcatcttcttgcgtgcgaagctgggaggtgggagtatacctttctgacagtgtggtcttcacactgttagttctgacaaagggagtcaaggagtcgtccttggaggaggcgatgaggccagtggaagaattgtggctggggacccctccactgctgagggagatgtcgatggactcacagctggtgtggaggctgctgacagactgaaagcccaggccatccttgctaactgcggaggagctgctggcgttggtgccccaggtgaggctgttggaaggggccgagtgggctgagctggggctggaggctagcggagactggttgaggtccacattcttgctgtagagaggactgctgctcccactgctcaggacgccactgcctgacggggagtctaggttaccttgctgagtcatggtggcatgaggattggagatgaccaccgaatttttcatgttttcagctgtggcgatgggcacttgcttggtaggcttcccaccaaagagtctgcggagtgtgggagaggccacatctgggtacttggctccaggctggagactggtctgagccggactggacacaggctgggctgccggattcactttcaccgagttacaggaagccacactctcgttgtctgatgagatgcctttctccttgtctgtttggttgaccagacctggtagagagctgcctagggctgttttggaaggctccctcagtttgggcactggcaggcctgcggacttgctgctaatgttggaatctatgctgctggtgctagacctgttcccagccccgttccggctgttggacttactgggcctcggcaaactccggtactgaaggtttgtccgggagcttagggctagatacccgtcatcctgattctgagccccatccatacttgacttccgaccagcagaccgactgacgagtgcagatgactttgggattttgcccagtgtggctgacctgctggtgacagtcaccccgctggctgtgatcatggccaggccggcggcggaaccactctgcttcttgaacccaaagctgttggcattggcagtaggtgtcctagagctgctggggaggggctttttggattcgtcaccactgctccggcctgcatctgatggggagcgcttcacctgggaggctttaggagaaagccttcctttctcagacacctttgcgtcgtctgtttttccagttcctggggtcttcagtgcgcctgccggggctgaaggcttcgtccttggcatggtgatgcccacctgagctgtcatgcctcgccgccatgagcctgtctgggagatgacaggattcttcttgcccgacgtgcttttgtcggactcgtcagacacatcagaaggattccgcctccacttggaacctggctccatttttatgccgctgtctgagcctccgtctgatttcttgacatcatcaccagaccacagggaattcctctccacctgtgagtgcttctcagcatcagtctgcacatccaggttttttcgagaggaggcaggtgtgttggcataagagctgatggaggagctggtgttgatgtcatcagtgctgaggttgtctatggtgtcgctgatgccgctgctgacggagctgctgtcgtcccagtaataaaaccacagccggtgagcagagatgaggttctctaactacggttctgaaaagcagtcttcacaaagcaaggatcctaatcctccccaaactccaaaggctgggtctgcttccaggaggcccttactgtccttggaaacagtct

SEQ ID NO: 17906 - RNA, 5806 nt, Homo sapiens
  source 1..5806: mol_type = other RNA
tcggctctctccctcaccctaggtggtgcccagagctcaaggatggagccaggcaggcatcaggcaatcctccttcctgaggttccctgcgtgcaacatgaaaaggacattcagatgggggcagagtggggaatcagcctcttgctaggaggctgcagggcttcccaaaggagaagaggcttgtccctgccaggccctgctcatctgatgcagcgccagggccttcccacctttacccaccctcaggaagcctcctaagatgcccagccacgtgcaccaaccccctttctgagctctttccaggctgtgctggcaccttggtctgactcttgtgagcagtgtctctgtgtggcctccctgtgcgtttcccaggatagcagagtacctgggaggcttcacggagtaggcagatgaggctctggctggggccatgcccagctttttgtccctcctctgccctgtgttacctggggcaattatttcctctttctgagccttgacttccccagcagggaagtggaacttggtcttttgccaagactccccctgcccacctctcattctcttttgctctggagaccacacagttatctccctcttcccactccagcccccttagtgatgaaggttccatgtcacggcacgggcaaggggtggtcctggctactccccgcccagctcccagccaaggctgcagctcctcccataaagtgggagaaggttgcccagccccacaggcttctgctgggtggccctgaacacatcgcctcccttctctgagcctcaggctcctcatctgagaaacgggtccctgccatgtctggactctctggctgggccggagagtctggctttccttctaggagacacccctcaaggcaggccctgcatcttgttcatctgcgagccacacccagtccggggctgggcagagtgggcactggtgtctgggagcctgtgggcagcaaggcacagcatagagcaaggggcccctagccacggctgacagggcgcctccagcataagggactctctgaggtcccttctggctttaacagtctgtgggtcacaagcatgctgtccctagaccagctcctggcatggggtcccggctggattcgggggtttgtgaggccccagaatgggaatatgtgaccccaacagctggcaagtttactaagaacaagttgtgaccccctgacctggaggtcattcacaaaccacaggggacagtggggcacaacgtccctgttctcagctcagctctgtcactaacccggaccttggacaggcctctttccctctcttgcctcagggtttccaactataaaataaggggcagatgagatgaccgcttctgacgtcccttccaacttattgggtctgagagagaagggccaggtctcctgggggatagggcatctgcccctgaatctgcccaggatgtccctggcacgattcagatggtgcatgtgcaaaaggagaaagaggggtgtctctccagaagccagtgcagctgctgctcaagagacccatggtggcacggaccctggtgggctgaggcggcagaaggaccagaacatcaactgaggtccttggagaggctctgtttgtaagaagagctgcagaagggctagctggctgctggggcccaatgggtgacacgaggccacatgtcaggcaaggaggttggcccaggacattctggggggactgaatttcccagcaaacgggagcaaaaccacagaacaggttgaacttagaggattccagagatccaggcagagggccccaaaggtggaaaagggacattcattatccttacttgctcaaaggttggaccaggcagactttagggtggtggcctagggcttgacctcagagttaaaggtagggttgtgagcacctgaacaaggggacacagtgatcaccaggggacagggtgggctcaccagtcaggccccagcagcccagcctccttgctctgacagggatagagttgagcagactggggctggggatggatctagtgcacctgacttccagcagggcgcctgacacaatcttctgcaattgccctgggagaagggggcaggaaatgcaattggaatgtgtcccccaaagaggatgcattaatgggccaatgtcaaacagggagaggccagcccggtccacacacctcaggtgagacccagggccaactcctcactgggcagatgtgctgggagagaggagagcagtggtcactgaatcagggtgcagagaaattccacaggctggaatgaatcgagtaagaaggaatggaaaaggaaagaggtcacggtccctcattcagtctaaacagtaagtgcagactgggtgcggtggctcacgcctgtaatcccagcactttgggaggccgaggcaggcggatcacctgaggtcgggggttggagaccagcctgaccaacatggagaaaccccgttgctactaaaaatacaaaattagctgggtgtggtggcgcatgcctgtaatctcagctactagggaggctgaggcatcagaatcacttgaacctgggaggcggaggttgtggtgagccgagatcgcgccattgcactccagcctgggcaacaagagcgaaactccgtctcaaacaaaacaaaacaaaacaaaacaaaacaaaacaaaacaaaacaaaacaaaacagtaggtgcccccatcctgcatatacacagaaaacagatgtggcttagctgtcacttgcgtgtggggcccagggatttagctacagcagggcagggtgaatctctaaggtcatgtggccaaatcattgtcttttgggccaaattaacagaggaagggtgccacagcaggagaggtgatgtgcctgctcacttctggccggctgacatcagtgggaaggtgaagtgatacctgccccacacctttagagggacagccggaggcctgctgggggacagtgttaagagggagagctggggaagcctggctctgggatgcaggacagcacagctgctgtgggctcgctgacctagtgagctccttgtcactggaggtatgtgaggggaggcagaggtggctggggagaggaccacattgcagatggggtgcccagcaggtgcttctgaagtccctgacccctggaggctctgttgtctggtctgatgctacctggttctgggggctccatctgcctctagagttggtggggcctggggctgccctccctgcccaggctgcccccatttgggcccaggctgggatacaactgggtccgatgcttcaagttcgcctcttcctctccccttcctccctttccaatcgctcttaagaactggggggtcccctgcctggcctccttttctctttctgacaaggcaggacagacccgctgagcatccctgtcccttctggtgtccccatacagctgtgtgtgtgtttgcgtgggtttgtctgcaagtgtgcatgtgtctgcacgtgcctctctgtccctttgcgcctgcccaggctcaggctccgagcccgcctcctgacagtgcctcccctcaggcccctctccactgctgctccagactcaggctgaggggtgtgcggttccaggcagtgggcctgcccccagaggccacccctgcccttgctggggcacaggtacacacgcttctcaggtcaccgcctcatgacaccattgtcctggggcttgcatggagggccatggacacagagaggacatttaaaaaaatagagagaatttaagcttcccaaaaaagagatggggaggaggcgatggaggccgaggtggggctgggaggcgagtggccgtccgagagctctgggtccctggggatgacaaggtctctgtgggcaggacacagcccctgcccaggctgtgcccatctaccggtctggctgtacccaacgggcacagtggtcaggcccagctggccgaggggagggcaccgtatggctgtctgtagtctgtgcggagagcagggcgggggtggccaggctggccgcagaggctggcagtcccccccaggcccctgcccaagcgtccgtgcgcctggctggctctcaggaggcgaagtaggaactctgcatggagtagagccggtcgatggggttccccacgcgggcctgcagggagcccacgtctgaggagccgaggaagcagtcgctgaggctggttaaggaggtatcgctgtcgatgtcatggaagatggagtcgttcccataggggttcatgtggtcacctggcatttggggcggcgtgaggccctgctggaaggggtcgctgctgccgtaggggctctgttccatggccacgatctgctgctgtggtggggccagcggcgtgtaggaagccatcatgccctccatgcggctggacaggacctcctggcccagccgctgggagttctgctgctcctgctgctgctggtgccgccgcgccagcttcttcatctttgctctttggttctgaaaccagacctggaccacgcgcacactgaggcccgtctcagctgccagtgtctctcggacctttcggcaaggcttcgacgagacctcgaaggaggccttgaaggctcttcgctgctgcgtggtgaggatggtccggggtcgcttgggcctccgcgggtccttcccgtcatccccgctgcccttgctctgactgccctgccccttggccggcttcatgtccccatcttcatcctcgctcttcacggagtcggactcgtcggggctcacggagctgagcaggtccttctccttctcgtagtcacccttgcacagcagctggccctccttgagcacgaattcgtcgcccttgcgtagctgccgttcacacacgcagcagcagaagcagcccaggtggtacacgcactccagcgcccgcatcacgaactcggtgggggcgatcttctccatgcagccgctgcacttggccgcgaagagctgttggtagtcttgtttgcagtacagtttccgatcccggaagtagcagctggtggtgagggcttgctgacacgccgcgcactgcaaacactcctcgtgccaggacgactcgttgactcgcatcaggaagcggtcggagatgggccgctggcagccctcgcagacggcgggatgcgggcagtcggagcccagcagcacccccagagtggcgggcccggggcgcagggcgtgctcctccatcttgatgccgtccaacatcttggcgcagtccgtctgcccgcgagggaagcacctctccagcgactcgggacctgttgctatatccatgggacgcggggcgcgctgcggaccccgccggccgggctgctcgcccgccggcccgtccacccgctctccgccgccgcggccctggaaccggggaggcgcggcccccgcagggcaggggttgcgccggcccccggcgatcgtggagcggcgacgcgctggccccgggccccggcgtcgtgcgggcgggccggggcggctgcagcccgcgccgcgctctcccggacacttgcagccacgcgcgccggctcctctgtcacctgcttgtcagtcccggaacccggcggcggcggctgctgcagacggagccgcggggaggaggcggcggcggcggtggcggtggcggcggcggcaggcgggggagggggtgggggtgcaggggcggccccgcgggccgcggggggggcgcgcggcgcagcggggtcccgggcggggcgcagcgggccgcggggctccgggcgcgctccccgcgctactccagtgccatggtgcgcccgctgagccgccgggtttagagctggggct

SEQ ID NO: 17907 - RNA, 5785 nt, Homo sapiens
  source 1..5785: mol_type = other RNA
tcggctctctccctcaccctaggtggtgcccagagctcaaggatggagccaggcaggcatcaggcaatcctccttcctgaggttccctgcgtgcaacatgaaaaggacattcagatgggggcagagtggggaatcagcctcttgctaggaggctgcagggcttcccaaaggagaagaggcttgtccctgccaggccctgctcatctgatgcagcgccagggccttcccacctttacccaccctcaggaagcctcctaagatgcccagccacgtgcaccaaccccctttctgagctctttccaggctgtgctggcaccttggtctgactcttgtgagcagtgtctctgtgtggcctccctgtgcgtttcccaggatagcagagtacctgggaggcttcacggagtaggcagatgaggctctggctggggccatgcccagctttttgtccctcctctgccctgtgttacctggggcaattatttcctctttctgagccttgacttccccagcagggaagtggaacttggtcttttgccaagactccccctgcccacctctcattctcttttgctctggagaccacacagttatctccctcttcccactccagcccccttagtgatgaaggttccatgtcacggcacgggcaaggggtggtcctggctactccccgcccagctcccagccaaggctgcagctcctcccataaagtgggagaaggttgcccagccccacaggcttctgctgggtggccctgaacacatcgcctcccttctctgagcctcaggctcctcatctgagaaacgggtccctgccatgtctggactctctggctgggccggagagtctggctttccttctaggagacacccctcaaggcaggccctgcatcttgttcatctgcgagccacacccagtccggggctgggcagagtgggcactggtgtctgggagcctgtgggcagcaaggcacagcatagagcaaggggcccctagccacggctgacagggcgcctccagcataagggactctctgaggtcccttctggctttaacagtctgtgggtcacaagcatgctgtccctagaccagctcctggcatggggtcccggctggattcgggggtttgtgaggccccagaatgggaatatgtgaccccaacagctggcaagtttactaagaacaagttgtgaccccctgacctggaggtcattcacaaaccacaggggacagtggggcacaacgtccctgttctcagctcagctctgtcactaacccggaccttggacaggcctctttccctctcttgcctcagggtttccaactataaaataaggggcagatgagatgaccgcttctgacgtcccttccaacttattgggtctgagagagaagggccaggtctcctgggggatagggcatctgcccctgaatctgcccaggatgtccctggcacgattcagatggtgcatgtgcaaaaggagaaagaggggtgtctctccagaagccagtgcagctgctgctcaagagacccatggtggcacggaccctggtgggctgaggcggcagaaggaccagaacatcaactgaggtccttggagaggctctgtttgtaagaagagctgcagaagggctagctggctgctggggcccaatgggtgacacgaggccacatgtcaggcaaggaggttggcccaggacattctggggggactgaatttcccagcaaacgggagcaaaaccacagaacaggttgaacttagaggattccagagatccaggcagagggccccaaaggtggaaaagggacattcattatccttacttgctcaaaggttggaccaggcagactttagggtggtggcctagggcttgacctcagagttaaaggtagggttgtgagcacctgaacaaggggacacagtgatcaccaggggacagggtgggctcaccagtcaggccccagcagcccagcctccttgctctgacagggatagagttgagcagactggggctggggatggatctagtgcacctgacttccagcagggcgcctgacacaatcttctgcaattgccctgggagaagggggcaggaaatgcaattggaatgtgtcccccaaagaggatgcattaatgggccaatgtcaaacagggagaggccagcccggtccacacacctcaggtgagacccagggccaactcctcactgggcagatgtgctgggagagaggagagcagtggtcactgaatcagggtgcagagaaattccacaggctggaatgaatcgagtaagaaggaatggaaaaggaaagaggtcacggtccctcattcagtctaaacagtaagtgcagactgggtgcggtggctcacgcctgtaatcccagcactttgggaggccgaggcaggcggatcacctgaggtcgggggttggagaccagcctgaccaacatggagaaaccccgttgctactaaaaatacaaaattagctgggtgtggtggcgcatgcctgtaatctcagctactagggaggctgaggcatcagaatcacttgaacctgggaggcggaggttgtggtgagccgagatcgcgccattgcactccagcctgggcaacaagagcgaaactccgtctcaaacaaaacaaaacaaaacaaaacaaaacaaaacaaaacaaaacaaaacaaaacagtaggtgcccccatcctgcatatacacagaaaacagatgtggcttagctgtcacttgcgtgtggggcccagggatttagctacagcagggcagggtgaatctctaaggtcatgtggccaaatcattgtcttttgggccaaattaacagaggaagggtgccacagcaggagaggtgatgtgcctgctcacttctggccggctgacatcagtgggaaggtgaagtgatacctgccccacacctttagagggacagccggaggcctgctgggggacagtgttaagagggagagctggggaagcctggctctgggatgcaggacagcacagctgctgtgggctcgctgacctagtgagctccttgtcactggaggtatgtgaggggaggcagaggtggctggggagaggaccacattgcagatggggtgcccagcaggtgcttctgaagtccctgacccctggaggctctgttgtctggtctgatgctacctggttctgggggctccatctgcctctagagttggtggggcctggggctgccctccctgcccaggctgcccccatttgggcccaggctgggatacaactgggtccgatgcttcaagttcgcctcttcctctccccttcctccctttccaatcgctcttaagaactggggggtcccctgcctggcctccttttctctttctgacaaggcaggacagacccgctgagcatccctgtcccttctggtgtccccatacagctgtgtgtgtgtttgcgtgggtttgtctgcaagtgtgcatgtgtctgcacgtgcctctctgtccctttgcgcctgcccaggctcaggctccgagcccgcctcctgacagtgcctcccctcaggcccctctccactgctgctccagactcaggctgaggggtgtgcggttccaggcagtgggcctgcccccagaggccacccctgcccttgctggggcacaggtacacacgcttctcaggtcaccgcctcatgacaccattgtcctggggcttgcatggagggccatggacacagagaggacatttaaaaaaatagagagaatttaagcttcccaaaaaagagatggggaggaggcgatggaggccgaggtggggctgggaggcgagtggccgtccgagagctctgggtccctggggatgacaaggtctctgtgggcaggacacagcccctgcccaggctgtgcccatctaccggtctggctgtacccaacgggcacagtggtcaggcccagctggccgaggggagggcaccgtatggctgtctgtagtctgtgcggagagcagggcgggggtggccaggctggccgcagaggctggcagtcccccccaggcccctgcccaagcgtccgtgcgcctggctggctctcaggaggcgaagtaggaactctgcatggagtagagccggtcgatggggttccccacgcgggcctgcagggagcccacgtctgaggagccgaggaagcagtcgctgaggctggttaaggaggtatcgctgtcgatgtcatggaagatggagtcgttccctggcatttggggcggcgtgaggccctgctggaaggggtcgctgctgccgtaggggctctgttccatggccacgatctgctgctgtggtggggccagcggcgtgtaggaagccatcatgccctccatgcggctggacaggacctcctggcccagccgctgggagttctgctgctcctgctgctgctggtgccgccgcgccagcttcttcatctttgctctttggttctgaaaccagacctggaccacgcgcacactgaggcccgtctcagctgccagtgtctctcggacctttcggcaaggcttcgacgagacctcgaaggaggccttgaaggctcttcgctgctgcgtggtgaggatggtccggggtcgcttgggcctccgcgggtccttcccgtcatccccgctgcccttgctctgactgccctgccccttggccggcttcatgtccccatcttcatcctcgctcttcacggagtcggactcgtcggggctcacggagctgagcaggtccttctccttctcgtagtcacccttgcacagcagctggccctccttgagcacgaattcgtcgcccttgcgtagctgccgttcacacacgcagcagcagaagcagcccaggtggtacacgcactccagcgcccgcatcacgaactcggtgggggcgatcttctccatgcagccgctgcacttggccgcgaagagctgttggtagtcttgtttgcagtacagtttccgatcccggaagtagcagctggtggtgagggcttgctgacacgccgcgcactgcaaacactcctcgtgccaggacgactcgttgactcgcatcaggaagcggtcggagatgggccgctggcagccctcgcagacggcgggatgcgggcagtcggagcccagcagcacccccagagtggcgggcccggggcgcagggcgtgctcctccatcttgatgccgtccaacatcttggcgcagtccgtctgcccgcgagggaagcacctctccagcgactcgggacctgttgctatatccatgggacgcggggcgcgctgcggaccccgccggccgggctgctcgcccgccggcccgtccacccgctctccgccgccgcggccctggaaccggggaggcgcggcccccgcagggcaggggttgcgccggcccccggcgatcgtggagcggcgacgcgctggccccgggccccggcgtcgtgcgggcgggccggggcggctgcagcccgcgccgcgctctcccggacacttgcagccacgcgcgccggctcctctgtcacctgcttgtcagtcccggaacccggcggcggcggctgctgcagacggagccgcggggaggaggcggcggcggcggtggcggtggcggcggcggcaggcgggggagggggtgggggtgcaggggcggccccgcgggccgcggggggggcgcgcggcgcagcggggtcccgggcggggcgcagcgggccgcggggctccgggcgcgctccccgcgctactccagtgccatggtgcgcccgctgagccgccgggtttagagctggggct

SEQ ID NO: 17908 - RNA, 5818 nt, Homo sapiens
  source 1..5818: mol_type = other RNA
tcggctctctccctcaccctaggtggtgcccagagctcaaggatggagccaggcaggcatcaggcaatcctccttcctgaggttccctgcgtgcaacatgaaaaggacattcagatgggggcagagtggggaatcagcctcttgctaggaggctgcagggcttcccaaaggagaagaggcttgtccctgccaggccctgctcatctgatgcagcgccagggccttcccacctttacccaccctcaggaagcctcctaagatgcccagccacgtgcaccaaccccctttctgagctctttccaggctgtgctggcaccttggtctgactcttgtgagcagtgtctctgtgtggcctccctgtgcgtttcccaggatagcagagtacctgggaggcttcacggagtaggcagatgaggctctggctggggccatgcccagctttttgtccctcctctgccctgtgttacctggggcaattatttcctctttctgagccttgacttccccagcagggaagtggaacttggtcttttgccaagactccccctgcccacctctcattctcttttgctctggagaccacacagttatctccctcttcccactccagcccccttagtgatgaaggttccatgtcacggcacgggcaaggggtggtcctggctactccccgcccagctcccagccaaggctgcagctcctcccataaagtgggagaaggttgcccagccccacaggcttctgctgggtggccctgaacacatcgcctcccttctctgagcctcaggctcctcatctgagaaacgggtccctgccatgtctggactctctggctgggccggagagtctggctttccttctaggagacacccctcaaggcaggccctgcatcttgttcatctgcgagccacacccagtccggggctgggcagagtgggcactggtgtctgggagcctgtgggcagcaaggcacagcatagagcaaggggcccctagccacggctgacagggcgcctccagcataagggactctctgaggtcccttctggctttaacagtctgtgggtcacaagcatgctgtccctagaccagctcctggcatggggtcccggctggattcgggggtttgtgaggccccagaatgggaatatgtgaccccaacagctggcaagtttactaagaacaagttgtgaccccctgacctggaggtcattcacaaaccacaggggacagtggggcacaacgtccctgttctcagctcagctctgtcactaacccggaccttggacaggcctctttccctctcttgcctcagggtttccaactataaaataaggggcagatgagatgaccgcttctgacgtcccttccaacttattgggtctgagagagaagggccaggtctcctgggggatagggcatctgcccctgaatctgcccaggatgtccctggcacgattcagatggtgcatgtgcaaaaggagaaagaggggtgtctctccagaagccagtgcagctgctgctcaagagacccatggtggcacggaccctggtgggctgaggcggcagaaggaccagaacatcaactgaggtccttggagaggctctgtttgtaagaagagctgcagaagggctagctggctgctggggcccaatgggtgacacgaggccacatgtcaggcaaggaggttggcccaggacattctggggggactgaatttcccagcaaacgggagcaaaaccacagaacaggttgaacttagaggattccagagatccaggcagagggccccaaaggtggaaaagggacattcattatccttacttgctcaaaggttggaccaggcagactttagggtggtggcctagggcttgacctcagagttaaaggtagggttgtgagcacctgaacaaggggacacagtgatcaccaggggacagggtgggctcaccagtcaggccccagcagcccagcctccttgctctgacagggatagagttgagcagactggggctggggatggatctagtgcacctgacttccagcagggcgcctgacacaatcttctgcaattgccctgggagaagggggcaggaaatgcaattggaatgtgtcccccaaagaggatgcattaatgggccaatgtcaaacagggagaggccagcccggtccacacacctcaggtgagacccagggccaactcctcactgggcagatgtgctgggagagaggagagcagtggtcactgaatcagggtgcagagaaattccacaggctggaatgaatcgagtaagaaggaatggaaaaggaaagaggtcacggtccctcattcagtctaaacagtaagtgcagactgggtgcggtggctcacgcctgtaatcccagcactttgggaggccgaggcaggcggatcacctgaggtcgggggttggagaccagcctgaccaacatggagaaaccccgttgctactaaaaatacaaaattagctgggtgtggtggcgcatgcctgtaatctcagctactagggaggctgaggcatcagaatcacttgaacctgggaggcggaggttgtggtgagccgagatcgcgccattgcactccagcctgggcaacaagagcgaaactccgtctcaaacaaaacaaaacaaaacaaaacaaaacaaaacaaaacaaaacaaaacaaaacagtaggtgcccccatcctgcatatacacagaaaacagatgtggcttagctgtcacttgcgtgtggggcccagggatttagctacagcagggcagggtgaatctctaaggtcatgtggccaaatcattgtcttttgggccaaattaacagaggaagggtgccacagcaggagaggtgatgtgcctgctcacttctggccggctgacatcagtgggaaggtgaagtgatacctgccccacacctttagagggacagccggaggcctgctgggggacagtgttaagagggagagctggggaagcctggctctgggatgcaggacagcacagctgctgtgggctcgctgacctagtgagctccttgtcactggaggtatgtgaggggaggcagaggtggctggggagaggaccacattgcagatggggtgcccagcaggtgcttctgaagtccctgacccctggaggctctgttgtctggtctgatgctacctggttctgggggctccatctgcctctagagttggtggggcctggggctgccctccctgcccaggctgcccccatttgggcccaggctgggatacaactgggtccgatgcttcaagttcgcctcttcctctccccttcctccctttccaatcgctcttaagaactggggggtcccctgcctggcctccttttctctttctgacaaggcaggacagacccgctgagcatccctgtcccttctggtgtccccatacagctgtgtgtgtgtttgcgtgggtttgtctgcaagtgtgcatgtgtctgcacgtgcctctctgtccctttgcgcctgcccaggctcaggctccgagcccgcctcctgacagtgcctcccctcaggcccctctccactgctgctccagactcaggctgaggggtgtgcggttccaggcagtgggcctgcccccagaggccacccctgcccttgctggggcacaggtacacacgcttctcaggtcaccgcctcatgacaccattgtcctggggcttgcatggagggccatggacacagagaggacatttaaaaaaatagagagaatttaagcttcccaaaaaagagatggggaggaggcgatggaggccgaggtggggctgggaggcgagtggccgtccgagagctctgggtccctggggatgacaaggtctctgtgggcaggacacagcccctgcccaggctgtgcccatctaccggtctggctgtacccaacgggcacagtggtcaggcccagctggccgaggggagggcaccgtatggctgtctgtagtctgtgcggagagcagggcgggggtggccaggctggccgcagaggctggcagtcccccccaggcccctgcccaagcgtccgtgcgcctggctggctctcaggaggcgaagtaggaactctgcatggagtagagccggtcgatggggttccccacgcgggcctgcagggagcccacgtctgaggagccgaggaagcagtcgctgaggctggttaaggaggtatcgctgtcgatgtcatggaagatggagtcgttccctggcatttggggcggcgtgaggccctgctggaaggggtcgctgctgccgtaggggctctgttccatggccacgatctgctgctgtggtggggccagcggcgtgtaggaagccatcatgccctccatgcggctggacaggacctcctggcccaggccctgccccggccccggctcaccctggcccagccgctgggagttctgctgctcctgctgctgctggtgccgccgcgccagcttcttcatctttgctctttggttctgaaaccagacctggaccacgcgcacactgaggcccgtctcagctgccagtgtctctcggacctttcggcaaggcttcgacgagacctcgaaggaggccttgaaggctcttcgctgctgcgtggtgaggatggtccggggtcgcttgggcctccgcgggtccttcccgtcatccccgctgcccttgctctgactgccctgccccttggccggcttcatgtccccatcttcatcctcgctcttcacggagtcggactcgtcggggctcacggagctgagcaggtccttctccttctcgtagtcacccttgcacagcagctggccctccttgagcacgaattcgtcgcccttgcgtagctgccgttcacacacgcagcagcagaagcagcccaggtggtacacgcactccagcgcccgcatcacgaactcggtgggggcgatcttctccatgcagccgctgcacttggccgcgaagagctgttggtagtcttgtttgcagtacagtttccgatcccggaagtagcagctggtggtgagggcttgctgacacgccgcgcactgcaaacactcctcgtgccaggacgactcgttgactcgcatcaggaagcggtcggagatgggccgctggcagccctcgcagacggcgggatgcgggcagtcggagcccagcagcacccccagagtggcgggcccggggcgcagggcgtgctcctccatcttgatgccgtccaacatcttggcgcagtccgtctgcccgcgagggaagcacctctccagcgactcgggacctgttgctatatccatgggacgcggggcgcgctgcggaccccgccggccgggctgctcgcccgccggcccgtccacccgctctccgccgccgcggccctggaaccggggaggcgcggcccccgcagggcaggggttgcgccggcccccggcgatcgtggagcggcgacgcgctggccccgggccccggcgtcgtgcgggcgggccggggcggctgcagcccgcgccgcgctctcccggacacttgcagccacgcgcgccggctcctctgtcacctgcttgtcagtcccggaacccggcggcggcggctgctgcagacggagccgcggggaggaggcggcggcggcggtggcggtggcggcggcggcaggcgggggagggggtgggggtgcaggggcggccccgcgggccgcggggggggcgcgcggcgcagcggggtcccgggcggggcgcagcgggccgcggggctccgggcgcgctccccgcgctactccagtgccatggtgcgcccgctgagccgccgggtttagagctggggct

SEQ ID NO: 17909 - RNA, 4855 nt, Homo sapiens
  source 1..4855: mol_type = other RNA
tcggctgtgtatctctgtgtccaagtttcccttttcttaaaagaacaccagttattggattagactagttattaaatccaatccagtatggcagtatgatattgtgttccaaaaataaaattctaaccccacgcacagactgaatggaccctcgtctcaaccaaggggatccaaagaaacctgaaaatctagtttggatcatgatgggatggtggagtggggcaggggatgttgaacatgactcattatactctcctctttttggaattcaggcacaaaattgaccagcattaacattataacagagatcctaagactgacagaacagactctttatagccataagataccaaattctaacctgtctctagtacagcattacatgacagcaaagtcctgaaagaaaaaacatattttgaaatagcactgcaaacctgtctcttgtggaggaagttttacactctatagagattctccttcctttactaggtctctccagagagcctgacacctttgataagagatgttcacatctattctctctgaagcctgctacccagaggcttcatctacataacaagaacctaggcttctctagccctcccaacttgccttaactcaggctagtttcaactcttcaggcacagcttcaccctttcaaccaattgctaatcagaaaatctttgaatccacctacgaccagtaagccctgccacttcaagttgtcctgcctttccttattaaaccaatgtatatttcatacatattgattgatgtcttatgttccctaaaacacataaaaccaagatgtaacccaaccaccttcggccaatgttcctaggacctcctaataggtcataatccttaaccttggcaaaataaacttcaaaattgattgagacctgtctcagttactttttgacttatgacatcatctttacttgattatatatgcaaagaccttatttccaaataaggtcatattcacaggtaccaagggattagaactgtaacatattttacaattcaatccacagcaggccacataggaaacctcagtttcaaaacataggaatagtatagatcatattctttgatcataatgcattaaaattagaaattaataacaaaaataggaaaataaatctttgccacatgaaaattttagaatatctcttaactcatgagaaatccaacatggaaattaaatccaacactgcaaaatccctaaaaactaatgataaataaaattttaatataaccacaagtcagaagaaaattcatagtttaaaacaaaaattactaaacaggaaaaaaaagaaaaataagaatttagaaaggaacttcaaattactcttaaagaaagtagaagaaagcaaattctataaataaaatccaatcaatgaatcagaaacagaaaagtaatggagctaatacatacattaaaagctggctctttgaaaaatgaacacacattaaaatgtataatccatgcgttagttacctaggcaagtatagtgaaagaaaaaaaatgagaaataaccacagtcacgaaacagatttataagataataatttagtccactttgtgcatataaattcaatgacaaagaagtttccccaaaaaactaaaaagttcccagattgattctagaattaatttctaggtttaggtaattataaaagttcatctccacagggtacagaggatgagtaaatgttatgtgggacccaggacatttttgcactttttcatgcactgttctatgcattgctccatgcatgttaggctttctagaattcctggccagtactcaccaaatactcatcaccaccccattactgtggtgaccacgcaactttctaaaacaccctagagacagacaaaccagttagacggctgttgtcataaatcagaggcaggagagggtagggcaggagtgagatgaagaggaaacacaggatttttgacacactatagtgattagagattggtttaggaaccagttggagggtaacacggagaagggtggtgagaaaattaggctgagtctgatttaggacacatgaaaattttagaatatctcttatacaaaatatctcatatacaaaaacatgagcgttattcagttgaatatgattttactttcttacatccaaacacatttattgtgttaggtacaagcatttgactacttcattatgtctaatatagttatttttagcatttgtaagctaaaatgaatattatattacaggtagatcattatgttagattttgcaaagtatgtgcatagcaggactatacttacctatgaatttcatttcaggaaaataagcgagttgcaaaatatagtccttttgattgtccccaaacccctccccagccatcctcctgaagggcctgttgccgaccccaagacactgcttccagcagactcaagtctttgcagaacccatgattatgacagttgtctctactctcagttaccaaatgccctgatatttataggctctctctacagacacaactgcaactgtccttctaagagtggctacaataaatcctaaagtcctgcagcctcagggagggcaggaaaatggtgggggctggctcaaattcctaaacacacacacacacacacacacacacacacacacacacacacacacacacacacacgccctctaagacaatacttagaacacatttaggtagcttacagcacgcgaagcagggaagtagtaagattttgtctctaataagcattatgcagcactaaatggaagaaaaaaccaaatagcgaaatcactctccctctccgaaagaaaactactagcaaataaaaatactattgtctgccagagtccacacggcgccacgtggaaagttccccaaattacatttcatggatgaagtttgatttagaaaagcacccccggcatagtgttctcaagagctttcaacacagagccatgcttcagacacgcaaagcttctgctctctcctatgctattaacattacatcatagccttcaattccctaaaagatagaatcttttctccccccactggcttaagaaaggctagtctactaaagaggttttgtccacctgctgcgggaaaaattggtgagtcactaataagaaaatttactcaccgttagaggaattaggaaaaggaggactattgggtgtgaactcaaagaatgggagtctctacagccttaaaaagtccagtatcagatagagtacattacattatcacattcattccttcatccatccactctgtcatctatccattcacccattaatcaagtatgaactgtgtgccagtcaaacaaaagcagaacaaaacaacaccttccccccaacacacacacaaaacacacacaagtgccataatacagggcaacaagcgccatgttaagagatgaatggatgtaccaggtggtaagggaccactcatgacaatgcacaaccagacttggagggagaattttgggacttcctgaaaagagcagtatttaggctgagacgtaaggttcagcgggagctggccaggtgtaggcaagatagtgatggagcagaggataaagggtctcagaggtatatttgaaaagtcctagggtcaagccaagaaaagagaaagttgcagccttgagtaagaatgggggcaacaagagagaagcctgaagaaacagagtgccaggatacaggcaagggatttagactccctcctaaagtcacagaaataaatgacgaatttaaacaaaggagtggtatgatccacctgtcctgctttattttacaacatacaatataaagtatttgcagtattttttttctttctgcttcccataactctggacatgtgcttcataaggacaaggtcctcaacagctttgttcactgcttaatccctaaagcaagaagcaaacaatgtctgacacgaagtagacaataaatatttgttgcattaatcaaaggagggatgcatgagtgtattcttccgtgtattcttagcacccaactgaatcccctagcacgtttactcagaaacttggtcacagggatatttctgtgctaaatttttcccattacccagtttcaagagacaactagtttgcattcgaagtacaaaatatcctacatttggaagctctggcagatcaaatgctactggaaaaatttaagggctaataaattatgaatgaaattaataaaatacacttttttaaaggaattttaaagtacctggtgaaagctagatttctaaggtggtaactttgagctgtttcagtagcaccgtgacagaataaacatcccttccctaagaaagcagcttacagctagtatttccacagagtcagtgcctaaagcccaagaggctctcatgaatttcatatgtggtttaacctacaaagatttgcatgtttcctttaacgtaaaaccaagtcaattgatgagaagctgctgtgtccatcacatatcttctaccaatttcctaaggcatggcttttctcctttctaaagaattttatttttggtaactctgggcaacttttcctcatccagttgttcacaatgaattgatgattaaattgtaagagtgccacattagtttgggactttattttctggattgaaaaaagagagcatacaggcatttttagcagaatgagagaaaactattcattaactcttcctcttctcactccctttacttttgttttccttattccttcttgcttctctctcacgcatatgcactctctcctgggtgagacatatagatatggatatagatatagatatagagatagatgtatatatatacacacatacatac

SEQ ID NO: 17910 - RNA, 622 nt, Homo sapiens
  source 1..622: mol_type = other RNA
tcggctgtgtatctctgtgtctataattatcaattgcaaatcccagaaagatgtctacagaactgaatcaggaagaaatggggtgctctctctcatctctcagcgcaaacaagccttgttcaagaccaattagcatgactggtggttccttcttcccgaaggttacacttccaggctgagagcatctgctgtacatctcttcatttctttcccattttgagcaatttggttcctaagctcagtttcctcgtggcttcctggagctctgatgacaaactgccatactttgttcctgtcctttaaggccctgaagggcaccttatccacagttggagtacaccagacatgaagcagaattatctttccattttcgtttttagatagttcagggtaacttagagttctgaattcctgaatgttggccaaggtgatgtcattaaatcagttgtgttttcggctggcatccactccaactggatgatgctcatgctgtattatatgttaaatattgttatcattattccaggagccaggcagagaataggcactcaataaatggcagcagttttcagtatttttctcctgcattcccagctgccatatcacctgcagcattcagtta

SEQ ID NO: 17911 - RNA, 4669 nt, Homo sapiens
  source 1..4669: mol_type = other RNA
tcgggcctggggttgggggagcaagagttctgttttagccttgtgaatttggaaatcactaatttgcccaagattactcaaatggttgctctagaatttaagaccagttttatctcataatcaaaacctgagctcttgagctcctgcgttgctgctaatatccagttcctagttgaaggttctcagctcttaaaacttcattaactcaatggtcatcctattttatctgggaaaagcttcaacttcagtgatatcttcacatcatcactagagaaatcttcataaatgagtatatttataccatgtatcttttttcactagtaaagaacattatccaaaaagcaattgaaagtgtgtaaaggggaaagacataagtagaattttagtcttgcccagccttagttaatatgaaatacaggtgtcctattaaaattacatttttcattctaatcaaagttttacgtaaggttgtaattatgaaaataaaaaaaaagtaaagatgaaaacagggatgaatttgtcctttcagtgtgaaaataaagggagtaatttcattggtgagaacatatgtaagtagtctctgggttataaatgacttcaggaataataaattagaaatgttattgtctgggcgcggtggctcacgcctgtaatcccagcactttgggaggccgaggagggcggatcacgaggtcaggagatcgagaccatcctgactaacacggtgaaaccccgtctctactaaaaatacaaaaaattagccaggagtggtggtgggcgcctgtagtcccagctactggggaggctgaggcaggagaatggcgtgaacctgggaggcggaagttgcagtgatccgagatcgcgccactgcactccagcctgggcgacagagcgagactctgtctcgaaaaaaaaaagaaaagaaaagaaagaaatattctttagattaaactagccggaaagaggagaaaagtagaaagacagatagatagagtcttttaatgctataatcatgaaactaattagtcttatttttgtctttaggaaaggtgtgaaaagatggttttaatatgttattagctaaatcctataactccatttttcataattaataggacttattttttacttcatattcatgccaaggctaatttactactaaaacagaaaataggaggtttataaatactttgttgccataaaataaagaaaggaaaatacctcttaagtgaaaaattgtcacaattttagaaagaaaaaaaacaaacaaacatatatgtatgccagtactggcctagtttctgtttatagttgtgatgaaagagtcttttggatgtgcttttgaaaggggaaactttaaaacagaagttcagaacccatacagttaacaaaactccaagcatcacactacattggaaaaaatctttcatgtaagtagagattgattcttaatttcattctttgtttctggcctagataaccgactgttgcactgcccagtccaaatgattgcacagtgtccacacagctaaaaacagtgcatttttttccagttctgtctgttttcattaaagggcaataatcagggcagggaaatacatttctatatgtgcaaaggatgtttatgagcaaggagacttcatttctgtgtgccctcatacacatggctcaaacttgcagagatgccttgcaattttaataatgcattatggcagttctggtggctgattacttaagggcctttgtaaaaggatgacctcaaccatcttttgtcaccttcagacacatcacttcaatctgtttgaaagcagctgatgtgggtcagctatatagctcaaagccaaacggactgacattaagtgggaatctattcagaaaatatttcacatgtgtgtatgtgcatgcatgcatatacaagtataaaatctttcctttgcttattgttgacttactagaaagagtatattttggtaactatacgactataattttgttcacgctgtattttgaccagctgaacaaaaatatttataagcattttaaaaataaacttttcattacggtatagcatatacctggaaaagtacacaaatcattaatgtacagcttgatgaactttcacaaattgaacataccatgtattaataatcacatccagatcaatggaacattactagcctcactcactctgcctcccaatcaataatctttcctccctaaatataattactattttgactcctgacaacttagaatagcttagtttctccagttttttaaatttacatggagtcatacagtatatattcttttctgcctgctttttttactctcctgtttacaagatccatcaatgctgtttaatgacataatagatttctattttcatcttaagccattgattaaaatgctgtacacaatggttttaaaaatttatatgcccccaaactgtcccaagaatgatagctttttaattacctcaccaacactgggaaattgtcaatgctataaagataccaatccagtggacaaaatgcaatggcatatattggtttatttctactttttatttatttgccattcatatgtattttataaatcatctgttaatgtactttacctttgttttgctattgttatatagtatgttgttaattatttataataattttgtatattacggattcaatgatttaacatttcttctgaaaatatttattgtgtgtctactttgtgtcagggaatgtgcaggccactgggaataaaatattcattaaggcagcatcactgccctcatggagcttatattgcagccctttttctgctatactgagcattcttcgaggttaaatctgagatctgtttattggacttgcgtaggcgtttatatcctgttttctcataaatgtgaaatgcagcgtttaaattaccttgaacatattaagtgaatatttagagtgtacatatcattgaattatccatgggccctctaagaagtggacaaatcaatgaccaagatattctagggatgagcatccctgattccttctcaacatacacattctcgtatggcagaagtgacattaaattttctttttgtcttccatgagcaggcaaattagttctcccatgtagggtacagaaaatttaaaatgtcctcccttaattttatattttccatacaaagaagatgaaatgtatagttttgatgactataacttaaagttatatttattcaatattaaatgaactgtgtgagaagcctgtaaggttggaggctaatagaagcctctgcatcctctagcacagtaaacaaattaacctatttcttttgtgtatactattctttcagctgaatgtagggttgacacctgaggagttaaaaccctgactgtaacattaaaacttgttcccagtaaattaactaggctaaggttataatatgagaagcaggtcattcccattggccaaaaccttaatacatcctgcatatttctatcatatcctaattccactggtctagtaggcttgaggtgcaaattaattaacattggaagttatgacctaaatttcaccgatatatttctctgcctgccttccaaatgaaatctagctgcctctttaaagcctatacagttagttttagaagttatctctcacactatcaacttatttcatggatattcatatggtttttatttacctatgacatcctctgaggcaaatattgagaagagggatgctagattaatgtgaaagaaacttacctacactttgtttatgttctttctttattagaaaattcttttgaaatggactttatacatttaagaaattcataatgatttagctttgttatttttcgttattttcactaatgaaaagcctattgatttatatatacatagcacactatttttattcagctaggaaacacataggtctggctttaatatctgtattctataataaaaaatgatttcattattgatgctcttgtacttgtgtccattcaaaaagaaaatgtgttctgatactttttaaagaatatagtaactaccaaagacatacagacttaagatatcatgcagtttctttgaccaaatttgaaataatgatcaagagaggcattttcatttattataaatgatctagtccaggcatcagtaaaccatatggcataagtcaaattatagccctttgcctcttttagaatggcccatgagctgagaataattttaaaatgtttaaatagttaaaataatatttttgatatgaaaaacgatatggaattcaaagttgggtatccattcatttttaatgtcaattcaaattgtggatatccataagtatttaacatgtccaatggaccactgctgcactcatccataaacttcttgtctgtggctgatctctgatattaacaaataatttaactctttgaaatagtcttttacatcctattctgactgacaaacagaatcagtctttggcagtattatgaagttagttcttatactactttatgccttacccccttgtgtgagtatattcccactaccttcccaccagtagtcctttctgtaacctccctatcccaccaacaatgggctcaactttacacattctagtacggcagaggtgacatatttatattaaaatacaatct

SEQ ID NO: 17912 - RNA, 641 nt, Homo sapiens
  source 1..641: mol_type = other RNA
tcgggcctggggttgggggagcagatggtccccatcctgagtttcctcctggccttcctaactgctagcatccctgttgttaacaaactggccagtctcagcccagtgccactcactcagtgatcatcacttcttgggctctgtggacgtttcagggcgacgcttgccacgccagtctttccaaaatgcctttctggctgggggacggggcaaacagatggatccttacccactagcactcacagtccccactctctccggcccagcctccgctccactcccttaatctgctcagtcccagctccgttaaacttcttatgttcccctctggagatgggggaaggtaggcccctagagataaatcttacataaactgaaagtccgaggagcagccacacccggagccactcacaagacaggtgcccacccagtgtacagacatgcctgcgggtccatacacaggtgcgcgcccgggcgcgccggctctagcctgatttatgtttctatatatgtcactgggctggtacacaagctgggcctgcctgctactcactcccccgcttctctgcacagacgccccctgccctgtggcttcctgaaagacacacagaagtgcagccggcggcaccaggactcccagc

SEQ ID NO: 17913 - RNA, 2962 nt, Homo sapiens
  source 1..2962: mol_type = other RNA
tcggggcatgggggagggaggctggcgggggacccgggatgcatattgtcgcacgttcctggggtacagctccacaatgtcacctgaagcatctatcttgaaatgtctttctggccagacatttagatgttttttcttgtaagagtcacattcattaatgacatagtatctgggggcgtggggcctgggaccctgtgccagcaaagtcgaggcctgtggtccacggtgaggagggttgatttgctgaaagtcttttcggaaaagaggttctgagtgtacatcttcgatgtgcgttgtaaatgtcataggtgtgcgcgatctgttcctgtgaaggtcactggtgcttgcacacagaccgtgcagatacctgttagtttcatgctctagcctggatttggggaccccagggagaggtgagctaggagccctgtcccctggcctcgggctctggggcatggactgtgcgactgtctctatcctgccactcttgctgctccctgagtcaaaatgggccacgttgccgttgttttggggtgtgcccgagtgcgctgaggacagctggctggtaagatcactgtcgtttggaagcttcttggtgctttcttcctgggtctggattcgggcttctaccatctgggcaacctttttcttatcctctgatcttgcgttttggatctgcattttgagctggtggttgctgagctttagagaccgtgcgatgctctggagataatagatgagcatgaaaagcaggagtactgcgggcaggatgaccacggggctactgatgtgtccaaccacggagccaaaccacacaggaaagtctttctcaatcgtttctgacacaatgtcataaattttctcttgtccactgaatggcccacagtttagagatggcttgtatcggacaatagcaaaaatggttggcagcatgcacagaaacagcataaacaggagcattgccaagtagaagttgttggatcttgaggctcgaaatacttgctggtggggcacattgcaggtcagcacagcccagcttctcaggtacatgagcccaatgagtttgagaacgttgaacgctgggagacatggggagaagaaggcccccatccaaatcattccttggttgtagactaaatgtagcacattctcagctattttgaattctccatattcaggaaacttgctctccagatcccaacaccagtagtcacttaagtaccgcacgaaaagtcctcggaagaagtctatgagcagaatgctcgccacggtgaagagcatgtcaatgatggagagcttcagcatctcctgaccaacgtatgtctcccagcactggtcttgtggactctgagtgtggaggctagtcttgttggcctttataagaggcatggtataagctgaaatgctggtctcttccaaggcccatgtgttgtttctcctgagccccattccaggccgagatgtggaccatttctcttcttcaggggctgtcctggttgcaaagaaggtggtggaatctatccaatgacttgtgttatttttggtagccatttcctcaatgctcatgctgttaactttgtccaggagagcaatgatcaggctgtagagatttcccaaatacagcacaaggacccttgcaagctggaagcgcagcgtggtcctggggtggtacatctctaaggcagcaatgaggtcaaaggctgatggtgctatcatggtgacgagggagaccaccacactgacctcattcttttcccaaagtgtcagctccttcttcgactgctccagcttctgggaccggtccaccacaaagtagatgagataaatgctcccagccagtgagagaagcaccaggatgttggcaataatcctcaggcagatggtcactgccaggtttttgcttttctttttctcctgttcttccaatatagcttccctgatgctgttcactatggcagctgttttgctctctgcagcctctgggtttccaatgaggtaatcccaggcacagaacacccgccagcagaaggtatagttttcattggaagcactggcaagactcgtgcgggagttcttagccatcttttttaaaagaatgatgaagctgtaagcaaacactgccatccccactaggaaatacgccaagggcagccggtagccagctctcccgatcttcctctccctgccgtaatatccgtagaagaggacagagtactggaggtagccccccagagaccagacggtgtccaggtcttgggcagacgaaacctgctccttggggatggtcttcctggctgtgcttccaaagggctggcctgcaatcagctctggaatgacaataaaagcacctgtcataatggtgagcacaatattaattccaaataaccatctcaagaatatgaaataggaggcaacgccagatccaaaatgactctcgattttctttatcctcatttcccagggaatgaagatgaccacaaagttacaggcgagacgagcaaatttccgccagagctctgcacctgctgcttggtagcctcgggtcctggtcagcctcccttcaaacttcagcacaatgttcttcgcttgtctcaatgccctcagcttctgtcccatagtccagggtctgcagcgaatgtttgccatgagatctttctggaactgtatattctggaagatttgttccggatcattgctgtcccctgtttcatcagcactaaagctgtcatccaagttgctgagcagcagagattcctggtagaggtagcactggctggcatttctccggatgcctctatagcgctgggatgccttcgaggttttcatgggagctaacccactgctaacaatcagaagctggccagagagctaggaagttggcaggcaaaggtctgttccgaggtttctgaatggaagcagcggagtttgctctgcccgctagttctcaggaagaagactgtgt

SEQ ID NO: 17914 - RNA, 2922 nt, Homo sapiens
  source 1..2922: mol_type = other RNA
tcggggcatgggggagggaggctgggattcagcgtcgttgtcatttcctgtgtggcttcttttccagctgagaaacttttttttcttttttactttttaaaaagaatcacagccaaaataagacattaactgcaaaatccaaaatggctgcgcttaccctatgtataaaaatgcgtccagtccggtcggggcacggcctatgctttcccggggatcttggcccgcttgcgtgcaatagcatcctccacggccttcagctgtttcagcagctcctcccgccgagacagcgtgctggccttccctgatttggtgctggcggcgccgggatccgaggctttgccgggcacgctcgtgaccttgctggagctcttggactggggtgacagctggcgcttcctgtcagccggggctgcaggggctttggagttctggcctctctgccgctctggcttcggggagcccagtctcccacctgacttccggtcccgagaacctcggtctggggatgtgttgggccgcttggctggaggagggctctgcctgtccttgtctgatggttcatagcgcttcctgcttcctttatcagccgccttattcaacagtgtcaacttgatctccttgtgggccacaaatgtgccctgctggggctgcccggggggtgcctgctggggtgtcgagggctgctgggaggacttcccccctgctggaggttttgcagatttgggtggttgtgtggacgaatcccttttccgcttttcctctttaacaccgtcttctttcttagattttcctttctccttcctggtctgggctggggccggggaccgagagctggctgaggacacggggctagccaggtctgcgtacatgtcctccgagtccacgctgtgtgcagagctgctgctcgacgtagcactggacactgaggagacgctgctcacgctcagggacctggatcgggagctggaaccactatagctgctaccactgccactgccgctgccgcttagcgtccgcctcctggggggggtcctggctggccgctccttcctcctggcttcccgagggtctcctggcttggtgggctcggggacaggagcagtggttttggtggcctgtggtggggctggaggcggggccggcttcttcactgacttctctcctgctttcccgggcggcggggccggctctcccttggttctgatggaaggtctatgtggggaaggtgttggggacggggacggggacgaagagaaggaccgggacctggaccggcttcctgagaacgagctgtgtctggaagagcggctggagtaggagctgtaggatgaagaccgggatcgcgaccgggaggagccggagccagagtaggacgatgaccgcgaagacgacctggaggaattagaggcagaggctgacgaggctgatgttttccgacgccttcgagcccggctcggggagaccgacaccccgagtttcttcttgggagacttggatcggcgccaagggtccttccactcatctgctctcttcacctgcggccccgtggtggcagcctccttctttggtggctcagcttggcggactgtgtctctgacatctctcgggatccgagaattccaatctcgaaaaacttcattttctttgtcaaattcccgttcgtcttcgccaatggtcaccgtaaaccttttctcttcaaaatcaggctcctgttcttttcgaatagttgctttttttaaaacctcctttgcatgccggagtcctcgttcccaggcactctctgttgggggctctggagggggtggaggcaaaatttcatcaactaccggcccaccccaagggttggcgggcatcagcgggtgaggtccgagaggcggggcaccattaggcgggaaggggtcggctttggtgattagggagtagttccccttgtcgttcactccagggtgtataaacctacaattcattccccaggtacagttccctttaacctggcctctgaatggtatggaattggatattggtggaagaagagtggataatggtgtcacaacatctttcatgaagaaccggcaggtgggacgaggcctcaccttcctgtcactggggtccttcacttcaccttcttccaggtcatcatcgtctatttccccatcatcgatttctccatcatcgtcctctttctttttctccttggcagcctccagggattccttttctcccacactctgaacaccagccttcccctcctccctgggagtgccttcgcctttctcctcatcatcctcagcccccgctttctcagcctcgtcctcctggacggcgggagctggctcctcaggaacctcctcatcgtagtctagctcatgctcatccagctccctggtgactgaggaggcctcatccctaaggtcgcttgtccggtcttcctccccttcgtccccctcctcctcgcagggggagctggtcgggccccggctcagctcattcacctctgagtcctggtcttgggatttaggctcacttgcccggtcctcctcgtcggagtgattatcttcctcctcctggctcggccccctggctgcactttcctcatcctccagatcagaagccctcacccccgccccgtccaaatcctgatcggacccgctgtccctcagaatgtcatcgtccgagagtccctgtggctgctcttcatcctctggagagtgaggatcccgttcagggctctcggccacatccatcggtacccacggttctcagcgctagggcggagaggaggccacggctcccctggagtcggagcggcgtggagaagacgtcccttggcccttccgctcttcacaggttctggctccaggctcgacacgggcggaacaaacgggctccactacccgcgggggccggccattgtgcgacgtc

SEQ ID NO: 17915 - RNA, 3309 nt, Homo sapiens
  source 1..3309: mol_type = other RNA
tcggggcatgggggagggaggctgggattcagcgtcgttgtcatttcctgtgtggcttcttttccagctgagaaacttttttttcttttttactttttaaaaagaatcacagccaaaataagacattaactgcaaaatccaaaatggctgcgcttaccctatgtataaaaatgcgtccagtccggtcggggcacggcctatgctttcccggggatcttggcccgcttgcgtgcaatagcatcctccacggccttcagctgtttcagcagctcctcccgccgagacagcgtgctggccttccctgatttggtgctggcggcgccgggatccgaggctttgccgggcacgctcgtgaccttgctggagctcttggactggggtgacagctggcgcttcctgtcagccggggctgcaggggctttggagttctggcctctctgccgctctggcttcggggagcccagtctcccacctgacttccggtcccgagaacctcggtctggggatgtgttgggccgcttggctggaggagggctctgcctgtccttgtctgatggttcatagcgcttcctgcttcctttatcagccgccttattcaacagtgtcaacttgatctccttgtgggccacaaatgtgccctgctggggctgcccggggggtgcctgctggggtgtcgagggctgctgggaggacttcccccctgctggaggttttgcagatttgggtggttgtgtggacgaatcccttttccgcttttcctctttaacaccgtcttctttcttagattttcctttctccttcctggtctgggctggggccggggaccgagagctggctgaggacacggggctagccaggtctgcgtacatgtcctccgagtccacgctgtgtgcagagctgctgctcgacgtagcactggacactgaggagacgctgctcacgctcagggacctggatcgggagctggaaccactatagctgctaccactgccactgccgctgccgcttagcgtccgcctcctggggggggtcctggctggccgctccttcctcctggcttcccgagggtctcctggcttggtgggctcggggacaggagcagtggttttggtggcctgtggtggggctggaggcggggccggcttcttcactgacttctctcctgctttcccgggcggcggggccggctctcccttggttctgatggaaggtctatgtggggaaggtgttggggacggggacggggacgaagagaaggaccgggacctggaccggcttcctgagaacgagctgtgtctggaagagcggctggagtaggagctgtaggatgaagaccgggatcgcgaccgggaggagccggagccagagtaggacgatgaccgcgaagacgacctggaggaattagaggcagaggctgacgaggctgatgttttccgacgccttcgagcccggctcggggagaccgacaccccgagtttcttcttgggagacttggatcggcgccaagggtccttccactcatctgctctcttcacctgcggccccgtggtggcagcctccttctttggtggctcagcttggcggcttggcggctgcggggagcggggcttgggcttccccttctccttctcccgctccttctcccggtcgcggtcacggtgctgccggtccttctcgtcccgcttggctcgctcacgctcccactcctccttcctccgctgccgctccttgtcgcgctcgcgctcccgctctcgctcgcgctccctctgccggcgctcccgctctcggtcccgctcccgctcccgctcgcgctcgcgctgtctgttctctctctctcgctcccgctccctttctcggtaattatgatacggctctgtttctgtatactgcaccctgaaattctcatactgtccgccacgccaaaaccgctcaatttcatagtcataataagggtctgcgtaaggctcgagtactgtgtctctgacatctctcgggatccgagaattccaatctcgaaaaacttcattttctttgtcaaattcccgttcgtcttcgccaatggtcaccgtaaaccttttctcttcaaaatcaggctcctgttcttttcgaatagttgctttttttaaaacctcctttgcatgccggagtcctcgttcccaggcactctctgttgggggctctggagggggtggaggcaaaatttcatcaactaccggcccaccccaagggttggcgggcatcagcgggtgaggtccgagaggcggggcaccattaggcgggaaggggtcggctttggtgattagggagtagttccccttgtcgttcactccagggtgtataaacctacaattcattccccaggtacagttccctttaacctggcctctgaatggtatggaattggatattggtggaagaagagtggataatggtgtcacaacatctttcatgaagaaccggcaggtgggacgaggcctcaccttcctgtcactggggtccttcacttcaccttcttccaggtcatcatcgtctatttccccatcatcgatttctccatcatcgtcctctttctttttctccttggcagcctccagggattccttttctcccacactctgaacaccagccttcccctcctccctgggagtgccttcgcctttctcctcatcatcctcagcccccgctttctcagcctcgtcctcctggacggcgggagctggctcctcaggaacctcctcatcgtagtctagctcatgctcatccagctccctggtgactgaggaggcctcatccctaaggtcgcttgtccggtcttcctccccttcgtccccctcctcctcgcagggggagctggtcgggccccggctcagctcattcacctctgagtcctggtcttgggatttaggctcacttgcccggtcctcctcgtcggagtgattatcttcctcctcctggctcggccccctggctgcactttcctcatcctccagatcagaagccctcacccccgccccgtccaaatcctgatcggacccgctgtccctcagaatgtcatcgtccgagagtccctgtggctgctcttcatcctctggagagtgaggatcccgttcagggctctcggccacatccatcggtacccacggttctcagcgctagggcggagaggaggccacggctcccctggagtcggagcggcgtggagaagacgtcccttggcccttccgctcttcacaggttctggctccaggctcgacacgggcggaacaaacgggctccactacccgcgggggccggccattgtgcgacgtc

SEQ ID NO: 17916 - RNA, 3237 nt, Homo sapiens
  source 1..3237: mol_type = other RNA
tcggggcatgggggagggaggctgggattcagcgtcgttgtcatttcctgtgtggcttcttttccagctgagaaacttttttttcttttttactttttaaaaagaatcacagccaaaataagacattaactgcaaaatccaaaatggctgcgcttaccctatgtataaaaatgcgtccagtccggtcggggcacggcctatgctttcccggggatcttggcccgcttgcgtgcaatagcatcctccacggccttcagctgtttcagcagctcctcccgccgagacagcgtgctggccttccctgatttggtgctggcggcgccgggatccgaggctttgccgggcacgctcgtgaccttgctggagctcttggactggggtgacagctggcgcttcctgtcagccggggctgcaggggctttggagttctggcctctctgccgctctggcttcggggagcccagtctcccacctgacttccggtcccgagaacctcggtctggggatgtgttgggccgcttggctggaggagggctctgcctgtccttgtctgatggttcatagcgcttcctgcttcctttatcagccgccttattcaacagtgtcaacttgatctccttgtgggccacaaatgtgccctgctggggctgcccggggggtgcctgctggggtgtcgagggctgctgggaggacttcccccctgctggaggttttgcagatttgggtggttgtgtggacgaatcccttttccgcttttcctctttaacaccgtcttctttcttagattttcctttctccttcctggtctgggctggggccggggaccgagagctggctgaggacacggggctagccaggtctgcgtacatgtcctccgagtccacgctgtgtgcagagctgctgctcgacgtagcactggacactgaggagacgctgctcacgctcagggacctggatcgggagctggaaccactatagctgctaccactgccactgccgctgccgcttagcgtccgcctcctggggggggtcctggctggccgctccttcctcctggcttcccgagggtctcctggcttggtgggctcggggacaggagcagtggttttggtggcctgtggtggggctggaggcggggccggcttcttcactgacttctctcctgctttcccgggcggcggggccggctctcccttggttctgatggaaggtctatgtggggaaggtgttggggacggggacggggacgaagagaaggaccgggacctggaccggcttcctgagaacgagctgtgtctggaagagcggctggagtaggagctgtaggatgaagaccgggatcgcgaccgggaggagccggagccagagtaggacgatgaccgcgaagacgacctggaggaattagaggcagaggctgacgaggctgatgttttccgacgccttcgagcccggctcggggagaccgacaccccgagtttcttcttgggagacttggatcggcgccaagggtccttccactcatctgctctcttcacctgcggccccgtggtggcagcctccttctttggtggctcagcttggcggcttggcggctgcggggagcggggcttgggcttccccttctccttctcccgctccttctcccggtcgcggtcacggtgctgccggtccttctcgtcccgcttggctcgctcacgctcccactcctccttcctccgctgccgctccttgtcgcgctcgcgctcccgctctcgctcgcgctccctctgccggcgctcccgctctcggtcccgctcccgctcccgctcgcgctcgcgctgtctgttctctctctctcgctcccgctccctttctcggtaattatgatacggctctgtttctgtatactgcaccctgaaattctcatactgtccgccacgccaaaaccgctcaatttcatagtcataataagggtctgcgtaaggctcgagtactgtgtctctgacatctctcgggatccgagaattccaatctcgaaaaacttcattttctttgtcaaattcccgttcgtcttcgccaatggtcaccgtaaaccttttctcttcaaaatcaggctcctgttcttttcgaatagttgctttttttaaaacctcctttgcatgccggagtcctcgttcccaggcactctctgttgggggctctggagggggtggaggcaaaatttcatcaactaccggcccaccccaagggttggcgggcatcagcgggtgaggtccgagaggcggggcaccattaggcgggaaggggtcggctttggtgattagggagtagttccccttgtcgttcactccagggtgtataaacctacaattcattccccaggtacagttccctttcatgaagaaccggcaggtgggacgaggcctcaccttcctgtcactggggtccttcacttcaccttcttccaggtcatcatcgtctatttccccatcatcgatttctccatcatcgtcctctttctttttctccttggcagcctccagggattccttttctcccacactctgaacaccagccttcccctcctccctgggagtgccttcgcctttctcctcatcatcctcagcccccgctttctcagcctcgtcctcctggacggcgggagctggctcctcaggaacctcctcatcgtagtctagctcatgctcatccagctccctggtgactgaggaggcctcatccctaaggtcgcttgtccggtcttcctccccttcgtccccctcctcctcgcagggggagctggtcgggccccggctcagctcattcacctctgagtcctggtcttgggatttaggctcacttgcccggtcctcctcgtcggagtgattatcttcctcctcctggctcggccccctggctgcactttcctcatcctccagatcagaagccctcacccccgccccgtccaaatcctgatcggacccgctgtccctcagaatgtcatcgtccgagagtccctgtggctgctcttcatcctctggagagtgaggatcccgttcagggctctcggccacatccatcggtacccacggttctcagcgctagggcggagaggaggccacggctcccctggagtcggagcggcgtggagaagacgtcccttggcccttccgctcttcacaggttctggctccaggctcgacacgggcggaacaaacgggctccactacccgcgggggccggccattgtgcgacgtc

SEQ ID NO: 17917 - RNA, 1701 nt, Homo sapiens
  source 1..1701: mol_type = other RNA
tcggggcatgggggagggaggctgggattcagcgtcgttgtcatttcctgtgtggcttcttttccagctgagaaacttttttttcttttttactttttaaaaagaatcacagccaaaataagacattaactgcaaaatccaaaatggctgcgcttaccctatgtataaaaatgcgtccagtccggtcggggcacggcctatgctttcccggggatcttggcccgcttgcgtgcaatagcatcctccacggccttcagctgtttcagcagctcctcccgccgagacagcgtgctggccttccctgatttggtgctggcggcgccgggatccgaggctttgccgggcacgctcgtgaccttgctggagctcttggactggggtgacagctggcgcttcctgtcagccggggctgcaggggctttggagttctggcctctctgccgctctggcttcggggagcccagtctcccacctgacttccggtcccgagaacctcggtctggggatgtgttgggccgcttggctggaggagggctctgcctgtccttgtctgatggttcatagcgcttcctgcttcctttatcagccgccttattcaacagtgtcaacttgatctccttgtgggccacaaatgtgccctgctggggctgcccggggggtgcctgctggggtgtcgagggctgctgggaggacttcccccctgctggaggttttgcagatttgggtggttgtgtggacgaatcccttttccgcttttcctctttaacaccgtcttctttcttagattttcctttctccttcctggtctgggctggggccggggaccgagagctggctgaggacacggggctagccaggtctgcgtacatgtcctccgagtccacgctgtgtgcagagctgctgctcgacgtagcactggacactgaggagacgctgctcacgctcagggacctggatcgggagctggaaccactatagctgctaccactgccactgccgctgccgcttagcgtccgcctcctggggggggtcctggctggccgctccttcctcctggcttcccgagggtctcctggcttggtgggctcggggacaggagcagtggttttggtggcctgtggtggggctggaggcggggccggcttcttcactgacttctctcctgctttcccgggcggcggggccggctctcccttggttctgatggaaggtctatgtggggaaggtgttggggacggggacggggacgaagagaaggaccgggacctggaccggcttcctgagaacgagctgtgtctggaagagcggctggagtaggagctgtaggatgaagaccgggatcgcgaccgggaggagccggagccagagtaggacgatgaccgcgaagacgacctggaggaattagaggcagaggctgacgaggctgatgttttccgacgccttcgagcccggctcggggagaccgacaccccgagtttcttcttgggagacttggatcggcgccaagggtccttccactcatctgctctcttcacctgcggccccgtggtggcagcctccttctttggtggctcagcttggcggtcggtaattatgatacggctctgtttctgtatactgcaccctgaaattctcatactgtccgccacgccaaaaccgctcaatttcatagtcataataagggtctgcgtaaggctcgag

SEQ ID NO: 17918 - RNA, 436 nt, Homo sapiens
  source 1..436: mol_type = other RNA
tcggggcatgggggagggaggctgggcatgagcggcactccctctggggctgcccaagttcggtctgtcccaggacccaagcccgtctggccgacctggctccctgcacactccctccctccgtgcccctcccactgtgcctctccgccctcggtcgtggccggtctgagcctccgctgcggtggccgtcggattctctgctggtgcctgcaggctcctctgcagacgttgcctcctccacatctccacgccagctgtgccaccgctgtgcagtccctgccacccctgacgacagacagcggcacgcaaagaggctcgggcgcagggggaagctcgtgttggccccggctggagtgcacatcagtcccggcttcggccgtggccacctccgcccagagccttgagtgggcattgagggggcgctgctctgcgtgag

SEQ ID NO: 17919 - RNA, 3501 nt, Homo sapiens
  source 1..3501: mol_type = other RNA
tcggggcatgggggagggaggctggggccttcccgagagacctaaaagattgcccactcttggcggcaagtgcaggtagttgctggcctccgaccatctgcttcgcctgcttcaccaggcccggggattggctaagaggccctggggtctgctcagcccctgcagaagctcttcctgaggcctgagttgttggctcatataaaaaggccttggcaggaggctgagaaagaagtctggcctgggtgagtgatttaacagcttgccaggggtcctctgaaggggctgctgctttcccagatgtctgaagaggatctgacacacagcctttctcaacagctctcggcatatgccccagacctttgctggcaggccatgaacttgactccaacactggcatcttctcatcagcctgtggtgtgacctgatgaggtgaagctgcccgctccttctggcgaggagttaggtctatgagatccatcaccaaagcagctctattttttgactgagtattctggtccacaggcctcagtgctttttctttagctacaagggtctggaccacagctgatagtactttctcaggaggtgggagtctctgggacaaagaggcatggggtttgtcagtaggcctgtctgaagtctggggtttgggactgctagtaatgagcagtctgtctggcggcggaagtctcaggccagtgggaactgaggttttctccagtgactggggccttgggctggcagcacctatggatttatccagccttgggtcagccgtccccagaggtctttccagtggttgggacctgactgagggtgaggagcttgggctggtcactggagagggtttgtcgcttagctggggtcttggtcctgccactgctggtggcctgtccagtggcctctggctggaaaccaaggattgggatttggtccctgacccagcgaggtctctgaccttatctaaaggctggggcctggagtcagttctctcaagaggtctttcaggtagcaatggcctctgacaagtccctgccagagcttttttggagagcgacagcatctggttggtgtcagcaggaggtttatctgacattttgggtgcctgagcagccattcctgttgattgctctgccaggtgagtgcttggccctggaggcagcggtactgggggaggcacatactcacggatctccccaggttccagaggattgggcccacaggggtcatgctcagtacaagacagacgcccatccagtttggaaatgaaaagcatcccttctcgatgctgcttacaaaaggagctggggcacatctcacagaaggaggctgcttccttcccgcagatgtcacactgatgccacggacattcccatttccctgctggtcgcttggtcagattgagacagtctgcgtggtaaacttttgggcagcctggtttcttgcaggagacgagctggccagcatccccacaactaaaacactcatcttctcgctcctttgtgatttcaccctgggtcctgcgctttccctgttgcttcttcttgaatttctttgacttttcttccgtggcaatgggttgattctttggccttacacccaagaagccactgcagttcggggctccacatttgcaaacagtctttccattcccaagacattctaggttgtagttgaaggtaagttcagtgcctgctttaatgtcacttagtgcaaaaaggcctacacgggtatctccattcacagaccacttctgtgtttcacagttgggctggcagcaatgattcatgaaccgagcatagtttcctttgggaccagcatcaatgattcggtctttgtctagggtgagcatatagaaattagtgatatcatgttcttgagcatagcgaattcgagctctgcattcttcttcatctataagctcacccacatactcattcacaaattcaccctttttaatatctgtttttgtccgtagaccccaaccccgctgtaatgtgcggaaaatttcaacctctggatattggcgcttggaaaagcactggttttgacagcgccctccggcaggacacactgtggggtggcactcatagagcagcatgcggttgatgcattcagagtctatcccacaggggttctcatcagtagctttacagttgcaacggggtatttcagataagtctgcagtgaagatctgtaccctgccaataggacggtttacctttatatgtttataaggtggtggcttcttgtcattctttcggtcttcctgcagctgtcttagctctttttgggcctttaattcctcaaaccttgctgcagcttcctgaagagcttttttatatgtcccatccactcctttgcccatcttatccttgctgctcacgtcaccctccatgtaagggaagactcgggcctggtgagtccacaaatagtcattagatccaaaaaagaggactgggaactctcccacatcatgtctcatcttatcaatgttggaaggaacagctcgaggatggcagatctcagctggccaccacctgtatcgtccaacttttacccagacaatctccctgtagtgtggctttttgcctgctttacagtcattgcaataccagtttccttcagggatatcaatgttcaggcattcacgatgaaaagcagcagggcaagaatcacagcacagaaggctgcctccttctgagcacacaaagcaccagctaacattaacatgctcatgatttcggcagccccgcctaggggtaaagtgattagggcagatgatactattagatgcaaggatctttgacccagcagccaggcaaaagtcattggcgtggtatgccacaggacagcggacacagcgcatcaaccgacctttagatgcagaaacattggctggattagcagcatgacaggttatacagatgtggagggagcaccggaagcccttgttctgcataacagtgggtgggtacttctggacacactcttcatggtaaaactttccacacaagggtagaaggcaccttttaacatcttccccactctgcttacatacaaaacaggtatggattcctgtgcgacattcattgcagataaattttcctcttggcatctcagtcaatccaaggcactccaggtggaaagccccacagcactgagcctcacataacagcagctcacccaatttttcacaattctgacagacattctccttgagtgcagctcctccaccgcgttcaccctgcatttttttagaggcaggcatcccgggatcgtgttctacaccttcctcaacagtctccttggggcttgtggccgtcctgtgaggcattagttctccagatgttcagccaatcactcgggcggactgcatgcaatgttagttctaaccctgctgtgattgggcgggtagtgggcgcctcatgccctgccactaactgctctgaggctgtttgttccactggaactttctgagctgttccattttaaggtttc

SEQ ID NO: 17920 - RNA, 7329 nt, Homo sapiens
  source 1..7329: mol_type = other RNA
tcggggcatgggggagggaggctggggccttcccgagagacctaaaagattgcccactcttggcggcaagtgcaggtagttgctggcctccgaccatctgcttcgcctgcttcaccaggcccggggattggctaagaggccctggggtctgctcagcccctgcagaagctcttcctgaggcctgagttgttggctcatataaaaaggccttggcaggaggctgagaaagaagtctggcctgggtgagtgatttaacagcttgccaggggtcctctgaaggggctgctgctttcccagatgtctgaagaggatctgacacacagcctttctcaacagctctcggcatatgccccagacctttgctggcaggccatgaacttgactccaacactggcatcttctcatcagcctgtggtgtgacctgatgaggtgaagctgcccgctccttctggcgaggagttaggtctatgagatccatcaccaaagcagctctattttttgactgagtattctggtccacaggcctcagtgctttttctttagctacaagggtctggaccacagctgatagtactttctcaggaggtgggagtctctgggacaaagaggcatggggtttgtcagtaggcctgtctgaagtctggggtttgggactgctagtaatgagcagtctgtctggcggcggaagtctcaggccagtgggaactgaggttttctccagtgactggggccttgggctggcagcacctatggatttatccagccttgggtcagccgtccccagaggtctttccagtggttgggacctgactgagggtgaggagcttgggctggtcactggagagggtttgtcgcttagctggggtcttggtcctgccactgctggtggcctgtccagtggcctctggctggaaaccaaggattgggatttggtccctgacccagcgaggtctctgaccttatctaaaggctggggcctggagtcagttctctcaagaggtctttcaggtagcaatggcctctgacaagtccctgccagagcttttttggagagcgacagcatctggttggtgtcagcaggaggtttatctgacattttgggtgcctgagcagccattcctgttgattgctctgccaggtgagtgcttggccctggaggcagcggtactgggggaggcacatactcacggatctccccaggttccagaggattgggcccacaggggtcatgctcagtacaagacagacgcccatccagtttggaaatgaaaagcatcccttctcgatgctgcttacaaaaggagctggggcacatctcacagaaggaggctgcttccttcccgcagatgtcacactgatgccacggacattcccatttccctgctggtcgcttggtcagattgagacagtctgcgtggtaaacttttgggcagcctggtttcttgcaggagacgagctggccagcatccccacaactaaaacactcatcttctcgctcctttgtgatttcaccctgggtcctgcgctttccctgttgcttcttcttgaatttctttgacttttcttccgtggcaatgggttgattctttggccttacacccaagaagccactgcagttcggggctccacatttgcaaacagtctttccattcccaagacattctaggttgtagttgaaggtaagttcagtgcctgctttaatgtcacttagtgcaaaaaggcctacacgggtatctccattcacagaccacttctgtgtttcacagttgggctggcagcaatgattcatgaaccgagcatagtttcctttgggaccagcatcaatgattcggtctttgtctagggtgagcatatagaaattagtgatatcatgttcttgagcatagcgaattcgagctctgcattcttcttcatctataagctcacccacatactcattcacaaattcaccctttttaatatctgtttttgtccgtagaccccaaccccgctgtaatgtgcggaaaatttcaacctctggatattggcgcttggaaaagcactggttttgacagcgccctccggcaggacacactgtggggtggcactcatagagcagcatgcggttgatgcattcagagtctatcccacaggggttctcatcagtagctttacagttgcaacggggtatttcagataagtctgcagtgaagatctgtaccctgccaataggacggtttacctttatatgtttataaggtggtggcttcttgtcattctttcggtcttcctgcagctgtcttagctctttttgggcctttaattcctcaaaccttgctgcagcttcctgaagagcttttttatatgtcccatccactcctttgcccatcttatccttgctgctcacgtcaccctccatgtaagggaagactcgggcctggtgagtccacaaatagtcattagatccaaaaaagaggactgggaactctcccacatcatgtctcatcttatcaatgttggaaggaacagctcgaggatggcagatctcagctggccaccacctgtatcgtccaacttttacccagacaatctccctgtagtgtggctttttgcctgctttacagtcattgcaataccagtttccttcagggatatcaatgttcaggcattcacgatgaaaagcagcagggcaagaatcacagcacagaaggctgcctccttctgagcacacaaagcaccagctaacattaacatgctcatgatttcggcagccccgcctaggggtaaagtgattagggcagatgatactattagatgcaaggatctttgacccagcagccaggcaaaagtcattggcgtggtatgccacaggacagcggacacagcgcatcaaccgacctttagatgcagaaacattggctggattagcagcatgacaggttatacagatgtggagggagcaccggaagcccttgttctgcataacagtgggtgggtacttctggacacactcttcatggtaaaactttccacacaagggtagaaggcaccttttaacatcttccccactctgcttacatacaaaacaggtatggattcctgtgcgacattcattgcagataaattttcctcttggcatctcagtcaatccaaggcactccaggtggaaagccccacagcactgagcctcacataacagcagctcacccaatttttcacaattctgacagacattctccttgagtgcagctcctccaccgcgttcaccctgcatttttttagaggcaggcatcccgggatcgtgttctacaccttcctcaacagtctccttggggcttgtggccgtcctgtgaggcattagttctccctctgagcctggaatctcttttgacgagtcatcatttttcacttttttacactgcatcttggctgcagcatgcctctgtcgttttcgcttccttggcttgtcaaatatcttggtagtgcctccaccaaaatcttttgaataagatgtggcacaagattcagttatgccattctccaggtgaccagcttcatagcactttttagaaaggccaaggtcccccttcttgggcataaatccagggtctaaatcattggattcaagaagtttcttagttggttttctttgacgtttactttcataatttcctggcgttttaactagcaattcctcagactcaagggcaggccgtggagagacttccggagccacaggcacagacaaggtcagctgcggcaactcagcatgtccacctccaagttctgactgagccaaggggccctccaaaaacggagcctccctttcaagaactggaggctcttctttggttgaaatcaaagaattctcgtccacctgcttgttctgagcactagatcgacctcgggctagaaggctttcctcttcacagcgggaacttaccttgtgcacctgctcctgtaccttcttttgttttttcttaggagcaaatatctgatcatattcttctgtatattccaaaagccacttgcttggcttcctaaggcgtttcttctctgaccgcacagctggttcagggagctcagcctgtggtgtcaaactgggaattcctggctccttttccatgtcaccaatgctggcactggatttatcacaaacatttaaccgtggcccagctgaatctaagcagtcagcatgattttgctctgtcagtggttcctcaagtatgcttgctgaaggagttctatgctctggaaactcatcccgcccctcctgcacagggtcactaggaagtaagaccctaaaggcacactcagagttttctttctctttaaatctgttcatgcgcttacgaggtttagtgcgcctttggtttaaacgctgccaccgctttttaggcaccacttgatttacaccattgagttcatcattctcactgttcattacagagtccagctctgggccttttccgttttcaaaagagagtcctttttcagaaattttaccaggatcagattgcttaaccttgctatcgaaatgcacatcagaaaaatggtcaccatcttcacttgttaagtggcccattatctgaaggggatcctctttactaggatcttctgccccacctctcaatgaacctccacgttctcggtctccctgcagtacagcatcaagagtcacacttggaagctgattcagttttcttttgcgctcggtctttaaggctttacggttcactgtgttctttaccatttgggctgaaaaagcatctcgcaatttggatgaaggctttgatcgtccacagttgcgcctagtaacacagtctgaacgacttttaccagaagcagggaggtctctcttgtcggacagtaagccaggtagggaagcagacaactcgccagataatgcagagtcacccccactagggctaggattggcggagttctgagtgccatctccctttttctctgaattgtgtgtggagcctcctgaaaccaaaaccttagagactcctacaggactattagtagaacagtccccacgaccaggactccggtaagagaccaggttttgagcagtcatcaaccgctgctccttcgtcttactatcatgcatatctttcaacatcattagcaatgtactgaatttgtagtctggttcaataggtatgtgattctgactagaagcagaagagaaaagtaatggttttgatggctttgatgttccagagtcactgacatcctcacctaaggatctgtaagagagttccttcaactcggataaaacatgtttcaccactgctgtttctatgtcacttgaatccctggttttctcatgcatattgttcagtagttttagaccatccactttcccacttttagaaatgctggccaaaggagagcctttggtatcagaagagcagcatttcaaactgcactcctcatttataactgggggttctgccataactggattttctttgtgtttgcactttatacttcggaacttgggctgtttgcttttcgaatgtaatagagcttgatttgctgccccaccctttattaacgagttctcactggatatgcttgatgacaggttgaattttggagagagagcatcatttgtaaaatctgactggggtttgtgaacaagagtagatgccttcagatcagagagattaacctgagacgtctcggttccaggctctgcactcttagtacaacccattaagtggtctgtatgtgagttactaatgagaggcttctgttttgcttttaccctagtgtttgtggcagcaaacctagaatactttatcttttcatttttctgcatagataacatgttctctgttctatcgaaagcatctggaatttcaaggacactgttatcagactctgagctgtgttctatgggatccaggtcactgcttccatcatcagaagtggtacagatactaatggaatcacttcgcttttcctcatcacctgctccaatatagcagagcttcacttttgaaccacacaccaggcttcgttggggtttattcttctctcgagaacactttgagatcaaagcaccctcaggcaagcccaataaagagtcaccatttgaagtctcaaattctttctttgcagtgttttttccacaggaagaaaacagaaaacttcctggggcagtgttggaccctgtgaggctatttgctatcctggaaagttcattagaggcctgcgtatcagatatatccccagagataaagtttaggccaaggttctctggaatctttcccctccgttcatctttatgtgcttcaaattgtatgtggccctttttcacactagtcctttttggattatcagagctctttctggctcgagatttagcgcaaggcttttccttctcatctgcagaatgttcagaatcaaaagccagtgatttcaaacagccattaagcaacaggtcatgttctgactcaggatcatttgtgcagtcttcaaatggcatatcttcttcactgtccaacttgattgaaccaggaatacattttcggttctttgaccccttgggaacatcatactgttctgcaagtccaacactggcttcccatttactcaaaattttctgaggaaccttatgcctatatcctttttctttctgtttccctcttctcctaaggacaggtagctcttcgaattgatgtctgccttcaaacatgacgattgcttttccagccacccaggctctctcagaaggatctccaaaagcctccacgtagtactgccgatagggcctccggttggaaactttcatttttgaatgtgtgttaatcaacggatcagaacaaatcctgcagggccaccatgggcgtctcttgaattttgcccagatgagatctccaacttcatacttcagtggcgtagactttttcttaggttgacaaaatggcaattcctgtgaagtagatgatgatgaagttccaggtaattctagcatgtttcctaatgtactggtactggaatctggatcatccgaaagggctgtccttgtcttcaggggcatctaaattcactggattggaaaagggcagcagacaatttcttctgggtagttcacaggtctgatccatcctgggccggcatcaaccgtgccccgcgccccctcccgggccagctggggggagggggtgaccctcattacactggggtgcgagcggagcggtggggagagagcggggccgctcgccgcacccccctccccccgcgtctctcttcaggggagaaggcagcgagcgcgacctgccccggcctattccgccgccgcctcctcctcctcacacccccaccgcgcgcgcc

SEQ ID NO: 17921 - RNA, 7220 nt, Homo sapiens
  source 1..7220: mol_type = other RNA
tcggggcatgggggagggaggctggggccttcccgagagacctaaaagattgcccactcttggcggcaagtgcaggtagttgctggcctccgaccatctgcttcgcctgcttcaccaggcccggggattggctaagaggccctggggtctgctcagcccctgcagaagctcttcctgaggcctgagttgttggctcatataaaaaggccttggcaggaggctgagaaagaagtctggcctgggtgagtgatttaacagcttgccaggggtcctctgaaggggctgctgctttcccagatgtctgaagaggatctgacacacagcctttctcaacagctctcggcatatgccccagacctttgctggcaggccatgaacttgactccaacactggcatcttctcatcagcctgtggtgtgacctgatgaggtgaagctgcccgctccttctggcgaggagttaggtctatgagatccatcaccaaagcagctctattttttgactgagtattctggtccacaggcctcagtgctttttctttagctacaagggtctggaccacagctgatagtactttctcaggaggtgggagtctctgggacaaagaggcatggggtttgtcagtaggcctgtctgaagtctggggtttgggactgctagtaatgagcagtctgtctggcggcggaagtctcaggccagtgggaactgaggttttctccagtgactggggccttgggctggcagcacctatggatttatccagccttgggtcagccgtccccagaggtctttccagtggttgggacctgactgagggtgaggagcttgggctggtcactggagagggtttgtcgcttagctggggtcttggtcctgccactgctggtggcctgtccagtggcctctggctggaaaccaaggattgggatttggtccctgacccagcgaggtctctgaccttatctaaaggctggggcctggagtcagttctctcaagaggtctttcaggtagcaatggcctctgacaagtccctgccagagcttttttggagagcgacagcatctggttggtgtcagcaggaggtttatctgacattttgggtgcctgagcagccattcctgttgattgctctgccaggtgagtgcttggccctggaggcagcggtactgggggaggcacatactcacggatctccccaggttccagaggattgggcccacaggggtcatgctcagtacaagacagacgcccatccagtttggaaatgaaaagcatcccttctcgatgctgcttacaaaaggagctggggcacatctcacagaaggaggctgcttccttcccgcagatgtcacactgatgccacggacattcccatttccctgctggtcgcttggtcagattgagacagtctgcgtggtaaacttttgggcagcctggtttcttgcaggagacgagctggccagcatccccacaactaaaacactcatcttctcgctcctttgtgatttcaccctgggtcctgcgctttccctgttgcttcttcttgaatttctttgacttttcttccgtggcaatgggttgattctttggccttacacccaagaagccactgcagttcggggctccacatttgcaaacagtctttccattcccaagacattctaggttgtagttgaaggtaagttcagtgcctgctttaatgtcacttagtgcaaaaaggcctacacgggtatctccattcacagaccacttctgtgtttcacagttgggctggcagcaatgattcatgaaccgagcatagtttcctttgggaccagcatcaatgattcggtctttgtctagggtgagcatatagaaattagtgatatcatgttcttgagcatagcgaattcgagctctgcattcttcttcatctataagctcacccacatactcattcacaaattcaccctttttaatatctgtttttgtccgtagaccccaaccccgctgtaatgtgcggaaaatttcaacctctggatattggcgcttggaaaagcactggttttgacagcgccctccggcaggacacactgtggggtggcactcatagagcagcatgcggttgatgcattcagagtctatcccacaggggttctcatcagtagctttacagttgcaacggggtatttcagataagtctgcagtgaagatctgtaccctgccaataggacggtttacctttatatgtttataaggtggtggcttcttgtcattctttcggtcttcctgcagctgtcttagctctttttgggcctttaattcctcaaaccttgctgcagcttcctgaagagcttttttatatgtcccatccactcctttgcccatcttatccttgctgctcacgtcaccctccatgtaagggaagactcgggcctggtgagtccacaaatagtcattagatccaaaaaagaggactgggaactctcccacatcatgtctcatcttatcaatgttggaaggaacagctcgaggatggcagatctcagctggccaccacctgtatcgtccaacttttacccagacaatctccctgtagtgtggctttttgcctgctttacagtcattgcaataccagtttccttcagggatatcaatgttcaggcattcacgatgaaaagcagcagggcaagaatcacagcacagaaggctgcctccttctgagcacacaaagcaccagctaacattaacatgctcatgatttcggcagccccgcctaggggtaaagtgattagggcagatgatactattagatgcaaggatctttgacccagcagccaggcaaaagtcattggcgtggtatgccacaggacagcggacacagcgcatcaaccgacctttagatgcagaaacattggctggattagcagcatgacaggttatacagatgtggagggagcaccggaagcccttgttctgcataacagtgggtgggtacttctggacacactcttcatggtaaaactttccacacaagggtagaaggcaccttttaacatcttccccactctgcttacatacaaaacaggtatggattcctgtgcgacattcattgcagataaattttcctcttggcatctcagtcaatccaaggcactccaggtggaaagccccacagcactgagcctcacataacagcagctcacccaatttttcacaattctgacagacattctccttgagtgcagctcctccaccgcgttcaccctgcatttttttagaggcaggcatcccgggatcgtgttctacaccttcctcaacagtctccttggggcttgtggccgtcctgtgaggcattagttctccctctgagcctggaatctcttttgacgagtcatcatttttcacttttttacactgcatcttggctgcagcatgcctctgtcgttttcgcttccttggcttgtcaaatatcttggtagtgcctccaccaaaatcttttgaataagatgtggcacaagattcagttatgccattctccaggtgaccagcttcatagcactttttagaaaggccaaggtcccccttcttgggcataaatccagggtctaaatcattggattcaagaagtttcttagttggttttctttgacgtttactttcataatttcctggcgttttaactagcaattcctcagactcaagggcaggccgtggagagacttccggagccacaggcacagacaaggtcagctgcggcaactcagcatgtccacctccaagttctgactgagccaaggggccctccaaaaacggagcctccctttcaagaactggaggctcttctttggttgaaatcaaagaattctcgtccacctgcttgttctgagcactagatcgacctcgggctagaaggctttcctcttcacagcgggaacttaccttgtgcacctgctcctgtaccttcttttgttttttcttaggagcaaatatctgatcatattcttctgtatattccaaaagccacttgcttggcttcctaaggcgtttcttctctgaccgcacagctggttcagggagctcagcctgtggtgtcaaactgggaattcctggctccttttccatgtcaccaatgctggcactggatttatcacaaacatttaaccgtggcccagctgaatctaagcagtcagcatgattttgctctgtcagtggttcctcaagtatgcttgctgaaggagttctatgctctggaaactcatcccgcccctcctgcacagggtcactaggaagtaagaccctaaaggcacactcagagttttctttctctttaaatctgttcatgcgcttacgaggtttagtgcgcctttggtttaaacgctgccaccgctttttaggcaccacttgatttacaccattgagttcatcattctcactgttcattacagagtccagctctgggccttttccgttttcaaaagagagtcctttttcagaaattttaccaggatcagattgcttaaccttgctatcgaaatgcacatcagaaaaatggtcaccatcttcacttgttaagtggcccattatctgaaggggatcctctttactaggatcttctgccccacctctcaatgaacctccacgttctcggtctccctgcagtacagcatcaagagtcacacttggaagctgattcagttttcttttgcgctcggtctttaaggctttacggttcactgtgttctttaccatttgggctgaaaaagcatctcgcaatttggatgaaggctttgatcgtccacagttgcgcctagtaacacagtctgaacgacttttaccagaagcagggaggtctctcttgtcggacagtaagccaggtagggaagcagacaactcgccagataatgcagagtcacccccactagggctaggattggcggagttctgagtgccatctccctttttctctgaattgtgtgtggagcctcctgaaaccaaaaccttagagactcctacaggactattagtagaacagtccccacgaccaggactccggtaagagaccaggttttgagcagtcatcaaccgctgctccttcgtcttactatcatgcatatctttcaacatcattagcaatgtactgaatttgtagtctggttcaataggtatgtgattctgactagaagcagaagagaaaagtaatggttttgatggctttgatgttccagagtcactgacatcctcacctaaggatctgtaagagagttccttcaactcggataaaacatgtttcaccactgctgtttctatgtcacttgaatccctggttttctcatgcatattgttcagtagttttagaccatccactttcccacttttagaaatgctggccaaaggagagcctttggtatcagaagagcagcatttcaaactgcactcctcatttataactgggggttctgccataactggattttctttgtgtttgcactttatacttcggaacttgggctgtttgcttttcgaatgtaatagagcttgatttgctgccccaccctttattaacgagttctcactggatatgcttgatgacaggttgaattttggagagagagcatcatttgtaaaatctgactggggtttgtgaacaagagtagatgccttcagatcagagagattaacctgagacgtctcggttccaggctctgcactcttagtacaacccattaagtggtctgtatgtgagttactaatgagaggcttctgttttgcttttaccctagtgtttgtggcagcaaacctagaatactttatcttttcatttttctgcatagataacatgttctctgttctatcgaaagcatctggaatttcaaggacactgttatcagactctgagctgtgttctatgggatccaggtcactgcttccatcatcagaagtggtacagatactaatggaatcacttcgcttttcctcatcacctgctccaatatagcagagcttcacttttgaaccacacaccaggcttcgttggggtttattcttctctcgagaacactttgagatcaaagcaccctcaggcaagcccaataaagagtcaccatttgaagtctcaaattctttctttgcagtgttttttccacaggaagaaaacagaaaacttcctggggcagtgttggaccctgtgaggctatttgctatcctggaaagttcattagaggcctgcgtatcagatatatccccagagataaagtttaggccaaggttctctggaatctttcccctccgttcatctttatgtgcttcaaattgtatgtggccctttttcacactagtcctttttggattatcagagctctttctggctcgagatttagcgcaaggcttttccttctcatctgcagaatgttcagaatcaaaagccagtgatttcaaacagccattaagcaacaggtcatgttctgactcaggatcatttgtgcagtcttcaaatggcatatcttcttcactgtccaacttgattgaaccaggaatacattttcggttctttgaccccttgggaacatcatactgttctgcaagtccaacactggcttcccatttactcaaaattttctgaggaaccttatgcctatatcctttttctttctgtttccctcttctcctaaggacaggtagctcttcgaattgatgtctgccttcaaacatgacgattgcttttccagccacccaggctctctcagaaggatctccaaaagcctccacgtagtactgccgatagggcctccggttggaaactttcatttttgaatgtgtgttaatcaacggatcagaacaaatcctgcagggccaccatgggcgtctcttgaattttgcccagatgagatctccaacttcatacttcagtggcgtagactttttcttaggttgacaaaatggcaattcctgtgaagtagatgatgatgaagttccaggtaattctagcatgtttcctaatgtactggtactggaatctggatcatccgaaagggctgtccttgtcttcaggggcatctaaattcactggattggaaaagggcagcagacaatttcttctgggtagttcacaggtctgatccatcctgggccggcatcaacctcaggagttacctggtccctagggcgctaagcgccttctcgctgttcagagaaagccggatccggccgccataaaaattccgcctcctccagaaagcct

SEQ ID NO: 17922 - RNA, 7137 nt, Homo sapiens
  source 1..7137: mol_type = other RNA
tcggggcatgggggagggaggctggggccttcccgagagacctaaaagattgcccactcttggcggcaagtgcaggtagttgctggcctccgaccatctgcttcgcctgcttcaccaggcccggggattggctaagaggccctggggtctgctcagcccctgcagaagctcttcctgaggcctgagttgttggctcatataaaaaggccttggcaggaggctgagaaagaagtctggcctgggtgagtgatttaacagcttgccaggggtcctctgaaggggctgctgctttcccagatgtctgaagaggatctgacacacagcctttctcaacagctctcggcatatgccccagacctttgctggcaggccatgaacttgactccaacactggcatcttctcatcagcctgtggtgtgacctgatgaggtgaagctgcccgctccttctggcgaggagttaggtctatgagatccatcaccaaagcagctctattttttgactgagtattctggtccacaggcctcagtgctttttctttagctacaagggtctggaccacagctgatagtactttctcaggaggtgggagtctctgggacaaagaggcatggggtttgtcagtaggcctgtctgaagtctggggtttgggactgctagtaatgagcagtctgtctggcggcggaagtctcaggccagtgggaactgaggttttctccagtgactggggccttgggctggcagcacctatggatttatccagccttgggtcagccgtccccagaggtctttccagtggttgggacctgactgagggtgaggagcttgggctggtcactggagagggtttgtcgcttagctggggtcttggtcctgccactgctggtggcctgtccagtggcctctggctggaaaccaaggattgggatttggtccctgacccagcgaggtctctgaccttatctaaaggctggggcctggagtcagttctctcaagaggtctttcaggtagcaatggcctctgacaagtccctgccagagcttttttggagagcgacagcatctggttggtgtcagcaggaggtttatctgacattttgggtgcctgagcagccattcctgttgattgctctgccaggtgagtgcttggccctggaggcagcggtactgggggaggcacatactcacggatctccccaggttccagaggattgggcccacaggggtcatgctcagtacaagacagacgcccatccagtttggaaatgaaaagcatcccttctcgatgctgcttacaaaaggagctggggcacatctcacagaaggaggctgcttccttcccgcagatgtcacactgatgccacggacattcccatttccctgctggtcgcttggtcagattgagacagtctgcgtggtaaacttttgggcagcctggtttcttgcaggagacgagctggccagcatccccacaactaaaacactcatcttctcgctcctttgtgatttcaccctgggtcctgcgctttccctgttgcttcttcttgaatttctttgacttttcttccgtggcaatgggttgattctttggccttacacccaagaagccactgcagttcggggctccacatttgcaaacagtctttccattcccaagacattctaggttgtagttgaaggtaagttcagtgcctgctttaatgtcacttagtgcaaaaaggcctacacgggtatctccattcacagaccacttctgtgtttcacagttgggctggcagcaatgattcatgaaccgagcatagtttcctttgggaccagcatcaatgattcggtctttgtctagggtgagcatatagaaattagtgatatcatgttcttgagcatagcgaattcgagctctgcattcttcttcatctataagctcacccacatactcattcacaaattcaccctttttaatatctgtttttgtccgtagaccccaaccccgctgtaatgtgcggaaaatttcaacctctggatattggcgcttggaaaagcactggttttgacagcgccctccggcaggacacactgtggggtggcactcatagagcagcatgcggttgatgcattcagagtctatcccacaggggttctcatcagtagctttacagttgcaacggggtatttcagataagtctgcagtgaagatctgtaccctgccaataggacggtttacctttatatgtttataaggtggtggcttcttgtcattctttcggtcttcctgcagctgtcttagctctttttgggcctttaattcctcaaaccttgctgcagcttcctgaagagcttttttatatgtcccatccactcctttgcccatcttatccttgctgctcacgtcaccctccatgtaagggaagactcgggcctggtgagtccacaaatagtcattagatccaaaaaagaggactgggaactctcccacatcatgtctcatcttatcaatgttggaaggaacagctcgaggatggcagatctcagctggccaccacctgtatcgtccaacttttacccagacaatctccctgtagtgtggctttttgcctgctttacagtcattgcaataccagtttccttcagggatatcaatgttcaggcattcacgatgaaaagcagcagggcaagaatcacagcacagaaggctgcctccttctgagcacacaaagcaccagctaacattaacatgctcatgatttcggcagccccgcctaggggtaaagtgattagggcagatgatactattagatgcaaggatctttgacccagcagccaggcaaaagtcattggcgtggtatgccacaggacagcggacacagcgcatcaaccgacctttagatgcagaaacattggctggattagcagcatgacaggttatacagatgtggagggagcaccggaagcccttgttctgcataacagtgggtgggtacttctggacacactcttcatggtaaaactttccacacaagggtagaaggcaccttttaacatcttccccactctgcttacatacaaaacaggtatggattcctgtgcgacattcattgcagataaattttcctcttggcatctcagtcaatccaaggcactccaggtggaaagccccacagcactgagcctcacataacagcagctcacccaatttttcacaattctgacagacattctccttgagtgcagctcctccaccgcgttcaccctgcatttttttagaggcaggcatcccgggatcgtgttctacaccttcctcaacagtctccttggggcttgtggccgtcctgtgaggcattagttctccctctgagcctggaatctcttttgacgagtcatcatttttcacttttttacactgcatcttggctgcagcatgcctctgtcgttttcgcttccttggcttgtcaaatatcttggtagtgcctccaccaaaatcttttgaataagatgtggcacaagattcagttatgccattctccaggtgaccagcttcatagcactttttagaaaggccaaggtcccccttcttgggcataaatccagggtctaaatcattggattcaagaagtttcttagttggttttctttgacgtttactttcataatttcctggcgttttaactagcaattcctcagactcaagggcaggccgtggagagacttccggagccacaggcacagacaaggtcagctgcggcaactcagcatgtccacctccaagttctgactgagccaaggggccctccaaaaacggagcctccctttcaagaactggaggctcttctttggttgaaatcaaagaattctcgtccacctgcttgttctgagcactagatcgacctcgggctagaaggctttcctcttcacagcgggaacttaccttgtgcacctgctcctgtaccttcttttgttttttcttaggagcaaatatctgatcatattcttctgtatattccaaaagccacttgcttggcttcctaaggcgtttcttctctgaccgcacagctggttcagggagctcagcctgtggtgtcaaactgggaattcctggctccttttccatgtcaccaatgctggcactggatttatcacaaacatttaaccgtggcccagctgaatctaagcagtcagcatgattttgctctgtcagtggttcctcaagtatgcttgctgaaggagttctatgctctggaaactcatcccgcccctcctgcacagggtcactaggaagtaagaccctaaaggcacactcagagttttctttctctttaaatctgttcatgcgcttacgaggtttagtgcgcctttggtttaaacgctgccaccgctttttaggcaccacttgatttacaccattgagttcatcattctcactgttcattacagagtccagctctgggccttttccgttttcaaaagagagtcctttttcagaaattttaccaggatcagattgcttaaccttgctatcgaaatgcacatcagaaaaatggtcaccatcttcacttgttaagtggcccattatctgaaggggatcctctttactaggatcttctgccccacctctcaatgaacctccacgttctcggtctccctgcagtacagcatcaagagtcacacttggaagctgattcagttttcttttgcgctcggtctttaaggctttacggttcactgtgttctttaccatttgggctgaaaaagcatctcgcaatttggatgaaggctttgatcgtccacagttgcgcctagtaacacagtctgaacgacttttaccagaagcagggaggtctctcttgtcggacagtaagccaggtagggaagcagacaactcgccagataatgcagagtcacccccactagggctaggattggcggagttctgagtgccatctccctttttctctgaattgtgtgtggagcctcctgaaaccaaaaccttagagactcctacaggactattagtagaacagtccccacgaccaggactccggtaagagaccaggttttgagcagtcatcaaccgctgctccttcgtcttactatcatgcatatctttcaacatcattagcaatgtactgaatttgtagtctggttcaataggtatgtgattctgactagaagcagaagagaaaagtaatggttttgatggctttgatgttccagagtcactgacatcctcacctaaggatctgtaagagagttccttcaactcggataaaacatgtttcaccactgctgtttctatgtcacttgaatccctggttttctcatgcatattgttcagtagttttagaccatccactttcccacttttagaaatgctggccaaaggagagcctttggtatcagaagagcagcatttcaaactgcactcctcatttataactgggggttctgccataactggattttctttgtgtttgcactttatacttcggaacttgggctgtttgcttttcgaatgtaatagagcttgatttgctgccccaccctttattaacgagttctcactggatatgcttgatgacaggttgaattttggagagagagcatcatttgtaaaatctgactggggtttgtgaacaagagtagatgccttcagatcagagagattaacctgagacgtctcggttccaggctctgcactcttagtacaacccattaagtggtctgtatgtgagttactaatgagaggcttctgttttgcttttaccctagtgtttgtggcagcaaacctagaatactttatcttttcatttttctgcatagataacatgttctctgttctatcgaaagcatctggaatttcaaggacactgttatcagactctgagctgtgttctatgggatccaggtcactgcttccatcatcagaagtggtacagatactaatggaatcacttcgcttttcctcatcacctgctccaatatagcagagcttcacttttgaaccacacaccaggcttcgttggggtttattcttctctcgagaacactttgagatcaaagcaccctcaggcaagcccaataaagagtcaccatttgaagtctcaaattctttctttgcagtgttttttccacaggaagaaaacagaaaacttcctggggcagtgttggaccctgtgaggctatttgctatcctggaaagttcattagaggcctgcgtatcagatatatccccagagataaagtttaggccaaggttctctggaatctttcccctccgttcatctttatgtgcttcaaattgtatgtggccctttttcacactagtcctttttggattatcagagctctttctggctcgagatttagcgcaaggcttttccttctcatctgcagaatgttcagaatcaaaagccagtgatttcaaacagccattaagcaacaggtcatgttctgactcaggatcatttgtgcagtcttcaaatggcatatcttcttcactgtccaacttgattgaaccaggaatacattttcggttctttgaccccttgggaacatcatactgttctgcaagtccaacactggcttcccatttactcaaaattttctgaggaaccttatgcctatatcctttttctttctgtttccctcttctcctaaggacaggtagctcttcgaattgatgtctgccttcaaacatgacgattgcttttccagccacccaggctctctcagaaggatctccaaaagcctccacgtagtactgccgatagggcctccggttggaaactttcatttttgaatgtgtgttaatcaacggatcagaacaaatcctgcagggccaccatgggcgtctcttgaattttgcccagatgagatctccaacttcatacttcagtggcgtagactttttcttaggttgacaaaatggcaattcctgtgaagtagatgatgatgaagttccaggtaattctagcatgtttcctaatgtactggtactggaatctggatcatccgaaagggctgtccttgtcttcaggggcatctaaattcactggattggaaaagggcagcagacaatttcttctgggtagttcacaggtctgatccatcctgggccggcatcaacctgaggggaggcggagg

SEQ ID NO: 17923 - RNA, 7260 nt, Homo sapiens
  source 1..7260: mol_type = other RNA
tcggggcatgggggagggaggctggggccttcccgagagacctaaaagattgcccactcttggcggcaagtgcaggtagttgctggcctccgaccatctgcttcgcctgcttcaccaggcccggggattggctaagaggccctggggtctgctcagcccctgcagaagctcttcctgaggcctgagttgttggctcatataaaaaggccttggcaggaggctgagaaagaagtctggcctgggtgagtgatttaacagcttgccaggggtcctctgaaggggctgctgctttcccagatgtctgaagaggatctgacacacagcctttctcaacagctctcggcatatgccccagacctttgctggcaggccatgaacttgactccaacactggcatcttctcatcagcctgtggtgtgacctgatgaggtgaagctgcccgctccttctggcgaggagttaggtctatgagatccatcaccaaagcagctctattttttgactgagtattctggtccacaggcctcagtgctttttctttagctacaagggtctggaccacagctgatagtactttctcaggaggtgggagtctctgggacaaagaggcatggggtttgtcagtaggcctgtctgaagtctggggtttgggactgctagtaatgagcagtctgtctggcggcggaagtctcaggccagtgggaactgaggttttctccagtgactggggccttgggctggcagcacctatggatttatccagccttgggtcagccgtccccagaggtctttccagtggttgggacctgactgagggtgaggagcttgggctggtcactggagagggtttgtcgcttagctggggtcttggtcctgccactgctggtggcctgtccagtggcctctggctggaaaccaaggattgggatttggtccctgacccagcgaggtctctgaccttatctaaaggctggggcctggagtcagttctctcaagaggtctttcaggtagcaatggcctctgacaagtccctgccagagcttttttggagagcgacagcatctggttggtgtcagcaggaggtttatctgacattttgggtgcctgagcagccattcctgttgattgctctgccaggtgagtgcttggccctggaggcagcggtactgggggaggcacatactcacggatctccccaggttccagaggattgggcccacaggggtcatgctcagtacaagacagacgcccatccagtttggaaatgaaaagcatcccttctcgatgctgcttacaaaaggagctggggcacatctcacagaaggaggctgcttccttcccgcagatgtcacactgatgccacggacattcccatttccctgctggtcgcttggtcagattgagacagtctgcgtggtaaacttttgggcagcctggtttcttgcaggagacgagctggccagcatccccacaactaaaacactcatcttctcgctcctttgtgatttcaccctgggtcctgcgctttccctgttgcttcttcttgaatttctttgacttttcttccgtggcaatgggttgattctttggccttacacccaagaagccactgcagttcggggctccacatttgcaaacagtctttccattcccaagacattctaggttgtagttgaaggtaagttcagtgcctgctttaatgtcacttagtgcaaaaaggcctacacgggtatctccattcacagaccacttctgtgtttcacagttgggctggcagcaatgattcatgaaccgagcatagtttcctttgggaccagcatcaatgattcggtctttgtctagggtgagcatatagaaattagtgatatcatgttcttgagcatagcgaattcgagctctgcattcttcttcatctataagctcacccacatactcattcacaaattcaccctttttaatatctgtttttgtccgtagaccccaaccccgctgtaatgtgcggaaaatttcaacctctggatattggcgcttggaaaagcactggttttgacagcgccctccggcaggacacactgtggggtggcactcatagagcagcatgcggttgatgcattcagagtctatcccacaggggttctcatcagtagctttacagttgcaacggggtatttcagataagtctgcagtgaagatctgtaccctgccaataggacggtttacctttatatgtttataaggtggtggcttcttgtcattctttcggtcttcctgcagctgtcttagctctttttgggcctttaattcctcaaaccttgctgcagcttcctgaagagcttttttatatgtcccatccactcctttgcccatcttatccttgctgctcacgtcaccctccatgtaagggaagactcgggcctggtgagtccacaaatagtcattagatccaaaaaagaggactgggaactctcccacatcatgtctcatcttatcaatgttggaaggaacagctcgaggatggcagatctcagctggccaccacctgtatcgtccaacttttacccagacaatctccctgtagtgtggctttttgcctgctttacagtcattgcaataccagtttccttcagggatatcaatgttcaggcattcacgatgaaaagcagcagggcaagaatcacagcacagaaggctgcctccttctgagcacacaaagcaccagctaacattaacatgctcatgatttcggcagccccgcctaggggtaaagtgattagggcagatgatactattagatgcaaggatctttgacccagcagccaggcaaaagtcattggcgtggtatgccacaggacagcggacacagcgcatcaaccgacctttagatgcagaaacattggctggattagcagcatgacaggttatacagatgtggagggagcaccggaagcccttgttctgcataacagtgggtgggtacttctggacacactcttcatggtaaaactttccacacaagggtagaaggcaccttttaacatcttccccactctgcttacatacaaaacaggtatggattcctgtgcgacattcattgcagataaattttcctcttggcatctcagtcaatccaaggcactccaggtggaaagccccacagcactgagcctcacataacagcagctcacccaatttttcacaattctgacagacattctccttgagtgcagctcctccaccgcgttcaccctgcatttttttagaggcaggcatcccgggatcgtgttctacaccttcctcaacagtctccttggggcttgtggccgtcctgtgaggcattagttctccctctgagcctggaatctcttttgacgagtcatcatttttcacttttttacactgcatcttggctgcagcatgcctctgtcgttttcgcttccttggcttgtcaaatatcttggtagtgcctccaccaaaatcttttgaataagatgtggcacaagattcagttatgccattctccaggtgaccagcttcatagcactttttagaaaggccaaggtcccccttcttgggcataaatccagggtctaaatcattggattcaagaagtttcttagttggttttctttgacgtttactttcataatttcctggcgttttaactagcaattcctcagactcaagggcaggccgtggagagacttccggagccacaggcacagacaaggtcagctgcggcaactcagcatgtccacctccaagttctgactgagccaaggggccctccaaaaacggagcctccctttcaagaactggaggctcttctttggttgaaatcaaagaattctcgtccacctgcttgttctgagcactagatcgacctcgggctagaaggctttcctcttcacagcgggaacttaccttgtgcacctgctcctgtaccttcttttgttttttcttaggagcaaatatctgatcatattcttctgtatattccaaaagccacttgcttggcttcctaaggcgtttcttctctgaccgcacagctggttcagggagctcagcctgtggtgtcaaactgggaattcctggctccttttccatgtcaccaatgctggcactggatttatcacaaacatttaaccgtggcccagctgaatctaagcagtcagcatgattttgctctgtcagtggttcctcaagtatgcttgctgaaggagttctatgctctggaaactcatcccgcccctcctgcacagggtcactaggaagtaagaccctaaaggcacactcagagttttctttctctttaaatctgttcatgcgcttacgaggtttagtgcgcctttggtttaaacgctgccaccgctttttaggcaccacttgatttacaccattgagttcatcattctcactgttcattacagagtccagctctgggccttttccgttttcaaaagagagtcctttttcagaaattttaccaggatcagattgcttaaccttgctatcgaaatgcacatcagaaaaatggtcaccatcttcacttgttaagtggcccattatctgaaggggatcctctttactaggatcttctgccccacctctcaatgaacctccacgttctcggtctccctgcagtacagcatcaagagtcacacttggaagctgattcagttttcttttgcgctcggtctttaaggctttacggttcactgtgttctttaccatttgggctgaaaaagcatctcgcaatttggatgaaggctttgatcgtccacagttgcgcctagtaacacagtctgaacgacttttaccagaagcagggaggtctctcttgtcggacagtaagccaggtagggaagcagacaactcgccagataatgcagagtcacccccactagggctaggattggcggagttctgagtgccatctccctttttctctgaattgtgtgtggagcctcctgaaaccaaaaccttagagactcctacaggactattagtagaacagtccccacgaccaggactccggtaagagaccaggttttgagcagtcatcaaccgctgctccttcgtcttactatcatgcatatctttcaacatcattagcaatgtactgaatttgtagtctggttcaataggtatgtgattctgactagaagcagaagagaaaagtaatggttttgatggctttgatgttccagagtcactgacatcctcacctaaggatctgtaagagagttccttcaactcggataaaacatgtttcaccactgctgtttctatgtcacttgaatccctggttttctcatgcatattgttcagtagttttagaccatccactttcccacttttagaaatgctggccaaaggagagcctttggtatcagaagagcagcatttcaaactgcactcctcatttataactgggggttctgccataactggattttctttgtgtttgcactttatacttcggaacttgggctgtttgcttttcgaatgtaatagagcttgatttgctgccccaccctttattaacgagttctcactggatatgcttgatgacaggttgaattttggagagagagcatcatttgtaaaatctgactggggtttgtgaacaagagtagatgccttcagatcagagagattaacctgagacgtctcggttccaggctctgcactcttagtacaacccattaagtggtctgtatgtgagttactaatgagaggcttctgttttgcttttaccctagtgtttgtggcagcaaacctagaatactttatcttttcatttttctgcatagataacatgttctctgttctatcgaaagcatctggaatttcaaggacactgttatcagactctgagctgtgttctatgggatccaggtcactgcttccatcatcagaagtggtacagatactaatggaatcacttcgcttttcctcatcacctgctccaatatagcagagcttcacttttgaaccacacaccaggcttcgttggggtttattcttctctcgagaacactttgagatcaaagcaccctcaggcaagcccaataaagagtcaccatttgaagtctcaaattctttctttgcagtgttttttccacaggaagaaaacagaaaacttcctggggcagtgttggaccctgtgaggctatttgctatcctggaaagttcattagaggcctgcgtatcagatatatccccagagataaagtttaggccaaggttctctggaatctttcccctccgttcatctttatgtgcttcaaattgtatgtggccctttttcacactagtcctttttggattatcagagctctttctggctcgagatttagcgcaaggcttttccttctcatctgcagaatgttcagaatcaaaagccagtgatttcaaacagccattaagcaacaggtcatgttctgactcaggatcatttgtgcagtcttcaaatggcatatcttcttcactgtccaacttgattgaaccaggaatacattttcggttctttgaccccttgggaacatcatactgttctgcaagtccaacactggcttcccatttactcaaaattttctgaggaaccttatgcctatatcctttttctttctgtttccctcttctcctaaggacaggtagctcttcgaattgatgtctgccttcaaacatgacgattgcttttccagccacccaggctctctcagaaggatctccaaaagcctccacgtagtactgccgatagggcctccggttggaaactttcatttttgaatgtgtgttaatcaacggatcagaacaaatcctgcagggccaccatgggcgtctcttgaattttgcccagatgagatctccaacttcatacttcagtggcgtagactttttcttaggttgacaaaatggcaattcctgtgaagtagatgatgatgaagttccaggtaattctagcatgtttcctaatgtactggtactggaatctggatcatccgaaagggctgtccttgtcttcaggggcatctaaattcactggattggaaaagggcagcagacaatttcttctgggtagttcacaggtctgatccatcctgggccggcatcaacctgggggcttgggctggggtcttcgaggcctcaggccccgagcagacgcggccgcaggcgaaccccctacccggccgcaccccaaacccacaccaccaccaccaccaccaccacagaccaagctgagcaggaaacaaaat

SEQ ID NO: 17924 - RNA, 7176 nt, Homo sapiens
  source 1..7176: mol_type = other RNA
tcggggcatgggggagggaggctggggccttcccgagagacctaaaagattgcccactcttggcggcaagtgcaggtagttgctggcctccgaccatctgcttcgcctgcttcaccaggcccggggattggctaagaggccctggggtctgctcagcccctgcagaagctcttcctgaggcctgagttgttggctcatataaaaaggccttggcaggaggctgagaaagaagtctggcctgggtgagtgatttaacagcttgccaggggtcctctgaaggggctgctgctttcccagatgtctgaagaggatctgacacacagcctttctcaacagctctcggcatatgccccagacctttgctggcaggccatgaacttgactccaacactggcatcttctcatcagcctgtggtgtgacctgatgaggtgaagctgcccgctccttctggcgaggagttaggtctatgagatccatcaccaaagcagctctattttttgactgagtattctggtccacaggcctcagtgctttttctttagctacaagggtctggaccacagctgatagtactttctcaggaggtgggagtctctgggacaaagaggcatggggtttgtcagtaggcctgtctgaagtctggggtttgggactgctagtaatgagcagtctgtctggcggcggaagtctcaggccagtgggaactgaggttttctccagtgactggggccttgggctggcagcacctatggatttatccagccttgggtcagccgtccccagaggtctttccagtggttgggacctgactgagggtgaggagcttgggctggtcactggagagggtttgtcgcttagctggggtcttggtcctgccactgctggtggcctgtccagtggcctctggctggaaaccaaggattgggatttggtccctgacccagcgaggtctctgaccttatctaaaggctggggcctggagtcagttctctcaagaggtctttcaggtagcaatggcctctgacaagtccctgccagagcttttttggagagcgacagcatctggttggtgtcagcaggaggtttatctgacattttgggtgcctgagcagccattcctgttgattgctctgccaggtgagtgcttggccctggaggcagcggtactgggggaggcacatactcacggatctccccaggttccagaggattgggcccacaggggtcatgctcagtacaagacagacgcccatccagtttggaaatgaaaagcatcccttctcgatgctgcttacaaaaggagctggggcacatctcacagaaggaggctgcttccttcccgcagatgtcacactgatgccacggacattcccatttccctgctggtcgcttggtcagattgagacagtctgcgtggtaaacttttgggcagcctggtttcttgcaggagacgagctggccagcatccccacaactaaaacactcatcttctcgctcctttgtgatttcaccctgggtcctgcgctttccctgttgcttcttcttgaatttctttgacttttcttccgtggcaatgggttgattctttggccttacacccaagaagccactgcagttcggggctccacatttgcaaacagtctttccattcccaagacattctaggttgtagttgaaggtaagttcagtgcctgctttaatgtcacttagtgcaaaaaggcctacacgggtatctccattcacagaccacttctgtgtttcacagttgggctggcagcaatgattcatgaaccgagcatagtttcctttgggaccagcatcaatgattcggtctttgtctagggtgagcatatagaaattagtgatatcatgttcttgagcatagcgaattcgagctctgcattcttcttcatctataagctcacccacatactcattcacaaattcaccctttttaatatctgtttttgtccgtagaccccaaccccgctgtaatgtgcggaaaatttcaacctctggatattggcgcttggaaaagcactggttttgacagcgccctccggcaggacacactgtggggtggcactcatagagcagcatgcggttgatgcattcagagtctatcccacaggggttctcatcagtagctttacagttgcaacggggtatttcagataagtctgcagtgaagatctgtaccctgccaataggacggtttacctttatatgtttataaggtggtggcttcttgtcattctttcggtcttcctgcagctgtcttagctctttttgggcctttaattcctcaaaccttgctgcagcttcctgaagagcttttttatatgtcccatccactcctttgcccatcttatccttgctgctcacgtcaccctccatgtaagggaagactcgggcctggtgagtccacaaatagtcattagatccaaaaaagaggactgggaactctcccacatcatgtctcatcttatcaatgttggaaggaacagctcgaggatggcagatctcagctggccaccacctgtatcgtccaacttttacccagacaatctccctgtagtgtggctttttgcctgctttacagtcattgcaataccagtttccttcagggatatcaatgttcaggcattcacgatgaaaagcagcagggcaagaatcacagcacagaaggctgcctccttctgagcacacaaagcaccagctaacattaacatgctcatgatttcggcagccccgcctaggggtaaagtgattagggcagatgatactattagatgcaaggatctttgacccagcagccaggcaaaagtcattggcgtggtatgccacaggacagcggacacagcgcatcaaccgacctttagatgcagaaacattggctggattagcagcatgacaggttatacagatgtggagggagcaccggaagcccttgttctgcataacagtgggtgggtacttctggacacactcttcatggtaaaactttccacacaagggtagaaggcaccttttaacatcttccccactctgcttacatacaaaacaggtatggattcctgtgcgacattcattgcagataaattttcctcttggcatctcagtcaatccaaggcactccaggtggaaagccccacagcactgagcctcacataacagcagctcacccaatttttcacaattctgacagacattctccttgagtgcagctcctccaccgcgttcaccctgcatttttttagaggcaggcatcccgggatcgtgttctacaccttcctcaacagtctccttggggcttgtggccgtcctgtgaggcattagttctccctctgagcctggaatctcttttgacgagtcatcatttttcacttttttacactgcatcttggctgcagcatgcctctgtcgttttcgcttccttggcttgtcaaatatcttggtagtgcctccaccaaaatcttttgaataagatgtggcacaagattcagttatgccattctccaggtgaccagcttcatagcactttttagaaaggccaaggtcccccttcttgggcataaatccagggtctaaatcattggattcaagaagtttcttagttggttttctttgacgtttactttcataatttcctggcgttttaactagcaattcctcagactcaagggcaggccgtggagagacttccggagccacaggcacagacaaggtcagctgcggcaactcagcatgtccacctccaagttctgactgagccaaggggccctccaaaaacggagcctccctttcaagaactggaggctcttctttggttgaaatcaaagaattctcgtccacctgcttgttctgagcactagatcgacctcgggctagaaggctttcctcttcacagcgggaacttaccttgtgcacctgctcctgtaccttcttttgttttttcttaggagcaaatatctgatcatattcttctgtatattccaaaagccacttgcttggcttcctaaggcgtttcttctctgaccgcacagctggttcagggagctcagcctgtggtgtcaaactgggaattcctggctccttttccatgtcaccaatgctggcactggatttatcacaaacatttaaccgtggcccagctgaatctaagcagtcagcatgattttgctctgtcagtggttcctcaagtatgcttgctgaaggagttctatgctctggaaactcatcccgcccctcctgcacagggtcactaggaagtaagaccctaaaggcacactcagagttttctttctctttaaatctgttcatgcgcttacgaggtttagtgcgcctttggtttaaacgctgccaccgctttttaggcaccacttgatttacaccattgagttcatcattctcactgttcattacagagtccagctctgggccttttccgttttcaaaagagagtcctttttcagaaattttaccaggatcagattgcttaaccttgctatcgaaatgcacatcagaaaaatggtcaccatcttcacttgttaagtggcccattatctgaaggggatcctctttactaggatcttctgccccacctctcaatgaacctccacgttctcggtctccctgcagtacagcatcaagagtcacacttggaagctgattcagttttcttttgcgctcggtctttaaggctttacggttcactgtgttctttaccatttgggctgaaaaagcatctcgcaatttggatgaaggctttgatcgtccacagttgcgcctagtaacacagtctgaacgacttttaccagaagcagggaggtctctcttgtcggacagtaagccaggtagggaagcagacaactcgccagataatgcagagtcacccccactagggctaggattggcggagttctgagtgccatctccctttttctctgaattgtgtgtggagcctcctgaaaccaaaaccttagagactcctacaggactattagtagaacagtccccacgaccaggactccggtaagagaccaggttttgagcagtcatcaaccgctgctccttcgtcttactatcatgcatatctttcaacatcattagcaatgtactgaatttgtagtctggttcaataggtatgtgattctgactagaagcagaagagaaaagtaatggttttgatggctttgatgttccagagtcactgacatcctcacctaaggatctgtaagagagttccttcaactcggataaaacatgtttcaccactgctgtttctatgtcacttgaatccctggttttctcatgcatattgttcagtagttttagaccatccactttcccacttttagaaatgctggccaaaggagagcctttggtatcagaagagcagcatttcaaactgcactcctcatttataactgggggttctgccataactggattttctttgtgtttgcactttatacttcggaacttgggctgtttgcttttcgaatgtaatagagcttgatttgctgccccaccctttattaacgagttctcactggatatgcttgatgacaggttgaattttggagagagagcatcatttgtaaaatctgactggggtttgtgaacaagagtagatgccttcagatcagagagattaacctgagacgtctcggttccaggctctgcactcttagtacaacccattaagtggtctgtatgtgagttactaatgagaggcttctgttttgcttttaccctagtgtttgtggcagcaaacctagaatactttatcttttcatttttctgcatagataacatgttctctgttctatcgaaagcatctggaatttcaaggacactgttatcagactctgagctgtgttctatgggatccaggtcactgcttccatcatcagaagtggtacagatactaatggaatcacttcgcttttcctcatcacctgctccaatatagcagagcttcacttttgaaccacacaccaggcttcgttggggtttattcttctctcgagaacactttgagatcaaagcaccctcaggcaagcccaataaagagtcaccatttgaagtctcaaattctttctttgcagtgttttttccacaggaagaaaacagaaaacttcctggggcagtgttggaccctgtgaggctatttgctatcctggaaagttcattagaggcctgcgtatcagatatatccccagagataaagtttaggccaaggttctctggaatctttcccctccgttcatctttatgtgcttcaaattgtatgtggccctttttcacactagtcctttttggattatcagagctctttctggctcgagatttagcgcaaggcttttccttctcatctgcagaatgttcagaatcaaaagccagtgatttcaaacagccattaagcaacaggtcatgttctgactcaggatcatttgtgcagtcttcaaatggcatatcttcttcactgtccaacttgattgaaccaggaatacattttcggttctttgaccccttgggaacatcatactgttctgcaagtccaacactggcttcccatttactcaaaattttctgaggaaccttatgcctatatcctttttctttctgtttccctcttctcctaaggacaggtagctcttcgaattgatgtctgccttcaaacatgacgattgcttttccagccacccaggctctctcagaaggatctccaaaagcctccacgtagtactgccgatagggcctccggttggaaactttcatttttgaatgtgtgttaatcaacggatcagaacaaatcctgcagggccaccatgggcgtctcttgaattttgcccagatgagatctccaacttcatacttcagtggcgtagactttttcttaggttgacaaaatggcaattcctgtgaagtagatgatgatgaagttccaggtaattctagcatgtttcctaatgtactggtactggaatctggatcatccgaaagggctgtccttgtcttcaggggcatctaaattcactggattggaaaagggcagcagacaatttcttctgggtagttcacaggtctgatccatcctgggccggcatcaactcttcggggttcagggcgggtgaagtcgggcttgtgagagcgccgcccaatcagcg

SEQ ID NO: 17925 - RNA, 8040 nt, Homo sapiens
  source 1..8040: mol_type = other RNA
tcggggcatgggggagggaggctggggccttcccgagagacctaaaagattgcccactcttggcggcaagtgcaggtagttgctggcctccgaccatctgcttcgcctgcttcaccaggcccggggattggctaagaggccctggggtctgctcagcccctgcagaagctcttcctgaggcctgagttgttggctcatataaaaaggccttggcaggaggctgagaaagaagtctggcctgggtgagtgatttaacagcttgccaggggtcctctgaaggggctgctgctttcccagatgtctgaagaggatctgacacacagcctttctcaacagctctcggcatatgccccagacctttgctggcaggccatgaacttgactccaacactggcatcttctcatcagcctgtggtgtgacctgatgaggtgaagctgcccgctccttctggcgaggagttaggtctatgagatccatcaccaaagcagctctattttttgactgagtattctggtccacaggcctcagtgctttttctttagctacaagggtctggaccacagctgatagtactttctcaggaggtgggagtctctgggacaaagaggcatggggtttgtcagtaggcctgtctgaagtctggggtttgggactgctagtaatgagcagtctgtctggcggcggaagtctcaggccagtgggaactgaggttttctccagtgactggggccttgggctggcagcacctatggatttatccagccttgggtcagccgtccccagaggtctttccagtggttgggacctgactgagggtgaggagcttgggctggtcactggagagggtttgtcgcttagctggggtcttggtcctgccactgctggtggcctgtccagtggcctctggctggaaaccaaggattgggatttggtccctgacccagcgaggtctctgaccttatctaaaggctggggcctggagtcagttctctcaagaggtctttcaggtagcaatggcctctgacaagtccctgccagagcttttttggagagcgacagcatctggttggtgtcagcaggaggtttatctgacattttgggtgcctgagcagccattcctgttgattgctctgccaggtgagtgcttggccctggaggcagcggtactgggggaggcacatactcacggatctccccaggttccagaggattgggcccacaggggtcatgctcagtacaagacagacgcccatccagtttggaaatgaaaagcatcccttctcgatgctgcttacaaaaggagctggggcacatctcacagaaggaggctgcttccttcccgcagatgtcacactgatgccacggacattcccatttccctgctggtcgcttggtcagattgagacagtctgcgtggtaaacttttgggcagcctggtttcttgcaggagacgagctggccagcatccccacaactaaaacactcatcttctcgctcctttgtgatttcaccctgggtcctgcgctttccctgttgcttcttcttgaatttctttgacttttcttccgtggcaatgggttgattctttggccttacacccaagaagccactgcagttcggggctccacatttgcaaacagtctttccattcccaagacattctaggttgtagttgaaggtaagttcagtgcctgctttaatgtcacttagtgcaaaaaggcctacacgggtatctccattcacagaccacttctgtgtttcacagttgggctggcagcaatgattcatgaaccgagcatagtttcctttgggaccagcatcaatgattcggtctttgtctagggtgagcatatagaaattagtgatatcatgttcttgagcatagcgaattcgagctctgcattcttcttcatctataagctcacccacatactcattcacaaattcaccctttttaatatctgtttttgtccgtagaccccaaccccgctgtaatgtgcggaaaatttcaacctctggatattggcgcttggaaaagcactggttttgacagcgccctccggcaggacacactgtggggtggcactcatagagcagcatgcggttgatgcattcagagtctatcccacaggggttctcatcagtagctttacagttgcaacggggtatttcagataagtctgcagtgaagatctgtaccctgccaataggacggtttacctttatatgtttataaggtggtggcttcttgtcattctttcggtcttcctgcagctgtcttagctctttttgggcctttaattcctcaaaccttgctgcagcttcctgaagagcttttttatatgtcccatccactcctttgcccatcttatccttgctgctcacgtcaccctccatgtaagggaagactcgggcctggtgagtccacaaatagtcattagatccaaaaaagaggactgggaactctcccacatcatgtctcatcttatcaatgttggaaggaacagctcgaggatggcagatctcagctggccaccacctgtatcgtccaacttttacccagacaatctccctgtagtgtggctttttgcctgctttacagtcattgcaataccagtttccttcagggatatcaatgttcaggcattcacgatgaaaagcagcagggcaagaatcacagcacagaaggctgcctccttctgagcacacaaagcaccagctaacattaacatgctcatgatttcggcagccccgcctaggggtaaagtgattagggcagatgatactattagatgcaaggatctttgacccagcagccaggcaaaagtcattggcgtggtatgccacaggacagcggacacagcgcatcaaccgacctttagatgcagaaacattggctggattagcagcatgacaggttatacagatgtggagggagcaccggaagcccttgttctgcataacagtgggtgggtacttctggacacactcttcatggtaaaactttccacacaagggtagaaggcaccttttaacatcttccccactctgcttacatacaaaacaggtatggattcctgtgcgacattcattgcagataaattttcctcttggcatctcagtcaatccaaggcactccaggtggaaagccccacagcactgagcctcacataacagcagctcacccaatttttcacaattctgacagacattctccttgagtgcagctcctccaccgcgttcaccctgcatttttttagaggcaggcatcccgggatcgtgttctacaccttcctcaacagtctccttggggcttgtggccgtcctgtgaggcattagttctccctctgagcctggaatctcttttgacgagtcatcatttttcacttttttacactgcatcttggctgcagcatgcctctgtcgttttcgcttccttggcttgtcaaatatcttggtagtgcctccaccaaaatcttttgaataagatgtggcacaagattcagttatgccattctccaggtgaccagcttcatagcactttttagaaaggccaaggtcccccttcttgggcataaatccagggtctaaatcattggattcaagaagtttcttagttggttttctttgacgtttactttcataatttcctggcgttttaactagcaattcctcagactcaagggcaggccgtggagagacttccggagccacaggcacagacaaggtcagctgcggcaactcagcatgtccacctccaagttctgactgagccaaggggccctccaaaaacggagcctccctttcaagaactggaggctcttctttggttgaaatcaaagaattctcgtccacctgcttgttctgagcactagatcgacctcgggctagaaggctttcctcttcacagcgggaacttaccttgtgcacctgctcctgtaccttcttttgttttttcttaggagcaaatatctgatcatattcttctgtatattccaaaagccacttgcttggcttcctaaggcgtttcttctctgaccgcacagctggttcagggagctcagcctgtggtgtcaaactgggaattcctggctccttttccatgtcaccaatgctggcactggatttatcacaaacatttaaccgtggcccagctgaatctaagcagtcagcatgattttgctctgtcagtggttcctcaagtatgcttgctgaaggagttctatgctctggaaactcatcccgcccctcctgcacagggtcactaggaagtaagaccctaaaggcacactcagagttttctttctctttaaatctgttcatgcgcttacgaggtttagtgcgcctttggtttaaacgctgccaccgctttttaggcaccacttgatttacaccattgagttcatcattctcactgttcattacagagtccagctctgggccttttccgttttcaaaagagagtcctttttcagaaattttaccaggatcagattgcttaaccttgctatcgaaatgcacatcagaaaaatggtcaccatcttcacttgttaagtggcccattatctgaaggggatcctctttactaggatcttctgccccacctctcaatgaacctccacgttctcggtctccctgcagtacagcatcaagagtcacacttggaagctgattcagttttcttttgcgctcggtctttaaggctttacggttcactgtgttctttaccatttgggctgaaaaagcatctcgcaatttggatgaaggctttgatcgtccacagttgcgcctagtaacacagtctgaacgacttttaccagaagcagggaggtctctcttgtcggacagtaagccaggtagggaagcagacaactcgccagataatgcagagtcacccccactagggctaggattggcggagttctgagtgccatctccctttttctctgaattgtgtgtggagcctcctgaaaccaaaaccttagagactcctacaggactattagtagaacagtccccacgaccaggactccggtaagagaccaggttttgagcagtcatcaaccgctgctccttcgtcttactatcatgcatatctttcaacatcattagcaatgtactgaatttgtagtctggttcaataggtatgtgattctgactagaagcagaagagaaaagtaatggttttgatggctttgatgttccagagtcactgacatcctcacctaaggatctgtaagagagttccttcaactcggataaaacatgtttcaccactgctgtttctatgtcacttgaatccctggttttctcatgcatattgttcagtagttttagaccatccactttcccacttttagaaatgctggccaaaggagagcctttggtatcagaagagcagcatttcaaactgcactcctcatttataactgggggttctgccataactggattttctttgtgtttgcactttatacttcggaacttgggctgtttgcttttcgaatgtaatagagcttgatttgctgccccaccctttattaacgagttctcactggatatgcttgatgacaggttgaattttggagagagagcatcatttgtaaaatctgactggggtttgtgaacaagagtagatgccttcagatcagagagattaacctgagacgtctcggttccaggctctgcactcttagtacaacccattaagtggtctgtatgtgagttactaatgagaggcttctgttttgcttttaccctagtgtttgtggcagcaaacctagaatactttatcttttcatttttctgcatagataacatgttctctgttctatcgaaagcatctggaatttcaaggacactgttatcagactctgagctgtgttctatgggatccaggtcactgcttccatcatcagaagtggtacagatactaatggaatcacttcgcttttcctcatcacctgctccaatatagcagagcttcacttttgaaccacacaccaggcttcgttggggtttattcttctctcgagaacactttgagatcaaagcaccctcaggcaagcccaataaagagtcaccatttgaagtctcaaattctttctttgcagtgttttttccacaggaagaaaacagaaaacttcctggggcagtgttggaccctgtgaggctatttgctatcctggaaagttcattagaggcctgcgtatcagatatatccccagagataaagtttaggccaaggttctctggaatctttcccctccgttcatctttatgtgcttcaaattgtatgtggccctttttcacactagtcctttttggattatcagagctctttctggctcgagatttagcgcaaggcttttccttctcatctgcagaatgttcagaatcaaaagccagtgatttcaaacagccattaagcaacaggtcatgttctgactcaggatcatttgtgcagtcttcaaatggcatatcttcttcactgtccaacttgattgaaccaggaatacattttcggttctttgaccccttgggaacatcatactgttctgcaagtccaacactggcttcccatttactcaaaattttctgaggaaccttatgcctatatcctttttctttctgtttccctcttctcctaaggacaggtagctcttcgaattgatgtctgccttcaaacatgacgattgcttttccagccacccaggctctctcagaaggatctccaaaagcctccacgtagtactgccgatagggcctccggttggaaactttcatttttgaatgtgtgttaatcaacggatcagaacaaatcctgcagggccaccatgggcgtctcttgaattttgcccagatgagatctccaacttcatacttcagtggcgtagactttttcttaggttgacaaaatggcaattcctgtgaagtagatgatgatgaagttccaggtaattctagcatgtttcctaatgtactggtactggaatctggatcatcctgaaaagataaatttattgagtttaattgctcttctattgtaatgtttgtgtctcctagtgaaaagggggctgggagaagggctgctttttcattgctgccgtccacttcatttctttgcttatttttctgtgtttcagtctgaggagctaatggcaagaatggcgatttgactgcaccgtgtctactctctggtgtgctgtcttgttcacttcccatggccacttttacaccattctctgatttagtctcataattgcaggtggcattggtctgagtttcctcaaagatctcctctatactctcatcctctgtgactggctgttctgggtccatttcagaatctacatctgcatcgtccacacaagtaaaattctcaaagtgcagaaagccattcttgatagtctttgttacttttacctggagttcaggggagttattacaagagggttcctgtttcatagcaagtgctgtaggaccaccaggactcaaggaagtgcaaacaattggcgtctgagctcttgaatcacttttttcagggtcttgaaaggattctgatccatcagcagacccatttaaatactctacattgatcatggaggccaaatcctgtagtctccgcagtggaatgtaacaagatggagaatcttgtccataagcattttgggatgttccactgacagtcgataactgcatagtacacccattaagtggctcagaaaaattggattgaccattaccgaaagggctgtccttgtcttcaggggcatctaaattcactggattggaaaagggcagcagacaatttcttctgggtagttcacaggtctgatccatcctgggccggcatcaaccgtgccccgcgccccctcccgggccagctggggggagggggtgaccctcattacactggggtgcgagcggagcggtggggagagagcggggccgctcgccgcacccccctccccccgcgtctctcttcaggggagaaggcagcgagcgcgacctgccccggcctattccgccgccgcctc

SEQ ID NO: 17926 - RNA, 8614 nt, Homo sapiens
  source 1..8614: mol_type = other RNA
tcggggcatgggggagggaggctggggccttcccgagagacctaaaagattgcccactcttggcggcaagtgcaggtagttgctggcctccgaccatctgcttcgcctgcttcaccaggcccggggattggctaagaggccctggggtctgctcagcccctgcagaagctcttcctgaggcctgagttgttggctcatataaaaaggccttggcaggaggctgagaaagaagtctggcctgggtgagtgatttaacagcttgccaggggtcctctgaaggggctgctgctttcccagatgtctgaagaggatctgacacacagcctttctcaacagctctcggcatatgccccagacctttgctggcaggccatgaacttgactccaacactggcatcttctcatcagcctgtggtgtgacctgatgaggtgaagctgcccgctccttctggcgaggagttaggtctatgagatccatcaccaaagcagctctattttttgactgagtattctggtccacaggcctcagtgctttttctttagctacaagggtctggaccacagctgatagtactttctcaggaggtgggagtctctgggacaaagaggcatggggtttgtcagtaggcctgtctgaagtctggggtttgggactgctagtaatgagcagtctgtctggcggcggaagtctcaggccagtgggaactgaggttttctccagtgactggggccttgggctggcagcacctatggatttatccagccttgggtcagccgtccccagaggtctttccagtggttgggacctgactgagggtgaggagcttgggctggtcactggagagggtttgtcgcttagctggggtcttggtcctgccactgctggtggcctgtccagtggcctctggctggaaaccaaggattgggatttggtccctgacccagcgaggtctctgaccttatctaaaggctggggcctggagtcagttctctcaagaggtctttcaggtagcaatggcctctgacaagtccctgccagagcttttttggagagcgacagcatctggttggtgtcagcaggaggtttatctgacattttgggtgcctgagcagccattcctgttgattgctctgccaggtgagtgcttggccctggaggcagcggtactgggggaggcacatactcacggatctccccaggttccagaggattgggcccacaggggtcatgctcagtacaagacagacgcccatccagtttggaaatgaaaagcatcccttctcgatgctgcttacaaaaggagctggggcacatctcacagaaggaggctgcttccttcccgcagatgtcacactgatgccacggacattcccatttccctgctggtcgcttggtcagattgagacagtctgcgtggtaaacttttgggcagcctggtttcttgcaggagacgagctggccagcatccccacaactaaaacactcatcttctcgctcctttgtgatttcaccctgggtcctgcgctttccctgttgcttcttcttgaatttctttgacttttcttccgtggcaatgggttgattctttggccttacacccaagaagccactgcagttcggggctccacatttgcaaacagtctttccattcccaagacattctaggttgtagttgaaggtaagttcagtgcctgctttaatgtcacttagtgcaaaaaggcctacacgggtatctccattcacagaccacttctgtgtttcacagttgggctggcagcaatgattcatgaaccgagcatagtttcctttgggaccagcatcaatgattcggtctttgtctagggtgagcatatagaaattagtgatatcatgttcttgagcatagcgaattcgagctctgcattcttcttcatctataagctcacccacatactcattcacaaattcaccctttttaatatctgtttttgtccgtagaccccaaccccgctgtaatgtgcggaaaatttcaacctctggatattggcgcttggaaaagcactggttttgacagcgccctccggcaggacacactgtggggtggcactcatagagcagcatgcggttgatgcattcagagtctatcccacaggggttctcatcagtagctttacagttgcaacggggtatttcagataagtctgcagtgaagatctgtaccctgccaataggacggtttacctttatatgtttataaggtggtggcttcttgtcattctttcggtcttcctgcagctgtcttagctctttttgggcctttaattcctcaaaccttgctgcagcttcctgaagagcttttttatatgtcccatccactcctttgcccatcttatccttgctgctcacgtcaccctccatgtaagggaagactcgggcctggtgagtccacaaatagtcattagatccaaaaaagaggactgggaactctcccacatcatgtctcatcttatcaatgttggaaggaacagctcgaggatggcagatctcagctggccaccacctgtatcgtccaacttttacccagacaatctccctgtagtgtggctttttgcctgctttacagtcattgcaataccagtttccttcagggatatcaatgttcaggcattcacgatgaaaagcagcagggcaagaatcacagcacagaaggctgcctccttctgagcacacaaagcaccagctaacattaacatgctcatgatttcggcagccccgcctaggggtaaagtgattagggcagatgatactattagatgcaaggatctttgacccagcagccaggcaaaagtcattggcgtggtatgccacaggacagcggacacagcgcatcaaccgacctttagatgcagaaacattggctggattagcagcatgacaggttatacagatgtggagggagcaccggaagcccttgttctgcataacagtgggtgggtacttctggacacactcttcatggtaaaactttccacacaagggtagaaggcaccttttaacatcttccccactctgcttacatacaaaacaggtatggattcctgtgcgacattcattgcagataaattttcctcttggcatctcagtcaatccaaggcactccaggtggaaagccccacagcactgagcctcacataacagcagctcacccaatttttcacaattctgacagacattctccttgagtgcagctcctccaccgcgttcaccctgcatttttttagaggcaggcatcccgggatcgtgttctacaccttcctcaacagtctccttggggcttgtggccgtcctgtgaggcattagttctccctctgagcctggaatctcttttgacgagtcatcatttttcacttttttacactgcatcttggctgcagcatgcctctgtcgttttcgcttccttggcttgtcaaatatcttggtagtgcctccaccaaaatcttttgaataagatgtggcacaagattcagttatgccattctccaggtgaccagcttcatagcactttttagaaaggccaaggtcccccttcttgggcataaatccagggtctaaatcattggattcaagaagtttcttagttggttttctttgacgtttactttcataatttcctggcgttttaactagcaattcctcagactcaagggcaggccgtggagagacttccggagccacaggcacagacaaggtcagctgcggcaactcagcatgtccacctccaagttctgactgagccaaggggccctccaaaaacggagcctccctttcaagaactggaggctcttctttggttgaaatcaaagaattctcgtccacctgcttgttctgagcactagatcgacctcgggctagaaggctttcctcttcacagcgggaacttaccttgtgcacctgctcctgtaccttcttttgttttttcttaggagcaaatatctgatcatattcttctgtatattccaaaagccacttgcttggcttcctaaggcgtttcttctctgaccgcacagctggttcagggagctcagcctgtggtgtcaaactgggaattcctggctccttttccatgtcaccaatgctggcactggatttatcacaaacatttaaccgtggcccagctgaatctaagcagtcagcatgattttgctctgtcagtggttcctcaagtatgcttgctgaaggagttctatgctctggaaactcatcccgcccctcctgcacagggtcactaggaagtaagaccctaaaggcacactcagagttttctttctctttaaatctgttcatgcgcttacgaggtttagtgcgcctttggtttaaacgctgccaccgctttttaggcaccacttgatttacaccattgagttcatcattctcactgttcattacagagtccagctctgggccttttccgttttcaaaagagagtcctttttcagaaattttaccaggatcagattgcttaaccttgctatcgaaatgcacatcagaaaaatggtcaccatcttcacttgttaagtggcccattatctgaaggggatcctctttactaggatcttctgccccacctctcaatgaacctccacgttctcggtctccctgcagtacagcatcaagagtcacacttggaagctgattcagttttcttttgcgctcggtctttaaggctttacggttcactgtgttctttaccatttgggctgaaaaagcatctcgcaatttggatgaaggctttgatcgtccacagttgcgcctagtaacacagtctgaacgacttttaccagaagcagggaggtctctcttgtcggacagtaagccaggtagggaagcagacaactcgccagataatgcagagtcacccccactagggctaggattggcggagttctgagtgccatctccctttttctctgaattgtgtgtggagcctcctgaaaccaaaaccttagagactcctacaggactattagtagaacagtccccacgaccaggactccggtaagagaccaggttttgagcagtcatcaaccgctgctccttcgtcttactatcatgcatatctttcaacatcattagcaatgtactgaatttgtagtctggttcaataggtatgtgattctgactagaagcagaagagaaaagtaatggttttgatggctttgatgttccagagtcactgacatcctcacctaaggatctgtaagagagttccttcaactcggataaaacatgtttcaccactgctgtttctatgtcacttgaatccctggttttctcatgcatattgttcagtagttttagaccatccactttcccacttttagaaatgctggccaaaggagagcctttggtatcagaagagcagcatttcaaactgcactcctcatttataactgggggttctgccataactggattttctttgtgtttgcactttatacttcggaacttgggctgtttgcttttcgaatgtaatagagcttgatttgctgccccaccctttattaacgagttctcactggatatgcttgatgacaggttgaattttggagagagagcatcatttgtaaaatctgactggggtttgtgaacaagagtagatgccttcagatcagagagattaacctgagacgtctcggttccaggctctgcactcttagtacaacccattaagtggtctgtatgtgagttactaatgagaggcttctgttttgcttttaccctagtgtttgtggcagcaaacctagaatactttatcttttcatttttctgcatagataacatgttctctgttctatcgaaagcatctggaatttcaaggacactgttatcagactctgagctgtgttctatgggatccaggtcactgcttccatcatcagaagtggtacagatactaatggaatcacttcgcttttcctcatcacctgctccaatatagcagagcttcacttttgaaccacacaccaggcttcgttggggtttattcttctctcgagaacactttgagatcaaagcaccctcaggcaagcccaataaagagtcaccatttgaagtctcaaattctttctttgcagtgttttttccacaggaagaaaacagaaaacttcctggggcagtgttggaccctgtgaggctatttgctatcctggaaagttcattagaggcctgcgtatcagatatatccccagagataaagtttaggccaaggttctctggaatctttcccctccgttcatctttatgtgcttcaaattgtatgtggccctttttcacactagtcctttttggattatcagagctctttctggctcgagatttagcgcaaggcttttccttctcatctgcagaatgttcagaatcaaaagccagtgatttcaaacagccattaagcaacaggtcatgttctgactcaggatcatttgtgcagtcttcaaatggcatatcttcttcactgtccaacttgattgaaccaggaatacattttcggttctttgaccccttgggaacatcatactgttctgcaagtccaacactggcttcccatttactcaaaattttctgaggaaccttatgcctatatcctttttctttctgtttccctcttctcctaaggacaggtagctcttcgaattgatgtctgccttcaaacatgacgattgcttttccagccacccaggctctctcagaaggatctccaaaagcctccacgtagtactgccgatagggcctccggttggaaactttcatttttgaatgtgtgttaatcaacggatcagaacaaatcctgcagggccaccatgggcgtctcttgaattttgcccagatgagatctccaacttcatacttcagtggcgtagactttttcttaggttgacaaaatggcaattcctgtgaagtagatgatgatgaagttccaggtaattctagcatgtttcctaatgtactggtactggaatctggatcatcctgaaaagataaatttattgagtttaattgctcttctattgtaatgtttgtgtctcctagtgaaaagggggctgggagaagggctgctttttcattgctgccgtccacttcatttctttgcttatttttctgtgtttcagtctgaggagctaatggcaagaatggcgatttgactgcaccgtgtctactctctggtgtgctgtcttgttcacttcccatggccacttttacaccattctctgatttagtctcataattgcaggtggcattggtctgagtttcctcaaagatctcctctatactctcatcctctgtgactggctgttctgggtccatttcagaatctacatctgcatcgtccacacaagtaaaattctcaaagtgcagaaagccattcttgatagtctttgttacttttacctggagttcaggggagttattacaagagggttcctgtttcatagcaagtgctgtaggaccaccaggactcaaggaagtgcaaacaattggcgtctgagctcttgaatcacttttttcagggtcttgaaaggattctgatccatcagcagacccatttaaatactctacattgatcatggaggccaaatcctgtagtctccgcagtggaatgtaacaagatggagaatcttgtccataagcattttgggatgttccactgacagtcgataactgcatagtacacccattaagtggctcagaaaaattggattgaccattaccgaaagggctgtccttgtcttcaggggcatctaaattcactggattggaaaagggcagcagacaatttcttctgggtagttcacaggtctgatccatcctgggccggcatcaacctcggggcacggcgctggcctcgggccgcacacggctcccgcaccctacgcgtctcgaaccccaacccaggcggcacctggcgcggctgaggcctgtccgatcgtcccgccagccctgctcgggcccgcgtcagtcccggcctccatcttaggttacagcccaggctccccatccactgggcacctgccctcagcccgctgggttcggcccgaggccaaggcaacccccctcctgccgcagggctcacctgggggcttgggctggggtcttcgaggcctcaggccccgagcagacgcggccgcaggcgaaccccctacccggccgcaccccaaacccacaccaccaccaccaccaccaccacagaccaagctgagcaggaaacaaaatggaggcagcagctcgggtctgcctccctgagccaagcctgtgcagccccagggctccctcctgtctcaggctcgacgcccgcgaggcagaggctggatcgtcccgggtgccgcgggcagccgccctacagcagcgcagacgggccggggactcggccctgcggtgcccacagcccctcacccaccaccccttcccttccccctccccccatccctctccctccccttgccgggccgtgcggggtgagcggctctggggagccgggtcgggttacccgccccggcactgctcgcccggccgtggcctccgcgggggaacgaagccaggcgaccccagcgctgagcccacccccggcaccgagccggg

SEQ ID NO: 17927 - RNA, 7965 nt, Homo sapiens
  source 1..7965: mol_type = other RNA
tcggggcatgggggagggaggctggggccttcccgagagacctaaaagattgcccactcttggcggcaagtgcaggtagttgctggcctccgaccatctgcttcgcctgcttcaccaggcccggggattggctaagaggccctggggtctgctcagcccctgcagaagctcttcctgaggcctgagttgttggctcatataaaaaggccttggcaggaggctgagaaagaagtctggcctgggtgagtgatttaacagcttgccaggggtcctctgaaggggctgctgctttcccagatgtctgaagaggatctgacacacagcctttctcaacagctctcggcatatgccccagacctttgctggcaggccatgaacttgactccaacactggcatcttctcatcagcctgtggtgtgacctgatgaggtgaagctgcccgctccttctggcgaggagttaggtctatgagatccatcaccaaagcagctctattttttgactgagtattctggtccacaggcctcagtgctttttctttagctacaagggtctggaccacagctgatagtactttctcaggaggtgggagtctctgggacaaagaggcatggggtttgtcagtaggcctgtctgaagtctggggtttgggactgctagtaatgagcagtctgtctggcggcggaagtctcaggccagtgggaactgaggttttctccagtgactggggccttgggctggcagcacctatggatttatccagccttgggtcagccgtccccagaggtctttccagtggttgggacctgactgagggtgaggagcttgggctggtcactggagagggtttgtcgcttagctggggtcttggtcctgccactgctggtggcctgtccagtggcctctggctggaaaccaaggattgggatttggtccctgacccagcgaggtctctgaccttatctaaaggctggggcctggagtcagttctctcaagaggtctttcaggtagcaatggcctctgacaagtccctgccagagcttttttggagagcgacagcatctggttggtgtcagcaggaggtttatctgacattttgggtgcctgagcagccattcctgttgattgctctgccaggtgagtgcttggccctggaggcagcggtactgggggaggcacatactcacggatctccccaggttccagaggattgggcccacaggggtcatgctcagtacaagacagacgcccatccagtttggaaatgaaaagcatcccttctcgatgctgcttacaaaaggagctggggcacatctcacagaaggaggctgcttccttcccgcagatgtcacactgatgccacggacattcccatttccctgctggtcgcttggtcagattgagacagtctgcgtggtaaacttttgggcagcctggtttcttgcaggagacgagctggccagcatccccacaactaaaacactcatcttctcgctcctttgtgatttcaccctgggtcctgcgctttccctgttgcttcttcttgaatttctttgacttttcttccgtggcaatgggttgattctttggccttacacccaagaagccactgcagttcggggctccacatttgcaaacagtctttccattcccaagacattctaggttgtagttgaaggtaagttcagtgcctgctttaatgtcacttagtgcaaaaaggcctacacgggtatctccattcacagaccacttctgtgtttcacagttgggctggcagcaatgattcatgaaccgagcatagtttcctttgggaccagcatcaatgattcggtctttgtctagggtgagcatatagaaattagtgatatcatgttcttgagcatagcgaattcgagctctgcattcttcttcatctataagctcacccacatactcattcacaaattcaccctttttaatatctgtttttgtccgtagaccccaaccccgctgtaatgtgcggaaaatttcaacctctggatattggcgcttggaaaagcactggttttgacagcgccctccggcaggacacactgtggggtggcactcatagagcagcatgcggttgatgcattcagagtctatcccacaggggttctcatcagtagctttacagttgcaacggggtatttcagataagtctgcagtgaagatctgtaccctgccaataggacggtttacctttatatgtttataaggtggtggcttcttgtcattctttcggtcttcctgcagctgtcttagctctttttgggcctttaattcctcaaaccttgctgcagcttcctgaagagcttttttatatgtcccatccactcctttgcccatcttatccttgctgctcacgtcaccctccatgtaagggaagactcgggcctggtgagtccacaaatagtcattagatccaaaaaagaggactgggaactctcccacatcatgtctcatcttatcaatgttggaaggaacagctcgaggatggcagatctcagctggccaccacctgtatcgtccaacttttacccagacaatctccctgtagtgtggctttttgcctgctttacagtcattgcaataccagtttccttcagggatatcaatgttcaggcattcacgatgaaaagcagcagggcaagaatcacagcacagaaggctgcctccttctgagcacacaaagcaccagctaacattaacatgctcatgatttcggcagccccgcctaggggtaaagtgattagggcagatgatactattagatgcaaggatctttgacccagcagccaggcaaaagtcattggcgtggtatgccacaggacagcggacacagcgcatcaaccgacctttagatgcagaaacattggctggattagcagcatgacaggttatacagatgtggagggagcaccggaagcccttgttctgcataacagtgggtgggtacttctggacacactcttcatggtaaaactttccacacaagggtagaaggcaccttttaacatcttccccactctgcttacatacaaaacaggtatggattcctgtgcgacattcattgcagataaattttcctcttggcatctcagtcaatccaaggcactccaggtggaaagccccacagcactgagcctcacataacagcagctcacccaatttttcacaattctgacagacattctccttgagtgcagctcctccaccgcgttcaccctgcatttttttagaggcaggcatcccgggatcgtgttctacaccttcctcaacagtctccttggggcttgtggccgtcctgtgaggcattagttctccctctgagcctggaatctcttttgacgagtcatcatttttcacttttttacactgcatcttggctgcagcatgcctctgtcgttttcgcttccttggcttgtcaaatatcttggtagtgcctccaccaaaatcttttgaataagatgtggcacaagattcagttatgccattctccaggtgaccagcttcatagcactttttagaaaggccaaggtcccccttcttgggcataaatccagggtctaaatcattggattcaagaagtttcttagttggttttctttgacgtttactttcataatttcctggcgttttaactagcaattcctcagactcaagggcaggccgtggagagacttccggagccacaggcacagacaaggtcagctgcggcaactcagcatgtccacctccaagttctgactgagccaaggggccctccaaaaacggagcctccctttcaagaactggaggctcttctttggttgaaatcaaagaattctcgtccacctgcttgttctgagcactagatcgacctcgggctagaaggctttcctcttcacagcgggaacttaccttgtgcacctgctcctgtaccttcttttgttttttcttaggagcaaatatctgatcatattcttctgtatattccaaaagccacttgcttggcttcctaaggcgtttcttctctgaccgcacagctggttcagggagctcagcctgtggtgtcaaactgggaattcctggctccttttccatgtcaccaatgctggcactggatttatcacaaacatttaaccgtggcccagctgaatctaagcagtcagcatgattttgctctgtcagtggttcctcaagtatgcttgctgaaggagttctatgctctggaaactcatcccgcccctcctgcacagggtcactaggaagtaagaccctaaaggcacactcagagttttctttctctttaaatctgttcatgcgcttacgaggtttagtgcgcctttggtttaaacgctgccaccgctttttaggcaccacttgatttacaccattgagttcatcattctcactgttcattacagagtccagctctgggccttttccgttttcaaaagagagtcctttttcagaaattttaccaggatcagattgcttaaccttgctatcgaaatgcacatcagaaaaatggtcaccatcttcacttgttaagtggcccattatctgaaggggatcctctttactaggatcttctgccccacctctcaatgaacctccacgttctcggtctccctgcagtacagcatcaagagtcacacttggaagctgattcagttttcttttgcgctcggtctttaaggctttacggttcactgtgttctttaccatttgggctgaaaaagcatctcgcaatttggatgaaggctttgatcgtccacagttgcgcctagtaacacagtctgaacgacttttaccagaagcagggaggtctctcttgtcggacagtaagccaggtagggaagcagacaactcgccagataatgcagagtcacccccactagggctaggattggcggagttctgagtgccatctccctttttctctgaattgtgtgtggagcctcctgaaaccaaaaccttagagactcctacaggactattagtagaacagtccccacgaccaggactccggtaagagaccaggttttgagcagtcatcaaccgctgctccttcgtcttactatcatgcatatctttcaacatcattagcaatgtactgaatttgtagtctggttcaataggtatgtgattctgactagaagcagaagagaaaagtaatggttttgatggctttgatgttccagagtcactgacatcctcacctaaggatctgtaagagagttccttcaactcggataaaacatgtttcaccactgctgtttctatgtcacttgaatccctggttttctcatgcatattgttcagtagttttagaccatccactttcccacttttagaaatgctggccaaaggagagcctttggtatcagaagagcagcatttcaaactgcactcctcatttataactgggggttctgccataactggattttctttgtgtttgcactttatacttcggaacttgggctgtttgcttttcgaatgtaatagagcttgatttgctgccccaccctttattaacgagttctcactggatatgcttgatgacaggttgaattttggagagagagcatcatttgtaaaatctgactggggtttgtgaacaagagtagatgccttcagatcagagagattaacctgagacgtctcggttccaggctctgcactcttagtacaacccattaagtggtctgtatgtgagttactaatgagaggcttctgttttgcttttaccctagtgtttgtggcagcaaacctagaatactttatcttttcatttttctgcatagataacatgttctctgttctatcgaaagcatctggaatttcaaggacactgttatcagactctgagctgtgttctatgggatccaggtcactgcttccatcatcagaagtggtacagatactaatggaatcacttcgcttttcctcatcacctgctccaatatagcagagcttcacttttgaaccacacaccaggcttcgttggggtttattcttctctcgagaacactttgagatcaaagcaccctcaggcaagcccaataaagagtcaccatttgaagtctcaaattctttctttgcagtgttttttccacaggaagaaaacagaaaacttcctggggcagtgttggaccctgtgaggctatttgctatcctggaaagttcattagaggcctgcgtatcagatatatccccagagataaagtttaggccaaggttctctggaatctttcccctccgttcatctttatgtgcttcaaattgtatgtggccctttttcacactagtcctttttggattatcagagctctttctggctcgagatttagcgcaaggcttttccttctcatctgcagaatgttcagaatcaaaagccagtgatttcaaacagccattaagcaacaggtcatgttctgactcaggatcatttgtgcagtcttcaaatggcatatcttcttcactgtccaacttgattgaaccaggaatacattttcggttctttgaccccttgggaacatcatactgttctgcaagtccaacactggcttcccatttactcaaaattttctgaggaaccttatgcctatatcctttttctttctgtttccctcttctcctaaggacaggtagctcttcgaattgatgtctgccttcaaacatgacgattgcttttccagccacccaggctctctcagaaggatctccaaaagcctccacgtagtactgccgatagggcctccggttggaaactttcatttttgaatgtgtgttaatcaacggatcagaacaaatcctgcagggccaccatgggcgtctcttgaattttgcccagatgagatctccaacttcatacttcagtggcgtagactttttcttaggttgacaaaatggcaattcctgtgaagtagatgatgatgaagttccaggtaattctagcatgtttcctaatgtactggtactggaatctggatcatcctgaaaagataaatttattgagtttaattgctcttctattgtaatgtttgtgtctcctagtgaaaagggggctgggagaagggctgctttttcattgctgccgtccacttcatttctttgcttatttttctgtgtttcagtctgaggagctaatggcaagaatggcgatttgactgcaccgtgtctactctctggtgtgctgtcttgttcacttcccatggccacttttacaccattctctgatttagtctcataattgcaggtggcattggtctgagtttcctcaaagatctcctctatactctcatcctctgtgactggctgttctgggtccatttcagaatctacatctgcatcgtccacacaagtaaaattctcaaagtgcagaaagccattcttgatagtctttgttacttttacctggagttcaggggagttattacaagagggttcctgtttcatagcaagtgctgtaggaccaccaggactcaaggaagtgcaaacaattggcgtctgagctcttgaatcacttttttcagggtcttgaaaggattctgatccatcagcagacccatttaaatactctacattgatcatggaggccaaatcctgtagtctccgcagtggaatgtaacaagatggagaatcttgtccataagcattttgggatgttccactgacagtcgataactgcatagtacacccattaagtggctcagaaaaattggattgaccattaccgaaagggctgtccttgtcttcaggggcatctaaattcactggattggaaaagggcagcagacaatttcttctgggtagttcacaggtctgatccatcctgggccggcatcaacctgaggggaggcggaggccgaggtgttcgcaggcggccggcggggcacgggccgcgccgggaggaagttcgcggcagcccggccagctaggcctgagcccggctg

SEQ ID NO: 17928 - RNA, 7990 nt, Homo sapiens
  source 1..7990: mol_type = other RNA
tcggggcatgggggagggaggctggggccttcccgagagacctaaaagattgcccactcttggcggcaagtgcaggtagttgctggcctccgaccatctgcttcgcctgcttcaccaggcccggggattggctaagaggccctggggtctgctcagcccctgcagaagctcttcctgaggcctgagttgttggctcatataaaaaggccttggcaggaggctgagaaagaagtctggcctgggtgagtgatttaacagcttgccaggggtcctctgaaggggctgctgctttcccagatgtctgaagaggatctgacacacagcctttctcaacagctctcggcatatgccccagacctttgctggcaggccatgaacttgactccaacactggcatcttctcatcagcctgtggtgtgacctgatgaggtgaagctgcccgctccttctggcgaggagttaggtctatgagatccatcaccaaagcagctctattttttgactgagtattctggtccacaggcctcagtgctttttctttagctacaagggtctggaccacagctgatagtactttctcaggaggtgggagtctctgggacaaagaggcatggggtttgtcagtaggcctgtctgaagtctggggtttgggactgctagtaatgagcagtctgtctggcggcggaagtctcaggccagtgggaactgaggttttctccagtgactggggccttgggctggcagcacctatggatttatccagccttgggtcagccgtccccagaggtctttccagtggttgggacctgactgagggtgaggagcttgggctggtcactggagagggtttgtcgcttagctggggtcttggtcctgccactgctggtggcctgtccagtggcctctggctggaaaccaaggattgggatttggtccctgacccagcgaggtctctgaccttatctaaaggctggggcctggagtcagttctctcaagaggtctttcaggtagcaatggcctctgacaagtccctgccagagcttttttggagagcgacagcatctggttggtgtcagcaggaggtttatctgacattttgggtgcctgagcagccattcctgttgattgctctgccaggtgagtgcttggccctggaggcagcggtactgggggaggcacatactcacggatctccccaggttccagaggattgggcccacaggggtcatgctcagtacaagacagacgcccatccagtttggaaatgaaaagcatcccttctcgatgctgcttacaaaaggagctggggcacatctcacagaaggaggctgcttccttcccgcagatgtcacactgatgccacggacattcccatttccctgctggtcgcttggtcagattgagacagtctgcgtggtaaacttttgggcagcctggtttcttgcaggagacgagctggccagcatccccacaactaaaacactcatcttctcgctcctttgtgatttcaccctgggtcctgcgctttccctgttgcttcttcttgaatttctttgacttttcttccgtggcaatgggttgattctttggccttacacccaagaagccactgcagttcggggctccacatttgcaaacagtctttccattcccaagacattctaggttgtagttgaaggtaagttcagtgcctgctttaatgtcacttagtgcaaaaaggcctacacgggtatctccattcacagaccacttctgtgtttcacagttgggctggcagcaatgattcatgaaccgagcatagtttcctttgggaccagcatcaatgattcggtctttgtctagggtgagcatatagaaattagtgatatcatgttcttgagcatagcgaattcgagctctgcattcttcttcatctataagctcacccacatactcattcacaaattcaccctttttaatatctgtttttgtccgtagaccccaaccccgctgtaatgtgcggaaaatttcaacctctggatattggcgcttggaaaagcactggttttgacagcgccctccggcaggacacactgtggggtggcactcatagagcagcatgcggttgatgcattcagagtctatcccacaggggttctcatcagtagctttacagttgcaacggggtatttcagataagtctgcagtgaagatctgtaccctgccaataggacggtttacctttatatgtttataaggtggtggcttcttgtcattctttcggtcttcctgcagctgtcttagctctttttgggcctttaattcctcaaaccttgctgcagcttcctgaagagcttttttatatgtcccatccactcctttgcccatcttatccttgctgctcacgtcaccctccatgtaagggaagactcgggcctggtgagtccacaaatagtcattagatccaaaaaagaggactgggaactctcccacatcatgtctcatcttatcaatgttggaaggaacagctcgaggatggcagatctcagctggccaccacctgtatcgtccaacttttacccagacaatctccctgtagtgtggctttttgcctgctttacagtcattgcaataccagtttccttcagggatatcaatgttcaggcattcacgatgaaaagcagcagggcaagaatcacagcacagaaggctgcctccttctgagcacacaaagcaccagctaacattaacatgctcatgatttcggcagccccgcctaggggtaaagtgattagggcagatgatactattagatgcaaggatctttgacccagcagccaggcaaaagtcattggcgtggtatgccacaggacagcggacacagcgcatcaaccgacctttagatgcagaaacattggctggattagcagcatgacaggttatacagatgtggagggagcaccggaagcccttgttctgcataacagtgggtgggtacttctggacacactcttcatggtaaaactttccacacaagggtagaaggcaccttttaacatcttccccactctgcttacatacaaaacaggtatggattcctgtgcgacattcattgcagataaattttcctcttggcatctcagtcaatccaaggcactccaggtggaaagccccacagcactgagcctcacataacagcagctcacccaatttttcacaattctgacagacattctccttgagtgcagctcctccaccgcgttcaccctgcatttttttagaggcaggcatcccgggatcgtgttctacaccttcctcaacagtctccttggggcttgtggccgtcctgtgaggcattagttctccctctgagcctggaatctcttttgacgagtcatcatttttcacttttttacactgcatcttggctgcagcatgcctctgtcgttttcgcttccttggcttgtcaaatatcttggtagtgcctccaccaaaatcttttgaataagatgtggcacaagattcagttatgccattctccaggtgaccagcttcatagcactttttagaaaggccaaggtcccccttcttgggcataaatccagggtctaaatcattggattcaagaagtttcttagttggttttctttgacgtttactttcataatttcctggcgttttaactagcaattcctcagactcaagggcaggccgtggagagacttccggagccacaggcacagacaaggtcagctgcggcaactcagcatgtccacctccaagttctgactgagccaaggggccctccaaaaacggagcctccctttcaagaactggaggctcttctttggttgaaatcaaagaattctcgtccacctgcttgttctgagcactagatcgacctcgggctagaaggctttcctcttcacagcgggaacttaccttgtgcacctgctcctgtaccttcttttgttttttcttaggagcaaatatctgatcatattcttctgtatattccaaaagccacttgcttggcttcctaaggcgtttcttctctgaccgcacagctggttcagggagctcagcctgtggtgtcaaactgggaattcctggctccttttccatgtcaccaatgctggcactggatttatcacaaacatttaaccgtggcccagctgaatctaagcagtcagcatgattttgctctgtcagtggttcctcaagtatgcttgctgaaggagttctatgctctggaaactcatcccgcccctcctgcacagggtcactaggaagtaagaccctaaaggcacactcagagttttctttctctttaaatctgttcatgcgcttacgaggtttagtgcgcctttggtttaaacgctgccaccgctttttaggcaccacttgatttacaccattgagttcatcattctcactgttcattacagagtccagctctgggccttttccgttttcaaaagagagtcctttttcagaaattttaccaggatcagattgcttaaccttgctatcgaaatgcacatcagaaaaatggtcaccatcttcacttgttaagtggcccattatctgaaggggatcctctttactaggatcttctgccccacctctcaatgaacctccacgttctcggtctccctgcagtacagcatcaagagtcacacttggaagctgattcagttttcttttgcgctcggtctttaaggctttacggttcactgtgttctttaccatttgggctgaaaaagcatctcgcaatttggatgaaggctttgatcgtccacagttgcgcctagtaacacagtctgaacgacttttaccagaagcagggaggtctctcttgtcggacagtaagccaggtagggaagcagacaactcgccagataatgcagagtcacccccactagggctaggattggcggagttctgagtgccatctccctttttctctgaattgtgtgtggagcctcctgaaaccaaaaccttagagactcctacaggactattagtagaacagtccccacgaccaggactccggtaagagaccaggttttgagcagtcatcaaccgctgctccttcgtcttactatcatgcatatctttcaacatcattagcaatgtactgaatttgtagtctggttcaataggtatgtgattctgactagaagcagaagagaaaagtaatggttttgatggctttgatgttccagagtcactgacatcctcacctaaggatctgtaagagagttccttcaactcggataaaacatgtttcaccactgctgtttctatgtcacttgaatccctggttttctcatgcatattgttcagtagttttagaccatccactttcccacttttagaaatgctggccaaaggagagcctttggtatcagaagagcagcatttcaaactgcactcctcatttataactgggggttctgccataactggattttctttgtgtttgcactttatacttcggaacttgggctgtttgcttttcgaatgtaatagagcttgatttgctgccccaccctttattaacgagttctcactggatatgcttgatgacaggttgaattttggagagagagcatcatttgtaaaatctgactggggtttgtgaacaagagtagatgccttcagatcagagagattaacctgagacgtctcggttccaggctctgcactcttagtacaacccattaagtggtctgtatgtgagttactaatgagaggcttctgttttgcttttaccctagtgtttgtggcagcaaacctagaatactttatcttttcatttttctgcatagataacatgttctctgttctatcgaaagcatctggaatttcaaggacactgttatcagactctgagctgtgttctatgggatccaggtcactgcttccatcatcagaagtggtacagatactaatggaatcacttcgcttttcctcatcacctgctccaatatagcagagcttcacttttgaaccacacaccaggcttcgttggggtttattcttctctcgagaacactttgagatcaaagcaccctcaggcaagcccaataaagagtcaccatttgaagtctcaaattctttctttgcagtgttttttccacaggaagaaaacagaaaacttcctggggcagtgttggaccctgtgaggctatttgctatcctggaaagttcattagaggcctgcgtatcagatatatccccagagataaagtttaggccaaggttctctggaatctttcccctccgttcatctttatgtgcttcaaattgtatgtggccctttttcacactagtcctttttggattatcagagctctttctggctcgagatttagcgcaaggcttttccttctcatctgcagaatgttcagaatcaaaagccagtgatttcaaacagccattaagcaacaggtcatgttctgactcaggatcatttgtgcagtcttcaaatggcatatcttcttcactgtccaacttgattgaaccaggaatacattttcggttctttgaccccttgggaacatcatactgttctgcaagtccaacactggcttcccatttactcaaaattttctgaggaaccttatgcctatatcctttttctttctgtttccctcttctcctaaggacaggtagctcttcgaattgatgtctgccttcaaacatgacgattgcttttccagccacccaggctctctcagaaggatctccaaaagcctccacgtagtactgccgatagggcctccggttggaaactttcatttttgaatgtgtgttaatcaacggatcagaacaaatcctgcagggccaccatgggcgtctcttgaattttgcccagatgagatctccaacttcatacttcagtggcgtagactttttcttaggttgacaaaatggcaattcctgtgaagtagatgatgatgaagttccaggtaattctagcatgtttcctaatgtactggtactggaatctggatcatcctgaaaagataaatttattgagtttaattgctcttctattgtaatgtttgtgtctcctagtgaaaagggggctgggagaagggctgctttttcattgctgccgtccacttcatttctttgcttatttttctgtgtttcagtctgaggagctaatggcaagaatggcgatttgactgcaccgtgtctactctctggtgtgctgtcttgttcacttcccatggccacttttacaccattctctgatttagtctcataattgcaggtggcattggtctgagtttcctcaaagatctcctctatactctcatcctctgtgactggctgttctgggtccatttcagaatctacatctgcatcgtccacacaagtaaaattctcaaagtgcagaaagccattcttgatagtctttgttacttttacctggagttcaggggagttattacaagagggttcctgtttcatagcaagtgctgtaggaccaccaggactcaaggaagtgcaaacaattggcgtctgagctcttgaatcacttttttcagggtcttgaaaggattctgatccatcagcagacccatttaaatactctacattgatcatggaggccaaatcctgtagtctccgcagtggaatgtaacaagatggagaatcttgtccataagcattttgggatgttccactgacagtcgataactgcatagtacacccattaagtggctcagaaaaattggattgaccattaccgaaagggctgtccttgtcttcaggggcatctaaattcactggattggaaaagggcagcagacaatttcttctgggtagttcacaggtctgatccatcctgggccggcatcaacctgggggcttgggctggggtcttcgaggcctcaggccccgagcagacgcggccgcaggcgaaccccctacccggccgcaccccaaacccacaccaccaccaccaccaccaccacagaccaagctgagcag

SEQ ID NO: 17929 - RNA, 7919 nt, Homo sapiens
  source 1..7919: mol_type = other RNA
tcggggcatgggggagggaggctggggccttcccgagagacctaaaagattgcccactcttggcggcaagtgcaggtagttgctggcctccgaccatctgcttcgcctgcttcaccaggcccggggattggctaagaggccctggggtctgctcagcccctgcagaagctcttcctgaggcctgagttgttggctcatataaaaaggccttggcaggaggctgagaaagaagtctggcctgggtgagtgatttaacagcttgccaggggtcctctgaaggggctgctgctttcccagatgtctgaagaggatctgacacacagcctttctcaacagctctcggcatatgccccagacctttgctggcaggccatgaacttgactccaacactggcatcttctcatcagcctgtggtgtgacctgatgaggtgaagctgcccgctccttctggcgaggagttaggtctatgagatccatcaccaaagcagctctattttttgactgagtattctggtccacaggcctcagtgctttttctttagctacaagggtctggaccacagctgatagtactttctcaggaggtgggagtctctgggacaaagaggcatggggtttgtcagtaggcctgtctgaagtctggggtttgggactgctagtaatgagcagtctgtctggcggcggaagtctcaggccagtgggaactgaggttttctccagtgactggggccttgggctggcagcacctatggatttatccagccttgggtcagccgtccccagaggtctttccagtggttgggacctgactgagggtgaggagcttgggctggtcactggagagggtttgtcgcttagctggggtcttggtcctgccactgctggtggcctgtccagtggcctctggctggaaaccaaggattgggatttggtccctgacccagcgaggtctctgaccttatctaaaggctggggcctggagtcagttctctcaagaggtctttcaggtagcaatggcctctgacaagtccctgccagagcttttttggagagcgacagcatctggttggtgtcagcaggaggtttatctgacattttgggtgcctgagcagccattcctgttgattgctctgccaggtgagtgcttggccctggaggcagcggtactgggggaggcacatactcacggatctccccaggttccagaggattgggcccacaggggtcatgctcagtacaagacagacgcccatccagtttggaaatgaaaagcatcccttctcgatgctgcttacaaaaggagctggggcacatctcacagaaggaggctgcttccttcccgcagatgtcacactgatgccacggacattcccatttccctgctggtcgcttggtcagattgagacagtctgcgtggtaaacttttgggcagcctggtttcttgcaggagacgagctggccagcatccccacaactaaaacactcatcttctcgctcctttgtgatttcaccctgggtcctgcgctttccctgttgcttcttcttgaatttctttgacttttcttccgtggcaatgggttgattctttggccttacacccaagaagccactgcagttcggggctccacatttgcaaacagtctttccattcccaagacattctaggttgtagttgaaggtaagttcagtgcctgctttaatgtcacttagtgcaaaaaggcctacacgggtatctccattcacagaccacttctgtgtttcacagttgggctggcagcaatgattcatgaaccgagcatagtttcctttgggaccagcatcaatgattcggtctttgtctagggtgagcatatagaaattagtgatatcatgttcttgagcatagcgaattcgagctctgcattcttcttcatctataagctcacccacatactcattcacaaattcaccctttttaatatctgtttttgtccgtagaccccaaccccgctgtaatgtgcggaaaatttcaacctctggatattggcgcttggaaaagcactggttttgacagcgccctccggcaggacacactgtggggtggcactcatagagcagcatgcggttgatgcattcagagtctatcccacaggggttctcatcagtagctttacagttgcaacggggtatttcagataagtctgcagtgaagatctgtaccctgccaataggacggtttacctttatatgtttataaggtggtggcttcttgtcattctttcggtcttcctgcagctgtcttagctctttttgggcctttaattcctcaaaccttgctgcagcttcctgaagagcttttttatatgtcccatccactcctttgcccatcttatccttgctgctcacgtcaccctccatgtaagggaagactcgggcctggtgagtccacaaatagtcattagatccaaaaaagaggactgggaactctcccacatcatgtctcatcttatcaatgttggaaggaacagctcgaggatggcagatctcagctggccaccacctgtatcgtccaacttttacccagacaatctccctgtagtgtggctttttgcctgctttacagtcattgcaataccagtttccttcagggatatcaatgttcaggcattcacgatgaaaagcagcagggcaagaatcacagcacagaaggctgcctccttctgagcacacaaagcaccagctaacattaacatgctcatgatttcggcagccccgcctaggggtaaagtgattagggcagatgatactattagatgcaaggatctttgacccagcagccaggcaaaagtcattggcgtggtatgccacaggacagcggacacagcgcatcaaccgacctttagatgcagaaacattggctggattagcagcatgacaggttatacagatgtggagggagcaccggaagcccttgttctgcataacagtgggtgggtacttctggacacactcttcatggtaaaactttccacacaagggtagaaggcaccttttaacatcttccccactctgcttacatacaaaacaggtatggattcctgtgcgacattcattgcagataaattttcctcttggcatctcagtcaatccaaggcactccaggtggaaagccccacagcactgagcctcacataacagcagctcacccaatttttcacaattctgacagacattctccttgagtgcagctcctccaccgcgttcaccctgcatttttttagaggcaggcatcccgggatcgtgttctacaccttcctcaacagtctccttggggcttgtggccgtcctgtgaggcattagttctccctctgagcctggaatctcttttgacgagtcatcatttttcacttttttacactgcatcttggctgcagcatgcctctgtcgttttcgcttccttggcttgtcaaatatcttggtagtgcctccaccaaaatcttttgaataagatgtggcacaagattcagttatgccattctccaggtgaccagcttcatagcactttttagaaaggccaaggtcccccttcttgggcataaatccagggtctaaatcattggattcaagaagtttcttagttggttttctttgacgtttactttcataatttcctggcgttttaactagcaattcctcagactcaagggcaggccgtggagagacttccggagccacaggcacagacaaggtcagctgcggcaactcagcatgtccacctccaagttctgactgagccaaggggccctccaaaaacggagcctccctttcaagaactggaggctcttctttggttgaaatcaaagaattctcgtccacctgcttgttctgagcactagatcgacctcgggctagaaggctttcctcttcacagcgggaacttaccttgtgcacctgctcctgtaccttcttttgttttttcttaggagcaaatatctgatcatattcttctgtatattccaaaagccacttgcttggcttcctaaggcgtttcttctctgaccgcacagctggttcagggagctcagcctgtggtgtcaaactgggaattcctggctccttttccatgtcaccaatgctggcactggatttatcacaaacatttaaccgtggcccagctgaatctaagcagtcagcatgattttgctctgtcagtggttcctcaagtatgcttgctgaaggagttctatgctctggaaactcatcccgcccctcctgcacagggtcactaggaagtaagaccctaaaggcacactcagagttttctttctctttaaatctgttcatgcgcttacgaggtttagtgcgcctttggtttaaacgctgccaccgctttttaggcaccacttgatttacaccattgagttcatcattctcactgttcattacagagtccagctctgggccttttccgttttcaaaagagagtcctttttcagaaattttaccaggatcagattgcttaaccttgctatcgaaatgcacatcagaaaaatggtcaccatcttcacttgttaagtggcccattatctgaaggggatcctctttactaggatcttctgccccacctctcaatgaacctccacgttctcggtctccctgcagtacagcatcaagagtcacacttggaagctgattcagttttcttttgcgctcggtctttaaggctttacggttcactgtgttctttaccatttgggctgaaaaagcatctcgcaatttggatgaaggctttgatcgtccacagttgcgcctagtaacacagtctgaacgacttttaccagaagcagggaggtctctcttgtcggacagtaagccaggtagggaagcagacaactcgccagataatgcagagtcacccccactagggctaggattggcggagttctgagtgccatctccctttttctctgaattgtgtgtggagcctcctgaaaccaaaaccttagagactcctacaggactattagtagaacagtccccacgaccaggactccggtaagagaccaggttttgagcagtcatcaaccgctgctccttcgtcttactatcatgcatatctttcaacatcattagcaatgtactgaatttgtagtctggttcaataggtatgtgattctgactagaagcagaagagaaaagtaatggttttgatggctttgatgttccagagtcactgacatcctcacctaaggatctgtaagagagttccttcaactcggataaaacatgtttcaccactgctgtttctatgtcacttgaatccctggttttctcatgcatattgttcagtagttttagaccatccactttcccacttttagaaatgctggccaaaggagagcctttggtatcagaagagcagcatttcaaactgcactcctcatttataactgggggttctgccataactggattttctttgtgtttgcactttatacttcggaacttgggctgtttgcttttcgaatgtaatagagcttgatttgctgccccaccctttattaacgagttctcactggatatgcttgatgacaggttgaattttggagagagagcatcatttgtaaaatctgactggggtttgtgaacaagagtagatgccttcagatcagagagattaacctgagacgtctcggttccaggctctgcactcttagtacaacccattaagtggtctgtatgtgagttactaatgagaggcttctgttttgcttttaccctagtgtttgtggcagcaaacctagaatactttatcttttcatttttctgcatagataacatgttctctgttctatcgaaagcatctggaatttcaaggacactgttatcagactctgagctgtgttctatgggatccaggtcactgcttccatcatcagaagtggtacagatactaatggaatcacttcgcttttcctcatcacctgctccaatatagcagagcttcacttttgaaccacacaccaggcttcgttggggtttattcttctctcgagaacactttgagatcaaagcaccctcaggcaagcccaataaagagtcaccatttgaagtctcaaattctttctttgcagtgttttttccacaggaagaaaacagaaaacttcctggggcagtgttggaccctgtgaggctatttgctatcctggaaagttcattagaggcctgcgtatcagatatatccccagagataaagtttaggccaaggttctctggaatctttcccctccgttcatctttatgtgcttcaaattgtatgtggccctttttcacactagtcctttttggattatcagagctctttctggctcgagatttagcgcaaggcttttccttctcatctgcagaatgttcagaatcaaaagccagtgatttcaaacagccattaagcaacaggtcatgttctgactcaggatcatttgtgcagtcttcaaatggcatatcttcttcactgtccaacttgattgaaccaggaatacattttcggttctttgaccccttgggaacatcatactgttctgcaagtccaacactggcttcccatttactcaaaattttctgaggaaccttatgcctatatcctttttctttctgtttccctcttctcctaaggacaggtagctcttcgaattgatgtctgccttcaaacatgacgattgcttttccagccacccaggctctctcagaaggatctccaaaagcctccacgtagtactgccgatagggcctccggttggaaactttcatttttgaatgtgtgttaatcaacggatcagaacaaatcctgcagggccaccatgggcgtctcttgaattttgcccagatgagatctccaacttcatacttcagtggcgtagactttttcttaggttgacaaaatggcaattcctgtgaagtagatgatgatgaagttccaggtaattctagcatgtttcctaatgtactggtactggaatctggatcatcctgaaaagataaatttattgagtttaattgctcttctattgtaatgtttgtgtctcctagtgaaaagggggctgggagaagggctgctttttcattgctgccgtccacttcatttctttgcttatttttctgtgtttcagtctgaggagctaatggcaagaatggcgatttgactgcaccgtgtctactctctggtgtgctgtcttgttcacttcccatggccacttttacaccattctctgatttagtctcataattgcaggtggcattggtctgagtttcctcaaagatctcctctatactctcatcctctgtgactggctgttctgggtccatttcagaatctacatctgcatcgtccacacaagtaaaattctcaaagtgcagaaagccattcttgatagtctttgttacttttacctggagttcaggggagttattacaagagggttcctgtttcatagcaagtgctgtaggaccaccaggactcaaggaagtgcaaacaattggcgtctgagctcttgaatcacttttttcagggtcttgaaaggattctgatccatcagcagacccatttaaatactctacattgatcatggaggccaaatcctgtagtctccgcagtggaatgtaacaagatggagaatcttgtccataagcattttgggatgttccactgacagtcgataactgcatagtacacccattaagtggctcagaaaaattggattgaccattaccgaaagggctgtccttgtcttcaggggcatctaaattcactggattggaaaagggcagcagacaatttcttctgggtagttcacaggtctgatccatcctgggccggcatcaactcttcggggttcagggcgggtgaagtcgggcttgtgagagcgccgcccaatcagcggag

SEQ ID NO: 17930 - RNA, 7631 nt, Homo sapiens
  source 1..7631: mol_type = other RNA
tcggggcatgggggagggaggctggggccttcccgagagacctaaaagattgcccactcttggcggcaagtgcaggtagttgctggcctccgaccatctgcttcgcctgcttcaccaggcccggggattggctaagaggccctggggtctgctcagcccctgcagaagctcttcctgaggcctgagttgttggctcatataaaaaggccttggcaggaggctgagaaagaagtctggcctgggtgagtgatttaacagcttgccaggggtcctctgaaggggctgctgctttcccagatgtctgaagaggatctgacacacagcctttctcaacagctctcggcatatgccccagacctttgctggcaggccatgaacttgactccaacactggcatcttctcatcagcctgtggtgtgacctgatgaggtgaagctgcccgctccttctggcgaggagttaggtctatgagatccatcaccaaagcagctctattttttgactgagtattctggtccacaggcctcagtgctttttctttagctacaagggtctggaccacagctgatagtactttctcaggaggtgggagtctctgggacaaagaggcatggggtttgtcagtaggcctgtctgaagtctggggtttgggactgctagtaatgagcagtctgtctggcggcggaagtctcaggccagtgggaactgaggttttctccagtgactggggccttgggctggcagcacctatggatttatccagccttgggtcagccgtccccagaggtctttccagtggttgggacctgactgagggtgaggagcttgggctggtcactggagagggtttgtcgcttagctggggtcttggtcctgccactgctggtggcctgtccagtggcctctggctggaaaccaaggattgggatttggtccctgacccagcgaggtctctgaccttatctaaaggctggggcctggagtcagttctctcaagaggtctttcaggtagcaatggcctctgacaagtccctgccagagcttttttggagagcgacagcatctggttggtgtcagcaggaggtttatctgacattttgggtgcctgagcagccattcctgttgattgctctgccaggtgagtgcttggccctggaggcagcggtactgggggaggcacatactcacggatctccccaggttccagaggattgggcccacaggggtcatgctcagtacaagacagacgcccatccagtttggaaatgaaaagcatcccttctcgatgctgcttacaaaaggagctggggcacatctcacagaaggaggctgcttccttcccgcagatgtcacactgatgccacggacattcccatttccctgctggtcgcttggtcagattgagacagtctgcgtggtaaacttttgggcagcctggtttcttgcaggagacgagctggccagcatccccacaactaaaacactcatcttctcgctcctttgtgatttcaccctgggtcctgcgctttccctgttgcttcttcttgaatttctttgacttttcttccgtggcaatgggttgattctttggccttacacccaagaagccactgcagttcggggctccacatttgcaaacagtctttccattcccaagacattctaggttgtagttgaaggtaagttcagtgcctgctttaatgtcacttagtgcaaaaaggcctacacgggtatctccattcacagaccacttctgtgtttcacagttgggctggcagcaatgattcatgaaccgagcatagtttcctttgggaccagcatcaatgattcggtctttgtctagggtgagcatatagaaattagtgatatcatgttcttgagcatagcgaattcgagctctgcattcttcttcatctataagctcacccacatactcattcacaaattcaccctttttaatatctgtttttgtccgtagaccccaaccccgctgtaatgtgcggaaaatttcaacctctggatattggcgcttggaaaagcactggttttgacagcgccctccggcaggacacactgtggggtggcactcatagagcagcatgcggttgatgcattcagagtctatcccacaggggttctcatcagtagctttacagttgcaacggggtatttcagataagtctgcagtgaagatctgtaccctgccaataggacggtttacctttatatgtttataaggtggtggcttcttgtcattctttcggtcttcctgcagctgtcttagctctttttgggcctttaattcctcaaaccttgctgcagcttcctgaagagcttttttatatgtcccatccactcctttgcccatcttatccttgctgctcacgtcaccctccatgtaagggaagactcgggcctggtgagtccacaaatagtcattagatccaaaaaagaggactgggaactctcccacatcatgtctcatcttatcaatgttggaaggaacagctcgaggatggcagatctcagctggccaccacctgtatcgtccaacttttacccagacaatctccctgtagtgtggctttttgcctgctttacagtcattgcaataccagtttccttcagggatatcaatgttcaggcattcacgatgaaaagcagcagggcaagaatcacagcacagaaggctgcctccttctgagcacacaaagcaccagctaacattaacatgctcatgatttcggcagccccgcctaggggtaaagtgattagggcagatgatactattagatgcaaggatctttgacccagcagccaggcaaaagtcattggcgtggtatgccacaggacagcggacacagcgcatcaaccgacctttagatgcagaaacattggctggattagcagcatgacaggttatacagatgtggagggagcaccggaagcccttgttctgcataacagtgggtgggtacttctggacacactcttcatggtaaaactttccacacaagggtagaaggcaccttttaacatcttccccactctgcttacatacaaaacaggtatggattcctgtgcgacattcattgcagataaattttcctcttggcatctcagtcaatccaaggcactccaggtggaaagccccacagcactgagcctcacataacagcagctcacccaatttttcacaattctgacagacattctccttgagtgcagctcctccaccgcgttcaccctgcatttttttagaggcaggcatcccgggatcgtgttctacaccttcctcaacagtctccttggggcttgtggccgtcctgtgaggcattagttctccctctgagcctggaatctcttttgacgagtcatcatttttcacttttttacactgcatcttggctgcagcatgcctctgtcgttttcgcttccttggcttgtcaaatatcttggtagtgcctccaccaaaatcttttgaataagatgtggcacaagattcagttatgccattctccaggtgaccagcttcatagcactttttagaaaggccaaggtcccccttcttgggcataaatccagggtctaaatcattggattcaagaagtttcttagttggttttctttgacgtttactttcataatttcctggcgttttaactagcaattcctcagactcaagggcaggccgtggagagacttccggagccacaggcacagacaaggtcagctgcggcaactcagcatgtccacctccaagttctgactgagccaaggggccctccaaaaacggagcctccctttcaagaactggaggctcttctttggttgaaatcaaagaattctcgtccacctgcttgttctgagcactagatcgacctcgggctagaaggctttcctcttcacagcgggaacttaccttgtgcacctgctcctgtaccttcttttgttttttcttaggagcaaatatctgatcatattcttctgtatattccaaaagccacttgcttggcttcctaaggcgtttcttctctgaccgcacagctggttcagggagctcagcctgtggtgtcaaactgggaattcctggctccttttccatgtcaccaatgctggcactggatttatcacaaacatttaaccgtggcccagctgaatctaagcagtcagcatgattttgctctgtcagtggttcctcaagtatgcttgctgaaggagttctatgctctggaaactcatcccgcccctcctgcacagggtcactaggaagtaagaccctaaaggcacactcagagttttctttctctttaaatctgttcatgcgcttacgaggtttagtgcgcctttggtttaaacgctgccaccgctttttaggcaccacttgatttacaccattgagttcatcattctcactgttcattacagagtccagctctgggccttttccgttttcaaaagagagtcctttttcagaaattttaccaggatcagattgcttaaccttgctatcgaaatgcacatcagaaaaatggtcaccatcttcacttgttaagtggcccattatctgaaggggatcctctttactaggatcttctgccccacctctcaatgaacctccacgttctcggtctccctgcagtacagcatcaagagtcacacttggaagctgattcagttttcttttgcgctcggtctttaaggctttacggttcactgtgttctttaccatttgggctgaaaaagcatctcgcaatttggatgaaggctttgatcgtccacagttgcgcctagtaacacagtctgaacgacttttaccagaagcagggaggtctctcttgtcggacagtaagccaggtagggaagcagacaactcgccagataatgcagagtcacccccactagggctaggattggcggagttctgagtgccatctccctttttctctgaattgtgtgtggagcctcctgaaaccaaaaccttagagactcctacaggactattagtagaacagtccccacgaccaggactccggtaagagaccaggttttgagcagtcatcaaccgctgctccttcgtcttactatcatgcatatctttcaacatcattagcaatgtactgaatttgtagtctggttcaataggtatgtgattctgactagaagcagaagagaaaagtaatggttttgatggctttgatgttccagagtcactgacatcctcacctaaggatctgtaagagagttccttcaactcggataaaacatgtttcaccactgctgtttctatgtcacttgaatccctggttttctcatgcatattgttcagtagttttagaccatccactttcccacttttagaaatgctggccaaaggagagcctttggtatcagaagagcagcatttcaaactgcactcctcatttataactgggggttctgccataactggattttctttgtgtttgcactttatacttcggaacttgggctgtttgcttttcgaatgtaatagagcttgatttgctgccccaccctttattaacgagttctcactggatatgcttgatgacaggttgaattttggagagagagcatcatttgtaaaatctgactggggtttgtgaacaagagtagatgccttcagatcagagagattaacctgagacgtctcggttccaggctctgcactcttagtacaacccattaagtggtctgtatgtgagttactaatgagaggcttctgttttgcttttaccctagtgtttgtggcagcaaacctagaatactttatcttttcatttttctgcatagataacatgttctctgttctatcgaaagcatctggaatttcaaggacactgttatcagactctgagctgtgttctatgggatccaggtcactgcttccatcatcagaagtggtacagatactaatggaatcacttcgcttttcctcatcacctgctccaatatagcagagcttcacttttgaaccacacaccaggcttcgttggggtttattcttctctcgagaacactttgagatcaaagcaccctcaggcaagcccaataaagagtcaccatttgaagtctcaaattctttctttgcagtgttttttccacaggaagaaaacagaaaacttcctggggcagtgttggaccctgtgaggctatttgctatcctggaaagttcattagaggcctgcgtatcagatatatccccagagataaagtttaggccaaggttctctggaatctttcccctccgttcatctttatgtgcttcaaattgtatgtggccctttttcacactagtcctttttggattatcagagctctttctggctcgagatttagcgcaaggcttttccttctcatctgcagaatgttcagaatcaaaagccagtgatttcaaacagccattaagcaacaggtcatgttctgactcaggatcatttgtgcagtcttcaaatggcatatcttcttcactgtccaacttgattgaaccaggaatacattttcggttctttgaccccttgggaacatcatactgttctgcaagtccaacactggcttcccatttactcaaaattttctgaggaaccttatgcctatatcctttttctttctgtttccctcttctcctaaggacaggtagctcttcgaattgatgtctgccttcaaacatgacgattgcttttccagccacccaggctctctcagaaggatctccaaaagcctccacgtagtactgccgatagggcctccggttggaaactttcatttttgaatgtgtgttaatcaacggatcagaacaaatcctgcagggccaccatgggcgtctcttgaattttgcccagatgagatctccaacttcatacttcagtggcgtagactttttcttaggttgacaaaatggcaattcctgtgaagtagatgatgatgaagttccaggtaattctagcatgtttcctaatgtactggtactggaatctggatcatcctggagttcaggggagttattacaagagggttcctgtttcatagcaagtgctgtaggaccaccaggactcaaggaagtgcaaacaattggcgtctgagctcttgaatcacttttttcagggtcttgaaaggattctgatccatcagcagacccatttaaatactctacattgatcatggaggccaaatcctgtagtctccgcagtggaatgtaacaagatggagaatcttgtccataagcattttgggatgttccactgacagtcgataactgcatagtacacccattaagtggctcagaaaaattggattgaccattaccgaaagggctgtccttgtcttcaggggcatctaaattcactggattggaaaagggcagcagacaatttcttctgggtagttcacaggtctgatccatcctgggccggcatcaaccgtgccccgcgccccctcccgggccagctggggggagggggtgaccctcattacactggggtgcgagcggagcggtggggagagagcggggccgctcgccgcacccccctccccccgcgtctctcttcaggggagaaggcagcgagcgcgacctgccccggcctattccgccgccgcctcctcctcctcac

SEQ ID NO: 17931 - RNA, 7014 nt, Homo sapiens
  source 1..7014: mol_type = other RNA
tcggggcatgggggagggaggctggggccttcccgagagacctaaaagattgcccactcttggcggcaagtgcaggtagttgctggcctccgaccatctgcttcgcctgcttcaccaggcccggggattggctaagaggccctggggtctgctcagcccctgcagaagctcttcctgaggcctgagttgttggctcatataaaaaggccttggcaggaggctgagaaagaagtctggcctgggtgagtgatttaacagcttgccaggggtcctctgaaggggctgctgctttcccagatgtctgaagaggatctgacacacagcctttctcaacagctctcggcatatgccccagacctttgctggcaggccatgaacttgactccaacactggcatcttctcatcagcctgtggtgtgacctgatgaggtgaagctgcccgctccttctggcgaggagttaggtctatgagatccatcaccaaagcagctctattttttgactgagtattctggtccacaggcctcagtgctttttctttagctacaagggtctggaccacagctgatagtactttctcaggaggtgggagtctctgggacaaagaggcatggggtttgtcagtaggcctgtctgaagtctggggtttgggactgctagtaatgagcagtctgtctggcggcggaagtctcaggccagtgggaactgaggttttctccagtgactggggccttgggctggcagcacctatggatttatccagccttgggtcagccgtccccagaggtctttccagtggttgggacctgactgagggtgaggagcttgggctggtcactggagagggtttgtcgcttagctggggtcttggtcctgccactgctggtggcctgtccagtggcctctggctggaaaccaaggattgggatttggtccctgacccagcgaggtctctgaccttatctaaaggctggggcctggagtcagttctctcaagaggtctttcaggtagcaatggcctctgacaagtccctgccagagcttttttggagagcgacagcatctggttggtgtcagcaggaggtttatctgacattttgggtgcctgagcagccattcctgttgattgctctgccaggtgagtgcttggccctggaggcagcggtactgggggaggcacatactcacggatctccccaggttccagaggattgggcccacaggggtcatgctcagtacaagacagacgcccatccagtttggaaatgaaaagcatcccttctcgatgctgcttacaaaaggagctggggcacatctcacagaaggaggctgcttccttcccgcagatgtcacactgatgccacggacattcccatttccctgctggtcgcttggtcagattgagacagtctgcgtggtaaacttttgggcagcctggtttcttgcaggagacgagctggccagcatccccacaactaaaacactcatcttctcgctcctttgtgatttcaccctgggtcctgcgctttccctgttgcttcttcttgaatttctttgacttttcttccgtggcaatgggttgattctttggccttacacccaagaagccactgcagttcggggctccacatttgcaaacagtctttccattcccaagacattctaggttgtagttgaaggtaagttcagtgcctgctttaatgtcacttagtgcaaaaaggcctacacgggtatctccattcacagaccacttctgtgtttcacagttgggctggcagcaatgattcatgaaccgagcatagtttcctttgggaccagcatcaatgattcggtctttgtctagggtgagcatatagaaattagtgatatcatgttcttgagcatagcgaattcgagctctgcattcttcttcatctataagctcacccacatactcattcacaaattcaccctttttaatatctgtttttgtccgtagaccccaaccccgctgtaatgtgcggaaaatttcaacctctggatattggcgcttggaaaagcactggttttgacagcgccctccggcaggacacactgtggggtggcactcatagagcagcatgcggttgatgcattcagagtctatcccacaggggttctcatcagtagctttacagttgcaacggggtatttcagataagtctgcagtgaagatctgtaccctgccaataggacggtttacctttatatgtttataaggtggtggcttcttgtcattctttcggtcttcctgcagctgtcttagctctttttgggcctttaattcctcaaaccttgctgcagcttcctgaagagcttttttatatgtcccatccactcctttgcccatcttatccttgctgctcacgtcaccctccatgtaagggaagactcgggcctggtgagtccacaaatagtcattagatccaaaaaagaggactgggaactctcccacatcatgtctcatcttatcaatgttggaaggaacagctcgaggatggcagatctcagctggccaccacctgtatcgtccaacttttacccagacaatctccctgtagtgtggctttttgcctgctttacagtcattgcaataccagtttccttcagggatatcaatgttcaggcattcacgatgaaaagcagcagggcaagaatcacagcacagaaggctgcctccttctgagcacacaaagcaccagctaacattaacatgctcatgatttcggcagccccgcctaggggtaaagtgattagggcagatgatactattagatgcaaggatctttgacccagcagccaggcaaaagtcattggcgtggtatgccacaggacagcggacacagcgcatcaaccgacctttagatgcagaaacattggctggattagcagcatgacaggttatacagatgtggagggagcaccggaagcccttgttctgcataacagtgggtgggtacttctggacacactcttcatggtaaaactttccacacaagggtagaaggcaccttttaacatcttccccactctgcttacatacaaaacaggtatggattcctgtgcgacattcattgcagataaattttcctcttggcatctcagtcaatccaaggcactccaggtggaaagccccacagcactgagcctcacataacagcagctcacccaatttttcacaattctgacagacattctccttgagtgcagctcctccaccgcgttcaccctgcatttttttagaggcaggcatcccgggatcgtgttctacaccttcctcaacagtctccttggggcttgtggccgtcctgtgaggcattagttctccctctgagcctggaatctcttttgacgagtcatcatttttcacttttttacactgcatcttggctgcagcatgcctctgtcgttttcgcttccttggcttgtcaaatatcttggtagtgcctccaccaaaatcttttgaataagatgtggcacaagattcagttatgccattctccaggtgaccagcttcatagcactttttagaaaggccaaggtcccccttcttgggcataaatccagggtctaaatcattggattcaagaagtttcttagttggttttctttgacgtttactttcataatttcctggcgttttaactagcaattcctcagactcaagggcaggccgtggagagacttccggagccacaggcacagacaaggtcagctgcggcaactcagcatgtccacctccaagttctgactgagccaaggggccctccaaaaacggagcctccctttcaagaactggaggctcttctttggttgaaatcaaagaattctcgtccacctgcttgttctgagcactagatcgacctcgggctagaaggctttcctcttcacagcgggaacttaccttgtgcacctgctcctgtaccttcttttgttttttcttaggagcaaatatctgatcatattcttctgtatattccaaaagccacttgcttggcttcctaaggcgtttcttctctgaccgcacagctggttcagggagctcagcctgtggtgtcaaactgggaattcctggctccttttccatgtcaccaatgctggcactggatttatcacaaacatttaaccgtggcccagctgaatctaagcagtcagcatgattttgctctgtcagtggttcctcaagtatgcttgctgaaggagttctatgctctggaaactcatcccgcccctcctgcacagggtcactaggaagtaagaccctaaaggcacactcagagttttctttctctttaaatctgttcatgcgcttacgaggtttagtgcgcctttggtttaaacgctgccaccgctttttaggcaccacttgatttacaccattgagttcatcattctcactgttcattacagagtccagctctgggccttttccgttttcaaaagagagtcctttttcagaaattttaccaggatcagattgcttaaccttgctatcgaaatgcacatcagaaaaatggtcaccatcttcacttgttaagtggcccattatctgaaggggatcctctttactaggatcttctgccccacctctcaatgaacctccacgttctcggtctccctgcagtacagcatcaagagtcacacttggaagctgattcagttttcttttgcgctcggtctttaaggctttacggttcactgtgttctttaccatttgggctgaaaaagcatctcgcaatttggatgaaggctttgatcgtccacagttgcgcctagtaacacagtctgaacgacttttaccagaagcagggaggtctctcttgtcggacagtaagccaggtagggaagcagacaactcgccagataatgcagagtcacccccactagggctaggattggcggagttctgagtgccatctccctttttctctgaattgtgtgtggagcctcctgaaaccaaaaccttagagactcctacaggactattagtagaacagtccccacgaccaggactccggtaagagaccaggttttgagcagtcatcaaccgctgctccttcgtcttactatcatgcatatctttcaacatcattagcaatgtactgaatttgtagtctggttcaataggtatgtgattctgactagaagcagaagagaaaagtaatggttttgatggctttgatgttccagagtcactgacatcctcacctaaggatctgtaagagagttccttcaactcggataaaacatgtttcaccactgctgtttctatgtcacttgaatccctggttttctcatgcatattgttcagtagttttagaccatccactttcccacttttagaaatgctggccaaaggagagcctttggtatcagaagagcagcatttcaaactgcactcctcatttataactgggggttctgccataactggattttctttgtgtttgcactttatacttcggaacttgggctgtttgcttttcgaatgtaatagagcttgatttgctgccccaccctttattaacgagttctcactggatatgcttgatgacaggttgaattttggagagagagcatcatttgtaaaatctgactggggtttgtgaacaagagtagatgccttcagatcagagagattaacctgagacgtctcggttccaggctctgcactcttagtacaacccattaagtggtctgtatgtgagttactaatgagaggcttctgttttgcttttaccctagtgtttgtggcagcaaacctagaatactttatcttttcatttttctgcatagataacatgttctctgttctatcgaaagcatctggaatttcaaggacactgttatcagactctgagctgtgttctatgggatccaggtcactgcttccatcatcagaagtggtacagatactaatggaatcacttcgcttttcctcatcacctgctccaatatagcagagcttcacttttgaaccacacaccaggcttcgttggggtttattcttctctcgagaacactttgagatcaaagcaccctcaggcaagcccaataaagagtcaccatttgaagtctcaaattctttctttgcagtgttttttccacaggaagaaaacagaaaacttcctggggcagtgttggaccctgtgaggctatttgctatcctggaaagttcattagaggcctgcgtatcagatatatccccagagataaagtttaggccaaggttctctggaatctttcccctccgttcatctttatgtgcttcaaattgtatgtggccctttttcacactagtcctttttggattatcagagctctttctggctcgagatttagcgcaaggcttttccttctcatctgcagaatgttcagaatcaaaagccagtgatttcaaacagccattaagcaacaggtcatgttctgactcaggatcatttgtgcagtcttcaaatggcatatcttcttcactgtccaacttgattgaaccaggaatacattttcggttctttgaccccttgggaacatcatactgttctgcaagtccaacactggcttcccatttactcaaaattttctgaggaaccttatgcctatatcctttttctttctgtttccctcttctcctaaggacaggtagctcttcgaattgatgtctgccttcaaacatgacgattgcttttccagccacccaggctctctcagaaggatctccaaaagcctccacgtagtactgccgatagggcctccggttggaaactttcatttttgaatgtgtgttaatcaacggatcagaacaaatcctgcagggccaccatgggcgtctcttgaattttgcccagatgagatctccaacttcatacttcagtggcgtagactttttcttaggttgacaccctcacaaccttacaagacagcattatctcgattttgcagataaagaaactgaggctcaaaaaggttaagtcacaggctgggtgcggtggctcatgc

SEQ ID NO: 17932 - RNA, 6691 nt, Homo sapiens
  source 1..6691: mol_type = other RNA
tcggggcatgggggagggaggctggggccttcccgagagacctaaaagattgcccactcttggcggcaagtgcaggtagttgctggcctccgaccatctgcttcgcctgcttcaccaggcccggggattggctaagaggccctggggtctgctcagcccctgcagaagctcttcctgaggcctgagttgttggctcatataaaaaggccttggcaggaggctgagaaagaagtctggcctgggtgagtgatttaacagcttgccaggggtcctctgaaggggctgctgctttcccagatgtctgaagaggatctgacacacagcctttctcaacagctctcggcatatgccccagacctttgctggcaggccatgaacttgactccaacactggcatcttctcatcagcctgtggtgtgacctgatgaggtgaagctgcccgctccttctggcgaggagttaggtctatgagatccatcaccaaagcagctctattttttgactgagtattctggtccacaggcctcagtgctttttctttagctacaagggtctggaccacagctgatagtactttctcaggaggtgggagtctctgggacaaagaggcatggggtttgtcagtaggcctgtctgaagtctggggtttgggactgctagtaatgagcagtctgtctggcggcggaagtctcaggccagtgggaactgaggttttctccagtgactggggccttgggctggcagcacctatggatttatccagccttgggtcagccgtccccagaggtctttccagtggttgggacctgactgagggtgaggagcttgggctggtcactggagagggtttgtcgcttagctggggtcttggtcctgccactgctggtggcctgtccagtggcctctggctggaaaccaaggattgggatttggtccctgacccagcgaggtctctgaccttatctaaaggctggggcctggagtcagttctctcaagaggtctttcaggtagcaatggcctctgacaagtccctgccagagcttttttggagagcgacagcatctggttggtgtcagcaggaggtttatctgacattttgggtgcctgagcagccattcctgttgattgctctgccaggtgagtgcttggccctggaggcagcggtactgggggaggcacatactcacggatctccccaggttccagaggattgggcccacaggggtcatgctcagtacaagacagacgcccatccagtttggaaatgaaaagcatcccttctcgatgctgcttacaaaaggagctggggcacatctcacagaaggaggctgcttccttcccgcagatgtcacactgatgccacggacattcccatttccctgctggtcgcttggtcagattgagacagtctgcgtggtaaacttttgggcagcctggtttcttgcaggagacgagctggccagcatccccacaactaaaacactcatcttctcgctcctttgtgatttcaccctgggtcctgcgctttccctgttgcttcttcttgaatttctttgacttttcttccgtggcaatgggttgattctttggccttacacccaagaagccactgcagttcggggctccacatttgcaaacagtctttccattcccaagacattctaggttgtagttgaaggtaagttcagtgcctgctttaatgtcacttagtgcaaaaaggcctacacgggtatctccattcacagaccacttctgtgtttcacagttgggctggcagcaatgattcatgaaccgagcatagtttcctttgggaccagcatcaatgattcggtctttgtctagggtgagcatatagaaattagtgatatcatgttcttgagcatagcgaattcgagctctgcattcttcttcatctataagctcacccacatactcattcacaaattcaccctttttaatatctgtttttgtccgtagaccccaaccccgctgtaatgtgcggaaaatttcaacctctggatattggcgcttggaaaagcactggttttgacagcgccctccggcaggacacactgtggggtggcactcatagagcagcatgcggttgatgcattcagagtctatcccacaggggttctcatcagtagctttacagttgcaacggggtatttcagataagtctgcagtgaagatctgtaccctgccaataggacggtttacctttatatgtttataaggtggtggcttcttgtcattctttcggtcttcctgcagctgtcttagctctttttgggcctttaattcctcaaaccttgctgcagcttcctgaagagcttttttatatgtcccatccactcctttgcccatcttatccttgctgctcacgtcaccctccatgtaagggaagactcgggcctggtgagtccacaaatagtcattagatccaaaaaagaggactgggaactctcccacatcatgtctcatcttatcaatgttggaaggaacagctcgaggatggcagatctcagctggccaccacctgtatcgtccaacttttacccagacaatctccctgtagtgtggctttttgcctgctttacagtcattgcaataccagtttccttcagggatatcaatgttcaggcattcacgatgaaaagcagcagggcaagaatcacagcacagaaggctgcctccttctgagcacacaaagcaccagctaacattaacatgctcatgatttcggcagccccgcctaggggtaaagtgattagggcagatgatactattagatgcaaggatctttgacccagcagccaggcaaaagtcattggcgtggtatgccacaggacagcggacacagcgcatcaaccgacctttagatgcagaaacattggctggattagcagcatgacaggttatacagatgtggagggagcaccggaagcccttgttctgcataacagtgggtgggtacttctggacacactcttcatggtaaaactttccacacaagggtagaaggcaccttttaacatcttccccactctgcttacatacaaaacaggtatggattcctgtgcgacattcattgcagataaattttcctcttggcatctcagtcaatccaaggcactccaggtggaaagccccacagcactgagcctcacataacagcagctcacccaatttttcacaattctgacagacattctccttgagtgcagctcctccaccgcgttcaccctgcatttttttagaggcaggcatcccgggatcgtgttctacaccttcctcaacagtctccttggggcttgtggccgtcctgtgaggcattagttctccctctgagcctggaatctcttttgacgagtcatcatttttcacttttttacactgcatcttggctgcagcatgcctctgtcgttttcgcttccttggcttgtcaaatatcttggtagtgcctccaccaaaatcttttgaataagatgtggcacaagattcagttatgccattctccaggtgaccagcttcatagcactttttagaaaggccaaggtcccccttcttgggcataaatccagggtctaaatcattggattcaagaagtttcttagttggttttctttgacgtttactttcataatttccttgtgcacctgctcctgtaccttcttttgttttttcttaggagcaaatatctgatcatattcttctgtatattccaaaagccacttgcttggcttcctaaggcgtttcttctctgaccgcacagctggttcagggagctcagcctgtggtgtcaaactgggaattcctggctccttttccatgtcaccaatgctggcactggatttatcacaaacatttaaccgtggcccagctgaatctaagcagtcagcatgattttgctctgtcagtggttcctcaagtatgcttgctgaaggagttctatgctctggaaactcatcccgcccctcctgcacagggtcactaggaagtaagaccctaaaggcacactcagagttttctttctctttaaatctgttcatgcgcttacgaggtttagtgcgcctttggtttaaacgctgccaccgctttttaggcaccacttgatttacaccattgagttcatcattctcactgttcattacagagtccagctctgggccttttccgttttcaaaagagagtcctttttcagaaattttaccaggatcagattgcttaaccttgctatcgaaatgcacatcagaaaaatggtcaccatcttcacttgttaagtggcccattatctgaaggggatcctctttactaggatcttctgccccacctctcaatgaacctccacgttctcggtctccctgcagtacagcatcaagagtcacacttggaagctgattcagttttcttttgcgctcggtctttaaggctttacggttcactgtgttctttaccatttgggctgaaaaagcatctcgcaatttggatgaaggctttgatcgtccacagttgcgcctagtaacacagtctgaacgacttttaccagaagcagggaggtctctcttgtcggacagtaagccaggtagggaagcagacaactcgccagataatgcagagtcacccccactagggctaggattggcggagttctgagtgccatctccctttttctctgaattgtgtgtggagcctcctgaaaccaaaaccttagagactcctacaggactattagtagaacagtccccacgaccaggactccggtaagagaccaggttttgagcagtcatcaaccgctgctccttcgtcttactatcatgcatatctttcaacatcattagcaatgtactgaatttgtagtctggttcaataggtatgtgattctgactagaagcagaagagaaaagtaatggttttgatggctttgatgttccagagtcactgacatcctcacctaaggatctgtaagagagttccttcaactcggataaaacatgtttcaccactgctgtttctatgtcacttgaatccctggttttctcatgcatattgttcagtagttttagaccatccactttcccacttttagaaatgctggccaaaggagagcctttggtatcagaagagcagcatttcaaactgcactcctcatttataactgggggttctgccataactggattttctttgtgtttgcactttatacttcggaacttgggctgtttgcttttcgaatgtaatagagcttgatttgctgccccaccctttattaacgagttctcactggatatgcttgatgacaggttgaattttggagagagagcatcatttgtaaaatctgactggggtttgtgaacaagagtagatgccttcagatcagagagattaacctgagacgtctcggttccaggctctgcactcttagtacaacccattaagtggtctgtatgtgagttactaatgagaggcttctgttttgcttttaccctagtgtttgtggcagcaaacctagaatactttatcttttcatttttctgcatagataacatgttctctgttctatcgaaagcatctggaatttcaaggacactgttatcagactctgagctgtgttctatgggatccaggtcactgcttccatcatcagaagtggtacagatactaatggaatcacttcgcttttcctcatcacctgctccaatatagcagagcttcacttttgaaccacacaccaggcttcgttggggtttattcttctctcgagaacactttgagatcaaagcaccctcaggcaagcccaataaagagtcaccatttgaagtctcaaattctttctttgcagtgttttttccacaggaagaaaacagaaaacttcctggggcagtgttggaccctgtgaggctatttgctatcctggaaagttcattagaggcctgcgtatcagatatatccccagagataaagtttaggccaaggttctctggaatctttcccctccgttcatctttatgtgcttcaaattgtatgtggccctttttcacactagtcctttttggattatcagagctctttctggctcgagatttagcgcaaggcttttccttctcatctgcagaatgttcagaatcaaaagccagtgatttcaaacagccattaagcaacaggtcatgttctgactcaggatcatttgtgcagtcttcaaatggcatatcttcttcactgtccaacttgattgaaccaggaatacattttcggttctttgaccccttgggaacatcatactgttctgcaagtccaacactggcttcccatttactcaaaattttctgaggaaccttatgcctatatcctttttctttctgtttccctcttctcctaaggacaggtagctcttcgaattgatgtctgccttcaaacatgacgattgcttttccagccacccaggctctctcagaaggatctccaaaagcctccacgtagtactgccgatagggcctccggttggaaactttcatttttgaatgtgtgttaatcaacggatcagaacaaatcctgcagggccaccatgggcgtctcttgaattttgcccagatgagatctccaacttcatacttcagtggcgtagactttttcttaggttgacaaaatggcaattcctgtgaagtagatgatgatgaagttccaggtaat

SEQ ID NO: 17933 - RNA, 260 nt, Homo sapiens
  source 1..260: mol_type = other RNA
tcggggcatgggggagggaggctgggtctctgtgaggccaggggttccagaaccccctcccccagtggctgtttaaagggataatcactccccccaccaccatcgcatacacccccgcagctctcaactgagtgactgcttagattcagatctcagctttgggggccgttacatgataggccgagtccttcttttatcattattatcattattattttttgagatggagtcttgctctgtcacccaggctggagcgcagt

SEQ ID NO: 17934 - RNA, 21 nt, Homo sapiens
  source 1..21: mol_type = other RNA
tcgtgcatatatctaccacat

SEQ ID NO: 17935 - RNA, 2563 nt, Homo sapiens
  source 1..2563: mol_type = other RNA
tcgtgtccctcttgtccacagctgtgctttggggcccacagtctgctgtaaaaggatgctggcttgtaagagatgagggtaggcagggagcaacctggatgtgagtttgcagatctgggcaaggaacttttcatctctgggtctctggttcttcatttggttacatcaattacctacaatattctagctctaatgtttatgattactgaattgcatccacatctagactaactagacgtgatgcttctggttcagcccagctagcaatcaagcattggatcagaaaggtgacatctacttttgaaaagggagagacattgagagagagaaaaagagagagagagagaaaagcaacatgttatctcagcaaaccaagctcagggacctataattctgtctggaattatggacatctataattttccctgatttctctgggggaatagcccggcacagatccatggaacctgccctgttgttgttgttgttgttttcccgtgggtctcgggtaaggtccaggcaactgtattttgcatactccaagtaatttaaaagcttgccaaattgtgaaggtctctgttttaaaccatttgcctcttgcctaaccagactttctggtcttgccttgttccagacttttggcatcctaatctgaacaaaatcatctaatctgaataagatcactacccacatttacgaagtggcccaaactatccttcatctagattctaccattaacagaagcctcaccaaggtatagaaagattaagacagtggcccagggagccatttatattctcaaaagttatctgaatcgtagcagaatgggcaacaggccttgcttgatgggattcctgggcctggctctgctttgaattttggcctcaaacattgcagaagctctctttgcctctcaagatatgaaatatccaaatgggcaaagtctagcatgaagacgaagcttggtcttcagccccatgacagacactaccaggaaactagactgcaaaccccaaggcccaagacttcctctacctgggggtattgggtgtggaattggcactcaacgccttcctggtggcaagtgttgcttgatgaaaccaaagtgtcctccaggtttcttcttgctcgttaggaaccagcccgcacagcaggagctgagcagcaggcaagcgagccaagcttcatctgtatttacagctgctccccatcactcgcattactgcctcagctccacctcctccattcttcctctatagtttcactgaaattctgcagattcatattcgatgctcttcaagtaaattaaagtggaggtcaggcctgaagaatctctgaaagaggtgggccaagatctgatttctagagttctgaggagaaacagcttttgccaagtaaagcacattttcagtcacggagcctggagaaaggactagcagcatccaggtggggagcagattcatccacctgccatcagggatccagggctgtgctccagagtcaccgttttcctaaagacctcgaggctcaaggtgagcaccatttgtcttctgggtgtccttctttccctcttttggtatctcctccctcttttggcatcctcatctattcagcaaacatcaatagaggacatcatatgtgccgaagactctctcaggggtgtctgccaagcctgtgctgtcagctgctgtcctgggaagcccagcaggtacttatgccaccggcattgacctcgtgaaagccttttttggagcctaacaaaactgcctcgagagctcgtttatgagccccctccactgcggcatttatctacacggtgaaaatcttgctctgagaagcaatgttgaatcccacagatgcttgtccctgggactcatcaggggacaaagacagagccacacagccctcattaatccacgtggaaataaaaaagattaagcagcatagaccctgtgaccactgagaaaatgacagaaataaagatcattatgtgcatctggttttccaggggaaagaaacggagataaagccttaagtctttaataaggctagaaattaaaactgggattaacaacaacacgaagcatttataagaagccgtccatgacattcctgcttaggttttgctggcctggtttctggaacattttttatattgttaatatttatcaccagctttttctttagttgaaaaaaaagtcactgcccactggtttcaggttcacagccttctctctagacatactagacctgcttcaagacgatacttgtttaaaaccaattattcagcaccattttcatgaggtttctgtagagataggggagtatgtattgcttaatttcaatgaagttttgaggtctggctttgctctgtgatacacagaggaaacagcttcccaggagagctgtccatgcaccacgcatcttaggcctgggaggggcaggaggggaggatggactatccccacatttagacaccccagattctcctaccagagatgcagtggacatcggcgcctatccaggaggctgtgttaaaatgtaactgtgccatttggttgaa

SEQ ID NO: 17936 - RNA, 443 nt, Homo sapiens
  source 1..443: mol_type = other RNA
tcgtttgcctttttctgcttctgctgcatgatctccgagtccctctgcttgcgggcggcagcagaaagcccgtcatctcggcgctttcccttaaccgagtcgctctgctttttcatattcttctggcgggcgagctcacgctggttaccgcaccgcggaagatccgggagggcctatgcctaacccgggagggtggtcccgtgaagtagccgtgggcaaagggctcgatttccgggcaccgagtgtgagggtggccacagagcgcgcccagagaaacgccttgctagggaagctacggaaggtcaaagccggcgcctcgccggtggtgtttagggtgaacggaaagaaaagggcaaggagaagggggctcggtgctcacgggtcatggcgacggcagcggctccaacctgcctccgttacgtcccctcgttctgtcggacgtt

SEQ ID NO: 17937 - RNA, 215 nt, Homo sapiens
  source 1..215: mol_type = other RNA
tcgtttgcctttttctgcttctgctgcatgatctccgagtccctctgcttgcgggcggcagcagaaagcccgtcatctcggcgctttcccttaaccgagtcgctctgctttttcatattcttctggcgggcgagctcacgctggttaccgcgggtcatggcgacggcagcggctccaacctgcctccgttacgtcccctcgttctgtcggacgtt

SEQ ID NO: 17938 - RNA, 559 nt, Homo sapiens
  source 1..559: mol_type = other RNA
tcgtttgcctttttctgcttctgctgcatgatctccgagtccctctgcttgcgggcggcagcagaaagcccgtcatctcggcgctttcccttaaccgagtcgctctgctttttcatattcttctggcgggcgagctcacgctggttaccgcgggtcatggcgacggcagcggctccaacctgcctccgttacgtcccctcgttctgtcggacgttgcaggtcccgccccttctggcaacgtagcacagtcgttcctttcctccccgccccttcgcgcccgggagccggctcccattggacaagaaaaagcacgtggatccacgggtcgtgcttgagccggggtgggtaagtggcggagggtcgcaggcggagcgctcagcgtggggcggggcttcccgagtgagacgtagggacgggcctggagaaactaggccgggtcacgtgggcaggttgggggtggaggggtgcggctggcgatgtggcgctcccgcgggctcgagcacgtgaccgtgcagagtgacctcatgcggggacagtttggggtactgacaaagtcgcc

SEQ ID NO: 17939 - RNA, 1101 nt, Homo sapiens
  source 1..1101: mol_type = other RNA
tcgtttgcctttttctgcttctgctgcatgatctccgagtccctctgcttgcgggcggcagcagaaagcccgtcatctcggcgctttcccttaaccgagtcgctctgctttttcatattcttctggcgggcgagctcacgctggttaccgcgggtcatggcgacggcagcggctccaacctgcctccgttacgtcccctcgttctgtcggacgttgcaggtcccgccccttctggcaacgtagcacagtcgttcctttcctccccgccccttcgcgcccgggagccggctcccattggacaagaaaaagcacgtggatccacgggtcgtgcttgagccggggtgggtaagtggcggagggtcgcaggcggagcgctcagcgtggggcggggcttcccgagtgagacgtagggacgggcctggagaaactaggccgggtcacgtgggcaggttgggggtggaggggtgcggctggcgatgtggcgctcccgcgggctcgagcacgtgaccgtgcagagtgacctcatgcggggacagtttggggtactgacaaagtcgccctgtagtccttagctactcaggaggctgagatgggaggattgcttgaatccaggaattcaaagttgtagtgagtcgtgatctcgccaccgtactccagcatgggtaacagagcaagactatgtctctctctgttagaaatcggtttcagagcggtggaaccgcgggcgggaaaaagcccaggcgctgtctcgggtgccccttcgtgtcagccatcctctggtctctcgggtctccgaagctcggggctaactgggcgcgaaccgctgagcccgcctaccaaccaggccctttctcccgcccctctgcggctgaaaccctcaaggggttgcaggttcagctttcacttagagacagcaactccaaattcagggtcgctggggaaactaaggcaggactggggactctgagtgagaggtcagacgctggtcgcggactctttctcccgagaactggggatagctcttccgatagcccaaagcgattcatgcggatcctagaagaaagcgccgaggtccgggcggttggccggggagagcgaagc

SEQ ID NO: 17940 - RNA, 582 nt, Homo sapiens
  source 1..582: mol_type = other RNA
tcgtttgcctttttctgcttctgctgcatgatctccgagtccctgggggtagagatgatggggcactctgcttgcgggcggcagcagaaagcccgtcatctcggcgctttcccttaaccgagtcgctctgctttttcatattcttctggcgggcgagctcacgctggttaccgcgggtcatggcgacggcagcggctccaacctgcctccgttacgtcccctcgttctgtcggacgttgcaggtcccgccccttctggcaacgtagcacagtcgttcctttcctccccgccccttcgcgcccgggagccggctcccattggacaagaaaaagcacgtggatccacgggtcgtgcttgagccggggtgggtaagtggcggagggtcgcaggcggagcgctcagcgtggggcggggcttcccgagtgagacgtagggacgggcctggagaaactaggccgggtcacgtgggcaggttgggggtggaggggtgcggctggcgatgtggcgctcccgcgggctcgagcacgtgaccgtgcagagtgacctcatgcggggacagtttggggtactgacaaagtcgcc

SEQ ID NO: 17941 - RNA, 693 nt, Homo sapiens
  source 1..693: mol_type = other RNA
tcgtttgcctttttctgcttctgctgcatgatctccgagtccctgggggtagagatgatggggcactgggaggtaccagagggcaaaaaggacaagatgcagggggatgaagggcacaaaggataagatggaagtggatgggactaagttcagcgtttggctgctgtactcccaccctctgcttgcgggcggcagcagaaagcccgtcatctcggcgctttcccttaaccgagtcgctctgctttttcatattcttctggcgggcgagctcacgctggttaccgcgggtcatggcgacggcagcggctccaacctgcctccgttacgtcccctcgttctgtcggacgttgcaggtcccgccccttctggcaacgtagcacagtcgttcctttcctccccgccccttcgcgcccgggagccggctcccattggacaagaaaaagcacgtggatccacgggtcgtgcttgagccggggtgggtaagtggcggagggtcgcaggcggagcgctcagcgtggggcggggcttcccgagtgagacgtagggacgggcctggagaaactaggccgggtcacgtgggcaggttgggggtggaggggtgcggctggcgatgtggcgctcccgcgggctcgagcacgtgaccgtgcagagtgacctcatgcggggacagtttggggtactgacaaagtcgcc

SEQ ID NO: 17942 - RNA, 3041 nt, Homo sapiens
  source 1..3041: mol_type = other RNA
tcgtttgcctttttctgctttcagagagaaaggtgtttgagcaagaaaacataggatatttcccaccacgaaacagacataattttgagggctcagcacaaaatgaaatcatggggcccttcttcaaacattattaagaatttccgctatagcagagccttgaaccaagtgtggggtccttctaagtgtgggccctgtgctgctacacaagttacacgctaagaaagccagccctgcctaggttccccgcctactcagattgccaaaaggagataaagtggctcaattgggttgtccagatgaaaagcaggtattttttttatgatgattcaaacactgtcatcaattgagaactaagtggcatttcactttccaaatggccggcaaatttctattcctaaaatctcatgttggactgattggttttcccctagatttctcattatacaaatggttatgctgggtctttaaatgccccttattttaatagagcaattaatcagacatgattaaatttctgtattaatcctacgtaattttttttttttaatctaagcatttcttaactgagaggggtctaaatatcactaaagcaacaggacatctttaagggaaaacagctgcaaaacagctttgcattctagagtgaaagccttagttttagcctatggtatattttgttcccttttaagaccacagtggtagtttttttccaaagagaactaataaacatattaagctatatggtaatttttctaacacccacattggtttcggtcagaagaattttactggaacctggaggtatcccattcttcataataataaaaaagaaatgtagtgtataaaagctccaggttacattactaagcaacgacatttccgggagtgaatatacttcctgtattccgcaagctgcttcaagtacatattcgacggccatctgtgcttttcaacaaaactgcgttcttccactgaaagatcctgaaattcaggcttttgactgaagatgaggtagttagtagcaatgaaatgaagtagccaggttgaaaggcaatcagagtggtgaaacttggcctttttaagcaggtcaactatatcaaggttcatggatgccagttccctgcttggcatgctctgcagctgggtaatgatgaacagctcacagatgtgctgcagtctggacacttggtacatctcggcacagatcaggagacacatggcctggaatatgccagctgggcagcaggagtctgtgtacaggtattctaaaaatgacaagaaagtctctttggaaacaccataaacgggaatcaggacactctttgcttccatgtaattaccattaaacatggctgccatcacttcacaacgggccaccaggatggccctgtgggctggcactgtcgtaccttgaatttcgaagacaacatcggcaagcatcggcttattaaggaaaaacttgagggaagtgttataaaaccacaaaggttttctggcttgataggttttgcaattccttaggcaattaatctttcctggtgtttttaaaatgcatttaactttctcgattacatttgaaacatccccagaatctttcaacttcttcctgatatcttcttccaattcttcccactgaaaagcacctgaataaatgaagcgaaggatgtctgataaacaagaacagaagagggcgtctttaacaatgactcgtaatggtgggttgcctgaagattcatggctagcacctggaaatgcagtatctctgtttatagcaaaaagatcctgggtagttcggatgatactggaatcctgaatgtcagtgggactcttcacattgaaaagcagcatgaaaacatggcttacagcgcagagaacgatcttgtgggcctctacaactttctttaaattggggttgtaaaataccacgtccacacactggcagcagaacagcaagttatttaagtcagagttataatgtgacgcttcagcctttaagacaggcattttttctggttgttcaagttgaggtggtctaattccatgaaaggagttgctcatttttcttttcttcattttttcacttgtcttctgatttaaggcttgaatcataaaatactccaacactcctccaaaatactttcctatgtagaagtcatcaaggctgtggagttcaagataggtcgctcctagttcttttgcaagttggatcccttcagttgtactaacacagctccctctgtctgaggtacatagtgggcatgtacaaggtaactcttcattttgtctggtaccaacagcagcaataattactggaactgaatttaatgctctttttatcactggaatataattatcctttacttcatggaatgaaaacttgtcattaacgttgtatttgatcacaatgatgtcagcgcccccaattagatttcgagaagtgtaccaatcactgtcaaatatgtcccagacgggacagtcgtggaccaccagcttgacattcccaaacgcactggcctgatactcggtgaacaccggacgcgcgaccgtgctggccgcgttcagcaacaagctgctctcgtccccggagaccagagggcttctccccaggtaagtgcggataagccccgacggccggttgtcctggtggaatgtgtccccctcgttccccagcgccacgatgtggatggacatgatctcaaatccaagggcagggcggcgactcggagaaaagcagcggctcacggcttcgcggggcccccgggcggcgagttcacccgcaatccgctcatccccggccgcgtccccctcgcgcgcctccaccgcggcggggccgacgcagagcggggccggggccgcgccagccagcgagcgagccggggaccagggcgggctagcgggcgggggataagctgccgctactcagggagtgcccgggaacatcgccgggcgcgggaccgccgcacagccccaagtggacgcagctgaccgcagtcccctctccgccgcgcctcctcggctggcagctgtcgcctcctgct

SEQ ID NO: 17943 - RNA, 2992 nt, Homo sapiens
  source 1..2992: mol_type = other RNA
tcgtttgcctttttctgctttcagagagaaaggtgtttgagcaagaaaacataggatatttcccaccacgaaacagacataattttgagggctcagcacaaaatgaaatcatggggcccttcttcaaacattattaagaatttccgctatagcagagccttgaaccaagtgtggggtccttctaagtgtgggccctgtgctgctacacaagttacacgctaagaaagccagccctgcctaggttccccgcctactcagattgccaaaaggagataaagtggctcaattgggttgtccagatgaaaagcaggtattttttttatgatgattcaaacactgtcatcaattgagaactaagtggcatttcactttccaaatggccggcaaatttctattcctaaaatctcatgttggactgattggttttcccctagatttctcattatacaaatggttatgctgggtctttaaatgccccttattttaatagagcaattaatcagacatgattaaatttctgtattaatcctacgtaattttttttttttaatctaagcatttcttaactgagaggggtctaaatatcactaaagcaacaggacatctttaagggaaaacagctgcaaaacagctttgcattctagagtgaaagccttagttttagcctatggtatattttgttcccttttaagaccacagtggtagtttttttccaaagagaactaataaacatattaagctatatggtaatttttctaacacccacattggtttcggtcagaagaattttactggaacctggaggtatcccattcttcataataataaaaaagaaatgtagtgtataaaagctccaggttacattactaagcaacgacatttccgggagtgaatatacttcctgtattccgcaagctgcttcaagtacatattcgacggccatctgtgcttttcaacaaaactgcgttcttccactgaaagatcctgaaattcaggcttttgactgaagatgaggtagttagtagcaatgaaatgaagtagccaggttgaaaggcaatcagagtggtgaaacttggcctttttaagcaggtcaactatatcaaggttcatggatgccagttccctgcttggcatgctctgcagctgggtaatgatgaacagctcacagatgtgctgcagtctggacacttggtacatctcggcacagatcaggagacacatggcctggaatatgccagctgggcagcaggagtctgtgtacaggtattctaaaaatgacaagaaagtctctttggaaacaccataaacgggaatcaggacactctttgcttccatgtaattaccattaaacatggctgccatcacttcacaacgggccaccaggatggccctgtgggctggcactgtcgtaccttgaatttcgaagacaacatcggcaagcatcggcttattaaggaaaaacttgagggaagtgttataaaaccacaaaggttttctggcttgataggttttgcaattccttaggcaattaatctttcctggtgtttttaaaatgcatttaactttctcgattacatttgaaacatccccagaatctttcaacttcttcctgatatcttcttccaattcttcccactgaaaagcacctgaataaatgaagcgaaggatgtctgataaacaagaacagaagagggcgtctttaacaatgactcgtaatggtgggttgcctgaagattcatggctagcacctggaaatgcagtatctctgtttatagcaaaaagatcctgggtagttcggatgatactggaatcctgaatgtcagtgggactcttcacattgaaaagcagcatgaaaacatggcttacagcgcagagaacgatcttgtgggcctctacaactttctttaaattggggttgtaaaataccacgtccacacactggcagcagaacagcaagttatttaagtcagagttataatgtgacgcttcagcctttaagacaggcattttttctggttgttcaagttgaggtggtctaattccatgaaaggagttgctcatttttcttttcttcattttttcacttgtcttctgatttaaggcttgaatcataaaatactccaacactcctccaaaatactttcctatgtagaagtcatcaaggctgtggagttcaagataggtcgctcctagttcttttgcaagttggatcccttcagttgtactaacacagctccctctgtctgaggtacatagtgggcatgtacaaggtaactcttcattttgtctggtaccaacagcagcaataattactggaactgaatttaatgctctttttatcactggaatataattatcctttacttcatggaatgaaaacttgtcattaacgttgtatttgatcacaatgatgtcagcgcccccaattagatttcgagaagtgtaccaatcactgtcaaatatgtcccagacgggacagtcgtggaccaccagcttgacattcccaaacgcactggcctgatactcggtgaacaccggacgcgcgaccgtgctggccgcgttcagcaacaagctgctctcgtccccggagaccagagggcttctccccaggtaagtgcggataagccccgacggccggttgtcctggtggaatgtgtccccctcgttccccagcgccacgatgtggatggaccttttcttttaaccctttgtttgtccctccaggcccgttcttcctcttctccatcctgctccatccactgggaagctagcttgtatatcgacagattcctttggcctctggcttctagttaggtttagtcaatgcagagatcagaggcagcagaatgagacaggatattttcttcccctggctcctccccttcagagtctcctttgtcaccaactgtattagctgagttataattctgcaggctgtacaggattctgcttctggggaggcctcaggaaatttccaatcatggcagaaggt

SEQ ID NO: 17944 - RNA, 3113 nt, Homo sapiens
  source 1..3113: mol_type = other RNA
tcgtttgcctttttctgctttcagagagaaaggtgtttgagcaagaaaacataggatatttcccaccacgaaacagacataattttgagggctcagcacaaaatgaaatcatggggcccttcttcaaacattattaagaatttccgctatagcagagccttgaaccaagtgtggggtccttctaagtgtgggccctgtgctgctacacaagttacacgctaagaaagccagccctgcctaggttccccgcctactcagattgccaaaaggagataaagtggctcaattgggttgtccagatgaaaagcaggtattttttttatgatgattcaaacactgtcatcaattgagaactaagtggcatttcactttccaaatggccggcaaatttctattcctaaaatctcatgttggactgattggttttcccctagatttctcattatacaaatggttatgctgggtctttaaatgccccttattttaatagagcaattaatcagacatgattaaatttctgtattaatcctacgtaattttttttttttaatctaagcatttcttaactgagaggggtctaaatatcactaaagcaacaggacatctttaagggaaaacagctgcaaaacagctttgcattctagagtgaaagccttagttttagcctatggtatattttgttcccttttaagaccacagtggtagtttttttccaaagagaactaataaacatattaagctatatggtaatttttctaacacccacattggtttcggtcagaagaattttactggaacctggaggtatcccattcttcataataataaaaaagaaatgtagtgtataaaagctccaggttacattactaagcaacgacatttccgggagtgaatatacttcctgtattccgcaagctgcttcaagtacatattcgacggccatctgtgcttttcaacaaaactgcgttcttccactgaaagatcctgaaattcaggcttttgactgaagatgaggtagttagtagcaatgaaatgaagtagccaggttgaaaggcaatcagagtggtgaaacttggcctttttaagcaggtcaactatatcaaggttcatggatgccagttccctgcttggcatgctctgcagctgggtaatgatgaacagctcacagatgtgctgcagtctggacacttggtacatctcggcacagatcaggagacacatggcctggaatatgccagctgggcagcaggagtctgtgtacaggtattctaaaaatgacaagaaagtctctttggaaacaccataaacgggaatcaggacactctttgcttccatgtaattaccattaaacatggctgccatcacttcacaacgggccaccaggatggccctgtgggctggcactgtcgtaccttgaatttcgaagacaacatcggcaagcatcggcttattaaggaaaaacttgagggaagtgttataaaaccacaaaggttttctggcttgataggttttgcaattccttaggcaattaatctttcctggtgtttttaaaatgcatttaactttctcgattacatttgaaacatccccagaatctttcaacttcttcctgatatcttcttccaattcttcccactgaaaagcacctgaataaatgaagcgaaggatgtctgataaacaagaacagaagagggcgtctttaacaatgactcgtaatggtgggttgcctgaagattcatggctagcacctggaaatgcagtatctctgtttatagcaaaaagatcctgggtagttcggatgatactggaatcctgaatgtcagtgggactcttcacattgaaaagcagcatgaaaacatggcttacagcgcagagaacgatcttgtgggcctctacaactttctttaaattggggttgtaaaataccacgtccacacactggcagcagaacagcaagttatttaagtcagagttataatgtgacgcttcagcctttaagacaggcattttttctggttgttcaagttgaggtggtctaattccatgaaaggagttgctcatttttcttttcttcattttttcacttgtcttctgatttaaggcttgaatcataaaatactccaacactcctccaaaatactttcctatgtagaagtcatcaaggctgtggagttcaagataggtcgctcctagttcttttgcaagttggatcccttcagttgtactaacacagctccctctgtctgaggtacatagtgggcatgtacaaggtaactcttcattttgtctggtaccaacagcagcaataattactggaactgaatttaatgctctttttatcactggaatataattatcctttacttcatggaatgaaaacttgtcattaacgttgtatttgatcacaatgatgtcagcgcccccaattagatttcgagaagtgtaccaatcactgtcaaatatgtcccagacgggacagtcgtggaccaccagcttgacattcccaaacgcactggcctgatactcggtgaacaccggacgcgcgaccgtgctggccgcgttcagcaacaagctgctctcgtccccggagaccagagggcttctccccaggtaagtgcggataagccccgacggccggttgtcctggtggaatgtgtccccctcgttccccagcgccacgatgtggatggaccttttcttttaaccctttgtttgtccctccaggcccgttcttcctcttctccatcctgctccatccactgggaagctagcttgtatatcgacagattcctttggcctctggcttctagttaggtttagtcaatgcagagatcagaggcagcagaatgagacaggatattttcttcccctggctcctccccttcagagtctcctttgtcaccaactgtattagctgagttatctgtctgatgtaaaggagatctaccttagattatctactggtgtgttagtctcttctcacacactataaagacatacctgcgactaggtaatttataaagaaaagagatttaatggctcacaattctgcaggctgtacaggattctgcttctggggaggcctcaggaaatttccaatcatggcagaaggt

SEQ ID NO: 17945 - RNA, 2945 nt, Homo sapiens
  source 1..2945: mol_type = other RNA
tcgtttgcctttttctgctttcagagagaaaggtgtttgagcaagaaaacataggatatttcccaccacgaaacagacataattttgagggctcagcacaaaatgaaatcatggggcccttcttcaaacattattaagaatttccgctatagcagagccttgaaccaagtgtggggtccttctaagtgtgggccctgtgctgctacacaagttacacgctaagaaagccagccctgcctaggttccccgcctactcagattgccaaaaggagataaagtggctcaattgggttgtccagatgaaaagcaggtattttttttatgatgattcaaacactgtcatcaattgagaactaagtggcatttcactttccaaatggccggcaaatttctattcctaaaatctcatgttggactgattggttttcccctagatttctcattatacaaatggttatgctgggtctttaaatgccccttattttaatagagcaattaatcagacatgattaaatttctgtattaatcctacgtaattttttttttttaatctaagcatttcttaactgagaggggtctaaatatcactaaagcaacaggacatctttaagggaaaacagctgcaaaacagctttgcattctagagtgaaagccttagttttagcctatggtatattttgttcccttttaagaccacagtggtagtttttttccaaagagaactaataaacatattaagctatatggtaatttttctaacacccacattggtttcggtcagaagaattttactggaacctggaggtatcccattcttcataataataaaaaagaaatgtagtgtataaaagctccaggttacattactaagcaacgacatttccgggagtgaatatacttcctgtattccgcaagctgcttcaagtacatattcgacggccatctgtgcttttcaacaaaactgcgttcttccactgaaagatcctgaaattcaggcttttgactgaagatgaggtagttagtagcaatgaaatgaagtagccaggttgaaaggcaatcagagtggtgaaacttggcctttttaagcaggtcaactatatcaaggttcatggatgccagttccctgcttggcatgctctgcagctgggtaatgatgaacagctcacagatgtgctgcagtctggacacttggtacatctcggcacagatcaggagacacatggcctggaatatgccagctgggcagcaggagtctgtgtacaggtattctaaaaatgacaagaaagtctctttggaaacaccataaacgggaatcaggacactctttgcttccatgtaattaccattaaacatggctgccatcacttcacaacgggccaccaggatggccctgtgggctggcactgtcgtaccttgaatttcgaagacaacatcggcaagcatcggcttattaaggaaaaacttgagggaagtgttataaaaccacaaaggttttctggcttgataggttttgcaattccttaggcaattaatctttcctggtgtttttaaaatgcatttaactttctcgattacatttgaaacatccccagaatctttcaacttcttcctgatatcttcttccaattcttcccactgaaaagcacctggttgttcaagttgaggtggtctaattccatgaaaggagttgctcatttttcttttcttcattttttcacttgtcttctgatttaaggcttgaatcataaaatactccaacactcctccaaaatactttcctatgtagaagtcatcaaggctgtggagttcaagataggtcgctcctagttcttttgcaagttggatcccttcagttgtactaacacagctccctctgtctgaggtacatagtgggcatgtacaaggtaactcttcattttgtctggtaccaacagcagcaataattactggaactgaatttaatgctctttttatcactggaatataattatcctttacttcatggaatgaaaacttgtcattaacgttgtatttgatcacaatgatgtcagcgcccccaattagatttcgagaagtgtaccaatcactgtcaaatatgtcccagacgggacagtcgtggaccaccagcttgacattcccaaacgcactggcctgatactcggtgaacaccggacgcgcgaccgtgctggccgcgttcagcaacaagctgctctcgtccccggagaccagagggcttctccccaggtaagtgcggataagccccgacggccggttgtcctggtggaatgtgtccccctcgttccccagcgccacgatgtggatggacatgatctcaaatccaagggcagggcggcgactcggagaaaagcagcggctcacggcttcgcggggcccccgggcggcgagttcacccgcaatccgctcatccccggccgcgtccccctcgcgcgcctccaccgcggcggggccgacgcagagcggggccggggccgcgccagccagcgagcgagccggggaccagggcgggctagcgggcgggggataagctgccgctactcagggagtgcccgggaacatcgccgggcgcgggaccgccgcacagccccaagtggacgcagctgaccgcagtcccctctccgccgcgcctcctcggctggcagctgtcgcctcctgctgccgctgccgctgctcctcctcctctaagcagagaaggggggtcggggagatcggggcctccgccccctcagcggaccgggcgcagcacgtgccagccccgggggtcgggcggatgcgggggacgcgctccccgcggaggccccgggagctccggtggcggcggctggacacaaaggagccgcccgcgcggggcgccgcggaatataaattaataaatacaacgccccagcccgagagctcccagccgccaatccgcctgcagcaagttt

SEQ ID NO: 17946 - RNA, 248 nt, Homo sapiens
  source 1..248: mol_type = other RNA
tctaggctggtactgctgacggtttcccactttctgcactcctgagaatctcggcaggcgtacctagaccggagcttctccaacttctccgagcctatgaatcacctgcagatccttcattcatgcaacttgggctttttcagattctgatacaggacacagcttctgttctgattctggcatgatcctgtagtcttggccatctcctccctcatgcaattcttgtgtcaattctaatgacctctctt

SEQ ID NO: 17947 - RNA, 452 nt, Homo sapiens
  source 1..452: mol_type = other RNA
tctaggctggtactgctgacggtttcccactttctgcactcctgagaatctcggcaggcgtacctagaccggagcttctccaacttctccgagcctatgaatcacctgcagatctggagtgctgttccgtccacagcctgccagacaggttctagacctgcaccagatacacatgctgtctgctactagcttctttgaggctaagagagcaaagtcatgattcaggttcccttataggcttatgaatgtcacatagaagaaacccatctttccagttgtctggatgacaaaatacaagctcttggccacagcagggtccttcattcatgcaacttgggctttttcagattctgatacaggacacagcttctgttctgattctggcatgatcctgtagtcttggccatctcctccctcatgcaattcttgtgtcaattctaatgacctctctt

SEQ ID NO: 17948 - RNA, 501 nt, Homo sapiens
  source 1..501: mol_type = other RNA
tctaggctggtactgctgacggtttcccactttctgcactcctgagaatctcggcaggcgtacctagaccggagcttctccaacttctccgagcctatgaatcacctgcagatctggagtgctgttccgtccacagcctgccagacaggttctagacctgcaccagatacacatgctgtctgctactagcttctttgaggctaagagagcaaagtcatgattcaggttcccttataggcttatgaatgtcacatagaagaaacccatctttccagttgtctggatgacaaaatacaagctcttggccacagcagggtctgagagaaagaatgtggatgtatcaggccaaccttcattcatgcaacttgggctttttcagattctgatacaggacacagcttctgttctgattctggcacacagagctgacgtgaacaggagtgtgcttgagggtggcgcttgacacaagtatcaatgtgcttttgtcttccagaaaaaaac

SEQ ID NO: 17949 - RNA, 484 nt, Homo sapiens
  source 1..484: mol_type = other RNA
tctaggctggtactgctgacggtttcccactttctgcactcctgagaatctcggcaggcgtacctagaccggagcttctccaacttctccgagcctatgaatcacctgcagatctggagtgctgttccgtccacagcctgccagacaggttctagacctgcaccagatacacatgctgtctgctactagcttctttgaggctaagagagcaaagtcatgattcaggttcccttataggcttatgaatgtcacatagaagaaacccatctttccagttgtctggatgacaaaatacaagctcttggccacagcagggtctgagagaaagaatgtggatgtatcaggccaaccttcattcatgcaacttgggctttttcagattctgatacaggacacagcttctgttctgattctggcatgatcctgtagtcttggccatctcctccctcatgcaattcttgtgtcaattctaatgacctctctt

SEQ ID NO: 17950 - RNA, 331 nt, Homo sapiens
  source 1..331: mol_type = other RNA
tctaggctggtactgctgatactgtaatcaccctttatgaacactgggatactgctagggcatttggagttgggggttgaataatttcagaacaaaacccttgggggtgtatcttcataattatgatgtatataaagtggtgtaagatagcagcatggaaaatgaacagtttctgaaaaagaaaacacactcatggattttgtttgtgactataagacttaactgttataattcaatattggtggattaaaaattgatcttagctattagatcttctcataattcattactccattccaaatacctttatccaatacctaccgtatgccag

SEQ ID NO: 17951 - RNA, 581 nt, Homo sapiens
  source 1..581: mol_type = other RNA
tctaggctggtactgctgatactgtaatcaccctttatgaacactgggatactgctagggcatttggagttgggggttgaataatttcagaacaaaacccttgggggtgtatcttcataattatgatgtatataaagtggtgtaagatagcagcatggaaaatgaacagtttcttctgcaactagatcaaggcgcttcccaggttctttcgcttgattttaccacatgattgtggccaccatcttccctgatttgtatcctcgatttcctctgttgttccctcaagtagctctctgcacatatgattgtattcccatgacagctgttgcttctcttggtgggcctgttagtccaactgaaaccaggaactctggcctgcagagatacattctgtgctgaggacatagtggttctgtaattcatctgagttccagtggttaagctcagttactaggcaacaccaccatgagaccacagatcctggttgcacatgtacatgccttctctggctcaccttctccattagcctcctttccctgggattcagagaaaagtctttggagactgggccagaagacaaa

SEQ ID NO: 17952 - RNA, 354 nt, Homo sapiens
  source 1..354: mol_type = other RNA
tctagtgcgggcgttcccgttcgcggggaggtcattggcaccctgaatcacccactgcgagcccttccaaccggattgtagacctgccagctccgggcccacctcccccaacagggcctttcccggagcaacccggccgggcctggaaaaactccgagagggattcccagcgcagggacgcccaccggagcgcagtgtctcgggctggataagaaggggacccggccacagctccttcgccaacctcaactcccgctcggcggcccactgcctgcccgggcacctcggggcgtccgctcgccggcctcgtctccacttgtcccggcaggcgcgcgtgggctcggcgtcccgcgc

SEQ ID NO: 17953 - RNA, 566 nt, Homo sapiens
  source 1..566: mol_type = other RNA
tctagtgcgggcgttcccgttcgcggggaggtcattggcaccctgaatcacccactgcgagcccttccaaccggattgtagacctgccagctccgggcccacctcccccaacagggcctttcccggagcaacccggccgggcctggaaaaactccgagagggattcccagcgcagggacgcccaccggagcgcagtgtctcgggctggataagaaggggacccggccacagctccttcgccaacctcggggcgtccgctcgccggcctcgtctccacttgtcccggcaggcgcgcgtgggctcggcgtcccgcgctccctcctcgaccgcgcggctccggcgctgccaggtttcctgtatagcactataaccagtgaggcaccggcggagagcgcccggcagaacttcctcccggactggggctgggctgcggttgcgagagacaatccccggcgtcctggcttcctgtcgcctctgggccaggcccgcgcctcctgggggccaggagtccagccccagggccctccgccttgggggtcttctgtttgggaattatctgcctctct

SEQ ID NO: 17954 - RNA, 3129 nt, Homo sapiens
  source 1..3129: mol_type = other RNA
tctcaccccaactctgccccagagcccaaagtgctcaagggagaactcctttgagaggagactgccccgcctttaatgtgaaaagcaggcctggaggcccagggtggacgtggtcctcagccagaccaagggcctcctctagtggaggggcttcctgggctctctctgcactgcccctcagggtgctttctggggtccagtcaatggatcttacacacccatgaacactgagcccttggggagacgtgtccaggcttcagtttcccctcccagctgacaacaaaagtaaataatggatgtgactatcctgtggggaaggactaggaatactgggagtcactctgggccaagaaacacacacatggggagacactgtgcctccaagacagcagccaagacatccccatcaaaacccacaggctgggccaagagtggtggctcacgcctgtaatcccagcacttcaggaggccgaggtgtgcgggtcacctaacatcaggagttcgagaccagtctggacaacatgatgaaaccctgtctctactaaaaatacaaaaattagccgggagtggtggtgggcgcctgtaatcccagctactcaggaggctgaggcaggagaatcacctgaacccgagaggcggaggttgcagtgagcggagattgtaccattgcactccagcctgggcaacaagagtgaaactccatcttaaaaaaacaacaacaacaacaaaaaaaaaaccaaaagacccacaggctggtggacgtagctcccctttcagctctgcgagcctcacatggaaaagccgactctttccgactttgcaaaaggcaaagttccattaacaactacacacatttacaaaagtatttcaaagtctctataagaagggaaaaaaatttcaaaatagcaaagtagaaaactttccagggccctttcttcaagtcaggccatccatccactccactccactgtttctcatggtgacagcaggcaggagatctctgcacaaaacaaaaatcccaggtccccgatgtctctatcgcccccatactggaagggccatgatctctggtcctcttggctgtggtacctaccagaggccttatcaaaaatatggcatcccttaagccttaaggcatcttttagaagtcaggaatgcagaaaaggcagcgaagagtgcaaacaggaaacagaaagcacccggtcacacacaatgtcaccagaagggcagctagcttcccatttgaatgggtaaaaacaacaaacctctctccatcccaggaaaaggaagaacctgcgtcaggcacaggggagagaccccgccaggggtcctctgtgggctcctgccaggtcagccctcctccttccggctgggccagggcaggggcaggctcccgtggcgggcgggggcggcagggaagtgtgggcccacctggcctcgggcgtgggtctgcatgtgcacggccaggtggtggttgcggttgaaggtccggccacactgggggcactggtagggccgctcaccggtgtggatgcgctggtgccggaagaggtccgagggccggcggaaggccttgccgcagtaggggcaggcgggccagccctggccattgccggtgtgcaggcgctggtgcagcagcaggctcttgcgctgctggaagaagcgcaggcactcgctgcagtggtacatcttgctggctgcaggccgccgccccaccaaggcacggccccctgccacggagcggcgaccctcaggctcctcggggagccagcggatgacagggccgggtaccaccacctcccccggctccagcatggcctggctgtccccgcagctggtgggcgagcggccgggggcctcctgccgcccctcctccacatgggtccgctgatgaatcgtcagattgatcttcaggcggaagctctgcccgcagtcggggcaggggaatgcccgctgccgcctgcgggagaggactcggggcgtctccccactggcccccggtggccgtggctcccctgcccgcaccctgggcatgccctgggcctgatgacggctggggcccccaggcctgttcctgggccctcgggggattctacactcggtctggcctcgggacacccccagaaagagccgctcaggcgtcatctcgtcttcagactgtgcctctgtcttgatggccacaccaccacctgcttctggcccggctggggccactctcgcctctgagtcctgctgctgcttgggggcctgcccttctttcagctcctcctgggcagggctaagtgggctggtgaggtgctctggatacggagggaggccagtgcccatcatccttggacgtcccacctctacttcattccccttctcctggccccaccggtcaagacaaggctcctctcccctctctatccgggtgaggatgtctggtttggagattgcataatccagggagaccagcgtctcgtagttgcccctcatcacgtgcttgtagagctccttctgccagtcctccagcttgccccactccagctcagagaaatacacggccacatcatcgaaggtcacgggcaccttgggggcctcccccttgctgcccgggggcagccgcaagatccagaagttcctgttgcgcagcaagttctccacattctccagccgcctctgcagcagcccgtactcctgcagcaaggtccccagcacggcccacttgccctccagctggttcccgaactccacagctgtcttctcgcagtcggccagcttcttctcggctgtccccgtgcgcccctccagagtcagcaagcgggtcaggcaggaatccaccttcttctccaaggcctgaatggcggccaccaccgtccacagtgtgatttccgtggagtagaggtacgagttcttctcagcagctggctggggcaagggtgtcgaaggactctggtcctctgtgtgcttgtctgtctcggggtcccgggcaggcgccgcttcggccatggctgcccgcgtccctcgctgggttgcagtccctggacccggcctgtcgggcccggggcggcgcggcagcgacggcggaagcggagcgggacccgcctaacctgagagctactgccgggcggcagcgaactgcgtccc

SEQ ID NO: 17955 - RNA, 3082 nt, Homo sapiens
  source 1..3082: mol_type = other RNA
tctcaccccaactctgccccagagcccaaagtgctcaagggagaactcctttgagaggagactgccccgcctttaatgtgaaaagcaggcctggaggcccagggtggacgtggtcctcagccagaccaagggcctcctctagtggaggggcttcctgggctctctctgcactgcccctcagggtgctttctggggtccagtcaatggatcttacacacccatgaacactgagcccttggggagacgtgtccaggcttcagtttcccctcccagctgacaacaaaagtaaataatggatgtgactatcctgtggggaaggactaggaatactgggagtcactctgggccaagaaacacacacatggggagacactgtgcctccaagacagcagccaagacatccccatcaaaacccacaggctgggccaagagtggtggctcacgcctgtaatcccagcacttcaggaggccgaggtgtgcgggtcacctaacatcaggagttcgagaccagtctggacaacatgatgaaaccctgtctctactaaaaatacaaaaattagccgggagtggtggtgggcgcctgtaatcccagctactcaggaggctgaggcaggagaatcacctgaacccgagaggcggaggttgcagtgagcggagattgtaccattgcactccagcctgggcaacaagagtgaaactccatcttaaaaaaacaacaacaacaacaaaaaaaaaaccaaaagacccacaggctggtggacgtagctcccctttcagctctgcgagcctcacatggaaaagccgactctttccgactttgcaaaaggcaaagttccattaacaactacacacatttacaaaagtatttcaaagtctctataagaagggaaaaaaatttcaaaatagcaaagtagaaaactttccagggccctttcttcaagtcaggccatccatccactccactccactgtttctcatggtgacagcaggcaggagatctctgcacaaaacaaaaatcccaggtccccgatgtctctatcgcccccatactggaagggccatgatctctggtcctcttggctgtggtacctaccagaggccttatcaaaaatatggcatcccttaagccttaaggcatcttttagaagtcaggaatgcagaaaaggcagcgaagagtgcaaacaggaaacagaaagcacccggtcacacacaatgtcaccagaagggcagctagcttcccatttgaatgggtaaaaacaacaaacctctctccatcccaggaaaaggaagaacctgcgtcaggcacaggggagagaccccgccaggggtcctctgtgggctcctgccaggtcagccctcctccttccggctgggccagggcaggggcaggctcccgtggcgggcgggggcggcagggaagtgtgggcccacctggcctcgggcgtgggtctgcatgtgcacggccaggtggtggttgcggttgaaggtccggccacactgggggcactggtagggccgctcaccggtgtggatgcgctggtgccggaagaggtccgagggccggcggaaggccttgccgcagtaggggcaggcgggccagccctggccattgccggtgtgcaggcgctggtgcagcagcaggctcttgcgctgctggaagaagcgcaggcactcgctgcagtggtacatcttgctggctgcaggccgccgccccaccaaggcacggccccctgccacggagcggcgaccctcaggctcctcggggagccagcggatgacagggccgggtaccaccacctcccccggctccagcatggcctggctgtccccgcagctggtgggcgagcggccgggggcctcctgccgcccctcctccacatgggtccgctgatgaatcgtcagattgatcttcaggcggaagctctgcccgcagtcggggcaggggaatgcccgctgccgcctgcgggagaggactcggggcgtctccccactggcccccggtggccgtggctcccctgcccgcaccctgggcatgccctgggcctgatgacggctggggcccccaggcctgttcctgggccctcgggggattctacactcggtctggcctcgggacacccccagaaagagccgctcaggcgtcatctcgtcttcagactgtgcctctgtcttgatggccacaccaccacctgcttctggcccggctggggccactctcgcctctgagtcctgctgctgcttgggggcctgcccttctttcagctcctcctgggcagggctaagtgggctggtgaggtgctctggatacggagggaggccagtgcccatcatccttggacgtcccacctctacttcattccccttctcctggccccaccggtcaagacaaggctcctctcccctctctatccgggtgaggatgtctggtttggagattgcataatccagggagaccagcgtctcgtagttgcccctcatcacgtgcttgtagagctccttctgccagtcctccagcttgccccactccagctcagagaaatacacggccacatcatcgaaggtcacgggcaccttgggggcctcccccttgctgcccgggggcagccgcaagatccagaagttcctgttgcgcagcaagttctccacattctccagccgcctctgcagcagcccgtactcctgcagcaaggtccccagcacggcccacttgccctccagctggttcccgaactccacagctgtcttctcgcagtcggccagcttcttctcggctgtccccgtgcgcccctccagagtcagcaagcgggtcaggcaggaatccaccttcttctccaaggcctgaatggcggccaccaccgtccacagtgtgatttccgtggagtagaggtacgagttcttctcagcagctggctggggcaagggtgtcgaaggactctggtcctctgtgtgcttgtctgtctcggggtcctcaaatccatccatgtttctccttctccactgccagtgtctagtccaagttcccatcaccttgcttggcctgggccactgcggtcctgcccacctgatttccccacttccagcc

SEQ ID NO: 17956 - RNA, 3242 nt, Homo sapiens
  source 1..3242: mol_type = other RNA
tctcaccccaactctgccccagagcccaaagtgctcaagggagaactcctttgagaggagactgccccgcctttaatgtgaaaagcaggcctggaggcccagggtggacgtggtcctcagccagaccaagggcctcctctagtggaggggcttcctgggctctctctgcactgcccctcagggtgctttctggggtccagtcaatggatcttacacacccatgaacactgagcccttggggagacgtgtccaggcttcagtttcccctcccagctgacaacaaaagtaaataatggatgtgactatcctgtggggaaggactaggaatactgggagtcactctgggccaagaaacacacacatggggagacactgtgcctccaagacagcagccaagacatccccatcaaaacccacaggctgggccaagagtggtggctcacgcctgtaatcccagcacttcaggaggccgaggtgtgcgggtcacctaacatcaggagttcgagaccagtctggacaacatgatgaaaccctgtctctactaaaaatacaaaaattagccgggagtggtggtgggcgcctgtaatcccagctactcaggaggctgaggcaggagaatcacctgaacccgagaggcggaggttgcagtgagcggagattgtaccattgcactccagcctgggcaacaagagtgaaactccatcttaaaaaaacaacaacaacaacaaaaaaaaaaccaaaagacccacaggctggtggacgtagctcccctttcagctctgcgagcctcacatggaaaagccgactctttccgactttgcaaaaggcaaagttccattaacaactacacacatttacaaaagtatttcaaagtctctataagaagggaaaaaaatttcaaaatagcaaagtagaaaactttccagggccctttcttcaagtcaggccatccatccactccactccactgtttctcatggtgacagcaggcaggagatctctgcacaaaacaaaaatcccaggtccccgatgtctctatcgcccccatactggaagggccatgatctctggtcctcttggctgtggtacctaccagaggccttatcaaaaatatggcatcccttaagccttaaggcatcttttagaagtcaggaatgcagaaaaggcagcgaagagtgcaaacaggaaacagaaagcacccggtcacacacaatgtcaccagaagggcagctagcttcccatttgaatgggtaaaaacaacaaacctctctccatcccaggaaaaggaagaacctgcgtcaggcacaggggagagaccccgccaggggtcctctgtgggctcctgccaggtcagccctcctccttccggctgggccagggcaggggcaggctcccgtggcgggcgggggcggcagggaagtgtgggcccacctggcctcgggcgtgggtctgcatgtgcacggccaggtggtggttgcggttgaaggtccggccacactgggggcactggtagggccgctcaccggtgtggatgcgctggtgccggaagaggtccgagggccggcggaaggccttgccgcagtaggggcaggcgggccagccctggccattgccggtgtgcaggcgctggtgcagcagcaggctcttgcgctgctggaagaagcgcaggcactcgctgcagtggtacatcttgctggctgcaggccgccgccccaccaaggcacggccccctgccacggagcggcgaccctcaggctcctcggggagccagcggatgacagggccgggtaccaccacctcccccggctccagcatggcctggctgtccccgcagctggtgggcgagcggccgggggcctcctgccgcccctcctccacatgggtccgctgatgaatcgtcagattgatcttcaggcggaagctctgcccgcagtcggggcaggggaatgcccgctgccgcctgcgggagaggactcggggcgtctccccactggcccccggtggccgtggctcccctgcccgcaccctgggcatgccctgggcctgatgacggctggggcccccaggcctgttcctgggccctcgggggattctacactcggtctggcctcgggacacccccagaaagagccgctcaggcgtcatctcgtcttcagactgtgcctctgtcttgatggccacaccaccacctgcttctggcccggctggggccactctcgcctctgagtcctgctgctgcttgggggcctgcccttctttcagctcctcctgggcagggctaagtgggctggtgaggtgctctggatacggagggaggcctggcagctagattccagtctaaagcctcatgtcccacagaaggaaactgcagcacaggaattcagcagacaggaaatcacggtaatgatcgccaggcaggtcatgacagaatcagtgcccatcatccttggacgtcccacctctacttcattccccttctcctggccccaccggtcaagacaaggctcctctcccctctctatccgggtgaggatgtctggtttggagattgcataatccagggagaccagcgtctcgtagttgcccctcatcacgtgcttgtagagctccttctgccagtcctccagcttgccccactccagctcagagaaatacacggccacatcatcgaaggtcacgggcaccttgggggcctcccccttgctgcccgggggcagccgcaagatccagaagttcctgttgcgcagcaagttctccacattctccagccgcctctgcagcagcccgtactcctgcagcaaggtccccagcacggcccacttgccctccagctggttcccgaactccacagctgtcttctcgcagtcggccagcttcttctcggctgtccccgtgcgcccctccagagtcagcaagcgggtcaggcaggaatccaccttcttctccaaggcctgaatggcggccaccaccgtccacagtgtgatttccgtggagtagaggtacgagttcttctcagcagctggctggggcaagggtgtcgaaggactctggtcctctgtgtgcttgtctgtctcggggtcccgggcaggcgccgcttcggccatggctgcccgcgtccctcgctgggttgcagtccctggacccggcctgtcgggcccggggcggcgcggcagcgacggcggaagcggagcgggacccgcctaacctgagagctactgccgggcggcagcgaactgcgtccc

SEQ ID NO: 17957 - RNA, 3176 nt, Homo sapiens
  source 1..3176: mol_type = other RNA
tctcaccccaactctgccccagagcccaaagtgctcaagggagaactcctttgagaggagactgccccgcctttaatgtgaaaagcaggcctggaggcccagggtggacgtggtcctcagccagaccaagggcctcctctagtggaggggcttcctgggctctctctgcactgcccctcagggtgctttctggggtccagtcaatggatcttacacacccatgaacactgagcccttggggagacgtgtccaggcttcagtttcccctcccagctgacaacaaaagtaaataatggatgtgactatcctgtggggaaggactaggaatactgggagtcactctgggccaagaaacacacacatggggagacactgtgcctccaagacagcagccaagacatccccatcaaaacccacaggctgggccaagagtggtggctcacgcctgtaatcccagcacttcaggaggccgaggtgtgcgggtcacctaacatcaggagttcgagaccagtctggacaacatgatgaaaccctgtctctactaaaaatacaaaaattagccgggagtggtggtgggcgcctgtaatcccagctactcaggaggctgaggcaggagaatcacctgaacccgagaggcggaggttgcagtgagcggagattgtaccattgcactccagcctgggcaacaagagtgaaactccatcttaaaaaaacaacaacaacaacaaaaaaaaaaccaaaagacccacaggctggtggacgtagctcccctttcagctctgcgagcctcacatggaaaagccgactctttccgactttgcaaaaggcaaagttccattaacaactacacacatttacaaaagtatttcaaagtctctataagaagggaaaaaaatttcaaaatagcaaagtagaaaactttccagggccctttcttcaagtcaggccatccatccactccactccactgtttctcatggtgacagcaggcaggagatctctgcacaaaacaaaaatcccaggtccccgatgtctctatcgcccccatactggaagggccatgatctctggtcctcttggctgtggtacctaccagaggccttatcaaaaatatggcatcccttaagccttaaggcatcttttagaagtcaggaatgcagaaaaggcagcgaagagtgcaaacaggaaacagaaagcacccggtcacacacaatgtcaccagaagggcagctagcttcccatttgaatgggtaaaaacaacaaacctctctccatcccaggaaaaggaagaacctgcgtcaggcacaggggagagaccccgccaggggtcctctgtgggctcctgccaggtcagccctcctccttccggctgggccagggcaggggcaggctcccgtggcgggcgggggcggcagggaagtgtgggcccacctggcctcgggcgtgggtctgcatgtgcacggccaggtggtggttgcggttgaaggtccggccacactgggggcactggtagggccgctcaccggtgtggatgcgctggtgccggaagaggtccgagggccggcggaaggccttgccgcagtaggggcaggcgggccagccctggccattgccggtgtgcaggcgctggtgcagcagcaggctcttgcgctgctggaagaagcgcaggcactcgctgcagtggtacatcttgctggctgcaggccgccgccccaccaaggcacggccccctgccacggagcggcgaccctcaggctcctcggggagccagcggatgacagggccgggtaccaccacctcccccggctccagcatggcctggctgtccccgcagctggtgggcgagcggccgggggcctcctgccgcccctcctccacatgggtccgctgatgaatcgtcagattgatcttcaggcggaagctctgcccgcagtcggggcaggggaatgcccgctgccgcctgcgggagaggactcggggcgtctccccactggcccccggtggccgtggctcccctgcccgcaccctgggcatgccctgggcctgatgacggctggggcccccaggcctgttcctgggccctcgggggattctacactcggtctggcctcgggacacccccagaaagagccgctcaggcgtcatctcgtcttcagactgtgcctctgtcttgatggccacaccaccacctgcttctggcccggctggggccactctcgcctctgagtcctgctgctgcttgggggcctgcccttctttcagctcctcctgggcagggctaagtgggctggtgaggtgctctggatacggagggaggcctggcagctagattccagtctaaagcctcatgtcccacagaaggaaactgcagcacaggaattcagcagacaggaaatcacggtaatgatcgccaggcaggtcatgacagaatcagtgcccatcatccttggacgtcccacctctacttcattccccttctcctggccccaccggtcaagacaaggctcctctcccctctctatccgggtgaggatgtctggtttggagattgcataatccagggagaccagcgtctcgtagttgcccctcatcacgtgcttgtagagctccttctgccagtcctccagcttgccccactccagctcagagaaatacacggccacatcatcgaaggtcacgggcaccttgggggcctcccccttgctgcccgggggcagccgcaagatccagaagttcctgttgcgcagcaagttctccacattctccagccgcctctgcagcagcccgtactcctgcagcaaggtccccagcacggcccacttgccctccagctggttcccgaactccacagctgtcttctcgcagtcggccagcttcttctcggctgtccccgtgcgcccctccagagtcagcaagcgggtcaggcaggaatccaccttcttctccaaggcctgaatggcggccaccaccgtccacagtgtgatttccgtggagtagaggtacgagttcttctcagcagctggctggggcaagggtgtcgaaggactctggtcctctgtgtgcttgtctgtctcggggtcctcaaatccatccatgtttctccttctccactgccagtgtctagtccaagttcccatcaccttgcttggcctgggccactgcggtcctgcccacct

SEQ ID NO: 17958 - RNA, 1025 nt, Homo sapiens
  source 1..1025: mol_type = other RNA
tctcagctgctgccctctccagggctccaggccgcggtgtaggccaggtttgtgctggggatgcagcagctcagctggaagccaggggaggtggcacaggagatggacagctgcagaaacgtgtgtgcggcgctatgtggctcctctgggccccgctgcaccacagaatctctgctgctttccaagccacagccttgctcctgtcctctgcctgccacccagtgcttaaccccagcaagcaaggtcccaggatggcccctttggtggacattccctgtccccaagaaggatttctgcccagtgatgggacatgttggagacgctgagggcagcctggccgtggctggaagtcacagacacctgtgtccctggctgcaggaggatgggactggggctccctgggtgcctcaggaaccagctcaggttggtggcctcctggctcagatggagagtcaggctcagcgtgtcaccaggcatctgcagctgggagttcaggttgaggatcccggggactgcagggaggcaggtgacaggggacccaggtggcagcaactggcagtacccgggttcgggatggctgaagacaaggcagccacaaggctggtggttgtggaggctttgacaaggagggtaatggaggcagatgctggtgttccactggtagccagagaggcaagcacaatagaaattccccttgtggttgacattacactctgttgtgagtctgaggccagtgagaagaggccttggggaagaggaagctgaggcagcagggagagtcagtgtcctggagagttcagggggccaggtcttatctggaaagtccagatgtacatagacggagaccagcgctgattcccctgctccattctcttggtccaggagctgcccagatccagattcccctccagcctgactctgtccctgaggcactgctgaactggttcgcaagcagtcactctacccccaagactaaaacggtataccccagatcaccacgcaagtgcggataccacagaaatccc

SEQ ID NO: 17959 - RNA, 1487 nt, Homo sapiens
  source 1..1487: mol_type = other RNA
tctcagctgctgccctctccagggctccaggccgcggtgtaggccaggtttgtgctggggatgcagcagctcagctggaagccaggggaggtggcacaggagatggacagctggtatggaagtcgagccacatctgtcgccttcaagggcaccctcaccacctcatacaggttccacttgaagccctgggcctcgaagcagctcatgtactcacctgcccagtgatgggacatgttggagacgctgagggcagcctggccgtggctggaagtcacagacacctgtgtccctggctgcaggaggatgggactggggctccctgggtgcctcaggaaccagctcaggttggtggcctcctggctcagatggagagtcaggctcagcgtgtcaccaggcatctgcagctgggagttcaggttgaggatcccggggacaggtggcagcaactggcagtacccgggttcgggatggctgaagacaaggcagccacaaggctggtggttgtggaggctttgacaaggagggtaatggaggcagatgctggtgttccactggtagccagagaggcaagcacaatagaaattccccttgtggttgacattacactctgttgtgagtctgaggccagtgagaagaggccttggggaagaggaagctgaggcagcagggagagtcagtgtcctggagagttcagggggccaggtcttatctggaaagtccagatgtacatagacggagaccagcgctgattcccctgctccattctcttggtccaggagctgcccagatccagattcccctccagcctgactctgtcccttctcgggcagcccagtctttgccatccttgcccagccggtgtggtgcttgtgtgtcacagccttgtagccgggagtcgctgccgagtgggcgctcagttttcgggtcgtcatggctggctacgaatacgtgagcccggagcagctggctggctttgataagtacaaggtaccgcgggccggcggatgcccctctccctgctcccggcctcgcccaggcggctgaggggcccgcgcggcgcggtccgtgtcaccttgtgccgcgtggctccgggcgggctggcgggcgttcctccggaggtcctgcgggtcctggggattgggggtcggggagcgtgggagcatcctaagcccgccgcccgtagtcggcaccccccgggagatttccttttccttaggagagcgctcagtgatcatggagcgagggaattcccttcctattttttttaaacttattattttcgtaagcccccgaaaggatggagttccttctgttgtgtcaatcgccttcattttagtgaagtttccactcgcctgtcatgcatacaacttcggaggaggagatgatcgtttggcagatgaggcccgggaggggagcgacttgccgatgccatcctgctgatgtctccacttctgctcccggcagggacttcctaagcggcagcttgt

SEQ ID NO: 17960 - RNA, 982 nt, Homo sapiens
  source 1..982: mol_type = other RNA
tctcagctgctgccctctccagggctccaggccgcggtgtaggccaggtttgtgctggggatgcagcagctcagctggaagccaggggaggtggcacaggagatggacagctggtatggaagtcgagccacatctgtcgccttcaagggcaccctcaccacctcatacaggttccacttgaagccctgggcctcgaagcagctcatgtactcacctgcccagtgatgggacatgttggagacgctgagggcagcctggccgtggctggaagtcacagacacctgtgtccctggctgcaggaggatgggactggggctccctgggtgcctcaggaaccagctcaggttggtggcctcctggctcagatggagagtcaggctcagcgtgtcaccaggcatctgcagctgggagttcaggttgaggatcccggggactgcagggaggcaggtgacaggggacccaggtggcagcaactggcagtacccgggttcgggatggctgaagacaaggcagccacaaggctggtggttgtggaggctttgacaaggagggtaatggaggcagatgctggtgttccactggtagccagagaggcaagcacaatagaaattccccttgtggttgacattacactctgttgtgagtctgaggccagtgagaagaggccttggggaagaggaagctgaggcagcagggagagtcagtgtcctggagagttcagggggccaggtcttatctggaaagtccagatgtacatagacggagaccagcgctgattcccctgctccattctcttggtccaggagctgcccagatccagattcccctccagcctgactctgtccaggttgggatgcttgggcaactggtgaccccagcaggggaagagttgtggccaggagcagcagtggggcagccgaacagaccatggctcagtgaagcagtccctacaagcccacgatgcaaatttccgcaaggaaga

SEQ ID NO: 17961 - RNA, 1419 nt, Homo sapiens
  source 1..1419: mol_type = other RNA
tctcagctgctgccctctccagggctccaggccgcggtgtaggccaggtttgtgctggggatgcagcagctcagctggaagccaggggaggtggcacaggagatggacagctggtatggaagtcgagccacatctgtcgccttcaagggcaccctcaccacctcatacaggttccacttgaagccctgggcctcgaagcagctcatgtactcacctgcccagtgatgggacatgttggagacgctgagggcagcctggccgtggctggaagtcacagacacctgtgtccctggctgcaggaggatgggactggggctccctgggtgcctcaggaaccagctcaggttggtggcctcctggctcagatggagagtcaggctcagcgtgtcaccaggcatctgcagctgggagttcaggttgaggatcccggggactgcagggaggcaggtgacaggggacccaggtggcagcaactggcagtacccgggttcgggatggctgaagacaaggcagccacaaggctggtggttgtggaggctttgacaaggagggtaatggaggcagatgctggtgttccactggtagccagagaggcaagcacaatagaaattccccttgtggttgacattacactctgttgtgagtctgaggccagtgagaagaggccttggggaagaggaagctgaggcagcagggagagtcagtgtcctggagagttcagggggccaggtcttatctggaaagtccagatgtacatagacggagaccagcgctgattcccctgctccattctcttggtccaggagctgcccagatccagattcccctccagcctgactctgtccaggttgggatgcttgggcaactggtgaccccagcaggggaagagttgtggccaggagcagcagtggggcagccgaacagaccatggctcagtgaagcagtccctacaagcccacgatgcaaatttccgcaaggaagagctggcagggcagtgtgcagatgggatgggagggaagaggggagggagccagggctgaatttacagaggaagcgctacagcctgtgactctgagtgaaatgggaatccaggtcactgtgggggccacctggagcccacatgccccagtgagaatggtgcccaggctcttcttaggctctggacccaaagctccgagagcaggagaggcttaggggttcgaagtcacaaccagcaacatgtctataagccaggttcagtcatgttcccaaggacctgggaaatctggattgttctgaactcctcaaaggctgaatcactgatcaaacagtcaaggttacaaatgaaaaataaagaaaagataaaaatatgagagctgatttttactctaaaataatttccagatagactagaatcctccctccctcccttccttccct

SEQ ID NO: 17962 - RNA, 1136 nt, Homo sapiens
  source 1..1136: mol_type = other RNA
tctcagctgctgccctctccagggctccaggccgcggtgtaggccaggtttgtgctggggatgcagcagctcagctggaagccaggggaggtggcacaggagatggacagctggtatggaagtcgagccacatctgtcgccttcaagggcaccctcaccacctcatacaggttccacttgaagccctgggcctcgaagcagctcatgtactcacctgcccagtgatgggacatgttggagacgctgagggcagcctggccgtggctggaagtcacagacacctgtgtccctggctgcaggaggatgggactggggctccctgggtgcctcaggaaccagctcaggttggtggcctcctggctcagatggagagtcaggctcagcgtgtcaccaggcatctgcagctgggagttcaggttgaggatcccggggactgcagggaggcaggtgacaggggacccaggtggcagcaactggcagtacccgggttcgggatggctgaagacaaggcagccacaaggctggtggttgtggaggctttgacaaggagggtaatggaggcagatgctggtgttccactggtagccagagaggcaagcacaatagaaattccccttgtggttgacattacactctgttgtgagtctgaggccagtgagaagaggccttggggaagaggaagctgaggcagcagggagagtcagtgtcctggagagttcagggggccaggtcttatctggaaagtccagatgtacatagacggagaccagcgctgattcccctgctccattctcttggtccaggagctgcccagatccagattcccctccagcctgactctgtcccaactcctcctctgtcagggtgagggtggaggtctgggcccacattgtctggcccttgggccatcggccaaagctagaagatagggggatggggcaggcagggaagggtctgtctatcctttcattccatgctttgtctctcccaatcaggggtccccattgtcgcctctgcagaccttccctgggtctcaccccagtctcacttacaggttgggatgcttgggcaactggtgaccccagcaggggaagagttgtggccaggagcagcagtggggcagccgaacagaccat

SEQ ID NO: 17963 - RNA, 1726 nt, Homo sapiens
  source 1..1726: mol_type = other RNA
tctcagctgctgccctctccagggctccaggccgcggtgtaggccaggtttgtgctggggatgcagcagctcagctggaagccaggggaggtggcacaggagatggacagctggtatggaagtcgagccacatctgtcgccttcaagggcaccctcaccacctcatacaggttccacttgaagccctgggcctcgaagcagctcatgtactcacctgcccagtgatgggacatgttggagacgctgagggcagcctggccgtggctggaagtcacagacacctgtgtccctggctgcaggaggatgggactggggctccctgggtgcctcaggaaccagctcaggttggtggcctcctggctcagatggagagtcaggctcagcgtgtcaccaggcatctgcagctgggagttcaggttgaggatcccggggactgcagggaggcaggtgacaggggacccaggtggcagcaactggcagtacccgggttcgggatggctgaagacaaggcagccacaaggctggtggttgtggaggctttgacaaggagggtaatggaggcagatgctggtgttccactggtagccagagaggcaagcacaatagaaattccccttgtggttgacattacactctgttgtgagtctgaggccagtgagaagaggccttggggaagaggaagctgaggcagcagggagagtcagtgtcctggagagttcagggggccaggtcttatctggaaagtccagatgtacatagacggagaccagcgctgattcccctgctccattctcttggtccaggagctgcccagatccagattcccctccagcctgactctgtccctcagctcaccaattttgacgctagcaaatgaagcgacgaagagagctggaaggcgggacttagtgttgcctgatccacgccgattggacaacagcagtgtcgggggacgggccgctcgagcgggctagcaaccccccctcgatgggcggggagaagcgtgggctgcgcttgcgcactgagaggcggccgaaggggccgaggcggctacgcgtgcgcggtgggcggagcgcggctctcctaccttctcgggcagcccagtctttgccatccttgcccagccggtgtggtgcttgtgtgtcacagccttgtagccgggagtcgctgccgagtgggcgctcagttttcgggtcgtcatggctggctacgaatacgtgagcccggagcagctggctggctttgataagtacaaggtaccgcgggccggcggatgcccctctccctgctcccggcctcgcccaggcggctgaggggcccgcgcggcgcggtccgtgtcaccttgtgccgcgtggctccgggcgggctggcgggcgttcctccggaggtcctgcgggtcctggggattgggggtcggggagcgtgggagcatcctaagcccgccgcccgtagtcggcaccccccgggagatttccttttccttaggagagcgctcagtgatcatggagcgagggaattcccttcctattttttttaaacttattattttcgtaagcccccgaaaggatggagttccttctgttgtgtcaatcgccttcattttagtgaagtttccactcgcctgtcatgcatacaacttcggaggaggagatgatcgtttggcagatgaggcccgggaggggagcgacttgccgatgccatcctgctgatgtctccacttctgctc

SEQ ID NO: 17964 - RNA, 1453 nt, Homo sapiens
  source 1..1453: mol_type = other RNA
tctcagctgctgccctctccagggctccaggccgcggtgtaggccaggtttgtgctggggatgcagcagctcagctggaagccaggggaggtggcacaggagatggacagctggtatggaagtcgagccacatctgtcgccttcaagggcaccctcaccacctcatacaggttccacttgaagccctgggcctcgaagcagctcatgtactcacctgcccagtgatgggacatgttggagacgctgagggcagcctggccgtggctggaagtcacagacacctgtgtccctggctgcaggaggatgggactggggctccctgggtgcctcaggaaccagctcaggttggtggcctcctggctcagatggagagtcaggctcagcgtgtcaccaggcatctgcagctgggagttcaggttgaggatcccggggactgcagggaggcaggtgacaggggacccaggtggcagcaactggcagtacccgggttcgggatggctgaagacaaggcagccacaaggctggtggttgtggaggctttgacaaggagggtaatggaggcagatgctggtgttccactggtagccagagaggcaagcacaatagaaattccccttgtggttgacattacactctgttgtgagtctgaggccagtgagaagaggccttggggaagaggaagctgaggcagcagggagagtcagtgtcctggagagttcagggggccaggtcttatctggaaagtccagatgtacatagacggagaccagcgctgattcccctgctccattctcttggtccaggagctgcccagatccagattcccctccagcctgactctgtccctggaacagaacacagaggggagacctcaagtcccttccaaaggcaccccaggggccagcctgactagtctcagccagcatgactcagtctcaaccagctcttctttttgccaggagtcaagtgtacacatcaggaagggaaagcaggcttctgttagggggtgccagggatgcaaccccaggaaccctgctatcccacccaagaccaggaaccaggcacgccctgggaagtcaacatgctttgtttaattccttcctgcgtttacctgtccctgggcctctaggctaattgaaatggcttggtctggagctccagcagcggagctggacattgctggctggggcccaggcgcttggggagtttattccttctgtaggatttgacagcagggtgagcagaaggcagcctctttcctccgtctttggttcctgtacattatttcctcaccaactcctcctctgtcagggtgagggtggaggtctgggcccacattgtctggcccttgggccatcggccaaagaggttgggatgcttgggcaactggtgaccccagcaggggaagagttgtggccaggagcagcagtggggcagccgaacagaccatggc

SEQ ID NO: 17965 - RNA, 1411 nt, Homo sapiens
  source 1..1411: mol_type = other RNA
tctcagctgctgccctctccagggctccaggccgcggtgtaggccaggtttgtgctggggatgcagcagctcagctggaagccaggggaggtggcacaggagatggacagctggtatggaagtcgagccacatctgtcgccttcaagggcaccctcaccacctcatacaggttccacttgaagccctgggcctcgaagcagctcatgtactcacctgcccagtgatgggacatgttggagacgctgagggcagcctggccgtggctggaagtcacagacacctgtgtccctggctgcaggaggatgggactggggctccctgggtgcctcaggaaccagctcaggttggtggcctcctggctcagatggagagtcaggctcagcgtgtcaccaggcatctgcagctgggagttcaggttgaggatcccggggactgcagggaggcaggtgacaggggacccaggtggcagcaactggcagtacccgggttcgggatggctgaagacaaggcagccacaaggctggtggttgtggaggctttgacaaggagggtaatggaggcagatgctggtgttccactggtagccagagaggcaagcacaatagaaattccccttgtggttgacattacactctgttgtgagtctgaggccagtgagaagaggccttggggaagaggaagctgaggcagcagggagagtcagtgtcctggagagttcagggggccaggtcttatctggaaagtccagatgtacatagacggagaccagcgctgattcccctgctccattctcttggtccaggagctgcccagatccagattcccctccagcctgactctgtccctgtccctgggcctctaggctaattgaaatggcttggtctggagctccagcagcggagctggacattgctggctggggcccaggcgcttggggagtttattccttctgtaggatttgacagcagggtgagcagaaggcagcctctttcctccgtctttggttcctgtacattatttcctcaccaactcctcctctgtcagggtgagggtggaggtctgggcccacattgtctggcccttgggccatcggccaaagctagaagatagggggatggggcaggcagggaagggtctgtctggtagggaggtgaggatggagctggcccaaggagagagaacatggcagtccttcctccaggaaatatggaggggctcactgtgtcacagacctgagccctgtctatatgcacctgcgtgtgcgtgtggatatctatccaaaaccagatattgatatagatacgagtatggataagacgtgagtataagctggtcacaatggcacgtgcctttagtcccagttacttgggaggctgaggtgggaggatcacttgagcccaggagttcaag

SEQ ID NO: 17966 - RNA, 959 nt, Homo sapiens
  source 1..959: mol_type = other RNA
tctcagctgctgccctctccagggctccaggccgcggtgtaggccaggtttgtgctggggatgcagcagctcagctggaagccaggggaggtggcacaggagatggacagctggtatggaagtcgagccacatctgtcgccttcaagggcaccctcaccacctcatacaggttccacttgaagccctgggcctcgaagcagctcatgtactcacctgcccagtgatgggacatgttggagacgctgagggcagcctggccgtggctggaagtcacagacacctgtgtccctggctgcaggaggatgggactggggctccctgggtgcctcaggaaccagctcaggttggtggcctcctggctcagatggagagtcaggctcagcgtgtcaccaggcatctgcagctgggagttcaggttgaggatcccggggactgcagggaggcaggtgacaggggacccaggtggcagcaactggcagtacccgggttcgggatggctgaagacaaggcagccacaaggctggtggttgtggaggctttgacaaggagggtaatggaggcagatgctggtgttccactggtagccagagaggcaagcacaatagaaattccccttgtggttgacattacactctgttgtgagtctgaggccagtgagaagaggccttggggaagaggaagctgaggcagcagggagagtcagtgtcctggagagttcagggggccaggtcttatctggaaagtccagatgtacatagacggagaccagcgctgattcccctgctccattctcttggtccaggagctgcccagatccagattcccctccagcctgactctgtcccttctcgggcagcccagtctttgccatccttgcccagccggtgtggtgcttgtgtgtcacagccttgtagccgggagtcgctgccgagtgggcgctcagttttcgggtcgtcat

SEQ ID NO: 17967 - RNA, 1094 nt, Homo sapiens
  source 1..1094: mol_type = other RNA
tctcagctgctgccctctccagggctccaggccgcggtgtaggccaggtttgtgctggggatgcagcagctcagctggaagccaggggaggtggcacaggagatggacagctggtatggaagtcgagccacatctgtcgccttcaagggcaccctcaccacctcatacaggttccacttgaagccctgggcctcgaagcagctcatgtactcacctgttgtgagtctgaggccagtgagaagaggccttggggaagaggaagctgaggcagcagggagagtcagtgtcctggagagttcagggggccaggtcttatctggaaagtccagatgtacatagacggagaccagcgctgattcccctgctccattctcttggtccaggagctgcccagatccagattcccctccagcctgactctgtcccttctcgggcagcccagtctttgccatccttgcccagccggtgtggtgcttgtgtgtcacagccttgtagccgggagtcgctgccgagtgggcgctcagttttcgggtcgtcatggctggctacgaatacgtgagcccggagcagctggctggctttgataagtacaaggtaccgcgggccggcggatgcccctctccctgctcccggcctcgcccaggcggctgaggggcccgcgcggcgcggtccgtgtcaccttgtgccgcgtggctccgggcgggctggcgggcgttcctccggaggtcctgcgggtcctggggattgggggtcggggagcgtgggagcatcctaagcccgccgcccgtagtcggcaccccccgggagatttccttttccttaggagagcgctcagtgatcatggagcgagggaattcccttcctattttttttaaacttattattttcgtaagcccccgaaaggatggagttccttctgttgtgtcaatcgccttcattttagtgaagtttccactcgcctgtcatgcatacaacttcggaggaggagatgatcgtttggcagatgaggcccgggaggggagcgacttgccgatgccatcctgctgatgtctccacttctgctcccggcagggacttcctaagcggcagcttgt

SEQ ID NO: 17968 - RNA, 247 nt, Homo sapiens
  source 1..247: mol_type = other RNA
tctcaggagtaaagacagagtttcaagaaaaagaaagtggtcacctgttccacattcttctgaggggtcaagtaaatttgtagtagtgcactgaccattgatttagcaatatggagtcatcagcaaccaatataaggcaatatatgtgtggagacaaaagcctgactggtgcttctgtgagaaaacaggaggttgagaaacagtatagttaatttatttttatttttatttttattattatacttta

SEQ ID NO: 17969 - RNA, 3129 nt, Homo sapiens
  source 1..3129: mol_type = other RNA
tctcaggagtaaagacagagtttcgccatgttggccaagctggtctcgaatttctgacctcaggtgatcctcccacttcggcctcccaaagtgctgggtttacaggtgtgagccactgcacctggtctcaataaacttttaaagaaacttgtgttttaatagtctcaagagcgtctatatatattaatatttgaaaaagagtcacacacatataaaacacatggtgtacatacagactgaaatatcacctgattcccaagaggtccgaggctaggaatgactacagtgtgtgacagatataaaaatgatcaccagaaagacactggagacattgctgtcacctcaaagagccttagttctaatggagataaaacaaatgtgcacaggagtttcatataagatagaatgtaaaacacaaactccagctccaaggctcaggagggtgtgacatagtgatgtggcaggcaatcagaggcttcatggtagaagcagtggaaaaatggttcagcaactctcgtgtaaatataatagaaatgttctcttttgtacctacaacaaggtgctcatatagaagatggaagaaagggtggccagaaatagcctatgcctggattgttttcttaaccttgggtatttagcccacagcatacttgacaactgtcaaagatgtggtgcccagacccaagtcagcaagcttgccccaaatcaggcagctatgaaactggactaagtcacatattcttctagtcacacattcaggctaaggacatttggctcctacctgaccagagccgtggtctccatgctgagatataacttaaatttttatttggtaacagtcacttttcaagataaatgtgcatctacaagatttgtatttggtaacagtcacctttcaagacaaatgcatctacccacctgtgaggccatttagtgagactgaagaggaagcctgaatacaaaccactagagaaaaacactgtcttatcaacaagattttactgctctctggttgtcaccatgcaatccactcccaactcatctgctaccagcatcctccaggtttttgagctacatttctcagtagttttctatccttcttcacatgactccaaaacagcttcccattcaaagcaaaataaacagcttcatgtgtaaacaagaatttagtgaattagcccaagtagaatcagattttgtgtgggagagtacacataatgcacacatactcatttgcctggacattacattgctgaagttccacgtgcaaatggtatcaatgcttccttgtctggatgagctgggaacgaggccactaggaaaaatgtgttcatactgaactgcctccagtttgaaagacactgatgcaggatctgacttactccattcaagagctgagatctagaaacagggacatctggtcctggaatctactgcattaatccatcactcatgagtgccacctaaatagcaaagtcccttacacagccctcgtgaaagcactgaagaaatcattcaaaaagatctttatttcaaattgcttgaataaacatgcaggtgtaaaataatgaaaaattattaagataaatttaggaaacaaagattctttccaaggttcttaaccgtcaatacggcaaaggagtacgacaggaatgggggaaattgattttgtgaaaggctattaaagagagtgctattctcatcagaaagtccctccccttttaaaatgtaatcaataatttaaagcaaagccaaaaatcatatcagttaaaaggaccaggacatttctttttgcacagtataggaggaaaattaaattagtgtctcttaagaaattactattatccttaagagaagtagtaggtaaaaattttaactcttttccacagcttgccattttactcactttaaaagaaagggttcaaagttaaacaatatgatactaagcatatcatcaaaataataataaatttcttttattactcagatatctgatttcctgccaaagtttaaaagatttatttaaaacttaacaggcacaaaacatacttcagcatttggcagaagttgttttctttctcagtttagcaatttttaaaatgtaaagttacacaatcatcagcgggaaggtttgacggtttgattacaaattatactgaacctattcttcattttaatgtgcctcgttctctttaagtattgatttgtgcctaaaggataagatggtctatttcatatttcatttttttttagatttgacctttcaatccaatggctaactctttgaaatgtatttaaaattagatagtcatcttttctgcaaaatgaaggactgcacacagtctctgtgtgtctaactctccgaactaggacgtgagaattctcatgagggttctggttgatggccacaaaatggaaaaggcagaagagcttcggtaagtagatatgtaccatcatgtttgtgagtgccctgtttctagaactcttttaaactataaatgattctgtgagctattaagcctctctctaagaatctagcagattcatcctaagcatgtgttgaatggtcacctctctagaatggagcagaagggaattagaaaggagagaagggtaaataaaagttaaggtccctcgaatgctaagatttcatggtcttccaccatattaaaatgagatttttatattcaaacattagtgttcaccagataaaattgatctctcaaaacctcgctgtccttgtctgaaatatacgaataattacaagcaggattattttgtgaactaaatgagataatggaaatgatcagactgttcatatggtgagaaacaaatggtcaccatgactaagtgactatgccccaaggataactcaaagccaattctgtcacaagaattccaaagtcatatcaaagccacacacaatcccaacagcaccagatccagacttaacccaaatgtgttattcccattgcacttgtgctggaagtctttattttgatgcatatgtacttgaattcaagttaattaaagtttactacttcccaacaacccactgttttgttttaaaatgccaggggctaggccaggaatggtggctcatgccctgtaatcccagcactttgggag

SEQ ID NO: 17970 - RNA, 31 nt, Homo sapiens
  source 1..31: mol_type = other RNA
tctcagtaagtggcactctgtcttctgagtc

SEQ ID NO: 17971 - RNA, 2626 nt, Homo sapiens
  source 1..2626: mol_type = other RNA
tctcagtaagtggcactctgttatagtcatatgggatgacattagaattcctgtttttacttttattttcttcttgatttccaatgtgctgtgtcctccagctcctatatgaaggaagtctctggaattcagcctctagtggagacggctcactgggtggatcccttttcttcatgttatgtagatatggatgtaattcagacaaattcacttctgtttctccaaactgattgtattccaccaaagcctgatggatcaagatgtactgggcctctacttgaaccatcaggcatctctgtcgccttagcttgacaacataaccataaacatccactttgttctcggcttccaggccttctagcatggcatcaattccgatataggttcctgtgcgcccaacaccagcactgcagtgcaccacaatgggaccactgaagaaattgctgaaggcattcactctccttctcagtttgaggagcaagtgaggatcctcaggcaccccgtggtctggccagctggtgaactgaatgtgagtcacctctcttccagttgctttttcttttttatttacaatgttcaatttctgaatgatgtaatctggacatcttttgtgctggttgatctttacaacaacatctccaaaagcccgagtgccctcttccattgacggccagtattctgcacacttgttcctgtttccttcttcacatcgagtgaccatgacaataactgtggctttctgttcccaaatcatcctccagaaatcatcaacagtttcatccctgggaccttgtgcagcaatgtatttcctgggttctttgaaaccatcaatatagctggcatttatgtagtttgaccctgcatctccgtttatctcagagagttcaacacggttataatcataaggaagaatgtcaacataacggtttttattctggttaaagggctttcgagcttcctttataggaaacttgctgaacacccgcgggatgctctgaaattcagccagaaaaagtcttccttcatcagcaatcttcctcttataagtttccaacaaaatatctgcatggattggctccacattcatcagttgtttttcatcatccctttcaacaagctcctgctgttcatctaaattgcaggatcttttcttatgtagatcatagattttgtagagaacaacaagcagggctattgatgtcacaataatcagaaatgccagaaatgctatcagtgccttagaattataagatgttgaatgatgtaaaataaagggttctccaggatagtctccattgtgaaaataggccttaaaagtgtagtctgttgaatattgaagatcttttacacggaaatcgcaattcttatgcgactcatttctaaccagagtatttccagcttcaacttccaaatggtaacgttcatgggggccattacggtccctgggaggcctacacttgacatgcatactattatctgatgtcatggagacagtcatgttccagacctggcttggaggagcacttttagttgtgaaatgacacattgcagcacttccattacgttgcacttttgcaatgatgtaggcatgtaatgataaaacatatttcgtataaggttttaaattttgcaaatcatatttgatcaggtttttatccagattgaggcaatctttttctgtctcttttatataacagagggtaaaattatgaaatgatctttgagggggattccaggtaattactccttgatgtgcagcttcacttctacaaaaaataatctgaggctctcctggactcccaaaatctgttttaataattttacttgcgttagtaaacttgtggttattatagagtatttctgagtcacacttatactcatgttcgggttcaaggttttctaatttaatttctttattatcaaatatcatattaccacactgaaatctgtaggtaatattctgtgtatcacaagtaaaggtttcaatatttttccattttaaacaaatagtagtatctgctttttcaacttgtgtacaatcatgtaactgaaacttttcaacccctggtggcacatctaatattaatgtcttatcaggagcagtacatgaattatgagatatggaaacagacgcatttttacattctgtaaggttatgcacctcattgtttgtgcaagtattgtttccacattccacattctcattaacatttagctttgctgtaaataatttagtttccttgttatataagtaatccacagtgatgtttgcatatttttcatcacatgttggcttagatggagtagtagctattgttgtggttgaaatgacagcgcttccagaagggctcagagtggttgtttcagaggcattaaggtaggcatcagtgggggaaggtgttgggctttgccctgtcacaaatacttctgtgtccagaaaggcaaagccaaatgccaagagtttaagccacaaatacatggtcatatctggaagtcagccgtgtccctaagaaacagcatgcgtcctttctccactgttgtcttatcagacgaggaacaatttcctcctctgttaccctaagaacaaaccacttgctagctgcatgaactgctaggtgatgatgtc

SEQ ID NO: 17972 - RNA, 2782 nt, Homo sapiens
  source 1..2782: mol_type = other RNA
tctcagtaagtggcactctgttatagtcatatgggatgacattagaattcctgtttttacttttattttcttcttgatttccaatgtgctgtgtcctccagctcctatatgaaggaagtctctggaattcagcctctagtggagacggctcactgggtggatcccttttcttcatgttatgtagatatggatgtaattcagacaaattcacttctgtttctccaaactgattgtattccaccaaagcctgatggatcaagatgtactgggcctctacttgaaccatcaggcatctctgtcgccttagcttgacaacataaccataaacatccactttgttctcggcttccaggccttctagcatggcatcaattccgatataggttcctgtgcgcccaacaccagcactgcagtgcaccacaatgggaccactgaagaaattgctgaaggcattcactctccttctcagtttgaggagcaagtgaggatcctcaggcaccccgtggtctggccagctggtgaactgaatgtgagtcacctctcttccagttgctttttcttttttatttacaatgttcaatttctgaatgatgtaatctggacatcttttgtgctggttgatctttacaacaacatctccaaaagcccgagtgccctcttccattgacggccagtattctgcacacttgttcctgtttccttcttcacatcgagtgaccatgacaataactgtggctttctgttcccaaatcatcctccagaaatcatcaacagtttcatccctgggaccttgtgcagcaatgtatttcctgggttctttgaaaccatcaatatagctggcatttatgtagtttgaccctgcatctccgtttatctcagagagttcaacacggttataatcataaggaagaatgtcaacataacggtttttattctggttaaagggctttcgagcttcctttataggaaacttgctgaacacccgcgggatgctctgaaattcagccagaaaaagtcttccttcatcagcaatcttcctcttataagtttccaacaaaatatctgcatggattggctccacattcatcagttgtttttcatcatccctttcaacaagctcctgctgttcatctaaattgcaggatcttttcttatgtagatcatagattttgtagagaacaacaagcagggctattgatgtcacaataatcagaaatgccagaaatgctatcagtgccttagaattataagatgttgaatgatgtaaaataaagggttctccaggatagtctccattgtgaaaataggccttaaaagtgtagtctgttgaatattgaagatcttttacacggaaatcgcaattcttatgcgactcatttctaaccagagtatttccagcttcaacttccaaatggtaacgttcatgggggccattacggtccctgggaggcctacacttgacatgcatactattatctgatgtcatggagacagtcatgttccagacctggcttggaggagcacttttagttgtgaaatgacacattgcagcacttccattacgttgcacttttgcaatgatgtaggcatgtaatgataaaacatatttcgtataaggttttaaattttgcaaatcatatttgatcaggtttttatccagattgaggcaatctttttctgtctcttttatataacagagggtaaaattatgaaatgatctttgagggggattccaggtaattactccttgatgtgcagcttcacttctacaaaaaataatctgaggctctcctggactcccaaaatctgttttaataattttacttgcgttagtaaacttgtggttattatagagtatttctgagtcacacttatactcatgttcgggttcaaggttttctaatttaatttctttattatcaaatatcatattaccacactgaaatctgtaggtaatattctgtgtatcacaagtaaaggtttcaatatttttccattttaaacaaatagtagtatctgctttttcaacttgtgtacaatcatgtaactgaaacttttcaacccctggtggcacatctaatattaatgtcttatcaggagcagtacatgaattatgagatatggaaacagacgcatttttacattctgtaaggttatgcacctcattgtttgtgcaagtattgtttccacattccacattctcattaacatttagctttgctgtaaataatttagtttccttgttatataagtaatccacagtgatgtttgcatatttttcatcacatgttggcttagatggagtagtagctattgttgtggttgaaatgacagcgcttccagaagggctcagagtggttgtttcagaggcattaaggtaggcatctgagatagcattgctgcctggggtagggttgagttttgcattggcggcggagccgctgaatgtctgcgtgtcagttccagcagagggcgtctgcgagtctgcgtgcgtgggaaggtgaggcgtctgtactgatgaaacaccagtgggggaaggtgttgggctttgccctgtcacaaatacttctgtgtccagaaaggcaaagccaaatgccaagagtttaagccacaaatacatggtcatatctggaagtcagccgtgtccctaagaaacagcatgcgtcctttctccactgttgtcttatcagacgaggaacaatttcctcctctgttaccctaagaacaaaccacttgctagctgcatgaactgctaggtgatgatgtcagattcggttttact

SEQ ID NO: 17973 - RNA, 2962 nt, Homo sapiens
  source 1..2962: mol_type = other RNA
tctcagtaagtggcactctgttatagtcatatgggatgacattagaattcctgtttttacttttattttcttcttgatttccaatgtgctgtgtcctccagctcctatatgaaggaagtctctggaattcagcctctagtggagacggctcactgggtggatcccttttcttcatgttatgtagatatggatgtaattcagacaaattcacttctgtttctccaaactgattgtattccaccaaagcctgatggatcaagatgtactgggcctctacttgaaccatcaggcatctctgtcgccttagcttgacaacataaccataaacatccactttgttctcggcttccaggccttctagcatggcatcaattccgatataggttcctgtgcgcccaacaccagcactgcagtgcaccacaatgggaccactgaagaaattgctgaaggcattcactctccttctcagtttgaggagcaagtgaggatcctcaggcaccccgtggtctggccagctggtgaactgaatgtgagtcacctctcttccagttgctttttcttttttatttacaatgttcaatttctgaatgatgtaatctggacatcttttgtgctggttgatctttacaacaacatctccaaaagcccgagtgccctcttccattgacggccagtattctgcacacttgttcctgtttccttcttcacatcgagtgaccatgacaataactgtggctttctgttcccaaatcatcctccagaaatcatcaacagtttcatccctgggaccttgtgcagcaatgtatttcctgggttctttgaaaccatcaatatagctggcatttatgtagtttgaccctgcatctccgtttatctcagagagttcaacacggttataatcataaggaagaatgtcaacataacggtttttattctggttaaagggctttcgagcttcctttataggaaacttgctgaacacccgcgggatgctctgaaattcagccagaaaaagtcttccttcatcagcaatcttcctcttataagtttccaacaaaatatctgcatggattggctccacattcatcagttgtttttcatcatccctttcaacaagctcctgctgttcatctaaattgcaggatcttttcttatgtagatcatagattttgtagagaacaacaagcagggctattgatgtcacaataatcagaaatgccagaaatgctatcagtgccttagaattataagatgttgaatgatgtaaaataaagggttctccaggatagtctccattgtgaaaataggccttaaaagtgtagtctgttgaatattgaagatcttttacacggaaatcgcaattcttatgcgactcatttctaaccagagtatttccagcttcaacttccaaatggtaacgttcatgggggccattacggtccctgggaggcctacacttgacatgcatactattatctgatgtcatggagacagtcatgttccagacctggcttggaggagcacttttagttgtgaaatgacacattgcagcacttccattacgttgcacttttgcaatgatgtaggcatgtaatgataaaacatatttcgtataaggttttaaattttgcaaatcatatttgatcaggtttttatccagattgaggcaatctttttctgtctcttttatataacagagggtaaaattatgaaatgatctttgagggggattccaggtaattactccttgatgtgcagcttcacttctacaaaaaataatctgaggctctcctggactcccaaaatctgttttaataattttacttgcgttagtaaacttgtggttattatagagtatttctgagtcacacttatactcatgttcgggttcaaggttttctaatttaatttctttattatcaaatatcatattaccacactgaaatctgtaggtaatattctgtgtatcacaagtaaaggtttcaatatttttccattttaaacaaatagtagtatctgctttttcaacttgtgtacaatcatgtaactgaaacttttcaacccctggtggcacatctaatattaatgtcttatcaggagcagtacatgaattatgagatatggaaacagacgcatttttacattctgtaaggttatgcacctcattgtttgtgcaagtattgtttccacattccacattctcattaacatttagctttgctgtaaataatttagtttccttgttatataagtaatccacagtgatgtttgcatatttttcatcacatgttggcttagatggagtagtagctattgttgtggttgaaatgacagcgcttccagaagggctcagagtggttgtttcagaggcattaaggtaggcatctgagatagcattgctgcctggggtagggttgagttttgcattggcggcggagccgctgaatgtctgcgtgtcagttccagcagagggcgtctgcgagtctgcgtgcgtgggaaggtgaggcgtctgtactgatgaaacacctgtggtattaaaagcactagcattatccaaagagtccggggatacttgggtggaagtattgtctggactaagagaagttgtggtctctgagaagtcattttctctttcaaaggtgcttgcgggtgagaatgcagtggtgtgagtaggtaaggggtcacttgaaagtggaacactgggcatctttgctgtagtcaatccagtgggggaaggtgttgggctttgccctgtcacaaatacttctgtgtccagaaaggcaaagccaaatgccaagagtttaagccacaaatacatggtcatatctggaagtcagccgtgtccctaagaaacagcatgcgtcctttctccactgttgtcttatcagacgaggaacaatttcctcctctgttaccctaagaacaaaccacttgctagctgcatgaactgctaggtgatgat

SEQ ID NO: 17974 - RNA, 2926 nt, Homo sapiens
  source 1..2926: mol_type = other RNA
tctcagtaagtggcactctgttatagtcatatgggatgacattagaattcctgtttttacttttattttcttcttgatttccaatgtgctgtgtcctccagctcctatatgaaggaagtctctggaattcagcctctagtggagacggctcactgggtggatcccttttcttcatgttatgtagatatggatgtaattcagacaaattcacttctgtttctccaaactgattgtattccaccaaagcctgatggatcaagatgtactgggcctctacttgaaccatcaggcatctctgtcgccttagcttgacaacataaccataaacatccactttgttctcggcttccaggccttctagcatggcatcaattccgatataggttcctgtgcgcccaacaccagcactgcagtgcaccacaatgggaccactgaagaaattgctgaaggcattcactctccttctcagtttgaggagcaagtgaggatcctcaggcaccccgtggtctggccagctggtgaactgaatgtgagtcacctctcttccagttgctttttcttttttatttacaatgttcaatttctgaatgatgtaatctggacatcttttgtgctggttgatctttacaacaacatctccaaaagcccgagtgccctcttccattgacggccagtattctgcacacttgttcctgtttccttcttcacatcgagtgaccatgacaataactgtggctttctgttcccaaatcatcctccagaaatcatcaacagtttcatccctgggaccttgtgcagcaatgtatttcctgggttctttgaaaccatcaatatagctggcatttatgtagtttgaccctgcatctccgtttatctcagagagttcaacacggttataatcataaggaagaatgtcaacataacggtttttattctggttaaagggctttcgagcttcctttataggaaacttgctgaacacccgcgggatgctctgaaattcagccagaaaaagtcttccttcatcagcaatcttcctcttataagtttccaacaaaatatctgcatggattggctccacattcatcagttgtttttcatcatccctttcaacaagctcctgctgttcatctaaattgcaggatcttttcttatgtagatcatagattttgtagagaacaacaagcagggctattgatgtcacaataatcagaaatgccagaaatgctatcagtgccttagaattataagatgttgaatgatgtaaaataaagggttctccaggatagtctccattgtgaaaataggccttaaaagtgtagtctgttgaatattgaagatcttttacacggaaatcgcaattcttatgcgactcatttctaaccagagtatttccagcttcaacttccaaatggtaacgttcatgggggccattacggtccctgggaggcctacacttgacatgcatactattatctgatgtcatggagacagtcatgttccagacctggcttggaggagcacttttagttgtgaaatgacacattgcagcacttccattacgttgcacttttgcaatgatgtaggcatgtaatgataaaacatatttcgtataaggttttaaattttgcaaatcatatttgatcaggtttttatccagattgaggcaatctttttctgtctcttttatataacagagggtaaaattatgaaatgatctttgagggggattccaggtaattactccttgatgtgcagcttcacttctacaaaaaataatctgaggctctcctggactcccaaaatctgttttaataattttacttgcgttagtaaacttgtggttattatagagtatttctgagtcacacttatactcatgttcgggttcaaggttttctaatttaatttctttattatcaaatatcatattaccacactgaaatctgtaggtaatattctgtgtatcacaagtaaaggtttcaatatttttccattttaaacaaatagtagtatctgctttttcaacttgtgtacaatcatgtaactgaaacttttcaacccctggtggcacatctaatattaatgtcttatcaggagcagtacatgaattatgagatatggaaacagacgcatttttacattctgtaaggttatgcacctcattgtttgtgcaagtattgtttccacattccacattctcattaacatttagctttgctgtaaataatttagtttccttgttatataagtaatccacagtgatgtttgcatatttttcatcacatgttggcttagatggagtagtagctattgttgtggttgaaatgacagcgcttccagaagggctcagagtggttgtttcagaggcattaaggtaggcatctgaggtgttcgctgtgatggtggtgttggaggtgcgtgcaggtaaggcagcagagctgtggtgtgcaaggctgagggtggttgtcaatggggaaactgggtctgtaggaaaggtgctggctgtactcctctctcctgggacatctgagatagcattgctgcctggggtagggttgagttttgcattggcggcggagccgctgaatgtctgcgtgtcagttccagcagagggcgtctgcgagtctgcgtgcgtgggaaggtgaggcgtctgtactgatgaaacaccagtgggggaaggtgttgggctttgccctgtcacaaatacttctgtgtccagaaaggcaaagccaaatgccaagagtttaagccacaaatacatggtcatatctggaagtcagccgtgtccctaagaaacagcatgcgtcctttctccactgttgtcttatcagacgaggaacaatttcctcctctgttaccctaagaacaaaccacttgctagctgcatgaactgctaggtgatgatgtcagattcggttttact

SEQ ID NO: 17975 - RNA, 3109 nt, Homo sapiens
  source 1..3109: mol_type = other RNA
tctcagtaagtggcactctgttatagtcatatgggatgacattagaattcctgtttttacttttattttcttcttgatttccaatgtgctgtgtcctccagctcctatatgaaggaagtctctggaattcagcctctagtggagacggctcactgggtggatcccttttcttcatgttatgtagatatggatgtaattcagacaaattcacttctgtttctccaaactgattgtattccaccaaagcctgatggatcaagatgtactgggcctctacttgaaccatcaggcatctctgtcgccttagcttgacaacataaccataaacatccactttgttctcggcttccaggccttctagcatggcatcaattccgatataggttcctgtgcgcccaacaccagcactgcagtgcaccacaatgggaccactgaagaaattgctgaaggcattcactctccttctcagtttgaggagcaagtgaggatcctcaggcaccccgtggtctggccagctggtgaactgaatgtgagtcacctctcttccagttgctttttcttttttatttacaatgttcaatttctgaatgatgtaatctggacatcttttgtgctggttgatctttacaacaacatctccaaaagcccgagtgccctcttccattgacggccagtattctgcacacttgttcctgtttccttcttcacatcgagtgaccatgacaataactgtggctttctgttcccaaatcatcctccagaaatcatcaacagtttcatccctgggaccttgtgcagcaatgtatttcctgggttctttgaaaccatcaatatagctggcatttatgtagtttgaccctgcatctccgtttatctcagagagttcaacacggttataatcataaggaagaatgtcaacataacggtttttattctggttaaagggctttcgagcttcctttataggaaacttgctgaacacccgcgggatgctctgaaattcagccagaaaaagtcttccttcatcagcaatcttcctcttataagtttccaacaaaatatctgcatggattggctccacattcatcagttgtttttcatcatccctttcaacaagctcctgctgttcatctaaattgcaggatcttttcttatgtagatcatagattttgtagagaacaacaagcagggctattgatgtcacaataatcagaaatgccagaaatgctatcagtgccttagaattataagatgttgaatgatgtaaaataaagggttctccaggatagtctccattgtgaaaataggccttaaaagtgtagtctgttgaatattgaagatcttttacacggaaatcgcaattcttatgcgactcatttctaaccagagtatttccagcttcaacttccaaatggtaacgttcatgggggccattacggtccctgggaggcctacacttgacatgcatactattatctgatgtcatggagacagtcatgttccagacctggcttggaggagcacttttagttgtgaaatgacacattgcagcacttccattacgttgcacttttgcaatgatgtaggcatgtaatgataaaacatatttcgtataaggttttaaattttgcaaatcatatttgatcaggtttttatccagattgaggcaatctttttctgtctcttttatataacagagggtaaaattatgaaatgatctttgagggggattccaggtaattactccttgatgtgcagcttcacttctacaaaaaataatctgaggctctcctggactcccaaaatctgttttaataattttacttgcgttagtaaacttgtggttattatagagtatttctgagtcacacttatactcatgttcgggttcaaggttttctaatttaatttctttattatcaaatatcatattaccacactgaaatctgtaggtaatattctgtgtatcacaagtaaaggtttcaatatttttccattttaaacaaatagtagtatctgctttttcaacttgtgtacaatcatgtaactgaaacttttcaacccctggtggcacatctaatattaatgtcttatcaggagcagtacatgaattatgagatatggaaacagacgcatttttacattctgtaaggttatgcacctcattgtttgtgcaagtattgtttccacattccacattctcattaacatttagctttgctgtaaataatttagtttccttgttatataagtaatccacagtgatgtttgcatatttttcatcacatgttggcttagatggagtagtagctattgttgtggttgaaatgacagcgcttccagaagggctcagagtggttgtttcagaggcattaaggtaggcatctgaggtgttcgctgtgatggtggtgttggaggtgcgtgcaggtaaggcagcagagctgtggtgtgcaaggctgagggtggttgtcaatggggaaactgggtctgtaggaaaggtgctggctgtactcctctctcctgggacatctgagatagcattgctgcctggggtagggttgagttttgcattggcggcggagccgctgaatgtctgcgtgtcagttccagcagagggcgtctgcgagtctgcgtgcgtgggaaggtgaggcgtctgtactgatgaaacacctgtggtattaaaagcactagcattatccaaagagtccggggatacttgggtggaagtattgtctggactaagagaagttgtggtctctgagaagtcattttctctttcaaaggtgcttgcgggtgagaatgcagtggtgtgagtaggtaaggggtcacttgaaagtggaacactgggcatctttgctgtagtcaatccagtgggggaaggtgttgggctttgccctgtcacaaatacttctgtgtccagaaaggcaaagccaaatgccaagagtttaagccacaaatacatggtcatatctggaagtcagccgtgtccctaagaaacagcatgcgtcctttctccactgttgtcttatcagacgaggaacaatttcctcctctgttaccctaagaacaaaccacttgctagctgcatgaactgctaggtgatgatgtc

SEQ ID NO: 17976 - RNA, 2342 nt, Homo sapiens
  source 1..2342: mol_type = other RNA
tctcgcatcaggaggcaaggagggatttggggaaaaatccatggacatgctgcagattccatctgcaaggtcacggccagcagtccaccctgcatcagggtcagggcacagggctgggggctgagcctccttccaaatacctgcaaggacttctcggctttcaaatacttcccaatcggtacgtcccgtgagaaggcgaatgtcacagcagggcagggagggagtgctcctccctttttgatagagctcattctctttttttttttttgaattgctggcctgaatgtccatcatggcccgggacagaagccctcaccttcctgagctgcaggctttcagtgggttagaaaacggattagaaggggttggggatactcaatggatgtccttcatccccctggagaggcagagtgtatggcagggaggcagcctggactgaatcccactttgccggtcactggcgctatgagcttgggcttgtttccagttatcttgatttgtcagctggggataatcacgaattatcggtaagatggaaatcagggtcatgagaatacaatgaattaaagaagggtgcctggcatacagtaggcacgcaaggaagatcagctttgttcctgttcttacgttcactgcccatgtgaagagcacgtcaggtgccatcacctgcaagctcgccgtggcgcagtgaacgctgcctggggttccagatagcgtggggtgtaactcactcctttgattcccgttagcccacccacgttggaatagacactttgtgacggttcaaatagacactttgtaacagttcaaagatgagaagcgtggacctggagaaggttagcgactggctcaaagtcacacagccaggtaagggtggacttggggctagaacccagcgctgtgcccacccactatccatgcctgctgccccagcactcctggggacatggacgtcatggtgctgtgtgcatgggcacccagtgggttgctggggatgaggatggagctgggcttcactctcatgggtggcctggcagatgctgaacctaaccctaatcctgcccgcatgcagcatggtggaggggtgcagaaccctgacctacgtgggatcctggtttctgtggccctttccttctgcccgtggtctgatgtgatctatgggcaaatcggagggtcataaaaatagccctacctggcacgccaggggcccagggggctgctgctgctcactgggatttcagtgggaggcagaagctgcggagacaggaggtaaaaatagcaagggtttccacaacagccccgcgctcccctgctccagcatttgacacggcagcacacgagatcctcttgtcccactgcgctggaatcttaaaggttcctgtccttggagacaccctatcttgccaggaaaatgaggagctcgcagctgcacacagcagaggctccaccttccctgaagtccttaaatcccccacatcaggctgactaggaaggccagaagtgggtgagggctgagcttcaaagcaaaagggttggtcccttcccagtgggtgaccccaggcaggttcctcaacctctctgagattcagcttctgcatcaagaataagcaggcagaccagaacagctcctgctggaaggcagagccagaaccatcggaccgctggaaccagctccatgagggcagggtccacgttgcccctggacacagctgcacccccagggcctggtacctgggagatgcccataaacaccgactacctgcacacacgtgcttataaactgtagagtactgtacaaagtgccacggtcatttctgatgtaggggtcatcacctcgtctaactggtttatcacaaaatggatgtgatccagggacatctccagaggctacagagaatgagcctggggtctggtgtccacagcccccgcctgtcaatctgctccctgatgccatgggtgatgggactggaggaatgtccctggcattcttggccctgtgactccttcgttggtgaaaaagtggggatggagaaagtgccagctcccagggggccatgaggagaacccatgagggtgtgtggaaagtgtctcagttgaaatccactcatccgtcacacccccatggcagggaggccctaagaggtccccaggagggagggctggagatagagttgtttacgctgttcttggcccaacaccagtctctaattacccagaaacatgcaggaatgacaggtgggactgatagctgtgtgttcttgcggtatacatgtgctgacacacgtgaacacgcatgtgaacatacacacacacattcatgtagcacaccggcatgcacaatg

SEQ ID NO: 17977 - RNA, 250 nt, Homo sapiens
  source 1..250: mol_type = other RNA
tctctcggctcctcgcggctcgcggcggccgacggttcctgggacacctgcttgcttggcccgtccggcggctcagggcttctctgctgcgctcccggttcgctggacgggaagaagggctgggccgtcccgtcccgtccccatcggaaccccaagtcgcgccgctgacccgtcgcagggcgagatgagcgcggacgcagcggccggggcgcccctgccccggctctgctgcctggagaagggtccgaac

SEQ ID NO: 17978 - RNA, 177 nt, Homo sapiens
  source 1..177: mol_type = other RNA
tctctcggctcctcgcggctcttctgcctccgaggcggtccctccctctggcctgcctcctccctccctccctttcttccttctttcctcccacctccttcccactaggctgcagaggcggggaagacccgccacaggctggcgtgcggagccccaggccggcggccttccgtgatt

SEQ ID NO: 17979 - RNA, 199 nt, Homo sapiens
  source 1..199: mol_type = other RNA
tctctcggctcctcgcggctcttctgcctccgaggcggtccctccctctggcctgcctcctccctccctccctttcttccttctttcctcccacctccttcccactaggctgcagaggcggggaagacccgccacaggctggcgtgcggagccccaggccggcggccttccgtgattaacgagtgtttacaagactcta

SEQ ID NO: 17980 - RNA, 589 nt, Homo sapiens
  source 1..589: mol_type = other RNA
tctctctgactccatggcatccctagtatgccagtgaacctgtgccacaaacaggttgaggcagaggagcaagcaggtagctgagatgaagctgagcatggataccttcagatccaagttggtggtcatgcttcctcgattaaggatccaagagctgaagagccagccaaggccagtaagtatggtaaagacagagatgagaaagaaggccctggaatattggagataatagggtggcttgggtgtgtggctccagcacagctcatggttgcataaggtccagagtcctgcgtagagctcaaggccattcttgatcaccagaaactgtacccagttcagtggggacatggcgatcagcattaggaggctaaaactacagaggctgccacagagcgttcggatgtagatgtgtgcctgatccataagctgctgctgcctttggcatgacatcgaggcacttggatgtttcttggcagggacggtaggcctttggtatttccggttcccctttattttgggaacctcaggactgtggaaagtcaaggttaaatgttcccttcgctccatcttggcagttagttctctaact

SEQ ID NO: 17981 - RNA, 568 nt, Homo sapiens
  source 1..568: mol_type = other RNA
tctctctgactccatggcatccctagtatgccagtgaacctgtgccacaaacaggttgaggcagaggagcaagcaggtagctgagatgaagctgagcatggataccttcagatccaagttggtggtcatgcttcctcgattaaggatccaagagctgaagagccagccaaggccagtaagtatggtaaagacagagatgagaaagaaggccctggaatattggagataatagggtggcttgggtgtgtggctccagcacagctcatggttgcataaggtccagagtcctgcgtagagctcaaggccattcttgatcaccagaaactgtacccagttcagtggggacatggcgatcagcattaggaggctaaaactacagaggctgccacagagcgttcggatgtagatgtgtgcctgatccataagctgctgctgcctttggcatgacatcgaggcacttggatgtttcttggcagggacggtaggctcctcaccctttggtatttccggttcccctttattttgggaacctcaggactgtggaaagtcaaggttaaatgttcccttc

SEQ ID NO: 17982 - RNA, 406 nt, Homo sapiens
  source 1..406: mol_type = other RNA
tctctctgactccatggcatccctagtatgccagtgaacctgtgccacaaacaggttgaggcagaggagcaagcaggtagctgagatgaagctgagcatggataccttcagatccaagttggtggtcatgcttcctcgattaaggatccaagagctgaagagccagccaaggccagtaagtatggtaaagacagagatgagaaagaaggccctggaatattggagataatccattgtttagttccattggtttttcacttccagctctatctggcatgtacaggccttgtcagcctatgacctttggtatttccggttcccctttattttgggaacctcaggactgtggaaagtcaaggttaaatgttcccttcgctccatcttggcagttagttctctaactgcc

SEQ ID NO: 17983 - RNA, 333 nt, Homo sapiens
  source 1..333: mol_type = other RNA
tctctctgactccatggcatccctagtatgccagtgaacctgtgccacaaacaggttgaggcagaggagcaagcaggtagctgagatgaagctgagcatggataccttcagatccaagttggtggtcatgcttcctcgattaaggatccaagagctgaagagccagccaaggccagtaagtatggtaaagacagagatgagaaagaaggccctggaatattggagataatcctttggtatttccggttcccctttattttgggaacctcaggactgtggaaagtcaaggttaaatgttcccttcgctccatcttggcagttagttctctaact

SEQ ID NO: 17984 - RNA, 34 nt, Homo sapiens
  source 1..34: mol_type = other RNA
tctctgagtaccatatgccttgtactgggctagg

SEQ ID NO: 17985 - RNA, 3409 nt, Homo sapiens
  source 1..3409: mol_type = other RNA
tctctggagggaagcactttctgaaccagtaatagttgcaacttcagcagagaaagcttgctgattaagactgcttgtttcagaatctatatgaagagtagttagactagccacttcctgctcttcagcactctgatgatggccagaacctgaatccacatcagcagaggacgtaaccccagtgtcggctccaaagccaaaattgtcaaatttttggccatcatattggaaagcgctgaaagaatccgaatgactatctgagctgataagatcactgctccctgcactggcaggagaagtccattctgagggcacacctgggtcatcaatagggcgcatctggttctgcttgtttagaatatcagggaggtctttgggaatttccaggctgcctggactacttcctcttcttgtcatagtcgaggcattaccacttcgaagtcattctgctataaactcatccatcagatcaggaacattagcactgctgctgccaatatcactattaagaggaggcagtttttggctcatgtcctctttattgactttggctcgttcaacagtgaatggttccaagatgtcagaagtgctgctacttcaaggcaatggctgctcctcattcaaagcaccaaaaacttcatttccagtttcttcactttgtgaaaaatgtctgactctagttgagcggggaagtatttgagcatcatcaatatcgacagttttttgccgtactatactcctcgccttttcggttcctggagaaccagtggttgttgcactcctctgtctcattggggcttggccaggctgatcacgactccatcctctagaaaatgacttgtcaactgaaactttctgaaattcatgtccaactcctttccctttgtgctttttttgtttctgttcactcagcttatccaatggtaaatcactgagatccaaactatataaattcctagctaaaactttagttaatgtctccatagtcagtgaccactcagtggccaactcttcccaataggtcaacgatgacaatactgacagtaagtcatcccaaagttctcgggagatgtacacatttaggtttgctttgatccaggcaactataagggtctggaaaagtggtcctgcaagtcgacctgccaaggtcatattttttttcccttggaactgtagaaaagcttgtgatggcatcttcagtacagattccgtgactctgagcaacacaagcagcatgtgttcccaagtctttttgtccattgatacttgtacaaccatgtaccgataaatgttaagaatgcgtttacacatatctgtgtgttcatccagaagattttttatttcatttgcaggttcaagaagaaatatatttgatgagtttataataaacacctgcaaaactgcctgggtaccagctcgtatgttttgttctgtggcttcttcagaggtgttatgaagagcaccttggtaggagccgttttttgcccaactggaatttcgaacatgatcagcagtattggtcccattttcctcttctcttttttctccttcttccattgaaatatcatggtctgtgacattttcaatgcaagggaggtctgaagaagtgatcacaatttcttcaggctcttgcatgaacaaaggtttttcctcttgttggatccattcttgatatacttttaccacttttctcatagctgctgcttcacaaattggtaataaaaatgcctgacgaaatatctctgtcacaaagtttacattactccttttagaagaaaaaactctgcgaactatttcaatgtctgtgagatgttcttcatcaatactacagagactagatgagctaggttctcgctccgtgagagtgcttgtattggaatgagactgttcgggttctgtagttctgtctgctttatcagcattatcatttttgctttcttctctggatactaaactagcagctgctctctgaatattctttggcaagacttcaccttccatcccaggaatatgaggtcctgtatgtggttttggctccagccagaaagaaaccagccaacgaatgacaataacacgagccttaatgaaaggctcctttgtacaatagattgcttcattggtttcagcatctttctttatcatgacataatgtggctttggtctcatctgcgggatgtcaagtataggatgatataaactgttttccttacagatgtttggaaaaatataaggcaagtaatatttcttaaaatgtgaaaacaaaaatgaaaatcccctttcttggttttctttgttcttccattctaaactttttacctgaatgactatgtattttagaagtgcttcaagaaaatagcttgtgagatcttcttgccctttatctcctgattgtggggggacaagaggagtgatttcttctatagtgacttgagtttcttaaaggttgagtggaggattaatgagattatctaaagttcgaggtccatgttcagactgtggtgctgaaaatccagggattaagcatgaaaacatccagagctgttctttgctacagttattctgaagagcttgcaaccatagtaagaaaagacgaacaccttcccgcctaatctttaaggagtctcctgtgtgaagtagcttctttaaatcaatccaatattatgaaactgccatggctgatgaattctttctggaagaagttgtaaaattttctcaaaaataaaaagtatagcatccagttcctctctttgagacttgtgacctttctgtttaagactagcttcgatagtcacaaaattttcaaagaacacatagtatatatgtaaaaaatgttgtcgaaaaactgtttaagatcaatagattctgcattctttttttcactaaataaacatcactttccaaaacaaatacgcatcaggaagacagctcgagataaactctgaactaggattcaggcatctggatgaatgcatcttcttcagccagttccaccattaactcgatgacgatgcgcaggtgcttgaggcgagtcagtgcgtccttcttggtgtctagcaccttctgggtggacttcttcacgtccccgtgcggcttcttggagaacatcctgccgctgccactgccactgccactgccactgccacagccggctcccagcggcagaaagtggagggagtggacggggaggagactagccagagaggctcattagctccccagccttgcgggccagggcagagccgactcctccccgatccaggccagggccgccacctccacccgcctcgcgccgcggctccaaggcaccttcggccccagctccaatatggcggatccctctcccggccctgcacggagcgaggtagacccgggctggccgcctgccgccgccgctcgtctccagcggccg

SEQ ID NO: 17986 - RNA, 4531 nt, Homo sapiens
  source 1..4531: mol_type = other RNA
tctctggagggaagcactttctgaaccagtaatagttgcaacttcagcagagaaagcttgctgattaagactgcttgtttcagaatctatatgaagagtagttagactagccacttcctgctcttcagcactctgatgatggccagaacctgaatccacatcagcagaggacgtaaccccagtgtcggttccaaagccaaaattgtcaaattttcggccatcatattggaaagcgctgaaagaatccgaatgactatctgagctgataagatcactgctccctgcactggcaggagaagtccattctgagggcacacctgggtcatcaatagggcgcatctggttctgcttgtttagaatatcagggaggtctttgggaatttccaggctgcctggactacttcctcttcttgtcatagtcgaggcattaccacttcgaagtcgttctgctataaactcatccatcagatcaggaacattagcactgctgccgccaatatcactattaagaggaggcagtttttggctcatgtcctctttattgactgcagctttccttccaaaatagcccattacatgactgtacagatccctcagtggagcctctggtggcattctgttctgcctctgtggggaaacatttgccttcggcttcgaaagagcatgtacaacagttttataaacgccacccagggagccctgctgtagtcctgcctcatgacttgatgacctaagagtactacgactacctaattgactacttgcaattccttctttttgtaatatggtggtgggaatctctgtggattccttcactgttttgctgcttactgatgcagtaccaagtgtatctagaggtctgtacacaccaggttttactagctctgtagcactatttgtgctggtatgggtgttgctagtgctgctattgctgctaccactactaaagccaccgagcttccgcagtctcatcttccatggagcctctttgttttccagaggattataaaactgaacggactcagtggatggcctaaaagtaacatgaacactatttcgttttttagtagcaattttcatgattttggctctatgagttactgtttcagacaagctccttttagttggagaaagtttgctagtacttgtaacatgaggcattctgcggttaacaggtgcttttagtgttgctttcttggcacgcataacatgtgggacagtgattttttcattaatttgcacactcttaagcttttcaactagtgttacatcaacacaagcatctaattctgtggctgcttgtctgtacagatgtttccttttttctttatcacaagggctatctaaactaggctctgatggctgtttatcagtgtttagttgcttagatttttcagaagtttgtgttctaaaaaaactgtctgactggttaggtgcgatattactcatgaagacagctgagtttggttctttctgaaactgtaggttttcaggagtcccaacaaaagaggtgatattttctgattcagtttcctgatctgtgcattctaatttatctaaggataatctttcacccctatttactgcaatagtcacttcctgagaagctgggtctttccctgtctcatttttactatgattttcctggttttccttaaaatattctttcagggtggaaagaagatcatcatctccttcaaggtcaatgtactggatttgttcaaaagctgaatctgcaagttctactggacctattaaatgacaaagatggtcatatatgctatcaccaacttccagagaagactctctactatgagtatcagtgatgtggctttcagtggatctagttattgaagaagcctctgtggaactctgcaagcttggtgcatgacgggatgaactgtcaatgacaggaactgcacctttggctcgttcaacagtgaatggttccaagatgtcagaagtgctgctacttcgaggcaatggctgctcctcattcaaagcaccaaaaacttcatttccagtttcttcactttgtgaaaaatgtctgactctagttgagcggggaagtatttgagcatcatcaatatcgacagttttttgccgtactatactcctcgccttttcggttcctggagaaccagtggttgttgcactcctctgtctcattggggcttggccaggctgatcacgactccatcctctagaaaatgacttgtcaactgaaactttctgaaattcatgtccaactcctttccctttgtgctttttttgtttctgttcactcagcttatccaatggtaaatcactgagatccaaactatataaattcctagctaaaactttagttaatgtctccatagtcagtgaccactcagtggccaactcttcccaataggtcagcgatgacaatactgacagtaagtcatcccaaagttctcgggagatgtacacatttaggtttgctttgatccaggcaactataagggtctggaaaagtggtcctgcaagtcgacctgccaaggtcatattttttttcccttggaactgtagaaaagcttgtgatggcatcttcagtacagattccgtgactctgagcaacacaagcagcatctgttcccaagtctttttgtccattgatacttgtacaaccatgtaccgataaatgttaagaatgcgtttacacatatctgtgtgttcatccagaagattttttatttcatttgcaggttcaagaagaaatatatttgatgagtttataataaacacctgcaaaactgcctgggtaccagctcgtatgttttgttctgtggcttcttcagaggcgttatgaagagcaccttggtaggagccgttttttgcccaactggaatttcgaacatgatcagcagtattggtcccattttcctcttctcttttttctccttcttccattgaaatatcatggtctgtgacattttcaatgcaagggaggtctgaagaagtgatcacaatttcttcaggctcttgcatgaacaaaggtttttcctcttgttggatccattcttgatatacttttaccacttttctcatagctgctgcttcacaaattggtaataaaaatgcctgacgaaatatctctgtcacaaagtttacattactccttttagaagaaaaaactctgcgaactatttcaatgtctgtgagatgttcttcatcaatactacagagactagatgagctaggttctcgctccgtgagagtgcttgtattggaatgagactgttcgggttctgtagttctgtctgttttatcagcattatcatttttgctttcttctctggatactaaactagcagctgctctctgaatattctttggcaagacttcaccttccatcccaggaatatgaggtcctgtatgtggttttggctccagccagaaagaaaccagccaacgaatgacaataacacgagccttaatgaaaggctcctttgtacaatagattgcttcattggtttcagcatctttctttatcacgacataatgtggctttggtctcatctgcgggatgtcaagtataggatgatataaactgttttccttacagatgtttggaaaaatataaggcaagtaatatttcttaaaatgtgaaaacaaaaatgaaaatcccctttcttggttttctttgttcttccattctaaactttttacctgaatgactatgtattttagaagtgcttcaagaaaatagcttgtgagatcttcttgccctttatctcctgattgtggggggacaagaggagtgatttcttctatagtgacttgagtttcttgaaggttgagtggaggattaatgagattatctaaagttcgaggtccatgttcagactgtggtgctgaaaatccagggattaagcatgaaaacatccagagctgttctttgctacagttattctgaagagcttgcaaccatagtaagaaaagacgaacaccttcccgcctaatctttaaggagtttcctgtgtgaagtagcttctttaaaatcaatccaatactatgaaactgccatcgctgatgaattctttctggaagaagttgtaaaattttctcaaaaataaaaagtatagcatccaattcctctctttgagacttgtgacctttctgtttaagactagcttcaatagtcacaaaattttcaaagaacacatagtatatatgtgaaaaatgttggtcgaaaaactgtttaagatcaatagattctgcattctcgatgacgatgcgcaggtgcttgaggcgagtcagtgcgtccttcttggtgtctagcaccttctgggtggacttcttcacgtccccgtgcggcttcttggagaacatcctgtcgctgccactgccactgccactgccacagccggctcccagccgggtcccggcggcagaaagtggagggagtggacggggaggagactagccagagaggctcattagctccccagccttgcgggccagggcagagccgactccttcccgatccaggccagggccgccacct

SEQ ID NO: 17987 - RNA, 4816 nt, Homo sapiens
  source 1..4816: mol_type = other RNA
tctctggagggaagcactttctgaaccagtaatagttgcaacttcagcagagaaagcttgctgattaagactgcttgtttcagaatctatatgaagagtagttagactagccacttcctgctcttcagcactctgatgatggccagaacctgaatccacatcagcagaggacgtaaccccagtgtcggttccaaagccaaaattgtcaaattttcggccatcatattggaaagcgctgaaagaatccgaatgactatctgagctgataagatcactgctccctgcactggcaggagaagtccattctgagggcacacctgggtcatcaatagggcgcatctggttctgcttgtttagaatatcagggaggtctttgggaatttccaggctgcctggactacttcctcttcttgtcatagtcgaggcattaccacttcgaagtcgttctgctataaactcatccatcagatcaggaacattagcactgctgccgccaatatcactattaagaggaggcagtttttggctcatgtcctctttattgactgcagctttccttccaaaatagcccattacatgactgtacagatccctcagtggagcctctggtggcattctgttctgcctctgtggggaaacatttgccttcggcttcgaaagagcatgtacaacagttttataaacgccacccagggagccctgctgtagtcctgcctcatgacttgatgacctaagagtactacgactacctaattgactacttgcaattccttctttttgtaatatggtggtgggaatctctgtggattccttcactgttttgctgcttactgatgcagtaccaagtgtatctagaggtctgtacacaccaggttttactagctctgtagcactatttgtgctggtatgggtgttgctagtgctgctattgctgctaccactactaaagccaccgagcttccgcagtctcatcttccatggagcctctttgttttccagaggattataaaactgaacggactcagtggatggcctaaaagtaacatgaacactatttcgttttttagtagcaattttcatgattttggctctatgagttactgtttcagacaagctccttttagttggagaaagtttgctagtacttgtaacatgaggcattctgcggttaacaggtgcttttagtgttgctttcttggcacgcataacatgtgggacagtgattttttcattaatttgcacactcttaagcttttcaactagtgttacatcaacacaagcatctaattctgtggctgcttgtctgtacagatgtttccttttttctttatcacaagggctatctaaactaggctctgatggctgtttatcagtgtttagttgcttagatttttcagaagtttgtgttctaaaaaaactgtctgactggttaggtgcgatattactcatgaagacagctgagtttggttctttctgaaactgtaggttttcaggagtcccaacaaaagaggtgatattttctgattcagtttcctgatctgtgcattctaatttatctaaggataatctttcacccctatttactgcaatagtcacttcctgagaagctgggtctttccctgtctcatttttactatgattttcctggttttccttaaaatattctttcagggtggaaagaagatcatcatctccttcaaggtcaatgtactggatttgttcaaaagctgaatctgcaagttctactggacctattaaatgacaaagatggtcatatatgctatcaccaacttccagagaagactctctactatgagtatcagtgatgtggctttcagtggatctagttattgaagaagcctctgtggaactctgcaagcttggtgcatgacgggatgaactgtcaatgacaggaactgcacctttggctcgttcaacagtgaatggttccaagatgtcagaagtgctgctacttcgaggcaatggctgctcctcattcaaagcaccaaaaacttcatttccagtttcttcactttgtgaaaaatgtctgactctagttgagcggggaagtatttgagcatcatcaatatcgacagttttttgccgtactatactcctcgccttttcggttcctggagaaccagtggttgttgcactcctctgtctcattggggcttggccaggctgatcacgactccatcctctagaaaatgacttgtcaactgaaactttctgaaattcatgtccaactcctttccctttgtgctttttttgtttctgttcactcagcttatccaatggtaaatcactgagatccaaactatataaattcctagctaaaactttagttaatgtctccatagtcagtgaccactcagtggccaactcttcccaataggtcagcgatgacaatactgacagtaagtcatcccaaagttctcgggagatgtacacatttaggtttgctttgatccaggcaactataagggtctggaaaagtggtcctgcaagtcgacctgccaaggtcatattttttttcccttggaactgtagaaaagcttgtgatggcatcttcagtacagattccgtgactctgagcaacacaagcagcatctgttcccaagtctttttgtccattgatacttgtacaaccatgtaccgataaatgttaagaatgcgtttacacatatctgtgtgttcatccagaagattttttatttcatttgcaggttcaagaagaaatatatttgatgagtttataataaacacctgcaaaactgcctgggtaccagctcgtatgttttgttctgtggcttcttcagaggcgttatgaagagcaccttggtaggagccgttttttgcccaactggaatttcgaacatgatcagcagtattggtcccattttcctcttctcttttttctccttcttccattgaaatatcatggtctgtgacattttcaatgcaagggaggtctgaagaagtgatcacaatttcttcaggctcttgcatgaacaaaggtttttcctcttgttggatccattcttgatatacttttaccacttttctcatagctgctgcttcacaaattggtaataaaaatgcctgacgaaatatctctgtcacaaagtttacattactccttttagaagaaaaaactctgcgaactatttcaatgtctgtgagatgttcttcatcaatactacagagactagatgagctaggttctcgctccgtgagagtgcttgtattggaatgagactgttcgggttctgtagttctgtctgttttatcagcattatcatttttgctttcttctctggatactaaactagcagctgctctctgaatattctttggcaagacttcaccttccatcccaggaatatgaggtcctgtatgtggttttggctccagccagaaagaaaccagccaacgaatgacaataacacgagccttaatgaaaggctcctttgtacaatagattgcttcattggtttcagcatctttctttatcacgacataatgtggctttggtctcatctgcgggatgtcaagtataggatgatataaactgttttccttacagatgtttggaaaaatataaggcaagtaatatttcttaaaatgtgaaaacaaaaatgaaaatcccctttcttggttttctttgttcttccattctaaactttttacctgaatgactatgtattttagaagtgcttcaagaaaatagcttgtgagatcttcttgccctttatctcctgattgtggggggacaagaggagtgatttcttctatagtgacttgagtttcttgaaggttgagtggaggattaatgagattatctaaagttcgaggtccatgttcagactgtggtgctgaaaatccagggattaagcatgaaaacatccagagctgttctttgctacagttattctgaagagcttgcaaccatagtaagaaaagacgaacaccttcccgcctaatctttaaggagtttcctgtgtgaagtagcttctttaaaatcaatccaatactatgaaactgccatcgctgatgaattctttctggaagaagttgtaaaattttctcaaaaataaaaagtatagcatccaattcctctctttgagacttgtgacctttctgtttaagactagcttcaatagtcacaaaattttcaaagaacacatagtatatatgtgaaaaatgttggtcgaaaaactgtttaagatcaatagattctgcattctcgatgacgatgcgcaggtgcttgaggcgagtcagtgcgtccttcttggtgtctagcaccttctgggtggacttcttcacgtccccgtgcggcttcttggagaacatcctgtcgctgccactgccactgccactgccacagccggctcccagccgggtcccggcggcagaaagtggagggagtggacggggaggagactagccagagaggctcattagctccccagccttgcgggccagggcagagccgactccttcccgatccaggccagggccgccacctccacccgcctcgcgccgcggctccaaggcaccttcggccccagctccaatatggcggatccctctcccggccctgcacggagcgaggcagacccgggctggccgcctgccgccgccgctcgtctccagcggccgccgctcgccgccacaggccggggccccggacccagagccacgaaggtggagctctcggcggcaggagcacaactctctccctgaggcccccttaaggttgaagcttctttagcagcttacaccctgcagaggccgaaacggagacgagtgt

SEQ ID NO: 17988 - RNA, 4672 nt, Homo sapiens
  source 1..4672: mol_type = other RNA
tctctggagggaagcactttctgaaccagtaatagttgcaacttcagcagagaaagcttgctgattaagactgcttgtttcagaatctatatgaagagtagttagactagccacttcctgctcttcagcactctgatgatggccagaacctgaatccacatcagcagaggacgtaaccccagtgtcggttccaaagccaaaattgtcaaattttcggccatcatattggaaagcgctgaaagaatccgaatgactatctgagctgataagatcactgctccctgcactggcaggagaagtccattctgagggcacacctgggtcatcaatagggcgcatctggttctgcttgtttagaatatcagggaggtctttgggaatttccaggctgcctggactacttcctcttcttgtcatagtcgaggcattaccacttcgaagtcgttctgctataaactcatccatcagatcaggaacattagcactgctgccgccaatatcactattaagaggaggcagtttttggctcatgtcctctttattgactgcagctttccttccaaaatagcccattacatgactgtacagatccctcagtggagcctctggtggcattctgttctgcctctgtggggaaacatttgccttcggcttcgaaagagcatgtacaacagttttataaacgccacccagggagccctgctgtagtcctgcctcatgacttgatgacctaagagtactacgactacctaattgactacttgcaattccttctttttgtaatatggtggtgggaatctctgtggattccttcactgttttgctgcttactgatgcagtaccaagtgtatctagaggtctgtacacaccaggttttactagctctgtagcactatttgtgctggtatgggtgttgctagtgctgctattgctgctaccactactaaagccaccgagcttccgcagtctcatcttccatggagcctctttgttttccagaggattataaaactgaacggactcagtggatggcctaaaagtaacatgaacactatttcgttttttagtagcaattttcatgattttggctctatgagttactgtttcagacaagctccttttagttggagaaagtttgctagtacttgtaacatgaggcattctgcggttaacaggtgcttttagtgttgctttcttggcacgcataacatgtgggacagtgattttttcattaatttgcacactcttaagcttttcaactagtgttacatcaacacaagcatctaattctgtggctgcttgtctgtacagatgtttccttttttctttatcacaagggctatctaaactaggctctgatggctgtttatcagtgtttagttgcttagatttttcagaagtttgtgttctaaaaaaactgtctgactggttaggtgcgatattactcatgaagacagctgagtttggttctttctgaaactgtaggttttcaggagtcccaacaaaagaggtgatattttctgattcagtttcctgatctgtgcattctaatttatctaaggataatctttcacccctatttactgcaatagtcacttcctgagaagctgggtctttccctgtctcatttttactatgattttcctggttttccttaaaatattctttcagggtggaaagaagatcatcatctccttcaaggtcaatgtactggatttgttcaaaagctgaatctgcaagttctactggacctattaaatgacaaagatggtcatatatgctatcaccaacttccagagaagactctctactatgagtatcagtgatgtggctttcagtggatctagttattgaagaagcctctgtggaactctgcaagcttggtgcatgacgggatgaactgtcaatgacaggaactgcacctttggctcgttcaacagtgaatggttccaagatgtcagaagtgctgctacttcgaggcaatggctgctcctcattcaaagcaccaaaaacttcatttccagtttcttcactttgtgaaaaatgtctgactctagttgagcggggaagtatttgagcatcatcaatatctgaaagctcatcagaaaggggagtgagaacaatatcaggcaagaagggtttggaagtatggatcagaacaggagcacttttagcactgcgtatataggccgatggcagagcacattcaccaatggatcggcttctcatggcgacagttttttgccgtactatactcctcgccttttcggttcctggagaaccagtggttgttgcactcctctgtctcattggggcttggccaggctgatcacgactccatcctctagaaaatgacttgtcaactgaaactttctgaaattcatgtccaactcctttccctttgtgctttttttgtttctgttcactcagcttatccaatggtaaatcactgagatccaaactatataaattcctagctaaaactttagttaatgtctccatagtcagtgaccactcagtggccaactcttcccaataggtcagcgatgacaatactgacagtaagtcatcccaaagttctcgggagatgtacacatttaggtttgctttgatccaggcaactataagggtctggaaaagtggtcctgcaagtcgacctgccaaggtcatattttttttcccttggaactgtagaaaagcttgtgatggcatcttcagtacagattccgtgactctgagcaacacaagcagcatctgttcccaagtctttttgtccattgatacttgtacaaccatgtaccgataaatgttaagaatgcgtttacacatatctgtgtgttcatccagaagattttttatttcatttgcaggttcaagaagaaatatatttgatgagtttataataaacacctgcaaaactgcctgggtaccagctcgtatgttttgttctgtggcttcttcagaggcgttatgaagagcaccttggtaggagccgttttttgcccaactggaatttcgaacatgatcagcagtattggtcccattttcctcttctcttttttctccttcttccattgaaatatcatggtctgtgacattttcaatgcaagggaggtctgaagaagtgatcacaatttcttcaggctcttgcatgaacaaaggtttttcctcttgttggatccattcttgatatacttttaccacttttctcatagctgctgcttcacaaattggtaataaaaatgcctgacgaaatatctctgtcacaaagtttacattactccttttagaagaaaaaactctgcgaactatttcaatgtctgtgagatgttcttcatcaatactacagagactagatgagctaggttctcgctccgtgagagtgcttgtattggaatgagactgttcgggttctgtagttctgtctgttttatcagcattatcatttttgctttcttctctggatactaaactagcagctgctctctgaatattctttggcaagacttcaccttccatcccaggaatatgaggtcctgtatgtggttttggctccagccagaaagaaaccagccaacgaatgacaataacacgagccttaatgaaaggctcctttgtacaatagattgcttcattggtttcagcatctttctttatcacgacataatgtggctttggtctcatctgcgggatgtcaagtataggatgatataaactgttttccttacagatgtttggaaaaatataaggcaagtaatatttcttaaaatgtgaaaacaaaaatgaaaatcccctttcttggttttctttgttcttccattctaaactttttacctgaatgactatgtattttagaagtgcttcaagaaaatagcttgtgagatcttcttgccctttatctcctgattgtggggggacaagaggagtgatttcttctatagtgacttgagtttcttgaaggttgagtggaggattaatgagattatctaaagttcgaggtccatgttcagactgtggtgctgaaaatccagggattaagcatgaaaacatccagagctgttctttgctacagttattctgaagagcttgcaaccatagtaagaaaagacgaacaccttcccgcctaatctttaaggagtttcctgtgtgaagtagcttctttaaaatcaatccaatactatgaaactgccatcgctgatgaattctttctggaagaagttgtaaaattttctcaaaaataaaaagtatagcatccaattcctctctttgagacttgtgacctttctgtttaagactagcttcaatagtcacaaaattttcaaagaacacatagtatatatgtgaaaaatgttggtcgaaaaactgtttaagatcaatagattctgcattctcgatgacgatgcgcaggtgcttgaggcgagtcagtgcgtccttcttggtgtctagcaccttctgggtggacttcttcacgtccccgtgcggcttcttggagaacatcctgtcgctgccactgccactgccactgccacagccggctcccagccgggtcccggcggcagaaagtggagggagtggacggggaggagactagccagagaggctcattagctccccagccttgcgggccagggcagagccgactccttcccgatccaggccagggccgccacct

SEQ ID NO: 17989 - RNA, 4957 nt, Homo sapiens
  source 1..4957: mol_type = other RNA
tctctggagggaagcactttctgaaccagtaatagttgcaacttcagcagagaaagcttgctgattaagactgcttgtttcagaatctatatgaagagtagttagactagccacttcctgctcttcagcactctgatgatggccagaacctgaatccacatcagcagaggacgtaaccccagtgtcggttccaaagccaaaattgtcaaattttcggccatcatattggaaagcgctgaaagaatccgaatgactatctgagctgataagatcactgctccctgcactggcaggagaagtccattctgagggcacacctgggtcatcaatagggcgcatctggttctgcttgtttagaatatcagggaggtctttgggaatttccaggctgcctggactacttcctcttcttgtcatagtcgaggcattaccacttcgaagtcgttctgctataaactcatccatcagatcaggaacattagcactgctgccgccaatatcactattaagaggaggcagtttttggctcatgtcctctttattgactgcagctttccttccaaaatagcccattacatgactgtacagatccctcagtggagcctctggtggcattctgttctgcctctgtggggaaacatttgccttcggcttcgaaagagcatgtacaacagttttataaacgccacccagggagccctgctgtagtcctgcctcatgacttgatgacctaagagtactacgactacctaattgactacttgcaattccttctttttgtaatatggtggtgggaatctctgtggattccttcactgttttgctgcttactgatgcagtaccaagtgtatctagaggtctgtacacaccaggttttactagctctgtagcactatttgtgctggtatgggtgttgctagtgctgctattgctgctaccactactaaagccaccgagcttccgcagtctcatcttccatggagcctctttgttttccagaggattataaaactgaacggactcagtggatggcctaaaagtaacatgaacactatttcgttttttagtagcaattttcatgattttggctctatgagttactgtttcagacaagctccttttagttggagaaagtttgctagtacttgtaacatgaggcattctgcggttaacaggtgcttttagtgttgctttcttggcacgcataacatgtgggacagtgattttttcattaatttgcacactcttaagcttttcaactagtgttacatcaacacaagcatctaattctgtggctgcttgtctgtacagatgtttccttttttctttatcacaagggctatctaaactaggctctgatggctgtttatcagtgtttagttgcttagatttttcagaagtttgtgttctaaaaaaactgtctgactggttaggtgcgatattactcatgaagacagctgagtttggttctttctgaaactgtaggttttcaggagtcccaacaaaagaggtgatattttctgattcagtttcctgatctgtgcattctaatttatctaaggataatctttcacccctatttactgcaatagtcacttcctgagaagctgggtctttccctgtctcatttttactatgattttcctggttttccttaaaatattctttcagggtggaaagaagatcatcatctccttcaaggtcaatgtactggatttgttcaaaagctgaatctgcaagttctactggacctattaaatgacaaagatggtcatatatgctatcaccaacttccagagaagactctctactatgagtatcagtgatgtggctttcagtggatctagttattgaagaagcctctgtggaactctgcaagcttggtgcatgacgggatgaactgtcaatgacaggaactgcacctttggctcgttcaacagtgaatggttccaagatgtcagaagtgctgctacttcgaggcaatggctgctcctcattcaaagcaccaaaaacttcatttccagtttcttcactttgtgaaaaatgtctgactctagttgagcggggaagtatttgagcatcatcaatatctgaaagctcatcagaaaggggagtgagaacaatatcaggcaagaagggtttggaagtatggatcagaacaggagcacttttagcactgcgtatataggccgatggcagagcacattcaccaatggatcggcttctcatggcgacagttttttgccgtactatactcctcgccttttcggttcctggagaaccagtggttgttgcactcctctgtctcattggggcttggccaggctgatcacgactccatcctctagaaaatgacttgtcaactgaaactttctgaaattcatgtccaactcctttccctttgtgctttttttgtttctgttcactcagcttatccaatggtaaatcactgagatccaaactatataaattcctagctaaaactttagttaatgtctccatagtcagtgaccactcagtggccaactcttcccaataggtcagcgatgacaatactgacagtaagtcatcccaaagttctcgggagatgtacacatttaggtttgctttgatccaggcaactataagggtctggaaaagtggtcctgcaagtcgacctgccaaggtcatattttttttcccttggaactgtagaaaagcttgtgatggcatcttcagtacagattccgtgactctgagcaacacaagcagcatctgttcccaagtctttttgtccattgatacttgtacaaccatgtaccgataaatgttaagaatgcgtttacacatatctgtgtgttcatccagaagattttttatttcatttgcaggttcaagaagaaatatatttgatgagtttataataaacacctgcaaaactgcctgggtaccagctcgtatgttttgttctgtggcttcttcagaggcgttatgaagagcaccttggtaggagccgttttttgcccaactggaatttcgaacatgatcagcagtattggtcccattttcctcttctcttttttctccttcttccattgaaatatcatggtctgtgacattttcaatgcaagggaggtctgaagaagtgatcacaatttcttcaggctcttgcatgaacaaaggtttttcctcttgttggatccattcttgatatacttttaccacttttctcatagctgctgcttcacaaattggtaataaaaatgcctgacgaaatatctctgtcacaaagtttacattactccttttagaagaaaaaactctgcgaactatttcaatgtctgtgagatgttcttcatcaatactacagagactagatgagctaggttctcgctccgtgagagtgcttgtattggaatgagactgttcgggttctgtagttctgtctgttttatcagcattatcatttttgctttcttctctggatactaaactagcagctgctctctgaatattctttggcaagacttcaccttccatcccaggaatatgaggtcctgtatgtggttttggctccagccagaaagaaaccagccaacgaatgacaataacacgagccttaatgaaaggctcctttgtacaatagattgcttcattggtttcagcatctttctttatcacgacataatgtggctttggtctcatctgcgggatgtcaagtataggatgatataaactgttttccttacagatgtttggaaaaatataaggcaagtaatatttcttaaaatgtgaaaacaaaaatgaaaatcccctttcttggttttctttgttcttccattctaaactttttacctgaatgactatgtattttagaagtgcttcaagaaaatagcttgtgagatcttcttgccctttatctcctgattgtggggggacaagaggagtgatttcttctatagtgacttgagtttcttgaaggttgagtggaggattaatgagattatctaaagttcgaggtccatgttcagactgtggtgctgaaaatccagggattaagcatgaaaacatccagagctgttctttgctacagttattctgaagagcttgcaaccatagtaagaaaagacgaacaccttcccgcctaatctttaaggagtttcctgtgtgaagtagcttctttaaaatcaatccaatactatgaaactgccatcgctgatgaattctttctggaagaagttgtaaaattttctcaaaaataaaaagtatagcatccaattcctctctttgagacttgtgacctttctgtttaagactagcttcaatagtcacaaaattttcaaagaacacatagtatatatgtgaaaaatgttggtcgaaaaactgtttaagatcaatagattctgcattctcgatgacgatgcgcaggtgcttgaggcgagtcagtgcgtccttcttggtgtctagcaccttctgggtggacttcttcacgtccccgtgcggcttcttggagaacatcctgtcgctgccactgccactgccactgccacagccggctcccagccgggtcccggcggcagaaagtggagggagtggacggggaggagactagccagagaggctcattagctccccagccttgcgggccagggcagagccgactccttcccgatccaggccagggccgccacctccacccgcctcgcgccgcggctccaaggcaccttcggccccagctccaatatggcggatccctctcccggccctgcacggagcgaggcagacccgggctggccgcctgccgccgccgctcgtctccagcggccgccgctcgccgccacaggccggggccccggacccagagccacgaaggtggagctctcggcggcaggagcacaactctctccctgaggcccccttaaggttgaagcttctttagcagcttacaccctgcagaggccgaaacggagacgagtgt

SEQ ID NO: 17990 - RNA, 2635 nt, Homo sapiens
  source 1..2635: mol_type = other RNA
tctctggagggaagcactttctgaaccagtaatagttgcaacttcagcagagaaagcttgctgattaagactgcttgtttcagaatctatatgaagagtagttagactagccacttcctgctcttcagcactctgatgatggccagaacctgaatccacatcagcagaggacgtaaccccagtgtcggttccaaagccaaaattgtcaaattttcggccatcatattggaaagcgctgaaagaatccgaatgactatctgagctgataagatcactgctccctgcactggcaggagaagtccattctgagggcacacctgggtcatcaatagggcgcatctggttctgcttgtttagaatatcagggaggtctttgggaatttccaggctgcctggactacttcctcttcttgtcatagtcgaggcattaccacttcgaagtcgttctgctataaactcatccatcagatcaggaacattagcactgctgccgccaatatcactattaagaggaggcagtttttggctcatgtcctctttattgactgcagctttccttccaaaatagcccattacatgactgtacagatccctcagtggagcctctggtggcattctgttctgcctctgtggggaaacatttgccttcggcttcgaaagagcatgtacaacagttttataaacgccacccagggagccctgctgtagtcctgcctcatgacttgatgacctaagagtactacgactacctaattgactacttgcaattccttctttttgtaatatggtggtgggaatctctgtggattccttcactgttttgctgcttactgatgcagtaccaagtgtatctagaggtctgtacacaccaggttttactagctctgtagcactatttgtgctggtatgggtgttgctagtgctgctattgctgctaccactactaaagccaccgagcttccgcagtctcatcttccatggagcctctttgttttccagaggattataaaactgaacggactcagtggatggcctaaaagtaacatgaacactatttcgttttttagtagcaattttcatgattttggctctatgagttactgtttcagacaagctccttttagttggagaaagtttgctagtacttgtaacatgaggcattctgcggttaacaggtgcttttagtgttgctttcttggcacgcataacatgtgggacagtgattttttcattaatttgcacactcttaagcttttcaactagtgttacatcaacacaagcatctaattctgtggctgcttgtctgtacagatgtttccttttttctttatcacaagggctatctaaactaggctctgatggctgtttatcagtgtttagttgcttagatttttcagaagtttgtgttctaaaaaaactgtctgactggttaggtgcgatattactcatgaagacagctgagtttggttctttctgaaactgtaggttttcaggagtcccaacaaaagaggtgatattttctgattcagtttcctgatctgtgcattctaatttatctaaggataatctttcacccctatttactgcaatagtcacttcctgagaagctgggtctttccctgtctcatttttactatgattttcctggttttccttaaaatattctttcagggtggaaagaagatcatcatctccttcaaggtcaatgtactggatttgttcaaaagctgaatctgcaagttctactggacctattaaatgacaaagatggtcatatatgctatcaccaacttccagagaagactctctactatgagtatcagtgatgtggctttcagtggatctagttattgaagaagcctctgtggaactctgcaagcttggtgcatgacgggatgaactgtcaatgacaggaactgcacctttggctcgttcaacagtgaatggttccaagatgtcagaagtgctgctacttcgaggcaatggctgctcctcattcaaagcaccaaaaacttcatttccagtttcttcactttgtgaaaaatgtctgactctagttgagcggggaagtatttgagcatcatcaatatctgaaagctcatcagaaaggggagtgagaacaatatcaggcaagaagggtttggaagtatggatcagaacaggagcacttttagcactgcgtatataggccgatggcagagcacattcaccaatggatcggcttctcatggctgaaattaacttgtatccttctcaagataaccaatttaacatggaagtcttcaattcagtcatccaaccttgaagcttgctcaagtctcagtctgaatcccagaagtgattatcagcaatttgcttcaagatcatcccacttttccagtgtgcttactgctcatcactccattttccactcatagttttattttggtcaaggaaatgagtaagaagagtcttagaggtttctctatttgcaaaccagtggtacgacgaaatgctagcaagaatatctaatagctccagaatatcaagttcactatgttgctggcaatacgagtcatgtaatgactttttaaaaagcccctttcttcccaattttttattaagaaaattttcaaatgtagaaaaaattaaaaga

SEQ ID NO: 17991 - RNA, 2494 nt, Homo sapiens
  source 1..2494: mol_type = other RNA
tctctggagggaagcactttctgaaccagtaatagttgcaacttcagcagagaaagcttgctgattaagactgcttgtttcagaatctatatgaagagtagttagactagccacttcctgctcttcagcactctgatgatggccagaacctgaatccacatcagcagaggacgtaaccccagtgtcggttccaaagccaaaattgtcaaattttcggccatcatattggaaagcgctgaaagaatccgaatgactatctgagctgataagatcactgctccctgcactggcaggagaagtccattctgagggcacacctgggtcatcaatagggcgcatctggttctgcttgtttagaatatcagggaggtctttgggaatttccaggctgcctggactacttcctcttcttgtcatagtcgaggcattaccacttcgaagtcgttctgctataaactcatccatcagatcaggaacattagcactgctgccgccaatatcactattaagaggaggcagtttttggctcatgtcctctttattgactgcagctttccttccaaaatagcccattacatgactgtacagatccctcagtggagcctctggtggcattctgttctgcctctgtggggaaacatttgccttcggcttcgaaagagcatgtacaacagttttataaacgccacccagggagccctgctgtagtcctgcctcatgacttgatgacctaagagtactacgactacctaattgactacttgcaattccttctttttgtaatatggtggtgggaatctctgtggattccttcactgttttgctgcttactgatgcagtaccaagtgtatctagaggtctgtacacaccaggttttactagctctgtagcactatttgtgctggtatgggtgttgctagtgctgctattgctgctaccactactaaagccaccgagcttccgcagtctcatcttccatggagcctctttgttttccagaggattataaaactgaacggactcagtggatggcctaaaagtaacatgaacactatttcgttttttagtagcaattttcatgattttggctctatgagttactgtttcagacaagctccttttagttggagaaagtttgctagtacttgtaacatgaggcattctgcggttaacaggtgcttttagtgttgctttcttggcacgcataacatgtgggacagtgattttttcattaatttgcacactcttaagcttttcaactagtgttacatcaacacaagcatctaattctgtggctgcttgtctgtacagatgtttccttttttctttatcacaagggctatctaaactaggctctgatggctgtttatcagtgtttagttgcttagatttttcagaagtttgtgttctaaaaaaactgtctgactggttaggtgcgatattactcatgaagacagctgagtttggttctttctgaaactgtaggttttcaggagtcccaacaaaagaggtgatattttctgattcagtttcctgatctgtgcattctaatttatctaaggataatctttcacccctatttactgcaatagtcacttcctgagaagctgggtctttccctgtctcatttttactatgattttcctggttttccttaaaatattctttcagggtggaaagaagatcatcatctccttcaaggtcaatgtactggatttgttcaaaagctgaatctgcaagttctactggacctattaaatgacaaagatggtcatatatgctatcaccaacttccagagaagactctctactatgagtatcagtgatgtggctttcagtggatctagttattgaagaagcctctgtggaactctgcaagcttggtgcatgacgggatgaactgtcaatgacaggaactgcacctttggctcgttcaacagtgaatggttccaagatgtcagaagtgctgctacttcgaggcaatggctgctcctcattcaaagcaccaaaaacttcatttccagtttcttcactttgtgaaaaatgtctgactctagttgagcggggaagtatttgagcatcatcaatatctgaaattaacttgtatccttctcaagataaccaatttaacatggaagtcttcaattcagtcatccaaccttgaagcttgctcaagtctcagtctgaatcccagaagtgattatcagcaatttgcttcaagatcatcccacttttccagtgtgcttactgctcatcactccattttccactcatagttttattttggtcaaggaaatgagtaagaagagtcttagaggtttctctatttgcaaaccagtggtacgacgaaatgctagcaagaatatctaatagctccagaatatcaagttcactatgttgctggcaatacgagtcatgtaatgactttttaaaaagcccctttcttcccaattttttattaagaaaattttcaaatgtagaaaaaattaaaaga

SEQ ID NO: 17992 - RNA, 1199 nt, Homo sapiens
  source 1..1199: mol_type = other RNA
tctctggagggaagcactttctgaaccagtaatagttgcaacttcagcagagaaagcttgctgattaagactgcttgtttcagaatctatatgaagagtagttagactagccacttcctgctcttcagcactctgatgatggccagaacctgaatccacatcagcagaggacgtaaccccagtgtcggttccaaagccaaaattgtcaaattttcggccatcatattggaaagcgctgaaagaatccgaatgactatctgagctgataagatcactgctccctgcactggcaggagaagtccattctgagggcacacctgggtcatcaatagggcgcatctggttctgcttgtttagaatatcagggaggtctttgggaatttccaggctgcctggactacttcctcttcttgtcatagtcgaggcattaccacttcgaagtcgttctgctataaactcatccatcagatcaggaacattagcactgctgccgccaatatcactattaagaggaggcagtttttggctcatgtcctctttattgactgcagctttccttccaaaatagcccattacatgactgtacagatccctcagtggagcctctggtggcattctgttctgcctctttggctcgttcaacagtgaatggttccaagatgtcagaagtgctgctacttcgaggcaatggctgctcctcattcaaagcaccaaaaacttcatttccagtttcttcactttgtgaaaaatgtctgactctagttgagcggggaagtatttgagcatcatcaatatctgaaattaacttgtatccttctcaagataaccaatttaacatggaagtcttcaattcagtcatccaaccttgaagcttgctcaagtctcagtctgaatcccagaagtgattatcagcaatttgcttcaagatcatcccacttttccagtgtgcttactgctcatcactccattttccactcatagttttattttggtcaaggaaatgagtaagaagagtcttagaggtttctctatttgcaaaccagtggtacgacgaaatgctagcaagaatatctaatagctccagaatatcaagttcactatgttgctggcaatacgagtcatgtaatgactttttaaaaagcccctttcttcccaattttttattaagaaaattttcaaatgtagaaaaaattaaaaga

SEQ ID NO: 17993 - RNA, 3439 nt, Homo sapiens
  source 1..3439: mol_type = other RNA
tctctggagggaagcactttctgaaccagtaatagttgcaacttcagcagagaaagcttgctgattaagactgcttgtttcagaatctatatgaagagtagttagactagccacttcctgctcttcagcactctgatgatggccagaacctgaatccacatcagcagaggacgtaaccccagtgtcggttccaaagccaaaattgtcaaattttcggccatcatattggaaagcgctgaaagaatccgaatgactatctgagctgataagatcactgctccctgcactggcaggagaagtccattctgagggcacacctgggtcatcaatagggcgcatctggttctgcttgtttagaatatcagggaggtctttgggaatttccaggctgcctggactacttcctcttcttgtcatagtcgaggcattaccacttcgaagtcgttctgctataaactcatccatcagatcaggaacattagcactgctgccgccaatatcactattaagaggaggcagtttttggctcatgtcctctttattgactttggctcgttcaacagtgaatggttccaagatgtcagaagtgctgctacttcgaggcaatggctgctcctcattcaaagcaccaaaaacttcatttccagtttcttcactttgtgaaaaatgtctgactctagttgagcggggaagtatttgagcatcatcaatatcgacagttttttgccgtactatactcctcgccttttcggttcctggagaaccagtggttgttgcactcctctgtctcattggggcttggccaggctgatcacgactccatcctctagaaaatgacttgtcaactgaaactttctgaaattcatgtccaactcctttccctttgtgctttttttgtttctgttcactcagcttatccaatggtaaatcactgagatccaaactatataaattcctagctaaaactttagttaatgtctccatagtcagtgaccactcagtggccaactcttcccaataggtcagcgatgacaatactgacagtaagtcatcccaaagttctcgggagatgtacacatttaggtttgctttgatccaggcaactataagggtctggaaaagtggtcctgcaagtcgacctgccaaggtcatattttttttcccttggaactgtagaaaagcttgtgatggcatcttcagtacagattccgtgactctgagcaacacaagcagcatctgttcccaagtctttttgtccattgatacttgtacaaccatgtaccgataaatgttaagaatgcgtttacacatatctgtgtgttcatccagaagattttttatttcatttgcaggttcaagaagaaatatatttgatgagtttataataaacacctgcaaaactgcctgggtaccagctcgtatgttttgttctgtggcttcttcagaggcgttatgaagagcaccttggtaggagccgttttttgcccaactggaatttcgaacatgatcagcagtattggtcccattttcctcttctcttttttctccttcttccattgaaatatcatggtctgtgacattttcaatgcaagggaggtctgaagaagtgatcacaatttcttcaggctcttgcatgaacaaaggtttttcctcttgttggatccattcttgatatacttttaccacttttctcatagctgctgcttcacaaattggtaataaaaatgcctgacgaaatatctctgtcacaaagtttacattactccttttagaagaaaaaactctgcgaactatttcaatgtctgtgagatgttcttcatcaatactacagagactagatgagctaggttctcgctccgtgagagtgcttgtattggaatgagactgttcgggttctgtagttctgtctgttttatcagcattatcatttttgctttcttctctggatactaaactagcagctgctctctgaatattctttggcaagacttcaccttccatcccaggaatatgaggtcctgtatgtggttttggctccagccagaaagaaaccagccaacgaatgacaataacacgagccttaatgaaaggctcctttgtacaatagattgcttcattggtttcagcatctttctttatcacgacataatgtggctttggtctcatctgcgggatgtcaagtataggatgatataaactgttttccttacagatgtttggaaaaatataaggcaagtaatatttcttaaaatgtgaaaacaaaaatgaaaatcccctttcttggttttctttgttcttccattctaaactttttacctgaatgactatgtattttagaagtgcttcaagaaaatagcttgtgagatcttcttgccctttatctcctgattgtggggggacaagaggagtgatttcttctatagtgacttgagtttcttgaaggttgagtggaggattaatgagattatctaaagttcgaggtccatgttcagactgtggtgctgaaaatccagggattaagcatgaaaacatccagagctgttctttgctacagttattctgaagagcttgcaaccatagtaagaaaagacgaacaccttcccgcctaatctttaaggagtttcctgtgtgaagtagcttctttaaaatcaatccaatactatgaaactgccatcgctgatgaattctttctggaagaagttgtaaaattttctcaaaaataaaaagtatagcatccaattcctctctttgagacttgtgacctttctgtttaagactagcttcaatagtcacaaaattttcaaagaacacatagtatatatgtgaaaaatgttggtcgaaaaactgtttaagatcaatagattctgcattctcgatgacgatgcgcaggtgcttgaggcgagtcagtgcgtccttcttggtgtctagcaccttctgggtggacttcttcacgtccccgtgcggcttcttggagaacatcctgtcgctgccactgccactgccactgccacagccggctcccagccgggtcccggcggcagaaagtggagggagtggacggggaggagactagccagagaggctcattagctccccagccttgcgggccagggcagagccgactccttcccgatccaggccagggccgccacctccacccgcctcgcgccgcggctccaaggcaccttcggccccagctccaatatggcggatccctctcccggccctgcacggagcgaggcagacccgggctggccgcctgccgccgccgctcgtctccagcggccgccgctcgccgccacaggccggggccccggacccagagccacgaaggtggagctctcggcggcaggagcacaactctctccctgaggcccccttaaggttgaagcttctttagcagcttacaccctgcagaggccgaaacggagacgagtgt

SEQ ID NO: 17994 - RNA, 3295 nt, Homo sapiens
  source 1..3295: mol_type = other RNA
tctctggagggaagcactttctgaaccagtaatagttgcaacttcagcagagaaagcttgctgattaagactgcttgtttcagaatctatatgaagagtagttagactagccacttcctgctcttcagcactctgatgatggccagaacctgaatccacatcagcagaggacgtaaccccagtgtcggttccaaagccaaaattgtcaaattttcggccatcatattggaaagcgctgaaagaatccgaatgactatctgagctgataagatcactgctccctgcactggcaggagaagtccattctgagggcacacctgggtcatcaatagggcgcatctggttctgcttgtttagaatatcagggaggtctttgggaatttccaggctgcctggactacttcctcttcttgtcatagtcgaggcattaccacttcgaagtcgttctgctataaactcatccatcagatcaggaacattagcactgctgccgccaatatcactattaagaggaggcagtttttggctcatgtcctctttattgactttggctcgttcaacagtgaatggttccaagatgtcagaagtgctgctacttcgaggcaatggctgctcctcattcaaagcaccaaaaacttcatttccagtttcttcactttgtgaaaaatgtctgactctagttgagcggggaagtatttgagcatcatcaatatctgaaagctcatcagaaaggggagtgagaacaatatcaggcaagaagggtttggaagtatggatcagaacaggagcacttttagcactgcgtatataggccgatggcagagcacattcaccaatggatcggcttctcatggcgacagttttttgccgtactatactcctcgccttttcggttcctggagaaccagtggttgttgcactcctctgtctcattggggcttggccaggctgatcacgactccatcctctagaaaatgacttgtcaactgaaactttctgaaattcatgtccaactcctttccctttgtgctttttttgtttctgttcactcagcttatccaatggtaaatcactgagatccaaactatataaattcctagctaaaactttagttaatgtctccatagtcagtgaccactcagtggccaactcttcccaataggtcagcgatgacaatactgacagtaagtcatcccaaagttctcgggagatgtacacatttaggtttgctttgatccaggcaactataagggtctggaaaagtggtcctgcaagtcgacctgccaaggtcatattttttttcccttggaactgtagaaaagcttgtgatggcatcttcagtacagattccgtgactctgagcaacacaagcagcatctgttcccaagtctttttgtccattgatacttgtacaaccatgtaccgataaatgttaagaatgcgtttacacatatctgtgtgttcatccagaagattttttatttcatttgcaggttcaagaagaaatatatttgatgagtttataataaacacctgcaaaactgcctgggtaccagctcgtatgttttgttctgtggcttcttcagaggcgttatgaagagcaccttggtaggagccgttttttgcccaactggaatttcgaacatgatcagcagtattggtcccattttcctcttctcttttttctccttcttccattgaaatatcatggtctgtgacattttcaatgcaagggaggtctgaagaagtgatcacaatttcttcaggctcttgcatgaacaaaggtttttcctcttgttggatccattcttgatatacttttaccacttttctcatagctgctgcttcacaaattggtaataaaaatgcctgacgaaatatctctgtcacaaagtttacattactccttttagaagaaaaaactctgcgaactatttcaatgtctgtgagatgttcttcatcaatactacagagactagatgagctaggttctcgctccgtgagagtgcttgtattggaatgagactgttcgggttctgtagttctgtctgttttatcagcattatcatttttgctttcttctctggatactaaactagcagctgctctctgaatattctttggcaagacttcaccttccatcccaggaatatgaggtcctgtatgtggttttggctccagccagaaagaaaccagccaacgaatgacaataacacgagccttaatgaaaggctcctttgtacaatagattgcttcattggtttcagcatctttctttatcacgacataatgtggctttggtctcatctgcgggatgtcaagtataggatgatataaactgttttccttacagatgtttggaaaaatataaggcaagtaatatttcttaaaatgtgaaaacaaaaatgaaaatcccctttcttggttttctttgttcttccattctaaactttttacctgaatgactatgtattttagaagtgcttcaagaaaatagcttgtgagatcttcttgccctttatctcctgattgtggggggacaagaggagtgatttcttctatagtgacttgagtttcttgaaggttgagtggaggattaatgagattatctaaagttcgaggtccatgttcagactgtggtgctgaaaatccagggattaagcatgaaaacatccagagctgttctttgctacagttattctgaagagcttgcaaccatagtaagaaaagacgaacaccttcccgcctaatctttaaggagtttcctgtgtgaagtagcttctttaaaatcaatccaatactatgaaactgccatcgctgatgaattctttctggaagaagttgtaaaattttctcaaaaataaaaagtatagcatccaattcctctctttgagacttgtgacctttctgtttaagactagcttcaatagtcacaaaattttcaaagaacacatagtatatatgtgaaaaatgttggtcgaaaaactgtttaagatcaatagattctgcattctcgatgacgatgcgcaggtgcttgaggcgagtcagtgcgtccttcttggtgtctagcaccttctgggtggacttcttcacgtccccgtgcggcttcttggagaacatcctgtcgctgccactgccactgccactgccacagccggctcccagccgggtcccggcggcagaaagtggagggagtggacggggaggagactagccagagaggctcattagctccccagccttgcgggccagggcagagccgactccttcccgatccaggccagggccgccacct

SEQ ID NO: 17995 - RNA, 3580 nt, Homo sapiens
  source 1..3580: mol_type = other RNA
tctctggagggaagcactttctgaaccagtaatagttgcaacttcagcagagaaagcttgctgattaagactgcttgtttcagaatctatatgaagagtagttagactagccacttcctgctcttcagcactctgatgatggccagaacctgaatccacatcagcagaggacgtaaccccagtgtcggttccaaagccaaaattgtcaaattttcggccatcatattggaaagcgctgaaagaatccgaatgactatctgagctgataagatcactgctccctgcactggcaggagaagtccattctgagggcacacctgggtcatcaatagggcgcatctggttctgcttgtttagaatatcagggaggtctttgggaatttccaggctgcctggactacttcctcttcttgtcatagtcgaggcattaccacttcgaagtcgttctgctataaactcatccatcagatcaggaacattagcactgctgccgccaatatcactattaagaggaggcagtttttggctcatgtcctctttattgactttggctcgttcaacagtgaatggttccaagatgtcagaagtgctgctacttcgaggcaatggctgctcctcattcaaagcaccaaaaacttcatttccagtttcttcactttgtgaaaaatgtctgactctagttgagcggggaagtatttgagcatcatcaatatctgaaagctcatcagaaaggggagtgagaacaatatcaggcaagaagggtttggaagtatggatcagaacaggagcacttttagcactgcgtatataggccgatggcagagcacattcaccaatggatcggcttctcatggcgacagttttttgccgtactatactcctcgccttttcggttcctggagaaccagtggttgttgcactcctctgtctcattggggcttggccaggctgatcacgactccatcctctagaaaatgacttgtcaactgaaactttctgaaattcatgtccaactcctttccctttgtgctttttttgtttctgttcactcagcttatccaatggtaaatcactgagatccaaactatataaattcctagctaaaactttagttaatgtctccatagtcagtgaccactcagtggccaactcttcccaataggtcagcgatgacaatactgacagtaagtcatcccaaagttctcgggagatgtacacatttaggtttgctttgatccaggcaactataagggtctggaaaagtggtcctgcaagtcgacctgccaaggtcatattttttttcccttggaactgtagaaaagcttgtgatggcatcttcagtacagattccgtgactctgagcaacacaagcagcatctgttcccaagtctttttgtccattgatacttgtacaaccatgtaccgataaatgttaagaatgcgtttacacatatctgtgtgttcatccagaagattttttatttcatttgcaggttcaagaagaaatatatttgatgagtttataataaacacctgcaaaactgcctgggtaccagctcgtatgttttgttctgtggcttcttcagaggcgttatgaagagcaccttggtaggagccgttttttgcccaactggaatttcgaacatgatcagcagtattggtcccattttcctcttctcttttttctccttcttccattgaaatatcatggtctgtgacattttcaatgcaagggaggtctgaagaagtgatcacaatttcttcaggctcttgcatgaacaaaggtttttcctcttgttggatccattcttgatatacttttaccacttttctcatagctgctgcttcacaaattggtaataaaaatgcctgacgaaatatctctgtcacaaagtttacattactccttttagaagaaaaaactctgcgaactatttcaatgtctgtgagatgttcttcatcaatactacagagactagatgagctaggttctcgctccgtgagagtgcttgtattggaatgagactgttcgggttctgtagttctgtctgttttatcagcattatcatttttgctttcttctctggatactaaactagcagctgctctctgaatattctttggcaagacttcaccttccatcccaggaatatgaggtcctgtatgtggttttggctccagccagaaagaaaccagccaacgaatgacaataacacgagccttaatgaaaggctcctttgtacaatagattgcttcattggtttcagcatctttctttatcacgacataatgtggctttggtctcatctgcgggatgtcaagtataggatgatataaactgttttccttacagatgtttggaaaaatataaggcaagtaatatttcttaaaatgtgaaaacaaaaatgaaaatcccctttcttggttttctttgttcttccattctaaactttttacctgaatgactatgtattttagaagtgcttcaagaaaatagcttgtgagatcttcttgccctttatctcctgattgtggggggacaagaggagtgatttcttctatagtgacttgagtttcttgaaggttgagtggaggattaatgagattatctaaagttcgaggtccatgttcagactgtggtgctgaaaatccagggattaagcatgaaaacatccagagctgttctttgctacagttattctgaagagcttgcaaccatagtaagaaaagacgaacaccttcccgcctaatctttaaggagtttcctgtgtgaagtagcttctttaaaatcaatccaatactatgaaactgccatcgctgatgaattctttctggaagaagttgtaaaattttctcaaaaataaaaagtatagcatccaattcctctctttgagacttgtgacctttctgtttaagactagcttcaatagtcacaaaattttcaaagaacacatagtatatatgtgaaaaatgttggtcgaaaaactgtttaagatcaatagattctgcattctcgatgacgatgcgcaggtgcttgaggcgagtcagtgcgtccttcttggtgtctagcaccttctgggtggacttcttcacgtccccgtgcggcttcttggagaacatcctgtcgctgccactgccactgccactgccacagccggctcccagccgggtcccggcggcagaaagtggagggagtggacggggaggagactagccagagaggctcattagctccccagccttgcgggccagggcagagccgactccttcccgatccaggccagggccgccacctccacccgcctcgcgccgcggctccaaggcaccttcggccccagctccaatatggcggatccctctcccggccctgcacggagcgaggcagacccgggctggccgcctgccgccgccgctcgtctccagcggccgccgctcgccgccacaggccggggccccggacccagagccacgaaggtggagctctcggcggcaggagcacaactctctccctgaggcccccttaaggttgaagcttctttagcagcttacaccctgcagaggccgaaacggagacgagtgt

SEQ ID NO: 17996 - RNA, 1521 nt, Homo sapiens
  source 1..1521: mol_type = other RNA
tctctggagggaagcactttctgaaccagtaatagttgcaacttcagcagagaaagcttgctgattaagactgcttgtttcagaatctatatgaagagtagttagactagccacttcctgctcttcagcactctgatgatggccagaacctgaatccacatcagcagaggacgtaaccccagtgtcggttccaaagccaaaattgtcaaattttcggccatcatattggaaagcgctgaaagaatccgaatgactatctgagctgataagatcactgctccctgcactggcaggagaagtccattctgagggcacacctgggtcatcaatagggcgcatctggttctgcttgtttagaatatcagggaggtctttgggaatttccaggctgcctggactacttcctcttcttgtcatagtcgaggcattaccacttcgaagtcgttctgctataaactcatccatcagatcaggaacattagcactgctgccgccaatatcactattaagaggaggcagtttttggctcatgtcctctttattgactttggctcgttcaacagtgaatggttccaagatgtcagaagtgctgctacttcgaggcaatggctgctcctcattcaaagcaccaaaaacttcatttccagtttcttcactttgtgaaaaatgtctgactctagttgagcggggaagtatttgagcatcatcaatatctgaaagctcatcagaaaggggagtgagaacaatatcaggcaagaagggtttggaagtatggatcagaacaggagcacttttagcactgcgtatataggccgatggcagagcacattcaccaatggatcggcttctcatggctgaaattaacttgtatccttctcaagataaccaatttaacatggaagtcttcaattcagtcatccaaccttgaagcttgctcaagtctcagtctgaatcccagaagtgattatcagcaatttgcttcaagatcatcccacttttccagtgtgcttactgctcatcactccattttccactcatagttttattttggtcaaggaaatgagtaagaagagtcttagaggtttctctatttgcaaaccagtggtacgacgaaatgctagcaagaatatctaatagctccagaatatcaagttcactatgttgctggcaatacgagtcatgtaatgactttttaaaaagcccctttcttcccaattttttattaagaaaattttcaaatgtagaaaaaattaaaagatggtgaggcatggtggctcatgcctataatcccagcactttgggaggccgaggagggtggatcacttgaggtcaggagttcaagaccagcctggtcaacatggtgaaaccccttctcactaaaaatacaaaaattagctaggcgtggtggtgtgcgcctatagtcccagctactctacttgggaggctgaggcaggagaatcacttgaacccaggaggcggaggttgcagtgagctgagatcgcaccactgcactccagcctg

SEQ ID NO: 17997 - RNA, 3478 nt, Homo sapiens
  source 1..3478: mol_type = other RNA
tctctggagggaagcactttctgaaccagtaatagttgcaacttcagcagagaaagcttgctgattaagactgcttgtttcagaatctatatgaagagtagttagactagccacttcctgctcttcagcactctgatgatggccagaacctgaatccacatcagcagaggacgtaaccccagtgtcggttccaaagccaaaattgtcaaattttcggccatcatattggaaagcgctgaaagaatccgaatgactatctgagctgataagatcactgctccctgcactggcaggagaagtccattctgagggcacacctgggtcatcaatagggcgcatctggttctgcttgtttagaatatcagggaggtctttgggaatttccaggctgcctggactacttcctcttcttgtcatagtcgaggcattaccacttcgaagtcgttctgctataaactcatccatcagatcaggaacattagcactgctgccgccaatatcactgcagctttccttccaaaatagcccattacatgactgtacagatccctcagtggagcctctggtggcattctgttctgcctctttggctcgttcaacagtgaatggttccaagatgtcagaagtgctgctacttcgaggcaatggctgctcctcattcaaagcaccaaaaacttcatttccagtttcttcactttgtgaaaaatgtctgactctagttgagcggggaagtatttgagcatcatcaatatcgacagttttttgccgtactatactcctcgccttttcggttcctggagaaccagtggttgttgcactcctctgtctcattggggcttggccaggctgatcacgactccatcctctagaaaatgacttgtcaactgaaactttctgaaattcatgtccaactcctttccctttgtgctttttttgtttctgttcactcagcttatccaatggtaaatcactgagatccaaactatataaattcctagctaaaactttagttaatgtctccatagtcagtgaccactcagtggccaactcttcccaataggtcagcgatgacaatactgacagtaagtcatcccaaagttctcgggagatgtacacatttaggtttgctttgatccaggcaactataagggtctggaaaagtggtcctgcaagtcgacctgccaaggtcatattttttttcccttggaactgtagaaaagcttgtgatggcatcttcagtacagattccgtgactctgagcaacacaagcagcatctgttcccaagtctttttgtccattgatacttgtacaaccatgtaccgataaatgttaagaatgcgtttacacatatctgtgtgttcatccagaagattttttatttcatttgcaggttcaagaagaaatatatttgatgagtttataataaacacctgcaaaactgcctgggtaccagctcgtatgttttgttctgtggcttcttcagaggcgttatgaagagcaccttggtaggagccgttttttgcccaactggaatttcgaacatgatcagcagtattggtcccattttcctcttctcttttttctccttcttccattgaaatatcatggtctgtgacattttcaatgcaagggaggtctgaagaagtgatcacaatttcttcaggctcttgcatgaacaaaggtttttcctcttgttggatccattcttgatatacttttaccacttttctcatagctgctgcttcacaaattggtaataaaaatgcctgacgaaatatctctgtcacaaagtttacattactccttttagaagaaaaaactctgcgaactatttcaatgtctgtgagatgttcttcatcaatactacagagactagatgagctaggttctcgctccgtgagagtgcttgtattggaatgagactgttcgggttctgtagttctgtctgttttatcagcattatcatttttgctttcttctctggatactaaactagcagctgctctctgaatattctttggcaagacttcaccttccatcccaggaatatgaggtcctgtatgtggttttggctccagccagaaagaaaccagccaacgaatgacaataacacgagccttaatgaaaggctcctttgtacaatagattgcttcattggtttcagcatctttctttatcacgacataatgtggctttggtctcatctgcgggatgtcaagtataggatgatataaactgttttccttacagatgtttggaaaaatataaggcaagtaatatttcttaaaatgtgaaaacaaaaatgaaaatcccctttcttggttttctttgttcttccattctaaactttttacctgaatgactatgtattttagaagtgcttcaagaaaatagcttgtgagatcttcttgccctttatctcctgattgtggggggacaagaggagtgatttcttctatagtgacttgagtttcttgaaggttgagtggaggattaatgagattatctaaagttcgaggtccatgttcagactgtggtgctgaaaatccagggattaagcatgaaaacatccagagctgttctttgctacagttattctgaagagcttgcaaccatagtaagaaaagacgaacaccttcccgcctaatctttaaggagtttcctgtgtgaagtagcttctttaaaatcaatccaatactatgaaactgccatcgctgatgaattctttctggaagaagttgtaaaattttctcaaaaataaaaagtatagcatccaattcctctctttgagacttgtgacctttctgtttaagactagcttcaatagtcacaaaattttcaaagaacacatagtatatatgtgaaaaatgttggtcgaaaaactgtttaagatcaatagattctgcattctcgatgacgatgcgcaggtgcttgaggcgagtcagtgcgtccttcttggtgtctagcaccttctgggtggacttcttcacgtccccgtgcggcttcttggagaacatcctgtcgctgccactgccactgccactgccacagccggctcccagccgggtcccggcggcagaaagtggagggagtggacggggaggagactagccagagaggctcattagctccccagccttgcgggccagggcagagccgactccttcccgatccaggccagggccgccacctccacccgcctcgcgccgcggctccaaggcaccttcggccccagctccaatatggcggatccctctcccggccctgcacggagcgaggcagacccgggctggccgcctgccgccgccgctcgtctccagcggccgccgctcgccgccacaggccggggccccggacccagagccacgaaggtggagctctcggcggcaggagcacaactctctccctgaggcccccttaaggttgaagcttctttagcagcttacaccctgcagaggccgaaacggagacgagtgt

SEQ ID NO: 17998 - RNA, 870 nt, Homo sapiens
  source 1..870: mol_type = other RNA
tctctgggcctgtgtcttaggctcagtgtcttgactcactgtgtgatagctcatgcttaataacagtggaataactttactataactctgagaagtaagaggtaggcaatacagagtccatattgtcatcctcattctctactaataaggaaacaggtacactgactttcccagatcaatagcaaatagcaaatctatagaaacccatatccatgaactcttaatcccctatatttgtcactccccaacctcacctaaaagtaaaaaaaatgaagttgcctaaaccctgaagctctgggtcggtagggaggatagaaatagaggctggtgttgtccaaggtttcccaaaagcaggattatgcccttacttgctccccacagtcctccctttccctgtgttgttttgacattgaacattgtttctgtttacattgattatatctgtaaatggccagtctctggaaaatgctccatttgaccaccagctccatgtaaaacctcttatccaccgagtagcatcagcttcttcctcctctagagaagggtcagtgatcagaggcagaggagcttattgtgcaggaacctactagaccccagtgagctcacagtggctactttagaaaatgccaccacaggcctcgattatatcacagaccagggaaaccctccccatgatacagagatttttgttgccagcatagtttgaggcagtcacaagaacatcgctggtccatgccggaaaccctagtgtacaattctgggccctggcctctgatagcctcactgtgcagctgagcaatgccttgatctgcttaaggaccaaagaggcagagcccagcactgtgagttctattttcaggctcagacaat

SEQ ID NO: 17999 - RNA, 4675 nt, Homo sapiens
  source 1..4675: mol_type = other RNA
tctgacatcagtgattctcctgcctcagtctccctcctgggctgggactatatacaggtgggccccaccatgcctggctgattttttgtattttttagtagagacggggtttcaccatattggccaggctggtcttgaactcctaacctcatgatccacccccatcagcctcccaaagtgctgggattacaggcaagagccaccgcgcccagcccatagaacttatttttgtcattaggatgaagaatgtgagatgatcttaaggcctagcaaagctgtgggaaatacacaggagggccaaggaagaacatgaacggaatttaaagtagaatcagaaggtaaacagatttgctgaatcacaaaggtttaatgataaatgtaggtaaatgaggaagaaaacatgataatgggatgggtttacagtcttgcaggctcaaatcaactgtgagaatcaggtaatgtgcaacctgaatccctagaaaggtgtggcttgaagtctctatggggacagcccctataaatggagactcagcccatgcctccttatgaagagaatcaccctggatatgagtgtcctagatcttatgcccagctcccagttacttgtcatatgcaacctccatacactgagagggtgacatccactagcttaggatggtaaaattgtttccttagtcaatgctacggcttcagtgtttgtgtggggggcgcctccgcccagccagccgaccagtccgggaggtggggggcgcttctgcccggccgcccctactgggaagtgaggagcccctctgcccggccaccaccacgtctgggaggtgtacccaacagctcattgagaacgggccatgatgacgatggtggttttgcggaatagaaaagggggaaatgtggggaaaagatagagaaatcacattgttgctgtgtctgtgtagaaagaagtagacatgggagacttcactttgttctgtactaagaaaaattcttctgccttgggatgctgttgatctatgatcttacccccaaccctgtgctctctgaaacatgtgctgtgtccactcagggttaaatggattaagggcggtgcaagatgtactttgttaaacagatgcttgaaggcagcatgctcgttaagagtcatcaccactccctaatctcaagtacccagggacacaaacactgcggaaggccgcagggtcctctgcctaggaaaaccagagacctttgttcacttgtttatctgctgaccttccctccactattgtcctatgaccctgccaaatccccctctgcgagaaacacccaagaatgatcaataaaaataaaaaaataaaaaataaaaaataaaagaaatatacagcatcctgagatgatacaagttagagatgagaaatagcattgctagaaaatgaagataattacagttaagacagaagaagtaagacctggtgttcaatagatcagtagggtaactagagttaatactaatctactgtacatttcaaaatagctagaagagagtaatttgaatgttactagcataaaggtaaatgtttaaggtgatggatatcccaattacactgattgattatatgaatatatcaaattaccacatataccctgacaatatttacatctattatgtatcaataagtttttttttaagaatcaaaaaaaggaaagaaagtgtagatattctaagagaggacactgtgcattatagaattatagttccttttcaaattaaatccacccatctctgtgcctaatggctggcttatggccaggaggggtgtcatccaaaataacagacagcatctgaagaaaaaacgtgaagttgggtttgtgttcctttccctagtacgctgattctgacatactagtgtacaggagaataaactagaatgtttaataaaactaaaattcctgggccctccttcctgagactctgattcagtaggtctggggtggggtcagcaacctggattaataacagggatcacactgaactctgatacagctcttctgtatggcagtgcttctcatactgtaatgtgcatacaaatctcctggagaccttgctaaaatgcagattctgattcaacacgcctgggacaggacaaaacctaggattctgcctttttttttttttttttctgagacaggatcttcagtccaagctgaagtgcagtggcactatcatagctcactgtaaccttgaactcccaggctcaagcaatcatcataccttagcctcccgaataactgagactacaggtgcgtgccaccatgccctactaactttttgaaatttttctgtagagacaaggtcttgccatattgcctaggctggtctcaaactcctggcctcaagcgaccgtcccaccacagcaactcaaaagcgttgggattacaggtgtgagccactgtgcccagcccgggttctgcatttctaacaagccccaagatgatcccaatgctggtgatctatggaccacacttggagtagctcactgttgaccgttttgggataaaaagattctgatgcaggcagaaagggcaggtggagaacttaccttcaacactgatatacctttctctctgtaaggagacgggcattccctcatcaaacagcgtttttactgacatccctgtcccaaatatagatcaggaggctgaagtccagtgaaacacaatgaccaaccctgggtcacctaggatggtggtatgttggcttcaccacaaattgtgggagttttaaatcacactgtactggtgggatttgccaacactaaaccaaatgttcatctgggtcttggctgcaattttaagaacttcattagaaggtcataattcctaagtgctggcactgctggcatagaagctgaagcatctcctttgcatgtgaagagaatctatctccacctatgtgtctgaaataatccagatgtggtactaagggcatcgggctggcctcagatagctcagatccaagaagactgtggaattactgcaaggggtttgagaatctatggacaatgtttttctatatatgtactactatttttaaaaggcatatggacattattaaaataaattttaaaaacaccttcagtgtaaacacattcaggttaggggatactgtatgctctctcatttaatggaaattaaaaaacaatcacatatcacttggggtctttacaatactttgacattaaaaagggtccttgtcttctagaacgtatgctagaagtggtttgtcataggaaaattcaaactctctggcatttcagagaataaatagtatatatatcattattaaatatgtttaacaaaaatcatgctcaagttctaagtgactacatttctcattttgtaaatcaaggaagaaaatactgcagaattcaacctgaaatgttttaatagtggaactgtgtacaggatcctctaaagagaccgcctggctgggtgctcaaaccacatgggccgacccaaaagacgccaaaaccaagagctgctcaggaggcactaaatgttgacggtcttggccggcttcacatcctcaatttcagcagacagccagcggtaagtgcgatgacgccgcagcacctcaatggccttgagttccagtggtgttgcctgaataccaaggtcttctaagccaggcaggtgaggcaatttcatgtctgtgatgtgcatccgctccactttatcccttgttatccagggctcaaatgggcttatttcaaagactcttgctacccatcgataggcaaaaagcggcaaggggaatgggaggaacaatctgtgagccacagcaaagatgtacttcaccaggtggaaaaggaggtaccgactgggaccaacgaaagcaaaggatttcccattggcatcaggatccttaactgcattaacaattcctttggatacatctacgacatatactggttgtttaactgtcttccagcccaaggaaccaaggggtataggaccaaaccgatgcatacttgcaaaagaattaaggaatctatcctctcttccaaagatgtccgacggctttacgataatggcttccggaaatgcatctctcactactttctctccaacagccttatttctcaaatatctagaagagcttttaatattcgcattcagatgtgaaacatgaatgaatttttcaactccagcttccttggacagttgagcaattgcttggggaatcttcacaaaaacatcctcaaaatcaaagtttttggtttcccagtctcgtccaataagattgatgaccacattgctgtgttgtactactcgtcggatagaatctttatctctcgcgtcccattccagaaacagaagctggcccaggtcacccatgggacgaaggtgcatgatgtcatatttatcacaccgatagggtatgattacctgtgaccccatgcgtccaaggtggttgacaacatatcgccccaggaatcctgttgctccaaacacagtggccacaatcccactgactgaggaacgtccacctttcccatgaggcatgagggcatgatgaagctggcgacagggtgggccgtgacacacagatgtggctattgcagtaatggcagaacgtgacattgacaggacccggacaacccgggattgtgcggcagccgccatcttttcccacaat

SEQ ID NO: 18000 - RNA, 1166 nt, Homo sapiens
  source 1..1166: mol_type = other RNA
tctgaggcctgcctctccccaccaacctcccagctggatgagacctcttcagcccctgggaacccggtctcgctgcccagcttccccagccaagctgggcactaggaagtgctcaaaaggacctcactgatgctgaacaggtaggtcatgatggcattggtgtagttgtagctgctgttggtggccagaaacactttcccaacctccttcatcttccccagcaggatggggaggcgtggatccttcttcacatatttctccaagtcctccagggtcttcttgagacagcccgactggtggatgttattcatggcatcagtcacatcctggaagaggcttcggaaggacatgaagaggttcccatgctgatagccggtgtcacaattagtgtaacgggagcagccagagaagaagtccaccaagcaggcatagaggtaggtttcaggcaggttgaagagcatgttgagtatgtagaaacactgcaggtcgtccctctgaatgaacttgctggggtagaagctccagatctctgccctgaggaggggtaggtccgagaggaaggtgaagccataggcacccagcagcacattcccgtgggcgtccaccttcagcaggttcccatagagttcatcgaacaccagccgcctggtggggaaggtggggtcgtaggtgtagcgcaggatctcatgcgggtacccaatgcacaccaggcgctccagcagcagctcgaaggtcagggcctcataagctggggacttgtaggcagccagagtgtagtccatgtcgaagccaaagcaacgaatcttccccagcgccaggctgcggttgacaaaaatcctggggagagagaggaggatgttggcatcagtccaccagccccccagaatccaaggcccaaggacagagggggtggaaaccccgcagaggagggcagagcaccccctgcagctgcagaaagcacaggggaagcaggtcaggccaagccagggccctgcctggacccatgtgtgtctgaaggcaagtgtgagtgtgcatgtaagcatgtgtgagcatgtgtgcaagcgtgcatctgagtgtgtgcgggcaatcagccgcttgctgtcccaccatgcaggcatgttataggcatccaaccctgtaagaaagtaggtgcagttgttggtgtg

SEQ ID NO: 18001 - RNA, 760 nt, Homo sapiens
  source 1..760: mol_type = other RNA
tctgaggcctgcctctccccacccttggtttggagatgagtctctcttggtccccatctccttccagagttttcgtgggggtctctctgcacccatcagcaacatccgtgtcctccttctccttgccctgtgggccgtgctgggcatcgctggaagcccactcttcatcctgtggggcagggagctgccgtctgattttgaactgaaccttgtacggctctgaatattgaaggattttgagagcatcttcatattttatgttttcaaagaacacggttgtactgagcagctgatccccttctctcaagttaaaaagcttggcggctgaggagtccttcagcacttgcttgacgaagatcccctggtccccaccacctgtgacactgtagccactggctcctgcctccacctctgtcttcagcgtcacctctgttgcctcctggacagcctctggacgactcatcctgaaaaatgtccgtgagtcccctgaatctcgcttccaccaggatctccgtctcccagcagaaccttgcctgccgggggcgtcttcctggagtccaaagtcggcagcctcagtcgtgtattcgtagacaggtgaagacccctgcggccgtggtcgaatgccctcatccgcaggcccttcagtcacagagtggtcatcttccgtttctgcacctggctccccgggctgcagctgacggccggacacaaggaagctacagacgctctcccaactggcccagaagcgaagatcccaact

SEQ ID NO: 18002 - RNA, 900 nt, Homo sapiens
  source 1..900: mol_type = other RNA
tctgaggcctgcctctccccacccttggtttggagatgagtctctcttggtccccatctccttccagagttttcgtgggggtctctctgcacccatcagcaacatccgtgtcctccttctccttgccctgtgggccgtgctgggcatcgctggaagcccactcttcatcctgtggggcagggagctgccgtctgattttgaactgaaccttgtacggctctgaatattgaaggattttgagagcatcttcatattttatgttttcaaagaacacggttgtactgagcagctgatccccttctctcaagttaaaaagcttggcggctgaggagtccttcagcacttgcttgacgaagatcccctggtccccaccacctgtgacactgtagccactggctcctgcctccacctctgtcttcagcgtcacctctgttgcctcctggacagcctctggacgactcatcctgaaaaatgtccgtgagtcccctgaatctcgcttccaccaggatctccgtctcccagcagaaccttgcctgccgggggcgtcttcctggagtccaaagtcggcagcctcagtcgtgtattcgtagacaggtgaagacccctgcggccgtggtcgaatgccctcatccgcaggcccttcagtcacagagtggtcatcttccgtttctgcacctggctccccgggctgcagctgacggccggacacgctgccgggggttccgggccaggtgggcagcaccatgtggaagcagtcgcacatcgcggcggccaggcggtgcgggcctggcggcccgtcgcgtccagtcgctggtcccggctccggcgcacggggcgggcgggcgggagccgcgctctgccccgctgccctgcgctgccgcgggcggccgacctcggact

SEQ ID NO: 18003 - RNA, 910 nt, Homo sapiens
  source 1..910: mol_type = other RNA
tctgaggcctgcctctccccacccttggtttggagatgagtctctcttggtccccatctccttccagagttttcgtgggggtctctctgcacccatcagcaacatccgtgtcctccttctccttgccctgtgggccgtgctgggcatcgctggaagcccactcttcatcctgtggggcagggagctgccgtctgattttgaactgaaccttgtacggctctgaatattgaaggattttgagagcatcttcatattttatgttttcaaagaacacggttgtactgagcagctgatccccttctctcaagttaaaaagcttggcggctgaggagtccttcagcacttgcttgacgaagatcccctggtccccaccacctgtgacactgtagccactggctcctgcctccacctctgtcttcagcgtcacctctgttgcctcctggacagcctctggacgactcatcctgaaaaatgtccgtgagtcccctgaatctcgcttccaccaggatctccgtctcccagcagaaccttgcctgccgggggcgtcttcctggagtccaaagtcggcagcctcagtcgtgtattcgtagacaggtgaagacccctgcggccgtggtcgaatgccctcatccgcaggcccttcagtcacagagtggtcatcttccgtttctgcacctggctccccgggctgcagctgacggccggacacgcttcacgggcctttccttgcccttctgcaagatggctcacagcccaggtcccctctggctctgctctcaggcctggcagggctggaggatggtgtctcctggaggaggttctctcaagcgaaggaagagaagggcaggaggtgagggcaggcagggctgggtcagtgccaggaggcatcaacactcacccccacgtcatc

SEQ ID NO: 18004 - RNA, 125 nt, Homo sapiens
  source 1..125: mol_type = other RNA
tctgaggtggaacagcagcaacaggagaagaagagagagacagagaaaggggtaggggatgaacaccccaactcaaaatttagaagaaaagagtcagaagaaacgttgtatgtgtttttcagttt

SEQ ID NO: 18005 - RNA, 876 nt, Homo sapiens
  source 1..876: mol_type = other RNA
tctgaggtggaacagcagcaacaggagaagaagagagagacagagaaaggggtaggggatgaacaccccaactcaaaatttagaagaaaagagtcagaagaaacgttgtatgtgtttttcagtttcccctttattctattaaatctcttgggttgtagctttcacaaataagtatgtattttaaacgaagaagacaatcgtataaaatttatatttttaatataaatgtactataaggatttcttccttcctggaaactccggactggctttaatgcctctaggtctctggtaggtaagcaccgtccccgtgaggctaagaagttcaaatttaaaggatgatgggccaaacaagacaaagcattcttgtgtttaacctctgttgagaagaaattatttacctgctagctactagttcccaggcatttgggctcaattacccaggaaacttctttcagagagggcctgcactcatccattctggtagcaaacaagtcagtgtgacatcgttcaaggtgctcgtgtgctcccagaccaatttcacatctcattgcttagttggacggaatttgattgtacatgctccctggactctctaacctggtgcagagaatcaaccagttctgaagcaaaacttggtttcattaaatggtgcatagtggaatgcagagtgaaaccactggaaataaaatctgggtaaaatgtctctatttataagtcagcctgctcttagtggggaggaagagaggatgttcactcttaagcccagtggcaccagccatcacctgatgtttactgtcacccaaagtagaaattcttatttcacacttgaaatatggaaatatggatctcaacagtaaaactgagaaccatatct

SEQ ID NO: 18006 - RNA, 9217 nt, Homo sapiens
  source 1..9217: mol_type = other RNA
tctgagttcctggagcctggtctacttttccagtctaattttctatcacccgccactacatacacaccctgtactccagttataccattctatgtgaagtccctgaacaaggcaagctgaaaacacaaatggcagaaatatttgaacaatttcctgggcttattaagggatagccagggtgacggcagcagagccatggcaggcaaccatgctcttcttatattaaataagactcagacatatataccattagggatccttgactcattatctttctgatcaatacttccacaaaatattcattcctttggccacacattttgcctgtgggctaggagttaaacattccctctccagacttattcaaggagctaattgtcttctacccagactatggaaatggtctcctaacctcttccccattgggtccactctctacactgaagctaaaattgcctttctaaaatgcaaatctgattatttaaaaagaaaattctttaatggcttgccattgcttgcagcgatttctaagcagagggtaccccctccctgccccacctcaccccagggagtaaacatatggaatatggggggcatatcagagccatctcagggatttttcaaagtttcacatacacacaggtatatgtggcatcatcaacacccctcacccatgtcccttttgctcccatacacatttcctatcccatgaaaatcgctgccatgcttgttgagtgatgggtgttatgttgtagccctcagttatgctgaggcataaaaatggttgagcagcctcatggcagaataaagtccagattccttagcatgtcctacaaagtcctgcacaatagcctccctgcttgccttttcagtttcatcttcacccattctccatcacacaccctgtgggccaacaccaccagtctggagaattcctgaaccaggtttgctttttcgtacttttttctttattctattccatttacccagaatgcacttctcctctcacacagctagtaaatttctgtttaacctttaagaaggcaccaacaattacatcttcagccacagcctgcccctggattccaggctggtacatctccacttggatttttagaaagtatcttaaacttaacatggctaaaacaacctcctggacccgcttcctactacttattcctcctgcagtcagccacatctcagttcattgcaactgactccccaactcataatccaagtctttgctgcagtctgtgagagcatgtatgatctgatcctattcctatcaccctcccctcccccactctgctctagccacactggcctcctagtcctaaatacaccaaacacatactgagctcagggccttcgaactgctgttctatctggaatgctcctctctcttagatgtccctgtgattcattcccttatttctttcaagtgtctgatcataagtaatcacatcagaaaccactgtttatgggacagtaccaattcaccatcaccttacatcccctccccttgctttattctccacagtacttaccactacttgacatcctgcactattactgttattatttgctcccactagaacataaactatacaagggccagcttttattattcctattctctaccatatcttcagttcctaaaacaatacttggcatatagtagatgctctgtaaacatgttattgtcattcgttatttgttaactcaactgaaaagtgctgtgggacttccatttaaacatactgcactcaatatataaatttccttcagttccttcctaaaaccccattaaattaacagcaaatagattttcaaaatgacacagagaatggaagtggagacatcaataaagcctaacctgatcaccacatttaaaattatggcctcctcttcccagtctccttaccctgacttttccttccatagcacctattatcttccaataagtataaagaatgggtaagagagctaaagcttcattagtaggcagttttagaccttattgtaaacaagtacacaatatatgtaacagccaaaagaattagaaattggttacttctgggaagtacaaactaagaatgagaggggaagggacagataatttattgttttgttttttaaataaggcttctagtactatactttttcaatcatgtatgttcataatttatgccaaataaaacttcaattaaaaaaatcccaaaaccaagagggaaactgtatatgcaagaagaaaagtcataatgcaactttgtctatttttattcttcacatagtgactatgtcttgtttaacagaatttgaacatattaaaatagatgaccaaatactaaatatttagactatgtagtggaacacatgatttatatcagtcatttcttgaaaacttatgagtacttcattgacattacatgcataaagcaaatatctagctgaaacattgctgaaaaaaaaatacgtcattttgccagtaaattaaataaactgcagaaagaaactacttctcaacatgaaagtaaagagaagagaatcaaggcaatgggctttgccacagacagggaatacacagcgaacagggaaaggatcaggccccccttgcttgaggcttgctttcctcatctgtagatttaggggtctcaatcaggtcatctcaagttccctaaacttgcttaaaaagcatcaaactttgagttagaccttcagacttccctaactccttttttcctgaattaagctatgacaaagatgaccatatgtcccagttcacctagtataatctcgatttatatctgttgtcctggaataacaattaattgctcctcctttaactctcaaaggtatctccagtcggaagataaattacatgcccctcatacctatgactatattcattttaatcttggtttagatttttaagaaaacacactaatttacttttaagcctacaaatatagcatttcatagcttgctttctcttaacacttggagaaatttcagattcttttgtgagtggtttgtgaactatcaaaaatttttttaacttggccgggcatgatgacctatgcctctaatcccagtactttggaaggctgaggcagaagaatcgcttaagatgggaagtttgcggctgcagtgagctacgatcacgccactacacttcagcctgggtgatgcagaaaggaccgtgtctctagaaataaaaataattttttaaaaactgagtaagtcaaatgtaaattttccttttcaaaaacaaattattcagtatgcaaaacattctgttaagacatattttctgataaccttagaatacgtggtacttaaaaactatgactaaaatatttgtggaagaattcattatcttaggtgatacattttaacaattaaaatagttccagaacacggtcttccacctgactttgacgattaaaacaatgttgtcaaaagaatgttctctctgaaaattctgggtctcatccaccaccataggtctcatctaccatcaactgaaataagctaatcagttataaacaagggaatatacttaaaaaaaaaaaaaagagagaaacacggtctcactctgtctccaaggctggagtgcagtggcacagtcatagctcactgcagcacagaactcctaagctcaggcaatactcccacctcagcttcccaggaatataccacttttactgcactgacaagctctgtatgctagtgattctcaaattttctttaaggctaggaccaagagtcctgccaatcccctgaacaacagctcacatattatcaaatgaacttgaaacattcctgtcatagtgagcagcattgaaacagattccataactgattactcagtttcaagggagatttaacattgctttgttttcaagttacaaaaagttccctagttttactcaaatatgcactatccctgattaaaaaaaacatgtttcattatgaagaggggtgatttgtttcagcatttttttttttcacttaaccacttaagtcactgcctgaggaagtttctttttaaggaaataaataccaggttcattagaagaaaaaaaaaaaacacataattttaattcattttgttttaaagatgcgtattttaaaaagactactttaaaatgaactaatatgttacactggatcatgctgtggcgactaacgtattgtcaagccttaacctaatgaaaacaaaagaaaagcgagtttggcactcacttgcacttttcatctctgttagaaagtatgtctcagtttggatctgagatcaggtttgcttggtaacctcaaagaataattttccttttttttttctttcaaaatttccttttgatcatttcagacagttcatccttttgagtgagaaagagtaaaagagaggaatgttgagtgaggttaagtaaatggagaatctgtcacataaagcaagtttaaatcctagtaagagcatccatgcaggacaaacggaagcattattcttttgaaaacattattcttttaaacagtgtgtaatgacatcctccctagagactttccatgagaggggaaaaaaattacttcctcagaagtcgttttctagattccaagcataataagtgaagcacagttaaaagtcaaacttgtgttttctttatgcaagaaggttcaaattagaactgcagaaaggtacttaaaagtttctctagcttgtcttttggttacatactggtattgctgtgaactaaaagagcaagtaagaggaaaggttactgttgttactttacacctataaatcagtgagtgtgtccttactgtaaaatttgagctgaacatattttgtttcaaaggagaaatatatgactcaaatatgctgaatgtatgataatttattaagttccttttaagtatatcattttcttatgctcaagtagaaactatggattatttttctagtattctatgctgctgttaccttctgaggagttgattgaaaattttatgcttttaaaagttgggtgctacttaaatatcagaattggctattgttttaaatatttaaaatatgcttaaacaacaattaaggttaataagcagagaaaatacttcttttgattcaaacactactttatatatttaatgaatacacgtccaaataaagatctctcttcaaaaattttggaaaatgttaatgcattttgaatataatggaacaaagaagaagaatactagagaaaattcacaattatgatgtttatttaggaaaataaacttgaagaaggttttctattaaaaaaacataagaatcatatccaaattttagactctccatcttctttggtatgaaaatcaacattcataatagaaaatattttcttttgaaaggtttagttgttattgggtctataacggttttccatataaggaaaatacagtattatctgtaatcatctcacttattgaacaaccaatgaatgcatgcaagtaaccaagcatatgtgtgcagagaccagcatcaaggaaatattcattcatagataaatgttttctaataaaatatattttaagtttttaatgatcttctgctatcattttttgccatgttatctgaatagccatccagatctgtagtaaaacatcctgttagttacataactcaagaagtacttccccaaggaagctcacaccatcataccaggacttagcaacatttatctttcaacatgagtataccattaaaatttttttatatttctcagaattgtattcttcagtcttttccacaatatagtatatggaaattgctaatagcattaaattaatattaataaaacccaattctatctaaacctttttctcataagaaaaaacattactttaaaaaatagactttttgtttcttctaaaagtagtactatatggactgctcaattagcaatgccaaatacttccaaaaacaccataggaccaccaagctatttctattgctttgataatttcttttcctgctccaatttctccacgttcctgctttcttgtgtcaaaatatcttcccttaatttgttaaaatgaatctgagggaaaaaaatctgataatctggggtaaagaaatttttttttttgcatagactcttgtgatcacaaaatgaccaggtaatttatagcttcagtgctaacactgtgattgggaacaagaagagtacaaccataataaaatacagctatctatgagaagaactgcataaagacatctttggccatgtaggctctgggccctctggaaataagtcagttgcattgccaacatgacaaagaaaatagcaatgttcagaatcaggaacaacctggtataggaagcagacagtgatggggccctgctgtgtgtagttgtcaccatccgtgcctgtccaaaccggcctttaatcaagcccccatttttatgtttctcgtatgttacatctgcaaaatctaaaaggtctttcatttcttcatcttcatctatgggtagttctttctgtgccaaaatctgagctttctgtctaatctttttctcattgacttcaatctgtgcaaaaatatcagggacagcatccacaaatttatagcgtttgcctgcccttcggtttttctttgacttgctttgctgctgctgttgctgtgatatggcaaaaatcctgtcaatggcctcctcagtctgtctcttatctgaaaatctcagcaggcgttcagcagtcttcctaaagctagctgtgttccggactcgggacagtatctgcttctccagcagctgaaacactggtttaaaatgctgcaagttctgttccacaatagcagcatagtccttcacctcagggacaatgctgctcttgatggctgaattccggtcaaacagaattttgtgacgatcagcaatgacctgtgcaaaggcagactgtcctgtggcctcacctgtccacaggtatgtggcgtaggcatgtttgctggtggctatgaacacatccagttgctgagagtctccgtggacagtgaagctctgaacatctatagatggccctatgaagaggtaagctgccctggtgatgggacttcggaggtgcatggtgacattcacatagtttgtcccattgtagggatagccccgaggatatgtcactgaggcaaaggttgctttctcgctgtagccagtatcgtccatccagtacattttatagagaccatctctctgcctgatgaaagccccatggacaccatctaccacagtctcctcaaaaggaacatccacattatggaagaagctcgctgctgtctccaagggactctcctctcccaggtgtatttggtctacaaggagaagcagctgtggatgtaggaggatgagattcctctgaacattcttcaggttgagctgggggttataagctcccacaccttctcctcggatgaaaaccaccccatttttctcctctgctgcaaccaccctcccctgacaactagctgccaggtcatgcttgtatttagaccattttgatgagcagtcttctgtgacctgacccacccagggagaaaagcagctctttgacacagctggggaaaacatcaaaacattgttgaagaaggtgtactttggcccgtacagagcctcagtaatgaaaggcacaccattgggagcaaaagtaaatgagttttgatcaggatgttcatgccctgcattaaaatttctccatcctttgatccaatctttgtatttgtttctgtggacaatgtcatatattgcacgtccccccagttttccagacttgaaggaaaggaaagatctattgatttctgcaggtagtgcacttccataagtcacgacaccccagtcttcaaaataatgcagtgtaggggtgccaaagtctggaggaggaaccgatttcaagctgccatcataccagagaaattctgtgtgcagagtgcaccagcgctgccctttggatggtgttcctggaccttccaccacacggttccttctgatttggtcagctagccagttaccactgccattacgcatgacaaatttatcaaggaacactaattggctttctggaccataaaaccagttgtaatttgagtccgcaatagccacagtcctttgaaaccctggcaggatggttctatacataaatgcaaagtgttgtttaagccacggatggccaaagtggttgatgttgaagtgcctctggacgagaaacatgtattggaagagtgatctagtggtgtagctgccatacgcaactccttcatagagggagccatccgtcacctccctgagcaagaccagagatttctccatgatggtcagaacttgtttggtccataagtaggcttcttgaagatatccttgattcatcaggactaggcttcccgtgagcaaagccatacagttggtgggctgatgattgtgcaggtattgaaatccccatcctctcctgtatgaagtttcatacatataccctgaggcattggcaatcacttcaagaaacttctcctgttgtgtcttgctcaggtagttgtacaagaagtcataagcagtggcaaaaccaaccagggagtgagcaagcgggacctcatcccaaggagcatctttcaccaaccaactaggctgcgctgccatcctctccatgtagtctttggccatgtctcgggcttcaatgttctcaggatacagcacacagaacattgccaaggcacccaagttgtttccaaaaatttcattccagcgggcactgtagtccttgggatcccagggagggaggtattccaaggggctggacagcatcgtgtgcacagcctccgtgaggcgggctgcaatgtgctcgtgcgagctggcagccctgagctgcagctccgccacttctgccctggagaagtacagcatgggatggctgtcgtagttggcattggtgaagggaatcataacttctgggttctcgtcggtgatgtaggctgacacaaagcaaagcaaatatatgaaaaacacactgggagccccccgtgtgtgagtcctcatcgtggcatcagatctccaaatctccaaggcagccaaaccatcttcgaaagatcccattcattagaatgagagatattttactgggagcagtgcttttctccatgagttctgaagggcacctccatccaattcctctatcctcagaggttctcacttctattt

SEQ ID NO: 18007 - RNA, 9283 nt, Homo sapiens
  source 1..9283: mol_type = other RNA
tctgagttcctggagcctggtctacttttccagtctaattttctatcacccgccactacatacacaccctgtactccagttataccattctatgtgaagtccctgaacaaggcaagctgaaaacacaaatggcagaaatatttgaacaatttcctgggcttattaagggatagccagggtgacggcagcagagccatggcaggcaaccatgctcttcttatattaaataagactcagacatatataccattagggatccttgactcattatctttctgatcaatacttccacaaaatattcattcctttggccacacattttgcctgtgggctaggagttaaacattccctctccagacttattcaaggagctaattgtcttctacccagactatggaaatggtctcctaacctcttccccattgggtccactctctacactgaagctaaaattgcctttctaaaatgcaaatctgattatttaaaaagaaaattctttaatggcttgccattgcttgcagcgatttctaagcagagggtaccccctccctgccccacctcaccccagggagtaaacatatggaatatggggggcatatcagagccatctcagggatttttcaaagtttcacatacacacaggtatatgtggcatcatcaacacccctcacccatgtcccttttgctcccatacacatttcctatcccatgaaaatcgctgccatgcttgttgagtgatgggtgttatgttgtagccctcagttatgctgaggcataaaaatggttgagcagcctcatggcagaataaagtccagattccttagcatgtcctacaaagtcctgcacaatagcctccctgcttgccttttcagtttcatcttcacccattctccatcacacaccctgtgggccaacaccaccagtctggagaattcctgaaccaggtttgctttttcgtacttttttctttattctattccatttacccagaatgcacttctcctctcacacagctagtaaatttctgtttaacctttaagaaggcaccaacaattacatcttcagccacagcctgcccctggattccaggctggtacatctccacttggatttttagaaagtatcttaaacttaacatggctaaaacaacctcctggacccgcttcctactacttattcctcctgcagtcagccacatctcagttcattgcaactgactccccaactcataatccaagtctttgctgcagtctgtgagagcatgtatgatctgatcctattcctatcaccctcccctcccccactctgctctagccacactggcctcctagtcctaaatacaccaaacacatactgagctcagggccttcgaactgctgttctatctggaatgctcctctctcttagatgtccctgtgattcattcccttatttctttcaagtgtctgatcataagtaatcacatcagaaaccactgtttatgggacagtaccaattcaccatcaccttacatcccctccccttgctttattctccacagtacttaccactacttgacatcctgcactattactgttattatttgctcccactagaacataaactatacaagggccagcttttattattcctattctctaccatatcttcagttcctaaaacaatacttggcatatagtagatgctctgtaaacatgttattgtcattcgttatttgttaactcaactgaaaagtgctgtgggacttccatttaaacatactgcactcaatatataaatttccttcagttccttcctaaaaccccattaaattaacagcaaatagattttcaaaatgacacagagaatggaagtggagacatcaataaagcctaacctgatcaccacatttaaaattatggcctcctcttcccagtctccttaccctgacttttccttccatagcacctattatcttccaataagtataaagaatgggtaagagagctaaagcttcattagtaggcagttttagaccttattgtaaacaagtacacaatatatgtaacagccaaaagaattagaaattggttacttctgggaagtacaaactaagaatgagaggggaagggacagataatttattgttttgttttttaaataaggcttctagtactatactttttcaatcatgtatgttcataatttatgccaaataaaacttcaattaaaaaaatcccaaaaccaagagggaaactgtatatgcaagaagaaaagtcataatgcaactttgtctatttttattcttcacatagtgactatgtcttgtttaacagaatttgaacatattaaaatagatgaccaaatactaaatatttagactatgtagtggaacacatgatttatatcagtcatttcttgaaaacttatgagtacttcattgacattacatgcataaagcaaatatctagctgaaacattgctgaaaaaaaaatacgtcattttgccagtaaattaaataaactgcagaaagaaactacttctcaacatgaaagtaaagagaagagaatcaaggcaatgggctttgccacagacagggaatacacagcgaacagggaaaggatcaggccccccttgcttgaggcttgctttcctcatctgtagatttaggggtctcaatcaggtcatctcaagttccctaaacttgcttaaaaagcatcaaactttgagttagaccttcagacttccctaactccttttttcctgaattaagctatgacaaagatgaccatatgtcccagttcacctagtataatctcgatttatatctgttgtcctggaataacaattaattgctcctcctttaactctcaaaggtatctccagtcggaagataaattacatgcccctcatacctatgactatattcattttaatcttggtttagatttttaagaaaacacactaatttacttttaagcctacaaatatagcatttcatagcttgctttctcttaacacttggagaaatttcagattcttttgtgagtggtttgtgaactatcaaaaatttttttaacttggccgggcatgatgacctatgcctctaatcccagtactttggaaggctgaggcagaagaatcgcttaagatgggaagtttgcggctgcagtgagctacgatcacgccactacacttcagcctgggtgatgcagaaaggaccgtgtctctagaaataaaaataattttttaaaaactgagtaagtcaaatgtaaattttccttttcaaaaacaaattattcagtatgcaaaacattctgttaagacatattttctgataaccttagaatacgtggtacttaaaaactatgactaaaatatttgtggaagaattcattatcttaggtgatacattttaacaattaaaatagttccagaacacggtcttccacctgactttgacgattaaaacaatgttgtcaaaagaatgttctctctgaaaattctgggtctcatccaccaccataggtctcatctaccatcaactgaaataagctaatcagttataaacaagggaatatacttaaaaaaaaaaaaaagagagaaacacggtctcactctgtctccaaggctggagtgcagtggcacagtcatagctcactgcagcacagaactcctaagctcaggcaatactcccacctcagcttcccaggaatataccacttttactgcactgacaagctctgtatgctagtgattctcaaattttctttaaggctaggaccaagagtcctgccaatcccctgaacaacagctcacatattatcaaatgaacttgaaacattcctgtcatagtgagcagcattgaaacagattccataactgattactcagtttcaagggagatttaacattgctttgttttcaagttacaaaaagttccctagttttactcaaatatgcactatccctgattaaaaaaaacatgtttcattatgaagaggggtgatttgtttcagcatttttttttttcacttaaccacttaagtcactgcctgaggaagtttctttttaaggaaataaataccaggttcattagaagaaaaaaaaaaaacacataattttaattcattttgttttaaagatgcgtattttaaaaagactactttaaaatgaactaatatgttacactggatcatgctgtggcgactaacgtattgtcaagccttaacctaatgaaaacaaaagaaaagcgagtttggcactcacttgcacttttcatctctgttagaaagtatgtctcagtttggatctgagatcaggtttgcttggtaacctcaaagaataattttccttttttttttctttcaaaatttccttttgatcatttcagacagttcatccttttgagtgagaaagagtaaaagagaggaatgttgagtgaggttaagtaaatggagaatctgtcacataaagcaagtttaaatcctagtaagagcatccatgcaggacaaacggaagcattattcttttgaaaacattattcttttaaacagtgtgtaatgacatcctccctagagactttccatgagaggggaaaaaaattacttcctcagaagtcgttttctagattccaagcataataagtgaagcacagttaaaagtcaaacttgtgttttctttatgcaagaaggttcaaattagaactgcagaaaggtacttaaaagtttctctagcttgtcttttggttacatactggtattgctgtgaactaaaagagcaagtaagaggaaaggttactgttgttactttacacctataaatcagtgagtgtgtccttactgtaaaatttgagctgaacatattttgtttcaaaggagaaatatatgactcaaatatgctgaatgtatgataatttattaagttccttttaagtatatcattttcttatgctcaagtagaaactatggattatttttctagtattctatgctgctgttaccttctgaggagttgattgaaaattttatgcttttaaaagttgggtgctacttaaatatcagaattggctattgttttaaatatttaaaatatgcttaaacaacaattaaggttaataagcagagaaaatacttcttttgattcaaacactactttatatatttaatgaatacacgtccaaataaagatctctcttcaaaaattttggaaaatgttaatgcattttgaatataatggaacaaagaagaagaatactagagaaaattcacaattatgatgtttatttaggaaaataaacttgaagaaggttttctattaaaaaaacataagaatcatatccaaattttagactctccatcttctttggtatgaaaatcaacattcataatagaaaatattttcttttgaaaggtttagttgttattgggtctataacggttttccatataaggaaaatacagtattatctgtaatcatctcacttattgaacaaccaatgaatgcatgcaagtaaccaagcatatgtgtgcagagaccagcatcaaggaaatattcattcatagataaatgttttctaataaaatatattttaagtttttaatgatcttctgctatcattttttgccatgttatctgaatagccatccagatctgtagtaaaacatcctgttagttacataactcaagaagtacttccccaaggaagctcacaccatcataccaggacttagcaacatttatctttcaacatgagtataccattaaaatttttttatatttctcagaattgtattcttcagtcttttccacaatatagtatatggaaattgctaatagcattaaattaatattaataaaacccaattctatctaaacctttttctcataagaaaaaacattactttaaaaaatagactttttgtttcttctaaaagtagtactatatggactgctcaattagcaatgccaaatacttccaaaaacaccataggaccaccaagctatttctattgctttgataatttcttttcctgctccaatttctccacgttcctgctttcttgtgtcaaaatatcttcccttaatttgttaaaatgaatctgagggaaaaaaatctgataatctggggtaaagaaatttttttttttgcatagactcttgtgatcacaaaatgaccaggtaatttatagcttcagtgctaacactgtgattgggaacaagaagagtacaaccataataaaatacagctatctatgagaagaactgcataaagacatctttggccatgtaggctctgggccctctggaaataagtcagttgcattgccaacatgacaaagaaaatagcaatgttcagaatcaggaacaacctggtataggaagcagacagtgatggggccctgctgtgtgtagttgtcaccatccgtgcctgtccaaaccggcctttaatcaagcccccatttttatgtttctcgtatgttacatctgcaaaatctaaaaggtctttcatttcttcatcttcatctatgggtagttctttctgtgccaaaatctgagctttctgtctaatctttttctcattgacttcaatctgtgcaaaaatatcagggacagcatccacaaatttatagcgtttgcctgcccttcggtttttctttgacttgctttgctgctgctgttgctgtgatatggcaaaaatcctgtcaatggcctcctcagtctgtctcttatctgaaaatctcagcaggcgttcagcagtcttcctaaagctagctgtgttccggactcgggacagtatctgcttctccagcagctgaaacactggtttaaaatgctgcaagttctgttccacaatagcagcatagtccttcacctcagggacaatgctgctcttgatggctgaattccggtcaaacagaattttgtgacgatcagcaatgacctgtgcaaaggcagactgtcctgtggcctcacctgtccacaggtatgtggcgtaggcatgtttgctggtggctatgaacacatccagttgctgagagtctccgtggacagtgaagctctgaacatctatagatggccctatgaagaggtaagctgccctggtgatgggacttcggaggtgcatggtgacattcacatagtttgtcccattgtagggatagccccgaggatatgtcactgaggcaaaggttgctttctcgctgtagccagtatcgtccatccagtacattttatagagaccatctctctgcctgatgaaagccccatggacaccatctaccacagtctcctcaaaaggaacatccacattatggaagaagctcgctgctgtctccaagggactctcctctcccaggtgtatttggtctacaaggagaagcagctgtggatgtaggaggatgagattcctctgaacattcttcaggttgagctgggggttataagctcccacaccttctcctcggatgaaaaccaccccatttttctcctctgctgcaaccaccctcccctgacaactagctgccaggtcatgcttgtatttagaccattttgatgagcagtcttctgtgacctgacccacccagggagaaaagcagctctttgacacagctggggaaaacatcaaaacattgttgaagaaggtgtactttggcccgtacagagcctcagtaatgaaaggcacaccattgggagcaaaagtaaatgagttttgatcaggatgttcatgccctgcattaaaatttctccatcctttgatccaatctttgtatttgtttctgtggacaatgtcatatattgcacgtccccccagttttccagacttgaaggaaaggaaagatctattgatttctgcaggtagtgcacttccataagtcacgacaccccagtcttcaaaataatgcagtgtaggggtgccaaagtctggaggaggaaccgatttcaagctgccatcataccagagaaattctgtgtgcagagtgcaccagcgctgccctttggatggtgttcctggaccttccaccacacggttccttctgatttggtcagctagccagttaccactgccattacgcatgacaaatttatcaaggaacactaattggctttctggaccataaaaccagttgtaatttgagtccgcaatagccacagtcctttgaaaccctggcaggatggttctatacataaatgcaaagtgttgtttaagccacggatggccaaagtggttgatgttgaagtgcctctggacgagaaacatgtattggaagagtgatctagtggtgtagctgccatacgcaactccttcatagagggagccatccgtcacctccctgagcaagaccagagatttctccatgatggtcagaacttgtttggtccataagtaggcttcttgaagatatccttgattcatcaggactaggcttcccgtgagcaaagccatacagttggtgggctgatgattgtgcaggtattgaaatccccatcctctcctgtatgaagtttcatacatataccctgaggcattggcaatcacttcaagaaacttctcctgttgtgtcttgctcaggtagttgtacaagaagtcataagcagtggcaaaaccaaccagggagtgagcaagcgggacctcatcccaaggagcatctttcaccaaccaactaggctgcgctgccatcctctccatgtagtctttggccatgtctcgggcttcaatgttctcaggatacagcacacagaacattgccaaggcacccaagttgtttccaaaaatttcattccagcgggcactgtagtccttgggatcccagggagggaggtattccaaggggctggacagcatcgtgtgcacagcctccgtgaggcgggctgcaatgtgctcgtgcgagctggcagccctgagctgcagctccgccacttctgccctggagaagtacagcatgggatggctgtcgtagttggcattggtgaagggaatcataacttctgggttctcgtcggtgatgtaggctgacacaaagcaaagcaaatatatgaaaaacacactgggagccccccgtgtgtgagtcctcatcgtggcatcagatctccaaatctccaaggcagccaaaccatcttcgaaagatccgctcccagccgaggcttcgttctctccggcgtcgcctccgcagcctccagagccagctcccggtcctcctcactccagggcgcccgggctcccggccccctccgaaccgagccctccgcgcccccgccgcgccatgccccgggatgcgctgctgcagcctcgggcgacgctact

SEQ ID NO: 18008 - RNA, 9755 nt, Homo sapiens
  source 1..9755: mol_type = other RNA
tctgagttcctggagcctggtctacttttccagtctaattttctatcacccgccactacatacacaccctgtactccagttataccattctatgtgaagtccctgaacaaggcaagctgaaaacacaaatggcagaaatatttgaacaatttcctgggcttattaagggatagccagggtgacggcagcagagccatggcaggcaaccatgctcttcttatattaaataagactcagacatatataccattagggatccttgactcattatctttctgatcaatacttccacaaaatattcattcctttggccacacattttgcctgtgggctaggagttaaacattccctctccagacttattcaaggagctaattgtcttctacccagactatggaaatggtctcctaacctcttccccattgggtccactctctacactgaagctaaaattgcctttctaaaatgcaaatctgattatttaaaaagaaaattctttaatggcttgccattgcttgcagcgatttctaagcagagggtaccccctccctgccccacctcaccccagggagtaaacatatggaatatggggggcatatcagagccatctcagggatttttcaaagtttcacatacacacaggtatatgtggcatcatcaacacccctcacccatgtcccttttgctcccatacacatttcctatcccatgaaaatcgctgccatgcttgttgagtgatgggtgttatgttgtagccctcagttatgctgaggcataaaaatggttgagcagcctcatggcagaataaagtccagattccttagcatgtcctacaaagtcctgcacaatagcctccctgcttgccttttcagtttcatcttcacccattctccatcacacaccctgtgggccaacaccaccagtctggagaattcctgaaccaggtttgctttttcgtacttttttctttattctattccatttacccagaatgcacttctcctctcacacagctagtaaatttctgtttaacctttaagaaggcaccaacaattacatcttcagccacagcctgcccctggattccaggctggtacatctccacttggatttttagaaagtatcttaaacttaacatggctaaaacaacctcctggacccgcttcctactacttattcctcctgcagtcagccacatctcagttcattgcaactgactccccaactcataatccaagtctttgctgcagtctgtgagagcatgtatgatctgatcctattcctatcaccctcccctcccccactctgctctagccacactggcctcctagtcctaaatacaccaaacacatactgagctcagggccttcgaactgctgttctatctggaatgctcctctctcttagatgtccctgtgattcattcccttatttctttcaagtgtctgatcataagtaatcacatcagaaaccactgtttatgggacagtaccaattcaccatcaccttacatcccctccccttgctttattctccacagtacttaccactacttgacatcctgcactattactgttattatttgctcccactagaacataaactatacaagggccagcttttattattcctattctctaccatatcttcagttcctaaaacaatacttggcatatagtagatgctctgtaaacatgttattgtcattcgttatttgttaactcaactgaaaagtgctgtgggacttccatttaaacatactgcactcaatatataaatttccttcagttccttcctaaaaccccattaaattaacagcaaatagattttcaaaatgacacagagaatggaagtggagacatcaataaagcctaacctgatcaccacatttaaaattatggcctcctcttcccagtctccttaccctgacttttccttccatagcacctattatcttccaataagtataaagaatgggtaagagagctaaagcttcattagtaggcagttttagaccttattgtaaacaagtacacaatatatgtaacagccaaaagaattagaaattggttacttctgggaagtacaaactaagaatgagaggggaagggacagataatttattgttttgttttttaaataaggcttctagtactatactttttcaatcatgtatgttcataatttatgccaaataaaacttcaattaaaaaaatcccaaaaccaagagggaaactgtatatgcaagaagaaaagtcataatgcaactttgtctatttttattcttcacatagtgactatgtcttgtttaacagaatttgaacatattaaaatagatgaccaaatactaaatatttagactatgtagtggaacacatgatttatatcagtcatttcttgaaaacttatgagtacttcattgacattacatgcataaagcaaatatctagctgaaacattgctgaaaaaaaaatacgtcattttgccagtaaattaaataaactgcagaaagaaactacttctcaacatgaaagtaaagagaagagaatcaaggcaatgggctttgccacagacagggaatacacagcgaacagggaaaggatcaggccccccttgcttgaggcttgctttcctcatctgtagatttaggggtctcaatcaggtcatctcaagttccctaaacttgcttaaaaagcatcaaactttgagttagaccttcagacttccctaactccttttttcctgaattaagctatgacaaagatgaccatatgtcccagttcacctagtataatctcgatttatatctgttgtcctggaataacaattaattgctcctcctttaactctcaaaggtatctccagtcggaagataaattacatgcccctcatacctatgactatattcattttaatcttggtttagatttttaagaaaacacactaatttacttttaagcctacaaatatagcatttcatagcttgctttctcttaacacttggagaaatttcagattcttttgtgagtggtttgtgaactatcaaaaatttttttaacttggccgggcatgatgacctatgcctctaatcccagtactttggaaggctgaggcagaagaatcgcttaagatgggaagtttgcggctgcagtgagctacgatcacgccactacacttcagcctgggtgatgcagaaaggaccgtgtctctagaaataaaaataattttttaaaaactgagtaagtcaaatgtaaattttccttttcaaaaacaaattattcagtatgcaaaacattctgttaagacatattttctgataaccttagaatacgtggtacttaaaaactatgactaaaatatttgtggaagaattcattatcttaggtgatacattttaacaattaaaatagttccagaacacggtcttccacctgactttgacgattaaaacaatgttgtcaaaagaatgttctctctgaaaattctgggtctcatccaccaccataggtctcatctaccatcaactgaaataagctaatcagttataaacaagggaatatacttaaaaaaaaaaaaaagagagaaacacggtctcactctgtctccaaggctggagtgcagtggcacagtcatagctcactgcagcacagaactcctaagctcaggcaatactcccacctcagcttcccaggaatataccacttttactgcactgacaagctctgtatgctagtgattctcaaattttctttaaggctaggaccaagagtcctgccaatcccctgaacaacagctcacatattatcaaatgaacttgaaacattcctgtcatagtgagcagcattgaaacagattccataactgattactcagtttcaagggagatttaacattgctttgttttcaagttacaaaaagttccctagttttactcaaatatgcactatccctgattaaaaaaaacatgtttcattatgaagaggggtgatttgtttcagcatttttttttttcacttaaccacttaagtcactgcctgaggaagtttctttttaaggaaataaataccaggttcattagaagaaaaaaaaaaaacacataattttaattcattttgttttaaagatgcgtattttaaaaagactactttaaaatgaactaatatgttacactggatcatgctgtggcgactaacgtattgtcaagccttaacctaatgaaaacaaaagaaaagcgagtttggcactcacttgcacttttcatctctgttagaaagtatgtctcagtttggatctgagatcaggtttgcttggtaacctcaaagaataattttccttttttttttctttcaaaatttccttttgatcatttcagacagttcatccttttgagtgagaaagagtaaaagagaggaatgttgagtgaggttaagtaaatggagaatctgtcacataaagcaagtttaaatcctagtaagagcatccatgcaggacaaacggaagcattattcttttgaaaacattattcttttaaacagtgtgtaatgacatcctccctagagactttccatgagaggggaaaaaaattacttcctcagaagtcgttttctagattccaagcataataagtgaagcacagttaaaagtcaaacttgtgttttctttatgcaagaaggttcaaattagaactgcagaaaggtacttaaaagtttctctagcttgtcttttggttacatactggtattgctgtgaactaaaagagcaagtaagaggaaaggttactgttgttactttacacctataaatcagtgagtgtgtccttactgtaaaatttgagctgaacatattttgtttcaaaggagaaatatatgactcaaatatgctgaatgtatgataatttattaagttccttttaagtatatcattttcttatgctcaagtagaaactatggattatttttctagtattctatgctgctgttaccttctgaggagttgattgaaaattttatgcttttaaaagttgggtgctacttaaatatcagaattggctattgttttaaatatttaaaatatgcttaaacaacaattaaggttaataagcagagaaaatacttcttttgattcaaacactactttatatatttaatgaatacacgtccaaataaagatctctcttcaaaaattttggaaaatgttaatgcattttgaatataatggaacaaagaagaagaatactagagaaaattcacaattatgatgtttatttaggaaaataaacttgaagaaggttttctattaaaaaaacataagaatcatatccaaattttagactctccatcttctttggtatgaaaatcaacattcataatagaaaatattttcttttgaaaggtttagttgttattgggtctataacggttttccatataaggaaaatacagtattatctgtaatcatctcacttattgaacaaccaatgaatgcatgcaagtaaccaagcatatgtgtgcagagaccagcatcaaggaaatattcattcatagataaatgttttctaataaaatatattttaagtttttaatgatcttctgctatcattttttgccatgttatctgaatagccatccagatctgtagtaaaacatcctgttagttacataactcaagaagtacttccccaaggaagctcacaccatcataccaggacttagcaacatttatctttcaacatgagtataccattaaaatttttttatatttctcagaattgtattcttcagtcttttccacaatatagtatatggaaattgctaatagcattaaattaatattaataaaacccaattctatctaaacctttttctcataagaaaaaacattactttaaaaaatagactttttgtttcttctaaaagtagtactatatggactgctcaattagcaatgccaaatacttccaaaaacaccataggaccaccaagctatttctattgctttgataatttcttttcctgctccaatttctccacgttcctgctttcttgtgtcaaaatatcttcccttaatttgttaaaatgaatctgagggaaaaaaatctgataatctggggtaaagaaatttttttttttgcatagactcttgtgatcacaaaatgaccaggtaatttatagcttcagtgctaacactgtgattgggaacaagaagagtacaaccataataaaatacagctatctatgagaagaactgcataaagacatctttggccatgtaggctctgggccctctggaaataagtcagttgcattgccaacatgacaaagaaaatagcaatgttcagaatcaggaacaacctggtataggaagcagacagtgatggggccctgctgtgtgtagttgtcaccatccgtgcctgtccaaaccggcctttaatcaagcccccatttttatgtttctcgtatgttacatctgcaaaatctaaaaggtctttcatttcttcatcttcatctatgggtagttctttctgtgccaaaatctgagctttctgtctaatctttttctcattgacttcaatctgtgcaaaaatatcagggacagcatccacaaatttatagcgtttgcctgcccttcggtttttctttgacttgctttgctgctgctgttgctgtgatatggcaaaaatcctgtcaatggcctcctcagtctgtctcttatctgaaaatctcagcaggcgttcagcagtcttcctaaagctagctgtgttccggactcgggacagtatctgcttctccagcagctgaaacactggtttaaaatgctgcaagttctgttccacaatagcagcatagtccttcacctcagggacaatgctgctcttgatggctgaattccggtcaaacagaattttgtgacgatcagcaatgacctgtgcaaaggcagactgtcctgtggcctcacctgtccacaggtatgtggcgtaggcatgtttgctggtggctatgaacacatccagttgctgagagtctccgtggacagtgaagctctgaacatctatagatggccctatgaagaggtaagctgccctggtgatgggacttcggaggtgcatggtgacattcacatagtttgtcccattgtagggatagccccgaggatatgtcactgaggcaaaggttgctttctcgctgtagccagtatcgtccatccagtacattttatagagaccatctctctgcctgatgaaagccccatggacaccatctaccacagtctcctcaaaaggaacatccacattatggaagaagctcgctgctgtctccaagggactctcctctcccaggtgtatttggtctacaaggagaagcagctgtggatgtaggaggatgagattcctctgaacattcttcaggttgagctgggggttataagctcccacaccttctcctcggatgaaaaccaccccatttttctcctctgctgcaaccaccctcccctgacaactagctgccaggtcatgcttgtatttagaccattttgatgagcagtcttctgtgacctgacccacccagggagaaaagcagctctttgacacagctggggaaaacatcaaaacattgttgaagaaggtgtactttggcccgtacagagcctcagtaatgaaaggcacaccattgggagcaaaagtaaatgagttttgatcaggatgttcatgccctgcattaaaatttctccatcctttgatccaatctttgtatttgtttctgtggacaatgtcatatattgcacgtccccccagttttccagacttgaaggaaaggaaagatctattgatttctgcaggtagtgcacttccataagtcacgacaccccagtcttcaaaataatgcagtgtaggggtgccaaagtctggaggaggaaccgatttcaagctgccatcataccagagaaattctgtgtgcagagtgcaccagcgctgccctttggatggtgttcctggaccttccaccacacggttccttctgatttggtcagctagccagttaccactgccattacgcatgacaaatttatcaaggaacactaattggctttctggaccataaaaccagttgtaatttgagtccgcaatagccacagtcctttgaaaccctggcaggatggttctatacataaatgcaaagtgttgtttaagccacggatggccaaagtggttgatgttgaagtgcctctggacgagaaacatgtattggaagagtgatctagtggtgtagctgccatacgcaactccttcatagagggagccatccgtcacctccctgagcaagaccagagatttctccatgatggtcagaacttgtttggtccataagtaggcttcttgaagatatccttgattcatcaggactaggcttcccgtgagcaaagccatacagttggtgggctgatgattgtgcaggtattgaaatccccatcctctcctgtatgaagtttcatacatataccctgaggcattggcaatcacttcaagaaacttctcctgttgtgtcttgctcaggtagttgtacaagaagtcataagcagtggcaaaaccaaccagggagtgagcaagcgggacctcatcccaaggagcatctttcaccaaccaactaggctgcgctgccatcctctccatgtagtctttggccatgtctcgggcttcaatgttctcaggatacagcacacagaacattgccaaggcacccaagttgtttccaaaaatttcattccagcgggcactgtagtccttgggatcccagggagggaggtattccaaggggctggacagcatcgtgtgcacagcctccgtgaggcgggctgcaatgtgctcgtgcgagctggcagccctgagctgcagctccgccacttctgccctggagaagtacagcatgggatggctgtcgtagttggcattggtgaagggaatcataacttctgggttctcgtcggtgatgtaggctgacacaaagcaaagcaaatatatgaaaaacacactgggagccccccgtgtgtgagtcctcatcgtggcatcagatctccaaatctccaaggcagccaaaccatcttcgaaagatcctcacagtgcagggtggtatgccgccaaatgcttccacaaagctcagtgtcccattgtggagcgccttactaactccatgatgatgcacggctgcaacaacggcaagaagctcatgactgtgtgcatcgtcaagcatgccttcgaggtcatacacctgctcacaggcgagaaccctctgcaggtcctggtgaacgccatcatcaacagtggtccccgggaggactccacacgcattgggtgcgccgggactgtgagacgacaggctgtggacgtgtccccacttcgccgtgtgaatcaggccatctggctgctgtgcacaggtgctcgtgaggctgccttccggaacattaagaccattgctgagtgcctggcagaggagctcatcaatgctgccaagggctcctccaactcctatgccattaagaagaaggacgtgtggccttcttggagcatgtggccaagtccaaccgctgattttcccagctgttgcccaataaacctgtctgcccttcagggcagccatgcttgagtctggtctacatccatttacgtaagtaaaactccccttccagactgacgaaattctttttgtgacaagaagacaaaggaatacgatggattgataagcgtagtcaaccgcgcagag

SEQ ID NO: 18009 - RNA, 9843 nt, Homo sapiens
  source 1..9843: mol_type = other RNA
tctgagttcctggagcctggtctacttttccagtctaattttctatcacccgccactacatacacaccctgtactccagttataccattctatgtgaagtccctgaacaaggcaagctgaaaacacaaatggcagaaatatttgaacaatttcctgggcttattaagggatagccagggtgacggcagcagagccatggcaggcaaccatgctcttcttatattaaataagactcagacatatataccattagggatccttgactcattatctttctgatcaatacttccacaaaatattcattcctttggccacacattttgcctgtgggctaggagttaaacattccctctccagacttattcaaggagctaattgtcttctacccagactatggaaatggtctcctaacctcttccccattgggtccactctctacactgaagctaaaattgcctttctaaaatgcaaatctgattatttaaaaagaaaattctttaatggcttgccattgcttgcagcgatttctaagcagagggtaccccctccctgccccacctcaccccagggagtaaacatatggaatatggggggcatatcagagccatctcagggatttttcaaagtttcacatacacacaggtatatgtggcatcatcaacacccctcacccatgtcccttttgctcccatacacatttcctatcccatgaaaatcgctgccatgcttgttgagtgatgggtgttatgttgtagccctcagttatgctgaggcataaaaatggttgagcagcctcatggcagaataaagtccagattccttagcatgtcctacaaagtcctgcacaatagcctccctgcttgccttttcagtttcatcttcacccattctccatcacacaccctgtgggccaacaccaccagtctggagaattcctgaaccaggtttgctttttcgtacttttttctttattctattccatttacccagaatgcacttctcctctcacacagctagtaaatttctgtttaacctttaagaaggcaccaacaattacatcttcagccacagcctgcccctggattccaggctggtacatctccacttggatttttagaaagtatcttaaacttaacatggctaaaacaacctcctggacccgcttcctactacttattcctcctgcagtcagccacatctcagttcattgcaactgactccccaactcataatccaagtctttgctgcagtctgtgagagcatgtatgatctgatcctattcctatcaccctcccctcccccactctgctctagccacactggcctcctagtcctaaatacaccaaacacatactgagctcagggccttcgaactgctgttctatctggaatgctcctctctcttagatgtccctgtgattcattcccttatttctttcaagtgtctgatcataagtaatcacatcagaaaccactgtttatgggacagtaccaattcaccatcaccttacatcccctccccttgctttattctccacagtacttaccactacttgacatcctgcactattactgttattatttgctcccactagaacataaactatacaagggccagcttttattattcctattctctaccatatcttcagttcctaaaacaatacttggcatatagtagatgctctgtaaacatgttattgtcattcgttatttgttaactcaactgaaaagtgctgtgggacttccatttaaacatactgcactcaatatataaatttccttcagttccttcctaaaaccccattaaattaacagcaaatagattttcaaaatgacacagagaatggaagtggagacatcaataaagcctaacctgatcaccacatttaaaattatggcctcctcttcccagtctccttaccctgacttttccttccatagcacctattatcttccaataagtataaagaatgggtaagagagctaaagcttcattagtaggcagttttagaccttattgtaaacaagtacacaatatatgtaacagccaaaagaattagaaattggttacttctgggaagtacaaactaagaatgagaggggaagggacagataatttattgttttgttttttaaataaggcttctagtactatactttttcaatcatgtatgttcataatttatgccaaataaaacttcaattaaaaaaatcccaaaaccaagagggaaactgtatatgcaagaagaaaagtcataatgcaactttgtctatttttattcttcacatagtgactatgtcttgtttaacagaatttgaacatattaaaatagatgaccaaatactaaatatttagactatgtagtggaacacatgatttatatcagtcatttcttgaaaacttatgagtacttcattgacattacatgcataaagcaaatatctagctgaaacattgctgaaaaaaaaatacgtcattttgccagtaaattaaataaactgcagaaagaaactacttctcaacatgaaagtaaagagaagagaatcaaggcaatgggctttgccacagacagggaatacacagcgaacagggaaaggatcaggccccccttgcttgaggcttgctttcctcatctgtagatttaggggtctcaatcaggtcatctcaagttccctaaacttgcttaaaaagcatcaaactttgagttagaccttcagacttccctaactccttttttcctgaattaagctatgacaaagatgaccatatgtcccagttcacctagtataatctcgatttatatctgttgtcctggaataacaattaattgctcctcctttaactctcaaaggtatctccagtcggaagataaattacatgcccctcatacctatgactatattcattttaatcttggtttagatttttaagaaaacacactaatttacttttaagcctacaaatatagcatttcatagcttgctttctcttaacacttggagaaatttcagattcttttgtgagtggtttgtgaactatcaaaaatttttttaacttggccgggcatgatgacctatgcctctaatcccagtactttggaaggctgaggcagaagaatcgcttaagatgggaagtttgcggctgcagtgagctacgatcacgccactacacttcagcctgggtgatgcagaaaggaccgtgtctctagaaataaaaataattttttaaaaactgagtaagtcaaatgtaaattttccttttcaaaaacaaattattcagtatgcaaaacattctgttaagacatattttctgataaccttagaatacgtggtacttaaaaactatgactaaaatatttgtggaagaattcattatcttaggtgatacattttaacaattaaaatagttccagaacacggtcttccacctgactttgacgattaaaacaatgttgtcaaaagaatgttctctctgaaaattctgggtctcatccaccaccataggtctcatctaccatcaactgaaataagctaatcagttataaacaagggaatatacttaaaaaaaaaaaaaagagagaaacacggtctcactctgtctccaaggctggagtgcagtggcacagtcatagctcactgcagcacagaactcctaagctcaggcaatactcccacctcagcttcccaggaatataccacttttactgcactgacaagctctgtatgctagtgattctcaaattttctttaaggctaggaccaagagtcctgccaatcccctgaacaacagctcacatattatcaaatgaacttgaaacattcctgtcatagtgagcagcattgaaacagattccataactgattactcagtttcaagggagatttaacattgctttgttttcaagttacaaaaagttccctagttttactcaaatatgcactatccctgattaaaaaaaacatgtttcattatgaagaggggtgatttgtttcagcatttttttttttcacttaaccacttaagtcactgcctgaggaagtttctttttaaggaaataaataccaggttcattagaagaaaaaaaaaaaacacataattttaattcattttgttttaaagatgcgtattttaaaaagactactttaaaatgaactaatatgttacactggatcatgctgtggcgactaacgtattgtcaagccttaacctaatgaaaacaaaagaaaagcgagtttggcactcacttgcacttttcatctctgttagaaagtatgtctcagtttggatctgagatcaggtttgcttggtaacctcaaagaataattttccttttttttttctttcaaaatttccttttgatcatttcagacagttcatccttttgagtgagaaagagtaaaagagaggaatgttgagtgaggttaagtaaatggagaatctgtcacataaagcaagtttaaatcctagtaagagcatccatgcaggacaaacggaagcattattcttttgaaaacattattcttttaaacagtgtgtaatgacatcctccctagagactttccatgagaggggaaaaaaattacttcctcagaagtcgttttctagattccaagcataataagtgaagcacagttaaaagtcaaacttgtgttttctttatgcaagaaggttcaaattagaactgcagaaaggtacttaaaagtttctctagcttgtcttttggttacatactggtattgctgtgaactaaaagagcaagtaagaggaaaggttactgttgttactttacacctataaatcagtgagtgtgtccttactgtaaaatttgagctgaacatattttgtttcaaaggagaaatatatgactcaaatatgctgaatgtatgataatttattaagttccttttaagtatatcattttcttatgctcaagtagaaactatggattatttttctagtattctatgctgctgttaccttctgaggagttgattgaaaattttatgcttttaaaagttgggtgctacttaaatatcagaattggctattgttttaaatatttaaaatatgcttaaacaacaattaaggttaataagcagagaaaatacttcttttgattcaaacactactttatatatttaatgaatacacgtccaaataaagatctctcttcaaaaattttggaaaatgttaatgcattttgaatataatggaacaaagaagaagaatactagagaaaattcacaattatgatgtttatttaggaaaataaacttgaagaaggttttctattaaaaaaacataagaatcatatccaaattttagactctccatcttctttggtatgaaaatcaacattcataatagaaaatattttcttttgaaaggtttagttgttattgggtctataacggttttccatataaggaaaatacagtattatctgtaatcatctcacttattgaacaaccaatgaatgcatgcaagtaaccaagcatatgtgtgcagagaccagcatcaaggaaatattcattcatagataaatgttttctaataaaatatattttaagtttttaatgatcttctgctatcattttttgccatgttatctgaatagccatccagatctgtagtaaaacatcctgttagttacataactcaagaagtacttccccaaggaagctcacaccatcataccaggacttagcaacatttatctttcaacatgagtataccattaaaatttttttatatttctcagaattgtattcttcagtcttttccacaatatagtatatggaaattgctaatagcattaaattaatattaataaaacccaattctatctaaacctttttctcataagaaaaaacattactttaaaaaatagactttttgtttcttctaaaagtagtactatatggactgctcaattagcaatgccaaatacttccaaaaacaccataggaccaccaagctatttctattgctttgataatttcttttcctgctccaatttctccacgttcctgctttcttgtgtcaaaatatcttcccttaatttgttaaaatgaatctgagggaaaaaaatctgataatctggggtaaagaaatttttttttttgcatagactcttgtgatcacaaaatgaccaggtaatttatagcttcagtgctaacactgtgattgggaacaagaagagtacaaccataataaaatacagctatctatgagaagaactgcataaagacatctttggccatgtaggctctgggccctctggaaataagtcagttgcattgccaacatgacaaagaaaatagcaatgttcagaatcaggaacaacctggtataggaagcagacagtgatggggccctgctgtgtgtagttgtcaccatccgtgcctgtccaaaccggcctttaatcaagcccccatttttatgtttctcgtatgttacatctgcaaaatctaaaaggtctttcatttcttcatcttcatctatgggtagttctttctgtgccaaaatctgagctttctgtctaatctttttctcattgacttcaatctgtgcaaaaatatcagggacagcatccacaaatttatagcgtttgcctgcccttcggtttttctttgacttgctttgctgctgctgttgctgtgatatggcaaaaatcctgtcaatggcctcctcagtctgtctcttatctgaaaatctcagcaggcgttcagcagtcttcctaaagctagctgtgttccggactcgggacagtatctgcttctccagcagctgaaacactggtttaaaatgctgcaagttctgttccacaatagcagcatagtccttcacctcagggacaatgctgctcttgatggctgaattccggtcaaacagaattttgtgacgatcagcaatgacctgtgcaaaggcagactgtcctgtggcctcacctgtccacaggtatgtggcgtaggcatgtttgctggtggctatgaacacatccagttgctgagagtctccgtggacagtgaagctctgaacatctatagatggccctatgaagaggtaagctgccctggtgatgggacttcggaggtgcatggtgacattcacatagtttgtcccattgtagggatagccccgaggatatgtcactgaggcaaaggttgctttctcgctgtagccagtatcgtccatccagtacattttatagagaccatctctctgcctgatgaaagccccatggacaccatctaccacagtctcctcaaaaggaacatccacattatggaagaagctcgctgctgtctccaagggactctcctctcccaggtgtatttggtctacaaggagaagcagctgtggatgtaggaggatgagattcctctgaacattcttcaggttgagctgggggttataagctcccacaccttctcctcggatgaaaaccaccccatttttctcctctgctgcaaccaccctcccctgacaactagctgccaggtcatgcttgtatttagaccattttgatgagcagtcttctgtgacctgacccacccagggagaaaagcagctctttgacacagctggggaaaacatcaaaacattgttgaagaaggtgtactttggcccgtacagagcctcagtaatgaaaggcacaccattgggagcaaaagtaaatgagttttgatcaggatgttcatgccctgcattaaaatttctccatcctttgatccaatctttgtatttgtttctgtggacaatgtcatatattgcacgtccccccagttttccagacttgaaggaaaggaaagatctattgatttctgcaggtagtgcacttccataagtcacgacaccccagtcttcaaaataatgcagtgtaggggtgccaaagtctggaggaggaaccgatttcaagctgccatcataccagagaaattctgtgtgcagagtgcaccagcgctgccctttggatggtgttcctggaccttccaccacacggttccttctgatttggtcagctagccagttaccactgccattacgcatgacaaatttatcaaggaacactaattggctttctggaccataaaaccagttgtaatttgagtccgcaatagccacagtcctttgaaaccctggcaggatggttctatacataaatgcaaagtgttgtttaagccacggatggccaaagtggttgatgttgaagtgcctctggacgagaaacatgtattggaagagtgatctagtggtgtagctgccatacgcaactccttcatagagggagccatccgtcacctccctgagcaagaccagagatttctccatgatggtcagaacttgtttggtccataagtaggcttcttgaagatatccttgattcatcaggactaggcttcccgtgagcaaagccatacagttggtgggctgatgattgtgcaggtattgaaatccccatcctctcctgtatgaagtttcatacatataccctgaggcattggcaatcacttcaagaaacttctcctgttgtgtcttgctcaggtagttgtacaagaagtcataagcagtggcaaaaccaaccagggagtgagcaagcgggacctcatcccaaggagcatctttcaccaaccaactaggctgcgctgccatcctctccatgtagtctttggccatgtctcgggcttcaatgttctcaggatacagcacacagaacattgccaaggcacccaagttgtttccaaaaatttcattccagcgggcactgtagtccttgggatcccagggagggaggtattccaaggggctggacagcatcgtgtgcacagcctccgtgaggcgggctgcaatgtgctcgtgcgagctggcagccctgagctgcagctccgccacttctgccctggagaagtacagcatgggatggctgtcgtagttggcattggtgaagggaatcataacttctgggttctcgtcggtgatgtaggctgacacaaagcaaagcaaatatatgaaaaacacactgggagccccccgtgtgtgagtcctcatcgtggcatcagatctccaaatctccaaggcagccaaaccatcttcgaaagatcctcacagtgcagggtggtatgccgccaaatgcttccacaaagctcagtgtcccattgtggagcgccttactaactccatgatgatgcacggctgcaacaacggcaagaagctcatgactgtgtgcatcgtcaagcatgccttcgaggtcatacacctgctcacaggcgagaaccctctgcaggtcctggtgaacgccatcatcaacagtggtccccgggaggactccacacgcattgggtgcgccgggactgtgagacgacaggctgtggacgtgtccccacttcgccgtgtgaatcaggccatctggctgctgtgcacaggtgctcgtgaggctgccttccggaacattaagaccattgctgagtgcctggcagaggagctcatcaatgctgccaagggctcctccaactcctatgccattaagaagaaggacgtgtggccttcttggagcatgtggccaagtccaaccgctgattttcccagctgttgcccaataaacctgtctgcccttcagggcagcccttaaagtaaatattttcagaaacaataggttaggtgccttagaaattcattcagaggcttagaaatccacattaacacagttcttacatgcttgagtctggtctacatccatttacgtaagtaaaactccccttccagactgacgaaattctttttgtgacaagaagacaaaggaatacgatggattgataagcgtagtcaaccgcgcagag

SEQ ID NO: 18010 - RNA, 9283 nt, Homo sapiens
  source 1..9283: mol_type = other RNA
tctgagttcctggagcctggtctacttttccagtctaattttctatcacccgccactacatacacaccctgtactccagttataccattctatgtgaagtccctgaacaaggcaagctgaaaacacaaatggcagaaatatttgaacaatttcctgggcttattaagggatagccagggtgacggcagcagagccatggcaggcaaccatgctcttcttatattaaataagactcagacatatataccattagggatccttgactcattatctttctgatcaatacttccacaaaatattcattcctttggccacacattttgcctgtgggctaggagttaaacattccctctccagacttattcaaggagctaattgtcttctacccagactatggaaatggtctcctaacctcttccccattgggtccactctctacactgaagctaaaattgcctttctaaaatgcaaatctgattatttaaaaagaaaattctttaatggcttgccattgcttgcagcgatttctaagcagagggtaccccctccctgccccacctcaccccagggagtaaacatatggaatatggggggcatatcagagccatctcagggatttttcaaagtttcacatacacacaggtatatgtggcatcatcaacacccctcacccatgtcccttttgctcccatacacatttcctatcccatgaaaatcgctgccatgcttgttgagtgatgggtgttatgttgtagccctcagttatgctgaggcataaaaatggttgagcagcctcatggcagaataaagtccagattccttagcatgtcctacaaagtcctgcacaatagcctccctgcttgccttttcagtttcatcttcacccattctccatcacacaccctgtgggccaacaccaccagtctggagaattcctgaaccaggtttgctttttcgtacttttttctttattctattccatttacccagaatgcacttctcctctcacacagctagtaaatttctgtttaacctttaagaaggcaccaacaattacatcttcagccacagcctgcccctggattccaggctggtacatctccacttggatttttagaaagtatcttaaacttaacatggctaaaacaacctcctggacccgcttcctactacttattcctcctgcagtcagccacatctcagttcattgcaactgactccccaactcataatccaagtctttgctgcagtctgtgagagcatgtatgatctgatcctattcctatcaccctcccctcccccactctgctctagccacactggcctcctagtcctaaatacaccaaacacatactgagctcagggccttcgaactgctgttctatctggaatgctcctctctcttagatgtccctgtgattcattcccttatttctttcaagtgtctgatcataagtaatcacatcagaaaccactgtttatgggacagtaccaattcaccatcaccttacatcccctccccttgctttattctccacagtacttaccactacttgacatcctgcactattactgttattatttgctcccactagaacataaactatacaagggccagcttttattattcctattctctaccatatcttcagttcctaaaacaatacttggcatatagtagatgctctgtaaacatgttattgtcattcgttatttgttaactcaactgaaaagtgctgtgggacttccatttaaacatactgcactcaatatataaatttccttcagttccttcctaaaaccccattaaattaacagcaaatagattttcaaaatgacacagagaatggaagtggagacatcaataaagcctaacctgatcaccacatttaaaattatggcctcctcttcccagtctccttaccctgacttttccttccatagcacctattatcttccaataagtataaagaatgggtaagagagctaaagcttcattagtaggcagttttagaccttattgtaaacaagtacacaatatatgtaacagccaaaagaattagaaattggttacttctgggaagtacaaactaagaatgagaggggaagggacagataatttattgttttgttttttaaataaggcttctagtactatactttttcaatcatgtatgttcataatttatgccaaataaaacttcaattaaaaaaatcccaaaaccaagagggaaactgtatatgcaagaagaaaagtcataatgcaactttgtctatttttattcttcacatagtgactatgtcttgtttaacagaatttgaacatattaaaatagatgaccaaatactaaatatttagactatgtagtggaacacatgatttatatcagtcatttcttgaaaacttatgagtacttcattgacattacatgcataaagcaaatatctagctgaaacattgctgaaaaaaaaatacgtcattttgccagtaaattaaataaactgcagaaagaaactacttctcaacatgaaagtaaagagaagagaatcaaggcaatgggctttgccacagacagggaatacacagcgaacagggaaaggatcaggccccccttgcttgaggcttgctttcctcatctgtagatttaggggtctcaatcaggtcatctcaagttccctaaacttgcttaaaaagcatcaaactttgagttagaccttcagacttccctaactccttttttcctgaattaagctatgacaaagatgaccatatgtcccagttcacctagtataatctcgatttatatctgttgtcctggaataacaattaattgctcctcctttaactctcaaaggtatctccagtcggaagataaattacatgcccctcatacctatgactatattcattttaatcttggtttagatttttaagaaaacacactaatttacttttaagcctacaaatatagcatttcatagcttgctttctcttaacacttggagaaatttcagattcttttgtgagtggtttgtgaactatcaaaaatttttttaacttggccgggcatgatgacctatgcctctaatcccagtactttggaaggctgaggcagaagaatcgcttaagatgggaagtttgcggctgcagtgagctacgatcacgccactacacttcagcctgggtgatgcagaaaggaccgtgtctctagaaataaaaataattttttaaaaactgagtaagtcaaatgtaaattttccttttcaaaaacaaattattcagtatgcaaaacattctgttaagacatattttctgataaccttagaatacgtggtacttaaaaactatgactaaaatatttgtggaagaattcattatcttaggtgatacattttaacaattaaaatagttccagaacacggtcttccacctgactttgacgattaaaacaatgttgtcaaaagaatgttctctctgaaaattctgggtctcatccaccaccataggtctcatctaccatcaactgaaataagctaatcagttataaacaagggaatatacttaaaaaaaaaaaaaagagagaaacacggtctcactctgtctccaaggctggagtgcagtggcacagtcatagctcactgcagcacagaactcctaagctcaggcaatactcccacctcagcttcccaggaatataccacttttactgcactgacaagctctgtatgctagtgattctcaaattttctttaaggctaggaccaagagtcctgccaatcccctgaacaacagctcacatattatcaaatgaacttgaaacattcctgtcatagtgagcagcattgaaacagattccataactgattactcagtttcaagggagatttaacattgctttgttttcaagttacaaaaagttccctagttttactcaaatatgcactatccctgattaaaaaaaacatgtttcattatgaagaggggtgatttgtttcagcatttttttttttcacttaaccacttaagtcactgcctgaggaagtttctttttaaggaaataaataccaggttcattagaagaaaaaaaaaaaacacataattttaattcattttgttttaaagatgcgtattttaaaaagactactttaaaatgaactaatatgttacactggatcatgctgtggcgactaacgtattgtcaagccttaacctaatgaaaacaaaagaaaagcgagtttggcactcacttgcacttttcatctctgttagaaagtatgtctcagtttggatctgagatcaggtttgcttggtaacctcaaagaataattttccttttttttttctttcaaaatttccttttgatcatttcagacagttcatccttttgagtgagaaagagtaaaagagaggaatgttgagtgaggttaagtaaatggagaatctgtcacataaagcaagtttaaatcctagtaagagcatccatgcaggacaaacggaagcattattcttttgaaaacattattcttttaaacagtgtgtaatgacatcctccctagagactttccatgagaggggaaaaaaattacttcctcagaagtcgttttctagattccaagcataataagtgaagcacagttaaaagtcaaacttgtgttttctttatgcaagaaggttcaaattagaactgcagaaaggtacttaaaagtttctctagcttgtcttttggttacatactggtattgctgtgaactaaaagagcaagtaagaggaaaggttactgttgttactttacacctataaatcagtgagtgtgtccttactgtaaaatttgagctgaacatattttgtttcaaaggagaaatatatgactcaaatatgctgaatgtatgataatttattaagttccttttaagtatatcattttcttatgctcaagtagaaactatggattatttttctagtattctatgctgctgttaccttctgaggagttgattgaaaattttatgcttttaaaagttgggtgctacttaaatatcagaattggctattgttttaaatatttaaaatatgcttaaacaacaattaaggttaataagcagagaaaatacttcttttgattcaaacactactttatatatttaatgaatacacgtccaaataaagatctctcttcaaaaattttggaaaatgttaatgcattttgaatataatggaacaaagaagaagaatactagagaaaattcacaattatgatgtttatttaggaaaataaacttgaagaaggttttctattaaaaaaacataagaatcatatccaaattttagactctccatcttctttggtatgaaaatcaacattcataatagaaaatattttcttttgaaaggtttagttgttattgggtctataacggttttccatataaggaaaatacagtattatctgtaatcatctcacttattgaacaaccaatgaatgcatgcaagtaaccaagcatatgtgtgcagagaccagcatcaaggaaatattcattcatagataaatgttttctaataaaatatattttaagtttttaatgatcttctgctatcattttttgccatgttatctgaatagccatccagatctgtagtaaaacatcctgttagttacataactcaagaagtacttccccaaggaagctcacaccatcataccaggacttagcaacatttatctttcaacatgagtataccattaaaatttttttatatttctcagaattgtattcttcagtcttttccacaatatagtatatggaaattgctaatagcattaaattaatattaataaaacccaattctatctaaacctttttctcataagaaaaaacattactttaaaaaatagactttttgtttcttctaaaagtagtactatatggactgctcaattagcaatgccaaatacttccaaaaacaccataggaccaccaagctatttctattgctttgataatttcttttcctgctccaatttctccacgttcctgctttcttgtgtcaaaatatcttcccttaatttgttaaaatgaatctgagggaaaaaaatctgataatctggggtaaagaaatttttttttttgcatagactcttgtgatcacaaaatgaccaggtaatttatagcttcagtgctaacactgtgattgggaacaagaagagtacaaccataataaaatacagctatctatgagaagaactgcataaagacatctttggccatgtaggctctgggccctctggaaataagtcagttgcattgccaacatgacaaagaaaatagcaatgttcagaatcaggaacaacctggtataggaagcagacagtgatggggccctgctgtgtgtagttgtcaccatccgtgcctgtccaaaccggcctttaatcaagcccccatttttatgtttctcgtatgttacatctgcaaaatctaaaaggtctttcatttcttcatcttcatctatgggtagttctttctgtgccaaaatctgagctttctgtctaatctttttctcattgacttcaatctgtgcaaaaatatcagggacagcatccacaaatttatagcgtttgcctgcccttcggtttttctttgacttgctttgctgctgctgttgctgtgatatggcaaaaatcctgtcaatggcctcctcagtctgtctcttatctgaaaatctcagcaggcgttcagcagtcttcctaaagctagctgtgttccggactcgggacagtatctgcttctccagcagctgaaacactggtttaaaatgctgcaagttctgttccacaatagcagcatagtccttcacctcagggacaatgctgctcttgatggctgaattccggtcaaacagaattttgtgacgatcagcaatgacctgtgcaaaggcagactgtcctgtggcctcacctgtccacaggtatgtggcgtaggcatgtttgctggtggctatgaacacatccagttgctgagagtctccgtggacagtgaagctctgaacatctatagatggccctatgaagaggtaagctgccctggtgatgggacttcggaggtgcatggtgacattcacatagtttgtcccattgtagggatagccccgaggatatgtcactgaggcaaaggttgctttctcgctgtagccagtatcgtccatccagtacattttatagagaccatctctctgcctgatgaaagccccatggacaccatctaccacagtctcctcaaaaggaacatccacattatggaagaagctcgctgctgtctccaagggactctcctctcccaggtgtatttggtctacaaggagaagcagctgtggatgtaggaggatgagattcctctgaacattcttcaggttgagctgggggttataagctcccacaccttctcctcggatgaaaaccaccccatttttctcctctgctgcaaccaccctcccctgacaactagctgccaggtcatgcttgtatttagaccattttgatgagcagtcttctgtgacctgacccacccagggagaaaagcagctctttgacacagctggggaaaacatcaaaacattgttgaagaaggtgtactttggcccgtacagagcctcagtaatgaaaggcacaccattgggagcaaaagtaaatgagttttgatcaggatgttcatgccctgcattaaaatttctccatcctttgatccaatctttgtatttgtttctgtggacaatgtcatatattgcacgtccccccagttttccagacttgaaggaaaggaaagatctattgatttctgcaggtagtgcacttccataagtcacgacaccccagtcttcaaaataatgcagtgtaggggtgccaaagtctggaggaggaaccgatttcaagctgccatcataccagagaaattctgtgtgcagagtgcaccagcgctgccctttggatggtgttcctggaccttccaccacacggttccttctgatttggtcagctagccagttaccactgccattacgcatgacaaatttatcaaggaacactaattggctttctggaccataaaaccagttgtaatttgagtccgcaatagccacagtcctttgaaaccctggcaggatggttctatacataaatgcaaagtgttgtttaagccacggatggccaaagtggttgatgttgaagtgcctctggacgagaaacatgtattggaagagtgatctagtggtgtagctgccatacgcaactccttcatagagggagccatccgtcacctccctgagcaagaccagagatttctccatgatggtcagaacttgtttggtccataagtaggcttcttgaagatatccttgattcatcaggactaggcttcccgtgagcaaagccatacagttggtgggctgatgattgtgcaggtattgaaatccccatcctctcctgtatgaagtttcatacatataccctgaggcattggcaatcacttcaagaaacttctcctgttgtgtcttgctcaggtagttgtacaagaagtcataagcagtggcaaaaccaaccagggagtgagcaagcgggacctcatcccaaggagcatctttcaccaaccaactaggctgcgctgccatcctctccatgtagtctttggccatgtctcgggcttcaatgttctcaggatacagcacacagaacattgccaaggcacccaagttgtttccaaaaatttcattccagcgggcactgtagtccttgggatcccagggagggaggtattccaaggggctggacagcatcgtgtgcacagcctccgtgaggcgggctgcaatgtgctcgtgcgagctggcagccctgagctgcagctccgccacttctgccctggagaagtacagcatgggatggctgtcgtagttggcattggtgaagggaatcataacttctgggttctcgtcggtgatgtaggctgacacaaagcaaagcaaatatatgaaaaacacactgggagccccccgtgtgtgagtcctcatcgtggcatcagatctccaaatctccaaggcagccaaaccatcttcgaaagatccttcctgcctcaaaaaagtgaagaccagaaaaacatttgttttcagacactggagagcaggcactgttacggctgtgattttacaactgctcctacatgctgggagcagtcgctagatgcatctcaaggtgggtcgtccgcgcttccagactcagcacaatcgacatttatttac

SEQ ID NO: 18011 - RNA, 9279 nt, Homo sapiens
  source 1..9279: mol_type = other RNA
tctgagttcctggagcctggtctacttttccagtctaattttctatcacccgccactacatacacaccctgtactccagttataccattctatgtgaagtccctgaacaaggcaagctgaaaacacaaatggcagaaatatttgaacaatttcctgggcttattaagggatagccagggtgacggcagcagagccatggcaggcaaccatgctcttcttatattaaataagactcagacatatataccattagggatccttgactcattatctttctgatcaatacttccacaaaatattcattcctttggccacacattttgcctgtgggctaggagttaaacattccctctccagacttattcaaggagctaattgtcttctacccagactatggaaatggtctcctaacctcttccccattgggtccactctctacactgaagctaaaattgcctttctaaaatgcaaatctgattatttaaaaagaaaattctttaatggcttgccattgcttgcagcgatttctaagcagagggtaccccctccctgccccacctcaccccagggagtaaacatatggaatatggggggcatatcagagccatctcagggatttttcaaagtttcacatacacacaggtatatgtggcatcatcaacacccctcacccatgtcccttttgctcccatacacatttcctatcccatgaaaatcgctgccatgcttgttgagtgatgggtgttatgttgtagccctcagttatgctgaggcataaaaatggttgagcagcctcatggcagaataaagtccagattccttagcatgtcctacaaagtcctgcacaatagcctccctgcttgccttttcagtttcatcttcacccattctccatcacacaccctgtgggccaacaccaccagtctggagaattcctgaaccaggtttgctttttcgtacttttttctttattctattccatttacccagaatgcacttctcctctcacacagctagtaaatttctgtttaacctttaagaaggcaccaacaattacatcttcagccacagcctgcccctggattccaggctggtacatctccacttggatttttagaaagtatcttaaacttaacatggctaaaacaacctcctggacccgcttcctactacttattcctcctgcagtcagccacatctcagttcattgcaactgactccccaactcataatccaagtctttgctgcagtctgtgagagcatgtatgatctgatcctattcctatcaccctcccctcccccactctgctctagccacactggcctcctagtcctaaatacaccaaacacatactgagctcagggccttcgaactgctgttctatctggaatgctcctctctcttagatgtccctgtgattcattcccttatttctttcaagtgtctgatcataagtaatcacatcagaaaccactgtttatgggacagtaccaattcaccatcaccttacatcccctccccttgctttattctccacagtacttaccactacttgacatcctgcactattactgttattatttgctcccactagaacataaactatacaagggccagcttttattattcctattctctaccatatcttcagttcctaaaacaatacttggcatatagtagatgctctgtaaacatgttattgtcattcgttatttgttaactcaactgaaaagtgctgtgggacttccatttaaacatactgcactcaatatataaatttccttcagttccttcctaaaaccccattaaattaacagcaaatagattttcaaaatgacacagagaatggaagtggagacatcaataaagcctaacctgatcaccacatttaaaattatggcctcctcttcccagtctccttaccctgacttttccttccatagcacctattatcttccaataagtataaagaatgggtaagagagctaaagcttcattagtaggcagttttagaccttattgtaaacaagtacacaatatatgtaacagccaaaagaattagaaattggttacttctgggaagtacaaactaagaatgagaggggaagggacagataatttattgttttgttttttaaataaggcttctagtactatactttttcaatcatgtatgttcataatttatgccaaataaaacttcaattaaaaaaatcccaaaaccaagagggaaactgtatatgcaagaagaaaagtcataatgcaactttgtctatttttattcttcacatagtgactatgtcttgtttaacagaatttgaacatattaaaatagatgaccaaatactaaatatttagactatgtagtggaacacatgatttatatcagtcatttcttgaaaacttatgagtacttcattgacattacatgcataaagcaaatatctagctgaaacattgctgaaaaaaaaatacgtcattttgccagtaaattaaataaactgcagaaagaaactacttctcaacatgaaagtaaagagaagagaatcaaggcaatgggctttgccacagacagggaatacacagcgaacagggaaaggatcaggccccccttgcttgaggcttgctttcctcatctgtagatttaggggtctcaatcaggtcatctcaagttccctaaacttgcttaaaaagcatcaaactttgagttagaccttcagacttccctaactccttttttcctgaattaagctatgacaaagatgaccatatgtcccagttcacctagtataatctcgatttatatctgttgtcctggaataacaattaattgctcctcctttaactctcaaaggtatctccagtcggaagataaattacatgcccctcatacctatgactatattcattttaatcttggtttagatttttaagaaaacacactaatttacttttaagcctacaaatatagcatttcatagcttgctttctcttaacacttggagaaatttcagattcttttgtgagtggtttgtgaactatcaaaaatttttttaacttggccgggcatgatgacctatgcctctaatcccagtactttggaaggctgaggcagaagaatcgcttaagatgggaagtttgcggctgcagtgagctacgatcacgccactacacttcagcctgggtgatgcagaaaggaccgtgtctctagaaataaaaataattttttaaaaactgagtaagtcaaatgtaaattttccttttcaaaaacaaattattcagtatgcaaaacattctgttaagacatattttctgataaccttagaatacgtggtacttaaaaactatgactaaaatatttgtggaagaattcattatcttaggtgatacattttaacaattaaaatagttccagaacacggtcttccacctgactttgacgattaaaacaatgttgtcaaaagaatgttctctctgaaaattctgggtctcatccaccaccataggtctcatctaccatcaactgaaataagctaatcagttataaacaagggaatatacttaaaaaaaaaaaaaagagagaaacacggtctcactctgtctccaaggctggagtgcagtggcacagtcatagctcactgcagcacagaactcctaagctcaggcaatactcccacctcagcttcccaggaatataccacttttactgcactgacaagctctgtatgctagtgattctcaaattttctttaaggctaggaccaagagtcctgccaatcccctgaacaacagctcacatattatcaaatgaacttgaaacattcctgtcatagtgagcagcattgaaacagattccataactgattactcagtttcaagggagatttaacattgctttgttttcaagttacaaaaagttccctagttttactcaaatatgcactatccctgattaaaaaaaacatgtttcattatgaagaggggtgatttgtttcagcatttttttttttcacttaaccacttaagtcactgcctgaggaagtttctttttaaggaaataaataccaggttcattagaagaaaaaaaaaaaacacataattttaattcattttgttttaaagatgcgtattttaaaaagactactttaaaatgaactaatatgttacactggatcatgctgtggcgactaacgtattgtcaagccttaacctaatgaaaacaaaagaaaagcgagtttggcactcacttgcacttttcatctctgttagaaagtatgtctcagtttggatctgagatcaggtttgcttggtaacctcaaagaataattttccttttttttttctttcaaaatttccttttgatcatttcagacagttcatccttttgagtgagaaagagtaaaagagaggaatgttgagtgaggttaagtaaatggagaatctgtcacataaagcaagtttaaatcctagtaagagcatccatgcaggacaaacggaagcattattcttttgaaaacattattcttttaaacagtgtgtaatgacatcctccctagagactttccatgagaggggaaaaaaattacttcctcagaagtcgttttctagattccaagcataataagtgaagcacagttaaaagtcaaacttgtgttttctttatgcaagaaggttcaaattagaactgcagaaaggtacttaaaagtttctctagcttgtcttttggttacatactggtattgctgtgaactaaaagagcaagtaagaggaaaggttactgttgttactttacacctataaatcagtgagtgtgtccttactgtaaaatttgagctgaacatattttgtttcaaaggagaaatatatgactcaaatatgctgaatgtatgataatttattaagttccttttaagtatatcattttcttatgctcaagtagaaactatggattatttttctagtattctatgctgctgttaccttctgaggagttgattgaaaattttatgcttttaaaagttgggtgctacttaaatatcagaattggctattgttttaaatatttaaaatatgcttaaacaacaattaaggttaataagcagagaaaatacttcttttgattcaaacactactttatatatttaatgaatacacgtccaaataaagatctctcttcaaaaattttggaaaatgttaatgcattttgaatataatggaacaaagaagaagaatactagagaaaattcacaattatgatgtttatttaggaaaataaacttgaagaaggttttctattaaaaaaacataagaatcatatccaaattttagactctccatcttctttggtatgaaaatcaacattcataatagaaaatattttcttttgaaaggtttagttgttattgggtctataacggttttccatataaggaaaatacagtattatctgtaatcatctcacttattgaacaaccaatgaatgcatgcaagtaaccaagcatatgtgtgcagagaccagcatcaaggaaatattcattcatagataaatgttttctaataaaatatattttaagtttttaatgatcttctgctatcattttttgccatgttatctgaatagccatccagatctgtagtaaaacatcctgttagttacataactcaagaagtacttccccaaggaagctcacaccatcataccaggacttagcaacatttatctttcaacatgagtataccattaaaatttttttatatttctcagaattgtattcttcagtcttttccacaatatagtatatggaaattgctaatagcattaaattaatattaataaaacccaattctatctaaacctttttctcataagaaaaaacattactttaaaaaatagactttttgtttcttctaaaagtagtactatatggactgctcaattagcaatgccaaatacttccaaaaacaccataggaccaccaagctatttctattgctttgataatttcttttcctgctccaatttctccacgttcctgctttcttgtgtcaaaatatcttcccttaatttgttaaaatgaatctgagggaaaaaaatctgataatctggggtaaagaaatttttttttttgcatagactcttgtgatcacaaaatgaccaggtaatttatagcttcagtgctaacactgtgattgggaacaagaagagtacaaccataataaaatacagctatctatgagaagaactgcataaagacatctttggccatgtaggctctgggccctctggaaataagtcagttgcattgccaacatgacaaagaaaatagcaatgttcagaatcaggaacaacctggtataggaagcagacagtgatggggccctgctgtgtgtagttgtcaccatccgtgcctgtccaaaccggcctttaatcaagcccccatttttatgtttctcgtatgttacatctgcaaaatctaaaaggtctttcatttcttcatcttcatctatgggtagttctttctgtgccaaaatctgagctttctgtctaatctttttctcattgacttcaatctgtgcaaaaatatcagggacagcatccacaaatttatagcgtttgcctgcccttcggtttttctttgacttgctttgctgctgctgttgctgtgatatggcaaaaatcctgtcaatggcctcctcagtctgtctcttatctgaaaatctcagcaggcgttcagcagtcttcctaaagctagctgtgttccggactcgggacagtatctgcttctccagcagctgaaacactggtttaaaatgctgcaagttctgttccacaatagcagcatagtccttcacctcagggacaatgctgctcttgatggctgaattccggtcaaacagaattttgtgacgatcagcaatgacctgtgcaaaggcagactgtcctgtggcctcacctgtccacaggtatgtggcgtaggcatgtttgctggtggctatgaacacatccagttgctgagagtctccgtggacagtgaagctctgaacatctatagatggccctatgaagaggtaagctgccctggtgatgggacttcggaggtgcatggtgacattcacatagtttgtcccattgtagggatagccccgaggatatgtcactgaggcaaaggttgctttctcgctgtagccagtatcgtccatccagtacattttatagagaccatctctctgcctgatgaaagccccatggacaccatctaccacagtctcctcaaaaggaacatccacattatggaagaagctcgctgctgtctccaagggactctcctctcccaggtgtatttggtctacaaggagaagcagctgtggatgtaggaggatgagattcctctgaacattcttcaggttgagctgggggttataagctcccacaccttctcctcggatgaaaaccaccccatttttctcctctgctgcaaccaccctcccctgacaactagctgccaggtcatgcttgtatttagaccattttgatgagcagtcttctgtgacctgacccacccagggagaaaagcagctctttgacacagctggggaaaacatcaaaacattgttgaagaaggtgtactttggcccgtacagagcctcagtaatgaaaggcacaccattgggagcaaaagtaaatgagttttgatcaggatgttcatgccctgcattaaaatttctccatcctttgatccaatctttgtatttgtttctgtggacaatgtcatatattgcacgtccccccagttttccagacttgaaggaaaggaaagatctattgatttctgcaggtagtgcacttccataagtcacgacaccccagtcttcaaaataatgcagtgtaggggtgccaaagtctggaggaggaaccgatttcaagctgccatcataccagagaaattctgtgtgcagagtgcaccagcgctgccctttggatggtgttcctggaccttccaccacacggttccttctgatttggtcagctagccagttaccactgccattacgcatgacaaatttatcaaggaacactaattggctttctggaccataaaaccagttgtaatttgagtccgcaatagccacagtcctttgaaaccctggcaggatggttctatacataaatgcaaagtgttgtttaagccacggatggccaaagtggttgatgttgaagtgcctctggacgagaaacatgtattggaagagtgatctagtggtgtagctgccatacgcaactccttcatagagggagccatccgtcacctccctgagcaagaccagagatttctccatgatggtcagaacttgtttggtccataagtaggcttcttgaagatatccttgattcatcaggactaggcttcccgtgagcaaagccatacagttggtgggctgatgattgtgcaggtattgaaatccccatcctctcctgtatgaagtttcatacatataccctgaggcattggcaatcacttcaagaaacttctcctgttgtgtcttgctcaggtagttgtacaagaagtcataagcagtggcaaaaccaaccagggagtgagcaagcgggacctcatcccaaggagcatctttcaccaactaggctgcgctgccatcctctccatgtagtctttggccatgtctcgggcttcaatgttctcaggatacagcacacagaacattgccaaggcacccaagttgtttccaaaaatttcattccagcgggcactgtagtccttgggatcccagggagggaggtattccaaggggctggacagcatcgtgtgcacagcctccgtgaggcgggctgcaatgtgctcgtgcgagctggcagccctgagctgcagctccgccacttctgccctggagaagtacagcatgggatggctgtcgtagttggcattggtgaagggaatcataacttctgggttctcgtcggtgatgtaggctgacacaaagcaaagcaaatatatgaaaaacacactgggagccccccgtgtgtgagtcctcatcgtggcatcagatctccaaatctccaaggcagccaaaccatcttcgaaagatccgctcccagccgaggcttcgttctctccggcgtcgcctccgcagcctccagagccagctcccggtcctcctcactccagggcgcccgggctcccggccccctccgaaccgagccctccgcgcccccgccgcgccatgccccgggatgcgctgctgcagcctcgggcgacgctact

SEQ ID NO: 18012 - RNA, 9839 nt, Homo sapiens
  source 1..9839: mol_type = other RNA
tctgagttcctggagcctggtctacttttccagtctaattttctatcacccgccactacatacacaccctgtactccagttataccattctatgtgaagtccctgaacaaggcaagctgaaaacacaaatggcagaaatatttgaacaatttcctgggcttattaagggatagccagggtgacggcagcagagccatggcaggcaaccatgctcttcttatattaaataagactcagacatatataccattagggatccttgactcattatctttctgatcaatacttccacaaaatattcattcctttggccacacattttgcctgtgggctaggagttaaacattccctctccagacttattcaaggagctaattgtcttctacccagactatggaaatggtctcctaacctcttccccattgggtccactctctacactgaagctaaaattgcctttctaaaatgcaaatctgattatttaaaaagaaaattctttaatggcttgccattgcttgcagcgatttctaagcagagggtaccccctccctgccccacctcaccccagggagtaaacatatggaatatggggggcatatcagagccatctcagggatttttcaaagtttcacatacacacaggtatatgtggcatcatcaacacccctcacccatgtcccttttgctcccatacacatttcctatcccatgaaaatcgctgccatgcttgttgagtgatgggtgttatgttgtagccctcagttatgctgaggcataaaaatggttgagcagcctcatggcagaataaagtccagattccttagcatgtcctacaaagtcctgcacaatagcctccctgcttgccttttcagtttcatcttcacccattctccatcacacaccctgtgggccaacaccaccagtctggagaattcctgaaccaggtttgctttttcgtacttttttctttattctattccatttacccagaatgcacttctcctctcacacagctagtaaatttctgtttaacctttaagaaggcaccaacaattacatcttcagccacagcctgcccctggattccaggctggtacatctccacttggatttttagaaagtatcttaaacttaacatggctaaaacaacctcctggacccgcttcctactacttattcctcctgcagtcagccacatctcagttcattgcaactgactccccaactcataatccaagtctttgctgcagtctgtgagagcatgtatgatctgatcctattcctatcaccctcccctcccccactctgctctagccacactggcctcctagtcctaaatacaccaaacacatactgagctcagggccttcgaactgctgttctatctggaatgctcctctctcttagatgtccctgtgattcattcccttatttctttcaagtgtctgatcataagtaatcacatcagaaaccactgtttatgggacagtaccaattcaccatcaccttacatcccctccccttgctttattctccacagtacttaccactacttgacatcctgcactattactgttattatttgctcccactagaacataaactatacaagggccagcttttattattcctattctctaccatatcttcagttcctaaaacaatacttggcatatagtagatgctctgtaaacatgttattgtcattcgttatttgttaactcaactgaaaagtgctgtgggacttccatttaaacatactgcactcaatatataaatttccttcagttccttcctaaaaccccattaaattaacagcaaatagattttcaaaatgacacagagaatggaagtggagacatcaataaagcctaacctgatcaccacatttaaaattatggcctcctcttcccagtctccttaccctgacttttccttccatagcacctattatcttccaataagtataaagaatgggtaagagagctaaagcttcattagtaggcagttttagaccttattgtaaacaagtacacaatatatgtaacagccaaaagaattagaaattggttacttctgggaagtacaaactaagaatgagaggggaagggacagataatttattgttttgttttttaaataaggcttctagtactatactttttcaatcatgtatgttcataatttatgccaaataaaacttcaattaaaaaaatcccaaaaccaagagggaaactgtatatgcaagaagaaaagtcataatgcaactttgtctatttttattcttcacatagtgactatgtcttgtttaacagaatttgaacatattaaaatagatgaccaaatactaaatatttagactatgtagtggaacacatgatttatatcagtcatttcttgaaaacttatgagtacttcattgacattacatgcataaagcaaatatctagctgaaacattgctgaaaaaaaaatacgtcattttgccagtaaattaaataaactgcagaaagaaactacttctcaacatgaaagtaaagagaagagaatcaaggcaatgggctttgccacagacagggaatacacagcgaacagggaaaggatcaggccccccttgcttgaggcttgctttcctcatctgtagatttaggggtctcaatcaggtcatctcaagttccctaaacttgcttaaaaagcatcaaactttgagttagaccttcagacttccctaactccttttttcctgaattaagctatgacaaagatgaccatatgtcccagttcacctagtataatctcgatttatatctgttgtcctggaataacaattaattgctcctcctttaactctcaaaggtatctccagtcggaagataaattacatgcccctcatacctatgactatattcattttaatcttggtttagatttttaagaaaacacactaatttacttttaagcctacaaatatagcatttcatagcttgctttctcttaacacttggagaaatttcagattcttttgtgagtggtttgtgaactatcaaaaatttttttaacttggccgggcatgatgacctatgcctctaatcccagtactttggaaggctgaggcagaagaatcgcttaagatgggaagtttgcggctgcagtgagctacgatcacgccactacacttcagcctgggtgatgcagaaaggaccgtgtctctagaaataaaaataattttttaaaaactgagtaagtcaaatgtaaattttccttttcaaaaacaaattattcagtatgcaaaacattctgttaagacatattttctgataaccttagaatacgtggtacttaaaaactatgactaaaatatttgtggaagaattcattatcttaggtgatacattttaacaattaaaatagttccagaacacggtcttccacctgactttgacgattaaaacaatgttgtcaaaagaatgttctctctgaaaattctgggtctcatccaccaccataggtctcatctaccatcaactgaaataagctaatcagttataaacaagggaatatacttaaaaaaaaaaaaaagagagaaacacggtctcactctgtctccaaggctggagtgcagtggcacagtcatagctcactgcagcacagaactcctaagctcaggcaatactcccacctcagcttcccaggaatataccacttttactgcactgacaagctctgtatgctagtgattctcaaattttctttaaggctaggaccaagagtcctgccaatcccctgaacaacagctcacatattatcaaatgaacttgaaacattcctgtcatagtgagcagcattgaaacagattccataactgattactcagtttcaagggagatttaacattgctttgttttcaagttacaaaaagttccctagttttactcaaatatgcactatccctgattaaaaaaaacatgtttcattatgaagaggggtgatttgtttcagcatttttttttttcacttaaccacttaagtcactgcctgaggaagtttctttttaaggaaataaataccaggttcattagaagaaaaaaaaaaaacacataattttaattcattttgttttaaagatgcgtattttaaaaagactactttaaaatgaactaatatgttacactggatcatgctgtggcgactaacgtattgtcaagccttaacctaatgaaaacaaaagaaaagcgagtttggcactcacttgcacttttcatctctgttagaaagtatgtctcagtttggatctgagatcaggtttgcttggtaacctcaaagaataattttccttttttttttctttcaaaatttccttttgatcatttcagacagttcatccttttgagtgagaaagagtaaaagagaggaatgttgagtgaggttaagtaaatggagaatctgtcacataaagcaagtttaaatcctagtaagagcatccatgcaggacaaacggaagcattattcttttgaaaacattattcttttaaacagtgtgtaatgacatcctccctagagactttccatgagaggggaaaaaaattacttcctcagaagtcgttttctagattccaagcataataagtgaagcacagttaaaagtcaaacttgtgttttctttatgcaagaaggttcaaattagaactgcagaaaggtacttaaaagtttctctagcttgtcttttggttacatactggtattgctgtgaactaaaagagcaagtaagaggaaaggttactgttgttactttacacctataaatcagtgagtgtgtccttactgtaaaatttgagctgaacatattttgtttcaaaggagaaatatatgactcaaatatgctgaatgtatgataatttattaagttccttttaagtatatcattttcttatgctcaagtagaaactatggattatttttctagtattctatgctgctgttaccttctgaggagttgattgaaaattttatgcttttaaaagttgggtgctacttaaatatcagaattggctattgttttaaatatttaaaatatgcttaaacaacaattaaggttaataagcagagaaaatacttcttttgattcaaacactactttatatatttaatgaatacacgtccaaataaagatctctcttcaaaaattttggaaaatgttaatgcattttgaatataatggaacaaagaagaagaatactagagaaaattcacaattatgatgtttatttaggaaaataaacttgaagaaggttttctattaaaaaaacataagaatcatatccaaattttagactctccatcttctttggtatgaaaatcaacattcataatagaaaatattttcttttgaaaggtttagttgttattgggtctataacggttttccatataaggaaaatacagtattatctgtaatcatctcacttattgaacaaccaatgaatgcatgcaagtaaccaagcatatgtgtgcagagaccagcatcaaggaaatattcattcatagataaatgttttctaataaaatatattttaagtttttaatgatcttctgctatcattttttgccatgttatctgaatagccatccagatctgtagtaaaacatcctgttagttacataactcaagaagtacttccccaaggaagctcacaccatcataccaggacttagcaacatttatctttcaacatgagtataccattaaaatttttttatatttctcagaattgtattcttcagtcttttccacaatatagtatatggaaattgctaatagcattaaattaatattaataaaacccaattctatctaaacctttttctcataagaaaaaacattactttaaaaaatagactttttgtttcttctaaaagtagtactatatggactgctcaattagcaatgccaaatacttccaaaaacaccataggaccaccaagctatttctattgctttgataatttcttttcctgctccaatttctccacgttcctgctttcttgtgtcaaaatatcttcccttaatttgttaaaatgaatctgagggaaaaaaatctgataatctggggtaaagaaatttttttttttgcatagactcttgtgatcacaaaatgaccaggtaatttatagcttcagtgctaacactgtgattgggaacaagaagagtacaaccataataaaatacagctatctatgagaagaactgcataaagacatctttggccatgtaggctctgggccctctggaaataagtcagttgcattgccaacatgacaaagaaaatagcaatgttcagaatcaggaacaacctggtataggaagcagacagtgatggggccctgctgtgtgtagttgtcaccatccgtgcctgtccaaaccggcctttaatcaagcccccatttttatgtttctcgtatgttacatctgcaaaatctaaaaggtctttcatttcttcatcttcatctatgggtagttctttctgtgccaaaatctgagctttctgtctaatctttttctcattgacttcaatctgtgcaaaaatatcagggacagcatccacaaatttatagcgtttgcctgcccttcggtttttctttgacttgctttgctgctgctgttgctgtgatatggcaaaaatcctgtcaatggcctcctcagtctgtctcttatctgaaaatctcagcaggcgttcagcagtcttcctaaagctagctgtgttccggactcgggacagtatctgcttctccagcagctgaaacactggtttaaaatgctgcaagttctgttccacaatagcagcatagtccttcacctcagggacaatgctgctcttgatggctgaattccggtcaaacagaattttgtgacgatcagcaatgacctgtgcaaaggcagactgtcctgtggcctcacctgtccacaggtatgtggcgtaggcatgtttgctggtggctatgaacacatccagttgctgagagtctccgtggacagtgaagctctgaacatctatagatggccctatgaagaggtaagctgccctggtgatgggacttcggaggtgcatggtgacattcacatagtttgtcccattgtagggatagccccgaggatatgtcactgaggcaaaggttgctttctcgctgtagccagtatcgtccatccagtacattttatagagaccatctctctgcctgatgaaagccccatggacaccatctaccacagtctcctcaaaaggaacatccacattatggaagaagctcgctgctgtctccaagggactctcctctcccaggtgtatttggtctacaaggagaagcagctgtggatgtaggaggatgagattcctctgaacattcttcaggttgagctgggggttataagctcccacaccttctcctcggatgaaaaccaccccatttttctcctctgctgcaaccaccctcccctgacaactagctgccaggtcatgcttgtatttagaccattttgatgagcagtcttctgtgacctgacccacccagggagaaaagcagctctttgacacagctggggaaaacatcaaaacattgttgaagaaggtgtactttggcccgtacagagcctcagtaatgaaaggcacaccattgggagcaaaagtaaatgagttttgatcaggatgttcatgccctgcattaaaatttctccatcctttgatccaatctttgtatttgtttctgtggacaatgtcatatattgcacgtccccccagttttccagacttgaaggaaaggaaagatctattgatttctgcaggtagtgcacttccataagtcacgacaccccagtcttcaaaataatgcagtgtaggggtgccaaagtctggaggaggaaccgatttcaagctgccatcataccagagaaattctgtgtgcagagtgcaccagcgctgccctttggatggtgttcctggaccttccaccacacggttccttctgatttggtcagctagccagttaccactgccattacgcatgacaaatttatcaaggaacactaattggctttctggaccataaaaccagttgtaatttgagtccgcaatagccacagtcctttgaaaccctggcaggatggttctatacataaatgcaaagtgttgtttaagccacggatggccaaagtggttgatgttgaagtgcctctggacgagaaacatgtattggaagagtgatctagtggtgtagctgccatacgcaactccttcatagagggagccatccgtcacctccctgagcaagaccagagatttctccatgatggtcagaacttgtttggtccataagtaggcttcttgaagatatccttgattcatcaggactaggcttcccgtgagcaaagccatacagttggtgggctgatgattgtgcaggtattgaaatccccatcctctcctgtatgaagtttcatacatataccctgaggcattggcaatcacttcaagaaacttctcctgttgtgtcttgctcaggtagttgtacaagaagtcataagcagtggcaaaaccaaccagggagtgagcaagcgggacctcatcccaaggagcatctttcaccaactaggctgcgctgccatcctctccatgtagtctttggccatgtctcgggcttcaatgttctcaggatacagcacacagaacattgccaaggcacccaagttgtttccaaaaatttcattccagcgggcactgtagtccttgggatcccagggagggaggtattccaaggggctggacagcatcgtgtgcacagcctccgtgaggcgggctgcaatgtgctcgtgcgagctggcagccctgagctgcagctccgccacttctgccctggagaagtacagcatgggatggctgtcgtagttggcattggtgaagggaatcataacttctgggttctcgtcggtgatgtaggctgacacaaagcaaagcaaatatatgaaaaacacactgggagccccccgtgtgtgagtcctcatcgtggcatcagatctccaaatctccaaggcagccaaaccatcttcgaaagatcctcacagtgcagggtggtatgccgccaaatgcttccacaaagctcagtgtcccattgtggagcgccttactaactccatgatgatgcacggctgcaacaacggcaagaagctcatgactgtgtgcatcgtcaagcatgccttcgaggtcatacacctgctcacaggcgagaaccctctgcaggtcctggtgaacgccatcatcaacagtggtccccgggaggactccacacgcattgggtgcgccgggactgtgagacgacaggctgtggacgtgtccccacttcgccgtgtgaatcaggccatctggctgctgtgcacaggtgctcgtgaggctgccttccggaacattaagaccattgctgagtgcctggcagaggagctcatcaatgctgccaagggctcctccaactcctatgccattaagaagaaggacgtgtggccttcttggagcatgtggccaagtccaaccgctgattttcccagctgttgcccaataaacctgtctgcccttcagggcagcccttaaagtaaatattttcagaaacaataggttaggtgccttagaaattcattcagaggcttagaaatccacattaacacagttcttacatgcttgagtctggtctacatccatttacgtaagtaaaactccccttccagactgacgaaattctttttgtgacaagaagacaaaggaatacgatggattgataagcgtagtcaaccgcgcagag

SEQ ID NO: 18013 - RNA, 9744 nt, Homo sapiens
  source 1..9744: mol_type = other RNA
tctgagttcctggagcctggtctacttttccagtctaattttctatcacccgccactacatacacaccctgtactccagttataccattctatgtgaagtccctgaacaaggcaagctgaaaacacaaatggcagaaatatttgaacaatttcctgggcttattaagggatagccagggtgacggcagcagagccatggcaggcaaccatgctcttcttatattaaataagactcagacatatataccattagggatccttgactcattatctttctgatcaatacttccacaaaatattcattcctttggccacacattttgcctgtgggctaggagttaaacattccctctccagacttattcaaggagctaattgtcttctacccagactatggaaatggtctcctaacctcttccccattgggtccactctctacactgaagctaaaattgcctttctaaaatgcaaatctgattatttaaaaagaaaattctttaatggcttgccattgcttgcagcgatttctaagcagagggtaccccctccctgccccacctcaccccagggagtaaacatatggaatatggggggcatatcagagccatctcagggatttttcaaagtttcacatacacacaggtatatgtggcatcatcaacacccctcacccatgtcccttttgctcccatacacatttcctatcccatgaaaatcgctgccatgcttgttgagtgatgggtgttatgttgtagccctcagttatgctgaggcataaaaatggttgagcagcctcatggcagaataaagtccagattccttagcatgtcctacaaagtcctgcacaatagcctccctgcttgccttttcagtttcatcttcacccattctccatcacacaccctgtgggccaacaccaccagtctggagaattcctgaaccaggtttgctttttcgtacttttttctttattctattccatttacccagaatgcacttctcctctcacacagctagtaaatttctgtttaacctttaagaaggcaccaacaattacatcttcagccacagcctgcccctggattccaggctggtacatctccacttggatttttagaaagtatcttaaacttaacatggctaaaacaacctcctggacccgcttcctactacttattcctcctgcagtcagccacatctcagttcattgcaactgactccccaactcataatccaagtctttgctgcagtctgtgagagcatgtatgatctgatcctattcctatcaccctcccctcccccactctgctctagccacactggcctcctagtcctaaatacaccaaacacatactgagctcagggccttcgaactgctgttctatctggaatgctcctctctcttagatgtccctgtgattcattcccttatttctttcaagtgtctgatcataagtaatcacatcagaaaccactgtttatgggacagtaccaattcaccatcaccttacatcccctccccttgctttattctccacagtacttaccactacttgacatcctgcactattactgttattatttgctcccactagaacataaactatacaagggccagcttttattattcctattctctaccatatcttcagttcctaaaacaatacttggcatatagtagatgctctgtaaacatgttattgtcattcgttatttgttaactcaactgaaaagtgctgtgggacttccatttaaacatactgcactcaatatataaatttccttcagttccttcctaaaaccccattaaattaacagcaaatagattttcaaaatgacacagagaatggaagtggagacatcaataaagcctaacctgatcaccacatttaaaattatggcctcctcttcccagtctccttaccctgacttttccttccatagcacctattatcttccaataagtataaagaatgggtaagagagctaaagcttcattagtaggcagttttagaccttattgtaaacaagtacacaatatatgtaacagccaaaagaattagaaattggttacttctgggaagtacaaactaagaatgagaggggaagggacagataatttattgttttgttttttaaataaggcttctagtactatactttttcaatcatgtatgttcataatttatgccaaataaaacttcaattaaaaaaatcccaaaaccaagagggaaactgtatatgcaagaagaaaagtcataatgcaactttgtctatttttattcttcacatagtgactatgtcttgtttaacagaatttgaacatattaaaatagatgaccaaatactaaatatttagactatgtagtggaacacatgatttatatcagtcatttcttgaaaacttatgagtacttcattgacattacatgcataaagcaaatatctagctgaaacattgctgaaaaaaaaatacgtcattttgccagtaaattaaataaactgcagaaagaaactacttctcaacatgaaagtaaagagaagagaatcaaggcaatgggctttgccacagacagggaatacacagcgaacagggaaaggatcaggccccccttgcttgaggcttgctttcctcatctgtagatttaggggtctcaatcaggtcatctcaagttccctaaacttgcttaaaaagcatcaaactttgagttagaccttcagacttccctaactccttttttcctgaattaagctatgacaaagatgaccatatgtcccagttcacctagtataatctcgatttatatctgttgtcctggaataacaattaattgctcctcctttaactctcaaaggtatctccagtcggaagataaattacatgcccctcatacctatgactatattcattttaatcttggtttagatttttaagaaaacacactaatttacttttaagcctacaaatatagcatttcatagcttgctttctcttaacacttggagaaatttcagattcttttgtgagtggtttgtgaactatcaaaaatttttttaacttggccgggcatgatgacctatgcctctaatcccagtactttggaaggctgaggcagaagaatcgcttaagatgggaagtttgcggctgcagtgagctacgatcacgccactacacttcagcctgggtgatgcagaaaggaccgtgtctctagaaataaaaataattttttaaaaactgagtaagtcaaatgtaaattttccttttcaaaaacaaattattcagtatgcaaaacattctgttaagacatattttctgataaccttagaatacgtggtacttaaaaactatgactaaaatatttgtggaagaattcattatcttaggtgatacattttaacaattaaaatagttccagaacacggtcttccacctgactttgacgattaaaacaatgttgtcaaaagaatgttctctctgaaaattctgggtctcatccaccaccataggtctcatctaccatcaactgaaataagctaatcagttataaacaagggaatatacttaaaaaaaaaaaaaagagagaaacacggtctcactctgtctccaaggctggagtgcagtggcacagtcatagctcactgcagcacagaactcctaagctcaggcaatactcccacctcagcttcccaggaatataccacttttactgcactgacaagctctgtatgctagtgattctcaaattttctttaaggctaggaccaagagtcctgccaatcccctgaacaacagctcacatattatcaaatgaacttgaaacattcctgtcatagtgagcagcattgaaacagattccataactgattactcagtttcaagggagatttaacattgctttgttttcaagttacaaaaagttccctagttttactcaaatatgcactatccctgattaaaaaaaacatgtttcattatgaagaggggtgatttgtttcagcatttttttttttcacttaaccacttaagtcactgcctgaggaagtttctttttaaggaaataaataccaggttcattagaagaaaaaaaaaaaacacataattttaattcattttgttttaaagatgcgtattttaaaaagactactttaaaatgaactaatatgttacactggatcatgctgtggcgactaacgtattgtcaagccttaacctaatgaaaacaaaagaaaagcgagtttggcactcacttgcacttttcatctctgttagaaagtatgtctcagtttggatctgagatcaggtttgcttggtaacctcaaagaataattttccttttttttttctttcaaaatttccttttgatcatttcagacagttcatccttttgagtgagaaagagtaaaagagaggaatgttgagtgaggttaagtaaatggagaatctgtcacataaagcaagtttaaatcctagtaagagcatccatgcaggacaaacggaagcattattcttttgaaaacattattcttttaaacagtgtgtaatgacatcctccctagagactttccatgagaggggaaaaaaattacttcctcagaagtcgttttctagattccaagcataataagtgaagcacagttaaaagtcaaacttgtgttttctttatgcaagaaggttcaaattagaactgcagaaaggtacttaaaagtttctctagcttgtcttttggttacatactggtattgctgtgaactaaaagagcaagtaagaggaaaggttactgttgttactttacacctataaatcagtgagtgtgtccttactgtaaaatttgagctgaacatattttgtttcaaaggagaaatatatgactcaaatatgctgaatgtatgataatttattaagttccttttaagtatatcattttcttatgctcaagtagaaactatggattatttttctagtattctatgctgctgttaccttctgaggagttgattgaaaattttatgcttttaaaagttgggtgctacttaaatatcagaattggctattgttttaaatatttaaaatatgcttaaacaacaattaaggttaataagcagagaaaatacttcttttgattcaaacactactttatatatttaatgaatacacgtccaaataaagatctctcttcaaaaattttggaaaatgttaatgcattttgaatataatggaacaaagaagaagaatactagagaaaattcacaattatgatgtttatttaggaaaataaacttgaagaaggttttctattaaaaaaacataagaatcatatccaaattttagactctccatcttctttggtatgaaaatcaacattcataatagaaaatattttcttttgaaaggtttagttgttattgggtctataacggttttccatataaggaaaatacagtattatctgtaatcatctcacttattgaacaaccaatgaatgcatgcaagtaaccaagcatatgtgtgcagagaccagcatcaaggaaatattcattcatagataaatgttttctaataaaatatattttaagtttttaatgatcttctgctatcattttttgccatgttatctgaatagccatccagatctgtagtaaaacatcctgttagttacataactcaagaagtacttccccaaggaagctcacaccatcataccaggacttagcaacatttatctttcaacatgagtataccattaaaatttttttatatttctcagaattgtattcttcagtcttttccacaatatagtatatggaaattgctaatagcattaaattaatattaataaaacccaattctatctaaacctttttctcataagaaaaaacattactttaaaaaatagactttttgtttcttctaaaagtagtactatatggactgctcaattagcaatgccaaatacttccaaaaacaccataggaccaccaagctatttctattgctttgataatttcttttcctgctccaatttctccacgttcctgctttcttgtgtcaaaatatcttcccttaatttgttaaaatgaatctgagggaaaaaaatctgataatctggggtaaagaaatttttttttttgcatagactcttgtgatcacaaaatgaccaggtaatttatagcttcagtgctaacactgtgattgggaacaagaagagtacaaccataataaaatacagctatctatgagaagaactgcataaagacatctttggccatgtaggctctgggccctctggaaataagtcagttgcattgccaacatgacaaagaaaatagcaatgttcagaatcaggaacaacctggtataggaagcagacagtgatggggccctgctgtgtgtagttgtcaccatccgtgcctgtccaaaccggcctttaatcaagcccccatttttatgtttctcgtatgttacatctgcaaaatctaaaaggtctttcatttcttcatcttcatctatgggtagttctttctgtgccaaaatctgagctttctgtctaatctttttctcattgacttcaatctgtgcaaaaatatcagggacagcatccacaaatttatagcgtttgcctgcccttcggtttttctttgacttgctttgctgctgctgttgctgtgatatggcaaaaatcctgtcaatggcctcctcagtctgtctcttatctgaaaatctcagcaggcgttcagcagtcttcctaaagctagctgtgttccggactcgggacagtatctgcttctccagcagctgaaacactggtttaaaatgctgcaagttctgttccacaatagcagcatagtccttcacctcagggacaatgctgctcttgatggctgaattccggtcaaacagaattttgtgacgatcagcaatgacctgtgcaaaggcagactgtcctgtggcctcacctgtccacaggtatgtggcgtaggcatgtttgctggtggctatgaacacatccagttgctgagagtctccgtggacagtgaagctctgaacatctatagatggccctatgaagaggtaagctgccctggtgatgggacttcggaggtgcatggtgacattcacatagtttgtcccattgtagggatagccccgaggatatgtcactgaggcaaaggttgctttctcgctgtagccagtatcgtccatccagtacattttatagagaccatctctctgcctgatgaaagccccatggacaccatctaccacagtctcctcaaaaggaacatccacattatggaagaagctcgctgctgtctccaagggactctcctctcccaggtgtatttggtctacaaggagaagcagctgtggatgtaggaggatgagattcctctgaacattcttcaggttgagctgggggttataagctcccacaccttctcctcggatgaaaaccaccccatttttctcctctgctgcaaccaccctcccctgacaactagctgccaggtcatgcttgtatttagaccattttgatgagcagtcttctgtgacctgacccacccagggagaaaagcagctctttgacacagctggggaaaacatcaaaacattgttgaagaaggtgtactttggcccgtacagagcctcagtaatgaaaggcacaccattgggagcaaaagtaaatgagttttgatcaggatgttcatgccctgcattaaaatttctccatcctttgatccaatctttgtatttgtttctgtggacaatgtcatatattgcacgtccccccagttttccagacttgaaggaaaggaaagatctattgatttctgcaggtagtgcacttccataagtcacgacaccccagtcttcaaaataatgcagtgtaggggtgccaaagtctggaggaggaaccgatttcaagctgccatcataccagagaaattctgtgtgcagagtgcaccagcgctgccctttggatggtgttcctggaccttccaccacacggttccttctgatttggtcagctagccagttaccactgccattacgcatgacaaatttatcaaggaacactaattggctttctggaccataaaaccagttgtaatttgagtccgcaatagccacagtcctttgaaacctccttcatagagggagccatccgtcacctccctgagcaagaccagagatttctccatgatggtcagaacttgtttggtccataagtaggcttcttgaagatatcctgaaggatgaaaacacatggaagcaatgactaaagccttgattcatcaggactaggcttcccgtgagcaaagccatacagttggtgggctgatgattgtgcaggtattgaaatccccatcctctcctgtatgaagtttcatacatataccctgaggcattggcaatcacttcaagaaacttctcctgttgtgtcttgctcaggtagttgtacaagaagtcataagcagtggcaaaaccaaccagggagtgagcaagcgggacctcatcccaaggagcatctttcaccaaccaactaggctgcgctgccatcctctccatgtagtctttggccatgtctcgggcttcaatgttctcaggatacagcacacagaacattgccaaggcacccaagttgtttccaaaaatttcattccagcgggcactgtagtccttgggatcccagggagggaggtattccaaggggctggacagcatcgtgtgcacagcctccgtgaggcgggctgcaatgtgctcgtgcgagctggcagccctgagctgcagctccgccacttctgccctggagaagtacagcatgggatggctgtcgtagttggcattggtgaagggaatcataacttctgggttctcgtcggtgatgtaggctgacacaaagcaaagcaaatatatgaaaaacacactgggagccccccgtgtgtgagtcctcatcgtggcatcagatctccaaatctccaaggcagccaaaccatcttcgaaagatcctcacagtgcagggtggtatgccgccaaatgcttccacaaagctcagtgtcccattgtggagcgccttactaactccatgatgatgcacggctgcaacaacggcaagaagctcatgactgtgtgcatcgtcaagcatgccttcgaggtcatacacctgctcacaggcgagaaccctctgcaggtcctggtgaacgccatcatcaacagtggtccccgggaggactccacacgcattgggtgcgccgggactgtgagacgacaggctgtggacgtgtccccacttcgccgtgtgaatcaggccatctggctgctgtgcacaggtgctcgtgaggctgccttccggaacattaagaccattgctgagtgcctggcagaggagctcatcaatgctgccaagggctcctccaactcctatgccattaagaagaaggacgtgtggccttcttggagcatgtggccaagtccaaccgctgattttcccagctgttgcccaataaacctgtctgcccttcagggcagcccttaaagtaaatattttcagaaacaataggttaggtgccttagaaattcattcagaggcttagaaatccacattaacacagttcttacatgcttgagtctggtctacatccatttacgtaagtaaaactccccttccagactgacgaaattctttttgtgacaagaagacaaaggaatacgatggattgataagcgtagtcaaccgcgcagag

SEQ ID NO: 18014 - RNA, 9075 nt, Homo sapiens
  source 1..9075: mol_type = other RNA
tctgagttcctggagcctggtctacttttccagtctaattttctatcacccgccactacatacacaccctgtactccagttataccattctatgtgaagtccctgaacaaggcaagctgaaaacacaaatggcagaaatatttgaacaatttcctgggcttattaagggatagccagggtgacggcagcagagccatggcaggcaaccatgctcttcttatattaaataagactcagacatatataccattagggatccttgactcattatctttctgatcaatacttccacaaaatattcattcctttggccacacattttgcctgtgggctaggagttaaacattccctctccagacttattcaaggagctaattgtcttctacccagactatggaaatggtctcctaacctcttccccattgggtccactctctacactgaagctaaaattgcctttctaaaatgcaaatctgattatttaaaaagaaaattctttaatggcttgccattgcttgcagcgatttctaagcagagggtaccccctccctgccccacctcaccccagggagtaaacatatggaatatggggggcatatcagagccatctcagggatttttcaaagtttcacatacacacaggtatatgtggcatcatcaacacccctcacccatgtcccttttgctcccatacacatttcctatcccatgaaaatcgctgccatgcttgttgagtgatgggtgttatgttgtagccctcagttatgctgaggcataaaaatggttgagcagcctcatggcagaataaagtccagattccttagcatgtcctacaaagtcctgcacaatagcctccctgcttgccttttcagtttcatcttcacccattctccatcacacaccctgtgggccaacaccaccagtctggagaattcctgaaccaggtttgctttttcgtacttttttctttattctattccatttacccagaatgcacttctcctctcacacagctagtaaatttctgtttaacctttaagaaggcaccaacaattacatcttcagccacagcctgcccctggattccaggctggtacatctccacttggatttttagaaagtatcttaaacttaacatggctaaaacaacctcctggacccgcttcctactacttattcctcctgcagtcagccacatctcagttcattgcaactgactccccaactcataatccaagtctttgctgcagtctgtgagagcatgtatgatctgatcctattcctatcaccctcccctcccccactctgctctagccacactggcctcctagtcctaaatacaccaaacacatactgagctcagggccttcgaactgctgttctatctggaatgctcctctctcttagatgtccctgtgattcattcccttatttctttcaagtgtctgatcataagtaatcacatcagaaaccactgtttatgggacagtaccaattcaccatcaccttacatcccctccccttgctttattctccacagtacttaccactacttgacatcctgcactattactgttattatttgctcccactagaacataaactatacaagggccagcttttattattcctattctctaccatatcttcagttcctaaaacaatacttggcatatagtagatgctctgtaaacatgttattgtcattcgttatttgttaactcaactgaaaagtgctgtgggacttccatttaaacatactgcactcaatatataaatttccttcagttccttcctaaaaccccattaaattaacagcaaatagattttcaaaatgacacagagaatggaagtggagacatcaataaagcctaacctgatcaccacatttaaaattatggcctcctcttcccagtctccttaccctgacttttccttccatagcacctattatcttccaataagtataaagaatgggtaagagagctaaagcttcattagtaggcagttttagaccttattgtaaacaagtacacaatatatgtaacagccaaaagaattagaaattggttacttctgggaagtacaaactaagaatgagaggggaagggacagataatttattgttttgttttttaaataaggcttctagtactatactttttcaatcatgtatgttcataatttatgccaaataaaacttcaattaaaaaaatcccaaaaccaagagggaaactgtatatgcaagaagaaaagtcataatgcaactttgtctatttttattcttcacatagtgactatgtcttgtttaacagaatttgaacatattaaaatagatgaccaaatactaaatatttagactatgtagtggaacacatgatttatatcagtcatttcttgaaaacttatgagtacttcattgacattacatgcataaagcaaatatctagctgaaacattgctgaaaaaaaaatacgtcattttgccagtaaattaaataaactgcagaaagaaactacttctcaacatgaaagtaaagagaagagaatcaaggcaatgggctttgccacagacagggaatacacagcgaacagggaaaggatcaggccccccttgcttgaggcttgctttcctcatctgtagatttaggggtctcaatcaggtcatctcaagttccctaaacttgcttaaaaagcatcaaactttgagttagaccttcagacttccctaactccttttttcctgaattaagctatgacaaagatgaccatatgtcccagttcacctagtataatctcgatttatatctgttgtcctggaataacaattaattgctcctcctttaactctcaaaggtatctccagtcggaagataaattacatgcccctcatacctatgactatattcattttaatcttggtttagatttttaagaaaacacactaatttacttttaagcctacaaatatagcatttcatagcttgctttctcttaacacttggagaaatttcagattcttttgtgagtggtttgtgaactatcaaaaatttttttaacttggccgggcatgatgacctatgcctctaatcccagtactttggaaggctgaggcagaagaatcgcttaagatgggaagtttgcggctgcagtgagctacgatcacgccactacacttcagcctgggtgatgcagaaaggaccgtgtctctagaaataaaaataattttttaaaaactgagtaagtcaaatgtaaattttccttttcaaaaacaaattattcagtatgcaaaacattctgttaagacatattttctgataaccttagaatacgtggtacttaaaaactatgactaaaatatttgtggaagaattcattatcttaggtgatacattttaacaattaaaatagttccagaacacggtcttccacctgactttgacgattaaaacaatgttgtcaaaagaatgttctctctgaaaattctgggtctcatccaccaccataggtctcatctaccatcaactgaaataagctaatcagttataaacaagggaatatacttaaaaaaaaaaaaaagagagaaacacggtctcactctgtctccaaggctggagtgcagtggcacagtcatagctcactgcagcacagaactcctaagctcaggcaatactcccacctcagcttcccaggaatataccacttttactgcactgacaagctctgtatgctagtgattctcaaattttctttaaggctaggaccaagagtcctgccaatcccctgaacaacagctcacatattatcaaatgaacttgaaacattcctgtcatagtgagcagcattgaaacagattccataactgattactcagtttcaagggagatttaacattgctttgttttcaagttacaaaaagttccctagttttactcaaatatgcactatccctgattaaaaaaaacatgtttcattatgaagaggggtgatttgtttcagcatttttttttttcacttaaccacttaagtcactgcctgaggaagtttctttttaaggaaataaataccaggttcattagaagaaaaaaaaaaaacacataattttaattcattttgttttaaagatgcgtattttaaaaagactactttaaaatgaactaatatgttacactggatcatgctgtggcgactaacgtattgtcaagccttaacctaatgaaaacaaaagaaaagcgagtttggcactcacttgcacttttcatctctgttagaaagtatgtctcagtttggatctgagatcaggtttgcttggtaacctcaaagaataattttccttttttttttctttcaaaatttccttttgatcatttcagacagttcatccttttgagtgagaaagagtaaaagagaggaatgttgagtgaggttaagtaaatggagaatctgtcacataaagcaagtttaaatcctagtaagagcatccatgcaggacaaacggaagcattattcttttgaaaacattattcttttaaacagtgtgtaatgacatcctccctagagactttccatgagaggggaaaaaaattacttcctcagaagtcgttttctagattccaagcataataagtgaagcacagttaaaagtcaaacttgtgttttctttatgcaagaaggttcaaattagaactgcagaaaggtacttaaaagtttctctagcttgtcttttggttacatactggtattgctgtgaactaaaagagcaagtaagaggaaaggttactgttgttactttacacctataaatcagtgagtgtgtccttactgtaaaatttgagctgaacatattttgtttcaaaggagaaatatatgactcaaatatgctgaatgtatgataatttattaagttccttttaagtatatcattttcttatgctcaagtagaaactatggattatttttctagtattctatgctgctgttaccttctgaggagttgattgaaaattttatgcttttaaaagttgggtgctacttaaatatcagaattggctattgttttaaatatttaaaatatgcttaaacaacaattaaggttaataagcagagaaaatacttcttttgattcaaacactactttatatatttaatgaatacacgtccaaataaagatctctcttcaaaaattttggaaaatgttaatgcattttgaatataatggaacaaagaagaagaatactagagaaaattcacaattatgatgtttatttaggaaaataaacttgaagaaggttttctattaaaaaaacataagaatcatatccaaattttagactctccatcttctttggtatgaaaatcaacattcataatagaaaatattttcttttgaaaggtttagttgttattgggtctataacggttttccatataaggaaaatacagtattatctgtaatcatctcacttattgaacaaccaatgaatgcatgcaagtaaccaagcatatgtgtgcagagaccagcatcaaggaaatattcattcatagataaatgttttctaataaaatatattttaagtttttaatgatcttctgctatcattttttgccatgttatctgaatagccatccagatctgtagtaaaacatcctgttagttacataactcaagaagtacttccccaaggaagctcacaccatcataccaggacttagcaacatttatctttcaacatgagtataccattaaaatttttttatatttctcagaattgtattcttcagtcttttccacaatatagtatatggaaattgctaatagcattaaattaatattaataaaacccaattctatctaaacctttttctcataagaaaaaacattactttaaaaaatagactttttgtttcttctaaaagtagtactatatggactgctcaattagcaatgccaaatacttccaaaaacaccataggaccaccaagctatttctattgctttgataatttcttttcctgctccaatttctccacgttcctgctttcttgtgtcaaaatatcttcccttaatttgttaaaatgaatctgagggaaaaaaatctgataatctggggtaaagaaatttttttttttgcatagactcttgtgatcacaaaatgaccaggtaatttatagcttcagtgctaacactgtgattgggaacaagaagagtacaaccataataaaatacagctatctatgagaagaactgcataaagacatctttggccatgtaggctctgggccctctggaaataagtcagttgcattgccaacatgacaaagaaaatagcaatgttcagaatcaggaacaacctggtataggaagcagacagtgatggggccctgctgtgtgtagttgtcaccatccgtgcctgtccaaaccggcctttaatcaagcccccatttttatgtttctcgtatgttacatctgcaaaatctaaaaggtctttcatttcttcatcttcatctatgggtagttctttctgtgccaaaatctgagctttctgtctaatctttttctcattgacttcaatctgtgcaaaaatatcagggacagcatccacaaatttatagcgtttgcctgcccttcggtttttctttgacttgctttgctgctgctgttgctgtgatatggcaaaaatcctgtcaatggcctcctcagtctgtctcttatctgaaaatctcagcaggcgttcagcagtcttcctaaagctagctgtgttccggactcgggacagtatctgcttctccagcagctgaaacactggtttaaaatgctgcaagttctgttccacaatagcagcatagtccttcacctcagggacaatgctgctcttgatggctgaattccggtcaaacagaattttgtgacgatcagcaatgacctgtgcaaaggcagactgtcctgtggcctcacctgtccacaggtatgtggcgtaggcatgtttgctggtggctatgaacacatccagttgctgagagtctccgtggacagtgaagctctgaacatctatagatggccctatgaagaggtaagctgccctggtgatgggacttcggaggtgcatggtgacattcacatagtttgtcccattgtagggatagccccgaggatatgtcactgaggcaaaggttgctttctcgctgtagccagtatcgtccatccagtacattttatagagaccatctctctgcctgatgaaagccccatggacaccatctaccacagtctcctcaaaaggaacatccacattatggaagaagctcgctgctgtctccaagggactctcctctcccaggtgtatttggtctacaaggagaagcagctgtggatgtaggaggatgagattcctctgaacattcttcaggttgagctgggggttataagctcccacaccttctcctcggatgaaaaccaccccatttttctcctctgctgcaaccaccctcccctgacaactagctgccaggtcatgcttgtatttagaccattttgatgagcagtcttctgtgacctgacccacccagggagaaaagcagctctttgacacagctggggaaaacatcaaaacattgttgaagaaggtgtactttggcccgtacagagcctcagtaatgaaaggcacaccattgggagcaaaagtaaatgagttttgatcaggatgttcatgccctgcattaaaatttctccatcctttgatccaatctttgtatttgtttctgtggacaatgtcatatattgcacgtccccccagttttccagacttgaaggaaaggaaagatctattgatttctgcaggtagtgcacttccataagtcacgacaccccagtcttcaaaataatgcagtgtaggggtgccaaagtctggaggaggaaccgatttcaagctgccatcatacctggcaggatggttctatacataaatgcaaagtgttgtttaagccacggatggccaaagtggttgatgttgaagtgcctctggacgagaaacatgtattggaagagtgatctagtggtgtagctgccatacgcaactccttcatagagggagccatccgtcacctccctgagcaagaccagagatttctccatgatggtcagaacttgtttggtccataagtaggcttcttgaagatatccttgattcatcaggactaggcttcccgtgagcaaagccatacagttggtgggctgatgattgtgcaggtattgaaatccccatcctctcctgtatgaagtttcatacatataccctgaggcattggcaatcacttcaagaaacttctcctgttgtgtcttgctcaggtagttgtacaagaagtcataagcagtggcaaaaccaaccagggagtgagcaagcgggacctcatcccaaggagcatctttcaccaaccaactaggctgcgctgccatcctctccatgtagtctttggccatgtctcgggcttcaatgttctcaggatacagcacacagaacattgccaaggcacccaagttgtttccaaaaatttcattccagcgggcactgtagtccttgggatcccagggagggaggtattccaaggggctggacagcatcgtgtgcacagcctccgtgaggcgggctgcaatgtgctcgtgcgagctggcagccctgagctgcagctccgccacttctgccctggagaagtacagcatgggatggctgtcgtagttggcattggtgaagggaatcataacttctgggttctcgtcggtgatgtaggctgacacaaagcaaagcaaatatatgaaaaacacactgggagccccccgtgtgtgagtcctcatcgtggcatcagatctccaaatctccaaggcagccaaaccatcttcgaaagatccgctcccagccgaggcttcgttctctccggcgtcgcctccgcagcctccagagccagctcccggtcctcctcactccagggcgcccgggctcccggccccctccgaaccgagccctccgcgcccccgccgcgccatgccccgggatgcgctgctgcagcctcgggcgacgctact

SEQ ID NO: 18015 - RNA, 9071 nt, Homo sapiens
  source 1..9071: mol_type = other RNA
tctgagttcctggagcctggtctacttttccagtctaattttctatcacccgccactacatacacaccctgtactccagttataccattctatgtgaagtccctgaacaaggcaagctgaaaacacaaatggcagaaatatttgaacaatttcctgggcttattaagggatagccagggtgacggcagcagagccatggcaggcaaccatgctcttcttatattaaataagactcagacatatataccattagggatccttgactcattatctttctgatcaatacttccacaaaatattcattcctttggccacacattttgcctgtgggctaggagttaaacattccctctccagacttattcaaggagctaattgtcttctacccagactatggaaatggtctcctaacctcttccccattgggtccactctctacactgaagctaaaattgcctttctaaaatgcaaatctgattatttaaaaagaaaattctttaatggcttgccattgcttgcagcgatttctaagcagagggtaccccctccctgccccacctcaccccagggagtaaacatatggaatatggggggcatatcagagccatctcagggatttttcaaagtttcacatacacacaggtatatgtggcatcatcaacacccctcacccatgtcccttttgctcccatacacatttcctatcccatgaaaatcgctgccatgcttgttgagtgatgggtgttatgttgtagccctcagttatgctgaggcataaaaatggttgagcagcctcatggcagaataaagtccagattccttagcatgtcctacaaagtcctgcacaatagcctccctgcttgccttttcagtttcatcttcacccattctccatcacacaccctgtgggccaacaccaccagtctggagaattcctgaaccaggtttgctttttcgtacttttttctttattctattccatttacccagaatgcacttctcctctcacacagctagtaaatttctgtttaacctttaagaaggcaccaacaattacatcttcagccacagcctgcccctggattccaggctggtacatctccacttggatttttagaaagtatcttaaacttaacatggctaaaacaacctcctggacccgcttcctactacttattcctcctgcagtcagccacatctcagttcattgcaactgactccccaactcataatccaagtctttgctgcagtctgtgagagcatgtatgatctgatcctattcctatcaccctcccctcccccactctgctctagccacactggcctcctagtcctaaatacaccaaacacatactgagctcagggccttcgaactgctgttctatctggaatgctcctctctcttagatgtccctgtgattcattcccttatttctttcaagtgtctgatcataagtaatcacatcagaaaccactgtttatgggacagtaccaattcaccatcaccttacatcccctccccttgctttattctccacagtacttaccactacttgacatcctgcactattactgttattatttgctcccactagaacataaactatacaagggccagcttttattattcctattctctaccatatcttcagttcctaaaacaatacttggcatatagtagatgctctgtaaacatgttattgtcattcgttatttgttaactcaactgaaaagtgctgtgggacttccatttaaacatactgcactcaatatataaatttccttcagttccttcctaaaaccccattaaattaacagcaaatagattttcaaaatgacacagagaatggaagtggagacatcaataaagcctaacctgatcaccacatttaaaattatggcctcctcttcccagtctccttaccctgacttttccttccatagcacctattatcttccaataagtataaagaatgggtaagagagctaaagcttcattagtaggcagttttagaccttattgtaaacaagtacacaatatatgtaacagccaaaagaattagaaattggttacttctgggaagtacaaactaagaatgagaggggaagggacagataatttattgttttgttttttaaataaggcttctagtactatactttttcaatcatgtatgttcataatttatgccaaataaaacttcaattaaaaaaatcccaaaaccaagagggaaactgtatatgcaagaagaaaagtcataatgcaactttgtctatttttattcttcacatagtgactatgtcttgtttaacagaatttgaacatattaaaatagatgaccaaatactaaatatttagactatgtagtggaacacatgatttatatcagtcatttcttgaaaacttatgagtacttcattgacattacatgcataaagcaaatatctagctgaaacattgctgaaaaaaaaatacgtcattttgccagtaaattaaataaactgcagaaagaaactacttctcaacatgaaagtaaagagaagagaatcaaggcaatgggctttgccacagacagggaatacacagcgaacagggaaaggatcaggccccccttgcttgaggcttgctttcctcatctgtagatttaggggtctcaatcaggtcatctcaagttccctaaacttgcttaaaaagcatcaaactttgagttagaccttcagacttccctaactccttttttcctgaattaagctatgacaaagatgaccatatgtcccagttcacctagtataatctcgatttatatctgttgtcctggaataacaattaattgctcctcctttaactctcaaaggtatctccagtcggaagataaattacatgcccctcatacctatgactatattcattttaatcttggtttagatttttaagaaaacacactaatttacttttaagcctacaaatatagcatttcatagcttgctttctcttaacacttggagaaatttcagattcttttgtgagtggtttgtgaactatcaaaaatttttttaacttggccgggcatgatgacctatgcctctaatcccagtactttggaaggctgaggcagaagaatcgcttaagatgggaagtttgcggctgcagtgagctacgatcacgccactacacttcagcctgggtgatgcagaaaggaccgtgtctctagaaataaaaataattttttaaaaactgagtaagtcaaatgtaaattttccttttcaaaaacaaattattcagtatgcaaaacattctgttaagacatattttctgataaccttagaatacgtggtacttaaaaactatgactaaaatatttgtggaagaattcattatcttaggtgatacattttaacaattaaaatagttccagaacacggtcttccacctgactttgacgattaaaacaatgttgtcaaaagaatgttctctctgaaaattctgggtctcatccaccaccataggtctcatctaccatcaactgaaataagctaatcagttataaacaagggaatatacttaaaaaaaaaaaaaagagagaaacacggtctcactctgtctccaaggctggagtgcagtggcacagtcatagctcactgcagcacagaactcctaagctcaggcaatactcccacctcagcttcccaggaatataccacttttactgcactgacaagctctgtatgctagtgattctcaaattttctttaaggctaggaccaagagtcctgccaatcccctgaacaacagctcacatattatcaaatgaacttgaaacattcctgtcatagtgagcagcattgaaacagattccataactgattactcagtttcaagggagatttaacattgctttgttttcaagttacaaaaagttccctagttttactcaaatatgcactatccctgattaaaaaaaacatgtttcattatgaagaggggtgatttgtttcagcatttttttttttcacttaaccacttaagtcactgcctgaggaagtttctttttaaggaaataaataccaggttcattagaagaaaaaaaaaaaacacataattttaattcattttgttttaaagatgcgtattttaaaaagactactttaaaatgaactaatatgttacactggatcatgctgtggcgactaacgtattgtcaagccttaacctaatgaaaacaaaagaaaagcgagtttggcactcacttgcacttttcatctctgttagaaagtatgtctcagtttggatctgagatcaggtttgcttggtaacctcaaagaataattttccttttttttttctttcaaaatttccttttgatcatttcagacagttcatccttttgagtgagaaagagtaaaagagaggaatgttgagtgaggttaagtaaatggagaatctgtcacataaagcaagtttaaatcctagtaagagcatccatgcaggacaaacggaagcattattcttttgaaaacattattcttttaaacagtgtgtaatgacatcctccctagagactttccatgagaggggaaaaaaattacttcctcagaagtcgttttctagattccaagcataataagtgaagcacagttaaaagtcaaacttgtgttttctttatgcaagaaggttcaaattagaactgcagaaaggtacttaaaagtttctctagcttgtcttttggttacatactggtattgctgtgaactaaaagagcaagtaagaggaaaggttactgttgttactttacacctataaatcagtgagtgtgtccttactgtaaaatttgagctgaacatattttgtttcaaaggagaaatatatgactcaaatatgctgaatgtatgataatttattaagttccttttaagtatatcattttcttatgctcaagtagaaactatggattatttttctagtattctatgctgctgttaccttctgaggagttgattgaaaattttatgcttttaaaagttgggtgctacttaaatatcagaattggctattgttttaaatatttaaaatatgcttaaacaacaattaaggttaataagcagagaaaatacttcttttgattcaaacactactttatatatttaatgaatacacgtccaaataaagatctctcttcaaaaattttggaaaatgttaatgcattttgaatataatggaacaaagaagaagaatactagagaaaattcacaattatgatgtttatttaggaaaataaacttgaagaaggttttctattaaaaaaacataagaatcatatccaaattttagactctccatcttctttggtatgaaaatcaacattcataatagaaaatattttcttttgaaaggtttagttgttattgggtctataacggttttccatataaggaaaatacagtattatctgtaatcatctcacttattgaacaaccaatgaatgcatgcaagtaaccaagcatatgtgtgcagagaccagcatcaaggaaatattcattcatagataaatgttttctaataaaatatattttaagtttttaatgatcttctgctatcattttttgccatgttatctgaatagccatccagatctgtagtaaaacatcctgttagttacataactcaagaagtacttccccaaggaagctcacaccatcataccaggacttagcaacatttatctttcaacatgagtataccattaaaatttttttatatttctcagaattgtattcttcagtcttttccacaatatagtatatggaaattgctaatagcattaaattaatattaataaaacccaattctatctaaacctttttctcataagaaaaaacattactttaaaaaatagactttttgtttcttctaaaagtagtactatatggactgctcaattagcaatgccaaatacttccaaaaacaccataggaccaccaagctatttctattgctttgataatttcttttcctgctccaatttctccacgttcctgctttcttgtgtcaaaatatcttcccttaatttgttaaaatgaatctgagggaaaaaaatctgataatctggggtaaagaaatttttttttttgcatagactcttgtgatcacaaaatgaccaggtaatttatagcttcagtgctaacactgtgattgggaacaagaagagtacaaccataataaaatacagctatctatgagaagaactgcataaagacatctttggccatgtaggctctgggccctctggaaataagtcagttgcattgccaacatgacaaagaaaatagcaatgttcagaatcaggaacaacctggtataggaagcagacagtgatggggccctgctgtgtgtagttgtcaccatccgtgcctgtccaaaccggcctttaatcaagcccccatttttatgtttctcgtatgttacatctgcaaaatctaaaaggtctttcatttcttcatcttcatctatgggtagttctttctgtgccaaaatctgagctttctgtctaatctttttctcattgacttcaatctgtgcaaaaatatcagggacagcatccacaaatttatagcgtttgcctgcccttcggtttttctttgacttgctttgctgctgctgttgctgtgatatggcaaaaatcctgtcaatggcctcctcagtctgtctcttatctgaaaatctcagcaggcgttcagcagtcttcctaaagctagctgtgttccggactcgggacagtatctgcttctccagcagctgaaacactggtttaaaatgctgcaagttctgttccacaatagcagcatagtccttcacctcagggacaatgctgctcttgatggctgaattccggtcaaacagaattttgtgacgatcagcaatgacctgtgcaaaggcagactgtcctgtggcctcacctgtccacaggtatgtggcgtaggcatgtttgctggtggctatgaacacatccagttgctgagagtctccgtggacagtgaagctctgaacatctatagatggccctatgaagaggtaagctgccctggtgatgggacttcggaggtgcatggtgacattcacatagtttgtcccattgtagggatagccccgaggatatgtcactgaggcaaaggttgctttctcgctgtagccagtatcgtccatccagtacattttatagagaccatctctctgcctgatgaaagccccatggacaccatctaccacagtctcctcaaaaggaacatccacattatggaagaagctcgctgctgtctccaagggactctcctctcccaggtgtatttggtctacaaggagaagcagctgtggatgtaggaggatgagattcctctgaacattcttcaggttgagctgggggttataagctcccacaccttctcctcggatgaaaaccaccccatttttctcctctgctgcaaccaccctcccctgacaactagctgccaggtcatgcttgtatttagaccattttgatgagcagtcttctgtgacctgacccacccagggagaaaagcagctctttgacacagctggggaaaacatcaaaacattgttgaagaaggtgtactttggcccgtacagagcctcagtaatgaaaggcacaccattgggagcaaaagtaaatgagttttgatcaggatgttcatgccctgcattaaaatttctccatcctttgatccaatctttgtatttgtttctgtggacaatgtcatatattgcacgtccccccagttttccagacttgaaggaaaggaaagatctattgatttctgcaggtagtgcacttccataagtcacgacaccccagtcttcaaaataatgcagtgtaggggtgccaaagtctggaggaggaaccgatttcaagctgccatcatacctggcaggatggttctatacataaatgcaaagtgttgtttaagccacggatggccaaagtggttgatgttgaagtgcctctggacgagaaacatgtattggaagagtgatctagtggtgtagctgccatacgcaactccttcatagagggagccatccgtcacctccctgagcaagaccagagatttctccatgatggtcagaacttgtttggtccataagtaggcttcttgaagatatccttgattcatcaggactaggcttcccgtgagcaaagccatacagttggtgggctgatgattgtgcaggtattgaaatccccatcctctcctgtatgaagtttcatacatataccctgaggcattggcaatcacttcaagaaacttctcctgttgtgtcttgctcaggtagttgtacaagaagtcataagcagtggcaaaaccaaccagggagtgagcaagcgggacctcatcccaaggagcatctttcaccaactaggctgcgctgccatcctctccatgtagtctttggccatgtctcgggcttcaatgttctcaggatacagcacacagaacattgccaaggcacccaagttgtttccaaaaatttcattccagcgggcactgtagtccttgggatcccagggagggaggtattccaaggggctggacagcatcgtgtgcacagcctccgtgaggcgggctgcaatgtgctcgtgcgagctggcagccctgagctgcagctccgccacttctgccctggagaagtacagcatgggatggctgtcgtagttggcattggtgaagggaatcataacttctgggttctcgtcggtgatgtaggctgacacaaagcaaagcaaatatatgaaaaacacactgggagccccccgtgtgtgagtcctcatcgtggcatcagatctccaaatctccaaggcagccaaaccatcttcgaaagatccttcctgcctcaaaaaagtgaagaccagaaaaacatttgttttcagacactggagagcaggcactgttacggctgtgattttacaactgctcctacatgctgggagcagtcgctagatgcatctcaaggtgggtcgtccgcgcttccagactcagcacaatcgacatttatttac

SEQ ID NO: 18016 - RNA, 8835 nt, Homo sapiens
  source 1..8835: mol_type = other RNA
tctgagttcctggagcctggtctacttttccagtctaattttctatcacccgccactacatacacaccctgtactccagttataccattctatgtgaagtccctgaacaaggcaagctgaaaacacaaatggcagaaatatttgaacaatttcctgggcttattaagggatagccagggtgacggcagcagagccatggcaggcaaccatgctcttcttatattaaataagactcagacatatataccattagggatccttgactcattatctttctgatcaatacttccacaaaatattcattcctttggccacacattttgcctgtgggctaggagttaaacattccctctccagacttattcaaggagctaattgtcttctacccagactatggaaatggtctcctaacctcttccccattgggtccactctctacactgaagctaaaattgcctttctaaaatgcaaatctgattatttaaaaagaaaattctttaatggcttgccattgcttgcagcgatttctaagcagagggtaccccctccctgccccacctcaccccagggagtaaacatatggaatatggggggcatatcagagccatctcagggatttttcaaagtttcacatacacacaggtatatgtggcatcatcaacacccctcacccatgtcccttttgctcccatacacatttcctatcccatgaaaatcgctgccatgcttgttgagtgatgggtgttatgttgtagccctcagttatgctgaggcataaaaatggttgagcagcctcatggcagaataaagtccagattccttagcatgtcctacaaagtcctgcacaatagcctccctgcttgccttttcagtttcatcttcacccattctccatcacacaccctgtgggccaacaccaccagtctggagaattcctgaaccaggtttgctttttcgtacttttttctttattctattccatttacccagaatgcacttctcctctcacacagctagtaaatttctgtttaacctttaagaaggcaccaacaattacatcttcagccacagcctgcccctggattccaggctggtacatctccacttggatttttagaaagtatcttaaacttaacatggctaaaacaacctcctggacccgcttcctactacttattcctcctgcagtcagccacatctcagttcattgcaactgactccccaactcataatccaagtctttgctgcagtctgtgagagcatgtatgatctgatcctattcctatcaccctcccctcccccactctgctctagccacactggcctcctagtcctaaatacaccaaacacatactgagctcagggccttcgaactgctgttctatctggaatgctcctctctcttagatgtccctgtgattcattcccttatttctttcaagtgtctgatcataagtaatcacatcagaaaccactgtttatgggacagtaccaattcaccatcaccttacatcccctccccttgctttattctccacagtacttaccactacttgacatcctgcactattactgttattatttgctcccactagaacataaactatacaagggccagcttttattattcctattctctaccatatcttcagttcctaaaacaatacttggcatatagtagatgctctgtaaacatgttattgtcattcgttatttgttaactcaactgaaaagtgctgtgggacttccatttaaacatactgcactcaatatataaatttccttcagttccttcctaaaaccccattaaattaacagcaaatagattttcaaaatgacacagagaatggaagtggagacatcaataaagcctaacctgatcaccacatttaaaattatggcctcctcttcccagtctccttaccctgacttttccttccatagcacctattatcttccaataagtataaagaatgggtaagagagctaaagcttcattagtaggcagttttagaccttattgtaaacaagtacacaatatatgtaacagccaaaagaattagaaattggttacttctgggaagtacaaactaagaatgagaggggaagggacagataatttattgttttgttttttaaataaggcttctagtactatactttttcaatcatgtatgttcataatttatgccaaataaaacttcaattaaaaaaatcccaaaaccaagagggaaactgtatatgcaagaagaaaagtcataatgcaactttgtctatttttattcttcacatagtgactatgtcttgtttaacagaatttgaacatattaaaatagatgaccaaatactaaatatttagactatgtagtggaacacatgatttatatcagtcatttcttgaaaacttatgagtacttcattgacattacatgcataaagcaaatatctagctgaaacattgctgaaaaaaaaatacgtcattttgccagtaaattaaataaactgcagaaagaaactacttctcaacatgaaagtaaagagaagagaatcaaggcaatgggctttgccacagacagggaatacacagcgaacagggaaaggatcaggccccccttgcttgaggcttgctttcctcatctgtagatttaggggtctcaatcaggtcatctcaagttccctaaacttgcttaaaaagcatcaaactttgagttagaccttcagacttccctaactccttttttcctgaattaagctatgacaaagatgaccatatgtcccagttcacctagtataatctcgatttatatctgttgtcctggaataacaattaattgctcctcctttaactctcaaaggtatctccagtcggaagataaattacatgcccctcatacctatgactatattcattttaatcttggtttagatttttaagaaaacacactaatttacttttaagcctacaaatatagcatttcatagcttgctttctcttaacacttggagaaatttcagattcttttgtgagtggtttgtgaactatcaaaaatttttttaacttggccgggcatgatgacctatgcctctaatcccagtactttggaaggctgaggcagaagaatcgcttaagatgggaagtttgcggctgcagtgagctacgatcacgccactacacttcagcctgggtgatgcagaaaggaccgtgtctctagaaataaaaataattttttaaaaactgagtaagtcaaatgtaaattttccttttcaaaaacaaattattcagtatgcaaaacattctgttaagacatattttctgataaccttagaatacgtggtacttaaaaactatgactaaaatatttgtggaagaattcattatcttaggtgatacattttaacaattaaaatagttccagaacacggtcttccacctgactttgacgattaaaacaatgttgtcaaaagaatgttctctctgaaaattctgggtctcatccaccaccataggtctcatctaccatcaactgaaataagctaatcagttataaacaagggaatatacttaaaaaaaaaaaaaagagagaaacacggtctcactctgtctccaaggctggagtgcagtggcacagtcatagctcactgcagcacagaactcctaagctcaggcaatactcccacctcagcttcccaggaatataccacttttactgcactgacaagctctgtatgctagtgattctcaaattttctttaaggctaggaccaagagtcctgccaatcccctgaacaacagctcacatattatcaaatgaacttgaaacattcctgtcatagtgagcagcattgaaacagattccataactgattactcagtttcaagggagatttaacattgctttgttttcaagttacaaaaagttccctagttttactcaaatatgcactatccctgattaaaaaaaacatgtttcattatgaagaggggtgatttgtttcagcatttttttttttcacttaaccacttaagtcactgcctgaggaagtttctttttaaggaaataaataccaggttcattagaagaaaaaaaaaaaacacataattttaattcattttgttttaaagatgcgtattttaaaaagactactttaaaatgaactaatatgttacactggatcatgctgtggcgactaacgtattgtcaagccttaacctaatgaaaacaaaagaaaagcgagtttggcactcacttgcacttttcatctctgttagaaagtatgtctcagtttggatctgagatcaggtttgcttggtaacctcaaagaataattttccttttttttttctttcaaaatttccttttgatcatttcagacagttcatccttttgagtgagaaagagtaaaagagaggaatgttgagtgaggttaagtaaatggagaatctgtcacataaagcaagtttaaatcctagtaagagcatccatgcaggacaaacggaagcattattcttttgaaaacattattcttttaaacagtgtgtaatgacatcctccctagagactttccatgagaggggaaaaaaattacttcctcagaagtcgttttctagattccaagcataataagtgaagcacagttaaaagtcaaacttgtgttttctttatgcaagaaggttcaaattagaactgcagaaaggtacttaaaagtttctctagcttgtcttttggttacatactggtattgctgtgaactaaaagagcaagtaagaggaaaggttactgttgttactttacacctataaatcagtgagtgtgtccttactgtaaaatttgagctgaacatattttgtttcaaaggagaaatatatgactcaaatatgctgaatgtatgataatttattaagttccttttaagtatatcattttcttatgctcaagtagaaactatggattatttttctagtattctatgctgctgttaccttctgaggagttgattgaaaattttatgcttttaaaagttgggtgctacttaaatatcagaattggctattgttttaaatatttaaaatatgcttaaacaacaattaaggttaataagcagagaaaatacttcttttgattcaaacactactttatatatttaatgaatacacgtccaaataaagatctctcttcaaaaattttggaaaatgttaatgcattttgaatataatggaacaaagaagaagaatactagagaaaattcacaattatgatgtttatttaggaaaataaacttgaagaaggttttctattaaaaaaacataagaatcatatccaaattttagactctccatcttctttggtatgaaaatcaacattcataatagaaaatattttcttttgaaaggtttagttgttattgggtctataacggttttccatataaggaaaatacagtattatctgtaatcatctcacttattgaacaaccaatgaatgcatgcaagtaaccaagcatatgtgtgcagagaccagcatcaaggaaatattcattcatagataaatgttttctaataaaatatattttaagtttttaatgatcttctgctatcattttttgccatgttatctgaatagccatccagatctgtagtaaaacatcctgttagttacataactcaagaagtacttccccaaggaagctcacaccatcataccaggacttagcaacatttatctttcaacatgagtataccattaaaatttttttatatttctcagaattgtattcttcagtcttttccacaatatagtatatggaaattgctaatagcattaaattaatattaataaaacccaattctatctaaacctttttctcataagaaaaaacattactttaaaaaatagactttttgtttcttctaaaagtagtactatatggactgctcaattagcaatgccaaatacttccaaaaacaccataggaccaccaagctatttctattgctttgataatttcttttcctgctccaatttctccacgttcctgctttcttgtgtcaaaatatcttcccttaatttgttaaaatgaatctgagggaaaaaaatctgataatctggggtaaagaaatttttttttttgcatagactcttgtgatcacaaaatgaccaggtaatttatagcttcagtgctaacactgtgattgggaacaagaagagtacaaccataataaaatacagctatctatgagaagaactgcataaagacatctttggccatgtaggctctgggccctctggaaataagtcagttgcattgccaacatgacaaagaaaatagcaatgttcagaatcaggaacaacctggtataggaagcagacagtgatggggccctgctgtgtgtagttgtcaccatccgtgcctgtccaaaccggcctttaatcaagcccccatttttatgtttctcgtatgttacatctgcaaaatctaaaaggtctttcatttcttcatcttcatctatgggtagttctttctgtgccaaaatctgagctttctgtctaatctttttctcattgacttcaatctgtgcaaaaatatcagggacagcatccacaaatttatagcgtttgcctgcccttcggtttttctttgacttgctttgctgctgctgttgctgtgatatggcaaaaatcctgtcaatggcctcctcagtctgtctcttatctgaaaatctcagcaggcgttcagcagtcttcctaaagctagctgtgttccggactcgggacagtatctgcttctccagcagctgaaacactggtttaaaatgctgcaagttctgttccacaatagcagcatagtccttcacctcagggacaatgctgctcttgatggctgaattccggtcaaacagaattttgtgacgatcagcaatgacctgtgcaaaggcagactgtcctgtggcctcacctgtccacaggtatgtggcgtaggcatgtttgctggtggctatgaacacatccagttgctgagagtctccgtggacagtgaagctctgaacatctatagatggccctatgaagaggtaagctgccctggtgatgggacttcggaggtgcatggtgacattcacatagtttgtcccattgtagggatagccccgaggatatgtcactgaggcaaaggttgctttctcgctgtagccagtatcgtccatccagtacattttatagagaccatctctctgcctgatgaaagccccatggacaccatctaccacagtctcctcaaaaggaacatccacattatggaagaagctcgctgctgtctccaagggactctcctctcccaggtgtatttggtctacaaggagaagcagctgtggatgtaggaggatgagattcctctgaacattcttcaggttgagctgggggttataagctcccacaccttctcctcggatgaaaaccaccccatttttctcctctgctgcaaccaccctcccctgacaactagctgccaggtcatgcttgtatttagaccattttgatgagcagtcttctgtgacctgacccacccagggagaaaagcagctctttgacacagctggggaaaacatcaaaacattgttgaagaaggtgtactttggcccgtacagagcctcagtaatgaaaggcacaccattgggagcaaaagtaaatgagttttgatcaggatgttcatgccctgcattaaaatttctccatcctttgatccaatctttgtatttgtttctgtggacaatgtcatatattgcacgtccccccagttttccagacttgaaggaaaggaaagatctattgatttctgcaggtagtgcacttccataagtcacgacaccccagtcttcaaaataatgcagtgtaggggtgccaaagtctggaggaggaaccgatttcaagctgccatcataccttgattcatcaggactaggcttcccgtgagcaaagccatacagttggtgggctgatgattgtgcaggtattgaaatccccatcctctcctgtatgaagtttcatacatataccctgaggcattggcaatcacttcaagaaacttctcctgttgtgtcttgctcaggtagttgtacaagaagtcataagcagtggcaaaaccaaccagggagtgagcaagcgggacctcatcccaaggagcatctttcaccaaccaactaggctgcgctgccatcctctccatgtagtctttggccatgtctcgggcttcaatgttctcaggatacagcacacagaacattgccaaggcacccaagttgtttccaaaaatttcattccagcgggcactgtagtccttgggatcccagggagggaggtattccaaggggctggacagcatcgtgtgcacagcctccgtgaggcgggctgcaatgtgctcgtgcgagctggcagccctgagctgcagctccgccacttctgccctggagaagtacagcatgggatggctgtcgtagttggcattggtgaagggaatcataacttctgggttctcgtcggtgatgtaggctgacacaaagcaaagcaaatatatgaaaaacacactgggagccccccgtgtgtgagtcctcatcgtggcatcagatctccaaatctccaaggcagccaaaccatcttcgaaagatccgctcccagccgaggcttcgttctctccggcgtcgcctccgcagcctccagagccagctcccggtcctcctcactccagggcgcccgggctcccggccccctccgaaccgagccctccgcgcccccgccgcgccatgccccgggatgcgctgctgcagcctcgggcgacgctact

SEQ ID NO: 18017 - RNA, 9395 nt, Homo sapiens
  source 1..9395: mol_type = other RNA
tctgagttcctggagcctggtctacttttccagtctaattttctatcacccgccactacatacacaccctgtactccagttataccattctatgtgaagtccctgaacaaggcaagctgaaaacacaaatggcagaaatatttgaacaatttcctgggcttattaagggatagccagggtgacggcagcagagccatggcaggcaaccatgctcttcttatattaaataagactcagacatatataccattagggatccttgactcattatctttctgatcaatacttccacaaaatattcattcctttggccacacattttgcctgtgggctaggagttaaacattccctctccagacttattcaaggagctaattgtcttctacccagactatggaaatggtctcctaacctcttccccattgggtccactctctacactgaagctaaaattgcctttctaaaatgcaaatctgattatttaaaaagaaaattctttaatggcttgccattgcttgcagcgatttctaagcagagggtaccccctccctgccccacctcaccccagggagtaaacatatggaatatggggggcatatcagagccatctcagggatttttcaaagtttcacatacacacaggtatatgtggcatcatcaacacccctcacccatgtcccttttgctcccatacacatttcctatcccatgaaaatcgctgccatgcttgttgagtgatgggtgttatgttgtagccctcagttatgctgaggcataaaaatggttgagcagcctcatggcagaataaagtccagattccttagcatgtcctacaaagtcctgcacaatagcctccctgcttgccttttcagtttcatcttcacccattctccatcacacaccctgtgggccaacaccaccagtctggagaattcctgaaccaggtttgctttttcgtacttttttctttattctattccatttacccagaatgcacttctcctctcacacagctagtaaatttctgtttaacctttaagaaggcaccaacaattacatcttcagccacagcctgcccctggattccaggctggtacatctccacttggatttttagaaagtatcttaaacttaacatggctaaaacaacctcctggacccgcttcctactacttattcctcctgcagtcagccacatctcagttcattgcaactgactccccaactcataatccaagtctttgctgcagtctgtgagagcatgtatgatctgatcctattcctatcaccctcccctcccccactctgctctagccacactggcctcctagtcctaaatacaccaaacacatactgagctcagggccttcgaactgctgttctatctggaatgctcctctctcttagatgtccctgtgattcattcccttatttctttcaagtgtctgatcataagtaatcacatcagaaaccactgtttatgggacagtaccaattcaccatcaccttacatcccctccccttgctttattctccacagtacttaccactacttgacatcctgcactattactgttattatttgctcccactagaacataaactatacaagggccagcttttattattcctattctctaccatatcttcagttcctaaaacaatacttggcatatagtagatgctctgtaaacatgttattgtcattcgttatttgttaactcaactgaaaagtgctgtgggacttccatttaaacatactgcactcaatatataaatttccttcagttccttcctaaaaccccattaaattaacagcaaatagattttcaaaatgacacagagaatggaagtggagacatcaataaagcctaacctgatcaccacatttaaaattatggcctcctcttcccagtctccttaccctgacttttccttccatagcacctattatcttccaataagtataaagaatgggtaagagagctaaagcttcattagtaggcagttttagaccttattgtaaacaagtacacaatatatgtaacagccaaaagaattagaaattggttacttctgggaagtacaaactaagaatgagaggggaagggacagataatttattgttttgttttttaaataaggcttctagtactatactttttcaatcatgtatgttcataatttatgccaaataaaacttcaattaaaaaaatcccaaaaccaagagggaaactgtatatgcaagaagaaaagtcataatgcaactttgtctatttttattcttcacatagtgactatgtcttgtttaacagaatttgaacatattaaaatagatgaccaaatactaaatatttagactatgtagtggaacacatgatttatatcagtcatttcttgaaaacttatgagtacttcattgacattacatgcataaagcaaatatctagctgaaacattgctgaaaaaaaaatacgtcattttgccagtaaattaaataaactgcagaaagaaactacttctcaacatgaaagtaaagagaagagaatcaaggcaatgggctttgccacagacagggaatacacagcgaacagggaaaggatcaggccccccttgcttgaggcttgctttcctcatctgtagatttaggggtctcaatcaggtcatctcaagttccctaaacttgcttaaaaagcatcaaactttgagttagaccttcagacttccctaactccttttttcctgaattaagctatgacaaagatgaccatatgtcccagttcacctagtataatctcgatttatatctgttgtcctggaataacaattaattgctcctcctttaactctcaaaggtatctccagtcggaagataaattacatgcccctcatacctatgactatattcattttaatcttggtttagatttttaagaaaacacactaatttacttttaagcctacaaatatagcatttcatagcttgctttctcttaacacttggagaaatttcagattcttttgtgagtggtttgtgaactatcaaaaatttttttaacttggccgggcatgatgacctatgcctctaatcccagtactttggaaggctgaggcagaagaatcgcttaagatgggaagtttgcggctgcagtgagctacgatcacgccactacacttcagcctgggtgatgcagaaaggaccgtgtctctagaaataaaaataattttttaaaaactgagtaagtcaaatgtaaattttccttttcaaaaacaaattattcagtatgcaaaacattctgttaagacatattttctgataaccttagaatacgtggtacttaaaaactatgactaaaatatttgtggaagaattcattatcttaggtgatacattttaacaattaaaatagttccagaacacggtcttccacctgactttgacgattaaaacaatgttgtcaaaagaatgttctctctgaaaattctgggtctcatccaccaccataggtctcatctaccatcaactgaaataagctaatcagttataaacaagggaatatacttaaaaaaaaaaaaaagagagaaacacggtctcactctgtctccaaggctggagtgcagtggcacagtcatagctcactgcagcacagaactcctaagctcaggcaatactcccacctcagcttcccaggaatataccacttttactgcactgacaagctctgtatgctagtgattctcaaattttctttaaggctaggaccaagagtcctgccaatcccctgaacaacagctcacatattatcaaatgaacttgaaacattcctgtcatagtgagcagcattgaaacagattccataactgattactcagtttcaagggagatttaacattgctttgttttcaagttacaaaaagttccctagttttactcaaatatgcactatccctgattaaaaaaaacatgtttcattatgaagaggggtgatttgtttcagcatttttttttttcacttaaccacttaagtcactgcctgaggaagtttctttttaaggaaataaataccaggttcattagaagaaaaaaaaaaaacacataattttaattcattttgttttaaagatgcgtattttaaaaagactactttaaaatgaactaatatgttacactggatcatgctgtggcgactaacgtattgtcaagccttaacctaatgaaaacaaaagaaaagcgagtttggcactcacttgcacttttcatctctgttagaaagtatgtctcagtttggatctgagatcaggtttgcttggtaacctcaaagaataattttccttttttttttctttcaaaatttccttttgatcatttcagacagttcatccttttgagtgagaaagagtaaaagagaggaatgttgagtgaggttaagtaaatggagaatctgtcacataaagcaagtttaaatcctagtaagagcatccatgcaggacaaacggaagcattattcttttgaaaacattattcttttaaacagtgtgtaatgacatcctccctagagactttccatgagaggggaaaaaaattacttcctcagaagtcgttttctagattccaagcataataagtgaagcacagttaaaagtcaaacttgtgttttctttatgcaagaaggttcaaattagaactgcagaaaggtacttaaaagtttctctagcttgtcttttggttacatactggtattgctgtgaactaaaagagcaagtaagaggaaaggttactgttgttactttacacctataaatcagtgagtgtgtccttactgtaaaatttgagctgaacatattttgtttcaaaggagaaatatatgactcaaatatgctgaatgtatgataatttattaagttccttttaagtatatcattttcttatgctcaagtagaaactatggattatttttctagtattctatgctgctgttaccttctgaggagttgattgaaaattttatgcttttaaaagttgggtgctacttaaatatcagaattggctattgttttaaatatttaaaatatgcttaaacaacaattaaggttaataagcagagaaaatacttcttttgattcaaacactactttatatatttaatgaatacacgtccaaataaagatctctcttcaaaaattttggaaaatgttaatgcattttgaatataatggaacaaagaagaagaatactagagaaaattcacaattatgatgtttatttaggaaaataaacttgaagaaggttttctattaaaaaaacataagaatcatatccaaattttagactctccatcttctttggtatgaaaatcaacattcataatagaaaatattttcttttgaaaggtttagttgttattgggtctataacggttttccatataaggaaaatacagtattatctgtaatcatctcacttattgaacaaccaatgaatgcatgcaagtaaccaagcatatgtgtgcagagaccagcatcaaggaaatattcattcatagataaatgttttctaataaaatatattttaagtttttaatgatcttctgctatcattttttgccatgttatctgaatagccatccagatctgtagtaaaacatcctgttagttacataactcaagaagtacttccccaaggaagctcacaccatcataccaggacttagcaacatttatctttcaacatgagtataccattaaaatttttttatatttctcagaattgtattcttcagtcttttccacaatatagtatatggaaattgctaatagcattaaattaatattaataaaacccaattctatctaaacctttttctcataagaaaaaacattactttaaaaaatagactttttgtttcttctaaaagtagtactatatggactgctcaattagcaatgccaaatacttccaaaaacaccataggaccaccaagctatttctattgctttgataatttcttttcctgctccaatttctccacgttcctgctttcttgtgtcaaaatatcttcccttaatttgttaaaatgaatctgagggaaaaaaatctgataatctggggtaaagaaatttttttttttgcatagactcttgtgatcacaaaatgaccaggtaatttatagcttcagtgctaacactgtgattgggaacaagaagagtacaaccataataaaatacagctatctatgagaagaactgcataaagacatctttggccatgtaggctctgggccctctggaaataagtcagttgcattgccaacatgacaaagaaaatagcaatgttcagaatcaggaacaacctggtataggaagcagacagtgatggggccctgctgtgtgtagttgtcaccatccgtgcctgtccaaaccggcctttaatcaagcccccatttttatgtttctcgtatgttacatctgcaaaatctaaaaggtctttcatttcttcatcttcatctatgggtagttctttctgtgccaaaatctgagctttctgtctaatctttttctcattgacttcaatctgtgcaaaaatatcagggacagcatccacaaatttatagcgtttgcctgcccttcggtttttctttgacttgctttgctgctgctgttgctgtgatatggcaaaaatcctgtcaatggcctcctcagtctgtctcttatctgaaaatctcagcaggcgttcagcagtcttcctaaagctagctgtgttccggactcgggacagtatctgcttctccagcagctgaaacactggtttaaaatgctgcaagttctgttccacaatagcagcatagtccttcacctcagggacaatgctgctcttgatggctgaattccggtcaaacagaattttgtgacgatcagcaatgacctgtgcaaaggcagactgtcctgtggcctcacctgtccacaggtatgtggcgtaggcatgtttgctggtggctatgaacacatccagttgctgagagtctccgtggacagtgaagctctgaacatctatagatggccctatgaagaggtaagctgccctggtgatgggacttcggaggtgcatggtgacattcacatagtttgtcccattgtagggatagccccgaggatatgtcactgaggcaaaggttgctttctcgctgtagccagtatcgtccatccagtacattttatagagaccatctctctgcctgatgaaagccccatggacaccatctaccacagtctcctcaaaaggaacatccacattatggaagaagctcgctgctgtctccaagggactctcctctcccaggtgtatttggtctacaaggagaagcagctgtggatgtaggaggatgagattcctctgaacattcttcaggttgagctgggggttataagctcccacaccttctcctcggatgaaaaccaccccatttttctcctctgctgcaaccaccctcccctgacaactagctgccaggtcatgcttgtatttagaccattttgatgagcagtcttctgtgacctgacccacccagggagaaaagcagctctttgacacagctggggaaaacatcaaaacattgttgaagaaggtgtactttggcccgtacagagcctcagtaatgaaaggcacaccattgggagcaaaagtaaatgagttttgatcaggatgttcatgccctgcattaaaatttctccatcctttgatccaatctttgtatttgtttctgtggacaatgtcatatattgcacgtccccccagttttccagacttgaaggaaaggaaagatctattgatttctgcaggtagtgcacttccataagtcacgacaccccagtcttcaaaataatgcagtgtaggggtgccaaagtctggaggaggaaccgatttcaagctgccatcataccttgattcatcaggactaggcttcccgtgagcaaagccatacagttggtgggctgatgattgtgcaggtattgaaatccccatcctctcctgtatgaagtttcatacatataccctgaggcattggcaatcacttcaagaaacttctcctgttgtgtcttgctcaggtagttgtacaagaagtcataagcagtggcaaaaccaaccagggagtgagcaagcgggacctcatcccaaggagcatctttcaccaaccaactaggctgcgctgccatcctctccatgtagtctttggccatgtctcgggcttcaatgttctcaggatacagcacacagaacattgccaaggcacccaagttgtttccaaaaatttcattccagcgggcactgtagtccttgggatcccagggagggaggtattccaaggggctggacagcatcgtgtgcacagcctccgtgaggcgggctgcaatgtgctcgtgcgagctggcagccctgagctgcagctccgccacttctgccctggagaagtacagcatgggatggctgtcgtagttggcattggtgaagggaatcataacttctgggttctcgtcggtgatgtaggctgacacaaagcaaagcaaatatatgaaaaacacactgggagccccccgtgtgtgagtcctcatcgtggcatcagatctccaaatctccaaggcagccaaaccatcttcgaaagatcctcacagtgcagggtggtatgccgccaaatgcttccacaaagctcagtgtcccattgtggagcgccttactaactccatgatgatgcacggctgcaacaacggcaagaagctcatgactgtgtgcatcgtcaagcatgccttcgaggtcatacacctgctcacaggcgagaaccctctgcaggtcctggtgaacgccatcatcaacagtggtccccgggaggactccacacgcattgggtgcgccgggactgtgagacgacaggctgtggacgtgtccccacttcgccgtgtgaatcaggccatctggctgctgtgcacaggtgctcgtgaggctgccttccggaacattaagaccattgctgagtgcctggcagaggagctcatcaatgctgccaagggctcctccaactcctatgccattaagaagaaggacgtgtggccttcttggagcatgtggccaagtccaaccgctgattttcccagctgttgcccaataaacctgtctgcccttcagggcagcccttaaagtaaatattttcagaaacaataggttaggtgccttagaaattcattcagaggcttagaaatccacattaacacagttcttacatgcttgagtctggtctacatccatttacgtaagtaaaactccccttccagactgacgaaattctttttgtgacaagaagacaaaggaatacgatggattgataagcgtagtcaaccgcgcagag

SEQ ID NO: 18018 - RNA, 800 nt, Homo sapiens
  source 1..800: mol_type = other RNA
tctgagttcctggagcctggtctcaggtaaatgaaaacacagggaacaaaaaagcaaaggaccacgatgcagtgggaggcacaggtctgaaaggctctgtgcctcccctctgaggtgtggatccgcaggatggaacagacgatggacacataagacagcactatcaggagaaagcagcccgaggccactagcccaatgtccacaaagatgaccatctcgttggctgaggtgtctgcacaggccagtttcaggatgggcggtgcatcacacaaatagtgctggatctggttgggtccacagtagggcaaatggaaagtcaatatggtctggacagcagagtgcagagagccactgagccaagtgctggtggccaggagggcacatctgctcccactcatcatgctggtgtacctgagcgggtaactgatggccaagtagcgatcataggacatgactgtgtagaggaaacactcggtgctccccaggaagtggaaaaaatagagctgagccacgcagctgtggaaggagatagccctgccgcttggggacaccaaggtcatcagcattttgggcaccgtgacagtggagaaccacatgtcaatgaaggacaggttggtgaggaagtagtacatgggggtgtggaggtgagaatccaccctgatcaccagcaggatgaggaggttccccagcacagtgagcacgtaaaccaccaggaagattccaaagagtggggcgtccagccctggggcatggggaaggcccgtgaggatgaacgctgtcacgaggctggtcttggacat

SEQ ID NO: 18019 - RNA, 716 nt, Homo sapiens
  source 1..716: mol_type = other RNA
tctgagttcctggagcctggtctcccctggtgctcttcttcctgcgcatagacgctcggacaaggtcagagccgaagtgggcattgtggtgccgctgggagcgtgcttcctggaaccagtcccctgtcaggatcttcagctgcccagggtctgccactgaggcccggagcttgctgacccgcccctcctccagctggcgcaggcgggcatctcgttggaggacgccagcaatggcctcctgctcctcctctgtcaggaagctgaggtccaacagtccttcagtctcaggctttggcccatgcgccatggggagggagggcagagcccaaagcccctcttgcgatgggtggcccctctggggcatcagctggggctgtgccccagctgggcacacggagcttccagagttaggtaggagtttggtcttctctgctgttttgacacggtgggacagacccattggtcaagaggagggtctgtccatctgtccagctgttccagttccagacatgtgcccacctcccccaaccccaaggtgctggagggtgctcaggataccaggtggcagtgcctgcgtctctggaccctggcaggggaccctggcaccgacacgtgttacctgtaggggtccagtatgggaggacaccttcgcaggtggctccagctcccctggcagccgagtttcagggaccgggagaagagccgtgagggaagaa

SEQ ID NO: 18020 - RNA, 513 nt, Homo sapiens
  source 1..513: mol_type = other RNA
tctgagttcctggagcctggtctcccctggtgctcttcttcctgcgcatagacgctcggacaaggtcagagccgaagtgggcattgtggtgccgctgggagcgtgcttcctggaaccagtcccctgtcaggatcttcagctgcccagggtctgccactgaggcccggagcttgctgacccgcccctcctccagctggcgcaggcgggcatctcgttggaggacgccagcaatggcctcctgctcctcctctgtcaggaagctgaggtccaacagtccttcagtctcaggctttggcccatgcgccatggggagggagggcagagcccaaagcccctcttgcgatgggtggcccctctggggcatcagctggggctgtgccccagctgggcacacggagcttcctgtaggggtccagtatgggaggacaccttcgcaggtggctccagctcccctggcagccgagtttcagggaccgggagaagagccgtgagggaagaaggctgactcaacag

SEQ ID NO: 18021 - RNA, 531 nt, Homo sapiens
  source 1..531: mol_type = other RNA
tctgagttcctggagcctggtctcccctggtgctcttcttcctgcgcatagacgctcggacaaggtcagagccgaagtgggcattgtggtgccgctgggagcgtgcttcctggaaccagtcccctgtcaggatcttcagctgcccagggtctgccactgaggcccggagcttgctgacccgcccctcctccagctggcgcaggcgggcatctcgttggaggacgccagcaatggcctcctgctcctcctctgtcaggaagctgaggtccaacagtccttcagtctcaggctttggcccatgcgccatggggagggagggcagagcccaaagcccctcttgcgatgggtggcccctctggggcatcagctggggctgtgccccagctgggcacacggagcttcctgtaggggtccagtatgggaggacaccttcgcaggtggctccagctcccctggcagccgagtttcagggaccgggagaagagccgtgagggaagaaggctgactcaacaggcagcccagccagcagct

SEQ ID NO: 18022 - RNA, 2898 nt, Homo sapiens
  source 1..2898: mol_type = other RNA
tctgcaagtgtcagaggcgaggtgggcgccgcaggcgtgggtgtggcagggctcaggccgctgttgtacatgggcgcccgctgcttgaactgcgctggcaacgtggggctcggggcgctgggctcctctggtgggcggctggcttcccgggaagatggggctgggggcgtctcggagctggggatgtaggaggaggcgggaaccacgctgggcgtggagggaaggtagctcgtggagggcagcgcaggctcattgttcagggacccaagtttctgcgtggacaccaggccggctgcgtagtccggggtggcgttctccaccaccgtttcctccttggccggcttctccaccacctccgcatcgagagtcttccttctccgcttcgcctctcggccagcgccaaccatatccagctcagagatgtccagcagcttcacacctcgttccttccgcagcagcgtcctggaaggcgggatgggggtccggttccctgtggggctgaagacgctgggcgccgtggggcttctgaagggcgcctgcttcgggatgcctttgagtggggtggtggtgtccatcttccgcagcagcccccggcccttggcgtggaagggcaccccggcgctccgcttcaactgctgggcggtctccgtggacttctgcagcagctccgcccgcagcgtggcgctcttgggtttccgctttaactgaaaatgcttcaccgggggagtgaggggtcccgcgagggtcgtcagggcgtttttgttcaagtactggcactccagtggcagcatggcagacgcttcacactcacccaccttttctctaagttctcccaaaatatcctgaacgttgggattctgctcctccagctccaggttaagcgagcctgtgtccggaaaggacttcaagatgtcggcgaccatgagcacccaggggtccgagtcgaggctggcgagctggatgatctccattagggcgcccttcatctcacacacccacttattggaatgacgcaaaacggcgtgtagaaaagagtaaaacggacacagagcgctccggacggccggggtctcgtccaccgtgcggcgcgggaggtgcagcgtcccgagtagcaacttgagcttcactgccgacgagaggccatggaagcagagacggatgttgtcgatgaccgcggccgtgagcagggacgcgatgctgggcggcgcccacagctcgtccgtggcccccagcttgttgtgcagccacaggcccgtgtcgctctcccgcatggacgccatcttgggggaaagcgcgcgccgctgccccggcatcttatgaagacacctacgcgtccctcgctaggaccccaacatggcggcgcccgtcgggctgcgggccgcagaggcggcgcaggtggcgcggtcccacgagcggggcttcccgggagagcgcttctgggtggcgaccgcgtctccgggtagcggccgcgtcttcgggaagctttgtggcaaagccgagagccggaaggacggggtgccgctgagcaaggactatcggcttccgtaaaacatcatggcggcgccctctgctggctctcgggaagaccgcaaaaaatgacgtcacgagcaggcgcgcgtattcgcgtcttgggagcccgggctgcggcctggcattcgcagtgcaggtgtcaagcgccgcagacttgctgctcgcgcggtggggcggaggctccctgtggcacctgccccgctgtccgctcttcgctttttccccgcttgggtctcggcgcggaccgtgtggacgccccgcccccgcgggcccagcacctgcacggagaggagccgcggccctgcggagcgagcctgcgggatcccggtcgcagcgctgagcttccgtcccccgctgagcccgctctgcccgtggcgcgccgccgacggggctgcgctgagcatgcgggtcggagggcgctcgggagctgtccaggggcactcgtgaccccacagtgcagggaggccccggcccccagtcgggctggagccgccaggcaggagccagtagtgaacttttcagttttaaaagcttgtcattagatacaaacatgagtaaaagttaaacttcattttattaaattcgttttacccttttgtctttttgacgaggccttcctatgttggccaggctggtctcaaactcctgggctcaagcgatccgcccgcccgcctctgcctcccagagtgctggggttacaggtcggggccgccttgcttggcttctgtattatatcttttttttaaaagatcttttccttattgttccactgccatgctcctgccgccgttcacagctattgccactgggcggtgggaacgccgggagaacagggctcagcccagctgctagcagtgccctggccctggcggcttgaacttggcagtcctgcggaagtcacacgggggaaacccgcaaatgctacaaatcagtgctggagcggtggttttgttgattgcttaaactgggagaagccctctaggtcatcaccacaccagcagccagtcctaatcggctgctacgacggctcctggaagcgaataggagaaaatattctcagaatattcctatgaaggtgcgatatccagaatctacaaggattcggttcagaagacaggagggtttggcagccttattgccacattttcttgatgtagaagtgttgcaatctgctgagctccagccacagatttcccacttcctcagcttttctcccgccggccttgcgctctggaggtctcgccccggcgccgcctcctccaggcagtcctctagactgcatccgccatgggcctggacgctgctcccgggggcagcccccggccagggccaggcacacccgattcctggagcgtcctaggttcctct

SEQ ID NO: 18023 - RNA, 1211 nt, Homo sapiens
  source 1..1211: mol_type = other RNA
tctgcaagtgtcagaggcgaggtgggcgccgcaggcgtgggtgtggcagggctcaggccgctgttgtacatgggcgcccgctgcttgaactgcgctggcaacgtggggctcggggcgctgggctcctctggtgggcggctggcttcccgggaagatggggctgggggcgtctcggagctggggatgtaggaggaggcgggaaccacgctgggcgtggagggaaggtagctcgtggagggcagcgcaggctcattgttcagggacccaagtttctgcgtggacaccaggccggctgcgtagtccggggtggcgttctccaccaccgtttcctccttggccggcttctccaccacctccgcatcgagagtcttccttctccgcttcgcctctcggccagcgccaaccatatccagctcagagatgtccagcagcttcacacctcgttccttccgcagcagcgtcctggaaggcgggatgggggtccggttccctgtggggctgaagacgctgggcgccgtggggcttctgaagggcgcctgcttcgggatgcctttgagtggggtggtggtgtccatcttccgcagcagcccccggcccttggcgtggaagggcaccccggcgctccgcttcaactgctgggcggtctccgtggacttctgcagcagctccgcccgcagcgtggcgctcttgggtttccgctttaactgaaaatgcttcaccgggggagtgaggggtcccgcgagggtcgtcagggcgtttttgttcaagtactggcactccagtggcagcatggcagacgcttcacactcacccaccttttctctaagttctcccaaaatatcctgaacgttgggattctgctcctccagctccaggttaagcgagcctgtgtccggaaaggacttcaagatgtcggcgaccatgagcacccaggggtccgagtcgaggctggcgagctggatgatctccattagggcgcccttcatctcgtccaccgtgcggcgcgggaggtgcagcgtcccgagtagcaacttgagcttcactgccgacgagaggccatggaagcagagacggatgttgtcgatgaccgcggccgtgagcagggacgcgatgctgggcggcgcccacagctcgtccgtggcccccagcttgttgtgcagccacaggcccgtgtcgctctcccgcatggacgccatcttgggggaaagcgc

SEQ ID NO: 18024 - RNA, 472 nt, Homo sapiens
  source 1..472: mol_type = other RNA
tctgcaggtcctggtgaacgccatcatcaacagtggtccccgggaggactccacacgcattgggtgcgccgggactgtgagacgacaggctgtggacgtgtccccacttcgccgtgtgaatcaggccatctggctgctgtgcacaggtgctcgtgaggctgccttccggaacattaagaccattgctgagtgcctggcagaggagctcatcaatgctgccaagggctcctccaactcctatgccattaagaagaaggacgtgtggccttcttggagcatgtggccaagtccaaccgctgattttcccagctgttgcccaataaacctgtctgcccttcagggcagccatgcttgagtctggtctacatccatttacgtaagtaaaactccccttccagactgacgaaattctttttgtgacaagaagacaaaggaatacgatggattgataagcgtagtcaaccgcgcagag

SEQ ID NO: 18025 - RNA, 560 nt, Homo sapiens
  source 1..560: mol_type = other RNA
tctgcaggtcctggtgaacgccatcatcaacagtggtccccgggaggactccacacgcattgggtgcgccgggactgtgagacgacaggctgtggacgtgtccccacttcgccgtgtgaatcaggccatctggctgctgtgcacaggtgctcgtgaggctgccttccggaacattaagaccattgctgagtgcctggcagaggagctcatcaatgctgccaagggctcctccaactcctatgccattaagaagaaggacgtgtggccttcttggagcatgtggccaagtccaaccgctgattttcccagctgttgcccaataaacctgtctgcccttcagggcagcccttaaagtaaatattttcagaaacaataggttaggtgccttagaaattcattcagaggcttagaaatccacattaacacagttcttacatgcttgagtctggtctacatccatttacgtaagtaaaactccccttccagactgacgaaattctttttgtgacaagaagacaaaggaatacgatggattgataagcgtagtcaaccgcgcagag

SEQ ID NO: 18026 - RNA, 30 nt, Homo sapiens
  source 1..30: mol_type = other RNA
tctgccatcctccctcccctacatcataat

SEQ ID NO: 18027 - RNA, 37 nt, Homo sapiens
  source 1..37: mol_type = other RNA
tctgccatcctccctcccctacatcataatacattat

SEQ ID NO: 18028 - RNA, 4330 nt, Homo sapiens
  source 1..4330: mol_type = other RNA
tctgccatcctccctcccctaccctcccacaactcccctcccccacccaccccaacccataaaaatcgcactcttgacagcctagtgaaaaccattgcaaaatccatatgggggcatgcacagttgcagcattgttgtaaatgatttcttgctctactagaaaaagttacattgtcttaaggtaacaaaacagttcttttgtgcttttcgatttctttgtttttttttttttctttttttctttttcttttttcttagaatgttagtgatgactgacagttctggtgcacagttacaatgtacaagtgaaatgaatatgatttgcattgttaaggcatccaatctgctggtttatatttatgtgaaagacagaggaaatatacaagcagacttaagaaagaaagtatgttcattgatttctatgaagtttctccctagaatttaatgcacaaaatgcgtcactccaaagggagagattccatgcatattaatagagtaaaacagcattagggttgttttgtaagcttccaaagcaaaggatacatttttttttaaatctactgaactaaatactacaagaataatatgctactatttttttttttttgccatatattggaaaaaacttcttaacttacaaataatacaaaaatagacaatgacttttgggtggaaattaaaaaaactgaagcatggtttataacaatactaaaaataactataaatgaaatgtttaaaaatcacattgaaacagctaatacaagtgtaggtgaccaaacaaatacgcacttttcacgtagcaaacatacacaataaaataaattgggggtggaaggaagaggaagaagggaaaagcaatgtacaaattcgaaagataaatacattatttatatggatattttacaaaatcccctttaaaacaaaaagccttttaattaactttgcaagtatgtgcaagctaaaggtagtgagctttttttctttgcaaaatacgcagtaaaatctttttgtgatattgaaaaaatgtcttaagacattaaaatgtataaatagaacaacaactttggcaaaaaatcacaaaaaaaaaatctacagtatttataactacatacaaaaacacaagagcaaagaaaaaaatatcaggcaaatgcatcctcagagctttgctgcatctttgctattaattcttatttttaagaacacttcccagataatgagagcaaaaattcccatagaacagaaaactatgttttggaggtctcaaccttcttttcctttctccacccccggttccctttaactcttaattccaaagcacttaacctgttgtttcaatctattatgttacaaatggtaagggtcgactgatagaggcagtatctggaatgggaaaatcgaaaatacctgccacgttgcttttatcaacttttggaagataggtatgaagtctgcatttaggacgagtaaactttaaacttgcaaatgggggagcgtacgtgaggttttggcttgttaactggagggcagagtgtggaattctgtgcctggaccctgttccatgaagtctcaaaggagattctcacacagtatgtgtgccaccaagctctcgagaggccatcggcttcagaagaaactgacttaagtaaaaggagagaatgagatcagatttaaatatgcagttttaacaatctgtctagaggcactggattttcgagtagagggaaaaatgtgatcacttacatcgcgttttaactttccaggctgcatttatttacacagttgcttaagacaacaatacaaaagagataaataagcttgcactgctaaggggtggcatgttaagttagatattgaaaatgcactgtctgagctaactaccatttgatatgctttaaggcgcaaaagccgacccttagtttttctaaaaaatctaactggcattcctattctgtcccatacaagcttttttttttttcctttttttctttttttttttttttacttttttgtaaatatcaccacttcattcttcctttacacagctttaaaaacatcataaattaaaacatggagtcttatttatagtgtcccttgtatagagctttacggtttataaaagacaaatgattgcagaattaagcttaaaaaaaaaaaagaaaaagaaaaagtggatttgcttttgtcaatacagaataaatatatcccccaaatacttgggaggtacaactttaaccaacaccctgcacttgcagatccctcttccaatttcagtatttgcaaggtcggtgattttgtttgtttaaaaatctgcagttattgtgattcctcttaaaaaggcctgagttaaaagttccactctgggacttgtatcagattactctctgtagcagaatccaacctcttcattaatacaattcttcaaggcaattctttcacataggaggaacaatcatgccagatatcgcttgcaggctgttcccgttggtgctggtgcaggtgggaggtggggaggtctggggtctgacgactggtgcgaaagcactcttctgtttcacggctgagaccatgttggctggtgagaaggagaagatgcccgaggagctgctgcagttggaggggaggcttgtggaggaggccatggtggggctggatggcactacctgattggtggcttgtgatgcctcggagacattcacggccagttgtccactgaacgaattcacgcccatcatccctgcgtggaccgaggtgttagcaagggccgggagttggttgtggttgcggggaacactgtacagggcctcggcaatgtcggccgctctcttcagaatgatttcctggttgttgtgtggcatcccatacagtgcttctaccagatccgcagcccttttgagtattacttcctttggcaaacgctcagggtcaccagggtgccgaggaatgaccttctgtaacctctggaaaccataatcgatggtgggttcgttgagcgctgtataaatgaatctgcctggtgttcctttgcagaactgcttagatttgtaggacagtgtgacttccacaacaccagggatgtgccgaggaggggtctgcacacggatggcatgaggagtgatcaactcactccagaccagcatggtaccgaatatgacctgtaacccatcaaagaaattgtcccctatgatgatcacagtcgcacctcccgtcgtccatccttcactcgggctgatggctttgatacagggagtagcatgttccagataagagggcgtaccttccgaggggtcaagcctccgagccctccgcccatgcttggaattattatggacaaacatgttatcagagactgccaggacatggccatccacattgactgtcgtagacaccacgacctggaatctccgcatgtcacgtgggtttcccgcattctttaggcaattttggttacatttgaggaaaaatttcaagaagaacctgtcaattatcactggatctgagggagtctcatttcggttgccacagcttttcttgtcacaacagcggctgcacatgatctcatgtgtgagcaagactcggcacatttctgggttcttgtcttggccttcatacactatggcttgttttgtcatggagtcaatgaggcgcacgtagaaatcctgctccgtccttatcccattgctgtagagaagctgaagccggtagtgaattccgttattggtcttttcgctgttggcttctttttccttctccacgaaccccacaaacgctgtcctctcgatctccacgggctggccctgtctgtcgtagagggccaggacgaagtggaagaagttggatttccgcagattggaaggcggctgcttctcaaagtgagcccgggccagacccaccccgctctgcgccgccgtgttggcgtccagcaccccggcgccctgcatccacgtccgcaccgcgttcatgccgctgcccagcggctcttccttcatgctgcttccactccgttggatgctttcctgaatcccaaacatgaaaacaaccttttcttgtggaaaatctcctcccccttgaaaaaaattaaaaaaaaaaaaaaaggaaagaaaagaaagaaaagaaaagaaacaaaaacgccaaccagagatttttttttttctcagacgatgaactcgcacttagaagatcaaggcgggctggaaagcaaatttttaaaaaatgtaaacctctgctcaaaactgagcgataacccgaaaaaaagaagaaagggaaaatccaacgaaaagaccaaaataataaaattagagatgtatgcttggctgttgggggttgtttggtt

SEQ ID NO: 18029 - RNA, 4806 nt, Homo sapiens
  source 1..4806: mol_type = other RNA
tctgccatcctccctcccctaccctcccacaactcccctcccccacccaccccaacccataaaaatcgcactcttgacagcctagtgaaaaccattgcaaaatccatatgggggcatgcacagttgcagcattgttgtaaatgatttcttgctctactagaaaaagttacattgtcttaaggtaacaaaacagttcttttgtgcttttcgatttctttgtttttttttttttctttttttctttttcttttttcttagaatgttagtgatgactgacagttctggtgcacagttacaatgtacaagtgaaatgaatatgatttgcattgttaaggcatccaatctgctggtttatatttatgtgaaagacagaggaaatatacaagcagacttaagaaagaaagtatgttcattgatttctatgaagtttctccctagaatttaatgcacaaaatgcgtcactccaaagggagagattccatgcatattaatagagtaaaacagcattagggttgttttgtaagcttccaaagcaaaggatacatttttttttaaatctactgaactaaatactacaagaataatatgctactatttttttttttttgccatatattggaaaaaacttcttaacttacaaataatacaaaaatagacaatgacttttgggtggaaattaaaaaaactgaagcatggtttataacaatactaaaaataactataaatgaaatgtttaaaaatcacattgaaacagctaatacaagtgtaggtgaccaaacaaatacgcacttttcacgtagcaaacatacacaataaaataaattgggggtggaaggaagaggaagaagggaaaagcaatgtacaaattcgaaagataaatacattatttatatggatattttacaaaatcccctttaaaacaaaaagccttttaattaactttgcaagtatgtgcaagctaaaggtagtgagctttttttctttgcaaaatacgcagtaaaatctttttgtgatattgaaaaaatgtcttaagacattaaaatgtataaatagaacaacaactttggcaaaaaatcacaaaaaaaaaatctacagtatttataactacatacaaaaacacaagagcaaagaaaaaaatatcaggcaaatgcatcctcagagctttgctgcatctttgctattaattcttatttttaagaacacttcccagataatgagagcaaaaattcccatagaacagaaaactatgttttggaggtctcaaccttcttttcctttctccacccccggttccctttaactcttaattccaaagcacttaacctgttgtttcaatctattatgttacaaatggtaagggtcgactgatagaggcagtatctggaatgggaaaatcgaaaatacctgccacgttgcttttatcaacttttggaagataggtatgaagtctgcatttaggacgagtaaactttaaacttgcaaatgggggagcgtacgtgaggttttggcttgttaactggagggcagagtgtggaattctgtgcctggaccctgttccatgaagtctcaaaggagattctcacacagtatgtgtgccaccaagctctcgagaggccatcggcttcagaagaaactgacttaagtaaaaggagagaatgagatcagatttaaatatgcagttttaacaatctgtctagaggcactggattttcgagtagagggaaaaatgtgatcacttacatcgcgttttaactttccaggctgcatttatttacacagttgcttaagacaacaatacaaaagagataaataagcttgcactgctaaggggtggcatgttaagttagatattgaaaatgcactgtctgagctaactaccatttgatatgctttaaggcgcaaaagccgacccttagtttttctaaaaaatctaactggcattcctattctgtcccatacaagcttttttttttttcctttttttctttttttttttttttacttttttgtaaatatcaccacttcattcttcctttacacagctttaaaaacatcataaattaaaacatggagtcttatttatagtgtcccttgtatagagctttacggtttataaaagacaaatgattgcagaattaagcttaaaaaaaaaaaagaaaaagaaaaagtggatttgcttttgtcaatacagaataaatatatcccccaaatacttgggaggtacaactttaaccaacaccctgcacttgcagatccctcttccaatttcagtatttgcaaggtcggtgattttgtttgtttaaaaatctgcagttattgtgattcctcttaaaaaggcctgagttaaaagttccactctgggacttgtatcagattactctctgtagcagaatccaacctcttcattaatacaattcttcaaggcaattctttcacataggaggaacaatcatgccagatatcgcttgcaggctgttcccgttggtgctggtgcaggtgggaggtggggaggtctggggtctgacgactggtgcgaaagcactcttctgtttcacggctgagaccatgttggctggtgagaaggagaagatgcccgaggagctgctgcagttggaggggaggcttgtggaggaggccatggtggggctggatggcactatggcatagggggagttggcagctgagccgttgaggaaggtgggggagccgcccaaattggacattgcggcagagccgtatccgttcatgctcgtggtgacggagttatagttggtctgctggggagtggtgctcggcacgtacccgtgtggtgatacgctgcttgagttgcgggtgaaaccctgattggtggcttgtgatgcctcggagacattcacggccagttgtccactgaacgaattcacgcccatcatccctgcgtggaccgaggtgttagcaagggccgggagttggttgtggttgcggggaacactgtacagggcctcggcaatgtcggccgctctcttcagaatgatttcctggttgttgtgtggcatcccatacagtgcttctaccagatccgcagcccttttgagtattacttcctttggcaaacgctcagggtcaccagggtgccgaggaatgaccttctgtaacctctggaaaccataatcgatggtgggttcgttgagcgctgtataaatgaatctgcctggtgttcctttgcagaactgcttagatttgtaggacagtgtgacttccacaacaccagggatgtgccgaggaggggtctgcacacggatggcatgaggagtgatcaactcactccagaccagcatggtaccgaatatgacctgtaacccatcaaagaaattgtcccctatgatgatcacagtcgcacctcccgtcgtccatccttcactcgggctgatggctttgatacagggagtagcatgttccagataagagggcgtaccttccgaggggtcaagcctccgagccctccgcccatgcttggaattattatggacaaacatgttatcagagactgccaggacatggccatccacattgactgtcgtagacaccacgacctggaatctccgcatgtcacgtgggtttcccgcattctttaggcaattttggttacatttgaggaaaaatttcaagaagaacctgtcaattatcactggatctgagggagtctcatttcggttgccacagcttttcttgtcacaacagcggctgcacatgatctcatgtgtgagcaagactcggcacatttctgggttcttgtcttggccttcatacactatggcttgttttgtcatggagtcaatgaggcgcacgtagaaatcctgctccgtccttatcccattgctgtagagaagctgaagccggtagtgaattccgttattggtcttttcgctgttggcttctttttccttctccacgaaccccacaaacgctgtcctctcgatctccacgggctggccctgtctgtcgtagagggccaggacgaagtggaagaagttggatttccgcagattggaaggcggctgcttctcaaagtgagcccgggccagacccaccccgctcctcttcccccaaaacatccagtgggcgctcttcacgccccttcaggcgacatagacccagctgacaacgggacacacatgtcccctcatgtcctcgtcctctccgccaaggacgggtgcgtcctcagaactcgctgaagaggtgtgaaagttttgtttgggttttgcgcgcgagatgaaactctataagcatttactcctacctgacacgcactgcgtggggaggaagaaaagtggcggtggatgaagtgaacccaccttcgcggagtagaacccacagttatattccggcacccctcgaatctcacgtctcagctagcagggcaggtgggaatggatggaaaacatgctcggcgtctcgccgcagcagccaccctccaggaacccctcaagctctggccaactgcgagtgcccggccttgggaagccacatccccccaccaccaaaaagcatgtggagaagggtccgagggcggggctcagaactgtcgcgggtggtcgctgtgaaaaagggaagaggggtgttttcttaaagacctgtcctaacaaagtttcgctgttccgcagaaatcctcacactcattccagaaatcctaaaggccagggctgctggctcagtgcgccggccggcgatgggaggctggagcgcctggggcgccaggcggccactgacagccggacctgcccaacacaagcgcgcacaggcacacacacacacatagaagaacac

SEQ ID NO: 18030 - RNA, 4646 nt, Homo sapiens
  source 1..4646: mol_type = other RNA
tctgccatcctccctcccctaccctcccacaactcccctcccccacccaccccaacccataaaaatcgcactcttgacagcctagtgaaaaccattgcaaaatccatatgggggcatgcacagttgcagcattgttgtaaatgatttcttgctctactagaaaaagttacattgtcttaaggtaacaaaacagttcttttgtgcttttcgatttctttgtttttttttttttctttttttctttttcttttttcttagaatgttagtgatgactgacagttctggtgcacagttacaatgtacaagtgaaatgaatatgatttgcattgttaaggcatccaatctgctggtttatatttatgtgaaagacagaggaaatatacaagcagacttaagaaagaaagtatgttcattgatttctatgaagtttctccctagaatttaatgcacaaaatgcgtcactccaaagggagagattccatgcatattaatagagtaaaacagcattagggttgttttgtaagcttccaaagcaaaggatacatttttttttaaatctactgaactaaatactacaagaataatatgctactatttttttttttttgccatatattggaaaaaacttcttaacttacaaataatacaaaaatagacaatgacttttgggtggaaattaaaaaaactgaagcatggtttataacaatactaaaaataactataaatgaaatgtttaaaaatcacattgaaacagctaatacaagtgtaggtgaccaaacaaatacgcacttttcacgtagcaaacatacacaataaaataaattgggggtggaaggaagaggaagaagggaaaagcaatgtacaaattcgaaagataaatacattatttatatggatattttacaaaatcccctttaaaacaaaaagccttttaattaactttgcaagtatgtgcaagctaaaggtagtgagctttttttctttgcaaaatacgcagtaaaatctttttgtgatattgaaaaaatgtcttaagacattaaaatgtataaatagaacaacaactttggcaaaaaatcacaaaaaaaaaatctacagtatttataactacatacaaaaacacaagagcaaagaaaaaaatatcaggcaaatgcatcctcagagctttgctgcatctttgctattaattcttatttttaagaacacttcccagataatgagagcaaaaattcccatagaacagaaaactatgttttggaggtctcaaccttcttttcctttctccacccccggttccctttaactcttaattccaaagcacttaacctgttgtttcaatctattatgttacaaatggtaagggtcgactgatagaggcagtatctggaatgggaaaatcgaaaatacctgccacgttgcttttatcaacttttggaagataggtatgaagtctgcatttaggacgagtaaactttaaacttgcaaatgggggagcgtacgtgaggttttggcttgttaactggagggcagagtgtggaattctgtgcctggaccctgttccatgaagtctcaaaggagattctcacacagtatgtgtgccaccaagctctcgagaggccatcggcttcagaagaaactgacttaagtaaaaggagagaatgagatcagatttaaatatgcagttttaacaatctgtctagaggcactggattttcgagtagagggaaaaatgtgatcacttacatcgcgttttaactttccaggctgcatttatttacacagttgcttaagacaacaatacaaaagagataaataagcttgcactgctaaggggtggcatgttaagttagatattgaaaatgcactgtctgagctaactaccatttgatatgctttaaggcgcaaaagccgacccttagtttttctaaaaaatctaactggcattcctattctgtcccatacaagcttttttttttttcctttttttctttttttttttttttacttttttgtaaatatcaccacttcattcttcctttacacagctttaaaaacatcataaattaaaacatggagtcttatttatagtgtcccttgtatagagctttacggtttataaaagacaaatgattgcagaattaagcttaaaaaaaaaaaagaaaaagaaaaagtggatttgcttttgtcaatacagaataaatatatcccccaaatacttgggaggtacaactttaaccaacaccctgcacttgcagatccctcttccaatttcagtatttgcaaggtcggtgattttgtttgtttaaaaatctgcagttattgtgattcctcttaaaaaggcctgagttaaaagttccactctgggacttgtatcagattactctctgtagcagaatccaacctcttcattaatacaattcttcaaggcaattctttcacataggaggaacaatcatgccagatatcgcttgcaggctgttcccgttggtgctggtgcaggtgggaggtggggaggtctggggtctgacgactggtgcgaaagcactcttctgtttcacggctgagaccatgttggctggtgagaaggagaagatgcccgaggagctgctgcagttggaggggaggcttgtggaggaggccatggtggggctggatggcactatggcatagggggagttggcagctgagccgttgaggaaggtgggggagccgcccaaattggacattgcggcagagccgtatccgttcatgctcgtggtgacggagttatagttggtctgctggggagtggtgctcggcacgtacccgtgtggtgatacgctgcttgagttgcgggtgaaaccctgattggtggcttgtgatgcctcggagacattcacggccagttgtccactgaacgaattcacgcccatcatccctgcgtggaccgaggtgttagcaagggccgggagttggttgtggttgcggggaacactgtacagggcctcggcaatgtcggccgctctcttcagaatgatttcctggttgttgtgtggcatcccatacagtgcttctaccagatccgcagcccttttgagtattacttcctttggcaaacgctcagggtcaccagggtgccgaggaatgaccttctgtaacctctggaaaccataatcgatggtgggttcgttgagcgctgtataaatgaatctgcctggtgttcctttgcagaactgcttagatttgtaggacagtgtgacttccacaacaccagggatgtgccgaggaggggtctgcacacggatggcatgaggagtgatcaactcactccagaccagcatggtaccgaatatgacctgtaacccatcaaagaaattgtcccctatgatgatcacagtcgcacctcccgtcgtccatccttcactcgggctgatggctttgatacagggagtagcatgttccagataagagggcgtaccttccgaggggtcaagcctccgagccctccgcccatgcttggaattattatggacaaacatgttatcagagactgccaggacatggccatccacattgactgtcgtagacaccacgacctggaatctccgcatgtcacgtgggtttcccgcattctttaggcaattttggttacatttgaggaaaaatttcaagaagaacctgtcaattatcactggatctgagggagtctcatttcggttgccacagcttttcttgtcacaacagcggctgcacatgatctcatgtgtgagcaagactcggcacatttctgggttcttgtcttggccttcatacactatggcttgttttgtcatggagtcaatgaggcgcacgtagaaatcctgctccgtccttatcccattgctgtagagaagctgaagccggtagtgaattccgttattggtcttttcgctgttggcttctttttccttctccacgaaccccacaaacgctgtcctctcgatctccacgggctggccctgtctgtcgtagagggccaggacgaagtggaagaagttggatttccgcagattggaaggcggctgcttctcaaagtgagcccgggccagacccaccccgctctgcgccgccgtgttggcgtccagcaccccggcgccctgcatccacgtccgcaccgcgttcatgccgctgcccagcggctcttccttcatgctgcttccactccgttggatgctttcctgaatcccaaacatgaaaacaaccttttcttgtggaaaatctcctcccccttgaaaaaaattaaaaaaaaaaaaaaaggaaagaaaagaaagaaaagaaaagaaacaaaaacgccaaccagagatttttttttttctcagacgatgaactcgcacttagaagatcaaggcgggctggaaagcaaatttttaaaaaatgtaaacctctgctcaaaactgagcgataacccgaaaaaaagaagaaagggaaaatccaacgaaaagaccaaaataataaaattagagatgtatgcttggctgttgggggttgtttggttggttgatttttggtttgggtgctttttttttttttttgcttttttttttttttttttgtaatgatcacaggccggtggaggacaggaggggctggagtttccttttgtagaggtacccttcacttgaagaagcagg

SEQ ID NO: 18031 - RNA, 4601 nt, Homo sapiens
  source 1..4601: mol_type = other RNA
tctgccatcctccctcccctaccctcccacaactcccctcccccacccaccccaacccataaaaatcgcactcttgacagcctagtgaaaaccattgcaaaatccatatgggggcatgcacagttgcagcattgttgtaaatgatttcttgctctactagaaaaagttacattgtcttaaggtaacaaaacagttcttttgtgcttttcgatttctttgtttttttttttttctttttttctttttcttttttcttagaatgttagtgatgactgacagttctggtgcacagttacaatgtacaagtgaaatgaatatgatttgcattgttaaggcatccaatctgctggtttatatttatgtgaaagacagaggaaatatacaagcagacttaagaaagaaagtatgttcattgatttctatgaagtttctccctagaatttaatgcacaaaatgcgtcactccaaagggagagattccatgcatattaatagagtaaaacagcattagggttgttttgtaagcttccaaagcaaaggatacatttttttttaaatctactgaactaaatactacaagaataatatgctactatttttttttttttgccatatattggaaaaaacttcttaacttacaaataatacaaaaatagacaatgacttttgggtggaaattaaaaaaactgaagcatggtttataacaatactaaaaataactataaatgaaatgtttaaaaatcacattgaaacagctaatacaagtgtaggtgaccaaacaaatacgcacttttcacgtagcaaacatacacaataaaataaattgggggtggaaggaagaggaagaagggaaaagcaatgtacaaattcgaaagataaatacattatttatatggatattttacaaaatcccctttaaaacaaaaagccttttaattaactttgcaagtatgtgcaagctaaaggtagtgagctttttttctttgcaaaatacgcagtaaaatctttttgtgatattgaaaaaatgtcttaagacattaaaatgtataaatagaacaacaactttggcaaaaaatcacaaaaaaaaaatctacagtatttataactacatacaaaaacacaagagcaaagaaaaaaatatcaggcaaatgcatcctcagagctttgctgcatctttgctattaattcttatttttaagaacacttcccagataatgagagcaaaaattcccatagaacagaaaactatgttttggaggtctcaaccttcttttcctttctccacccccggttccctttaactcttaattccaaagcacttaacctgttgtttcaatctattatgttacaaatggtaagggtcgactgatagaggcagtatctggaatgggaaaatcgaaaatacctgccacgttgcttttatcaacttttggaagataggtatgaagtctgcatttaggacgagtaaactttaaacttgcaaatgggggagcgtacgtgaggttttggcttgttaactggagggcagagtgtggaattctgtgcctggaccctgttccatgaagtctcaaaggagattctcacacagtatgtgtgccaccaagctctcgagaggccatcggcttcagaagaaactgacttaagtaaaaggagagaatgagatcagatttaaatatgcagttttaacaatctgtctagaggcactggattttcgagtagagggaaaaatgtgatcacttacatcgcgttttaactttccaggctgcatttatttacacagttgcttaagacaacaatacaaaagagataaataagcttgcactgctaaggggtggcatgttaagttagatattgaaaatgcactgtctgagctaactaccatttgatatgctttaaggcgcaaaagccgacccttagtttttctaaaaaatctaactggcattcctattctgtcccatacaagcttttttttttttcctttttttctttttttttttttttacttttttgtaaatatcaccacttcattcttcctttacacagctttaaaaacatcataaattaaaacatggagtcttatttatagtgtcccttgtatagagctttacggtttataaaagacaaatgattgcagaattaagcttaaaaaaaaaaaagaaaaagaaaaagtggatttgcttttgtcaatacagaataaatatatcccccaaatacttgggaggtacaactttaaccaacaccctgcacttgcagatccctcttccaatttcagtatttgcaaggtcggtgattttgtttgtttaaaaatctgcagttattgtgattcctcttaaaaaggcctgagttaaaagttccactctgggacttgtatcagattactctctgtagcagaatccaacctcttcattaatacaattcttcaaggcaattctttcacataggaggaacaatcatgccagatatcgcttgcaggctgttcccgttggtgctggtgcaggtgggaggtggggaggtctggggtctgacgactggtgcgaaagcactcttctgtttcacggctgagaccatgttggctggtgagaaggagaagatgcccgaggagctgctgcagttggaggggaggcttgtggaggaggccatggtggggctggatggcactatggcatagggggagttggcagctgagccgttgaggaaggtgggggagccgcccaaattggacattgcggcagagccgtatccgttcatgctcgtggtgacggagttatagttggtctgctggggagtggtgctcggcacgtacccgtgtggtgatacgctgcttgagttgcgggtgaaaccctgattggtggcttgtgatgcctcggagacattcacggccagttgtccactgaacgaattcacgcccatcatccctgcgtggaccgaggtgttagcaagggccgggagttggttgtggttgcggggaacactgtacagggcctcggcaatgtcggccgctctcttcagaatgatttcctggttgttgtgtggcatcccatacagtgcttctaccagatccgcagcccttttgagtattacttcctttggcaaacgctcagggtcaccagggtgccgaggaatgaccttctgtaacctctggaaaccataatcgatggtgggttcgttgagcgctgtataaatgaatctgcctggtgttcctttgcagaactgcttagatttgtaggacagtgtgacttccacaacaccagggatgtgccgaggaggggtctgcacacggatggcatgaggagtgatcaactcactccagaccagcatggtaccgaatatgacctgtaacccatcaaagaaattgtcccctatgatgatcacagtcgcacctcccgtcgtccatccttcactcgggctgatggctttgatacagggagtagcatgttccagataagagggcgtaccttccgaggggtcaagcctccgagccctccgcccatgcttggaattattatggacaaacatgttatcagagactgccaggacatggccatccacattgactgtcgtagacaccacgacctggaatctccgcatgtcacgtgggtttcccgcattctttaggcaattttggttacatttgaggaaaaatttcaagaagaacctgtcaattatcactggatctgagggagtctcatttcggttgccacagcttttcttgtcacaacagcggctgcacatgatctcatgtgtgagcaagactcggcacatttctgggttcttgtcttggccttcatacactatggcttgttttgtcatggagtcaatgaggcgcacgtagaaatcctgctccgtccttatcccattgctgtagagaagctgaagccggtagtgaattccgttattggtcttttcgctgttggcttctttttccttctccacgaaccccacaaacgctgtcctctcgatctccacgggctggccctgtctgtcgtagagggccaggacgaagtggaagaagttggatttccgcagattggaaggcggctgcttctcaaagtgagcccgggccagacccaccccgctgacacgcactgcgtggggaggaagaaaagtggcggtggatgaagtgaacccaccttcgcggagtagaacccacagttatattccggcacccctcgaatctcacgtctcagctagcagggcaggtgggaatggatggaaaacatgctcggcgtctcgccgcagcagccaccctccaggaacccctcaagctctggccaactgcgagtgcccggccttgggaagccacatccccccaccaccaaaaagcatgtggagaagggtccgagggcggggctcagaactgtcgcgggtggtcgctgtgaaaaagggaagaggggtgttttcttaaagacctgtcctaacaaagtttcgctgttccgcagaaatcctcacactcattccagaaatcctaaaggccagggctgctggctcagtgcgccggccggcgatgggaggctggagcgcctggggcgccaggcggccactgacagccggacctgcccaacacaagcgcgcacaggcacacacacacacatagaagaacac

SEQ ID NO: 18032 - RNA, 24265 nt, Homo sapiens
  source 1..24265: mol_type = other RNA
tctgccatcctccctcccctaccctcccacaactcccctcccccacccaccccaacccataaaaatcgcactcttgacagcctagtgaaaaccattgcaaaatccatatgggggcatgcacagttgcagcattgttgtaaatgatttcttgctctactagaaaaagttacattgtcttaaggtaacaaaacagttcttttgtgcttttcgatttctttgtttttttttttttctttttttctttttcttttttcttagaatgttagtgatgactgacagttctggtgcacagttacaatgtacaagtgaaatgaatatgatttgcattgttaaggcatccaatctgctggtttatatttatgtgaaagacagaggaaatatacaagcagacttaagaaagaaagtatgttcattgatttctatgaagtttctccctagaatttaatgcacaaaatgcgtcactccaaagggagagattccatgcatattaatagagtaaaacagcattagggttgttttgtaagcttccaaagcaaaggatacatttttttttaaatctactgaactaaatactacaagaataatatgctactatttttttttttttgccatatattggaaaaaacttcttaacttacaaataatacaaaaatagacaatgacttttgggtggaaattaaaaaaactgaagcatggtttataacaatactaaaaataactataaatgaaatgtttaaaaatcacattgaaacagctaatacaagtgtaggtgaccaaacaaatacgcacttttcacgtagcaaacatacacaataaaataaattgggggtggaaggaagaggaagaagggaaaagcaatgtacaaattcgaaagataaatacattatttatatggatattttacaaaatcccctttaaaacaaaaagccttttaattaactttgcaagtatgtgcaagctaaaggtagtgagctttttttctttgcaaaatacgcagtaaaatctttttgtgatattgaaaaaatgtcttaagacattaaaatgtataaatagaacaacaactttggcaaaaaatcacaaaaaaaaaatctacagtatttataactacatacaaaaacacaagagcaaagaaaaaaatatcaggcaaatgcatcctcagagctttgctgcatctttgctattaattcttatttttaagaacacttcccagataatgagagcaaaaattcccatagaacagaaaactatgttttggaggtctcaaccttcttttcctttctccacccccggttccctttaactcttaattccaaagcacttaacctgttgtttcaatctattatgttacaaatggtaagggtcgactgatagaggcagtatctggaatgggaaaatcgaaaatacctgccacgttgcttttatcaacttttggaagataggtatgaagtctgcatttaggacgagtaaactttaaacttgcaaatgggggagcgtacgtgaggttttggcttgttaactggagggcagagtgtggaattctgtgcctggaccctgttccatgaagtctcaaaggagattctcacacagtatgtgtgccaccaagctctcgagaggccatcggcttcagaagaaactgacttaagtaaaaggagagaatgagatcagatttaaatatgcagttttaacaatctgtctagaggcactggattttcgagtagagggaaaaatgtgatcacttacatcgcgttttaactttccaggctgcatttatttacacagttgcttaagacaacaatacaaaagagataaataagcttgcactgctaaggggtggcatgttaagttagatattgaaaatgcactgtctgagctaactaccatttgatatgctttaaggcgcaaaagccgacccttagtttttctaaaaaatctaactggcattcctattctgtcccatacaagcttttttttttttcctttttttctttttttttttttttacttttttgtaaatatcaccacttcattcttcctttacacagctttaaaaacatcataaattaaaacatggagtcttatttatagtgtcccttgtatagagctttacggtttataaaagacaaatgattgcagaattaagcttaaaaaaaaaaaagaaaaagaaaaagtggatttgcttttgtcaatacagaataaatatatcccccaaatacttgggaggtacaactttaaccaacaccctgcacttgcagatccctcttccaatttcagtatttgcaaggtcggtgattttgtttgtttaaaaatctgcagttattgtgattcctcttaaaaaggcctgagttaaaagttccactctgggacttgtatcagattactctctgtagcagaatccaacctcttcattaatacaattcttcaaggcaattctttcacataggaggaacaatcatgccagatatcgcttgcaggctgttcccgttggtgctggtgcaggtgggaggtggggaggtctggggtctgacgactggtgcgaaagcactcttctgtttcacggctgagaccatgttggctggtgagaaggagaagatgcccgaggagctgctgcagttggaggggaggcttgtggaggaggccatggtggggctggatggcactatggcatagggggagttggcagctgagccgttgaggaaggtgggggagccgcccaaattggacattgcggcagagccgtatccgttcatgctcgtggtgacggagttatagttggtctgctggggagtggtgctcggcacgtacccgtgtggtgatacgctgcttgagttgcgggtgaaaccctgattggtggcttgtgatgcctcggagacattcacggccagttgtccactgaacgaattcacgcccatcatccctgcgtggaccgaggtgttagcaagggccgggagttggttgtggttgcggggaacactgtacagggcctcggcaatgtcggccgctctcttcagaatgatttcctggttgttgtgtggcatcccatacagtgcttctaccagatccgcagcccttttgagtattacttcctttggcaaacgctcagggtcaccagggtgccgaggaatgaccttctgtaacctctggaaaccataatcgatggtgggttcgttgagcgctgtataaatgaatctgcctggtgttcctttgcagaactgcttagatttgtaggacagtgtgacttccacaacaccagggatgtgccgaggaggggtctgcacacggatggcatgaggagtgatcaactcactccagaccagcatggtaccgaatatgacctgtaacccatcaaagaaattgtcccctatgatgatcacagtcgcacctcccgtcgtccatccttcactcgggctgatggctttgatacagggagtagcatgttccagataagagggcgtaccttccgaggggtcaagcctccgagccctccgcccatgcttggaattattatggacaaacatgttatcagagactgccaggacatggccatccacattgactgtcgtagacaccacgacctggaatctccgcatgtcacgtgggtttcccgcattctttaggcaattttggttacatttgaggaaaaatttcaagaagaacctttggcaggaacccagggcaggttcaggaaacggttccgtgttcctgcccttagctttgtgtcaatgaagcctggcacatcttttttgtggttgtaatttaaatgagacaaccaactgcacagctgtctcggtcaaattatgcagggccatgtggcctttcttccatctttaaaaagtctggggcacctctgaccatgtttgaaggaagcccaggggagcaatgaccaacaaaaggaatagcgattacgccagcaaaggatggaaatttgcctaaatgaatatattaagggctgcgcttagaaaatggaaatgttagtttttaaatagaggcagaatagtgttatgattaaaaccctgatctttggggtcagacactgcaaggttggcatcccagctccaccacttaatagctatgttgacgttgggcaagttatttaaccaactgaagccccagtttcctcatctgtaaaatgggagaaataagaatactcagcacatagaattgctgtaaggattaaatgagagaatacccagaattcagctaatatgtggcttcataaatggttagttatcatcagtaattacagtaatgacaataacacatagaacatgcaaaacgccaatgccagtcactgccacaccagtcatctgtaaccaagaaaagactaattttactctgcctctggccccttattttacatattacagggatttattcttgcaggcaaaactaatgtgactgaagtttctatcattcaagttttatttattctgttgatctggcattgggtattttaacccctctctccctctctctctctctctcacacacacacacacacacacacacacacacaccccagacatgggaatgtgagtataagcatctgcatagatgcacactacaccaatacaagccagcagatatgcagacacaaaatgagtatatgtaccccggaataaaaggaacataattaccaactttattttgacaactcttttcaatgatacccaattaggcattgcatggcaaaaataaactctttaaaatactgaaagcacaacccattgtatatttgctcctaagggccctttaaaagctgaggttaaattaccatcagatggcaagaggataaggacctcgccttagggcacttccttgggataaatggccagttcttgtcctctttggaaggggttgctggcccaaagcaccatgaggccagtgaccccttgctggtcattaatcgttaccgaattccctagaaccaaggtcattattgctaatataaacttaaataaaaattccagagacatatggatttcttttaatagttagtcttatttctttgctttttatagggcatttctatagaattaatgttctatacattagctctgtagttggtttgtcttaacacttgatcctgcttaaagtaaaaggtttattggacctaaaataagaagcgaaggaaagcaaacaaaaaaacaggaaatcctgaaagggcctattctgtacctggaattctcagaaaaatcattatccatgggactcacaattttatttctttggaaacctgtcaaaatattataatgtttatatttaacggttggataatttaaaatttaaaaaatagagagagagatctggttcccatcctggacaaagttttctgtttctcagtctctctctcgtctcctctgcacatagaaaaaaatttttttcaagattttatgaaattccaatttcttcaagcttaaggaatatatactgtattgtcactcacaagcaaaggatattagcagagcatataatttcatagcttcattccaaagatgctcagcattatttgccttaaaaggaattatacaccctaaaagtacagaaacaaagtggatatgcagaaaatgaacaattatttaatgagcatgtactatgtgcaacttagtgtagattctctgtatatcaacattaggctgcttcatctggaagacaagtctcaaccagattaagagacaacttgaggatgttgcacaggcaacctctgcccacaaccttttggggttactatctcacagagacaaatgtgttggtccacgtgcctcacattttacaagcctacaattttctttttactagatcccttccccatcttgcccaagttatgctaccaataaatttaaatataacaactcaattagccttgtaaggtgcatcatctaaagatctcacccactagcttcctgccttaaggtagattttagcaatagacatgggctgtacctgctgccttatcttcttattacctggctgatcccttggatgaggtaaggaagaagaactgaaagttgattgagaatattgttggttattcagttctgacctctgtgaggttgctatttaccttatagtacatgctacttaagcacatgtttaataataggtactgtccaatgtcagatatgagaggtaaccagatttataagggtagagaggattaaagtcattgagagaggtaaccttaaagatcctaagtgtttacttctctcgttctataaataagaaagctgaaatccagagaagttaagagacacacagacacagaggctcacatatctaaataacagcaggggcagtactcaaaaccaggtctcctgtgtcccagttcagcattctacatgaggttccttctcatttcataatgaatgagaagtcccatatcagaatgagcaatttaatgtgtcgagcctttaacagaaccaaagcatgctttctccttaacagaagaatatgcacaaatttgggttcatattagaactattagtaccttgaagatgaaaattattagcatagtagggaattaacctacactaaatctgatgagtagtgaattactttaaatctctttttggaggtgggaccttaccctgggaatggccaggtaatggcaggagaaagatgaatggcaatggatttggtggtgatttggaaaagagaaagagattctacaccaaatccaatttccttaataggtgagtgccctgggaggaccacaaagtgcttctggggcagtccccaatctgggattgggggtacaacttattttatatagtagatgcttcacgaacatttattgaataaattaacatgctgggtcctttgtttctcctgtctgaggtcaatgaactcaacagctgcttgtcctcaccacctctgtgaatgtaaacaatggtttctaaaggagagactaaccctacatgaaaccattttttaataggtttagcatgattatcctttctggcttctggtatcaaactatttgggagcagaaaggaatccagcctgttgaatgatttatgacaatttgggaagagaaaaagagaagaaaagagtatacataaattcaaaattccaccttttaaaattaattttagtggattgatactgggaagaaagatttagttggttgactacattcagtcatatatttctgtggagacggaaaaaattaaatttttccaaatcagcacaatcttttcagccagaccagatagtcaaataattcagaggtgaaataattgtcacttcctcctttgccccatactctgaaacagtacagaagctgccaactccccacctctccctctagcttaccaggcgaatgaatgcccctttgccttctggaatcattctcctgcagttcagcatgagactatgccaggggctaataatttctctcagcaccatacccatgacttctgcccttccttggcaattccaaatgtgtgacaaacctcttcgggcttaggcaaaactgtacacaaaagtggtttgagtaggaagaaatacagtgtacttttttcccctttcactacaattttttcagaattatattctgcaacaatgcctcacttcctttattattatttttggaaagggtactttcaatttgtttaggtttaaataaaagaaaaattttattaagacttactttgaaaattgccaacgtcaatatttatgtatgtcagtaccttccagagaaagataatagtcagagacaactgctcatggtaagacatctggaatagaaagaccttttgtaaaattcctactgaaagatgactattgatgaaatacctctggcaaacaaaaacaaaaattgcaatttgtcgcacggtgttatatgacatagtatgaacaagcacagttgcaaataaatgaaatatgtgggcttttaaaaataaagtaatattttatgatgggatattctgtagcttcctcctccctgtgactgttataatttctttcttttcttttcttttcttttttttttttttttttttgagatggagtctcactctgtcacccaggctgaagtgcaatggcaccatcttggctcactgcaacctccgcctcctgggttcaagtgattctcctgcctcagcctcctgagtagctgagattacaggcatgtgccatcataccaagctcatttttgtatttttagtagagacgaggttttgccattttggccaggctggtctcgaactcctaatctcaggtgatccacctgcctcagcctccaaaagtgctgggattactaagcatgagccaccgcgcctgacggactgttataatttctgagaaacaatttaacttgtgctccgtgcacaatgctaggccttgttagagatacaggacttaggggcttccttggacccaaacccagaaaagacacgttgtacccttccctaaggctgattgcacacaaggtgaaatggagagcagagcaggacccagatggcccagagtagtagtagaaaagccactggaaccagagccagggacttggcttatggtcctggctctgagactaattaggtctttgggcaacattgctgtgcttctcttggcctcagctttctcatctttaaaatgaaggggctgaactgtaatctctgagagtccactcagcttaaatggaatcgtggtctcttcctacaggaatctagattttttggaaaacctgcctttgggatctagctaggctatgtattagcgttcttaagctattcattctccatatttgtgaaatgatacaaaaaaatcctgcttacctcactgtgttgtcatgaaaactaaaaagagctgaacccatgtgagatctttatgtcattccctcgaagaggtatgtgaatgatagaattaaagtgctagccttccctaagttttgtatgtcttggtatacattgaaggttcttagctaaagggatgagattctgacagtggaattccaagcatcagccagaattgggtgggaaaacctttcctgcattctcatgagctctgcagatagtctttattgtttttaaacccagccgtttaatcagacctcaaggaggcttttctattggagcttacagacttgtccaaactaaaaagaatatctaaacctggaggagggggatgtaggagggagaatgagtaagaaaatgttttgttaatgaataaagatcctgtatttcattcctgaaagctctcactttgctttaggaccatcagcagaagcacagagctagcttaataagctgtaggacgtgaaaaagtcactggtaggtccagggaagttctcagctgaaggggaccctggggaattgtccagtccacccccagccctaccttgcaaccagacaaatgaagctgtctgctagaaaatctggagataccctttcacatttccacaatgacaaagttgtgtgtgggagtccccaggaatcatttataactgaaagaaaaggaaaagccaccttcaaactccagttccaatagacctgagatctttccggaaacccaaaggaactgcctcatttggttttcccagagaatatgaacaacagatcaaactaatccaacctagtggaagaaggatctgtagagtttgggctaatttcttagtaatattcagctgcagccacttcccttctgtttaattttcacgtatcttagtgcttgaattcgtaattcatacccttgttttgaattcccactaccaacagattccataaggccattcatgtcaaacaccctccaaacagttccaagaaaaggactgagctagaattcttttctgaacagtcagaggggctatggacctggtttatatgagtagcatgttctcataacccccaaatccttgacagacattccagggacatggccacttctgccatgtagccaccatttcaatcaggcctcctcaaacaacttactcctaatttctacaatatgtaggtggcaactgtagcccaacgggtgtccgtagatacaaaccaaagctggctaaaaccatgtctggaaagctgacaaatttccaggcaatctaccctgagcagcagacagaaataaaagagctggtaagaagagaaacagacatataatataacagagtttcctgaaattcattataccaaacttccaggatagatcaaggaattggacctaattctgccctgattattttgggtatgtcattatcaatgttgcagaaacatttttaagccactgtctatcaacaatttgatgaaaaaaaaaaaactaacatttcacgagtaatgttgagtgcacagtgattttgaaagaatcactattagtaaactaaacagcactctaaataaagaaaatgactgctgttaagacatactgtctgagaattctcaggaagaacaccacaacgctaactctgctgtatataagaaattattccagtatgcatttgagtaattctgcattttaatttaaccctttgaaacattaatcaaaccatggctaattataggaattaaggaattaaacgatggaatcttctaaaagatattatttaaaaggcagtttatacaattacttgtatagatgtttgctttaaagaggaaaacagttctactgtaatgaaaagggtcttagaaaattaaattaacaaggggggaccaggctgatatgaaactaaattagcatcaaatgcaaattacagggtacttaatggtagaaacaggtgcagagaagaaccctaaatgagataaatgaataaaacatccctctccacaaatgtggaagctgacacaaagtcaatgatatgaataattcagcagcctccacactgctgttgaggtcagcctgccttgacctttgaaacaggaagtaaaattcagttcaaatttgagtgactagaaatataacagtcatttgttttttatattaaaaaatcaacagaattttttaaaaatacaaatacagaaaatataaaatagaattacagtttgaactagagacattatacaatcaaagtacttagtaaacaaacaaaataatttgataagattttacccaaaccatacttcaatatggaaatcctaaaaataaaaataattaaaaacatatataccagtgctcagcttaatgaaactccctgtgagaataaatttttaaatcgttatcctttcttcaaagtattttgttgtgttgctatcaatgtaaaaaaagcatgtcataatttttaaaagccacatattcttattagtaatgcaaaataatttctcatatttgaaagataaaatttggttaaactagatttttaaaaatctatgtaaagttgctattttttaattcttcaattcctgattgaataaatactgcatcctccaaaactattcaccttagaaaaatgcaacctaggttctaaaaacaaactattctcataaccgaatatctattgtggttttacgtgtcttttatcctttttttttctttttgcatgcttcaaaagtattttgtacagtcaaatagtgaaagtactctcctcatttcaaattgaatttagtgctgttagagattaacagggtatgacaacaaaccaatttctacaagctagaaagacagcaaaatatatatggtatatcaccctcgtccttattttacaggatggcataaaagatgtttgataatagcagttatctctgccctccaattggttctattaaggggacccacaacttggctatctacctttcatctatctactgtgcttgtcagataaaagattatgttgaaagatgagcttaattttattttctagatttagagagggttaaagctacatacacacacacacacacacacacacacacacacacacacatacccctcagccatctatgagagagcagtggtaaactaggtctatgattgtaatcactgtaggaagaagtttgagaaatgttccttccaaaccggagtgtttagttgaggcaaaattaaagatgcagggtgtgctgggtatttcttaattattattattattattatcatatctgctaaatcactcctcgctcgacatttaatacagggtgatagacaaaacactgctgatttggggtttgccataatgactgacctgagcaaaggctttgtgtacaaagtggctccccattaaataagggctctgtggaaccagctggttctcattttgaaacaaccggtttctgtatccccaagtgctaaagaaaataatccctgccatctatgactgcacactttcacagaggcagcaacgagaatttgattgtggagataattaaagtcattcctggaacttccaagaaaaaaaaaaaggtggaaagaggtggggtagaaagaaagaatagtcaatgatagtgtttaaaattaaactatgacaaatcattttgagtggagaagagggaggaggagcccccgccctttatggaattcagttgaaacagctctgttttcttccccactcggctgctccagagggaggtccgagatgcgattagtcagggcgacggcccccagtgtccggctcggaagccgaagaatcgaaacatggctcaagaagctacttgtcactgatgacacatcacaatgagattgttttgttttttttttttttacgtttcaatcctaaataaaatagccgcggaggaatctaactggactcttcaacaaacattctttcctagttgatctgaaatgctgaggttagtttaatataatattaagaaaaaaaagagtgtatcagacattcagagacactcatctttcaatcttgaggagagcttattcttttattattttttgaatgctacattgttctacaataagaatccatgttcaaatagcctgaatgacattcagctgaacctacgttccctgcctgcctacattatttcataagcttttgggaaaaaactaaaatatgtgtaatctgtctgtctgcgctatctgcctttaacaggaagaagagatgggctcaatgaggacgactcacggcctctcaattaacctgattagttcagcacattgctctcatgaatgacaccttatcttaaaataagggagaacttccttcctcgagtagacacaggagccccctaaagccacaaagatgcagcctatcaaatgtgagggcctctgcttctcctccctcttcccagctcgcaggtcagagagactagcaggccaggcgcctgattggattttgtgtcctaaggacagaaggcaagctcccgtctgcccaggtggccttggagaaggctggggaaagggatgccctgtgggtaacttcaagccccttctttcagagtcaaccaggcacatgatgggattgggggtgggggacaggaagattggggagggggagggagggaaagagaattcattaacccttcaatctccagagtatcaggtcaatgctatacctgcctgaaagaaaaactggtgaattctgaagtcttctaatagtatataaaacaaaggcgctgcttgcacaggggtctttctaacactgatttcgcgtttgacataatagaggatggctgaatttttgccctgcaaaaatcaagccttctcccaaactctctgaaatctggtggtttgcaaaggatgccacatatatatgtttttacaaaataagaaattcccattatcatgtgtaatacacatagttaatagaatatattcttgaaaatatgctttgtgagaatgtcaacagcagagattttcacttgtctgctctgtgatttacttgatcaattaaacagttaggcaatgaggagatttgcatggtaatcgtgtgaagattaacatttttaagtgtaacaaatttaatattttatcttacattttctgttcctcatcattctttaatggcagtgccatttcactttattgtgtagttataacaagcttgtctttagacagagagatgagaccaccagattcaacaactgcatttctagttcctgtcattccttcttttcacaaaaacaagccctaagcatctagtacacaggagggaggcactgtgctcaacgtagtcactgccctcttaggcttacaacctaccctccaaagcgctcatctacctgcctgtgctcagcaataccacaaacagctaaaattagaattccatagttggaaagggtcttagagatctcttccttcagtcttaaccaacatgtagactgcctcagaagagtgcaataaagccgtggaatttgcccaagttcgatacctctgggtatgagctaaaaggtgactttaacccggggatatttttcttctgcatcatgatcccagtgtaaaatggcattcttctatttttaaaacatatatatcaatatattctttgtttatacttgctattactattccaactatttttgggggactgggggcagagatcaaccctgagacactgagaaagctgcatgaagccaggaactatgtttgtctttttcactgttatacccccaaccctgaaaacagtgcatgacatataatagaggcttaataaatatttgtggaaacaaaacaatgaatgagtctttatctaaggagacttagctaccatgattaacttcagtaaggtaattgtgctcaaaggaagtcccatggcaatgatcacattaagaatgaaaatccacatggaatatacgatgctcaaattgcaagagctacctgattttaagcacctgttatgtgccaagcccagtgctaggtgtttcaatcctcacaacgcttcaaaatagaagtgacttttcccattttgaagatgagaaaactgagccccctgaggctcagctactaataagtagctgtggaggaactggatcccttagccaatgcactccaaaatctatgcctttgccatcatactgtgccttctcccagatttctgtatggattactgatgtttttttcaagcaaatacacaatcaaattaaatgaggacataagaactcaaacattgctccagcaatgagtacaataaacagtgtcacatatgtatatatgcatatatgtgtgtgtatatatatgtgtttatatatatgtgtgtgtatatatacatataaaatcctgaaagttaattgtgacatcaactaagaaagctggcttggtaaataggtttagagtaatacatgaaaatgtgctgtggatagcaagaaaaatgaaataaaagagacattatgaaatactgaaaacagtgtttttagctgagcaattgagaaaagggaaaaaaatcagtctgggagataggagatgtggagtttctaatcacttgctttgtcaccaataaagtggatagttccttaggctgtgtgcctcagtttacagatctgtcaaatggagtcaatttgtgcaaagagaattttctgagatggtataccccgacgtgctctaaaacgctggaagtgccatttaggtgtaagctactattaaactcacagtgatcaggggttttgcttgctttgttttaaggtgctcatagaccaggattcagatgctggtcttcacgagccagatcagggcactcccatttctacagctacaggaagaacaactcagtgtttaaaaccatattctgagacatatcccatatatctaacattagaatctggctttaggaaaacaacaagactgtgtagagaaacatgggttttcaactgttggtaacagcttcaaagataaccaggtgaacccttaaccaactttcttttctaaagaactttttaaaaaatgaaaaagagactgctctcttttcatctttttttttttttttttttttttttggtctctgtagagtatgtgcgtgtgtgtatgtgcgtatgtgtgtggtgtgtgtagctaaacctgatgcaggtccatagttcttcaaattaactttccattctgtgagggggcttcagccaatagtgcacccaagagtgttaaaagtgatattttcagatattactaacagatcagaatacttatgaacgagaagcacattaaaaacaggtggggaaaatctcagtagtttacctctggaaaacaataaataaattgcaagcagcatgactgtctgatattcaggtggagtaataaagagctttagtcaaatcatggttgcttcaggaaggtggaggagggaacaaccttttgaccattagaaaagttacccagctgggctcctgactcctcggcatgcaccagcagagtctaagtcgcgtgcaccacccggcaaaggcggagaattcacggcactggcggggagcagcaccacatcaaaaagcagcagctgatgtcatgaaacaaaataccctatcattttactttgataattttcaattcatcaattaaaaaagaaaagaaaaaaagttatttcagccttgaagatgtcatgtcctgagccccagtgttcacaccctacagaagggctcttcctacccacacatggtatcaatattaagttaattgagcagcaaatgagcaaaaaagttcttgagggattcttgatattgattaaaaggacattaaaaaaaaaacccaccacaacctttacatgaaccaaaatttgagaatgtcgccaaagccccataaaatatgtataatagtgacagtgtccagattaaaaatgtacatgggcagcttgattactattttctggttttttccctgccctggctctgaaagtgttaaagaaaacaataaaagaacaagtgagtgtacagggtaggatttactggcatttacttttaatctatggcccttcactctgtagcttatcgggcctctgtcagtcctttttccccctttatatttcatgaggagccccccatgctgctactgagagacagagcccaagtgtctatgagctttttgtcaggtaaaaagagaagaaaaaggaaaggaacaagaggaaaagcaaagctaagaggcatctattagatgtcactaggcttttgtattcatgtcaatgattcaggattagagtatttgaaataatcttattgagaggaatcaaaaggcccaccgagtgagaggctgctctgtagcatatggcaaaggcacgaacaatatcttattaaagatgtgttggctaacaccattactttatattatattacaaaactattgtgcctcaaacagttagcaggatggtatagttaccaagtgccattttggaggttattgtgtaggatcaatctatataatttgccagcatgtctagctcagtcatgacaagtagggtttagggcatgtttgcaactggaaccaagcacttcactttcaaaaatagaaattcccaaagcacacagaagaccactctgttcccaccgaaagtggagtacacatttcatagatggaacgccaatggcctgtccttccccagaatcagtttaattaagtttgcatcatttaacatatgtgacaccccctgccccacccatgaaaaatgtaacaaagattttttttttttgcatgactcccctccctattaggaatacatgcacagacacacacacacacacacacacactcagcttcacactttagcaggattagggcaattaaaattctattagaataagtactgtaacgttaaaaccttcttttgcttctggacaaagacttgtaactggagaaatagtttgtaagggagatttttcttcctctacccacacctttcaaggcagggagcaatgaaagacaaacctgtactgttcaccatatttcattgattgcaataggagtattgaggtcacttttatattgtcctggatagtatgtagttacgcggtttgtaaagagaggaatgggatggggggctgtgagaaggaagaattagtggtcgatttcagataacatctcatgcaaattaaagtgaccaaaataccatctctttacgcaggaaccactaaatggagttttttaaatctggtcaatttttattagagagttaaccgggtgctggcaggagagggaaatgaggaaatgaggggaatttatcaatggagagttacacttggagagagtttttccccccattctaagcaacttcttttaggaaagtaaaagcatgtttaatatactcatatattctcattacaaaatgattgtgcatagttactaatgggacacacagaggacttcgtactgcttttctgtatttttccagaactgttacaaaagcaaagttatgatgacatgggattaaaaacctacaccacgggctgatacccgggccatgctacacatacacactactgattctctgaagctccgttaaatacatttcttggaagttgctgccattatttcctttacaggaaaaccactgttgttcattatacagtgtctgcaatagtattataccatgtaaaagtactttgcattatgatacattgtcagcgtattcgaaatgcattttaatgcatcctggttgtgtatttgggaatagctgatagcaaatggaatatagactgcgattagcttattgtattagttattttcttatcacggtagcaaactgcacacaaatgtacggggctcatctcatattcagaatggtattatctgatatgtgataaaatttagaatgatactcattcacataagtctcatcgctaataatcacatatgaattcccactgagaagacaaatgtttaaacacactaaggttaataaacagtcttaaattcatgctcagtgtcaatgctggcttttcacttttgaaaaaatgcaaacctctcaaaccaaccaaaaacacaataattatcctgcctagggcaattttagagagtgaattcctcctccttttattttaaccaagcagtcaaggttacaaatcaggtggtataaaaggtttatcggaacgctgagaaatgcatttacacctctggttcttcataccccacacagccatttgtgtatagtgcagaatgattatgcattggtggtggttggtccttctaaaaactggatgaagaccaaaataagaagagttgaaagggcattgaaatgaaatcatgaaactaactaaaagcctcatttgcaactttaataaaattatatatttatgttcatgttaattgaggactttatgtggatgacaaaaaataaataaatattggaatttacctctgattataaaagacagaggaaagccattgattgttgaaaggcccagatgcctttacaatccttggcaaatacataccacacccgacccaatggtaaaaagtatgtgggtgggtggatggatggatggatggatggatggatggatggatggttagatagatagatctctcctaactctaaagtttttatattgttttcctattatacatatgggcatatatgttatataaatacattggtgtcaatttaatgaagaaaattagcttggtgataaggcaacactgcacttttctgaaaagtcttaccacagaatttacacctcttagaaaaagaatgagtcttcaataaacttgtttatctgagcaaccataacatggttaagcttttccgttcatatgatgtacatcatataaaatcaacaggcaaatgggcattctaatattttcattactgaacattctatttcagataatcataaaacaaacccaattcgtgttacctaaatggaagtgatctagatgtggaagatctttagacaaatctggaaaaaagaaatacaggcatttttttcctttataggagacccttgcgtaagtgtgacccgaagtaattccaaacagactaggtttttcattttacaaaatttgtgtattttttttatgtcacatgtcaaggcctacatcccatagccatacacatagatacaggaattcttaaaaatgggggaaaaaggcatggtaattctgttaatattacaataaacaaactcaaaattcttacaggtacataagttgacaagcttttaacatccaagttttaaatatcggctttgaggaacccaaaacttttaggttactggagctacattatatccttaaaaaactaggtctaaattcacaccaataggagaacataatttgagatggaatttcatcctttagtatttctatctactaaaaaaaaaatccacttgttaacagataaggattcattgcacaaggaatgatgctcacattgtcacccttacttaatggttcatttcatcaattgcactaattctaaattcaaacaaacaaacaaacaaacaaacattaagctgccccctatcccaccccactgcaaataagcaacagaaatctagccagaaacttcaggagtctgtgtgaaaagaagcctccagcatactttggagaaagaaatgtttttataagaccatctgtattcatccatgtcattgctcaaagatagtttaggaaaataaagagtttggggaagcaaattaagaatgaatggtcatcctaaccagatatggaataacagtctgcatacttaatatattcagttccgacatttattaaaaagtttccatatagaaagattttttaatagatgcagaaaaactgggttcccaattcagactaccctatgtgacttttgtcattatcatcttttctgattcttacaaagtaaacctaattaagaacctccctcattagtcttccagaaaaattagcacagcttatgctaattactcctgcaaaatttaataaactcgttgaaatgggaatagtctaatgaggttttatttattgaactaagataactccaaggaaaaaggttaggacacaaggatatccaatgtggtaataaaactcctatttattcaatttctaaacatgaagtttattgcaaaccttttaaattcaaatattagttactgtgtcaatatgtaaaatcaatctccaccttaattcaataactggaagtcattttttgctttttactttaacaataattaccacacatagccctttacctcaaaaataatgaaatctgctgttatcagttcctggttatttgctattaaacataacacatttgacttttcccatgtctatgcagctcaaatatctggatcactgagtgcaggctgggttatgtgcttcttaatcaagctatttggcaccacacagaaatgtaacctggcattcaactccagatgtgcacttcctgcatttacagcaatttttctataaacttttttgaagtgacttgacaaattgtcatgattgtaaaaagaattggggtcatatgtttctcagtctgtgcatgccataaggatgaagtataatagaagccccttttctaaatcacagtttgcaactgctgattttgttaattctacttttttgatagaatatgccaggctgatgtcccaaagtcagtggcagcaaataatacagccaaaatttaacacagaaatagcttgccctgcacgattgcactatgaccagaaagtctcttctctctaccctataaatagttttcctgaataaaccactgctaaaagtcttttgactgataaaaatagtagtgttctcccaaattccgaaggacaagcaaagagagctaaaaattattggtgctcaaaagttgactgcgtgttaaaactatgctaaatcctaacgcaaggatggcctgtaccctcagctctgtaattgcatattgtatgcatcttttgaaaacagttactattgctactgaatgcaggcctcatagcctattttcacaaaatattcagggatttgcatccataaatctgaaagcaaatcaaaccctaagcacgtaacacagatattatgcaatcagtaatatagaatcaaattggaaactatgaaattcaaacacggttgccatcattttttcccctttgcagcaattttatggaattgaaaaatcttttctattttgccctttcttgcataagttcttctcttgttgttattctcttctctcgctgttaagaatgggagtttcacatatcagcacagacaggactggagcttttaaaacctttggcagcctgaaggacaaataaattctgaaaactcaggtgcaaataaaaatagctaaatggggttttgcatatcaactggcatcactgcatgaaaagatagttcatcagaaacaatggcaacagccagcgaataaacatatgctgtggggcttgtgcacatacactgagtttcagctgtttttaaagtactcctatctgaagagaccaagattggctacacactgttttctactttgtcaaaccaaaagggaaaaaaaatgaaaaggataaatgtcatgagtaatatccccaaagccaccaacagcataaagtgcatacttattttgcctaaattgtttgaactaccccagccaagaaaaggttttaagtacccttctgggacagatgcaaagcggcaacaatagaagccacactaatgcaatccaggtaacacaatcctgtttcaaaaacaggggccgggctaattacagtgctgctgagtcaagtttcttatgccatcgcaacccacaggaacaggtcaaaatcaaatgttattcaaaccacagtcatatcaaccttctatatcagagtcacagcttcaaaccaaacgaagaacttaaaagcttaacccattcacaagcgaaaaaaaaaaaaaagtcttttcattgagggtggcaaggtaaggttcttgtcatcatctaaaccaaaaggaactacatggcagaacaaaatgcttatagtttcaaagttttggggactatttgggctggtcctttgatccgtacactttcttttcaacagaggaggaagaaaaatgcttaaaataacaaatgatattttggagaggtaaatttaaataaaacaaaccagcataaaggttaaatttacttgtgaccttattcatttggagacttatgttcaatcacagaaaaagcaactatatgaacagtatatctgcttttgtagataaacatgttatcctaattctataggtagcacacacatcaccatatgtcaaactttctcatcttttaactttgaatcaaatatactaatactcttatatggagcaaaaatatatatattttagtgaatactagtgaggaatatttagttaaaatatctgattgaaatgtaacctttataaagcttcttggcaatcaattgggtttatgcctgaagactcacataagtcaaaatcaacaatcgatcttttggcataaattatgttgaagcgaagtaaacatcttgttttttgttgttgtcattgttaactgaaaaatgataaaacaagcccaaaaaaggtagaaagaaagatgggtttttttttcttttgttgttgttgtcaaaaatcaatattgctgaaacccaaaaagggacttgtgttcaaccattggtttcctcaatgagggatcggtcagtcttattggcaagactctttttccagctagtacaagatgctagctcttttcctagctgacaattgacagtatctataaaccttccaggccatttaactctcaatgagtaatgctatgtaacaaatggtttatcatacatgtttccatacaatgaatttcaataattaaaatgtaaaatgaatatttggaatgcgactttgcataatgcgtgcacactgactcaaaattacaccgaacaactaaaacagatttattgttctacggtgatttacttggtcatgtcagattagtaatatggatctgtttaaaaacacaaaaattaagacaagcaggataaattaatcaacttacaatatggtctcatactgcaatcaaatccggcaaataacagtagaaaatcttggttcacagatctctttaaactgcttttatgcataaataaaaccttaaagtgtagatggattacgtccaacagaactactgtagctaaaagtgataatgattcaaacatttttcaaataaaagttaaatatttataagcacccaaccacatttcataaatcacaaactattattattttatttctgaagcttcctggcacagcatgaggattgagccacagaaagtcaggaaagaaaaaatatattcctttaggagcatgaatcagacaaaaaccggagcaatccaaggaacaggcctctaaaagaacattccatatggctttcccaggaatcaaaatcgctcagcacagcgtaagtcatgaccaacaggcaaatttcagccacatgcattcctaaccctcgcccatgagcaacacaagggcaggtgtttcattataatgaggaataagaatccagtgaaagaagagtggt

SEQ ID NO: 18033 - RNA, 4649 nt, Homo sapiens
  source 1..4649: mol_type = other RNA
tctgccatcctccctcccctaccctcccacaactcccctcccccacccaccccaacccataaaaatcgcactcttgacagcctagtgaaaaccattgcaaaatccatatgggggcatgcacagttgcagcattgttgtaaatgatttcttgctctactagaaaaagttacattgtcttaaggtaacaaaacagttcttttgtgcttttcgatttctttgtttttttttttttctttttttctttttcttttttcttagaatgttagtgatgactgacagttctggtgcacagttacaatgtacaagtgaaatgaatatgatttgcattgttaaggcatccaatctgctggtttatatttatgtgaaagacagaggaaatatacaagcagacttaagaaagaaagtatgttcattgatttctatgaagtttctccctagaatttaatgcacaaaatgcgtcactccaaagggagagattccatgcatattaatagagtaaaacagcattagggttgttttgtaagcttccaaagcaaaggatacatttttttttaaatctactgaactaaatactacaagaataatatgctactatttttttttttttgccatatattggaaaaaacttcttaacttacaaataatacaaaaatagacaatgacttttgggtggaaattaaaaaaactgaagcatggtttataacaatactaaaaataactataaatgaaatgtttaaaaatcacattgaaacagctaatacaagtgtaggtgaccaaacaaatacgcacttttcacgtagcaaacatacacaataaaataaattgggggtggaaggaagaggaagaagggaaaagcaatgtacaaattcgaaagataaatacattatttatatggatattttacaaaatcccctttaaaacaaaaagccttttaattaactttgcaagtatgtgcaagctaaaggtagtgagctttttttctttgcaaaatacgcagtaaaatctttttgtgatattgaaaaaatgtcttaagacattaaaatgtataaatagaacaacaactttggcaaaaaatcacaaaaaaaaaatctacagtatttataactacatacaaaaacacaagagcaaagaaaaaaatatcaggcaaatgcatcctcagagctttgctgcatctttgctattaattcttatttttaagaacacttcccagataatgagagcaaaaattcccatagaacagaaaactatgttttggaggtctcaaccttcttttcctttctccacccccggttccctttaactcttaattccaaagcacttaacctgttgtttcaatctattatgttacaaatggtaagggtcgactgatagaggcagtatctggaatgggaaaatcgaaaatacctgccacgttgcttttatcaacttttggaagataggtatgaagtctgcatttaggacgagtaaactttaaacttgcaaatgggggagcgtacgtgaggttttggcttgttaactggagggcagagtgtggaattctgtgcctggaccctgttccatgaagtctcaaaggagattctcacacagtatgtgtgccaccaagctctcgagaggccatcggcttcagaagaaactgacttaagtaaaaggagagaatgagatcagatttaaatatgcagttttaacaatctgtctagaggcactggattttcgagtagagggaaaaatgtgatcacttacatcgcgttttaactttccaggctgcatttatttacacagttgcttaagacaacaatacaaaagagataaataagcttgcactgctaaggggtggcatgttaagttagatattgaaaatgcactgtctgagctaactaccatttgatatgctttaaggcgcaaaagccgacccttagtttttctaaaaaatctaactggcattcctattctgtcccatacaagcttttttttttttcctttttttctttttttttttttttacttttttgtaaatatcaccacttcattcttcctttacacagctttaaaaacatcataaattaaaacatggagtcttatttatagtgtcccttgtatagagctttacggtttataaaagacaaatgattgcagaattaagcttaaaaaaaaaaaagaaaaagaaaaagtggatttgcttttgtcaatacagaataaatatatcccccaaatacttgggaggtacaactttaaccaacaccctgcacttgcagatccctcttccaatttcagtatttgcaaggtcggtgattttgtttgtttaaaaatctgcagttattgtgattcctcttaaaaaggcctgagttaaaagttccactctgggacttgtatcagattactctctgtagcagaatccaacctcttcattaatacaattcttcaaggcaattctttcacataggaggaacaatcatgccagatatcgcttgcaggctgttcccgttggtgctggtgcaggtgggaggtggggaggtctggggtctgacgactggtgcgaaagcactcttctgtttcacggctgagaccatgttggctggtgagaaggagaagatgcccgaggagctgctgcagttggaggggaggcttgtggaggaggccatggtggggctggatggcactatggcatagggggagttggcagctgagccgttgaggaaggtgggggagccgcccaaattggacattgcggcagagccgtatccgttcatgctcgtggtgacggagttatagttggtctgctggggagtggtgctcggcacgtacccgtgtggtgatacgctgcttgagttgcgggtgaaaccctgattggtggcttgtgatgcctcggagacattcacggccagttgtccactgaacgaattcacgcccatcatccctgcgtggaccgaggtgttagcaagggccgggagttggttgtggttgcggggaacactgtacagggcctcggcaatgtcggccgctctcttcagaatgatttcctggttgttgtgtggcatcccatacagtgcttctaccagatccgcagcccttttgagtattacttcctttggcaaacgctcagggtcaccagggtgccgaggaatgaccttctgtaacctctggaaaccataatcgatggtgggttcgttgagcgctgtataaatgaatctgcctggtgttcctttgcagaactgcttagatttgtaggacagtgtgacttccacaacaccagggatgtgccgaggaggggtctgcacacggatggcatgaggagtgatcaactcactccagaccagcatggtaccgaatatgacctgtaacccatcaaagaaattgtcccctatgatgatcacagtcgcacctcccgtcgtccatccttcactcgggctgatggctttgatacagggagtagctgcatgttccagataagagggcgtaccttccgaggggtcaagcctccgagccctccgcccatgcttggaattattatggacaaacatgttatcagagactgccaggacatggccatccacattgactgtcgtagacaccacgacctggaatctccgcatgtcacgtgggtttcccgcattctttaggcaattttggttacatttgaggaaaaatttcaagaagaacctgtcaattatcactggatctgagggagtctcatttcggttgccacagcttttcttgtcacaacagcggctgcacatgatctcatgtgtgagcaagactcggcacatttctgggttcttgtcttggccttcatacactatggcttgttttgtcatggagtcaatgaggcgcacgtagaaatcctgctccgtccttatcccattgctgtagagaagctgaagccggtagtgaattccgttattggtcttttcgctgttggcttctttttccttctccacgaaccccacaaacgctgtcctctcgatctccacgggctggccctgtctgtcgtagagggccaggacgaagtggaagaagttggatttccgcagattggaaggcggctgcttctcaaagtgagcccgggccagacccaccccgctctgcgccgccgtgttggcgtccagcaccccggcgccctgcatccacgtccgcaccgcgttcatgccgctgcccagcggctcttccttcatgctgcttccactccgttggatgctttcctgaatcccaaacatgaaaacaaccttttcttgtggaaaatctcctcccccttgaaaaaaattaaaaaaaaaaaaaaaggaaagaaaagaaagaaaagaaaagaaacaaaaacgccaaccagagatttttttttttctcagacgatgaactcgcacttagaagatcaaggcgggctggaaagcaaatttttaaaaaatgtaaacctctgctcaaaactgagcgataacccgaaaaaaagaagaaagggaaaatccaacgaaaagaccaaaataataaaattagagatgtatgcttggctgttgggggttgtttggttggttgatttttggtttgggtgctttttttttttttttgcttttttttttttttttttgtaatgatcacaggccggtggaggacaggaggggctggagtttccttttgtagaggtacccttcacttgaagaagcagg

SEQ ID NO: 18034 - RNA, 4744 nt, Homo sapiens
  source 1..4744: mol_type = other RNA
tctgccatcctccctcccctaccctcccacaactcccctcccccacccaccccaacccataaaaatcgcactcttgacagcctagtgaaaaccattgcaaaatccatatgggggcatgcacagttgcagcattgttgtaaatgatttcttgctctactagaaaaagttacattgtcttaaggtaacaaaacagttcttttgtgcttttcgatttctttgtttttttttttttctttttttctttttcttttttcttagaatgttagtgatgactgacagttctggtgcacagttacaatgtacaagtgaaatgaatatgatttgcattgttaaggcatccaatctgctggtttatatttatgtgaaagacagaggaaatatacaagcagacttaagaaagaaagtatgttcattgatttctatgaagtttctccctagaatttaatgcacaaaatgcgtcactccaaagggagagattccatgcatattaatagagtaaaacagcattagggttgttttgtaagcttccaaagcaaaggatacatttttttttaaatctactgaactaaatactacaagaataatatgctactatttttttttttttgccatatattggaaaaaacttcttaacttacaaataatacaaaaatagacaatgacttttgggtggaaattaaaaaaactgaagcatggtttataacaatactaaaaataactataaatgaaatgtttaaaaatcacattgaaacagctaatacaagtgtaggtgaccaaacaaatacgcacttttcacgtagcaaacatacacaataaaataaattgggggtggaaggaagaggaagaagggaaaagcaatgtacaaattcgaaagataaatacattatttatatggatattttacaaaatcccctttaaaacaaaaagccttttaattaactttgcaagtatgtgcaagctaaaggtagtgagctttttttctttgcaaaatacgcagtaaaatctttttgtgatattgaaaaaatgtcttaagacattaaaatgtataaatagaacaacaactttggcaaaaaatcacaaaaaaaaaatctacagtatttataactacatacaaaaacacaagagcaaagaaaaaaatatcaggcaaatgcatcctcagagctttgctgcatctttgctattaattcttatttttaagaacacttcccagataatgagagcaaaaattcccatagaacagaaaactatgttttggaggtctcaaccttcttttcctttctccacccccggttccctttaactcttaattccaaagcacttaacctgttgtttcaatctattatgttacaaatggtaagggtcgactgatagaggcagtatctggaatgggaaaatcgaaaatacctgccacgttgcttttatcaacttttggaagataggtatgaagtctgcatttaggacgagtaaactttaaacttgcaaatgggggagcgtacgtgaggttttggcttgttaactggagggcagagtgtggaattctgtgcctggaccctgttccatgaagtctcaaaggagattctcacacagtatgtgtgccaccaagctctcgagaggccatcggcttcagaagaaactgacttaagtaaaaggagagaatgagatcagatttaaatatgcagttttaacaatctgtctagaggcactggattttcgagtagagggaaaaatgtgatcacttacatcgcgttttaactttccaggctgcatttatttacacagttgcttaagacaacaatacaaaagagataaataagcttgcactgctaaggggtggcatgttaagttagatattgaaaatgcactgtctgagctaactaccatttgatatgctttaaggcgcaaaagccgacccttagtttttctaaaaaatctaactggcattcctattctgtcccatacaagcttttttttttttcctttttttctttttttttttttttacttttttgtaaatatcaccacttcattcttcctttacacagctttaaaaacatcataaattaaaacatggagtcttatttatagtgtcccttgtatagagctttacggtttataaaagacaaatgattgcagaattaagcttaaaaaaaaaaaagaaaaagaaaaagtggatttgcttttgtcaatacagaataaatatatcccccaaatacttgggaggtacaactttaaccaacaccctgcacttgcagatccctcttccaatttcagtatttgcaaggtcggtgattttgtttgtttaaaaatctgcagttattgtgattcctcttaaaaaggcctgagttaaaagttccactctgggacttgtatcagattactctctgtagcagaatccaacctcttcattaatacaattcttcaaggcaattctttcacataggaggaacaatcatgccagatatcgcttgcaggctgttcccgttggtgctggtgcaggtgggaggtggggaggtctggggtctgacgactggtgcgaaagcactcttctgtttcacggctgagaccatgttggctggtgagaaggagaagatgcccgaggagctgctgcagttggaggggaggcttgtggaggaggccatggtggggctggatggcactatggcatagggggagttggcagctgagccgttgaggaaggtgggggagccgcccaaattggacattgcggcagagccgtatccgttcatgctcgtggtgacggagttatagttggtctgctggggagtggtgctcggcacgtacccgtgtggtgatacgctgcttgagttgcgggtgaaaccctgattggtggcttgtgatgcctcggagacattcacggccagttgtccactgaacgaattcacgcccatcatccctgcgtggaccgaggtgttagcaagggccgggagttggttgtggttgcggggaacactgtacagggcctcggcaatgtcggccgctctcttcagaatgatttcctggttgttgtgtggcatcccatacagtgcttctaccagatccgcagcccttttgagtattacttcctttggcaaacgctcagggtcaccagggtgccgaggaatgaccttctgtaacctctggaaaccataatcgatggtgggttcgttgagcgctgtataaatgaatctgcctggtgttcctttgcagaactgcttagatttgtaggacagtgtgacttccacaacaccagggatgtgccgaggaggggtctgcacacggatggcatgaggagtgatcaactcactccagaccagcatggtaccgaatatgacctgtaacccatcaaagaaattgtcccctatgatgatcacagtcgcacctcccgtcgtccatccttcactcgggctgatggctttgatacagggagtagctgcatgttccagataagagggcgtaccttccgaggggtcaagcctccgagccctccgcccatgcttggaattattatggacaaacatgttatcagagactgccaggacatggccatccacattgactgtcgtagacaccacgacctggaatctccgcatgtcacgtgggtttcccgcattctttaggcaattttggttacatttgaggaaaaatttcaagaagaacctgtcaattatcactggatctgagggagtctcatttcggttgccacagcttttcttgtcacaacagcggctgcacatgatctcatgtgtgagcaagactcggcacatttctgggttcttgtcttggccttcatacactatggcttgttttgtcatggagtcaatgaggcgcacgtagaaatcctgctccgtccttatcccttcgctggaggatttcgtccacctggagctccctgcgccccctgcccagacccggagccccagggtgaggccatagacccgacccgggcctcaccattgctgtagagaagctgaagccggtagtgaattccgttattggtcttttcgctgttggcttctttttccttctccacgaaccccacaaacgctgtcctctcgatctccacgggctggccctgtctgtcgtagagggccaggacgaagtggaagaagttggatttccgcagattggaaggcggctgcttctcaaagtgagcccgggccagacccaccccgctctgcgccgccgtgttggcgtccagcaccccggcgccctgcatccacgtccgcaccgcgttcatgccgctgcccagcggctcttccttcatgctgcttccactccgttggatgctttcctgaatcccaaacatgaaaacaaccttttcttgtggaaaatctcctcccccttgaaaaaaattaaaaaaaaaaaaaaaggaaagaaaagaaagaaaagaaaagaaacaaaaacgccaaccagagatttttttttttctcagacgatgaactcgcacttagaagatcaaggcgggctggaaagcaaatttttaaaaaatgtaaacctctgctcaaaactgagcgataacccgaaaaaaagaagaaagggaaaatccaacgaaaagaccaaaataataaaattagagatgtatgcttggctgttgggggttgtttggttggttgatttttggtttgggtgctttttttttttttttgcttttttttttttttttttgtaatgatcacaggccggtggaggacaggaggggctggagtttccttttgtagaggtacccttcacttgaagaagcagg

SEQ ID NO: 18035 - RNA, 4625 nt, Homo sapiens
  source 1..4625: mol_type = other RNA
tctgccatcctccctcccctaccctcccacaactcccctcccccacccaccccaacccataaaaatcgcactcttgacagcctagtgaaaaccattgcaaaatccatatgggggcatgcacagttgcagcattgttgtaaatgatttcttgctctactagaaaaagttacattgtcttaaggtaacaaaacagttcttttgtgcttttcgatttctttgtttttttttttttctttttttctttttcttttttcttagaatgttagtgatgactgacagttctggtgcacagttacaatgtacaagtgaaatgaatatgatttgcattgttaaggcatccaatctgctggtttatatttatgtgaaagacagaggaaatatacaagcagacttaagaaagaaagtatgttcattgatttctatgaagtttctccctagaatttaatgcacaaaatgcgtcactccaaagggagagattccatgcatattaatagagtaaaacagcattagggttgttttgtaagcttccaaagcaaaggatacatttttttttaaatctactgaactaaatactacaagaataatatgctactatttttttttttttgccatatattggaaaaaacttcttaacttacaaataatacaaaaatagacaatgacttttgggtggaaattaaaaaaactgaagcatggtttataacaatactaaaaataactataaatgaaatgtttaaaaatcacattgaaacagctaatacaagtgtaggtgaccaaacaaatacgcacttttcacgtagcaaacatacacaataaaataaattgggggtggaaggaagaggaagaagggaaaagcaatgtacaaattcgaaagataaatacattatttatatggatattttacaaaatcccctttaaaacaaaaagccttttaattaactttgcaagtatgtgcaagctaaaggtagtgagctttttttctttgcaaaatacgcagtaaaatctttttgtgatattgaaaaaatgtcttaagacattaaaatgtataaatagaacaacaactttggcaaaaaatcacaaaaaaaaaatctacagtatttataactacatacaaaaacacaagagcaaagaaaaaaatatcaggcaaatgcatcctcagagctttgctgcatctttgctattaattcttatttttaagaacacttcccagataatgagagcaaaaattcccatagaacagaaaactatgttttggaggtctcaaccttcttttcctttctccacccccggttccctttaactcttaattccaaagcacttaacctgttgtttcaatctattatgttacaaatggtaagggtcgactgatagaggcagtatctggaatgggaaaatcgaaaatacctgccacgttgcttttatcaacttttggaagataggtatgaagtctgcatttaggacgagtaaactttaaacttgcaaatgggggagcgtacgtgaggttttggcttgttaactggagggcagagtgtggaattctgtgcctggaccctgttccatgaagtctcaaaggagattctcacacagtatgtgtgccaccaagctctcgagaggccatcggcttcagaagaaactgacttaagtaaaaggagagaatgagatcagatttaaatatgcagttttaacaatctgtctagaggcactggattttcgagtagagggaaaaatgtgatcacttacatcgcgttttaactttccaggctgcatttatttacacagttgcttaagacaacaatacaaaagagataaataagcttgcactgctaaggggtggcatgttaagttagatattgaaaatgcactgtctgagctaactaccatttgatatgctttaaggcgcaaaagccgacccttagtttttctaaaaaatctaactggcattcctattctgtcccatacaagcttttttttttttcctttttttctttttttttttttttacttttttgtaaatatcaccacttcattcttcctttacacagctttaaaaacatcataaattaaaacatggagtcttatttatagtgtcccttgtatagagctttacggtttataaaagacaaatgattgcagaattaagcttaaaaaaaaaaaagaaaaagaaaaagtggatttgcttttgtcaatacagaataaatatatcccccaaatacttgggaggtacaactttaaccaacaccctgcacttgcagatccctcttccaatttcagtatttgcaaggtcggtgattttgtttgtttaaaaatctgcagttattgtgattcctcttaaaaaggcctgagttaaaagttccactctgggacttgtatcagattactctctgtagcagaatccaacctcttcattaatacaattcttcaaggcaattctttcacataggaggaacaatcatgccagatatcgcttgcaggctgttcccgttggtgctggtgcaggtgggaggtggggaggtctggggtctgacgactggtgcgaaagcactcttctgtttcacggctgagaccatgttggctggtgagaaggagaagatgcccgaggagctgctgcagttggaggggaggcttgtggaggaggccatggtggggctggatggcactatggcatagggggagttggcagctgagccgttgaggaaggtgggggagccgcccaaattggacattgcggcagagccgtatccgttcatgctcgtggtgacggagttatagttggtctgctggggagtggtgctcggcacgtacccgtgtggtgatacgctgcttgagttgcgggtgaaaccctgattggtggcttgtgatgcctcggagacattcacggccagttgtccactgaacgaattcacgcccatcatccctgcgtggaccgaggtgttagcaagggccgggagttggttgtggttgcggggaacactgtacagggcctcggcaatgtcggccgctctcttcagaatgatttcctggttgttgtgtggcatcccatacagtgcttctaccagatccgcagcccttttgagtattacttcctttggcaaacgctcagggtcaccagggtgccgaggaatgaccttctgtaacctctggaaaccataatcgatggtgggttcgttgagcgctgtataaatgaatctgcctggtgttcctttgcagaactgcttagatttgtaggacagtgtgacttccacaacaccagggatgtgccgaggaggggtctgcacacggatggcatgaggagtgatcaactcactccagaccagcatggtaccgaatatgacctgtaacccatcaaagaaattgtcccctatgatgatcacagtcgcacctcccgtcgtccatccttcactcgggctgatggctttgatacagggagtagctgcttccgaggggtcaagcctccgagccctccgcccatgcttggaattattatggacaaacatgttatcagagactgccaggacatggccatccacattgactgtcgtagacaccacgacctggaatctccgcatgtcacgtgggtttcccgcattctttaggcaattttggttacatttgaggaaaaatttcaagaagaacctgtcaattatcactggatctgagggagtctcatttcggttgccacagcttttcttgtcacaacagcggctgcacatgatctcatgtgtgagcaagactcggcacatttctgggttcttgtcttggccttcatacactatggcttgttttgtcatggagtcaatgaggcgcacgtagaaatcctgctccgtccttatcccattgctgtagagaagctgaagccggtagtgaattccgttattggtcttttcgctgttggcttctttttccttctccacgaaccccacaaacgctgtcctctcgatctccacgggctggccctgtctgtcgtagagggccaggacgaagtggaagaagttggatttccgcagattggaaggcggctgcttctcaaagtgagcccgggccagacccaccccgctctgcgccgccgtgttggcgtccagcaccccggcgccctgcatccacgtccgcaccgcgttcatgccgctgcccagcggctcttccttcatgctgcttccactccgttggatgctttcctgaatcccaaacatgaaaacaaccttttcttgtggaaaatctcctcccccttgaaaaaaattaaaaaaaaaaaaaaaggaaagaaaagaaagaaaagaaaagaaacaaaaacgccaaccagagatttttttttttctcagacgatgaactcgcacttagaagatcaaggcgggctggaaagcaaatttttaaaaaatgtaaacctctgctcaaaactgagcgataacccgaaaaaaagaagaaagggaaaatccaacgaaaagaccaaaataataaaattagagatgtatgcttggctgttgggggttgtttggttggttgatttttggtttgggtgctttttttttttttttgcttttttttttttttttttgtaatgatcacaggccggtggaggacaggaggggctggagtttccttttgtagaggtacccttcacttgaagaagcagg

SEQ ID NO: 18036 - RNA, 4553 nt, Homo sapiens
  source 1..4553: mol_type = other RNA
tctgccatcctccctcccctaccctcccacaactcccctcccccacccaccccaacccataaaaatcgcactcttgacagcctagtgaaaaccattgcaaaatccatatgggggcatgcacagttgcagcattgttgtaaatgatttcttgctctactagaaaaagttacattgtcttaaggtaacaaaacagttcttttgtgcttttcgatttctttgtttttttttttttctttttttctttttcttttttcttagaatgttagtgatgactgacagttctggtgcacagttacaatgtacaagtgaaatgaatatgatttgcattgttaaggcatccaatctgctggtttatatttatgtgaaagacagaggaaatatacaagcagacttaagaaagaaagtatgttcattgatttctatgaagtttctccctagaatttaatgcacaaaatgcgtcactccaaagggagagattccatgcatattaatagagtaaaacagcattagggttgttttgtaagcttccaaagcaaaggatacatttttttttaaatctactgaactaaatactacaagaataatatgctactatttttttttttttgccatatattggaaaaaacttcttaacttacaaataatacaaaaatagacaatgacttttgggtggaaattaaaaaaactgaagcatggtttataacaatactaaaaataactataaatgaaatgtttaaaaatcacattgaaacagctaatacaagtgtaggtgaccaaacaaatacgcacttttcacgtagcaaacatacacaataaaataaattgggggtggaaggaagaggaagaagggaaaagcaatgtacaaattcgaaagataaatacattatttatatggatattttacaaaatcccctttaaaacaaaaagccttttaattaactttgcaagtatgtgcaagctaaaggtagtgagctttttttctttgcaaaatacgcagtaaaatctttttgtgatattgaaaaaatgtcttaagacattaaaatgtataaatagaacaacaactttggcaaaaaatcacaaaaaaaaaatctacagtatttataactacatacaaaaacacaagagcaaagaaaaaaatatcaggcaaatgcatcctcagagctttgctgcatctttgctattaattcttatttttaagaacacttcccagataatgagagcaaaaattcccatagaacagaaaactatgttttggaggtctcaaccttcttttcctttctccacccccggttccctttaactcttaattccaaagcacttaacctgttgtttcaatctattatgttacaaatggtaagggtcgactgatagaggcagtatctggaatgggaaaatcgaaaatacctgccacgttgcttttatcaacttttggaagataggtatgaagtctgcatttaggacgagtaaactttaaacttgcaaatgggggagcgtacgtgaggttttggcttgttaactggagggcagagtgtggaattctgtgcctggaccctgttccatgaagtctcaaaggagattctcacacagtatgtgtgccaccaagctctcgagaggccatcggcttcagaagaaactgacttaagtaaaaggagagaatgagatcagatttaaatatgcagttttaacaatctgtctagaggcactggattttcgagtagagggaaaaatgtgatcacttacatcgcgttttaactttccaggctgcatttatttacacagttgcttaagacaacaatacaaaagagataaataagcttgcactgctaaggggtggcatgttaagttagatattgaaaatgcactgtctgagctaactaccatttgatatgctttaaggcgcaaaagccgacccttagtttttctaaaaaatctaactggcattcctattctgtcccatacaagcttttttttttttcctttttttctttttttttttttttacttttttgtaaatatcaccacttcattcttcctttacacagctttaaaaacatcataaattaaaacatggagtcttatttatagtgtcccttgtatagagctttacggtttataaaagacaaatgattgcagaattaagcttaaaaaaaaaaaagaaaaagaaaaagtggatttgcttttgtcaatacagaataaatatatcccccaaatacttgggaggtacaactttaaccaacaccctgcacttgcagatccctcttccaatttcagtatttgcaaggtcggtgattttgtttgtttaaaaatctgcagttattgtgattcctcttaaaaaggcctgagttaaaagttccactctgggacttgtatcagattactctctgtagcagaatccaacctcttcattaatacaattcttcaaggcaattctttcacataggaggaacaatcatgccagatatcgcttgcaggctgttcccgttggtgctggtgcaggtgggaggtggggaggtctggggtctgacgactggtgcgaaagcactcttctgtttcacggctgagaccatgttggctggtgagaaggagaagatgcccgaggagctgctgcagttggaggggaggcttgtggaggaggccatggtggggctggatggcactatggcatagggggagttggcagctgagccgttgaggaaggtgggggagccgcccaaattggacattgcggcagagccgtatccgttcatgctcgtggtgacggagttatagttggtctgctggggagtggtgctcggcacgtacccgtgtggtgatacgctgcttgagttgcgggtgaaaccctgattggtggcttgtgatgcctcggagacattcacggccagttgtccactgaacgaattcacgcccatcatccctgcgtggaccgaggtgttagcaagggccgggagttggttgtggttgcggggaacactgtacagggcctcggcaatgtcggccgctctcttcagaatgatttcctggttgttgtgtggcatcccatacagtgcttctaccagatccgcagcccttttgagtattacttcctttggcaaacgctcagggtcaccagggtgccgaggaatgaccttctgtaacctctggaaaccataatcgatggtgggttcgttgagcgctgtataaatgaatctgcctggtgttcctttgcagaactgcttagatttgtaggacagtgtgacttccacaacaccagggatgtgccgaggaggggtctgcacacggatggcatgaggagtgatcaactcactccagaccagcatggtaccgaatatgacctgtaacccatcaaagaaattgtcccctatgatgatcacagtcgcacctcccgtcgtccatccttcactcgggctgatggctttgatacagggagtagcttccgaggggtcaagcctccgagccctccgcccatgcttggaattattatggacaaacatgttatcagagactgccaggacatggccatccacattgactgtcgtagacaccacgacctggaatctccgcatgtcacgtgggtttcccgcattctttaggcaattttggttacatttgaggaaaaatttcaagaagaacctgcacatgatctcatgtgtgagcaagactcggcacatttctgggttcttgtcttggccttcatacactatggcttgttttgtcatggagtcaatgaggcgcacgtagaaatcctgctccgtccttatcccattgctgtagagaagctgaagccggtagtgaattccgttattggtcttttcgctgttggcttctttttccttctccacgaaccccacaaacgctgtcctctcgatctccacgggctggccctgtctgtcgtagagggccaggacgaagtggaagaagttggatttccgcagattggaaggcggctgcttctcaaagtgagcccgggccagacccaccccgctctgcgccgccgtgttggcgtccagcaccccggcgccctgcatccacgtccgcaccgcgttcatgccgctgcccagcggctcttccttcatgctgcttccactccgttggatgctttcctgaatcccaaacatgaaaacaaccttttcttgtggaaaatctcctcccccttgaaaaaaattaaaaaaaaaaaaaaaggaaagaaaagaaagaaaagaaaagaaacaaaaacgccaaccagagatttttttttttctcagacgatgaactcgcacttagaagatcaaggcgggctggaaagcaaatttttaaaaaatgtaaacctctgctcaaaactgagcgataacccgaaaaaaagaagaaagggaaaatccaacgaaaagaccaaaataataaaattagagatgtatgcttggctgttgggggttgtttggttggttgatttttggtttgggtgctttttttttttttttgcttttttttttttttttttgtaatgatcacaggccggtggaggacaggaggggctggagtttccttttgtagaggtacccttcacttgaagaagcagg

SEQ ID NO: 18037 - RNA, 4622 nt, Homo sapiens
  source 1..4622: mol_type = other RNA
tctgccatcctccctcccctaccctcccacaactcccctcccccacccaccccaacccataaaaatcgcactcttgacagcctagtgaaaaccattgcaaaatccatatgggggcatgcacagttgcagcattgttgtaaatgatttcttgctctactagaaaaagttacattgtcttaaggtaacaaaacagttcttttgtgcttttcgatttctttgtttttttttttttctttttttctttttcttttttcttagaatgttagtgatgactgacagttctggtgcacagttacaatgtacaagtgaaatgaatatgatttgcattgttaaggcatccaatctgctggtttatatttatgtgaaagacagaggaaatatacaagcagacttaagaaagaaagtatgttcattgatttctatgaagtttctccctagaatttaatgcacaaaatgcgtcactccaaagggagagattccatgcatattaatagagtaaaacagcattagggttgttttgtaagcttccaaagcaaaggatacatttttttttaaatctactgaactaaatactacaagaataatatgctactatttttttttttttgccatatattggaaaaaacttcttaacttacaaataatacaaaaatagacaatgacttttgggtggaaattaaaaaaactgaagcatggtttataacaatactaaaaataactataaatgaaatgtttaaaaatcacattgaaacagctaatacaagtgtaggtgaccaaacaaatacgcacttttcacgtagcaaacatacacaataaaataaattgggggtggaaggaagaggaagaagggaaaagcaatgtacaaattcgaaagataaatacattatttatatggatattttacaaaatcccctttaaaacaaaaagccttttaattaactttgcaagtatgtgcaagctaaaggtagtgagctttttttctttgcaaaatacgcagtaaaatctttttgtgatattgaaaaaatgtcttaagacattaaaatgtataaatagaacaacaactttggcaaaaaatcacaaaaaaaaaatctacagtatttataactacatacaaaaacacaagagcaaagaaaaaaatatcaggcaaatgcatcctcagagctttgctgcatctttgctattaattcttatttttaagaacacttcccagataatgagagcaaaaattcccatagaacagaaaactatgttttggaggtctcaaccttcttttcctttctccacccccggttccctttaactcttaattccaaagcacttaacctgttgtttcaatctattatgttacaaatggtaagggtcgactgatagaggcagtatctggaatgggaaaatcgaaaatacctgccacgttgcttttatcaacttttggaagataggtatgaagtctgcatttaggacgagtaaactttaaacttgcaaatgggggagcgtacgtgaggttttggcttgttaactggagggcagagtgtggaattctgtgcctggaccctgttccatgaagtctcaaaggagattctcacacagtatgtgtgccaccaagctctcgagaggccatcggcttcagaagaaactgacttaagtaaaaggagagaatgagatcagatttaaatatgcagttttaacaatctgtctagaggcactggattttcgagtagagggaaaaatgtgatcacttacatcgcgttttaactttccaggctgcatttatttacacagttgcttaagacaacaatacaaaagagataaataagcttgcactgctaaggggtggcatgttaagttagatattgaaaatgcactgtctgagctaactaccatttgatatgctttaaggcgcaaaagccgacccttagtttttctaaaaaatctaactggcattcctattctgtcccatacaagcttttttttttttcctttttttctttttttttttttttacttttttgtaaatatcaccacttcattcttcctttacacagctttaaaaacatcataaattaaaacatggagtcttatttatagtgtcccttgtatagagctttacggtttataaaagacaaatgattgcagaattaagcttaaaaaaaaaaaagaaaaagaaaaagtggatttgcttttgtcaatacagaataaatatatcccccaaatacttgggaggtacaactttaaccaacaccctgcacttgcagatccctcttccaatttcagtatttgcaaggtcggtgattttgtttgtttaaaaatctgcagttattgtgattcctcttaaaaaggcctgagttaaaagttccactctgggacttgtatcagattactctctgtagcagaatccaacctcttcattaatacaattcttcaaggcaattctttcacataggaggaacaatcatgccagatatcgcttgcaggctgttcccgttggtgctggtgcaggtgggaggtggggaggtctggggtctgacgactggtgcgaaagcactcttctgtttcacggctgagaccatgttggctggtgagaaggagaagatgcccgaggagctgctgcagttggaggggaggcttgtggaggaggccatggtggggctggatggcactatggcatagggggagttggcagctgagccgttgaggaaggtgggggagccgcccaaattggacattgcggcagagccgtatccgttcatgctcgtggtgacggagttatagttggtctgctggggagtggtgctcggcacgtacccgtgtggtgatacgctgcttgagttgcgggtgaaaccctgattggtggcttgtgatgcctcggagacattcacggccagttgtccactgaacgaattcacgcccatcatccctgcgtggaccgaggtgttagcaagggccgggagttggttgtggttgcggggaacactgtacagggcctcggcaatgtcggccgctctcttcagaatgatttcctggttgttgtgtggcatcccatacagtgcttctaccagatccgcagcccttttgagtattacttcctttggcaaacgctcagggtcaccagggtgccgaggaatgaccttctgtaacctctggaaaccataatcgatggtgggttcgttgagcgctgtataaatgaatctgcctggtgttcctttgcagaactgcttagatttgtaggacagtgtgacttccacaacaccagggatgtgccgaggaggggtctgcacacggatggcatgaggagtgatcaactcactccagaccagcatggtaccgaatatgacctgtaacccatcaaagaaattgtcccctatgatgatcacagtcgcacctcccgtcgtccatccttcactcgggctgatggctttgatacagggagtagcttccgaggggtcaagcctccgagccctccgcccatgcttggaattattatggacaaacatgttatcagagactgccaggacatggccatccacattgactgtcgtagacaccacgacctggaatctccgcatgtcacgtgggtttcccgcattctttaggcaattttggttacatttgaggaaaaatttcaagaagaacctgtcaattatcactggatctgagggagtctcatttcggttgccacagcttttcttgtcacaacagcggctgcacatgatctcatgtgtgagcaagactcggcacatttctgggttcttgtcttggccttcatacactatggcttgttttgtcatggagtcaatgaggcgcacgtagaaatcctgctccgtccttatcccattgctgtagagaagctgaagccggtagtgaattccgttattggtcttttcgctgttggcttctttttccttctccacgaaccccacaaacgctgtcctctcgatctccacgggctggccctgtctgtcgtagagggccaggacgaagtggaagaagttggatttccgcagattggaaggcggctgcttctcaaagtgagcccgggccagacccaccccgctctgcgccgccgtgttggcgtccagcaccccggcgccctgcatccacgtccgcaccgcgttcatgccgctgcccagcggctcttccttcatgctgcttccactccgttggatgctttcctgaatcccaaacatgaaaacaaccttttcttgtggaaaatctcctcccccttgaaaaaaattaaaaaaaaaaaaaaaggaaagaaaagaaagaaaagaaaagaaacaaaaacgccaaccagagatttttttttttctcagacgatgaactcgcacttagaagatcaaggcgggctggaaagcaaatttttaaaaaatgtaaacctctgctcaaaactgagcgataacccgaaaaaaagaagaaagggaaaatccaacgaaaagaccaaaataataaaattagagatgtatgcttggctgttgggggttgtttggttggttgatttttggtttgggtgctttttttttttttttgcttttttttttttttttttgtaatgatcacaggccggtggaggacaggaggggctggagtttccttttgtagaggtacccttcacttgaagaagcagg

SEQ ID NO: 18038 - RNA, 4577 nt, Homo sapiens
  source 1..4577: mol_type = other RNA
tctgccatcctccctcccctaccctcccacaactcccctcccccacccaccccaacccataaaaatcgcactcttgacagcctagtgaaaaccattgcaaaatccatatgggggcatgcacagttgcagcattgttgtaaatgatttcttgctctactagaaaaagttacattgtcttaaggtaacaaaacagttcttttgtgcttttcgatttctttgtttttttttttttctttttttctttttcttttttcttagaatgttagtgatgactgacagttctggtgcacagttacaatgtacaagtgaaatgaatatgatttgcattgttaaggcatccaatctgctggtttatatttatgtgaaagacagaggaaatatacaagcagacttaagaaagaaagtatgttcattgatttctatgaagtttctccctagaatttaatgcacaaaatgcgtcactccaaagggagagattccatgcatattaatagagtaaaacagcattagggttgttttgtaagcttccaaagcaaaggatacatttttttttaaatctactgaactaaatactacaagaataatatgctactatttttttttttttgccatatattggaaaaaacttcttaacttacaaataatacaaaaatagacaatgacttttgggtggaaattaaaaaaactgaagcatggtttataacaatactaaaaataactataaatgaaatgtttaaaaatcacattgaaacagctaatacaagtgtaggtgaccaaacaaatacgcacttttcacgtagcaaacatacacaataaaataaattgggggtggaaggaagaggaagaagggaaaagcaatgtacaaattcgaaagataaatacattatttatatggatattttacaaaatcccctttaaaacaaaaagccttttaattaactttgcaagtatgtgcaagctaaaggtagtgagctttttttctttgcaaaatacgcagtaaaatctttttgtgatattgaaaaaatgtcttaagacattaaaatgtataaatagaacaacaactttggcaaaaaatcacaaaaaaaaaatctacagtatttataactacatacaaaaacacaagagcaaagaaaaaaatatcaggcaaatgcatcctcagagctttgctgcatctttgctattaattcttatttttaagaacacttcccagataatgagagcaaaaattcccatagaacagaaaactatgttttggaggtctcaaccttcttttcctttctccacccccggttccctttaactcttaattccaaagcacttaacctgttgtttcaatctattatgttacaaatggtaagggtcgactgatagaggcagtatctggaatgggaaaatcgaaaatacctgccacgttgcttttatcaacttttggaagataggtatgaagtctgcatttaggacgagtaaactttaaacttgcaaatgggggagcgtacgtgaggttttggcttgttaactggagggcagagtgtggaattctgtgcctggaccctgttccatgaagtctcaaaggagattctcacacagtatgtgtgccaccaagctctcgagaggccatcggcttcagaagaaactgacttaagtaaaaggagagaatgagatcagatttaaatatgcagttttaacaatctgtctagaggcactggattttcgagtagagggaaaaatgtgatcacttacatcgcgttttaactttccaggctgcatttatttacacagttgcttaagacaacaatacaaaagagataaataagcttgcactgctaaggggtggcatgttaagttagatattgaaaatgcactgtctgagctaactaccatttgatatgctttaaggcgcaaaagccgacccttagtttttctaaaaaatctaactggcattcctattctgtcccatacaagcttttttttttttcctttttttctttttttttttttttacttttttgtaaatatcaccacttcattcttcctttacacagctttaaaaacatcataaattaaaacatggagtcttatttatagtgtcccttgtatagagctttacggtttataaaagacaaatgattgcagaattaagcttaaaaaaaaaaaagaaaaagaaaaagtggatttgcttttgtcaatacagaataaatatatcccccaaatacttgggaggtacaactttaaccaacaccctgcacttgcagatccctcttccaatttcagtatttgcaaggtcggtgattttgtttgtttaaaaatctgcagttattgtgattcctcttaaaaaggcctgagttaaaagttccactctgggacttgtatcagattactctctgtagcagaatccaacctcttcattaatacaattcttcaaggcaattctttcacataggaggaacaatcatgccagatatcgcttgcaggctgttcccgttggtgctggtgcaggtgggaggtggggaggtctggggtctgacgactggtgcgaaagcactcttctgtttcacggctgagaccatgttggctggtgagaaggagaagatgcccgaggagctgctgcagttggaggggaggcttgtggaggaggccatggtggggctggatggcactatggcatagggggagttggcagctgagccgttgaggaaggtgggggagccgcccaaattggacattgcggcagagccgtatccgttcatgctcgtggtgacggagttatagttggtctgctggggagtggtgctcggcacgtacccgtgtggtgatacgctgcttgagttgcgggtgaaaccctgattggtggcttgtgatgcctcggagacattcacggccagttgtccactgaacgaattcacgcccatcatccctgcgtggaccgaggtgttagcaagggccgggagttggttgtggttgcggggaacactgtacagggcctcggcaatgtcggccgctctcttcagaatgatttcctggttgttgtgtggcatcccatacagtgcttctaccagatccgcagcccttttgagtattacttcctttggcaaacgctcagggtcaccagggtgccgaggaatgaccttctgtaacctctggaaaccataatcgatggtgggttcgttgagcgctgtataaatgaatctgcctggtgttcctttgcagaactgcttagatttgtaggacagtgtgacttccacaacaccagggatgtgccgaggaggggtctgcacacggatggcatgaggagtgatcaactcactccagaccagcatggtaccgaatatgacctgtaacccatcaaagaaattgtcccctatgatgatcacagtcgcacctcccgtcgtccatccttcactcgggctgatggctttgatacagggagtagcttccgaggggtcaagcctccgagccctccgcccatgcttggaattattatggacaaacatgttatcagagactgccaggacatggccatccacattgactgtcgtagacaccacgacctggaatctccgcatgtcacgtgggtttcccgcattctttaggcaattttggttacatttgaggaaaaatttcaagaagaacctgtcaattatcactggatctgagggagtctcatttcggttgccacagcttttcttgtcacaacagcggctgcacatgatctcatgtgtgagcaagactcggcacatttctgggttcttgtcttggccttcatacactatggcttgttttgtcatggagtcaatgaggcgcacgtagaaatcctgctccgtccttatcccattgctgtagagaagctgaagccggtagtgaattccgttattggtcttttcgctgttggcttctttttccttctccacgaaccccacaaacgctgtcctctcgatctccacgggctggccctgtctgtcgtagagggccaggacgaagtggaagaagttggatttccgcagattggaaggcggctgcttctcaaagtgagcccgggccagacccaccccgctgacacgcactgcgtggggaggaagaaaagtggcggtggatgaagtgaacccaccttcgcggagtagaacccacagttatattccggcacccctcgaatctcacgtctcagctagcagggcaggtgggaatggatggaaaacatgctcggcgtctcgccgcagcagccaccctccaggaacccctcaagctctggccaactgcgagtgcccggccttgggaagccacatccccccaccaccaaaaagcatgtggagaagggtccgagggcggggctcagaactgtcgcgggtggtcgctgtgaaaaagggaagaggggtgttttcttaaagacctgtcctaacaaagtttcgctgttccgcagaaatcctcacactcattccagaaatcctaaaggccagggctgctggctcagtgcgccggccggcgatgggaggctggagcgcctggggcgccaggcggccactgacagccggacctgcccaacacaagcgcgcacaggcacacacacacacatagaagaacac

SEQ ID NO: 18039 - RNA, 4538 nt, Homo sapiens
  source 1..4538: mol_type = other RNA
tctgccatcctccctcccctaccctcccacaactcccctcccccacccaccccaacccataaaaatcgcactcttgacagcctagtgaaaaccattgcaaaatccatatgggggcatgcacagttgcagcattgttgtaaatgatttcttgctctactagaaaaagttacattgtcttaaggtaacaaaacagttcttttgtgcttttcgatttctttgtttttttttttttctttttttctttttcttttttcttagaatgttagtgatgactgacagttctggtgcacagttacaatgtacaagtgaaatgaatatgatttgcattgttaaggcatccaatctgctggtttatatttatgtgaaagacagaggaaatatacaagcagacttaagaaagaaagtatgttcattgatttctatgaagtttctccctagaatttaatgcacaaaatgcgtcactccaaagggagagattccatgcatattaatagagtaaaacagcattagggttgttttgtaagcttccaaagcaaaggatacatttttttttaaatctactgaactaaatactacaagaataatatgctactatttttttttttttgccatatattggaaaaaacttcttaacttacaaataatacaaaaatagacaatgacttttgggtggaaattaaaaaaactgaagcatggtttataacaatactaaaaataactataaatgaaatgtttaaaaatcacattgaaacagctaatacaagtgtaggtgaccaaacaaatacgcacttttcacgtagcaaacatacacaataaaataaattgggggtggaaggaagaggaagaagggaaaagcaatgtacaaattcgaaagataaatacattatttatatggatattttacaaaatcccctttaaaacaaaaagccttttaattaactttgcaagtatgtgcaagctaaaggtagtgagctttttttctttgcaaaatacgcagtaaaatctttttgtgatattgaaaaaatgtcttaagacattaaaatgtataaatagaacaacaactttggcaaaaaatcacaaaaaaaaaatctacagtatttataactacatacaaaaacacaagagcaaagaaaaaaatatcaggcaaatgcatcctcagagctttgctgcatctttgctattaattcttatttttaagaacacttcccagataatgagagcaaaaattcccatagaacagaaaactatgttttggaggtctcaaccttcttttcctttctccacccccggttccctttaactcttaattccaaagcacttaacctgttgtttcaatctattatgttacaaatggtaagggtcgactgatagaggcagtatctggaatgggaaaatcgaaaatacctgccacgttgcttttatcaacttttggaagataggtatgaagtctgcatttaggacgagtaaactttaaacttgcaaatgggggagcgtacgtgaggttttggcttgttaactggagggcagagtgtggaattctgtgcctggaccctgttccatgaagtctcaaaggagattctcacacagtatgtgtgccaccaagctctcgagaggccatcggcttcagaagaaactgacttaagtaaaaggagagaatgagatcagatttaaatatgcagttttaacaatctgtctagaggcactggattttcgagtagagggaaaaatgtgatcacttacatcgcgttttaactttccaggctgcatttatttacacagttgcttaagacaacaatacaaaagagataaataagcttgcactgctaaggggtggcatgttaagttagatattgaaaatgcactgtctgagctaactaccatttgatatgctttaaggcgcaaaagccgacccttagtttttctaaaaaatctaactggcattcctattctgtcccatacaagcttttttttttttcctttttttctttttttttttttttacttttttgtaaatatcaccacttcattcttcctttacacagctttaaaaacatcataaattaaaacatggagtcttatttatagtgtcccttgtatagagctttacggtttataaaagacaaatgattgcagaattaagcttaaaaaaaaaaaagaaaaagaaaaagtggatttgcttttgtcaatacagaataaatatatcccccaaatacttgggaggtacaactttaaccaacaccctgcacttgcagatccctcttccaatttcagtatttgcaaggtcggtgattttgtttgtttaaaaatctgcagttattgtgattcctcttaaaaaggcctgagttaaaagttccactctgggacttgtatcagattactctctgtagcagaatccaacctcttcattaatacaattcttcaaggcaattctttcacataggaggaacaatcatgccagatatcgttcaggagaaggccagtcccgggagagaccctgcactggagaacttgctagagtccacaaaagactgatcttgcaggctgttcccgttggtgctggtgcaggtgggaggtggggaggtctggggtctgacgactggtgcgaaagcactcttctgtttcacggctgagaccatgttggctggtgagaaggagaagatgcccgaggagctgctgcagttggaggggaggcttgtggaggaggccatggtggggctggatggcactacctgattggtggcttgtgatgcctcggagacattcacggccagttgtccactgaacgaattcacgcccatcatccctgcgtggaccgaggtgttagcaagggccgggagttggttgtggttgcggggaacactgtacagggcctcggcaatgtcggccgctctcttcagaatgatttcctggttgttgtgtggcatcccatacagtgcttctaccagatccgcagcccttttgagtattacttcctttggcaaacgctcagggtcaccagggtgccgaggaatgaccttctgtaacctctggaaaccataatcgatggtgggttcgttgagcgctgtataaatgaatctgcctggtgttcctttgcagaactgcttagatttgtaggacagtgtgacttccacaacaccagggatgtgccgaggaggggtctgcacacggatggcatgaggagtgatcaactcactccagaccagcatggtaccgaatatgacctgtaacccatcaaagaaattgtcccctatgatgatcacagtcgcacctcccgtcgtccatccttcactcgggctgatggctttgatacagggagtagctgcatgttccagataagagggcgtaccttccgaggggtcaagcctccgagccctccgcccatgcttggaattattatggacaaacatgttatcagagactgccaggacatggccatccacattgactgtcgtagacaccacgacctggaatctccgcatgtcacgtgggtttcccgcattctttaggcaattttggttacatttgaggaaaaatttcaagaagaacctgtcaattatcactggatctgagggagtctcatttcggttgccacagcttttcttgtcacaacagcggctgcacatgatctcatgtgtgagcaagactcggcacatttctgggttcttgtcttggccttcatacactatggcttgttttgtcatggagtcaatgaggcgcacgtagaaatcctgctccgtccttatcccattgctgtagagaagctgaagccggtagtgaattccgttattggtcttttcgctgttggcttctttttccttctccacgaaccccacaaacgctgtcctctcgatctccacgggctggccctgtctgtcgtagagggccaggacgaagtggaagaagttggatttccgcagattggaaggcggctgcttctcaaagtgagcccgggccagacccaccccgctctgcgccgccgtgttggcgtccagcaccccggcgccctgcatccacgtccgcaccgcgttcatgccgctgcccagcggctcttccttcatgctgcttccactccgttggatgctttcctgaatcccaaacatgaaaacaaccttttcttgtggaaaatctcctcccccttgaaaaaaattaaaaaaaaaaaaaaaggaaagaaaagaaagaaaagaaaagaaacaaaaacgccaaccagagatttttttttttctcagacgatgaactcgcacttagaagatcaaggcgggctggaaagcaaatttttaaaaaatgtaaacctctgctcaaaactgagcgataacccgaaaaaaagaagaaagggaaaatccaacgaaaagaccaaaataataaaattagagatgtatgcttggctgttgggggttgtttggttggttgatttttggtttgggtgctttttttttttttttgcttttttttttttttttttgtaatgatcacaggccggtggaggacaggaggggctggagtttccttttgtagaggtacccttcacttgaagaagcagg

SEQ ID NO: 18040 - RNA, 4715 nt, Homo sapiens
  source 1..4715: mol_type = other RNA
tctgccatcctccctcccctaccctcccacaactcccctcccccacccaccccaacccataaaaatcgcactcttgacagcctagtgaaaaccattgcaaaatccatatgggggcatgcacagttgcagcattgttgtaaatgatttcttgctctactagaaaaagttacattgtcttaaggtaacaaaacagttcttttgtgcttttcgatttctttgtttttttttttttctttttttctttttcttttttcttagaatgttagtgatgactgacagttctggtgcacagttacaatgtacaagtgaaatgaatatgatttgcattgttaaggcatccaatctgctggtttatatttatgtgaaagacagaggaaatatacaagcagacttaagaaagaaagtatgttcattgatttctatgaagtttctccctagaatttaatgcacaaaatgcgtcactccaaagggagagattccatgcatattaatagagtaaaacagcattagggttgttttgtaagcttccaaagcaaaggatacatttttttttaaatctactgaactaaatactacaagaataatatgctactatttttttttttttgccatatattggaaaaaacttcttaacttacaaataatacaaaaatagacaatgacttttgggtggaaattaaaaaaactgaagcatggtttataacaatactaaaaataactataaatgaaatgtttaaaaatcacattgaaacagctaatacaagtgtaggtgaccaaacaaatacgcacttttcacgtagcaaacatacacaataaaataaattgggggtggaaggaagaggaagaagggaaaagcaatgtacaaattcgaaagataaatacattatttatatggatattttacaaaatcccctttaaaacaaaaagccttttaattaactttgcaagtatgtgcaagctaaaggtagtgagctttttttctttgcaaaatacgcagtaaaatctttttgtgatattgaaaaaatgtcttaagacattaaaatgtataaatagaacaacaactttggcaaaaaatcacaaaaaaaaaatctacagtatttataactacatacaaaaacacaagagcaaagaaaaaaatatcaggcaaatgcatcctcagagctttgctgcatctttgctattaattcttatttttaagaacacttcccagataatgagagcaaaaattcccatagaacagaaaactatgttttggaggtctcaaccttcttttcctttctccacccccggttccctttaactcttaattccaaagcacttaacctgttgtttcaatctattatgttacaaatggtaagggtcgactgatagaggcagtatctggaatgggaaaatcgaaaatacctgccacgttgcttttatcaacttttggaagataggtatgaagtctgcatttaggacgagtaaactttaaacttgcaaatgggggagcgtacgtgaggttttggcttgttaactggagggcagagtgtggaattctgtgcctggaccctgttccatgaagtctcaaaggagattctcacacagtatgtgtgccaccaagctctcgagaggccatcggcttcagaagaaactgacttaagtaaaaggagagaatgagatcagatttaaatatgcagttttaacaatctgtctagaggcactggattttcgagtagagggaaaaatgtgatcacttacatcgcgttttaactttccaggctgcatttatttacacagttgcttaagacaacaatacaaaagagataaataagcttgcactgctaaggggtggcatgttaagttagatattgaaaatgcactgtctgagctaactaccatttgatatgctttaaggcgcaaaagccgacccttagtttttctaaaaaatctaactggcattcctattctgtcccatacaagcttttttttttttcctttttttctttttttttttttttacttttttgtaaatatcaccacttcattcttcctttacacagctttaaaaacatcataaattaaaacatggagtcttatttatagtgtcccttgtatagagctttacggtttataaaagacaaatgattgcagaattaagcttaaaaaaaaaaaagaaaaagaaaaagtggatttgcttttgtcaatacagaataaatatatcccccaaatacttgggaggtacaactttaaccaacaccctgcacttgcagatccctcttccaatttcagtatttgcaaggtcggtgattttgtttgtttaaaaatctgcagttattgtgattcctcttaaaaaggcctgagttaaaagttccactctgggacttgtatcagattactctctgtagcagaatccaacctcttcattaatacaattcttcaaggcaattctttcacataggaggaacaatcatgccagatatcgttcaggagaaggccagtcccgggagagaccctgcactggagaacttgctagagtccacaaaagactgatcttgcaggctgttcccgttggtgctggtgcaggtgggaggtggggaggtctggggtctgacgactggtgcgaaagcactcttctgtttcacggctgagaccatgttggctggtgagaaggagaagatgcccgaggagctgctgcagttggaggggaggcttgtggaggaggccatggtggggctggatggcactatggcatagggggagttggcagctgagccgttgaggaaggtgggggagccgcccaaattggacattgcggcagagccgtatccgttcatgctcgtggtgacggagttatagttggtctgctggggagtggtgctcggcacgtacccgtgtggtgatacgctgcttgagttgcgggtgaaaccctgattggtggcttgtgatgcctcggagacattcacggccagttgtccactgaacgaattcacgcccatcatccctgcgtggaccgaggtgttagcaagggccgggagttggttgtggttgcggggaacactgtacagggcctcggcaatgtcggccgctctcttcagaatgatttcctggttgttgtgtggcatcccatacagtgcttctaccagatccgcagcccttttgagtattacttcctttggcaaacgctcagggtcaccagggtgccgaggaatgaccttctgtaacctctggaaaccataatcgatggtgggttcgttgagcgctgtataaatgaatctgcctggtgttcctttgcagaactgcttagatttgtaggacagtgtgacttccacaacaccagggatgtgccgaggaggggtctgcacacggatggcatgaggagtgatcaactcactccagaccagcatggtaccgaatatgacctgtaacccatcaaagaaattgtcccctatgatgatcacagtcgcacctcccgtcgtccatccttcactcgggctgatggctttgatacagggagtagcatgttccagataagagggcgtaccttccgaggggtcaagcctccgagccctccgcccatgcttggaattattatggacaaacatgttatcagagactgccaggacatggccatccacattgactgtcgtagacaccacgacctggaatctccgcatgtcacgtgggtttcccgcattctttaggcaattttggttacatttgaggaaaaatttcaagaagaacctgtcaattatcactggatctgagggagtctcatttcggttgccacagcttttcttgtcacaacagcggctgcacatgatctcatgtgtgagcaagactcggcacatttctgggttcttgtcttggccttcatacactatggcttgttttgtcatggagtcaatgaggcgcacgtagaaatcctgctccgtccttatcccattgctgtagagaagctgaagccggtagtgaattccgttattggtcttttcgctgttggcttctttttccttctccacgaaccccacaaacgctgtcctctcgatctccacgggctggccctgtctgtcgtagagggccaggacgaagtggaagaagttggatttccgcagattggaaggcggctgcttctcaaagtgagcccgggccagacccaccccgctctgcgccgccgtgttggcgtccagcaccccggcgccctgcatccacgtccgcaccgcgttcatgccgctgcccagcggctcttccttcatgctgcttccactccgttggatgctttcctgaatcccaaacatgaaaacaaccttttcttgtggaaaatctcctcccccttgaaaaaaattaaaaaaaaaaaaaaaggaaagaaaagaaagaaaagaaaagaaacaaaaacgccaaccagagatttttttttttctcagacgatgaactcgcacttagaagatcaaggcgggctggaaagcaaatttttaaaaaatgtaaacctctgctcaaaactgagcgataacccgaaaaaaagaagaaagggaaaatccaacgaaaagaccaaaataataaaattagagatgtatgcttggctgttgggggttgtttggttggttgatttttggtttgggtgctttttttttttttttgcttttttttttttttttttgtaatgatcacaggccggtggaggacaggaggggctggagtttccttttgtagaggtacccttcacttgaagaagcagg

SEQ ID NO: 18041 - RNA, 4878 nt, Homo sapiens
  source 1..4878: mol_type = other RNA
tctgccatcctccctcccctaccctcccacaactcccctcccccacccaccccaacccataaaaatcgcactcttgacagcctagtgaaaaccattgcaaaatccatatgggggcatgcacagttgcagcattgttgtaaatgatttcttgctctactagaaaaagttacattgtcttaaggtaacaaaacagttcttttgtgcttttcgatttctttgtttttttttttttctttttttctttttcttttttcttagaatgttagtgatgactgacagttctggtgcacagttacaatgtacaagtgaaatgaatatgatttgcattgttaaggcatccaatctgctggtttatatttatgtgaaagacagaggaaatatacaagcagacttaagaaagaaagtatgttcattgatttctatgaagtttctccctagaatttaatgcacaaaatgcgtcactccaaagggagagattccatgcatattaatagagtaaaacagcattagggttgttttgtaagcttccaaagcaaaggatacatttttttttaaatctactgaactaaatactacaagaataatatgctactatttttttttttttgccatatattggaaaaaacttcttaacttacaaataatacaaaaatagacaatgacttttgggtggaaattaaaaaaactgaagcatggtttataacaatactaaaaataactataaatgaaatgtttaaaaatcacattgaaacagctaatacaagtgtaggtgaccaaacaaatacgcacttttcacgtagcaaacatacacaataaaataaattgggggtggaaggaagaggaagaagggaaaagcaatgtacaaattcgaaagataaatacattatttatatggatattttacaaaatcccctttaaaacaaaaagccttttaattaactttgcaagtatgtgcaagctaaaggtagtgagctttttttctttgcaaaatacgcagtaaaatctttttgtgatattgaaaaaatgtcttaagacattaaaatgtataaatagaacaacaactttggcaaaaaatcacaaaaaaaaaatctacagtatttataactacatacaaaaacacaagagcaaagaaaaaaatatcaggcaaatgcatcctcagagctttgctgcatctttgctattaattcttatttttaagaacacttcccagataatgagagcaaaaattcccatagaacagaaaactatgttttggaggtctcaaccttcttttcctttctccacccccggttccctttaactcttaattccaaagcacttaacctgttgtttcaatctattatgttacaaatggtaagggtcgactgatagaggcagtatctggaatgggaaaatcgaaaatacctgccacgttgcttttatcaacttttggaagataggtatgaagtctgcatttaggacgagtaaactttaaacttgcaaatgggggagcgtacgtgaggttttggcttgttaactggagggcagagtgtggaattctgtgcctggaccctgttccatgaagtctcaaaggagattctcacacagtatgtgtgccaccaagctctcgagaggccatcggcttcagaagaaactgacttaagtaaaaggagagaatgagatcagatttaaatatgcagttttaacaatctgtctagaggcactggattttcgagtagagggaaaaatgtgatcacttacatcgcgttttaactttccaggctgcatttatttacacagttgcttaagacaacaatacaaaagagataaataagcttgcactgctaaggggtggcatgttaagttagatattgaaaatgcactgtctgagctaactaccatttgatatgctttaaggcgcaaaagccgacccttagtttttctaaaaaatctaactggcattcctattctgtcccatacaagcttttttttttttcctttttttctttttttttttttttacttttttgtaaatatcaccacttcattcttcctttacacagctttaaaaacatcataaattaaaacatggagtcttatttatagtgtcccttgtatagagctttacggtttataaaagacaaatgattgcagaattaagcttaaaaaaaaaaaagaaaaagaaaaagtggatttgcttttgtcaatacagaataaatatatcccccaaatacttgggaggtacaactttaaccaacaccctgcacttgcagatccctcttccaatttcagtatttgcaaggtcggtgattttgtttgtttaaaaatctgcagttattgtgattcctcttaaaaaggcctgagttaaaagttccactctgggacttgtatcagattactctctgtagcagaatccaacctcttcattaatacaattcttcaaggcaattctttcacataggaggaacaatcatgccagatatcgttcaggagaaggccagtcccgggagagaccctgcactggagaacttgctagagtccacaaaagactgatcttgcaggctgttcccgttggtgctggtgcaggtgggaggtggggaggtctggggtctgacgactggtgcgaaagcactcttctgtttcacggctgagaccatgttggctggtgagaaggagaagatgcccgaggagctgctgcagttggaggggaggcttgtggaggaggccatggtggggctggatggcactatggcatagggggagttggcagctgagccgttgaggaaggtgggggagccgcccaaattggacattgcggcagagccgtatccgttcatgctcgtggtgacggagttatagttggtctgctggggagtggtgctcggcacgtacccgtgtggtgatacgctgcttgagttgcgggtgaaaccctgattggtggcttgtgatgcctcggagacattcacggccagttgtccactgaacgaattcacgcccatcatccctgcgtggaccgaggtgttagcaagggccgggagttggttgtggttgcggggaacactgtacagggcctcggcaatgtcggccgctctcttcagaatgatttcctggttgttgtgtggcatcccatacagtgcttctaccagatccgcagcccttttgagtattacttcctttggcaaacgctcagggtcaccagggtgccgaggaatgaccttctgtaacctctggaaaccataatcgatggtgggttcgttgagcgctgtataaatgaatctgcctggtgttcctttgcagaactgcttagatttgtaggacagtgtgacttccacaacaccagggatgtgccgaggaggggtctgcacacggatggcatgaggagtgatcaactcactccagaccagcatggtaccgaatatgacctgtaacccatcaaagaaattgtcccctatgatgatcacagtcgcacctcccgtcgtccatccttcactcgggctgatggctttgatacagggagtagctgcatgttccagataagagggcgtaccttccgaggggtcaagcctccgagccctccgcccatgcttggaattattatggacaaacatgttatcagagactgccaggacatggccatccacattgactgtcgtagacaccacgacctggaatctccgcatgtcacgtgggtttcccgcattctttaggcaattttggttacatttgaggaaaaatttcaagaagaacctgtcaattatcactggatctgagggagtctcatttcggttgccacagcttttcttgtcacaacagcggctgcacatgatctcatgtgtgagcaagactcggcacatttctgggttcttgtcttggccttcatacactatggcttgttttgtcatggagtcaatgaggcgcacgtagaaatcctgctccgtccttatcccattgctgtagagaagctgaagccggtagtgaattccgttattggtcttttcgctgttggcttctttttccttctccacgaaccccacaaacgctgtcctctcgatctccacgggctggccctgtctgtcgtagagggccaggacgaagtggaagaagttggatttccgcagattggaaggcggctgcttctcaaagtgagcccgggccagacccaccccgctcctcttcccccaaaacatccagtgggcgctcttcacgccccttcaggcgacatagacccagctgacaacgggacacacatgtcccctcatgtcctcgtcctctccgccaaggacgggtgcgtcctcagaactcgctgaagaggtgtgaaagttttgtttgggttttgcgcgcgagatgaaactctataagcatttactcctacctgacacgcactgcgtggggaggaagaaaagtggcggtggatgaagtgaacccaccttcgcggagtagaacccacagttatattccggcacccctcgaatctcacgtctcagctagcagggcaggtgggaatggatggaaaacatgctcggcgtctcgccgcagcagccaccctccaggaacccctcaagctctggccaactgcgagtgcccggccttgggaagccacatccccccaccaccaaaaagcatgtggagaagggtccgagggcggggctcagaactgtcgcgggtggtcgctgtgaaaaagggaagaggggtgttttcttaaagacctgtcctaacaaagtttcgctgttccgcagaaatcctcacactcattccagaaatcctaaaggccagggctgctggctcagtgcgccggccggcgatgggaggctggagcgcctggggcgccaggcggccactgacagccggacctgcccaacacaagcgcgcacaggcacacacacacacatagaagaacac

SEQ ID NO: 18042 - RNA, 4718 nt, Homo sapiens
  source 1..4718: mol_type = other RNA
tctgccatcctccctcccctaccctcccacaactcccctcccccacccaccccaacccataaaaatcgcactcttgacagcctagtgaaaaccattgcaaaatccatatgggggcatgcacagttgcagcattgttgtaaatgatttcttgctctactagaaaaagttacattgtcttaaggtaacaaaacagttcttttgtgcttttcgatttctttgtttttttttttttctttttttctttttcttttttcttagaatgttagtgatgactgacagttctggtgcacagttacaatgtacaagtgaaatgaatatgatttgcattgttaaggcatccaatctgctggtttatatttatgtgaaagacagaggaaatatacaagcagacttaagaaagaaagtatgttcattgatttctatgaagtttctccctagaatttaatgcacaaaatgcgtcactccaaagggagagattccatgcatattaatagagtaaaacagcattagggttgttttgtaagcttccaaagcaaaggatacatttttttttaaatctactgaactaaatactacaagaataatatgctactatttttttttttttgccatatattggaaaaaacttcttaacttacaaataatacaaaaatagacaatgacttttgggtggaaattaaaaaaactgaagcatggtttataacaatactaaaaataactataaatgaaatgtttaaaaatcacattgaaacagctaatacaagtgtaggtgaccaaacaaatacgcacttttcacgtagcaaacatacacaataaaataaattgggggtggaaggaagaggaagaagggaaaagcaatgtacaaattcgaaagataaatacattatttatatggatattttacaaaatcccctttaaaacaaaaagccttttaattaactttgcaagtatgtgcaagctaaaggtagtgagctttttttctttgcaaaatacgcagtaaaatctttttgtgatattgaaaaaatgtcttaagacattaaaatgtataaatagaacaacaactttggcaaaaaatcacaaaaaaaaaatctacagtatttataactacatacaaaaacacaagagcaaagaaaaaaatatcaggcaaatgcatcctcagagctttgctgcatctttgctattaattcttatttttaagaacacttcccagataatgagagcaaaaattcccatagaacagaaaactatgttttggaggtctcaaccttcttttcctttctccacccccggttccctttaactcttaattccaaagcacttaacctgttgtttcaatctattatgttacaaatggtaagggtcgactgatagaggcagtatctggaatgggaaaatcgaaaatacctgccacgttgcttttatcaacttttggaagataggtatgaagtctgcatttaggacgagtaaactttaaacttgcaaatgggggagcgtacgtgaggttttggcttgttaactggagggcagagtgtggaattctgtgcctggaccctgttccatgaagtctcaaaggagattctcacacagtatgtgtgccaccaagctctcgagaggccatcggcttcagaagaaactgacttaagtaaaaggagagaatgagatcagatttaaatatgcagttttaacaatctgtctagaggcactggattttcgagtagagggaaaaatgtgatcacttacatcgcgttttaactttccaggctgcatttatttacacagttgcttaagacaacaatacaaaagagataaataagcttgcactgctaaggggtggcatgttaagttagatattgaaaatgcactgtctgagctaactaccatttgatatgctttaaggcgcaaaagccgacccttagtttttctaaaaaatctaactggcattcctattctgtcccatacaagcttttttttttttcctttttttctttttttttttttttacttttttgtaaatatcaccacttcattcttcctttacacagctttaaaaacatcataaattaaaacatggagtcttatttatagtgtcccttgtatagagctttacggtttataaaagacaaatgattgcagaattaagcttaaaaaaaaaaaagaaaaagaaaaagtggatttgcttttgtcaatacagaataaatatatcccccaaatacttgggaggtacaactttaaccaacaccctgcacttgcagatccctcttccaatttcagtatttgcaaggtcggtgattttgtttgtttaaaaatctgcagttattgtgattcctcttaaaaaggcctgagttaaaagttccactctgggacttgtatcagattactctctgtagcagaatccaacctcttcattaatacaattcttcaaggcaattctttcacataggaggaacaatcatgccagatatcgttcaggagaaggccagtcccgggagagaccctgcactggagaacttgctagagtccacaaaagactgatcttgcaggctgttcccgttggtgctggtgcaggtgggaggtggggaggtctggggtctgacgactggtgcgaaagcactcttctgtttcacggctgagaccatgttggctggtgagaaggagaagatgcccgaggagctgctgcagttggaggggaggcttgtggaggaggccatggtggggctggatggcactatggcatagggggagttggcagctgagccgttgaggaaggtgggggagccgcccaaattggacattgcggcagagccgtatccgttcatgctcgtggtgacggagttatagttggtctgctggggagtggtgctcggcacgtacccgtgtggtgatacgctgcttgagttgcgggtgaaaccctgattggtggcttgtgatgcctcggagacattcacggccagttgtccactgaacgaattcacgcccatcatccctgcgtggaccgaggtgttagcaagggccgggagttggttgtggttgcggggaacactgtacagggcctcggcaatgtcggccgctctcttcagaatgatttcctggttgttgtgtggcatcccatacagtgcttctaccagatccgcagcccttttgagtattacttcctttggcaaacgctcagggtcaccagggtgccgaggaatgaccttctgtaacctctggaaaccataatcgatggtgggttcgttgagcgctgtataaatgaatctgcctggtgttcctttgcagaactgcttagatttgtaggacagtgtgacttccacaacaccagggatgtgccgaggaggggtctgcacacggatggcatgaggagtgatcaactcactccagaccagcatggtaccgaatatgacctgtaacccatcaaagaaattgtcccctatgatgatcacagtcgcacctcccgtcgtccatccttcactcgggctgatggctttgatacagggagtagctgcatgttccagataagagggcgtaccttccgaggggtcaagcctccgagccctccgcccatgcttggaattattatggacaaacatgttatcagagactgccaggacatggccatccacattgactgtcgtagacaccacgacctggaatctccgcatgtcacgtgggtttcccgcattctttaggcaattttggttacatttgaggaaaaatttcaagaagaacctgtcaattatcactggatctgagggagtctcatttcggttgccacagcttttcttgtcacaacagcggctgcacatgatctcatgtgtgagcaagactcggcacatttctgggttcttgtcttggccttcatacactatggcttgttttgtcatggagtcaatgaggcgcacgtagaaatcctgctccgtccttatcccattgctgtagagaagctgaagccggtagtgaattccgttattggtcttttcgctgttggcttctttttccttctccacgaaccccacaaacgctgtcctctcgatctccacgggctggccctgtctgtcgtagagggccaggacgaagtggaagaagttggatttccgcagattggaaggcggctgcttctcaaagtgagcccgggccagacccaccccgctctgcgccgccgtgttggcgtccagcaccccggcgccctgcatccacgtccgcaccgcgttcatgccgctgcccagcggctcttccttcatgctgcttccactccgttggatgctttcctgaatcccaaacatgaaaacaaccttttcttgtggaaaatctcctcccccttgaaaaaaattaaaaaaaaaaaaaaaggaaagaaaagaaagaaaagaaaagaaacaaaaacgccaaccagagatttttttttttctcagacgatgaactcgcacttagaagatcaaggcgggctggaaagcaaatttttaaaaaatgtaaacctctgctcaaaactgagcgataacccgaaaaaaagaagaaagggaaaatccaacgaaaagaccaaaataataaaattagagatgtatgcttggctgttgggggttgtttggttggttgatttttggtttgggtgctttttttttttttttgcttttttttttttttttttgtaatgatcacaggccggtggaggacaggaggggctggagtttccttttgtagaggtacccttcacttgaagaagcagg

SEQ ID NO: 18043 - RNA, 4691 nt, Homo sapiens
  source 1..4691: mol_type = other RNA
tctgccatcctccctcccctaccctcccacaactcccctcccccacccaccccaacccataaaaatcgcactcttgacagcctagtgaaaaccattgcaaaatccatatgggggcatgcacagttgcagcattgttgtaaatgatttcttgctctactagaaaaagttacattgtcttaaggtaacaaaacagttcttttgtgcttttcgatttctttgtttttttttttttctttttttctttttcttttttcttagaatgttagtgatgactgacagttctggtgcacagttacaatgtacaagtgaaatgaatatgatttgcattgttaaggcatccaatctgctggtttatatttatgtgaaagacagaggaaatatacaagcagacttaagaaagaaagtatgttcattgatttctatgaagtttctccctagaatttaatgcacaaaatgcgtcactccaaagggagagattccatgcatattaatagagtaaaacagcattagggttgttttgtaagcttccaaagcaaaggatacatttttttttaaatctactgaactaaatactacaagaataatatgctactatttttttttttttgccatatattggaaaaaacttcttaacttacaaataatacaaaaatagacaatgacttttgggtggaaattaaaaaaactgaagcatggtttataacaatactaaaaataactataaatgaaatgtttaaaaatcacattgaaacagctaatacaagtgtaggtgaccaaacaaatacgcacttttcacgtagcaaacatacacaataaaataaattgggggtggaaggaagaggaagaagggaaaagcaatgtacaaattcgaaagataaatacattatttatatggatattttacaaaatcccctttaaaacaaaaagccttttaattaactttgcaagtatgtgcaagctaaaggtagtgagctttttttctttgcaaaatacgcagtaaaatctttttgtgatattgaaaaaatgtcttaagacattaaaatgtataaatagaacaacaactttggcaaaaaatcacaaaaaaaaaatctacagtatttataactacatacaaaaacacaagagcaaagaaaaaaatatcaggcaaatgcatcctcagagctttgctgcatctttgctattaattcttatttttaagaacacttcccagataatgagagcaaaaattcccatagaacagaaaactatgttttggaggtctcaaccttcttttcctttctccacccccggttccctttaactcttaattccaaagcacttaacctgttgtttcaatctattatgttacaaatggtaagggtcgactgatagaggcagtatctggaatgggaaaatcgaaaatacctgccacgttgcttttatcaacttttggaagataggtatgaagtctgcatttaggacgagtaaactttaaacttgcaaatgggggagcgtacgtgaggttttggcttgttaactggagggcagagtgtggaattctgtgcctggaccctgttccatgaagtctcaaaggagattctcacacagtatgtgtgccaccaagctctcgagaggccatcggcttcagaagaaactgacttaagtaaaaggagagaatgagatcagatttaaatatgcagttttaacaatctgtctagaggcactggattttcgagtagagggaaaaatgtgatcacttacatcgcgttttaactttccaggctgcatttatttacacagttgcttaagacaacaatacaaaagagataaataagcttgcactgctaaggggtggcatgttaagttagatattgaaaatgcactgtctgagctaactaccatttgatatgctttaaggcgcaaaagccgacccttagtttttctaaaaaatctaactggcattcctattctgtcccatacaagcttttttttttttcctttttttctttttttttttttttacttttttgtaaatatcaccacttcattcttcctttacacagctttaaaaacatcataaattaaaacatggagtcttatttatagtgtcccttgtatagagctttacggtttataaaagacaaatgattgcagaattaagcttaaaaaaaaaaaagaaaaagaaaaagtggatttgcttttgtcaatacagaataaatatatcccccaaatacttgggaggtacaactttaaccaacaccctgcacttgcagatccctcttccaatttcagtatttgcaaggtcggtgattttgtttgtttaaaaatctgcagttattgtgattcctcttaaaaaggcctgagttaaaagttccactctgggacttgtatcagattactctctgtagcagaatccaacctcttcattaatacaattcttcaaggcaattctttcacataggaggaacaatcatgccagatatcgttcaggagaaggccagtcccgggagagaccctgcactggagaacttgctagagtccacaaaagactgatcttgcaggctgttcccgttggtgctggtgcaggtgggaggtggggaggtctggggtctgacgactggtgcgaaagcactcttctgtttcacggctgagaccatgttggctggtgagaaggagaagatgcccgaggagctgctgcagttggaggggaggcttgtggaggaggccatggtggggctggatggcactatggcatagggggagttggcagctgagccgttgaggaaggtgggggagccgcccaaattggacattgcggcagagccgtatccgttcatgctcgtggtgacggagttatagttggtctgctggggagtggtgctcggcacgtacccgtgtggtgatacgctgcttgagttgcgggtgaaaccctgattggtggcttgtgatgcctcggagacattcacggccagttgtccactgaacgaattcacgcccatcatccctgcgtggaccgaggtgttagcaagggccgggagttggttgtggttgcggggaacactgtacagggcctcggcaatgtcggccgctctcttcagaatgatttcctggttgttgtgtggcatcccatacagtgcttctaccagatccgcagcccttttgagtattacttcctttggcaaacgctcagggtcaccagggtgccgaggaatgaccttctgtaacctctggaaaccataatcgatggtgggttcgttgagcgctgtataaatgaatctgcctggtgttcctttgcagaactgcttagatttgtaggacagtgtgacttccacaacaccagggatgtgccgaggaggggtctgcacacggatggcatgaggagtgatcaactcactccagaccagcatggtaccgaatatgacctgtaacccatcaaagaaattgtcccctatgatgatcacagtcgcacctcccgtcgtccatccttcactcgggctgatggctttgatacagggagtagcttccgaggggtcaagcctccgagccctccgcccatgcttggaattattatggacaaacatgttatcagagactgccaggacatggccatccacattgactgtcgtagacaccacgacctggaatctccgcatgtcacgtgggtttcccgcattctttaggcaattttggttacatttgaggaaaaatttcaagaagaacctgtcaattatcactggatctgagggagtctcatttcggttgccacagcttttcttgtcacaacagcggctgcacatgatctcatgtgtgagcaagactcggcacatttctgggttcttgtcttggccttcatacactatggcttgttttgtcatggagtcaatgaggcgcacgtagaaatcctgctccgtccttatcccattgctgtagagaagctgaagccggtagtgaattccgttattggtcttttcgctgttggcttctttttccttctccacgaaccccacaaacgctgtcctctcgatctccacgggctggccctgtctgtcgtagagggccaggacgaagtggaagaagttggatttccgcagattggaaggcggctgcttctcaaagtgagcccgggccagacccaccccgctctgcgccgccgtgttggcgtccagcaccccggcgccctgcatccacgtccgcaccgcgttcatgccgctgcccagcggctcttccttcatgctgcttccactccgttggatgctttcctgaatcccaaacatgaaaacaaccttttcttgtggaaaatctcctcccccttgaaaaaaattaaaaaaaaaaaaaaaggaaagaaaagaaagaaaagaaaagaaacaaaaacgccaaccagagatttttttttttctcagacgatgaactcgcacttagaagatcaaggcgggctggaaagcaaatttttaaaaaatgtaaacctctgctcaaaactgagcgataacccgaaaaaaagaagaaagggaaaatccaacgaaaagaccaaaataataaaattagagatgtatgcttggctgttgggggttgtttggttggttgatttttggtttgggtgctttttttttttttttgcttttttttttttttttttgtaatgatcacaggccggtggaggacaggaggggctggagtttccttttgtagaggtacccttcacttgaagaagcagg

SEQ ID NO: 18044 - RNA, 667 nt, Homo sapiens
  source 1..667: mol_type = other RNA
tctgccccctccgctgctgccaaccacgttgccacagacatcggtgtggtcactgccccgcagctcaccattgaggtagagggagttggcgagacccttgtcctctgaggggtagcggcccggcctctccctgctggccccactgccactgcctcgggggccagggaaactgccctggctgcccccaccccctgtgcgggtacccacgctcttcatggcaaactcctgggcatgggccaccccactgcccacgctgcccatggccaggcgggggtccgggggtccaagctcggagggccgtggggcaaaggccaggagaggatcccgccctgggtcagcgcgcacaggcagcgtctccagcttcgccatgactaagccaggggggcacagcgcaggcttctctccttgcctttccaaggggttgaggggccgacgggtcctcaagcctgggaccctccgaggcccggtctgcaggggccatgtgcctcactctcgcagtcggggctcggcccgaaccagctgcgcgactttggaggggccgactgagccatcccggactgcagttttctccttcgctgcctcagggtccggcgcggggtctccgacacgggcgccaccggccccgcttgctggcgcagcccgaagcacgcccggcggggcgcgctgc

SEQ ID NO: 18045 - RNA, 706 nt, Homo sapiens
  source 1..706: mol_type = other RNA
tctgccccctccgctgctgccaaccacgttgccacagacatcggtgtggtcactgccccgcagctcaccattgaggtagagggagttggcgagacccttgtcctctgaggggtagcggcccggcctctccctgctggccccactgccactgcctcgggggccagggaaactgccctggctgcccccaccccctgtgcgggtacccacgctcttcatggcaaactcctgggcatgggccaccccactgcccacgctgcccatggccaggcgggggtccgggggtccaagctcggagggccgtggggcaaaggccaggagaggatcccgccctgggtcagcgcgcacaggcagcgtctccagcttcgccatgactaagccaggggggcactaagtgttgcagtcagggcagaagtggaagctcactaccagcgcaggcttctctccttgcctttccaaggggttgaggggccgacgggtcctcaagcctgggaccctccgaggcccggtctgcaggggccatgtgcctcactctcgcagtcggggctcggcccgaaccagctgcgcgactttggaggggccgactgagccatcccggactgcagttttctccttcgctgcctcagggtccggcgcggggtctccgacacgggcgccaccggccccgcttgctggcgcagcccgaagcacgcccggcggggcgcgctgc

SEQ ID NO: 18046 - RNA, 701 nt, Homo sapiens
  source 1..701: mol_type = other RNA
tctgccccctccgctgctgccaaccacgttgccacagacatcggtgtggtcactgccccgcagctcaccattgaggtagagggagttggcgagacccttgtcctctgaggggtagcggcccggcctctccctgctggccccactgccactgcctcgggggccagggaaactgccctggctgcccccaccccctgtgcgggtacccacgctcttcatggcaaactcctgggcatgggccaccccactgcccacgctgcccatggccaggcgggggtccgggggtccaagctcggagggccgtggggcaaaggccaggagaggatcccgccctgggtcagcgcgcacaggcagcgtctccagcttcgccatgactaagccaggggggcacttgcggggctgccgcgtgccaggcgccccgaggcggcgagcgcctgaggaaacgggggtctgggggagggtgggtaggcgacgcacatctgggtcgcgggtgggcgccgccaagggcacagcctgtccctcccggatggacgggggccgcggctgcagtaggtggcaggcctgccctccccaaggtcttcccagctcggccgcaccggggccctgggaagacagggcccccttcccgggatcagtcctccgcagaggtcccagggctggctgaggccggggcaggggacgcagtggcgccagctgctggcact

SEQ ID NO: 18047 - RNA, 2329 nt, Homo sapiens
  source 1..2329: mol_type = other RNA
tctgccccctccgctgctgccaaccacgttgccacagacatcggtgtggtcactgccccgcagctcaccattgaggtagagggagttggcgagacccttgtcctctgaggggtagcggcccggcctctccctgctggccccactgccactgcctcgggggccagggaaactgccctggctgcccccaccccctgtgcgggtacccacgctcttcatggcaaactcctgggcatgggccaccccactgcccacgctgcccatggccaggcgggggtccgggggtccaagctcggagggccgtggggcaaaggccaggagaggatcccgccctgggtcagcgcgcacaggcagcgtctccagcttcgccatgactaagccaggggggcactttccaaggggttgaggggccgacgggtcctcaagcctgggaccctccgaggcccggtctgcaggggccatgtgcctcactctcgcagtcggggctcggcccgaaccagctgcgcgactttggaggggccgactgagccatcccggactgcagttttctcctatctgggtcgcgggtgggcgccgccaagggcacagcctgtccctcccggatggacgggggccgcggctgcagtaggtggcaggcctgccctccccaaggtcttcccagctcggccgcaccggggccctgggaagacagggcccccttcccgggatcagtcctccgcagaggtcccagggctggctgaggccggggcaggggacgcagtggcgccagctgctggcactgacggagcctctctcagggcctgcgtttcccacaggtgggaggggggaggggaggggaggggccgctgcagggtgcgcggccccaaggatcctgcgcctgccgaaccccgcaaagaattcactgccaccaggaagacttcccggattactaccctctcccgctccctgtggaccttgaccctgctcagcttaccgtgaagccctctgagtccttctgtgggtgcgcgtccccctcccccaaggccggcccacaagcgcagggggagccaggcctcgggttacctgtgctcagggaggccgtgcttcctcgttcctttgtctcaagttcgcacctgggaacacctgccccagagatctgcataatgcagccgggcaggagcaccaggcagtgtctgcctcgggttagaccctcaaataagtgtgtgggaaatgggagagggcgcccttcaggccttttcccactacaccctgcataaaccaggcagggagccctccttccctatcaagttaaggggcccacgtggcaccctatggccccacagaccgtcttctacccagatgcccagttctaatgctgagtccctggcccagaccaagggcacctgacaaaactgttgtccttcgggagtcttctggcccccacaccaggaatgagagctctaggttgttggaaagttcactaccaagcctgtccactgtctctgtagaattccattctcagcatctgtccccacaggtgtggagaagagcacttcgccaccctcctcccttggacccgtctgtccccataagcaagggccaggactaggatgaggacagagagccacgtagggcacaaatgaagggcacaaacagcaagtacacagccctgagggtgacagcctccttccctttgtgccttgggtccctctctggcctcactctagtccctgctctgcctctactccccagcatactccagccccctatgcctcagccctgcaaccccctcctaccttaagtatggacccttctcttgccacctctgggtgcaatgtggggagcagctggggactgggaggatgaagcctgaaaggcctgaggcttggaaccagtaggaaggcctgggcagggtttgggaaagaactggcaaaatttcatacagatgaggtcaggtggtggggacaagggataatgctggactgggcaccagcgtgcgtgtgacactgttaacatgatagggggagactgcttggggaaaatagttgctttgggaaacaccagaggaagatacctctcaagcactaaatggaggccaagcaaggtggctcatgcctgtaatcccagcactttgggaggtcaaggtgggcagattacttgaggccaagagttcaagaccatcctggccaaattggtggaaccccatctctactaaaaatacaaaaattagctgggtgcggtatgcattcctgtaatcccagctacttgggaggctgaggcacgagaacccccttgaacccaggaggcagaggttgcagtgagctgtaattgcaccactgcactccagcctggg

SEQ ID NO: 18048 - RNA, 1909 nt, Homo sapiens
  source 1..1909: mol_type = other RNA
tctgccccctccgctgctgccaaccacgttgccacagacatcggtgtggtcactgccccgcagctcaccattgaggtagagggagttggcgagacccttgtcctctgaggggtagcggcccggcctctccctgctggccccactgccactgcctcgggggccagggaaactgccctggctgcccccaccccctgtgcgggtacccacgctcttcatggcaaactcctgggcatgggccaccccactgcccacgctgcccatggccaggcgggggtccgggggtccaagctcggagggccgtggggcaaaggccaggagaggatcccgccctgggtcagcgcgcacaggcagcgtctccagcttcgccatgactaagccaggggggcactttccaaggggttgaggggccgacgggtcctcaagcctgggaccctccgaggcccggtctgcaggggccatgtgcctcactctcgcagtcggggctcggcccgaaccagctgcgcgactttggaggggccgactgagccatcccggactgcagttttctcctcgtgaagccctctgagtccttctgtgggtgcgcgtccccctcccccaaggccggcccacaagcgcagggggagccaggcctcgggttacctgtgctcagggaggccgtgcttcctcgttcctttgtctcaagttcgcacctgggaacacctgccccagagatctgcataatgcagccgggcaggagcaccaggcagtgtctgcctcgggttagaccctcaaataagtgtgtgggaaatgggagagggcgcccttcaggccttttcccactacaccctgcataaaccaggcagggagccctccttccctatcaagttaaggggcccacgtggcaccctatggccccacagaccgtcttctacccagatgcccagttctaatgctgagtccctggcccagaccaagggcacctgacaaaactgttgtccttcgggagtcttctggcccccacaccaggaatgagagctctaggttgttggaaagttcactaccaagcctgtccactgtctctgtagaattccattctcagcatctgtccccacaggtgtggagaagagcacttcgccaccctcctcccttggacccgtctgtccccataagcaagggccaggactaggatgaggacagagagccacgtagggcacaaatgaagggcacaaacagcaagtacacagccctgagggtgacagcctccttccctttgtgccttgggtccctctctggcctcactctagtccctgctctgcctctactccccagcatactccagccccctatgcctcagccctgcaaccccctcctaccttaagtatggacccttctcttgccacctctgggtgcaatgtggggagcagctggggactgggaggatgaagcctgaaaggcctgaggcttggaaccagtaggaaggcctgggcagggtttgggaaagaactggcaaaatttcatacagatgaggtcaggtggtggggacaagggataatgctggactgggcaccagcgtgcgtgtgacactgttaacatgatagggggagactgcttggggaaaatagttgctttgggaaacaccagaggaagatacctctcaagcactaaatggaggccaagcaaggtggctcatgcctgtaatcccagcactttgggaggtcaaggtgggcagattacttgaggccaagagttcaagaccatcctggccaaattggtggaaccccatctctactaaaaatacaaaaattagctgggtgcggtatgcattcctgtaatcccagctacttgggaggctgaggcacgagaacccccttgaacccaggaggcagaggttgcagtgagctgtaattgcaccactgcactccagcctggg

SEQ ID NO: 18049 - RNA, 645 nt, Homo sapiens
  source 1..645: mol_type = other RNA
tctgccccctccgctgctgccaaccacgttgccacagacatcggtgtggtcactgccccgcagctcaccattgaggtagagggagttggcgagacccttgtcctctgaggggtagcggcccggcctctccctgctggccccactgccactgcctcgggggccagggaaactgccctggctgcccccaccccctgtgcgggtacccacgctcttcatggcaaactcctgggcatgggccaccccactgcccacgctgcccatggccaggcgggggtccgggggtccaagctcggagggccgtggggcaaaggccaggagaggatcccgccctgggtcagcgcgcacaggcagcgtctccagcttcgccatgactaagccaggggggcactttccaaggggttgaggggccgacgggtcctcaagcctgggaccctccgaggcccggtctgcaggggccatgtgcctcactctcgcagtcggggctcggcccgaaccagctgcgcgactttggaggggccgactgagccatcccggactgcagttttctccttcgctgcctcagggtccggcgcggggtctccgacacgggcgccaccggccccgcttgctggcgcagcccgaagcacgcccggcggggcgcgctgc

SEQ ID NO: 18050 - RNA, 482 nt, Homo sapiens
  source 1..482: mol_type = other RNA
tctgccccctccgctgctgccaaccacgttgccacagacatcggtgtggtcactgccccgcagctcaccattgaggtagagggagttggcgagacccttgtcctctgaggggtagcggcccggcctctccctgctggccccactgccactgcctcgggggccagggaaactgccctggctgcccccaccccctgtgcgggtacccacgctcttcatggcaaactcctgggcatgggccaccccactgcccacgctgcccatggccaggcgggggtccgggggtccaagctcggagggccgtggggcaaaggccaggagaggatcccgccctgggtcagcgcgcacaggcagcgtctccagcttcgccatgactaagccaggggggcatcgctgcctcagggtccggcgcggggtctccgacacgggcgccaccggccccgcttgctggcgcagcccgaagcacgcccggcggggcgcgctgc

SEQ ID NO: 18051 - RNA, 40 nt, Homo sapiens
  source 1..40: mol_type = other RNA
tctgccccctccgctgctgccacggcaacccgggccttgt

SEQ ID NO: 18052 - RNA, 80 nt, Homo sapiens
  source 1..80: mol_type = other RNA
tctgccccctccgctgctgccatggccggttttgtttcgccccacgtacccttcagtccccccaaatacacatacacacg

SEQ ID NO: 18053 - RNA, 130 nt, Homo sapiens
  source 1..130: mol_type = other RNA
tctgccccctccgctgctgccatggccggttttgtttcgccccacgtacccttcagtccccccaaatacacatacacacgccccaacaaaccagaaaccacctcctgcccacgatcgttgggcaggcttc

SEQ ID NO: 18054 - RNA, 62 nt, Homo sapiens
  source 1..62: mol_type = other RNA
tctggcaagtaaaaaactctcattttttaaggaaaatgagagttttttacttgccagaggaa

SEQ ID NO: 18055 - RNA, 65 nt, Homo sapiens
  source 1..65: mol_type = other RNA
tctggccagctacgtccccacggcccttgtcagtgtggaaggtagacggccagagaggtgacccc

SEQ ID NO: 18056 - RNA, 6168 nt, Homo sapiens
  source 1..6168: mol_type = other RNA
tctggctccgtgtcttcactcccaggaaggttgcgggggtggggggcgtggggggagggttggcagcggtggtggcggtggtggtggcagcggtggtggcaataggaggtgtgtgtcaaggtggatgttaaacagtgtgaattcccttccagatggctccagagagggagaaaggtgcaggactgcaccgggtaaggcgctcagcttcttttcttagagagacaaatccacagggtcaatacacagccaaaagcatatactcaggattaacatatcacgctagcttccagaagtttaagatatagtcatcaacaccccccacccctacccctttcccccctccccccacccccctccccgatccacagctaagtcaaactcccaaggacagtctgtctggtagagagatgttgagagagaagcctcatgcctgcagcaacagcccctgagctgggctgggccgggctaggcgggctcctaggcctgcactgggtctccccaggcagacgttttcatcaggtaccttacccaaaatgagtggggtgatcccagatgcttgctccctagtggactgagctgccctgcccatcagtgaggggcagggcactttggggatggctggtgtggagctactggacctggaggtgagggctcaccaggctgccggccagttgggccgctgcaaacagcctagtgtggctgttttctgcagacatctcacccaggcacaggccctcagggtggcatctaccaggtgagtgtgagcccaaggtggatggggacatctggactgagcgccctctcccctcggcacggcaatgtggcctgctgctactgccactgctcccagcaggggagccgatgccacgaggagctcaaagcctgagggtccgcttgcttcaggccctggctcccccagcgcccaacacggattgagcaggaagtgagcctgatgtcacctctcagccccagagaagagataaaatacagctctgctgtgagcagagtgaagaggggcctttgccctcacagtgaggcccagaggccagggaaggggtgaggacacccagggcggcagctaagcctgcagcccttaagagagagcctcaatcaagagagtttccactccccggagactgatgggctcttggaccctgactggcccagcagacacacacacactcaccacaagatgcaaggaccacaaagctcaaacctggggccatggttggggaagggggacaggtgtgggcagatgccctacttaataagggtttttaaggagtgggtgaatgtgctcataacagtcgccgaagttggggagcctggtggatgctctgtggctgcccctgcagctgctgccacctgctgctgctgctgctgctgttgttgttgctgctgctgttgttgttgctgctgctgctgttgttgttgctgctgctgctggttaaggttacgggctgtggactcctcagctgcacgcagcaggaaggtgtagttcctcaccacctcttctaccttggccagcagctcttggcgctgggcctcggagcgcacaatgaacaccagccgcacgaaggtctcaatgaggctgctcagcacctggaagctgcccgtgatggctgccagcatgtgagttgggctcttgtccacattggccacacggcggcaggaggcccggagctccttgaacttgagagctagctcaagcttatactcggagatctgagacacatagggcttgggggcacgggcctcggggctggccacacactgccgcaggactgtcagcagctcgttggtgtccagccgggcagccaggaagccatcagggaggccataggcatgggcccgcagggcattgatcttggccaggctcccctcgaaggtggacacacggaggtcaatctcctgagtgcgggaggcctcagggctgctgctgctgcaggtagcagcatccagcacctgcagggtcctgctcaccacaggcaccacctgctcgtccagcttcatgccaggcaggatcttcatggggatagagtaggagagctcatccttgccatcactggcatcatctgccatgtcacacttgcggtagtagaagcagtagcggatggagcagcacttgctgctctcactgtcctcgtctagctcggcaggcttccggtacacctcctcgggcagtgagaacacggccatctgtctggggcctttggtctctggggcaacctggacgtaggaggggtctcccagcgtcggtgactccagagacctgcttttgggacccaaggctatggggaggcttgcctctacctccttggcctccctgggcagcatgcccaggggaggatgtgggtagacatccgaggtcagcgaggccctgtcaccctggtccagctcactgatactgtagcggcgcatcagtttcctgtaattgggagctcccagacactcgccccccgaggcacacgtggtcaggcacgaaacaccactctcagggtccgatcggcactctcgggactccaggctggtagaacgaatgcgctggacattgatggggctgctgaggctcacgcctgggccagcctctggctgcctctggctagggaggactctgtccctttccctcccccggaggctgggcactggtgtctgggtggcttgtggccggcccccccggcagatgcgcttgcagtcacagctgcgcctctgctcacgggacatgccaggcccctgctgcacagggctgctgcggagctggcagctgcagcggccaggtgctggaggttgcaggtactcggtgcctggcagctccccctggcttggtggctttagaagttcctcaaggaactccagttcatactgctttaccttctgcagttgggcctgccgctcatctgtctccttcttctggcgggttgggaaggtggcagagaataaattgcgtagccggaaaggacctcgggatgacttgggtttggcagggccttcagaggtcgagtgggctccattgagagttgtttcaagcttcctagagggcatggtgctcacctgccggctggcagcctgagacctcagtgggctctggcctcgaggttggcagctggggctctgacctcgagactggctgctggggctgtggccatgaggctggcagctggggctgtggcttcttgactggcagctggggctctgcagagccatggggtaggtagctcggggaaccaggctggtctcttcgagcttgcttcttttgggtgtgctctccagctgcgccttctccccttggctggagatggtgccctgcttctgcagggtgggcttaccacccactggcccgcctttgcctgccacctcccctgtagcttgcttgcccactgactctcggcttgttcgcaaaagatagcttttgggagggaaattttgaacaggcagactgtcctcttgttgggagaggtgcaggctgtcagcccggctgcctgtgggtgctctggggctggaagagacctctgcacccagctgatgttgagaattccatgaggtctctggagcactggggctaattttgaacttcagattcttactggcactgctgctcatcatgctaacctctggcctccccatgctggcctccagccttctctcacccctgctgggggggttccccaaagccccaccagcagtgactagactcttattgtgaaccacttgctgtagggcggccgagatgatggcaggggtcacactgctctttgggtcgaggataagcttggggctcaacctgacctccttgggcaggttgtccctcagctcagagacctgctcttcactgagggatgatgtggctgccctcagtgacatttctaggcctgccctagtgtggccaggccctttgtcctcaggaactggggacagcagactcagattcttctgttcactaagctgtggggacagtgctgggtgcactgccaaggagtatgttcgttctccctgtacctggccctctgactggggcagcttcctccgagcgccaggggggccaggactctggcctgtggcaatgggttggagagatgggttgggatccgggcgcccaagagagtaaggggccgtaagaacggcctgggctgcacagctctggatccggaagggcaggtccttgcgggcaaggaggctgtccttgttgaggtgctgggccaggaagtaggtggtgttctggtgctgcttcatggccgacatcatctctgacatgtctgtgagctctgaagagttggtttcatgacctgagtccagcgatgattcaggagtgattgtggccagcacaatcagacctgcagtctgtgggggtggtgggtgtggtccatcctcggatgcagccagggcttctagagcctgcagagtggacaccagggcatcatctagctcctgggcatgatctcgaactgtccgggtctgcacactgtcaatcaatgtcactggaatctcatcgtacagaagcccacgcaggtggcgtccttgttcctggctctggacagcccggcgcttggggtcatcctcatcagagctgttgtctcggaaaccagggggtggggcagcaatggctggcaacagagaagttgtctcatcttcctcctcctcctcctcctcactcccaggtggtgggagggacatcaaatctactatattgtcacgagaggagccaggcttcccacctttgcgagggcccagctgctcctgaagtttggctttgcaagagtcacagtagaaattcagggcttcagccccaagggaattgtccaaggtgtaggaccgggccctgctggcacaaggctcgtggtctaggctagctgcatcaaagtcatcagggactacctcataaccttggccagagcttttggatgtggggtcagacttggttcggggcctggtctcctcaaagaagattaggttctcgttgacatctgtccggctttcctgctccttcctttgttcccgcatatggaggtagcagaagctgacaagctcagagtcggcaggtgggggcgtgcagcggctcgatttcctggggctggtgcccacgctgcccacataactactctcctttttccccaggtggcccccagtgacagggcggtgggcgctgtgcatgtaatctgccttgatcattggaggtggaagtggctggctggcaggcctggagaagaccatcttcctggaatccagcaagaggcggcagtaccccgcgatcaggcaggcaaagttggtggcttcaggccactccatcaacagcaccagaggcttggcatccatgatgctggtctccacccgggccacgccctggttctcccggaacagctggatcttgctgatcttgctgaactcggacagcacagtggtgaggttggttttgaggtcaataacatggctgatgccatgacggggtcccaccaggagcgtggtggccgactgcttctcatccaggcctacagtgttgaacaaaacgcccgtgaaggtaggaagttcattcagaattcgtagatactggagctttgcctgaattgcagagcccttggtgccgcaggaaggatgtgtttggtgagccttcagttgctgagagagagatttccggaggttcttctctttgatgacctgcaggagggaggggggaagaaagggttccaggccccactccttctccacattcttgagcgagatcttctgactaggtcgagtggctgagacagtgatatagatgtggagcgcagcaaggcccaaaagcatctctggcttgggatccattccaaagcgttctcgaataacatcattccgactctggatgtataggtactcaaaagcagcaggatcccgacgcagcagctccacagggtctttgggaaagaagcttattcggaagaggcatttcattccatgatagtgtgtccgctgtaccacataagccaggggttgcttgtcctgaagaagcagaaacttgtgattctgttctggcccggcatactcaaggacaagagcaaagtgctcaatgaacctcagggaaaggcggtcctgtaatgtcaacatcacatcctgataagttctatgagtctctccctcggggcttcactcacgtcttcctcattaatagccacaatctggtcaccagccaggagc

SEQ ID NO: 18057 - RNA, 6595 nt, Homo sapiens
  source 1..6595: mol_type = other RNA
tctggctccgtgtcttcactcccaggaaggttgcgggggtggggggcgtggggggagggttggcagcggtggtggcggtggtggtggcagcggtggtggcaataggaggtgtgtgtcaaggtggatgttaaacagtgtgaattcccttccagatggctccagagagggagaaaggtgcaggactgcaccgggtaaggcgctcagcttcttttcttagagagacaaatccacagggtcaatacacagccaaaagcatatactcaggattaacatatcacgctagcttccagaagtttaagatatagtcatcaacaccccccacccctacccctttcccccctccccccacccccctccccgatccacagctaagtcaaactcccaaggacagtctgtctggtagagagatgttgagagagaagcctcatgcctgcagcaacagcccctgagctgggctgggccgggctaggcgggctcctaggcctgcactgggtctccccaggcagacgttttcatcaggtaccttacccaaaatgagtggggtgatcccagatgcttgctccctagtggactgagctgccctgcccatcagtgaggggcagggcactttggggatggctggtgtggagctactggacctggaggtgagggctcaccaggctgccggccagttgggccgctgcaaacagcctagtgtggctgttttctgcagacatctcacccaggcacaggccctcagggtggcatctaccaggtgagtgtgagcccaaggtggatggggacatctggactgagcgccctctcccctcggcacggcaatgtggcctgctgctactgccactgctcccagcaggggagccgatgccacgaggagctcaaagcctgagggtccgcttgcttcaggccctggctcccccagcgcccaacacggattgagcaggaagtgagcctgatgtcacctctcagccccagagaagagataaaatacagctctgctgtgagcagagtgaagaggggcctttgccctcacagtgaggcccagaggccagggaaggggtgaggacacccagggcggcagctaagcctgcagcccttaagagagagcctcaatcaagagagtttccactccccggagactgatgggctcttggaccctgactggcccagcagacacacacacactcaccacaagatgcaaggaccacaaagctcaaacctggggccatggttggggaagggggacaggtgtgggcagatgccctacttaataagggtttttaaggagtgggtgaatgtgctcataacagtcgccgaagttggggagcctggtggatgctctgtggctgcccctgcagctgctgccacctgctgctgctgctgctgctgttgttgttgctgctgctgttgttgttgctgctgctgctgttgttgttgctgctgctgctggttaaggttacgggctgtggactcctcagctgcacgcagcaggaaggtgtagttcctcaccacctcttctaccttggccagcagctcttggcgctgggcctcggagcgcacaatgaacaccagccgcacgaaggtctcaatgaggctgctcagcacctggaagctgcccgtgatggctgccagcatgtgagttgggctcttgtccacattggccacacggcggcaggaggcccggagctccttgaacttgagagctagctcaagcttatactcggagatctgagacacatagggcttgggggcacgggcctcggggctggccacacactgccgcaggactgtcagcagctcgttggtgtccagccgggcagccaggaagccatcagggaggccataggcatgggcccgcagggcattgatcttggccaggctcccctcgaaggtggacacacggaggtcaatctcctgagtgcgggaggcctcagggctgctgctgctgcaggtagcagcatccagcacctgcagggtcctgctcaccacaggcaccacctgctcgtccagcttcatgccaggcaggatcttcatggggatagagtaggagagctcatccttgccatcactggcatcatctgccatgtcacacttgcggtagtagaagcagtagcggatggagcagcacttgctgctctcactgtcctcgtctagctcggcaggcttccggtacacctcctcgggcagtgagaacacggccatctgtctggggcctttggtctctggggcaacctggacgtaggaggggtctcccagcgtcggtgactccagagacctgcttttgggacccaaggctatggggaggcttgcctctacctccttggcctccctgggcagcatgcccaggggaggatgtgggtagacatccgaggtcagcgaggccctgtcaccctggtccagctcactgatactgtagcggcgcatcagtttcctgtaattgggagctcccagacactcgccccccgaggcacacgtggtcaggcacgaaacaccactctcagggtccgatcggcactctcgggactccaggctggtagaacgaatgcgctggacattgatggggctgctgaggctcacgcctgggccagcctctggctgcctctggctagggaggactctgtccctttccctcccccggaggctgggcactggtgtctgggtggcttgtggccggcccccccggcagatgcgcttgcagtcacagctgcgcctctgctcacgggacatgccaggcccctgctgcacagggctgctgcggagctggcagctgcagcggccaggtgctggaggttgcaggtactcggtgcctggcagctccccctggcttggtggctttagaagttcctcaaggaactccagttcatactgctttaccttctgcagttgggcctgccgctcatctgtctccttcttctggcgggttgggaaggtggcagagaataaattgcgtagccggaaaggacctcgggatgacttgggtttggcagggccttcagaggtcgagtgggctccattgagagttgtttcaagcttcctagagggcatggtgctcacctgccggctggcagcctgagacctcagtgggctctggcctcgaggttggcagctggggctctgacctcgagactggctgctggggctgtggccatgaggctggcagctggggctgtggcttcttgactggcagctggggctctgcagagccatggggtaggtagctcggggaaccaggctggtctcttcgagcttgcttcttttgggtgtgctctccagctgcgccttctccccttggctggagatggtgccctgcttctgcagggtgggcttaccacccactggcccgcctttgcctgccacctcccctgtagcttgcttgcccactgactctcggcttgttcgcaaaagatagcttttgggagggaaattttgaacaggcagactgtcctcttgttgggagaggtgcaggctgtcagcccggctgcctgtgggtgctctggggctggaagagacctctgcacccagctgatgttgagaattccatgaggtctctggagcactggggctaattttgaacttcagattcttactggcactgctgctcatcatgctaacctctggcctccccatgctggcctccagccttctctcacccctgctgggggggttccccaaagccccaccagcagtgactagactcttattgtgaaccacttgctgtagggcggccgagatgatggcaggggtcacactgctctttgggtcgaggataagcttggggctcaacctgacctccttgggcaggttgtccctcagctcagagacctgctcttcactgagggatgatgtggctgccctcagtgacatttctaggcctgccctagtgtggccaggccctttgtcctcaggaactggggacagcagactcagattcttctgttcactaagctgtggggacagtgctgggtgcactgccaaggagtatgttcgttctccctgtacctggccctctgactggggcagcttcctccgagcgccaggggggccaggactctggcctgtggcaatgggttggagagatgggttgggatccgggcgcccaagagagtaaggggccgtaagaacggcctgggctgcacagctctggatccggaagggcaggtccttgcgggcaaggaggctgtccttgttgaggtgctgggccaggaagtaggtggtgttctggtgctgcttcatggccgacatcatctctgacatgtctgtgagctctgaagagttggtttcatgacctgagtccagcgatgattcaggagtgattgtggccagcacaatcagacctgcagtctgtgggggtggtgggtgtggtccatcctcggatgcagccagggcttctagagcctgcagagtggacaccagggcatcatctagctcctgggcatgatctcgaactgtccgggtctgcacactgtcaatcaatgtcactggaatctcatcgtacagaagcccacgcaggtggcgtccttgttcctggctctggacagcccggcgcttggggtcatcctcatcagagctgttgtctcggaaaccagggggtggggcagcaatggctggcaacagagaagttgtctcatcttcctcctcctcctcctcctcactcccaggtggtgggagggacatcaaatctactatattgtcacgagaggagccaggcttcccacctttgcgagggcccagctgctcctgaagtttggctttgcaagagtcacagtagaaattcagggcttcagccccaagggaattgtccaaggtgtaggaccgggccctgctggcacaaggctcgtggtctaggctagctgcatcaaagtcatcagggactacctcataaccttggccagagcttttggatgtggggtcagacttggttcggggcctggtctcctcaaagaagattaggttctcgttgacatctgtccggctttcctgctccttcctttgttcccgcatatggaggtagcagaagctgacaagctcagagtcggcaggtgggggcgtgcagcggctcgatttcctggggctggtgcccacgctgcccacataactactctcctttttccccaggtggcccccagtgacagggcggtgggcgctgtgcatgtaatctgccttgatcattggaggtggaagtggctggctggcaggcctggagaagaccatcttcctggaatccagcaagaggcggcagtaccccgcgatcaggcaggcaaagttggtggcttcaggccactccatcaacagcaccagaggcttggcatccatgatgctggtctccacccgggccacgccctggttctcccggaacagctggatcttgctgatcttgctgaactcggacagcacagtggtgaggttggttttgaggtcaataacatggctgatgccatgacggggtcccaccaggagcgtggtggccgactgcttctcatccaggcctacagtgttgaacaaaacgcccgtgaaggtaggaagttcattcagaattcgtagatactggagctttgcctgaattgcagagcccttggtgccgcaggaaggatgtgtttggtgagccttcagttgctgagagagagatttccggaggttcttctctttgatgacctgcaggagggaggggggaagaaagggttccaggccccactccttctccacattcttgagcgagatcttctgactaggtcgagtggctgagacagtgatatagatgtggagcgcagcaaggcccaaaagcatctctggcttgggatccattccaaagcgttctcgaataacatcattccgactctggatgtataggtactcaaaagcagcaggatcccgacgcagcagctccacagggtctttgggaaagaagcttattcggaagaggcatttcattccatgatagtgtgtccgctgtaccacataagccaggggttgcttgtcctgaagaagcagaaacttgtgattctgttctggcccggcatactcaaggacaagagcaaagtgctcaatgaacctcagggaaaggcggtcctgtaatgtcaacatcacatccttaacagtggtccgaccatcaaatgtgaatgacttgatctgcccattttctaagaaaaccttcaggacattagggatgaggaggagagcttccttcttcatcattttcaaatccaagtcatacgtcctctgggttttcaagcattcaggacacacatatcctcctggtgacttggacctcggggtctgtttcacccactgcatggccttttctggtcaagatgtggagttgcaagatcacttaaatgtgaagagagctcaatttcaccagccactcattccctgagtcttcaggaagccattatttccttcctgttttgcatctgtttctccaactgccacctgctcagaaaatcgaaccttcacaggattggacctcaacttggccttcttcgcagcactgatgaaagcagatttgggggactgataagttctatgagtctctccctcggggcttcactcacgtcttcctcattaatagccacaatctggtcaccagccaggagcttgt

SEQ ID NO: 18058 - RNA, 6669 nt, Homo sapiens
  source 1..6669: mol_type = other RNA
tctggctccgtgtcttcactcccaggaaggttgcgggggtggggggcgtggggggagggttggcagcggtggtggcggtggtggtggcagcggtggtggcaataggaggtgtgtgtcaaggtggatgttaaacagtgtgaattcccttccagatggctccagagagggagaaaggtgcaggactgcaccgggtaaggcgctcagcttcttttcttagagagacaaatccacagggtcaatacacagccaaaagcatatactcaggattaacatatcacgctagcttccagaagtttaagatatagtcatcaacaccccccacccctacccctttcccccctccccccacccccctccccgatccacagctaagtcaaactcccaaggacagtctgtctggtagagagatgttgagagagaagcctcatgcctgcagcaacagcccctgagctgggctgggccgggctaggcgggctcctaggcctgcactgggtctccccaggcagacgttttcatcaggtaccttacccaaaatgagtggggtgatcccagatgcttgctccctagtggactgagctgccctgcccatcagtgaggggcagggcactttggggatggctggtgtggagctactggacctggaggtgagggctcaccaggctgccggccagttgggccgctgcaaacagcctagtgtggctgttttctgcagacatctcacccaggcacaggccctcagggtggcatctaccaggtgagtgtgagcccaaggtggatggggacatctggactgagcgccctctcccctcggcacggcaatgtggcctgctgctactgccactgctcccagcaggggagccgatgccacgaggagctcaaagcctgagggtccgcttgcttcaggccctggctcccccagcgcccaacacggattgagcaggaagtgagcctgatgtcacctctcagccccagagaagagataaaatacagctctgctgtgagcagagtgaagaggggcctttgccctcacagtgaggcccagaggccagggaaggggtgaggacacccagggcggcagctaagcctgcagcccttaagagagagcctcaatcaagagagtttccactccccggagactgatgggctcttggaccctgactggcccagcagacacacacacactcaccacaagatgcaaggaccacaaagctcaaacctggggccatggttggggaagggggacaggtgtgggcagatgccctacttaataagggtttttaaggagtgggtgaatgtgctcataacagtcgccgaagttggggagcctggtggatgctctgtggctgcccctgcagctgctgccacctgctgctgctgctgctgctgttgttgttgctgctgctgttgttgttgctgctgctgctgttgttgttgctgctgctgctggttaaggttacgggctgtggactcctcagctgcacgcagcaggaaggtgtagttcctcaccacctcttctaccttggccagcagctcttggcgctgggcctcggagcgcacaatgaacaccagccgcacgaaggtctcaatgaggctgctcagcacctggaagctgcccgtgatggctgccagcatgtgagttgggctcttgtccacattggccacacggcggcaggaggcccggagctccttgaacttgagagctagctcaagcttatactcggagatctgagacacatagggcttgggggcacgggcctcggggctggccacacactgccgcaggactgtcagcagctcgttggtgtccagccgggcagccaggaagccatcagggaggccataggcatgggcccgcagggcattgatcttggccaggctcccctcgaaggtggacacacggaggtcaatctcctgagtgcgggaggcctcagggctgctgctgctgcaggtagcagcatccagcacctgcagggtcctgctcaccacaggcaccacctgctcgtccagcttcatgccaggcaggatcttcatggggatagagtaggagagctcatccttgccatcactggcatcatctgccatgtcacacttgcggtagtagaagcagtagcggatggagcagcacttgctgctctcactgtcctcgtctagctcggcaggcttccggtacacctcctcgggcagtgagaacacggccatctgtctggggcctttggtctctggggcaacctggacgtaggaggggtctcccagcgtcggtgactccagagacctgcttttgggacccaaggctatggggaggcttgcctctacctccttggcctccctgggcagcatgcccaggggaggatgtgggtagacatccgaggtcagcgaggccctgtcaccctggtccagctcactgatactgtagcggcgcatcagtttcctgtaattgggagctcccagacactcgccccccgaggcacacgtggtcaggcacgaaacaccactctcagggtccgatcggcactctcgggactccaggctggtagaacgaatgcgctggacattgatggggctgctgaggctcacgcctgggccagcctctggctgcctctggctagggaggactctgtccctttccctcccccggaggctgggcactggtgtctgggtggcttgtggccggcccccccggcagatgcgcttgcagtcacagctgcgcctctgctcacgggacatgccaggcccctgctgcacagggctgctgcggagctggcagctgcagcggccaggtgctggaggttgcaggtactcggtgcctggcagctccccctggcttggtggctttagaagttcctcaaggaactccagttcatactgctttaccttctgcagttgggcctgccgctcatctgtctccttcttctggcgggttgggaaggtggcagagaataaattgcgtagccggaaaggacctcgggatgacttgggtttggcagggccttcagaggtcgagtgggctccattgagagttgtttcaagcttcctagagggcatggtgctcacctgccggctggcagcctgagacctcagtgggctctggcctcgaggttggcagctggggctctgacctcgagactggctgctggggctgtggccatgaggctggcagctggggctgtggcttcttgactggcagctggggctctgcagagccatggggtaggtagctcggggaaccaggctggtctcttcgagcttgcttcttttgggtgtgctctccagctgcgccttctccccttggctggagatggtgccctgcttctgcagggtgggcttaccacccactggcccgcctttgcctgccacctcccctgtagcttgcttgcccactgactctcggcttgttcgcaaaagatagcttttgggagggaaattttgaacaggcagactgtcctcttgttgggagaggtgcaggctgtcagcccggctgcctgtgggtgctctggggctggaagagacctctgcacccagctgatgttgagaattccatgaggtctctggagcactggggctaattttgaacttcagattcttactggcactgctgctcatcatgctaacctctggcctccccatgctggcctccagccttctctcacccctgctgggggggttccccaaagccccaccagcagtgactagactcttattgtgaaccacttgctgtagggcggccgagatgatggcaggggtcacactgctctttgggtcgaggataagcttggggctcaacctgacctccttgggcaggttgtccctcagctcagagacctgctcttcactgagggatgatgtggctgccctcagtgacatttctaggcctgccctagtgtggccaggccctttgtcctcaggaactggggacagcagactcagattcttctgttcactaagctgtggggacagtgctgggtgcactgccaaggagtatgttcgttctccctgtacctggccctctgactggggcagcttcctccgagcgccaggggggccaggactctggcctgtggcaatgggttggagagatgggttgggatccgggcgcccaagagagtaaggggccgtaagaacggcctgggctgcacagctctggatccggaagggcaggtccttgcgggcaaggaggctgtccttgttgaggtgctgggccaggaagtaggtggtgttctggtgctgcttcatggccgacatcatctctgacatgtctgtgagctctgaagagttggtttcatgacctgagtccagcgatgattcaggagtgattgtggccagcacaatcagacctgcagtctgtgggggtggtgggtgtggtccatcctcggatgcagccagggcttctagagcctgcagagtggacaccagggcatcatctagctcctgggcatgatctcgaactgtccgggtctgcacactgtcaatcaatgtcactggaatctcatcgtacagaagcccacgcaggtggcgtccttgttcctggctctggacagcccggcgcttggggtcatcctcatcagagctgttgtctcggaaaccagggggtggggcagcaatggctggcaacagagaagttgtctcatcttcctcctcctcctcctcctcactcccaggtggtgggagggacatcaaatctactatattgtcacgagaggagccaggcttcccacctttgcgagggcccagctgctcctgaagtttggctttgcaagagtcacagtagaaattcagggcttcagccccaagggaattgtccaaggtgtaggaccgggccctgctggcacaaggctcgtggtctaggctagctgcatcaaagtcatcagggactacctcataaccttggccagagcttttggatgtggggtcagacttggttcggggcctggtctcctcaaagaagattaggttctcgttgacatctgtccggctttcctgctccttcctttgttcccgcatatggaggtagcagaagctgacaagctcagagtcggcaggtgggggcgtgcagcggctcgatttcctggggctggtgcccacgctgcccacataactactctcctttttccccaggtggcccccagtgacagggcggtgggcgctgtgcatgtaatctgccttgatcattggaggtggaagtggctggctggcaggcctggagaagaccatcttcctggaatccagcaagaggcggcagtaccccgcgatcaggcaggcaaagttggtggcttcaggccactccatcaacagcaccagaggcttggcatccatgatgctggtctccacccgggccacgccctggttctcccggaacagctggatcttgctgatcttgctgaactcggacagcacagtggtgaggttggttttgaggtcaataacatggctgatgccatgacggggtcccaccaggagcgtggtggccgactgcttctcatccaggcctacagtgttgaacaaaacgcccgtgaaggtaggaagttcattcagaattcgtagatactggagctttgcctgaattgcagagcccttggtgccgcaggaaggatgtgtttggtgagccttcagttgctgagagagagatttccggaggttcttctctttgatgacctgcaggagggaggggggaagaaagggttccaggccccactccttctccacattcttgagcgagatcttctgactaggtcgagtggctgagacagtgatatagatgtggagcgcagcaaggcccaaaagcatctctggcttgggatccattccaaagcgttctcgaataacatcattccgactctggatgtataggtactcaaaagcagcaggatcccgacgcagcagctccacagggtctttgggaaagaagcttattcggaagaggcatttcattccatgatagtgtgtccgctgtaccacataagccaggggttgcttgtcctgaagaagcagaaacttgtgattctgttctggcccggcatactcaaggacaagagcaaagtgctcaatgaacctcagggaaaggcggtcctgtaatgtcaacatcacatccttaacagtggtccgaccatcaaatgtgaatgacttgatctgcccattttctaagaaaaccttcaggacattagggatgaggaggagagcttccttcttcatcattttcaaatccaagtcatacgtcctctgggttttcaagcattcaggacacacatatcctcctggtgacttggacctcggggtctgtttcaccctgatttgcagggactccatattactccttttcccctctgctcatcaatgatcacttctcttaaaacttttcttcactgcatggccttttctggtcaagatgtggagttgcaagatcacttaaatgtgaagagagctcaatttcaccagccactcattccctgagtcttcaggaagccattatttccttcctgttttgcatctgtttctccaactgccacctgctcagaaaatcgaaccttcacaggattggacctcaacttggccttcttcgcagcactgatgaaagcagatttgggggactgataagttctatgagtctctccctcggggcttcactcacgtcttcctcattaatagccacaatctggtcaccagccaggagcttgt

SEQ ID NO: 18059 - RNA, 6507 nt, Homo sapiens
  source 1..6507: mol_type = other RNA
tctggctccgtgtcttcactcccaggaaggttgcgggggtggggggcgtggggggagggttggcagcggtggtggcggtggtggtggcagcggtggtggcaataggaggtgtgtgtcaaggtggatgttaaacagtgtgaattcccttccagatggctccagagagggagaaaggtgcaggactgcaccgggtaaggcgctcagcttcttttcttagagagacaaatccacagggtcaatacacagccaaaagcatatactcaggattaacatatcacgctagcttccagaagtttaagatatagtcatcaacaccccccacccctacccctttcccccctccccccacccccctccccgatccacagctaagtcaaactcccaaggacagtctgtctggtagagagatgttgagagagaagcctcatgcctgcagcaacagcccctgagctgggctgggccgggctaggcgggctcctaggcctgcactgggtctccccaggcagacgttttcatcaggtaccttacccaaaatgagtggggtgatcccagatgcttgctccctagtggactgagctgccctgcccatcagtgaggggcagggcactttggggatggctggtgtggagctactggacctggaggtgagggctcaccaggctgccggccagttgggccgctgcaaacagcctagtgtggctgttttctgcagacatctcacccaggcacaggccctcagggtggcatctaccaggtgagtgtgagcccaaggtggatggggacatctggactgagcgccctctcccctcggcacggcaatgtggcctgctgctactgccactgctcccagcaggggagccgatgccacgaggagctcaaagcctgagggtccgcttgcttcaggccctggctcccccagcgcccaacacggattgagcaggaagtgagcctgatgtcacctctcagccccagagaagagataaaatacagctctgctgtgagcagagtgaagaggggcctttgccctcacagtgaggcccagaggccagggaaggggtgaggacacccagggcggcagctaagcctgcagcccttaagagagagcctcaatcaagagagtttccactccccggagactgatgggctcttggaccctgactggcccagcagacacacacacactcaccacaagatgcaaggaccacaaagctcaaacctggggccatggttggggaagggggacaggtgtgggcagatgccctacttaataagggtttttaaggagtgggtgaatgtgctcataacagtcgccgaagttggggagcctggtggatgctctgtggctgcccctgcagctgctgccacctgctgctgctgctgctgctgttgttgttgctgctgctgttgttgttgctgctgctgctgttgttgttgctgctgctgctggttaaggttacgggctgtggactcctcagctgcacgcagcaggaaggtgtagttcctcaccacctcttctaccttggccagcagctcttggcgctgggcctcggagcgcacaatgaacaccagccgcacgaaggtctcaatgaggctgctcagcacctggaagctgcccgtgatggctgccagcatgtgagttgggctcttgtccacattggccacacggcggcaggaggcccggagctccttgaacttgagagctagctcaagcttatactcggagatctgagacacatagggcttgggggcacgggcctcggggctggccacacactgccgcaggactgtcagcagctcgttggtgtccagccgggcagccaggaagccatcagggaggccataggcatgggcccgcagggcattgatcttggccaggctcccctcgaaggtggacacacggaggtcaatctcctgagtgcgggaggcctcagggctgctgctgctgcaggtagcagcatccagcacctgcagggtcctgctcaccacaggcaccacctgctcgtccagcttcatgccaggcaggatcttcatggggatagagtaggagagctcatccttgccatcactggcatcatctgccatgtcacacttgcggtagtagaagcagtagcggatggagcagcacttgctgctctcactgtcctcgtctagctcggcaggcttccggtacacctcctcgggcagtgagaacacggccatctgtctggggcctttggtctctggggcaacctggacgtaggaggggtctcccagcgtcggtgactccagagacctgcttttgggacccaaggctatggggaggcttgcctctacctccttggcctccctgggcagcatgcccaggggaggatgtgggtagacatccgaggtcagcgaggccctgtcaccctggtccagctcactgatactgtagcggcgcatcagtttcctgtaattgggagctcccagacactcgccccccgaggcacacgtggtcaggcacgaaacaccactctcagggtccgatcggcactctcgggactccaggctggtagaacgaatgcgctggacattgatggggctgctgaggctcacgcctgggccagcctctggctgcctctggctagggaggactctgtccctttccctcccccggaggctgggcactggtgtctgggtggcttgtggccggcccccccggcagatgcgcttgcagtcacagctgcgcctctgctcacgggacatgccaggcccctgctgcacagggctgctgcggagctggcagctgcagcggccaggtgctggaggttgcaggtactcggtgcctggcagctccccctggcttggtggctttagaagttcctcaaggaactccagttcatactgctttaccttctgcagttgggcctgccgctcatctgtctccttcttctggcgggttgggaaggtggcagagaataaattgcgtagccggaaaggacctcgggatgacttgggtttggcagggccttcagaggtcgagtgggctccattgagagttgtttcaagcttcctagagggcatggtgctcacctgccggctggcagcctgagacctcagtgggctctggcctcgaggttggcagctggggctctgacctcgagactggctgctggggctgtggccatgaggctggcagctggggctgtggcttcttgactggcagctggggctctgcagagccatggggtaggtagctcggggaaccaggctggtctcttcgagcttgcttcttttgggtgtgctctccagctgcgccttctccccttggctggagatggtgccctgcttctgcagggtgggcttaccacccactggcccgcctttgcctgccacctcccctgtagcttgcttgcccactgactctcggcttgttcgcaaaagatagcttttgggagggaaattttgaacaggcagactgtcctcttgttgggagaggtgcaggctgtcagcccggctgcctgtgggtgctctggggctggaagagacctctgcacccagctgatgttgagaattccatgaggtctctggagcactggggctaattttgaacttcagattcttactggcactgctgctcatcatgctaacctctggcctccccatgctggcctccagccttctctcacccctgctgggggggttccccaaagccccaccagcagtgactagactcttattgtgaaccacttgctgtagggcggccgagatgatggcaggggtcacactgctctttgggtcgaggataagcttggggctcaacctgacctccttgggcaggttgtccctcagctcagagacctgctcttcactgagggatgatgtggctgccctcagtgacatttctaggcctgccctagtgtggccaggccctttgtcctcaggaactggggacagcagactcagattcttctgttcactaagctgtggggacagtgctgggtgcactgccaaggagtatgttcgttctccctgtacctggccctctgactggggcagcttcctccgagcgccaggggggccaggactctggcctgtggcaatgggttggagagatgggttgggatccgggcgcccaagagagtaaggggccgtaagaacggcctgggctgcacagctctggatccggaagggcaggtccttgcgggcaaggaggctgtccttgttgaggtgctgggccaggaagtaggtggtgttctggtgctgcttcatggccgacatcatctctgacatgtctgtgagctctgaagagttggtttcatgacctgagtccagcgatgattcaggagtgattgtggccagcacaatcagacctgcagtctgtgggggtggtgggtgtggtccatcctcggatgcagccagggcttctagagcctgcagagtggacaccagggcatcatctagctcctgggcatgatctcgaactgtccgggtctgcacactgtcaatcaatgtcactggaatctcatcgtacagaagcccacgcaggtggcgtccttgttcctggctctggacagcccggcgcttggggtcatcctcatcagagctgttgtctcggaaaccagggggtggggcagcaatggctggcaacagagaagttgtctcatcttcctcctcctcctcctcctcactcccaggtggtgggagggacatcaaatctactatattgtcacgagaggagccaggcttcccacctttgcgagggcccagctgctcctgaagtttggctttgcaagagtcacagtagaaattcagggcttcagccccaagggaattgtccaaggtgtaggaccgggccctgctggcacaaggctcgtggtctaggctagctgcatcaaagtcatcagggactacctcataaccttggccagagcttttggatgtggggtcagacttggttcggggcctggtctcctcaaagaagattaggttctcgttgacatctgtccggctttcctgctccttcctttgttcccgcatatggaggtagcagaagctgacaagctcagagtcggcaggtgggggcgtgcagcggctcgatttcctggggctggtgcccacgctgcccacataactactctcctttttccccaggtggcccccagtgacagggcggtgggcgctgtgcatgtaatctgccttgatcattggaggtggaagtggctggctggcaggcctggagaagaccatcttcctggaatccagcaagaggcggcagtaccccgcgatcaggcaggcaaagttggtggcttcaggccactccatcaacagcaccagaggcttggcatccatgatgctggtctccacccgggccacgccctggttctcccggaacagctggatcttgctgatcttgctgaactcggacagcacagtggtgaggttggttttgaggtcaataacatggctgatgccatgacggggtcccaccaggagcgtggtggccgactgcttctcatccaggcctacagtgttgaacaaaacgcccgtgaaggtaggaagttcattcagaattcgtagatactggagctttgcctgaattgcagagcccttggtgccgcaggaaggatgtgtttggtgagccttcagttgctgagagagagatttccggaggttcttctctttgatgacctgcaggagggaggggggaagaaagggttccaggccccactccttctccacattcttgagcgagatcttctgactaggtcgagtggctgagacagtgatatagatgtggagcgcagcaaggcccaaaagcatctctggcttgggatccattccaaagcgttctcgaataacatcattccgactctggatgtataggtactcaaaagcagcaggatcccgacgcagcagctccacagggtctttgggaaagaagcttattcggaagaggcatttcattccatgatagtgtgtccgctgtaccacataagccaggggttgcttgtcctgaagaagcagaaacttgtgattctgttctggcccggcatactcaaggacaagagcaaagtgctcaatgaacctcagggaaaggcggtcctgtaatgtcaacatcacatccttaacagtggtccgaccatcaaatgtgaatgacttgatctgcccattttctaagaaaaccttcaggacattagggatgaggaggagagcttccttcttcatcattttcactgcatggccttttctggtcaagatgtggagttgcaagatcacttaaatgtgaagagagctcaatttcaccagccactcattccctgagtcttcaggaagccattatttccttcctgttttgcatctgtttctccaactgccacctgctcagaaaatcgaaccttcacaggattggacctcaacttggccttcttcgcagcactgatgaaagcagatttgggggactgataagttctatgagtctctccctcggggcttcactcacgtcttcctcattaatagccacaatctggtcaccagccaggagcttgt

SEQ ID NO: 18060 - RNA, 6754 nt, Homo sapiens
  source 1..6754: mol_type = other RNA
tctggctccgtgtcttcactcccaggaaggttgcgggggtggggggcgtggggggagggttggcagcggtggtggcggtggtggtggcagcggtggtggcaataggaggtgtgtgtcaaggtggatgttaaacagtgtgaattcccttccagatggctccagagagggagaaaggtgcaggactgcaccgggtaaggcgctcagcttcttttcttagagagacaaatccacagggtcaatacacagccaaaagcatatactcaggattaacatatcacgctagcttccagaagtttaagatatagtcatcaacaccccccacccctacccctttcccccctccccccacccccctccccgatccacagctaagtcaaactcccaaggacagtctgtctggtagagagatgttgagagagaagcctcatgcctgcagcaacagcccctgagctgggctgggccgggctaggcgggctcctaggcctgcactgggtctccccaggcagacgttttcatcaggtaccttacccaaaatgagtggggtgatcccagatgcttgctccctagtggactgagctgccctgcccatcagtgaggggcagggcactttggggatggctggtgtggagctactggacctggaggtgagggctcaccaggctgccggccagttgggccgctgcaaacagcctagtgtggctgttttctgcagacatctcacccaggcacaggccctcagggtggcatctaccaggtgagtgtgagcccaaggtggatggggacatctggactgagcgccctctcccctcggcacggcaatgtggcctgctgctactgccactgctcccagcaggggagccgatgccacgaggagctcaaagcctgagggtccgcttgcttcaggccctggctcccccagcgcccaacacggattgagcaggaagtgagcctgatgtcacctctcagccccagagaagagataaaatacagctctgctgtgagcagagtgaagaggggcctttgccctcacagtgaggcccagaggccagggaaggggtgaggacacccagggcggcagctaagcctgcagcccttaagagagagcctcaatcaagagagtttccactccccggagactgatgggctcttggaccctgactggcccagcagacacacacacactcaccacaagatgcaaggaccacaaagctcaaacctggggccatggttggggaagggggacaggtgtgggcagatgccctacttaataagggtttttaaggagtgggtgaatgtgctcataacagtcgccgaagttggggagcctggtggatgctctgtggctgcccctgcagctgctgccacctgctgctgctgctgctgctgttgttgttgctgctgctgttgttgttgctgctgctgctgttgttgttgctgctgctgctggttaaggttacgggctgtggactcctcagctgcacgcagcaggaaggtgtagttcctcaccacctcttctaccttggccagcagctcttggcgctgggcctcggagcgcacaatgaacaccagccgcacgaaggtctcaatgaggctgctcagcacctggaagctgcccgtgatggctgccagcatgtgagttgggctcttgtccacattggccacacggcggcaggaggcccggagctccttgaacttgagagctagctcaagcttatactcggagatctgagacacatagggcttgggggcacgggcctcggggctggccacacactgccgcaggactgtcagcagctcgttggtgtccagccgggcagccaggaagccatcagggaggccataggcatgggcccgcagggcattgatcttggccaggctcccctcgaaggtggacacacggaggtcaatctcctgagtgcgggaggcctcagggctgctgctgctgcaggtagcagcatccagcacctgcagggtcctgctcaccacaggcaccacctgctcgtccagcttcatgccaggcaggatcttcatggggatagagtaggagagctcatccttgccatcactggcatcatctgccatgtcacacttgcggtagtagaagcagtagcggatggagcagcacttgctgctctcactgtcctcgtctagctcggcaggcttccggtacacctcctcgggcagtgagaacacggccatctgtctggggcctttggtctctggggcaacctggacgtaggaggggtctcccagcgtcggtgactccagagacctgcttttgggacccaaggctatggggaggcttgcctctacctccttggcctccctgggcagcatgcccaggggaggatgtgggtagacatccgaggtcagcgaggccctgtcaccctggtccagctcactgatactgtagcggcgcatcagtttcctgtaattgggagctcccagacactcgccccccgaggcacacgtggtcaggcacgaaacaccactctcagggtccgatcggcactctcgggactccaggctggtagaacgaatgcgctggacattgatggggctgctgaggctcacgcctgggccagcctctggctgcctctggctagggaggactctgtccctttccctcccccggaggctgggcactggtgtctgggtggcttgtggccggcccccccggcagatgcgcttgcagtcacagctgcgcctctgctcacgggacatgccaggcccctgctgcacagggctgctgcggagctggcagctgcagcggccaggtgctggaggttgcaggtactcggtgcctggcagctccccctggcttggtggctttagaagttcctcaaggaactccagttcatactgctttaccttctgcagttgggcctgccgctcatctgtctccttcttctggcgggttgggaaggtggcagagaataaattgcgtagccggaaaggacctcgggatgacttgggtttggcagggccttcagaggtcgagtgggctccattgagagttgtttcaagcttcctagagggcatggtgctcacctgccggctggcagcctgagacctcagtgggctctggcctcgaggttggcagctggggctctgacctcgagactggctgctggggctgtggccatgaggctggcagctggggctgtggcttcttgactggcagctggggctctgcagagccatggggtaggtagctcggggaaccaggctggtctcttcgagcttgcttcttttgggtgtgctctccagctgcgccttctccccttggctggagatggtgccctgcttctgcagggtgggcttaccacccactggcccgcctttgcctgccacctcccctgtagcttgcttgcccactgactctcggcttgttcgcaaaagatagcttttgggagggaaattttgaacaggcagactgtcctcttgttgggagaggtgcaggctgtcagcccggctgcctgtgggtgctctggggctggaagagacctctgcacccagctgatgttgagaattccatgaggtctctggagcactggggctaattttgaacttcagattcttactggcactgctgctcatcatgctaacctctggcctccccatgctggcctccagccttctctcacccctgctgggggggttccccaaagccccaccagcagtgactagactcttattgtgaaccacttgctgtagggcggccgagatgatggcaggggtcacactgctctttgggtcgaggataagcttggggctcaacctgacctccttgggcaggttgtccctcagctcagagacctgctcttcactgagggatgatgtggctgccctcagtgacatttctaggcctgccctagtgtggccaggccctttgtcctcaggaactggggacagcagactcagattcttctgttcactaagctgtggggacagtgctgggtgcactgccaaggagtatgttcgttctccctgtacctggccctctgactggggcagcttcctccgagcgccaggggggccaggactctggcctgtggcaatgggttggagagatgggttgggatccgggcgcccaagagagtaaggggccgtaagaacggcctgggctgcacagctctggatccggaagggcaggtccttgcgggcaaggaggctgtccttgttgaggtgctgggccaggaagtaggtggtgttctggtgctgcttcatggccgacatcatctctgacatgtctgtgagctctgaagagttggtttcatgacctgagtccagcgatgattcaggagtgattgtggccagcacaatcagacctgcagtctgtgggggtggtgggtgtggtccatcctcggatgcagccagggcttctagagcctgcagagtggacaccagggcatcatctagctcctgggcatgatctcgaactgtccgggtctgcacactgtcaatcaatgtcactggaatctcatcgtacagaagcccacgcaggtggcgtccttgttcctggctctggacagcccggcgcttggggtcatcctcatcagagctgttgtctcggaaaccagggggtggggcagcaatggctggcaacagagaagttgtctcatcttcctcctcctcctcctcctcactcccaggtggtgggagggacatcaaatctactatattgtcacgagaggagccaggcttcccacctttgcgagggcccagctgctcctgaagtttggctttgcaagagtcacagtagaaattcagggcttcagccccaagggaattgtccaaggtgtaggaccgggccctgctggcacaaggctcgtggtctaggctagctgcatcaaagtcatcagggactacctcataaccttggccagagcttttggatgtggggtcagacttggttcggggcctggtctcctcaaagaagattaggttctcgttgacatctgtccggctttcctgctccttcctttgttcccgcatatggaggtagcagaagctgacaagctcagagtcggcaggtgggggcgtgcagcggctcgatttcctggggctggtgcccacgctgcccacataactactctcctttttccccaggtggcccccagtgacagggcggtgggcgctgtgcatgtaatctgccttgatcattggaggtggaagtggctggctggcaggcctggagaagaccatcttcctggaatccagcaagaggcggcagtaccccgcgatcaggcaggcaaagttggtggcttcaggccactccatcaacagcaccagaggcttggcatccatgatgctggtctccacccgggccacgccctggttctcccggaacagctggatcttgctgatcttgctgaactcggacagcacagtggtgaggttggttttgaggtcaataacatggctgatgccatgacggggtcccaccaggagcgtggtggccgactgcttctcatccaggcctacagtgttgaacaaaacgcccgtgaaggtaggaagttcattcagaattcgtagatactggagctttgcctgaattgcagagcccttggtgccgcaggaaggatgtgtttggtgagccttcagttgctgagagagagatttccggaggttcttctctttgatgacctgcaggagggaggggggaagaaagggttccaggccccactccttctccacattcttgagcgagatcttctgactaggtcgagtggctgagacagtgatatagatgtggagcgcagcaaggcccaaaagcatctctggcttgggatccattccaaagcgttctcgaataacatcattccgactctggatgtataggtactcaaaagcagcaggatcccgacgcagcagctccacagggtctttgggaaagaagcttattcggaagaggcatttcattccatgatagtgtgtccgctgtaccacataagccaggggttgcttgtcctgaagaagcagaaacttgtgattctgttctggcccggcatactcaaggacaagagcaaagtgctcaatgaacctcagggaaaggcggtcctgtaatgtcaacatcacatccttaacagtggtccgaccatcaaatgtgaatgacttgatctgcccattttctaagaaaaccttcaggacattagggatgaggaggagagcttccttcttcatcatttttgcatctgtttctccaactgccacctgctcagaaaatcgaaccttcacaggattggacctcaacttggccttcttcgcagcactgatgaaagcagatttgggggactgataagttctatgagtctctccctcggggcttcactcacgtcttcctcattaatagccacaatctggtcaccagccaggagcttgttctcagaggggcctccttcctccccctcctcttcctcctcctcttcctcctcctcctcctcctcctccgcctcctcagcggcgcggcagcggcggcgcagcggcggcggcggcggcggcggcagcgggactagggcacccgtgcccccgagcccggcatgggcttggggctcagtggcgccgggcggcggggcgggcagaggttggcagggcggcagcagctggcccgggacgcggggagctggcgcgcaggcggcgggctgcgggcaggatggcaggagcgcgcgcgggctcctcgggcgggcttcatggctgcgccgcgggcggcaccatcgccgtggctcgctcgtcgctctctcgctccaggagt

SEQ ID NO: 18061 - RNA, 6693 nt, Homo sapiens
  source 1..6693: mol_type = other RNA
tctggctccgtgtcttcactcccaggaaggttgcgggggtggggggcgtggggggagggttggcagcggtggtggcggtggtggtggcagcggtggtggcaataggaggtgtgtgtcaaggtggatgttaaacagtgtgaattcccttccagatggctccagagagggagaaaggtgcaggactgcaccgggtaaggcgctcagcttcttttcttagagagacaaatccacagggtcaatacacagccaaaagcatatactcaggattaacatatcacgctagcttccagaagtttaagatatagtcatcaacaccccccacccctacccctttcccccctccccccacccccctccccgatccacagctaagtcaaactcccaaggacagtctgtctggtagagagatgttgagagagaagcctcatgcctgcagcaacagcccctgagctgggctgggccgggctaggcgggctcctaggcctgcactgggtctccccaggcagacgttttcatcaggtaccttacccaaaatgagtggggtgatcccagatgcttgctccctagtggactgagctgccctgcccatcagtgaggggcagggcactttggggatggctggtgtggagctactggacctggaggtgagggctcaccaggctgccggccagttgggccgctgcaaacagcctagtgtggctgttttctgcagacatctcacccaggcacaggccctcagggtggcatctaccaggtgagtgtgagcccaaggtggatggggacatctggactgagcgccctctcccctcggcacggcaatgtggcctgctgctactgccactgctcccagcaggggagccgatgccacgaggagctcaaagcctgagggtccgcttgcttcaggccctggctcccccagcgcccaacacggattgagcaggaagtgagcctgatgtcacctctcagccccagagaagagataaaatacagctctgctgtgagcagagtgaagaggggcctttgccctcacagtgaggcccagaggccagggaaggggtgaggacacccagggcggcagctaagcctgcagcccttaagagagagcctcaatcaagagagtttccactccccggagactgatgggctcttggaccctgactggcccagcagacacacacacactcaccacaagatgcaaggaccacaaagctcaaacctggggccatggttggggaagggggacaggtgtgggcagatgccctacttaataagggtttttaaggagtgggtgaatgtgctcataacagtcgccgaagttggggagcctggtggatgctctgtggctgcccctgcagctgctgccacctgctgctgctgctgctgctgttgttgttgctgctgctgttgttgttgctgctgctgctgttgttgttgctgctgctgctggttaaggttacgggctgtggactcctcagctgcacgcagcaggaaggtgtagttcctcaccacctcttctaccttggccagcagctcttggcgctgggcctcggagcgcacaatgaacaccagccgcacgaaggtctcaatgaggctgctcagcacctggaagctgcccgtgatggctgccagcatgtgagttgggctcttgtccacattggccacacggcggcaggaggcccggagctccttgaacttgagagctagctcaagcttatactcggagatctgagacacatagggcttgggggcacgggcctcggggctggccacacactgccgcaggactgtcagcagctcgttggtgtccagccgggcagccaggaagccatcagggaggccataggcatgggcccgcagggcattgatcttggccaggctcccctcgaaggtggacacacggaggtcaatctcctgagtgcgggaggcctcagggctgctgctgctgcaggtagcagcatccagcacctgcagggtcctgctcaccacaggcaccacctgctcgtccagcttcatgccaggcaggatcttcatggggatagagtaggagagctcatccttgccatcactggcatcatctgccatgtcacacttgcggtagtagaagcagtagcggatggagcagcacttgctgctctcactgtcctcgtctagctcggcaggcttccggtacacctcctcgggcagtgagaacacggccatctgtctggggcctttggtctctggggcaacctggacgtaggaggggtctcccagcgtcggtgactccagagacctgcttttgggacccaaggctatggggaggcttgcctctacctccttggcctccctgggcagcatgcccaggggaggatgtgggtagacatccgaggtcagcgaggccctgtcaccctggtccagctcactgatactgtagcggcgcatcagtttcctgtaattgggagctcccagacactcgccccccgaggcacacgtggtcaggcacgaaacaccactctcagggtccgatcggcactctcgggactccaggctggtagaacgaatgcgctggacattgatggggctgctgaggctcacgcctgggccagcctctggctgcctctggctagggaggactctgtccctttccctcccccggaggctgggcactggtgtctgggtggcttgtggccggcccccccggcagatgcgcttgcagtcacagctgcgcctctgctcacgggacatgccaggcccctgctgcacagggctgctgcggagctggcagctgcagcggccaggtgctggaggttgcaggtactcggtgcctggcagctccccctggcttggtggctttagaagttcctcaaggaactccagttcatactgctttaccttctgcagttgggcctgccgctcatctgtctccttcttctggcgggttgggaaggtggcagagaataaattgcgtagccggaaaggacctcgggatgacttgggtttggcagggccttcagaggtcgagtgggctccattgagagttgtttcaagcttcctagagggcatggtgctcacctgccggctggcagcctgagacctcagtgggctctggcctcgaggttggcagctggggctctgacctcgagactggctgctggggctgtggccatgaggctggcagctggggctgtggcttcttgactggcagctggggctctgcagagccatggggtaggtagctcggggaaccaggctggtctcttcgagcttgcttcttttgggtgtgctctccagctgcgccttctccccttggctggagatggtgccctgcttctgcagggtgggcttaccacccactggcccgcctttgcctgccacctcccctgtagcttgcttgcccactgactctcggcttgttcgcaaaagatagcttttgggagggaaattttgaacaggcagactgtcctcttgttgggagaggtgcaggctgtcagcccggctgcctgtgggtgctctggggctggaagagacctctgcacccagctgatgttgagaattccatgaggtctctggagcactggggctaattttgaacttcagattcttactggcactgctgctcatcatgctaacctctggcctccccatgctggcctccagccttctctcacccctgctgggggggttccccaaagccccaccagcagtgactagactcttattgtgaaccacttgctgtagggcggccgagatgatggcaggggtcacactgctctttgggtcgaggataagcttggggctcaacctgacctccttgggcaggttgtccctcagctcagagacctgctcttcactgagggatgatgtggctgccctcagtgacatttctaggcctgccctagtgtggccaggccctttgtcctcaggaactggggacagcagactcagattcttctgttcactaagctgtggggacagtgctgggtgcactgccaaggagtatgttcgttctccctgtacctggccctctgactggggcagcttcctccgagcgccaggggggccaggactctggcctgtggcaatgggttggagagatgggttgggatccgggcgcccaagagagtaaggggccgtaagaacggcctgggctgcacagctctggatccggaagggcaggtccttgcgggcaaggaggctgtccttgttgaggtgctgggccaggaagtaggtggtgttctggtgctgcttcatggccgacatcatctctgacatgtctgtgagctctgaagagttggtttcatgacctgagtccagcgatgattcaggagtgattgtggccagcacaatcagacctgcagtctgtgggggtggtgggtgtggtccatcctcggatgcagccagggcttctagagcctgcagagtggacaccagggcatcatctagctcctgggcatgatctcgaactgtccgggtctgcacactgtcaatcaatgtcactggaatctcatcgtacagaagcccacgcaggtggcgtccttgttcctggctctggacagcccggcgcttggggtcatcctcatcagagctgttgtctcggaaaccagggggtggggcagcaatggctggcaacagagaagttgtctcatcttcctcctcctcctcctcctcactcccaggtggtgggagggacatcaaatctactatattgtcacgagaggagccaggcttcccacctttgcgagggcccagctgctcctgaagtttggctttgcaagagtcacagtagaaattcagggcttcagccccaagggaattgtccaaggtgtaggaccgggccctgctggcacaaggctcgtggtctaggctagctgcatcaaagtcatcagggactacctcataaccttggccagagcttttggatgtggggtcagacttggttcggggcctggtctcctcaaagaagattaggttctcgttgacatctgtccggctttcctgctccttcctttgttcccgcatatggaggtagcagaagctgacaagctcagagtcggcaggtgggggcgtgcagcggctcgatttcctggggctggtgcccacgctgcccacataactactctcctttttccccaggtggcccccagtgacagggcggtgggcgctgtgcatgtaatctgccttgatcattggaggtggaagtggctggctggcaggcctggagaagaccatcttcctggaatccagcaagaggcggcagtaccccgcgatcaggcaggcaaagttggtggcttcaggccactccatcaacagcaccagaggcttggcatccatgatgctggtctccacccgggccacgccctggttctcccggaacagctggatcttgctgatcttgctgaactcggacagcacagtggtgaggttggttttgaggtcaataacatggctgatgccatgacggggtcccaccaggagcgtggtggccgactgcttctcatccaggcctacagtgttgaacaaaacgcccgtgaaggtaggaagttcattcagaattcgtagatactggagctttgcctgaattgcagagcccttggtgccgcaggaaggatgtgtttggtgagccttcagttgctgagagagagatttccggaggttcttctctttgatgacctgcaggagggaggggggaagaaagggttccaggccccactccttctccacattcttgagcgagatcttctgactaggtcgagtggctgagacagtgatatagatgtggagcgcagcaaggcccaaaagcatctctggcttgggatccattccaaagcgttctcgaataacatcattccgactctggatgtataggtactcaaaagcagcaggatcccgacgcagcagctccacagggtctttgggaaagaagcttattcggaagaggcatttcattccatgatagtgtgtccgctgtaccacataagccaggggttgcttgtcctgaagaagcagaaacttgtgattctgttctggcccggcatactcaaggacaagagcaaagtgctcaatgaacctcagggaaaggcggtcctgtaatgtcaacatcacatccttaacagtggtccgaccatcaaatgtgaatgacttgatctgcccattttctaagaaaaccttcaggacattagggatgaggaggagagcttccttcttcatcatttttgcatctgtttctccaactgccacctgctcagaaaatcgaaccttcacaggattggacctcaacttggccttcttcgcagcactgatgaaagcagatttgggggactgatgagtgtgcagaactgtaagaacgatgaattccttagcgctcctgataagttctatgagtctctccctcggggcttcactcacgtcttcctcattaatagccacaatctggtcaccagccaggagcttgttctcagaggggcctcctggcctcacagatcgaaccaccacaggcctctcactgccagccacgaagccaaagccatatatagggtctcggtgaacggtcacttgtcgcagtatctctgctggcagctgctcacattccatatcatttgcgctctcttcctgcatcacatgactggaaaagagttcctgttggccagaaggggagctgcatcctggggctgccagcaggcggtcctggaccctctggctatccagagtctccat

SEQ ID NO: 18062 - RNA, 6955 nt, Homo sapiens
  source 1..6955: mol_type = other RNA
tctggctccgtgtcttcactcccaggaaggttgcgggggtggggggcgtggggggagggttggcagcggtggtggcggtggtggtggcagcggtggtggcaataggaggtgtgtgtcaaggtggatgttaaacagtgtgaattcccttccagatggctccagagagggagaaaggtgcaggactgcaccgggtaaggcgctcagcttcttttcttagagagacaaatccacagggtcaatacacagccaaaagcatatactcaggattaacatatcacgctagcttccagaagtttaagatatagtcatcaacaccccccacccctacccctttcccccctccccccacccccctccccgatccacagctaagtcaaactcccaaggacagtctgtctggtagagagatgttgagagagaagcctcatgcctgcagcaacagcccctgagctgggctgggccgggctaggcgggctcctaggcctgcactgggtctccccaggcagacgttttcatcaggtaccttacccaaaatgagtggggtgatcccagatgcttgctccctagtggactgagctgccctgcccatcagtgaggggcagggcactttggggatggctggtgtggagctactggacctggaggtgagggctcaccaggctgccggccagttgggccgctgcaaacagcctagtgtggctgttttctgcagacatctcacccaggcacaggccctcagggtggcatctaccaggtgagtgtgagcccaaggtggatggggacatctggactgagcgccctctcccctcggcacggcaatgtggcctgctgctactgccactgctcccagcaggggagccgatgccacgaggagctcaaagcctgagggtccgcttgcttcaggccctggctcccccagcgcccaacacggattgagcaggaagtgagcctgatgtcacctctcagccccagagaagagataaaatacagctctgctgtgagcagagtgaagaggggcctttgccctcacagtgaggcccagaggccagggaaggggtgaggacacccagggcggcagctaagcctgcagcccttaagagagagcctcaatcaagagagtttccactccccggagactgatgggctcttggaccctgactggcccagcagacacacacacactcaccacaagatgcaaggaccacaaagctcaaacctggggccatggttggggaagggggacaggtgtgggcagatgccctacttaataagggtttttaaggagtgggtgaatgtgctcataacagtcgccgaagttggggagcctggtggatgctctgtggctgcccctgcagctgctgccacctgctgctgctgctgctgctgttgttgttgctgctgctgttgttgttgctgctgctgctgttgttgttgctgctgctgctggttaaggttacgggctgtggactcctcagctgcacgcagcaggaaggtgtagttcctcaccacctcttctaccttggccagcagctcttggcgctgggcctcggagcgcacaatgaacaccagccgcacgaaggtctcaatgaggctgctcagcacctggaagctgcccgtgatggctgccagcatgtgagttgggctcttgtccacattggccacacggcggcaggaggcccggagctccttgaacttgagagctagctcaagcttatactcggagatctgagacacatagggcttgggggcacgggcctcggggctggccacacactgccgcaggactgtcagcagctcgttggtgtccagccgggcagccaggaagccatcagggaggccataggcatgggcccgcagggcattgatcttggccaggctcccctcgaaggtggacacacggaggtcaatctcctgagtgcgggaggcctcagggctgctgctgctgcaggtagcagcatccagcacctgcagggtcctgctcaccacaggcaccacctgctcgtccagcttcatgccaggcaggatcttcatggggatagagtaggagagctcatccttgccatcactggcatcatctgccatgtcacacttgcggtagtagaagcagtagcggatggagcagcacttgctgctctcactgtcctcgtctagctcggcaggcttccggtacacctcctcgggcagtgagaacacggccatctgtctggggcctttggtctctggggcaacctggacgtaggaggggtctcccagcgtcggtgactccagagacctgcttttgggacccaaggctatggggaggcttgcctctacctccttggcctccctgggcagcatgcccaggggaggatgtgggtagacatccgaggtcagcgaggccctgtcaccctggtccagctcactgatactgtagcggcgcatcagtttcctgtaattgggagctcccagacactcgccccccgaggcacacgtggtcaggcacgaaacaccactctcagggtccgatcggcactctcgggactccaggctggtagaacgaatgcgctggacattgatggggctgctgaggctcacgcctgggccagcctctggctgcctctggctagggaggactctgtccctttccctcccccggaggctgggcactggtgtctgggtggcttgtggccggcccccccggcagatgcgcttgcagtcacagctgcgcctctgctcacgggacatgccaggcccctgctgcacagggctgctgcggagctggcagctgcagcggccaggtgctggaggttgcaggtactcggtgcctggcagctccccctggcttggtggctttagaagttcctcaaggaactccagttcatactgctttaccttctgcagttgggcctgccgctcatctgtctccttcttctggcgggttgggaaggtggcagagaataaattgcgtagccggaaaggacctcgggatgacttgggtttggcagggccttcagaggtcgagtgggctccattgagagttgtttcaagcttcctagagggcatggtgctcacctgccggctggcagcctgagacctcagtgggctctggcctcgaggttggcagctggggctctgacctcgagactggctgctggggctgtggccatgaggctggcagctggggctgtggcttcttgactggcagctggggctctgcagagccatggggtaggtagctcggggaaccaggctggtctcttcgagcttgcttcttttgggtgtgctctccagctgcgccttctccccttggctggagatggtgccctgcttctgcagggtgggcttaccacccactggcccgcctttgcctgccacctcccctgtagcttgcttgcccactgactctcggcttgttcgcaaaagatagcttttgggagggaaattttgaacaggcagactgtcctcttgttgggagaggtgcaggctgtcagcccggctgcctgtgggtgctctggggctggaagagacctctgcacccagctgatgttgagaattccatgaggtctctggagcactggggctaattttgaacttcagattcttactggcactgctgctcatcatgctaacctctggcctccccatgctggcctccagccttctctcacccctgctgggggggttccccaaagccccaccagcagtgactagactcttattgtgaaccacttgctgtagggcggccgagatgatggcaggggtcacactgctctttgggtcgaggataagcttggggctcaacctgacctccttgggcaggttgtccctcagctcagagacctgctcttcactgagggatgatgtggctgccctcagtgacatttctaggcctgccctagtgtggccaggccctttgtcctcaggaactggggacagcagactcagattcttctgttcactaagctgtggggacagtgctgggtgcactgccaaggagtatgttcgttctccctgtacctggccctctgactggggcagcttcctccgagcgccaggggggccaggactctggcctgtggcaatgggttggagagatgggttgggatccgggcgcccaagagagtaaggggccgtaagaacggcctgggctgcacagctctggatccggaagggcaggtccttgcgggcaaggaggctgtccttgttgaggtgctgggccaggaagtaggtggtgttctggtgctgcttcatggccgacatcatctctgacatgtctgtgagctctgaagagttggtttcatgacctgagtccagcgatgattcaggagtgattgtggccagcacaatcagacctgcagtctgtgggggtggtgggtgtggtccatcctcggatgcagccagggcttctagagcctgcagagtggacaccagggcatcatctagctcctgggcatgatctcgaactgtccgggtctgcacactgtcaatcaatgtcactggaatctcatcgtacagaagcccacgcaggtggcgtccttgttcctggctctggacagcccggcgcttggggtcatcctcatcagagctgttgtctcggaaaccagggggtggggcagcaatggctggcaacagagaagttgtctcatcttcctcctcctcctcctcctcactcccaggtggtgggagggacatcaaatctactatattgtcacgagaggagccaggcttcccacctttgcgagggcccagctgctcctgaagtttggctttgcaagagtcacagtagaaattcagggcttcagccccaagggaattgtccaaggtgtaggaccgggccctgctggcacaaggctcgtggtctaggctagctgcatcaaagtcatcagggactacctcataaccttggccagagcttttggatgtggggtcagacttggttcggggcctggtctcctcaaagaagattaggttctcgttgacatctgtccggctttcctgctccttcctttgttcccgcatatggaggtagcagaagctgacaagctcagagtcggcaggtgggggcgtgcagcggctcgatttcctggggctggtgcccacgctgcccacataactactctcctttttccccaggtggcccccagtgacagggcggtgggcgctgtgcatgtaatctgccttgatcattggaggtggaagtggctggctggcaggcctggagaagaccatcttcctggaatccagcaagaggcggcagtaccccgcgatcaggcaggcaaagttggtggcttcaggccactccatcaacagcaccagaggcttggcatccatgatgctggtctccacccgggccacgccctggttctcccggaacagctggatcttgctgatcttgctgaactcggacagcacagtggtgaggttggttttgaggtcaataacatggctgatgccatgacggggtcccaccaggagcgtggtggccgactgcttctcatccaggcctacagtgttgaacaaaacgcccgtgaaggtaggaagttcattcagaattcgtagatactggagctttgcctgaattgcagagcccttggtgccgcaggaaggatgtgtttggtgagccttcagttgctgagagagagatttccggaggttcttctctttgatgacctgcaggagggaggggggaagaaagggttccaggccccactccttctccacattcttgagcgagatcttctgactaggtcgagtggctgagacagtgatatagatgtggagcgcagcaaggcccaaaagcatctctggcttgggatccattccaaagcgttctcgaataacatcattccgactctggatgtataggtactcaaaagcagcaggatcccgacgcagcagctccacagggtctttgggaaagaagcttattcggaagaggcatttcattccatgatagtgtgtccgctgtaccacataagccaggggttgcttgtcctgaagaagcagaaacttgtgattctgttctggcccggcatactcaaggacaagagcaaagtgctcaatgaacctcagggaaaggcggtcctgtaatgtcaacatcacatccttaacagtggtccgaccatcaaatgtgaatgacttgatctgcccattttctaagaaaaccttcaggacattagggatgaggaggagagcttccttcttcatcatttttgcatctgtttctccaactgccacctgctcagaaaatcgaaccttcacaggattggacctcaacttggccttcttcgcagcactgatgaaagcagatttgggggactgatgagtgtgcagaactgtaagaacgatgaattccttagcgctcctgataagttctatgagtctctccctcggggcttcactcacgtcttcctcattaatagccacaatctggtcaccagccaggagcttgttctcagaggggcctcctggcctcacagatcgaaccaccacaggcctctcactgccagccacgaagccaaagccatatatagggtctcggtgaacggtcacttgtcgcagtatctctgctggcagctgctcacattccatatcatttgcgctctcttcctgcatcacatgacttcctccccctcctcttcctcctcctcttcctcctcctcctcctcctcctccgcctcctcagcggcgcggcagcggcggcgcagcggcggcggcggcggcggcggcagcgggactagggcacccgtgcccccgagcccggcatgggcttggggctcagtggcgccgggcggcggggcgggcagaggttggcagggcggcagcagctggcccgggacgcggggagctggcgcgcaggcggcgggctgcgggcaggatggcaggagcgcgcgcgggctcctcgggcgggcttcatggctgcgccgcgggcggcaccatcgccgtggctcgctcgtcgctctctcgctccaggagt

SEQ ID NO: 18063 - RNA, 6825 nt, Homo sapiens
  source 1..6825: mol_type = other RNA
tctggctccgtgtcttcactcccaggaaggttgcgggggtggggggcgtggggggagggttggcagcggtggtggcggtggtggtggcagcggtggtggcaataggaggtgtgtgtcaaggtggatgttaaacagtgtgaattcccttccagatggctccagagagggagaaaggtgcaggactgcaccgggtaaggcgctcagcttcttttcttagagagacaaatccacagggtcaatacacagccaaaagcatatactcaggattaacatatcacgctagcttccagaagtttaagatatagtcatcaacaccccccacccctacccctttcccccctccccccacccccctccccgatccacagctaagtcaaactcccaaggacagtctgtctggtagagagatgttgagagagaagcctcatgcctgcagcaacagcccctgagctgggctgggccgggctaggcgggctcctaggcctgcactgggtctccccaggcagacgttttcatcaggtaccttacccaaaatgagtggggtgatcccagatgcttgctccctagtggactgagctgccctgcccatcagtgaggggcagggcactttggggatggctggtgtggagctactggacctggaggtgagggctcaccaggctgccggccagttgggccgctgcaaacagcctagtgtggctgttttctgcagacatctcacccaggcacaggccctcagggtggcatctaccaggtgagtgtgagcccaaggtggatggggacatctggactgagcgccctctcccctcggcacggcaatgtggcctgctgctactgccactgctcccagcaggggagccgatgccacgaggagctcaaagcctgagggtccgcttgcttcaggccctggctcccccagcgcccaacacggattgagcaggaagtgagcctgatgtcacctctcagccccagagaagagataaaatacagctctgctgtgagcagagtgaagaggggcctttgccctcacagtgaggcccagaggccagggaaggggtgaggacacccagggcggcagctaagcctgcagcccttaagagagagcctcaatcaagagagtttccactccccggagactgatgggctcttggaccctgactggcccagcagacacacacacactcaccacaagatgcaaggaccacaaagctcaaacctggggccatggttggggaagggggacaggtgtgggcagatgccctacttaataagggtttttaaggagtgggtgaatgtgctcataacagtcgccgaagttggggagcctggtggatgctctgtggctgcccctgcagctgctgccacctgctgctgctgctgctgctgttgttgttgctgctgctgttgttgttgctgctgctgctgttgttgttgctgctgctgctggttaaggttacgggctgtggactcctcagctgcacgcagcaggaaggtgtagttcctcaccacctcttctaccttggccagcagctcttggcgctgggcctcggagcgcacaatgaacaccagccgcacgaaggtctcaatgaggctgctcagcacctggaagctgcccgtgatggctgccagcatgtgagttgggctcttgtccacattggccacacggcggcaggaggcccggagctccttgaacttgagagctagctcaagcttatactcggagatctgagacacatagggcttgggggcacgggcctcggggctggccacacactgccgcaggactgtcagcagctcgttggtgtccagccgggcagccaggaagccatcagggaggccataggcatgggcccgcagggcattgatcttggccaggctcccctcgaaggtggacacacggaggtcaatctcctgagtgcgggaggcctcagggctgctgctgctgcaggtagcagcatccagcacctgcagggtcctgctcaccacaggcaccacctgctcgtccagcttcatgccaggcaggatcttcatggggatagagtaggagagctcatccttgccatcactggcatcatctgccatgtcacacttgcggtagtagaagcagtagcggatggagcagcacttgctgctctcactgtcctcgtctagctcggcaggcttccggtacacctcctcgggcagtgagaacacggccatctgtctggggcctttggtctctggggcaacctggacgtaggaggggtctcccagcgtcggtgactccagagacctgcttttgggacccaaggctatggggaggcttgcctctacctccttggcctccctgggcagcatgcccaggggaggatgtgggtagacatccgaggtcagcgaggccctgtcaccctggtccagctcactgatactgtagcggcgcatcagtttcctgtaattgggagctcccagacactcgccccccgaggcacacgtggtcaggcacgaaacaccactctcagggtccgatcggcactctcgggactccaggctggtagaacgaatgcgctggacattgatggggctgctgaggctcacgcctgggccagcctctggctgcctctggctagggaggactctgtccctttccctcccccggaggctgggcactggtgtctgggtggcttgtggccggcccccccggcagatgcgcttgcagtcacagctgcgcctctgctcacgggacatgccaggcccctgctgcacagggctgctgcggagctggcagctgcagcggccaggtgctggaggttgcaggtactcggtgcctggcagctccccctggcttggtggctttagaagttcctcaaggaactccagttcatactgctttaccttctgcagttgggcctgccgctcatctgtctccttcttctggcgggttgggaaggtggcagagaataaattgcgtagccggaaaggacctcgggatgacttgggtttggcagggccttcagaggtcgagtgggctccattgagagttgtttcaagcttcctagagggcatggtgctcacctgccggctggcagcctgagacctcagtgggctctggcctcgaggttggcagctggggctctgacctcgagactggctgctggggctgtggccatgaggctggcagctggggctgtggcttcttgactggcagctggggctctgcagagccatggggtaggtagctcggggaaccaggctggtctcttcgagcttgcttcttttgggtgtgctctccagctgcgccttctccccttggctggagatggtgccctgcttctgcagggtgggcttaccacccactggcccgcctttgcctgccacctcccctgtagcttgcttgcccactgactctcggcttgttcgcaaaagatagcttttgggagggaaattttgaacaggcagactgtcctcttgttgggagaggtgcaggctgtcagcccggctgcctgtgggtgctctggggctggaagagacctctgcacccagctgatgttgagaattccatgaggtctctggagcactggggctaattttgaacttcagattcttactggcactgctgctcatcatgctaacctctggcctccccatgctggcctccagccttctctcacccctgctgggggggttccccaaagccccaccagcagtgactagactcttattgtgaaccacttgctgtagggcggccgagatgatggcaggggtcacactgctctttgggtcgaggataagcttggggctcaacctgacctccttgggcaggttgtccctcagctcagagacctgctcttcactgagggatgatgtggctgccctcagtgacatttctaggcctgccctagtgtggccaggccctttgtcctcaggaactggggacagcagactcagattcttctgttcactaagctgtggggacagtgctgggtgcactgccaaggagtatgttcgttctccctgtacctggccctctgactggggcagcttcctccgagcgccaggggggccaggactctggcctgtggcaatgggttggagagatgggttgggatccgggcgcccaagagagtaaggggccgtaagaacggcctgggctgcacagctctggatccggaagggcaggtccttgcgggcaaggaggctgtccttgttgaggtgctgggccaggaagtaggtggtgttctggtgctgcttcatggccgacatcatctctgacatgtctgtgagctctgaagagttggtttcatgacctgagtccagcgatgattcaggagtgattgtggccagcacaatcagacctgcagtctgtgggggtggtgggtgtggtccatcctcggatgcagccagggcttctagagcctgcagagtggacaccagggcatcatctagctcctgggcatgatctcgaactgtccgggtctgcacactgtcaatcaatgtcactggaatctcatcgtacagaagcccacgcaggtggcgtccttgttcctggctctggacagcccggcgcttggggtcatcctcatcagagctgttgtctcggaaaccagggggtggggcagcaatggctggcaacagagaagttgtctcatcttcctcctcctcctcctcctcactcccaggtggtgggagggacatcaaatctactatattgtcacgagaggagccaggcttcccacctttgcgagggcccagctgctcctgaagtttggctttgcaagagtcacagtagaaattcagggcttcagccccaagggaattgtccaaggtgtaggaccgggccctgctggcacaaggctcgtggtctaggctagctgcatcaaagtcatcagggactacctcataaccttggccagagcttttggatgtggggtcagacttggttcggggcctggtctcctcaaagaagattaggttctcgttgacatctgtccggctttcctgctccttcctttgttcccgcatatggaggtagcagaagctgacaagctcagagtcggcaggtgggggcgtgcagcggctcgatttcctggggctggtgcccacgctgcccacataactactctcctttttccccaggtggcccccagtgacagggcggtgggcgctgtgcatgtaatctgccttgatcattggaggtggaagtggctggctggcaggcctggagaagaccatcttcctggaatccagcaagaggcggcagtaccccgcgatcaggcaggcaaagttggtggcttcaggccactccatcaacagcaccagaggcttggcatccatgatgctggtctccacccgggccacgccctggttctcccggaacagctggatcttgctgatcttgctgaactcggacagcacagtggtgaggttggttttgaggtcaataacatggctgatgccatgacggggtcccaccaggagcgtggtggccgactgcttctcatccttggtgccgcaggaaggatgtgtttggtgagccttcagttgctgagagagagatttccggaggttcttctctttgatgacctgcaggagggaggggggaagaaagggttccaggccccactccttctccacattcttgagcgagatcttctgactaggtcgagtggctgagacagtgatatagatgtggagcgcagcaaggcccaaaagcatctctggcttgggatccattccaaagcgttctcgaataacatcattccgactctggatgtataggtactcaaaagcagcaggatcccgacgcagcagctccacagggtctttgggaaagaagcttattcggaagaggcatttcattccatgatagtgtgtccgctgtaccacataagccaggggttgcttgtcctgaagaagcagaaacttgtgattctgttctggcccggcatactcaaggacaagagcaaagtgctcaatgaacctcagggaaaggcggtcctgtaatgtcaacatcacatccttaacagtggtccgaccatcaaatgtgaatgacttgatctgcccattttctaagaaaaccttcaggacattagggatgaggaggagagcttccttcttcatcatttttgcatctgtttctccaactgccacctgctcagaaaatcgaaccttcacaggattggacctcaacttggccttcttcgcagcactgatgaaagcagatttgggggactgatgagtgtgcagaactgtaagaacgatgaattccttagcgctcctgataagttctatgagtctctccctcggggcttcactcacgtcttcctcattaatagccacaatctggtcaccagccaggagcttgttctcagaggggcctcctggcctcacagatcgaaccaccacaggcctctcactgccagccacgaagccaaagccatatatagggtctcggtgaacggtcacttgtcgcagtatctctgctggcagctgctcacattccatatcatttgcgctctcttcctgcatcacatgactggggaaaagggaaggtgggagcaaaacaagatgcacagggaactaagcctcagaaccagcagggagagatgccagttagggttctggccctggcacccaggagtttacagcttagcttcctacatcctctggagccaacagagatgatgactgcctcatatttcagattggagaaagagaaatctagaaagtagaagctactgtcttcagggctacagccaatagaagaaactgacgtcatgagcctgaaattagagtcagacccttcctctcagatattggaactccagaaggaacccaatgcaaatattc

SEQ ID NO: 18064 - RNA, 593 nt, Homo sapiens
  source 1..593: mol_type = other RNA
tctggctccgtgtcttcactcccgtggcctctgtgcccacgggcctgcccaccatgctctgcaaagacctcctcacctgagacaccctcatctccgactttgtggtcttgggacctgtggcctgggagtaggtgcccatattccttggagacatcttcatcctccttttcacggtctgggtggctccagaaatgatgcccattctctgtggaaacatccttgttctcatctggatggtctctagggctgtggaggtggtggcgaagctctgctgatgcctcctcggagagcccggcgactccagtgctgttgttccggtttctgaagcctagcccatcccctctgagctgctgggtcatggccggggggaggagcaggctggccaccccagcccagaggacagaagcgtgcagccatggcctatggtggcccatggggacggacaggcagcactggctccagctgcctctgcggcaatgtggacaaacgttggggtctttgtccctttggggttggtctctttttttctctgtgtctctcctttgtcctttcggtctctgtccaccttcctctggtccttgctgcctggctct

SEQ ID NO: 18065 - RNA, 661 nt, Homo sapiens
  source 1..661: mol_type = other RNA
tctggctccgtgtcttcactcccgtggcctctgtgcccacgggcctgcccaccatgctctgcaaagacctcctcacctgagacaccctcatctccgactttgtggtcttgggacctgtggcctgggagtaggtgcccatattccttggagacatcttcatcctccttttcacggtctgggtggctccagaaatgatgcccattctctgtggaaacatccttgttctcatctggatggtctctagggctgtggaggtggtggcgaagctctgctgatgcctcctcggagagcccggcgactccagtgctgttgttccggtttctgaagcctagcccatcccctctgagctgctgggtcatggccggggggaggagcaggctggccaccccagcccagaggacagaagcgtgcagccatggcctatggtggcccatggggacggacaggcagcactggctccagctgcctctgcggcaatgtggacaaacgttggggtctttgtccctttggggttggtctctttttttctctgtgtctctcctttgtcctttcggtctctgtccaccttcctctggtccttgctgcctggctctggacacccctctgaggctgtctccggagccccctgacccccctctggggccctccctccccattcccc

SEQ ID NO: 18066 - RNA, 57 nt, Homo sapiens
  source 1..57: mol_type = other RNA
tctggctgtgctgtaatgcagcagggtgcagactgcattacagcacagccagactgc

SEQ ID NO: 18067 - RNA, 1569 nt, Homo sapiens
  source 1..1569: mol_type = other RNA
tctggctgtgctgtaatgcaggaggactccagaagccctgttgtctggacttagagaacatgcctccagccctgggtcaaagtcctgttatgattaactccagggaactggtatggattgaggatgaaggtacagagactttcagctatgaaaatcggtctgcagtcaggattccaagtttaatctctgtgaaaccgatgggccagtgtggccatgcttactaattagacagcagcaatgtaattgatcaaatcaattcccttcatgacgcaaagccaaagaatccagggacagctggagcttggaagagcttgcagaaagccagagaatgtgaatccctctcccagagatgttaacgtggttaagctaaatttttgtgctaattgctggctcctttctcaataacggataatatggtgatgcaatgtagctcccgtgtccctcacgtggccagactctaggctggagagatttaaattgtgctcattcatttctttcctggatttacagcaagcattcaacgtcttcaagcttaaagagcctttgctttcaagcggtagagcgatgaagaagggtagccagcacaagatgaacataccgaccacaatgcccaacgtcttagctgctttcttttccctggagaacttaaaaagtttgacagctatggaactcctggggttgtggcccttggccttggtactgctaagggtgtcctcgtgaaagttcttggaatggatcctcagggtcagctccttggagttggacatctccttcatgactcctgcctctaggttcttggtggttctcttggccactatatagacacggcagtacatgactagaatgaccgccagagggatgtagaaggagcccagagaggagaagagggcatagaagggttcttcggtgaccccgcactccttgtcatcgttgggtgccggctccttccacccaaggagaggcccgatggagatgacggtggacaagacccagacactgagcagcgccaagatggccttcctccgggtgaccagcgtgggatactgcagagagtagcgcaccccgatgtagcgatcgatggagatggcgcacaggctcagaatggacgctgtgcagcacaggacatccacggctgcccagatgtcacagaagatccgccccagcacccagtagccgagcacctctagggccgctgagaagggcaggacggtgaagctcaacagcaggtcggccatggccaggttgacaatgaagtagttggtgggcgtccgcaggtgccggttgcaggccacagacaagatgactaggatgttgcccacgatggcaaagaggatgaaggcgcccagcaccaggcccacagagatggccctggtgatgtccagctggggcagtgtggagttgctcgaggtctggttggggccagtgaagttggcatttttcaactctccccagtgggcaggtgctgatgtgttgtggccggtgtccaggtcgggattcatcttagagtccgccctccatagccagggggatgattgggctcggaagggctgcggcgaaggctcctcagct

SEQ ID NO: 18068 - RNA, 1677 nt, Homo sapiens
  source 1..1677: mol_type = other RNA
tctggctgtgctgtaatgcaggaggactccagaagccctgttgtctggacttagagaacatgcctccagccctgggtcaaagtcctgttatgattaactccagggaactggtatggattgaggatgaaggtacagagactttcagctatgaaaatcggtctgcagtcaggattccaagtttaatctctgtgaaaccgatgggccagtgtggccatgcttactaattagacagcagcaatgtaattgatcaaatcaattcccttcatgacgcaaagccaaagaatccagggacagctggagcttggaagagcttgcagaaagccagagaatgtgaatccctctcccagagatgttaacgtggttaagctaaatttttgtgctaattgctggctcctttctcaataacggataatatggtgatgcaatgtagctcccgtgtccctcacgtggccagactctaggctggagagatttaaattgtgctcattcatttctttcctggatttacagcaagcattcaacgtcttcaagcttaaagagcctttgctttctgatcttgtggcatcaagaggcaggaccagaggcagattcatgatggaagagtgtccccatggtgctggcaccacacgtaggtgggtgggtggtggtgaatccgggtcaagcggtagagcgatgaagaagggtagccagcacaagatgaacataccgaccacaatgcccaacgtcttagctgctttcttttccctggagaacttaaaaagtttgacagctatggaactcctggggttgtggcccttggccttggtactgctaagggtgtcctcgtgaaagttcttggaatggatcctcagggtcagctccttggagttggacatctccttcatgactcctgcctctaggttcttggtggttctcttggccactatatagacacggcagtacatgactagaatgaccgccagagggatgtagaaggagcccagagaggagaagagggcatagaagggttcttcggtgaccccgcactccttgtcatcgttgggtgccggctccttccacccaaggagaggcccgatggagatgacggtggacaagacccagacactgagcagcgccaagatggccttcctccgggtgaccagcgtgggatactgcagagagtagcgcaccccgatgtagcgatcgatggagatggcgcacaggctcagaatggacgctgtgcagcacaggacatccacggctgcccagatgtcacagaagatccgccccagcacccagtagccgagcacctctagggccgctgagaagggcaggacggtgaagctcaacagcaggtcggccatggccaggttgacaatgaagtagttggtgggcgtccgcaggtgccggttgcaggccacagacaagatgactaggatgttgcccacgatggcaaagaggatgaaggcgcccagcaccaggcccacagagatggccctggtgatgtccagctggggcagtgtggagttgctcgaggtctggttggggccagtgaagttggcatttttcaactctccccagtgggcaggtgctgatgtgttgtggccggtgtccaggtcgggattcatcttagagtccgccctccatagccagggggatgattgggctcggaagggctgcggcgaaggctcctcagct

SEQ ID NO: 18069 - RNA, 4488 nt, Homo sapiens
  source 1..4488: mol_type = other RNA
tctgggcaacaaagtgagacctacaaaaaaacaaaaataaaataaaaataaagcaaagtttgactgtttaaagggtaatttaagtatgagaaactggtgattggaaatcactgccaaaaagggaagtcttcccagagccttgctgctcacagtgtggtctgaagctgagatcccccgggaggttgtaagaaaggtaacatcccagcttatctgaatccagatctgcattttaaaaagatctccagatgtttgtgtccatatgtacattaaaggttgagaagtccggctctggagagttccttcacttgctttctgaagtgatggactccttggattgggcctgttctgaccaaccaactgagcacaggtctgccagttccttcacgtagtcagttggagcataaccagcacatgctggggacaagctgcacatgtgcagacaagagtggggaaatccccactcttaccacttcaagaaagccactttctgaaaatttcaagattctactctagtaatagctttgactgggaaggagatgtggtatctaccctggagtctgtgggcaagacaggtggtcatgatctgggttaggtgagagactgtaactatgttgattctggggatttcctaaggactagcagcactagctttaactgctttagtaagcgaaatcttatgtctgcaatccgaggtcatgggaaatctctttctggacctgagggaatcctatctccctaaggtcttctactagatgcagatccaggtaggactggcattctactccccaagtttcacctgaacctagctattctgttttttcttctttttcttttattctttttttttttttttttttttttttttttttttttgagacggagttttgctctttcgcccaggctggagtgtagtggcccgatcttggctcactgcaacctccgccttccggtttcaagcaattctgcctcggcttcccgagtagctgggattacaggcgcctgccaccacgcccggctaatttttgtgtttttagtacaggcggggtttcatcatgttggccaggctagtctcgaactcttgacctcatgatccacccgcctcagcctcccaaaatgctgggattacaggtgtgagccaccgcgcccggccacctagctgttctttatcaagtgactgtagtcatcatcccacctgcctgcttgtatttatttaaatatctgcattaattactgttaactaacttatttatacatataagaagtattcagagtaactttcaaaaacacatatgagataaattattaagtgaggaaaccttggcaattggagtatttgttttaagagggcaatagtattataatgaaaacctcctgacctgtggctctggggttcatgtttcttcttatcgaggtctcaggccttccagtccaatatattttgctccaaattttacttcaaggagagatcaagtatcaaatacctcatcaaattggagactttagggagtaaggcttaggaaaaatcaagagaatcaagggacccaattttcagtgggttttataatcataaagccacatgagtagttgactatcttcctgaataaattgttccatgttatcattaaatgtctcagcctggccagctctcgcattggtaaagcattggtggggatggaatatccctgagagatccatattcagagctctttcacaagtccagaaatgttcagtgtgcttttctgcttgtccaacactttcttgagcaattgatatcttctgaagctgacacatgacagggtggaagtatgtttcatctcagagggagaatcttgagctataagtgcttaaaatttagtttggtaagatccctggtgcattgatatgtcaaagccttctgattatggagactggcaagtcccataatctgttgtctgcaagctggagaccaaggaaagttgatggtgtagtcccagtccaagtctaaaagtctgagaaccaggtaagccaatggtgaaagttctagtccaagtctagtcagaaatacaattcctgggttaaagcaagcaaagctgcttttctaataactcccattttctatgcataccctgggtccagcattccatcttccaggtatggttagaaaagagatcagaccttagtgactgctggtgaagtgaattgcatgctgcagcccctcatcagcatctttgtacagctcagtttcgtgttttctgcagaatcaggagctgacaatcaaaatggcccctcactcacattcattggtcagactgggcttgtgataacaatttagactaatcactgacaagcagggatggggagcactgaagtcagctattggctgtgtcccggagcagttgggcattctgccactggatgctgcttttgtaatcttgtcatatgacaaagcattatgatgttcttttgttttccttggattggcttaagggctggtgagaagcaggaaatattctgccatgggaagtctactgacctgcaaaaatttatcaaaatacacagaagcaggaatggaaggtggaaaaattacaaactgtgataatcagctccaagagcatgtaggggtaaaaggaggtaggtaatacctctccttactcattgtaagagtcatggctgacactcctataacaaaagacaagttaacaagagaaaagcataacaaatttacttaatcaaagttttatgtgatatgagagccttcagaaatgaagacccaaagatccagggaaaactgtttttgtgcttaggttccatgaagaatgggcagctctgtagagatgtgtttggacaagagtatgatctaatggtaatagactgggttcaaattcttcttggactctctgtgtagcatttcttctttgcaagtatggggcaggattcctctggattaagggtcttcaaatgagaagggagaagggagagagtgaccttcctaagttttatggcttgctttggggaaagggcttctagtttctatcattgtcttgcggaagaggaattctagtttccatggttcactccaggggagaaagaagcatgaaagacaagagggcaggagaaggtcaaagagatctttcttcggaggcccttccaatgtctttcagttcaaagtactcagcacaccgaggcgctatactttgggcatcatgttctgagagccaacagctacagtgaagaagtatgagagcagtcactgagtagggagggagctttcaactaacttagaggagcagggcctgaccctagcaagcattcctggggcctcccgattgccatatggggcagtacttatgtgtgggacagtgatatgaggagctacactcaggaagcttcctgatctcaatttttattatgatttgtttctgatttgggatcttcctaactgaattaaagaacttatattaatttctagcttaattcaggcaggagttagtccaagtatcattcgacaaactttattaatcttttaaaagtgccttggctttgggtttagacctatttcaacctcacctccaccacttagtatctctacagtgttgggaaaaatcacctaacctctgtgaccctaagatattcctacataaaacctgggaataataaattatacctcacagaagattaaatgtgtttccttacaagcattatggtagaccagatatacacagaacaaaaagcctgtgtatcacaatgaaaaatgctatataatctgcaaaacatattttttaaatgcacagctgcatttataagagagtaaggaattccctgaagtccagaaatgacaggaaagtgaaaatccaccagaataagcatgtgttcatttgtgttggtgatctacatcactttctcatggactacattacattatgaaggagatggaagacaaagtctggggcctgcacgtggtacattgtatcatagaactcacataaaaccaggacccattcagaggttaaactggagaacaaactccttgcagacgtaaatgatggggctacacatgcctgtttttggctttggccctaagtaaagcagggaggaaaaaaagtcattgataatttctaatcttaagtggagaagcatgattgttttgggctgaaattctcactatccatgcggcaagaaaaaaaaaaaaaaacctcaagtagaaaatttcattttaagcaattctggcttggtagtgctcccatgcacctaacaaaagcaaataaaaacacccctcaaagggaaacactttttacatagttctcaaagaatttccaagtttgataaagttccaaggaatatcaggtcataatacaaaatcaaagaatacacacaaataaataagccacaatgtgcaaaagttgccagataataaacgataagccagagcaacaaaactgcagatattgtaattgaatagagaataaaaaagaatgtatttagtacactttgggaggccgaggcaggtgt

SEQ ID NO: 18070 - RNA, 4419 nt, Homo sapiens
  source 1..4419: mol_type = other RNA
tctgggcaacaaagtgagacctacaaaaaaacaaaaataaaataaaaataaagcaaagtttgactgtttaaagggtaatttaagtatgagaaactggtgattggaaatcactgccaaaaagggaagtcttcccagagccttgctgctcacagtgtggtctgaagctgagatcccccgggaggttgtaagaaaggtaacatcccagcttatctgaatccagatctgcattttaaaaagatctccagatgtttgtgtccatatgtacattaaaggttgagaagtccggctctggagagttccttcacttgctttctgaagtgatggactccttggattgggcctgttctgaccaaccaactgagcacaggtctgccagttccttcacgtagtcagttggagcataaccagcacatgctggggacaagctgcacatgtgcagacaagagtggggaaatccccactcttaccacttcaagaaagccactttctgaaaatttcaagattctactctagtaatagctttgactgggaaggagatgtggtatctaccctggagtctgtgggcaagacaggtggtcatgatctgggttaggtgagagactgtaactatgttgattctggggatttcctaaggactagcagcactagctttaactgctttagtaagcgaaatcttatgtctgcaatccgaggtcatgggaaatctctttctggacctgagggaatcctatctccctaaggtcttctactagatgcagatccaggtaggactggcattctactccccaagtttcacctgaacctagctattctgttttttcttctttttcttttattctttttttttttttttttttttttttttttttttttgagacggagttttgctctttcgcccaggctggagtgtagtggcccgatcttggctcactgcaacctccgccttccggtttcaagcaattctgcctcggcttcccgagtagctgggattacaggcgcctgccaccacgcccggctaatttttgtgtttttagtacaggcggggtttcatcatgttggccaggctagtctcgaactcttgacctcatgatccacccgcctcagcctcccaaaatgctgggattacaggtgtgagccaccgcgcccggccacctagctgttctttatcaagtgactgtagtcatcatcccacctgcctgcttgtatttatttaaatatctgcattaattactgttaactaacttatttatacatataagaagtattcagagtaactttcaaaaacacatatgagataaattattaagtgaggaaaccttggcaattggagtatttgttttaagagggcaatagtattataatgaaaacctcctgacctgtggctctggggttcatgtttcttcttatcgaggtctcaggccttccagtccaatatattttgctccaaattttacttcaaggagagatcaagtatcaaatacctcatcaaattggagactttagggagtaaggcttaggaaaaatcaagagaatcaagggacccaattttcagtgggttttataatcataaagccacatgagtagttgactatcttcctgaataaattgttccatgttatcattaaatgtctcagcctggccagctctcgcattggtaaagcattggtggggatggaatatccctgagagatccatattcagagctctttcacaagtccagaaatgttcagtgtgcttttctgcttgtccaacactttcttgagcaattgatatcttctgaagctgacacatgacagggtggaagtatgtttcatctcagagggagaatcttgagctataagtgcttaaaatttagtttggtaagatccctggtgcattgatatgtcaaagccttctgattatggagactggcaagtcccataatctgttgtctgcaagctggagaccaaggaaagttgatggtgtagtcccagtccaagtctaaaagtctgagaaccaggtaagccaatggtgaaagttctagtccaagtctagtcctgggtccagcattccatcttccaggtatggttagaaaagagatcagaccttagtgactgctggtgaagtgaattgcatgctgcagcccctcatcagcatctttgtacagctcagtttcgtgttttctgcagaatcaggagctgacaatcaaaatggcccctcactcacattcattggtcagactgggcttgtgataacaatttagactaatcactgacaagcagggatggggagcactgaagtcagctattggctgtgtcccggagcagttgggcattctgccactggatgctgcttttgtaatcttgtcatatgacaaagcattatgatgttcttttgttttccttggattggcttaagggctggtgagaagcaggaaatattctgccatgggaagtctactgacctgcaaaaatttatcaaaatacacagaagcaggaatggaaggtggaaaaattacaaactgtgataatcagctccaagagcatgtaggggtaaaaggaggtaggtaatacctctccttactcattgtaagagtcatggctgacactcctataacaaaagacaagttaacaagagaaaagcataacaaatttacttaatcaaagttttatgtgatatgagagccttcagaaatgaagacccaaagatccagggaaaactgtttttgtgcttaggttccatgaagaatgggcagctctgtagagatgtgtttggacaagagtatgatctaatggtaatagactgggttcaaattcttcttggactctctgtgtagcatttcttctttgcaagtatggggcaggattcctctggattaagggtcttcaaatgagaagggagaagggagagagtgaccttcctaagttttatggcttgctttggggaaagggcttctagtttctatcattgtcttgcggaagaggaattctagtttccatggttcactccaggggagaaagaagcatgaaagacaagagggcaggagaaggtcaaagagatctttcttcggaggcccttccaatgtctttcagttcaaagtactcagcacaccgaggcgctatactttgggcatcatgttctgagagccaacagctacagtgaagaagtatgagagcagtcactgagtagggagggagctttcaactaacttagaggagcagggcctgaccctagcaagcattcctggggcctcccgattgccatatggggcagtacttatgtgtgggacagtgatatgaggagctacactcaggaagcttcctgatctcaatttttattatgatttgtttctgatttgggatcttcctaactgaattaaagaacttatattaatttctagcttaattcaggcaggagttagtccaagtatcattcgacaaactttattaatcttttaaaagtgccttggctttgggtttagacctatttcaacctcacctccaccacttagtatctctacagtgttgggaaaaatcacctaacctctgtgaccctaagatattcctacataaaacctgggaataataaattatacctcacagaagattaaatgtgtttccttacaagcattatggtagaccagatatacacagaacaaaaagcctgtgtatcacaatgaaaaatgctatataatctgcaaaacatattttttaaatgcacagctgcatttataagagagtaaggaattccctgaagtccagaaatgacaggaaagtgaaaatccaccagaataagcatgtgttcatttgtgttggtgatctacatcactttctcatggactacattacattatgaaggagatggaagacaaagtctggggcctgcacgtggtacattgtatcatagaactcacataaaaccaggacccattcagaggttaaactggagaacaaactccttgcagacgtaaatgatggggctacacatgcctgtttttggctttggccctaagtaaagcagggaggaaaaaaagtcattgataatttctaatcttaagtggagaagcatgattgttttgggctgaaattctcactatccatgcggcaagaaaaaaaaaaaaaaacctcaagtagaaaatttcattttaagcaattctggcttggtagtgctcccatgcacctaacaaaagcaaataaaaacacccctcaaagggaaacactttttacatagttctcaaagaatttccaagtttgataaagttccaaggaatatcaggtcataatacaaaatcaaagaatacacacaaataaataagccacaatgtgcaaaagttgccagataataaacgataagccagagcaacaaaactgcagatattgtaattgaatagagaataaaaaagaatgtatttagtacactttgggaggccgaggcaggtgt

SEQ ID NO: 18071 - RNA, 4369 nt, Homo sapiens
  source 1..4369: mol_type = other RNA
tctgggcaacaaagtgagacctacaaaaaaacaaaaataaaataaaaataaagcaaagtttgactgtttaaagggtaatttaagtatgagaaactggtgattggaaatcactgccaaaaagggaagtcttcccagagccttgctgctcacagtgtggtctgaagctgagatcccccgggaggttgtaagaaaggtaacatcccagcttatctgaatccagatctgcattttaaaaagatctccagatgtttgtgtccatatgtacattaaaggttgagaagtccggctctggagagttccttcacttgctttctgaagtgatggactccttggattgggcctgttctgaccaaccaactgagcacaggtctgccagttccttcacgtagtcagttggagcataaccagcacatgctggggacaagctgcacatgtgcagacaagagtggggaaatccccactcttaccacttcaagaaagccactttctgaaaatttcaagattctactctagtaatagctttgactgggaaggagatgtggtatctaccctggagtctgtgggcaagacaggtggtcatgatctgggttaggtgagagactgtaactatgttgattctggggatttcctaaggactagcagcactagctttaactgctttagtaagcgaaatcttatgtctgcaatccgaggtcatgggaaatctctttctggacctgagggaatcctatctccctaaggtcttctactagatgcagatccaggtaggactggcattctactccccaagtttcacctgaacctagctattctgttttttcttctttttcttttattctttttttttttttttttttttttttttttttttttgagacggagttttgctctttcgcccaggctggagtgtagtggcccgatcttggctcactgcaacctccgccttccggtttcaagcaattctgcctcggcttcccgagtagctgggattacaggcgcctgccaccacgcccggctaatttttgtgtttttagtacaggcggggtttcatcatgttggccaggctagtctcgaactcttgacctcatgatccacccgcctcagcctcccaaaatgctgggattacaggtgtgagccaccgcgcccggccacctagctgttctttatcaagtgactgtagtcatcatcccacctgcctgcttgtatttatttaaatatctgcattaattactgttaactaacttatttatacatataagaagtattcagagtaactttcaaaaacacatatgagataaattattaagtgaggaaaccttggcaattggagtatttgttttaagagggcaatagtattataatgaaaacctcctgacctgtggctctggggttcatgtttcttcttatcgaggtctcaggccttccagtccaatatattttgctccaaattttacttcaaggagagatcaagtatcaaatacctcatcaaattggagactttagggagtaaggcttaggaaaaatcaagagaatcaagggacccaattttcagtgggttttataatcataaagccacatgagtagttgactatcttcctgaataaattgttccatgttatcattaaatgtctcagcctggccagctctcgcattggtaaagcattggtggggatggaatatccctgagagatccatattcagagctctttcacaagtccagaaatgttcagtgtgcttttctgcttgtccaacactttcttgagcaattgatatcttctgaagctgacacatgacagggtggaagtatgtttcatctcagagggagaatcttgagctataagtgcttaaaatttagtttggtaagatccctggtgcattgatatgtcaaagccttctgattatggagactggcaagtcccataatctgttgtctgcaagctggagaccaaggaaagttgatggtgtagtcccagtccaagtctaaaagtctgagaaccaggtaagccaatggtgaaagttctagtccaagtctagtcttagtgactgctggtgaagtgaattgcatgctgcagcccctcatcagcatctttgtacagctcagtttcgtgttttctgcagaatcaggagctgacaatcaaaatggcccctcactcacattcattggtcagactgggcttgtgataacaatttagactaatcactgacaagcagggatggggagcactgaagtcagctattggctgtgtcccggagcagttgggcattctgccactggatgctgcttttgtaatcttgtcatatgacaaagcattatgatgttcttttgttttccttggattggcttaagggctggtgagaagcaggaaatattctgccatgggaagtctactgacctgcaaaaatttatcaaaatacacagaagcaggaatggaaggtggaaaaattacaaactgtgataatcagctccaagagcatgtaggggtaaaaggaggtaggtaatacctctccttactcattgtaagagtcatggctgacactcctataacaaaagacaagttaacaagagaaaagcataacaaatttacttaatcaaagttttatgtgatatgagagccttcagaaatgaagacccaaagatccagggaaaactgtttttgtgcttaggttccatgaagaatgggcagctctgtagagatgtgtttggacaagagtatgatctaatggtaatagactgggttcaaattcttcttggactctctgtgtagcatttcttctttgcaagtatggggcaggattcctctggattaagggtcttcaaatgagaagggagaagggagagagtgaccttcctaagttttatggcttgctttggggaaagggcttctagtttctatcattgtcttgcggaagaggaattctagtttccatggttcactccaggggagaaagaagcatgaaagacaagagggcaggagaaggtcaaagagatctttcttcggaggcccttccaatgtctttcagttcaaagtactcagcacaccgaggcgctatactttgggcatcatgttctgagagccaacagctacagtgaagaagtatgagagcagtcactgagtagggagggagctttcaactaacttagaggagcagggcctgaccctagcaagcattcctggggcctcccgattgccatatggggcagtacttatgtgtgggacagtgatatgaggagctacactcaggaagcttcctgatctcaatttttattatgatttgtttctgatttgggatcttcctaactgaattaaagaacttatattaatttctagcttaattcaggcaggagttagtccaagtatcattcgacaaactttattaatcttttaaaagtgccttggctttgggtttagacctatttcaacctcacctccaccacttagtatctctacagtgttgggaaaaatcacctaacctctgtgaccctaagatattcctacataaaacctgggaataataaattatacctcacagaagattaaatgtgtttccttacaagcattatggtagaccagatatacacagaacaaaaagcctgtgtatcacaatgaaaaatgctatataatctgcaaaacatattttttaaatgcacagctgcatttataagagagtaaggaattccctgaagtccagaaatgacaggaaagtgaaaatccaccagaataagcatgtgttcatttgtgttggtgatctacatcactttctcatggactacattacattatgaaggagatggaagacaaagtctggggcctgcacgtggtacattgtatcatagaactcacataaaaccaggacccattcagaggttaaactggagaacaaactccttgcagacgtaaatgatggggctacacatgcctgtttttggctttggccctaagtaaagcagggaggaaaaaaagtcattgataatttctaatcttaagtggagaagcatgattgttttgggctgaaattctcactatccatgcggcaagaaaaaaaaaaaaaaacctcaagtagaaaatttcattttaagcaattctggcttggtagtgctcccatgcacctaacaaaagcaaataaaaacacccctcaaagggaaacactttttacatagttctcaaagaatttccaagtttgataaagttccaaggaatatcaggtcataatacaaaatcaaagaatacacacaaataaataagccacaatgtgcaaaagttgccagataataaacgataagccagagcaacaaaactgcagatattgtaattgaatagagaataaaaaagaatgtatttagtacactttgggaggccgaggcaggtgt

SEQ ID NO: 18072 - RNA, 117 nt, Homo sapiens
  source 1..117: mol_type = other RNA
tctgggcaacaaagtgagacctcaactcttttgatgcatccatcatcccttcagattctctcctgcaatgccagggaagactctatctctgatgcctggtgcttccacacagtcggt

SEQ ID NO: 18073 - RNA, 3224 nt, Homo sapiens
  source 1..3224: mol_type = other RNA
tctgggcaacaaagtgagacctcatctctacaaaaattagccaggcatggtggtatgggcctgtggtcccagcaacttgggaggctcagatgggaggatcgcttgagccctgggagggaaaggctgcggttagccatgatcacaccactgcactccaacctgggtgactgggtgaggccctttctcaccaaaaacaaacaaacaaacaaaaaacaaagacgtttgtatatatttttatttttttagaaacgaactcaaactcctgggctcagcctccctaagtagggagcctgggattacaggcatgagccattgtgctcagccctaaaatagttttgaagaatatttatacataggaaaaaatgctattttttatgcattataataattttgtaaataagaaatgtacgtgcaacaaatctacaaatatagtaaaatatagtgatgatctctctcaaaaaattgtgggaaagttgattttatattttttcctgaattgttggtgttttctacaataatgttttaaaattacagaaggcaaaagaaggcaaattcttaagatgtaaaatactcttaactcaaactacaaaacttcttcagtatcttacactaaattgaacctaaattaaacttacagttcattcaatcacagaatgtaaactccatgaaggtaacttgatttttcctgcttaatatactgttgtgcctctaatggctacatcagtacctggcacctgagtacttgttcaatgaaaggtgaagagaaaaatgaactggcagtgtatttccatcatactagcaagatgtttatttaaaaacatttaaaaactgttttttaaaaaacattctagttaagacgagataattcaatgttcaagctaataattctataccattttaagagtctgaatttacttttaagtaaaaaaaggcagagaaaaagagtgaaggatacagaattatcttgattatgcactgctgttactattcccatgctaaagaccccttttgtttcaataaaactatcaatatttactgagaatgacagctctgaatcaaaggcaagagaaagagacctgtaaatagtgctgttcatactagttgcccccagtagttcccaggcctcacttccaagctgccttaagtaatttttactttctgaatataaagccaactgtggaggggtcagacagctgaggactgaacttcttaaaaattggcttcagagaaaagcataacattacaactgaggcggccaagcacagtggctcacgtctgtaatctcagcactttgggaggctgacgcaggtggatcaccagatcaggagatagagaccatcctggctaacacagtgaaccccatctctactaaaaatacaaaaattacccgggcatggtggcatgcacctgcagtgccagctactcgggaggctgaggcaggagaattgcttgaacccgggaggcggacgttgcagtgagcagagatcgcgccactgcactccagcctgggtgacagagcaggacaccgtctcagaaaaaaaaaaaaaagttacaactgaggcatcaggtcttaaggtttaaaacagtctcataattgtcacattatcatattatgtcaactctgaaaataaatgcacactcatcccagagtctccaaaatctttatctttagaatccaaccttgttttaagaagtagtaaaatgaaggagcattgttagtagtcacctgacaaaagctgtccattattcttgacattaaaaattgaatgcaatgatttaaaaaacataatacattaacatttacataatatatttagaatcacatggtttccagtgattagatttcagtcatgcctggaaaggagaagacagtggctaggagcacattccttataaaggatacataaatggtatacttaggatgactaatattaagaatttaaacacggtgcatttttttcctcaaaggaagcaattttagtttctaaagagcatttacttctgacatctcgattcctgatttcagtggctgcagactgtgtacttctgtgccacacttaggacaagtaaagtacacgtcaaataagaaactactcttagcacagaaataacagaaaatatgctcacatcctatggtgtgaggcatggtgggccactctccacatagagcgcattctttgccactggtggctaatgtattgtcactattaggtgcaccagtaagaggaatacaccatgaagacagcttggctttcaacttctggacattgataagtggtaagagaaaaatcagaaattcagcaaaaccatgccagagaagttccctattcatgtattcaaagccaacttcacatatgttttgaggcttgcaaaatacagaatgaatacctaggagacgttctgtcaaagttgcaaactttcccctctgaaggaaaatcaaaaaattaatcagcccacctaatttcaaaagtccaatcacaaaattcacacactgcttgactttcccaaatgatgctaaatgatggtttcgaaacaaatcatagcatcgttcttctaaccacctgccaccaattgtacaaacagcataccagattttttgatttttactgggtggctgatatctcaggttaggggaaaaatcatttttgtacttaatattcaaaactgactgtcccactgtggcatttttggagtagatggtgaatctccacaagaaaacccataagcacgctttcacctctggctcaaagcgagctaacagcccaggtttaaatccatgaaagcactgagtaaactgggaccaaactagctgctccagggccttgtttagttcaagtgcatccaactggcttattcttagcactctgtttgcactcttcgcattctcttttctggaagccatgtcttctctgaaggtctcttaggagtctgcgaaacgcccacgctccacgtaactttctctgaaacattctctggaaagcttgtcttttcctagccgaatctggattaccaaggcttccggaactcgcaggcttccggagcgacgcaggagccggaagtggcaggcagtgacatgtagccgttgaggatcgccactgccttctcgttctgtggtatgaatggcagtgtctctctagagagttagtgcttaagtttgaatgatggcaggcacttcaggattccagcacgtagtagggtttaagaacgtcttagttcttacctcc

SEQ ID NO: 18074 - RNA, 3150 nt, Homo sapiens
  source 1..3150: mol_type = other RNA
tctgggcaacaaagtgagacctcatctctacaaaaattagccaggcatggtggtatgggcctgtggtcccagcaacttgggaggctcagatgggaggatcgcttgagccctgggagggaaaggctgcggttagccatgatcacaccactgcactccaacctgggtgactgggtgaggccctttctcaccaaaaacaaacaaacaaacaaaaaacaaagacgtttgtatatatttttatttttttagaaacgaactcaaactcctgggctcagcctccctaagtagggagcctgggattacaggcatgagccattgtgctcagccctaaaatagttttgaagaatatttatacataggaaaaaatgctattttttatgcattataataattttgtaaataagaaatgtacgtgcaacaaatctacaaatatagtaaaatatagtgatgatctctctcaaaaaattgtgggaaagttgattttatattttttcctgaattgttggtgttttctacaataatgttttaaaattacagaaggcaaaagaaggcaaattcttaagatgtaaaatactcttaactcaaactacaaaacttcttcagtatcttacactaaattgaacctaaattaaacttacagttcattcaatcacagaatgtaaactccatgaaggtaacttgatttttcctgcttaatatactgttgtgcctctaatggctacatcagtacctggcacctgagtacttgttcaatgaaaggtgaagagaaaaatgaactggcagtgtatttccatcatactagcaagatgtttatttaaaaacatttaaaaactgttttttaaaaaacattctagttaagacgagataattcaatgttcaagctaataattctataccattttaagagtctgaatttacttttaagtaaaaaaaggcagagaaaaagagtgaaggatacagaattatcttgattatgcactgctgttactattcccatgctaaagaccccttttgtttcaataaaactatcaatatttactgagaatgacagctctgaatcaaaggcaagagaaagagacctgtaaatagtgctgttcatactagttgcccccagtagttcccaggcctcacttccaagctgccttaagtaatttttactttctgaatataaagccaactgtggaggggtcagacagctgaggactgaacttcttaaaaattggcttcagagaaaagcataacattacaactgaggcggccaagcacagtggctcacgtctgtaatctcagcactttgggaggctgacgcaggtggatcaccagatcaggagatagagaccatcctggctaacacagtgaaccccatctctactaaaaatacaaaaattacccgggcatggtggcatgcacctgcagtgccagctactcgggaggctgaggcaggagaattgcttgaacccgggaggcggacgttgcagtgagcagagatcgcgccactgcactccagcctgggtgacagagcaggacaccgtctcagaaaaaaaaaaaaaagttacaactgaggcatcaggtcttaaggtttaaaacagtctcataattgtcacattatcatattatgtcaactctgaaaataaatgcacactcatcccagagtctccaaaatctttatctttagaatccaaccttgttttaagaagtagtaaaatgaaggagcattgttagtagtcacctgacaaaagctgtccattattcttgacattaaaaattgaatgcaatgatttaaaaaacataatacattaacatttacataatatatttagaatcacatggtttccagtgattagatttcagtcatgcctggaaaggagaagacagtggctaggagcacattccttataaaggatacataaatggtatacttaggatgactaatattaagaatttaaacacggtgcatttttttcctcaaaggaagcaattttagtttctaaagagcatttacttctgacatctcgattcctgatttcagtggctgcagactgtgtacttctgtgccacacttaggacaagtaaagtacacgtcaaataagaaactactcttagcacagaaataacagaaaatatgctcacatcctatggtgtgaggcatggtgggccactctccacatagagcgcattctttgccactggtggctaatgtattgtcactattaggtgcaccagtaagaggaatacaccatgaagacagcttggctttcaacttctggacattgataagtggtaagagaaaaatcagaaattcagcaaaaccatgccagagaagttccctattcatgtattcaaagccaacttcacatatgttttgaggcttgcaaaatacagaatgaatacctaggagacgttctgtcaaagttgcaaactttcccctctgaaggaaaatcaaaaaattaatcagcccacctaatttcaaaagtccaatcacaaaattcacacactgcttgactttcccaaatgatgctaaatgatggtttcgaaacaaatcatagcatcgttcttctaaccacctgccaccaattgtacaaacagcataccagattttttgatttttactgggtggctgatatctcaggttaggggaaaaatcatttttgtacttaatattcaaaactgactgtcccactgtggcatttttggagtagatggtgaatctccacaagaaaacccataagcacgctttcacctctggctcaaagcgagctaacagcccaggtttaaatccatgaaagcactgagtaaactgggaccaaactagctgctccagggccttgtttagttcaagtgcatccaactggcttattcttagcactctgtttgcactcttcgcattctcttttctggaagccatgtcttctctgaaggtctctttttcctgttcctgcagctccctcaagactggacagcctatagctatgacagtgggaatttttgctccaagttcttctgtgaaatccttgcctcatacttgccagaagctcagagacactgcaggttaggttccagaccacttaggagtctgcgaaacgcccacgctccacgtaactttctctgaaacattctctggaaagcttgtcttttcctagccgaatctggatt

SEQ ID NO: 18075 - RNA, 3366 nt, Homo sapiens
  source 1..3366: mol_type = other RNA
tctgggcaacaaagtgagacctcatctctacaaaaattagccaggcatggtggtatgggcctgtggtcccagcaacttgggaggctcagatgggaggatcgcttgagccctgggagggaaaggctgcggttagccatgatcacaccactgcactccaacctgggtgactgggtgaggccctttctcaccaaaaacaaacaaacaaacaaaaaacaaagacgtttgtatatatttttatttttttagaaacgaactcaaactcctgggctcagcctccctaagtagggagcctgggattacaggcatgagccattgtgctcagccctaaaatagttttgaagaatatttatacataggaaaaaatgctattttttatgcattataataattttgtaaataagaaatgtacgtgcaacaaatctacaaatatagtaaaatatagtgatgatctctctcaaaaaattgtgggaaagttgattttatattttttcctgaattgttggtgttttctacaataatgttttaaaattacagaaggcaaaagaaggcaaattcttaagatgtaaaatactcttaactcaaactacaaaacttcttcagtatcttacactaaattgaacctaaattaaacttacagttcattcaatcacagaatgtaaactccatgaaggtaacttgatttttcctgcttaatatactgttgtgcctctaatggctacatcagtacctggcacctgagtacttgttcaatgaaaggtgaagagaaaaatgaactggcagtgtatttccatcatactagcaagatgtttatttaaaaacatttaaaaactgttttttaaaaaacattctagttaagacgagataattcaatgttcaagctaataattctataccattttaagagtctgaatttacttttaagtaaaaaaaggcagagaaaaagagtgaaggatacagaattatcttgattatgcactgctgttactattcccatgctaaagaccccttttgtttcaataaaactatcaatatttactgagaatgacagctctgaatcaaaggcaagagaaagagacctgtaaatagtgctgttcatactagttgcccccagtagttcccaggcctcacttccaagctgccttaagtaatttttactttctgaatataaagccaactgtggaggggtcagacagctgaggactgaacttcttaaaaattggcttcagagaaaagcataacattacaactgaggcggccaagcacagtggctcacgtctgtaatctcagcactttgggaggctgacgcaggtggatcaccagatcaggagatagagaccatcctggctaacacagtgaaccccatctctactaaaaatacaaaaattacccgggcatggtggcatgcacctgcagtgccagctactcgggaggctgaggcaggagaattgcttgaacccgggaggcggacgttgcagtgagcagagatcgcgccactgcactccagcctgggtgacagagcaggacaccgtctcagaaaaaaaaaaaaaagttacaactgaggcatcaggtcttaaggtttaaaacagtctcataattgtcacattatcatattatgtcaactctgaaaataaatgcacactcatcccagagtctccaaaatctttatctttagaatccaaccttgttttaagaagtagtaaaatgaaggagcattgttagtagtcacctgacaaaagctgtccattattcttgacattaaaaattgaatgcaatgatttaaaaaacataatacattaacatttacataatatatttagaatcacatggtttccagtgattagatttcagtcatgcctggaaaggagaagacagtggctaggagcacattccttataaaggatacataaatggtatacttaggatgactaatattaagaatttaaacacggtgcatttttttcctcaaaggaagcaattttagtttctaaagagcatttacttctgacatctcgattcctgatttcagtggctgcagactgtgtacttctgtgccacacttaggacaagtaaagtacacgtcaaataagaaactactcttagcacagaaataacagaaaatatgctcacatcctatggtgtgaggcatggtgggccactctccacatagagcgcattctttgccactggtggctaatgtattgtcactattaggtgcaccagtaagaggaatacaccatgaagacagcttggctttcaacttctggacattgataagtggtaagagaaaaatcagaaattcagcaaaaccatgccagagaagttccctattcatgtattcaaagccaacttcacatatgttttgaggcttgcaaaatacagaatgaatacctaggagacgttctgtcaaagttgcaaactttcccctctgaaggaaaatcaaaaaattaatcagcccacctaatttcaaaagtccaatcacaaaattcacacactgcttgactttcccaaatgatgctaaatgatggtttcgaaacaaatcatagcatcgttcttctaaccacctgccaccaattgtacaaacagcataccagattttttgatttttactgggtggctgatatctcaggttaggggaaaaatcatttttgtacttaatattcaaaactgactgtcccactgtggcatttttggagtagatggtgaatctccacaagaaaacccataagcacgctttcacctctggctcaaagcgagctaacagcccaggtttaaatccatgaaagcactgagtaaactgggaccaaactagctgctccagggccttgtttagttcaagtgcatccaactggcttattcttagcactctgtttgcactcttcgcattctcttttctggaagccatgtcttctctgaaggtctctttttcctgttcctgcagctccctcaagactggacagcctatagctatgacagtgggaatttttgctccaagttcttctgtgaaatccttgcctcatacttgccagaagctcagagacactgcaggttaggttccagaccacttaggagtctgcgaaacgcccacgctccacgtaactttctctgaaacattctctggaaagcttgtcttttcctagccgaatctggattaccaaggcttccggaactcgcaggcttccggagcgacgcaggagccggaagtggcaggcagtgacatgtagccgttgaggatcgccactgccttctcgttctgtggtatgaatggcagtgtctctctagagagttagtgcttaagtttgaatgatggcaggcacttcaggattccagcacgtagtagggtttaagaacgtcttagttcttacctcc

SEQ ID NO: 18076 - RNA, 3118 nt, Homo sapiens
  source 1..3118: mol_type = other RNA
tctgggcaacaaagtgagacctcatctctacaaaaattagccaggcatggtggtatgggcctgtggtcccagcaacttgggaggctcagatgggaggatcgcttgagccctgggagggaaaggctgcggttagccatgatcacaccactgcactccaacctgggtgactgggtgaggccctttctcaccaaaaacaaacaaacaaacaaaaaacaaagacgtttgtatatatttttatttttttagaaacgaactcaaactcctgggctcagcctccctaagtagggagcctgggattacaggcatgagccattgtgctcagccctaaaatagttttgaagaatatttatacataggaaaaaatgctattttttatgcattataataattttgtaaataagaaatgtacgtgcaacaaatctacaaatatagtaaaatatagtgatgatctctctcaaaaaattgtgggaaagttgattttatattttttcctgaattgttggtgttttctacaataatgttttaaaattacagaaggcaaaagaaggcaaattcttaagatgtaaaatactcttaactcaaactacaaaacttcttcagtatcttacactaaattgaacctaaattaaacttacagttcattcaatcacagaatgtaaactccatgaaggtaacttgatttttcctgcttaatatactgttgtgcctctaatggctacatcagtacctggcacctgagtacttgttcaatgaaaggtgaagagaaaaatgaactggcagtgtatttccatcatactagcaagatgtttatttaaaaacatttaaaaactgttttttaaaaaacattctagttaagacgagataattcaatgttcaagctaataattctataccattttaagagtctgaatttacttttaagtaaaaaaaggcagagaaaaagagtgaaggatacagaattatcttgattatgcactgctgttactattcccatgctaaagaccccttttgtttcaataaaactatcaatatttactgagaatgacagctctgaatcaaaggcaagagaaagagacctgtaaatagtgctgttcatactagttgcccccagtagttcccaggcctcacttccaagctgccttaagtaatttttactttctgaatataaagccaactgtggaggggtcagacagctgaggactgaacttcttaaaaattggcttcagagaaaagcataacattacaactgaggcggccaagcacagtggctcacgtctgtaatctcagcactttgggaggctgacgcaggtggatcaccagatcaggagatagagaccatcctggctaacacagtgaaccccatctctactaaaaatacaaaaattacccgggcatggtggcatgcacctgcagtgccagctactcgggaggctgaggcaggagaattgcttgaacccgggaggcggacgttgcagtgagcagagatcgcgccactgcactccagcctgggtgacagagcaggacaccgtctcagaaaaaaaaaaaaaagttacaactgaggcatcaggtcttaaggtttaaaacagtctcataattgtcacattatcatattatgtcaactctgaaaataaatgcacactcatcccagagtctccaaaatctttatctttagaatccaaccttgttttaagaagtagtaaaatgaaggagcattgttagtagtcacctgacaaaagctgtccattattcttgacattaaaaattgaatgcaatgatttaaaaaacataatacattaacatttacataatatatttagaatcacatggtttccagtgattagatttcagtcatgcctggaaaggagaagacagtggctaggagcacattccttataaaggatacataaatggtatacttaggatgactaatattaagaatttaaacacggtgcatttttttcctcaaaggaagcaattttagtttctaaagagcatttacttctgacatctcgattcctgatttcagtggctgcagactgtgtacttctgtgccacacttaggacaagtaaagtacacgtcaaataagaaactactcttagcacagaaataacagaaaatatgctcacatcctatggtgtgaggcatggtgggccactctccacatagagcgcattctttgccactggtggctaatgtattgtcactattaggtgcaccagtaagaggaatacaccatgaagacagcttggctttcaacttctggacattgataagtggtaagagaaaaatcagaaattcagcaaaaccatgccagagaagttccctattcatgtattcaaagccaacttcacatatgttttgaggcttgcaaaatacagaatgaatacctaggagacgttctgtcaaagttgcaaactttcccctctgaaggaaaatcaaaaaattaatcagcccacctaatttcaaaagtccaatcacaaaattcacacactgcttgactttcccaaatgatgctaaatgatggtttcgaaacaaatcatagcatcgttcttctaaccacctgccaccaattgtacaaacagcataccagattttttgatttttactgggtggctgatatctcaggttaggggaaaaatcatttttgtacttaatattcaaaactgactgtcccactgtggcatttttggagtagatggtgaatctccacaagaaaacccataagcacgctttcacctctggctcaaagcgagctaacagcccaggtttaaatccatgaaagcactgagtaaactgggaccaaactagctgctccagggccttgtttagttcaagtgcatccaactggcttattcttagcactctgtttgcactcttcgcattctcttttctggaagccatgtcttctctgaaggtctctttttcctgttcctgcagctccctcaagactggacagcctatagctatgacagtgggaatttttgctccaagttcttctgtgaaatccttgcctcatacttgccagaagcttaggagtctgcgaaacgcccacgctccacgtaactttctctgaaacattctctggaaagcttgtcttttcctagccgaatctggatt

SEQ ID NO: 18077 - RNA, 192 nt, Homo sapiens
  source 1..192: mol_type = other RNA
tctgggcaacaaagtgagacctcgtctctaccaaaataaaaacaaaaaaattagccaggcattttggtgcccgcctgtggccccagctaaacagaagcctgaggcaagaggatcgcttgagcccagaaggtcaagggtgcagtgagccatgttcatgcccctgcaccccagcctgggcaacagagtaaaacc

SEQ ID NO: 18078 - RNA, 6527 nt, Homo sapiens
  source 1..6527: mol_type = other RNA
tctgggcaacaaagtgagaccttgtgtcttaaaaaaacaaaaaccactaaaatagcaacaagagcagtttacttggcttggaggtcaaagctgcatttgataaattcccagagtggtcagggggagaacagatattcaggaacactggggtttgggagtttttttcgcttctttcttacacccataaagccacctatccattcattcattttattctcttgcctatagcaaaactgaaagggccattaaactccagtttaaattttattcccaagatcctctaaatagcagcagctctcaaatcccagctccagcttagtggcttgctagcagtgacactgtgaaaaaaaatctagctggcagaacctcggtttctccatttgtgaaatgaaagtactggatgataatcctggctctgccaatttcctgggctttcacctgcttcttgcacttgaagatggtctctgatatcgtcccagttgggctggaatgtcctgggttttgcgttaggtttttggcatgtccagcatttgcggaaaaagaagatgtcctaactatcttcagaaggcacaaaactaggggtttttcttgtttttggtttcgagacggagtctcactctgtcgcccaggctggagtgcagtgacgcaatctcggctcactgcaacctctgcctcctgggttcaagcgattctcctgcctcagcctcccgagtagctgacttcaggtgatccgcccacctcagcctcccaaagtggcgtgagccactgcacccagcccaaactaggttttgaaggtggaataagttctcctagctcagaaggatctcaacctcttgcaagttacttttcacttttaagggcccttaaagaagcatttgcttagctctgtatccaggccatctctccctccccgaagagcaacagaccagcaactgacattaaggtcacatgggtgggtggggagtagaattgcgggggtgacagttccagccaatccagacaacgaatcattgtttggaggaaccagagcctcaaagggtgagtgcactgactagggctggctctccatctgttcacacacttgttgagtgcctactctatgccaaagcactgtgttttggtgccctggggaacacaaaattgggatagctcctgccctcagggcttaataaagtagctctcagtcaagggttagagcaagggttgacaaactacagcccaaaagggccacccgtttgtgtaaataaagttttattggaacaccagccacactcattcgtgttcatgtagtgtctgtggcagcttttacattacaacagcagggctgagcatttgcagcagaggctatatggcctgcaaagcctaaaatcttcactttctacccctttacaaaaaagtttgccaattcctgctagagaagagatgacatacaactaagaacttaaacgagtgatcagggaacacaaattatttacataataaaatttcagagagggggggctggctgaatttaaaaagcatgaattacgtgaggcttgattactgtgaagagataagtcaacttaaagttacttacatttaacatacaatttatatgcactggtttaaaacacgcacacacacacacaaaatgtaacacaagccaactactgatctggtacagatgacaaaagggtgatcagttccaacttcaaaaggaaaactggctatgatgagtccatattgaaaaagtcactgtcatttatgggtggtccaagggatttttttcaagggtaattttacctgcttcattgttcatttaagggtacacactgaactttggaactaacgcttgcatgggtttgtgcctccaaagcagtcaacactgaagtcttggctgggctcagtggctcctgcctgtaatcccagcgctttgggagactgaggcgggaggctcacttaagtccaggagttcgagaccagcctgggcaacacagtgagaccccatctctatttcaaaaattataaaataataaaaagaaaataatctctctgcataagcaacaacaacaaaccccactaaggtgttgaaggacccattttaatgaatagttaagaatggtttgtatgttatactctgcttttttatgttttgacttttaaacaaagaaaaataggctgcttttgcatttagggttgatcaaagcagtctgtcttttttttgttgttttggtagagacagggtctcgccatgtttacccaggctggtcttgaagtcctgagctcaagcaatcctcccaccttggccctcctcaaagtgctgagattacaggcgggagccaccgcacctagcatctttgctatttgaaacatcaaatgaaatcatactaatgtgagagctgaattccattgaaaggaaaagctcattaaataacaatcgccattgtctggccatggggagactactagaattaatgagtgtttatagttcttgccctctcatcctcaaacatcttagataaaatcccaagagactgctgctgaaagcgtcctgctgtaaattacaagaaaatcagcccagcttcaagcagaaaatgccaaggaccagggctggggagcagatttcacgtaagaacatccagacactaagaaaacaccaaggaatactgtataagagacattgcagtcacgttgtgggagctgccactgagatgcagagtgtgggtctgcttggagaaaaggctctcacattccaagccgctgtccttacgtgtaaaagctttgaggtgcaccctcttccacactagctgatgtaggagttagaggtagtaaacgtgtgcatacaaaactcaaacctgttttgaaaagcccaccgtagaaagcatgcttaaaagatggaattcggctgtatgccagaaaatcagtagcattatggaaggaaattgaactagaagtttaaaaaacagccaacatgcaggcccttccccacagtagaagggagcctgggtattgtgcaatctcacacccactgaaaaaatgccacgcatgcctctaaatgctctgagaaagaatgctttgcactaagccacggcaatacacgccccgtgacttaggaaagccagcgtgaagtgcttcatttctcatcccgatgcacaaaacacagggctccatgggcccgacatttcagtccagcctgaaaagactagtgagcacagccctaaaattgtccattcaaggcaaaaagcactttcttatatctcgtgacaaaaaaaaaaaaagaaataaaaatgaaaatagaaccacaaaatgggcaggcatggtggctcacacctgtaatcccagcactttgggaggctgaggcaggtggatcacctgaggttaggagttcgagaccagcctggccaacatggtgaaaccccatctctactaaaaatgcaaaaattagctgagtgtggtggtgtgcaccagtaatcccagctacttgggaggctgaggcaggagaatcacttgaacccaggaggcggaggttgcagtgagctaagatcatgtcactgcactccagcctgggtgacagagcaagactctgtctcaaaacaaacaaacaaacaaacaaaaaaaaccacacacaaaacggtatgttggttcattaggctgcttcttcaagccccacttccccaaaatactgccctaagagacagctatagagtctctgctggtagctgccaaggagcaaagacatttttcaagagtcaaaaaatgaaatataaaatttgattttacaacacacttaaaaatgcttcccctccccaaactaaataagttgttgttgttgtttttttaatctttcctcctagcccgtttgcttgggactagccggcagtgattttcctggttactcctccatctgggcccaggcctcttcagccttttggtagtactggttggccagtcggcccttcatggcttccatcgctgcctctgctgcctgggtatacaagtcccctgatctctgcgggtccttctccagcccgtagcctcctgtgaacagcatctcggcctccctggccagcatcatgtaccggggctcgtcctgcattccgtcgtactcaccgccctcatcacagtccgtcatctccagggcagtgttgtaccagtgcagggcctctagccagtcttggcacctgtccgggctgaggttctggccagagtcaaaagctcgcgccactaggatcatggactgcctgtcgccagcttcagcggcctttagtaagtaatcaaatcctttggttttgttctcttctgtctccttcagagagacatcggctaggatgtgatgaggcaactgcgagtacatgagtcccaggcccacgatggcctccagctcgcccaggttggctgcgtgctccaggtggaagacagccgactcctggtcccactcctcgcccttctcgcagaagcgcccaccctcgtggtagcgcaccatggccagatggaccttccccaaaatggacttcccgattttcttttcgaggtccagagcattaagcctttgcacttccagggccacggccgaagccctcggcaggtggaggcgggaggagttgaggagattccacttctctacacatacccgtccagagctgcccaggctgtcttcgtcagactcgtacttccgattactgtatgagtggccatgttctcggggctcagggtcatccagctcaccccgcttctcactggggtatccgctgtccccactattctcagactcccggtggttgtctagatgatcatggtctctggatgccatgttatcgaggtcactgaacactggccaatggaggtggtctagcttctggctgtgtggtgtggccgaagatggggaagaagggagagagtcgaaggtcacgtcgctcatgttctcgtctccagagttctctgaaaggggacggagcaggggtggccggctcccagagagggtccttacttgggggctcccacatttttcctctgttcctctcaagatggtcttggctgattgcagcagcttggtgttctgattcactgcatccctctcccggggcgagaggtcaaagggagcaaggcccatgctctcgcaaatccggttgcaggcatgagagtagaagaagagcgccatcccgcggacacctaggttgccgtctccaaagtcagtgcccgtctccgtgtggatctgtgggtcagtgtagagatccccaactccctggatgtccaccactatcagctgatggccggaacgctcaaaagtgaagtggctgaaggcctgcggcgtcaggcggatgttgtcatcgcggacaaagccagagttggagttgtacttgatgtacttgccctcgatgtagtgctccaggtggaagaggggcttgcccggtctgtccttcagctcgatgatgcacatctgcatgatgtccacctgcttggggggcttgtgccgattatactcctccccccagagcttggcctccatctgtagacgcacgtcctcaaagtacacatcccggtctacgggctcgatgtagcgcttcgccacgtagttggaggcgcccttccactgctgggcatgcaagaagttggagagcttcttcgtccggaagcactccctcattgctcctcggccgaagggctgagatgccatcttgatcagaacttcatcatccagccattccccggtgacggcgttgtacctgtgtcgagtagcacgttcggtggcaatatcttccaggtggaactcagcccaggggtcgggcatgtgcttggccttctggattgcgtgcttccaggcttccttgaagtggaaggagtttgccggggacccgctggagctataccgctcactttttgttaggttgctgtagtacttattaaccttggaattgacattctggttcgagcttgggtcatccgtgatggggcagatgaagtaaccttcctcatcgtcgctgtccccatcagaatcaccatcatggccagctcggggggactggccgccatcaacgccttccaggcggaagatgagatcttcgtctgccatgttcctggggtgcccgttttacccaagcagtatccggcacagccagagttactggacaaatgcagaggcgaaggtcctccctcgggcagacaggcgcggcagccgctgcccacggccgcgagggtccagaggagttggcagaggctcgcggcccggagctccagggtgcagggcgggcgggccccccgagagtgccggggagcggagagcggggagcgctagctggcgctccgggcaagcagctggggccacgcggggtagatggaccgatcccagggcgcgcggggcagtcggagtgatcccaggaagggcgcaggggccgttgggacgatcccgggatgtgggagcgcgtgccaggggggactcgcgtgcaggcgacagcgagcgggactcgggtggctgcagggccgggagtgcgggcgctcgatccaggaaggaggggagctgaggctgaagctggggctggtctaggttgagc

SEQ ID NO: 18079 - RNA, 1866 nt, Homo sapiens
  source 1..1866: mol_type = other RNA
tctgggcacaggcggatggacaggccggtgagcacatctgtgcgctgcatgagcagcaaagatttgccatcaatttcctgctcttggaaagctgtcgcctgctccgggaatccagcctcagtaaaatattcgacgacatccatcacggtccactcgacgggatcagatggcttctctttgcgcccgggaggacagccaaagggggtcccgtcggccccaggtagggctggtttgcctgggggcaaaggcacgggggacggggagtctggcccggtggcaacagaagctgttcccccttccttgttcatggctgccatggagaacacctggcgggtgccgctgcccggggctggcccccgcccttcatcctggccctggtgcggtccgcagggggtccactccttgaccctctccttggcactctgaggtccccgctcgccgttaagctggtggtgctgggcacctgcaggacggtcactctcgggcacttcagagccctctgacacatcatcttcttcatcttcatcttcatcatcatcttcttcctcttctttctcaagtactcgctcttctccacctctcttgctgcgagacgggcgggcgctggcggccggcggcgcccgtccgggcctgtccccgcggggcagcgcaagcgctccgagacgggtgcgctccagacggcctcgagccgccgcctcctcctccagcagcccctgcacgcggccgcgggttaggcgaccgccggcgccgccgctgcccccgaggtagcgcacgacttcccgcaggctcacgggccgcgccgcgccgccggcccgcaccgcgcccccctccggcggcggctgtggctgcggcggcggcggctgctgctgctgtggcggcgccggcggctgtggcggcggcggcagcggcggctcccgggcggcgacggcgggcgggggggcgcggcgcgggccggccgggggcgccaccgccgggggagcggctggcgcgggcggcggcgcggccaggggcgcggcccgctgcgcgcgggggcccggctgcgcggggccaggcgaggggggcgctgtggcggcggcggcggccgcgcggggcgcccgggccggggcggcggcggcgacgggcgcgggcggtggcggcggggcgggcgtgggcggcggcgcggcggcggcggcggcggcgggggccccgcggggggcgcgcggcggggccggcggggtggctccgcgccggggcggctggacgcgcgccgcgttgcggtacgagatgctccccttgtagctgacccggagcacggcgcgctgctggatcagtttctcgagctcggcgcgcgtgcgctccggctccgggccgtgccgccgccgcaccatccggcagatgcgctccaggtccggccgcgccttgcgcgagcgcagcgagtcgatggtgtccaggatccactcttggtagtgcggggaagcggcggacgacgaggcggcggccgccgtggtggcggccgccgccgtctccggcgggggtagggccgggggccccgccatgcctcccgcccggcccggctgcaccgtgcgcgctgcctccctcccagcgcggcgcccccctccccggctcccctccctccgccgctgcccgcctcctccgcctccccccccggggggcgcagcgcctcggcggagcggcggcggcgctgctgtttctttgcaaaaaaaaaaaaaaaaaaaagagagagagagggagagagagagagaggaaaaaacagtgagagagaaagaaaagagagaaaaaaatatgcacacactcactcactcgcacgcacgcacacacagacccgcttctgctgggcgcgcgcggggccggggatgcgagggggag

SEQ ID NO: 18080 - RNA, 5904 nt, Homo sapiens
  source 1..5904: mol_type = other RNA
tctgggtgcagtgggggtttggctgtggcagggaaaaggcatgtgagcttatatttttaaaaaattgtagtgggtaaacatcaacataaacctgcccaggaaaatagagcaggacttaaaagtttaaaaaaccataacaaaatagagctctaactataaactacagaaaacaggctcggagcttccgaggacatatgcccttcaagatgcctgtcccgctgccccctgtgaagggccacctgtcggagcatgggctttggggtttcctagttgtgctgctgctcttgcctagggaatctgctcttgctttggcctcttttcttggggcaagagtgagggggacagggagcttcaagtcagccctccatgttgaagtttggtagaagctctgcccacaccttggacgggaacccagccatgccaatccccatgatcaccaatccgaaccccttgaagtagaattttcacaccctactgactaatcaccttcttagccaggccatagccattcagcagtgcctccttcctctgggtagacaaacagccttgaacagaaaggtggaagactcgagttcttaacccagccccatctcttctgggctgtgtgaccttgggaatcccagaccctctctggaccacctccatttcctcatctgtaaagtgaggggcttgaagaagttgagctctaaggcttcttccagctctgacgttctgtgactggtagtatacccagagctcaggaaaggatggcccatttattaacccctttttctccggggaaatgcaagcagtccaaggccgtctgggagcggatctggccaggtggtcctaggtatacctgggagcaggcagggccacatttatcctctgcccttcccagaaacctcccaataccaggacacacagcatgaatgctgcattcccctcccaggcaggagtgagtcagtgctgggagagcagagtctggggctgcaggtcggggaggccgagctgactgcaggcagcactggagaggtgggcgcatgattggccatctcctgcccaaaccctggagggactgtgcagaatgggtcttggaggggtgggagaccccaccaagacaagccctttagtcacccagccacctgaagtggcgctgtcaatcgggatgacagggtcaggttggcagtgttggctgagagggcatcgtcacctgggttgtgactatctcagaccaaggctggtgcccctttccaccaagggccctggcctctcaactctttttggctcccaccccaaacagcctggagtatcacccccctcaaagctgaaggggctcaggctcccagcctcaggcatcggggcgctggttctcagccgcttgggcaggcaggagcccctagggagttatcggggacagcgtcagggtccttgctgctgctcgagggagaaggcgggagagctcttggtcccagggcttgcccttcttccttagactgaaggatggtgaggtgtgcacttcgctccagttcttcaacctgttcatgtctggtgttcctgccgggcctaggactgctctcaagtggcggagtccgtatagggtcccagagggccatctctgctgagttgaagacatgtttttaaaacccccttcttcccatgggcctgttccttccctccaggcagcctagagctcaggtataggcgtcagtgtcatcatggaagttactgcctggtgcctctcaatttaaagaaaatccttgcgtgggttctatcctgcggcagaatataaaatatcctacctcctacaaaaagggcactgtttaaagtaggtatttaaaaccagccactctctggcacagtgtcaggccaccttggcagcaggaaggggctggctgtgtccgtcggaggtggcgtccagctgcggcgcagagggaggggttccaggatcagagctccagggagcctatgaggatcagcatcgccacggagtgggaaatgacggtgccagggtgtggtgctgggcggactgccatgttctccaccatcatgcttgtgcagggccagctgcaggcctgggagcggacggctgggtggtcttctcagtccgactcctacggtgctttgtaggccgtttgctattgctggttggtcctcagcctccccctgcaccctgcgcccttccctggccctcggggatgttctgggggctgggtagaaaggtggcggcgaggcagttctaagactactttgcacttggttcctgcctgccttccactttcctttgcgggtagagattggagttggcctgggtgggaatgatcctctcaggtatctgggtggatcctgaatctctcgaggggataagggtaggggaggagcagcacctccattcctcacgatgtggacttctgcagggatcccatcccctccgggccctgtggtccgaatttgtaccagggcatggccaatgtcttcaggcactgggatttctatccagttcttgccggtgaggtggagcgtgggagtcaggtgtaagtcattctggtacagcatcttatagccggtgactgcagactcatttcggaaagggaccacagggtcccacttaatgctaagactagagcttgagaaagtccaggagatgttgccaggaggtcgccgcggagggggcttcatggtcgtggcgttggcagaagggctggcaggcccagtgccagcccggttgtaggccctcacggtcacatggtacttggtgttgggatgcaggccgctgactcgggcactggtgtccagccctgctgtcctcactcggtccgcagctgcttctttgtccccagctttccagtagcggatctcataccccaggaggataccattcatgtcctgctgcacgggttcccaggtcacgttcatctctgaggatgagacccctttggcccacaccttggtaggggccaccctgggctcttcctcagctgagtacacgagtgcagtgaggctctcgggcccatccccgcggcggttgtagctgcggatcttgacctcaaagggcgtgtagggccggacgctctcgttgctgtagacaaagtactgggcatcggcgccaggcacccgggcggtctgccagtgagtgctgccctgcctgcggaaggacagcaggtagccgaagccgtctccgttctggtactcccgtgacatgggcgtccagttgacgatgagctctccgggggctccacctcctccgctgagtcctgagggtgccaccgagggggctgcttccctggtccggattttgctggagggcccactaggctccccagtgcccagaatgttgctggctatgacccggaactcatagtccatccagggggtgaggcccagcacctgtgcagtctcggcattgccctcgatgtttgcaggattggtccgaacctgcttccacttccctgcaggtggagtgcgagcttgcagggtgtacttagcgatggggctgtggttgtcgaagccacggctccagctgagctggatggtggtgtcgccaatgtccctcaccaccacacctcctgggggacctggcggacctcggaccaggactgtggcctccttggacgcgctgtccaccaccgtctgggccatgcacgtgtacttccccccatggcgcagctgggcgttcaggatggtcagatccccaatggtctccttcacattagttctccggtagtgccctccaggcttatcaaagtcgatggggaagtcgtccagggtccaggtgaaggtgaggtccatggtggggtcgtgggaggcatggcactgtagggtcaggttgtcacccaagttgatgtcggcacttgagggggctagagtgattttggttgcatctcgcacagataggattccagtgctgttggctttgcccatgaagttctcagcaaagcaggtgtatttgccttcatctgaccggctgatgtttcttatgatcaaggtgccatctggagttacagtcactctgctgctgttgaccaaaatctccgtgcctttgctccagagcaccacggcctttggagctgcccggggctggcaggggataaggatctctcccccgcgggccgcggggatcagacgcctcacgggattcagcctgaagtcaggggcgagtgcttgcacggctagctcggcgctggcgtagatggtaccgtgcttattctctgccacacactggtacatgcccgagtcttccaggctcagcttggagaaccgcaggtccccagccaacacctccacccggttctgggaggccagaggctccccgttccgcagccagcgcactgtaggccggggcttgccggcggctgcacagccccaacgcaggttggagccaatgtcagcctctgtgtccgagatcacttttagccactcaggctgagcctgcacgatgatgcggccctgcacggtgtctcggcccttggagttctccgcctcacactcgtaggtgccctcatcctcaaagctgacgctggggatctgcagggtgggctcagctgtggtccactgcggggacagggagccgtccactttgcgccacttgatccgggggacagggttcccaaaggcgaagcactccagggtgacctgctgccccaccagtgcataggtctctgctgggaaccgggccttgatgctgggtgcaaagagccgggtatcttcagcagccaggttgagctgagcaaacttgctgaagacgctcttggtggagaagtccatgtggctggtggccaaacaggagtagttgcccaggtctgaggcattggttcgggcaatgtacaggttccctgtggtctgggacacgaagtgacgcccgtccgtcgggatgaagttggggaactcgttgaggagccagcggtaggacaagcctgggtagtgggcaggtgggttacagggcaacatcaccccccagccttcatgagctttcactgggtctcgctcctccttggagaattcctgcagaaagccgaagcggaggatggcctccctgctgacaacggtgcccactgggttggaggccaggcactggtagaccccggcatcctgtgccttggtggggttcatgatgaccaggttgccccccaccagctggtgacgggaacctggctccagcttcatctcggtaccattcatcttccaccgataggtggctggagggctggcccgggcgcggcatgccagcaacacctgctcctccgtggactcctctgggaatagcacactgaggggctggtcttcaaagacaggcccgaaggtggtttgggatcccagggctgaactccaagagaagaactgatctgtggggtgtgaggtgcatgagacgtcgccagccacaaacatgcagagaggatgtgtgtccctggagcctaatacccttactggggcagtgtggaccaacgaggcctgggcctggggactaggctggccctctactagctgtgggaccttgggaaagttatagaactcttctgagcctcagtatcttcacctgaagaggagacaagggccacagcagctaccagcagcaggtgtggcttcctcctggtggctgtccccatggtggatgtccgggcagaggtggggatcggaggagaagagcctcagctcagcttggggacagcccagctggaggctgagaaaggacctggggcgagagaagggtgttggctggggcaggtggatgctgcccgagtcggtgagccggggccggccgggccgccagcccctgtctgggccgctgtcctttgggccctggcggcctcagccgctcgctgtccgggtgcggcggcggccgcggcggcggtggcgggtgagggcgcgtgtgtgtgagcgcgcccggagccactgcagcatctctgcatcaagatgtgctcctccctc

SEQ ID NO: 18081 - RNA, 5389 nt, Homo sapiens
  source 1..5389: mol_type = other RNA
tctgggtgcagtgggggtttggctgtggcagggaaaaggcatgtgagcttatatttttaaaaaattgtagtgggtaaacatcaacataaacctgcccaggaaaatagagcaggacttaaaagtttaaaaaaccataacaaaatagagctctaactataaactacagaaaacaggctcggagcttccgaggacatatgcccttcaagatgcctgtcccgctgccccctgtgaagggccacctgtcggagcatgggctttggggtttcctagttgtgctgctgctcttgcctagggaatctgctcttgctttggcctcttttcttggggcaagagtgagggggacagggagcttcaagtcagccctccatgttgaagtttggtagaagctctgcccacaccttggacgggaacccagccatgccaatccccatgatcaccaatccgaaccccttgaagtagaattttcacaccctactgactaatcaccttcttagccaggccatagccattcagcagtgcctccttcctctgggtagacaaacagccttgaacagaaaggtggaagactcgagttcttaacccagccccatctcttctgggctgtgtgaccttgggaatcccagaccctctctggaccacctccatttcctcatctgtaaagtgaggggcttgaagaagttgagctctaaggcttcttccagctctgacgttctgtgactggtagtatacccagagctcaggaaaggatggcccatttattaacccctttttctccggggaaatgcaagcagtccaaggccgtctgggagcggatctggccaggtggtcctaggtatacctgggagcaggcagggccacatttatcctctgcccttcccagaaacctcccaataccaggacacacagcatgaatgctgcattcccctcccaggcaggagtgagtcagtgctgggagagcagagtctggggctgcaggtcggggaggccgagctgactgcaggcagcactggagaggtgggcgcatgattggccatctcctgcccaaaccctggagggactgtgcagaatgggtcttggaggggtgggagaccccaccaagacaagccctttagtcacccagccacctgaagtggcgctgtcaatcgggatgacagggtcaggttggcagtgttggctgagagggcatcgtcacctgggttgtgactatctcagaccaaggctggtgcccctttccaccaagggccctggcctctcaactctttttggctcccaccccaaacagcctggagtatcacccccctcaaagctgaaggggctcaggctcccagcctcaggcatcggggcgctggttctcagccgcttgggcaggcaggagcccctagggagttatcggggacagcgtcagggtccttgctgctgctcgagggagaaggcgggagagctcttggtcccagggcttgcccttcttccttagactgaaggatggtgaggtgtgcacttcgctccagttcttcaacctgttcatgtctggtgttcctgccgggcctaggactgctctcaagtggcggagtccgtatagggtcccagagggccatctctgctgagttgaagacatgtttttaaaacccccttcttcccatgggcctgttccttccctccaggcagcctagagctcaggtataggcgtcagtgtcatcatggaagttactgcctggtgcctctcaatttaaagaaaatccttgcgtgggttctatcctgcggcagaatataaaatatcctacctcctacaaaaagggcactgtttaaagtaggtatttaaaaccagccactctctggcacagtgtcaggccaccttggcagcaggaaggggctggctgtgtccgtcggaggtggcgtccagctgcggcgcagagggaggggttccaggatcagagctccagggagcctatgaggatcagcatcgccacggagtgggaaatgacggtgccagggtgtggtgctgggcggactgccatgttctccaccatcatgcttgtgcagggccagctgcaggcctgggagcggacggctgggtggtcttctcagtccgactcctacggtgctttgtaggccgtttgctattgctggttggtcctcagcctccccctgcaccctgcgcccttccctggccctcggggatgttctgggggctgggtagaaaggtggcggcgaggcagttctaagactactttgcacttggttcctgcctgccttccactttcctttgcgggtagagattggagttggcctgggtgggaatgatcctctcaggtatctgggtggatcctgaatctctcgaggggataagggtaggggaggagcagcacctccattcctcacgatgtggacttctgcagggatcccatcccctccgggccctgtggtccgaatttgtaccagggcatggccaatgtcttcaggcactgggatttctatccagttcttgccggtgaggtggagcgtgggagtcaggtgtaagtcattctggtacagcatcttatagccggtgactgcagactcatttcggaaagggaccacagggtcccacttaatgctaagactagagcttgagaaagtccaggagatgttgccaggaggtcgccgcggagggggcttcatggtcgtggcgttggcagaagggctggcaggcccagtgccagcccggttgtaggccctcacggtcacatggtacttggtgttgggatgcaggccgctgactcgggcactggtgtccagccctgctgtcctcactcggtccgcagctgcttctttgtccccagctttccagtagcggatctcataccccaggaggataccattcatgtcctgctgcacgggttcccaggtcacgttcatctctgaggatgagacccctttggcccacaccttggtaggggccaccctgggctcttcctcagctgagtacacgagtgcagtgaggctctcgggcccatccccgcggcggttgtagctgcggatcttgacctcaaagggcgtgtagggccggacgctctcgttgctgtagacaaagtactgggcatcggcgccaggcacccgggcggtctgccagtgagtgctgccctgcctgcggaaggacagcaggtagccgaagccgtctccgttctggtactcccgtgacatgggcgtccagttgacgatgagctctccgggggctccacctcctccgctgagtcctgagggtgccaccgagggggctgcttccctggtccggattttgctggagggcccactaggctccccagtgcccagaatgttgctggctatgacccggaactcatagtccatccagggggtgaggcccagcacctgtgcagtctcggcattgccctcgatgtttgcaggattggtccgaacctgcttccacttccctgcaggtggagtgcgagcttgcagggtgtacttagcgatggggctgtggttgtcgaagccacggctccagctgagctggatggtggtgtcgccaatgtccctcaccaccacacctcctgggggacctggcggacctcggaccaggactgtggcctccttggacgcgctgtccaccaccgtctgggccatgcacgtgtacttccccccatggcgcagctgggcgttcaggatggtcagatccccaatggtctccttcacattagttctccggtagtgccctccaggcttatcaaagtcgatggggaagtcgtccagggtccaggtgaaggtgaggtccatggtggggtcgtgggaggcatggcactgtagggtcaggttgtcacccaagttgatgtcggcacttgagggggctagagtgattttggttgcatctcgcacagataggattccagtgctgttggctttgcccatgaagttctcagcaaagcaggtgtatttgccttcatctgaccggctgatgtttcttatgatcaaggtgccatctggagttacagtcactctgctgctgttgaccaaaatctccgtgcctttgctccagagcaccacggcctttggagctgcccggggctggcaggggataaggatctctcccccgcgggccgcggggatcagacgcctcacgggattcagcctgaagtcaggggcgagtgcttgcacggctagctcggcgctggcgtagatggtaccgtgcttattctctgccacacactggtacatgcccgagtcttccaggctcagcttggagaaccgcaggtccccagccaacacctccacccggttctgggaggccagaggctccccgttccgcagccagcgcactgtaggccggggcttgccggcggctgcacagccccaacgcaggttggagccaatgtcagcctctgtgtccgagatcacttttagccactcaggctgagcctgcacgatgatgcggccctgcacggtgtctcggcccttggagttctccgcctcacactcgtaggtgccctcatcctcaaagctgacgctggggatctgcagggtgggctcagctgtggtccactgcggggacagggagccgtccactttgcgccacttgatccgggggacagggttcccaaaggcgaagcactccagggtgacctgctgccccaccagtgcataggtctctgctgggaaccgggccttgatgctgggtgcaaagagccgggtatcttcagcagccaggttgagctgagcaaacttgctgaagacgctcttggtggagaagtccatgtggctggtggccaaacaggagtagttgcccaggtctgaggcattggttcgggcaatgtacaggttccctgtggtctgggacacgaagtgacgcccgtccgtcgggatgaagttggggaactcgttgaggagccagcggtaggacaagcctgggtagtgggcaggtgggttacagggcaacatcaccccccagccttcatgagctttcactgggtctcgctcctccttggagaattcctgcagaaagccgaagcggaggatggcctccctgctgacaacggtgcccactgggttggaggccaggcactggtagaccccggcatcctgtgccttggtggggttcatgatgaccaggttgccccccaccagctggtgacgggaacctggctccagcttcatctcggtaccattcatcttccaccgataggtggctggagggctggcccgggcgcggcatgccagcaacacctgctcctccgtggactcctctgggaatagcacactgaggggctggtcttcaaagacaggcccgaaggtggtttgggatcccagggctgaactccaagctgaagaggagacaagggccacagcagctaccagcagcaggtgtggcttcctcctggtggctgtccccatggtggatgtc

SEQ ID NO: 18082 - RNA, 6415 nt, Homo sapiens
  source 1..6415: mol_type = other RNA
tctgggtgcagtgggggtttggctgtggcagggaaaaggcatgtgagcttatatttttaaaaaattgtagtgggtaaacatcaacataaacctgcccaggaaaatagagcaggacttaaaagtttaaaaaaccataacaaaatagagctctaactataaactacagaaaacaggctcggagcttccgaggacatatgcccttcaagatgcctgtcccgctgccccctgtgaagggccacctgtcggagcatgggctttggggtttcctagttgtgctgctgctcttgcctagggaatctgctcttgctttggcctcttttcttggggcaagagtgagggggacagggagcttcaagtcagccctccatgttgaagtttggtagaagctctgcccacaccttggacgggaacccagccatgccaatccccatgatcaccaatccgaaccccttgaagtagaattttcacaccctactgactaatcaccttcttagccaggccatagccattcagcagtgcctccttcctctgggtagacaaacagccttgaacagaaaggtggaagactcgagttcttaacccagccccatctcttctgggctgtgtgaccttgggaatcccagaccctctctggaccacctccatttcctcatctgtaaagtgaggggcttgaagaagttgagctctaaggcttcttccagctctgacgttctgtgactggtagtatacccagagctcaggaaaggatggcccatttattaacccctttttctccggggaaatgcaagcagtccaaggccgtctgggagcggatctggccaggtggtcctaggtatacctgggagcaggcagggccacatttatcctctgcccttcccagaaacctcccaataccaggacacacagcatgaatgctgcattcccctcccaggcaggagtgagtcagtgctgggagagcagagtctggggctgcaggtcggggaggccgagctgactgcaggcagcactggagaggtgggcgcatgattggccatctcctgcccaaaccctggagggactgtgcagaatgggtcttggaggggtgggagaccccaccaagacaagccctttagtcacccagccacctgaagtggcgctgtcaatcgggatgacagggtcaggttggcagtgttggctgagagggcatcgtcacctgggttgtgactatctcagaccaaggctggtgcccctttccaccaagggccctggcctctcaactctttttggctcccaccccaaacagcctggagtatcacccccctcaaagctgaaggggctcaggctcccagcctcaggcatcggggcgctggttctcagccgcttgggcaggcaggagcccctagggagttatcggggacagcgtcagggtccttgctgctgctcgagggagaaggcgggagagctcttggtcccagggcttgcccttcttccttagactgaaggatggtgaggtgtgcacttcgctccagttcttcaacctgttcatgtctggtgttcctgccgggcctaggactgctctcaagtggcggagtccgtatagggtcccagagggccatctctgctgagttgaagacatgtttttaaaacccccttcttcccatgggcctgttccttccctccaggcagcctagagctcaggtataggcgtcagtgtcatcatggaagttactgcctggtgcctctcaatttaaagaaaatccttgcgtgggttctatcctgcggcagaatataaaatatcctacctcctacaaaaagggcactgtttaaagtaggtatttaaaaccagccactctctggcacagtgtcaggccaccttggcagcaggaaggggctggctgtgtccgtcggaggtggcgtccagctgcggcgcagagggaggggttccaggatcagagctccagggagcctatgaggatcagcatcgccacggagtgggaaatgacggtgccagggtgtggtgctgggcggactgccatgttctccaccatcatgcttgtgcagggccagctgcaggcctgggagcggacggctgggtggtcttctcagtccgactcctacggtgctttgtaggccgtttgctattgctggttggtcctcagcctccccctgcaccctgcgcccttccctggccctcggggatgttctgggggctgggtagaaaggtggcggcgaggcagttctaagactactttgcacttggttcctgcctgccttccactttcctttgcgggtagagattggagttggcctgggtgggaatgatcctctcaggtatctgggtggatcctgaatctctcgaggggataagggtaggggaggagcagcacctccattcctcacgatgtggacttctgcagggatcccatcccctccgggccctgtggtccgaatttgtaccagggcatggccaatgtcttcaggcactgggatttctatccagttcttgccggtgaggtggagcgtgggagtcaggtgtaagtcattctggtacagcatcttatagccggtgactgcagactcatttcggaaagggaccacagggtcccacttaatgctaagactagagcttgagaaagtccaggagatgttgccaggaggtcgccgcggagggggcttcatggtcgtggcgttggcagaagggctggcaggcccagtgccagcccggttgtaggccctcacggtcacatggtacttggtgttgggatgcaggccgctgactcgggcactggtgtccagccctgctgtcctcactcggtccgcagctgcttctttgtccccagctttccagtagcggatctcataccccaggaggataccattcatgtcctgctgcacgggttcccaggtcacgttcatctctgaggatgagacccctttggcccacaccttggtaggggccaccctgggctcttcctcagctgagtacacgagtgcagtgaggctctcgggcccatccccgcggcggttgtagctgcggatcttgacctcaaagggcgtgtagggccggacgctctcgttgctgtagacaaagtactgggcatcggcgccaggcacccgggcggtctgccagtgagtgctgccctgcctgcggaaggacagcaggtagccgaagccgtctccgttctggtactcccgtgacatgggcgtccagttgacgatgagctctccgggggctccacctcctccgctgagtcctgagggtgccaccgagggggctgcttccctggtccggattttgctggagggcccactaggctccccagtgcccagaatgttgctggctatgacccggaactcatagtccatccagggggtgaggcccagcacctgtgcagtctcggcattgccctcgatgtttgcaggattggtccgaacctgcttccacttccctgcaggtggagtgcgagcttgcagggtgtacttagcgatggggctgtggttgtcgaagccacggctccagctgagctggatggtggtgtcgccaatgtccctcaccaccacacctcctgggggacctggcggacctcggaccaggactgtggcctccttggacgcgctgtccaccaccgtctgggccatgcacgtgtacttccccccatggcgcagctgggcgttcaggatggtcagatccccaatggtctccttcacattagttctccggtagtgccctccaggcttatcaaagtcgatggggaagtcgtccagggtccaggtgaaggtgaggtccatggtggggtcgtgggaggcatggcactgtagggtcaggttgtcacccaagttgatgtcggcacttgagggggctagagtgattttggttgcatctcgcacagataggattccagtgctgttggctttgcccatgaagttctcagcaaagcaggtgtatttgccttcatctgaccggctgatgtttcttatgatcaaggtgccatctggagttacagtcactctgctgctgttgaccaaaatctccgtgcctttgctccagagcaccacggcctttggagctgcccggggctggcaggggataaggatctctcccccgcgggccgcggggatcagacgcctcacgggattcagcctgaagtcaggggcgagtgcttgcacggctagctcggcgctggcgtagatggtaccgtgcttattctctgccacacactggtacatgcccgagtcttccaggctcagcttggagaaccgcaggtccccagccaacacctccacccggttctgggaggccagaggctccccgttccgcagccagcgcactgtaggccggggcttgccggcggctgcacagccccaacgcaggttggagccaatgtcagcctctgtgtccgagatcacttttagccactcaggctgagcctgcacgatgatgcggccctgcacggtgtctcggcccttggagttctccgcctcacactcgtaggtgccctcatcctcaaagctgacgctggggatctgcagggtgggctcagctgtggtccactgcggggacagggagccgtccactttgcgccacttgatccgggggacagggttcccaaaggcgaagcactccagggtgacctgctgccccaccagtgcataggtctctgctgggaaccgggccttgatgctgggtgcaaagagccgggtatcttcagcagccaggttgagctgagcaaacttgctgaagacgctcttggtggagaagtccatgtggctggtggccaaacaggagtagttgcccaggtctgaggcattggttcgggcaatgtacaggttccctgtggtctgggacacgaagtgacgcccgtccgtcgggatgaagttggggaactcgttgaggagccagcggtaggacaagcctgggtagtgggcaggtgggttacagggcaacatcaccccccagccttcatgagctttcactgggtctcgctcctccttggagaattcctgcagaaagccgaagcggaggatggcctccctgctgacaacggtgcccactgggttggaggccaggcactggtagaccccggcatcctgtgccttggtggggttcatgatgaccaggttgccccccaccagctggtgacgggaacctggctccagcttcatctcggtaccattcatcttccaccgataggtggctggagggctggcccgggcgcggcatgccagcaacacctgctcctccgtggactcctctgggaatagcacactgaggggctggtcttcaaagacaggcccgaaggtggtttgggatcccagggctgaactccaagctgcaggtgatgacaccaccagatgcctcagagccttggcctggctggagcctggcctcttgggctgtgctgtccagtaaaactttctctgatgatgggaatgtcccattttctgcactgttcaatgtggtaaccactagccacgtagggctatcgagcacttgacatgtggctattgcgactgaagaacgacattttacattttatattacttaattaatttaaatttgaatttaaataggctgggcaggccccatctggccatactagttcaatcaatcacccatcctacacttaggtattgagcacctgctctatacccagcactgggctagagactggcttgtaaagatgattaagacacagtccctcttcttcaaggggcttgcggtccaaggagggagacaggaaattgacagtgcaaggtagcaaatgccataaagttcaagatgctggggcctcagaatggaagcagttctacctcccagggggctttcaagggacccttacagaagaactgatctgtggggtgtgaggtgcatgagacgtcgccagccacaaacatgcagagaggatgtgtgtccctggagcctaatacccttactggggcagtgtggaccaacgaggcctgggcctggggactaggctggccctctactagctgtgggaccttgggaaagttatagaactcttctgagcctcagtatcttcacctgaagaggagacaagggccacagcagctaccagcagcaggtgtggcttcctcctggtggctgtccccatggtggatgtccgggcagaggtggggatcggaggagaagagcctcagctcagcttggggacagcccagctggaggctgagaaaggacctggggcgagagaagggtgttggctggggcaggtggatgctgcccgagtcggtgagccggggccggccgggccgccagcccctgtctgggccgctgtcctttgggccctggcggcctcagccgctcgctgtccgggtgcggcggcggccgcggcggcggtggcgggtgagggcgcgtgtgtgtgagcgcgcccggagccactgcagcatctctgcatcaagatgtgctcctccctct

SEQ ID NO: 18083 - RNA, 5911 nt, Homo sapiens
  source 1..5911: mol_type = other RNA
tctgggtgcagtgggggtttggctgtggcagggaaaaggcatgtgagcttatatttttaaaaaattgtagtgggtaaacatcaacataaacctgcccaggaaaatagagcaggacttaaaagtttaaaaaaccataacaaaatagagctctaactataaactacagaaaacaggctcggagcttccgaggacatatgcccttcaagatgcctgtcccgctgccccctgtgaagggccacctgtcggagcatgggctttggggtttcctagttgtgctgctgctcttgcctagggaatctgctcttgctttggcctcttttcttggggcaagagtgagggggacagggagcttcaagtcagccctccatgttgaagtttggtagaagctctgcccacaccttggacgggaacccagccatgccaatccccatgatcaccaatccgaaccccttgaagtagaattttcacaccctactgactaatcaccttcttagccaggccatagccattcagcagtgcctccttcctctgggtagacaaacagccttgaacagaaaggtggaagactcgagttcttaacccagccccatctcttctgggctgtgtgaccttgggaatcccagaccctctctggaccacctccatttcctcatctgtaaagtgaggggcttgaagaagttgagctctaaggcttcttccagctctgacgttctgtgactggtagtatacccagagctcaggaaaggatggcccatttattaacccctttttctccggggaaatgcaagcagtccaaggccgtctgggagcggatctggccaggtggtcctaggtatacctgggagcaggcagggccacatttatcctctgcccttcccagaaacctcccaataccaggacacacagcatgaatgctgcattcccctcccaggcaggagtgagtcagtgctgggagagcagagtctggggctgcaggtcggggaggccgagctgactgcaggcagcactggagaggtgggcgcatgattggccatctcctgcccaaaccctggagggactgtgcagaatgggtcttggaggggtgggagaccccaccaagacaagccctttagtcacccagccacctgaagtggcgctgtcaatcgggatgacagggtcaggttggcagtgttggctgagagggcatcgtcacctgggttgtgactatctcagaccaaggctggtgcccctttccaccaagggccctggcctctcaactctttttggctcccaccccaaacagcctggagtatcacccccctcaaagctgaaggggctcaggctcccagcctcaggcatcggggcgctggttctcagccgcttgggcaggcaggagcccctagggagttatcggggacagcgtcagggtccttgctgctgctcgagggagaaggcgggagagctcttggtcccagggcttgcccttcttccttagactgaaggatggtgaggtgtgcacttcgctccagttcttcaacctgttcatgtctggtgttcctgccgggcctaggactgctctcaagtggcggagtccgtatagggtcccagagggccatctctgctgagttgaagacatgtttttaaaacccccttcttcccatgggcctgttccttccctccaggcagcctagagctcaggtataggcgtcagtgtcatcatggaagttactgcctggtgcctctcaatttaaagaaaatccttgcgtgggttctatcctgcggcagaatataaaatatcctacctcctacaaaaagggcactgtttaaagtaggtatttaaaaccagccactctctggcacagtgtcaggccaccttggcagcaggaaggggctggctgtgtccgtcggaggtggcgtccagctgcggcgcagagggaggggttccaggatcagagctccagggagcctatgaggatcagcatcgccacggagtgggaaatgacggtgccagggtgtggtgctgggcggactgccatgttctccaccatcatgcttgtgcagggccagctgcaggcctgggagcggacggctgggtggtcttctcagtccgactcctacggtgctttgtaggccgtttgctattgctggttggtcctcagcctccccctgcaccctgcgcccttccctggccctcggggatgttctgggggctgggtagaaaggtggcggcgaggcagttctaagactactttgcacttggttcctgcctgccttccactttcctttgcgggtagagattggagttggcctgggtgggaatgatcctctcaggtatctgggtggatcctgaatctctcgaggggataagggtaggggaggagcagcacctccattcctcacgatgtggacttctgcagggatcccatcccctccgggccctgtggtccgaatttgtaccagggcatggccaatgtcttcaggcactgggatttctatccagttcttgccggtgaggtggagcgtgggagtcaggtgtaagtcattctggtacagcatcttatagccggtgactgcagactcatttcggaaagggaccacagggtcccacttaatgctaagactagagcttgagaaagtccaggagatgttgccaggaggtcgccgcggagggggcttcatggtcgtggcgttggcagaagggctggcaggcccagtgccagcccggttgtaggccctcacggtcacatggtacttggtgttgggatgcaggccgctgactcgggcactggtgtccagccctgctgtcctcactcggtccgcagctgcttctttgtccccagctttccagtagcggatctcataccccaggaggataccattcatgtcctgctgcacgggttcccaggtcacgttcatctctgaggatgagacccctttggcccacaccttggtaggggccaccctgggctcttcctcagctgagtacacgagtgcagtgaggctctcgggcccatccccgcggcggttgtagctgcggatcttgacctcaaagggcgtgtagggccggacgctctcgttgctgtagacaaagtactgggcatcggcgccaggcacccgggcggtctgccagtgagtgctgccctgcctgcggaaggacagcaggtagccgaagccgtctccgttctggtactcccgtgacatgggcgtccagttgacgatgagctctccgggggctccacctcctccgctgagtcctgagggtgccaccgagggggctgcttccctggtccggattttgctggagggcccactaggctccccagtgcccagaatgttgctggctatgacccggaactcatagtccatccagggggtgaggcccagcacctgtgcagtctcggcattgccctcgatgtttgcaggattggtccgaacctgcttccacttccctgcaggtggagtgcgagcttgcagggtgtacttagcgatggggctgtggttgtcgaagccacggctccagctgagctggatggtggtgtcgccaatgtccctcaccaccacacctcctgggggacctggcggacctcggaccaggactgtggcctccttggacgcgctgtccaccaccgtctgggccatgcacgtgtacttccccccatggcgcagctgggcgttcaggatggtcagatccccaatggtctccttcacattagttctccggtagtgccctccaggcttatcaaagtcgatggggaagtcgtccagggtccaggtgaaggtgaggtccatggtggggtcgtgggaggcatggcactgtagggtcaggttgtcacccaagttgatgtcggcacttgagggggctagagtgattttggttgcatctcgcacagataggattccagtgctgttggctttgcccatgaagttctcagcaaagcaggtgtatttgccttcatctgaccggctgatgtttcttatgatcaaggtgccatctggagttacagtcactctgctgctgttgaccaaaatctccgtgcctttgctccagagcaccacggcctttggagctgcccggggctggcaggggataaggatctctcccccgcgggccgcggggatcagacgcctcacgggattcagcctgaagtcaggggcgagtgcttgcacggctagctcggcgctggcgtagatggtaccgtgcttattctctgccacacactggtacatgcccgagtcttccaggctcagcttggagaaccgcaggtccccagccaacacctccacccggttctgggaggccagaggctccccgttccgcagccagcgcactgtaggccggggcttgccggcggctgcacagccccaacgcaggttggagccaatgtcagcctctgtgtccgagatcacttttagccactcaggctgagcctgcacgatgatgcggccctgcacggtgtctcggcccttggagttctccgcctcacactcgtaggtgccctcatcctcaaagctgacgctggggatctgcagggtgggctcagctgtggtccactgcggggacagggagccgtccactttgcgccacttgatccgggggacagggttcccaaaggcgaagcactccagggtgacctgctgccccaccagtgcataggtctctgctgggaaccgggccttgatgctgggtgcaaagagccgggtatcttcagcagccaggttgagctgagcaaacttgctgaagacgctcttggtggagaagtccatgtggctggtggccaaacaggagtagttgcccaggtctgaggcattggttcgggcaatgtacaggttccctgtggtctgggacacgaagtgacgcccgtccgtcgggatgaagttggggaactcgttgaggagccagcggtaggacaagcctgggtagtgggcaggtgggttacagggcaacatcaccccccagccttcatgagctttcactgggtctcgctcctccttggagaattcctgcagaactggaggcagagaccaggggctcaggcactgtcctcctggcctgcgagcccctccccgactcatccttcacggagaagcagcagttcactaaggcatgtcatgtgaggtcaggaaggcccggcttgagggtgtcccttatcctttctcagtaatttctcctagccccctctccccctcccccaaagtgtcttggtcccccgcgggtctcacagccgaagcggaggatggcctccctgctgacaacggtgcccactgggttggaggccaggcactggtagaccccggcatcctgtgccttggtggggttcatgatgaccaggttgccccccaccagctggtgacgggaacctggctccagcttcatctcggtaccattcatcttccaccgataggtggctggagggctggcccgggcgcggcatgccagcaacacctgctcctccgtggactcctctgggaatagcacactgaggggctggtcttcaaagacaggcccgaaggtggtttgggatcccagggctgaactccaagctgaagaggagacaagggccacagcagctaccagcagcaggtgtggcttcctcctggtggctgtccccatggtggatgtccgggcagaggtggggatcggaggagaagagcctcagctcagcttggggacagcccagctggaggctgagaaaggacctggggcgagagaagggtgttggctggggcaggtggatgctgcccgagtcggtgagccggggccggccgggccgccagcccctgtctgggccgctgtcctttgggccctggcggcctcagccgctcgctgtccgggtgcggcggcggccgcggcggcggtggcgggtgagggcgcgtgtgtgtgagcgcgcccggagccactgcagcatctctgcatcaagatgtgctcctccct

SEQ ID NO: 18084 - RNA, 6495 nt, Homo sapiens
  source 1..6495: mol_type = other RNA
tctgggtgcagtgggggtttggctgtggcagggaaaaggcatgtgagcttatatttttaaaaaattgtagtgggtaaacatcaacataaacctgcccaggaaaatagagcaggacttaaaagtttaaaaaaccataacaaaatagagctctaactataaactacagaaaacaggctcggagcttccgaggacatatgcccttcaagatgcctgtcccgctgccccctgtgaagggccacctgtcggagcatgggctttggggtttcctagttgtgctgctgctcttgcctagggaatctgctcttgctttggcctcttttcttggggcaagagtgagggggacagggagcttcaagtcagccctccatgttgaagtttggtagaagctctgcccacaccttggacgggaacccagccatgccaatccccatgatcaccaatccgaaccccttgaagtagaattttcacaccctactgactaatcaccttcttagccaggccatagccattcagcagtgcctccttcctctgggtagacaaacagccttgaacagaaaggtggaagactcgagttcttaacccagccccatctcttctgggctgtgtgaccttgggaatcccagaccctctctggaccacctccatttcctcatctgtaaagtgaggggcttgaagaagttgagctctaaggcttcttccagctctgacgttctgtgactggtagtatacccagagctcaggaaaggatggcccatttattaacccctttttctccggggaaatgcaagcagtccaaggccgtctgggagcggatctggccaggtggtcctaggtatacctgggagcaggcagggccacatttatcctctgcccttcccagaaacctcccaataccaggacacacagcatgaatgctgcattcccctcccaggcaggagtgagtcagtgctgggagagcagagtctggggctgcaggtcggggaggccgagctgactgcaggcagcactggagaggtgggcgcatgattggccatctcctgcccaaaccctggagggactgtgcagaatgggtcttggaggggtgggagaccccaccaagacaagccctttagtcacccagccacctgaagtggcgctgtcaatcgggatgacagggtcaggttggcagtgttggctgagagggcatcgtcacctgggttgtgactatctcagaccaaggctggtgcccctttccaccaagggccctggcctctcaactctttttggctcccaccccaaacagcctggagtatcacccccctcaaagctgaaggggctcaggctcccagcctcaggcatcggggcgctggttctcagccgcttgggcaggcaggagcccctagggagttatcggggacagcgtcagggtccttgctgctgctcgagggagaaggcgggagagctcttggtcccagggcttgcccttcttccttagactgaaggatggtgaggtgtgcacttcgctccagttcttcaacctgttcatgtctggtgttcctgccgggcctaggactgctctcaagtggcggagtccgtatagggtcccagagggccatctctgctgagttgaagacatgtttttaaaacccccttcttcccatgggcctgttccttccctccaggcagcctagagctcaggtataggcgtcagtgtcatcatggaagttactgcctggtgcctctcaatttaaagaaaatccttgcgtgggttctatcctgcggcagaatataaaatatcctacctcctacaaaaagggcactgtttaaagtaggtatttaaaaccagccactctctggcacagtgtcaggccaccttggcagcaggaaggggctggctgtgtccgtcggaggtggcgtccagctgcggcgcagagggaggggttccaggatcagagctccagggagcctatgaggatcagcatcgccacggagtgggaaatgacggtgccagggtgtggtgctgggcggactgccatgttctccaccatcatgcttgtgcagggccagctgcaggcctgggagcggacggctgggtggtcttctcagtccgactcctacggtgctttgtaggccgtttgctattgctggttggtcctcagcctccccctgcaccctgcgcccttccctggccctcggggatgttctgggggctgggtagaaaggtggcggcgaggcagttctaagactactttgcacttggttcctgcctgccttccactttcctttgcgggtagagattggagttggcctgggtgggaatgatcctctcaggtatctgggtggatcctgaatctctcgaggggataagggtaggggaggagcagcacctccattcctcacgatgtggacttctgcagggatcccatcccctccgggccctgtggtccgaatttgtaccagggcatggccaatgtcttcaggcactgggatttctatccagttcttgccggtgaggtggagcgtgggagtcaggtgtaagtcattctggtacagcatcttatagccggtgactgcagactcatttcggaaagggaccacagggtcccacttaatgctaagactagagcttgagaaagtccaggagatgttgccaggaggtcgccgcggagggggcttcatggtcgtggcgttggcagaagggctggcaggcccagtgccagcccggttgtaggccctcacggtcacatggtacttggtgttgggatgcaggccgctgactcgggcactggtgtccagccctgctgtcctcactcggtccgcagctgcttctttgtccccagctttccagtagcggatctcataccccaggaggataccattcatgtcctgctgcacgggttcccaggtcacgttcatctctgaggatgagacccctttggcccacaccttggtaggggccaccctgggctcttcctcagctgagtacacgagtgcagtgaggctctcgggcccatccccgcggcggttgtagctgcggatcttgacctcaaagggcgtgtagggccggacgctctcgttgctgtagacaaagtactgggcatcggcgccaggcacccgggcggtctgccagtgagtgctgccctgcctgcggaaggacagcaggtagccgaagccgtctccgttctggtactcccgtgacatgggcgtccagttgacgatgagctctccgggggctccacctcctccgctgagtcctgagggtgccaccgagggggctgcttccctggtccggattttgctggagggcccactaggctccccagtgcccagaatgttgctggctatgacccggaactcatagtccatccagggggtgaggcccagcacctgtgcagtctcggcattgccctcgatgtttgcaggattggtccgaacctgcttccacttccctgcaggtggagtgcgagcttgcagggtgtacttagcgatggggctgtggttgtcgaagccacggctccagctgagctggatggtggtgtcgccaatgtccctcaccaccacacctcctgggggacctggcggacctcggaccaggactgtggcctccttggacgcgctgtccaccaccgtctgggccatgcacgtgtacttccccccatggcgcagctgggcgttcaggatggtcagatccccaatggtctccttcacattagttctccggtagtgccctccaggcttatcaaagtcgatggggaagtcgtccagggtccaggtgaaggtgaggtccatggtggggtcgtgggaggcatggcactgtagggtcaggttgtcacccaagttgatgtcggcacttgagggggctagagtgattttggttgcatctcgcacagataggattccagtgctgttggctttgcccatgaagttctcagcaaagcaggtgtatttgccttcatctgaccggctgatgtttcttatgatcaaggtgccatctggagttacagtcactctgctgctgttgaccaaaatctccgtgcctttgctccagagcaccacggcctttggagctgcccggggctggcaggggataaggatctctcccccgcgggccgcggggatcagacgcctcacgggattcagcctgaagtcaggggcgagtgcttgcacggctagctcggcgctggcgtagatggtaccgtgcttattctctgccacacactggtacatgcccgagtcttccaggctcagcttggagaaccgcaggtccccagccaacacctccacccggttctgggaggccagaggctccccgttccgcagccagcgcactgtaggccggggcttgccggcggctgcacagccccaacgcaggttggagccaatgtcagcctctgtgtccgagatcacttttagccactcaggctgagcctgcacgatgatgcggccctgcacggtgtctcggcccttggagttctccgcctcacactcgtaggtgccctcatcctcaaagctgacgctggggatctgcagggtgggctcagctgtggtccactgcggggacagggagccgtccactttgcgccacttgatccgggggacagggttcccaaaggcgaagcactccagggtgacctgctgccccaccagtgcataggtctctgctgggaaccgggccttgatgctgggtgcaaagagccgggtatcttcagcagccaggttgagctgagcaaacttgctgaagacgctcttggtggagaagtccatgtggctggtggccaaacaggagtagttgcccaggtctgaggcattggttcgggcaatgtacaggttccctgtggtctgggacacgaagtgacgcccgtccgtcgggatgaagttggggaactcgttgaggagccagcggtaggacaagcctgggtagtgggcaggtgggttacagggcaacatcaccccccagccttcatgagctttcactgggtctcgctcctccttggagaattcctgcagaactggaggcagagaccaggggctcaggcactgtcctcctggcctgcgagcccctccccgactcatccttcacggagaagcagcagttcactaaggcatgtcatgtgaggtcaggaaggcccggcttgagggtgtcccttatcctttctcagtaatttctcctagccccctctccccctcccccaaagtgtcttggtcccccgcgggtctcacagccgaagcggaggatggcctccctgctgacaacggtgcccactgggttggaggccaggcactggtagaccccggcatcctgtgccttggtggggttcatgatgaccaggttgccccccaccagctggtgacgggaacctggctccagcttcatctcggtaccattcatcttccaccgataggtggctggagggctggcccgggcgcggcatgccagcaacacctgctcctccgtggactcctctgggaatagcacactgaggggctggtcttcaaagacaggcccgaaggtggtttgggatcccagggctgaactccaagctgcaggtgatgacaccaccagatgcctcagagccttggcctggctggagcctggcctcttgggctgtgctgtccagtaaaactttctctgatgatgggaatgtcccattttctgcactgttcaatgtggtaaccactagccacgtagggctatcgagcacttgacatgtggctattgcgactgaagaacgacattttacattttatattacttaattaatttaaatttgaatttaaataggctgggcaggccccatctggccatactagttcaatcaatcacccatcctacacttaggtattgagcacctgctctatacccagcactgggctagagactggcttgtaaagatgattaagacacagtccctcttcttcaaggggcttgcggtccaaggagggagacaggaaattgacagtgcaaggtagcaaatgccataaagttcaagatgctggggcctcagaatggaagcagttctacctcccagggggctttcaagggacccttacagaagaactgatctgtggggtgtgaggtgcatgagacgtcgccagccacaaacatgcagagaggatgtgtgtccctggagcctaatacccttactggggcagtgtggaccaacgaggcctgggcctggggactaggctggccctctactagctgtgggaccttgggaaagttatagaactcttctgagcctcagtatcttcacctgaagaggagacaagggccacagcagctaccagcagcaggtgtggcttcctcctggtggctgtccccatggtggatgtccgggcagaggtggggatcggaggagaagagcctcagctcagcttggggacagcccagctggaggctgagaaaggacctcatttgctgtcatttaaggaccagggagcgagcccagcgcgcgtcttccataatgcatgggccgctcatggacaggccgcggggcgctgtctggcccgcctgcc

SEQ ID NO: 18085 - RNA, 5261 nt, Homo sapiens
  source 1..5261: mol_type = other RNA
tctgggtgcagtgggggtttggctgtggcagggaaaaggcatgtgagcttatatttttaaaaaattgtagtgggtaaacatcaacataaacctgcccaggaaaatagagcaggacttaaaagtttaaaaaaccataacaaaatagagctctaactataaactacagaaaacaggctcggagcttccgaggacatatgcccttcaagatgcctgtcccgctgccccctgtgaagggccacctgtcggagcatgggctttggggtttcctagttgtgctgctgctcttgcctagggaatctgctcttgctttggcctcttttcttggggcaagagtgagggggacagggagcttcaagtcagccctccatgttgaagtttggtagaagctctgcccacaccttggacgggaacccagccatgccaatccccatgatcaccaatccgaaccccttgaagtagaattttcacaccctactgactaatcaccttcttagccaggccatagccattcagcagtgcctccttcctctgggtagacaaacagccttgaacagaaaggtggaagactcgagttcttaacccagccccatctcttctgggctgtgtgaccttgggaatcccagaccctctctggaccacctccatttcctcatctgtaaagtgaggggcttgaagaagttgagctctaaggcttcttccagctctgacgttctgtgactggtagtatacccagagctcaggaaaggatggcccatttattaacccctttttctccggggaaatgcaagcagtccaaggccgtctgggagcggatctggccaggtggtcctaggtatacctgggagcaggcagggccacatttatcctctgcccttcccagaaacctcccaataccaggacacacagcatgaatgctgcattcccctcccaggcaggagtgagtcagtgctgggagagcagagtctggggctgcaggtcggggaggccgagctgactgcaggcagcactggagaggtgggcgcatgattggccatctcctgcccaaaccctggagggactgtgcagaatgggtcttggaggggtgggagaccccaccaagacaagccctttagtcacccagccacctgaagtggcgctgtcaatcgggatgacagggtcaggttggcagtgttggctgagagggcatcgtcacctgggttgtgactatctcagaccaaggctggtgcccctttccaccaagggccctggcctctcaactctttttggctcccaccccaaacagcctggagtatcacccccctcaaagctgaaggggctcaggctcccagcctcaggcatcggggcgctggttctcagccgcttgggcaggcaggagcccctagggagttatcggggacagcgtcagggtccttgctgctgctcgagggagaaggcgggagagctcttggtcccagggcttgcccttcttccttagactgaaggatggtgaggtgtgcacttcgctccagttcttcaacctgttcatgtctggtgttcctgccgggcctaggactgctctcaagtggcggagtccgtatagggtcccagagggccatctctgctgagttgaagacatgtttttaaaacccccttcttcccatgggcctgttccttccctccaggcagcctagagctcaggtataggcgtcagtgtcatcatggaagttactgcctggtgcctctcaatttaaagaaaatccttgcgtgggttctatcctgcggcagaatataaaatatcctacctcctacaaaaagggcactgtttaaagtaggtatttaaaaccagccactctctggcacagtgtcaggccaccttggcagcaggaaggggctggctgtgtccgtcggaggtggcgtccagctgcggcgcagagggaggggttccaggatcagagctccagggagcctatgaggatcagcatcgccacggagtgggaaatgacggtgccagggtgtggtgctgggcggactgccatgttctccaccatcatgcttgtgcctccattcctcacgatgtggacttctgcagggatcccatcccctccgggccctgtggtccgaatttgtaccagggcatggccaatgtcttcaggcactgggatttctatccagttcttgccggtgaggtggagcgtgggagtcaggtgtaagtcattctggtacagcatcttatagccggtgactgcagactcatttcggaaagggaccacagggtcccacttaatgctaagactagagcttgagaaagtccaggagatgttgccaggaggtcgccgcggagggggcttcatggtcgtggcgttggcagaagggctggcaggcccagtgccagcccggttgtaggccctcacggtcacatggtacttggtgttgggatgcaggccgctgactcgggcactggtgtccagccctgctgtcctcactcggtccgcagctgcttctttgtccccagctttccagtagcggatctcataccccaggaggataccattcatgtcctgctgcacgggttcccaggtcacgttcatctctgaggatgagacccctttggcccacaccttggtaggggccaccctgggctcttcctcagctgagtacacgagtgcagtgaggctctcgggcccatccccgcggcggttgtagctgcggatcttgacctcaaagggcgtgtagggccggacgctctcgttgctgtagacaaagtactgggcatcggcgccaggcacccgggcggtctgccagtgagtgctgccctgccgtccagttgacgatgagctctccgggggctccacctcctccgctgagtcctgagggtgccaccgagggggctgcttccctggtccggattttgctggagggcccactaggctccccagtgcccagaatgttgctggctatgacccggaactcatagtccatccagggggtgaggcccagcacctgtgcagtctcggcattgccctcgatgtttgcaggattggtccgaacctgcttccacttccctgcaggtggagtgcgagcttgcagggtgtacttagcgatggggctgtggttgtcgaagccacggctccagctgagctggatggtggtgtcgccaatgtccctcaccaccacacctcctgggggacctggcggacctcggaccaggactgtggcctccttggacgcgctgtccaccaccgtctgggccatgcacgtgtacttccccccatggcgcagctgggcgttcaggatggtcagatccccaatggtctccttcacattagttctccggtagtgccctccaggcttatcaaagtcgatggggaagtcgtccagggtccaggtgaaggtgaggtccatggtggggtcgtgggaggcatggcactgtagggtcaggttgtcacccaagttgatgtcggcacttgagggggctagagtgattttggttgcatctcgcacagataggattccagtgctgttggctttgcccatgaagttctcagcaaagcaggtgtatttgccttcatctgaccggctgatgtttcttatgatcaaggtgccatctggagttacagtcactctgctgctgttgaccaaaatctccgtgcctttgctccagagcaccacggcctttggagctgcccggggctggcaggggataaggatctctcccccgcgggccgcggggatcagacgcctcacgggattcagcctgaagtcaggggcgagtgcttgcacggctagctcggcgctggcgtagatggtaccgtgcttattctctgccacacactggtacatgcccgagtcttccaggctcagcttggagaaccgcaggtccccagccaacacctccacccggttctgggaggccagaggctccccgttccgcagccagcgcactgtaggccggggcttgccggcggctgcacagccccaacgcaggttggagccaatgtcagcctctgtgtccgagatcacttttagccactcaggctgagcctgcacgatgatgcggccctgcacggtgtctcggcccttggagttctccgcctcacactcgtaggtgccctcatcctcaaagctgacgctggggatctgcagggtgggctcagctgtggtccactgcggggacagggagccgtccactttgcgccacttgatccgggggacagggttcccaaaggcgaagcactccagggtgacctgctgccccaccagtgcataggtctctgctgggaaccgggccttgatgctgggtgcaaagagccgggtatcttcagcagccaggttgagctgagcaaacttgctgaagacgctcttggtggagaagtccatgtggctggtggccaaacaggagtagttgcccaggtctgaggcattggttcgggcaatgtacaggttccctgtggtctgggacacgaagtgacgcccgtccgtcgggatgaagttggggaactcgttgaggagccagcggtaggacaagcctgggtagtgggcaggtgggttacagggcaacatcaccccccagccttcatgagctttcactgggtctcgctcctccttggagaattcctgcagaaagccgaagcggaggatggcctccctgctgacaacggtgcccactgggttggaggccaggcactggtagaccccggcatcctgtgccttggtggggttcatgatgaccaggttgccccccaccagctggtgacgggaacctggctccagcttcatctcggtaccattcatcttccaccgataggtggctggagggctggcccgggcgcggcatgccagcaacacctgctcctccgtggactcctctgggaatagcacactgaggggctggtcttcaaagacaggcccgaaggtggtttgggatcccagggctgaactccaagctgaagaggagacaagggccacagcagctaccagcagcaggtgtggcttcctcctggtggctgtccccatggtggatgtccgggcagaggtggggatcggaggagaagagcctcagctcagcttggggacagcccagctggaggctgagaaaggacctggggcgagagaagggtgttggctggggcaggtggatgctgcccgagtcggtgagccggggccggccgggccgccagcccctgtctgggccgctgtcctttgggccctggcggcctcagccgctcgctgtccgggtgcggcggcggccgcggcggcggtggcgggtgagggcgcgtgtgtgt

SEQ ID NO: 18086 - RNA, 5231 nt, Homo sapiens
  source 1..5231: mol_type = other RNA
tctgggtgcagtgggggtttggctgtggcagggaaaaggcatgtgagcttatatttttaaaaaattgtagtgggtaaacatcaacataaacctgcccaggaaaatagagcaggacttaaaagtttaaaaaaccataacaaaatagagctctaactataaactacagaaaacaggctcggagcttccgaggacatatgcccttcaagatgcctgtcccgctgccccctgtgaagggccacctgtcggagcatgggctttggggtttcctagttgtgctgctgctcttgcctagggaatctgctcttgctttggcctcttttcttggggcaagagtgagggggacagggagcttcaagtcagccctccatgttgaagtttggtagaagctctgcccacaccttggacgggaacccagccatgccaatccccatgatcaccaatccgaaccccttgaagtagaattttcacaccctactgactaatcaccttcttagccaggccatagccattcagcagtgcctccttcctctgggtagacaaacagccttgaacagaaaggtggaagactcgagttcttaacccagccccatctcttctgggctgtgtgaccttgggaatcccagaccctctctggaccacctccatttcctcatctgtaaagtgaggggcttgaagaagttgagctctaaggcttcttccagctctgacgttctgtgactggtagtatacccagagctcaggaaaggatggcccatttattaacccctttttctccggggaaatgcaagcagtccaaggccgtctgggagcggatctggccaggtggtcctaggtatacctgggagcaggcagggccacatttatcctctgcccttcccagaaacctcccaataccaggacacacagcatgaatgctgcattcccctcccaggcaggagtgagtcagtgctgggagagcagagtctggggctgcaggtcggggaggccgagctgactgcaggcagcactggagaggtgggcgcatgattggccatctcctgcccaaaccctggagggactgtgcagaatgggtcttggaggggtgggagaccccaccaagacaagccctttagtcacccagccacctgaagtggcgctgtcaatcgggatgacagggtcaggttggcagtgttggctgagagggcatcgtcacctgggttgtgactatctcagaccaaggctggtgcccctttccaccaagggccctggcctctcaactctttttggctcccaccccaaacagcctggagtatcacccccctcaaagctgaaggggctcaggctcccagcctcaggcatcggggcgctggttctcagccgcttgggcaggcaggagcccctagggagttatcggggacagcgtcagggtccttgctgctgctcgagggagaaggcgggagagctcttggtcccagggcttgcccttcttccttagactgaaggatggtgaggtgtgcacttcgctccagttcttcaacctgttcatgtctggtgttcctgccgggcctaggactgctctcaagtggcggagtccgtatagggtcccagagggccatctctgctgagttgaagacatgtttttaaaacccccttcttcccatgggcctgttccttccctccaggcagcctagagctcaggtataggcgtcagtgtcatcatggaagttactgcctggtgcctctcaatttaaagaaaatccttgcgtgggttctatcctgcggcagaatataaaatatcctacctcctacaaaaagggcactgtttaaagtaggtatttaaaaccagccactctctggcacagtgtcaggccaccttggcagcaggaaggggctggctgtgtccgtcggaggtggcgtccagctgcggcgcagagggaggggttccaggatcagagctccagggagcctatgaggatcagcatcgccacggagtgggaaatgacggtgccagggtgtggtgctgggcggactgccatgttctccaccatcatgcttgtgcctccattcctcacgatgtggacttctgcagggatcccatcccctccgggccctgtggtccgaatttgtaccagggcatggccaatgtcttcaggcactgggatttctatccagttcttgccggtgaggtggagcgtgggagtcaggtgtaagtcattctggtacagcatcttatagccggtgactgcagactcatttcggaaagggaccacagggtcccacttaatgctaagactagagcttgagaaagtccaggagatgttgccaggaggtcgccgcggagggggcttcatggtcgtggcgttggcagaagggctggcaggcccagtgccagcccggttgtaggccctcacggtcacatggtacttggtgttgggatgcaggccgctgactcgggcactggtgtccagccctgctgtcctcactcggtccgcagctgcttctttgtccccagctttccagtagcggatctcataccccaggaggataccattcatgtcctgctgcacgggttcccaggtcacgttcatctctgaggatgagacccctttggcccacaccttggtaggggccaccctgggctcttcctcagctgagtacacgagtgcagtgaggctctcgggcccatccccgcggcggttgtagctgcggatcttgacctcaaagggcgtgtagggccggacgctctcgttgctgtagacaaagtactgggcatcggcgccaggcacccgggcggtctgccagtgagtgctgccctgcctgcggaaggacagcaggtagccgaagccgtctccgttctggtactcccgtgacatgggcgtccagttgacgatgagctctccgggggctccacctcctccgctgagtcctgagggtgccaccgagggggctgcttccctggtccggattttgctggagggcccactaggctccccagtgcccagaatgttgctggctatgacccggaactcatagtccatccagggggtgaggcccagcacctgtgcagtctcggcattgccctcgatgtttgcaggattggtccgaacctgcttccacttccctgcaggtggagtgcgagcttgcagggtgtacttagcgatggggctgtggttgtcgaagccacggctccagctgagctggatggtggtgtcgccaatgtccctcaccaccacacctcctgggggacctggcggacctcggaccaggactgtggcctccttggacgcgctgtccaccaccgtctgggccatgcacgtgtacttccccccatggcgcagctgggcgttcaggatggtcagatccccaatggtctccttcacattagttctccggtagtgccctccaggcttatcaaagtcgatggggaagtcgtccagggtccaggtgaaggtgaggtccatggtggggtcgtgggaggcatggcactgtagggtcaggttgtcacccaagttgatgtcggcacttgagggggctagagtgattttggttgcatctcgcacagataggattccagtgctgttggctttgcccatgaagttctcagcaaagcaggtgtatttgccttcatctgaccggctgatgtttcttatgatcaaggtgccatctggagttacagtcactctgctgctgttgaccaaaatctccgtgcctttgctccagagcaccacggcctttggagctgcccggggctggcaggggataaggatctctcccccgcgggccgcggggatcagacgcctcacgggattcagcctgaagtcaggggcgagtgcttgcacggctagctcggcgctggcgtagatggtaccgtgcttattctctgccacacactggtacatgcccgagtcttccaggctcagcttggagaaccgcaggtccccagccaacacctccacccggttctgggaggccagaggctccccgttccgcagccagcgcactgtaggccggggcttgccggcggctgcacagccccaacgcaggttggagccaatgtcagcctctgtgtccgagatcacttttagccactcaggctgagcctgcacgatgatgcggccctgcacggtgtctcggcccttggagttctccgcctcacactcgtaggtgccctcatcctcaaagctgacgctggggatctgcagggtgggctcagctgtggtccactgcggggacagggagccgtccactttgcgccacttgatccgggggacagggttcccaaaggcgaagcactccagggtgacctgctgccccaccagtgcataggtctctgctgggaaccgggccttgatgctgggtgcaaagagccgggtatcttcagcagccaggttgagctgagcaaacttgctgaagacgctcttggtggagaagtccatgtggctggtggccaaacaggagtagttgcccaggtctgaggcattggttcgggcaatgtacaggttccctgtggtctgggacacgaagtgacgcccgtccgtcgggatgaagttggggaactcgttgaggagccagcggtaggacaagcctgggtagtgggcaggtgggttacagggcaacatcaccccccagccttcatgagctttcactgggtctcgctcctccttggagaattcctgcagaaagccgaagcggaggatggcctccctgctgacaacggtgcccactgggttggaggccaggcactggtagaccccggcatcctgtgccttggtggggttcatgatgaccaggttgccccccaccagctggtgacgggaacctggctccagcttcatctcggtaccattcatcttccaccgataggtggctggagggctggcccgggcgcggcatgccagcaacacctgctcctccgtggactcctctgggaatagcacactgaggggctggtcttcaaagacaggcccgaaggtggtttgggatcccagggctgaactccaagctgaagaggagacaagggccacagcagctaccagcagcaggtgtggcttcctcctggtggctgtccccatggtggatgtccgggcagaggtggggatcggaggagaagagcctcagctcagcttggggacagcccagctggaggctgagaaaggacctcatttgctgtcatttaaggaccagggagcgagcccagcgcgcgtcttccataatgcatgggccgctcatggacaggccgcggggcgctgtct

SEQ ID NO: 18087 - RNA, 5320 nt, Homo sapiens
  source 1..5320: mol_type = other RNA
tctgggtgcagtgggggtttggctgtggcagggaaaaggcatgtgagcttatatttttaaaaaattgtagtgggtaaacatcaacataaacctgcccaggaaaatagagcaggacttaaaagtttaaaaaaccataacaaaatagagctctaactataaactacagaaaacaggctcggagcttccgaggacatatgcccttcaagatgcctgtcccgctgccccctgtgaagggccacctgtcggagcatgggctttggggtttcctagttgtgctgctgctcttgcctagggaatctgctcttgctttggcctcttttcttggggcaagagtgagggggacagggagcttcaagtcagccctccatgttgaagtttggtagaagctctgcccacaccttggacgggaacccagccatgccaatccccatgatcaccaatccgaaccccttgaagtagaattttcacaccctactgactaatcaccttcttagccaggccatagccattcagcagtgcctccttcctctgggtagacaaacagccttgaacagaaaggtggaagactcgagttcttaacccagccccatctcttctgggctgtgtgaccttgggaatcccagaccctctctggaccacctccatttcctcatctgtaaagtgaggggcttgaagaagttgagctctaaggcttcttccagctctgacgttctgtgactggtagtatacccagagctcaggaaaggatggcccatttattaacccctttttctccggggaaatgcaagcagtccaaggccgtctgggagcggatctggccaggtggtcctaggtatacctgggagcaggcagggccacatttatcctctgcccttcccagaaacctcccaataccaggacacacagcatgaatgctgcattcccctcccaggcaggagtgagtcagtgctgggagagcagagtctggggctgcaggtcggggaggccgagctgactgcaggcagcactggagaggtgggcgcatgattggccatctcctgcccaaaccctggagggactgtgcagaatgggtcttggaggggtgggagaccccaccaagacaagccctttagtcacccagccacctgaagtggcgctgtcaatcgggatgacagggtcaggttggcagtgttggctgagagggcatcgtcacctgggttgtgactatctcagaccaaggctggtgcccctttccaccaagggccctggcctctcaactctttttggctcccaccccaaacagcctggagtatcacccccctcaaagctgaaggggctcaggctcccagcctcaggcatcggggcgctggttctcagccgcttgggcaggcaggagcccctagggagttatcggggacagcgtcagggtccttgctgctgctcgagggagaaggcgggagagctcttggtcccagggcttgcccttcttccttagactgaaggatggtgaggtgtgcacttcgctccagttcttcaacctgttcatgtctggtgttcctgccgggcctaggactgctctcaagtggcggagtccgtatagggtcccagagggccatctctgctgagttgaagacatgtttttaaaacccccttcttcccatgggcctgttccttccctccaggcagcctagagctcaggtataggcgtcagtgtcatcatggaagttactgcctggtgcctctcaatttaaagaaaatccttgcgtgggttctatcctgcggcagaatataaaatatcctacctcctacaaaaagggcactgtttaaagtaggtatttaaaaccagccactctctggcacagtgtcaggccaccttggcagcaggaaggggctggctgtgtccgtcggaggtggcgtccagctgcggcgcagagggaggggttccaggatcagagctccagggagcctatgaggatcagcatcgccacggagtgggaaatgacggtgccagggtgtggtgctgggcggactgccatgttctccaccatcatgcttgtgcctccattcctcacgatgtggacttctgcagggatcccatcccctccgggccctgtggtccgaatttgtaccagggcatggccaatgtcttcaggcactgggatttctatccagttcttgccggtgaggtggagcgtgggagtcaggtgtaagtcattctggtacagcatcttatagccggtgactgcagactcatttcggaaagggaccacagggtcccacttaatgctaagactagagcttgagaaagtccaggagatgttgccaggaggtcgccgcggagggggcttcatggtcgtggcgttggcagaagggctggcaggcccagtgccagcccggttgtaggccctcacggtcacatggtacttggtgttgggatgcaggccgctgactcgggcactggtgtccagccctgctgtcctcactcggtccgcagctgcttctttgtccccagctttccagtagcggatctcataccccaggaggataccattcatgtcctgctgcacgggttcccaggtcacgttcatctctgaggatgagacccctttggcccacaccttggtaggggccaccctgggctcttcctcagctgagtacacgagtgcagtgaggctctcgggcccatccccgcggcggttgtagctgcggatcttgacctcaaagggcgtgtagggccggacgctctcgttgctgtagacaaagtactgggcatcggcgccaggcacccgggcggtctgccagtgagtgctgccctgcctgcggaaggacagcaggtagccgaagccgtctccgttctggtactcccgtgacatgggcgtccagttgacgatgagctctccgggggctccacctcctccgctgagtcctgagggtgccaccgagggggctgcttccctggtccggattttgctggagggcccactaggctccccagtgcccagaatgttgctggctatgacccggaactcatagtccatccagggggtgaggcccagcacctgtgcagtctcggcattgccctcgatgtttgcaggattggtccgaacctgcttccacttccctgcaggtggagtgcgagcttgcagggtgtacttagcgatggggctgtggttgtcgaagccacggctccagctgagctggatggtggtgtcgccaatgtccctcaccaccacacctcctgggggacctggcggacctcggaccaggactgtggcctccttggacgcgctgtccaccaccgtctgggccatgcacgtgtacttccccccatggcgcagctgggcgttcaggatggtcagatccccaatggtctccttcacattagttctccggtagtgccctccaggcttatcaaagtcgatggggaagtcgtccagggtccaggtgaaggtgaggtccatggtggggtcgtgggaggcatggcactgtagggtcaggttgtcacccaagttgatgtcggcacttgagggggctagagtgattttggttgcatctcgcacagataggattccagtgctgttggctttgcccatgaagttctcagcaaagcaggtgtatttgccttcatctgaccggctgatgtttcttatgatcaaggtgccatctggagttacagtcactctgctgctgttgaccaaaatctccgtgcctttgctccagagcaccacggcctttggagctgcccggggctggcaggggataaggatctctcccccgcgggccgcggggatcagacgcctcacgggattcagcctgaagtcaggggcgagtgcttgcacggctagctcggcgctggcgtagatggtaccgtgcttattctctgccacacactggtacatgcccgagtcttccaggctcagcttggagaaccgcaggtccccagccaacacctccacccggttctgggaggccagaggctccccgttccgcagccagcgcactgtaggccggggcttgccggcggctgcacagccccaacgcaggttggagccaatgtcagcctctgtgtccgagatcacttttagccactcaggctgagcctgcacgatgatgcggccctgcacggtgtctcggcccttggagttctccgcctcacactcgtaggtgccctcatcctcaaagctgacgctggggatctgcagggtgggctcagctgtggtccactgcggggacagggagccgtccactttgcgccacttgatccgggggacagggttcccaaaggcgaagcactccagggtgacctgctgccccaccagtgcataggtctctgctgggaaccgggccttgatgctgggtgcaaagagccgggtatcttcagcagccaggttgagctgagcaaacttgctgaagacgctcttggtggagaagtccatgtggctggtggccaaacaggagtagttgcccaggtctgaggcattggttcgggcaatgtacaggttccctgtggtctgggacacgaagtgacgcccgtccgtcgggatgaagttggggaactcgttgaggagccagcggtaggacaagcctgggtagtgggcaggtgggttacagggcaacatcaccccccagccttcatgagctttcactgggtctcgctcctccttggagaattcctgcagaaagccgaagcggaggatggcctccctgctgacaacggtgcccactgggttggaggccaggcactggtagaccccggcatcctgtgccttggtggggttcatgatgaccaggttgccccccaccagctggtgacgggaacctggctccagcttcatctcggtaccattcatcttccaccgataggtggctggagggctggcccgggcgcggcatgccagcaacacctgctcctccgtggactcctctgggaatagcacactgaggggctggtcttcaaagacaggcccgaaggtggtttgggatcccagggctgaactccaagctgaagaggagacaagggccacagcagctaccagcagcaggtgtggcttcctcctggtggctgtccccatggtggatgtccgggcagaggtggggatcggaggagaagagcctcagctcagcttggggacagcccagctggaggctgagaaaggacctggggcgagagaagggtgttggctggggcaggtggatgctgcccgagtcggtgagccggggccggccgggccgccagcccctgtctgggccgctgtcctttgggccctggcggcctcagccgctcgctgtccgggtgcggcggcggccgcggcggcggtggcgggtgagggcgcgtgtgtgt

SEQ ID NO: 18088 - RNA, 6076 nt, Homo sapiens
  source 1..6076: mol_type = other RNA
tctgggtgcagtgggggtttggctgtggcagggaaaaggcatgtgagcttatatttttaaaaaattgtagtgggtaaacatcaacataaacctgcccaggaaaatagagcaggacttaaaagtttaaaaaaccataacaaaatagagctctaactataaactacagaaaacaggctcggagcttccgaggacatatgcccttcaagatgcctgtcccgctgccccctgtgaagggccacctgtcggagcatgggctttggggtttcctagttgtgctgctgctcttgcctagggaatctgctcttgctttggcctcttttcttggggcaagagtgagggggacagggagcttcaagtcagccctccatgttgaagtttggtagaagctctgcccacaccttggacgggaacccagccatgccaatccccatgatcaccaatccgaaccccttgaagtagaattttcacaccctactgactaatcaccttcttagccaggccatagccattcagcagtgcctccttcctctgggtagacaaacagccttgaacagaaaggtggaagactcgagttcttaacccagccccatctcttctgggctgtgtgaccttgggaatcccagaccctctctggaccacctccatttcctcatctgtaaagtgaggggcttgaagaagttgagctctaaggcttcttccagctctgacgttctgtgactggtagtatacccagagctcaggaaaggatggcccatttattaacccctttttctccggggaaatgcaagcagtccaaggccgtctgggagcggatctggccaggtggtcctaggtatacctgggagcaggcagggccacatttatcctctgcccttcccagaaacctcccaataccaggacacacagcatgaatgctgcattcccctcccaggcaggagtgagtcagtgctgggagagcagagtctggggctgcaggtcggggaggccgagctgactgcaggcagcactggagaggtgggcgcatgattggccatctcctgcccaaaccctggagggactgtgcagaatgggtcttggaggggtgggagaccccaccaagacaagccctttagtcacccagccacctgaagtggcgctgtcaatcgggatgacagggtcaggttggcagtgttggctgagagggcatcgtcacctgggttgtgactatctcagaccaaggctggtgcccctttccaccaagggccctggcctctcaactctttttggctcccaccccaaacagcctggagtatcacccccctcaaagctgaaggggctcaggctcccagcctcaggcatcggggcgctggttctcagccgcttgggcaggcaggagcccctagggagttatcggggacagcgtcagggtccttgctgctgctcgagggagaaggcgggagagctcttggtcccagggcttgcccttcttccttagactgaaggatggtgaggtgtgcacttcgctccagttcttcaacctgttcatgtctggtgttcctgccgggcctaggactgctctcaagtggcggagtccgtatagggtcccagagggccatctctgctgagttgaagacatgtttttaaaacccccttcttcccatgggcctgttccttccctccaggcagcctagagctcaggtataggcgtcagtgtcatcatggaagttactgcctggtgcctctcaatttaaagaaaatccttgcgtgggttctatcctgcggcagaatataaaatatcctacctcctacaaaaagggcactgtttaaagtaggtatttaaaaccagccactctctggcacagtgtcaggccaccttggcagcaggaaggggctggctgtgtccgtcggaggtggcgtccagctgcggcgcagagggaggggttccaggatcagagctccagggagcctatgaggatcagcatcgccacggagtgggaaatgacggtgccagggtgtggtgctgggcggactgccatgttctccaccatcatgcttgtgcctccattcctcacgatgtggacttctgcagggatcccatcccctccgggccctgtggtccgaatttgtaccagggcatggccaatgtcttcaggcactgggatttctatccagttcttgccggtgaggtggagcgtgggagtcaggtgtaagtcattctggtacagcatcttatagccggtgactgcagactcatttcggaaagggaccacagggtcccacttaatgctaagactagagcttgagaaagtccaggagatgttgccaggaggtcgccgcggagggggcttcatggtcgtggcgttggcagaagggctggcaggcccagtgccagcccggttgtaggccctcacggtcacatggtacttggtgttgggatgcaggccgctgactcgggcactggtgtccagccctgctgtcctcactcggtccgcagctgcttctttgtccccagctttccagtagcggatctcataccccaggaggataccattcatgtcctgctgcacgggttcccaggtcacgttcatctctgaggatgagacccctttggcccacaccttggtaggggccaccctgggctcttcctcagctgagtacacgagtgcagtgaggctctcgggcccatccccgcggcggttgtagctgcggatcttgacctcaaagggcgtgtagggccggacgctctcgttgctgtagacaaagtactgggcatcggcgccaggcacccgggcggtctgccagtgagtgctgccctgcctgcggaaggacagcaggtagccgaagccgtctccgttctggtactcccgtgacatgggcgtccagttgacgatgagctctccgggggctccacctcctccgctgagtcctgagggtgccaccgagggggctgcttccctggtccggattttgctggagggcccactaggctccccagtgcccagaatgttgctggctatgacccggaactcatagtccatccagggggtgaggcccagcacctgtgcagtctcggcattgccctcgatgtttgcaggattggtccgaacctgcttccacttccctgcaggtggagtgcgagcttgcagggtgtacttagcgatggggctgtggttgtcgaagccacggctccagctgagctggatggtggtgtcgccaatgtccctcaccaccacacctcctgggggacctggcggacctcggaccaggactgtggcctccttggacgcgctgtccaccaccgtctgggccatgcacgtgtacttccccccatggcgcagctgggcgttcaggatggtcagatccccaatggtctccttcacattagttctccggtagtgccctccaggcttatcaaagtcgatggggaagtcgtccagggtccaggtgaaggtgaggtccatggtggggtcgtgggaggcatggcactgtagggtcaggttgtcacccaagttgatgtcggcacttgagggggctagagtgattttggttgcatctcgcacagataggattccagtgctgttggctttgcccatgaagttctcagcaaagcaggtgtatttgccttcatctgaccggctgatgtttcttatgatcaaggtgccatctggagttacagtcactctgctgctgttgaccaaaatctccgtgcctttgctccagagcaccacggcctttggagctgcccggggctggcaggggataaggatctctcccccgcgggccgcggggatcagacgcctcacgggattcagcctgaagtcaggggcgagtgcttgcacggctagctcggcgctggcgtagatggtaccgtgcttattctctgccacacactggtacatgcccgagtcttccaggctcagcttggagaaccgcaggtccccagccaacacctccacccggttctgggaggccagaggctccccgttccgcagccagcgcactgtaggccggggcttgccggcggctgcacagccccaacgcaggttggagccaatgtcagcctctgtgtccgagatcacttttagccactcaggctgagcctgcacgatgatgcggccctgcacggtgtctcggcccttggagttctccgcctcacactcgtaggtgccctcatcctcaaagctgacgctggggatctgcagggtgggctcagctgtggtccactgcggggacagggagccgtccactttgcgccacttgatccgggggacagggttcccaaaggcgaagcactccagggtgacctgctgccccaccagtgcataggtctctgctgggaaccgggccttgatgctgggtgcaaagagccgggtatcttcagcagccaggttgagctgagcaaacttgctgaagacgctcttggtggagaagtccatgtggctggtggccaaacaggagtagttgcccaggtctgaggcattggttcgggcaatgtacaggttccctgtggtctgggacacgaagtgacgcccgtccgtcgggatgaagttggggaactcgttgaggagccagcggtaggacaagcctgggtagtgggcaggtgggttacagggcaacatcaccccccagccttcatgagctttcactgggtctcgctcctccttggagaattcctgcagaaagccgaagcggaggatggcctccctgctgacaacggtgcccactgggttggaggccaggcactggtagaccccggcatcctgtgccttggtggggttcatgatgaccaggttgccccccaccagctggtgacgggaacctggctccagcttcatctcggtaccattcatcttccaccgataggtggctggagggctggcccgggcgcggcatgccagcaacacctgctcctccgtggactcctctgggaatagcacactgaggggctggtcttcaaagacaggcccgaaggtggtttgggatcccagggctgaactccaagctgcaggtgatgacaccaccagatgcctcagagccttggcctggctggagcctggcctcttgggctgtgctgtccagtaaaactttctctgatgatgggaatgtcccattttctgcactgttcaatgtggtaaccactagccacgtagggctatcgagcacttgacatgtggctattgcgactgaagaacgacattttacattttatattacttaattaatttaaatttgaatttaaataggctgggcaggccccatctggccatactagttcaatcaatcacccatcctacacttaggtattgagcacctgctctatacccagcactgggctagagactggcttgtaaagatgattaagacacagtccctcttcttcaaggggcttgcggtccaaggagggagacaggaaattgacagtgcaaggtagcaaatgccataaagttcaagatgctggggcctcagaatggaagcagttctacctcccagggggctttcaagggacccttacagaagaactgatctgtggggtgtgaggtgcatgagacgtcgccagccacaaacatgcagagaggatgtgtgtccctggagcctaatacccttactggggcagtgtggaccaacgaggcctgggcctggggactaggctggccctctactagctgtgggaccttgggaaagttatagaactcttctgagcctcagtatcttcacctgaagaggagacaagggccacagcagctaccagcagcaggtgtggcttcctcctggtggctgtccccatggtggatgtccgggcagaggtggggatcggaggagaagagcctcagctcagcttggggacagcccagctggaggctgagaaaggacctggggcgagagaagggtgttggctggggcaggtggatgctgcccgagtcggtgagccggggccggccgggccgccagcccctgtctgggccgctgtcctttgggccctggcggcctcagccgctcgctgtccgggtgcggcggcggccgcggcggcggtggcgggtgagggcgcgtgtgtgtgagcgcgcccggagccactgcagcatctctgcatcaagatgtg

SEQ ID NO: 18089 - RNA, 1666 nt, Homo sapiens
  source 1..1666: mol_type = other RNA
tctggtcctggacaggaggcaatttcttagccgaatcccaggactcacgagtgcccttggattcgtttgctttcctttgtttatctccaagtgcagtggtggcagattttccagtctttttcttttgcttccgcaactgatcgtaggtgaggtatttttcacatgacagagtgggctgctcgaattcctcagccatatctacctcctccacctcagagagggagctcacggacgttctgtccaaatgagcagtcggtggcttcccctcttgagtctctcggtcgttggaaagctgctctttctcctcgggcgacaggccgtgtgtcccatttcctgggtcccggccgtctagactgggcctcttcttgttcgagtgactgtgctgaggcctcttctggtgactgtctggagcctcctccaaggcagggacacgctggccgctgccagcttgccccccttccttgtctgtcttgaagtccgaaggctgcctgtccctggcacttgcccaggagggcatccttggggtttcctctcttaagcaggccccgcatgatttctccctgatcaaagtaggggagtgccaatctccctgggcacacaaggggcgtttttcctggcgagacgatttgtgccccttgctgtggctcacaacggctttcccctggggttggccctggcagcctggacacagcagaggcccgccctgagccgcgtgagtgtggcctcttccgggttgcttcccgggcgcagcgggctcagggccctcgggcatccggaggggagctgtgcgcgttggagaggcccgatagcggccggaatcagctggggctattctggggcactttctctcagctctgggctcgcgactgtgagacctcgggtgaggtctctgttgccccggaggtgttctgcgtgctgtccgtctgtgctcagggctgtgagatgggctcctgggggccgtcgcgttttctgggaagccccaggccttttcctggtcctgaagagcctccccgaagcgctgtcgggaagcgctctcctcagggtcctgtgggccaggccgggtgtttcggtccacgagcaccagcttcttccaccgggccgctaagtctctggcaaagtcgcccacgtgctggtgcttccgcaggcgcttcaccgtctttctgattccagtctccgccaggatgtctgccgtcatgggcaaggcggagagtttctgcaaatatttctctagctttttcggctccgtcttagtggccagacgcacctgcagcttctccactgcgtgcagcgtagtggaccctgccgccatctcaccagagctgtgcaggcgtcgctgtcccggcggtcgcagctctgtctttggggctgcgggacaggaagtctggggtggccggtcctcgctgcccggtcgccaggcagcgacctcgggatgtggagtcacagcctggagcgagctgggtcctcggagcagcaggccacttggtctggaacggccgtccttgcagacagctgagcaggcccgcttttgttcctcgggatgtggagccacagcctggagtgacctctgcagtttgctgtgcaacaaagaatgaagctctggtgccagagctgggccttatgtagcccatcccaggctgacactcacggctctagccctgaccctctt

SEQ ID NO: 18090 - RNA, 113 nt, Homo sapiens
  source 1..113: mol_type = other RNA
tctgtagcctgggagcaatggggtgtcggtgtcaggggacgtgatgggggaggcaagggagacagagagaaggggacgaggcccagacgccgacagggggtgggggcggagag

SEQ ID NO: 18091 - RNA, 68 nt, Homo sapiens
  source 1..68: mol_type = other RNA
tctgtgatagagattctttgctttgttagaaacaaaaagcaaagaatctctatcacagaaaaaagata

SEQ ID NO: 18092 - RNA, 67 nt, Homo sapiens
  source 1..67: mol_type = other RNA
tctgtgatagagattctttgctttttgtttctaacaaagcaaagaatctctatcacagaaaaaagac

SEQ ID NO: 18093 - RNA, 1791 nt, Homo sapiens
  source 1..1791: mol_type = other RNA
tctgtgctactggatgaagagtgcattctagtctctgctgaccttagacgctggttctaagtagttcattcatagtagaaactctgctcttttggacctgtctgatcaacctaagggaaaaggatggaatatagtcctagcatagaaccagcgtgttgtgcagggaaactgaggcccagtctcctaacttcagataaggtggcatgaaggagggaagggatttggtgagcaggccagtcctaggggtccattcaggaaagccaacttccagggccagtatgtacagctgtgtgagtgcataattccagggataagaatgttcatgttgtgcttggcgtggtgcagtgcataacctgcacaactgtatatgatgatcctccttggaattcacgctaccacaattctggtccctacttattggtaggaatgatgacttgctaatcccagtgacaggccggtcccaattctacattctccaaggctgatctcaggaactggagaaggctgagggctgaggtcatgatggagaattgacttctcgaagggatgtttgagggatgaatagcaaacatttcttatctttgcagctcttgaaggtgtgtagctacctttgtaaacccaatggcagaaccaactgtataatttagttcctggtgcaaaataaaactgtgaaccccttacttgaaaagcaggaaaaaagtattattaaagggactaaagcataagccgttttcatttttttcagcagattctctcattttgtagtgttttttatttgtatttttcatgtttttctaactaaaaaataagctttaaattattagcgtggattttactgtttatgttgtgccatgacaattttaaatttggctatagtagcaattaactcttacataaaattacccaaatttcacagttcatatgttgcagttcctatgtgtccatgaatttagttcttaccaggacactggaaatgctgcacgaaacaagctcacctgttttcctttcacttcttgatacgtgcacgtttcatccgcactctttaccttcctctcacagggaatgagggggactgagaggaacgggaaatctgggccctgccctcccctttcctcctaaacaccaatttcaatgggcatagttggccaatgcagggaagcaacacgagtaaggaaggatgtgagggggtcccttgccctggtgtctgttagaatcctggtgccttctttcttcatttgatgcaaatcctggtttggatagaaaatatgacttaccttggactcactttgagcctctctgaactcccatgctggcgggtccctcacaattccacattcatggggcatctggggcatcatgagcatgctgcattaatgggcagcaaggaaaggtgaacacacccattgcacttccctcctccgctcacggacacgctccagtgtgccatcagatttcacgggttcccagccccaaggaaacacttctctgctctgttatctgttgctggagttgccctttatgaaatccatttcccaggctgcggtatccttggcttcctgttgcgttgtgccaatggaagtcacaggaaggagacaggaagttaggaggagtaaaaagaactttattcttggtgtttcttattccttttcagtgttgctccagcagcagcagcaattgactctatctctaccttctttctccattcccagaaccagacttctcacagcttcttagacccacaaacagcagctgataagaccttctttgcagggctctgccctcttttgagtc

SEQ ID NO: 18094 - RNA, 1051 nt, Homo sapiens
  source 1..1051: mol_type = other RNA
tctgtgctactggatgaagagttttttaatggttacgagaagtgaagtccattcttctcttctctcattctgcaccaccactttgtaaaagtcttcatagaatctccccttgtgatcctgtcgaattgaggctcggtttatttcaggaaattcatcaacagattttgcatcatagaaagttctagaaaacaggaccactgtcacttcatgactacagttcttctccttccacttggtaaatagatcagcaaggaaaccattcacagctttctcaaaatacaaatccccataaatatcaaaatcccacatttcacagctcatctgaataaatatgtaaaccatagccgacgtagaacgaaacaccaccctggtatcttcactgatgtagccacacatgaccttctcattcttaacccacagttcaccagcctgtgctctgatgccagcaaactccaccttctgggtgatataggcacatgtgctgaccaaacttttctttagtcgccacatatccccacggccaatatactgatccttaaaagttaattccactaggtcaagggtcacatccttagggtctacgacattaacatagacatcctgataaggtctcagccggaacacttgagtcacagtctggtccacactgatagtttccttctgtaaatcttccttaagagacttgacctgcaaaagcagagggctgtattcatcgttggggtgtgcaatctctacaatgtctccaagcttgatgtgagggaacactttggggttcacaactagctcatcatcactgcccccaaagcccttcttgtggatgacgagtttgtagacctttgttgttctcatcttgcactgtttttccctttagctgttccaagcttggggcagagaagtcatcttgcctcccgaagctctagagccccttcccgcctctggccggggcactgagggctggaccctctccaggttccctgcgcctcctccagataccccgcctacgcccgcgcggcccgcgctgttccgcccctaagcctgaagcgcctactag

SEQ ID NO: 18095 - RNA, 1055 nt, Homo sapiens
  source 1..1055: mol_type = other RNA
tctgtgctactggatgaagagttttttaatggttacgagaagtgaagtccattcttctcttctctcattctgcaccaccactttgtaaaagtcttcatagaatctccccttgtgatcctgtcgaattgaggctcggtttatttcaggaaattcatcaacagattttgcatcatagaaagttctagaaaacaggaccactgtcacttcatgactacagttcttctccttccacttggtaaatagatcagcaaggaaaccattcacagctttctcaaaatacaaatccccataaatatcaaaatcccacatttcacagctcatctgaataaatatgtaaaccatagccgacgtagaacgaaacaccaccctggtatcttcactgatgtagccacacatgaccttctcattcttaacccacagttcaccagcctgtgctctgatgccagcaaactccaccttctgggtgatataggcacatgtgctgaccaaacttttctttagtcgccacatatccccacggccaatatactgatccttaaaagttaattccactaggtcaagggtcacatccttagggtctacgacattaacatagacatcctgataaggtctcagccggaacacttgagtcacagtctggtccacactgatagtttccttctgtaaatcttccttaagagacttgacctgcaaaagcagagggctgtattcatcgttggggtgtgcaatctctacaatgtctccaagcttgatgtgagggaacactttggggttcacaactagctcatcatcactgcccccaaagcccttcttgtggatgacgagtttgtagacctttgttgttctcatcttgcactgtttttccctttagctgttccaagcttggggcagagaagtcatcttgcctcccgaagctctagagccccttcccgcctctggccggggcactgagggctggaccctctccaggttccctgcgcctcctccagataccccgcctacgcccgcgcggcccgcgctgttccgcccctaagcctgaagcgcctactaggccc

SEQ ID NO: 18096 - RNA, 1058 nt, Homo sapiens
  source 1..1058: mol_type = other RNA
tctgtgctactggatgaagagttttttaatggttacgagaagtgaagtccattcttctcttctctcattctgcaccaccactttgtaaaagtcttcatagaatctccccttgtgatcctgtcgaattgaggctcggtttatttcaggaaattcatcaacagattttgcatcatagaaagttctagaaaacaggaccactgtcacttcatgactacagttcttctccttccacttggtaaatagatcagcaaggaaaccattcacagctttctcaaaatacaaatccccataaatatcaaaatcccacatttcacagctcatctgaataaatatgtaaaccatagccgacgtagaacgaaacaccaccctggtatcttcactgatgtagccacacatgaccttctcattcttaacccacagttcaccagcctgtgctctgatgccagcaaactccaccttctgggtgatataggcacatgtgctgaccaaacttttctttagtcgccacatatccccacggccaatatactgatccttaaaagttaattccactaggtcaagggtcacatccttagggtctacgacattaacatagacatcctgataaggtctcagccggaacacttgagtcacagtctggtccacactgatagtttccttctgtaaatcttccttaagagacttgacctgcaaaagcagagggctgtattcatcgttggggtgtgcaatctctacaatgtctccaagcttgatgtgagggaacactttggggttcacaactagctcatcatcactgcccccaaagcccttcttgtggatgacgagtttgtagacctttgttgttctcatcttgcactgtttttccctttagctgttccaagcttggggcagagaagtcatcttgcctcccgaagctctagagccccttcccgcctctggccggggcactgagggctggaccctctccaggttccctgcgcctcctccagataccccgcctacgcccgcgcggcccgcgctgttccgcccctaagcctgaagcgcctactaggcccgcc

SEQ ID NO: 18097 - RNA, 938 nt, Homo sapiens
  source 1..938: mol_type = other RNA
tctgtgctactggatgaagagttttttaatggttacgagaagtgaagtccattcttctcttctctcattctgcaccaccactttgtaaaagtcttcatagaatctccccttgtgatcctgtcgaattgaggctcggtttatttcaggaaattcatcaacagattttgcatcatagaaagttctagaaaacaggaccactgtcacttcatgactacagttcttctccttccacttggtaaatagatcagcaaggaaaccattcacagctttctcaaaatacaaatccccataaatatcaaaatcccacatttcacagctcatctgaataaatatgtaaaccatagccgacgtagaacgaaacaccaccctggtatcttcactgatgtagccacacatgaccttctcattcttaacccacagttcaccagcctgtgctctgatgccagcaaactccaccttctgggtgatataggcacatgtgctgaccaaacttttctttagtcgccacatatccccacggccaatatactgatccttaaaagttaattccactaggtcaagggtcacatccttagggtctacgacattaacatagacatcctgataaggtctcagccggaacacttgagtcacagtctggtccacactgatagtttccttctgtaaatcttccttaagagacttgacctgcaaaagcagagggctgtattcatcgttggggtgtgcaatctctacaatgtctccaagcttgatgtgagggaacactttggggttcacaactagctcatcatcactgcccccaaagcccttcttgtggatgacgagtttgtagacctttgttgttctcatcttgcactgtttttccctttagctgttccaagcttggggcagagaagtcatcttgcctccctgagaacccgcgccgctccggtggctcc

SEQ ID NO: 18098 - RNA, 967 nt, Homo sapiens
  source 1..967: mol_type = other RNA
tctgtgctactggatgaagagttttttaatggttacgagaagtgaagtccattcttctcttctctcattctgcaccaccactttgtaaaagtcttcatagaatctccccttgtgatcctgtcgaattgaggctcggtttatttcaggaaattcatcaacagattttgcatcatagaaagttctagaaaacaggaccactgtcacttcatgactacagttcttctccttccacttggtaaatagatcagcaaggaaaccattcacagctttctcaaaatacaaatccccataaatatcaaaatcccacatttcacagctcatctgaataaatatgtaaaccatagccgacgtagaacgaaacaccaccctggtatcttcactgatgtagccacacatgaccttctcattcttaacccacagttcaccagcctgtgctctgatgccagcaaactccaccttctgggtgatataggcacatgtgctgaccttagggtctacgacattaacatagacatcctgataaggtctcagccggaacacttgagtcacagtctggtccacactgatagtttccttctgtaaatcttccttaagagacttgacctgcaaaagcagagggctgtattcatcgttggggtgtgcaatctctacaatgtctccaagcttgatgtgagggaacactttggggttcacaactagctcatcatcactgcccccaaagcccttcttgtggatgacgagtttgtagacctttgttgttctcatcttgcactgtttttccctttagctgttccaagcttggggcagagaagtcatcttgcctcccgaagctctagagccccttcccgcctctggccggggcactgagggctggaccctctccaggttccctgcgcctcctccagataccccgcctacgcccgcgcggcccgcgctgttccgcccctaagcctgaagcgcctactag

SEQ ID NO: 18099 - RNA, 854 nt, Homo sapiens
  source 1..854: mol_type = other RNA
tctgtgctactggatgaagagttttttaatggttacgagaagtgaagtccattcttctcttctctcattctgcaccaccactttgtaaaagtcttcatagaatctccccttgtgatcctgtcgaattgaggctcggtttatttcaggaaattcatcaacagattttgcatcatagaaagttctagaaaacaggaccactgtcacttcatgactacagttcttctccttccacttggtaaatagatcagcaaggaaaccattcacagctttctcaaaatacaaatccccataaatatcaaaatcccacatttcacagctcatctgaataaatatgtaaaccatagccgacgtagaacgaaacaccaccctggtatcttcactgatgtagccacacatgaccttctcattcttaacccacagttcaccagcctgtgctctgatgccagcaaactccaccttctgggtgatataggcacatgtgctgaccttagggtctacgacattaacatagacatcctgataaggtctcagccggaacacttgagtcacagtctggtccacactgatagtttccttctgtaaatcttccttaagagacttgacctgcaaaagcagagggctgtattcatcgttggggtgtgcaatctctacaatgtctccaagcttgatgtgagggaacactttggggttcacaactagctcatcatcactgcccccaaagcccttcttgtggatgacgagtttgtagacctttgttgttctcatcttgcactgtttttccctttagctgttccaagcttggggcagagaagtcatcttgcctccctgagaacccgcgccgctccggtggctcc

SEQ ID NO: 18100 - RNA, 39 nt, Homo sapiens
  source 1..39: mol_type = other RNA
tcttactccctcaggcactgcaccagccagcaaagcatc

SEQ ID NO: 18101 - RNA, 40 nt, Homo sapiens
  source 1..40: mol_type = other RNA
tcttactccctcaggcactgcaccagccagcaaagcatca

SEQ ID NO: 18102 - RNA, 13604 nt, Homo sapiens
  source 1..13604: mol_type = other RNA
tcttactccctcaggcactgctaaacaataccgttatgtttacataaaaacttactgacacatggacacaagaaaagcttctccaagaaatcatctgacattttctttttctaaaaaattctattttattttatattttgtagagacagggtcttgatatgttttcccaggctagtctcaaacacctgcctcaagtgattcctcctaacttggcctcccaaagcactgggattacagttgtgagccatagaacccagccacatttaacattttcagcagggaaatattgtatatactttgtttcactgtatttgataaagattgcttctgtaattcatctataattatttgggtgacatattatacaatttgggtttcgacccagcaatgtgaacaaacaaaacaaaaaaatttaattcatagtaagaaaaacacaaattaaaactacattgagtttcttactaatcagattggcaaaaattcaacaacttggtaactcactccactggcaggcctatgggtaagggaatgttctcacactacagtgaaaatgcagaatggtacaactcttacagaggggatttggcaaactgacagagcatttgttgccctttgacctccttctgggaattcactctgaaaatatacttctaaaaatacaaaaaaagatgcatgaggttattcattacagcttatttgtaatagcaaaatactgaaatacaacataaatacccatacaaagaagacagacagaataaactatagtacatccgctaagcagctgtaataaaaggatgaggaagacctctataaactgatatagagtgatttccatgatatattgttaagttgaaaagcaaaatgcaaaagtagacttacagcagggtttctcaacaacggcactttggcttattgaaccagataattctttattgtcgagggctaccctgtgtacagtaggatgtttagcattatgcctgatgtctacccactagatgtcagcagcaccccttcctgtagtgaacaaaaataattgtctccagataatgccaaatgtccctgggggacaaaatcttcccggttgagaaccacttctatgtaaaaagaaagcaaaatgaaatatagacatacccatttatatttaaaaaaggaaacacaggaagagtaaacctgaaactagtgaagttggttagctacaggaggtgggaggaacaaggtggaatggataggcaggaaaaggcctacgtatcctttctattaataaagtttttacttttggaatccctcaaagtgttactattcaataaataaataaaattaaaccaacaagaacgaaggaagaaaccttaaaattgaatacaaatagaaacaatttaactgaacagtatgtccaaaggataaagtaaccacacagcgaaggggatggaggtggggatgaattaatccatgtaatttttgaacttggctatataatttcagtcaaagacagaaagaatcaggcggaaattttaaactttacttgcaagtttatttttgctaatgatataggggtagcaattctgaaactattttatgtatattgtaggattggttacgtaagtaaatggtttggtaatgttaggagcaagggttctcactgtggaagaagaaagatacaaacatgctgtgtgggaaggcaagagaaaaactaattttaatttgagtatcagtatgaatttatgttttttaataaaaaaatttctagccctatctacatctggaacagtctaatattatcctttgagaagcacacagcatcatttcagtaatgcaataaattcaattgtggacccaaaaagatccatcttaatccagacccccccatatctgtaaatgaaaccttatttaggaacagagtctttgcagatttaattaaggttcttgagacgagatcatcctggattaaccagatgagtcctaaatccaataaatgctcttatcaaatgagaagaaacacaggaaagaaaagaaagccacgtgaagaaggagacagagatgggagttactgccgccacaaacgaaggaatgcttggcaccaccagaagctggaaaagaggcaggaaataattctccccaagagccttcagagggcgtggattgccaatactttgacttcgggtgttcaggaatgcgagaaaataaatttctgttgttcaaaccgccaagtgtttggtaatttgtagcccttagaaactaatacaagtagtatttctgtaaaaagtttataacctgaatcacatcacggagaaactatcagacaaacccaaattgaggtgttctcttaaaaaaaaaaagcaatagtctggcattctttaaaaatatcaatgtcatataaaataaagaaatgctgagaaactctttcgaataaaagaaactataataaatagacatggcaactaagtgcagtgcatgacaatggattgggaaaaacaagttgctctataaagtacagtgttatgacaattgctgaaatttaaatatggactgtattttagatactaatatataaatgtcagatttcctgaatttgataagtatactgtagttacctaagagaatatccctgttctttgaaaatataccctaaattaattaggggtaaaggtgtatgattactgcaacttgattaaaaaatacaaggtgtatattgtgtgtgtatgcctggagagagaaagaaagagaaggagaggttttcaaatacaaaatgtgttttgtggatgaattatctacctattttcccatggtacacaagccattaggttgaaggatagacagcacaagcttattttataatatatttaattattatttgaattcaaaatgtttatattttacttgtacatgtgtatgttcatataagaagactttgcaatgaaattattacaaatataaggaagctttggtctgggttttttttttttttttttttgagacggagtctcgctttgtcgcccaggctggagtgcagtggcgccatctcggtggctcactgcaagctccgcctcccgggttctcgctgttctcttgtcagcctcccaagtagctgggactacaggcgtctgtcaccacgcctggctaattttttgtatttttagtagagacggggttttaccgtgttagccaggatggtcttgatctcctgacctcgtgttccgcccacctcggcctcccaaagtgctgggattacaggtgtgagccaccgcacccagccctatctgagctattgttatttaaatgatgtaacgatgtataaaaattgctcactttgaaaactgatgtgaatgagaatgttgatgaatatgtataaaagtattcataagcttatatatttattgaggactaatcaaatattgttttattaaagttcaattttttgtcaattattgttttatgatcatgtgaaatggtaaaaataatacattctatatatgtttgatgtacatagcaactaaagccgcttaggtttttattaaaataatgattttaaaatattattataatgttaaagccaccactgaattctctggaaagactgtgtcaagaaaattcgggatgacatttactcaatttgaaagcacaaggaaacggaggaccctatagccaatgtttatataattagtttgcatgtgattctctttccagctcaaagttctggaatttaacattttgagtcagttcaagtttctgtagtcctaccaaagttatacataatagataagcactcaaagtaccctttactaaactttcctttctagatatatagacctattcagataatcttctaaatatttcaggtagatcaattaccatgttagaatgttactggctcacttgctctggctcattacaaaggagatcatgcaacatatctaacataagcaacaaaagaaatggtcagattgctcctcattagtagctatcaaaaaagaaatattaactagttttaatttactttctataagtaaaacccagaatcatctctatatgttatggaaaagatagcaaaataaatccataggtgtcacatgtggatcatttaacaaataatccttatttaaacaattataataattataataattgttttttcttgggaatctacaattctttcaaatgtatatatagttaaaattcaattataatagtaaaattatttgagataaaattcattccccatgattatggctttttatagttttgttactaatgtctcaaggtgcttttatactttgcattatattcccacttttctgcattaacatctaagtaatctgacagtgattttttttttttggtaaaatgtattgatgtttgttagagttacttttttattattctctaagacaaagctagaaagaatgggaaagcactgagaagtgttagctgtatctatgtgcttggagcttctgaatgacacaaaattctaaatatttcctaaattgagagcaaaaaaccaattcaaatccagaggagaaaaaaaagtgtgacatgaaaggcctatatgcagagaaaacaaatttttaaagtaatcatataaaatttaattggaacaatattgataaaaattttgcagcaatgttaactgtatttaaggcatgagatgtgttaagtttaagaataatgtaccactaagtactgctgtgttgtcgtagcaaaagaagttaacaatctgaaaggcataaaatttaactatcaataattcacataactatacatgctggaaccaatcattgcatcagggtttttcatgcatagaaagaactagatttgagtcatttatagtattcttaaaaaatgtgtgataataagaagaaatattcaagtgaaaatagatatttactattactgaaattatatcttttggataagatatttctagattccaaaacagagatgagaatagcctcttaagagcagggatgaggtttatttccaagtaataaaaataatattaggccaggtgcagtggctcgcatctgtaatccccgtaatttgggaggccaagctgggtgaatcacctgaggtcagaagtttgagaccagcctgctcaacatggtgaaaccccatctctactaaaaatgcaaaaattagccaggtgtggtggcacacacctgtaatcccagctacttgggaggctgaggcacaagaatctcttgaaccctggagacagaggttgcagtgagccaagattgtgtcactgaactccagcctgggcaatagagtgagacactgtctcaataagtaaataaataaatatattattagtggaagaattaaagtattgctaagctgttaaaaatgcaaatttctgtaaaagtcaactttaagagtatttatcattatatcagattaccatttaaattgctgatatttgacctataaaaattgcagttccatatggtttaatgtaatagtactcataaaatgagaaaaacttttgagtgagaggggagttttttcattattacttttataaatgagcccttagaaaagttaaagattttaaaaagtatctttagcattcttccaagccatagaaagctatagaaaattgtgtttacatttatagatctctttaaaagagatttaaaaaaactgaactgtaccaactactacacaggaggaactaaaatgtacaacttctatttctgtcaactgactgcccaaaggtatttatacaaagattacttggctgtaagtctaacagtcagaaagcaaggaatagaagtcaatttgctacagcaatgctactaagccttccttgtggttaaaataattttctaaaaaaggacatgttaaatgacagatatttatccccatcataaagagaattttgcaacatacctactgcaagcagcaaaataaatagattgctcataattagtgtaaggtaccagattgacttggcagtagaaaccaaatctgtggagatgttcattcattcagtcaatcacttatcagatatttattgcacaattacaatatatttactaggatcctaccagtgctgtacagagacatgtggttgccttttctagcttttaatctataaaagtttgttcaacagtgactcaacaagggcaaagtctgttccagtacaacccctactcccaaagccatatttctttgctttgagggcagcaggacaatagatatgtaacctacatacacattggcacagtacataggtatagagttctgtgaggagctctggattaagccacatcacattcctcctttattccagtggcttttatagacccatattccactcaggcagtggcctgctagtctgcctctttcttaaataaacacactccttgtcctcaagaggtgcaccctgtttgccttttggcagctagatattcattaagaattgacaggtccaaaagctagagacctataggaaaattgagattaagatatttaaaacagcataccccagattcttgcttagatccttttccagaccacatcctcatttttaaaatctgagatcttggataaaaagaaaaaaagcaaggatctcactgagaatactttaacagcaccctttctgtcctccatagagaaaagaggcaaatcagttcttctgacctgatctcatatgctttctagttaatagccatcatctggttttatatgtgtgggttaaacaatgttgatatataacacagagttccctgatccctacaaagaagaaatcttagatttggaagtcattcatatagaaacaatagaaaatggaacttcacagcttttatttttttgttttatttttatttttattcttttgagatagcatctcactctgttgcccaggccagagtgcagtggtgcaatcatggctcactgcagcctcaacttcccagactcaagcagccctcccacctcagcctcttaagtagctgggactacaggcaagtaccaccatatccagctacttttttattatttgtattgacggggtccccctatgttgccagggctaaccttaaattcctggcctcaagtgattatccaacctcagcctcctaaagtgctgggattacagtcatgagccaccaggcccagcccagaacttcatattttaaaatatccataaagcttatttggtgcaagtacttcttagtgcacagggcagttgtgccaatgttggtattatcgtccttcaagccctttctgcagaacttctgaaataaaacaccgtcttcactgttgcaagcgacaatctcttcttttgatgacataaagggtaagtcatgatctttttaagccataatgcatcctgaaaattaaggtttgcttgttttatatctcaacaagaattctgatttaaaattaagggactatttttgaaaaattctttaaaattttatggagaaatgaattttagaagaataggaaagagtagagaataaaatttaatttgaaaatgaattgaacaccaataaattttttaaaatttcactttcatatgagaatatagcttccttcaccttaacatatctgaatgatggccaagtacctatgctaaaatgtatgttaaaattgacttaattgccatgtacatcgaggattatgaggacctctgcctccaaaccacagcttgatattagtacagatcagcacaccaagaaaacaaccttagctggtgatacttgcaaggtcaggataaagggtagtaatttttcatacacatgcccctgttgataccaataaggcaaaatgactttagggtaaggcacatctgagttcaaattctagctccagcatttatccactggaggacttaaacctctttaagttttctcacaaaatagggatactaataccaactttataggttgtcatacagaaaaataagaaacttatatatgtagaattgtgactagcacacactaattgtttgacatattgttaattacaaaaaataacaataccctagagatgctcaatcctggttcaggatgcctaggacccaacagttatctcaagaggtcacaacattctcaggataaaatcaattttaatgcatataattttttaaaacacacacactatatcattaaaaggaagaagtggaaatgccatcaaagaaaatatagatatcaattaaagataccaaagaaaacataaatatactagtacttgtaaaggctgagatttcatgtcttaagctcttcttccttagaaaaacagttgaagaatacaatggccaggtagagtggctcacgtgtttaatcccagcactttgggaggccaaggcgggtggatcacttgaggccaggagttcgagaccggcctggccaacgtgatgaaaccccaactctactaaaaatacaaaaattctctgggtttcgtggtgggcgcctgtaatcccagttacttgggaagctgaggtgcgataatcacttgaggccaggagttcaagattagccctggcaaggtaggaaaaccctgtcaatacaaataataaaaaattagccgtgcatggtggtaccatggtgaacccaggaggcagaggctgcagtgagccaagattgtgccactgcactccagcctgggtgacagagtgacactctgtttcaaaaaaagaaaaagaaaaaagaagatagctgaagatacagatatttttgaaaagtgaagacaaattataaagaatgatattttgttattcctcagaaagttgggaaagtaatacagactgtgttatgattatctgagaaaatatttaagatcaaaaacagtaggatttttttcatcttaagatgcttaaatgtgataatcttattaatctgaaaatgagaggcagtgagtacagaagatttgtattcaaagacttggtatagtctaactctggctttgaaattccatataacgctaagtaaagtatgtagtccctttgaaattcaatttaattacttaaaaatactctatttagcataacttatacagaacataattaatatgtattattcatgcataacaagatagaaataaagttattatctatatttaatttcctgtacaatctaattagtgatgtttaccattcctgcttacaatcaaatttaagacttttatgttgcatttaattttaaaatgtgattcataactttatttatcaagtagtatttatatttaatctaggagattaagtaacatggtacttgtgcacacaaccctgtgaatgaagtagtagttactagttagaaataaacaaatattgagctgataagtaaaatgttactcataatttcagaatatcttctgaaaacaggaaacaaaaaataatgagtgttgtggaagcaagctaccgtcatcttttattatgctttttgagaagtaatttagcacataaaattgtgtcacttacttatagagagcaggttgagctccttagctagagactgggaaaatggcaaacatccaaattactaaaaaaccttaaaaaattaaatcaaagaacttcagctaaaagaaacagtgcagcaaacgagtaaggactgagaggatgagcactatcatttccagtatgtactgatgacttcttattagtggggatgagtctaagaaatgctttcttttctcagcatcgtgtgttagaggagagtaggaaagaacattatgctatccagaagtgtccaaaaaacaaaaacttctgcttacttgaatctgtggtatttcttacctatttagaaattggagaaactgatgcaatccatggcaactgttcaaatcctgaattactttcaaaactcaggtcaaatgacacactgttctattttttcctcattttgaacatccatagcatttcttgcctttcttgaggcacttatttctggtttttatttccattagttgaatgtttttatttataactaaatgatacataaacatcataagattatatgctaattattgtctatcctaaaaagactaaatgaaaaaaaaattgttatctctctgacatgaaacacaatactccagctatttctccctttttttctttttctttctttaaaaaaagtatttgatcagatttaattctatacttatatataatccttctttcactttctgaaccttttgtttctcagactccaaagtcatgggtgggcagaagtttatacaagttacctttttgtacaccattgtgggaagcctgaatctatttcagatcttgtgggccttagtatttgggcctgcatagtaagtttgaatagtaagaaaattacgattaaaatttctttttcaagatatttctgccaaggaagcgtaggtagtaagagcatacgtgttagaattacatgatgggttggtgcccagggtggaactggttccaggaccccagaaaacaccaaaatccacagatgcctttatataaaatggccacagtatttgcatatcaccaacacacatccccctatatactttaaatcatctttagattacttgtaatacctaacacaatacaaatactatgcattggttttttgtttgtatgattttttatggttatgttgttgttttcagtgtttattttaaaaatattttttattcatggtgggttgaatccaaggttgtggaagctgcagatacagaggcccaactgtaatgtgatgtatgcaaatgatcttctggagtattatttttaaaaactagtacaaaagaaagcaagattttactctgagcaaaatatattttgtcagcaaatatctattatcatctgtctttcttccttctgtcccttcctctgttgcttctctcccactctctctctacccccaactcccactaaatattccaatttattattttgatgattgttagcatactataaaattttgttagcaggtgaacaaaataaacaagtaaaagggtgggtttaggggctttcatggatgaagacagaaacttaccaggggattaggaagtaacaaataggccataaattagtggatttgtgaaagtgagagcaggggatcacaaatctctccttagggacttggaaagacagataaactttgtggaatataaaacatatgttgaggaggtggtttatagaggactccttcatacacaggccagagcccacttagaattctgaagagagaacttttcccacaaccattgggaccagttatcaaaagatgcattccttcttctactttgaagtttagcctggaagccaccacttctcctgctggtgtaattatgggaacattttcacaaataattccgtgatccacatcaataacttttcctttaattgccaatgtgtcactgagaggtaattctaccttagctccattcttgctatggctttcagattcttgaatgacagcagttctcttataaatgcctctttttacttcatcaaagacccaaaacatattgtacactcgagcagtgtagcctgctaattcagtgacctctttgtatgaagacataatcctttcaatagcatcagctccagaggccagtaaatttcgagcagtggtaaaggcttctgtccgttcactaaccataacttgcttttggccatcctcaccatctgcaaagccagttgcagtgataataggtatagccaccataattagtccactgctgctccaaacatacttcatcaggaactgttctatcatgatgtaccacaaacgtttggataaaatgaggttcatctgatctgctaaagctttgtaacttttctgaagttgtttcatttctaccttatgtcctctgtaaaaggcaatttcttctacattggctataattctcgagtgcacataccgcaaatagccttttctatgtgcttcctctgccaccagtttgccaaatttgggagaacaggcttttaacactttagcagtggcatacaccacaagtcctgctagtagggtgggcccaattgggcttgctcctctggatgtagcagtttgaatgagtgtataggaggtcagcattacatctaaaataggtttggtcagattggaatacaagtgagccacagattgggagaacatcataatatcctccgtaagagattggtcagggtttgccagcctcccatccatattgatcactttataataagtctgatttgtaaaataggtttcataggcgtggtctactaggcgagttctgaaggccaaagccaatttgcattccaggtaccttattgcactgttgacgaaggtagcagggatggcaatcataagccacttgattaatttgatgatgaaagtccgaggcttcttttccacaatgcttttcacgatttttccatccagaccagccacatagatagaaagaaaggttcttgagattagagccactgagtgcaggcagagccaccctgtttcagtggtcacaagttttggaaacaaaattttccgaagttctagtagctgtttgaagaaatctgcattcactccaggcgaaggtttttcacaaatggtctcggtgcaatgcagtatttctgtgttctctgcagcagggtaagctgctgcttttttcttcccgtggccagattgctttaaacgcttgccaatgatgggatagagggttttcagagcatatgccgcagccaccaggcaggcagccctcttagcagcactcgatctggtccatttcactcgatcagctgctgcatttagcatatgtgtcattttcccagttacccaaaccggcttccaaaagaattcgttttaaaagatcatgcttcacagaaatccccagcaaatgttttagaaagtcctacagcgtcccatagtctgcagcgtttctcttccactgttgtgtttttaattttgttctgctgtgacagatgcagcagagctcagactccgctgcatctaccgggaatgattctctcagaagctcaagctgcaccaagctcctccctcccaggcccctcattggctgtgagggcggtgggaccttggaatcctcgcagcttccctttgaaccttgaaaatgaggagagagcaaagcgaattacatccttccttaaacaggagttcagagagttaaaatgtctatttttggagaggtcgaatcaggccatctgctggcgaacaaaaccggctctagctactgagcatgctcagtgtcacttagaaacccacagaagtttcagaatatacatcacttcggtaagatttcagtagataccgcaaacagaagagcaagcagaaagggagatttccaagcgaacaaaaccggccctagctactgagcatgctcaatgtcacttagaaacccgcagaagtttcagaatatacatcacttcggtaagatttcagcagctaccgcaaacagaagagcaagcagaaagggagatttgcaagagttttaatgagacgaggagggagaaggaaccacgaaaatgagggaggagggacaagaggatcaacataaaatgaatatgaaaaggatatggaatgaatctgaaacggatcagaaaagaaagtgacaagtgggagggacaccggagaatgccaaatatcaaatacacttggatctgtttttcacagatccccccggcttttttgggggtc

SEQ ID NO: 18103 - RNA, 2327 nt, Homo sapiens
  source 1..2327: mol_type = other RNA
tcttcacctgcctctgcctgcacagctccgtccctgcttcctccagctcctgggtggacagggaggccccggcttcccgcagcaacccaatgacacccggatgcatgagctgaccggccccactgcacacccaaacgctgatcacaccccgtggtgacctcctcagccaggcgcaggggacactgaatcaatccggccgactgcccttgggtaggagtgggggcagggcacccggacagtggagtcccactcaggcacagcagggccaggcaggcggcctcagggagcctggcagcggagcgaggctgggagaccggttgggggcgtgctgtgagcctggtcctgccccgcacggccagcagcagcgggctgaagccatccgtgtcccgggtgttcacgtccacacctctctgcagcagcatggtgactgcctctgtgtggcctccccgggcggccgcgtgcagtggggtttggccgttaaagtccaccaggcccaggtcactgcccagctccacaagcgcctgcagcgcctccacgtcaccggcgtgggcagcagcacaggccaggctgggcaccagggcattccgcagggcatctgcctcctggctgccgctcagactgaggagccaggagaccccaccgcccagcgtgttgccctgcagtgagggccggcgctcttccaccgagggtggcgtcatctccccccgaaggtccttggtcagcagctccttcctgacatccaggctcagccctggctggcccagcacatacgatagcttggccagggcggcctccgatgtcatgtcgaagcctgagatgacgccggctcccgccatggccatgccagctgcatagtctgtggtcacagccccctggaggcagtgggtacagttgacgatgaccaggccgcgctcggtggccacccgcagctcctgcagcaggtcgggcttggtgggtccgttccctgaaccgaaggtctccatgaccacgcccttcaggggaggctgcaagaaggcccgaaccagggcggcagggatcccagggtagaggcgcagcaggcccacgtcctgctccatgctgctgtgcaccaccagcccagccttcccgtccaccttccgcaccagctccctgttgattgtgatgtcagcacccactgtggccagaggcagcaggttcggggagcagaaagctgcgaacctccgagcgtctaccttggttgcccggttgccccgaaacagctgattctggaagaaaaggcagacctctgggatcacatactggccagccatgagcagtgcccccagcaggttctcacggccgtcgctccacagggcatggatgggcacctgggccccagtgaggatgacagtcttctgcaggttctccagcatgaaggacagcatcgaggcagcaaaggccatggtgtcggtgccgtggatgaccacaaagccgtggtactgctcgtagtgcctcttgatggtctgggcaaggcaaacccactcagcgatggtcatgtcactggagtcgaagaggggctggcactccagcacggtgtagagaatcctctggttgcggctggccgggctgcgggacagaaacagcaggaggcggaacagcaggctcccgctctgcacctcctcctgctctaaatgccctgacccgctctgttcccctctggcagagctggggcccctacgccaagggctccgcacatagcaagttctcagcatcccaggtacggggcccggccccccttccacctggagctccccacagaggcaaggacgtaggtcaggatgggccactcccagcagtcttcttcccacaccagctcgaagaggggggctgggaccagccatccccaggcaggagaggatgcttgcaggaggctcgcctgtggcggctgtggtggtcagccaccacgagggcaactcccagctcacccccagctgtgggggacatcagggagctgggcccagagctgagaaatggaaggacctctatgctgggggcaaggccacctgggccagctggctcctgatatacaggatccctagacggggcgccctcatcacacttgccgaagcagcctggctgggggtgtgggaggagggtggggagggaaggtgggaccaggcacggggcaccctcagaggttcaggctctggtggaaggcgactgctggtcagtcctaaagccctgtaagctgaggggatgttagagacaggggtgagcaaatggctcacgtgggcctggccagcagtgcccagcctcaggatcggtgcccctcagcagccatgccctgtccgggactgggaggagcccac

SEQ ID NO: 18104 - RNA, 2089 nt, Homo sapiens
  source 1..2089: mol_type = other RNA
tcttcacctgcctctgcctgcacagctccgtccctgcttcctccagctcctgggtggacagggaggccccggcttcccgcagcaacccaatgacacccggatgcctgccccgcacggccagcagcagcgggctgaagccatccgtgtcccgggtgttcacgtccacacctctctgcagcagcatggtgactgcctctgtgtggcctccccgggcggccgcgtgcagtggggtttggccgttaaagtccaccaggcccaggtcactgcccagctccacaagcgcctgcagcgcctccacgtcaccggcgtgggcagcagcacaggccaggctgggcaccagggcattccgcagggcatctgcctcctggctgccgctcagactgaggagccaggagaccccaccgcccagcgtgttgccctgcagtgagggccggcgctcttccaccgagggtggcgtcatctccccccgaaggtccttggtcagcagctccttcctgacatccaggctcagccctggctggcccagcacatacgatagcttggccagggcggcctccgatgtcatgtcgaagcctgagatgacgccggctcccgccatggccatgccagctgcatagtctgtggtcacagccccctggaggcagtgggtacagttgacgatgaccaggccgcgctcggtggccacccgcagctcctgcagcaggtcgggcttggtgggtccgttccctgaaccgaaggtctccatgaccacgcccttcaggggaggctgcaagaaggcccgaaccagggcggcagggatcccagggtagaggcgcagcaggcccacgtcctgctccatgctgctgtgcaccaccagcccagccttcccgtccaccttccgcaccagctccctgttgattgtgatgtcagcacccactgtggccagaggcagcaggttcggggagcagaaagctgcgaacctccgagcgtctaccttggttgcccggttgccccgaaacagctgattctggaagaaaaggcagacctctgggatcacatactggccagccatgagcagtgcccccagcaggttctcacggccgtcgctccacagggcatggatgggcacctgggccccagtgaggatgacagtcttctgcaggttctccagcatgaaggacagcatcgaggcagcaaaggccatggtgtcggtgccgtggatgaccacaaagccgtggtactgctcgtagtgcctcttgatggtctgggcaaggcaaacccactcagcgatggtcatgtcactggagtcgaagaggggctggcactccagcacggtgtagagaatcctctggttgcggctggccgggctgcgggacagaaacagcaggaggcggaacagcaggctcccgctctgcacctcctcctgctctaaatgccctgacccgctctgttcccctctggcagagctggggcccctacgccaagggctccgcacatagcaagttctcagcatcccaggtacggggcccggccccccttccacctggagctccccacagaggcaaggacgtaggtcaggatgggccactcccagcagtcttcttcccacaccagctcgaagaggggggctgggaccagccatccccaggcaggagaggatgcttgcaggaggctcgcctgtggcggctgtggtggtcagccaccacgagggcaactcccagctcacccccagctgtgggggacatcagggagctgggcccagagctgagaaatggaaggacctctatgctgggggcaaggccacctgggccagctggctcctgatatacaggatccctagacggggcgccctcatcacacttgccgaagcagcctggctgggggtgtgggaggagggtggggagggaaggtgggaccaggcacggggcaccctcagaggttcaggctctggtggaaggcgactgctggtcagtcctaaagccctgtaagctgaggggatgttagagacaggggtgagcaaatggctcacgtgggcctggccagcagtgcccagcctcaggatcggtgcccctcagcagccatgccctgtccgggactgggaggagcccac

SEQ ID NO: 18105 - RNA, 2794 nt, Homo sapiens
  source 1..2794: mol_type = other RNA
tcttcacctgcctctgcctgcagcttcctgcgtgccagctgctccttagcaaacaccaccttgggctcagagacgcggagccggaagtccacagagtcctcgcccacgcggcaggagtaggtgccttcatcctgcctggtgactgtggctgccaccagccggtgccgcgtccccacatcctcctgcaagaagcgctcaccggagtggcccagctccatgccatccttgtaccagtgcacgtggacgtgggcttcggaggtctcacactcaaactgcgccgggcccccagccacggcatccacacagctgcccgccatgtccttgtgcagaaagcgcgcgaggccttgcacggagagctggtaggcgatgcggcccccgcggctgacgcactcgtagaggcctgcatcgtcccgggccacatctcgcacaaggagcacccgccgcccggccgatgcctgcacctcatacttggggcctggggacagtgtgcgaccatccttcagccacgtcacagccgcagcctgatctgacagctcagccagcagctgcgcctcctcgtgcagccgagccagcacctcccgggcagctgcggctggcggcttgttggcagtcagccctggggccgcccggacctccatccggatgctgctctcaatgccgttggccacgaacttcagctgcgccccgtgcaggctggcgggcacctcccggatggtgagcgtgtgccgggtgcgatcacagtggatctcatacacactgctggccttcagggcctgcccatccaggaaccactcacccgctgaggccaccgtgaggtccacggagaaagtgacctcgccaccctctaccgcctgcaccgccttcagcggtgtcctcacggccagcttgggggccaggtggacagtccccgggaactcgaggtagggactctgaccaaagctgttgagagcggacactcggaactggaagttcccctcctccgccacatcagccacggtcagctcaggtgtagccacccattcagcctcgtggcacctgatccaggtgtaggtgccaagcttcttcttctctaccaggtagccgtcgatagtgacagggcgttccccatggggtggtggggaccagctgagaatcacggaactctccatcctggcctttaccacaggatccacagggggttgcaggggaggcttcctgggggccgacacgcagaactgggtggacgtctggcagtcgccagccataaaggccacctggcccacatcctccaggcagcactgggagatggttagtgtgtggcgcgtgccctccgcggagatggccacgcggccccccgccaccacttcctcctggttccgcagccagtggacggggcccaccgggaccgccagctccacgcaaaacatagccgtgtcgcccacgcgcaccgccgtcttccgagggagctttcggaggaggtttccttggactgcgagctccgccaccgtgcggctgccctctggcgtctcgcagatgtacaccgcgtcgtcgtcggccgagacattgcgcacggtcaggcggcgctcggtgccctcctcctcgatgccgtacttggcgctcgcccacaaccgcgtctcctccttgaaccacgcggcctcagtggacggctggggcacctcacataggaacgtggccgactccttctcccgcacctccagatcttgcagccgctttttgaagggaaccgcgggctcgcgcactacgaccagcacagagctgtaggtctggcccacgaggttggacgccgtgcaggtgtagaggccgcggtccgactgcttgcagaagaggatcttgagcacgaagttctcctgcgcgtcctcgtacaccacgtggcgccggccctcggtcaccagctggccgtccttcttccacaccgtctcgggcttgggctcgccggtcacgtagcagctgaggcgcgcgtgcttgccttcagtcaccgtgcaggtgcgcgtgccggtgctgggcggtgaggcgggggcgccctcggcgcgcatagcctcgcgccgccgctgcaggtgcgccaggagcgcggccgtggaggtcccgggccggctggccgtgtccgcggcgtccgagtccaccactagcgccgcggcggcgctggcagcgcccagcgggttctcggcgcggacctcgtaagtgccgccgtcgcgcggccgcgccgcccgaatgcgcagcgcacttgcctcgccgagctcctccacgcgcacgcgggggccgtcgggctcacccaggcgccgcccgtccttggaccagctcactgccggcctcggggagccacccacgcggcagcggaaggtggcctctgagccctcgcgcacgcggatggacgtgggccgcagcaggaagtgcggcgcctgctcggcgcacgcggcctccgcgtccacctgcaggcccacagcagcgaaggcctcgcctatggcattgcgcgcgcggcacacgtattgcccactgtcgcccagcgccaggtccaggatagtgaggcggtagaggtcgccgtcctgggccagacggaagcgcgcgccggccgccaccggctgctggtccttctcccagctcacctgtggcgtgggattacccacgatctggcagctgagggtggcgtccttgcccaccgacaccacgaaggccttgggccgggtgagaaagcggggcgccccgctgaactgtggctgatccatgagggtggcggcggggacctctctctatgggggctctgggcagcacgcaggctgggggcacaggctgggaggca

SEQ ID NO: 18106 - RNA, 2880 nt, Homo sapiens
  source 1..2880: mol_type = other RNA
tcttcacctgcctctgcctgcagcttcctgcgtgccagctgctccttagcaaacaccaccttgggctcagagacgcggagccggaagtccacagagtcctcgcccacgcggcaggagtaggtgccttcatcctgcctggtgactgtggctgccaccagccggtgccgcgtccccacatcctcctgcaagaagcgctcaccggagtggcccagctccatgccatccttgtaccagtgcacgtggacgtgggcttcggaggtctcacactcaaactgcgccgggcccccagccacggcatccacacagctgcccgccatgtccttgtgcagaaagcgcgcgaggccttgcacggagagctggtaggcgatgcggcccccgcggctgacgcactcgtagaggcctgcatcgtcccgggccacatctcgcacaaggagcacccgccgcccggccgatgcctgcacctcatacttggggcctggggacagtgtgcgaccatccttcagccacgtcacagccgcagcctgatctgacagctcagccagcagctgcgcctcctcgtgcagccgagccagcacctcccgggcagctgcggctggcggcttgttggcagtcagccctggggccgcccggacctccatccggatgctgctctcaatgccgttggccacgaacttcagctgcgccccgtgcaggctggcgggcacctcccggatggtgagcgtgtgccgggtgcgatcacagtggatctcatacacactgctggccttcagggcctgcccatccaggaaccactcacccgctgaggccaccgtgaggtccacggagaaagtgacctcgccaccctctaccgcctgcaccgccttcagcggtgtcctcacggccagcttgggggccaggtggacagtccccgggaactcgaggtagggactctgaccaaagctgttgagagcggacactcggaactggaagttcccctcctccgccacatcagccacggtcagctcaggtgtagccacccattcagcctcgtggcacctgatccaggtgtaggtgccaagcttcttcttctctaccaggtagccgtcgatagtgacagggcgttccccatggggtggtggggaccagctgagaatcacggaactctccatcctggcctttaccacaggatccacagggggttgcaggggaggcttcctgggggccgacacgcagaactgggtggacgtctggcagtcgccagccataaaggccacctggcccacatcctccaggcagcactgggagatggttagtgtgtggcgcgtgccctccgcggagatggccacgcggccccccgccaccacttcctcctggttccgcagccagtggacggggcccaccgggaccgccagctccacgcaaaacatagccgtgtcgcccacgcgcaccgccgtcttccgagggagctttcggaggaggtttccttggactgcgagctccgccaccgtgcggctgccctctggcgtctcgcagatgtacaccgcgtcgtcgtcggccgagacattgcgcacggtcaggcggcgctcggtgccctcctcctcgatgccgtacttggcgctcgcccacaaccgcgtctcctccttgaaccacgcggcctcagtggacggctggggcacctcacataggaacgtggccgactccttctcccgcacctccagatcttgcagccgctttttgaagggaaccgcgggctcgcgcactacgaccagcacagagctgtaggtctggcccacgaggttggacgccgtgcaggtgtagaggccgcggtccgactgcttgcagaagaggatcttgagcacgaagttctcctgcgcgtcctcgtacaccacgtggcgccggccctcggtcaccagctggccgtccttcttccacaccgtctcgggcttgggctcgccggtcacgtagcagctgaggcgcgcgtgcttgccttcagtcaccgtgcaggtgcgcgtgccggtgctgggcggtgaggcgggggcgccctcggcgcgcatagcctcgcgccgccgctgcaggtgcgccaggagcgcggccgtggaggtcccgggccggctggccgtgtccgcggcgtccgagtccaccactagcgccgcggcggcgctggcagcgcccagcgggttctcggcgcggacctcgtaagtgccgccgtcgcgcggccgcgccgcccgaatgcgcagcgcacttgcctcgccgagctcctccacgcgcacgcgggggccgtcgggctcacccaggcgccgcccgtccttggaccagctcactgccggcctcggggagccacccacgcggcagcggaaggtggcctctgagccctcgcgcacgcggatggacgtgggccgcagcaggaagtgcggcgcctgctcggcgcacgcggcctccgcgtccacctgcaggcccacagcagcgaaggcctcgcctatggcattgcgcgcgcggcacacgtattgcccactgtcgcccagcgccaggtccaggatagtgaggcggtagaggtcgccgtcctgggccagacggaagcgcgcgccggccgccaccggctgctggtccttctcccagctcacctgtggcgtgggattacccacgatctggcagctgagggtggcgtccttgcccaccgacaccacgaaggccttgggccgggtgagaaagcggggcgccccgctgaactgtggctgatccatgagggtggcggcggggacctctctctatgggggctctgggcagcacgcaggctgggggcacaggctgggaggcaggggctgccgggtctcacctccctccgagggcccaggaccagcaggctgcctaccagcagcccacactccggccgctcctcaaact

SEQ ID NO: 18107 - RNA, 3070 nt, Homo sapiens
  source 1..3070: mol_type = other RNA
tcttcacctgcctctgcctgcagcttcctgcgtgccagctgctccttagcaaacaccaccttgggctctgcaacgtccaggcggaaggagaccctctgtcccctggcctcacagctgtactctccggagtctgcctggcccacctgctgcaccaccagcctccgcatacagcccacagcctccacgtgcactttcgagctggagctcaacttcttcccgtccttgtaccacgtcacctccatctggtcctgggccacctcacagctcagcgtggcgctggcccccacctcagcctgcacctccctgcacgccggctgctccttggcaaacaccgccttgggctcagagacgcggagccggaagtccacagagtcctcgcccacgcggcaggagtaggtgccttcatcctgcctggtgactgtggctgccaccagccggtgccgcgtccccacatcctcctgcaagaagcgctcaccggagtggcccagctccatgccatccttgtaccagtgcacgtggacgtgggcttcggaggtctcacactcaaactgcgccgggcccccagccacggcatccacacagctgcccgccatgtccttgtgcagaaagcgcgcgaggccttgcacggagagctggtaggcgatgcggcccccgcggctgacgcactcgtagaggcctgcatcgtcccgggccacatctcgcacaaggagcacccgccgcccggccgatgcctgcacctcatacttggggcctggggacagtgtgcgaccatccttcagccacgtcacagccgcagcctgatctgacagctcagccagcagctgcgcctcctcgtgcagccgagccagcacctcccgggcagctgcggctggcggcttgttggcagtcagccctggggccgcccggacctccatccggatgctgctctcaatgccgttggccacgaacttcagctgcgccccgtgcaggctggcgggcacctcccggatggtgagcgtgtgccgggtgcgatcacagtggatctcatacacactgctggccttcagggcctgcccatccaggaaccactcacccgctgaggccaccgtgaggtccacggagaaagtgacctcgccaccctctaccgcctgcaccgccttcagcggtgtcctcacggccagcttgggggccaggtggacagtccccgggaactcgaggtagggactctgaccaaagctgttgagagcggacactcggaactggaagttcccctcctccgccacatcagccacggtcagctcaggtgtagccacccattcagcctcgtggcacctgatccaggtgtaggtgccaagcttcttcttctctaccaggtagccgtcgatagtgacagggcgttccccatggggtggtggggaccagctgagaatcacggaactctccatcctggcctttaccacaggatccacagggggttgcaggggaggcttcctgggggccgacacgcagaactgggtggacgtctggcagtcgccagccataaaggccacctggcccacatcctccaggcagcactgggagatggttagtgtgtggcgcgtgccctccgcggagatggccacgcggccccccgccaccacttcctcctggttccgcagccagtggacggggcccaccgggaccgccagctccacgcaaaacatagccgtgtcgcccacgcgcaccgccgtcttccgagggagctttcggaggaggtttccttggactgcgagctccgccaccgtgcggctgccctctggcgtctcgcagatgtacaccgcgtcgtcgtcggccgagacattgcgcacggtcaggcggcgctcggtgccctcctcctcgatgccgtacttggcgctcgcccacaaccgcgtctcctccttgaaccacgcggcctcagtggacggctggggcacctcacataggaacgtggccgactccttctcccgcacctccagatcttgcagccgctttttgaagggaaccgcgggctcgcgcactacgaccagcacagagctgtaggtctggcccacgaggttggacgccgtgcaggtgtagaggccgcggtccgactgcttgcagaagaggatcttgagcacgaagttctcctgcgcgtcctcgtacaccacgtggcgccggccctcggtcaccagctggccgtccttcttccacaccgtctcgggcttgggctcgccggtcacgtagcagctgaggcgcgcgtgcttgccttcagtcaccgtgcaggtgcgcgtgccggtgctgggcggtgaggcgggggcgccctcggcgcgcatagcctcgcgccgccgctgcaggtgcgccaggagcgcggccgtggaggtcccgggccggctggccgtgtccgcggcgtccgagtccaccactagcgccgcggcggcgctggcagcgcccagcgggttctcggcgcggacctcgtaagtgccgccgtcgcgcggccgcgccgcccgaatgcgcagcgcacttgcctcgccgagctcctccacgcgcacgcgggggccgtcgggctcacccaggcgccgcccgtccttggaccagctcactgccggcctcggggagccacccacgcggcagcggaaggtggcctctgagccctcgcgcacgcggatggacgtgggccgcagcaggaagtgcggcgcctgctcggcgcacgcggcctccgcgtccacctgcaggcccacagcagcgaaggcctcgcctatggcattgcgcgcgcggcacacgtattgcccactgtcgcccagcgccaggtccaggatagtgaggcggtagaggtcgccgtcctgggccagacggaagcgcgcgccggccgccaccggctgctggtccttctcccagctcacctgtggcgtgggattacccacgatctggcagctgagggtggcgtccttgcccaccgacaccacgaaggccttgggccgggtgagaaagcggggcgccccgctgaactgtggctgatccatgagggtggcggcggggacctctctctatgggggctctgggcagcacgcaggctgggggcacaggctgggaggca

SEQ ID NO: 18108 - RNA, 3156 nt, Homo sapiens
  source 1..3156: mol_type = other RNA
tcttcacctgcctctgcctgcagcttcctgcgtgccagctgctccttagcaaacaccaccttgggctctgcaacgtccaggcggaaggagaccctctgtcccctggcctcacagctgtactctccggagtctgcctggcccacctgctgcaccaccagcctccgcatacagcccacagcctccacgtgcactttcgagctggagctcaacttcttcccgtccttgtaccacgtcacctccatctggtcctgggccacctcacagctcagcgtggcgctggcccccacctcagcctgcacctccctgcacgccggctgctccttggcaaacaccgccttgggctcagagacgcggagccggaagtccacagagtcctcgcccacgcggcaggagtaggtgccttcatcctgcctggtgactgtggctgccaccagccggtgccgcgtccccacatcctcctgcaagaagcgctcaccggagtggcccagctccatgccatccttgtaccagtgcacgtggacgtgggcttcggaggtctcacactcaaactgcgccgggcccccagccacggcatccacacagctgcccgccatgtccttgtgcagaaagcgcgcgaggccttgcacggagagctggtaggcgatgcggcccccgcggctgacgcactcgtagaggcctgcatcgtcccgggccacatctcgcacaaggagcacccgccgcccggccgatgcctgcacctcatacttggggcctggggacagtgtgcgaccatccttcagccacgtcacagccgcagcctgatctgacagctcagccagcagctgcgcctcctcgtgcagccgagccagcacctcccgggcagctgcggctggcggcttgttggcagtcagccctggggccgcccggacctccatccggatgctgctctcaatgccgttggccacgaacttcagctgcgccccgtgcaggctggcgggcacctcccggatggtgagcgtgtgccgggtgcgatcacagtggatctcatacacactgctggccttcagggcctgcccatccaggaaccactcacccgctgaggccaccgtgaggtccacggagaaagtgacctcgccaccctctaccgcctgcaccgccttcagcggtgtcctcacggccagcttgggggccaggtggacagtccccgggaactcgaggtagggactctgaccaaagctgttgagagcggacactcggaactggaagttcccctcctccgccacatcagccacggtcagctcaggtgtagccacccattcagcctcgtggcacctgatccaggtgtaggtgccaagcttcttcttctctaccaggtagccgtcgatagtgacagggcgttccccatggggtggtggggaccagctgagaatcacggaactctccatcctggcctttaccacaggatccacagggggttgcaggggaggcttcctgggggccgacacgcagaactgggtggacgtctggcagtcgccagccataaaggccacctggcccacatcctccaggcagcactgggagatggttagtgtgtggcgcgtgccctccgcggagatggccacgcggccccccgccaccacttcctcctggttccgcagccagtggacggggcccaccgggaccgccagctccacgcaaaacatagccgtgtcgcccacgcgcaccgccgtcttccgagggagctttcggaggaggtttccttggactgcgagctccgccaccgtgcggctgccctctggcgtctcgcagatgtacaccgcgtcgtcgtcggccgagacattgcgcacggtcaggcggcgctcggtgccctcctcctcgatgccgtacttggcgctcgcccacaaccgcgtctcctccttgaaccacgcggcctcagtggacggctggggcacctcacataggaacgtggccgactccttctcccgcacctccagatcttgcagccgctttttgaagggaaccgcgggctcgcgcactacgaccagcacagagctgtaggtctggcccacgaggttggacgccgtgcaggtgtagaggccgcggtccgactgcttgcagaagaggatcttgagcacgaagttctcctgcgcgtcctcgtacaccacgtggcgccggccctcggtcaccagctggccgtccttcttccacaccgtctcgggcttgggctcgccggtcacgtagcagctgaggcgcgcgtgcttgccttcagtcaccgtgcaggtgcgcgtgccggtgctgggcggtgaggcgggggcgccctcggcgcgcatagcctcgcgccgccgctgcaggtgcgccaggagcgcggccgtggaggtcccgggccggctggccgtgtccgcggcgtccgagtccaccactagcgccgcggcggcgctggcagcgcccagcgggttctcggcgcggacctcgtaagtgccgccgtcgcgcggccgcgccgcccgaatgcgcagcgcacttgcctcgccgagctcctccacgcgcacgcgggggccgtcgggctcacccaggcgccgcccgtccttggaccagctcactgccggcctcggggagccacccacgcggcagcggaaggtggcctctgagccctcgcgcacgcggatggacgtgggccgcagcaggaagtgcggcgcctgctcggcgcacgcggcctccgcgtccacctgcaggcccacagcagcgaaggcctcgcctatggcattgcgcgcgcggcacacgtattgcccactgtcgcccagcgccaggtccaggatagtgaggcggtagaggtcgccgtcctgggccagacggaagcgcgcgccggccgccaccggctgctggtccttctcccagctcacctgtggcgtgggattacccacgatctggcagctgagggtggcgtccttgcccaccgacaccacgaaggccttgggccgggtgagaaagcggggcgccccgctgaactgtggctgatccatgagggtggcggcggggacctctctctatgggggctctgggcagcacgcaggctgggggcacaggctgggaggcaggggctgccgggtctcacctccctccgagggcccaggaccagcaggctgcctaccagcagcccacactccggccgctcctcaaact

SEQ ID NO: 18109 - RNA, 1090 nt, Homo sapiens
  source 1..1090: mol_type = other RNA
tcttcacctgcctctgcctgcatggcaactcaccgtccagagcctttccacttggcttgggcttctcacagtgcagtaatcttggggtaatcacatttcttgcatgtgatcacacttcaaccctgtgctttattggtcaaaataatcacagggcctcccagattcaaggaagtgaagaaatacactccagcttttgatgttcagaattggacaaggtcacatgacaggagagcatgcagaatgtgtatcattgttgaggtcccctttgaaaaatataatctaactaatctgcagaggaaattcaacagtttcatttgaaagtgcattggcgtaaaatgcacaatatatacatcgaggagtcaaaaattagaatgtctaaaatgaataaaccaaccactttagaccaaccagccaataaacaaacatatagactaacattttattaagagaatctgcgcaattagattctggtctctggtccacctgataactataaaatgatggcctgttggtgttatggtaaactattctttgattaaattgaatgcaataatcactaattatattgtagaagctcttgctgtatcacatatagtgatgacaccacccaccatggtattctgtccataaatggccttgaatttagtttaaagtcgaacttcttaagacacttatgacgttttcagtttggctcttcactttcaggtggcatcaatcccaatcttacagtattcttttaagttctgcaaatctgccatcttagaaactgtagataaagaatcttttccagaggtcttggaatcaaacatccttcactgaaacattatgtttaacatcaatgtcttgaccacttctggaatcttcttgaatcttctctgctggaatcccaggactttgggaggccaggtttggagaatagcttgagcccaggagttcatgatcagcctaggcaacatagccagaccatgtctcttctgcttcggccacccggtgcggctccagcaccgcgcgctctcccggcacggttcccggagaaagtcccccaatcaccagctacggcacttgtagcctctgcacgccgctcggctcc

SEQ ID NO: 18110 - RNA, 655 nt, Homo sapiens
  source 1..655: mol_type = other RNA
tcttggagtaggtcattgggtggatcctctatttccttacgtgggccactggatggctcctccatgtcttggagtagatcagtgggcagctcttccatttcctggagtgggccactggggggctccttcttttcctgggctgggccgctggctggccctgcctctccccgcactccactgcccgacgtcgcctcggtggtgttggatgagccctcggaggactccatttgttttgatgatggattcttatgctccatcatcgtctcaaatgagtcttcagagggttctatcatttcgtcggatggaaaggagtgtattctgaagattggtaaggttgtgatggcgtccagtcagtagctgggaccgtggagatcagaaccttggctgcaagcgttcaagtggatctcctcccgtcctgtgccactcgatcctcgctgcttgcttccccgggcccagtcccaagcgtgaggctggggatgaagtgatgccggtggcttagtgatgccggtggcttcctgtcctcgaagctcagtcggtcgtctctcagctggtgtgaggctgggccaggatggaaccccagactctccgaggctccccaccacaccctgctgctgaaggctgctcagcgaggctgtgccgagtgctgggggggtgt

SEQ ID NO: 18111 - RNA, 6826 nt, Homo sapiens
  source 1..6826: mol_type = other RNA
tcttttctttgagactcacttttcaaaactgctgttgttagatgatccttataaacatgttgctgagggaaagaagccaaacgcaaagtaatcaaatctacatgactccatttatatacttttaaaaggagcttcactgatccatggtgttaagaggtcaggatagaggttacctatggggagtagggaggaggcagagattgaggcaggtcccaagggttgcttctgggttgctgttaatgctgtttcttaatctggatgctggttctttggatctgtttgtgaaaatcctttttgatccagagtctctctctttttttttttgagacagaaaatcccaaagcgctgggattataggcgtgagccaccatgcctggcctcttttttttttttttttttttgagatggagtctcgctctgtcacccaggctggagtgcactggtgccatctcagttcactgcaacctccgcctccagggttcaagtgattctcctgccttagcctcccaagtagctgggattacaggtgcctgccaccactcctggctagtttttgtattttttagtagagatggggtttcaccatgttggccaggctggtcttgaacccctgacctcaggtgatccacccgcctcagcctcacaaagtgctgggattacaggcatcagccaccgcccccaaccgatagtgaaggtcttttcaatcaataattcccagatgttatctcacaggtaatcactacctgcagtgaaagctaatcacagcaggaaagattctgaaagctacttgcctggaagtttttcaggtttcatgatctacatgggaaccagaatttggagtaccagcaacaggtttttcaggatatttgctttcagaagcagccaccctattcccctgccctcagccagaagcagcacaatacctgtgggccctcccagtctccccacactcctcactagcacatgtgtggttcctgcgcctcctgctgcatctcccatgaacttgctctaaaagcttttttgttgttttgttttgtttctgagacagtcttaatctgtcacccaggccgaagtttagtggcaagatctcagcttactgcaacctcctcctcccaggtttaagtgattctcatgcctcagtcacccagtagctgagatgacaaacctgcgccaccaagcctggctaaacttttttgaatttttagttgagatggggtttcatgttgcccaggctggtctcgaactcccggcctgaagtgatccacccgcctcagcctcccaaagtgctgggattacaagctgggtatggtgtctcacccctgttatcacagcactttgggaggctaaggcaggcagatcacttgaaatcaggagttcgagaccagcctggccaacatggcgaaaccctgtctctacaaaaaaatacaaaaaatagccggacacagtggctcgtgcctgtagtcccaactactcgggaagccaagacaagagacttgattaaacctgggagacagaggttacagtgagccgagatcacaccactgcactctagcctgggcgacagagagagactcgagactccgtctcaaaaaaaaaaaaaaatacacgccactgtgcccagctgaatatttgcattttcaaaagatcaatggtgattatctctaggtggtgggagtataggtaactggcaccttttattattttttgcatttttatttttattttatttttgagatggagtctcgcctgtcacctaggctgccgggatctcgactcactgcaacctccgcctcctgagttcaagcaattctcctgcctcagtgtcctgagtagctgggattacagacacgcgccaccatgcccagctaatttttgtatttttagtaaagacggggtgtcaccatgttggtcagactagtcttgaacttctgacctcgtgatccacacacccaggtctcccaaagtgctgggattacaggcgtgagccactgcgcccagccgattttttgcatttttctaactgcccacggtgactctgtattatcttcagtataataagattcattgggatcctgtatctaattacaaaagcattttgtgctcaatgcagaaaacttggaaagcacaaagaagaacgtccccttaaccccatcatttaaaggtaacagctgttgccaggtgcggtggctcacgcctgtaatcccaacactttgggaggctgaggcaggcggatcacgaggtcaggagattgagatcatcctggctaatacggtgaaaccctatctctactaaaaatacaaaaaattagccgggcgtggtggcaggcacctgtagtcccagctactcgggaggctgaggcaggagaatggcgtgaacctgggaggcagagcttgcagtgagctcagatcgcgcaattgcactccagcctgggcgacagagtgagactcggtctcaaaaaaaaaaaaaaaaagataacagctgttaacattttggcatatgtctttccagacttttctctctataaaaatctttcatctttgtgatctcaaaaaaagtaaacatttaagagacaaagctggggccaggtgtggtggctcaggactgtaatcccagcactttgggaggccaaggcaggcagatcacttgaggtcatgagttcaagaccaccctggccaacatggcgaaaccacatctctactaaaaatacaaaaattacctgggcatggtagtgagcccctgtaatcccagctactctggtgactgaggcacaagaatcgcttgaacccaggaggcagaggttgcagtgaaccaagatcacaccatgcactccagcctgggcaacacagtgagactgtctcaaaaaaaaagaaaaaaaaaaagagacaaaaccttaggtctttagtcttcaattttatttctattttaaacagcaactaacagcttggaaatgtccctaacagctaggacccgccccatgcattccagaggctcccccaccaaggctggggtccaggttccaggaattccccctcatcaggcctgatttctctctggagacttgggacagaagaggctgtccagttagaggggaagttggcactaaaggtcaccgtttagaagggttgggctcagacacagctgcctttgttagtcttaggatattttgagatttggtagcgtgctcagattgtgggtatggagaagggttcctgaactcctctccggcctcacttgctcctgggcaagcctcacagcaccccttcctcttgctggctcggcacgctgcctttggaagaggggcacctgataggctgggtactccagcatgcctttgtgtgacccggtcagctgcagggaagcatgctcccctcaacttctcctggcgtaggcagggtgcggaatcagaaagatggtgaagattcagacctgagataccaaccccttaccaaccctcacctaaaagggaatattacaaggacatctctttgtgacttggaggggcacacctggatatttaaaccccaagtgtggtaatagctgggccaccaggctggaggcagctcaatgcatgcacttaagcagcaggggcagctcagcaggagggtagggcccacagagctggacctgccctccccacactgccatccacacccatggtaaccatggaaacataaccaccccactcctgccagctgcctgggttcagacaaccaggactggcccacttccatcaagccaaggcctaaactgatgccaggctggccacagagtggttgcaggaagaactgggattgggtgatttggtcagtccgggcttcccagcacagcttgggaggactaccacaggagcctccacaccttgctgtctgggctggggtcagacggggcttagtcagccagctcagtggccaccagagccggccaaatggccccgatgccctctgcctgtgggctaacagctactgtgtggcagtagcccttgctgcagcagcaaaagcctctgtgtctcattgaggggactctctggctggtgctctgcctgccctggctgctcagccagccctccgggggtgagtatgtaccgacagtcactgggagtgccacccactgcccccatgccactgccatccccagccccactgtagggctgatccctgccaggtagctccaggctgcctcccgcagtgggctcctcagctctctcgatgttgatgtataaggggtcctggctggcagatagcacagacagctggcccaagatgttctccagttccattcgcagacaagtaaagctcgggcgctgcttggggtcagcactccagcactggtacatgagatcatacacgtcctccatacactccggaggctgtttcaggcggttcccgccaatgaggtagttgtaaatctcagcgttttcgatgccagcatatggcgtctgcccacgtgtcatgatctcccacatggtcaccccgaacgcccacacgtcactctgcacagtatacaggttgtcggccaggctctccagggccagccacttgacaggcagtttggaggcacagccttgacgatagtagtccccactgtagatcttccgggagagtccgaagtcagccacacacactgtcatgtcctctgccagcatgcaattccgagcagccaggtctcggtggatgaagttccgagagctcaggtactccatgccgcaggcaatgtccaccatgaaccggatcagggtctggaggggtaggttaaaggggttctccccaatccgggaggcgagcaggaaggcatgcaggtccccatgcttcatgaagggcaagatgaccatggggatggggagacggcctttagccctgctccggaggcttaccccaacaagtttggccacgtgtggatggtcaaactccttcatgcaagctgcttccctgaggaactcttcaatgtcgcttgaggcaatgatgtcagctttcagcatcttcacagccactttcacaaaggagccatcctcttgcttcagctgggcctcccgcactgaaccaaactctcctttgcccaacatccggcccagggtgaactgctgctctgggatgagcacatcctccagtttttcctttagttcatcgctgatgcccaagctgtccaatgtggcctcgatgcgctcgggcctttctcgattgaaggaccgggctgcccggaagtgaacggctggctctccccgggccatgacactgtcaaaggcttgcccaaaccgcgtctctttccgtctctttcgaagcaggatgagggccagggcagcagccgtcaccagggccgttagcacaccaaggaccacaggtacccaggatgtgcggctgtgaggagggccctgctggcctgcacggtcatgagaagagaccaccagtggctgactccagggtccacagccaactgcattggagacgcacacacgtacgatcaggtccttttggggatcccagcctgtcaaattggccctggtcccctccactgtcagctcatcctgggttccattgtcttgaacccaggacagtttgtagggtcccagggggccttccaaaggggcctcggggatcacttcttcccactccaagatgaggcctgaatctgtgcggatggcatggaggttttggggagcgctggctggggctagacccttggtctgaaagggcacccagtcagcatagggagagggccccaaggcattggcacagcgcaccctgaggctgtagttggtggcaggcaccaggtcccggagcaggcaggtaaaggggggcacagggaccacaacagccaggacttcccagcctcctggggcctgtgtcacctgaactgtacaggactgtagcagagctcggccatcagcacctggcatccaggccacactagcgttgctgctggaaagctttgtcacggtgatgttgaagggggctgcaggcagtgcttgaaggtgaacagtggctgtgcgagaagaggccaggccttttaggttgtgagcttcacaggaaaacatggtgctctgggtcacccctgttacatttaaaacagatggagagggagcgggtcccccgatcttcgtagttcctctccaccagacaatggtaacaggttcagggggacccacagcctcacaagacagttggaaaggggcattgggtggcactgccagatcttttggctccactgtgaaaaatggcacaccttctaccgtgagccacactggctgggagatctcggtttcacccccatcctccacctggcaccagtaccggccggcgtcagagcgctccactgacttcaggctgaggaagccgatccagtgctgctcgctgactgggatgtacaactggtccaagttctggaccacagccccatccttcacccactggatgtcaggctcctccatcccctccacactgcagttgagcttcaccggctgcccctgagacactgtcagcttcaccggggctcccatgagcttcagaccctttgctgtgtgactctaggcaaagtcgtgggctccctgagcatcaggtccgcacctttcggcttgtaaatactcgtcaccccgtttcccttcccttccctgagaggctgatatggcaaggaatgctgtctcaagagaagatgccagcgggtggccgctgtcctggcctgtggctcttccctgctcccttcaccctctcaggaccagtcacaggatgggggccagcctcccgctccctatatgcccatcagtccccgaggtgcggggtgggaacttggagagcaccgtgctgcatggaacgctcttgtcaccagcaaatgcctc

SEQ ID NO: 18112 - RNA, 6671 nt, Homo sapiens
  source 1..6671: mol_type = other RNA
tcttttctttgagactcacttttcaaaactgctgttgttagatgatccttataaacatgttgctgagggaaagaagccaaacgcaaagtaatcaaatctacatgactccatttatatacttttaaaaggagcttcactgatccatggtgttaagaggtcaggatagaggttacctatggggagtagggaggaggcagagattgaggcaggtcccaagggttgcttctgggttgctgttaatgctgtttcttaatctggatgctggttctttggatctgtttgtgaaaatcctttttgatccagagtctctctctttttttttttgagacagaaaatcccaaagcgctgggattataggcgtgagccaccatgcctggcctcttttttttttttttttttttgagatggagtctcgctctgtcacccaggctggagtgcactggtgccatctcagttcactgcaacctccgcctccagggttcaagtgattctcctgccttagcctcccaagtagctgggattacaggtgcctgccaccactcctggctagtttttgtattttttagtagagatggggtttcaccatgttggccaggctggtcttgaacccctgacctcaggtgatccacccgcctcagcctcacaaagtgctgggattacaggcatcagccaccgcccccaaccgatagtgaaggtcttttcaatcaataattcccagatgttatctcacaggtaatcactacctgcagtgaaagctaatcacagcaggaaagattctgaaagctacttgcctggaagtttttcaggtttcatgatctacatgggaaccagaatttggagtaccagcaacaggtttttcaggatatttgctttcagaagcagccaccctattcccctgccctcagccagaagcagcacaatacctgtgggccctcccagtctccccacactcctcactagcacatgtgtggttcctgcgcctcctgctgcatctcccatgaacttgctctaaaagcttttttgttgttttgttttgtttctgagacagtcttaatctgtcacccaggccgaagtttagtggcaagatctcagcttactgcaacctcctcctcccaggtttaagtgattctcatgcctcagtcacccagtagctgagatgacaaacctgcgccaccaagcctggctaaacttttttgaatttttagttgagatggggtttcatgttgcccaggctggtctcgaactcccggcctgaagtgatccacccgcctcagcctcccaaagtgctgggattacaagctgggtatggtgtctcacccctgttatcacagcactttgggaggctaaggcaggcagatcacttgaaatcaggagttcgagaccagcctggccaacatggcgaaaccctgtctctacaaaaaaatacaaaaaatagccggacacagtggctcgtgcctgtagtcccaactactcgggaagccaagacaagagacttgattaaacctgggagacagaggttacagtgagccgagatcacaccactgcactctagcctgggcgacagagagagactcgagactccgtctcaaaaaaaaaaaaaaatacacgccactgtgcccagctgaatatttgcattttcaaaagatcaatggtgattatctctaggtggtgggagtataggtaactggcaccttttattattttttgcatttttatttttattttatttttgagatggagtctcgcctgtcacctaggctgccgggatctcgactcactgcaacctccgcctcctgagttcaagcaattctcctgcctcagtgtcctgagtagctgggattacagacacgcgccaccatgcccagctaatttttgtatttttagtaaagacggggtgtcaccatgttggtcagactagtcttgaacttctgacctcgtgatccacacacccaggtctcccaaagtgctgggattacaggcgtgagccactgcgcccagccgattttttgcatttttctaactgcccacggtgactctgtattatcttcagtataataagattcattgggatcctgtatctaattacaaaagcattttgtgctcaatgcagaaaacttggaaagcacaaagaagaacgtccccttaaccccatcatttaaaggtaacagctgttgccaggtgcggtggctcacgcctgtaatcccaacactttgggaggctgaggcaggcggatcacgaggtcaggagattgagatcatcctggctaatacggtgaaaccctatctctactaaaaatacaaaaaattagccgggcgtggtggcaggcacctgtagtcccagctactcgggaggctgaggcaggagaatggcgtgaacctgggaggcagagcttgcagtgagctcagatcgcgcaattgcactccagcctgggcgacagagtgagactcggtctcaaaaaaaaaaaaaaaaagataacagctgttaacattttggcatatgtctttccagacttttctctctataaaaatctttcatctttgtgatctcaaaaaaagtaaacatttaagagacaaagctggggccaggtgtggtggctcaggactgtaatcccagcactttgggaggccaaggcaggcagatcacttgaggtcatgagttcaagaccaccctggccaacatggcgaaaccacatctctactaaaaatacaaaaattacctgggcatggtagtgagcccctgtaatcccagctactctggtgactgaggcacaagaatcgcttgaacccaggaggcagaggttgcagtgaaccaagatcacaccatgcactccagcctgggcaacacagtgagactgtctcaaaaaaaaagaaaaaaaaaaagagacaaaaccttaggtctttagtcttcaattttatttctattttaaacagcaactaacagcttggaaatgtccctaacagctaggacccgccccatgcattccagaggctcccccaccaaggctggggtccaggttccaggaattccccctcatcaggcctgatttctctctggagacttgggacagaagaggctgtccagttagaggggaagttggcactaaaggtcaccgtttagaagggttgggctcagacacagctgcctttgttagtcttaggatattttgagatttggtagcgtgctcagattgtgggtatggagaagggttcctgaactcctctccggcctcacttgctcctgggcaagcctcacagcaccccttcctcttgctggctcggcacgctgcctttggaagaggggcacctgataggctgggtactccagcatgcctttgtgtgacccggtcagctgcagggaagcatgctcccctcaacttctcctggcgtaggcagggtgcggaatcagaaagatggtgaagattcagacctgagataccaaccccttaccaaccctcacctaaaagggaatattacaaggacatctctttgtgacttggaggggcacacctggatatttaaaccccaagtgtggtaatagctgggccaccaggctggaggcagctcaatgcatgcacttaagcagcaggggcagctcagcaggagggtagggcccacagagctggacctgccctccccacactgccatccacacccatggtaaccatggaaacataaccaccccactcctgccagctgcctgggttcagacaaccaggactggcccacttccatcaagccaaggcctaaactgatgccaggctggccacagagtggttgcaggaagaactgggattgggtgatttggtcagtccgggcttcccagcacagcttgggaggactaccacaggagcctccacaccttgctgtctgggctggggtcagacggggcttagtcagccagctcagtggccaccagagccggccaaatggccccgatgccctctgcctgtgggctaacagctactgtgtggcagtagcccttgctgcagcagcaaaagcctctgtgtctcattgaggggactctctggctggtgctctgcctgccctggctgctcagccagccctccgggggtgagtatgtaccgacagtcactgggagtgccacccactgcccccatgccactgccatccccagccccactgtagggctgatccctgccaggtagctccaggctgcctcccgcagtgggctcctcagctctctcgatgttgatgtataaggggtcctggctggcagatagcacagacagctggcccaagatgttctccagttccattcgcagacaagtaaagctcgggcgctgcttggggtcagcactccagcactggtacatgagatcatacacgtcctccatacactccggaggctgtttcaggcggttcccgccaatgaggtagttgtaaatctcagcgttttcgatgccagcatatggcgtctgcccacgtgtcatgatctcccacatggtcaccccgaacgcccacacgtcactctgcacagtatacaggttgtcggccaggctctccagggccagccacttgacaggcagtttggaggcacagccttgacgatagtagtccccactgtagatcttccgggagagtccgaagtcagccacacacactgtcatgtcctctgccagcatgcaattccgagcagccaggtctcggtggatgaagttccgagagctcaggtactccatgccgcaggcaatgtccaccatgaaccggatcagggtctggaggggtaggttaaaggggttctccccaatccgggaggcgagcaggaaggcatgcaggtccccatgcttcatgaagggcaagatgaccatggggatggggagacggcctttagccctgctccggaggcttaccccaacaagtttggccacgtgtggatggtcaaactccttcatgcaagctgcttccctgaggaactcttcaatgtcgcttgaggcaatgatgtcagctttcagcatcttcacagccactttcacaaaggagccatcctcttgcttcagctgggcctcccgcactgaaccaaactctcctttgcccaacatccggcccagggtgaactgctgctctgggatgagcacatcctccagtttttcctttagttcatcgctgatgcccaagctgtccaatgtggcctcgatgcgctcgggcctttctcgattgaaggaccgggctgcccggaagtgaacggctggctctccccgggccatgacactgtcaaaggcttgcccaaaccgcgtctctttccgtctctttcgaagcaggatgagggccagggcagcagccgtcaccagggccgttagcacaccaaggaccacaggtacccaggatgtgcggctgtgaggagggccctgctggcctgcacggtcatgagaagagaccaccagtggctgactccagggtccacagccaactgcattggagacgcacacacgtacgatcaggtccttttggggatcccagcctgtcaaattggccctggtcccctccactgtcagctcatcctgggttccattgtcttgaacccaggacagtttgtagggtcccagggggccttccaaaggggcctcggggatcacttcttcccactccaagatgaggcctgaatctgtgcggatggcatggaggttttggggagcgctggctggggctagacccttggtctgaaagggcacccagtcagcatagggagagggccccaaggcattggcacagcgcaccctgaggctgtagttggtggcaggcaccaggtcccggagcaggcaggtaaaggggggcacagggaccacaacagccaggacttcccagcctcctggggcctgtgtcacctgaactgtacaggactgtagcagagctcggccatcagcacctggcatccaggccacactagcgttgctgctggaaagctttgtcacggtgatgttgaagggggctgcaggcagtgcttgaaggtgaacagtggctgtgcgagaagaggccaggccttttaggttgtgagcttcacaggaaaacatggtgctctgggtcacccctgttacatttaaaacagatggagagggagcgggtcccccgatcttcgtagttcctctccaccagacaatggtaacaggttcagggggacccacagcctcacaagacagttggaaaggggcattgggtggcactgccagatcttttggctccactgtgaaaaatggcacaccttctaccgtgagccacactggctgggagatctcggtttcacccccatcctccacctggcaccagtaccggccggcgtcagagcgctccactgacttcaggctgaggaagccgatccagtgctgctcgctgactgggatgtacaactggtccaagttctggaccacagccccatccttcacccactggatgtcaggctcctccatcccctccacactgcagttgagcttcaccggctgcccctgagacactgtcagcttcaccggggctcccatgagcttcagacctgcggcggcggactccgggagcagcagagaagccagagccgccagcagcagcccgagccgcggtggcggcggcagcggcagcggcgggagccccggccgccccatgctccgcctcagcgccatcggcggcgacgccgcaccatgccgggcccggcccgcgagcgaggag

SEQ ID NO: 18113 - RNA, 546 nt, Homo sapiens
  source 1..546: mol_type = other RNA
tgaagccagctctggtctgggcgtcctggcctcagatgcaagttcgagtttatctctctgcaggcccctgccagcagtgagcaagacagatggcttacctcctttccttcttccacagaaagaaaacttgggcagagccgcctcacagatgggataggagaaattcaaaacagatgagccttgagacatgagagctaggtcaagaaaaagctctttgatgtcctctctcagaataattccaaatctaatgttgatatttgattttaattgcttggaacacttttcaacagaaaagccaaaatcttgtaatggatcgcaactctggtagagcacttccaagccgctgtcgctacagaccacgtgtgtgggccaggctttcccaccgccgcctccactgcagctgggaaaaatcagagtccagaggaagagagtggctgtgaaacccttcatggtgggggcctgtatgggacacacagaaaaataaccggccaataaaaagcctgtaaaatttcttcctctcccctcaccaaggcagttggatgttca

SEQ ID NO: 18114 - RNA, 869 nt, Homo sapiens
  source 1..869: mol_type = other RNA
tgaagcgcctgtgctctgccgagagaggggaattgagtcactgcgtggggtcttccatggtgccctggagggcacttggaggaagctaactagaacaaactgggcactgtccacgtcgctgggctcagcaggggtcacccttcccagggtggggactatgaggtcttcactcaactgtgatgccacaccagattatcttgctatccagcatgtcctcagtctgaactgtgctctgaccagacaatcacaccaagacccaactcccccacacaatgcgactgagatctgtgtttttggagatgattgcctgatttctcccaaaaagggttttaacttttcatagacagggggattctaggagcctcatgactttccctaattttccctccacctccaacacgtacctgcccacctcgtccaagccccgggcttgacaggtgtcccctctgagaacattactgcactgactttgtccccgagggtgaggtgaaccgctggggactgatgccagggactggggagtggccgtgccctgaaggaaggtcaaggcacaggagtcatgtaacgcaccttctccaaccacagcacaaccatgtgaggactgatgacaagaacggagtggaaaatacccggccatcccatctctgggcacagctggctcaggggcccaggccccctcctgaaggaagaagttcacacagatctgcgactggggctcccagactcccacttcctcctctcactgtcacccctcttgtgggccttactcctttaggggcagggctgggagaagaaggggccgggtgacactggtgtgggaaggggaagcagctaggggcatctctaaggctgctctgagctggcccagg

SEQ ID NO: 18115 - RNA, 1055 nt, Homo sapiens
  source 1..1055: mol_type = other RNA
tgaagcgcctgtgctctgccgagagaggggaattgagtcactgcgtggggtcttccatggtgccctggagggcacttggaggaagctaactagaacaaactgggcactgtccacgtcgctgggctcagcaggggtcacccttcccagggtggggactatgaggtcttcactcaactgtgatgccacaccagattatcttgctatccagcatgtcctcagtctgaactgtgctctgaccagacaatcacaccaagacccaactcccccacacaatgcgactgagatctgtgtttttggagatgattgcctgatttctcccaaaaagggttttaacttttcatagacagggggattctaggagcctcatgactttccctaattttccctccacctccaacacgtacctgcccacctcgtccaagccccgggcttgacaggtgtcccctctgagaacattactgcactgactttgtccccgagggtgaggtgaaccgctggggactgatgccagggactggggagtggccgtgccctgaaggaaggtcaaggcacaggagtcatgtaacgcaccttctccaaccacagcacaaccatgtgaggactgatgacaagaacggagtggaaaatacccggccatctgggaattacaaaaacaacccatcagccaaacaagaaaccataatggaaaccgatatttggaactgaatgatgaaaaagtacttcacagtaaaacttgtaggatccacctaaaattgcatggaaggataattctatggatttaaatggttatattagaaaagaaggatgtctgaaaagtaatgagccgaacatccagctcaataaactagaaaaaggggaacaaagaaagaaggaaataaaaaaataagagcagaaattaatgaaatggaaaacaatatacaaaacaaaggaataactaacgccagaagcttgatctttgaaaggacatcagttttagtgatctgtttcattgcagtgaccgcagttaataataatgcattttatgtttttaaattcttaaaagaatagattttaaa

SEQ ID NO: 18116 - RNA, 3443 nt, Homo sapiens
  source 1..3443: mol_type = other RNA
tgaagcgcctgtgctctgccgagaggaggtgctgttaacgggatcgggcaccggtgcgagaaggctgggcgggttctttttgtgaacgctattcataccaggcattttagtgattttacaggctttgctactagaactcgagttcttacgcttttttccttctgatttgtcaaaagagaggggcagagaagacacagcattgtgtgaggccagagagaggtcccctgcgtggagcgcaagggagggcacagagaggggacaggagtcactgctgcctcccaccgcgcccacctgtctcactatgtccgcggggccgccgggcagcgaggtccgtcctgagggctccagtttggcactgagtgggctcaccccattgtttgagttgtgcacagacaggctgttatagggaggggccgcctgataggagttcaaagcagaactggcattcaaaacacagttctttttgtgaggccctgacagtggagacgagagggatgtctgcaaggaagaggaggaggaggaggaggaggaggaagtcgaagactgtggcttcctttttttgttacttggagactcgtcgctacgggtggacaggtctttgacttttgaggatttgctggttttggttttggatggcttgtgggatggggaagggatgacggctggtatcggggacacggcggatggggccttgaaggttgagtccatgatgctgagggttgcggccacatgagggaaagctgtggtgtgggacatgagggcgctcgggtccggcgatgtcacgaaagctgcgtttgagagcatggctgatgtcattatgtaagaagaggtgagcctcgagctgatgggagctgaaggaagatacacagcactggggttgctgaaaggctgcaaaacggatgctggaacgggggtggtgatgtgggctgctggcgagggcagggggctatctgccgcaggagggatcttcctggctgaaagagaatactgtgttggcggctcctgatgcagagttaaatgcttgttaaagaaaaaagagtcttggccgttccttttcttcctaatgtcttccacgcccccatcggctgccatccctccaggttcgggcccgccggggcctggggtttgggcagcgaggttgagagggtagcggggtgctacgctctccagagttgacacccaggcagccccaatgttgctcagtgacagcagattggttaggcaagtcctgaacaggggggagggacctgatgccctgtggctcgggtttctgtgcttccacatctgtgaattcaggtgtttttctaccatggagtttagtgcgaatcgaaaacgatcccatcttctatcaaacacatagtaccctcgtcccatgaggcgactcccaaatgagcaaaacgccagaggtctggggtggtgcgtggagaactgacagtctagcttctcggattcgtcggctccgtccatctccccttcatcactggacagtcggctggcgaggtcacctccaaccggtgggagtgggggctctggagtgtggccgctatgatttgaagatgtgctgctgcttatgctatttgcagatgatggtctaggaagtacagagttgggtggtctggattttgcaggggatgcaacttttggttctggcccagagctccctgaagaccctagcagagaatcctgtgccggcccggattggcttggaagtatttccctcgtggaagtcaggagatgctctttatctttaacttctttttcccgggactttgctttgtgttctgccaggaggaggtcaaattgctttttccggcctgggactgccctccgatggcttagcgaatgtgtcttgcaggtgagggatcttgtgcaaggtttctttgtctcgggatccaatactccacagtgtttatttgggtcaaattctctctctgaaagtctcctgtaaggcttgttgctgtttttggtgccattttggtgtttcttgtctatggtggttggcagaattcctttgccatttaagatcttctctggtgaaggtggcactgacttggacatcaggacaggcttaattaaaggaggggtggagacggcagaggacgaggtggaggaggcagaaactgcagtagtggttgtggagttcattttgacattggcaccatctgccttcactaggttaggaattttctctaaactgactacaggaactggaacacatggtttatcccttgatcctttcgcaggaaagactgtgtgctgtttgctgctggaggtaagtagattgtctttgggcgttttgaatggctttgaggtgctgctggcagagtgatggccgctgagacaggcttttgttttcacctgtactagtgatgtcctgggattggaggctggagacactggagagggagaaggtctacacattgaaccgtgtcttctctcgcagtgcgactggaaaacctgtggcttgacgacctggttacaggcactgcacactacgagatagaagtcgtcatgtgctgggtaatggccaaataagtgcatatcttctttattaagcctcataacctccctgctttttccaccctcttttccagcctcttctaaatctacattgtcggagcagtgtaatttggcggcgtcgatccaggaggaccagggtttgcccagaaacgcctccggactgggcactttgcgatccagtgtcgccattgctcttccttcttgttgctttttccctgttccttcggcagcagcagccgagagacacgggattcgagaacgctccgacgtcatcttcggaacgttccgacattgagtgttccccgtcacccctttcttctctttcctggaggactttggaccatggagattctgcagttgttgctctaggagctgaaaccagtgggtagatgtcgttctgaaacgcaggtgagtttggagcgctacgagctaccttcccatctcaggctgcggggcgtgcaaaactcaaaagttagggcccccggacccccgggttccccgcgcggtgcgtatctccggctctcagagaaccactgcatggactttgctccagggtcagcagagcgggagggcgaatttacggctcttggaagacgacgctaacgggcctagcccctgagccgtttccagcgctccctgccgtgagacgagggtggcccgggtttgcgcaggcaacctttggccaggaatctgattcctgggagaattcacttcaggcttaactgctctagccagctagaaagggagcgctagatttcctctggattttggacgttgggtgctttagttgagattttcaccctttaaagaaggctttaaaaagtcttctgttacttctttttaacaaatccttttgtttactagaattatctaaactatatggacaccgccctcaccccacaagcgacatatttttttttctc

SEQ ID NO: 18117 - RNA, 9492 nt, Homo sapiens
  source 1..9492: mol_type = other RNA
tgaagctctgacattcctgcagctgaagaatatgacctgctttggcctctaggacttggacaggtcataagggacatgactggggcagcgccgacaccctctgggggcagatgggacatgcagtccacaggagtggtcatctcctcttactaagcaggtgaagcagaacttccagaggctgagacagcagcctcgacatagctctgtgctttctactctaggccaacataataagactcactcctgccttcatcagctatgacaagagctatggcagtgagtgacccaccaggaaggaccccccccatcagtctcctaatgaagaacctaagtccgtgctgtcctatacagcaaccagtagtcaggtgtggctattgaacactggaaatagggctgggccagactgagatgttttctaagaggaaaatcacattggattttgaagacttcatttggaaaaaagaatgtaaaatatcccagtaatttttatattgattccatgctgaagtgatactatttttgacatgttaggttaaaatgtagtctaaaaattaatttcactgattttagctgtttctttggactttaaaaaatgtggctactagaatattttaaattgcatatgtggcttggatcatggttccattggatgacgctggtctatactaccttcctgaagctggttccatcactgtgacccagcagaggagaggaaagttgggattgaaggtgcctctaatcatgggttgggtcactggccaagctcgacgtgcctcccctctctggggcagctggtcttctcagtcctgcagggagacagctgtttatgctgcagatttacctaatccctgctcctctttcctacttcctattacttcagggttactgctttgaggatccttctctgctgccttgctgaggattttctggtgcttctgccatctgtccttcccaaagctccgttcatcttacctctgctcccaacccacatcttctgcctactgcctccacgccaccactgcctccaccatcttcagtcttatttggtagcaacccttggccagactccctgcttctgacactgcaagccacatttatatggtgagtcataaattacaaagcaattcacacatcatctccttggatgctctttctcctaccccagcccagtgcagcaaagctcagtcagtagagactgatagtaaaatgagatcgtcaaagtgggtgggaaaaggaatctgagaatgaaacggtagatagaaggctctggactctgagtgcaaactggctgctagctcaaggtcactttctgaggggcgaaagcagaggccaggagtagcagagagaaaacatctcctaatttacctccatgcagtaagcacgcactagcaagggctcaaagtctctctagaaatagcagcaaaatacacaaggggactgcgcacccccagagccctggaagcccctgatccccatttggctgagaagacgtggagacaaggtgaggtaatgagactcccccaaggccctgagtgagccggtgacagggccactcatgccaccccagagtcaggtctttgtcatgacccttgccatgacccttcaaacattgctgatttacttttattttgggggaagtgcattctactttacagggaaaaacctttagaacagagagttctaagcagacactgatgactgtgagagaaacaaccagaaaaaaacctcctgtgtcaatggtatccctcccttcatatcccaccctaactcaggattttagggccgtccacagaagtcctcagaaaactaagggctacatcattgcatttgtttaatctcaatctccctcccctttattttcagttttcacttttatttgtacatttttacagatagtcttgaatagcaaaacagtcacaccatgggtggaaatggggaaggagtatgagaatgagttcatgaaagctcttcacaggaaaggcttcgtcacgctcacaacacagacgcactggtacagacggagagggtctatgggtgacccggaaaggaaaggaaaagctcagccagtgggaggaatggggttctggagaggagagagggatacagagttccttaaggagcaacacctggtccttgggaatgaagtgtaggagttgcatttgctgaggttggtgtttgccaaagagatgccagcttcttcgaactactgctgtgcaactcttcatgttcagacccagttttctgtttttcacacctgaacatacacccccctgcagttgggtggctcccccgttaccagctgggctctatctacagagagagcaatggcttcccttcccttgaaggaagtctcaccctcacaaggacacttgatccgctgcaaagcagaaagtgtgcggaccctttgggaagggcgttcttttcttgtttagaacctaggattctgtttttcccaaacaggatcacacccagacacgtcttagtgaatgtaccatctaaagggcttccttatatgaattcatatgtttttgacgaagctactggcttcagcaactgacaagagaaagaagatcccagctccttgagacttggtctcatcctaaacttgaaagatcattgaaacctttcagaatctgatttgcttccacccattccttttgggaatgtacagctagaaataacgttaggagaattaaaaaaaaaaatactaaggcattgaccatgtgccttggttaacagttaactggtttagctcatatatgctatttgccccatatggtttactcattctgtcacctctgggaataactgagatggataaaagtgccctttgcaaaactggctctagacaaaaggaagtctaggaataggtaaagaaaaataaggagccaatttctctgggggacctgaatgaagaatagaatcctttaagtgtgcttaagtgcgacaggtccagccctgttcagcaacaaagatgaccttgcactctgggttatccttcagcagcgaggcacagacacttgatgtgagaattccattccagcggggggtcttctgagggataattagaacatacataactcatatgacacttcatgtttgcaaatcactttgcaatttctttgtcacccttaatataccatgaggtaaggtgttatcacttatcctcattttgtagatgaggaagttcaagtatggagaagacacagtgcccagagtcacaaatcatttcagtgcagagctgtagtgaaatttacagtaactgttacacaagtgtagcttaatgagtgagttactctggcttccgcattcttacatctatgattagattgagatggcaactgaccaaaaaaaaaaaggaaagaaaaggaaggaaggaaagcaggcagacaggcccaaagagacatcttttagccctgctccatcctgcccctaaggtctggcattaaacttttaggcctctttgctatctctgggggctcagggccctgcactcttgctgccaggaacacagggtcaactcaacgcagaccagtgcggttctgtggtgtacactgctcacatggccccagctgccaacccagagacaagcactcattggggaagttttgaggtcatgaccatttggattgggcccgcggtagatgcctcagagtgactggattatgaaaaatcttgtagtcttttttgtattttatttttcttattttctacaatgagcagttattattcaggaaagaaatccaatactcagtaatcacatattctaagaaccaggaataatgtttaagaaacattttgcatcatggcagcatcaatgaaaagagggcaaacacagccccagacattgagagctttgagagacagacacgagaatcacgtgtgtatgtcaactctggtggggttcttaaaaatctgcccccttagtctatcccacaccagctggaagatggcatggaaggcaaccctgctggtgtgcaccagctcttcctatctgcactgaaatcacctctcactcagaaacatcgtatttccctggaaagggctggctgtgtcccctgggatggatgtgtcccctgggatgggtaagtcccctgaagacagggaacattttcagaaaagcaacttcactttaactacaagaatcaaccaagtatcccccacaaaccacaccaaaggatgaccagagtgtatctcttcccactccttcccccagatatttgaaaaatcacttaacactcagcacataatccaggtgaagagagagtccattctaaatgcctctgggtgatgtacctgagttcattattctgaatttgacccaggtgggcatctttggagacctaagcagcacatcctcccactaaatcaagacagctacacacagtgcattcatttccggcatcttatcatgagtgtggatgaatattgagatatagggcccagtctcagagtcctaggatatcctaccctcttgtcacaggagaggcaagcattgctaggtgggaccactcatccctgatgggaagatatgcacctgggctcagggcgcttaagaaagtctttgtctagatttggaggagttgtccagtctctgtgactccatgatccctgaagttgaaagggtagggttgttgaaaagctaaggcttggaggaggattgaagctggaacaggcacagattttatttttcatattttgatgccagggagccacagacctccttataaaacctacagccacaatgaacaaggaagggggctgcttggagtctaggagcctctctacagatgaatcacttgtctatgttaattgaccaaagttgatgcaggagaaagtaggagtgagtagagagagaggaaacggaaacagaagaagaaaccgtaactcccaaaataaggagaaaaagatatgggacctctctctaggtagaatacctcactttcctgaatctcaaggtagtagagtagggaaggaaataaaagttgcaatgggccccaggctcaaggttgacttgcatggagctcaaagcacatacatgttcatatgccagtaagaagtttgaacttgacctggggttgcggctggtgactttagtgaggtcattgaccctaaatgccctcataaggttgggttccactttgatttggagttagcagagtctgacctacagagcctcacaagtcaaggctcctctcttcctcctcctcatctccctcagctacctcacagccagaaagcttccgtaactggttggagtcacatgttttaatctgtggtcaagcccttatgctagagggatcaaggtcacctgagaagtcctcccattggccaggacttgccgtctgaaaggggcctctatcctggtcatgtggctgggcgtcttttgcttcccagcaggatcagatcccaaagtgtgttcgtatttatctggtcctgctatcaaagaagtcactcaaagcccctgctctgggctggtgagttgagcccaggttgtttacgtctttcctgggagctttctaacatttcaggaactctcaaggtttcaaagggatgcagtaagctttgctaaatgtctgtcacaaagacaataattggatagagcagataatctattcattgaaagtatgggatttttttttaaaaagaggatataaataatgataggtctgtgagccagcatcctcaaacatgattacttacaaaaagtttaaatggttcatagcaaatttccccatttagaatttttcccctctctcctgcaactggaaaaaagctggaatttcagtgtggtcatagacaagccctctcccccaaatggatgcttgtgaacctgtctgtcccttcctcggcagagccccttcaggacgcttggaaggaagacaaaaggcctctcaatctgagatacttttcttcacttttccttaagcccaagtatgcccttccccttaagggagaaatctaacttttcaaagaaaattagaaataaaatgcccaattgaaaaactgggttttcctgaaaattatttcccttctcatagaataaatcctttgttttaaaaataatccttagaaccccaactggaagctaacaacttttcccgttgcacaccttaccctatcgcccagcacacccacacacagggaactcacacatgagaccttttgcagaagctgaccagagtccccggtaaggaagtcttgagtagggcacccacacctgtgtgcaggtgtgtactgacacaaacgtacacaaaatgcaccagagagatacacatacagagagatccacattcaaccccattcatgcacatcagatgtcatatcatatccagatatgaattacatacacgcagttcaaaggagcagatgagggtggaagatagaagagagagaaggtaagtggttagtaggtgagaaaaggaggagagtggtaggaagatgggttggaagacgtgtaaatgaaacagattacacagcagtggaagaaaggctgctgagtgcctggcaaagctcccaaagcatatttgtttatgaaacaaggggattctctgctacacagttgaccatggctacaccagctcagggattctcacctggcctccccagggctgctgggcaccagcaggctcactgagatgactgtgagcggctccagcccactccagcagactcccacccctacagcgttcacaactctctggctgactttgcttgccagcacctgcagtgctaatttgctcaaatgagcccgagacactggggtggatttattccacctctgtttgggtgctagccactaagactgttattttgggattcatggccttgaatatcaagagggaaaggaagaggatggaaagagtcaagagttctgcattaatttacacaatatcatacaaacttgagcccatgggaaatggaggtgctctctctgcatgtgacccacttcctttcgtttgtacagaggtcacccctagggaaaggggagatgtccagtgacaaaggacagcttctataatggggagtgaaggtcttgttggtttatgttcttgtacaacagcaaccagagcaacatttcttctctctcctgaactgtgtgttccccctcttctctcatggcttatgtgcccagctgtgtcttgaacttccaaaattagaggactaaatcgtgcagagtcccagagctgtaatgtggagaaccacgggggtcctctggcccagtggctttgttcttggttctgccctctggaaatttcagctataccagaaacaatttaaaaaaacacaacacaaacaataaaaccccacgctcaagaaacatccaccacacacacacacacacacacacacacacacacacacgcacacacacaccactccagggatctgtagctgcagaattggcacccttataggcctgtccctcatgacaatttctaggtctctgggcctctatctggggccatgaaaccactacagtgataagagagacaacagtcataatgcagtatttccatttaaaaggtagaaaagaaaaaaaggaaaccgcccaaagtacacatgcacgcacacccacacacacacatcacagcatgactccaaggctccagtctgcccagggagtgcaggtgcggctggggacagggtggcctcttgtttcactgggtgtaaggcagctggaaggtaagactgggttgtctgagcatccaccgaagcgtcctttcattgatgcagatcttgcctctcagcatgttctcttcccttcccacctatgaaacatggtccaaaagtttggcagcaaagagaaaacgtccttctcagtttgttttctcttccactccttgtgtgttgctggtgggctgggaaggaagtccgaacaggaagagcaggagaagaagtgattctgaaaatggcctcaataatttggttacattctaggaactgagggctttgttaccctgtgatatgactggttaggggtggcgtcctctcccgttgacccagtgggtggcacttccttctctacatctgtgctgcctcagaccccttccactgtcccttcaccaccccatcctcgccagtgatggggatcaagacgcggtcgcaagtggtggtgtttgctctgtcttcaagagaccatgaagccaaaagtcaagaactgatggaagagccacaggatggaaaaactttccccatctcagagatgaggcaacacaaagtccggcgagatgcaggtgcctgagccaactcaactctaccttggcactggcatcgtcttgatttagttttgttttgttttatatatgtatattatatatatatatttatatatatatatgtatgtatgggtttgttttttagcacactgtcccattctcgggtctggatttagggtagttggtcctcgggacaggttgaacagaaggggctaaggtacagaagaatcccgagatgagtgtgaggcccaggcccccccatgcacagaacatggaccagccatagccatggctgatgtcatcagggagtccgtacaggtagcgtgggtagcgtgacagctcaaagttgatcccggccacacaggtgcacagtgaaatgatgcagaaggttcctcccatgaggaagagcagccctgccacgtactgcataaggcctcggtcccagcagcagcccagcacgccgatgatccagccaaagaggatgatggccaccgccatgcccatgaagccagccgtcattctgcgcaggtgtagggcatgccactcatcctgacggatggtcttcgtgatattgaaagtgaggttcctggggatggttgctgaggagtagtggtatttgatgtacgtacatcgctcaatttctcctttccgaatgagggcggcgatctcggggtcgaagccctgccggtggcacttcctccagaggcccatgttggtggagttgtactgccggctgcactcgtccgcggggctcatggcgaacagctgccggcgattccgggcccggaggagtttgccctcccagcggtccaggcgcgagcggctcgcccggagcggcaagttgttgttattgttgtaaatgaagccggggtcgacccggcgggtgttgaaggccttgcacctgtccctgtgcttcctggcgtccgtctcgtaccagtggtccgagcagatggccacggccagcatgccgagggcgcagagcgctagcgagaggccagtgtagagcagtaaccttccggcagccatgcctccgcttggcggctacaccatgggcatgatccgccgcagcctcgccttccctcgccgcacccggaacaaagcggcgggcggccgagctgggggagggggcaggagagggactcgcgccgcggcgccccctcggcccccgcctaccggagcacggcccggggactgcggggatgggggcgggcggcctaaaaagttctgatccggagaggctcccgcgggctcctgggcatcctctgaggcaggt

SEQ ID NO: 18118 - RNA, 89 nt, Homo sapiens
  source 1..89: mol_type = other RNA
tgaagctctgacattcctgcagggcggggcctctcctgtccatgtctgcagagctacctgctctaacaaaacaagaaatcttcggtaga

SEQ ID NO: 18119 - RNA, 3589 nt, Homo sapiens
  source 1..3589: mol_type = other RNA
tgaaggtctactgtgtgccaggaaaacaatgtcgcatgtagaacatggcccctatttctttaatatctgtaaagttaatgattgataatgattaataacaataacaagggccgggtacggtggctcacgcctgtaatcccagcactttcggaggcagaggtgggtggctcacctgaggtcaggagtttgagatcagcctggcaaacatggtgaaaccctgtgtctactaaaagtacaaaaattagccaggcgtggtggcaggcacctgtaatcccagcttctcaggaggttgaggctggagaattgcttgaacccaggaagcagaggttgcagtaagccgagatcacgccattgcactccagcctgggcaacaagagtgaaaactcagtctcaaaaaacaaacaaacaaagaaacaaaaacaataacaagaaaaatggtttgtaaatttcagatttttttaagagctagaatggctctcaggtttaatctaggccagggattttcaaactcttcagagtccctgtggacccccatgtacgtaatcaaagagatgaaggtttgtaggtgctctggatgtccaaaccctgcttataattcacataggaattcagctttttgacgttttatatgttggggattcattgaaagatttatttgaacaaagagttgtaaggttaaaacatgttcgagaatcgtttcctagtgtaatctaatttgacaaataaggaaacaagcttgtagaagttaagtgacttgttcaagtcaatccagtcaataatgccaaagctaaggatagaaatctatcttctagcccaatgttctttggataacacataccatgtccacaatttctcaatatagggagcaaagcagctttctagtcattacatctacttaatacagtttattcttacctattgtaaacctggcttcctatagaatatgcgttctttgcccagactgttatttcttaacatttgaagcattgtttcttacacttaaggaaaaatccaaaattagggacccctatagtttgctttaagttggttactggtagtaatcttaaattttataccagaactcctcactaggagaactcaaggtagtcaatgcttagtctccatggctctgctctgtcctgtgaactatagtttctagatgtcacttgtggtaaatccagctacagatttccttccacccttactttaatcaaaatctatcaatccattccttctgggagaaaactttgtctgtaatgaaggttgaattttaaaactctggaaaagggtaccatagtcccagtctagaattacccatcaaacacatttgctatagtcctactatgtattcatttttagggggagaactgggattgatcagtatttataaggatagtatagtttaccttttaggtaggcaattctaaaggatccatcaataagaagctctaggattaaaaataaaatacctctatggaatacaaattaggattcttgggacagtctggcacaaaaaggcattcagggacaggaagcaaagacaggcagtgtttggcttgtaacaaacagaaaagccctatacaaaacgaagcagcgctaatgacgcttttactgttcagtgttccctcagctcagagtaagtaggccgactgtccacaggtccttggatccaaaacagtcccctacccagagccttcatttcagcccatgcgtgttcattagggaaaagtgagggtcctggggtgtgctccctgccccacctctttctttgtccttcccgttgctctctctgctgctgaccatgcttcaaggtgaaagcccaggcatgcttcccagtgcatccttgagatgttaggtctttctgagctaaaagaacaaaaggatgacattgctggactgaaaatggcccttcaggctgtagtcattttgcagctgcagctgacctggaggtttagttcctgtcttccttggctaccataacactggcaggggaggatgaggcagttgaggccagcagtcgtttttggtgtagctcttcccacttacttctgtttgtagctactgaatctagcatcggcttcagtttcacgttgaccttcaccagtgcctgatacaaaggcatgcagatgctatcaatccactccagttgcaaccgaggcagttcatccttccggttccgatcaaaaattgctgaaggagtgagtttgagctctaatctctcccgatctccttgttcgaagaactcactggttacaagttctgccacctgtctggagatctcccacggtttggtcacggctccaaggtcacaggctgtcattaacattgatcgaaatatatcacgatggtttttgatgttccaatcgtattctcctttactgacaagttcaaagaattcagttctcctctcaaagtacagcgtgaggtctgttgccaatattgactgcttcaaaagctgcataaggtcactatattccttggaggacaggttagcaaagatattgtgaccctcactttgaaggatcatcacggcgtggttgaaatggtgatgctccaaggtagcagaggttccatagagttgggccagggcagagccactcttagcttggaaggcattgttggttcccctgtggtcgaggtcatgacacaggcatcccacaatcaccgctaaaatttccacctcggtcagaatgtcttgaaacccagcagtggttaacatcgcgaacatcagctgacacacgttgaaggcatgtctccagttgtggtatagaaccatccgatagtttttcctcactgtcaaaagccacctacacagtgtctcatagtcaattttaaatttctgtaccatccccagctccatgaacatccggagagcagctgtgatcatggcatcaacgtcgagagaaaagtcatcaaaatgaatgtcatcgatggcaagttctgacaccagagggatgttggctgccttaaacttgtcaacttcagcttttgaacatgttgcatggtatgatagcacatcaagagccacagactgcttggcccaggacttcttcacttgatcatacataattgtgttgttgatgccaagtccacaaaagatgacaaaagcctcaaaaagtcgttgatctgcatcatcaaaaggtttcccatcaagtctgtttaacacttgagccactccaattatttggtggttgctattccaaatagggacacaaagaacagatcttatgtgaaaaccagatatctggtctgcctctgcatcaaagcgcggatcctggtaggcatcactgatgttcactggaaggcctgttgaagcaaccagctcagcaatgctgttatttattagccagtcggagtatgatgatttctccatgctttctttgaaactgttctcagcatcagcactgcactttggggacatcaattcaaaggatttggtaaatttcaccacctgttgagagaggcaatccacaaaaccaagccatgcatgtcaggactttaaggccctagttcagttctcaggattgtatttgcagtgagcaaacctgggagatgaagtaacatctttccacagacaaacatcaggctt

SEQ ID NO: 18120 - RNA, 3812 nt, Homo sapiens
  source 1..3812: mol_type = other RNA
tgaaggtctactgtgtgccaggaaaacaatgtcgcatgtagaacatggcccctatttctttaatatctgtaaagttaatgattgataatgattaataacaataacaagggccgggtacggtggctcacgcctgtaatcccagcactttcggaggcagaggtgggtggctcacctgaggtcaggagtttgagatcagcctggcaaacatggtgaaaccctgtgtctactaaaagtacaaaaattagccaggcgtggtggcaggcacctgtaatcccagcttctcaggaggttgaggctggagaattgcttgaacccaggaagcagaggttgcagtaagccgagatcacgccattgcactccagcctgggcaacaagagtgaaaactcagtctcaaaaaacaaacaaacaaagaaacaaaaacaataacaagaaaaatggtttgtaaatttcagatttttttaagagctagaatggctctcaggtttaatctaggccagggattttcaaactcttcagagtccctgtggacccccatgtacgtaatcaaagagatgaaggtttgtaggtgctctggatgtccaaaccctgcttataattcacataggaattcagctttttgacgttttatatgttggggattcattgaaagatttatttgaacaaagagttgtaaggttaaaacatgttcgagaatcgtttcctagtgtaatctaatttgacaaataaggaaacaagcttgtagaagttaagtgacttgttcaagtcaatccagtcaataatgccaaagctaaggatagaaatctatcttctagcccaatgttctttggataacacataccatgtccacaatttctcaatatagggagcaaagcagctttctagtcattacatctacttaatacagtttattcttacctattgtaaacctggcttcctatagaatatgcgttctttgcccagactgttatttcttaacatttgaagcattgtttcttacacttaaggaaaaatccaaaattagggacccctatagtttgctttaagttggttactggtagtaatcttaaattttataccagaactcctcactaggagaactcaaggtagtcaatgcttagtctccatggctctgctctgtcctgtgaactatagtttctagatgtcacttgtggtaaatccagctacagatttccttccacccttactttaatcaaaatctatcaatccattccttctgggagaaaactttgtctgtaatgaaggttgaattttaaaactctggaaaagggtaccatagtcccagtctagaattacccatcaaacacatttgctatagtcctactatgtattcatttttagggggagaactgggattgatcagtatttataaggatagtatagtttaccttttaggtaggcaattctaaaggatccatcaataagaagctctaggattaaaaataaaatacctctatggaatacaaattaggattcttgggacagtctggcacaaaaaggcattcagggacaggaagcaaagacaggcagtgtttggcttgtaacaaacagaaaagccctatacaaaacgaagcagcgctaatgacgcttttactgttcagtgttccctcagctcagagtaagtaggccgactgtccacaggtccttggatccaaaacagtcccctacccagagccttcatttcagcccatgcgtgttcattagggaaaagtgagggtcctggggtgtgctccctgccccacctctttctttgtccttcccgttgctctctctgctgctgaccatgcttcaaggtgaaagcccaggcatgcttcccagtgcatccttgagatgttaggtctttctgagctaaaagaacaaaaggatgacattgctggactgaaaatggcccttcaggctgtagtcattttgcagctgcagctgacctggaggtttagttcctgtcttccttggctaccataacactggcaggggaggatgaggcagttgaggccagcagtcgtttttggtgtagctcttcccacttacttctgtttgtagctactgaatctagcatcggcttcagtttcacgttgaccttcaccagtgcctgatacaaaggcatgcagatgctatcaatccactccagttgcaaccgaggcagttcatccttccggttccgatcaaaaattgctgaaggagtgagtttgagctctaatctctcccgatctccttgttcgaagaactcactggttacaagttctgccacctgtctggagatctcccacggtttggtcacggctccaaggtcacaggctgtcattaacattgatcgaaatatatcacgatggtttttgatgttccaatcgtattctcctttactgacaagttcaaagaattcagttctcctctcaaagtacagcgtgaggtctgttgccaatattgactgcttcaaaagctgcataaggtcactatattccttggaggacaggttagcaaagatattgtgaccctcactttgaaggatcatcacggcgtggttgaaatggtgatgctccaaggtagcagaggttccatagagttgggccagggcagagccactcttagcttggaaggcattgttggttcccctgtggtcgaggtcatgacacaggcatcccacaatcaccgctaaaatttccacctcggtcagaatgtcttgaaacccagcagtggttaacatcgcgaacatcagctgacacacgttgaaggcatgtctccagttgtggtatagaaccatccgatagtttttcctcactgtcaaaagccacctacacagtgtctcatagtcaattttaaatttctgtaccatccccagctccatgaacatccggagagcagctgtgatcatggcatcaacgtcgagagaaaagtcatcaaaatgaatgtcatcgatggcaagttctgacaccagagggatgttggctgccttaaacttgtcaacttcagcttttgaacatgttgcatggtatgatagcacatcaagagccacagactgcttggcccaggacttcttcacttgatcatacataattgtgttgttgatgccaagtccacaaaagatgacaaaagcctcaaaaagtcgttgatctgcatcatcaaaaggtttcccatcaagtctgtttaacacttgagccactccaattatttggtggttgctattccaaatagggacacaaagaacagatcttatgtgaaaaccagatatctggtctgcctctgcatcaaagcgcggatcctggtaggcatcactgatgttcactggaaggcctgttgaagcaaccagctcagcaatgctgttatttattagccagtcggagtatgatgatttctccatgctttctttgaaactgttctcagcatcagcactgcactttggggacatcaattcaaaggatttggtaaatttcaccactggtgattcgatgtcctctaggagtaaaacagaacagcgttcacatttcagcagagtttgggcccgatgcattattttcttgacaattttctccaggtcagtctgttcttcaaagaggtcattaaccacctctagcaaagctctgcttctttcatattctttccttgaggcagcaaagagctgagcgttagatatggcgattccacaaaatggaagatacatctgcataacctttctggctgttccatggcttcctattgcttacagggcctacactcaaagcccttcataatctattcccaacacacagtggacttttcttgactcatcttccagcactcttctccctctacatttcttg

SEQ ID NO: 18121 - RNA, 5093 nt, Homo sapiens
  source 1..5093: mol_type = other RNA
tgaaggtctactgtgtgccaggaaaacaatgtcgcatgtagaacatggcccctatttctttaatatctgtaaagttaatgattgataatgattaataacaataacaagggccgggtacggtggctcacgcctgtaatcccagcactttcggaggcagaggtgggtggctcacctgaggtcaggagtttgagatcagcctggcaaacatggtgaaaccctgtgtctactaaaagtacaaaaattagccaggcgtggtggcaggcacctgtaatcccagcttctcaggaggttgaggctggagaattgcttgaacccaggaagcagaggttgcagtaagccgagatcacgccattgcactccagcctgggcaacaagagtgaaaactcagtctcaaaaaacaaacaaacaaagaaacaaaaacaataacaagaaaaatggtttgtaaatttcagatttttttaagagctagaatggctctcaggtttaatctaggccagggattttcaaactcttcagagtccctgtggacccccatgtacgtaatcaaagagatgaaggtttgtaggtgctctggatgtccaaaccctgcttataattcacataggaattcagctttttgacgttttatatgttggggattcattgaaagatttatttgaacaaagagttgtaaggttaaaacatgttcgagaatcgtttcctagtgtaatctaatttgacaaataaggaaacaagcttgtagaagttaagtgacttgttcaagtcaatccagtcaataatgccaaagctaaggatagaaatctatcttctagcccaatgttctttggataacacataccatgtccacaatttctcaatatagggagcaaagcagctttctagtcattacatctacttaatacagtttattcttacctattgtaaacctggcttcctatagaatatgcgttctttgcccagactgttatttcttaacatttgaagcattgtttcttacacttaaggaaaaatccaaaattagggacccctatagtttgctttaagttggttactggtagtaatcttaaattttataccagaactcctcactaggagaactcaaggtagtcaatgcttagtctccatggctctgctctgtcctgtgaactatagtttctagatgtcacttgtggtaaatccagctacagatttccttccacccttactttaatcaaaatctatcaatccattccttctgggagaaaactttgtctgtaatgaaggttgaattttaaaactctggaaaagggtaccatagtcccagtctagaattacccatcaaacacatttgctatagtcctactatgtattcatttttagggggagaactgggattgatcagtatttataaggatagtatagtttaccttttaggtaggcaattctaaaggatccatcaataagaagctctaggattaaaaataaaatacctctatggaatacaaattaggattcttgggacagtctggcacaaaaaggcattcagggacaggaagcaaagacaggcagtgtttggcttgtaacaaacagaaaagccctatacaaaacgaagcagcgctaatgacgcttttactgttcagtgttccctcagctcagagtaagtaggccgactgtccacaggtccttggatccaaaacagtcccctacccagagccttcatttcagcccatgcgtgttcattagggaaaagtgagggtcctggggtgtgctccctgccccacctctttctttgtccttcccgttgctctctctgctgctgaccatgcttcaaggtgaaagcccaggcatgcttcccagtgcatccttgagatgttaggtctttctgagctaaaagaacaaaaggatgacattgctggactgaaaatggcccttcaggctgtagtcattttgcagctgcagctgacctggaggtttagttcctgtcttccttggctaccataacactggcaggggaggatgaggcagttgaggccagcagtcgtttttggtgtagctcttcccacttacttctgtttgtagctactgaatctagcatcggcttcagtttcacgttgaccttcaccagtgcctgatacaaaggcatgcagatgctatcaatccactccagttgcaaccgaggcagttcatccttccggttccgatcaaaaattgctgaaggagtgagtttgagctctaatctctcccgatctccttgttcgaagaactcactggttacaagttctgccacctgtctggagatctcccacggtttggtcacggctccaaggtcacaggctgtcattaacattgatcgaaatatatcacgatggtttttgatgttccaatcgtattctcctttactgacaagttcaaagaattcagttctcctctcaaagtacagcgtgaggtctgttgccaatattgactgcttcaaaagctgcataaggtcactatattccttggaggacaggttagcaaagatattgtgaccctcactttgaaggatcatcacggcgtggttgaaatggtgatgctccaaggtagcagaggttccatagagttgggccagggcagagccactcttagcttggaaggcattgttggttcccctgtggtcgaggtcatgacacaggcatcccacaatcaccgctaaaatttccacctcggtcagaatgtcttgaaacccagcagtggttaacatcgcgaacatcagctgacacacgttgaaggcatgtctccagttgtggtatagaaccatccgatagtttttcctcactgtcaaaagccacctacacagtgtctcatagtcaattttaaatttctgtaccatccccagctccatgaacatccggagagcagctgtgatcatggcatcaacgtcgagagaaaagtcatcaaaatgaatgtcatcgatggcaagttctgacaccagagggatgttggctgccttaaacttgtcaacttcagcttttgaacatgttgcatggtatgatagcacatcaagagccacagactgcttggcccaggacttcttcacttgatcatacataattgtgttgttgatgccaagtccacaaaagatgacaaaagcctcaaaaagtcgttgatctgcatcatcaaaaggtttcccatcaagtctgtttaacacttgagccactccaattatttggtggttgctattccaaatagggacacaaagaacagatcttatgtgaaaaccagatatctggtctgcctctgcatcaaagcgcggatcctggtaggcatcactgatgttcactggaaggcctgttgaagcaaccagctcagcaatgctgttatttattagccagtcggagtatgatgatttctccatgctttctttgaaactgttctcagcatcagcactgcactttggggacatcaattcaaaggatttggtaaatttcaccactggtgattcgatgtcctctaggagtaaaacagaacagcgttcacatttcagcagagtttgggcccgatgcattattttcttgacaattttctccaggtcagtctgttcttcaaagaggtcattaaccacctctagcaaagctctgcttctttcatattctttccttgaggcagcaaagagctgagcgttagatatggcgattccacaaaatggaagatacatctgcataactttttcatcatcttcagtaaatggagctccttcaggaatcttatttatcgcttgggccacaccaataatctcaccatcactgcttcggataggcatgcacaataatgattttgtcttgtatccagttagcttgtcgatttcatcattgaatcgtcgatcctggtaggcatcaggaatgttgaccgtttctccatgctccccgacatagccaatgatacctttgccccaggggacctgcacctcatttgagttctctgtgctgctgcaaggcagcagaggtgttcctgcatgcacatcaaagaatttggagaccaaggtcttcttgccagcagctgccccttccaccaggaaaagagagcagcggtcagcatccaccataaggcagacaaagatgagaatcttgtagctcaggctggtgaggtcaaggtcattggagatatctttgaccaattccagaaagaactgacgctcattatgctttttcagatggcacttgtagtcgatggctgtagggggataccgaggcagattcactctcgattccagcagcgcactgagaatatgggctgtggtggggggcagggagcttgccttccggagaagtgccctccgtcgtacactactcaggggttcctgagcccgggaggtcacctgttcatcgtaggtcctgttcacgtggatggccttggagcgggcaaaactcttccttagctctttctgagaagctctccgctgcaggttcccatcgcccctgctgccaccggcccagctgggactcaagggaaccccaccacagtccccgccaccgggaaggggctggctgtgggcagagccatttggtccagtgccaccaccaacgctgctgccacctctgcaggtgctgtgagccaagctgctggtaccagccaaagagggccttggacctaaagccccctgaccctgactgtgcctctgcagccacttttcaaccatctcctgcttccccttccgcatcaagtaatcttcaaacaactctgggtgcctgtccaggaaagtttccacctccccaaagtccaggcgggaggctgccatggtcccagacagctttccttgcctgtttacacgtgaaccaaatgttttcctgccccgaggcctctagctgttcctgcacatgttcacccccaccagtattcccagttcagcgccacctcccctggagattattcccagcagtggaatctgggagatgccccttccttctctggctcagagtggctggcgccgaccccaccccgtggtcctgctactcctgctccgcacaggtgcccagcactgagctgccgccgctgccccggctcctgttccggaaacccgagctatcgctgctcctgttctggctgccgccgctgctgctggaactgctgctgtaacc

SEQ ID NO: 18122 - RNA, 4102 nt, Homo sapiens
  source 1..4102: mol_type = other RNA
tgaaggtctactgtgtgccaggaaaacaatgtcgcatgtagaacatggcccctatttctttaatatctgtaaagttaatgattgataatgattaataacaataacaagggccgggtacggtggctcacgcctgtaatcccagcactttcggaggcagaggtgggtggctcacctgaggtcaggagtttgagatcagcctggcaaacatggtgaaaccctgtgtctactaaaagtacaaaaattagccaggcgtggtggcaggcacctgtaatcccagcttctcaggaggttgaggctggagaattgcttgaacccaggaagcagaggttgcagtaagccgagatcacgccattgcactccagcctgggcaacaagagtgaaaactcagtctcaaaaaacaaacaaacaaagaaacaaaaacaataacaagaaaaatggtttgtaaatttcagatttttttaagagctagaatggctctcaggtttaatctaggccagggattttcaaactcttcagagtccctgtggacccccatgtacgtaatcaaagagatgaaggtttgtaggtgctctggatgtccaaaccctgcttataattcacataggaattcagctttttgacgttttatatgttggggattcattgaaagatttatttgaacaaagagttgtaaggttaaaacatgttcgagaatcgtttcctagtgtaatctaatttgacaaataaggaaacaagcttgtagaagttaagtgacttgttcaagtcaatccagtcaataatgccaaagctaaggatagaaatctatcttctagcccaatgttctttggataacacataccatgtccacaatttctcaatatagggagcaaagcagctttctagtcattacatctacttaatacagtttattcttacctattgtaaacctggcttcctatagaatatgcgttctttgcccagactgttatttcttaacatttgaagcattgtttcttacacttaaggaaaaatccaaaattagggacccctatagtttgctttaagttggttactggtagtaatcttaaattttataccagaactcctcactaggagaactcaaggtagtcaatgcttagtctccatggctctgctctgtcctgtgaactatagtttctagatgtcacttgtggtaaatccagctacagatttccttccacccttactttaatcaaaatctatcaatccattccttctgggagaaaactttgtctgtaatgaaggttgaattttaaaactctggaaaagggtaccatagtcccagtctagaattacccatcaaacacatttgctatagtcctactatgtattcatttttagggggagaactgggattgatcagtatttataaggatagtatagtttaccttttaggtaggcaattctaaaggatccatcaataagaagctctaggattaaaaataaaatacctctatggaatacaaattaggattcttgggacagtctggcacaaaaaggcattcagggacaggaagcaaagacaggcagtgtttggcttgtaacaaacagaaaagccctatacaaaacgaagcagcgctaatgacgcttttactgttcagtgttccctcagctcagagtaagtaggccgactgtccacaggtccttggatccaaaacagtcccctacccagagccttcatttcagcccatgcgtgttcattagggaaaagtgagggtcctggggtgtgctccctgccccacctctttctttgtccttcccgttgctctctctgctgctgaccatgcttcaaggtgaaagcccaggcatgcttcccagtgcatccttgagatgttaggtctttctgagctaaaagaacaaaaggatgacattgctggactgaaaatggcccttcaggctgtagtcattttgcagctgcagctgacctggaggtttagttcctgtcttccttggctaccataacactggcaggggaggatgaggcagttgaggccagcagtcgtttttggtgtagctcttcccacttacttctgtttgtagctactgaatctagcatcggcttcagtttcacgttgaccttcaccagtgcctgatacaaaggcatgcagatgctatcaatccactccagttgcaaccgaggcagttcatccttccggttccgatcaaaaattgctgaaggagtgagtttgagctctaatctctcccgatctccttgttcgaagaactcactggttacaagttctgccacctgtctggagatctcccacggtttggtcacggctccaaggtcacaggctgtcattaacattgatcgaaatatatcacgatggtttttgatgttccaatcgtattctcctttactgacaagttcaaagaattcagttctcctctcaaagtacagcgtgaggtctgttgccaatattgactgcttcaaaagctgcataaggtcactatattccttggaggacaggttagcaaagatattgtgaccctcactttgaaggatcatcacggcgtggttgaaatggtgatgctccaaggtagcagaggttccatagagttgggccagggcagagccactcttagcttggaaggcattgttggttcccctgtggtcgaggtcatgacacaggcatcccacaatcaccgctaaaatttccacctcggtcagaatgtcttgaaacccagcagtggttaacatcgcgaacatcagctgacacacgttgaaggcatgtctccagttgtggtatagaaccatccgatagtttttcctcactgtcaaaagccacctacacagtgtctcatagtcaattttaaatttctgtaccatccccagctccatgaacatccggagagcagctgtgatcatggcatcaacgtcgagagaaaagtcatcaaaatgaatgtcatcgatggcaagttctgacaccagagggatgttggctgccttaaacttgtcaacttcagcttttgaacatgttgcatggtatgatagcacatcaagagccacagactgcttggcccaggacttcttcacttgatcatacataattgtgttgttgatgccaagtccacaaaagatgacaaaagcctcaaaaagtcgttgatctgcatcatcaaaaggtttcccatcaagtctgtttaacacttgagccactccaattatttggtggttgctattccaaatagggacacaaagaacagatcttatgtgaaaaccagatatctggtctgcctctgcatcaaagcgcggatcctggtaggcatcactgatgttcactggaaggcctgttgaagcaaccagctcagcaatgctgttatttattagccagtcggagtatgatgatttctccatgctttctttgaaactgttctcagcatcagcactgcactttggggacatcaattcaaaggatttggtaaatttcaccactggtgattcgatgtcctctaggagtaaaacagaacagcgttcacatttcagcagagtttgggcccgatgcattattttcttgacaattttctccaggtcagtctgttcttcaaagaggtcattaaccacctctagcaaagctctgcttctttcatattctttccttgaggcagcaaagagctgagcgttagatatggcgattccacaaaatggaagatacatctgcataactttttcatcatcttcagtaaatggagctccttcaggaatcttatttatcgcttgggccacaccaataatctcaccatcactgcttcggataggcatgcacaataatgattttgtcttgtatccagttagcttgtcgatttcatcattgaatcgtcgatcctttgtttttgtttgcctctgtataagaaaatcctggtgcttttcctgtttttcagccaaagaggccccagagatttggaccagtcttgtgattttcacctttttccactgtgtggcactgagcacatttctgaataaaggtcttcttgcctgcttcagcatctcccatgttgctctggaacagccacctggccagagtccacgcctcaacttcgaggctggcgatccagaaagagcacctcacgccctgggctgcaagcg

SEQ ID NO: 18123 - RNA, 1204 nt, Homo sapiens
  source 1..1204: mol_type = other RNA
tgaaggtctactgtgtgccaggaacagagccagcacttggaaatgccaagacaatctaagtctcttccatttcatttttcccccacagtgctgcatctctttcctccgagggttttcaaagaaagacaagccttaaatacatgccttaaaaggaagaagtgatctgttaattgctctgggtcgttgctttgggtgggtgacacatttactcaattcagcggagctgtaccttcttagtcccaggtcctgaggggcagagagtgaggcaattccaggacccattaccctgggcagagtgcacagatgttgcaagggaggtcaagagcatggggaggcccggaggaggaggaggggggagggggagaagggagcgagcttcctcctggggtccatcagtctcagcttggggttggggggcacttaagtgaggctctgcgaagaagagatgggggagtgggggtggatgggctccaggtggctgggaagggcattcttccaacagctggagcagaggtgaaaggaggcagcacatgacactgtgtcatgaggaccctgtaaggagcctgtggatgtgggagcagagggaggaaaaggaggtcagacggggctggagaagtttctggggcagattttgagggtctgagctccagccaagtgggtgcttacctgatgaggagcctcttcagagctggtcacattcatcccagtgtccccagcacctggctggtgcccagtgggtgtttgtggactggctggactcttcctctgtaggcctcgggttcctcacatttgtggtcaggcgaggtcacctggcacctcccttcctactctgaagagctctcaggagttctggatgcttgtgcaggggaaggcctcaccactctccctgtctcctgcctcagggttctctgggttgccccagcagggctggggccatggtgccctgagtgggggacagccctcccgctgccagggaactttgcccctcgtgctttctcccttcagcagttggccccctgagcccagaaggacattccttggtgtcccgtgactgggagtggcagtggcattgagcgcatgctgcagcttagcacggggagggagctctgcttccatctatgtgaaaatgggcagccaggtgtggtagctcatgcctataatcccaacactttgggaggccgaggcgggcagatcacttgaggtc

SEQ ID NO: 18124 - RNA, 784 nt, Homo sapiens
  source 1..784: mol_type = other RNA
tgaaggtctactgtgtgccaggaacagagccagcacttggaaatgccaagacaatctaagtctcttccatttcatttttcccccacagtgctgcatctctttcctccgagggttttcaaagaaagacaagccttaaatacatgccttaaaaggaagaagtgatctgttaattgctctgggtcgttgctttgggtgggtgacacatttactcaattcagcggagctgtaccttcttagtcccaggtcctgatgaggagcctcttcagagctggtcacattcatcccagtgtccccagcacctggctggtgcccagtgggtgtttgtggactggctggactcttcctctgtaggcctcgggttcctcacatttgtggtcaggcgaggtcacctggcacctcccttcctactctgaagagctctcaggagttctggatgcttgtgcaggggaaggcctcaccactctccctgtctcctgcctcagggttctctgggttgccccagcagggctggggccatggtgccctgagtgggggacagccctcccgctgccagggaactttgcccctcgtgctttctcccttcagcagttggccccctgagcccagaaggacattccttggtgtcccgtgactgggagtggcagtggcattgagcgcatgctgcagcttagcacggggagggagctctgcttccatctatgtgaaaatgggcagccaggtgtggtagctcatgcctataatcccaacactttgggaggccgaggcgggcagatcacttgaggtc

SEQ ID NO: 18125 - RNA, 710 nt, Homo sapiens
  source 1..710: mol_type = other RNA
tgaaggtctactgtgtgccaggagatgtgctaagtattttacacgtattcatttatctcaggctcacaattgcactcaaagggagacaccatcaccctcagtttacagatggtggaactgaagcacagagataaatgaacttaagtaatagtgtcaggaaatgatggtacccagattataatcaagataacctgtctcttccaatgttcctgcttgtaaccactctgctgtattgggagcaaacttgtccctctgggtgaggtgagctatgaagggtgcaagacatgctcctgtggtgctgagattccacccgaggaggtcatctgtgcctttcttggctcccaaagcacagggttctatgtaggccactgagcatatggctctttgaggcaggtcacatttgcagctgaggaagattgcctgatgccgcgtggaactcttgctaggggaacatgccctcatttgtagaaagagcacatttccaaagtgttccatgcagtgatactccccgaagcttgtcttgggtctccaaatggacttttagtttttgttttgttttgttttatttttatttttattttttttgcttaaatacatatttatatatgtatttaaaatatgcatgagctacaatgcaaactcattctaatggggaggtggcattctctgccagctctgaaatctcagtcacactcaccttctgtgtttgt

SEQ ID NO: 18126 - RNA, 4085 nt, Homo sapiens
  source 1..4085: mol_type = other RNA
tgaaggtctactgtgtgccaggcactattctgggaactgaggattcaacaatgaataaataaagcttcgtaagacattgtcctcactgctatatctccaccccctagaagaatgcccagcacatactgggtgctcaattatatgtgtgaaatcaatttgagttggaaatgggcaatctgctggttctcaccatggggcatgcataccctgaatgtctggctgggaggtgttaaagcactagtagtagggattttggccaggattttattctggtttcattctcttaaaggattgacttatgcaaaaaactcccacaggtgggacagaaccagaaataacccagatcctcatgggcctttagatttgtgacttgcattaggggaggcagctaaccaatctcacactttttttcctttccagtctccacagaatcaaagcggtcagggttggacaggaatgacagagctgtctccgtattacttgatcaaggaaaccagtatcggggaagtcaaaagatttacacaagtcacatgatgtgttggtgacagagctgtgactaaaactaaaacctagacctaagacctgtgatttctttattcatctgggagccttcaggcccctaaaaaaatatgttgacattttcagaggaaagagcttacttacgtgcctgtggaaccatcaggggctctacaaggtagtagcttagttttgtacacctcctagtttttctcttatgaaagaagatgaaagaagtatctctgaggtgtagcagcaaaggagaaagtatatggaaacccgagcaattggattttactcttctggatattagcttgtgtgcttcacttttatactccattgcagtttccttcagtgccagctttccccctacagactaaaacaaaggtcttccccaaattccctgcctaaaggaaaggcaatctgtaatactcttaatactttattaacttaaaacatcactctaataaatatgtattaacaaacataatgcttaccagaagatctaaaaacatttaccaacctcatcaaagtgaaaataccacctttcccccctctatggtacacatggagggtcaaagagttgaagacagagccttccttcccacatgcctgctagctcagaaatctttaaaatatcagcttaacaataaaaaactgaatatacacacatatctttgaagtaactgttcagctttttgtttacacctgataaaatccaaaagggtcaaaagggaaggtttacaattctgtgctgtcttctcagaattccctccaagagtaagaacagacccagccacttggaggtgcaaccgttagcttttgaggagcagtcaggggttgtgacttcagtctctcttccccaatacctagcatggtgcctggtaccttggtagccggtgatccatgaacatttgctgagtgaatgaatgacatcttgtccacaggcattgcttgtgcttttacctccagtgatgaggttttcacagccctactgaagggaggacctctaatcccctctcattaccaacttctcttctgcttcttcttgggggtagcctcgatggtgcatctcatgacttcaaagtattaaattccttccccaagtcagtttctgaatcagtttttgaggaggagaaatgattcctccaagatttataggcagcacccaaaagaaaggagtcaacagaccccccagaaggaaaaaaataaaagttaacactcactcttctttctagataaaaatattagcatttgtccaccttgtaaatggtgattcctcctcttccacacaaatatctggggtaggtcaagaggggggagggaagaaacctgaagggcattcctgtctgtagattagggctggaaatgggaaggactgtggggtctaagatttattctggtccccatttgactttgcctttgtcttcaggtgtagaggagcctatttgtgtccgaagcctagagagtcacttggttctcactctcggctgcactttgaaaaggtacctcatttcttctggcagctccaggaggtaaggcgaaggaggagcaacctggtaggatctgcagactggacctggggtctggaaagtcagaagggagtggaggcaagcagggagcagagtggtggcaagcagggaggctgccctctgtagtgttgtgtagctgctgcttgcagccagccagggtgctcatttgagcccatgctgcgtctcccggtgccttcggaggtccaccttcctctggaaacccttcccacagaggtcgcagccgaagggcttgaagcctgtgtgtttgcggctgtgggtgatgaggttggagctctggctgaatgccttgccgcacacctggcacttgtgaggcttctcaccagtgtggatgaaagtgtgtttcttcatgtctgacttctggtggaacctcttgccacagtactgacaggggtagggccgagtgtctgagtggataagcaggtgtgtggacagtgtggatgacctcttgaagctcttcccacagatcttacagtcaaagctccgttcctgcgagtgcacggctttgtgctgctccaggctcaccgcgtgcccgaaggtcttgccgcacatctcgcaggcaaagggtctggtaccgctgtgggacctgcgcacgtgcacctcgagcccgtgcggcgtggagaacaccttgctgcacttgatgcacttgtaggagccgccgcccagcagcaggcgggtgcacagcagctccgactccaccttgacgccagcgcccttgtctgcgtgcagcccgtggccacgctcggggtacagcaagcccgccgctgccgtgggcctctcatacagcccggctgccgcagacccgaagtcgccgtagagccctaggccagggccagcggtggcaccggcccctgcgctgcagctccctggcgccccggcccccgcgccgccggcagcccgcttcgggccgtacagcgcggccgggtggccaggctccggggcgggttcgcagaagaggcccaggccagcgccacgctccagggccccacacggtcggtagctctgcaccaggtgccgcaggtcagaacccgccaggccgctccatgagtacggtttgaaaggcagggggaagggctgggcttcgtccagcgatgggcacattgacttctccgaggctggagacgcggagggtgacgggggcctccagaagtcctcaaactccgagctccgttcgcagacgctgccttcgcagctgtctggggatgcggaggctctgtctggggcttcggtcagctgcgattcgggggacaaacggtcccggggctccgccttcgccccgcctgcatttgaagtgctgtctgctcggctaggcgccggtacattctctaaacggagggaatagtctggtcctggggagcgcggctggtggtagctgtgagccttcttgcttttgacgagaaatgagcgcggcatggtggtccggcactttccccactgcgccccaagagtccctggagccgctgtcacccacggtcactccgagggcttgctcagccccagcccggaggagaccaaaaaatcttgtcctagggaggtggagcccgatccacgaacgttgactgggaaatgctaggtgtcccgagtcggtagtgcaccgacaatttagcagacaaaaaagacaggacgccagagcgcgcaggctgcattagcagagagcgggggtcgggcccgggcccgggagggaactagctgcccggggcgtcgctctcattaacccccaatcagttcacctaataccaggtcgaaatctgagcgcagcgggagggcgtggctgcgcctgccgctaggctccagccggctccgggggcggtaccccacagtcgaggtggtctggagtaaacgaatctgccttcctcccggggtgaaggcgatggtgaccgggttcacacgtgagctgcagtacagcagttctccgtggcctcggctggttcagaaacgagggtgctgggaactctgggccggggcaggacctgcagtcctccggcttcgcgctgtttccactgccggactaggagcccc

SEQ ID NO: 18127 - RNA, 3658 nt, Homo sapiens
  source 1..3658: mol_type = other RNA
tgaaggtctactgtgtgccaggcactattctgggaactgaggattcaacaatgaataaataaagcttcgtaagacattgtcctcactgctatatctccaccccctagaagaatgcccagcacatactgggtgctcaattatatgtgtgaaatcaatttgagttggaaatgggcaatctgctggttctcaccatggggcatgcataccctgaatgtctggctgggaggtgttaaagcactagtagtagggattttggccaggattttattctggtttcattctcttaaaggattgacttatgcaaaaaactcccacaggtgggacagaaccagaaataacccagatcctcatgggcctttagatttgtgacttgcattaggggaggcagctaaccaatctcacactttttttcctttccagtctccacagaatcaaagcggtcagggttggacaggaatgacagagctgtctccgtattacttgatcaaggaaaccagtatcggggaagtcaaaagatttacacaagtcacatgatgtgttggtgacagagctgtgactaaaactaaaacctagacctaagacctgtgatttctttattcatctgggagccttcaggcccctaaaaaaatatgttgacattttcagaggaaagagcttacttacgtgcctgtggaaccatcaggggctctacaaggtagtagcttagttttgtacacctcctagtttttctcttatgaaagaagatgaaagaagtatctctgaggtgtagcagcaaaggagaaagtatatggaaacccgagcaattggattttactcttctggatattagcttgtgtgcttcacttttatactccattgcagtttccttcagtgccagctttccccctacagactaaaacaaaggtcttccccaaattccctgcctaaaggaaaggcaatctgtaatactcttaatactttattaacttaaaacatcactctaataaatatgtattaacaaacataatgcttaccagaagatctaaaaacatttaccaacctcatcaaagtgaaaataccacctttcccccctctatggtacacatggagggtcaaagagttgaagacagagccttccttcccacatgcctgctagctcagaaatctttaaaatatcagcttaacaataaaaaactgaatatacacacatatctttgaagtaactgttcagctttttgtttacacctgataaaatccaaaagggtcaaaagggaaggtttacaattctgtgctgtcttctcagaattccctccaagagtaagaacagacccagccacttggaggtgcaaccgttagcttttgaggagcagtcaggggttgtgacttcagtctctcttccccaatacctagcatggtgcctggtaccttggtagccggtgatccatgaacatttgctgagtgaatgaatgacatcttgtccacaggcattgcttgtgcttttacctccagtgatgaggttttcacagccctactgaagggaggacctctaatcccctctcattaccaacttctcttctgcttcttcttgggggtagcctcgatggtgcatctcatgacttcaaagtattaaattccttccccaagtcagtttctgaatcagtttttgaggaggagaaatgattcctccaagatttataggcagcacccaaaagaaaggagtcaacagaccccccagaaggaaaaaaataaaagttaacactcactcttctttctagataaaaatattagcatttgtccaccttgtaaatggtgattcctcctcttccacacaaatatctggggtaggtcaagaggggggagggaagaaacctgaagggcattcctgtctgtagattagggctggaaatgggaaggactgtggggtctaagatttattctggtccccatttgactttgcctttgtcttcaggtgtagaggagcctatttgtgtccgaagcctagagagtcacttggttctcactctcggctgcactttgaaaaggtacctcatttcttctggcagctccaggaggtaaggcgaaggaggagcaacctggtaggatctgcagactggacctggggtctggaaagtcagaagggagtggaggcaagcagggagcagagtggtggcaagcagggaggctgccctctgtagtgttgtgtagctgctgcttgcagccagccagggtgctcatttgagcccatgctgcgtctcccggtgccttcggaggtccaccttcctctggaaacccttcccacagaggtcgcagccgaagggcttgaagcctgtgtgtttgcggctgtgggtgatgaggttggagctctggctgaatgccttgccgcacacctggcacttgtgaggcttctcaccagtgtggatgaaagtgtgtttcttcatgtctgacttctggtggaacctcttgccacagtactgacaggggtagggccgagtgtctgagtggataagcaggtgtgtggacagtgtggatgacctcttgaagctcttcccacagatcttacagtcaaagctccgttcctgcgagtgcacggctttgtgctgctccaggctcaccgcgtgcccgaaggtcttgccgcacatctcgcaggcaaagggtctggtaccgctgtgggacctgcgcacgtgcacctcgagcccgtgcggcgtggagaacaccttgctgcacttgatgcacttgtaggagccgccgcccagcagcaggcgggtgcacagcagctccgactccaccttgacgccagcgcccttgtctgcgtgcagcccgtggccacgctcggggtacagcaagcccgccgctgccgtgggcctctcatacagcccggctgccgcagacccgaagtcgccgtagagccctaggccagggccagcggtggcaccggcccctgcgctgcagctccctggcgccccggcccccgcgccgccggcagcccgcttcgggccgtacagcgcggccgggtggccaggctccggggcgggttcgcagaagaggcccaggccagcgccacgctccagggccccacacggtcggtagctctgcaccaggtgccgcaggtcagaacccgccaggccgctccatgagtacggtttgaaaggcagggggaagggctgggcttcgtccagcgatgggcacattgacttctccgaggctggagacgcggagggtgacgggggcctccagaagtcctcaaactccgagctccgttcgcagacgctgccttcgcagctgtctggggatgcggaggctctgtctggggcttcggtcagctgcgattcgggggacaaacggtcccggggctccgccttcgccccgcctgcatttgaagtgctgtctgctcggctaggcgccggtacattctctaaacggagggaatagtctggtcctggggagcgcggctggtggtagctgtgagccttcttgcttttgacgagaaatgagcgcggcatggtggtccggcactttccccactgcgccccaagagtccctggagccgctgtcacccacggtcactccgagggcttgctcagccccagcccggaggagaccaggtggcacttggacaggtggcgcgaacccgccgtcgttgccgccgccgccactgacacagctcagcggtaaaacctgt

SEQ ID NO: 18128 - RNA, 3847 nt, Homo sapiens
  source 1..3847: mol_type = other RNA
tgaaggtctactgtgtgccaggcactattctgggaactgaggattcaacaatgaataaataaagcttcgtaagacattgtcctcactgctatatctccaccccctagaagaatgcccagcacatactgggtgctcaattatatgtgtgaaatcaatttgagttggaaatgggcaatctgctggttctcaccatggggcatgcataccctgaatgtctggctgggaggtgttaaagcactagtagtagggattttggccaggattttattctggtttcattctcttaaaggattgacttatgcaaaaaactcccacaggtgggacagaaccagaaataacccagatcctcatgggcctttagatttgtgacttgcattaggggaggcagctaaccaatctcacactttttttcctttccagtctccacagaatcaaagcggtcagggttggacaggaatgacagagctgtctccgtattacttgatcaaggaaaccagtatcggggaagtcaaaagatttacacaagtcacatgatgtgttggtgacagagctgtgactaaaactaaaacctagacctaagacctgtgatttctttattcatctgggagccttcaggcccctaaaaaaatatgttgacattttcagaggaaagagcttacttacgtgcctgtggaaccatcaggggctctacaaggtagtagcttagttttgtacacctcctagtttttctcttatgaaagaagatgaaagaagtatctctgaggtgtagcagcaaaggagaaagtatatggaaacccgagcaattggattttactcttctggatattagcttgtgtgcttcacttttatactccattgcagtttccttcagtgccagctttccccctacagactaaaacaaaggtcttccccaaattccctgcctaaaggaaaggcaatctgtaatactcttaatactttattaacttaaaacatcactctaataaatatgtattaacaaacataatgcttaccagaagatctaaaaacatttaccaacctcatcaaagtgaaaataccacctttcccccctctatggtacacatggagggtcaaagagttgaagacagagccttccttcccacatgcctgctagctcagaaatctttaaaatatcagcttaacaataaaaaactgaatatacacacatatctttgaagtaactgttcagctttttgtttacacctgataaaatccaaaagggtcaaaagggaaggtttacaattctgtgctgtcttctcagaattccctccaagagtaagaacagacccagccacttggaggtgcaaccgttagcttttgaggagcagtcaggggttgtgacttcagtctctcttccccaatacctagcatggtgcctggtaccttggtagccggtgatccatgaacatttgctgagtgaatgaatgacatcttgtccacaggcattgcttgtgcttttacctccagtgatgaggttttcacagccctactgaagggaggacctctaatcccctctcattaccaacttctcttctgcttcttcttgggggtagcctcgatggtgcatctcatgacttcaaagtattaaattccttccccaagtcagtttctgaatcagtttttgaggaggagaaatgattcctccaagatttataggcagcacccaaaagaaaggagtcaacagaccccccagaaggaaaaaaataaaagttaacactcactcttctttctagataaaaatattagcatttgtccaccttgtaaatggtgattcctcctcttccacacaaatatctggggtaggtcaagaggggggagggaagaaacctgaagggcattcctgtctgtagattagggctggaaatgggaaggactgtggggtctaagatttattctggtccccatttgactttgcctttgtcttcaggtgtagaggagcctatttgtgtccgaagcctagagagtcacttggttctcactctcggctgcactttgaaaaggtacctcatttcttctggcagctccaggaggtaaggcgaaggaggagcaacctggtaggatctgcagactggacctggggtctggaaagtcagaagggagtggaggcaagcagggagcagagtggtggcaagcagggaggctgccctctgtagtgttgtgtagctgctgcttgcagccagccagggtgctcatttgagcccatgctgcgtctcccggtgccttcggaggtccaccttcctctggaaacccttcccacagaggtcgcagccgaagggcttgaagcctgtgtgtttgcggctgtgggtgatgaggttggagctctggctgaatgccttgccgcacacctggcacttgtgaggcttctcaccagtgtggatgaaagtgtgtttcttcatgtctgacttctggtggaacctcttgccacagtactgacaggggtagggccgagtgtctgagtggataagcaggtgtgtggacagtgtggatgacctcttgaagctcttcccacagatcttacagtcaaagctccgttcctgcgagtgcacggctttgtgctgctccaggctcaccgcgtgcccgaaggtcttgccgcacatctcgcaggcaaagggtctggtaccgctgtgggacctgcgcacgtgcacctcgagcccgtgcggcgtggagaacaccttgctgcacttgatgcacttgtaggagccgccgcccagcagcaggcgggtgcacagcagctccgactccaccttgacgccagcgcccttgtctgcgtgcagcccgtggccacgctcggggtacagcaagcccgccgctgccgtgggcctctcatacagcccggctgccgcagacccgaagtcgccgtagagccctaggccagggccagcggtggcaccggcccctgcgctgcagctccctggcgccccggcccccgcgccgccggcagcccgcttcgggccgtacagcgcggccgggtggccaggctccggggcgggttcgcagaagaggcccaggccagcgccacgctccagggccccacacggtcggtagctctgcaccaggtgccgcaggtcagaacccgccaggccgctccatgagtacggtttgaaaggcagggggaagggctgggcttcgtccagcgatgggcacattgacttctccgaggctggagacgcggagggtgacgggggcctccagaagtcctcaaactccgagctccgttcgcagacgctgccttcgcagctgtctggggatgcggaggctctgtctggggcttcggtcagctgcgattcgggggacaaacggtcccggggctccgccttcgccccgcctgcatttgaagtgctgtctgctcggctaggcgccggtacattctctaaacggagggaatagtctggtcctggggagcgcggctggtggtagctgtgagccttcttgcttttgacgagaaatgagcgcggcatggtggtccggcactttccccactgcgccccaagagtccctggagccgctgtcacccacggtcactccgagggcttgctcagccccagcccggaggagaccgtccgggcccaggaaggagggagccgagggcgctaagggggcgtcctcccgagcgcagctgccgccgcctccccaccagatgtttccttccctggtggatttggctcccctgccgaaccaccagaccgcctgctgcgcgcccccagctccagatttccagtcacactgcgcgggtcgcgccctaacccagctgccggagctctctgggctcccgcacggcggtccgcagcaggtgggaaaccgcccgcgccctctgatcgcccccgca

SEQ ID NO: 18129 - RNA, 4571 nt, Homo sapiens
  source 1..4571: mol_type = other RNA
tgaaggtctactgtgtgccaggcactattctgggaactgaggattcaacaatgaataaataaagcttcgtaagacattgtcctcactgctatatctccaccccctagaagaatgcccagcacatactgggtgctcaattatatgtgtgaaatcaatttgagttggaaatgggcaatctgctggttctcaccatggggcatgcataccctgaatgtctggctgggaggtgttaaagcactagtagtagggattttggccaggattttattctggtttcattctcttaaaggattgacttatgcaaaaaactcccacaggtgggacagaaccagaaataacccagatcctcatgggcctttagatttgtgacttgcattaggggaggcagctaaccaatctcacactttttttcctttccagtctccacagaatcaaagcggtcagggttggacaggaatgacagagctgtctccgtattacttgatcaaggaaaccagtatcggggaagtcaaaagatttacacaagtcacatgatgtgttggtgacagagctgtgactaaaactaaaacctagacctaagacctgtgatttctttattcatctgggagccttcaggcccctaaaaaaatatgttgacattttcagaggaaagagcttacttacgtgcctgtggaaccatcaggggctctacaaggtagtagcttagttttgtacacctcctagtttttctcttatgaaagaagatgaaagaagtatctctgaggtgtagcagcaaaggagaaagtatatggaaacccgagcaattggattttactcttctggatattagcttgtgtgcttcacttttatactccattgcagtttccttcagtgccagctttccccctacagactaaaacaaaggtcttccccaaattccctgcctaaaggaaaggcaatctgtaatactcttaatactttattaacttaaaacatcactctaataaatatgtattaacaaacataatgcttaccagaagatctaaaaacatttaccaacctcatcaaagtgaaaataccacctttcccccctctatggtacacatggagggtcaaagagttgaagacagagccttccttcccacatgcctgctagctcagaaatctttaaaatatcagcttaacaataaaaaactgaatatacacacatatctttgaagtaactgttcagctttttgtttacacctgataaaatccaaaagggtcaaaagggaaggtttacaattctgtgctgtcttctcagaattccctccaagagtaagaacagacccagccacttggaggtgcaaccgttagcttttgaggagcagtcaggggttgtgacttcagtctctcttccccaatacctagcatggtgcctggtaccttggtagccggtgatccatgaacatttgctgagtgaatgaatgacatcttgtccacaggcattgcttgtgcttttacctccagtgatgaggttttcacagccctactgaagggaggacctctaatcccctctcattaccaacttctcttctgcttcttcttgggggtagcctcgatggtgcatctcatgacttcaaagtattaaattccttccccaagtcagtttctgaatcagtttttgaggaggagaaatgattcctccaagatttataggcagcacccaaaagaaaggagtcaacagaccccccagaaggaaaaaaataaaagttaacactcactcttctttctagataaaaatattagcatttgtccaccttgtaaatggtgattcctcctcttccacacaaatatctggggtaggtcaagaggggggagggaagaaacctgaagggcattcctgtctgtagattagggctggaaatgggaaggactgtggggtctaagatttattctggtccccatttgactttgcctttgtcttcaggtgtagaggagcctatttgtgtccgaagcctagagagtcacttggttctcactctcggctgcactttgaaaaggtacctcatttcttctggcagctccaggaggtaaggcgaaggaggagcaacctggtaggatctgcagactggacctggggtctggaaagtcagaagggagtggaggcaagcagggagcagagtggtggcaagcagggaggctgccctctgtagtgttgtgtagctgctgcttgcagccagccagggtgctcatttgagcccatgctgcgtctcccggtgccttcggaggtccaccttcctctggaaacccttcccacagaggtcgcagccgaagggcttgaagcctgtgtgtttgcggctgtgggtgatgaggttggagctctggctgaatgccttgccgcacacctggcacttgtgaggcttctcaccagtgtggatgaaagtgtgtttcttcatgtctgacttctggtggaacctcttgccacagtactgacaggggtagggccgagtgtctgagtggataagcaggtgtgtggacagtgtggatgacctcttgaagctcttcccacagatcttacagtcaaagctccgttcctgcgagtgcacggctttgtgctgctccaggctcaccgcgtgcccgaaggtcttgccgcacatctcgcaggcaaagggtctggtaccgctgtgggacctgcgcacgtgcacctcgagcccgtgcggcgtggagaacaccttgctgcacttgatgcacttgtaggagccgccgcccagcagcaggcgggtgcacagcagctccgactccaccttgacgccagcgcccttgtctgcgtgcagcccgtggccacgctcggggtacagcaagcccgccgctgccgtgggcctctcatacagcccggctgccgcagacccgaagtcgccgtagagccctaggccagggccagcggtggcaccggcccctgcgctgcagctccctggcgccccggcccccgcgccgccggcagcccgcttcgggccgtacagcgcggccgggtggccaggctccggggcgggttcgcagaagaggcccaggccagcgccacgctccagggccccacacggtcggtagctctgcaccaggtgccgcaggtcagaacccgccaggccgctccatgagtacggtttgaaaggcagggggaagggctgggcttcgtccagcgatgggcacattgacttctccgaggctggagacgcggagggtgacgggggcctccagaagtcctcaaactccgagctccgttcgcagacgctgccttcgcagctgtctggggatgcggaggctctgtctggggcttcggtcagctgcgattcgggggacaaacggtcccggggctccgccttcgccccgcctgcatttgaagtgctgtctgctcggctaggcgccggtacattctctaaacggagggaatagtctggtcctggggagcgcggctggtggtagctgtgagccttcttgcttttgacgagaaatgagcgcggcatggtggtccggcactttccccactgcgccccaagagtccctggagccgctgtcacccacggtcactccgagggcttgctcagccccagcccggaggagacctaataccaggtcgaaatctgagcgcagcgggagggcgtggctgcgcctgccgctaggctccagccggctccgggggcggtaccccacagtcgaggtggtctggagtaaacgaatctgccttcctcccggggtgaaggcgatggtgaccgggttcacacgtgagctgcagtacagcagttctccgtggcctcggctggttcagaaacgagggtgctgggaactctgggccggggcaggacctgcagtcctccggcttcgcgctgtttccactgccggactaggagcccctcggcttcctaggcaagatgcaggccacacagtctacgtctgtccgttggcgctctcagctcaaacgagtcctacaggccttggtccctgtagggtgcaggccccctgctccagatccccagccccattgtgtccccttctccggaggaatgggaatagacctgggagaaaagacgcctgggacgtgtcgcggggctcccgcgaagtttcccgctacccaagcgccagaatgcccctaggggtgagagtgccatccgcctccctccggggtggctcctagggctagagctttgtcgcttcctgcacttctcgtccgtacaattagacgccacaaaccccaaacccaattctttaaacagccacgaaactcggaagaaaagaaaaacggagtggcgttgtcccgagggtcccgctgcagcttggacccacgttggctgggagcgggacagatgggggcggggtaactgtcagcgccggagctgggtctgggctggcgccaccagagaccaggcggacgcggaggccgcctccccacccgggctgtaagcccacgcctctctcgcaccccggcccgctttgctggttcctgtggggagcgacagagtttggaggagataggggccccggggcctgggccgagcgcgtgggaaggcaaccccgcgctgcagctggcgcgggaggtggggcggcccctccgcgcgctc

SEQ ID NO: 18130 - RNA, 3664 nt, Homo sapiens
  source 1..3664: mol_type = other RNA
tgaaggtctactgtgtgccaggcactattctgggaactgaggattcaacaatgaataaataaagcttcgtaagacattgtcctcactgctatatctccaccccctagaagaatgcccagcacatactgggtgctcaattatatgtgtgaaatcaatttgagttggaaatgggcaatctgctggttctcaccatggggcatgcataccctgaatgtctggctgggaggtgttaaagcactagtagtagggattttggccaggattttattctggtttcattctcttaaaggattgacttatgcaaaaaactcccacaggtgggacagaaccagaaataacccagatcctcatgggcctttagatttgtgacttgcattaggggaggcagctaaccaatctcacactttttttcctttccagtctccacagaatcaaagcggtcagggttggacaggaatgacagagctgtctccgtattacttgatcaaggaaaccagtatcggggaagtcaaaagatttacacaagtcacatgatgtgttggtgacagagctgtgactaaaactaaaacctagacctaagacctgtgatttctttattcatctgggagccttcaggcccctaaaaaaatatgttgacattttcagaggaaagagcttacttacgtgcctgtggaaccatcaggggctctacaaggtagtagcttagttttgtacacctcctagtttttctcttatgaaagaagatgaaagaagtatctctgaggtgtagcagcaaaggagaaagtatatggaaacccgagcaattggattttactcttctggatattagcttgtgtgcttcacttttatactccattgcagtttccttcagtgccagctttccccctacagactaaaacaaaggtcttccccaaattccctgcctaaaggaaaggcaatctgtaatactcttaatactttattaacttaaaacatcactctaataaatatgtattaacaaacataatgcttaccagaagatctaaaaacatttaccaacctcatcaaagtgaaaataccacctttcccccctctatggtacacatggagggtcaaagagttgaagacagagccttccttcccacatgcctgctagctcagaaatctttaaaatatcagcttaacaataaaaaactgaatatacacacatatctttgaagtaactgttcagctttttgtttacacctgataaaatccaaaagggtcaaaagggaaggtttacaattctgtgctgtcttctcagaattccctccaagagtaagaacagacccagccacttggaggtgcaaccgttagcttttgaggagcagtcaggggttgtgacttcagtctctcttccccaatacctagcatggtgcctggtaccttggtagccggtgatccatgaacatttgctgagtgaatgaatgacatcttgtccacaggcattgcttgtgcttttacctccagtgatgaggttttcacagccctactgaagggaggacctctaatcccctctcattaccaacttctcttctgcttcttcttgggggtagcctcgatggtgcatctcatgacttcaaagtattaaattccttccccaagtcagtttctgaatcagtttttgaggaggagaaatgattcctccaagatttataggcagcacccaaaagaaaggagtcaacagaccccccagaaggaaaaaaataaaagttaacactcactcttctttctagataaaaatattagcatttgtccaccttgtaaatggtgattcctcctcttccacacaaatatctggggtaggtcaagaggggggagggaagaaacctgaagggcattcctgtctgtagattagggctggaaatgggaaggactgtggggtctaagatttattctggtccccatttgactttgcctttgtcttcaggtgtagaggagcctatttgtgtccgaagcctagagagtcacttggttctcactctcggctgcactttgaaaaggtacctcatttcttctggcagctccaggaggtaaggcgaaggaggagcaacctggtaggatctgcagactggacctggggtctggaaagtcagaagggagtggaggcaagcagggagcagagtggtggcaagcagggaggctgccctctgtagtgttgtgtagctgctgcttgcagccagccagggtgctcatttgagcccatgctgcgtctcccggtgccttcggaggtccaccttcctctggaaacccttcccacagaggtcgcagccgaagggcttgaagcctgtgtgtttgcggctgtgggtgatgaggttggagctctggctgaatgccttgccgcacacctggcacttgtgaggcttctcaccagtgtggatgaaagtgtgtttcttcatgtctgacttctggtggaacctcttgccacagtactgacaggggtagggccgagtgtctgagtggataagcaggtgtgtggacagtgtggatgacctcttgaagctcttcccacagatcttacagtcaaagctccgttcctgcgagtgcacggctttgtgctgctccaggctcaccgcgtgcccgaaggtcttgccgcacatctcgcaggcaaagggtctggtaccgctgtgggacctgcgcacgtgcacctcgagcccgtgcggcgtggagaacaccttgctgcacttgatgcacttgtaggagccgccgcccagcagcaggcgggtgcacagcagctccgactccaccttgacgccagcgcccttgtctgcgtgcagcccgtggccacgctcggggtacagcaagcccgccgctgccgtgggcctctcatacagcccggctgccgcagacccgaagtcgccgtagagccctaggccagggccagcggtggcaccggcccctgcgctgcagctccctggcgccccggcccccgcgccgccggcagcccgcttcgggccgtacagcgcggccgggtggccaggctccggggcgggttcgcagaagaggcccaggccagcgccacgctccagggccccacacggtcggtagctctgcaccaggtgccgcaggtcagaacccgccaggccgctccatgagtacggtttgaaaggcagggggaagggctgggcttcgtccagcgatgggcacattgacttctccgaggctggagacgcggagggtgacgggggcctccagaagtcctcaaactccgagctccgttcgcagacgctgccttcgcagctgtctggggatgcggaggctctgtctggggcttcggtcagctgcgattcgggggacaaacggtcccggggctccgccttcgccccgcctgcatttgaagtgctgtctgctcggctaggcgccggtacattctctaaacggagggaatagtctggtcctggggagcgcggctggtggtagctgtgagccttcttgcttttgacgagaaatgagcgcggcatggtggtccggcactttccccactgcgccccaagagtccctggagccgctgtcacccacggtcactccgagggcttgctcagccccagcccggaggagacctgcggagtcacggcgcgggcaccgcgctaggagagttttcaaacggaatcttgctttcgggagagaccgctctatctctctgact

SEQ ID NO: 18131 - RNA, 3778 nt, Homo sapiens
  source 1..3778: mol_type = other RNA
tgaaggtctactgtgtgccaggcactattctgggaactgaggattcaacaatgaataaataaagcttcgtaagacattgtcctcactgctatatctccaccccctagaagaatgcccagcacatactgggtgctcaattatatgtgtgaaatcaatttgagttggaaatgggcaatctgctggttctcaccatggggcatgcataccctgaatgtctggctgggaggtgttaaagcactagtagtagggattttggccaggattttattctggtttcattctcttaaaggattgacttatgcaaaaaactcccacaggtgggacagaaccagaaataacccagatcctcatgggcctttagatttgtgacttgcattaggggaggcagctaaccaatctcacactttttttcctttccagtctccacagaatcaaagcggtcagggttggacaggaatgacagagctgtctccgtattacttgatcaaggaaaccagtatcggggaagtcaaaagatttacacaagtcacatgatgtgttggtgacagagctgtgactaaaactaaaacctagacctaagacctgtgatttctttattcatctgggagccttcaggcccctaaaaaaatatgttgacattttcagaggaaagagcttacttacgtgcctgtggaaccatcaggggctctacaaggtagtagcttagttttgtacacctcctagtttttctcttatgaaagaagatgaaagaagtatctctgaggtgtagcagcaaaggagaaagtatatggaaacccgagcaattggattttactcttctggatattagcttgtgtgcttcacttttatactccattgcagtttccttcagtgccagctttccccctacagactaaaacaaaggtcttccccaaattccctgcctaaaggaaaggcaatctgtaatactcttaatactttattaacttaaaacatcactctaataaatatgtattaacaaacataatgcttaccagaagatctaaaaacatttaccaacctcatcaaagtgaaaataccacctttcccccctctatggtacacatggagggtcaaagagttgaagacagagccttccttcccacatgcctgctagctcagaaatctttaaaatatcagcttaacaataaaaaactgaatatacacacatatctttgaagtaactgttcagctttttgtttacacctgataaaatccaaaagggtcaaaagggaaggtttacaattctgtgctgtcttctcagaattccctccaagagtaagaacagacccagccacttggaggtgcaaccgttagcttttgaggagcagtcaggggttgtgacttcagtctctcttccccaatacctagcatggtgcctggtaccttggtagccggtgatccatgaacatttgctgagtgaatgaatgacatcttgtccacaggcattgcttgtgcttttacctccagtgatgaggttttcacagccctactgaagggaggacctctaatcccctctcattaccaacttctcttctgcttcttcttgggggtagcctcgatggtgcatctcatgacttcaaagtattaaattccttccccaagtcagtttctgaatcagtttttgaggaggagaaatgattcctccaagatttataggcagcacccaaaagaaaggagtcaacagaccccccagaaggaaaaaaataaaagttaacactcactcttctttctagataaaaatattagcatttgtccaccttgtaaatggtgattcctcctcttccacacaaatatctggggtaggtcaagaggggggagggaagaaacctgaagggcattcctgtctgtagattagggctggaaatgggaaggactgtggggtctaagatttattctggtccccatttgactttgcctttgtcttcaggtgtagaggagcctatttgtgtccgaagcctagagagtcacttggttctcactctcggctgcactttgaaaaggtacctcatttcttctggcagctccaggaggtaaggcgaaggaggagcaacctggtaggatctgcagactggacctggggtctggaaagtcagaagggagtggaggcaagcagggagcagagtggtggcaagcagggaggctgccctctgtagtgttgtgtagctgctgcttgcagccagccagggtgctcatttgagcccatgctgcgtctcccggtgccttcggaggtccaccttcctctggaaacccttcccacagaggtcgcagccgaagggcttgaagcctgtgtgtttgcggctgtgggtgatgaggttggagctctggctgaatgccttgccgcacacctggcacttgtgaggcttctcaccagtgtggatgaaagtgtgtttcttcatgtctgacttctggtggaacctcttgccacagtactgacaggggtagggccgagtgtctgagtggataagcaggtgtgtggacagtgtggatgacctcttgaagctcttcccacagatcttacagtcaaagctccgttcctgcgagtgcacggctttgtgctgctccaggctcaccgcgtgcccgaaggtcttgccgcacatctcgcaggcaaagggtctggtaccgctgtgggacctgcgcacgtgcacctcgagcccgtgcggcgtggagaacaccttgctgcacttgatgcacttgtaggagccgccgcccagcagcaggcgggtgcacagcagctccgactccaccttgacgccagcgcccttgtctgcgtgcagcccgtggccacgctcggggtacagcaagcccgccgctgccgtgggcctctcatacagcccggctgccgcagacccgaagtcgccgtagagccctaggccagggccagcggtggcaccggcccctgcgctgcagctccctggcgccccggcccccgcgccgccggcagcccgcttcgggccgtacagcgcggccgggtggccaggctccggggcgggttcgcagaagaggcccaggccagcgccacgctccagggccccacacggtcggtagctctgcaccaggtgccgcaggtcagaacccgccaggccgctccatgagtacggtttgaaaggcagggggaagggctgggcttcgtccagcgatgggcacattgacttctccgaggctggagacgcggagggtgacgggggcctccagaagtcctcaaactccgagctccgttcgcagacgctgccttcgcagctgtctggggatgcggaggctctgtctggggcttcggtcagctgcgattcgggggacaaacggtcccggggctccgccttcgccccgcctgcatttgaagtgctgtctgctcggctaggcgccggtacattctctaaacggagggaatagtctggtcctggggagcgcggctggtggtagctgtgagccttcttgcttttgacgagaaatgagcgcggcatggtggtccggcactttccccactgcgccccaagagtccctggagccgctgtcacccacggtcactccgagggcttgctcagccccagcccggaggagaccttgacacccaatccgagaggtttgctcatttcccttcggatttaggtaatggttaaatttggaagaggtgggcgagcgccgagcccccggcggagagggccctggcggcgcgtcccgcgggcgcccggcgggaccggtgggcgcaccctccctgcgcggagctcgccggctctcgaccgggtccgctcagccttcgact

SEQ ID NO: 18132 - RNA, 5238 nt, Homo sapiens
  source 1..5238: mol_type = other RNA
tgaaggtctactgtgtgccaggcactgtgctaggcacttttcgtacaatatctaatttaaatcctcacaacaaccctgtgaggtaggtattattatcatcattttacatacgagggaactgaggctcagagaggttaaataactctatcacacaaccaaaaatagtagagctggaattcaaacccaaaaccacctaactccaaatcccatgctccaatgaattaaagtagagaggggagagggagggccaaattcaagacagagtgttggagtgaaatggatatgatatgctgataagatatgggaagaaggaatgtaagctcataaatgtttctagctggtgagcctatgtagattgtgatgaagtaaccaggagaggaattcaggaggaacatacttggttgggcagatgagttgagtctatacggaactgtccatagagatgtccagtaggtaataccaatacagatctaaagtctgggggaagttgggggttggagctatgtatttgggaatcaccagcatatcagcagcaattgaggacatcaggatgaatgactccattttgggagtaaatagaaaggaaagagaagtgaatcaaagatggaacgatggaagcactgatactgacaggcatgagcaatcgttgagaaattctcaagagagtcggacaagacagagtcagagagagaagtacatgaaacagccctgtagtggtggctagaagccatggactgggttgggaacaattctagagctcccagaaggcaggcaagattgagtcacacttccaacaaagccctctgcacaccaaaaccccaggaagtattgtttttctttgttagtttgcttttgagacagaatctcactctgtcacccaggctggagtgcgatctcaactcactgcaacctccgcttgcttcctggattcaagcgattcttgtgcctcagcctcctgagtagctgagattacaggcaggtgccaaaacacccatctaatttttgtatttttagtagagacagggttttgctatgttggccaggctggtctcgaactcccgacctcaagtgatccacctgtctcagcctcccaaagtgctgggattacagacgtgagccaccgcacccgtccaaggaagtattgttaattgaaataaatgccaaaatgttcctaccttggtttaccccaaaacctggagctaagaacttcatctcacttttgacaccccagcccccaaaatatggaagcccaggagagccaggagaatttatagcagaggcttaaagagaaagttatgatttgtttaaagtagagaataaggtgaaaaataaaacctggtactctgtctggaagtcctggaagtctccttgcccaacctcaactggcctgtgggctcctgtgtccttgctctgggatgccatggtgaatgtgaaaacaggggaggttgtgtgtgggggtgggaatggcctgtcggttgcaaggcgagtcctttgctgagcccagcctgagacccagcttatgggctttatccaggtgagaaaatgctggggacatgtgtgcgaggtttaaggtctaccaggaaggggagaagggtgtcaggggaccagccccacaacctaggagaggattaggagggtccagccctttgggcagggaccagccctgaggcttaaatgaacttgcataggcacctgtgtatgcatctctgtgcatgtatgcatacatgagtgagagagaaagataaagagagctaaagaggcccccctccccccgccgcaggctgccacacgtggtgcgatccgattctctctggaaaggaggagagtctctcatgcatgggtgaagttgggccctccccagaagcctagtgactcattatgttaacgtgtgggtgtgggggctggacatccttgggaagccctgaggggctgctgaagcagggttcctggtctcctcggaggctgggcctcccctcgctgggggctcacagaaagtcaaacagcccgaaattcttggctgctccaggcccagggtaaattgggggaggaaaaaagaaagaaaagaaatgtttcaggcctggaggtgagatgagcctgctggttagtagggttaggggtctgaaggaaccagcacgcagggcaggcatggggcaggggtagagcagagatgctccctggaagccaccagctgctcaggcaactgagggggccctctgggcctctgatctaggcacaggcagggatggcatggatggctattggaggcgactacagctttaggttgcaggactgaggcagcaggcagggggatggttagtaggggcagatgaagcaaatatattttggtttcagtaatgtggggtaaagtcaagaggtttgcacacgtgcctgatggggtggggttaatagagggatgatgtagctgaataaatggtgaaagggagctaaaggggaaacgagagaatgagggagtgagcgtgccaccaaggtcattgctggggtcaactcccaaaatgggggttgcagaggggagtaaggggtagcaccaacaagtctggtcccagagacaaaaggggtcctgggaagtcctgcgcagggattagtgggcagaggaaacgaactggggccagaggcaggttagggggctgcagagccaatcggtaggtgcaccccaccctcgcagcaccctgcgagcagttagcgcacctggatttagttccttttatttccctttcaggtaccagacaaagtaaaaaagacggacggatggagagaggaacgcagccggctggggtgggagcggaatggagctgggggaggggccctgctcacatcacatccacaaagaactcactggggtttcccatggccatgcggaaggactgtctgctggcggtcagttccgggggcactgaggccaggtcgcggcccggaggggctcctgggggccccatggccgcgggcggcgggggcatcatcagcatgggggggccgtagagagggggcactccgggaggaccgtagctcgggtgtgtgtggtggctgcgaaggctgctggccagggaatggtggctgcggtggctgtgctcgctggccgccggccctgagcgctcgctgggcgcccgctcccgcggcccccgcaggctgctgcgtgtggtgtggtccgattcgctgccgctgcccccggacttggagtccccggccttcgggtccttctccttcctccgatcgctgccgctacggttggagccactgctccgactgccttcgctgtgctgactgctggcgctgcccccgccgtagctgtagcccagctccgggaagcccgggtgcgggttgtatgggtgcgggggtggcgggtactggtacgggaaagccatgggccaaggggcggcccccgggtgcggcaaaggggccagtgtgtcctggtcagaggcgccactggagccatcgtgatcgtggagagacaggttggccatgttgccgcagaggtcaccgaagatgtagtagcactgctcggagaaggtgatcttgttgacggtatggcggatgaagccagctttcagcaggttgctggcatacttgcgggcctccctccggtccgtgaagccttccacattgtggtacagccagtccaccacatctgagccgatgaaagcattagggatggtaatcttgagccacatgcggtcacggacctccaaccctgattcaggggaggccatggcttttacgatggcagccatgtcactgtggatggacaagtggaagtcgtctaggcgctctgtgtcagggatggaactggtgatggaggagctggtggaggtgatggtgctcagggaggggctcatgccgtatgcagggaaggtgccggtcatggctgcagtgtgggagacccaggccgcagggtcaatgggccggatgggctcgctcctgggcaatgtgaagcaaccacgtggacttgggtcccagcacttggctacagtcagggtgatgggccccggtttgtgcacaatctcccgcagtacccggactgcatcgtcattactcatgttctcaaagttgatctcgtttacctgtaacaacatatctcctggctcgatgcgtccatcagcagccacggccccacccttcatgatagagccaatgtagatgccgccgtcaccacgctcgttgctttggcccacaatggagatgcccaagaagttatatttttccatgttgagagtgaccgtgatgatgttgagtgacatggtggagtccgtgatgctgctgaaggacgaggaccgctcaatccgagaaaccttctgcttccgccgccgccgcttgtgtcttctcatcaggcgtgaggcactgctctgttctgtggagctgctgaacctgctggtggagtcatcctcatctgagtcaaagaagctggtggtctccagctcactgctcataagggtggatgagctatcataaccccctggttctcgccgccgttcccccttcgcagttccatttagccgggttgcatgctctgggccatccctccggcgtggccgctctcgctgggcagacaccaaagagtccgtctctgtgtcattgtccaggttctcctggctgcccccaccagcatgagggtggaaggatgggggtcgggagtccccgatgcctcccgtgcgctccataggtggtggcagctccgatgggttatcagcacagaagggggctgggtctgggtgtgagccctcagctgacaccagccaggacaccacccggccattgaagcatggtagcttggcattgtcatccgagatctcctccttcaccactccgaaatcgtcgtccatagacttgaagaagaacttatagctgggtcgctgcaaaacgcccttaaagtccgccaaggtgacgcgctcggcgggcaggggcagcttcacaaggtacggcgtctcctgcccatccaagtggtagatgatcttggtctcgcccatggctctggcctcgggcccggcggcccgcgcgcggcctgctcgggcggccgggccgagcctcccagacggcggcggcgcgcggcgcggcccagcggctcaacccagctcggcggctgctggcggcgccagctcccttgttctccggccgctaccgggtcccagcgccgcccgccgccgccgcggccgccgcttccgctccccactctcccgactggactggcgaccgcgactcttccggtggccgcggccctcccggccc

SEQ ID NO: 18133 - RNA, 4907 nt, Homo sapiens
  source 1..4907: mol_type = other RNA
tgaaggtctactgtgtgccaggcactgtgctaggcacttttcgtacaatatctaatttaaatcctcacaacaaccctgtgaggtaggtattattatcatcattttacatacgagggaactgaggctcagagaggttaaataactctatcacacaaccaaaaatagtagagctggaattcaaacccaaaaccacctaactccaaatcccatgctccaatgaattaaagtagagaggggagagggagggccaaattcaagacagagtgttggagtgaaatggatatgatatgctgataagatatgggaagaaggaatgtaagctcataaatgtttctagctggtgagcctatgtagattgtgatgaagtaaccaggagaggaattcaggaggaacatacttggttgggcagatgagttgagtctatacggaactgtccatagagatgtccagtaggtaataccaatacagatctaaagtctgggggaagttgggggttggagctatgtatttgggaatcaccagcatatcagcagcaattgaggacatcaggatgaatgactccattttgggagtaaatagaaaggaaagagaagtgaatcaaagatggaacgatggaagcactgatactgacaggcatgagcaatcgttgagaaattctcaagagagtcggacaagacagagtcagagagagaagtacatgaaacagccctgtagtggtggctagaagccatggactgggttgggaacaattctagagctcccagaaggcaggcaagattgagtcacacttccaacaaagccctctgcacaccaaaaccccaggaagtattgtttttctttgttagtttgcttttgagacagaatctcactctgtcacccaggctggagtgcgatctcaactcactgcaacctccgcttgcttcctggattcaagcgattcttgtgcctcagcctcctgagtagctgagattacaggcaggtgccaaaacacccatctaatttttgtatttttagtagagacagggttttgctatgttggccaggctggtctcgaactcccgacctcaagtgatccacctgtctcagcctcccaaagtgctgggattacagacgtgagccaccgcacccgtccaaggaagtattgttaattgaaataaatgccaaaatgttcctaccttggtttaccccaaaacctggagctaagaacttcatctcacttttgacaccccagcccccaaaatatggaagcccaggagagccaggagaatttatagcagaggcttaaagagaaagttatgatttgtttaaagtagagaataaggtgaaaaataaaacctggtactctgtctggaagtcctggaagtctccttgcccaacctcaactggcctgtgggctcctgtgtccttgctctgggatgccatggtgaatgtgaaaacaggggaggttgtgtgtgggggtgggaatggcctgtcggttgcaaggcgagtcctttgctgagcccagcctgagacccagcttatgggctttatccaggtgagaaaatgctggggacatgtgtgcgaggtttaaggtctaccaggaaggggagaagggtgtcaggggaccagccccacaacctaggagaggattaggagggtccagccctttgggcagggaccagccctgaggcttaaatgaacttgcataggcacctgtgtatgcatctctgtgcatgtatgcatacatgagtgagagagaaagataaagagagctaaagaggcccccctccccccgccgcaggctgccacacgtggtgcgatccgattctctctggaaaggaggagagtctctcatgcatgggtgaagttgggccctccccagaagcctagtgactcattatgttaacgtgtgggtgtgggggctggacatccttgggaagccctgaggggctgctgaagcagggttcctggtctcctcggaggctgggcctcccctcgctgggggctcacagaaagtcaaacagcccgaaattcttggctgctccaggcccagggtaaattgggggaggaaaaaagaaagaaaagaaatgtttcaggcctggaggtgagatgagcctgctggttagtagggttaggggtctgaaggaaccagcacgcagggcaggcatggggcaggggtagagcagagatgctccctggaagccaccagctgctcaggcaactgagggggccctctgggcctctgatctaggcacaggcagggatggcatggatggctattggaggcgactacagctttaggttgcaggactgaggcagcaggcagggggatggttagtaggggcagatgaagcaaatatattttggtttcagtaatgtggggtaaagtcaagaggtttgcacacgtgcctgatggggtggggttaatagagggatgatgtagctgaataaatggtgaaagggagctaaaggggaaacgagagaatgagggagtgagcgtgccaccaaggtcattgctggggtcaactcccaaaatgggggttgcagaggggagtaaggggtagcaccaacaagtctggtcccagagacaaaaggggtcctgggaagtcctgcgcagggattagtgggcagaggaaacgaactggggccagaggcaggttagggggctgcagagccaatcggtaggtgcaccccaccctcgcagcaccctgcgagcagttagcgcacctggatttagttccttttatttccctttcaggtaccagacaaagtaaaaaagacggacggatggagagaggaacgcagccggctggggtgggagcggaatggagctgggggaggggccctgctcacatcacatccacaaagaactcactggggtttcccatggccatgcggaaggactgtctgctggcggtcagttccgggggcactgaggccaggtcgcggcccggaggggctcctgggggccccatggccgcgggcggcgggggcatcatcagcatgggggggccgtagagagggggcactccgggaggaccgtagctcgggtgtgtgtggtggctgcgaaggctgctggccagggaatggtggctgcggtggctgtgctcgctggccgccggccctgagcgctcgctgggcgcccgctcccgcggcccccgcaggctgctgcgtgtggtgtggtccgattcgctgccgctgcccccggacttggagtccccggccttcgggtccttctccttcctccgatcgctgccgctacggttggagccactgctccgactgccttcgctgtgctgactgctggcgctgcccccgccgtagctgtagcccagctccgggaagcccgggtgcgggttgtatgggtgcgggggtggcgggtactggtacgggaaagccatgggccaaggggcggcccccgggtgcggcaaaggggccagtgtgtcctggtcagaggcgccactggagccatcgtgatcgtggagagacaggttggccatgttgccgcagaggtcaccgaagatgtagtagcactgctcggagaaggtgatcttgttgacggtatggcggatgaagccagctttcagcaggttgctggcatacttgcgggcctccctccggtccgtgaagccttccacattgtggtacagccagtccaccacatctgagccgatgaaagcattagggatggtaatcttgagccacatgcggtcacggacctccaaccctgattcaggggaggccatggcttttacgatggcagccatgtcactgtggatggacaagtggaagtcgtctaggcgctctgtgtcagggatggaactggtgatggaggagctggtggaggtgatggtgctcagggaggggctcatgccgtatgcagggaaggtgccggtcatggctgcagtgtgggagacccaggccgcagggtcaatgggccggatgggctcgctcctgggcaatgtgaagcaaccacgtggacttgggtcccagcacttggctacagtcagggtgatgggccccggtttgtgcacaatctcccgcagtacccggactgcatcgtcattactcatgttctcaaagttgatctcgtttacctgtaacaacatatctcctggctcgatgcgtccatcagcagccacggccccacccttcatgatagagccaatgtagatgccgccgtcaccacgctcgttgctttggcccacaatggagatgcccaagaagttatatttttccatgttgagagtgaccgtgatgatgttgagtgacatggtggagtccgtgatgctgctgaaggacgaggaccgctcaatccgagaaaccttctgcttccgccgccgccgcttgtgtcttctcatcaggcgtgaggcactgctctgttctgtggagctgctgaacctgtggggcccacagtcgttccccaccaggctggcccagccctgcccccatgaggggaggcactgcagggcctgggtccccaacacaaagcccataagcctcccaggggccccgcatcctcagggtttagggctcctccagggtcacctgccccacaatacccatgaaactcaagccccacctgctggtggagtcatcctcatctgagtcaaagaagctggtggtctccagctcactgctcataagggtggatgagctatcataaccccctggttctcgccgccgttcccccttcgcagttccatttagccgggttgcatgctctgggccatccctccggcgtggccgctctcgctgggcagacaccaaagagtccgtctctgtgtcattgtccaggttctcctggctgcccccaccagcatgagggctgcagggaagagatggaaggatgggggtcgggagtccccgatgcctcccgtgcgctccataggtggtggcagctccgatgggttatcagcacagaaggg

SEQ ID NO: 18134 - RNA, 4467 nt, Homo sapiens
  source 1..4467: mol_type = other RNA
tgaaggtctactgtgtgccaggcactgtgctaggcacttttcgtacaatatctaatttaaatcctcacaacaaccctgtgaggtaggtattattatcatcattttacatacgagggaactgaggctcagagaggttaaataactctatcacacaaccaaaaatagtagagctggaattcaaacccaaaaccacctaactccaaatcccatgctccaatgaattaaagtagagaggggagagggagggccaaattcaagacagagtgttggagtgaaatggatatgatatgctgataagatatgggaagaaggaatgtaagctcataaatgtttctagctggtgagcctatgtagattgtgatgaagtaaccaggagaggaattcaggaggaacatacttggttgggcagatgagttgagtctatacggaactgtccatagagatgtccagtaggtaataccaatacagatctaaagtctgggggaagttgggggttggagctatgtatttgggaatcaccagcatatcagcagcaattgaggacatcaggatgaatgactccattttgggagtaaatagaaaggaaagagaagtgaatcaaagatggaacgatggaagcactgatactgacaggcatgagcaatcgttgagaaattctcaagagagtcggacaagacagagtcagagagagaagtacatgaaacagccctgtagtggtggctagaagccatggactgggttgggaacaattctagagctcccagaaggcaggcaagattgagtcacacttccaacaaagccctctgcacaccaaaaccccaggaagtattgtttttctttgttagtttgcttttgagacagaatctcactctgtcacccaggctggagtgcgatctcaactcactgcaacctccgcttgcttcctggattcaagcgattcttgtgcctcagcctcctgagtagctgagattacaggcaggtgccaaaacacccatctaatttttgtatttttagtagagacagggttttgctatgttggccaggctggtctcgaactcccgacctcaagtgatccacctgtctcagcctcccaaagtgctgggattacagacgtgagccaccgcacccgtccaaggaagtattgttaattgaaataaatgccaaaatgttcctaccttggtttaccccaaaacctggagctaagaacttcatctcacttttgacaccccagcccccaaaatatggaagcccaggagagccaggagaatttatagcagaggcttaaagagaaagttatgatttgtttaaagtagagaataaggtgaaaaataaaacctggtactctgtctggaagtcctggaagtctccttgcccaacctcaactggcctgtgggctcctgtgtccttgctctgggatgccatggtgaatgtgaaaacaggggaggttgtgtgtgggggtgggaatggcctgtcggttgcaaggcgagtcctttgctgagcccagcctgagacccagcttatgggctttatccaggtgagaaaatgctggggacatgtgtgcgaggtttaaggtctaccaggaaggggagaagggtgtcaggggaccagccccacaacctaggagaggattaggagggtccagccctttgggcagggaccagccctgaggcttaaatgaacttgcataggcacctgtgtatgcatctctgtgcatgtatgcatacatgagtgagagagaaagataaagagagctaaagaggcccccctccccccgccgcaggctgccacacgtggtgcgatccgattctctctggaaaggaggagagtctctcatgcatgggtgaagttgggccctccccagaagcctagtgactcattatgttaacgtgtgggtgtgggggctggacatccttgggaagccctgaggggctgctgaagcagggttcctggtctcctcggaggctgggcctcccctcgctgggggctcacagaaagtcaaacagcccgaaattcttggtggggtttcccatggccatgcggaaggactgtctgctggcggtcagttccgggggcactgaggccaggtcgcggcccggaggggctcctgggggccccatggccgcgggcggcgggggcatcatcagcatgggggggccgtagagagggggcactccgggaggaccgtagctcgggtgtgtgtggtggctgcgaaggctgctggccagggaatggtggctgcggtggctgtgctcgctggccgccggccctgagcgctcgctgggcgcccgctcccgcggcccccgcaggctgctgcgtgtggtgtggtccgattcgctgccgctgcccccggacttggagtccccggccttcgggtccttctccttcctccgatcgctgccgctacggttggagccactgctccgactgccttcgctgtgctgactgctggcgctgcccccgccgtagctgtagcccagctccgggaagcccgggtgcgggttgtatgggtgcgggggtggcgggtactggtacgggaaagccatgggccaaggggcggcccccgggtgcggcaaaggggccagtgtgtcctggtcagaggcgccactggagccatcgtgatcgtggagagacaggttggccatgttgccgcagaggtcaccgaagatgtagtagcactgctcggagaaggtgatcttgttgacggtatggcggatgaagccagctttcagcaggttgctggcatacttgcgggcctccctccggtccgtgaagccttccacattgtggtacagccagtccaccacatctgagccgatgaaagcattagggatggtaatcttgagccacatgcggtcacggacctccaaccctgattcaggggaggccatggcttttacgatggcagccatgtcactgtggatggacaagtggaagtcgtctaggcgctctgtgtcagggatggaactggtgatggaggagctggtggaggtgatggtgctcagggaggggctcatgccgtatgcagggaaggtgccggtcatggctgcagtgtgggagacccaggccgcagggtcaatgggccggatgggctcgctcctgggcaatgtgaagcaaccacgtggacttgggtcccagcacttggctacagtcagggtgatgggccccggtttgtgcacaatctcccgcagtacccggactgcatcgtcattactcatgttctcaaagttgatctcgtttacctgtaacaacatatctcctggctcgatgcgtccatcagcagccacggccccacccttcatgatagagccaatgtagatgccgccgtcaccacgctcgttgctttggcccacaatggagatgcccaagaagttatatttttccatgttgagagtgaccgtgatgatgttgagtgacatggtggagtccgtgatgctgctgaaggacgaggaccgctcaatccgagaaaccttctgcttccgccgccgccgcttgtgtcttctcatcaggcgtgaggcactgctctgttctgtggagctgctgaacctgctggtggagtcatcctcatctgagtcaaagaagctggtggtctccagctcactgctcataagggtggatgagctatcataaccccctggttctcgccgccgttcccccttcgcagttccatttagccgggttgcatgctctgggccatccctccggcgtggccgctctcgctgggcagacaccaaagagtccgtctctgtgtcattgtccaggttctcctggctgcccccaccagcatgagggtggaaggatgggggtcgggagtccccgatgcctcccgtgcgctccataggtggtggcagctccgatgggttatcagcacagaagggggctgggtctgggtgtgagccctcagctgacaccagccaggacaccacccggccattgaagcatggtagcttggcattgtcatccgagatctcctccttcaccactccgaaatcgtcgtccatagacttgaagaagaacttatagctgggtcgctgcaaaacgcccttaaagtccgccaaggtgacgcgctcggcgggcaggggcagcttcacaaggtacggcgtctcctgcccatccaagtggtagatgatcttggtctcgcccatggctctggcctcgggcccggcggcccgcgcgcggcctgctcgggcggccgggccgagcctcccagacggcggcggcgcgcggcgcggcccagcggctcaacccagctcggcggctgctggcggcgccagctcccttgttctccggccgctaccgggtcccagcgccgcccgccgccgccgcggccgccgcttccgctccccactctcccgactggactggcgaccgcgactcttccggtggccgcggccctcccggcccagggcttcgtccgggcccgctcccctcctccggcccggcgcggccccgccccggcgcgccccgccc

SEQ ID NO: 18135 - RNA, 3794 nt, Homo sapiens
  source 1..3794: mol_type = other RNA
tgaaggtctactgtgtgccaggcagtgtgcaaggcgctttacatacattatcgcattaaatcctcacaacaaccctgcgaggtaggtgtttataaacccccatttgacagatgaggaaactgaggctcagggaggtgaagtgatgtggccaagttcacatggctaataaatggcagacagaggaggtgtccaaggatcggagagaaaaaaaaaaagacttcggtgtctgagtcccaagccggctggggtggatgagtacaaagatgggcccggcgggctctagaagtctgggaggccggaggcctgctcccggccccgcacggctggagactgcaaggcgggggacccgcgctcgggaactagggataggattgagtggcagagccgggattagcaactggggagatccgcgacctgcgcgcgccctgtagtggctatagagagtatcacaccccacgcctgctggcttctggtgaccggcctctttccttgcctggccggtttctggaagaggccaagatgggagaaattctcaggattttttcaggtgggcgataccacctgggagggagatcgtggccacgcctcagagcatcactaaggagcatcggggtggaggaaaaggggaaggcctaaagaggtcccaagctgattcattggtgtccttccctccccagctcagaccaccacaggccagggtcagtgacagggccgctatcttgccctgccttggggagccctcaaccaaacctgggagactgggataggagtgcctcactcccttacctcttctgcaagccttgggcagtctcctgaattgatcatgactttgggtgacacggaggccgcccagaaaccctcaaactctgttcacttattcccaattctcattcttggcttgtcgaggggaggatgagatagagtcctttccaaagatctcaaaatgtcagagacggaaggatggaccttagaataccatcattttatataccaggaggcctggaggcctggagagggaaagtgactggcctcagtcaaccagcaactcagtggcagagttgggattgaaatccaagacttgtgacaccaaggtgagccctccttctgctttgttggttgttgctggacctatgcctcttctcccaagaacccctctgtcatctgatcactctgtcaccaggtccaaagcctctccttcactttttccctcctcctcagaggccctaccctaccctgccctcctatggctgccaccatccctgccctcctgcctgatcctggttaggcctctctgctcagctccacacccagtgcatcagcccctgcgaagagctcacccttgtgccctgaacataacagacattaattaaatctgctcattctcacctctcctgaaacaaaatcattaatgggcatatgcttcccttcctttcatttatatttcaaggatgagaacaggtatgggtaaagatacaaggaaaagagaagcaaaggaagtctgtggggaagaatggggaccagtggacccaaggatggatgcgttggggacacaaatacaagaaggggcctctcactgcctcttcctatttccctgttgggtccctctgatgtccctcaccccgaagaggacctcctcggtttggcttatgacatctaggatctccccgacactgtcgctcagttccgctgtcttcccatcttcctctggcgaactgtttccaacctcgggcagggtcctctcattccgccaggaggcgcccggggcttctgtgtcgcttccatcagaggagccgctatggacgctgagctcctcagcttcgtccgtgtccgagtcaggggctgtgtggcggcggatacgggacacggcttctcgcagggccccggcgtagggccctggggtccgcgcccagccccggccggcgcgccgctggaccaccgccacttccgacccctcggctctgccctgggctcccgaagctgctgggcctaaggcttggtgctctgggctacctggctgcgtgggggcgtcccgcaggtttacttcgggggccgggagccccaagatgcggaaagtgcgctcctccagtgtggagtcccccggcctcccgccctcagcttcgcccccgcggcccccgccgggctggtgtaaaaggcgactgctcgacagccgcttttgacaaggggaaggaaagaccgtggccccttcaccctcctccttgccgggcttcgattggctgggggaatcccccaccacgcgtgtcaccccagagggcaaaagctgcacctgctgggttcggggggttggaacatattgggatcgtatcactacgcacgtggcgtcaatgacaaagacgccttccccacgggacaggccctgggaactgcggggcaaggtgtgggcacggcgggtcgccttccaaccctccagggtctccggtcctgccccctctccaagacccagagattctctccatccggtgcctccgggagcccagggtctggggagtgtctggctatggcggggcggctgctttttaggggagggaatccagcatttgggaaaccagatctgttctccttctttcccttccctcgagcccttgaggtggtgcctggatctgggagcgggatgcggggcacagggagccgcagttgcagaccccgcaggagctatctcggtgcctgcgctccctgtagctttggcttggggatggctgtcgctaccactgttcaggtcagcagcagccagccccaggcttttctccacgacccccttgccgggctctggccttgctctggccgctccacagcctggggatccccccaagagaccttgcccctgtcggagaccccaagccccgaggacgtcccggtagatccgaggatccagcctcttctttgtgcgccctccgtctgtcctggctggagtcgcagctggggctgatgaagtgggcacctgagagttcccggggcctctcttagtccccaaggtcctatgggggccttcgtaagaaggtggagccacgtagggtggcggccggtcccagcggcgtcgtggggcggtcccggcagaacctctcagcagcaggtgagcctcgtagcttgggggcccgggccgccgacctccccagggccccgcccacgccgaccctgggtcgctctgcggctgcgcggatggacggggcgctcgccccacaggcgccaggcgctccggccgcaagggagcagggagccctgccagctgggccacccgaggggcgttgcggggctccgggcggggtcgacccggggggctccgtcgggccccaccagccttgcgcctttttcgctcggtctccttggcctcccgctcctgcgacgccgctttccttttctcttgctcccgagctcggacctcggccaggggccccgcccgccagttggtcgcctcctgcagcaccctggaggcccagggccggcggggcggcggctgtggggatcccgggcgcggcccacacgtgcggttctggaacccgcgagcccagtggctggcctggaagtccatgggctgtcgagaaggggcgcggcgactataatgacaggaaatagtcttcacttctatcaccaatagcttggacttctgcacccagaggcagctgccagactcctcatcctggagctcccgggggctgtcaggcccctcggagaacagtgggccatccagcatcctgccccaccccaccccggccccccaccctcccacccgccccaggagccccctcccagcccagggagccggcgcccactgcagagcc

SEQ ID NO: 18136 - RNA, 4330 nt, Homo sapiens
  source 1..4330: mol_type = other RNA
tgaaggtctactgtgtgccaggcagtgtgcaaggcgctttacatacattatcgcattaaatcctcacaacaaccctgcgaggtaggtgtttataaacccccatttgacagatgaggaaactgaggctcagggaggtgaagtgatgtggccaagttcacatggctaataaatggcagacagaggaggtgtccaaggatcggagagaaaaaaaaaaagacttcggtgtctgagtcccaagccggctggggtggatgagtacaaagatgggcccggcgggctctagaagtctgggaggccggaggcctgctcccggccccgcacggctggagactgcaaggcgggggacccgcgctcgggaactagggataggattgagtggcagagccgggattagcaactggggagatccgcgacctgcgcgcgccctgtagtggctatagagagtatcacaccccacgcctgctggcttctggtgaccggcctctttccttgcctggccggtttctggaagaggccaagatgggagaaattctcaggattttttcaggtgggcgataccacctgggagggagatcgtggccacgcctcagagcatcactaaggagcatcggggtggaggaaaaggggaaggcctaaagaggtcccaagctgattcattggtgtccttccctccccagctcagaccaccacaggccagggtcagtgacagggccgctatcttgccctgccttggggagccctcaaccaaacctgggagactgggataggagtgcctcactcccttacctcttctgcaagccttgggcagtctcctgaattgatcatgactttgggtgacacggaggccgcccagaaaccctcaaactctgttcacttattcccaattctcattcttggcttgtcgaggggaggatgagatagagtcctttccaaagatctcaaaatgtcagagacggaaggatggaccttagaataccatcattttatataccaggaggcctggaggcctggagagggaaagtgactggcctcagtcaaccagcaactcagtggcagagttgggattgaaatccaagacttgtgacaccaaggtgagccctccttctgctttgttggttgttgctggacctatgcctcttctcccaagaacccctctgtcatctgatcactctgtcaccaggtccaaagcctctccttcactttttccctcctcctcagaggccctaccctaccctgccctcctatggctgccaccatccctgccctcctgcctgatcctggttaggcctctctgctcagctccacacccagtgcatcagcccctgcgaagagctcacccttgtgccctgaacataacagacattaattaaatctgctcattctcacctctcctgaaacaaaatcattaatgggcatatgcttcccttcctttcatttatatttcaaggatgagaacaggtatgggtaaagatacaaggaaaagagaagcaaaggaagtctgtggggaagaatggggaccagtggacccaaggatggatgcgttggggacacaaatacaagaaggggcctctcactgcctcttcctatttccctgttgggtccctctgatgtccctcaccccgaagaggacctcctcggtttggcttatgacatctaggatctccccgacactgtcgctcagttccgctgtcttcccatcttcctctggcgaactgtttccaacctcgggcagggtcctctcattccgccaggaggcgcccggggcttctgtgtcgcttccatcagaggagccgctatggacgctgagctcctcagcttcgtccgtgtccgagtcaggggctgtgtggcggcggatacgggacacggcttctcgcagggccccggcgtagggccctggggtccgcgcccagccccggccggcgcgccgctggaccaccgccacttccgacccctcggctctgccctgggctcccgaagctgctgggcctaaggcttggtgctctgggctacctggctgcgtgggggcgtcccgcaggtttacttcgggggccgggagccccaagatgcggaaagtgcgctcctccagtgtggagtcccccggcctcccgccctcagcttcgcccccgcggcccccgccgggctggtgtaaaaggcgactgctcgacagccgcttttgacaaggggaaggaaagaccgtggccccttcaccctcctccttgccgggcttcgattggctgggggaatcccccaccacgcgtgtcaccccagagggcaaaagctgcacctgctgggttcggggggttggaacatattgggatcgtatcactacgcacgtggcgtcaatgacaaagacgccttccccacgggacaggccctgggaactgcggggcaaggtgtgggcacggcgggtcgccttccaaccctccagggtctccggtcctgccccctctccaagacccagagattctctccatccggtgcctccgggagcccagggtctggggagtgtctggctatggcggggcggctgctttttaggggagggaatccagcatttgggaaaccagatctgttctccttctttcccttccctcgagcccttgaggtggtgcctggatctgggagcgggatgcggggcacagggagccgcagttgcagaccccgcaggagctatctcggtgcctgcgctccctgtagctttggcttggggatggctgtcgctaccactgttcaggtcagcagcagccagccccaggcttttctccacgacccccttgccgggctctggccttgctctggccgctccacagcctggggatccccccaagagaccttgcccctgtcggagaccccaagccccgaggacgtcccggtagatccgaggatccagcctcttctttgtgcgccctccgtctgtcctggctggagtcgcagctggggctgatgaagtgggcacctgagagttcccggggcctctcttagtccccaaggtcctatgggggccttcgtaagaaggtggagccacgtagggtggcggccggtcccagcggcgtcgtggggcggtcccggcagaacctctcagcagcaggtgagcctcgtagcttgggggcccgggccgccgacctccccagggccccgcccacgccgaccctgggtcgctctgcggctgcgcggatggacggggcgctcgccccacaggcgccaggcgctccggccgcaagggagcagggagccctgccagctgggccacccgaggggcgttgcggggctccgggcggggtcgacccggggggctccgtcgggccccaccagccttgcgcctttttcgctcggtctccttggcctcccgctcctgcgacgccgctttccttttctcttgctcccgagctcggacctcggccaggggccccgcccgccagttggtcgcctcctgcagcaccctggaggcccagggccggcggggcggcggctgtggggatcccgggcgcggcccacacgtgcggttctggaacccgcgagcccagtggctggcctggaagtccatgggctgtcgagaaggggcgcggcgactgccagctgcactgatgacttgactcgaagatgcttccttccaccctaggtcccactagagtcctgaggctttttaaagcccttgcctcctccctaggcaaatcttccttaatgagggaatgtgacataaggggccatctgtcctttccaccatgtgcttaccctcctgacacataaacatactctaattctaataacttggaagccttcctcccccaaggttgagaatgtgctgtgagagctgtaaaggggtgaaggcagaagcaggggctcctccacagccatgatgcaacactgaaagctgagctctgatgagggccaccttctttttttaaaataagcttcctcaggtcgaatctgatgagggccttgatgcttttccctgtgttccatcaggagaacccagtatgccctggctggagggttatcagaggggttaggcactgtggggcaggggcaaggaatgactccgaaattgctcctggcttggatgggaaactgtatcatacctgcaaggctggggtgagctggcacccaaatttagctcatactccagtctagcagttcttctgatgttgggtgctgactgctgtttgggtctacatgctttcaatacagggaatggatctgatggagtgaccactgccctgctgttctcccaccatccagctcattctcaccttggaagaggcaagggatttgtaggtttaaagatagtgctggccgggtgcggtggctcatgcctgtaatcccagcactt

SEQ ID NO: 18137 - RNA, 533 nt, Homo sapiens
  source 1..533: mol_type = other RNA
tgaaggtctactgtgtgccaggcatccatctacaagttgagaatacagcagcaaacatagcaatgtaaatcctggtcttatgtcccagtgcttaaaacacaccttcattgtttaatgtaattttaaactattatattgctccttctcaaaaaaatagaaacctcacccacatttaaaggagtcctgattgccacttgatcatatcattaagtcaataatatgttaagctatcagtgttaaaaaattatccttgaaatccatattagcagaagctagtttaatcagcacataaatggagaactggaaaacgatgagaggggatgtcatgttgatgaaatggtgtgctattttcctcttgattagaaggaggaagagtgccagaagagattgtgagagaattctcaggagtcagttgtgacagaagatggattgcagagggatgttttaagagtgaagtaatttcttgatctctttctttctgaatatggtatcaactaatctagcctgagatttcctctgtatcacttggtgct

SEQ ID NO: 18138 - RNA, 8929 nt, Homo sapiens
  source 1..8929: mol_type = other RNA
tgaaggtctactgtgtgccaggccatacacttcatacttggaattcagagataagtgaaagatagcccaggatctcttggggcctacaatctggtagggagaaaccaacatcgggggccatgcaaagaatgtttcagggtctttgtagggaaacaggagcaaaaaatagtgactgatcaatttttccagagggcaaggaacacttttctgaaggtggcccttgagctgagttgaaagatgagtaattatgtaggtgggagagagaaaaggggcattcaggaagcatattctgggcagagggaacaatggagcacagatgccagaaaggagaaacagcttggtctgttcaggaaaccctgaatgccaagccagtgtttagagtgcatcatggacagtgatatataggagctagcttgtattggcttgcaagagctgttaaagtttcaggaattttgtgaactggctgacatcacataacttgaaatctgtcatggtgggagcatttacaccacataaataatcatacactaaaaatcactcccttttcctactcattccactgctaaatcttggagacagttgagagcttttgaaaactgctttttttttttttttgacatgagagtgctattatgggaatgctgtttatagctaatctgtaaaaaatgcataagatggtttagagcagggaaaactgacaaatcagttggaaagtcaagagtttagacaactgataagggcttgacaaaagagatggaaacaaatggatattttcattttcaagaggccctacaagagtagacagaattcagtaacagatacagggttggcagaggtagcagtggatacaaggtggatgagttaaaaagtaaggagtagtaaacaaatacatttgttaatgatggcagaaaaaatatctcctattaattgctacatctctcttgcctttaacttacagccttcttacatatatgcctataaccactgtctacattttcttagcacaaagttccttcttaagttctgttatatggcttccattacccatgttgatgctgaaacttcttactctagaaggccacttcttcagtggggacactgaccttgcggataccacaagtcccatgctaactttaaaataaaacatttctggtggagtgaattaaatttataaatacttcttataatgctacttttcctactatcacaaaagattgaggaaaggtgtatagctctatattacagggacaatgtaaagactgatattaaaaaagagacctttgaattacattgaagagaggattatacacatgcaaagaaattattaggcctatgtcatttgttgttttatatgcatatattcaaaacgcatagcccatcctccttgagaccccctaaacatgttacgaatttgaagtgtctctgcattattcaagtgaggcaggaaaaagttactctaagtgatctttcttttttatattttatttgaatacaattctaataatttgacattaatgcagtaaagggttaacctagcagcctcaggttactccagccctgcacttttcaaagagaggtgtcttcacgtactggcccttccttgactagctcctgggaaatgacctgagctcgtggaatttccagtttgataatagtgttctagtatgcctgaggccttgggctgcattttgttagtttgacgagatagtttatgctaacagtatgaatcatggcgaatgtctgtttttgaatggctgaagccctgggccatgaggtatcactacacccctggggtcttgagactcaacgggtaaggtcagtcacatgggtgatgcatgcctatgtgactgacttccagtaaacaccttggacaccaaggattggttgagcttccttggttggcaatattttgcacatgctgtcacacatttctgggagaattaagcatgtccccatgtgactcaacaaggaagaggcaccaggaagcttgtgactgaactgatacagaaatagggtactgcaaataacaaagcctaatataacaaattgacttagggttggagagaagaatttagggagtggggacacaaataccacagactggaaaactggtgacttgtttggtggtgtattagggtcctctagagggacagaactaatagatgtatatatgaaggggagtttcttaggaaaattgactcacacaatcacaaggtgaagtcccacagtctgcaagctgagaagccaggaagccagtctgagtcccaaaacctcaaaagcagacaagcagatggtgcagcccttcagtctgtggctgaaggcctgatagtccctggcaaatcactggtggaagtccaagagtccaaaagctgaagaacttggagtctgatgttcaagggcagaagacatgcagcacaggagaaagacggaggccagaagacttagccagtgtagtccttccaccttcctctgcctgcttttatcctagctatgctggcagttgattagatggtgcacaaccagattgagggtggatctgcttcttgagcccactgactcaaatgttaatcttctttggcaataccctcacagacacacccaggaacaatattttgcatcatttaatccaatcaagttgacactcaatattaaccatcacaaacggcaaaaaaatatttggtctaactgtcaacagctgtctttggaaagaagaccaaatactgattgaggctgtagccttaggggaaatgctaggagaaaaactaaaaattttgcatgggatggctctttcttgctgtgttcagcaaggttctagaagaaaaaaatgtatttttttctcgattgaaattagctagcctgcagagttggaggaaaatatcatcttgttaacgaaagcagtttttgccatttttttctctttattataaaggttatatatgaacaagaatatataaaatatatatgtataaagagtattttaaaagtgaacatccatgcaatcaccacccaagacaagaaatagaacattgccagcatcccagaagcaccaggtgccactccccaatcacactgctgtacttctccacagaggaaatcattattctggttctggggacagcaaaacacttgcttttctttacagttgtatctcatatatataactatatacccttaaaacaatatagttgttcagtttatactgttttaaactttatacaaatggaatcatgttgatggcatccttctgtgatttgcttcttttgctctatgctatgtctgtgatattcatctatgttgtggttagctatttccttcattttcaccactgtgtagaattctactgtttcaatataaatgccatggtacaatttaaccattctaccattgctgaatatttggttcatttctaacttttggatattgcagtgctgctatgaacattaaaaaatttttttcttggccaccttcctgactgggaagaactttcttgtacatgcttcctaggatacatgttcattagttttcccaaggcattgtattagttagggtcctgacagggaaaaaaataactgtaatgaaagataacctgcaaagatgtatacttcagagtgcaattgctaggttttgagcatgtttatctttaaatttactgagggacaaatttttccacagtgattgttttcaatgtaagagctgacatcatcaccaaaacttagtatcattagatcatttcatttttgcaaataaggtaaagatgtaatacctccttgtagttttattttttacttctcaaatattaatatggctgggaatattttcatgtttcttggtcatctggatttcctttcacttgaaatgccatataaagtcttttgtccaaatttctattgactgtctttttcttactgattcatagggatcatttatatattctggacactagtttttcaccagttatatatattgcaaatacggtggttctttatattaggtttatattaggttcactaagtaggtgagattatgcatgcttattaccagttcttgtagttttgctgtattttcttcaaatgccccaaatcaaaattataataaaaagaaaatgggttggatataatagacaaaacaggtagtaaagaatgtgaagaaaattctgggcacagaaaacaaaagtgaaggcataagagggaggaagagtggaaaagtagaaaaccatctctattagatcaattaaagctttaaattttatttcaaatgattaaatattactaaatgataatattcaactacataaatccttaaatgaaaataatttagcatttattctaatattgaagataataaaaataaacctaaggcaagacagaaaataattcactatggtactatttacctttcagtacattaaatcagtgtttcattgaacttaaatttgtacataatttacataagtaaatcacaccatcaagaaccataatactacaactttgtatttgccatagtgtataataacatcagtcatgggattggattggcatgctagcaggcattaagcctaatttgaagaatctagtaattaaaagtctagttaccactttgtcaaagtctgtgagttcttaattaagctattcctaaaatattataatatacaaaatatatatttagatcataagctaaaatatgaaacgcaaggggagagaaaacaaaaatataaaagatttagctccttaaagaagtaacagaaaatggcttccaacttcatgttgcaattaaataataactattattatattattgagacagagtctcgctcttcaggctggagtacagtggcaagatcttggctgactgcagctttgacctcccaggttcaagtagttctcctgcctcagccatctgagtagctgggattacaggcgtgtgccaccaagcctggctaattttttttttttttttatcgttttagtagagacagggtctcaccatgttggcgaggctggtctcaaactcctgacctcaagtgatctgcccattcggcctcccaaagggctggcattacaggtgtgagccattgtgcctggcctaactaattattttttgagaagaactcattgatagcacaaaagtacttggagaaactacttaagctaactactattaagctgtcttctttcacaaatattaataaaagtactgatagaaatgtaactaagatacataatgtgttttaatacacattaatcttttgaattacacattttctcttgaggattataataaaatgatggtacaatttatccttctttatagatttgtggaaagtaccaacataattgacaagaaatgaaatactgccatttaaaagtcctgtattaaaataaaactactttgaatcatcttagactaaatattttaaaaactgattcaagtgcttattcataagataatggaattttaaataagaaaagccaaattaaaaattatattttaggcaaaaaccattttaacacagataatactgtgatatttattttcctgaagaaaaccacttatgctagttacattaatactcttcatagaacttaagataaattttaattatgaatgctcatgaagtatttaaagacactaggatcaatgccaacaaagtagttaagtgctgaaaaattcttatgataatataggcatgtgtgaatctttgagagcccttacaaatgtttttatattcagtataaaaataataaaaaaatcaccttcttatcccattcctaatttcccttttaagaattatctcttaacaggattgatttccaattgatgtataatggaagtaaaattctcatggttataaaaaagatacacagaatcagtatatgtatcttagaaaagcaaacatcatctgaggaaggattattgcacttgccttcactaaataaatctgcaaacttaaaatcagaaagaacaaattcattgattataaaataactagtttcaattaaaaattaatgataaaatgttcaatgtttacttaaaaaatatatcaagggtatgtttgggattgtttggttttattttctttgatgttgagtactttgtcatcaatcctggcctttttgttcttgttacagccttctgtactccacttgagctaccagtacttctggagctttctttgggttgattaactgggttaaatttatcctttcttaattcttggataaaacttttatttaagcaaacatccacatgcacattgaacagggttagatctgaagtcttttgttctacgttacaaacaggacaaactagagcttggcctgttttcacttcacataagtaaggctggcggtattcttgtctaaatgatccaacatcttcgttttccaatgaaacagtagaagaagaattctgatgacagtgttcaatattaaaagacttgcttgggagactagaacattcttccttgctatgcttattacttaaagcatctatgctttctgctttagatgagttatctatagtatctactaaagctatacaatctactgaagatatttctttaatttttggatgggcttcataatcttgcttctcacaaagtgaagaagcaggaacattttctttcttgttaactttggtagcagaaacatgtgaacacgagaacattttaaagttttcactgattgaaggtccatcaagacattcatctacatgtttattcaaggcttccagactgatgcacccttgagccctaaagcaaacaggacaggtaagtatctgacagtcatctgaattctctgatatttccaaattctcattcatcttcttctttaaaacttggaatggttgtgatgtctggaaactttgtttattcacggcttcacatttaaatgtatcttggtgactccatttcctttctgatcgttttttatcaaagaaactcttcttatgagacatttctagaggttttacaaacttatctttgtcagttttctctaatgtacactcagtggctgacagggcttggtttccagcctgtaaaaagccaataatgctcctttgttggtgtttcctgtcctcttcattgggaaaactagatatccgaacacccataagccttaatctcaagggatgtggaaaatcagcatcaatttctgtttttagcaattccttagcaatggcaaatatttcttctgcagtagaaacaacagatgaaactgtagatgcacgagtttttacttcaaaattcacattcttcaacttaatggtaacagttctacccttaagtctttctttctgtagatcctgagcaagctcactgcaaagttcttgacataggctgtattgctcttccgctttatttatctcactgaatgtcctctcaacgctcatacttttcctctctccatccctcgtcaggtgtgttgaacctagacccaaggagatatgaaggaaataatgccaagatgtttcagagaaaaggagagaaagcaatgccctctgttggtaaagttctgtacatgtaataattccaagggcctttaacattttctctgtaacttttcctattccagaaacctttctaatgggtaaatccttgatgaagtccatcacagcttgtctattgggaagaatttggtattgtccatttggtttattcttatcactgcatacttttgctaacattgtatttggggcaatgcctgcactggctgtcagtgttgttttctgctcaattctgaaacgaatttcctttaccacttcctgggctgatgttccaaaaacaactgagttttggagtatttgaggattgttttgttcttcaaagttcacttggaaaggatctcctgggggctgcacatcagaaggactctcttcaaaaagtagtggagagatggatcgttcatgctcactcagtttattaacttcctttcctggattatcattttctacagagcttcccattttgatgaaataccttcttttatcctcaggccaattttgtctttcttctaagtgctttgttatattcaagtaggcttcatcaagactcatggccataaaattgggatcataatcagcaagtatttccttaacctctttactcacagctcggtatttgtcaaagttggggggcactattataagttgtgggcacagcctcttagcaataaatcctggcatggctgcacgaacaccaaatctccttgcatggtaatttgaagtagacagcatactcattgatcctacagcaatgggtttatccttcaattctggattgtccctcatttctacagctgcatagaaagcatccatgtcaatgtgcactatggtattgctcaaatttcggctttgttctaattccattgcaaatctgtcaacctctttggcatatgatgtttatgctgaacaggaaggtacaactgaagatactgtagcataatgtaaatgttcctctgtagaattgcttttataatgttaaaatttgatgttaatctgtaattgtgcttttcttagctgttggctggtgatttgagctttttgttgcatcatattttcaattcgttggttgacttgcttttctttcttgagctcatttccataaaatctggaccccttcgtggcttccattataattttgttaattttctctttatctaatccttccattcctgctttattatcattaagtcccatcctaagcagaagatcatctttgtaactgtcacacttctcctttgtgctatccatggtataaacttatccgttacctcaggatcgcgactacaactcccaggaggctgcgcgagcgacggaccaacgcccttcccagaatgcagcacagctgcatccctaccccgccctctcctttctccgctcctcctgcttttctacccgtcgtcacccgggagagccggaggtagggttc

SEQ ID NO: 18139 - RNA, 8667 nt, Homo sapiens
  source 1..8667: mol_type = other RNA
tgaaggtctactgtgtgccaggccatacacttcatacttggaattcagagataagtgaaagatagcccaggatctcttggggcctacaatctggtagggagaaaccaacatcgggggccatgcaaagaatgtttcagggtctttgtagggaaacaggagcaaaaaatagtgactgatcaatttttccagagggcaaggaacacttttctgaaggtggcccttgagctgagttgaaagatgagtaattatgtaggtgggagagagaaaaggggcattcaggaagcatattctgggcagagggaacaatggagcacagatgccagaaaggagaaacagcttggtctgttcaggaaaccctgaatgccaagccagtgtttagagtgcatcatggacagtgatatataggagctagcttgtattggcttgcaagagctgttaaagtttcaggaattttgtgaactggctgacatcacataacttgaaatctgtcatggtgggagcatttacaccacataaataatcatacactaaaaatcactcccttttcctactcattccactgctaaatcttggagacagttgagagcttttgaaaactgctttttttttttttttgacatgagagtgctattatgggaatgctgtttatagctaatctgtaaaaaatgcataagatggtttagagcagggaaaactgacaaatcagttggaaagtcaagagtttagacaactgataagggcttgacaaaagagatggaaacaaatggatattttcattttcaagaggccctacaagagtagacagaattcagtaacagatacagggttggcagaggtagcagtggatacaaggtggatgagttaaaaagtaaggagtagtaaacaaatacatttgttaatgatggcagaaaaaatatctcctattaattgctacatctctcttgcctttaacttacagccttcttacatatatgcctataaccactgtctacattttcttagcacaaagttccttcttaagttctgttatatggcttccattacccatgttgatgctgaaacttcttactctagaaggccacttcttcagtggggacactgaccttgcggataccacaagtcccatgctaactttaaaataaaacatttctggtggagtgaattaaatttataaatacttcttataatgctacttttcctactatcacaaaagattgaggaaaggtgtatagctctatattacagggacaatgtaaagactgatattaaaaaagagacctttgaattacattgaagagaggattatacacatgcaaagaaattattaggcctatgtcatttgttgttttatatgcatatattcaaaacgcatagcccatcctccttgagaccccctaaacatgttacgaatttgaagtgtctctgcattattcaagtgaggcaggaaaaagttactctaagtgatctttcttttttatattttatttgaatacaattctaataatttgacattaatgcagtaaagggttaacctagcagcctcaggttactccagccctgcacttttcaaagagaggtgtcttcacgtactggcccttccttgactagctcctgggaaatgacctgagctcgtggaatttccagtttgataatagtgttctagtatgcctgaggccttgggctgcattttgttagtttgacgagatagtttatgctaacagtatgaatcatggcgaatgtctgtttttgaatggctgaagccctgggccatgaggtatcactacacccctggggtcttgagactcaacgggtaaggtcagtcacatgggtgatgcatgcctatgtgactgacttccagtaaacaccttggacaccaaggattggttgagcttccttggttggcaatattttgcacatgctgtcacacatttctgggagaattaagcatgtccccatgtgactcaacaaggaagaggcaccaggaagcttgtgactgaactgatacagaaatagggtactgcaaataacaaagcctaatataacaaattgacttagggttggagagaagaatttagggagtggggacacaaataccacagactggaaaactggtgacttgtttggtggtgtattagggtcctctagagggacagaactaatagatgtatatatgaaggggagtttcttaggaaaattgactcacacaatcacaaggtgaagtcccacagtctgcaagctgagaagccaggaagccagtctgagtcccaaaacctcaaaagcagacaagcagatggtgcagcccttcagtctgtggctgaaggcctgatagtccctggcaaatcactggtggaagtccaagagtccaaaagctgaagaacttggagtctgatgttcaagggcagaagacatgcagcacaggagaaagacggaggccagaagacttagccagtgtagtccttccaccttcctctgcctgcttttatcctagctatgctggcagttgattagatggtgcacaaccagattgagggtggatctgcttcttgagcccactgactcaaatgttaatcttctttggcaataccctcacagacacacccaggaacaatattttgcatcatttaatccaatcaagttgacactcaatattaaccatcacaaacggcaaaaaaatatttggtctaactgtcaacagctgtctttggaaagaagaccaaatactgattgaggctgtagccttaggggaaatgctaggagaaaaactaaaaattttgcatgggatggctctttcttgctgtgttcagcaaggttctagaagaaaaaaatgtatttttttctcgattgaaattagctagcctgcagagttggaggaaaatatcatcttgttaacgaaagcagtttttgccatttttttctctttattataaaggttatatatgaacaagaatatataaaatatatatgtataaagagtattttaaaagtgaacatccatgcaatcaccacccaagacaagaaatagaacattgccagcatcccagaagcaccaggtgccactccccaatcacactgctgtacttctccacagaggaaatcattattctggttctggggacagcaaaacacttgcttttctttacagttgtatctcatatatataactatatacccttaaaacaatatagttgttcagtttatactgttttaaactttatacaaatggaatcatgttgatggcatccttctgtgatttgcttcttttgctctatgctatgtctgtgatattcatctatgttgtggttagctatttccttcattttcaccactgtgtagaattctactgtttcaatataaatgccatggtacaatttaaccattctaccattgctgaatatttggttcatttctaacttttggatattgcagtgctgctatgaacattaaaaaatttttttcttggccaccttcctgactgggaagaactttcttgtacatgcttcctaggatacatgttcattagttttcccaaggcattgtattagttagggtcctgacagggaaaaaaataactgtaatgaaagataacctgcaaagatgtatacttcagagtgcaattgctaggttttgagcatgtttatctttaaatttactgagggacaaatttttccacagtgattgttttcaatgtaagagctgacatcatcaccaaaacttagtatcattagatcatttcatttttgcaaataaggtaaagatgtaatacctccttgtagttttattttttacttctcaaatattaatatggctgggaatattttcatgtttcttggtcatctggatttcctttcacttgaaatgccatataaagtcttttgtccaaatttctattgactgtctttttcttactgattcatagggatcatttatatattctggacactagtttttcaccagttatatatattgcaaatacggtggttctttatattaggtttatattaggttcactaagtaggtgagattatgcatgcttattaccagttcttgtagttttgctgtattttcttcaaatgccccaaatcaaaattataataaaaagaaaatgggttggatataatagacaaaacaggtagtaaagaatgtgaagaaaattctgggcacagaaaacaaaagtgaaggcataagagggaggaagagtggaaaagtagaaaaccatctctattagatcaattaaagctttaaattttatttcaaatgattaaatattactaaatgataatattcaactacataaatccttaaatgaaaataatttagcatttattctaatattgaagataataaaaataaacctaaggcaagacagaaaataattcactatggtactatttacctttcagtacattaaatcagtgtttcattgaacttaaatttgtacataatttacataagtaaatcacaccatcaagaaccataatactacaactttgtatttgccatagtgtataataacatcagtcatgggattggattggcatgctagcaggcattaagcctaatttgaagaatctagtaattaaaagtctagttaccactttgtcaaagtctgtgagttcttaattaagctattcctaaaatattataatatacaaaatatatatttagatcataagctaaaatatgaaacgcaaggggagagaaaacaaaaatataaaagatttagctccttaaagaagtaacagaaaatggcttccaacttcatgttgcaattaaataataactattattatattattgagacagagtctcgctcttcaggctggagtacagtggcaagatcttggctgactgcagctttgacctcccaggttcaagtagttctcctgcctcagccatctgagtagctgggattacaggcgtgtgccaccaagcctggctaattttttttttttttttatcgttttagtagagacagggtctcaccatgttggcgaggctggtctcaaactcctgacctcaagtgatctgcccattcggcctcccaaagggctggcattacaggtgtgagccattgtgcctggcctaactaattattttttgagaagaactcattgatagcacaaaagtacttggagaaactacttaagctaactactattaagctgtcttctttcacaaatattaataaaagtactgatagaaatgtaactaagatacataatgtgttttaatacacattaatcttttgaattacacattttctcttgaggattataataaaatgatggtacaatttatccttctttatagatttgtggaaagtaccaacataattgacaagaaatgaaatactgccatttaaaagtcctgtattaaaataaaactactttgaatcatcttagactaaatattttaaaaactgattcaagtgcttattcataagataatggaattttaaataagaaaagccaaattaaaaattatattttaggcaaaaaccattttaacacagataatactgtgatatttattttcctgaagaaaaccacttatgctagttacattaatactcttcatagaacttaagataaattttaattatgaatgctcatgaagtatttaaagacactaggatcaatgccaacaaagtagttaagtgctgaaaaattcttatgataatataggcatgtgtgaatctttgagagcccttacaaatgtttttatattcagtataaaaataataaaaaaatcaccttcttatcccattcctaatttcccttttaagaattatctcttaacaggattgatttccaattgatgtataatggaagtaaaattctcatggttataaaaaagatacacagaatcagtatatgtatcttagaaaagcaaacatcatctgaggaaggattattgcacttgccttcactaaataaatctgcaaacttaaaatcagaaagaacaaattcattgattataaaataactagtttcaattaaaaattaatgataaaatgttcaatgtttacttaaaaaatatatcaagggtatgtttgggattgtttggttttattttctttgatgttgagtactttgtcatcaatcctggcctttttgttcttgttacagccttctgtactccacttgagctaccagtacttctggagctttctttgggttgattaactgggttaaatttatcctttcttaattcttggataaaacttttatttaagcaaacatccacatgcacattgaacagggttagatctgaagtcttttgttctacgttacaaacaggacaaactagagcttggcctgttttcacttcacataagtaaggctggcggtattcttgtctaaatgatccaacatcttcgttttccaatgaaacagtagaagaagaattctgatgacagtgttcaatattaaaagacttgcttgggagactagaacattcttccttgctatgcttattacttaaagcatctatgctttctgctttagatgagttatctatagtatctactaaagctatacaatctactgaagatatttctttaatttttggatgggcttcataatcttgcttctcacaaagtgaagaagcaggaacattttctttcttgttaactttggtagcagaaacatgtgaacacgagaacattttaaagttttcactgattgaaggtccatcaagacattcatctacatgtttattcaaggcttccagactgatgcacccttgagccctaaagcaaacaggacaggtaagtatctgacagtcatctgaattctctgatatttccaaattctcattcatcttcttctttaaaacttggaatggttgtgatgtctggaaactttgtttattcacggcttcacatttaaatgtatcttggtgactccatttcctttctgatcgttttttatcaaagaaactcttcttatgagacatttctagaggttttacaaacttatctttgtcagttttctctaatgtacactcagtggctgacagggcttggtttccagcctgtaaaaagccaataatgctcctttgttggtgtttcctgtcctcttcattgggaaaactagatatccgaacacccataagccttaatctcaagggatgtggaaaatcagcatcaatttctgtttttagcaattccttagcaatggcaaatatttcttctgcagtagaaacaacagatgaaactgtagatgcacgagtttttacttcaaaattcacattcttcaacttaatggtaacagttctacccttaagtctttctttctgtagatcctgagcaagctcactgcaaagttcttgacataggctgtattgctcttccgctttatttatctcactgaatgtcctctcaacgctcatacttttcctctctccatccctcgtcaggtgtgttgaacctagacccaaggagatatgaaggaaataatgccaagatgtttcagagaaaaggagagaaagcaatgccctctgttggtaaagttctgtacatgtaataattccaagggcctttaacattttctctgtaacttttcctattccagaaacctttctaatgggtaaatccttgatgaagtccatcacagcttgtctattgggaagaatttggtattgtccatttggtttattcttatcactgcatacttttgctaacattgtatttggggcaatgcctgcactggctgtcagtgttgttttctgctcaattctgaaacgaatttcctttaccacttcctgggctgatgttccaaaaacaactgagttttggagtatttgaggattgttttgttcttcaaagttcacttggaaaggatctcctgggggctgcacatcagaaggactctcttcaaaaagtagtggagagatggatcgttcatgctcactcagtttattaacttcctttcctggattatcattttctacagagcttcccattttgatgaaataccttcttttatcctcaggccaattttgtctttcttctaagtgctttgttatattcaagtaggcttcatcaagactcatggccataaaattgggatcataatcagcaagtatttccttaacctctttactcacagctcggtatttgtcaaagttggggggcactattataagttgtgggcacagcctcttagcaataaatcctggcatggctgcacgaacaccaaatctccttgcatggtaatttgaagtagacagcatactcattgatcctacagcaatgggtttatccttcaattctggattgtccctcatttctacagctgcatagaaagcatccatgtcaatgtgcactatggtattgctcaaatttcggctttgttctaattccattgcaaatctgtcaacctgtaattgtgcttttcttagctgttggctggtgatttgagctttttgttgcatcatattttcaattcgttggttgacttgcttttctttcttgagctcatttccataaaatctggacccccgttacctcaggatcgcgactacaactcccaggaggctgcgcgagcgacggaccaacgcccttcccagaatgcagcacagctgcatccctaccccgccctctcctttctccgctcctcctgcttttctacccgtcgtcacccgggagagccggaggtagggttc

SEQ ID NO: 18140 - RNA, 8643 nt, Homo sapiens
  source 1..8643: mol_type = other RNA
tgaaggtctactgtgtgccaggccatacacttcatacttggaattcagagataagtgaaagatagcccaggatctcttggggcctacaatctggtagggagaaaccaacatcgggggccatgcaaagaatgtttcagggtctttgtagggaaacaggagcaaaaaatagtgactgatcaatttttccagagggcaaggaacacttttctgaaggtggcccttgagctgagttgaaagatgagtaattatgtaggtgggagagagaaaaggggcattcaggaagcatattctgggcagagggaacaatggagcacagatgccagaaaggagaaacagcttggtctgttcaggaaaccctgaatgccaagccagtgtttagagtgcatcatggacagtgatatataggagctagcttgtattggcttgcaagagctgttaaagtttcaggaattttgtgaactggctgacatcacataacttgaaatctgtcatggtgggagcatttacaccacataaataatcatacactaaaaatcactcccttttcctactcattccactgctaaatcttggagacagttgagagcttttgaaaactgctttttttttttttttgacatgagagtgctattatgggaatgctgtttatagctaatctgtaaaaaatgcataagatggtttagagcagggaaaactgacaaatcagttggaaagtcaagagtttagacaactgataagggcttgacaaaagagatggaaacaaatggatattttcattttcaagaggccctacaagagtagacagaattcagtaacagatacagggttggcagaggtagcagtggatacaaggtggatgagttaaaaagtaaggagtagtaaacaaatacatttgttaatgatggcagaaaaaatatctcctattaattgctacatctctcttgcctttaacttacagccttcttacatatatgcctataaccactgtctacattttcttagcacaaagttccttcttaagttctgttatatggcttccattacccatgttgatgctgaaacttcttactctagaaggccacttcttcagtggggacactgaccttgcggataccacaagtcccatgctaactttaaaataaaacatttctggtggagtgaattaaatttataaatacttcttataatgctacttttcctactatcacaaaagattgaggaaaggtgtatagctctatattacagggacaatgtaaagactgatattaaaaaagagacctttgaattacattgaagagaggattatacacatgcaaagaaattattaggcctatgtcatttgttgttttatatgcatatattcaaaacgcatagcccatcctccttgagaccccctaaacatgttacgaatttgaagtgtctctgcattattcaagtgaggcaggaaaaagttactctaagtgatctttcttttttatattttatttgaatacaattctaataatttgacattaatgcagtaaagggttaacctagcagcctcaggttactccagccctgcacttttcaaagagaggtgtcttcacgtactggcccttccttgactagctcctgggaaatgacctgagctcgtggaatttccagtttgataatagtgttctagtatgcctgaggccttgggctgcattttgttagtttgacgagatagtttatgctaacagtatgaatcatggcgaatgtctgtttttgaatggctgaagccctgggccatgaggtatcactacacccctggggtcttgagactcaacgggtaaggtcagtcacatgggtgatgcatgcctatgtgactgacttccagtaaacaccttggacaccaaggattggttgagcttccttggttggcaatattttgcacatgctgtcacacatttctgggagaattaagcatgtccccatgtgactcaacaaggaagaggcaccaggaagcttgtgactgaactgatacagaaatagggtactgcaaataacaaagcctaatataacaaattgacttagggttggagagaagaatttagggagtggggacacaaataccacagactggaaaactggtgacttgtttggtggtgtattagggtcctctagagggacagaactaatagatgtatatatgaaggggagtttcttaggaaaattgactcacacaatcacaaggtgaagtcccacagtctgcaagctgagaagccaggaagccagtctgagtcccaaaacctcaaaagcagacaagcagatggtgcagcccttcagtctgtggctgaaggcctgatagtccctggcaaatcactggtggaagtccaagagtccaaaagctgaagaacttggagtctgatgttcaagggcagaagacatgcagcacaggagaaagacggaggccagaagacttagccagtgtagtccttccaccttcctctgcctgcttttatcctagctatgctggcagttgattagatggtgcacaaccagattgagggtggatctgcttcttgagcccactgactcaaatgttaatcttctttggcaataccctcacagacacacccaggaacaatattttgcatcatttaatccaatcaagttgacactcaatattaaccatcacaaacggcaaaaaaatatttggtctaactgtcaacagctgtctttggaaagaagaccaaatactgattgaggctgtagccttaggggaaatgctaggagaaaaactaaaaattttgcatgggatggctctttcttgctgtgttcagcaaggttctagaagaaaaaaatgtatttttttctcgattgaaattagctagcctgcagagttggaggaaaatatcatcttgttaacgaaagcagtttttgccatttttttctctttattataaaggttatatatgaacaagaatatataaaatatatatgtataaagagtattttaaaagtgaacatccatgcaatcaccacccaagacaagaaatagaacattgccagcatcccagaagcaccaggtgccactccccaatcacactgctgtacttctccacagaggaaatcattattctggttctggggacagcaaaacacttgcttttctttacagttgtatctcatatatataactatatacccttaaaacaatatagttgttcagtttatactgttttaaactttatacaaatggaatcatgttgatggcatccttctgtgatttgcttcttttgctctatgctatgtctgtgatattcatctatgttgtggttagctatttccttcattttcaccactgtgtagaattctactgtttcaatataaatgccatggtacaatttaaccattctaccattgctgaatatttggttcatttctaacttttggatattgcagtgctgctatgaacattaaaaaatttttttcttggccaccttcctgactgggaagaactttcttgtacatgcttcctaggatacatgttcattagttttcccaaggcattgtattagttagggtcctgacagggaaaaaaataactgtaatgaaagataacctgcaaagatgtatacttcagagtgcaattgctaggttttgagcatgtttatctttaaatttactgagggacaaatttttccacagtgattgttttcaatgtaagagctgacatcatcaccaaaacttagtatcattagatcatttcatttttgcaaataaggtaaagatgtaatacctccttgtagttttattttttacttctcaaatattaatatggctgggaatattttcatgtttcttggtcatctggatttcctttcacttgaaatgccatataaagtcttttgtccaaatttctattgactgtctttttcttactgattcatagggatcatttatatattctggacactagtttttcaccagttatatatattgcaaatacggtggttctttatattaggtttatattaggttcactaagtaggtgagattatgcatgcttattaccagttcttgtagttttgctgtattttcttcaaatgccccaaatcaaaattataataaaaagaaaatgggttggatataatagacaaaacaggtagtaaagaatgtgaagaaaattctgggcacagaaaacaaaagtgaaggcataagagggaggaagagtggaaaagtagaaaaccatctctattagatcaattaaagctttaaattttatttcaaatgattaaatattactaaatgataatattcaactacataaatccttaaatgaaaataatttagcatttattctaatattgaagataataaaaataaacctaaggcaagacagaaaataattcactatggtactatttacctttcagtacattaaatcagtgtttcattgaacttaaatttgtacataatttacataagtaaatcacaccatcaagaaccataatactacaactttgtatttgccatagtgtataataacatcagtcatgggattggattggcatgctagcaggcattaagcctaatttgaagaatctagtaattaaaagtctagttaccactttgtcaaagtctgtgagttcttaattaagctattcctaaaatattataatatacaaaatatatatttagatcataagctaaaatatgaaacgcaaggggagagaaaacaaaaatataaaagatttagctccttaaagaagtaacagaaaatggcttccaacttcatgttgcaattaaataataactattattatattattgagacagagtctcgctcttcaggctggagtacagtggcaagatcttggctgactgcagctttgacctcccaggttcaagtagttctcctgcctcagccatctgagtagctgggattacaggcgtgtgccaccaagcctggctaattttttttttttttttatcgttttagtagagacagggtctcaccatgttggcgaggctggtctcaaactcctgacctcaagtgatctgcccattcggcctcccaaagggctggcattacaggtgtgagccattgtgcctggcctaactaattattttttgagaagaactcattgatagcacaaaagtacttggagaaactacttaagctaactactattaagctgtcttctttcacaaatattaataaaagtactgatagaaatgtaactaagatacataatgtgttttaatacacattaatcttttgaattacacattttctcttgaggattataataaaatgatggtacaatttatccttctttatagatttgtggaaagtaccaacataattgacaagaaatgaaatactgccatttaaaagtcctgtattaaaataaaactactttgaatcatcttagactaaatattttaaaaactgattcaagtgcttattcataagataatggaattttaaataagaaaagccaaattaaaaattatattttaggcaaaaaccattttaacacagataatactgtgatatttattttcctgaagaaaaccacttatgctagttacattaatactcttcatagaacttaagataaattttaattatgaatgctcatgaagtatttaaagacactaggatcaatgccaacaaagtagttaagtgctgaaaaattcttatgataatataggcatgtgtgaatctttgagagcccttacaaatgtttttatattcagtataaaaataataaaaaaatcaccttcttatcccattcctaatttcccttttaagaattatctcttaacaggattgatttccaattgatgtataatggaagtaaaattctcatggttataaaaaagatacacagaatcagtatatgtatcttagaaaagcaaacatcatctgaggaaggattattgcacttgccttcactaaataaatctgcaaacttaaaatcagaaagaacaaattcattgattataaaataactagtttcaattaaaaattaatgataaaatgttcaatgtttacttaaaaaatatatcaagggtatgtttgggattgtttggttttattttctttgatgttgagtactttgtcatcaatcctggcctttttgttcttgttacagccttctgtactccacttgagctaccagtacttctggagctttctttgggttgattaactgggttaaatttatcctttcttaattcttggataaaacttttatttaagcaaacatccacatgcacattgaacagggttagatctgaagtcttttgttctacgttacaaacaggacaaactagagcttggcctgttttcacttcacataagtaaggctggcggtattcttgtctaaatgatccaacatcttcgttttccaatgaaacagtagaagaagaattctgatgacagtgttcaatattaaaagacttgcttgggagactagaacattcttccttgctatgcttattacttaaagcatctatgctttctgctttagatgagttatctatagtatctactaaagctatacaatctactgaagatatttctttaatttttggatgggcttcataatcttgcttctcacaaagtgaagaagcaggaacattttctttcttgttaactttggtagcagaaacatgtgaacacgagaacattttaaagttttcactgattgaaggtccatcaagacattcatctacatgtttattcaaggcttccagactgatgcacccttgagccctaaagcaaacaggacaggtaagtatctgacagtcatctgaattctctgatatttccaaattctcattcatcttcttctttaaaacttggaatggttgtgatgtctggaaactttgtttattcacggcttcacatttaaatgtatcttggtgactccatttcctttctgatcgttttttatcaaagaaactcttcttatgagacatttctagaggttttacaaacttatctttgtcagttttctctaatgtacactcagtggctgacagggcttggtttccagcctgtaaaaagccaataatgctcctttgttggtgtttcctgtcctcttcattgggaaaactagatatccgaacaccttaagtctttctttctgtagatcctgagcaagctcactgcaaagttcttgacataggctgtattgctcttccgctttatttatctcactgaatgtcctctcaacgctcatacttttcctctctccatccctcgtcaggtgtgttgaacctagacccaaggagatatgaaggaaataatgccaagatgtttcagagaaaaggagagaaagcaatgccctctgttggtaaagttctgtacatgtaataattccaagggcctttaacattttctctgtaacttttcctattccagaaacctttctaatgggtaaatccttgatgaagtccatcacagcttgtctattgggaagaatttggtattgtccatttggtttattcttatcactgcatacttttgctaacattgtatttggggcaatgcctgcactggctgtcagtgttgttttctgctcaattctgaaacgaatttcctttaccacttcctgggctgatgttccaaaaacaactgagttttggagtatttgaggattgttttgttcttcaaagttcacttggaaaggatctcctgggggctgcacatcagaaggactctcttcaaaaagtagtggagagatggatcgttcatgctcactcagtttattaacttcctttcctggattatcattttctacagagcttcccattttgatgaaataccttcttttatcctcaggccaattttgtctttcttctaagtgctttgttatattcaagtaggcttcatcaagactcatggccataaaattgggatcataatcagcaagtatttccttaacctctttactcacagctcggtatttgtcaaagttggggggcactattataagttgtgggcacagcctcttagcaataaatcctggcatggctgcacgaacaccaaatctccttgcatggtaatttgaagtagacagcatactcattgatcctacagcaatgggtttatccttcaattctggattgtccctcatttctacagctgcatagaaagcatccatgtcaatgtgcactatggtattgctcaaatttcggctttgttctaattccattgcaaatctgtcaacctgtaattgtgcttttcttagctgttggctggtgatttgagctttttgttgcatcatattttcaattcgttggttgacttgcttttctttcttgagctcatttccataaaatctggaccccttcgtggcttccattataattttgttaattttctctttatctaatccttccattcctgctttattatcattaagtcccatcctaagcagaagatcatctttgtaactgtcacacttctcctttgtgctatccatggtataaacttatccgttacctcaggatcgcgactacaactcccaggaggctgcgcgagcgacggaccaacgcccttcccagaatgcagcacagctgcatccctaccccgccctctcctttctccgctcctcctgcttttctacccgtcgtcacccgggagagccggaggtagggttc

SEQ ID NO: 18141 - RNA, 4982 nt, Homo sapiens
  source 1..4982: mol_type = other RNA
tgaaggtctactgtgtgccaggccccatgtcagctcttctaagtacattatttcagtctaaagtcatacaccctgtaagcagcagaaccatgattttagccacattgatctgatcccaaagcccacttttcctctcaagtctttcctctgtgttttgctaagccacatatttcaaaggacctatcacctataattacagcaataacaaagtgcgtcagtggctatgctttttcaagggctgagtatgaggctctgattcacttgtagccccaatgctgtggattggtcactcttggtactaagttcctttagctcaaataatggaaaagtaaactagagcctactccttttccagatgaccaaattcacaaatcagtggcatccaaattaatgccattttgttactaatatacttaaagcatacacatgctaaattaagcctcctaaaataatgcattgtgcttccctcaaatggcttcccgttgcccaaactccatattctgtcattcaaaccctcttcaaggtgagtctccaatctcccttccagttcagttttgcctcattcttccaggttatgtgacactgaatgagtaagaagcggtgggtgtgggaaagttggacaggaagtggaataatattgttggggcgaaggaacctacaggggaaagtcagttagtgagtcctgattctgttctctgcaactggttgtttggaagggtcttcttttcttcagaggttgtttcctggtattgagaaacagtttggggagatccttgttggggaaaatacactcatgggatagagttttgggactgagctaatcatgagctgcctacttgttatacctgaatttctggaataatctgtccagcttcgctttgcagaaggggtgaaaatccttcttaggtaactgggaagtaactcaccaggcccatgaagtggacactcctcagagcgtgccatgtttgtgtccattgacttatctaaaggttcacgagtctttggaacaggtggggaattttagggtacctgtgtgatatttgcttttataccccaaattgtataatatttacctctttaagtaatatatcctgccttggcaactgtattgtaagcctctggagggcaaggactggctattcttcgagtccctaacactttgcccagagtatagatttaaaacacgttggtcctgattgttatgatatcattggctccatttgctaccagcaacctcctccccatccttctttccttagtaaagaggcccacatgcataaagcactggaatgaattgtctgtcccaaagacagctacccacttgattgatggactgtttgctgaccttggaaaagaaatagaagacaaaaatgtctctgatttctactttctctgaagagtacgcaataattttttattatgttggaaggtgagattgccactcagcacaggctactgaattcactccctaccgggctggtgaaattcaagagattttggcaagggcagccatgccagctgtctgtttacctaaagagtcataatgactacaaaaccaggctggatttgtattctctcatcgctttaaagcaactggtaatggaaatgaactgacttagaaaacagacacctggaaatttcctccaaagactgtgcgggggatggtcactgccctcctctgctgtcttttacctgcagtcactgtggcctctatctctgggctccagcacatcctcttctgagccagtactcactaaagcagactgtgcatcctcagccccagctggcagcatccagattagctgaactgctgtaatctatgtttctggtattccagggtgagctcaggccatgccaatgttccctgggtcacagcttttctggagtgatcttgagtctatcagtctctatggttctgcttggcttccaaccttgtgctgcagatcctcacagactagaggcctgcccagaatcttgatccagttagtgggctatttctacacccttctaccaagtctgcaccccaggcaggggtctgctcctactggagctggtgcttttatgatgatatctttgactattgcccttcctgggaacgctggttatagtttcttacctggcagattttttcccctgttaaattatgctcaagctccttggatatgaagatagaattgctggccatccttttctgaagtctacctcccaaccaactcagagccccctgttctgattctacctccttctggctccttttctttcctgccagtaggtgccatcatggtaccagtatgacccttgattgggttcattcatttattcactcaaccatcattatttgctgagtaatgagtatgtgcagacattgtgccaggtgctgggttgtgacggtgaacaagatggtctgttttgcctcaagaaacataggggcgatactatgcctgagagacaaccgctctttccaatgtctgcgtttgctttatgacaactctctagttgtttccaaagctataaactacctctatatggcagccggaggcccgccttcctgtgaaacattggtagtcatgaagtgttgaaaataacccggatgttaagagggtctttcttcctgaaataatgaacaagtctgtggctctccaggcctttgcatgagaggaggaagtgaaggcacgacttggaatatggaaaagaggaatttggagacaaaattttggagtctttgtctggcaacatataagtgagaaggtccctaggcttgtcatcttgagctaaaattatttttttaggcaaattcctatctttatatcagaaagaggggccccaaagaaagtacatatagaatagaacaaaagaacatttaagaatcccaagattctgaatgcatgatagatttttttttgtggcaacagaaattttgcatgtggtaataatgtatcaactttatttgctttaattcatgtgtttaatttgtctaaatatttccctatgttactatttacttgattcatttattgaggaaaactcttcaaaagtagcaaagagtcagcctgccacccagtcttgtttgacttatcaccacatctgatttactggtgtttttcttcctagttatcttgtgggcaacatcttcaaagattttttccagcctgctcctaaaatacagtcttatcgtagagactcaaaaggagcatgcttcttaatcagggggagatagcctgtttataagccacgggacatgtacagtgaatctaatggggcagggcattagacttttacttggcaaggaaagttaggtcaataacctaatacacagctgtcattttttgaacagactattatgtacctcaagccccttatatacttaatctttactataaaaatgcgagacaggttctgaaacagactccaggtaaacctgtccaggatcaccctggaaagtcaaggggctgggatgtgaaataaagattttcgactcaatatcctgtattcttaattcctccattatcctgcagttatagagcagttgttttcgctttgatgtttcaggtctcagtttgttgaatttcaggtttcattcaaatggcatttctctaaacagtgatatgacatggatccgctcaaagttattgaaccttgttgctactgcagtcaggctgtttttcatataaatcaggagaaaaaaacaggggtcttcatttatttaatgttgaatttggaaccttgtgtctaactttaggtcattttcttttcttcaaagattgtgactttccaacccagcagccagtacaaagcaaatcctgatcagggttaacagggatgagcatcaactgggccgcactgccacatcttgggtgttcaagatcaagggtgtagagcgtacatcacagtgtgtggtggtgatgatgacagaactggagataaaagagaggccatcgttcatgctgacctggagtgcagctttcatgccaacttcttttaagataggcgctggacacagtaaataagtatcttccacagaaaagggcttctcattgagtgtgaccgagtcattgatcttgaagctgcagaggaccctgtccacgttgcgggcatgtcggaagccgtttcctctcacgacaacttgaaatgactctcctgcacatatggtggatggttcagctgctagaatttcgatgcaggacttcttcaaaattgagtggatgatgccttgcagagcctgaaagccgtcattcacgggaaacacatgatccttactgtccgcaatccgggccagctgtgtctcattgaaatctttcacaccaacacagtaaacaattgcaccaagatctcgagacctattagcctccctctctgaatagaaaaagagatcttcatggagttctccatcagtcaaagcaatgatgacgctggctgtcctgtacccttgtctgttttcataataaatctgctcactggccctttcaaatccttcatgcatgtaagtgtctcctcctggcagaactttctggagttcttctaggccttgacggatttgttctctgtcttctgtcagtttcattaaggttgttcctcgggtggagaaaacaataaaggacattctcaactgtgggctgatgaatttgtgagccaactgttccacaaagtaatagatttcattccagtggtgcagcacacttcctgatttgtccaaaatgaagtacaggtcaaatccgccgtagcaggctggacccccatcctccctgcgtcccccttgcccggcgcagatgagcaccagagtggccaaagagagccactggaagccgatgccgagggctctccgctccgccgtggccatggcccgcagcccggggagagcagggtccgctccttcccacgctccgcgaactcgccacgaccctcagggacgcgccatccgcgggcccttcctcgcgggtcctttattccccctcgctccctcgcaactccccggaagcaattgt

SEQ ID NO: 18142 - RNA, 35 nt, Homo sapiens
  source 1..35: mol_type = other RNA
tgaaggtctactgtgtgccaggccccgctgctcca

SEQ ID NO: 18143 - RNA, 176 nt, Homo sapiens
  source 1..176: mol_type = other RNA
tgaaggtctactgtgtgccaggccccgctgctccagggccctggggtggggcggggcgggggtgggtccctgccctggtggtggtgcctggagacagacagagacaaattcacaagctgaattcctggcaggtcagatggtggggacagttctgcagaaaaaccagccgggagaat

SEQ ID NO: 18144 - RNA, 2738 nt, Homo sapiens
  source 1..2738: mol_type = other RNA
tgaaggtctactgtgtgccaggccctagggtgggcactgagaacccagtggtgaaatgaacagatgtggcctgggccccacagatcctctccggccctttctggtcccaactccatccctaacaccaccccctgcaacatggccatcgaccctgtggccttggctctcccaggttcatctgtccccacacccccgcccatggggatgcccactgcctcaaaggctgccagcgagctctggggtggctgctgcagccaggcacgcactcggtggccagcccgcctggaccttggctgtacccagccagcagagacctcactgctgccactgccgcaaggctctccacaggctgcctctcagcatctcagagggcccacccacctctgcctgcctggccaccacgccagccacagagccatctgatttgaatgaaacttcaaacttaatgactttcatgctggttatttaaaacacaatgtaattttctaaaacaccctattatttcttttgatagctacaaagcttcccccagtcccataagcatgtttatttttagggaaaagagtggtttgcagttggtcatagagaccataaggagagggaacccacacagcagggcaaagagtcaaccctagcagctcagaggcctgtgctgccctgcctcctgcttagcgggttttccaccggacaccggggtctcccgggcaggccctgccctactctcacaaacatgttggcagtgactctcgtccagcattggacagtggccaagtaaacaccagactagcaccctcccagtgctccccctccttggggccactgtgtcctcttctgtaagatggttccactagctttccaataaggttcctaccagcattccaggcatgacaagcctggggaagggtcctgagaccaccacctcaccctcagcagcctcctcctggctctcccagacattctgccttgggtacagccacagggcctgaagctttcaccagctgagtgagacctgtgcccagataaattggctccaggcagtggctgcccacactgggagggtgagtgggtggggccctgccagtcggggctccctggcaagggaggtggcctggtggtgggtgggtgtgcgtgcagaggtcagctgagccccaccaatgcggggcgtcctctgggagcagctatttttaagtcccaggctttcatgtggccaaatgatgtggagtttacaaagcatcagtaatgcgtttcagatggcggcccagcaggccaggaggctgggcccgctgccaccagagccaggtcagagttagtcagaatccctcggcctagactcccatcacctgtccctccctccccatgaccccttcttgcctggtggggaggctggctctggagcaatgcttgcaaggagctgcccagcaaaccccggctgaggcccacccagcacacaggcctctccatggccagggattcctaccccatttaagaaactgagacctagagaggttcacagatttgcgtgaggtcacacagcagggggagggatggcttccttcccatcacagctccctgccctcatgggaaaactgggtttcctgggaggaggtgatttgccaccactggcacccaaaccagctcagacatggtggagtgggggcaggcctaaccgtgtaaacccccaaagtccacacccactgttccctggggccacgtcctgcccatccatgcctggagcctctgccgcacactcatcatttggaagcacatggtgtggggcccagacagctttcctgcccttgaagagcaagctagtggttttaatggggggcagggcgggggggttaggaggaagcttatttggcagagtgtctgctcctctgatctctagggagttctagctatggagttggggctgcggggtgagggctttgtgtccccaggcttgctccggctctagagtagtctgctagcagagcccaggcaggtgacctcctcccaggagaaggccagactcaggctcaccccaggccagagtccctatccagcaagggacagagaccctctactccctggggaactgggcaagaggagccccatgttccagcagaaagcaggggaagggggaaccctctgaggaggacaagcccacccaggctgtagacagcttgtgtgcagcagcagaagcaggccacacatttttaagggaggaaggcggtttcccaggtccagaccccaagcatgacaggtctgcgaaacaggacagcaaactgcctgaaccaagaagctgacaatgtcctggtttctcagagatgcccaccctccacccctgccaaagcccctgggaccctggagctctgctagagacagagctggtcagagatgctctccacaccctggctgagtcaccaatgggccttgggacctgagcgagccactgacctctggggtagagttcccctcagtaatcagggggccagaccctaggatcccgaaccccgagagagcatgagggtcaaatggaaggatgggaaaatggaaagttctcacctctgaggtacccctgccttgcactgcccaacacccttgggtcttctccacccaaagcctacctctcccttggctctgttcgagttcctcccatgatccccatgcctcctagcatccaccctgccccagcagctggctctccccgcctttgtccgccatgtccaattcacaccatctgtgggtgggtaccg

SEQ ID NO: 18145 - RNA, 2000 nt, Homo sapiens
  source 1..2000: mol_type = other RNA
tgaaggtctactgtgtgccaggccttgagcggcactaaggaggcccaggtgagagaggcagctccccgtcaggttccaggcccccggctcctgtcacaagccttctcacagtgggttccccgcacagactcggaacatggaatcgagtgcccaggcaggaggaagggccaggctggaggccacgtttctgcccatactttcagtcagttcagatagctttcctgtttccctctacctcctctgcccagcagtcaggcagttctcaagcaatactaatacagtcaatcaaagaagggtctcccaacctgttcctgtggtctctcaaggagctgggtcaagtttcatgcccactgacctagacccaaccaatgtcacctagtcagtccttctgtccctcatctcctcagccaccacactgtcagaatctacttcctaaattacagatttggtctcagtgctggaatctatgcattttggcaacctagaatttatagatcctctggtctgcaaatttaagtcaaaatgcttagcacagtactccaggataaggacctgccctccaccgaccttccagcttcatctcccttaaaccatacccaactacttcccactctgtgaactgcccatatttccatctccccaagtcatcacccacgctctcctctctgcctgaagggcttttcttctcccacctccaccccctaatcctactcagtcttccagctccaggacaaagtccacctgttctttggaactttctctaactctgcagttccaatgaatctttcttatctacattttcaaagcactttgtttatattacattcttgagtatgtttaccatatgataaattatatgtggaaaaagctttgcaaactgtatcctctataaaggtaaagtatcatttcttccacttattaacctttgatcctttccctttctgtatctccctccaagaacccatcaaagagtaggagctcaataaataataaataccagccatcaatcaaacgaaattcctcccacccacaaaagagaagcagagtcatcatatggtacacatatgcacaacactttcaccttcagaagtcctctgtgaaagaaagttaaacctttgtatagcatagctataggctggtttttgttcagttctaaggactgctgaaagtcttcatgggctgttgcatagtcctctgatatgaagtacagggttccccgatgtctgtacagccgtgctgagggctgcagttggatagctttagtgaggtcattcactgcttcattaattcgtcccagaggggacagaatttctgctcgctgctcaaatacctctggacgatctggttccaaggtaattactcggctcagttcgaacagagcaagctcagcattcttaatgtcatgtagtcccttctttccataggctatccctcggccataaattgcactaaccagatcaggctcctcctgaagcattgttgaaaaatgccgtattgcttcatcatacagaccactgccaatcaagacataagcaatagctaactcttcatttgtgctgtcattatcagtggcaaacgggaatctcttctgttctgcaatagacttggcctggctcagaatcttctcagtgttgagggaaagcaaggagtcacagggtgatgatcccttgggttcgcagtctgagtcatggaagttcaaaaaggatgactcgccgcactcggcagagtactggtccccccagtccccggactgcgggctgcagccgccgccgcccgccggggcctcctgctgctgccggtgctgcagctcctgcttgagcagggagagcggcgagtagtgctcggtggccagggcgcctggccgcagcccggcggacaggacccccagcagcagcagcagcaggacacgccgggcggcgcccgcggcggccacagcgccgccccagaagcagcagcagcagcagcagccggcaggtgccatcttccctcaaggcgcatgc

SEQ ID NO: 18146 - RNA, 1784 nt, Homo sapiens
  source 1..1784: mol_type = other RNA
tgaaggtctactgtgtgccaggctctgggtgaagtgctgaggactcgaagatgacttaggttcaaggctttgccctttcatcaaaggaatccaggcaccgaagggtatgccctgtgtgacaccctttaaaatgctcacaaccaggtgcacaggtctccatttgcaggggcgtcaagctgggctgcagctgctttcccctgcttggtcccaggttggagttggtgggaagaggaaagtgagagggatctggaagttggaagtggagcagctgccacgacccccgaaagtccttgtggctgtcctgagaggggaggaagcttccgctcttctggcctcccggatccgccagggctcctgctgctcccacttccgccacccaggagggccaggccgccgtcttgagtttccctccagcctggcctagggacgactcttcttcagtgccgccttctccaccgagtcctcgcatattaagattccagaaggttctgatctcctggtgcttcagtgtaaacgagtgtgtttggggatagctggcctgtggggatccactcattctttcacagatatccaggactgggttagggagcctggtggtggcaggaggccgccctccagctcgctggctgccgtgtggaagtcctttctcctcggattctgatctagggacggcccacaagctcctggcgaggatgaactgagttcagtgatgtcaagctcggcacagtgcctgtccacaatgagcccaataatttttagctattgtcacgtcgacggtaccacccacctggatgccactcacctggacaccattcacctgggtgatgcccctcacctggacaccactcacctgggtgccaccacctggacaccacttacctggatgccactcacctggacaccattcacctgggtgatgccactcacctggacaccattcacctggctgtcactcacctgggcaccactcgcctgggtgccaccacctggaccccacttacctggatgtgactcacttgggcaccactcaactgggtgccactcacctgggtgttatgcacctggacaatgctagtcacgtggatgccactcgcctgggtgtcactcacctgaatgctactcacctgggtgccatttacctggatgatgtcactcacctggatgtcgtcactcacctggatgtcacctaggtgccacttacctggatgatatcactcacctggatgccactcacccaggtgtcacctggataatgccactcacccgaatgccactcacctgggtgccactcacctggaagctactcacctggatgatgccactcacacagacgccactaacctgaatgtcactcacctaggtgtcactcacctggatgctactcacctgggtgccactcaactgggatgtcactcacctgggtgccacccacctgaacaccactcacctgggtgtgtgagaacagtggaagttcctggaacatagttggcattcatccttcccaatgcttgctctcatacacagccagcccttacatggttatttcttcatgtcatctgccacctctgggcagccaggctcccccagactcaagccctcagactctgccaagaactgtccggccccagggcctttgcaagcgcaggtcgcacggcctgggatgccctctcccagctcaccacatggctggctctttcccattcattggcctcagcccagtggcctccttctcgtcagagaggccgcccctgcctgccctggctggccggcccctcccccacaat

SEQ ID NO: 18147 - RNA, 3646 nt, Homo sapiens
  source 1..3646: mol_type = other RNA
tgaaggtctactgtgtgccaggtactgttctaggcgtttcagagtcatccatggaagaaaaaggccataaatccttgccctcgtggagcttaccttctaataaggagagacagagggtgagaaacaaacaaacaaaaatatgtgagttaacacagagtgttggagggtgtcaggtgctatgggagaaacgtggagcatgtcaaggagagagcaggcaagagggcattctggaaaggcctaggaagatggtgacatttgaccttcatatccaccaacccccagcacaaagcatttgccagaggcagacagaggagggcaatggacagtaggcgtccatgcacccaagtgagggagagagacatgcagacactctagagaagagtgtccaggcaggggaacggccctgttcgttcatcatttcatcctcatgagatatgttacgtgttatccccattcgaaagatggtgaagctgagactcaagagaggttaaagtcacatgagagggtcacagagctagcaagggacagcacttactggttgcaagtccatgctaaatataagaccttgtcatgacccagggcttggtgccccttatagtgaagatcagaagaggaatggatcgtcatcttcctctgcttgctaccctcgctggtttcaagacctaccctcagctctgcctccaggaatctagcaccgactgtgtctcacgtggccttgcctcatgccctccaagggatgcagcactaaaaaaatgttggtagagtgtcttctcttgccaggcagtggtcaagatggcagggattcagcgggaaacatgctcccagtcctcctggagttggttagtgccctgcttccatttgtttcctgagcaccctttggtgttaagtcctagccactggggagagggagggcacaggaatgaggaatgcagagtttctacattcaaagggcttcccaaggagagagaaaggtgctctctgcacacacagctcagccacagggaactctagaacagagagatatttgttttaaatagtgtatctaggaagtcttactggaggaagtggcatctgcattgagcgctctaaggataggaagaatttggcaggagttgaggtgtgcacctacctggtcttggaggaggcatcttgaggagggatgtcaaactccaatttgtctcacaggaaactgaagcaaaggctatgttgagggtaggaaaagttggcactttttattcctcccttcttttatatttttcccccttcccaagtgcctactacgcaccaggagctatacgaggcaccagggaagcaacaatgaacaaggctgtagggatccctctgggaaaccacagactgatgggatttcagtgcagctgagttggagaagagagacagagagggagacttaaatagcagaacgaggggtttgtgtttgctccttcagcaatggggagccacggagggttttgagcagggaaatgacatgatctgaactggacaagtaataattatttgggcagcacgcaaggatgggtttgaaggggaccagaggcaaggaagccagctcgcatcaaaagataacccttaagtacatctgcctttgttggggcgctctggtttcccgtgcccctttgtggtggggaggtgagggatggagcatcaggggagggagaacaggctgcaggtctgagaagggatgaagggtttccatggcaaccttttgcttgcctgtagccaaggtagctatgcaaattccccaggcaccattcctgtggaccttgaagccagcatccccggctgctgagagcctgactttagaaaaactgggatgcagtaaaattgaacaagagagacgagagacaaagatgttcggctggaacaggggtgcaggctcccaggcagcccttgaattcccttgaacctgttctgcaggctccttctccctcctctagggagggactctcccaagcccacccttccccatttggcatgcattttacaccatggggacttgggccacctggaaaatgggctgacctgatggtggtgcctcctttaagtttttgtgatgacttgcaatattgtttgccaagcttcgtacacaatgcctgggtcagggtaagcaggtcaaaatgctagcagttattgttatttggcattgtgattaaagaatgctggctcttagaacaccaggtcctcctctgagagtggccgctgattgatgtgtgaccttgagaaagtcacttcccttctctttaatcttcctgttcttatgtgtcagatggggatgctggctctacagtctctttattagcattttattgttgttgttgttgctgctactgctgctattgtcaccattattattagtattgctgttttatcattgctattattataacacctatgttgctgctacctgctacaaagggcaatgatgatgattcctgtaaatactccacgtagttagaacgtgaaactctatgccaaagcagaccatgcaaaaatgagttttcgagaaattgttacatgaagagtttataaaaatgaaatgctgtattctacacatatcaagacaggattgcttgtgggtgttgaaacttattaggcgaggtagtccttagacattcacttgtcttagtcttaataattgaccaaatctcctctccttgagttctcacactgggtctgggttccatgtccgtttccattctaggtgatcctaaattcaattgagaatcctgagttcagacccttgtaagacacagcctctcctgttgtagaaagacaccttcctttacctaacacagatttagtccacatcgtattactaaccctaaccctaacccaacctgagtatttggcatgtaatagacactcacatttgttgaaaggaagaaaagaaagaattagaaggaagaaaatggggcacactgctttctaatcccaagaccctctagttattaatctagagaggaaggtagaagccaactctctcatattcgtctcagtggaaaagccatttttcccctctaactccagactttctgtcttctttttttactcaccaatgcccaaaggaaaaaaaaaaggtatttccaagtacgaaagtacaaagtttcaaacccactcgtgctcctccttacaatgcagtcgattaatcccacaacatttctcctgggtggttgccgttaattgaattaaatgagataatatttgttgagtacgtagcactgcgcctggaaatgtttattgcatagaattgaatcaaggatgaaacacaagtggaaaactcatgggaaatgttcatccttcgtagaggtcaagtgaatgcacctgcaactacccttgagggaccacattacaccaactaaattagcttagaatgtttaaaccaataacacttggtgttggcaaggttattagaacattggtaagctcaggggctttgtgatttgaaagaccccttaggaaagcaacacggcaattctgtccagctagagcggtaaaactgttcatgccctttgaccaaaggatttcattccagggaatttctgcttgaagatggattcaactgtagcaaaagttgtatacacaaagatgctcattaactacagctagcactgaaaaagaaaaaggaaga

SEQ ID NO: 18148 - RNA, 3883 nt, Homo sapiens
  source 1..3883: mol_type = other RNA
tgaaggtctactgtgtgccaggtactgttctaggcgtttcagagtcatccatggaagaaaaaggccataaatccttgccctcgtggagcttaccttctaataaggagagacagagggtgagaaacaaacaaacaaaaatatgtgagttaacacagagtgttggagggtgtcaggtgctatgggagaaacgtggagcatgtcaaggagagagcaggcaagagggcattctggaaaggcctaggaagatggtgacatttgaccttcatatccaccaacccccagcacaaagcatttgccagaggcagacagaggagggcaatggacagtaggcgtccatgcacccaagtgagggagagagacatgcagacactctagagaagagtgtccaggcaggggaacggccctgttcgttcatcatttcatcctcatgagatatgttacgtgttatccccattcgaaagatggtgaagctgagactcaagagaggttaaagtcacatgagagggtcacagagctagcaagggacagcacttactggttgcaagtccatgctaaatataagaccttgtcatgacccagggcttggtgccccttatagtgaagatcagaagaggaatggatcgtcatcttcctctgcttgctaccctcgctggtttcaagacctaccctcagctctgcctccaggaatctagcaccgactgtgtctcacgtggccttgcctcatgccctccaagggatgcagcactggacagaggcaaaagaaagggaaatgtcaccttcttcttctgggcttggctcctccgtcttggaaagcgagtctcagaacatctgttaaaccaagccccagcatattaaacagccactgaaaatgtattgttgcttcgttcaatacatagcaattacacggcgagttttgctcattagcgggaaattgacacagaggcaatcctgctttttaaattaccactaatctcactgcacctaaaaaaatgttggtagagtgtcttctcttgccaggcagtggtcaagatggcagggattcagcgggaaacatgctcccagtcctcctggagttggttagtgccctgcttccatttgtttcctgagcaccctttggtgttaagtcctagccactggggagagggagggcacaggaatgaggaatgcagagtttctacattcaaagggcttcccaaggagagagaaaggtgctctctgcacacacagctcagccacagggaactctagaacagagagatatttgttttaaatagtgtatctaggaagtcttactggaggaagtggcatctgcattgagcgctctaaggataggaagaatttggcaggagttgaggtgtgcacctacctggtcttggaggaggcatcttgaggagggatgtcaaactccaatttgtctcacaggaaactgaagcaaaggctatgttgagggtaggaaaagttggcactttttattcctcccttcttttatatttttcccccttcccaagtgcctactacgcaccaggagctatacgaggcaccagggaagcaacaatgaacaaggctgtagggatccctctgggaaaccacagactgatgggatttcagtgcagctgagttggagaagagagacagagagggagacttaaatagcagaacgaggggtttgtgtttgctccttcagcaatggggagccacggagggttttgagcagggaaatgacatgatctgaactggacaagtaataattatttgggcagcacgcaaggatgggtttgaaggggaccagaggcaaggaagccagctcgcatcaaaagataacccttaagtacatctgcctttgttggggcgctctggtttcccgtgcccctttgtggtggggaggtgagggatggagcatcaggggagggagaacaggctgcaggtctgagaagggatgaagggtttccatggcaaccttttgcttgcctgtagccaaggtagctatgcaaattccccaggcaccattcctgtggaccttgaagccagcatccccggctgctgagagcctgactttagaaaaactgggatgcagtaaaattgaacaagagagacgagagacaaagatgttcggctggaacaggggtgcaggctcccaggcagcccttgaattcccttgaacctgttctgcaggctccttctccctcctctagggagggactctcccaagcccacccttccccatttggcatgcattttacaccatggggacttgggccacctggaaaatgggctgacctgatggtggtgcctcctttaagtttttgtgatgacttgcaatattgtttgccaagcttcgtacacaatgcctgggtcagggtaagcaggtcaaaatgctagcagttattgttatttggcattgtgattaaagaatgctggctcttagaacaccaggtcctcctctgagagtggccgctgattgatgtgtgaccttgagaaagtcacttcccttctctttaatcttcctgttcttatgtgtcagatggggatgctggctctacagtctctttattagcattttattgttgttgttgttgctgctactgctgctattgtcaccattattattagtattgctgttttatcattgctattattataacacctatgttgctgctacctgctacaaagggcaatgatgatgattcctgtaaatactccacgtagttagaacgtgaaactctatgccaaagcagaccatgcaaaaatgagttttcgagaaattgttacatgaagagtttataaaaatgaaatgctgtattctacacatatcaagacaggattgcttgtgggtgttgaaacttattaggcgaggtagtccttagacattcacttgtcttagtcttaataattgaccaaatctcctctccttgagttctcacactgggtctgggttccatgtccgtttccattctaggtgatcctaaattcaattgagaatcctgagttcagacccttgtaagacacagcctctcctgttgtagaaagacaccttcctttacctaacacagatttagtccacatcgtattactaaccctaaccctaacccaacctgagtatttggcatgtaatagacactcacatttgttgaaaggaagaaaagaaagaattagaaggaagaaaatggggcacactgctttctaatcccaagaccctctagttattaatctagagaggaaggtagaagccaactctctcatattcgtctcagtggaaaagccatttttcccctctaactccagactttctgtcttctttttttactcaccaatgcccaaaggaaaaaaaaaaggtatttccaagtacgaaagtacaaagtttcaaacccactcgtgctcctccttacaatgcagtcgattaatcccacaacatttctcctgggtggttgccgttaattgaattaaatgagataatatttgttgagtacgtagcactgcgcctggaaatgtttattgcatagaattgaatcaaggatgaaacacaagtggaaaactcatgggaaatgttcatccttcgtagaggtcaagtgaatgcacctgcaactacccttgagggaccacattacaccaactaaattagcttagaatgtttaaaccaataacacttggtgttggcaaggttattagaacattggtaagctcaggggctttgtgatttgaaagaccccttaggaaagcaacacggcaattctgtccagctagagcggtaaaactgttcatgccctttgaccaaaggatttcattccagggaatttctgcttgaagatggattcaactgtagcaaaagttgtatacacaaagatgctcattaactacagctagcactgaaaaagaaaaaggaaga

SEQ ID NO: 18149 - RNA, 2722 nt, Homo sapiens
  source 1..2722: mol_type = other RNA
tgaaggtctactgtgtgccaggtactgttctaggcgtttcagagtcatccatggaagaaaaaggccataaatccttgccctcgtggagcttaccttctaataaggagagacagagggtgagaaacaaacaaacaaaaatatgtgagttaacacagagtgttggagggtgtcaggtgctatgggagaaacgtggagcatgtcaaggagagagcaggcaagagggcattctggaaaggcctaggaagatggtgacatttgaccttcatatccaccaacccccagcacaaagcatttgccagaggcagacagaggagggcaatggacagtaggcgtccatgcacccaagtgagggagagagacatgcagacactctagagaagagtgtccaggcaggggaacggccctgttcgttcatcatttcatcctcatgagatatgttacgtgttatccccattcgaaagatggtgaagctgagactcaagagaggttaaagtcacatgagagggtcacagagctagcaagggacagcacttactggttgcaagtccatgctaaatataagaccttgtcatgacccagggcttggtgccccttatagtgaagatcagaagaggaatggatcgtcatcttcctctgcttgctaccctcgctggtttcaagacctaccctcagctctgcctccaggaatctagcaccgactgtgtctcacgtggccttgcctcatgccctccaagggatgcagcactggacagaggcaaaagaaagggaaatgtcaccttcttcttctgggcttggctcctccgtcttggaaagcgagtctcagaacatctgttaaaccaagccccagcatattaaacagccactgaaaatgtattgttgcttcgttcaatacatagcaattacacggcgagttttgctcattagcgggaaattgacacagaggcaatcctgctttttaaattaccactaatctcactgcacctgtttgggaagaaggcaggaggagaaaggaaaaaagttgataataaccatttcattacattttaaaaacaaacacttctaaaattcccttaaatatagcttttgggctctcagattcccatcttatcttaggaggagcctctttgcctcatgccacaggctggagtaactctccattaatgtcacaggcttaatggcacatgagtctgggcaccaaggacaccgggaggacaagctaggctcccttaaggtttatttaaagtgagattctgtgattaactatggttaagggacttggtgcacattgaggagagccaccatacctcagaggctcatggaaaactgacttattcagtgggtgggcaggtgttaggggaggtggatgcagatgccgctacaggtgtctccagagctcaaagacaaggtgtcacttgaccaaatcaaacagctgtcagtgaagctggcattcagacttgctgcccaggcaggttgctgaaatcatggagccccaattccccatttctgtctcagtgcacggggttgcatgccatgcccagcacagaggctgacttcacacagtaggcactcaataaatgcttcctaacacaacctcggggctgcttcctgagatgctccttcactgatatcctccagtccatggggccaggctcattctgtatgaggcacactgccctgggctcaagcccctccctggctgggtgatcttggacaaacctctctacctctctgagtcttggcttccttatttggaaaatcgggataatgatagtaagtccagctcaagctcgtggcttgctggcttgttggtgagggtcttgtgtgatcatagggctgaaagtgcttgagaaactggaaaagtggtttaagaaccacgactattgatacccgtggaaatggagagagaaaaaagaaaaataaaagcaatgtaaaaaagaacaattattattattctggagttggttgctccttggaagaggagatgctggggcctcggattaacatgaaacttaccagaacttaacatagcactgtacacatagtggttcttgatgaagacttgaaaaatgaattcttttatttacctaaaaaaatgttggtagagtgtcttctcttgccaggcagtggtcaagatggcagggattcagcgggaaacatgctcccagtcctcctggagttggttagtgccctgcttccatttgtttcctgagcaccctttggtgttaagtcctagccactggggagagggagggcacaggaatgaggaatgcagagtttctacattcaaagggcttcccaaggagagagaaaggtgctctctgcacacacagctcagccacagggaactcaaggatgaaacacaagtggaaaactcatgggaaatgttcatccttcgtagaggtcaagtgaatgcacctgcaactacccttgagggaccacattacaccaactaaattagcttagaatgtttaaaccaataacacttggtgttggcaaggttattagaacattggtaagctcaggggctttgtgatttgaaagaccccttaggaaagcaacacggcaattctgtccagctagagcggtaaaactgttcatgccctttgaccaaaggatttcattccagggaatttctgcttgaagatggattcaactgtagcaaaagttgtatacacaaagatgctcattaactacagctagcactgaaaaagaaaaaggaaga

SEQ ID NO: 18150 - RNA, 4986 nt, Homo sapiens
  source 1..4986: mol_type = other RNA
tgaaggtctactgtgtgccaggtactgttctaggcgtttcagagtcatccatggaagaaaaaggccataaatccttgccctcgtggagcttaccttctaataaggagagacagagggtgagaaacaaacaaacaaaaatatgtgagttaacacagagtgttggagggtgtcaggtgctatgggagaaacgtggagcatgtcaaggagagagcaggcaagagggcattctggaaaggcctaggaagatggtgacatttgaccttcatatccaccaacccccagcacaaagcatttgccagaggcagacagaggagggcaatggacagtaggcgtccatgcacccaagtgagggagagagacatgcagacactctagagaagagtgtccaggcaggggaacggccctgttcgttcatcatttcatcctcatgagatatgttacgtgttatccccattcgaaagatggtgaagctgagactcaagagaggttaaagtcacatgagagggtcacagagctagcaagggacagcacttactggttgcaagtccatgctaaatataagaccttgtcatgacccagggcttggtgccccttatagtgaagatcagaagaggaatggatcgtcatcttcctctgcttgctaccctcgctggtttcaagacctaccctcagctctgcctccaggaatctagcaccgactgtgtctcacgtggccttgcctcatgccctccaagggatgcagcactggacagaggcaaaagaaagggaaatgtcaccttcttcttctgggcttggctcctccgtcttggaaagcgagtctcagaacatctgttaaaccaagccccagcatattaaacagccactgaaaatgtattgttgcttcgttcaatacatagcaattacacggcgagttttgctcattagcgggaaattgacacagaggcaatcctgctttttaaattaccactaatctcactgcacctgtttgggaagaaggcaggaggagaaaggaaaaaagttgataataaccatttcattacattttaaaaacaaacacttctaaaattcccttaaatatagcttttgggctctcagattcccatcttatcttaggaggagcctctttgcctcatgccacaggctggagtaactctccattaatgtcacaggcttaatggcacatgagtctgggcaccaaggacaccgggaggacaagctaggctcccttaaggtttatttaaagtgagattctgtgattaactatggttaagggacttggtgcacattgaggagagccaccatacctcagaggctcatggaaaactgacttattcagtgggtgggcaggtgttaggggaggtggatgcagatgccgctacaggtgtctccagagctcaaagacaaggtgtcacttgaccaaatcaaacagctgtcagtgaagctggcattcagacttgctgcccaggcaggttgctgaaatcatggagccccaattccccatttctgtctcagtgcacggggttgcatgccatgcccagcacagaggctgacttcacacagtaggcactcaataaatgcttcctaacacaacctcggggctgcttcctgagatgctccttcactgatatcctccagtccatggggccaggctcattctgtatgaggcacactgccctgggctcaagcccctccctggctgggtgatcttggacaaacctctctacctctctgagtcttggcttccttatttggaaaatcgggataatgatagtaagtccagctcaagctcgtggcttgctggcttgttggtgagggtcttgtgtgatcatagggctgaaagtgcttgagaaactggaaaagtggtttaagaaccacgactattgatacccgtggaaatggagagagaaaaaagaaaaataaaagcaatgtaaaaaagaacaattattattattctggagttggttgctccttggaagaggagatgctggggcctcggattaacatgaaacttaccagaacttaacatagcactgtacacatagtggttcttgatgaagacttgaaaaatgaattcttttatttacctaaaaaaatgttggtagagtgtcttctcttgccaggcagtggtcaagatggcagggattcagcgggaaacatgctcccagtcctcctggagttggttagtgccctgcttccatttgtttcctgagcaccctttggtgttaagtcctagccactggggagagggagggcacaggaatgaggaatgcagagtttctacattcaaagggcttcccaaggagagagaaaggtgctctctgcacacacagctcagccacagggaactctagaacagagagatatttgttttaaatagtgtatctaggaagtcttactggaggaagtggcatctgcattgagcgctctaaggataggaagaatttggcaggagttgaggtgtgcacctacctggtcttggaggaggcatcttgaggagggatgtcaaactccaatttgtctcacaggaaactgaagcaaaggctatgttgagggtaggaaaagttggcactttttattcctcccttcttttatatttttcccccttcccaagtgcctactacgcaccaggagctatacgaggcaccagggaagcaacaatgaacaaggctgtagggatccctctgggaaaccacagactgatgggatttcagtgcagctgagttggagaagagagacagagagggagacttaaatagcagaacgaggggtttgtgtttgctccttcagcaatggggagccacggagggttttgagcagggaaatgacatgatctgaactggacaagtaataattatttgggcagcacgcaaggatgggtttgaaggggaccagaggcaaggaagccagctcgcatcaaaagataacccttaagtacatctgcctttgttggggcgctctggtttcccgtgcccctttgtggtggggaggtgagggatggagcatcaggggagggagaacaggctgcaggtctgagaagggatgaagggtttccatggcaaccttttgcttgcctgtagccaaggtagctatgcaaattccccaggcaccattcctgtggaccttgaagccagcatccccggctgctgagagcctgactttagaaaaactgggatgcagtaaaattgaacaagagagacgagagacaaagatgttcggctggaacaggggtgcaggctcccaggcagcccttgaattcccttgaacctgttctgcaggctccttctccctcctctagggagggactctcccaagcccacccttccccatttggcatgcattttacaccatggggacttgggccacctggaaaatgggctgacctgatggtggtgcctcctttaagtttttgtgatgacttgcaatattgtttgccaagcttcgtacacaatgcctgggtcagggtaagcaggtcaaaatgctagcagttattgttatttggcattgtgattaaagaatgctggctcttagaacaccaggtcctcctctgagagtggccgctgattgatgtgtgaccttgagaaagtcacttcccttctctttaatcttcctgttcttatgtgtcagatggggatgctggctctacagtctctttattagcattttattgttgttgttgttgctgctactgctgctattgtcaccattattattagtattgctgttttatcattgctattattataacacctatgttgctgctacctgctacaaagggcaatgatgatgattcctgtaaatactccacgtagttagaacgtgaaactctatgccaaagcagaccatgcaaaaatgagttttcgagaaattgttacatgaagagtttataaaaatgaaatgctgtattctacacatatcaagacaggattgcttgtgggtgttgaaacttattaggcgaggtagtccttagacattcacttgtcttagtcttaataattgaccaaatctcctctccttgagttctcacactgggtctgggttccatgtccgtttccattctaggtgatcctaaattcaattgagaatcctgagttcagacccttgtaagacacagcctctcctgttgtagaaagacaccttcctttacctaacacagatttagtccacatcgtattactaaccctaaccctaacccaacctgagtatttggcatgtaatagacactcacatttgttgaaaggaagaaaagaaagaattagaaggaagaaaatggggcacactgctttctaatcccaagaccctctagttattaatctagagaggaaggtagaagccaactctctcatattcgtctcagtggaaaagccatttttcccctctaactccagactttctgtcttctttttttactcaccaatgcccaaaggaaaaaaaaaaggtatttccaagtacgaaagtacaaagtttcaaacccactcgtgctcctccttacaatgcagtcgattaatcccacaacatttctcctgggtggttgccgttaattgaattaaatgagataatatttgttgagtacgtagcactgcgcctggaaatgtttattgcatagaattgaatcaaggatgaaacacaagtggaaaactcatgggaaatgttcatccttcgtagaggtcaagtgaatgcacctgcaactacccttgagggaccacattacaccaactaaattagcttagaatgtttaaaccaataacacttggtgttggcaaggttattagaacattggtaagctcaggggctttgtgatttgaaagaccccttaggaaagcaacacggcaattctgtccagctagagcggtaaaactgttcatgccctttgaccaaaggatttcattccagggaatttctgcttgaagatggattcaactgtagcaaaagttgtatacacaaagatgctcattaactacagctagcactgaaaaagaaaaaggaaga

SEQ ID NO: 18151 - RNA, 2794 nt, Homo sapiens
  source 1..2794: mol_type = other RNA
tgaaggtctactgtgtgccaggtactgttctaggcgtttcagagtcatccatggaagaaaaaggccataaatccttgccctcgtggagcttaccttctaataaggagagacagagggtgagaaacaaacaaacaaaaatatgtgagttaacacagagtgttggagggtgtcaggtgctatgggagaaacgtggagcatgtcaaggagagagcaggcaagagggcattctggaaaggcctaggaagatggtgacatttgaccttcatatccaccaacccccagcacaaagcatttgccagaggcagacagaggagggcaatggacagtaggcgtccatgcacccaagtgagggagagagacatgcagacactctagagaagagtgtccaggcaggggaacggccctgttcgttcatcatttcatcctcatgagatatgttacgtgttatccccattcgaaagatggtgaagctgagactcaagagaggttaaagtcacatgagagggtcacagagctagcaagggacagcacttactggttgcaagtccatgctaaatataagaccttgtcatgacccagggcttggtgccccttatagtgaagatcagaagaggaatggatcgtcatcttcctctgcttgctaccctcgctggtttcaagacctaccctcagctctgcctccaggaatctagcaccgactgtgtctcacgtggccttgcctcatgccctccaagggatgcagcactggacagaggcaaaagaaagggaaatgtcaccttcttcttctgggcttggctcctccgtcttggaaagcgagtctcagaacatctgttaaaccaagccccagcatattaaacagccactgaaaatgtattgttgcttcgttcaatacatagcaattacacggcgagttttgctcattagcgggaaattgacacagaggcaatcctgctttttaaattaccactaatctcactgcacctgtttgggaagaaggcaggaggagaaaggaaaaaagttgataataaccatttcattacattttaaaaacaaacacttctaaaattcccttaaatatagcttttgggctctcagattcccatcttatcttaggaggagcctctttgcctcatgccacaggctggagtaactctccattaatgtcacaggcttaatggcacatgagtctgggcaccaaggacaccgggaggacaagctaggctcccttaaggtttatttaaagtgagattctgtgattaactatggttaagggacttggtgcacattgaggagagccaccatacctcagaggctcatggaaaactgacttattcagtgggtgggcaggtgttaggggaggtggatgcagatgccgctacaggtgtctccagagctcaaagacaaggtgtcacttgaccaaatcaaacagctgtcagtgaagctggcattcagacttgctgcccaggcaggttgctgaaatcatggagccccaattccccatttctgtctcagtgcacggggttgcatgccatgcccagcacagaggctgacttcacacagtaggcactcaataaatgcttcctaacacaacctcggggctgcttcctgagatgctccttcactgatatcctccagtccatggggccaggctcattctgtatgaggcacactgccctgggctcaagcccctccctggctgggtgatcttggacaaacctctctacctctctgagtcttggcttccttatttggaaaatcgggataatgatagtaagtccagctcaagctcgtggcttgctggcttgttggtgagggtcttgtgtgatcatagggctgaaagtgcttgagaaactggaaaagtggtttaagaaccacgactattgatacccgtggaaatggagagagaaaaaagaaaaataaaagcaatgtaaaaaagaacaattattattattctggagttggttgctccttggaagaggagatgctggggcctcggattaacatgaaacttaccagaacttaacatagcactgtacacatagtggttcttgatgaagacttgaaaaatgaattcttttatttacctaaaaaaatgttggtagagtgtcttctcttgccaggcagtggtcaagatggcagggattcagcgggaaacatgctcccagtcctcctggagttggttagtgccctgcttccatttgtttcctgagcaccctttggtgttaagtcctagccactggggagagggagggcacaggaatgaggaatgcagagtttctacattcaaagggcttcccaaggagagagaaaggtgctctctgcacacacagctcagccacagggaactctggtcttggaggaggcatcttgaggagggatgtcaaactccaatttgtctcacaggaaactgaagcaaaggcaaggatgaaacacaagtggaaaactcatgggaaatgttcatccttcgtagaggtcaagtgaatgcacctgcaactacccttgagggaccacattacaccaactaaattagcttagaatgtttaaaccaataacacttggtgttggcaaggttattagaacattggtaagctcaggggctttgtgatttgaaagaccccttaggaaagcaacacggcaattctgtccagctagagcggtaaaactgttcatgccctttgaccaaaggatttcattccagggaatttctgcttgaagatggattcaactgtagcaaaagttgtatacacaaagatgctcattaactacagctagcactgaaaaagaaaaaggaaga

SEQ ID NO: 18152 - RNA, 4864 nt, Homo sapiens
  source 1..4864: mol_type = other RNA
tgaaggtctactgtgtgccaggtactgttctaggcgtttcagagtcatccatggaagaaaaaggccataaatccttgccctcgtggagcttaccttctaataaggagagacagagggtgagaaacaaacaaacaaaaatatgtgagttaacacagagtgttggagggtgtcaggtgctatgggagaaacgtggagcatgtcaaggagagagcaggcaagagggcattctggaaaggcctaggaagatggtgacatttgaccttcatatccaccaacccccagcacaaagcatttgccagaggcagacagaggagggcaatggacagtaggcgtccatgcacccaagtgagggagagagacatgcagacactctagagaagagtgtccaggcaggggaacggccctgttcgttcatcatttcatcctcatgagatatgttacgtgttatccccattcgaaagatggtgaagctgagactcaagagaggttaaagtcacatgagagggtcacagagctagcaagggacagcacttactggttgcaagtccatgctaaatataagaccttgtcatgacccagggcttggtgccccttatagtgaagatcagaagaggaatggatcgtcatcttcctctgcttgctaccctcgctggtttcaagacctaccctcagctctgcctccaggaatctagcaccgactgtgtctcacgtggccttgcctcatgccctccaagggatgcagcactggacagaggcaaaagaaagggaaatgtcaccttcttcttctgggcttggctcctccgtcttggaaagcgagtctcagaacatctgttaaaccaagccccagcatattaaacagccactgaaaatgtattgttgcttcgttcaatacatagcaattacacggcgagttttgctcattagcgggaaattgacacagaggcaatcctgctttttaaattaccactaatctcactgcacctgtttgggaagaaggcaggaggagaaaggaaaaaagttgataataaccatttcattacattttaaaaacaaacacttctaaaattcccttaaatatagcttttgggctctcagattcccatcttatcttaggaggagcctctttgcctcatgccacaggctggagtaactctccattaatgtcacaggcttaatggcacatgagtctgggcaccaaggacaccgggaggacaagctaggctcccttaaggtttatttaaagtgagattctgtgattaactatggttaagggacttggtgcacattgaggagagccaccatacctcagaggctcatggaaaactgacttattcagtgggtgggcaggtgttaggggaggtggatgcagatgccgctacaggtgtctccagagctcaaagacaaggtgtcacttgaccaaatcaaacagctgtcagtgaagctggcattcagacttgctgcccaggcaggttgctgaaatcatggagccccaattccccatttctgtctcagtgcacggggttgcatgccatgcccagcacagaggctgacttcacacagtaggcactcaataaatgcttcctaacacaacctcggggctgcttcctgagatgctccttcactgatatcctccagtccatggggccaggctcattctgtatgaggcacactgccctgggctcaagcccctccctggctgggtgatcttggacaaacctctctacctctctgagtcttggcttccttatttggaaaatcgggataatgatagtaagtccagctcaagctcgtggcttgctggcttgttggtgagggtcttgtgtgatcatagggctgaaagtgcttgagaaactggaaaagtggtttaagaaccacgactattgatacccgtggaaatggagagagaaaaaagaaaaataaaagcaatgtaaaaaagaacaattattattattctggagttggttgctccttggaagaggagatgctggggcctcggattaacatgaaacttaccagaacttaacatagcactgtacacatagtggttcttgatgaagacttgaaaaatgaattcttttatttacctaaaaaaatgttggtagagtgtcttctcttgccaggcagtggtcaagatggcagggattcagcgggaaacatgctcccagtcctcctggagttggttagtgccctgcttccatttgtttcctgagcaccctttggtgttaagtcctagccactggggagagggagggcacaggaatgaggaatgcagagtttctacattcaaagggcttcccaaggagagagaaaggtgctctctgcacacacagctcagccacagggaactctggtcttggaggaggcatcttgaggagggatgtcaaactccaatttgtctcacaggaaactgaagcaaaggctatgttgagggtaggaaaagttggcactttttattcctcccttcttttatatttttcccccttcccaagtgcctactacgcaccaggagctatacgaggcaccagggaagcaacaatgaacaaggctgtagggatccctctgggaaaccacagactgatgggatttcagtgcagctgagttggagaagagagacagagagggagacttaaatagcagaacgaggggtttgtgtttgctccttcagcaatggggagccacggagggttttgagcagggaaatgacatgatctgaactggacaagtaataattatttgggcagcacgcaaggatgggtttgaaggggaccagaggcaaggaagccagctcgcatcaaaagataacccttaagtacatctgcctttgttggggcgctctggtttcccgtgcccctttgtggtggggaggtgagggatggagcatcaggggagggagaacaggctgcaggtctgagaagggatgaagggtttccatggcaaccttttgcttgcctgtagccaaggtagctatgcaaattccccaggcaccattcctgtggaccttgaagccagcatccccggctgctgagagcctgactttagaaaaactgggatgcagtaaaattgaacaagagagacgagagacaaagatgttcggctggaacaggggtgcaggctcccaggcagcccttgaattcccttgaacctgttctgcaggctccttctccctcctctagggagggactctcccaagcccacccttccccatttggcatgcattttacaccatggggacttgggccacctggaaaatgggctgacctgatggtggtgcctcctttaagtttttgtgatgacttgcaatattgtttgccaagcttcgtacacaatgcctgggtcagggtaagcaggtcaaaatgctagcagttattgttatttggcattgtgattaaagaatgctggctcttagaacaccaggtcctcctctgagagtggccgctgattgatgtgtgaccttgagaaagtcacttcccttctctttaatcttcctgttcttatgtgtcagatggggatgctggctctacagtctctttattagcattttattgttgttgttgttgctgctactgctgctattgtcaccattattattagtattgctgttttatcattgctattattataacacctatgttgctgctacctgctacaaagggcaatgatgatgattcctgtaaatactccacgtagttagaacgtgaaactctatgccaaagcagaccatgcaaaaatgagttttcgagaaattgttacatgaagagtttataaaaatgaaatgctgtattctacacatatcaagacaggattgcttgtgggtgttgaaacttattaggcgaggtagtccttagacattcacttgtcttagtcttaataattgaccaaatctcctctccttgagttctcacactgggtctgggttccatgtccgtttccattctaggtgatcctaaattcaattgagaatcctgagttcagacccttgtaagacacagcctctcctgttgtagaaagacaccttcctttacctaacacagatttagtccacatcgtattactaaccctaaccctaacccaacctgagtatttggcatgtaatagacactcacatttgttgaaaggaagaaaagaaagaattagaaggaagaaaatggggcacactgctttctaatcccaagaccctctagttattaatctagagaggaaggtagaagccaactctctcatattcgtctcagtggaaaagccatttttcccctctaactccagactttctgtcttctttttttactcaccaatgcccaaaggaaaaaaaaaaggtatttccaagtacgaaagtacaaagtttcaaacccactcgtgctcctccttacaatgcagtcgattaatcccacaacatttctcctgggtggttgccgttaattgaattaaatgagataatatttgttgagtacgtagcactgcgcctggaaatgtttattgcatagaattgaatcaaggatgaaacacaagtggaaaactcatgggaaatgttcatccttcgtagaggtcaagtgaatgcacctgcaactacccttgagggaccacattacaccaactaaattagcttagaatgtttaaaccaataacacttggtgttggcaaggttattagaacattggtaagctcaggggctttgtgatttgaaagaccccttaggaaagcaacacggcaattctgtccagctagagcggtaaaactgttcatgccctttgaccaaaggatttcattccagggaatttctgcttgaagatggattcaactgtagcaaaagttgtatacacaaagatgctcattaactacagctagcactgaaaaagaaaaaggaaga

SEQ ID NO: 18153 - RNA, 4547 nt, Homo sapiens
  source 1..4547: mol_type = other RNA
tgaaggtctactgtgtgccaggtactgttctaggcgtttcagagtcatccatggaagaaaaaggccataaatccttgccctcgtggagcttacctttggttgcaagtccatgctaaatataagaccttgtcatgacccagggcttggtgccccttatagtgaagatcagaagaggaatggatcgtcatcttcctctgcttgctaccctcgctggtttcaagacctaccctcagctctgcctccaggaatctagcaccgactgtgtctcacgtggccttgcctcatgccctccaagggatgcagcactggacagaggcaaaagaaagggaaatgtcaccttcttcttctgggcttggctcctccgtcttggaaagcgagtctcagaacatctgttaaaccaagccccagcatattaaacagccactgaaaatgtattgttgcttcgttcaatacatagcaattacacggcgagttttgctcattagcgggaaattgacacagaggcaatcctgctttttaaattaccactaatctcactgcacctgtttgggaagaaggcaggaggagaaaggaaaaaagttgataataaccatttcattacattttaaaaacaaacacttctaaaattcccttaaatatagcttttgggctctcagattcccatcttatcttaggaggagcctctttgcctcatgccacaggctggagtaactctccattaatgtcacaggcttaatggcacatgagtctgggcaccaaggacaccgggaggacaagctaggctcccttaaggtttatttaaagtgagattctgtgattaactatggttaagggacttggtgcacattgaggagagccaccatacctcagaggctcatggaaaactgacttattcagtgggtgggcaggtgttaggggaggtggatgcagatgccgctacaggtgtctccagagctcaaagacaaggtgtcacttgaccaaatcaaacagctgtcagtgaagctggcattcagacttgctgcccaggcaggttgctgaaatcatggagccccaattccccatttctgtctcagtgcacggggttgcatgccatgcccagcacagaggctgacttcacacagtaggcactcaataaatgcttcctaacacaacctcggggctgcttcctgagatgctccttcactgatatcctccagtccatggggccaggctcattctgtatgaggcacactgccctgggctcaagcccctccctggctgggtgatcttggacaaacctctctacctctctgagtcttggcttccttatttggaaaatcgggataatgatagtaagtccagctcaagctcgtggcttgctggcttgttggtgagggtcttgtgtgatcatagggctgaaagtgcttgagaaactggaaaagtggtttaagaaccacgactattgatacccgtggaaatggagagagaaaaaagaaaaataaaagcaatgtaaaaaagaacaattattattattctggagttggttgctccttggaagaggagatgctggggcctcggattaacatgaaacttaccagaacttaacatagcactgtacacatagtggttcttgatgaagacttgaaaaatgaattcttttatttacctaaaaaaatgttggtagagtgtcttctcttgccaggcagtggtcaagatggcagggattcagcgggaaacatgctcccagtcctcctggagttggttagtgccctgcttccatttgtttcctgagcaccctttggtgttaagtcctagccactggggagagggagggcacaggaatgaggaatgcagagtttctacattcaaagggcttcccaaggagagagaaaggtgctctctgcacacacagctcagccacagggaactctagaacagagagatatttgttttaaatagtgtatctaggaagtcttactggaggaagtggcatctgcattgagcgctctaaggataggaagaatttggcaggagttgaggtgtgcacctacctggtcttggaggaggcatcttgaggagggatgtcaaactccaatttgtctcacaggaaactgaagcaaaggctatgttgagggtaggaaaagttggcactttttattcctcccttcttttatatttttcccccttcccaagtgcctactacgcaccaggagctatacgaggcaccagggaagcaacaatgaacaaggctgtagggatccctctgggaaaccacagactgatgggatttcagtgcagctgagttggagaagagagacagagagggagacttaaatagcagaacgaggggtttgtgtttgctccttcagcaatggggagccacggagggttttgagcagggaaatgacatgatctgaactggacaagtaataattatttgggcagcacgcaaggatgggtttgaaggggaccagaggcaaggaagccagctcgcatcaaaagataacccttaagtacatctgcctttgttggggcgctctggtttcccgtgcccctttgtggtggggaggtgagggatggagcatcaggggagggagaacaggctgcaggtctgagaagggatgaagggtttccatggcaaccttttgcttgcctgtagccaaggtagctatgcaaattccccaggcaccattcctgtggaccttgaagccagcatccccggctgctgagagcctgactttagaaaaactgggatgcagtaaaattgaacaagagagacgagagacaaagatgttcggctggaacaggggtgcaggctcccaggcagcccttgaattcccttgaacctgttctgcaggctccttctccctcctctagggagggactctcccaagcccacccttccccatttggcatgcattttacaccatggggacttgggccacctggaaaatgggctgacctgatggtggtgcctcctttaagtttttgtgatgacttgcaatattgtttgccaagcttcgtacacaatgcctgggtcagggtaagcaggtcaaaatgctagcagttattgttatttggcattgtgattaaagaatgctggctcttagaacaccaggtcctcctctgagagtggccgctgattgatgtgtgaccttgagaaagtcacttcccttctctttaatcttcctgttcttatgtgtcagatggggatgctggctctacagtctctttattagcattttattgttgttgttgttgctgctactgctgctattgtcaccattattattagtattgctgttttatcattgctattattataacacctatgttgctgctacctgctacaaagggcaatgatgatgattcctgtaaatactccacgtagttagaacgtgaaactctatgccaaagcagaccatgcaaaaatgagttttcgagaaattgttacatgaagagtttataaaaatgaaatgctgtattctacacatatcaagacaggattgcttgtgggtgttgaaacttattaggcgaggtagtccttagacattcacttgtcttagtcttaataattgaccaaatctcctctccttgagttctcacactgggtctgggttccatgtccgtttccattctaggtgatcctaaattcaattgagaatcctgagttcagacccttgtaagacacagcctctcctgttgtagaaagacaccttcctttacctaacacagatttagtccacatcgtattactaaccctaaccctaacccaacctgagtatttggcatgtaatagacactcacatttgttgaaaggaagaaaagaaagaattagaaggaagaaaatggggcacactgctttctaatcccaagaccctctagttattaatctagagaggaaggtagaagccaactctctcatattcgtctcagtggaaaagccatttttcccctctaactccagactttctgtcttctttttttactcaccaatgcccaaaggaaaaaaaaaaggtatttccaagtacgaaagtacaaagtttcaaacccactcgtgctcctccttacaatgcagtcgattaatcccacaacatttctcctgggtggttgccgttaattgaattaaatgagataatatttgttgagtacgtagcactgcgcctggaaatgtttattgcatagaattgaatcaaggatgaaacacaagtggaaaactcatgggaaatgttcatccttcgtagaggtcaagtgaatgcacctgcaactacccttgagggaccacattacaccaactaaattagcttagaatgtttaaaccaataacacttggtgttggcaaggttattagaacattggtaagctcaggggctttgtgatttgaaagaccccttaggaaagcaacacggcaattctgtccagctagagcggtaaaactgttcatgccctttgaccaaaggatttcattccagggaatttctgcttgaagatggattcaactgtagcaaaagttgtatacacaaagatgctcattaactacagctagcactgaaaaagaaaaaggaaga

SEQ ID NO: 18154 - RNA, 16202 nt, Homo sapiens
  source 1..16202: mol_type = other RNA
tgaaggtctactgtgtgccaggtattgcgtaacgttattgacattcattatttcattcactccctccaataaactcaagggttagtgatatattaagtgctcgtgggttgcacaaagctaagaaaattcaaggaatactctggaggggctgctgatgctgagaaagtgttgatgaaatcattatccacaatagacagtggctcaagaaatgcaaattgagtcaagttgaagcagataaacaagcctcgctaatttgcagtagccacatataccctgggagtctggcggtcagcaaagatgctttgttttctgtctttcaaaccctgacatatttatagagacagcaaacacaccactccatcaacaggactgatacattctttcccacacttcaggctgtattgcaggcttggcctgtggcccactatggcccctaggtcttcttcagtcatttctgtaacaaaccagcattttgcccatcatacctgaaatgtttagttagagaccctcagtgtagggtctttccataaatacatttccacgttcacacatgtccttgacctcaacacttcaggggcctattcatagagtgatatgaactgtcccagaaagaggttttttgctgaagaaggttttttggtatggcaagacagaactgggggccccagagacatcagagacacaggtcgcaagagtcgatagagggaaagtgaagcaaaagaggaacaggaatgaaaaatgcattagagagaagggctcatggccaacccatctatagccaagatgcccatggacttcaggacccaatgcagggcactaagaaatagagacacatccttcactgtgtggaggcaggcagagacagagacagacacagagacagacagacagagagagagagagagagagagagagagagagagagaggtctgtagagccagagagggatgcagagcaggcctgaggtggcctgagtactggtctgactccagcaagcacaaaactctcctcagacatcttcccccacaggacaccaaggctaacagtaggaaccagagcatgctggggaaagaagtcaaggtctccacatctgagccagggcaccctctgtttggagatggagactccagggtcccaaaatcaggctttggggaaagcagggaaaggcaggcaagtgccagggggcaggattttagccacttgcagttaccctcaataaatcatgatcttgcctctgagtccacacataggctgttccttctgtctgacacaccgttccctaccattctactcaaatttcaagacagggttcagaagtctcctcctctgagaatccttcctggagggtctttctctgggttgggagctcctgtggggcctcgggaccctactggaactcctccctctcttcatcggactcctagtaccctgaaggcagcacccacttttctccattttttccagaatcacaggaggcacttaacaaatatttactaaatgactatataaaatgaagatttggggaatgaagggacaaggttgctccacgctgggctctgctgagggtgtagtgaatggggctggggacatgagcctttgaaatacaagcaaaattttcttagaatccttcggctgctcaactgtaggcatttgaaatccaccaatgtacccaaaaatagggctatgaggaaactagaggaccggggcccagaagcagtgccttgtggaatatgggacagctatgggagctcatggagaacagagactccaaattggatgccatcttggaagtggagtcagagaagctcatgtgacagcatgcctgacatgccaccatatgggcttctggcctctgtgctccaagccttggggctttatgaggattgattccagacgcaaagtcagggtgtgttttgatggggtggggagtacaatctatgatattccttgataggttaggaccgcagaggccctcaggaggagatagacttccgaaaagaaggaagaaggagccaggcaaagatttatgcatcacacagttgggcagaagcctgaccaaggacagcccctcccttaatgctccagtcgagccaggactgtccagatagctttgaaggggcagggtgtgcagtgctccctagaaggctggctaggagggaaagggggccggggcagggggcctcggtgtggcagggcaagtaccttagagtaccttgatgcccatgctgtagctacatagcagttacttgaacttacacaagttcatatgtacccatctaaacattattacttgtaacacatgtagaaaaataagcagaggaaaatggctagaatcttacaggaccaatacattacatttgttgtccaggacgcacttaagctgccaatgccccaacctgggcagggctgtgttggggagaggttgaccccatctagggcagagccccagccaactcaactgtcttcttggaaggtgtcccaattcccaaagcaattttccaagatctggtcttttgcagtgcccgactcgtcctctctgttacccttcccaatcctgggactgccggaagctccagggatttgattctaggggtaaaacagctggacctacagaggccatcctcacccactgcctgtctccatgcccaaatcagtcacacgggactggacagaactgccacatcttgtccagactgtctatgttgttgcttcattgctaccagagacagccattctaacccggcctgactctcttcttcacagtgaactgggaattgcaaggaaggtagaaaaggcccttcactatctgggagactttccttcctggggaatacagaagggctttccctgagtagcctcagaaagcaacaccaagattgccggatgcaagtctcaagatttcagctcagcaagaggatctgcttcttagaagggctgtggaaggatggagagaatgactggagatttcagcccctgtccgtgcagacggtgaaaggcaagtccacattctccttacctagacagccttcaaaccactggtgatgctaactagtgctttaaaaacctatttccctgcaatgttcacttaaggagtcccctccttgtgttttcctgttctcctctgatttcctttctcccatggaaggttgcagatggcaggatgctggatttgaatcctagtcgcgtggcctggagacaactcaggggacatctggcaatgtctggagatggttttggatgtcacactttggatgtcaactggaggcttttgaaatccaccaacatacccaaaaatagggctatgctggaactagaggaccgtggcccagaagcaatgccttgtggaatatgggacagctatgggagctcatggagaacagagactccaaactggatgccatatcagaagtgggggtcagagaagctcaggtgacaccatgcctgacatgccaccatatgggcttccagcctctgtgctccaaggcttggggctttatgaggattgattccagacagcaaagtcagggtgtgtctggggatgtttttggatgtcaccagtaccaggtgctactggtatcttgtggggagagttgaggaagctgcttaacatcctccaatgcccaggacagtcgccacctcaaagaattatctggccccaaatagctcaacagtactgaggttgagaaaccctggcttagaatgaacatctctttatccttctcttcctttagatcttgacttaaatgtcacctcctcagaaagacctttgtcagcagctctcccacagtataccctctcccatgtttctggtcccccgtgagttttctttccatagatctacatgagttgcaaatttatatatttgtggttgacttgcttcttgtctctcttccccattgggctttaggcttcagaacaggtgagacattgtatcactcatcactgaatgcccagggtctaacacatagtagatgctcaacaaatcacccactgaatgaatggttggtgaagaaatctctgtcagagaggacagaggttcactgaattccagacaaacccagaatgccagcatctgtgtgaggacacaaagacctctcttctaccttgttcatcctgtcgcccaccactcagaaaaggcctctggttattgttggcctgtatttatttcctcctgatatcctggtaccagcctttccaaaattctcactgtagtgctggaggtcagggtatttttaaactagaagaactagccaagctggttttttttttttaagtggtggaaaagaaaaactaagatttgtttttaatcattagactttcaaatttaagaaggcgcgatgcaaatagcatgttggcataaacaagtgctgcccgctcaatggagggagggagcctttcttctgagctaatttaagctaaatacatggcagctatttttcatctctacaattgtgcaactttctcctcagtttacaatacaggggagatattatcgggcagaagttggatgggggataagtgaagacgagaaggaaaagaagaggcagtggacaagaaggtactctcagccaccgagctggtgattagaggtatttcaagagctcaggagtagagctggtggtccactaggacctcaagatcttatctgggtggaaacttgattttgagccttccattcagggaagaaaccaaagagcaattggagtcaggctccttttcctgccctttatatgcagcaccccctgacttcccagaagcccagactgaacagcagaaattttacaaacctcctcaagaaagaaaagcccttgcagctctcctgcacaccaccacgcacactgttattccttaaggcccccatatgccgtgacttccagcccagctgttactagactgggcatagcattcaggccttgtggtgaagccgtcccagaagataaatgatttttctccaagcaggcagattaccgagtaggatcatacacagagtcttagagacagaatctttctttctgcattttccaagttccctaactgagaagaaacatctgcagagcgctgatagactgtccaccaactacagcccaaatggcttggcttctggaagtttctgaggcctgagttctaaacctacctctgcctcttagaagggacctgacttaggggagtttattatagcttccctctctgggcctcagatcctgcttctgtgaaaggagaagagtgagataagggagggtcactcatatccatcttaagtggtaactcgaatgccctgaagctacatctgtgatcagtgggaaggcatgctgtgatggattagtgatgtctgccaagagtacagcaggggacactggtggtagatccattacatatttgtactccttggaccagatctttatccttctagatcttagaggtccttctagatcaccatcccaatgacttggttgaagatgaaaactcaggtgaaaacttaacccttctgagggtgttacatcttatatacttttcacattggcctccaagccatggtatgttggagaagccaccaacacacagcagatttgacccctccattggaagacaccatcagccagatgtggtgttcttgttcatggaaccactgtccacatggatggaatcgggctctaagctacctttctcatctcctagcagtgtctatgaatgctagtggtcagctcttttctgtgggccagtacattgacattgcctccttcagtaccaggtaaggtatcaagtctcattcacagaggttgaccttgttggagattcagaaacaagcctgggaaagcttgggaagaacagcctcctatcaggcatttagagattcaaccacacaatagtgtcttaaaagttctgataagtcctgcaatcaagaaattagtttcattttacctaagcatttccaatgcatgcttgtcccaggaccctttcaataatgcaaatccggcgagttttccatggaatgaaaggtctatgggacatgcttgggaaacaaggtcttatttagatcaggcacattctagacagagtccatctcctccagctcagtcctcagtggaaggaggacagccattctcaaccccatgagatgaatccttcatattcttggtgttaggaaatgggagctgcatgatcccaatgagtgggaaggaagggccctttcccacccctgagagggaagagcactcactgatgtacgcctctcaggaacacgggaccacagtgcaacatccagcaggagagacggaggggataggaagcctggagcagggatactggagggacccaggagggactctgccaacccagatgtacatttcctggaaatccgggctgctgctggcagcctgtcagtttgagaacataagttcaagcttccgtgcaaactcccagtatggtccctgccagcccctgcaccctcccttccacaacttcctgcttttcctctctctctttcctggttccaagttgccaataagtctcagaggctgggattgtaacatccccatgagcagctggacatgaaccccttgacctggaggtgggttcctgggaatggatgagcccaaagactcgtttttaaaatgctgggtctgcaatttggaggctggtttctgtccctgtaccacagttgccccattggaacgagaataagactactgatctccccaaaccatcataggaattccagcctggcacgtagtaagtgctctgtgaatgagggctgttcagggtggattgttactctgcctcctagacatcctgggccacctgactcaatgggtcgcttcatacgtcacagatattaaacctggcaaactggctcagcacaatggcttagccctgtaatcccagtgctttgggaggctgaagcagggggattgcttgagaccaggagttcaagaccagcgcgggcaacatagcaagaccctgtctgtacaacaaataaaaaattagccaggcatgatggtgtgcacctgtagtaccagcaacttgagaggctaaggtgggaggattgcttgtggccaggagttcgaggctgcagtgagctatgatcacgctgtactccagcctgggtgacagagcaagactctaactctaaaccacaacaacaaacctaacaaacaaactcattggggttgatatggcacccacaacatggtctggcaaaggggaatcccaataccatccagccctgccaatggtgcccttctaactccctgtgccagggtcttactcttacccagcaaacctctctgtctgcattctgtaaacatttcttgagcacttactatgtgccaggcactactaagacaagtccaggaggtcactgggaccgcagattttccatcaacctcctgccccactactggtttcaaaactaaactggtaacagaatgggtatggattgcagggcctcgagaagggagtctgggatttgggttaatatcatagtcaggcactgaccagagaggacagaggttcactgcggctccacattccaggacccagactgacatttgctgcctgtcactccccttggagttcaaagtgattcccttgcaggtgtgtgcaggtgagggtgaggtggtacgggaggaggtgaggctgggagccagggagagtggccacatgagtctgcctaggaacttccccacatcacaggcaaagccaaaaaaggaaacagcaaaatgtagctcatcaaaatccactcctttgtcaatgaacaagagtatagataaaatcagatgctgtgtcaccaactgctttggatagggtcatgaggcacattcaggggtcaagtgacagtccgctacagacaagccacttacacacaggctgttcccatacagccacagaactgagatccagagctgttggaattcagtgatgggacgtgttgattggggcaagcttggtaagcatgacagcaacagcctgaccttgtagaccaggaattctggggaatctatcttcaagggcacctgggttctacagtggaggaccagtcaaggcacaagagaaaatgtcttagagggtgttataagttgtggtgtccccaacaaaaaaaaaaaaaaaaaaaaaaagacatgttgaagtcctcattcctagtacctcagaatgagacttcatttggagagagggtctttgcagatataattagttaagatgaggtcatactgaaatagggtgggcccttaatccaatgtgactcgtgtccttataagaagatggccatatgaagatagggacacacagagagatgatgagggcagggattggactgacacagctgcaagccaaggaatgccaatgatgaccaggaaagcaccaggaattcagaagccgccaggaaggattcccttacagatttcagggggaacatggccctgctaacactttgattttggacttctggcatccagatgggtgagagatgatacatctgttgttgtaggccccagtgggtggtggtttgctgcagcagtcctaggagcctcacggaggtgaggggggcttggggatatggtggcacagtggaacaagaccagcctgcaggggatggatgggtgaagtgaaggtaggcacaggatgaggatagggagggcatatttcgggactcaagattgagaaccagtgtggggaaagaaagccggggatgggaataaaatcacagagcgttggaaccctaatctaataagattgttgtctttatcagaagaggaggagatactggggatgtgcagtcacagaggaaaggccacgtgaggtcacgatcagagggcagctgtctgcaagccaaagaaagaggcctcaccagaaaccaaccctgctgacaccttgatcttgggacttccagcctcaagaattgtgaggaataaattcgtgttgtttaagccactcagtgtgtgacattttgttattatggccccccttagcaaacgaagagttttaaagtccagggagttggtccagccttcagggcctgaattgcctccatatcacacaggccaagcagtcaacatctgctccaccctatccaaggacagggagttctctacttccggaggcagcccgctgcatcttggggcaagctggccttcttccgctgaaacaagttctctccccctccaacttcctgttcctcccctgagagccatatccaaccctctctatcaaaggctcctgttcctcccctgacagccatatccaatcctctctatcaaaggctagcaaagttaggaaagggccagattgtaaaagtttttgactgtgtgggccacatcgtctctgttgcaaatagctggctctgtcacagttgcataggagcagccgtggttgtgtaaatggagaggtgactgtgctccaataacattttgtttattgacatgaaatttgaatgttatagaattttcatgtcatgaaatattattcttttgatttttcctcaattaaaacatgtaaaaaccatttggcaggctgggtatggcctatggggcatagcctgacagccctgggtttagatttctcaagataatgattggcctgagctccgtgtctactacttcctccgtgtacctttgatgatcagctgtaggtggggatgggaatggtggaaggtgagataaggctggtttcgtgtgtttgtggggaggggcatgatgtgtgtatatggcatgggaggtgagaaaaagggaagaactaggttccctggatacaaaagtctagtggtcaatatcagtcaagggcttctattgactgacaatccaaggtagctgtggagacaagtggatggggtgaggatgggggggtccatggcaagatgaaaattttctctttgatcagtaaaaggaataccaggacaaaatggatctaagcaatgactttgggtttccagcttggctctggggatggggacacaaggggcacgtcctcccacagggggccaagaaggaagctccttggttttatgaataatctgtatcctggaagagttgggtgaaatttatgtgcaaatccacatgccctttaaagaaagctgagatgtttctctctgcaaagccaaggcttcctggtgaatcttcaccctgtggactggtcccctcgggaagcccatgtatatgacggtttgctaaaagcaagactgactggaacaactcgctgctgagtcagtgacttatgtgtacagggcacctgtgtgcagctgtgatgggacaagggcaaacacacaaatcttggtcgtgtcattgtatagaatgagttgcaggtgaggctggtaattatgatgtaaaaatatacagcctctttcctctttttttttcctccctgcgtaagatgaatataacctcctcccaaaacctcatcagcgaataaagatggaagccagcagggaaagcagcggtttggttcttcctggatttaaatgtgtgcaaattaaagctggtttctcaacaagtcagggcggtgtagaggggacagggtaggggcgtcaggaaggcactgaaggccaggatcctggcctggctgcagcagagaccaatgcaggtggggacagagtagtgaagtggggaaagatcgagaagtcaagagcaagtgactcagattcagggatggacccaaggcaccctgttccacaaagggctgggttttcccctggatcactcaggccctgtccttaatcccaaactggtgctcatgaatgaatggaaaaatcagctgttggagatcatgctaggccttgccaaaggctgtggttggacattttagttaattctggaaacaagagaggcaagagtgagaaggtgccagttcttgtggacatttcagctgcagggtagtagaccctggctgcctcttcccttcctcatatcctgtctcttggcacaagggaacatgacaaggactggagcctgtggacccaagaagtcctggtgtgatggaagagaagtgagtggttgggtttcaggcactcagtaggctgctgggcagagccaagacaggtgcaagtccaggcccagggctgggacacagagtgttgtgttgggatggggaggtgtccattgacaagagccatccccagcaaccccagagtggctggggctcaggcaaacatatataaaatgcctccaagacacacacacgtcgtcaagccaagagccatagatgtccccagaagagcagtgtctgcttaggagcagcccaagccggggtctttagtcctctagtcccagtaagctgggagtgttggaaaggcaattcaggagggccctttgggaaacacaggggtttcctgtagccaggctcctgggaagcatgactgatctcaccattcttcccggtttggaagcaggtttggcccccagagcatgaaccagtctgggagtcacccaaggtggggaagagatcctcataggtctatttggattttgaaagtaagatcaggtagggtttttgaagttccagttcctctctctggccctctaggagggagatgcctggatagatagtagctacaagaaaactaaggcccaggtagtacccaggaaacacagaggggctgtggccgccctgggcttcctgttcactgcccagataatcctgctattgctctgcttggggacagatttcccttttgtatcaggtcacatgcagggggtcagggctttgaaaacatgggcaaatgacccagaggttctcctctcccatctgcatgcccagcctgctctcggcatccttcctacagatacagaacaccaggggcttccccaacatggtcaggaagagtcgccggcccaggttgggatcaagaggagggagggaaggtggggcactgagggaacacacacaggtgagggacacaggcttccgatggggaagctacttgaggaccccgcaccaggctagagcaaagaacgcagaagtgtaacaaacatcctccctttgtgctcccccaacaggactcctcaagggtgacaggcagggaaatcttttgcaaacgtgttatcataggtacagccacataacccaacatggacgtaccccaagaacccgcatccaccttggtgggggaataagcttcactggtgtgagtagcagagaagagggaagaaaaggaatgtcctagaactccctgcccagagccctgattctcagggaccagacttcagggggtgccctgaatgacggtgagctctaaggagcccctcagaagtcatcttggctttccaaatggcaaggaggtgcgggcagtgaggtgaaaagggatgctactctcagagaacaggagaaaacagcagaaatgggggaataggtcccccagagagacccagaactcaaaagacgttctaactttcctactgtacttcagagctctatgcaaaggtgccacacgccatgacaggctcgggttggggtgtctgaaaacagatatttccaaaggaacgagcttagccactcccgaccttccctgctcgatcttggctcagtagccttgactaagctgccactcggctctgtaccctcctcttagcttcccagatggtacagctggaacctaccacatacagacagaactgaggagtgccccgtcattgggacagtctggctcttgcttgtcaaggggaaacaagagtgaacaacgtcaaacacacagacacacacacacatagccccgtctgtgagcccccccacgtggggtctcctgtcctagtcccatagcccaaaggcaccacgtgcagcctgcagtgctctcattagtgctgtcccctgggccgcactgatcaataacgcatcaccctggctggtccggttcagtcctagctcgggggtccccaaccctgcccgaggaaaagggctcaagtctgaggtgcagggaggccgccgagcagttgtccagtgctcccaggtcggtcggggttggtaccctctgatgctgagtctctggcctcctgagctggcagaggacagagtagggagggagaggtgacgggagcccaggcagctgggcgccgtcccgatgtccaaaggtcacagctctgcagacttccagaaatgtccagggtgagacaggcgacggtttcgctttggcagtttctccagcatgtccatgagcttggtgaaggtaggtctctcttcttgttcaaaggcccagcagaagagaagaatgtccgagatttcttttcccatgccaatctggctgaggttgggtttcatgcctgtgcccatttgccagattattgcctctgctggttgggtcttgaaaggccattccctggcgtggagttcataccagattgtgccaagggcaaagacgtcagagtgcttggagaaggggagcttatcctcctctgtgtcgggggacagctggcggatgatctctggtgccaggtggcatagccagccattctggatgcgcagtttgtcctcccgcctgccagcctgcagcaccccagaaatgctgaagagtccaaagtccgtgatgaccactttgccgttgtcatagaagacgttctttgacttgaggtccttgtgtaggattcccttggcgtggaggtagcccatgcccttcacaatttcttgagcaatctgcctggttttgttgacatccaaaacgattttggcatccctcacaacggaatagagcgtccgtcccttacagaggctggtgatgatggccaggtgaggcgggctcatgcaggcacccatgaaaagcaccacgttctcatgccgtgtctgcctgtaggccatcacctcccgcttgaaggccttgagctggtcctcgttgtccctctcaatgtcaatcagccggatggccacctcgccatgccagcggccgtggtacacttgcccaaagcggccctttccaatgagctcgccgatctccagctgctcaaaggggatgtcccactcctgaaggaagatgctggtctggctggccttgcgtgggaagctccgggccgagaggagggacaggttcatctcctcgaagtcatcctctgactcttcggcctcatcatggacctcttcattctccgacgttggctccacttcaatttgaagtaatggatttccttccaagattggattcgaggtcaccggatgcaggatgacctggggcgcccgggtcggcgtctccggcaccggcaccacatctgggaagatgaactgctgcttgtatttgtagtagtgggatgctggcaggttgaagttcttctgctgccgtgtgcactgtggggaagggtgtaggggagaaggcggcgtggcactaggagggagggggggtgctggcgaggagggcgtggaggacgtcgtggaggaggggttgctgctggagtctggctggtaagggacagggatgtggtccttgttgattttgttggttttggggagcgtctgactgatgtgcaggtctgaatagcgaggtggcttccgtagagggttgttgatgtcacacggaacggactctgtccggactaaccttgctcctcggtggatgatcagaagatgacagggtggggcttctttggtgcatttgttgtggcactttaacttgcagtttttacacttgaggccaaaaagcatccctttcccacagactgtgcacgtctgagacatccagtacttggtggaaaacctgtgcttgatggagttgccgagatctctgcgagggatctgcggggaccagcgtggcactgacagtgtgtttgcagagaagttggcctcagtgtgaacaggaggggtggaaggcaggaaaggtgcgtgtcccacaaagaaggagcggagggagcgctcggacagcagcggggagcgctgctgagaggggatgttctcgcagctgcctacgctgctgtggatcttgaggttcaagggtttgctcttcttcttggctttgggcgtgtgggcctcgtccacgcggtgccccagctggaactcgtgggatttgctccgatgcagcgcggtgaatcccgggatcaagtgtatcagttttcgggaggagggcggtggggtccccgggggcttcagcttgttcttcttcctcatgggcggcgtgcccggcggggtcacggtggtgacgatgttgggggtgcgcggcggggtgcggaccgcgtgccgctgccggggcgatgggggcagggaacggtggcccgactccagtggcgggggcgggcacaagcccgggtaggcgtccacggtaagcctgtccacgtgggtgtacacaggggccccgggagtggggctggtgtgacaatagtgctggacgcacttggacgggaccctggggctctgggagagatgggtgcggatccacggggtgggctccggggggcacacgggattgttctccttccccgtctctgtcgtgggccactggatggtccagtcttgtttggaaaggttgcctcctgacatgtggacattcctgaggcaggagagggaggcgttgaggcgggcacactcctcccggttggctccgtatttctccacagtctcgcacacctgttcatccgtcatctccaagaggtcctccaggctcagctggccgggggagatttcctccaggacctccttgcgcacatcgacgattcggaaccagtgccgtagctgggggaagccgtccagctccgcgttgcgctcctgcaaggctaccttctttttgcaggacagctgccggctgaagtacttcaccagcttgctctccagggtccggatttctttttgtgtgaggtcgttggaggtagcacatttggtcctaagcccttccaggttggagatgctcaagtctatcatgttttggaccagttcgcactgctgtaaggctttttgcaaactcagaggctgctgctcctcgcttttcgtcatgttttcctcatccatcgcttgctctgcaacccccttcccctcctcctcctcccagagagaaaaaagaggggggggagtagaggtagtctaccctccgcctctccaaccactgcgacttctcaacaatgtctcatgaagaagaaatccaacatctcacacagggttgagggggtgggagtgggaggaggggacaagagccaaaatttattattttattttgggatatcaagcggactccattagaatgtctcctctctctctgagtctctggtccctgaaaaggagagatgctgtttctcagaagcaaaccaggtgat

SEQ ID NO: 18155 - RNA, 14659 nt, Homo sapiens
  source 1..14659: mol_type = other RNA
tgaaggtctactgtgtgccaggtattgcgtaacgttattgacattcattatttcattcactccctccaataaactcaagggttagtgatatattaagtgctcgtgggttgcacaaagctaagaaaattcaaggaatactctggaggggctgctgatgctgagaaagtgttgatgaaatcattatccacaatagacagtggctcaagaaatgcaaattgagtcaagttgaagcagataaacaagcctcgctaatttgcagtagccacatataccctgggagtctggcggtcagcaaagatgctttgttttctgtctttcaaaccctgacatatttatagagacagcaaacacaccactccatcaacaggactgatacattctttcccacacttcaggctgtattgcaggcttggcctgtggcccactatggcccctaggtcttcttcagtcatttctgtaacaaaccagcattttgcccatcatacctgaaatgtttagttagagaccctcagtgtagggtctttccataaatacatttccacgttcacacatgtccttgacctcaacacttcaggggcctattcatagagtgatatgaactgtcccagaaagaggttttttgctgaagaaggttttttggtatggcaagacagaactgggggccccagagacatcagagacacaggtcgcaagagtcgatagagggaaagtgaagcaaaagaggaacaggaatgaaaaatgcattagagagaagggctcatggccaacccatctatagccaagatgcccatggacttcaggacccaatgcagggcactaagaaatagagacacatccttcactgtgtggaggcaggcagagacagagacagacacagagacagacagacagagagagagagagagagagagagagagagagagagaggtctgtagagccagagagggatgcagagcaggcctgaggtggcctgagtactggtctgactccagcaagcacaaaactctcctcagacatcttcccccacaggacaccaaggctaacagtaggaaccagagcatgctggggaaagaagtcaaggtctccacatctgagccagggcaccctctgtttggagatggagactccagggtcccaaaatcaggctttggggaaagcagggaaaggcaggcaagtgccagggggcaggattttagccacttgcagttaccctcaataaatcatgatcttgcctctgagtccacacataggctgttccttctgtctgacacaccgttccctaccattctactcaaatttcaagacagggttcagaagtctcctcctctgagaatccttcctggagggtctttctctgggttgggagctcctgtggggcctcgggaccctactggaactcctccctctcttcatcggactcctagtaccctgaaggcagcacccacttttctccattttttccagaatcacaggaggcacttaacaaatatttactaaatgactatataaaatgaagatttggggaatgaagggacaaggttgctccacgctgggctctgctgagggtgtagtgaatggggctggggacatgagcctttgaaatacaagcaaaattttcttagaatccttcggctgctcaactgtaggcatttgaaatccaccaatgtacccaaaaatagggctatgaggaaactagaggaccggggcccagaagcagtgccttgtggaatatgggacagctatgggagctcatggagaacagagactccaaattggatgccatcttggaagtggagtcagagaagctcatgtgacagcatgcctgacatgccaccatatgggcttctggcctctgtgctccaagccttggggctttatgaggattgattccagacgcaaagtcagggtgtgttttgatggggtggggagtacaatctatgatattccttgataggttaggaccgcagaggccctcaggaggagatagacttccgaaaagaaggaagaaggagccaggcaaagatttatgcatcacacagttgggcagaagcctgaccaaggacagcccctcccttaatgctccagtcgagccaggactgtccagatagctttgaaggggcagggtgtgcagtgctccctagaaggctggctaggagggaaagggggccggggcagggggcctcggtgtggcagggcaagtaccttagagtaccttgatgcccatgctgtagctacatagcagttacttgaacttacacaagttcatatgtacccatctaaacattattacttgtaacacatgtagaaaaataagcagaggaaaatggctagaatcttacaggaccaatacattacatttgttgtccaggacgcacttaagctgccaatgccccaacctgggcagggctgtgttggggagaggttgaccccatctagggcagagccccagccaactcaactgtcttcttggaaggtgtcccaattcccaaagcaattttccaagatctggtcttttgcagtgcccgactcgtcctctctgttacccttcccaatcctgggactgccggaagctccagggatttgattctaggggtaaaacagctggacctacagaggccatcctcacccactgcctgtctccatgcccaaatcagtcacacgggactggacagaactgccacatcttgtccagactgtctatgttgttgcttcattgctaccagagacagccattctaacccggcctgactctcttcttcacagtgaactgggaattgcaaggaaggtagaaaaggcccttcactatctgggagactttccttcctggggaatacagaagggctttccctgagtagcctcagaaagcaacaccaagattgccggatgcaagtctcaagatttcagctcagcaagaggatctgcttcttagaagggctgtggaaggatggagagaatgactggagatttcagcccctgtccgtgcagacggtgaaaggcaagtccacattctccttacctagacagccttcaaaccactggtgatgctaactagtgctttaaaaacctatttccctgcaatgttcacttaaggagtcccctccttgtgttttcctgttctcctctgatttcctttctcccatggaaggttgcagatggcaggatgctggatttgaatcctagtcgcgtggcctggagacaactcaggggacatctggcaatgtctggagatggttttggatgtcacactttggatgtcaactggaggcttttgaaatccaccaacatacccaaaaatagggctatgctggaactagaggaccgtggcccagaagcaatgccttgtggaatatgggacagctatgggagctcatggagaacagagactccaaactggatgccatatcagaagtgggggtcagagaagctcaggtgacaccatgcctgacatgccaccatatgggcttccagcctctgtgctccaaggcttggggctttatgaggattgattccagacagcaaagtcagggtgtgtctggggatgtttttggatgtcaccagtaccaggtgctactggtatcttgtggggagagttgaggaagctgcttaacatcctccaatgcccaggacagtcgccacctcaaagaattatctggccccaaatagctcaacagtactgaggttgagaaaccctggcttagaatgaacatctctttatccttctcttcctttagatcttgacttaaatgtcacctcctcagaaagacctttgtcagcagctctcccacagtataccctctcccatgtttctggtcccccgtgagttttctttccatagatctacatgagttgcaaatttatatatttgtggttgacttgcttcttgtctctcttccccattgggctttaggcttcagaacaggtgagacattgtatcactcatcactgaatgcccagggtctaacacatagtagatgctcaacaaatcacccactgaatgaatggttggtgaagaaatctctgtcagagaggacagaggttcactgaattccagacaaacccagaatgccagcatctgtgtgaggacacaaagacctctcttctaccttgttcatcctgtcgcccaccactcagaaaaggcctctggttattgttggcctgtatttatttcctcctgatatcctggtaccagcctttccaaaattctcactgtagtgctggaggtcagggtatttttaaactagaagaactagccaagctggttttttttttttaagtggtggaaaagaaaaactaagatttgtttttaatcattagactttcaaatttaagaaggcgcgatgcaaatagcatgttggcataaacaagtgctgcccgctcaatggagggagggagcctttcttctgagctaatttaagctaaatacatggcagctatttttcatctctacaattgtgcaactttctcctcagtttacaatacaggggagatattatcgggcagaagttggatgggggataagtgaagacgagaaggaaaagaagaggcagtggacaagaaggtactctcagccaccgagctggtgattagaggtatttcaagagctcaggagtagagctggtggtccactaggacctcaagatcttatctgggtggaaacttgattttgagccttccattcagggaagaaaccaaagagcaattggagtcaggctccttttcctgccctttatatgcagcaccccctgacttcccagaagcccagactgaacagcagaaattttacaaacctcctcaagaaagaaaagcccttgcagctctcctgcacaccaccacgcacactgttattccttaaggcccccatatgccgtgacttccagcccagctgttactagactgggcatagcattcaggccttgtggtgaagccgtcccagaagataaatgatttttctccaagcaggcagattaccgagtaggatcatacacagagtcttagagacagaatctttctttctgcattttccaagttccctaactgagaagaaacatctgcagagcgctgatagactgtccaccaactacagcccaaatggcttggcttctggaagtttctgaggcctgagttctaaacctacctctgcctcttagaagggacctgacttaggggagtttattatagcttccctctctgggcctcagatcctgcttctgtgaaaggagaagagtgagataagggagggtcactcatatccatcttaagtggtaactcgaatgccctgaagctacatctgtgatcagtgggaaggcatgctgtgatggattagtgatgtctgccaagagtacagcaggggacactggtggtagatccattacatatttgtactccttggaccagatctttatccttctagatcttagaggtccttctagatcaccatcccaatgacttggttgaagatgaaaactcaggtgaaaacttaacccttctgagggtgttacatcttatatacttttcacattggcctccaagccatggtatgttggagaagccaccaacacacagcagatttgacccctccattggaagacaccatcagccagatgtggtgttcttgttcatggaaccactgtccacatggatggaatcgggctctaagctacctttctcatctcctagcagtgtctatgaatgctagtggtcagctcttttctgtgggccagtacattgacattgcctccttcagtaccaggtaaggtatcaagtctcattcacagaggttgaccttgttggagattcagaaacaagcctgggaaagcttgggaagaacagcctcctatcaggcatttagagattcaaccacacaatagtgtcttaaaagttctgataagtcctgcaatcaagaaattagtttcattttacctaagcatttccaatgcatgcttgtcccaggaccctttcaataatgcaaatccggcgagttttccatggaatgaaaggtctatgggacatgcttgggaaacaaggtcttatttagatcaggcacattctagacagagtccatctcctccagctcagtcctcagtggaaggaggacagccattctcaaccccatgagatgaatccttcatattcttggtgttaggaaatgggagctgcatgatcccaatgagtgggaaggaagggccctttcccacccctgagagggaagagcactcactgatgtacgcctctcaggaacacgggaccacagtgcaacatccagcaggagagacggaggggataggaagcctggagcagggatactggagggacccaggagggactctgccaacccagatgtacatttcctggaaatccgggctgctgctggcagcctgtcagtttgagaacataagttcaagcttccgtgcaaactcccagtatggtccctgccagcccctgcaccctcccttccacaacttcctgcttttcctctctctctttcctggttccaagttgccaataagtctcagaggctgggattgtaacatccccatgagcagctggacatgaaccccttgacctggaggtgggttcctgggaatggatgagcccaaagactcgtttttaaaatgctgggtctgcaatttggaggctggtttctgtccctgtaccacagttgccccattggaacgagaataagactactgatctccccaaaccatcataggaattccagcctggcacgtagtaagtgctctgtgaatgagggctgttcagggtggattgttactctgcctcctagacatcctgggccacctgactcaatgggtcgcttcatacgtcacagatattaaacctggcaaactggctcagcacaatggcttagccctgtaatcccagtgctttgggaggctgaagcagggggattgcttgagaccaggagttcaagaccagcgcgggcaacatagcaagaccctgtctgtacaacaaataaaaaattagccaggcatgatggtgtgcacctgtagtaccagcaacttgagaggctaaggtgggaggattgcttgtggccaggagttcgaggctgcagtgagctatgatcacgctgtactccagcctgggtgacagagcaagactctaactctaaaccacaacaacaaacctaacaaacaaactcattggggttgatatggcacccacaacatggtctggcaaaggggaatcccaataccatccagccctgccaatggtgcccttctaactccctgtgccagggtcttactcttacccagcaaacctctctgtctgcattctgtaaacatttcttgagcacttactatgtgccaggcactactaagacaagtccaggaggtcactgggaccgcagattttccatcaacctcctgccccactactggtttcaaaactaaactggtaacagaatgggtatggattgcagggcctcgagaagggagtctgggatttgggttaatatcatagtcaggcactgaccagagaggacagaggttcactgcggctccacattccaggacccagactgacatttgctgcctgtcactccccttggagttcaaagtgattcccttgcaggtgtgtgcaggtgagggtgaggtggtacgggaggaggtgaggctgggagccagggagagtggccacatgagtctgcctaggaacttccccacatcacaggcaaagccaaaaaaggaaacagcaaaatgtagctcatcaaaatccactcctttgtcaatgaacaagagtatagataaaatcagatgctgtgtcaccaactgctttggatagggtcatgaggcacattcaggggtcaagtgacagtccgctacagacaagccacttacacacaggctgttcccatacagccacagaactgagatccagagctgttggaattcagtgatgggacgtgttgattggggcaagcttggtaagcatgacagcaacagcctgaccttgtagaccaggaattctggggaatctatcttcaagggcacctgggttctacagtggaggaccagtcaaggcacaagagaaaatgtcttagagggtgttataagttgtggtgtccccaacaaaaaaaaaaaaaaaaaaaaaaagacatgttgaagtcctcattcctagtacctcagaatgagacttcatttggagagagggtctttgcagatataattagttaagatgaggtcatactgaaatagggtgggcccttaatccaatgtgactcgtgtccttataagaagatggccatatgaagatagggacacacagagagatgatgagggcagggattggactgacacagctgcaagccaaggaatgccaatgatgaccaggaaagcaccaggaattcagaagccgccaggaaggattcccttacagatttcagggggaacatggccctgctaacactttgattttggacttctggcatccagatgggtgagagatgatacatctgttgttgtaggccccagtgggtggtggtttgctgcagcagtcctaggagcctcacggaggtgaggggggcttggggatatggtggcacagtggaacaagaccagcctgcaggggatggatgggtgaagtgaaggtaggcacaggatgaggatagggagggcatatttcgggactcaagattgagaaccagtgtggggaaagaaagccggggatgggaataaaatcacagagcgttggaaccctaatctaataagattgttgtctttatcagaagaggaggagatactggggatgtgcagtcacagaggaaaggccacgtgaggtcacgatcagagggcagctgtctgcaagccaaagaaagaggcctcaccagaaaccaaccctgctgacaccttgatcttgggacttccagcctcaagaattgtgaggaataaattcgtgttgtttaagccactcagtgtgtgacattttgttattatggccccccttagcaaacgaagagttttaaagtccagggagttggtccagccttcagggcctgaattgcctccatatcacacaggccaagcagtcaacatctgctccaccctatccaaggacagggagttctctacttccggaggcagcccgctgcatcttggggcaagctggccttcttccgctgaaacaagttctctccccctccaacttcctgttcctcccctgagagccatatccaaccctctctatcaaaggctcctgttcctcccctgacagccatatccaatcctctctatcaaaggctagcaaagttaggaaagggccagattgtaaaagtttttgactgtgtgggccacatcgtctctgttgcaaatagctggctctgtcacagttgcataggagcagccgtggttgtgtaaatggagaggtgactgtgctccaataacattttgtttattgacatgaaatttgaatgttatagaattttcatgtcatgaaatattattcttttgatttttcctcaattaaaacatgtaaaaaccatttggcaggctgggtatggcctatggggcatagcctgacagccctgggtttagatttctcaagataatgattggcctgagctccgtgtctactacttcctccgtgtacctttgatgatcagctgtaggtggggatgggaatggtggaaggtgagataaggctggtttcgtgtgtttgtggggaggggcatgatgtgtgtatatggcatgggaggtgagaaaaagggaagaactaggttccctggatacaaaagtctagtggtcaatatcagtcaagggcttctattgactgacaatccaaggtagctgtggagacaagtggatggggtgaggatgggggggtccatggcaagatgaaaattttctctttgatcagtaaaaggaataccaggacaaaatggatctaagcaatgactttgggtttccagcttggctctggggatggggacacaaggggcacgtcctcccacagggggccaagaaggaagctccttggttttatgaataatctgtatcctggaagagttgggtgaaatttatgtgcaaatccacatgccctttaaagaaagctgagatgtttctctctgcaaagccaaggcttcctggtgaatcttcaccctgtggactggtcccctcgggaagcccatgtatatgacggtttgctaaaagcaagactgactggaacaactcgctgctgagtcagtgacttatgtgtacagggcacctgtgtgcagctgtgatgggacaagggcaaacacacaaatcttggtcgtgtcattgtatagaatgagttgcaggtgaggctggtaattatgatgtaaaaatatacagcctctttcctctttttttttcctccctgcgtaagatgaatataacctcctcccaaaacctcatcagcgaataaagatggaagccagcagggaaagcagcggtttggttcttcctggatttaaatgtgtgcaaattaaagctggtttctcaacaagtcagggcggtgtagaggggacagggtaggggcgtcaggaaggcactgaaggccaggatcctggcctggctgcagcagagaccaatgcaggtggggacagagtagtgaagtggggaaagatcgagaagtcaagagcaagtgactcagattcagggatggacccaaggcaccctgttccacaaagggctgggttttcccctggatcactcaggccctgtccttaatcccaaactggtgctcatgaatgaatggaaaaatcagctgttggagatcatgctaggccttgccaaaggctgtggttggacattttagttaattctggaaacaagagaggcaagagtgagaaggtgccagttcttgtggacatttcagctgcagggtagtagaccctggctgcctcttcccttcctcatatcctgtctcttggcacaagggaacatgacaaggactggagcctgtggacccaagaagtcctggtgtgatggaagagaagtgagtggttgggtttcaggcactcagtaggctgctgggcagagccaagacaggtgcaagtccaggcccagggctgggacacagagtgttgtgttgggatggggaggtgtccattgacaagagccatccccagcaaccccagagtggctggggctcaggcaaacatatataaaatgcctccaagacacacacacgtcgtcaagccaagagccatagatgtccccagaagagcagtgtctgcttaggagcagcccaagccggggtctttagtcctctagtcccagtaagctgggagtgttggaaaggcaattcaggagggccctttgggaaacacaggggtttcctgtagccaggctcctgggaagcatgactgatctcaccattcttcccggtttggaagcaggtttggcccccagagcatgaaccagtctgggagtcacccaaggtggggaagagatcctcataggtctatttggattttgaaagtaagatcaggtagggtttttgaagttccagttcctctctctggccctctaggagggagatgcctggatagatagtagctacaagaaaactaaggcccaggtagtacccaggaaacacagaggggctgtggccgccctgggcttcctgttcactgcccagataatcctgctattgctctgcttggggacagatttcccttttgtatcaggtcacatgcagggggtcagggctttgaaaacatgggcaaatgacccagaggttctcctctcccatctgcatgcccagcctgctctcggcatccttcctacagatacagaacaccaggggcttccccaacatggtcaggaagagtcgccggcccaggttgggatcaagaggagggagggaaggtggggcactgagggaacacacacaggtgagggacacaggcttccgatggggaagctacttgaggaccccgcaccaggctagagcaaagaacgcagaagtgtaacaaacatcctccctttgtgctcccccaacaggactcctcaagggtgacaggcagggaaatcttttgcaaacgtgttatcataggtacagccacataacccaacatggacgtaccccaagaacccgcatccaccttggtgggggaataagcttcactggtgtgagtagcagagaagagggaagaaaaggaatgtcctagaactccctgcccagagccctgattctcagggaccagacttcagggggtgccctgaatgacggtgagctctaaggagcccctcagaagtcatcttggctttccaaatggcaaggaggtgcgggcagtgaggtgaaaagggatgctactctcagagaacaggagaaaacagcagaaatgggggaataggtcccccagagagacccagaactcaaaagacgttctaactttcctactgtacttcagagctctatgcaaaggtgccacacgccatgacaggctcgggttggggtgtctgaaaacagatatttccaaaggaacgagcttagccactcccgaccttccctgctcgatcttggctcagtagccttgactaagctgccactcggctctgtaccctcctcttagcttcccagatggtacagctggaacctaccacatacagacagaactgaggagtgccccgtcattgggacagtctggctcttgcttgtcaaggggaaacaagagtgaacaacgtcaaacacacagacacacacacacatagccccgtctgtgagcccccccacgtggggtctcctgtcctagtcccatagcccaaaggcaccacgtgcagcctgcagtgctctcattagtgctgtcccctgggccgcactgatcaataacgcatcaccctggctggtccggttcagtcctagctcgggggtccccaaccctgcccgaggaaaagggctcaagtctgaggtgcagggaggccgccgagcagttgtccagtgctcccaggtcggtcggggttggtaccctctgatgctgagtctctggcctcctgagctggcagaggacagagtagggagggagaggtgacgggagcccaggcagctgggcgccgtcccgatgtccaaaggtcacagctctgcagacttccagaaatgtccagggtgagacaggcgacggtttcgctttggcagtttctccagcatgtccatgagcttggtgaaggtaggtctctcttcttgttcaaaggcccagcagaagagaagaatgtccgagatttcttttcccatgccaatctggctgaggttgggtttcatgcctgtgcccatttgccagattattgcctctgctggttgggtcttgaaaggccattccctggcgtggagttcataccagattgtgccaagggcaaagacgtcagagtgcttggagaaggggagcttatcctcctctgtgtcgggggacagctggcggatgatctctggtgccaggtggcatagccagccattctggatgcgcagtttgtcctcccgcctgccagcctgcagcaccccagaaatgctgaagagtccaaagtccgtgatgaccactttgccgttgtcatagaagacgttctttgacttgaggtccttgtgtaggattcccttggcgtggaggtagcccatgcccttcacaatttcttgagcaatctgcctggttttgttgacatccaaaacgattttggcatccctcacaacggaatagagcgtccgtcccttacagaggctggtgatgatggccaggtgaggcgggctcatgcaggcacccatgaaaagcaccacgttctcatgccgtgtctgcctgtaggccatcacctcccgcttgaaggccttgagctggtcctcgttgtccctctcaatgtcaatcagccggatggccacctcgccatgccagcggccgtggtacacttgcccaaagcggccctttccaatgagctcgccgatctccagctgctcaaaggggatgtcccactcctgaaggaagatgctggtctggctggccttgcgtgggaagctccgggccgagaggagggacaggttcatctcctcgaagtcatcctctgactcttcggcctcatcatggacctcttcattctccgacgttggctccacttcaatttgaagtaatggatttccttccaagattggattcgaggtcaccggatgcaggatgacctggggcgcccgggtcggcgtctccggcaccggcaccacatctgggaagatgaactgctgcttgtatttgtagtagtgggatgctggcaggttgaagttcttctgctgccgtgtgcactgtggggaagggtgtaggggagaaggcggcgtggcactaggagggagggggggtgctggcgaggagggcgtggaggacgtcgtggaggaggggttgctgctggagtctggctggtaagggacagggatgtggtccttgttgattttgttggttttggggagcgtctgactgatgtgcaggtctgaatagcgaggtggcttccgtagagggttgttgatgtcacacggaacggactctgtccggactaaccttgctggatctcctcggtggatgatcagaagatgacagggtggggcttctttggtgcatttgttgtggcactttaaccttactaggggaacgaacatgggtctcactcctacagaagtgggcagtaacctcaattgcagtttttacacttgaggc

SEQ ID NO: 18156 - RNA, 16668 nt, Homo sapiens
  source 1..16668: mol_type = other RNA
tgaaggtctactgtgtgccaggtattgcgtaacgttattgacattcattatttcattcactccctccaataaactcaagggttagtgatatattaagtgctcgtgggttgcacaaagctaagaaaattcaaggaatactctggaggggctgctgatgctgagaaagtgttgatgaaatcattatccacaatagacagtggctcaagaaatgcaaattgagtcaagttgaagcagataaacaagcctcgctaatttgcagtagccacatataccctgggagtctggcggtcagcaaagatgctttgttttctgtctttcaaaccctgacatatttatagagacagcaaacacaccactccatcaacaggactgatacattctttcccacacttcaggctgtattgcaggcttggcctgtggcccactatggcccctaggtcttcttcagtcatttctgtaacaaaccagcattttgcccatcatacctgaaatgtttagttagagaccctcagtgtagggtctttccataaatacatttccacgttcacacatgtccttgacctcaacacttcaggggcctattcatagagtgatatgaactgtcccagaaagaggttttttgctgaagaaggttttttggtatggcaagacagaactgggggccccagagacatcagagacacaggtcgcaagagtcgatagagggaaagtgaagcaaaagaggaacaggaatgaaaaatgcattagagagaagggctcatggccaacccatctatagccaagatgcccatggacttcaggacccaatgcagggcactaagaaatagagacacatccttcactgtgtggaggcaggcagagacagagacagacacagagacagacagacagagagagagagagagagagagagagagagagagagaggtctgtagagccagagagggatgcagagcaggcctgaggtggcctgagtactggtctgactccagcaagcacaaaactctcctcagacatcttcccccacaggacaccaaggctaacagtaggaaccagagcatgctggggaaagaagtcaaggtctccacatctgagccagggcaccctctgtttggagatggagactccagggtcccaaaatcaggctttggggaaagcagggaaaggcaggcaagtgccagggggcaggattttagccacttgcagttaccctcaataaatcatgatcttgcctctgagtccacacataggctgttccttctgtctgacacaccgttccctaccattctactcaaatttcaagacagggttcagaagtctcctcctctgagaatccttcctggagggtctttctctgggttgggagctcctgtggggcctcgggaccctactggaactcctccctctcttcatcggactcctagtaccctgaaggcagcacccacttttctccattttttccagaatcacaggaggcacttaacaaatatttactaaatgactatataaaatgaagatttggggaatgaagggacaaggttgctccacgctgggctctgctgagggtgtagtgaatggggctggggacatgagcctttgaaatacaagcaaaattttcttagaatccttcggctgctcaactgtaggcatttgaaatccaccaatgtacccaaaaatagggctatgaggaaactagaggaccggggcccagaagcagtgccttgtggaatatgggacagctatgggagctcatggagaacagagactccaaattggatgccatcttggaagtggagtcagagaagctcatgtgacagcatgcctgacatgccaccatatgggcttctggcctctgtgctccaagccttggggctttatgaggattgattccagacgcaaagtcagggtgtgttttgatggggtggggagtacaatctatgatattccttgataggttaggaccgcagaggccctcaggaggagatagacttccgaaaagaaggaagaaggagccaggcaaagatttatgcatcacacagttgggcagaagcctgaccaaggacagcccctcccttaatgctccagtcgagccaggactgtccagatagctttgaaggggcagggtgtgcagtgctccctagaaggctggctaggagggaaagggggccggggcagggggcctcggtgtggcagggcaagtaccttagagtaccttgatgcccatgctgtagctacatagcagttacttgaacttacacaagttcatatgtacccatctaaacattattacttgtaacacatgtagaaaaataagcagaggaaaatggctagaatcttacaggaccaatacattacatttgttgtccaggacgcacttaagctgccaatgccccaacctgggcagggctgtgttggggagaggttgaccccatctagggcagagccccagccaactcaactgtcttcttggaaggtgtcccaattcccaaagcaattttccaagatctggtcttttgcagtgcccgactcgtcctctctgttacccttcccaatcctgggactgccggaagctccagggatttgattctaggggtaaaacagctggacctacagaggccatcctcacccactgcctgtctccatgcccaaatcagtcacacgggactggacagaactgccacatcttgtccagactgtctatgttgttgcttcattgctaccagagacagccattctaacccggcctgactctcttcttcacagtgaactgggaattgcaaggaaggtagaaaaggcccttcactatctgggagactttccttcctggggaatacagaagggctttccctgagtagcctcagaaagcaacaccaagattgccggatgcaagtctcaagatttcagctcagcaagaggatctgcttcttagaagggctgtggaaggatggagagaatgactggagatttcagcccctgtccgtgcagacggtgaaaggcaagtccacattctccttacctagacagccttcaaaccactggtgatgctaactagtgctttaaaaacctatttccctgcaatgttcacttaaggagtcccctccttgtgttttcctgttctcctctgatttcctttctcccatggaaggttgcagatggcaggatgctggatttgaatcctagtcgcgtggcctggagacaactcaggggacatctggcaatgtctggagatggttttggatgtcacactttggatgtcaactggaggcttttgaaatccaccaacatacccaaaaatagggctatgctggaactagaggaccgtggcccagaagcaatgccttgtggaatatgggacagctatgggagctcatggagaacagagactccaaactggatgccatatcagaagtgggggtcagagaagctcaggtgacaccatgcctgacatgccaccatatgggcttccagcctctgtgctccaaggcttggggctttatgaggattgattccagacagcaaagtcagggtgtgtctggggatgtttttggatgtcaccagtaccaggtgctactggtatcttgtggggagagttgaggaagctgcttaacatcctccaatgcccaggacagtcgccacctcaaagaattatctggccccaaatagctcaacagtactgaggttgagaaaccctggcttagaatgaacatctctttatccttctcttcctttagatcttgacttaaatgtcacctcctcagaaagacctttgtcagcagctctcccacagtataccctctcccatgtttctggtcccccgtgagttttctttccatagatctacatgagttgcaaatttatatatttgtggttgacttgcttcttgtctctcttccccattgggctttaggcttcagaacaggtgagacattgtatcactcatcactgaatgcccagggtctaacacatagtagatgctcaacaaatcacccactgaatgaatggttggtgaagaaatctctgtcagagaggacagaggttcactgaattccagacaaacccagaatgccagcatctgtgtgaggacacaaagacctctcttctaccttgttcatcctgtcgcccaccactcagaaaaggcctctggttattgttggcctgtatttatttcctcctgatatcctggtaccagcctttccaaaattctcactgtagtgctggaggtcagggtatttttaaactagaagaactagccaagctggttttttttttttaagtggtggaaaagaaaaactaagatttgtttttaatcattagactttcaaatttaagaaggcgcgatgcaaatagcatgttggcataaacaagtgctgcccgctcaatggagggagggagcctttcttctgagctaatttaagctaaatacatggcagctatttttcatctctacaattgtgcaactttctcctcagtttacaatacaggggagatattatcgggcagaagttggatgggggataagtgaagacgagaaggaaaagaagaggcagtggacaagaaggtactctcagccaccgagctggtgattagaggtatttcaagagctcaggagtagagctggtggtccactaggacctcaagatcttatctgggtggaaacttgattttgagccttccattcagggaagaaaccaaagagcaattggagtcaggctccttttcctgccctttatatgcagcaccccctgacttcccagaagcccagactgaacagcagaaattttacaaacctcctcaagaaagaaaagcccttgcagctctcctgcacaccaccacgcacactgttattccttaaggcccccatatgccgtgacttccagcccagctgttactagactgggcatagcattcaggccttgtggtgaagccgtcccagaagataaatgatttttctccaagcaggcagattaccgagtaggatcatacacagagtcttagagacagaatctttctttctgcattttccaagttccctaactgagaagaaacatctgcagagcgctgatagactgtccaccaactacagcccaaatggcttggcttctggaagtttctgaggcctgagttctaaacctacctctgcctcttagaagggacctgacttaggggagtttattatagcttccctctctgggcctcagatcctgcttctgtgaaaggagaagagtgagataagggagggtcactcatatccatcttaagtggtaactcgaatgccctgaagctacatctgtgatcagtgggaaggcatgctgtgatggattagtgatgtctgccaagagtacagcaggggacactggtggtagatccattacatatttgtactccttggaccagatctttatccttctagatcttagaggtccttctagatcaccatcccaatgacttggttgaagatgaaaactcaggtgaaaacttaacccttctgagggtgttacatcttatatacttttcacattggcctccaagccatggtatgttggagaagccaccaacacacagcagatttgacccctccattggaagacaccatcagccagatgtggtgttcttgttcatggaaccactgtccacatggatggaatcgggctctaagctacctttctcatctcctagcagtgtctatgaatgctagtggtcagctcttttctgtgggccagtacattgacattgcctccttcagtaccaggtaaggtatcaagtctcattcacagaggttgaccttgttggagattcagaaacaagcctgggaaagcttgggaagaacagcctcctatcaggcatttagagattcaaccacacaatagtgtcttaaaagttctgataagtcctgcaatcaagaaattagtttcattttacctaagcatttccaatgcatgcttgtcccaggaccctttcaataatgcaaatccggcgagttttccatggaatgaaaggtctatgggacatgcttgggaaacaaggtcttatttagatcaggcacattctagacagagtccatctcctccagctcagtcctcagtggaaggaggacagccattctcaaccccatgagatgaatccttcatattcttggtgttaggaaatgggagctgcatgatcccaatgagtgggaaggaagggccctttcccacccctgagagggaagagcactcactgatgtacgcctctcaggaacacgggaccacagtgcaacatccagcaggagagacggaggggataggaagcctggagcagggatactggagggacccaggagggactctgccaacccagatgtacatttcctggaaatccgggctgctgctggcagcctgtcagtttgagaacataagttcaagcttccgtgcaaactcccagtatggtccctgccagcccctgcaccctcccttccacaacttcctgcttttcctctctctctttcctggttccaagttgccaataagtctcagaggctgggattgtaacatccccatgagcagctggacatgaaccccttgacctggaggtgggttcctgggaatggatgagcccaaagactcgtttttaaaatgctgggtctgcaatttggaggctggtttctgtccctgtaccacagttgccccattggaacgagaataagactactgatctccccaaaccatcataggaattccagcctggcacgtagtaagtgctctgtgaatgagggctgttcagggtggattgttactctgcctcctagacatcctgggccacctgactcaatgggtcgcttcatacgtcacagatattaaacctggcaaactggctcagcacaatggcttagccctgtaatcccagtgctttgggaggctgaagcagggggattgcttgagaccaggagttcaagaccagcgcgggcaacatagcaagaccctgtctgtacaacaaataaaaaattagccaggcatgatggtgtgcacctgtagtaccagcaacttgagaggctaaggtgggaggattgcttgtggccaggagttcgaggctgcagtgagctatgatcacgctgtactccagcctgggtgacagagcaagactctaactctaaaccacaacaacaaacctaacaaacaaactcattggggttgatatggcacccacaacatggtctggcaaaggggaatcccaataccatccagccctgccaatggtgcccttctaactccctgtgccagggtcttactcttacccagcaaacctctctgtctgcattctgtaaacatttcttgagcacttactatgtgccaggcactactaagacaagtccaggaggtcactgggaccgcagattttccatcaacctcctgccccactactggtttcaaaactaaactggtaacagaatgggtatggattgcagggcctcgagaagggagtctgggatttgggttaatatcatagtcaggcactgaccagagaggacagaggttcactgcggctccacattccaggacccagactgacatttgctgcctgtcactccccttggagttcaaagtgattcccttgcaggtgtgtgcaggtgagggtgaggtggtacgggaggaggtgaggctgggagccagggagagtggccacatgagtctgcctaggaacttccccacatcacaggcaaagccaaaaaaggaaacagcaaaatgtagctcatcaaaatccactcctttgtcaatgaacaagagtatagataaaatcagatgctgtgtcaccaactgctttggatagggtcatgaggcacattcaggggtcaagtgacagtccgctacagacaagccacttacacacaggctgttcccatacagccacagaactgagatccagagctgttggaattcagtgatgggacgtgttgattggggcaagcttggtaagcatgacagcaacagcctgaccttgtagaccaggaattctggggaatctatcttcaagggcacctgggttctacagtggaggaccagtcaaggcacaagagaaaatgtcttagagggtgttataagttgtggtgtccccaacaaaaaaaaaaaaaaaaaaaaaaagacatgttgaagtcctcattcctagtacctcagaatgagacttcatttggagagagggtctttgcagatataattagttaagatgaggtcatactgaaatagggtgggcccttaatccaatgtgactcgtgtccttataagaagatggccatatgaagatagggacacacagagagatgatgagggcagggattggactgacacagctgcaagccaaggaatgccaatgatgaccaggaaagcaccaggaattcagaagccgccaggaaggattcccttacagatttcagggggaacatggccctgctaacactttgattttggacttctggcatccagatgggtgagagatgatacatctgttgttgtaggccccagtgggtggtggtttgctgcagcagtcctaggagcctcacggaggtgaggggggcttggggatatggtggcacagtggaacaagaccagcctgcaggggatggatgggtgaagtgaaggtaggcacaggatgaggatagggagggcatatttcgggactcaagattgagaaccagtgtggggaaagaaagccggggatgggaataaaatcacagagcgttggaaccctaatctaataagattgttgtctttatcagaagaggaggagatactggggatgtgcagtcacagaggaaaggccacgtgaggtcacgatcagagggcagctgtctgcaagccaaagaaagaggcctcaccagaaaccaaccctgctgacaccttgatcttgggacttccagcctcaagaattgtgaggaataaattcgtgttgtttaagccactcagtgtgtgacattttgttattatggccccccttagcaaacgaagagttttaaagtccagggagttggtccagccttcagggcctgaattgcctccatatcacacaggccaagcagtcaacatctgctccaccctatccaaggacagggagttctctacttccggaggcagcccgctgcatcttggggcaagctggccttcttccgctgaaacaagttctctccccctccaacttcctgttcctcccctgagagccatatccaaccctctctatcaaaggctcctgttcctcccctgacagccatatccaatcctctctatcaaaggctagcaaagttaggaaagggccagattgtaaaagtttttgactgtgtgggccacatcgtctctgttgcaaatagctggctctgtcacagttgcataggagcagccgtggttgtgtaaatggagaggtgactgtgctccaataacattttgtttattgacatgaaatttgaatgttatagaattttcatgtcatgaaatattattcttttgatttttcctcaattaaaacatgtaaaaaccatttggcaggctgggtatggcctatggggcatagcctgacagccctgggtttagatttctcaagataatgattggcctgagctccgtgtctactacttcctccgtgtacctttgatgatcagctgtaggtggggatgggaatggtggaaggtgagataaggctggtttcgtgtgtttgtggggaggggcatgatgtgtgtatatggcatgggaggtgagaaaaagggaagaactaggttccctggatacaaaagtctagtggtcaatatcagtcaagggcttctattgactgacaatccaaggtagctgtggagacaagtggatggggtgaggatgggggggtccatggcaagatgaaaattttctctttgatcagtaaaaggaataccaggacaaaatggatctaagcaatgactttgggtttccagcttggctctggggatggggacacaaggggcacgtcctcccacagggggccaagaaggaagctccttggttttatgaataatctgtatcctggaagagttgggtgaaatttatgtgcaaatccacatgccctttaaagaaagctgagatgtttctctctgcaaagccaaggcttcctggtgaatcttcaccctgtggactggtcccctcgggaagcccatgtatatgacggtttgctaaaagcaagactgactggaacaactcgctgctgagtcagtgacttatgtgtacagggcacctgtgtgcagctgtgatgggacaagggcaaacacacaaatcttggtcgtgtcattgtatagaatgagttgcaggtgaggctggtaattatgatgtaaaaatatacagcctctttcctctttttttttcctccctgcgtaagatgaatataacctcctcccaaaacctcatcagcgaataaagatggaagccagcagggaaagcagcggtttggttcttcctggatttaaatgtgtgcaaattaaagctggtttctcaacaagtcagggcggtgtagaggggacagggtaggggcgtcaggaaggcactgaaggccaggatcctggcctggctgcagcagagaccaatgcaggtggggacagagtagtgaagtggggaaagatcgagaagtcaagagcaagtgactcagattcagggatggacccaaggcaccctgttccacaaagggctgggttttcccctggatcactcaggccctgtccttaatcccaaactggtgctcatgaatgaatggaaaaatcagctgttggagatcatgctaggccttgccaaaggctgtggttggacattttagttaattctggaaacaagagaggcaagagtgagaaggtgccagttcttgtggacatttcagctgcagggtagtagaccctggctgcctcttcccttcctcatatcctgtctcttggcacaagggaacatgacaaggactggagcctgtggacccaagaagtcctggtgtgatggaagagaagtgagtggttgggtttcaggcactcagtaggctgctgggcagagccaagacaggtgcaagtccaggcccagggctgggacacagagtgttgtgttgggatggggaggtgtccattgacaagagccatccccagcaaccccagagtggctggggctcaggcaaacatatataaaatgcctccaagacacacacacgtcgtcaagccaagagccatagatgtccccagaagagcagtgtctgcttaggagcagcccaagccggggtctttagtcctctagtcccagtaagctgggagtgttggaaaggcaattcaggagggccctttgggaaacacaggggtttcctgtagccaggctcctgggaagcatgactgatctcaccattcttcccggtttggaagcaggtttggcccccagagcatgaaccagtctgggagtcacccaaggtggggaagagatcctcataggtctatttggattttgaaagtaagatcaggtagggtttttgaagttccagttcctctctctggccctctaggagggagatgcctggatagatagtagctacaagaaaactaaggcccaggtagtacccaggaaacacagaggggctgtggccgccctgggcttcctgttcactgcccagataatcctgctattgctctgcttggggacagatttcccttttgtatcaggtcacatgcagggggtcagggctttgaaaacatgggcaaatgacccagaggttctcctctcccatctgcatgcccagcctgctctcggcatccttcctacagatacagaacaccaggggcttccccaacatggtcaggaagagtcgccggcccaggttgggatcaagaggagggagggaaggtggggcactgagggaacacacacaggtgagggacacaggcttccgatggggaagctacttgaggaccccgcaccaggctagagcaaagaacgcagaagtgtaacaaacatcctccctttgtgctcccccaacaggactcctcaagggtgacaggcagggaaatcttttgcaaacgtgttatcataggtacagccacataacccaacatggacgtaccccaagaacccgcatccaccttggtgggggaataagcttcactggtgtgagtagcagagaagagggaagaaaaggaatgtcctagaactccctgcccagagccctgattctcagggaccagacttcagggggtgccctgaatgacggtgagctctaaggagcccctcagaagtcatcttggctttccaaatggcaaggaggtgcgggcagtgaggtgaaaagggatgctactctcagagaacaggagaaaacagcagaaatgggggaataggtcccccagagagacccagaactcaaaagacgttctaactttcctactgtacttcagagctctatgcaaaggtgccacacgccatgacaggctcgggttggggtgtctgaaaacagatatttccaaaggaacgagcttagccactcccgaccttccctgctcgatcttggctcagtagccttgactaagctgccactcggctctgtaccctcctcttagcttcccagatggtacagctggaacctaccacatacagacagaactgaggagtgccccgtcattgggacagtctggctcttgcttgtcaaggggaaacaagagtgaacaacgtcaaacacacagacacacacacacatagccccgtctgtgagcccccccacgtggggtctcctgtcctagtcccatagcccaaaggcaccacgtgcagcctgcagtgctctcattagtgctgtcccctgggccgcactgatcaataacgcatcaccctggctggtccggttcagtcctagctcgggggtccccaaccctgcccgaggaaaagggctcaagtctgaggtgcagggaggccgccgagcagttgtccagtgctcccaggtcggtcggggttggtaccctctgatgctgagtctctggcctcctgagctggcagaggacagagtagggagggagaggtgacgggagcccaggcagctgggcgccgtcccgatgtccaaaggtcacagctctgcagacttccagaaatgtccagggtgagacaggcgacggtttcgctttggcagtttctccagcatgtccatgagcttggtgaaggtaggtctctcttcttgttcaaaggcccagcagaagagaagaatgtccgagatttcttttcccatgccaatctggctgaggttgggtttcatgcctgtgcccatttgccagattattgcctctgctggttgggtcttgaaaggccattccctggcgtggagttcataccagattgtgccaagggcaaagacgtcagagtgcttggagaaggggagcttatcctcctctgtgtcgggggacagctggcggatgatctctggtgccaggtggcatagccagccattctggatgcgcagtttgtcctcccgcctgccagcctgcagcaccccagaaatgctgaagagtccaaagtccgtgatgaccactttgccgttgtcatagaagacgttctttgacttgaggtccttgtgtaggattcccttggcgtggaggtagcccatgcccttcacaatttcttgagcaatctgcctggttttgttgacatccaaaacgattttggcatccctcacaacggaatagagcgtccgtcccttacagaggctggtgatgatggccaggtgaggcgggctcatgcaggcacccatgaaaagcaccacgttctcatgccgtgtctgcctgtaggccatcacctcccgcttgaaggccttgagctggtcctcgttgtccctctcaatgtcaatcagccggatggccacctcgccatgccagcggccgtggtacacttgcccaaagcggccctttccaatgagctcgccgatctccagctgctcaaaggggatgtcccactcctgaaggaagatgctggtctggctggccttgcgtgggaagctccgggccgagaggagggacaggttcatctcctcgaagtcatcctctgactcttcggcctcatcatggacctcttcattctccgacgttggctccacttcaatttgaagtaatggatttccttccaagattggattcgaggtcaccggatgcaggatgacctggggcgcccgggtcggcgtctccggcaccggcaccacatctgggaagatgaactgctgcttgtatttgtagtagtgggatgctggcaggttgaagttcttctgctgccgtgtgcactgtggggaagggtgtaggggagaaggcggcgtggcactaggagggagggggggtgctggcgaggagggcgtggaggacgtcgtggaggaggggttgctgctggagtctggctggtaagggacagggatgtggtccttgttgattttgttggttttggggagcgtctgactgatgtgcaggtctgaatagcgaggtggcttccgtagagggttgttgatgtcacacggaacggactctgtccggactaaccttgctggatctcctcggtggatgatcagaagatgacagggtggggcttctttggtgcatttgttgtggcactttaacttgcagtttttacacttgaggccaaaaagcatccctttcccacagactgtgcacgtctgagacatccagtacttggtggaaaacctgtgcttgatggagttgccgagatctctgcgagggatctgcggggaccagcgtggcactgacagtgtgtttgcagagaagttggcctcagtgtgaacaggaggggtggaaggcaggaaaggtgcgtgtcccacaaagaaggagcggagggagcgctcggacagcagcggggagcgctgctgagaggggatgttctcgcagctgcctacgctgctgtggatcttgaggttcaagggtttgctcttcttcttggctttgggcgtgtgggcctcgtccacgcggtgccccagctggaactcgtgggatttgctccgatgcagcgcggtgaatcccgggatcaagtgtatcagttttcgggaggagggcggtggggtccccgggggcttcagcttgttcttcttcctcatgggcggcgtgcccggcggggtcacggtggtgacgatgttgggggtgcgcggcggggtgcggaccgcgtgccgctgccggggcgatgggggcagggaacggtggcccgactccagtggcgggggcgggcacaagcccgggtaggcgtccacggtaagcctgtccacgtgggtgtacacaggggccccgggagtggggctggtgtgacaatagtgctggacgcacttggacgggaccctggggctctgggagagatgggtgcggatccacggggtgggctccggggggcacacgggattgttctccttccccgtctctgtcgtgggccactggatggtccagtcttgtttggaaaggttgcctcctgacatgtggacattcctgaggcaggagagggaggcgttgaggcgggcacactcctcccggttggctccgtatttctccacagtctcgcacacctgttcatccgtcatctccaagaggtcctccaggctcagctggccgggggagatttcctccaggacctccttgcgcacatcgacgattcggaaccagtgccgtagctgggggaagccgtccagctccgcgttgcgctcctgcaaggctaccttctttttgcaggacagctgccggctgaagtacttcaccagcttgctcggcgagagctcttctgtcagctttaggcataaacagccctttccgttccttcaggtgtcacctctgcccaagctcctctcaatgccaccatcacgccgccctgctttctttccttggtggcactttgctatctcacaaatcatcctgtttattggtttccatggttacgcctcccccccaccaccaccacacacccatcatgtcagctcaagagagcacgggctttgcctgtcatttccccagcgttcagatccgtgcctggcatacagtcggtgctcaatacatttttcttggtctttcaataaaccaacatccttggtggttaaacgccaggccactaaaaataaatcccaagtccttttccaagcgggcacagtgcacctgcaggaccgggtccctggttgtgttattaaggttctcgggtgagcagaccccgtgcgggtaatgaaatcgcggcagccacagccagcagccccgacgccttcccgccgttgccagggcgaccattgtcataacatccctggcgcttggcggcccagctgacgggggagagaattatttgactggagaacgtctcaagtaaccggccaatttgcatccacaagaaaatcccctgctgagggagggctggaggcctgggagaggcgcccttccttctctccccagccctggatcccaatgagaaccggatccctgaggccaggcagagggacccaacagtctggggcagtcccgccgaatgctggaacacaggcagctgcctctgcaggaaggaagagcccccctctccgctgtctcactattgctgatggtttttccttttctctacgttattactgctgatggatattacaaacaatagaaaaaagggtttatatatttaatgagcacttactagacagcaggtccagtagtaataacttccttacacgatccttata

SEQ ID NO: 18157 - RNA, 16641 nt, Homo sapiens
  source 1..16641: mol_type = other RNA
tgaaggtctactgtgtgccaggtattgcgtaacgttattgacattcattatttcattcactccctccaataaactcaagggttagtgatatattaagtgctcgtgggttgcacaaagctaagaaaattcaaggaatactctggaggggctgctgatgctgagaaagtgttgatgaaatcattatccacaatagacagtggctcaagaaatgcaaattgagtcaagttgaagcagataaacaagcctcgctaatttgcagtagccacatataccctgggagtctggcggtcagcaaagatgctttgttttctgtctttcaaaccctgacatatttatagagacagcaaacacaccactccatcaacaggactgatacattctttcccacacttcaggctgtattgcaggcttggcctgtggcccactatggcccctaggtcttcttcagtcatttctgtaacaaaccagcattttgcccatcatacctgaaatgtttagttagagaccctcagtgtagggtctttccataaatacatttccacgttcacacatgtccttgacctcaacacttcaggggcctattcatagagtgatatgaactgtcccagaaagaggttttttgctgaagaaggttttttggtatggcaagacagaactgggggccccagagacatcagagacacaggtcgcaagagtcgatagagggaaagtgaagcaaaagaggaacaggaatgaaaaatgcattagagagaagggctcatggccaacccatctatagccaagatgcccatggacttcaggacccaatgcagggcactaagaaatagagacacatccttcactgtgtggaggcaggcagagacagagacagacacagagacagacagacagagagagagagagagagagagagagagagagagagaggtctgtagagccagagagggatgcagagcaggcctgaggtggcctgagtactggtctgactccagcaagcacaaaactctcctcagacatcttcccccacaggacaccaaggctaacagtaggaaccagagcatgctggggaaagaagtcaaggtctccacatctgagccagggcaccctctgtttggagatggagactccagggtcccaaaatcaggctttggggaaagcagggaaaggcaggcaagtgccagggggcaggattttagccacttgcagttaccctcaataaatcatgatcttgcctctgagtccacacataggctgttccttctgtctgacacaccgttccctaccattctactcaaatttcaagacagggttcagaagtctcctcctctgagaatccttcctggagggtctttctctgggttgggagctcctgtggggcctcgggaccctactggaactcctccctctcttcatcggactcctagtaccctgaaggcagcacccacttttctccattttttccagaatcacaggaggcacttaacaaatatttactaaatgactatataaaatgaagatttggggaatgaagggacaaggttgctccacgctgggctctgctgagggtgtagtgaatggggctggggacatgagcctttgaaatacaagcaaaattttcttagaatccttcggctgctcaactgtaggcatttgaaatccaccaatgtacccaaaaatagggctatgaggaaactagaggaccggggcccagaagcagtgccttgtggaatatgggacagctatgggagctcatggagaacagagactccaaattggatgccatcttggaagtggagtcagagaagctcatgtgacagcatgcctgacatgccaccatatgggcttctggcctctgtgctccaagccttggggctttatgaggattgattccagacgcaaagtcagggtgtgttttgatggggtggggagtacaatctatgatattccttgataggttaggaccgcagaggccctcaggaggagatagacttccgaaaagaaggaagaaggagccaggcaaagatttatgcatcacacagttgggcagaagcctgaccaaggacagcccctcccttaatgctccagtcgagccaggactgtccagatagctttgaaggggcagggtgtgcagtgctccctagaaggctggctaggagggaaagggggccggggcagggggcctcggtgtggcagggcaagtaccttagagtaccttgatgcccatgctgtagctacatagcagttacttgaacttacacaagttcatatgtacccatctaaacattattacttgtaacacatgtagaaaaataagcagaggaaaatggctagaatcttacaggaccaatacattacatttgttgtccaggacgcacttaagctgccaatgccccaacctgggcagggctgtgttggggagaggttgaccccatctagggcagagccccagccaactcaactgtcttcttggaaggtgtcccaattcccaaagcaattttccaagatctggtcttttgcagtgcccgactcgtcctctctgttacccttcccaatcctgggactgccggaagctccagggatttgattctaggggtaaaacagctggacctacagaggccatcctcacccactgcctgtctccatgcccaaatcagtcacacgggactggacagaactgccacatcttgtccagactgtctatgttgttgcttcattgctaccagagacagccattctaacccggcctgactctcttcttcacagtgaactgggaattgcaaggaaggtagaaaaggcccttcactatctgggagactttccttcctggggaatacagaagggctttccctgagtagcctcagaaagcaacaccaagattgccggatgcaagtctcaagatttcagctcagcaagaggatctgcttcttagaagggctgtggaaggatggagagaatgactggagatttcagcccctgtccgtgcagacggtgaaaggcaagtccacattctccttacctagacagccttcaaaccactggtgatgctaactagtgctttaaaaacctatttccctgcaatgttcacttaaggagtcccctccttgtgttttcctgttctcctctgatttcctttctcccatggaaggttgcagatggcaggatgctggatttgaatcctagtcgcgtggcctggagacaactcaggggacatctggcaatgtctggagatggttttggatgtcacactttggatgtcaactggaggcttttgaaatccaccaacatacccaaaaatagggctatgctggaactagaggaccgtggcccagaagcaatgccttgtggaatatgggacagctatgggagctcatggagaacagagactccaaactggatgccatatcagaagtgggggtcagagaagctcaggtgacaccatgcctgacatgccaccatatgggcttccagcctctgtgctccaaggcttggggctttatgaggattgattccagacagcaaagtcagggtgtgtctggggatgtttttggatgtcaccagtaccaggtgctactggtatcttgtggggagagttgaggaagctgcttaacatcctccaatgcccaggacagtcgccacctcaaagaattatctggccccaaatagctcaacagtactgaggttgagaaaccctggcttagaatgaacatctctttatccttctcttcctttagatcttgacttaaatgtcacctcctcagaaagacctttgtcagcagctctcccacagtataccctctcccatgtttctggtcccccgtgagttttctttccatagatctacatgagttgcaaatttatatatttgtggttgacttgcttcttgtctctcttccccattgggctttaggcttcagaacaggtgagacattgtatcactcatcactgaatgcccagggtctaacacatagtagatgctcaacaaatcacccactgaatgaatggttggtgaagaaatctctgtcagagaggacagaggttcactgaattccagacaaacccagaatgccagcatctgtgtgaggacacaaagacctctcttctaccttgttcatcctgtcgcccaccactcagaaaaggcctctggttattgttggcctgtatttatttcctcctgatatcctggtaccagcctttccaaaattctcactgtagtgctggaggtcagggtatttttaaactagaagaactagccaagctggttttttttttttaagtggtggaaaagaaaaactaagatttgtttttaatcattagactttcaaatttaagaaggcgcgatgcaaatagcatgttggcataaacaagtgctgcccgctcaatggagggagggagcctttcttctgagctaatttaagctaaatacatggcagctatttttcatctctacaattgtgcaactttctcctcagtttacaatacaggggagatattatcgggcagaagttggatgggggataagtgaagacgagaaggaaaagaagaggcagtggacaagaaggtactctcagccaccgagctggtgattagaggtatttcaagagctcaggagtagagctggtggtccactaggacctcaagatcttatctgggtggaaacttgattttgagccttccattcagggaagaaaccaaagagcaattggagtcaggctccttttcctgccctttatatgcagcaccccctgacttcccagaagcccagactgaacagcagaaattttacaaacctcctcaagaaagaaaagcccttgcagctctcctgcacaccaccacgcacactgttattccttaaggcccccatatgccgtgacttccagcccagctgttactagactgggcatagcattcaggccttgtggtgaagccgtcccagaagataaatgatttttctccaagcaggcagattaccgagtaggatcatacacagagtcttagagacagaatctttctttctgcattttccaagttccctaactgagaagaaacatctgcagagcgctgatagactgtccaccaactacagcccaaatggcttggcttctggaagtttctgaggcctgagttctaaacctacctctgcctcttagaagggacctgacttaggggagtttattatagcttccctctctgggcctcagatcctgcttctgtgaaaggagaagagtgagataagggagggtcactcatatccatcttaagtggtaactcgaatgccctgaagctacatctgtgatcagtgggaaggcatgctgtgatggattagtgatgtctgccaagagtacagcaggggacactggtggtagatccattacatatttgtactccttggaccagatctttatccttctagatcttagaggtccttctagatcaccatcccaatgacttggttgaagatgaaaactcaggtgaaaacttaacccttctgagggtgttacatcttatatacttttcacattggcctccaagccatggtatgttggagaagccaccaacacacagcagatttgacccctccattggaagacaccatcagccagatgtggtgttcttgttcatggaaccactgtccacatggatggaatcgggctctaagctacctttctcatctcctagcagtgtctatgaatgctagtggtcagctcttttctgtgggccagtacattgacattgcctccttcagtaccaggtaaggtatcaagtctcattcacagaggttgaccttgttggagattcagaaacaagcctgggaaagcttgggaagaacagcctcctatcaggcatttagagattcaaccacacaatagtgtcttaaaagttctgataagtcctgcaatcaagaaattagtttcattttacctaagcatttccaatgcatgcttgtcccaggaccctttcaataatgcaaatccggcgagttttccatggaatgaaaggtctatgggacatgcttgggaaacaaggtcttatttagatcaggcacattctagacagagtccatctcctccagctcagtcctcagtggaaggaggacagccattctcaaccccatgagatgaatccttcatattcttggtgttaggaaatgggagctgcatgatcccaatgagtgggaaggaagggccctttcccacccctgagagggaagagcactcactgatgtacgcctctcaggaacacgggaccacagtgcaacatccagcaggagagacggaggggataggaagcctggagcagggatactggagggacccaggagggactctgccaacccagatgtacatttcctggaaatccgggctgctgctggcagcctgtcagtttgagaacataagttcaagcttccgtgcaaactcccagtatggtccctgccagcccctgcaccctcccttccacaacttcctgcttttcctctctctctttcctggttccaagttgccaataagtctcagaggctgggattgtaacatccccatgagcagctggacatgaaccccttgacctggaggtgggttcctgggaatggatgagcccaaagactcgtttttaaaatgctgggtctgcaatttggaggctggtttctgtccctgtaccacagttgccccattggaacgagaataagactactgatctccccaaaccatcataggaattccagcctggcacgtagtaagtgctctgtgaatgagggctgttcagggtggattgttactctgcctcctagacatcctgggccacctgactcaatgggtcgcttcatacgtcacagatattaaacctggcaaactggctcagcacaatggcttagccctgtaatcccagtgctttgggaggctgaagcagggggattgcttgagaccaggagttcaagaccagcgcgggcaacatagcaagaccctgtctgtacaacaaataaaaaattagccaggcatgatggtgtgcacctgtagtaccagcaacttgagaggctaaggtgggaggattgcttgtggccaggagttcgaggctgcagtgagctatgatcacgctgtactccagcctgggtgacagagcaagactctaactctaaaccacaacaacaaacctaacaaacaaactcattggggttgatatggcacccacaacatggtctggcaaaggggaatcccaataccatccagccctgccaatggtgcccttctaactccctgtgccagggtcttactcttacccagcaaacctctctgtctgcattctgtaaacatttcttgagcacttactatgtgccaggcactactaagacaagtccaggaggtcactgggaccgcagattttccatcaacctcctgccccactactggtttcaaaactaaactggtaacagaatgggtatggattgcagggcctcgagaagggagtctgggatttgggttaatatcatagtcaggcactgaccagagaggacagaggttcactgcggctccacattccaggacccagactgacatttgctgcctgtcactccccttggagttcaaagtgattcccttgcaggtgtgtgcaggtgagggtgaggtggtacgggaggaggtgaggctgggagccagggagagtggccacatgagtctgcctaggaacttccccacatcacaggcaaagccaaaaaaggaaacagcaaaatgtagctcatcaaaatccactcctttgtcaatgaacaagagtatagataaaatcagatgctgtgtcaccaactgctttggatagggtcatgaggcacattcaggggtcaagtgacagtccgctacagacaagccacttacacacaggctgttcccatacagccacagaactgagatccagagctgttggaattcagtgatgggacgtgttgattggggcaagcttggtaagcatgacagcaacagcctgaccttgtagaccaggaattctggggaatctatcttcaagggcacctgggttctacagtggaggaccagtcaaggcacaagagaaaatgtcttagagggtgttataagttgtggtgtccccaacaaaaaaaaaaaaaaaaaaaaaaagacatgttgaagtcctcattcctagtacctcagaatgagacttcatttggagagagggtctttgcagatataattagttaagatgaggtcatactgaaatagggtgggcccttaatccaatgtgactcgtgtccttataagaagatggccatatgaagatagggacacacagagagatgatgagggcagggattggactgacacagctgcaagccaaggaatgccaatgatgaccaggaaagcaccaggaattcagaagccgccaggaaggattcccttacagatttcagggggaacatggccctgctaacactttgattttggacttctggcatccagatgggtgagagatgatacatctgttgttgtaggccccagtgggtggtggtttgctgcagcagtcctaggagcctcacggaggtgaggggggcttggggatatggtggcacagtggaacaagaccagcctgcaggggatggatgggtgaagtgaaggtaggcacaggatgaggatagggagggcatatttcgggactcaagattgagaaccagtgtggggaaagaaagccggggatgggaataaaatcacagagcgttggaaccctaatctaataagattgttgtctttatcagaagaggaggagatactggggatgtgcagtcacagaggaaaggccacgtgaggtcacgatcagagggcagctgtctgcaagccaaagaaagaggcctcaccagaaaccaaccctgctgacaccttgatcttgggacttccagcctcaagaattgtgaggaataaattcgtgttgtttaagccactcagtgtgtgacattttgttattatggccccccttagcaaacgaagagttttaaagtccagggagttggtccagccttcagggcctgaattgcctccatatcacacaggccaagcagtcaacatctgctccaccctatccaaggacagggagttctctacttccggaggcagcccgctgcatcttggggcaagctggccttcttccgctgaaacaagttctctccccctccaacttcctgttcctcccctgagagccatatccaaccctctctatcaaaggctcctgttcctcccctgacagccatatccaatcctctctatcaaaggctagcaaagttaggaaagggccagattgtaaaagtttttgactgtgtgggccacatcgtctctgttgcaaatagctggctctgtcacagttgcataggagcagccgtggttgtgtaaatggagaggtgactgtgctccaataacattttgtttattgacatgaaatttgaatgttatagaattttcatgtcatgaaatattattcttttgatttttcctcaattaaaacatgtaaaaaccatttggcaggctgggtatggcctatggggcatagcctgacagccctgggtttagatttctcaagataatgattggcctgagctccgtgtctactacttcctccgtgtacctttgatgatcagctgtaggtggggatgggaatggtggaaggtgagataaggctggtttcgtgtgtttgtggggaggggcatgatgtgtgtatatggcatgggaggtgagaaaaagggaagaactaggttccctggatacaaaagtctagtggtcaatatcagtcaagggcttctattgactgacaatccaaggtagctgtggagacaagtggatggggtgaggatgggggggtccatggcaagatgaaaattttctctttgatcagtaaaaggaataccaggacaaaatggatctaagcaatgactttgggtttccagcttggctctggggatggggacacaaggggcacgtcctcccacagggggccaagaaggaagctccttggttttatgaataatctgtatcctggaagagttgggtgaaatttatgtgcaaatccacatgccctttaaagaaagctgagatgtttctctctgcaaagccaaggcttcctggtgaatcttcaccctgtggactggtcccctcgggaagcccatgtatatgacggtttgctaaaagcaagactgactggaacaactcgctgctgagtcagtgacttatgtgtacagggcacctgtgtgcagctgtgatgggacaagggcaaacacacaaatcttggtcgtgtcattgtatagaatgagttgcaggtgaggctggtaattatgatgtaaaaatatacagcctctttcctctttttttttcctccctgcgtaagatgaatataacctcctcccaaaacctcatcagcgaataaagatggaagccagcagggaaagcagcggtttggttcttcctggatttaaatgtgtgcaaattaaagctggtttctcaacaagtcagggcggtgtagaggggacagggtaggggcgtcaggaaggcactgaaggccaggatcctggcctggctgcagcagagaccaatgcaggtggggacagagtagtgaagtggggaaagatcgagaagtcaagagcaagtgactcagattcagggatggacccaaggcaccctgttccacaaagggctgggttttcccctggatcactcaggccctgtccttaatcccaaactggtgctcatgaatgaatggaaaaatcagctgttggagatcatgctaggccttgccaaaggctgtggttggacattttagttaattctggaaacaagagaggcaagagtgagaaggtgccagttcttgtggacatttcagctgcagggtagtagaccctggctgcctcttcccttcctcatatcctgtctcttggcacaagggaacatgacaaggactggagcctgtggacccaagaagtcctggtgtgatggaagagaagtgagtggttgggtttcaggcactcagtaggctgctgggcagagccaagacaggtgcaagtccaggcccagggctgggacacagagtgttgtgttgggatggggaggtgtccattgacaagagccatccccagcaaccccagagtggctggggctcaggcaaacatatataaaatgcctccaagacacacacacgtcgtcaagccaagagccatagatgtccccagaagagcagtgtctgcttaggagcagcccaagccggggtctttagtcctctagtcccagtaagctgggagtgttggaaaggcaattcaggagggccctttgggaaacacaggggtttcctgtagccaggctcctgggaagcatgactgatctcaccattcttcccggtttggaagcaggtttggcccccagagcatgaaccagtctgggagtcacccaaggtggggaagagatcctcataggtctatttggattttgaaagtaagatcaggtagggtttttgaagttccagttcctctctctggccctctaggagggagatgcctggatagatagtagctacaagaaaactaaggcccaggtagtacccaggaaacacagaggggctgtggccgccctgggcttcctgttcactgcccagataatcctgctattgctctgcttggggacagatttcccttttgtatcaggtcacatgcagggggtcagggctttgaaaacatgggcaaatgacccagaggttctcctctcccatctgcatgcccagcctgctctcggcatccttcctacagatacagaacaccaggggcttccccaacatggtcaggaagagtcgccggcccaggttgggatcaagaggagggagggaaggtggggcactgagggaacacacacaggtgagggacacaggcttccgatggggaagctacttgaggaccccgcaccaggctagagcaaagaacgcagaagtgtaacaaacatcctccctttgtgctcccccaacaggactcctcaagggtgacaggcagggaaatcttttgcaaacgtgttatcataggtacagccacataacccaacatggacgtaccccaagaacccgcatccaccttggtgggggaataagcttcactggtgtgagtagcagagaagagggaagaaaaggaatgtcctagaactccctgcccagagccctgattctcagggaccagacttcagggggtgccctgaatgacggtgagctctaaggagcccctcagaagtcatcttggctttccaaatggcaaggaggtgcgggcagtgaggtgaaaagggatgctactctcagagaacaggagaaaacagcagaaatgggggaataggtcccccagagagacccagaactcaaaagacgttctaactttcctactgtacttcagagctctatgcaaaggtgccacacgccatgacaggctcgggttggggtgtctgaaaacagatatttccaaaggaacgagcttagccactcccgaccttccctgctcgatcttggctcagtagccttgactaagctgccactcggctctgtaccctcctcttagcttcccagatggtacagctggaacctaccacatacagacagaactgaggagtgccccgtcattgggacagtctggctcttgcttgtcaaggggaaacaagagtgaacaacgtcaaacacacagacacacacacacatagccccgtctgtgagcccccccacgtggggtctcctgtcctagtcccatagcccaaaggcaccacgtgcagcctgcagtgctctcattagtgctgtcccctgggccgcactgatcaataacgcatcaccctggctggtccggttcagtcctagctcgggggtccccaaccctgcccgaggaaaagggctcaagtctgaggtgcagggaggccgccgagcagttgtccagtgctcccaggtcggtcggggttggtaccctctgatgctgagtctctggcctcctgagctggcagaggacagagtagggagggagaggtgacgggagcccaggcagctgggcgccgtcccgatgtccaaaggtcacagctctgcagacttccagaaatgtccagggtgagacaggcgacggtttcgctttggcagtttctccagcatgtccatgagcttggtgaaggtaggtctctcttcttgttcaaaggcccagcagaagagaagaatgtccgagatttcttttcccatgccaatctggctgaggttgggtttcatgcctgtgcccatttgccagattattgcctctgctggttgggtcttgaaaggccattccctggcgtggagttcataccagattgtgccaagggcaaagacgtcagagtgcttggagaaggggagcttatcctcctctgtgtcgggggacagctggcggatgatctctggtgccaggtggcatagccagccattctggatgcgcagtttgtcctcccgcctgccagcctgcagcaccccagaaatgctgaagagtccaaagtccgtgatgaccactttgccgttgtcatagaagacgttctttgacttgaggtccttgtgtaggattcccttggcgtggaggtagcccatgcccttcacaatttcttgagcaatctgcctggttttgttgacatccaaaacgattttggcatccctcacaacggaatagagcgtccgtcccttacagaggctggtgatgatggccaggtgaggcgggctcatgcaggcacccatgaaaagcaccacgttctcatgccgtgtctgcctgtaggccatcacctcccgcttgaaggccttgagctggtcctcgttgtccctctcaatgtcaatcagccggatggccacctcgccatgccagcggccgtggtacacttgcccaaagcggccctttccaatgagctcgccgatctccagctgctcaaaggggatgtcccactcctgaaggaagatgctggtctggctggccttgcgtgggaagctccgggccgagaggagggacaggttcatctcctcgaagtcatcctctgactcttcggcctcatcatggacctcttcattctccgacgttggctccacttcaatttgaagtaatggatttccttccaagattggattcgaggtcaccggatgcaggatgacctggggcgcccgggtcggcgtctccggcaccggcaccacatctgggaagatgaactgctgcttgtatttgtagtagtgggatgctggcaggttgaagttcttctgctgccgtgtgcactgtggggaagggtgtaggggagaaggcggcgtggcactaggagggagggggggtgctggcgaggagggcgtggaggacgtcgtggaggaggggttgctgctggagtctggctggtaagggacagggatgtggtccttgttgattttgttggttttggggagcgtctgactgatgtgcaggtctgaatagcgaggtggcttccgtagagggttgttgatgtcacacggaacggactctgtccggactaaccttgctggatctcctcggtggatgatcagaagatgacagggtggggcttctttggtgcatttgttgtggcactttaacttgcagtttttacacttgaggccaaaaagcatccctttcccacagactgtgcacgtctgagacatccagtacttggtggaaaacctgtgcttgatggagttgccgagatctctgcgagggatctgcggggaccagcgtggcactgacagtgtgtttgcagagaagttggcctcagtgtgaacaggaggggtggaaggcaggaaaggtgcgtgtcccacaaagaaggagcggagggagcgctcggacagcagcggggagcgctgctgagaggggatgttctcgcagctgcctacgctgctgtggatcttgaggttcaagggtttgctcttcttcttggctttgggcgtgtgggcctcgtccacgcggtgccccagctggaactcgtgggatttgctccgatgcagcgcggtgaatcccgggatcaagtgtatcagttttcgggaggagggcggtggggtccccgggggcttcagcttgttcttcttcctcatgggcggcgtgcccggcggggtcacggtggtgacgatgttgggggtgcgcggcggggtgcggaccgcgtgccgctgccggggcgatgggggcagggaacggtggcccgactccagtggcgggggcgggcacaagcccgggtaggcgtccacggtaagcctgtccacgtgggtgtacacaggggccccgggagtggggctggtgtgacaatagtgctggacgcacttggacgggaccctggggctctgggagagatgggtgcggatccacggggtgggctccggggggcacacgggattgttctccttccccgtctctgtcgtgggccactggatggtccagtcttgtttggaaaggttgcctcctgacatgtggacattcctgaggcaggagagggaggcgttgaggcgggcacactcctcccggttggctccgtatttctccacagtctcgcacacctgttcatccgtcatctccaagaggtcctccaggctcagctggccgggggagatttcctccaggacctccttgcgcacatcgacgattcggaaccagtgccgtagctgggggaagccgtccagctccgcgttgcgctcctgcaaggctaccttctttttgcaggacagctgccggctgaagtacttcaccagcttgctctccagggtccggatttctttttgtgtgaggtcgttggaggtagcacatttggtcctaagcccttccaggttggagatgctcaagtctatcatgttttggaccagttcgcactgctgtaaggctttttgcaaactcagaggctgctgctcctcgcttttcgtcatgttttcctcatccatcgcttgctctgcaacccccttcccctcctcctcctcccagagagaaaaaagaggggggggagtagaggtagtctaccctccgcctctccaaccactgcgacttctcaacaatgtctcatgaagaagaaatccaacatctcacacagggttgagggggtgggagtgggaggaggggacaagagccaaaatttattattttattttgggatatcaagcggactccattagaatgtctcctctctctctgagtctctggtccctgaaaaggagagatgctgtttctcagaagcaaaccaggtgatgtgatgctgtctgtacacttagggaggaggaggaggaggaaaaagaagaggagaaggaggagagagaggaggagggagaggaggaggagggagaggaggaggaggagaaggaaaatagcgctcactctttacacaccggctccttgaaggacaaaattatatatttttggctggcttgcttttatgtcaaaaaaaatctggttttcccccctcccagttgcagggacacggcatggtccacggtttggagtgctttagcgcgttctcaaggtgctgtctgcattgctcccgcggctgcggcggctactgcggctggctgctgtctcctccccgcgctgctgctgctgctgctgctgccgccgccgggctccgggggtgacggttgctgcaatcgctcctgcctcgctccacaccgacatcttgcctgtcaatc

SEQ ID NO: 18158 - RNA, 3061 nt, Homo sapiens
  source 1..3061: mol_type = other RNA
tgaaggtctactgtgtgccaggtgcaccacactagatgcaacggatactaacagtaaataagatacggtccctgccctcagagcttacatttcaacagtttaaagtgcatctcaggtatttcagataacagaagtaattctaccactctcaaatttttttttttaatgcaagacacaacacaatcataggccagagttataaaatacaatgttagaaagaaacgtttggtatcattcgtccagatcccattttacagaaaagaaactacaggagtggccatttgcacctatgttctgatttcaagtttggtgttttacccattgccaggcctctcataaaacaatattcagatttgccatgtatatatcaatatccaaacgctggtagtatacctgtgcagttgtctcctgctagacaaggaccatataatttatagcttatttaagtgtccactttctttatcccatcctattctttgtgataaaccagagggatcaggcttaaccaagtgctgaactttggggcaacttcatgccctaggattcaagatggccagcggctacatgccgggtctgcctgccaggaccttacttcccattttttgcagttttcctggactgccgggaggcagctgtacaagctttataagcctcaggctgtaagtgaacttgctttctgcattttccagccatgtgccattgaccaggagtgaactcaagtataaattgcaaagggctacttgtcaagatgacaaatatctatcctactgtttcaactatgaacatattctgaaatgccatatgccaggcgccataccagatactagggacataaatatgaaaaagtctttgcccctcaggagtaatattggttgtactggaacatttgtagctgaaggaaaatctccaaaaaagatttcaaagagactaaagtaggaatgggtgctggagaatgagcaagaagggtgagagtcccacgggtgaagggagaaagcagcagagaatgaatataagcccggagaatgaacataaatgtgaggggaagaggccagaggccaacactggaaggacagtgagggccaagaaaggaactactaatgtttctgagacctgcagggaaccatggtattaagctctcattaccagcacctaattttttagaggctggttttccaacttaagtgaaagaaattcaccctgtttttagcaattatgacgcactatatttacttctgtcacattagctgattctgtggtggactgggtaatttgaaaagctcctttgaacatgaattgtttttaaacttacagtctagcaataagcctaatttttaaaacagaatgcttaatttctccctgtacaatcagtaagattttgatttttaacaagtttacatgtccaattacatgtagataaaaggaatgaaaaccagtaaagacaccttttataatctgaaaatagatttttaaaccttcctttaatgtgaaattttctctttaatgtgttatgaattctatcaaatataaccatttaggattatttatagtatgtcactgatcacttctactagtatagacaaataaatttataaacattattttgaatgtaactaattagcataattttatttaagagttagactgtgttgtcaatactgacatttttgggaatatatagtatagtttatgagtcaagcttctgaaccaaaagttttactttgagccctattcctaccttacaagctagcaggtgaccttgggcaagccaacctattagaaccctgggttcacgtccatacagtgaagacatcataacctgtcctacctacttcacaagcttcctctaccgatcaactagatcaatatatgtaagattttttttgacaactgtaaagtactataaaatgacacttacagataagtcagtgaagttaaccatcaaaacaatattcatgcctataaccaaaagcttttaaacaaaacagcttaataaaaagtggtcaggtaagcaaataaagattatattacacaaactatgttcctcacctactctcatactgagtctaatctttggaaagataattcattttaaggggaaaaaaatctgttaagatattttttagtatttatacaaacaagctgcaactactattcaaaaataggtttttttcatccaataggagtatactctttaatagaactgtatttgaataagaattccatacaaatagaatatataccttaacacaagaaagcaagaaaagaatattttacattacatagaacattcaggtgattcgatcaaattatccctccaactaaatacttattttccctatttactacaaatattgcagtcagtcagtatatgccaataatcatatagttttaacatctagtagtgtgaagtacacttgactgtttccaaagggagagaggtgatgtagtcttcatttcaggggagaagaatggactgaattactgtctgctttttaatgtttcaactaaccattccattgcctcatcaaggccggtgcctttggttgctgacgttttgaatatctgccattttcggtccttcaaggcaggtaacccaagtgaatttgccatctctgaggaagtcatggcctgttccatgtcctgtttatttgcaaacaccactaaaatggcttttctcagctcttcttcctccaacatggcaactaactctgatttggaaatgccaattcggtctcggtcacaactgtctactacataaatgactgcatctgtgtttgaatagtaacatctccagtatggcctgatacttgtctgtcctcctaaatcccagacttggaatttaaggtttttgtacgtcaccgtctctacattaaatccaatggccatgatgaaccccctgtcctccctcgccgatcttcagtgattccttggccttcggctgcagctccgaggcggtttcctcgcaagcccagtcagccagcaacttccacgtcggactccaggcgggggcgggagcgagggtcagctgcgactgcgcgccgggaacggtggcctgagcatc

SEQ ID NO: 18159 - RNA, 3151 nt, Homo sapiens
  source 1..3151: mol_type = other RNA
tgaaggtctactgtgtgccaggtgcaccacactagatgcaacggatactaacagtaaataagatacggtccctgccctcagagcttacatttcaacagtttaaagtgcatctcaggtatttcagataacagaagtaattctaccactctcaaatttttttttttaatgcaagacacaacacaatcataggccagagttataaaatacaatgttagaaagaaacgtttggtatcattcgtccagatcccattttacagaaaagaaactacaggagtggccatttgcacctatgttctgatttcaagtttggtgttttacccattgccaggcctctcataaaacaatattcagatttgccatgtatatatcaatatccaaacgctggtagtatacctgtgcagttgtctcctgctagacaaggaccatataatttatagcttatttaagtgtccactttctttatcccatcctattctttgtgataaaccagagggatcaggcttaaccaagtgctgaactttggggcaacttcatgccctaggattcaagatggccagcggctacatgccgggtctgcctgccaggaccttacttcccattttttgcagttttcctggactgccgggaggcagctgtacaagctttataagcctcaggctgtaagtgaacttgctttctgcattttccagccatgtgccattgaccaggagtgaactcaagtataaattgcaaagggctacttgtcaagatgacaaatatctatcctactgtttcaactatgaacatattctgaaatgccatatgccaggcgccataccagatactagggacataaatatgaaaaagtctttgcccctcaggagtaatattggttgtactggaacatttgtagctgaaggaaaatctccaaaaaagatttcaaagagactaaagtaggaatgggtgctggagaatgagcaagaagggtgagagtcccacgggtgaagggagaaagcagcagagaatgaatataagcccggagaatgaacataaatgtgaggggaagaggccagaggccaacactggaaggacagtgagggccaagaaaggaactactaatgtttctgagacctgcagggaaccatggtattaagctctcattaccagcacctaattttttagaggctggttttccaacttaagtgaaagaaattcaccctgtttttagcaattatgacgcactatatttacttctgtcacattagctgattctgtggtggactgggtaatttgaaaagctcctttgaacatgaattgtttttaaacttacagtctagcaataagcctaatttttaaaacagaatgcttaatttctccctgtacaatcagtaagattttgatttttaacaagtttacatgtccaattacatgtagataaaaggaatgaaaaccagtaaagacaccttttataatctgaaaatagatttttaaaccttcctttaatgtgaaattttctctttaatgtgttatgaattctatcaaatataaccatttaggattatttatagtatgtcactgatcacttctactagtatagacaaataaatttataaacattattttgaatgtaactaattagcataattttatttaagagttagactgtgttgtcaatactgacatttttgggaatatatagtatagtttatgagtcaagcttctgaaccaaaagttttactttgagccctattcctaccttacaagctagcaggtgaccttgggcaagccaacctattagaaccctgggttcacgtccatacagtgaagacatcataacctgtcctacctacttcacaagcttcctctaccgatcaactagatcaatatatgtaagattttttttgacaactgtaaagtactataaaatgacacttacagataagtcagtgaagttaaccatcaaaacaatattcatgcctataaccaaaagcttttaaacaaaacagcttaataaaaagtggtcaggtaagcaaataaagattatattacacaaactatgttcctcacctactctcatactgagtctaatctttggaaagataattcattttaaggggaaaaaaatctgttaagatattttttagtatttatacaaacaagctgcaactactattcaaaaataggtttttttcatccaataggagtatactctttaatagaactgtatttgaataagaattccatacaaatagaatatataccttaacacaagaaagcaagaaaagaatattttacattacatagaacattcaggtgattcgatcaaattatccctccaactaaatacttattttccctatttactacaaatattgcagtcagtcagtatatgccaataatcatatagttttaacatctagtagtgtgaagtacacttgactgtttccaaagggagagaggtgatgtagtcttcatttcaggggagaagaatggactgaattactgtctgctttttaatgtttcaactaaccattccattgcctcatcaaggccggtgcctttggttgctgacgttttgaatatctgccattttcggtccttcaaggcaggtaacccaagtgaatttgccatctctgaggaagtcatggcctgttccatgtcctgtttatttgcaaacaccactaaaatggcttttctcagctcttcttcctccaacatggcaactaactctgatttggaaatgccaattcggtctcggtcacaactgtctactacataaatgactgcatctgtgtttgaatagtaacatctccagtatggcctgatacttgtctgtcctcctaaatcccagacttggaatttaaggtttttgtacgtcaccgtctctacattaaatccaatggtaggtatagtagtaacaacttctcccacttgtaatctgtacaaaattgtggtttttcctgctccatctaatcccaaaattaaaattctcatttcccgagttccaaacagactggaaaatatacttgagaaaaagccacccatgatgaaccccctgtcctccctcgccgatcttcagtgattccttggccttcggctgcagctccgaggcggtttcctcgcaagcccagtcagccagcaacttccacgtcggactccaggcgggggcggg

SEQ ID NO: 18160 - RNA, 4860 nt, Homo sapiens
  source 1..4860: mol_type = other RNA
tgaaggtctactgtgtgccaggttccaggctagattgtttacattgtttcattgaatatgcccaaaagcccaaggtcagttttgtcatttccactttatttattcagaaactgagacccaaagaggttcacacatctatcaagtggagaacccaaatacaagcccaatttaatctggctctaaagcccacgctctttcccctgggccaatctctgtgctggacaggtatcacactggctgcagcaggttcatgacaggggatgtggtcactgattctgcccatctgtcccatcagagtaaaccttgggtcttgctgttgaatgagtccaagtcacagcacataactcacacctcacattggtctgttccttcttaaccatcacatcagacaaaaggcagcattgtgccctcttacctctcttgaagaagaggagaccactatctgtctccccttattcctctgtagtaatttttgagctagacaagtggccaagccaaagactatacttcccagggtttcttgcagctgagtgtagccatgtgactatcaagatgtgagcagacttaatgtgtgccatgagtttggatgtgtgccttgagttttgatgttttgatgtgtgtcttgagttttgcctttaaaggaaggaaagagcgttttcacatcttcttgctgtctggaatttagatctgatggtaggtgttgaaggtggcttctagaagctggaaaaaggcaaggaaagataatcctcccgagagcctcagccagccctgccgacattgagacctaacccagtgacgatgattttggacttcccacctccagaactgtaaaataataaatttgtgttgttctaaggcattaagttggagaaacttattatggctgcaataggaaatataatgggggaatccagataaaaggagaatccagtccatgaaggaaagggcatgccagggtgaagcaataacgctgttctgcatgctcccaaatcccatcagtgatcttctccccaaccttcaaggtccagcagcagcctcctctcagaagccttcctggaccacaccaagcaactggcttccatgctgatctcatcagagaaactacatactggtatagaaagatagggcctcttggggaggaagtgaatgtagccccagccctgctaatccagagcctagcacaagctgcccttccttgtggaacacctggcaccatagttaccatctgtgcagaccatggtgccttggagtttcagccattcagaagaacaaagtaggcccaaaggaggaaagaaggaggtacacaggcagtattccttctagcgaggctagtgtgtgttggcctgaaggcccaacaggcaagatctatctctccaaaggggaagggaccatcctagaattgccaatatggcacctgtctgctcccttcccacctcccctcaccaggttgtgaaaacttgacctcacaatccttcccctgttaagagaacttgacctcacaatcgttctcacatagagttccagaaggccaccaccaagtggttggaacttgccatccctgccccagaccttaaaagtaagaaaagcaataattaaaacggcttcaccatttgcataacaaccaccactatgattattactggcaggaatcatcaatggctgccaaaattactgcaaaaatgtatgatggggaacagtgtctctgcataatctcaaagcatttcctcataagacacatattaattataaaggaaaaaaatcatagtttacatattttatagttgagaaaactgacagatactaccttaatcatgtgataaaagtggacattgccaggaatgaccatcatgttcctcttgatacactgcactgagaaggacacaatgtcactgctgtggtctcctggcaaaaaaaaaagcacaatctgaatctaatcatgaagaaacatcaggcaatcctgaattgggactgtctgcaaaataactaacctgtactcttcaaaagtgtcaaggtcatgaaagacaaaggaagactgaggacccacgggaatgtaagctccacaagggcaggaaccaggtctcttctgattcaaagttacatccctggtgcctcttaaatgctcagcaccatggatgatcaatgaagatgagatgtcctttgcagggacacggatgacttgtagtcctgacattctgattctatggagttgatcagaaaaccacttaaggcacccgggccccagtggtacagcgttttccctggatccgattcctttttccctgtggcttgtcatgtgggatggtgttctgagggttaacgtaaatacagttcgtagaggtgcgtctcactcctggagctggtgttcctgactgagggactgcaagtctgaatagtgtaaatggaatctgacttccccacggcagcaatgctataatgtgggattatgtgaatgggaattttctgtggaaggatcctaccagatgaatgaatgggcttaattctcatcggaatctaccagaatgtatatgttccagtgaatgtttatcttaatgtctcctgactctacagtcagaggagacattcccaaggctgatgctcatttcttttctctgtcccctcctcctttgtgctcccattgtatgcttcaggcttgaatcacatgtcctggggaggaaggctgtggactagagcacagtgtcccctgccttcaccctttgccccgctcagatccacttgctttgaaaaaagcctgggaacagccattccaggattctgggggaaacataacagaaatattagtggaacaaactacaacccctgctgtcgcagctgctcccaaagccaccactgatatctattgcttcccttctctactactcattctaaactctcctcccccttggcaagaatctctgctactttccattgcttactactgggcaaacccagagtctcatccacaaggggtctgagctcctgctaaccatgccatttgggtttacaaaccaggcaagggattttgacttcttactggaatggctgctttcagcctcctgtgatccattttcgatttcttttgcctgtatagatgaacaatacccttgttggctgccctcccatcttgcacttagggatgacatgttttattagatccaaagatctctgcaggtctggtctctctggccgccactccaaacttgctactaattatgatgattgcacccaccaggtctgtattatttcaggaccttgtcatcctccttgatacctggggcccagttctgtcatgacatcttctaccctcagtcctggcctgcagggatgtgggtgcccttctagcaccttccttcaattcattgctggaatgaatgtccccagcctctctcgcagagcagaggcatccagtggatttgggggtacctagcatacctgctccagcagtctcctcactctgagctttcctgttcttgcctccaccctctgtcacatcagttctgacatttcttcttagtgtcagccaccattttctccaagccaagcagcttataacatcagggcagcactttttccctgggtccttgcgggttgttcaatctcctatcgataaactctcccttgacccactttatagtccgtttccccttgacccagcacctgctaaatccagtcccatttcagtggctatgttgggtacatgttggtgaggacctacagctcctatgggagatggttctttccctgtcctagcaggtccagcactttggcagccaggttgtaccatgacttaacccaagtcactccagtggggggcatgtgtagttttgcatgggagaagcctctgcattatcttcaagcaaagaaagaggaacgccggctttgaacagggaggagctggccatgtaggcaggcccgaggagggttcactggaatcgggggttcaagattgttcaagtgcatcaacccagagaaccccgttcacctctgtcagggctctgaccctggggcagaagatttttagaggtgagttcagcctctggagctgtgcttctccatgggctgagcctgctcatgtttggctgtaggagatgaagctctccttagatgttaaggagtctcagagagactttctctctctgagagaaagccagaggctttcacatttagcctctactgggtgattaatcacccttcagcttttcattgtcttttttccagagcactccacaacagtcatccaagtccatcgtctttataatttttcctttcccttacttttcaattcctgccacgtggtaccctccagcacatcgccctccatcagcacgccatacaagcatcaccaaggaaagttttaacaattgtgcagccaagcgtgccagaggctgtccatgagggcccacgaccagtgatgggtccttcttttcatggttcaatgggtggctcagctcccaaactccatttttgaatctgttttcttgggacactcctggtgggttctttgggatgcagactatgtgtgagagaggtctgcacataggaagtttatggagcagtgttctcgggatcagcatctgtaaggaaatgcccaggcctgggcagacagagaggttgagctgggatgcagttcagtgaagccttcagtcaatgctcaagggagttctggagctgggatggcctttccaagtggttttgaaatggagcttggggctgggtcttttatttttatttatttattttttttttgaggcggagactcaccatccttagcaccttccttacgacttgctgagtctctgtcacccagagtctcactctcttgcctgggctggagtgcagtggcacaatctcggcttgttgcaa

SEQ ID NO: 18161 - RNA, 22 nt, Homo sapiens
  source 1..22: mol_type = other RNA
tgaagtaccagctactcgagag

SEQ ID NO: 18162 - RNA, 2225 nt, Homo sapiens
  source 1..2225: mol_type = other RNA
tgaagtaccagctactcgagagactgaggcgggaggattgcttgagcccaggaggtagaggttgcagtgagccatgatcgcaccacagcactccagcctgggtgacagagaaagaccctatctacaaaacacacacacacacacacacacacacacaaaacagatgagaaaactgaggcaccaagaggtgtttctggaatccaaacttggcaggaaggctaggagcagggttgggagctgcccttgtctcctccacaggcaggaagcttgtcctccctctccagcacctcagctgcccctgccacccccacccctctcagccctgaccctgtggtccagaaaggcctctggaggccagctgtgggtggcagggcctctggcttacaccagcgggcagcagggagtgtagtcacctgctcactcgtgtctggtgctctttgtggctataggaagcagaggacaggtgctgggaggagggctggcctgaggggaaactgaggcctgggactgcggggtcagggcttggtctctgccactgagtttgcacctggcttcccctcatgcctggccatttggttccggctcttgaaatagatcctctgcccacctggtagctggccggccatgggccgtgccacgccacctgcctgctgcagcccagcccggtcaccccgaaacgctgacaaaagccagctgctctcccagcagtcgctcggcaggcagacacccggaggcgtgacgcctgccctcgtctggcaccgaggctgccaggagggcgctgacgcagctctccccactcccactcccaggggctccgcagctcctttctggaatggcttcccgatgaggtaatgcagctcggagcacaggaggaggccactgggaaacgctgctggccaggccccagctccccgggaagatggctgccgtggcctccctgccctgcctgcccgacgccaccgcacaagggcctggcaggctgagaacaggagccggacttcaggccggaggcttggcggcctcactctggagtggccagggggacccagacatttactcatctcccggccgaggtggtgcaggcctcagcctgggcctgcagcctcactctgatccttagaggcccctgccctgagaacacgccgcccccgggcacacgcggagaaacagaggccgtgcccagggttatagcaggaatcaaggtctgttctcgccctgcagccctgggggcaagggcaggcctccctccacacgcatcgcatcgggtctgggaacagcaccatgagcttgctccgacctgccaagcggctttttcctggaacatgagtcttttccgggcacggagcagagcactcaggccaccggccctcctatgctgggagcagggggagatgccggctggccgagcaaggaggcccctggggctgtccacccggtgtccctctcagggcccctcttggccccatgaaaaggcggcacccccaccccttgcctctcctagcgctgccaggctcccctgcaggtgtgacctgcctcgcagaagctgctgagaggcaggaactgagcagggaagtgtcccaaggggtgactcacttccctcacccacgtttccccctctccctgccaggccctgcgctgggcgggccctagggccacagggaccagcatggcccggcagccccggacctcccaggtggaaggaaggacccggagaactggaaacatccttgcatagcagcccccgagttggaggcagccactcggcacctggcacctggcccaggggggcctcctgcggactcacgtgggctctgggaggtggaggagggtcacttcccccaggggagagcggagaaggctggcaggaccctgctgtgggtgtgactgggaccgtgctgggccctgcgttggccagcagtgtcccgagcgggcctccgcgccggcaggcccagctgggcctatttctgactcgaatttgttgcgaaacgtcggcaaatcccctgccctggctgggcctcaatttccccatctgcagacaggaggcgggcgagagggccccctggacttcagggcccgtgggtctgacggccagggctgcagctgaatctccgagttggagatgcctggtggggtgcagcacaccctgcgtgcacagatgagggccgggctggctccaggcgtgcgggaggcagcagtggagctgggatcggagtctggactcctct

SEQ ID NO: 18163 - RNA, 139 nt, Homo sapiens
  source 1..139: mol_type = other RNA
tgaagtaccagctactcgagaggacgaggcaggagaattgcttgaacccgggaggcggaggttgcagtgagccgaggtcgcgccactgctctacggcttgggcaacagagcaagactctgtctcaaaaaaaaaaaaaaa

SEQ ID NO: 18164 - RNA, 4256 nt, Homo sapiens
  source 1..4256: mol_type = other RNA
tgaagtaccagctactcgagaggatgaggtaggagaatggagtgaacctgggaggcggagcttgcagtgatctgagattgggccactgcacttcagcctgggtgacagagcaagactgtgtcttaaaaaaaaaaaaaaattgttaagtggctgtaaagggaacatttcattagagtatttgtgtgtgtgtgtaattttcaaagatagatatatttttagttatagaaactgaaaacagggctgggcacagtggctcattcctgtaatcctggcactttgggaggctgaggtgagtggattgcttgagcccaggagttctgagatcagcctgggcaatgtggtgtaaccctgtctctacaaaaaatacaaaaactagccaggtgtggtggcacacgcctgtggtctcagctactagggaggctcaggcaggaataccacttgagccccagaagtggaggttgcagtgagttgagatcatgccactgcactccagcctgactgacagagtgaaactctgtctcaaaaaaaaaacacctgaaaacatttctggagcaatatttatttttagagtccctcgaatacagaagtgaaaatgtactattcaagacttgtatttaacttcataaaatttctttcctagatgggtattacctcttattaaacaactaataaaatatgtgctatataatcatacatttaaaacatggaaagacaactaatatcttacagtacatgaagacaaacttcaggagacaaacattaaatatatccaaaaactaaatggacctggactttgcttacaaattgcttaaatggaaatgaaatttgtgtttaagaaatgttttcactgatggaaaaataaatctaacaaaaccattatgtaaaaacatactgatttacaaagccaatgtgtctcagttttaatttgtatataccctagatgaggtttatattaaatgagaataaaatattaaaagtccatcaatgtgtagaaaagaaatacagctgctcaagtactagatagaacttcatattctttaaatctatttctagaactgaattgactttttaaaattttataatttatcaactactccttaaggttattaacaatagcaggaattatgacgacatattatgtcatttgtttctcctactgcttttatctctacattacaatataaaattttcaatccagcattttatagctctgtgtttaagttaattagtaccttaaaaaaataaaattctaaatataaacttggtggattaaggctcagtaaacagtaatcaaacaaacaacagatttgtcctcacaaagagaatatgaaagccaaagttttttttcttttgtgatcctgcttcatattattctgttctgtccaatttcttttctgtagggaaacgccaaagagatataaaaaagagatataaaacagtggtgagtggcttccaaatgactgtttgcccttgctttttaagccaaaatcctctaaaaataggtctttaattctggcagcagattaggacaaatgctcaaaaattcatgttttcttcaaaaaatttcaactggcgagctttcacactgtaagttgtatacttttcacccatgtgctcccgcaaacgtacctctctatcaaattcatcctcctcctccaaaagatcatacacctgctctaaaagctgaactcccaggccacgaattacatcagttctcaagacttcaactagtctcctgatcttttcagaacctggcataatagctgaaggtagctctttaaaatggatttcctctgcctcttctgcaaccttcccatgaagtatcagtgtgtcccgatatttccgatgaagtttgaattctgacactgggtttgctaccgggacatcttcacagctctctttagaatccagtttcagggtctgagtcatcaattgtaccaaggcattaatttcatttgtctgacctttcccttccccgtaatccccatctgacttatcagttgaacttgtagaagaacttaactcatcctcagacagacaatgaatctgtttcctttcctgagtgacgctgcagtcagaggagagccgtcgggcaggcaagggctggtcttcttcctggggttttcctggccctgctacactcagagacgctttcctcactgaagggcctgaagaggacatttcttcctgtgactgctttagtcgcctcctctctctggctgataatggtcgatcctttgatgatgacatctcactgctccttgaactgctcacagacccagtgaccactctacgttggttttcagcctctttttgtgttgatgtgacatccactttcccaacaatgggatgagaaggcaaaaatcgaggaggcgactcttggaaagcaaagagatctctgcggacctgtctcttttcccctctgtgctcagtctgttctctcctcttttgccgtcgctgtcgagacagggaaggttcagacccagagttgtgtggctgtaaatctgggtggattctgccctgtttttctataatacattcaccagcaacttgatcctgggcgtggtggcacacgcctgtaatcccagctactcgggaggctgaggctggagaatcacttgaacccaggaggcggaggttgctgtgagccaagattgtgccactgcactccagcttgggcgacagggcaagactctggtcctttggcttttgttctttgattaggggctgcagaggcttcactggttcattcttttccccagtgacaatgtcagaggaccacatgggaatcaggttttcaggctgggcactggatttagtgttgtcctgcagcatctcctcttccacttgagaaatactgcatatacctcctaactcattagaggcatccaaatatcttggctgattctcctgaacaaagccatcactcactgaatccctcccttttgcaggtaagatgtcaatatttacgctactgattgtggctagttctgtggtattgctcaagtcctgtttgcaggtatgggctttcagactggcaggtgacttcaagagaccagaggccctgggtttctcctgggacaaacatttgccttcacccattatatatgtctgggagccctcagaagagagtggttgggggtggattacttcatgatttgattctgcctctccagaaaccactgtagcaaaaggcttggattgagagtcaccatttttaatgttatttttggaggtttttatctttgtggcctccaaaaagaaggagatttgccgctttatataaggctgcctcaggatgctcctcacagacggcctttcttcaggccttttgctcagcattgttcttatcagttctgccagctctgggctgtaatctcttggcattggtggcagctttccttcaataatccgataaactaaagaattcatatcttttgcattgaaagcatgcttcaaggtggccatttcatagacacagcatcctagagcccaaacatcagacttatagttgtagggtttgtttgagaacaattcagggctcatgtagtagggtgtgccaatgagggtgctagccatgtcacagtggttctctaacactcgggcaattcctaggtcccctactttgatgatgtttgttcttgttaggaagacattttgagttttcagatctcgatgaaggatgtgtttttcatgtaaatactgcaaagccatggcgatctgtacaaaccactctaccacctgattctcaggcagaagctgccctttctgctccttgagctttcggtacaaatcacctccttcacagaagcccatgacaatgtagagcagaccatctcctccttcccatgactccttgtaggtgacaatgttgggatgcttcaactgagacaagagctgggcttcctgttcagcagctcgccgctctcggctagaggcatttcggaggttcagttttttgatgacatactgcttgccgtcccgccggtgcttcacaagcgtcacctctccatagctccccttgcccacgacccgcaggtagcagtaggcggccaggggcatgttcccagcgctggcccagagtcgggatgcggcggcagcggcgggtagggcagcgggcggcaacaagaagctcggttcatgcccgagagggggcagtgggggcggctgttgaggcagccgggcccgggcgggattgctggggcccggcccgcgacgacgccgctgccatagcgatccgggccgggagcagttct

SEQ ID NO: 18165 - RNA, 4218 nt, Homo sapiens
  source 1..4218: mol_type = other RNA
tgaagtaccagctactcgagaggatgaggtaggagaatggagtgaacctgggaggcggagcttgcagtgatctgagattgggccactgcacttcagcctgggtgacagagcaagactgtgtcttaaaaaaaaaaaaaaattgttaagtggctgtaaagggaacatttcattagagtatttgtgtgtgtgtgtaattttcaaagatagatatatttttagttatagaaactgaaaacagggctgggcacagtggctcattcctgtaatcctggcactttgggaggctgaggtgagtggattgcttgagcccaggagttctgagatcagcctgggcaatgtggtgtaaccctgtctctacaaaaaatacaaaaactagccaggtgtggtggcacacgcctgtggtctcagctactagggaggctcaggcaggaataccacttgagccccagaagtggaggttgcagtgagttgagatcatgccactgcactccagcctgactgacagagtgaaactctgtctcaaaaaaaaaacacctgaaaacatttctggagcaatatttatttttagagtccctcgaatacagaagtgaaaatgtactattcaagacttgtatttaacttcataaaatttctttcctagatgggtattacctcttattaaacaactaataaaatatgtgctatataatcatacatttaaaacatggaaagacaactaatatcttacagtacatgaagacaaacttcaggagacaaacattaaatatatccaaaaactaaatggacctggactttgcttacaaattgcttaaatggaaatgaaatttgtgtttaagaaatgttttcactgatggaaaaataaatctaacaaaaccattatgtaaaaacatactgatttacaaagccaatgtgtctcagttttaatttgtatataccctagatgaggtttatattaaatgagaataaaatattaaaagtccatcaatgtgtagaaaagaaatacagctgctcaagtactagatagaacttcatattctttaaatctatttctagaactgaattgactttttaaaattttataatttatcaactactccttaaggttattaacaatagcaggaattatgacgacatattatgtcatttgtttctcctactgcttttatctctacattacaatataaaattttcaatccagcattttatagctctgtgtttaagttaattagtaccttaaaaaaataaaattctaaatataaacttggtggattaaggctcagtaaacagtaatcaaacaaacaacagatttgtcctcacaaagagaatatgaaagccaaagttttttttcttttgtgatcctgcttcatattattctgttctgtccaatttcttttctgtagggaaacgccaaagagatataaaaaagagatataaaacagtggtgagtggcttccaaatgactgtttgcccttgctttttaagccaaaatcctctaaaaataggtctttaattctggcagcagattaggacaaatgctcaaaaattcatgttttcttcaaaaaatttcaactggcgagctttcacactgtaagttgtatacttttcacccatgtgctcccgcaaacgtacctctctatcaaattcatcctcctcctccaaaagatcatacacctgctctaaaagctgaactcccaggccacgaattacatcagttctcaagacttcaactagtctcctgatcttttcagaacctggcataatagctgaaggtagctctttaaaatggatttcctctgcctcttctgcaaccttcccatgaagtatcagtgtgtcccgatatttccgatgaagtttgaattctgacactgggtttgctaccgggacatcttcacagctctctttagaatccagtttcagggtctgagtcatcaattgtaccaaggcattaatttcatttgtctgacctttcccttccccgtaatccccatctgacttatcagttgaacttgtagaagaacttaactcatcctcagacagacaatgaatctgtttcctttcctgagtgacgctgcagtcagaggagagccgtcgggcaggcaagggctggtcttcttcctggggttttcctggccctgctacactcagagacgctttcctcactgaagggcctgaagaggacatttcttcctgtgactgctttagtcgcctcctctctctggctgataatggtcgatcctttgatgatgacatctcactgctccttgaactgctcacagacccagtgaccactctacgttggttttcagcctctttttgtgttgatgtgacatccactttcccaacaatgggatgagaaggcaaaaatcgaggaggcgactcttggaaagcaaagagatctctgcggacctgtctcttttcccctctgtgctcagtctgttctctcctcttttgccgtcgctgtcgagacagggaaggttcagacccagagttgtgtggctgtaaatctgggtggattctgccctgtttttctataatacattcaccagcaacttgatcctgggcgtggtggcacacgcctgtaatcccagctactcgggaggctgaggctggagaatcacttgaacccaggaggcggaggttgctgtgagccaagattgtgccactgcactccagcttgggcgacagggcaagactctggtcctttggcttttgttctttgattaggggctgcagaggcttcactggttcattcttttccccagtgacaatgtcagaggaccacatgggaatcaggttttcaggctgggcactggatttagtgttgtcctgcagcatctcctcttccacttgagaaatactgcatatacctcctaactcattagaggcatccaaatatcttggctgattctcctgaacaaagccatcactcactgaatccctcccttttgcaggtaagatgtcaatatttacgctactgattgtggctagttctgtggtattgctcaagtcctgtttgcaggtatgggctttcagactggcaggtgacttcaagagaccagaggccctgggtttctcctgggacaaacatttgccttcacccattatatatgtctgggagccctcagaagagagtggttgggggtggattacttcatgatttgattctgcctctccagaaaccactgtagcaaaaggcttggattgagagtcaccatttttaatgttatttttggaggtttttatctttgtggcctccaaaaagaaggagatttgccgctttatataaggctgcctcaggatgctcctcacagacggcctttcttcaggccttttgctcagcattgttcttatcagttctgccagctctgggctgtaatctcttggcattggtggcagctttccttcaataatccgataaactaaagaattcatatcttttgcattgaaagcatgcttcaaggtggccatttcatagacacagcatcctagagcccaaacatcagacttatagttgtagggtttgtttgagaacaattcagggctcatgtagtagggtgtgccaatgagggtgctagccatgtcacagtggttctctaacactcgggcaattcctaggtcccctactttgatgatgtttgttcttgttaggaagacattttgagttttcagatctcgatgaaggatgtgtttttcatgtaaatactgcaaagccatggcgatctgtacaaaccactctaccacctgattctcaggcagaagctgccctttctgctccttgagctttcggtacaaatcacctccttcacagaagcccatgacaatgtagagcagaccatctcctccttcccatgactccttgtaggtgacaatgttgggatgcttcaactgagacaagagctgggcttcctgttcagcagctcgccgctctcggctgcttgccgtcccgccggtgcttcacaagcgtcacctctccatagctccccttgcccacgacccgcaggtagcagtaggcggccaggggcatgttcccagcgctggcccagagtcgggatgcggcggcagcggcgggtagggcagcgggcggcaacaagaagctcggttcatgcccgagagggggcagtgggggcggctgttgaggcagccgggcccgggcgggattgctggggcccggcccgcgacgacgccgctgccatagcgatccgggccgggagcagttct

SEQ ID NO: 18166 - RNA, 3989 nt, Homo sapiens
  source 1..3989: mol_type = other RNA
tgaagtaccagctactcgagaggatgaggtaggagaatggagtgaacctgggaggcggagcttgcagtgatctgagattgggccactgcacttcagcctgggtgacagagcaagactgtgtcttaaaaaaaaaaaaaaattgttaagtggctgtaaagggaacatttcattagagtatttgtgtgtgtgtgtaattttcaaagatagatatatttttagttatagaaactgaaaacagggctgggcacagtggctcattcctgtaatcctggcactttgggaggctgaggtgagtggattgcttgagcccaggagttctgagatcagcctgggcaatgtggtgtaaccctgtctctacaaaaaatacaaaaactagccaggtgtggtggcacacgcctgtggtctcagctactagggaggctcaggcaggaataccacttgagccccagaagtggaggttgcagtgagttgagatcatgccactgcactccagcctgactgacagagtgaaactctgtctcaaaaaaaaaacacctgaaaacatttctggagcaatatttatttttagagtccctcgaatacagaagtgaaaatgtactattcaagacttgtatttaacttcataaaatttctttcctagatgggtattacctcttattaaacaactaataaaatatgtgctatataatcatacatttaaaacatggaaagacaactaatatcttacagtacatgaagacaaacttcaggagacaaacattaaatatatccaaaaactaaatggacctggactttgcttacaaattgcttaaatggaaatgaaatttgtgtttaagaaatgttttcactgatggaaaaataaatctaacaaaaccattatgtaaaaacatactgatttacaaagccaatgtgtctcagttttaatttgtatataccctagatgaggtttatattaaatgagaataaaatattaaaagtccatcaatgtgtagaaaagaaatacagctgctcaagtactagatagaacttcatattctttaaatctatttctagaactgaattgactttttaaaattttataatttatcaactactccttaaggttattaacaatagcaggaattatgacgacatattatgtcatttgtttctcctactgcttttatctctacattacaatataaaattttcaatccagcattttatagctctgtgtttaagttaattagtaccttaaaaaaataaaattctaaatataaacttggtggattaaggctcagtaaacagtaatcaaacaaacaacagatttgtcctcacaaagagaatatgaaagccaaagttttttttcttttgtgatcctgcttcatattattctgttctgtccaatttcttttctgtagggaaacgccaaagagatataaaaaagagatataaaacagtggtgagtggcttccaaatgactgtttgcccttgctttttaagccaaaatcctctaaaaataggtctttaattctggcagcagattaggacaaatgctcaaaaattcatgttttcttcaaaaaatttcaactggcgagctttcacactgtaagttgtatacttttcacccatgtgctcccgcaaacgtacctctctatcaaattcatcctcctcctccaaaagatcatacacctgctctaaaagctgaactcccaggccacgaattacatcagttctcaagacttcaactagtctcctgatcttttcagaacctggcataatagctgaaggtagctctttaaaatggatttcctctgcctcttctgcaaccttcccatgaagtatcagtgtgtcccgatatttccgatgaagtttgaattctgacactgggtttgctaccgggacatcttcacagctctctttagaatccagtttcagggtctgagtcatcaattgtaccaaggcattaatttcatttgtctgacctttcccttccccgtaatccccatctgacttatcagttgaacttgtagaagaacttaactcatcctcagacagacaatgaatctgtttcctttcctgagtgacgctgcagtcagaggagagccgtcgggcaggcaagggctggtcttcttcctggggttttcctggccctgctacactcagagacgctttcctcactgaagggcctgaagaggacatttcttcctgtgactgctttagtcgcctcctctctctggctgataatggtcgatcctttgatgatgacatctcactgctccttgaactgctcacagacccagtgaccactctacgttggttttcagcctctttttgtgttgatgtgacatccactttcccaacaatgggatgagaaggcaaaaatcgaggaggcgactcttggaaagcaaagagatctctgcggacctgtctcttttcccctctgtgctcagtctgttctctcctcttttgccgtcgctgtcgagacagggaaggttcagacccagagttgtgtggctgtaaatctgggtggattctgccctgtttttctataatacattcaccagcaacttgatcctgggcgtggtggcacacgcctgtaatcccagctactcgggaggctgaggctggagaatcacttgaacccaggaggcggaggttgctgtgagccaagattgtgccactgcactccagcttgggcgacagggcaagactctggtcctttggcttttgttctttgattaggggctgcagaggcttcactggttcattcttttccccagtgacaatgtcagaggaccacatgggaatcaggttttcaggctgggcactggatttagtgttgtcctgcagcatctcctcttccacttgagaaatactgcatatacctcctaactcattagaggcatccaaatatcttggctgattctcctgaacaaagccatcactcactgaatccctcccttttgcaggtaagatgtcaatatttacgctactgattgtggctagttctgtggtattgctcaagtcctgtttgcaggtatgggctttcagactggcaggtgacttcaagagaccagaggccctgggtttctcctgggacaaacatttgccttcacccattatatatgtctgggagccctcagaagagagtggttgggggtggattacttcatgatttgattctgcctctccagaaaccactgtagcaaaaggcttggattgagagtcaccatttttaatgttatttttggaggtttttatctttgtggcctccaaaaagaaggagatttgccgctttatataaggctgcctcaggatgctcctcacagacggcctttcttcaggccttttgctcagcattgttcttatcagttctgccagctctgggctgtaatctcttggcattggtggcagctttccttcaataatccgataaactaaagaattcatatcttttgcattgaaagcatgcttcaaggtggccatttcatagacacagcatcctagagcccaaacatcagacttatagttgtagggtttgtttgagaacaattcagggctcatgtagtagggtgtgccaatgagggtgctagccatgtcacagtggttctctaacactcgggcaattcctaggtcccctactttgatgatgtttgttcttgttaggaagacattttgagttttcagatctcgatgaaggatgtgtttttcatgtaaatactgcttgccgtcccgccggtgcttcacaagcgtcacctctccatagctccccttgcccacgacccgcaggtagcagtaggcggccaggggcatgttcccagcgctggcccagagtcgggatgcggcggcagcggcgggtagggcagcgggcggcaacaagaagctcggttcatgcccgagagggggcagtgggggcggctgttgaggcagccgggcccgggcgggattgctggggcccggcccgcgacgacgccgctgccatagcgatccgggccgggagcagttct

SEQ ID NO: 18167 - RNA, 4118 nt, Homo sapiens
  source 1..4118: mol_type = other RNA
tgaagtaccagctactcgagaggatgaggtaggagaatggagtgaacctgggaggcggagcttgcagtgatctgagattgggccactgcacttcagcctgggtgacagagcaagactgtgtcttaaaaaaaaaaaaaaattgttaagtggctgtaaagggaacatttcattagagtatttgtgtgtgtgtgtaattttcaaagatagatatatttttagttatagaaactgaaaacagggctgggcacagtggctcattcctgtaatcctggcactttgggaggctgaggtgagtggattgcttgagcccaggagttctgagatcagcctgggcaatgtggtgtaaccctgtctctacaaaaaatacaaaaactagccaggtgtggtggcacacgcctgtggtctcagctactagggaggctcaggcaggaataccacttgagccccagaagtggaggttgcagtgagttgagatcatgccactgcactccagcctgactgacagagtgaaactctgtctcaaaaaaaaaacacctgaaaacatttctggagcaatatttatttttagagtccctcgaatacagaagtgaaaatgtactattcaagacttgtatttaacttcataaaatttctttcctagatgggtattacctcttattaaacaactaataaaatatgtgctatataatcatacatttaaaacatggaaagacaactaatatcttacagtacatgaagacaaacttcaggagacaaacattaaatatatccaaaaactaaatggacctggactttgcttacaaattgcttaaatggaaatgaaatttgtgtttaagaaatgttttcactgatggaaaaataaatctaacaaaaccattatgtaaaaacatactgatttacaaagccaatgtgtctcagttttaatttgtatataccctagatgaggtttatattaaatgagaataaaatattaaaagtccatcaatgtgtagaaaagaaatacagctgctcaagtactagatagaacttcatattctttaaatctatttctagaactgaattgactttttaaaattttataatttatcaactactccttaaggttattaacaatagcaggaattatgacgacatattatgtcatttgtttctcctactgcttttatctctacattacaatataaaattttcaatccagcattttatagctctgtgtttaagttaattagtaccttaaaaaaataaaattctaaatataaacttggtggattaaggctcagtaaacagtaatcaaacaaacaacagatttgtcctcacaaagagaatatgaaagccaaagttttttttcttttgtgatcctgcttcatattattctgttctgtccaatttcttttctgtagggaaacgccaaagagatataaaaaagagatataaaacagtggtgagtggcttccaaatgactgtttgcccttgctttttaagccaaaatcctctaaaaataggtctttaattctggcagcagattaggacaaatgctcaaaaattcatgttttcttcaaaaaatttcaactggcgagctttcacactgtaagttgtatacttttcacccatgtgctcccgcaaacgtacctctctatcaaattcatcctcctcctccaaaagatcatacacctgctctaaaagctgaactcccaggccacgaattacatcagttctcaagacttcaactagtctcctgatcttttcagaacctggcataatagctgaaggtagctctttaaaatggatttcctctgcctcttctgcaaccttcccatgaagtatcagtgtgtcccgatatttccgatgaagtttgaattctgacactgggtttgctaccgggacatcttcacagctctctttagaatccagtttcagggtctgagtcatcaattgtaccaaggcattaatttcatttgtctgacctttcccttccccgtaatccccatctgacttatcagttgaacttgtagaagaacttaactcatcctcagacagacaatgaatctgtttcctttcctgagtgacgctgcagtcagaggagagccgtcgggcaggcaagggctggtcttcttcctggggttttcctggccctgctacactcagagacgctttcctcactgaagggcctgaagaggacatttcttcctgtgactgctttagtcgcctcctctctctggctgataatggtcgatcctttgatgatgacatctcactgctccttgaactgctcacagacccagtgaccactctacgttggttttcagcctctttttgtgttgatgtgacatccactttcccaacaatgggatgagaaggcaaaaatcgaggaggcgactcttggaaagcaaagagatctctgcggacctgtctcttttcccctctgtgctcagtctgttctctcctcttttgccgtcgctgtcgagacagggaaggttcagacccagagttgtgtggctgtaaatctgggtggattctgccctgtttttctataatacattcaccagcaacttgatcctggtcctttggcttttgttctttgattaggggctgcagaggcttcactggttcattcttttccccagtgacaatgtcagaggaccacatgggaatcaggttttcaggctgggcactggatttagtgttgtcctgcagcatctcctcttccacttgagaaatactgcatatacctcctaactcattagaggcatccaaatatcttggctgattctcctgaacaaagccatcactcactgaatccctcccttttgcaggtaagatgtcaatatttacgctactgattgtggctagttctgtggtattgctcaagtcctgtttgcaggtatgggctttcagactggcaggtgacttcaagagaccagaggccctgggtttctcctgggacaaacatttgccttcacccattatatatgtctgggagccctcagaagagagtggttgggggtggattacttcatgatttgattctgcctctccagaaaccactgtagcaaaaggcttggattgagagtcaccatttttaatgttatttttggaggtttttatctttgtggcctccaaaaagaaggagatttgccgctttatataaggctgcctcaggatgctcctcacagacggcctttcttcaggccttttgctcagcattgttcttatcagttctgccagctctgggctgtaatctcttggcattggtggcagctttccttcaataatccgataaactaaagaattcatatcttttgcattgaaagcatgcttcaaggtggccatttcatagacacagcatcctagagcccaaacatcagacttatagttgtagggtttgtttgagaacaattcagggctcatgtagtagggtgtgccaatgagggtgctagccatgtcacagtggttctctaacactcgggcaattcctaggtcccctactttgatgatgtttgttcttgttaggaagacattttgagttttcagatctcgatgaaggatgtgtttttcatgtaaatactgcaaagccatggcgatctgtacaaaccactctaccacctgattctcaggcagaagctgccctttctgctccttgagctttcggtacaaatcacctccttcacagaagcccatgacaatgtagagcagaccatctcctccttcccatgactccttgtaggtgacaatgttgggatgcttcaactgagacaagagctgggcttcctgttcagcagctcgccgctctcggctagaggcatttcggaggttcagttttttgatgacatactgcttgccgtcccgccggtgcttcacaagcgtcacctctccatagctccccttgcccacgacccgcaggtagcagtaggcggccaggggcatgttcccagcgctggcccagagtcgggatgcggcggcagcggcgggtagggcagcgggcggcaacaagaagctcggttcatgcccgagagggggcagtgggggcggctgttgaggcagccgggcccgggcgggattgctggggcccggcccgcgacgacgccgctgccatagcgatccgggccgggagcagttct

SEQ ID NO: 18168 - RNA, 318 nt, Homo sapiens
  source 1..318: mol_type = other RNA
tgaagtaccagctactcgagaggctaaggcaggaggatcacttgagcccaggaggtcgagggctgcagccatctacaattgcaccactgtactccagcctgagacacagagtgagaccctggacgtaacaagacggaagggctgggcgctgaggtcctgccagcccggccgccagagggagctgagcgccagaggaggacaagccgaacccttcaggaggccgggcgtctccggagaccgaagcgccggaggacccgaggaggtctgccccgcgcgctgctctggagactcccggggcgggtggcgctcggcctttcc

SEQ ID NO: 18169 - RNA, 994 nt, Homo sapiens
  source 1..994: mol_type = other RNA
tgaagtaccagctactcgagaggctagggcatgagaattgcttgaacctgggaggtggaggttgcagtgtgctgagatcataccctccaacctgggcaacagggtgagactccatttcaaaaaaaatcaaaaaaagaaaaagaaaagaaatgttctctctgagctgcccaagacagtggtggccatagggagctactgagcactggaaatgggactaacgccattcaatttttaattttacttaaatagtccctgtggctagcgcaaccattccccacagtctgccaggaggacccccgtgctgctttcgcgtctgctttgttaccccctagaccaggccaacctccgccccctgcacagctgacacaggctcctaaggggggctgcctcctccagtcttggccaccctcccatctgctgttcacagttaccaggcaatcattttaaacctaactctatcttatgcatctgatgcttccagccccagtgttttcccagctcccctagaggacagaggcacagcctcccggctggcacagcctcccagacacacacaaagtcaaccctccttgggaggccagcccactggctgggcaccaggatagagaaggcctcccctccagcgtgctccccagcttgactcttctacccagggaaccccccactactcagacccccaagagacagcggagcacatgggcagaatcgggcgtccctctagggcagcggtctccagctccaggccacggctcactcgccactgtctcagcccctgggcgggtgccaggccgaagaccatgaggatccccagtgcagcgcccccacaagggccctccagagccacccggcacaaccccaaacaccgcgaccccaaagctgtgcccatcccgggccgacgtcaggggtcccgcgtggggtctgcccctctacgagcgggagaccctgagcaggctgctcggcagcgctggaccttccctggtgtgtaaagtgaggg

SEQ ID NO: 18170 - RNA, 667 nt, Homo sapiens
  source 1..667: mol_type = other RNA
tgaagtaccagctactcgagaggctcaggccggggaggatcacttgggcccagaagttcgaggtcagcctggacaacactgacctatttgaaaggtcaacatctctgcattgcacttttccccagtttcaccacctcaaataatgtgacaggctccccttccccattctgttgagggtgtccattagctcttccacggcctgctcctctaattccagcttcaattctgctcttctcacctggagattttcgaggtttcttatttgtagatggaggccggccaggacgacccctttttctttttcctttgacctctgtttcttcaagctcgctgccagcatcggaatgggcagtagtttcattagttgaatcctgtaacactggtaattctgaagtaatcattgctggagaggtcctttcacaatgcagcaaaataatcaagtgctgtacaactcaaaacttttaaaataacctcaaaggcaatcctcagctgcccatccgggcgccgccgaccatcgacctagtttccccccaaaagtctccggtgtgttattcccgatgtgggggggttgttacggggtggtcgccgggggttcgggagcgggggccgcgccttcaacggagctgcaatcctaacccgccatctggtggcattttccacacgccaa

SEQ ID NO: 18171 - RNA, 2945 nt, Homo sapiens
  source 1..2945: mol_type = other RNA
tgaagtaccagctactcgagaggctgaagcaggagaatcgcttgaacccgggaggtggaggtggcagtgaacggagattgaaccactgccacctcagcctgggtgacacagtgagactccatctcaaaaacaaaacaaaaatcttgaaactgtctcaaaaaaaaaatcttgaaagaagacacagcggggttcttgaaagaagacacagagaaggctcaaggcttctctctgccttgctcaggagacctggtaccttagctggggctgcaggtgtggagctgagaatagcttggggggtggctgtttttgaaaggagggtgtctgtgcaaatatcacacccagaattttctcaagttgcgccttgcatcaagagtcccaaagtcctccccagccacccaaactcgtttttctcacttttggtgattattctgtgccccaaatagtgcaactgagcaatgaggtctgagaatgaggaatggacctcagccgccatcccctccccacctccagccgtggtttccgggcctcagagagacggggagaagtcgtcaagtggcagctgatgaaatttggggaagctgtggatttgggctctggatggtcagagaggaggcctctagctcctcaggacagtggttctgtagtcgcacgaagttgcccagagaaggtggcaggaggaatacattcgaaaaggagaaatcggtgcaggactaggggccagggaagaaaatgcagaaattctttgtaccgccaggtgaggtggcttacgcctgtaatcccacactttgggaggccaacacgggcggatcatgaggtcaggagttcgagaccagcctggccaacatggtgaaaccccgtctctactaaaaatacaaaaaaaaaaaaaattacctgggcgtggtggtaggcacctgtaatcccagctactcaggaggctcaggctggagaatcgcttgaacctgggaggtggaggttgcagtgagctgagaccgtaccactgcactctccagcctgggcaacagagcgagacttcatctcaaaaaaaaaaaaaaaaaaaaaaaaaaaaaaaaaaaaagccgggcacggtggctcacgcctgtaatcccagcactttgggaggccgaggcgggcggatcacgaggtcaggagatcaagaccatcctggctaacacggtgaaaccccatctctactaaaggtacaaaaaattagccaggtgtggtggcaggcgcctatagtcccagctacttgggaggctgaggcaggagaacgacatgaacccaggaggcggagcttgcggtgagccgagatcacgccactgcactccagcctgggcagcagtgcaagattccgtctcaaaaaaaaaaaaaaatcctttgtaccaggtggtaaagtgctcctgccctgagctccccttaaatgctgcctgccctcaccctggctcttcacaggtcccctgccctggcctccccaggatccagttctaaaggggtcacactagccactggactggccctcaggaccgcactgcaacactgctatgtgactagtcagtgccttatctggcctttccaggtgtgaaatatttgcaacatcacccaggtctgtggggcgggggcatctggctcagtagccccaagtctctatctggggtcacccagtggcctctccatgaacccctctgccctggcctggttgttggtccacccccaccctcagaccaccgtgttgccctccagaaacgtgggtgacgtgggcatgtgcatgcccctctccagggagctggagctgcggagtggcaggaggtggtggcccggggtcccgccccgcctccgtccttgcacccccacccccggcctccagcactgcagcggccgaagcacctcccgccgcaggtcccggctgcgccacgtgtagatgacggggttgagcagggaattcagggtggagacggcgaaaaagtagtgggctttgtagaggatcgggcaggagtggacgggacaggcatagtccagaaggaggatgctgaaggcgggcagccagcagacgataaagacgcctagcacgatggtgaccgtcttgagcagggctagcgtctgcggggcggccatgtcagcgtggcttgagcggaccacgcagtagatgcgcacgtacagggccacgatggccaacaggatgatggagaagatggtcaccacgcacagcacataatgcttggcgtagagaggcaggacagtggagcaggcctcgaggtggcccaggcagttccagccaaggatgggcaggccaccgaggaccagcgagatgagccacgaggccccgatgagcagaagcatgcggcagctcttgtcgctgccatacagcttgaccttggcaatggccacgtggcgctcaatggcgatggccaggaggctgaagacagaggccgagagcgtgatgaaggcagagccctcccgggcaaaccactgcacaggcgtcagcctcagcgtgacagagccagagagcaaggtattggctacgaaggccacgcctgccagtagatcggaggcggccaggttgcccagaaacaggtacattgccgagtggaacttgctgtttcgggccaccgcaatgagcaccagaaggttttccaccacaatggcgcaacagaggatgacgatgaaggccgaggccacctggcgggaggtcgtctcctgcgtttccagcgtctccttggtataattatagtgttcctggaccttgttggggttcaggtactccgagtacaagctgcccatggtggggctcagaggcctgctggggccatggggctttcagaactggctaggccggcccggctcccggccctggccggaggggccttggcgtctgcgtccccagggcggccgcggctggggctggggttgccagccgggctcggctaagtcccggggctgggacgagggac

SEQ ID NO: 18172 - RNA, 5954 nt, Homo sapiens
  source 1..5954: mol_type = other RNA
tgaagtaccagctactcgagaggctgagacaggagaatggcatgaacccgggaggcggagcttgcagtgagccgagatcacgccactgcactctagcctgggtgacagagcgagactctgtctcaaaaaacaaaaaaacagaaaaacaaaaacagaaggccaggcgcggtggctcacgcctgtaatcccagcactttgggaggccgaggcgggtggatcacgaggtcaggagattgagactatcctggctaacacggtgaaaccccgtctctactaaaaatacaagaaattagccgggcatggtgtcgggcgcctgtagtcccagctacttgggagactgaggcaggagaatagcgtgaacccgggaggcggagcttgcagtgagccgagatcgcgccactgcactccagcctgggcgacagagcgagactccgtctcaaaaaagaaaaaaaccagagtactggggttcttgagacactggtgctgagttcacttctgtgggcttcagtcttctcattcatacacttgggctagataggtctttcttggatctttaaaaccaccaaaaactcaatgatccttctgggtctaatcagtgtgattcaaggcatattatttttaatgtcatataattcatgtcacttgcaataaagtgacatgaacaatatatagcagaccccattttgcaataagagtataatctcctttgagaattattcctgaaatcacaaccaggcttctcccgtcccctctcatcagtgaacacactcctcaaacagggaagcattcttctcatcagacattggcagaaccatacaaatgttcagaggcagactttcaggaggttcttttaaagtctaacaattctatgaaacatgacaaagacactgacataagcgctgtcgggttaaaggagtctttgaaatctcttttgtgatgtgaaatgtgaacattctttgccttttgttaaacgtttagattgacactctccccacacacaaaaggaatatcacatcttattcctacatgctttagatgttgggattagtaggtttcctgcaatagatctgtgggcatttgggggatgatgcggtgaattgcagatggaagataatggtgacagtattatacaggtatacttaatgctgtttctgaattgaagatatttatcccttccagatttgcattttgtgttcaacactgggacactgtgtggggtaccctgcgtgacagttaatactgtgtaatgaattccacaagattgctaaatttcatgtcttctgttattaaattttatggctttcattttagtaagcaatttataaagttttctcactgatctcaaagattaaaggctgtatatacagcaattagcattattctggcaataatgcctaagatttattagttccattcttacctcttccaaaagcatagagaagtttaataaataaatgagatctaatgcccatctatgattcaatgaaggtgtataacatgtgacaggctaaggctggcttagctattgatcatctggttctttagttctatccctgaaaatacagactgaccctaaaccaatgttcctagacgacattaagttgtgccttcactgggttaagaagcaccattataacctctgtctccattttgcatcttttttacattctgaagaaatgttcctatatacagaccctcatgctgtagttcaagaggaaattagcctctgcacataagtttttttactgtgaaaagcaaaaagtgttttagcagccagaaaattcagaaccaaacttactgtctaaatgttacttgctacattgactcgtataaaactgtgtacttctattttactgttatgtcttctttaaaggctctgtattttgtaggcctcttcaagaccttataaatagaaatcaaatttcaaaaacaaaaatgtagttacaagtgactatagtttagcatactgtattatttgctattataatctaaagattaaatataggtttaacagctattttaaaaaatgaataattttacatagaaaatatgctaacttcccttttatcatcataagatcatagttgttgttatattaagtatttattatgctgttcaaatgttagctggtgtaagttacctactaaaatgcttattcagcataactactgaaaaaacttagctgtctctggtattagttcattgaatattatatgcatcaagtcttttcatgtttccacgttatatttttaaaacaagaaactaggctgacttaaaaaaatttaaatcatgaatacattatgtataggtttttctgtctcctaaatattatctacttttttaaaaaacaaaaattttgatacaagaaagcactctgaggcagtatatgtgtattaaatttaaggtcacaattttcactaatctgagaaaacacatatatgtaatatttaaaagttaatgaaatccagtgaaacttcaacttatttcattgagaatttactaacaaaatatagaaaacaagaatttacctcttttaaatggcatgtctgtattacttacaatttgataaatgagttcctttccatacataccttaagatccacaaccttggtggcataaataacatgattaaagggtcaggtacaatgtatattttaatatgggatttgtgtagtgatttagagcataaatatcacacagtgaaaaatttatcacaaactaaatacagtaacaaaaggaaagaaagagcttatgtccacatttccaaggtctttacaataagttatagcgtccaggtccaacacagcatatttgcatacaaagccactgatgtgaacactgaaaggaatctgtcctgtaggtctttcatcttgatttaataaagtttgtacagtatcaaataatatcaaaagtctaaaaaacacaatgagcttttatgtttataaattattgtttttataccataaaaaaagtcaaaagtgcagtttaaaaaaaagtggaagttgttattcttgataagagctagaaaaatgtcatgtcccagttaagaagcaatctcaaggctcatccaatttctaaggaattttaactggcatctaaccttggttaccatatgctgtaagcaaaaccaacagaatgggagctatgtaacaatctagcgaagagaaacattgcaaataaatgtaattataggcctctcccaaagtgaatgaaatgattctttactggaatgaatgggctgtcactgaatgtgactatacttggtaaacttcaaaggcttgctagaaatttttatctttttcaaatttttagtcatagctgacaatggtacatatatcccaggattatgaaattttctagtataactgagaaaaatataattgaaaggtaataaatcatatcatctattatttctcacagaaaataaggaataagggcccagtaattaaaaggcagaagtacagagattagccaagaagaaacagatgggtgaaatacaactgggtcttaattggcacagtaactagctgtattttgacacactcaagaacaaatgcctatactgaagtatgtggtacattaaccacttgtacttatgtaagaaaatgaaatggtaaaacgataggcttataaaacaaattaaatttagagaaaggaaaaataaaaggaatgtaaagaaaaatcaagtttattgtggcatcaaaatattgacagagctgttatcagtcaagagcagtcttcttgttgctaaaacgaagaggcagcctgagcctggctccatccaaccacctcttctaatgctctttaactggcagtgcttcctataaatgacaccaagcaatagagatgattattgtttccactgaatagagtaagttccttgattggtttaacatatatagactgcctgagagaataaaaacatcaccatacaataggttaacggtaaatcaaggtcttcgtagttgtgatgggagaaaagggttggctgctggaaacagtatggtgccctggaggctgcgtacgtacacaccctaagaattcacatcaccattagcagaagattagaagtcaatggatatggatgcttgtgcagaatcttctcgccccctgacataaatttcacagggaatctcctccattactcggtcttccagggcctgctcagggcactcatgtccctgtttgaaagtgtaactacttttcttgaaggtgctattaaatgttttcattggctgtggttgtgcaaagtcatttcggaaaggaagttccatggaactgaggttggtcctgctttgtttgacgctggaggcctgcgacccacagtggtggtcgtggatgcagcgggaggcggtggaggagcgccgcatcttctggtagttgtccaattcttccgacaagtctgccaggtctgcagaaatctctttgtcccttagtgaaaacagttcataatgaggaggatcaaacacttcttggaacccggttttattaaaagcggttttgcaagccatgaccttttttcgaggctgtttcacttgtactaaaatagaaataatgagaaggaccaagacaatccctgaagtaatgccaataattgttccatgagtcttagtgatttgttcaaatactcctgcttttttcttttctttacaatgattttcatcccaagggtatgcacaattttggacaccattacagactaaagaattattgatgcacatgttgctatggcaaaagaaagtgctgcttgtgcagggaggctccacaaaggaagtaaagagcattcgaaacctgctaagccgactaccttcatctgcccacattcgaatcactccaattcctgttttaagcattacatcattggccacagtgctgcaaaacttggccttcaggttttcaatagaactgcttccatcatagactgcaacgaagtttctcttgcattcatttgagtgctccatttgataatctaggaacctcaaataaatcttagcttttggagtggctttaatggtccagatgcaatcaacggcttggcctggttttgttttctcctcttgttctacctgactagagcgcactattccatcagctcccgagagctcgaactgacaatctcctaggtaagtaaagtctggatctggaataaatgaatattttgctcgaaatcccagtccttcaagctcttcatcagaactaaacttaatccacatgaatctccctgttgatctaattaatggagggcttttcacgccacagtaacgatctataagaggagagaaaccaaatggcccatctcgaacttccaagtgatcaaaccgacactcaaatgatggttctatataataatgttcatcaaaggtcaactctattctttgacgtggagcagcttccaaaatgtagatacactccttgtttggtggatatgagtcaggataatttggcgaagcaaaatgacctccattgctggttcgaacccaaatgccacactgggttgcaggaatatgcttgattccaatattttgtccatcttgggttttttgggccacggcaatcccttccactaccagtactgttattaacaacactttgaggaccgagcagagccgctccagggccatgttcccgagctgcccggcgcttcgcgaagggctgaggtagcggcggcggtggctcggcgctcacggctcggcgcggcggcgacggccccactccgtccccatcgccggccagcagctgcctccccgctcccctgaggagagctcaggtcctgcggcccgccatgcccgagccccacagtgggctcccgcgcggcccgagcaccccgacgggcgccgcctcctgctccgcggcgccccgtcccatcgaccgcccgagggccgaggagtgcggacgcgcggcgcgggaccggcaggcagctccgcccgcggccccggcgcgggatccactgaagt

SEQ ID NO: 18173 - RNA, 5975 nt, Homo sapiens
  source 1..5975: mol_type = other RNA
tgaagtaccagctactcgagaggctgagacaggagaatggcatgaacccgggaggcggagcttgcagtgagccgagatcacgccactgcactctagcctgggtgacagagcgagactctgtctcaaaaaacaaaaaaacagaaaaacaaaaacagaaggccaggcgcggtggctcacgcctgtaatcccagcactttgggaggccgaggcgggtggatcacgaggtcaggagattgagactatcctggctaacacggtgaaaccccgtctctactaaaaatacaagaaattagccgggcatggtgtcgggcgcctgtagtcccagctacttgggagactgaggcaggagaatagcgtgaacccgggaggcggagcttgcagtgagccgagatcgcgccactgcactccagcctgggcgacagagcgagactccgtctcaaaaaagaaaaaaaccagagtactggggttcttgagacactggtgctgagttcacttctgtgggcttcagtcttctcattcatacacttgggctagataggtctttcttggatctttaaaaccaccaaaaactcaatgatccttctgggtctaatcagtgtgattcaaggcatattatttttaatgtcatataattcatgtcacttgcaataaagtgacatgaacaatatatagcagaccccattttgcaataagagtataatctcctttgagaattattcctgaaatcacaaccaggcttctcccgtcccctctcatcagtgaacacactcctcaaacagggaagcattcttctcatcagacattggcagaaccatacaaatgttcagaggcagactttcaggaggttcttttaaagtctaacaattctatgaaacatgacaaagacactgacataagcgctgtcgggttaaaggagtctttgaaatctcttttgtgatgtgaaatgtgaacattctttgccttttgttaaacgtttagattgacactctccccacacacaaaaggaatatcacatcttattcctacatgctttagatgttgggattagtaggtttcctgcaatagatctgtgggcatttgggggatgatgcggtgaattgcagatggaagataatggtgacagtattatacaggtatacttaatgctgtttctgaattgaagatatttatcccttccagatttgcattttgtgttcaacactgggacactgtgtggggtaccctgcgtgacagttaatactgtgtaatgaattccacaagattgctaaatttcatgtcttctgttattaaattttatggctttcattttagtaagcaatttataaagttttctcactgatctcaaagattaaaggctgtatatacagcaattagcattattctggcaataatgcctaagatttattagttccattcttacctcttccaaaagcatagagaagtttaataaataaatgagatctaatgcccatctatgattcaatgaaggtgtataacatgtgacaggctaaggctggcttagctattgatcatctggttctttagttctatccctgaaaatacagactgaccctaaaccaatgttcctagacgacattaagttgtgccttcactgggttaagaagcaccattataacctctgtctccattttgcatcttttttacattctgaagaaatgttcctatatacagaccctcatgctgtagttcaagaggaaattagcctctgcacataagtttttttactgtgaaaagcaaaaagtgttttagcagccagaaaattcagaaccaaacttactgtctaaatgttacttgctacattgactcgtataaaactgtgtacttctattttactgttatgtcttctttaaaggctctgtattttgtaggcctcttcaagaccttataaatagaaatcaaatttcaaaaacaaaaatgtagttacaagtgactatagtttagcatactgtattatttgctattataatctaaagattaaatataggtttaacagctattttaaaaaatgaataattttacatagaaaatatgctaacttcccttttatcatcataagatcatagttgttgttatattaagtatttattatgctgttcaaatgttagctggtgtaagttacctactaaaatgcttattcagcataactactgaaaaaacttagctgtctctggtattagttcattgaatattatatgcatcaagtcttttcatgtttccacgttatatttttaaaacaagaaactaggctgacttaaaaaaatttaaatcatgaatacattatgtataggtttttctgtctcctaaatattatctacttttttaaaaaacaaaaattttgatacaagaaagcactctgaggcagtatatgtgtattaaatttaaggtcacaattttcactaatctgagaaaacacatatatgtaatatttaaaagttaatgaaatccagtgaaacttcaacttatttcattgagaatttactaacaaaatatagaaaacaagaatttacctcttttaaatggcatgtctgtattacttacaatttgataaatgagttcctttccatacataccttaagatccacaaccttggtggcataaataacatgattaaagggtcaggtacaatgtatattttaatatgggatttgtgtagtgatttagagcataaatatcacacagtgaaaaatttatcacaaactaaatacagtaacaaaaggaaagaaagagcttatgtccacatttccaaggtctttacaataagttatagcgtccaggtccaacacagcatatttgcatacaaagccactgatgtgaacactgaaaggaatctgtcctgtaggtctttcatcttgatttaataaagtttgtacagtatcaaataatatcaaaagtctaaaaaacacaatgagcttttatgtttataaattattgtttttataccataaaaaaagtcaaaagtgcagtttaaaaaaaagtggaagttgttattcttgataagagctagaaaaatgtcatgtcccagttaagaagcaatctcaaggctcatccaatttctaaggaattttaactggcatctaaccttggttaccatatgctgtaagcaaaaccaacagaatgggagctatgtaacaatctagcgaagagaaacattgcaaataaatgtaattataggcctctcccaaagtgaatgaaatgattctttactggaatgaatgggctgtcactgaatgtgactatacttggtaaacttcaaaggcttgctagaaatttttatctttttcaaatttttagtcatagctgacaatggtacatatatcccaggattatgaaattttctagtataactgagaaaaatataattgaaaggtaataaatcatatcatctattatttctcacagaaaataaggaataagggcccagtaattaaaaggcagaagtacagagattagccaagaagaaacagatgggtgaaatacaactgggtcttaattggcacagtaactagctgtattttgacacactcaagaacaaatgcctatactgaagtatgtggtacattaaccacttgtacttatgtaagaaaatgaaatggtaaaacgataggcttataaaacaaattaaatttagagaaaggaaaaataaaaggaatgtaaagaaaaatcaagtttattgtggcatcaaaatattgacagagctgttatcagtcaagagcagtcttcttgttgctaaaacgaagaggcagcctgagcctggctccatccaaccacctcttctaatgctctttaactggcagtgcttcctataaatgacaccaagcaatagagatgattattgtttccactgaatagagtaagttccttgattggtttaacatatatagactgcctgagagaataaaaacatcaccatacaataggttaacggtaaatcaaggtcttcgtagttgtgatgggagaaaagggttggctgctggaaacagtatggtgccctggaggctgcgtacgtacacaccctaagaattcacatcaccattagcagaagattagaagtcaatggatatggatgcttgtgcagaatcttctcgccccctgacataaatttcacagggaatctcctccattactcggtcttccagggcctgctcagggcactcatgtccctgtttgaaagtgtaactacttttcttgaaggtgctattaaatgttttcattggctgtggttgtgcaaagtcatttcggaaaggaagttccatggaactgaggttggtcctgctttgtttgacgctggaggcctgcgacccacagtggtggtcgtggatgcagcgggaggcggtggaggagcgccgcatcttctggtagttgtccaattcttccgacaagtctgccaggtctgcagaaatctctttgtcccttagtgaaaacagttcataatgaggaggatcaaacacttcttggaacccggttttattaaaagcggttttgcaagccatgaccttttttcgaggctgtttcacttgtactaaaatagaaataatgagaaggaccaagacaatccctgaagtaatgccaataattgttccatgagtcttagtgatttgttcaaatactcctgcttttttcttttctttacaatgattttcatcccaagggtatgcacaattttggacaccattacagactaaagaattattgatgcacatgttgctatggcaaaagaaagtgctgcttgtgcagggaggctccacaaaggaagtaaagagcattcgaaacctgctaagccgactaccttcatctgcccacattcgaatcactccaattcctgttttaagcattacatcattggccacagtgctgcaaaacttggccttcaggttttcaatagaactgcttccatcatagactgcaacgaagtttctcttgcattcatttgagtgctccatttgataatctaggaacctcaaataaatcttagcttttggagtggctttaatggtccagatgcaatcaacggcttggcctggttttgttttctcctcttgttctacctgactagagcgcactattccatcagctcccgagagctcgaactgacaatctggaatgggatttaaaatacctcctaggtaagtaaagtctggatctggaataaatgaatattttgctcgaaatcccagtccttcaagctcttcatcagaactaaacttaatccacatgaatctccctgttgatctaattaatggagggcttttcacgccacagtaacgatctataagaggagagaaaccaaatggcccatctcgaacttccaagtgatcaaaccgacactcaaatgatggttctatataataatgttcatcaaaggtcaactctattctttgacgtggagcagcttccaaaatgtagatacactccttgtttggtggatatgagtcaggataatttggcgaagcaaaatgacctccattgctggttcgaacccaaatgccacactgggttgcaggaatatgcttgattccaatattttgtccatcttgggttttttgggccacggcaatcccttccactaccagtactgttattaacaacactttgaggaccgagcagagccgctccagggccatgttcccgagctgcccggcgcttcgcgaagggctgaggtagcggcggcggtggctcggcgctcacggctcggcgcggcggcgacggccccactccgtccccatcgccggccagcagctgcctccccgctcccctgaggagagctcaggtcctgcggcccgccatgcccgagccccacagtgggctcccgcgcggcccgagcaccccgacgggcgccgcctcctgctccgcggcgccccgtcccatcgaccgcccgagggccgaggagtgcggacgcgcggcgcgggaccggcaggcagctccgcccgcggccccggcgcgggatccactgaagt

SEQ ID NO: 18174 - RNA, 5256 nt, Homo sapiens
  source 1..5256: mol_type = other RNA
tgaagtaccagctactcgagaggctgagacaggagaattgcttgaacccaggaggcagaggttgcagtgagccgagatcgctccattgcacttcatcctgggcaaccaagtaagactctgtctcaaaaaaacaaaacaaaacaaaacaaaacaaaaaaacctcaactttgtcagctgctcagagttaaaacaattcaaatgtttcagactagaagtgagtttttaaaaacatctgaaatattcaagaaaatttgggttttggtacttttccttatgctctgaacaatgtgaactcccaacattgtttatccttgttcctcttactgcatgaagttcaaactaggtcttaaagacaacttttctgtacttaagaaaaagtgcaaagatagaaaatgaaatgtaaggtgttttgcaagaaatgctccctcgagaatggtgtttggatgtgggtggggggaaaacgatttttgttctccattgtaatctgacacctacgaatgaccttgtcttcaatgtccacaacactagtaagcatgtaataatcacggacatcgcaagattaaaaattaagtagcaaattccactaaaacacttgtattcattctatacaatcgaatggaaatccgtgagtgctactgaaaaaggtgttcacatgcacatgtccaatatgtgcattccactgaaggctaaaagcttaaaattctatttccagtgtttatgaatagcttcaatatctacattcatagccagcattctgcttgagttacctcttactttaatacttcacaaatgagtaagtacgtcttgggagattaggaaggtacctgttgtcaataactttctcttatgcttagaatgtgctgcaattgtttttaaactatttaaaatgaacacccctataataatgaaacactttatgccaagaagaaaattgatttgtttttagccaatcaagactaccctgcagatctgaaaactgtagattacatccttaggaaaggagaaaaggaggctcacaaatataaaggaatcctgacttttacacggacaaatttttaaaaagataaaatgtattacataagcgccataaacagtgaaatctgcttatattaaaaaaaataagtgaagctttgtttggacattatttccttgcaagagcagtacatatccttagtaaacaactaccatatttacaagttaatttccttgatacttagataggattgaaagccagaagaaatcatggaagagtgagctttgaaataatctttacagctaagttggtaacagtgaaggtacccagacaattcctaaagcagacttgtttattttgtagagtatttgactacgtctgggtagctagcttgctttgataaaggccaaggacaagttcaatccctattttggcctgttaaagcttttcccagaagaacaaatatctgctccatagtcattctaatcctaaccccagctagtctcaaaaaagaaattaggcaagaagactggggttatcatgaagttactcttactactaagaaaccaacataaagtgcatgtccatagatagcgagtcagcagtctcattttcatatatgggcagcacaattaaaatttgaatttcaaataacccaacatgactttcaacaaaggataaaaatcccttaatcttcaactggtctttaaatttgagatgttaggactgtgttagagatagtaatgaaatatgatcaagtgtgcactggtaccttaaatgacaaatctcaaaaacaacacaaattcgagactttcctattaacacacacatgtgtaccaactgcaattcatatgctaaaagtggttttatagtctctttcctccattttttcatttttgaggagcagacttgtaaatttaacttgtgctaggtagtagtggtttgtttttcttaaaccaaaactctgccaaacttgctgatcttctgcttcatctactcaggtagaataccaggtcaagctgctgctgtggctgctctcaccatatgaaaccagtttgtgtctgcattattactgtcttcaggaaaactttaaattcttcagttttctttactcctcccatatttcacttcctgcctaaatccaagttaaattatacaatttccactggtcttcaacacggtttaattctgcactgtcctttcctttgcatgtcacagtagctgttcacacattaaatattatagatatgttctgctcttgacatctacacacttacaaaagcagctttgtactttgtttggtgtgtttgttactatgttggctcacaaaaagcagttttctcagttctaagcatggtactttacaatttttaatgcattcatacaacagtgcattggaaaagtactgagcctctacaaaatagctttacatttttaaacaaatgaatgtgattttttttcacttacacaagcataggctttttaatatttccacaagataaatatctcaattaaactataagctcactctacagtgtgccacagtgatgggcttaggagacagttatacacttagaagatcctaaccttagtgttatttacactgacatgtccagtatcaccaagtctgaaaggtgaacaaacaatactcagaatgtggctgaatttgtgttaactaataactgggaatgatatagctttaatcacttatgaaacacatactgtaacttagtctaaactggtaatttcctttgctcctctcttatggtgtgggaaaatttaaagatcaacatgaaaaaggagccattgctaaggcagatcttttaagataacaaaggaaaaattgacaagtgtatatgataaattatcagtaacagtgatgctaccaatttaactggtacggaaatcagatttttaggtcctataacgtggcttttaaaatatttccttttattctggaacaaaaactggagaaaggacaatgattccttcagaaagcaatgactcaattcaggttgttactttacatttaagtaccactcaaaaagtggacataaaagcaagtgattcctgtttgcccatcactatatcagctacatagctgagagttcagatcttaattacacaacactttctctgttaccagaagctaagactgctctgcgacaaataggacaggtagaattctcagataaccagcgatcgatgcagtggacatggtactcatgggaacaaggtagtttacgaagtttgttgccttctgtatattctgtaatgcaaacactacaggtttttaatgcatcattttcaccaaaacttctcattgccaagttgtcaatctgttctttggtgagtcctctaggttggtcatcatcatcctcatttaagaggaaaaactgagccaggctaaggaagggcaaagagccactttcatcaaatgtgactggggccctatgtcgaccctctcgcctggcacctgatgagcctgatgatgagcttccttcattactgccttcaaataaatctgagctagtttctgaactttcaccaccggaactggaactaggactggaactggaacttgaactggaactggaactcgaactggaactggaactcgaactggaaccagaactactaccaccaccagaacctcctcttccactccgtgactctgccctttccatatttcgatttgagactgagccagtaggctctgagtcgctatcactgtacataaaatagcttaactcaccaaaacctgtcattatctgccttaacatggtctgaattgcaacagatgtagtctcacttaaaccagtatttaagattctacgaatgggaattctgatggtactgacataggttctcacacctgcccgctcagaacgtgaaaatgtacgcctaaaacctcctcgttcactttcataggtgacagtgttgtttggtgtctgagacctagaccgagttctgctggctatgctatctctctgccgatattctccaggacgaactcttcttacttgaagatcaaggactatggttggaggtctctgtcctgatcctgtagattcaccactggcagctgtgtctgaagaacctgctccttgagaagcatttcttgttccagaagctgcaaaaagacctctacttagcaactcaggcccagatatttgctgcctcaatgtcacatggtgccgggttctagaacttccctccgtctcatttaccaaaggatgttcaaaagtctgagatgagatactatgatgagatcttcgtggaatttcactcattggatgcagaggtgacctacttctttcagctcttgctctggttctccgatggtctgggctcctgcttcttgccctcctctgacctctggtaggtgggacctctgttaacgcttcagttgaatttcgttctgatctagatggccttgcagatgttgattcagatcgtgggttttccacttgcctttggctgttgttttccacattttctccactagaacgtcttgcagatggctcattttcattctctgaattttggctcccattattacggttaacatttatctctaaactgaatctgaaatcaccactgtttggattagtccgactcactgctctccaagattggtttcctctttgcccacttcttgttgtatttccagtttgtctgacagagttaagccagtctattatagagtcaccattagacacatcatctgaagagtctcctcctctattttcatctgagttttgcggtggtgggccttctttaatttgctgtagtcgtctcagcaactcttcctcagtactttcacctggggtgcctagcaaattgttatctctcataagcctataatcttcttcactcaggttatttacaaattgatagaaagcttcttctcgatccaatcggtccatctgacttctgcgctgtgctgcagactgatcaccacttcctttgtcattggaatctgagttttccatattgatgaacaagtggaaaatacctgactgttatgacatagtattgaaatacaataaactggattttagttttcttcactctgcttaggttttagggtcaggatccgactcggttggttcggccgccgccgccgaggctgctccgcacctccctggccgccgctctcaagcccgcctccaatgagtagctggttgagacccgcctctagcccagcgcctgctcggagacgttgctcaggcagccattatcttccccattgttaccaagcagcgacaggaaacgactgc

SEQ ID NO: 18175 - RNA, 5194 nt, Homo sapiens
  source 1..5194: mol_type = other RNA
tgaagtaccagctactcgagaggctgagacaggagaattgcttgaacccaggaggcagaggttgcagtgagccgagatcgctccattgcacttcatcctgggcaaccaagtaagactctgtctcaaaaaaacaaaacaaaacaaaacaaaacaaaaaaacctcaactttgtcagctgctcagagttaaaacaattcaaatgtttcagactagaagtgagtttttaaaaacatctgaaatattcaagaaaatttgggttttggtacttttccttatgctctgaacaatgtgaactcccaacattgtttatccttgttcctcttactgcatgaagttcaaactaggtcttaaagacaacttttctgtacttaagaaaaagtgcaaagatagaaaatgaaatgtaaggtgttttgcaagaaatgctccctcgagaatggtgtttggatgtgggtggggggaaaacgatttttgttctccattgtaatctgacacctacgaatgaccttgtcttcaatgtccacaacactagtaagcatgtaataatcacggacatcgcaagattaaaaattaagtagcaaattccactaaaacacttgtattcattctatacaatcgaatggaaatccgtgagtgctactgaaaaaggtgttcacatgcacatgtccaatatgtgcattccactgaaggctaaaagcttaaaattctatttccagtgtttatgaatagcttcaatatctacattcatagccagcattctgcttgagttacctcttactttaatacttcacaaatgagtaagtacgtcttgggagattaggaaggtacctgttgtcaataactttctcttatgcttagaatgtgctgcaattgtttttaaactatttaaaatgaacacccctataataatgaaacactttatgccaagaagaaaattgatttgtttttagccaatcaagactaccctgcagatctgaaaactgtagattacatccttaggaaaggagaaaaggaggctcacaaatataaaggaatcctgacttttacacggacaaatttttaaaaagataaaatgtattacataagcgccataaacagtgaaatctgcttatattaaaaaaaataagtgaagctttgtttggacattatttccttgcaagagcagtacatatccttagtaaacaactaccatatttacaagttaatttccttgatacttagataggattgaaagccagaagaaatcatggaagagtgagctttgaaataatctttacagctaagttggtaacagtgaaggtacccagacaattcctaaagcagacttgtttattttgtagagtatttgactacgtctgggtagctagcttgctttgataaaggccaaggacaagttcaatccctattttggcctgttaaagcttttcccagaagaacaaatatctgctccatagtcattctaatcctaaccccagctagtctcaaaaaagaaattaggcaagaagactggggttatcatgaagttactcttactactaagaaaccaacataaagtgcatgtccatagatagcgagtcagcagtctcattttcatatatgggcagcacaattaaaatttgaatttcaaataacccaacatgactttcaacaaaggataaaaatcccttaatcttcaactggtctttaaatttgagatgttaggactgtgttagagatagtaatgaaatatgatcaagtgtgcactggtaccttaaatgacaaatctcaaaaacaacacaaattcgagactttcctattaacacacacatgtgtaccaactgcaattcatatgctaaaagtggttttatagtctctttcctccattttttcatttttgaggagcagacttgtaaatttaacttgtgctaggtagtagtggtttgtttttcttaaaccaaaactctgccaaacttgctgatcttctgcttcatctactcaggtagaataccaggtcaagctgctgctgtggctgctctcaccatatgaaaccagtttgtgtctgcattattactgtcttcaggaaaactttaaattcttcagttttctttactcctcccatatttcacttcctgcctaaatccaagttaaattatacaatttccactggtcttcaacacggtttaattctgcactgtcctttcctttgcatgtcacagtagctgttcacacattaaatattatagatatgttctgctcttgacatctacacacttacaaaagcagctttgtactttgtttggtgtgtttgttactatgttggctcacaaaaagcagttttctcagttctaagcatggtactttacaatttttaatgcattcatacaacagtgcattggaaaagtactgagcctctacaaaatagctttacatttttaaacaaatgaatgtgattttttttcacttacacaagcataggctttttaatatttccacaagataaatatctcaattaaactataagctcactctacagtgtgccacagtgatgggcttaggagacagttatacacttagaagatcctaaccttagtgttatttacactgacatgtccagtatcaccaagtctgaaaggtgaacaaacaatactcagaatgtggctgaatttgtgttaactaataactgggaatgatatagctttaatcacttatgaaacacatactgtaacttagtctaaactggtaatttcctttgctcctctcttatggtgtgggaaaatttaaagatcaacatgaaaaaggagccattgctaaggcagatcttttaagataacaaaggaaaaattgacaagtgtatatgataaattatcagtaacagtgatgctaccaatttaactggtacggaaatcagatttttaggtcctataacgtggcttttaaaatatttccttttattctggaacaaaaactggagaaaggacaatgattccttcagaaagcaatgactcaattcaggttgttactttacatttaagtaccactcaaaaagtggacataaaagcaagtgattcctgtttgcccatcactatatcagctacatagctgagagttcagatcttaattacacaacactttctctgttaccagaagctaagactgctctgcgacaaataggacaggtagaattctcagataaccagcgatcgatgcagtggacatggtactcatgggaacaaggtagtttacgaagtttgttgccttctgtatattctgtaatgcaaacactacaggtttttaatgcatcattttcaccaaaacttctcattgccaagttgtcaatctgttctttggtgagtcctctaggttggtcatcatcatcctcatttaagaggaaaaactgagccaggctaaggaagggcaaagagccactttcatcaaatgtgactggggccctatgtcgaccctctcgcctggcacctgatgagcctgatgatgagcttccttcattactgccttcaaataaatctgagctagtttctgaactttcaccaccggaactggaactaggactggaactggaacttgaactggaactggaactcgaactggaactggaactcgaactggaaccagaactactaccaccaccagaacctcctcttccactccgtgactctgccctttccatatttcgatttgagactgagccagtaggctctgagtcgctatcactgtacataaaatagcttaactcaccaaaacctgtcattatctgccttaacatggtctgaattgcaacagatgtagtctcacttaaaccagtatttaagattctacgaatgggaattctgatggtactgacataggttctcacacctgcccgctcagaacgtgaaaatgtacgcctaaaacctcctcgttcactttcataggtgacagtgttgtttggtgtctgagacctagaccgagttctgctggctatgctatctctctgccgatattctccaggacgaactcttcttacttgaagatcaaggactatggttggaggtctctgtcctgatcctgtagattcaccactggcagctgtgtctgaagaacctgctccttgagaagcatttcttgttccagaagctgcaaaaagacctctacttagcaactcaggcccagatatttgctgcctcaatgtcacatggtgccgggttctagaacttccctccgtctcatttaccaaaggatgttcaaaagtctgagatgagatactatgatgagatcttcgtggaatttcactcattggatgcagaggtgacctacttctttcagctcttgctctggttctccgatggtctgggctcctgcttcttgccctcctctgacctctggtaggtgggacctctgttaacgcttcagttgaatttcgttctgatctagatggccttgcagatgttgattcagatcgtgggttttccacttgcctttggctgttgttttccacattttctccactagaacgtcttgcagatggctcattttcattctctgaattttggctcccattattacggttaacatttatctctaaactgaatctgaaatcaccactgtttggattagtccgactcactgctctccaagattggtttcctctttgcccacttcttgttgtatttccagtttgtctgacagagttaagccagtctattatagagtcaccattagacacatcatctgaagagtctcctcctctattttcatctgagttttgcggtggtgggccttctttaatttgctgtagtcgtctcagcaactcttcctcagtactttcacctggggtgcctagcaaattgttatctctcataagcctataatcttcttcactcaggttatttacaaattgatagaaagcttcttctcgatccaatcggtccatctgacttctgcgctgtgctgcagactgatcaccacttcctttgtcattggaatctgagttttccatattgatgaacaagtggaaaatactaggttttagggtcaggatccgactcggttggttcggccgccgccgccgaggctgctccgcacctccctggccgccgctctcaagcccgcctccaatgagtagctggttgagacccgcctctagcccagcgcctgctcggagacgttgctcaggcagccattatcttccccattgttaccaagcagcgacaggaaacgactgc

SEQ ID NO: 18176 - RNA, 45 nt, Homo sapiens
  source 1..45: mol_type = other RNA
tgaagtaccagctactcgagaggctgagactggagaattgctgga

SEQ ID NO: 18177 - RNA, 1517 nt, Homo sapiens
  source 1..1517: mol_type = other RNA
tgaagtaccagctactcgagaggctgagatgggaggatcacctgagcctcgggaggtcgaggctggaggctgcattgactcatgattgcaccgctgcattctagcctggttgacagaacaagaccatctcaaaaaaaagaaagaaagaaaaaagctagcccccaagtatcacacaggaggtggaggctggggatgagtctttaaattcctcacgtattaccataactcagattttctttcagtctatttctagatgtttctatagccccctagcctgggcacaatgctggcacattacagatgctcaatacacacaaataagcaaataagtacaatgaattaatagaaaggatgaatcccagttgcttgggaggctgaggcaggaggatcgtctaagtccaggagttcaagaccagcctcggcaatgtcgaagacccccccccccccaaaacaactcctctaaaaaagtccattcacaaactcaggatcctctttaaatagaaatatatatatatatataatatatataatatattatctgagctcaggctcagaataaatatcaaggtccaacttggggaaggagtgggtgaggagggtcctcaaggggaggtcagcagcagggacccctgccaagccccttgaggtagagaaagcagcagggacccagcaccaggggtctccatgaaggatggagtaggattcggactctgtccaggtgggctgcacccaggctggacgttattccgacctcggtgaagggagtccggctgggatttcgggggtcacccggaagagtcccaagactgtggcgccctgggtaagctgccaggcatggcgtgccctggcctcagtgtgaagatggacgcccaggcgctggccggcactcaggtgcagcaagcggccctggaaaccgaaggccgagttccgagcctcggaggaggcgggtggcaggtccacggtcaaagccagggcggcggccccagcagcagagcgcagtggctgcaggtgcagcgcaagtgaaacggagcctgagccctcgccggccaccacgcgccgcagctctagttgaaagaagacatagtagactccagccttggccaccaccagctccttcgtgtcctctttgtagctcaggccccccgtcagggacacgcctgccaggcctgggtcactgtaccagctcaggggcccatcgatcagcagaacattttgggccaccagctgcgcaaacatgccctgccgcaggtccaagaggccggcgggatcgtcgggcgaaagctcgggaccctcgcggagtctcgggctggccgcggagccgggcgaggcgcgagccccggacacggcccaggggcaggcgaggaagacggcgcaggcggcagcgagcagcagcagcagcagcagccccgcgaccagggcccaaggcagtacgcggcaggcgcgagcgcggggcgcgggaggccacggggcttcggggtccagtgaagcgtcagaggcgtattccatgacgagagact

SEQ ID NO: 18178 - RNA, 940 nt, Homo sapiens
  source 1..940: mol_type = other RNA
tgaagtaccagctactcgagaggctgagcaccaaaatggggatgctagtcacacttacgtcctagggttcttggggatgaaatgggttcttacttgtacaactcttgaagtggtgtgcctggcatgtgacaagcatgcagcagatgtgatgctagctttcattattattggctatttgccatatccacggatgtcatcttgtcccttgtctcctttaattattgacagaagttgacacaagtgatcatctcatcctttaaaaagtgctttctctcttcccttggctactaggacactttactgtcgtcgttcttttccagtgtcattggccattttcagctccttcattagtttctctcccacttgtcttttaaatgcatgtatttctcaaggatctcttcatctaaatgtccttccctcaaattgctgtcttgtgcattttcctttttagttaatactattatatcctccaagtcactcaggattgttaccgtgaaatcatccagaattctgtctcctcctttgtctcccttttcagaccactccaaagctgaccttttttcaaattttgttgattggacctaccccatcttatgcatggccttctcatgttcgatgctacgatcccattttggatatctggtcattctctttttctgtcttctcattactgtcagagttctctttcttaaagttcagccctaatgtcactccccattgcatgaagtggtggtctccaaagaggggcgtgtagcaaagagagttgacgtgaggctcaagtcatcttagggctcatcatcaaatgccatgcttgaagaactttgtgaaatcttggacaactcatagttctgttgaaggaggccatcatctttcctccatgtttgcaacatatttttcttcaatcctggaggctgggaagtccaagatcaagttgccggca

SEQ ID NO: 18179 - RNA, 1010 nt, Homo sapiens
  source 1..1010: mol_type = other RNA
tgaagtaccagctactcgagaggctgagcaccaaaatggggatgctagtcacacttacgtcctagggttcttggggatgaaatgggttcttacttgtacaactcttgaagtggtgtgcctggcatgtgacaagcatgcagcagatgtgatgctagctttcattattattggctatttgccatatccacggatgtcatcttgtcccttgtctcctttaattattgacagaagttgacacaagtgatcatctcatcctttaaaaagtgctttctctcttcccttggctactaggacactttactgtcgtcgttcttttccagtgtcattggccattttcagctccttcattagtttctctcccacttgtcttttaaatgcatgtatttctcaaggatctcttcatctaaatgtccttccctcaaattgctgtcttgtgcattttcctttttagttaatactattatatcctccaagtcactcaggattgttaccgtgaaatcatccagaattctgtctcctcctttgtctcccttttcagaccactccaaagctgaccttttttcaaattttgttgattggacctaccccatcttatgcatggccttctcatgttcgatgctacgatcccattttggatatctggtcattctctttttctgtcttctcattactgtcagagttctctttcttaaagttcagccctaatgtcactccccattgcatgaagtggtggtctccaaagaggggcgtgtagcaaagagagttgacgtgaggctcaagtcatcttagggctcatcatcaaatgccatgcttgaagaactttgtgaaatcttggacaactcatagttctgttgaaggaggccatcatctttcctccatgtttgcaacatatttttcttcctaggtttgtaaaaagccaattagcatcatcaatctagtgaatattttttatttccaaatcatgtatttcctactagtctttttatttttattttatttttatttattta

SEQ ID NO: 18180 - RNA, 487 nt, Homo sapiens
  source 1..487: mol_type = other RNA
tgaagtaccagctactcgagaggctgaggcaagagaattgcttgaactcgggaggcagaggttgcagtgagtcgagatcacaccaccgcactccagcctgggcgacagaatgagattctgggggtttggctaccatctcctgtctcttcctattccagggctcttttccttgctccaaacaggttatcaggtgaggcttagagacagcaatacccaggaagaccaggtttctgtagttctcaaacatcactttcctatataaattccgttgtgcagtgtccaggcattgccactcctccagagagaattctatggccacatccctaaatgtcagtggtcccatttctaggcttccaggtggtcctggcatcttagctgtgcatctcccaatacctgcagataacggagtcacagaggctgggcctctaggagcagaatacacagagcagtaaagactagacctggagctcccgcagcagctagagac

SEQ ID NO: 18181 - RNA, 551 nt, Homo sapiens
  source 1..551: mol_type = other RNA
tgaagtaccagctactcgagaggctgaggcaagagaattgcttgaactcgggaggcagaggttgcagtgagtcgagatcacaccaccgcactccagcctgggcgacagaatgagattctgggggtttggctaccatctcctgtctcttcctattccagggctcttttccttgctccaaacaggttatcaggtgaggcttagagacagcaatacccaggaagaccaggtttctgtagttctcaaacatcactttcctatataaattccgttgtgcagtgtccaggcattgccactcctccagagagaattctatggccacatccctaaatgtcagtggtcccatttctaggcttccaggtggtcctggcatcttagctgtgcatctcccaatacctgcagataacggagtcacagaggctgggcctctaggagcagaatacacagagcagtaaagactagacctggagctcccgcagcagctagagacaaaggccccgccaaatcccggaagccgtcctgtccgctccagctgcgtgcctgattggacgggt

SEQ ID NO: 18182 - RNA, 819 nt, Homo sapiens
  source 1..819: mol_type = other RNA
tgaagtaccagctactcgagaggctgaggcaagagaattgcttgaactcgggaggcagaggttgcagtgagtcgagatcacaccaccgcactccagcctgggcgacagaatgagattctgggggtttggctaccatctcctgtctcttcctattccagggctcttttccttgctccaaacaggttatcaggtgaggcttagagacagcaatacccaggaagaccaggtttctgtagttctcaaacatcactttcctatataaattccgttgtgcagtgtccaggcattgccactcctccagagagaattctatggccacatccctaaatgtcagtggtccctcttttacaccattcgtaaatattttaccttttaatttcctttacaaatttttcactatttgtctttcactcttttttcatcattttttttcactatttttctgcccccttagagaatccagaaattatttctatgtttttccctcaataccagcatctgattgaccagcaatgtgtcccaaggaaacggaagctgagttgggtgaagacaatcttaatgtctcaaggtgtcagcctttccaaggaagagtgcaccaggagatttctctcagctccagggcatccacctgctccctcgagaggctacactttgtacctcaggcagtccatttctaggcttccaggtggtcctggcatcttagctgtgcatctcccaatacctgcagataacggagtcacagaggctgggcctctaggagcagaatacacagagcagtaaagactagacctggagctcccgcagcagctagagacaaag

SEQ ID NO: 18183 - RNA, 560 nt, Homo sapiens
  source 1..560: mol_type = other RNA
tgaagtaccagctactcgagaggctgaggcaagagaattgcttgaactcgggaggcagaggttgcagtgagtcgagatcacaccaccgcactccagcctgggcgacagaatgagatttctctaatcatcccaaactcctcccagccacagtctgggagagaccgtgcccttccagaggcctggaggaagacagccatttatagccacgcaggcaggcctgcagaccttgtcctttactgtggtttctgaagcagttcgatgactcagttccagctccctgagccacagttcacggccagttctgcctgggggtttggctaccatctcctgtctcttcctattccagggctcttttccttgctccaaacaggttatcaggtgaggcttagagacagcaataccatttctaggcttccaggtggtcctggcatcttagctgtgcatctcccaatacctgcagataacggagtcacagaggctgggcctctaggagcagaatacacagagcagtaaagactagacctggagctcccgcagcagctagagacaaaggccccgcc

SEQ ID NO: 18184 - RNA, 630 nt, Homo sapiens
  source 1..630: mol_type = other RNA
tgaagtaccagctactcgagaggctgaggcaagagaattgcttgaactcgggaggcagaggttgcagtgagtcgagatcacaccaccgcactccagcctgggcgacagaatgagatttctctaatcatcccaaactcctcccagccacagtctgggagagaccgtgcccttccagaggcctggaggaagacagccatttatagccacgcaggcaggcctgcagaccttgtcctttactgtggtttctgaagcagttcgatgactcagttccagctccctgagccacagttcacggccagttctgcctgggggtttggctaccatctcctgtctcttcctattccagggctcttttccttgctccaaacaggttatcaggtgaggcttagagacagcaatacccaggaagaccaggtttctgtagttctcaaacatcactttcctatataaattccgttgtgcagtgtccaggcattgccactcctccagagagaattctatggccacatccctaaatgtcagtggtcccatttctaggcttccaggtggtcctggcatcttagctgtgcatctcccaatacctgcagataacggagtcacagaggctgggcctctaggagcagaatacac

SEQ ID NO: 18185 - RNA, 1007 nt, Homo sapiens
  source 1..1007: mol_type = other RNA
tgaagtaccagctactcgagaggctgaggcaagagaattgcttgaactcgggaggcagaggttgcagtgagtcgagatcacaccaccgcactccagcctgggcgacagaatgagatttctctaatcatcccaaactcctcccagccacagtctgggagagaccgtgcccttccagaggcctggaggaagacagccatttatagccacgcaggcaggcctgcagaccttgtcctttactgtggtttctgaagcagttcgatgactcagttccagctccctgagccacagttcacggccagttctgcctgggggtttggctaccatctcctgtctcttcctattccagggctcttttccttgctccaaacaggttatcaggtgaggcttagagacagcaatacccaggaagaccaggtttctgtagttctcaaacatcactttcctatataaattccgttgtgcagtgtccaggcattgccactcctccagagagaattctatggccacatccctaaatgtcagtggtccctcttttacaccattcgtaaatattttaccttttaatttcctttacaaatttttcactatttgtctttcactcttttttcatcattttttttcactatttttctgcccccttagagaatccagaaattatttctatgtttttccctcaataccagcatctgattgaccagcaatgtgtcccaaggaaacggaagctgagttgggtgaagacaatcttaatgtctcaaggtgtcagcctttccaaggaagagtgcaccaggagatttctctcagctccagggcatccacctgctccctcgagaggctacactttgtacctcaggcagtccatttctaggcttccaggtggtcctggcatcttagctgtgcatctcccaatacctgcagataacggagtcacagaggctgggcctctaggagcagaatacacagagcagtaaagactagacctggagctcccgcagcagctagagacaaag

SEQ ID NO: 18186 - RNA, 1126 nt, Homo sapiens
  source 1..1126: mol_type = other RNA
tgaagtaccagctactcgagaggctgaggcacaagaatcgcttgaacccaggaggcagaggttgcagtgagccaagatcacaccactgcactccagcctggcgacagagtgagactctgcctcaaaaaaaaaaaaaaaaaaaaaaaagcaagacagaaaataacaaagactccttagcccaaattgtaccagcaagactaaagaaaataatttttctacttcacgattcctttccttaactgtaaattgatgacactgtacttaatactttaaaaacccagtcaaagcaaaccaatgacttgatcctaccaactctaaggaaactaagggtatacaccctaagttatccaaacacaactgaggttgaggtcattaaaccggtaagtatacgccctatactaactcacagctgaaagtgtacatggagcaaaaaacaaagaatacatatcccaagcgaatattttgtctggtgacacatcaggaagccacaagctccacttcatttaaaaaattatttgggtatcagcggtgtggcaaacattcaaaattctccttcaaacagttggaagaaaacatgtaatacattccagagcaaagatgaatcaaaaagtatctttttgctcaggaaaagaatttcttcattcaattacagcataattcattgaaaggggaagtcatgagtctcttatgagagttcctgaacagtttataaatacaacaagaacatttattcaataaataagtggttcctaaagtctttactgatgatctccaggattgtccatcgctatggtccaggccagctccactttctctgacaggctttagctgccagtggaatgggatgtttcctgtctttaggtgactcttcttgtgtcatacagactttcatcaatatgtctcttcatagtctgaatccaggcactcagcgcaacggacacaaagcctcgccatacacgcctcttcctcctcctgatcagtgcctggaagaacaggacgcccagcagagggaagagagcgcagccacggcttccagctgctcctctctgctgcatcccggcagctcttcagatgcttgcacaccttgtttacagctcccggtaacgacacaggtaacaccggaagt

SEQ ID NO: 18187 - RNA, 1634 nt, Homo sapiens
  source 1..1634: mol_type = other RNA
tgaagtaccagctactcgagaggctgaggcacaagaatcgcttgaacccaggaggcagaggttgcagtgagccaagatcacaccactgcactccagcctggcgacagagtgagactctgcctcaaaaaaaaaaaaaaaaaaaaaaaagcaagacagaaaataacaaagactccttagcccaaattgtaccagcaagactaaagaaaataatttttctacttcacgattcctttccttaactgtaaattgatgacactgtacttaatactttaaaaacccagtcaaagcaaaccaatgacttgatcctaccaactctaaggaaactaagggtatacaccctaagttatccaaacacaactgaggttgaggtcattaaaccggtaagtatacgccctatactaactcacagctgaaagtgtacatggagcaaaaaacaaagaatacatatcccaagcgaatattttgtctggtgacacatcaggaagccacaagctccacttcatttaaaaaattatttgggtatcagcggtgtggcaaacattcaaaattctccttcaaacagttggaagaaaacatgtaatacattccagagcaaagatgaatcaaaaagtatctttttgctcaggaaaagaatttcttcattcaattacagcataattcattgaaaggggaagtcatgagtctcttatgagagttcctgaacagtttataaatacaacaagaacatttattcaataaataagtggttcctaaagtctttactgatgatctccaggattgtccatcgctatggtccaggccagctccactttctctgacaggctttagctgccagtggaatgggatgtttcctgtctttaggtgactcttcttgtgtcatacagactttcatcaatatgtctcttcatagtctgaatccaggcactcagcgcaacggacacaaagcctcgccatacacgcctcttcctcctcctgatcagtgtcatcggaaacctcaatagatgacttcttatagccagacctgctcctcttcttcagcccagcagccttcctccccattctcaccagcagcagagcaaccaccacggctgagggcacaaagacaaggatggaaagaagggccacagaggaaagcatggtgccaaaacccctttctgtgactgttagctctgtcatgggaatattatgatgcacatctgggggattcttcacagcacagctgaatgtcccattgtcctttatggtagggttgcttatacttatagatgcatcccctttgtatacatttccaacccaggaaatccgatcccgaaatgtgcctgctgtggttgggtactggaaagactgataatgaaatattgatactgtgtggctgctgctgggagggcgatatgtccagtctatagtaagtttgtcagtgacatctgaagttgacttgaaagtgcatttcaacttgatcttttctccaacataacctcggacatgggcatcctggaagaacaggacgcccagcagagggaagagagcgcagccacggcttccagctgctcctctctgctgcatcccggcagctcttcagatgcttgcacaccttgtttacagctcccggtaacgacacaggtaacaccggaagt

SEQ ID NO: 18188 - RNA, 1784 nt, Homo sapiens
  source 1..1784: mol_type = other RNA
tgaagtaccagctactcgagaggctgaggcacaagaatcgcttgaacccaggaggcagaggttgcagtgagccaagatcacaccactgcactccagcctggcgacagagtgagactctgcctcaaaaaaaaaaaaaaaaaaaaaaaagcaagacagaaaataacaaagactccttagcccaaattgtaccagcaagactaaagaaaataatttttctacttcacgattcctttccttaactgtaaattgatgacactgtacttaatactttaaaaacccagtcaaagcaaaccaatgacttgatcctaccaactctaaggaaactaagggtatacaccctaagttatccaaacacaactgaggttgaggtcattaaaccggtaagtatacgccctatactaactcacagctgaaagtgtacatggagcaaaaaacaaagaatacatatcccaagcgaatattttgtctggtgacacatcaggaagccacaagctccacttcatttaaaaaattatttgggtatcagcggtgtggcaaacattcaaaattctccttcaaacagttggaagaaaacatgtaatacattccagagcaaagatgaatcaaaaagtatctttttgctcaggaaaagaatttcttcattcaattacagcataattcattgaaaggggaagtcatgagtctcttatgagagttcctgaacagtttataaatacaacaagaacatttattcaataaataagtggttcctaaagtctttactgatgatctccaggattgtccatcgctatggtccaggccagctccactttctctgacaggctttagctgccagtggaatgggatgtttcctgtctttaggtgactcttcttgtgtcatacagactttcatcaatatgtctcttcatagtctgaatccaggcactcagcgcaacggacacaaagcctcgccatacacgcctcttcctcctcctgatcagtgtcatcggaaacctcaatagatgacttcttatagccagacctgctcctcttcttcagcccagcagccttcctccccattctcaccagcagcagagcaaccaccacggctgagggcacaaagacaaggatggaaagaagggccacagaggaaagcatggtgccaaaacccctttctgtgactgttagctctgtcatgggaatattatgatgcacatctgggggattcttcacagcacagctgaatgtcccattgtcctttatggtagggttgcttatacttatagatgcatcccctttgtatacatttccaacccaggaaatccgatcccgaaatgtgcctgctgtggttgggtactggaaagactgataatgaaatattgatactgtgtggctgctgctgggagggcgatatgtccagtctatagtaagtttgtcagtgacatctgaagttgacttgaaagtgcatttcaacttgatcttttctccaacataacctcggacatgggcatctgcacgaatctccaaggaaaagacgatataaacaccccaagtatagcatggttgcatcatgaagctaccattgcctcatcaacagcaaaatgagaataggaagtaagaatgggagaatttatttcaaataattttctaaaactgcccccaaggtactatctagtttttccctttttcttaaagctggctgaggaatcacacatccattaaaagtaaatcatggagaagaaaacagaataggtaaatgcattctagcaagtaaaaataaggtaccattttaaaacccactagag

SEQ ID NO: 18189 - RNA, 1670 nt, Homo sapiens
  source 1..1670: mol_type = other RNA
tgaagtaccagctactcgagaggctgaggcacaagaatcgcttgaacccaggaggcagaggttgcagtgagccaagatcacaccactgcactccagcctggcgacagagtgagactctgcctcaaaaaaaaaaaaaaaaaaaaaaaagcaagacagaaaataacaaagactccttagcccaaattgtaccagcaagactaaagaaaataatttttctacttcacgattcctttccttaactgtaaattgatgacactgtacttaatactttaaaaacccagtcaaagcaaaccaatgacttgatcctaccaactctaaggaaactaagggtatacaccctaagttatccaaacacaactgaggttgaggtcattaaaccggtaagtatacgccctatactaactcacagctgaaagtgtacatggagcaaaaaacaaagaatacatatcccaagcgaatattttgtctggtgacacatcaggaagccacaagctccacttcatttaaaaaattatttgggtatcagcggtgtggcaaacattcaaaattctccttcaaacagttggaagaaaacatgtaatacattccagagcaaagatgaatcaaaaagtatctttttgctcaggaaaagaatttcttcattcaattacagcataattcattgaaaggggaagtcatgagtctcttatgagagttcctgaacagtttataaatacaacaagaacatttattcaataaataagtggttcctaaagtctttactgatgatctccaggattgtccatcgctatggtccaggccagctccactttctctgacaggctttagctgccagtggaatgggatgtttcctgtctttaggtgactcttcttgtgtcatacagactttcatcaatatgtctcttcatagtctgaatccaggcactcagcgcaacggacacaaagcctcgccatacacgcctcttcctcctcctgatcagtgtcatcggaaacctcaatagatgacttcttatagccagacctgctcctcttcttcagcccagcagccttcctccccattctcaccagcagcagagcaaccaccacggctgagggcacaaagacaaggatggaaagaagggccacagaggaaagcatggtgccaaaacccctttctgtgactgttagctctgtcatgggaatattatgatgcacatctgggggattcttcacagcacagctgaatgtcccattgtcctttatggtagggttgcttatacttatagatgcatcccctttgtatacatttccaacccaggaaatccgatcccgaaatgtgcctgctgtggttgggtactggaaagactgataatgaaatattgatactgtgtggctgctgctgggagggcgatatgtccagtctatagtaagtttgtcagtgacatctgaagttgacttgaaagtgcatttcaacttgatcttttctccaacataacctcggacatgggcatctgcacgaatctccaaggaaaagacgatataaacaccctggaagaacaggacgcccagcagagggaagagagcgcagccacggcttccagctgctcctctctgctgcatcccggcagctcttcagatgcttgcacaccttgtttacagctcccggtaacgacacaggtaacaccggaagt

SEQ ID NO: 18190 - RNA, 2025 nt, Homo sapiens
  source 1..2025: mol_type = other RNA
tgaagtaccagctactcgagaggctgaggcacaagaatcgcttgaacccaggaggcagaggttgcagtgagccaagatcacaccactgcactccagcctggcgacagagtgagactctgcctcaaaaaaaaaaaaaaaaaaaaaaaagcaagacagaaaataacaaagactccttagcccaaattgtaccagcaagactaaagaaaataatttttctacttcacgattcctttccttaactgtaaattgatgacactgtacttaatactttaaaaacccagtcaaagcaaaccaatgacttgatcctaccaactctaaggaaactaagggtatacaccctaagttatccaaacacaactgaggttgaggtcattaaaccggtaagtatacgccctatactaactcacagctgaaagtgtacatggagcaaaaaacaaagaatacatatcccaagcgaatattttgtctggtgacacatcaggaagccacaagctccacttcatttaaaaaattatttgggtatcagcggtgtggcaaacattcaaaattctccttcaaacagttggaagaaaacatgtaatacattccagagcaaagatgaatcaaaaagtatctttttgctcaggaaaagaatttcttcattcaattacagcataattcattgaaaggggaagtcatgagtctcttatgagagttcctgaacagtttataaatacaacaagaacatttattcaataaataagtggttcctaaagtctttactgatgatctccaggattgtccatcgctatggtccaggccagctccactttctctgacaggctttagctgccagtggaatgggatgtttcctgtctttaggtgactcttcttgtgtcatacagactttcatcaatatgtctcttcatagtctgaatccaggcactcagcgcaacggacacaaagcctcgccatacacgcctcttcctcctcctgatcagtgtcatcggaaacctcaatagatgacttcttatagccagacctgctcctcttcttcagcccagcagccttcctccccattctcaccagcagcagagcaaccaccacggctgagggcacaaagacaaggatggaaagaagggccacagaggaaagcatggtgccaaaacccctttctgtgactgttagctctgtcatgggaatattatgatgcacatctgggggattcttcacagcacagctgaatgtcccattgtcctttatggtagggttgcttatacttatagatgcatcccctttgtatacatttccaacccaggaaatccgatcccgaaatgtgcctgctgtggttgggtactggaaagactgataatgaaatattgatactgtgtggctgctgctgggagggcgatatgtccagtctatagtaagtttgtcagtgacatctgaagttgacttgaaagtgcatttcaacttgatcttttctccaacataacctcggacatgggcatctgcacgaatctccaaggaaaagacgatataaacacgtcttccaaaaccactcatttatccaactctgacacttcatctctctgaaaagggctggcactttgttctaaccagttccttctgctttcagagaacaaaaacttatctttccctacaggggcatattttaggaaatgacattgccagtactttgttcttcctgcttccttatctacctcaagaagccatgaatcttctgctggccaagataaacagagcagcaagatttcagaaaagtgcaaacccacacgctgtcctgaaaatcggcagtgcttctggtacaggcagaatggtgttgtgattgagcacgcaggccacggctcctacaccagagggtctgggttcaaatcccggccctgtcacctgctggctctgcagccttagtaagttaccgtacttcttcagtcttctcagcctcatgggaatgataataacagtacttacctcagaaggccactgtgaggattaaaagagttaaaacacatacaacactaagaa

SEQ ID NO: 18191 - RNA, 1459 nt, Homo sapiens
  source 1..1459: mol_type = other RNA
tgaagtaccagctactcgagaggctgaggcacaagaatcgcttgaacccaggaggcagaggttgcagtgagccaagatcacaccactgcactccagcctggcgacagagtgagactctgcctcaaaaaaaaaaaaaaaaaaaaaaaagcaagacagaaaataacaaagactccttagcccaaattgtaccagcaagactaaagaaaataatttttctacttcacgattcctttccttaactgtaaattgatgacactgtacttaatactttaaaaacccagtcaaagcaaaccaatgacttgatcctaccaactctaaggaaactaagggtatacaccctaagttatccaaacacaactgaggttgaggtcattaaaccggtaagtatacgccctatactaactcacagctgaaagtgtacatggagcaaaaaacaaagaatacatatcccaagcgaatattttgtctggtgacacatcaggaagccacaagctccacttcatttaaaaaattatttgggtatcagcggtgtggcaaacattcaaaattctccttcaaacagttggaagaaaacatgtaatacattccagagcaaagatgaatcaaaaagtatctttttgctcaggaaaagaatttcttcattcaattacagcataattcattgaaaggggaagtcatgagtctcttatgagagttcctgaacagtttataaatacaacaagaacatttattcaataaataagtggttcctaaagtctttactgatgatctccaggattgtccatcgctatggtccaggccagctccactttctctgacaggctttagctgccagtggaatgggatgtttcctgtctttaggtgactcttcttgtgtcatacagactttcatcaatatgtctcttcatagtctgaatccaggcactcagcgcaacggacacaaagcctcgccatacacgcctcttcctcctcctgatcagtgtcatcggaaacctcaatagatgacttcttatagccagacctgctcctcttcttcagcccagcagccttcctccccattctcaccagcagcagagcaaccaccacggctgagggcacaaagacaaggatggaaagaagggccacagaggaaagcatggtgccaaaactgatactgtgtggctgctgctgggagggcgatatgtccagtctatagtaagtttgtcagtgacatctgaagttgacttgaaagtgcatttcaacttgatcttttctccaacataacctcggacatgggcatctgcacgaatctccaaggaaaagacgatataaacaccctggaagaacaggacgcccagcagagggaagagagcgcagccacggcttccagctgctcctctctgctgcatcccggcagctcttcagatgcttgcacaccttgtttacagctcccggtaacgacacaggtaacaccggaagt

SEQ ID NO: 18192 - RNA, 3925 nt, Homo sapiens
  source 1..3925: mol_type = other RNA
tgaagtaccagctactcgagaggctgaggcacgagaatcgcttgaacctggtaggcagagattgcagtgagctgagattataccaccgcactccagcctgagtgacagagtgagatatggcctcaaaaaacaaaaaaaagccacacagaatacaagcaagaaagtacttttagattaaaattcgtcttatgtgaattatggcaaatgaaatcaccccactgtttacctgttttatgagtttttacatttgcttaaaattagcatacttgatcttttacagttcccatctccaccaattagtattggcagatttccactatatgtagaagtcaaaagatcagactgtaaaaatatcagatattgtaattaagagctccaaacaagtcttgcagtttcaaaggtagaaacccacccagccagttcagctgcttggacttcaaagccctccgcctagccatctcagccaggctcaggttccttctcccacccatcaggccaagcaggacttgtcaaacatacacattcaagttcctagcacacagtaggtgctaagtgggaattgattataaacttgaattcttccatcaacaaatatccacctctcctgtccagcttgcctcagatcttcaggttctctcttctctgaggcagctaagcttctacatccttcatgaagtttcctttacttctcgacagaagacagttccctttaggcctatcatctctaaatgcaactggctttccattttccacttactcaacactccacaaagtacacttgctacatggtatttattcaatgactgtatatttagtcaccacctcaatcactgctaagctctcttcatgtctatctgtaccacagtttcccatcttagactgtgacgtcagctggcaagggctggctgttggccgattcatcatgactgacatggtgtgtcacaaagagctccaagtaaatgctgtgaaggaagaggatgaggatggagatgaggatcctgagaagggcccagactggctgcccaacccatggacctgaggcctgagtaaggcctgggagctgctttcccctctgcccaggaactctgtccaggggcgattctaaggcacagtggtgaaggacatgattggtcccccaagtgtggtcctcaggtctcatggcagccactcgcctgggaacagtgcaacaagcattccatttagaagatcttccagaacacacacaagaagcattgtctaatgaaaatggagacaaggtctttcttggaagagagtgcccaagtagatactctctgccccaagactaaccaggtcccttttaaggtccctgagaacagcagcctgggagcaaccaagcctttcaaaggctgacaaggcacagagtggatgaatggaacgaacgatacatgaaaaaaacactttggctgataaaacctccaacctgaggcagggacagtgtcgctcgctgacatgcagaaacatgactgtagcagagatgatgatgatgagaaatgcttcgcatttcccacactgccgatatcccaagccctgtgctaccaccctctccccgaacacacacacacacacacacacacacacacacacacacacacacacagagcatctgcagaataagtcagaggttgacacccagagcctgacgtcaggataggactcttggcactccgcactgaaacaccgtgattagtcctgactagacagcaaaagtaacgccagcctaagcttgaaatgaagggtccatcttgtgaaaagttaggctgcgcccaagacagccaggtctgggaagtctttcacttctcctacttcgctgaaaggctgtccaccttggttgaatgtcagcttgtaccgtaagcggataggttctttgtgtggattgtcaagcagcagcatctgagatatcacagctggaggcatcaaaggactgaatgcaggaagcttggagctggatgccggctgcagcttcactctcattgactttggcacagccacttgaaacatgatatcccagacaggctggggagccgtgctcatcatggtcaagagcagcacctgtacctctgggtgcccaggggctcccgtctgggagaagtggagcagaattctgaatccattccggtcatacacaatgagaggcggcaggctgctgggcttaacagactccaaagggacaaacacttgagccagaggtgtattctgtgaagatggggaaggagccaacgggccagcctcccaggaccaacctggagaggacttagtacctggtggcacttccttggggacacttttctgcgaaacataattcagagggcacggagctggctgtgctgagaggaggtccagcaaattcctgtctgcagaagggttctgaacaccaccgcctggcagcgtgctggaggagggattcctcttttcctcacagcaattctgaccagaaaccatgcctgtaacaggagcatcactgattcccaaggctgccaggtcctgatgaagcaaagatggcaccacagtccccatctgcgcaggtccattgtccacctccaagtcaatcagggggcaggtcttcatgcagcctgctggattctgaaagactctggagacagggatgtctcccaatgagctggtcactctgtttccaaaggtgacccggccctccatcacctgtttgtacagcagaactccttgggtgaggaggtcatttgcctggagaatttccgcgagtgcatcatcgtcatcagtggtgtcactcgccaaccggaacagcgtgggccgcagcttttcacacctctcatacacgacctgcagggcctcctggtcgggcggggcctgccctggcctgcggtacatgctcagcatctcctgcagcaccttcacatggcttcgcacttcctccaccgcactgaccctcttggacaccttctccgatttttcttgttcctccttgaccaaattcttgattaaccggtttgcagcctgaaggtcctcggggtggttgctctttagaagccttgtcagaagcttggacttttcttcatcagcatcaaagatggagctcttgggccagggagatggtgggggtaagattttatccactggtagtttagggtcttgttttataattccttgtttcttcagcatctgataagcgtctcgaatcttgatgtcttccggaaaccagactgtccaactgaagagtatttcaatgactcttcctttaacttttcctgtggcccaggaccccaggtactttggggacaacactttgatcagttcgttcaggaaacgaaatttggccacctcgctgtggaacttctccccacagtggttcatgcacatctccagcaccgttaaggcataaagagcttccttctcttgcggagactggatcttgtgggccagtagccagggcgcatgtgtggggccattggggtcagtgttcacctgctcacagaaattctggatagctgaccaatcctgttccgacatgcttgggtctgtggctttgtacagcacagtccgagttgaatttttcctgactgcagtcacatttatgtcacgtggaagtcatgtgtctagatagggagggtcaacggacaggtaatcaccatcttcctgcccactgactccattctaagtgaagagagaacacaagggcgagggaaggatcagtgattgattcctatattctcctccccacccccgcaaagctctctcccatgttccgtatcttaaaatcctatctacccttgagtcccaagtcacattccaccctaaagacttctctgacctttttatctcccgtccccataaaacaaaagctgtctcctcctcctctgaacagatattttatctgccccttctccgatagggatctccagctacacccattagtcacatgtacttggac

SEQ ID NO: 18193 - RNA, 3698 nt, Homo sapiens
  source 1..3698: mol_type = other RNA
tgaagtaccagctactcgagaggctgaggcacgagaatcgcttgaacctggtaggcagagattgcagtgagctgagattataccaccgcactccagcctgagtgacagagtgagatatggcctcaaaaaacaaaaaaaagccacacagaatacaagcaagaaagtacttttagattaaaattcgtcttatgtgaattatggcaaatgaaatcaccccactgtttacctgttttatgagtttttacatttgcttaaaattagcatacttgatcttttacagttcccatctccaccaattagtattggcagatttccactatatgtagaagtcaaaagatcagactgtaaaaatatcagatattgtaattaagagctccaaacaagtcttgcagtttcaaaggtagaaacccacccagccagttcagctgcttggacttcaaagccctccgcctagccatctcagccaggctcaggttccttctcccacccatcaggccaagcaggacttgtcaaacatacacattcaagttcctagcacacagtaggtgctaagtgggaattgattataaacttgaattcttccatcaacaaatatccacctctcctgtccagcttgcctcagatcttcaggttctctcttctctgaggcagctaagcttctacatccttcatgaagtttcctttacttctcgacagaagacagttccctttaggcctatcatctctaaatgcaactggctttccattttccacttactcaacactccacaaagtacacttgctacatggtatttattcaatgactgtatatttagtcaccacctcaatcactgctaagctctcttcatgtctatctgtaccacagtttcccatcttagactgtgacgtcagctggcaagggctggctgttggccgattcatcatgactgacatggtgtgtcacaaagagctccaagtaaatgctgtgaaggaagaggatgaggatggagatgaggatcctgagaagggcccagactggctgcccaacccatggacctgaggcctgagtaaggcctgggagctgctttcccctctgcccaggaactctgtccaggggcgattctaaggcacagtggtgaaggacatgattggtcccccaagtgtggtcctcaggtctcatggcagccactcgcctgggaacagtgcaacaagcattccatttagaagatcttccagaacacacacaagaagcattgtctaatgaaaatggagacaaggtctttcttggaagagagtgcccaagtagatactctctgccccaagactaaccaggtcccttttaaggtccctgagaacagcagcctgggagcaaccaagcctttcaaaggctgacaaggcacagagtggatgaatggaacgaacgatacatgaaaaaaacactttggctgataaaacctccaacctgaggcagggacagtgtcgctcgctgacatgcagaaacatgactgtagcagagatgatgatgatgagaaatgcttcgcatttcccacactgccgatatcccaagccctgtgctaccaccctctccccgaacacacacacacacacacacacacacacacacacacacacacacacagagcatctgcagaataagtcagaggttgacacccagagcctgacgtcaggataggactcttggcactccgcactgaaacaccgtgattagtcctgactagacagcaaaagtaacgccagcctaagcttgaaatgaagggtccatcttgtgaaaagttaggctgcgcccaagacagccaggtctgggaagtctttcacttctcctacttcgctgaaaggctgtccaccttggttgaatgtcagcttgtaccgtaagcggataggttctttgtgtggattgtcaagcagcagcatctgagatatcacagctggaggcatcaaaggactgaatgcaggaagcttggagctggatgccggctgcagcttcactctcattgactttggcacagccacttgaaacatgatatcccagacaggctggggagccgtgctcatcatggtcaagagcagcacctgtacctctgggtgcccaggggctcccgtctgggagaagtggagcagaattctgaatccattccggtcatacacaatgagaggcggcaggctgctgggcttaacagactccaaagggacaaacacttgagccagaggtgtattctgtgaagatggggaaggagccaacgggccagcctcccaggaccaacctggagaggacttagtacctggtggcacttccttggggacacttttctgcgaaacataattcagagggcacggagctggctgtgctgagaggaggtccagcaaattcctgtctgcagaagggttctgaacaccaccgcctggcagcgtgctggaggagggattcctcttttcctcacagcaattctgaccagaaaccatgcctgtaacaggagcatcactgattcccaaggctgccaggtcctgatgaagcaaagatggcaccacagtccccatctgcgcaggtccattgtccacctccaagtcaatcagggggcaggtcttcatgcagcctgctggattctgaaagactctggagacagggatgtctcccaatgagctggtcactctgtttccaaaggtgacccggccctccatcacctgtttgtacagcagaactccttgggtgaggaggtcatttgcctggagaatttccgcgagtgcatcatcgtcatcagtggtgtcactcgccaaccggaacagcgtgggccgcagcttttcacacctctcatacacgacctgcagggcctcctggtcgggcggggcctgccctggcctgcggtacatgctcagcatctcctgcagcaccttcacatggcttcgcacttcctccaccgcactgaccctcttggacaccttctccgatttttcttgttcctccttgaccaaattcttgattaaccggtttgcagcctgaaggtcctcggggtggttgctctttagaagccttgtcagaagcttggacttttcttcatcagcatcaaagatggagctcttgggccagggagatggtgggggtaagattttatccactggtagtttagggtcttgttttataattccttgtttcttcagcatctgataagcgtctcgaatcttgatgtcttccggaaaccagactgtccaactgaagagtatttcaatgactcttcctttaacttttcctgtggcccaggaccccaggtactttggggacaacactttgatcagttcgttcaggaaacgaaatttggccacctcgctgtggaacttctccccacagtggttcatgcacatctccagcaccgttaaggcataaagagcttccttctcttgcggagactggatcttgtgggccagtagccagggcgcatgtgtggggccattggggtcagtgttcacctgctcacagaaattctggatagctgaccaatcctgttccgacatgcttgggtctgtggctttgttgagccacagctccagcgacgctgccgggcccgggggaccctgggccgactcggttcccgccacagccgccgccaccgcggtcgccgccatcgctccagccccgacgctgcggccgcgggcgccactgcctcttcagccgctgtagcgtcctggcgctctcctctgctgactgc

SEQ ID NO: 18194 - RNA, 3701 nt, Homo sapiens
  source 1..3701: mol_type = other RNA
tgaagtaccagctactcgagaggctgaggcacgagaatcgcttgaacctggtaggcagagattgcagtgagctgagattataccaccgcactccagcctgagtgacagagtgagatatggcctcaaaaaacaaaaaaaagccacacagaatacaagcaagaaagtacttttagattaaaattcgtcttatgtgaattatggcaaatgaaatcaccccactgtttacctgttttatgagtttttacatttgcttaaaattagcatacttgatcttttacagttcccatctccaccaattagtattggcagatttccactatatgtagaagtcaaaagatcagactgtaaaaatatcagatattgtaattaagagctccaaacaagtcttgcagtttcaaaggtagaaacccacccagccagttcagctgcttggacttcaaagccctccgcctagccatctcagccaggctcaggttccttctcccacccatcaggccaagcaggacttgtcaaacatacacattcaagttcctagcacacagtaggtgctaagtgggaattgattataaacttgaattcttccatcaacaaatatccacctctcctgtccagcttgcctcagatcttcaggttctctcttctctgaggcagctaagcttctacatccttcatgaagtttcctttacttctcgacagaagacagttccctttaggcctatcatctctaaatgcaactggctttccattttccacttactcaacactccacaaagtacacttgctacatggtatttattcaatgactgtatatttagtcaccacctcaatcactgctaagctctcttcatgtctatctgtaccacagtttcccatcttagactgtgacgtcagctggcaagggctggctgttggccgattcatcatgactgacatggtgtgtcacaaagagctccaagtaaatgctgtgaaggaagaggatgaggatggagatgaggatcctgagaagggcccagactggctgcccaacccatggacctgaggcctgagtaaggcctgggagctgctttcccctctgcccaggaactctgtccaggggcgattctaaggcacagtggtgaaggacatgattggtcccccaagtgtggtcctcaggtctcatggcagccactcgcctgggaacagtgcaacaagcattccatttagaagatcttccagaacacacacaagaagcattgtctaatgaaaatggagacaaggtctttcttggaagagagtgcccaagtagatactctctgccccaagactaaccaggtcccttttaaggtccctgagaacagcagcctgggagcaaccaagcctttcaaaggctgacaaggcacagagtggatgaatggaacgaacgatacatgaaaaaaacactttggctgataaaacctccaacctgaggcagggacagtgtcgctcgctgacatgcagaaacatgactgtagcagagatgatgatgatgagaaatgcttcgcatttcccacactgccgatatcccaagccctgtgctaccaccctctccccgaacacacacacacacacacacacacacacacacacacacacacacacagagcatctgcagaataagtcagaggttgacacccagagcctgacgtcaggataggactcttggcactccgcactgaaacaccgtgattagtcctgactagacagcaaaagtaacgccagcctaagcttgaaatgaagggtccatcttgtgaaaagttaggctgcgcccaagacagccaggtctgggaagtctttcacttctcctacttcgctgaaaggctgtccaccttggttgaatgtcagcttgtaccgtaagcggataggttctttgtgtggattgtcaagcagcagcatctgagatatcacagctggaggcatcaaaggactgaatgcaggaagcttggagctggatgccggctgcagcttcactctcattgactttggcacagccacttgaaacatgatatcccagacaggctggggagccgtgctcatcatggtcaagagcagcacctgtacctctgggtgcccaggggctcccgtctgggagaagtggagcagaattctgaatccattccggtcatacacaatgagaggcggcaggctgctgggcttaacagactccaaagggacaaacacttgagccagaggtgtattctgtgaagatggggaaggagccaacgggccagcctcccaggaccaacctggagaggacttagtacctggtggcacttccttggggacacttttctgcgaaacataattcagagggcacggagctggctgtgctgagaggaggtccagcaaattcctgtctgcagaagggttctgaacaccaccgcctggcagcgtgctggaggagggattcctcttttcctcacagcaattctgaccagaaaccatgcctgtaacaggagcatcactgattcccaaggctgccaggtcctgatgaagcaaagatggcaccacagtccccatctgcgcaggtccattgtccacctccaagtcaatcagggggcaggtcttcatgcagcctgctggattctgaaagactctggagacagggatgtctcccaatgagctggtcactctgtttccaaaggtgacccggccctccatcacctgtttgtacagcagaactccttgggtgaggaggtcatttgcctggagaatttccgcgagtgcatcatcgtcatcagtggtgtcactcgccaaccggaacagcgtgggccgcagcttttcacacctctcatacacgacctgcagggcctcctggtcgggcggggcctgccctggcctgcggtacatgctcagcatctcctgcagcaccttcacatggcttcgcacttcctccaccgcactgaccctcttggacaccttctccgatttttcttgttcctccttgaccaaattcttgattaaccggtttgcagcctgaaggtcctcggggtggttgctctttagaagccttgtcagaagcttggacttttcttcatcagcatcaaagatggagctcttgggccagggagatggtgggggtaagattttatccactggtagtttagggtcttgttttataattccttgtttcttcagcatctgataagcgtctcgaatcttgatgtcttccggaaaccagactgtccaactgaagagtatttcaatgactcttcctttaacttttcctgtggcccaggaccccaggtactttggggacaacactttgatcagttcgttcaggaaacgaaatttggccacctcgctgtggaacttctccccacagtggttcatgcacatctccagcaccgttaaggcataaagagcttccttctcttgcggagactggatcttgtgggccagtagccagggcgcatgtgtggggcttacccattggggtcagtgttcacctgctcacagaaattctggatagctgaccaatcctgttccgacatgcttgggtctgtggctttgttgagccacagctccagcgacgctgccgggcccgggggaccctgggccgactcggttcccgccacagccgccgccaccgcggtcgccgccatcgctccagccccgacgctgcggccgcgggcgccactgcctcttcagccgctgtagcgtcctggcgctctcctctgctgact

SEQ ID NO: 18195 - RNA, 48 nt, Homo sapiens
  source 1..48: mol_type = other RNA
tgaagtaccagctactcgagaggctgaggcagaagaagaatcacttga

SEQ ID NO: 18196 - RNA, 572 nt, Homo sapiens
  source 1..572: mol_type = other RNA
tgaagtaccagctactcgagaggctgaggcagaagaagaatcacttgaacacagaaggcagaggctgcagtgagccaaatttgcaccactgcactgcattccagcctggatgacagaggaagactgtctgtcttaatcacacaacttgactctaatcttaatcttgaacatccactgttgctgtactgcgcagcaaaacaattctatcttcttaatagttcttctatgtctttcccagcggacggacgtgcgggcggccggcgacggtggcgggtgctgcaggccggcctttctctggagcactgggccgggctccggctggtggggcgggcggagggagggaggaggggccgagctcggagctgacaaaaagcggcccagctccccggcacgggcccgccgtcagcacgtcacgtcaccgcccgggagagagacccaggaaaatgcggaagggtagacaggccccctcctccgcccggtgggtcctcctggcaccccgtgtcggcgccgctcccgccccgcgaccggggagcccagtggcctcgctgcggcggggtctccggcggccggag

SEQ ID NO: 18197 - RNA, 414 nt, Homo sapiens
  source 1..414: mol_type = other RNA
tgaagtaccagctactcgagaggctgaggcagaagaagaatcacttgaacacagaaggcagaggctgcagtgagccaaatttgcaccactgcactgcattccagcctggatgacagaggaagactgtctgtcttaatcacacaacttgactctaatcttaatcttgaacatccactgttgctgtactgcgcagcaaaacaattctatcttcttaatagttcttctatgtctttcccagcgtaaagcacagctcagggaacagacggcagtgacaggcgggcagtgggaggcgggagaacggcttgagcccaggagttcgagaccagcctggggcaatatagcaagaaccggacggacgtgcgggcggccggcgacggtggcgggtgctgcaggccggcctttctctggagcact

SEQ ID NO: 18198 - RNA, 479 nt, Homo sapiens
  source 1..479: mol_type = other RNA
tgaagtaccagctactcgagaggctgaggcagaagaagaatcacttgaacacagaaggcagaggctgcagtgagccaaatttgcaccactgcactgcattccagcctggatgacagaggaagactgtctgtcttaatcacacaacttgactctaatcttaatcttgaacatccactgttgctgtactgcgcagcaaaacaattctatcttcttaatagttcttctatgtctttcccagcgtaaagcacagctcagggaacagacggcagtgacaggcgggcagtgggaggcgggagaacggcttgagcccaggagttcgagaccagcctggggcaatatagcaagaacctgtctcaaaataaaaaataagtaaataacaaggtgcagctcaggtgtgccatcactcttctagttgagggcacccccgctgcctaccccattgagtataagcccctccacctggcaagcaagcccttctg

SEQ ID NO: 18199 - RNA, 424 nt, Homo sapiens
  source 1..424: mol_type = other RNA
tgaagtaccagctactcgagaggctgaggcagaatcgcttgaacccgagaggtgaggttgcagtgagccaaggtcatgccactgcactccagtctgagcaagagagcaagattccatcttatctcactaaatgcagaaactactgggagtgaggctgccataaatctcttctggagaattttactggccataaagaagacagagaagaccgcttgcacctcgcccgcggctccggaagcggctgcggccccgaccggaaagcccccagcatcgcccgaaggaatcgcggctggcctgcggctccggcccggcctcgggtaccacgcgcctagtgggaagccgcactgacgcctgcagcatctcgcgagatttcgggctcagcccaagtactgcgagttcaccaaagcggggggaaaaaaaaaaa

SEQ ID NO: 18200 - RNA, 659 nt, Homo sapiens
  source 1..659: mol_type = other RNA
tgaagtaccagctactcgagaggctgaggcagaatcgcttgaacccgagaggtgaggttgcagtgagccaaggtcatgccactgcactccagtctgagcaagagagcaagattccatcttatctcactaaatgcagaaactactgggagtgaggctgccataaatctcttctggagaattttactggccataaagaagacagagaagaccgcttgcaccttggaacatcagcttttaaaataaaggtgtcatcagaagtgtgtagacacccactgcatcacaactggaactgatctctggttatgccaatctaggtctgcctggcagggtgagtctaccgctcgaaagctgcacagaggaaatcctccctcctccaggttcaggcccggagttacgagcggagattcgcggcggcgggtcagagcccagagcaaaccaggctggggaacgcacctcgcccgcggctccggaagcggctgcggccccgaccggaaagcccccagcatcgcccgaaggaatcgcggctggcctgcggctccggcccggcctcgggtaccacgcgcctagtgggaagccgcactgacgcctgcagcatctcgcgagatttcgggctcagcccaagtactgcgagttcaccaaagcggggggaaaaaaaaaaa

SEQ ID NO: 18201 - RNA, 4226 nt, Homo sapiens
  source 1..4226: mol_type = other RNA
tgaagtaccagctactcgagaggctgaggcagataattgcttgaacccaggaagcagaggttgcagtgagctgcagaggttgcagtgatcacaccactgcagtccagcctgggcaacagagcaagactccgtcttaagaaaaaaaaacaacaaaaaaaaacaaacaaacaaaaaacctgtggaagacttagtgatgttccaaataaggcctcagactttccttatccacttaaaacacatctttaccttttaatcaaagccaacttgagtgttaagtttttaaagtttgctaactgtaactgagaaataacagatcagcctgaacttgccgagtgtgaagtcataattagcacccgttctctggtccacagagccatcacttcttttccatccccctcactaggtaagacagagttccctctcaggcttctcaaagagaactgtgggagtcatgtctggatactcatttgcttttcagaaaaacataaagacatggaggtgaaattgtatgaaaacattctacctagaaacatcttaacctctatgtttcaattaccaaagatatttaaaagaaaatatctttactctttaaaaatactagtgtccttattttccttctaattcttcacctgagtagtctctctgaagagcatgacttacaaaatgctctctcatgcatccctggatctttcatgttattgtaaatttaatacttttcattatagattttaaacaactactacttggggttgtgtgtataaatatgtaaaataagcaatacacacaggtacatgatatatatgtgtatatatataattcagggtacatttacatacataaagttgcaaaagatcctataagccatgagttacctctaggagattccaaaatgcagtcctcagtaagtgtcatttgtagcacacaaccattccaagatgaagccgcacagacagaataatcaaaatacaacatgagcaagcacagtttttcaataaggttttctaaaagtttgctacgctgacaaaagatgtaaataatccaaagaaagccaaaagaagtatatttgaaaagtaaacacgaacccagccactgctctttactcagcaaagccagggacgcaacagctcaaatggaaactttcactgtcaagtggtctgaaaatattaagcaagacaagtaaatgacttccatgttatgataattagacctgactgtaaaatctcccatttatattagtagatgtctctgacaattttattgtgagaaatgtatggggaaaaaaatgagtcaacatgaatactttcagagttaccaatataaagttaccttaagttaatggtcttagaagagtaccatcaaggtaagcaaggtaaatatttaaataaatataaaattctaagatataaaacttcggtatagaatcagggattactttattaaaagtaactagcatgttgccagttttccctatttattaaacaaactgaatagaattcagaacacactactgagcaaaatgtatatttaaaaaaaagtcaactagaagtaataattctatttgtacacagcataaatcaatatacagtattgtatgtgaatgagactgattggctttaaaatgaattttctgcttcaaggccaatatctctacaaacgttctgtagaagtattgttagggcaggccaacttctttatgatgtcgcattatgtgctggttcttttctgaaggtcttcggaagcctttcttgcagtactcacaccggtgaggatagtctttcgtgtgaatggaaataacgtgccgtttaaagcctgaggcatctgtagtgctatactcacagtactcacactgatacactttcctgccactgtgtgtcttcatatgctttttaagctcactctgttgcctaaatccctttctacatctcttgcacctaaatggaagatcctttgtgtgaactgagagaatatggcgacttagaacaaatggatctgcaatcttaaagtcacaatgtctacactggtgcatttttttgcccttgtgggcagccacgtgtttcttgagttctgaaggcctgtgaaagcctttatcacacatgtcacacttatgggggtagtctttcgtgtgaactgaaattatgtgtcgtttcaaatcacttgagttcgaactcttgtggtcgcaatgcaaacactggtgtgttttgctttcttggtggataagagcatgttgctgcacctctttggtatccgagaaagtcagaagacaaatgtcacacttgaatggcatctctttactatgcttagttttgacatgcgttttcaagttagaagagtctgcagacctatattcgcagtactggcattggtacggcttctccccagtatggattctcatgtgctttttgagctctgacgggtgacgaaaacccttaccacactccacacaaatatgaggaaagttcttgctgtggactgccaagaggtggcgattcaataacccttgttcagctgtctcgtattcacagaatttacacttgtgcattttgttggctcctttttccttatgcaccattttgtgagtaaacaaagcccctgcatgagagaaatgcttcccacactcatcgcattcaatggccttctctgccttgctggtcagcttgtggctctccaggtggttgtgtaaacttatcttcttgttggtagtgtaatcacagtcagtacagcggtatttcttcttggcaaggtgttcgggatggtttttcatgtgccttttcaaaaaacctctcgacttaaacttcttcccacaaatcatgcaaggatagacagtcaaaggatgtccatcagggccaataattattgcataagctgctgcccatgcaatcggcatgaaggttttgatttcattgtcatccatttgctgctcgtgcacggcggcggctgccgctgctgctgcagcatcctcctctcctacgatcacttccatataaacttcgtcagcgatttcagcaacatttaaatcttcatcttctggctgagagtcattgacagtcatataaaccatcttttccctgggaacacgaatactgctgttctgatcaagcagttcaactccatgatcattctcaggctcactctccacaatgtctacagttccacctaagtcatcttctccagggtcagctttaaaaatgtacaccttgatgacctcagggcaagtgccatccactttacaaggatcaatttccgactctgtgtccatggtcattccagaagaaccatcgtgttctattttgccagcatcatccaaggaaatcataaggtagtcctcacagttgcctttgtcatcatcctgctggtccacagggatcccattggcatctatgactgcttcagaggcacagtctgctaccaatacttcttctgaaactacgtcggtagtcagaggatcagtgacaatttctgcttccactacactatcatgaaccacatgttcaacatgtccaacatgtccaacatgtccaacgtcagacacatgtatagaatcacccgtcaagacgtgttctggcatagacattgaggctgaagtaatgtcagaagctaaaacatcatctgggactgtgcaatgtgctaaagaaacttcttcagttacatctgagtccagcacttgctcaggaatgatgaccgtttcagacacatctgcttcttccatgatatctgggcactgaacatcttctataacaacgtcctcaataacatcttggattacaactgaatctgggtcatcaggaacaaagttatgcacagttatgtctgaatccacaacatctgaaacaaaaacagtttcttgtacttccacaacaatttgatcaccatccatgtgtgtaccatcagctccggacggacgtgcgggcggccggcgacggtggcgggtgctgcaggccggcctttctctggagcactgggccgggctccggctggtggggcgggcggagggagggaggaggggccgagctcggagctgacaaaaagcggcccagctccccggcacgggcccgccgtcagcacgtcacgtcaccgcccgggagagagacccaggaaaatgcggaagggtagacaggccccctcctccgcccggtgggtcctcctggcaccccgtgtcggcgccgctcccgccccgcgaccggggagcccagtggcctcgctgcggcggggtctccggcggccggagt

SEQ ID NO: 18202 - RNA, 4143 nt, Homo sapiens
  source 1..4143: mol_type = other RNA
tgaagtaccagctactcgagaggctgaggcagataattgcttgaacccaggaagcagaggttgcagtgagctgcagaggttgcagtgatcacaccactgcagtccagcctgggcaacagagcaagactccgtcttaagaaaaaaaaacaacaaaaaaaaacaaacaaacaaaaaacctgtggaagacttagtgatgttccaaataaggcctcagactttccttatccacttaaaacacatctttaccttttaatcaaagccaacttgagtgttaagtttttaaagtttgctaactgtaactgagaaataacagatcagcctgaacttgccgagtgtgaagtcataattagcacccgttctctggtccacagagccatcacttcttttccatccccctcactaggtaagacagagttccctctcaggcttctcaaagagaactgtgggagtcatgtctggatactcatttgcttttcagaaaaacataaagacatggaggtgaaattgtatgaaaacattctacctagaaacatcttaacctctatgtttcaattaccaaagatatttaaaagaaaatatctttactctttaaaaatactagtgtccttattttccttctaattcttcacctgagtagtctctctgaagagcatgacttacaaaatgctctctcatgcatccctggatctttcatgttattgtaaatttaatacttttcattatagattttaaacaactactacttggggttgtgtgtataaatatgtaaaataagcaatacacacaggtacatgatatatatgtgtatatatataattcagggtacatttacatacataaagttgcaaaagatcctataagccatgagttacctctaggagattccaaaatgcagtcctcagtaagtgtcatttgtagcacacaaccattccaagatgaagccgcacagacagaataatcaaaatacaacatgagcaagcacagtttttcaataaggttttctaaaagtttgctacgctgacaaaagatgtaaataatccaaagaaagccaaaagaagtatatttgaaaagtaaacacgaacccagccactgctctttactcagcaaagccagggacgcaacagctcaaatggaaactttcactgtcaagtggtctgaaaatattaagcaagacaagtaaatgacttccatgttatgataattagacctgactgtaaaatctcccatttatattagtagatgtctctgacaattttattgtgagaaatgtatggggaaaaaaatgagtcaacatgaatactttcagagttaccaatataaagttaccttaagttaatggtcttagaagagtaccatcaaggtaagcaaggtaaatatttaaataaatataaaattctaagatataaaacttcggtatagaatcagggattactttattaaaagtaactagcatgttgccagttttccctatttattaaacaaactgaatagaattcagaacacactactgagcaaaatgtatatttaaaaaaaagtcaactagaagtaataattctatttgtacacagcataaatcaatatacagtattgtatgtgaatgagactgattggctttaaaatgaattttctgcttcaaggccaatatctctacaaacgttctgtagaagtattgttagggcaggccaacttctttatgatgtcgcattatgtgctggttcttttctgaaggtcttcggaagcctttcttgcagtactcacaccggtgaggatagtctttcgtgtgaatggaaataacgtgccgtttaaagcctgaggcatctgtagtgctatactcacagtactcacactgatacactttcctgccactgtgtgtcttcatatgctttttaagctcactctgttgcctaaatccctttctacatctcttgcacctaaatggaagatcctttgtgtgaactgagagaatatggcgacttagaacaaatggatctgcaatcttaaagtcacaatgtctacactggtgcatttttttgcccttgtgggcagccacgtgtttcttgagttctgaaggcctgtgaaagcctttatcacacatgtcacacttatgggggtagtctttcgtgtgaactgaaattatgtgtcgtttcaaatcacttgagttcgaactcttgtggtcgcaatgcaaacactggtgtgttttgctttcttggtggataagagcatgttgctgcacctctttggtatccgagaaagtcagaagacaaatgtcacacttgaatggcatctctttactatgcttagttttgacatgcgttttcaagttagaagagtctgcagacctatattcgcagtactggcattggtacggcttctccccagtatggattctcatgtgctttttgagctctgacgggtgacgaaaacccttaccacactccacacaaatatgaggaaagttcttgctgtggactgccaagaggtggcgattcaataacccttgttcagctgtctcgtattcacagaatttacacttgtgcattttgttggctcctttttccttatgcaccattttgtgagtaaacaaagcccctgcatgagagaaatgcttcccacactcatcgcattcaatggccttctctgccttgctggtcagcttgtggctctccaggtggttgtgtaaacttatcttcttgttggtagtgtaatcacagtcagtacagcggtatttcttcttggcaaggtgttcgggatggtttttcatgtgccttttcaaaaaacctctcgacttaaacttcttcccacaaatcatgcaaggatagacagtcaaaggatgtccatcagggccaataattattgcataagctgctgcccatgcaatcggcatgaaggttttgatttcattgtcatccatttgctgctcgtgcacggcggcggctgccgctgctgctgcagcatcctcctctcctacgatcacttccatataaacttcgtcagcgatttcagcaacatttaaatcttcatcttctggctgagagtcattgacagtcatataaaccatcttttccctgggaacacgaatactgctgttctgatcaagcagttcaactccatgatcattctcaggctcactctccacaatgtctacagttccacctaagtcatcttctccagggtcagctttaaaaatgtacaccttgatgacctcagggcaagtgccatccactttacaaggatcaatttccgactctgtgtccatggtcattccagaagaaccatcgtgttctattttgccagcatcatccaaggaaatcataaggtagtcctcacagttgcctttgtcatcatcctgctggtccacagggatcccattggcatctatgactgcttcagaggcacagtctgctaccaatacttcttctgaaactacgtcggtagtcagaggatcagtgacaatttctgcttccactacactatcatgaaccacatgttcaacatgtccaacatgtccaacatgtccaacgtcagacacatgtatagaatcacccgtcaagacgtgttctggcatagacattgaggctgaagtaatgtcagaagctaaaacatcatctgggactgtgcaatgtgctaaagaaacttcttcagttacatctgagtccagcacttgctcaggaatgatgaccgtttcagacacatctgcttcttccatgatatctgggcactgaacatcttctataacaacgtcctcaataacatcttggattacaactgaatctgggtcatcaggaacaaagttatgcacagttatgtctgaatccacaacatctgaaacaaaaacagtttcttgtacttccacaacaatttgatcaccatccatgtgtgtaccatcagctcctgtagccccagttactcgggaagctgagcagatcacttgagcctgggaggcggaggttgcagtggacccagatggcgccactgtgctccagcctgggtgacagaacgagaccctgtctgttgcatcaaaaaatgagtttggctcttgttgtaattcaagcccatcttcatccatggcctttaattctcatcagtcacagctcctgtaatcccagctactcgagaggctgaggcagaagaagaatcacttga

SEQ ID NO: 18203 - RNA, 4315 nt, Homo sapiens
  source 1..4315: mol_type = other RNA
tgaagtaccagctactcgagaggctgaggcagataattgcttgaacccaggaagcagaggttgcagtgagctgcagaggttgcagtgatcacaccactgcagtccagcctgggcaacagagcaagactccgtcttaagaaaaaaaaacaacaaaaaaaaacaaacaaacaaaaaacctgtggaagacttagtgatgttccaaataaggcctcagactttccttatccacttaaaacacatctttaccttttaatcaaagccaacttgagtgttaagtttttaaagtttgctaactgtaactgagaaataacagatcagcctgaacttgccgagtgtgaagtcataattagcacccgttctctggtccacagagccatcacttcttttccatccccctcactaggtaagacagagttccctctcaggcttctcaaagagaactgtgggagtcatgtctggatactcatttgcttttcagaaaaacataaagacatggaggtgaaattgtatgaaaacattctacctagaaacatcttaacctctatgtttcaattaccaaagatatttaaaagaaaatatctttactctttaaaaatactagtgtccttattttccttctaattcttcacctgagtagtctctctgaagagcatgacttacaaaatgctctctcatgcatccctggatctttcatgttattgtaaatttaatacttttcattatagattttaaacaactactacttggggttgtgtgtataaatatgtaaaataagcaatacacacaggtacatgatatatatgtgtatatatataattcagggtacatttacatacataaagttgcaaaagatcctataagccatgagttacctctaggagattccaaaatgcagtcctcagtaagtgtcatttgtagcacacaaccattccaagatgaagccgcacagacagaataatcaaaatacaacatgagcaagcacagtttttcaataaggttttctaaaagtttgctacgctgacaaaagatgtaaataatccaaagaaagccaaaagaagtatatttgaaaagtaaacacgaacccagccactgctctttactcagcaaagccagggacgcaacagctcaaatggaaactttcactgtcaagtggtctgaaaatattaagcaagacaagtaaatgacttccatgttatgataattagacctgactgtaaaatctcccatttatattagtagatgtctctgacaattttattgtgagaaatgtatggggaaaaaaatgagtcaacatgaatactttcagagttaccaatataaagttaccttaagttaatggtcttagaagagtaccatcaaggtaagcaaggtaaatatttaaataaatataaaattctaagatataaaacttcggtatagaatcagggattactttattaaaagtaactagcatgttgccagttttccctatttattaaacaaactgaatagaattcagaacacactactgagcaaaatgtatatttaaaaaaaagtcaactagaagtaataattctatttgtacacagcataaatcaatatacagtattgtatgtgaatgagactgattggctttaaaatgaattttctgcttcaaggccaatatctctacaaacgttctgtagaagtattgttagggcaggccaacttctttatgatgtcgcattatgtgctggttcttttctgaaggtcttcggaagcctttcttgcagtactcacaccggtgaggatagtctttcgtgtgaatggaaataacgtgccgtttaaagcctgaggcatctgtagtgctatactcacagtactcacactgatacactttcctgccactgtgtgtcttcatatgctttttaagctcactctgttgcctaaatccctttctacatctcttgcacctaaatggaagatcctttgtgtgaactgagagaatatggcgacttagaacaaatggatctgcaatcttaaagtcacaatgtctacactggtgcatttttttgcccttgtgggcagccacgtgtttcttgagttctgaaggcctgtgaaagcctttatcacacatgtcacacttatgggggtagtctttcgtgtgaactgaaattatgtgtcgtttcaaatcacttgagttcgaactcttgtggtcgcaatgcaaacactggtgtgttttgctttcttggtggataagagcatgttgctgcacctctttggtatccgagaaagtcagaagacaaatgtcacacttgaatggcatctctttactatgcttagttttgacatgcgttttcaagttagaagagtctgcagacctatattcgcagtactggcattggtacggcttctccccagtatggattctcatgtgctttttgagctctgacgggtgacgaaaacccttaccacactccacacaaatatgaggaaagttcttgctgtggactgccaagaggtggcgattcaataacccttgttcagctgtctcgtattcacagaatttacacttgtgcattttgttggctcctttttccttatgcaccattttgtgagtaaacaaagcccctgcatgagagaaatgcttcccacactcatcgcattcaatggccttctctgccttgctggtcagcttgtggctctccaggtggttgtgtaaacttatcttcttgttggtagtgtaatcacagtcagtacagcggtatttcttcttggcaaggtgttcgggatggtttttcatgtgccttttcaaaaaacctctcgacttaaacttcttcccacaaatcatgcaaggatagacagtcaaaggatgtccatcagggccaataattattgcataagctgctgcccatgcaatcggcatgaaggttttgatttcattgtcatccatttgctgctcgtgcacggcggcggctgccgctgctgctgcagcatcctcctctcctacgatcacttccatataaacttcgtcagcgatttcagcaacatttaaatcttcatcttctggctgagagtcattgacagtcatataaaccatcttttccctgggaacacgaatactgctgttctgatcaagcagttcaactccatgatcattctcaggctcactctccacaatgtctacagttccacctaagtcatcttctccagggtcagctttaaaaatgtacaccttgatgacctcagggcaagtgccatccactttacaaggatcaatttccgactctgtgtccatggtcattccagaagaaccatcgtgttctattttgccagcatcatccaaggaaatcataaggtagtcctcacagttgcctttgtcatcatcctgctggtccacagggatcccattggcatctatgactgcttcagaggcacagtctgctaccaatacttcttctgaaactacgtcggtagtcagaggatcagtgacaatttctgcttccactacactatcatgaaccacatgttcaacatgtccaacatgtccaacatgtccaacgtcagacacatgtatagaatcacccgtcaagacgtgttctggcatagacattgaggctgaagtaatgtcagaagctaaaacatcatctgggactgtgcaatgtgctaaagaaacttcttcagttacatctgagtccagcacttgctcaggaatgatgaccgtttcagacacatctgcttcttccatgatatctgggcactgaacatcttctataacaacgtcctcaataacatcttggattacaactgaatctgggtcatcaggaacaaagttatgcacagttatgtctgaatccacaacatctgaaacaaaaacagtttcttgtacttccacaacaatttgatcaccatccatgtgtgtaccatcagctcctgtagccccagttactcgggaagctgagcagatcacttgagcctgggaggcggaggttgcagtggacccagatggcgccactgtgctccagcctgggtgacagaacgagaccctgtctgttgcatcaaaaaatgagtttggctcttgttgtaattcaagcccatcttcatccatggcctttaattctcatcagtcacagctcctgtcttaatcacacaacttgactctaatcttaatcttgaacatccactgttgctgtactgcgcagcaaaacaattctatcttcttaatagttcttctatgtctttcccagcgtaaagcacagctcagggaacagacggcagtgacaggcgggcagtgggaggcgggagaacggcttgagcccaggagttcgagaccagcctggggcaatatagcaagaac

SEQ ID NO: 18204 - RNA, 4237 nt, Homo sapiens
  source 1..4237: mol_type = other RNA
tgaagtaccagctactcgagaggctgaggcagataattgcttgaacccaggaagcagaggttgcagtgagctgcagaggttgcagtgatcacaccactgcagtccagcctgggcaacagagcaagactccgtcttaagaaaaaaaaacaacaaaaaaaaacaaacaaacaaaaaacctgtggaagacttagtgatgttccaaataaggcctcagactttccttatccacttaaaacacatctttaccttttaatcaaagccaacttgagtgttaagtttttaaagtttgctaactgtaactgagaaataacagatcagcctgaacttgccgagtgtgaagtcataattagcacccgttctctggtccacagagccatcacttcttttccatccccctcactaggtaagacagagttccctctcaggcttctcaaagagaactgtgggagtcatgtctggatactcatttgcttttcagaaaaacataaagacatggaggtgaaattgtatgaaaacattctacctagaaacatcttaacctctatgtttcaattaccaaagatatttaaaagaaaatatctttactctttaaaaatactagtgtccttattttccttctaattcttcacctgagtagtctctctgaagagcatgacttacaaaatgctctctcatgcatccctggatctttcatgttattgtaaatttaatacttttcattatagattttaaacaactactacttggggttgtgtgtataaatatgtaaaataagcaatacacacaggtacatgatatatatgtgtatatatataattcagggtacatttacatacataaagttgcaaaagatcctataagccatgagttacctctaggagattccaaaatgcagtcctcagtaagtgtcatttgtagcacacaaccattccaagatgaagccgcacagacagaataatcaaaatacaacatgagcaagcacagtttttcaataaggttttctaaaagtttgctacgctgacaaaagatgtaaataatccaaagaaagccaaaagaagtatatttgaaaagtaaacacgaacccagccactgctctttactcagcaaagccagggacgcaacagctcaaatggaaactttcactgtcaagtggtctgaaaatattaagcaagacaagtaaatgacttccatgttatgataattagacctgactgtaaaatctcccatttatattagtagatgtctctgacaattttattgtgagaaatgtatggggaaaaaaatgagtcaacatgaatactttcagagttaccaatataaagttaccttaagttaatggtcttagaagagtaccatcaaggtaagcaaggtaaatatttaaataaatataaaattctaagatataaaacttcggtatagaatcagggattactttattaaaagtaactagcatgttgccagttttccctatttattaaacaaactgaatagaattcagaacacactactgagcaaaatgtatatttaaaaaaaagtcaactagaagtaataattctatttgtacacagcataaatcaatatacagtattgtatgtgaatgagactgattggctttaaaatgaattttctgcttcaaggccaatatctctacaaacgttctgtagaagtattgttagggcaggccaacttctttatgatgtcgcattatgtgctggttcttttctgaaggtcttcggaagcctttcttgcagtactcacaccggtgaggatagtctttcgtgtgaatggaaataacgtgccgtttaaagcctgaggcatctgtagtgctatactcacagtactcacactgatacactttcctgccactgtgtgtcttcatatgctttttaagctcactctgttgcctaaatccctttctacatctcttgcacctaaatggaagatcctttgtgtgaactgagagaatatggcgacttagaacaaatggatctgcaatcttaaagtcacaatgtctacactggtgcatttttttgcccttgtgggcagccacgtgtttcttgagttctgaaggcctgtgaaagcctttatcacacatgtcacacttatgggggtagtctttcgtgtgaactgaaattatgtgtcgtttcaaatcacttgagttcgaactcttgtggtcgcaatgcaaacactggtgtgttttgctttcttggtggataagagcatgttgctgcacctctttggtatccgagaaagtcagaagacaaatgtcacacttgaatggcatctctttactatgcttagttttgacatgcgttttcaagttagaagagtctgcagacctatattcgcagtactggcattggtacggcttctccccagtatggattctcatgtgctttttgagctctgacgggtgacgaaaacccttaccacactccacacaaatatgaggaaagttcttgctgtggactgccaagaggtggcgattcaataacccttgttcagctgtctcgtattcacagaatttacacttgtgcattttgttggctcctttttccttatgcaccattttgtgagtaaacaaagcccctgcatgagagaaatgcttcccacactcatcgcattcaatggccttctctgccttgctggtcagcttgtggctctccaggtggttgtgtaaacttatcttcttgttggtagtgtaatcacagtcagtacagcggtatttcttcttggcaaggtgttcgggatggtttttcatgtgccttttcaaaaaacctctcgacttaaacttcttcccacaaatcatgcaaggatagacagtcaaaggatgtccatcagggccaataattattgcataagctgctgcccatgcaatcggcatgaaggttttgatttcattgtcatccatttgctgctcgtgcacggcggcggctgccgctgctgctgcagcatcctcctctcctacgatcacttccatataaacttcgtcagcgatttcagcaacatttaaatcttcatcttctggctgagagtcattgacagtcatataaaccatcttttccctgggaacacgaatactgctgttctgatcaagcagttcaactccatgatcattctcaggctcactctccacaatgtctacagttccacctaagtcatcttctccagggtcagctttaaaaatgtacaccttgatgacctcagggcaagtgccatccactttacaaggatcaatttccgactctgtgtccatggtcattccagaagaaccatcgtgttctattttgccagcatcatccaaggaaatcataaggtagtcctcacagttgcctttgtcatcatcctgctggtccacagggatcccattggcatctatgactgcttcagaggcacagtctgctaccaatacttcttctgaaactacgtcggtagtcagaggatcagtgacaatttctgcttccactacactatcatgaaccacatgttcaacatgtccaacatgtccaacatgtccaacgtcagacacatgtatagaatcacccgtcaagacgtgttctggcatagacattgaggctgaagtaatgtcagaagctaaaacatcatctgggactgtgcaatgtgctaaagaaacttcttcagttacatctgagtccagcacttgctcaggaatgatgaccgtttcagacacatctgcttcttccatgatatctgggcactgaacatcttctataacaacgtcctcaataacatcttggattacaactgaatctgggtcatcaggaacaaagttatgcacagttatgtctgaatccacaacatctgaaacaaaaacagtttcttgtacttccacaacaatttgatcaccatccatgtgtgtaccatcagctcctgttgcatcaaaaaatgagtttggctcttgttgtaattcaagcccatcttcatccatggcctttaattctcatcagtcacagctccgcctctcgcgccggtcctggccgaggctccagctcgagttgtttgcaggccctcagacccccgcccgcagtaaatgtgttttcttcatccccgtggctggggaggaagataaatttagcaacccccgccgtcccctgccttcgcttaaaaaaaaaaaatctttgaaataaaatgaaaacgggcttgccagtctaaatgggtgtgcgggaaggggggtggagtggggggagaagggttatccctagagcacctaccaggc

SEQ ID NO: 18205 - RNA, 4366 nt, Homo sapiens
  source 1..4366: mol_type = other RNA
tgaagtaccagctactcgagaggctgaggcagataattgcttgaacccaggaagcagaggttgcagtgagctgcagaggttgcagtgatcacaccactgcagtccagcctgggcaacagagcaagactccgtcttaagaaaaaaaaacaacaaaaaaaaacaaacaaacaaaaaacctgtggaagacttagtgatgttccaaataaggcctcagactttccttatccacttaaaacacatctttaccttttaatcaaagccaacttgagtgttaagtttttaaagtttgctaactgtaactgagaaataacagatcagcctgaacttgccgagtgtgaagtcataattagcacccgttctctggtccacagagccatcacttcttttccatccccctcactaggtaagacagagttccctctcaggcttctcaaagagaactgtgggagtcatgtctggatactcatttgcttttcagaaaaacataaagacatggaggtgaaattgtatgaaaacattctacctagaaacatcttaacctctatgtttcaattaccaaagatatttaaaagaaaatatctttactctttaaaaatactagtgtccttattttccttctaattcttcacctgagtagtctctctgaagagcatgacttacaaaatgctctctcatgcatccctggatctttcatgttattgtaaatttaatacttttcattatagattttaaacaactactacttggggttgtgtgtataaatatgtaaaataagcaatacacacaggtacatgatatatatgtgtatatatataattcagggtacatttacatacataaagttgcaaaagatcctataagccatgagttacctctaggagattccaaaatgcagtcctcagtaagtgtcatttgtagcacacaaccattccaagatgaagccgcacagacagaataatcaaaatacaacatgagcaagcacagtttttcaataaggttttctaaaagtttgctacgctgacaaaagatgtaaataatccaaagaaagccaaaagaagtatatttgaaaagtaaacacgaacccagccactgctctttactcagcaaagccagggacgcaacagctcaaatggaaactttcactgtcaagtggtctgaaaatattaagcaagacaagtaaatgacttccatgttatgataattagacctgactgtaaaatctcccatttatattagtagatgtctctgacaattttattgtgagaaatgtatggggaaaaaaatgagtcaacatgaatactttcagagttaccaatataaagttaccttaagttaatggtcttagaagagtaccatcaaggtaagcaaggtaaatatttaaataaatataaaattctaagatataaaacttcggtatagaatcagggattactttattaaaagtaactagcatgttgccagttttccctatttattaaacaaactgaatagaattcagaacacactactgagcaaaatgtatatttaaaaaaaagtcaactagaagtaataattctatttgtacacagcataaatcaatatacagtattgtatgtgaatgagactgattggctttaaaatgaattttctgcttcaaggccaatatctctacaaacgttctgtagaagtattgttagggcaggccaacttctttatgatgtcgcattatgtgctggttcttttctgaaggtcttcggaagcctttcttgcagtactcacaccggtgaggatagtctttcgtgtgaatggaaataacgtgccgtttaaagcctgaggcatctgtagtgctatactcacagtactcacactgatacactttcctgccactgtgtgtcttcatatgctttttaagctcactctgttgcctaaatccctttctacatctcttgcacctaaatggaagatcctttgtgtgaactgagagaatatggcgacttagaacaaatggatctgcaatcttaaagtcacaatgtctacactggtgcatttttttgcccttgtgggcagccacgtgtttcttgagttctgaaggcctgtgaaagcctttatcacacatgtcacacttatgggggtagtctttcgtgtgaactgaaattatgtgtcgtttcaaatcacttgagttcgaactcttgtggtcgcaatgcaaacactggtgtgttttgctttcttggtggataagagcatgttgctgcacctctttggtatccgagaaagtcagaagacaaatgtcacacttgaatggcatctctttactatgcttagttttgacatgcgttttcaagttagaagagtctgcagacctatattcgcagtactggcattggtacggcttctccccagtatggattctcatgtgctttttgagctctgacgggtgacgaaaacccttaccacactccacacaaatatgaggaaagttcttgctgtggactgccaagaggtggcgattcaataacccttgttcagctgtctcgtattcacagaatttacacttgtgcattttgttggctcctttttccttatgcaccattttgtgagtaaacaaagcccctgcatgagagaaatgcttcccacactcatcgcattcaatggccttctctgccttgctggtcagcttgtggctctccaggtggttgtgtaaacttatcttcttgttggtagtgtaatcacagtcagtacagcggtatttcttcttggcaaggtgttcgggatggtttttcatgtgccttttcaaaaaacctctcgacttaaacttcttcccacaaatcatgcaaggatagacagtcaaaggatgtccatcagggccaataattattgctgtttggtactgcctggaatcaggtcttctccttttctttggtttttgtttagccagtctgccgaggccagcagactcatctatgtgcaagagggcacttgcagtgccattccggttttcaattccatcagaattattaccataagctgctgcccatgcaatcggcatgaaggttttgatttcattgtcatccatttgctgctcgtgcacggcggcggctgccgctgctgctgcagcatcctcctctcctacgatcacttccatataaacttcgtcagcgatttcagcaacatttaaatcttcatcttctggctgagagtcattgacagtcatataaaccatcttttccctgggaacacgaatactgctgttctgatcaagcagttcaactccatgatcattctcaggctcactctccacaatgtctacagttccacctaagtcatcttctccagggtcagctttaaaaatgtacaccttgatgacctcagggcaagtgccatccactttacaaggatcaatttccgactctgtgtccatggtcattccagaagaaccatcgtgttctattttgccagcatcatccaaggaaatcataaggtagtcctcacagttgcctttgtcatcatcctgctggtccacagggatcccattggcatctatgactgcttcagaggcacagtctgctaccaatacttcttctgaaactacgtcggtagtcagaggatcagtgacaatttctgcttccactacactatcatgaaccacatgttcaacatgtccaacatgtccaacatgtccaacgtcagacacatgtatagaatcacccgtcaagacgtgttctggcatagacattgaggctgaagtaatgtcagaagctaaaacatcatctgggactgtgcaatgtgctaaagaaacttcttcagttacatctgagtccagcacttgctcaggaatgatgaccgtttcagacacatctgcttcttccatgatatctgggcactgaacatcttctataacaacgtcctcaataacatcttggattacaactgaatctgggtcatcaggaacaaagttatgcacagttatgtctgaatccacaacatctgaaacaaaaacagtttcttgtacttccacaacaatttgatcaccatccatgtgtgtaccatcagctccggacggacgtgcgggcggccggcgacggtggcgggtgctgcaggccggcctttctctggagcactgggccgggctccggctggtggggcgggcggagggagggaggaggggccgagctcggagctgacaaaaagcggcccagctccccggcacgggcccgccgtcagcacgtcacgtcaccgcccgggagagagacccaggaaaatgcggaagggtagacaggccccctcctccgcccggtgggtcctcctggcaccccgtgtcggcgccgctcccgccccgcgaccggggagcccagtggcctcgctgcggcggggtctccggcggccggag

SEQ ID NO: 18206 - RNA, 4746 nt, Homo sapiens
  source 1..4746: mol_type = other RNA
tgaagtaccagctactcgagaggctgaggcagataattgcttgaacccaggaagcagaggttgcagtgagctgcagaggttgcagtgatcacaccactgcagtccagcctgggcaacagagcaagactccgtcttaagaaaaaaaaacaacaaaaaaaaacaaacaaacaaaaaacctgtggaagacttagtgatgttccaaataaggcctcagactttccttatccacttaaaacacatctttaccttttaatcaaagccaacttgagtgttaagtttttaaagtttgctaactgtaactgagaaataacagatcagcctgaacttgccgagtgtgaagtcataattagcacccgttctctggtccacagagccatcacttcttttccatccccctcactaggtaagacagagttccctctcaggcttctcaaagagaactgtgggagtcatgtctggatactcatttgcttttcagaaaaacataaagacatggaggtgaaattgtatgaaaacattctacctagaaacatcttaacctctatgtttcaattaccaaagatatttaaaagaaaatatctttactctttaaaaatactagtgtccttattttccttctaattcttcacctgagtagtctctctgaagagcatgacttacaaaatgctctctcatgcatccctggatctttcatgttattgtaaatttaatacttttcattatagattttaaacaactactacttggggttgtgtgtataaatatgtaaaataagcaatacacacaggtacatgatatatatgtgtatatatataattcagggtacatttacatacataaagttgcaaaagatcctataagccatgagttacctctaggagattccaaaatgcagtcctcagtaagtgtcatttgtagcacacaaccattccaagatgaagccgcacagacagaataatcaaaatacaacatgagcaagcacagtttttcaataaggttttctaaaagtttgctacgctgacaaaagatgtaaataatccaaagaaagccaaaagaagtatatttgaaaagtaaacacgaacccagccactgctctttactcagcaaagccagggacgcaacagctcaaatggaaactttcactgtcaagtggtctgaaaatattaagcaagacaagtaaatgacttccatgttatgataattagacctgactgtaaaatctcccatttatattagtagatgtctctgacaattttattgtgagaaatgtatggggaaaaaaatgagtcaacatgaatactttcagagttaccaatataaagttaccttaagttaatggtcttagaagagtaccatcaaggtaagcaaggtaaatatttaaataaatataaaattctaagatataaaacttcggtatagaatcagggattactttattaaaagtaactagcatgttgccagttttccctatttattaaacaaactgaatagaattcagaacacactactgagcaaaatgtatatttaaaaaaaagtcaactagaagtaataattctatttgtacacagcataaatcaatatacagtattgtatgtgaatgagactgattggctttaaaatgaattttctgcttcaaggccaatatctctacaaacgttctgtagaagtattgttagggcaggccaacttctttatgatgtcgcattatgtgctggttcttttctgaaggtcttcggaagcctttcttgcagtactcacaccggtgaggatagtctttcgtgtgaatggaaataacgtgccgtttaaagcctgaggcatctgtagtgctatactcacagtactcacactgatacactttcctgccactgtgtgtcttcatatgctttttaagctcactctgttgcctaaatccctttctacatctcttgcacctaaatggaagatcctttgtgtgaactgagagaatatggcgacttagaacaaatggatctgcaatcttaaagtcacaatgtctacactggtgcatttttttgcccttgtgggcagccacgtgtttcttgagttctgaaggcctgtgaaagcctttatcacacatgtcacacttatgggggtagtctttcgtgtgaactgaaattatgtgtcgtttcaaatcacttgagttcgaactcttgtggtcgcaatgcaaacactggtgtgttttgctttcttggtggataagagcatgttgctgcacctctttggtatccgagaaagtcagaagacaaatgtcacacttgaatggcatctctttactatgcttagttttgacatgcgttttcaagttagaagagtctgcagacctatattcgcagtactggcattggtacggcttctccccagtatggattctcatgtgctttttgagctctgacgggtgacgaaaacccttaccacactccacacaaatatgaggaaagttcttgctgtggactgccaagaggtggcgattcaataacccttgttcagctgtctcgtattcacagaatttacacttgtgcattttgttggctcctttttccttatgcaccattttgtgagtaaacaaagcccctgcatgagagaaatgcttcccacactcatcgcattcaatggccttctctgccttgctggtcagcttgtggctctccaggtggttgtgtaaacttatcttcttgttggtagtgtaatcacagtcagtacagcggtatttcttcttggcaaggtgttcgggatggtttttcatgtgccttttcaaaaaacctctcgacttaaacttcttcccacaaatcatgcaaggatagacagtcaaaggatgtccatcagggccaataattattgctgtttggtactgcctggaatcaggtcttctccttttctttggtttttgtttagccagtctgccgaggccagcagactcatctatgtgcaagagggcacttgcagtgccattccggttttcaattccatcagaattattaccataagctgctgcccatgcaatcggcatgaaggttttgatttcattgtcatccatttgctgctcgtgcacggcggcggctgccgctgctgctgcagcatcctcctctcctacgatcacttccatataaacttcgtcagcgatttcagcaacatttaaatcttcatcttctggctgagagtcattgacagtcatataaaccatcttttccctgggaacacgaatactgctgttctgatcaagcagttcaactccatgatcattctcaggctcactctccacaatgtctacagttccacctaagtcatcttctccagggtcagctttaaaaatgtacaccttgatgacctcagggcaagtgccatccactttacaaggatcaatttccgactctgtgtccatggtcattccagaagaaccatcgtgttctattttgccagcatcatccaaggaaatcataaggtagtcctcacagttgcctttgtcatcatcctgctggtccacagggatcccattggcatctatgactgcttcagaggcacagtctgctaccaatacttcttctgaaactacgtcggtagtcagaggatcagtgacaatttctgcttccactacactatcatgaaccacatgttcaacatgtccaacatgtccaacatgtccaacgtcagacacatgtatagaatcacccgtcaagacgtgttctggcatagacattgaggctgaagtaatgtcagaagctaaaacatcatctgggactgtgcaatgtgctaaagaaacttcttcagttacatctgagtccagcacttgctcaggaatgatgaccgtttcagacacatctgcttcttccatgatatctgggcactgaacatcttctataacaacgtcctcaataacatcttggattacaactgaatctgggtcatcaggaacaaagttatgcacagttatgtctgaatccacaacatctgaaacaaaaacagtttcttgtacttccacaacaatttgatcaccatccatgtgtgtaccatcagctcctcacaggactgtggtgatgatcaaatgggaatgtatgggaagtgttctgaaaaactgttgcatcaaaaaatgagtttggctcttgttgtaattcaagcccatcttcatccatggcctttaattctcatcagtcacagctcctgtaatcccagctactcgagaggctgaggcagaagaagaatcacttgaacacagaaggcagaggctgcagtgagccaaatttgcaccactgcactgcattccagcctggatgacagaggaagactgtctgtcttaatcacacaacttgactctaatcttaatcttgaacatccactgttgctgtactgcgcagcaaaacaattctatcttcttaatagttcttctatgtctttcccagcggacggacgtgcgggcggccggcgacggtggcgggtgctgcaggccggcctttctctggagcactgggccgggctccggctggtggggcgggcggagggagggaggaggggccgagctcggagctgacaaaaagcggcccagctccccggcacgggcccgccgtcagcacgtcacgtcaccgcccgggagagagacccaggaaaatgcggaagggtagacaggccccctcctccgcccggtgggtcctcctggcaccccgtgtcggcgccgctcccgccccgcgaccggggagcccagtggcctcgctgcggcggggtctccggcggccggag

SEQ ID NO: 18207 - RNA, 4134 nt, Homo sapiens
  source 1..4134: mol_type = other RNA
tgaagtaccagctactcgagaggctgaggcagataattgcttgaacccaggaagcagaggttgcagtgagctgcagaggttgcagtgatcacaccactgcagtccagcctgggcaacagagcaagactccgtcttaagaaaaaaaaacaacaaaaaaaaacaaacaaacaaaaaacctgtggaagacttagtgatgttccaaataaggcctcagactttccttatccacttaaaacacatctttaccttttaatcaaagccaacttgagtgttaagtttttaaagtttgctaactgtaactgagaaataacagatcagcctgaacttgccgagtgtgaagtcataattagcacccgttctctggtccacagagccatcacttcttttccatccccctcactaggtaagacagagttccctctcaggcttctcaaagagaactgtgggagtcatgtctggatactcatttgcttttcagaaaaacataaagacatggaggtgaaattgtatgaaaacattctacctagaaacatcttaacctctatgtttcaattaccaaagatatttaaaagaaaatatctttactctttaaaaatactagtgtccttattttccttctaattcttcacctgagtagtctctctgaagagcatgacttacaaaatgctctctcatgcatccctggatctttcatgttattgtaaatttaatacttttcattatagattttaaacaactactacttggggttgtgtgtataaatatgtaaaataagcaatacacacaggtacatgatatatatgtgtatatatataattcagggtacatttacatacataaagttgcaaaagatcctataagccatgagttacctctaggagattccaaaatgcagtcctcagtaagtgtcatttgtagcacacaaccattccaagatgaagccgcacagacagaataatcaaaatacaacatgagcaagcacagtttttcaataaggttttctaaaagtttgctacgctgacaaaagatgtaaataatccaaagaaagccaaaagaagtatatttgaaaagtaaacacgaacccagccactgctctttactcagcaaagccagggacgcaacagctcaaatggaaactttcactgtcaagtggtctgaaaatattaagcaagacaagtaaatgacttccatgttatgataattagacctgactgtaaaatctcccatttatattagtagatgtctctgacaattttattgtgagaaatgtatggggaaaaaaatgagtcaacatgaatactttcagagttaccaatataaagttaccttaagttaatggtcttagaagagtaccatcaaggtaagcaaggtaaatatttaaataaatataaaattctaagatataaaacttcggtatagaatcagggattactttattaaaagtaactagcatgttgccagttttccctatttattaaacaaactgaatagaattcagaacacactactgagcaaaatgtatatttaaaaaaaagtcaactagaagtaataattctatttgtacacagcataaatcaatatacagtattgtatgtgaatgagactgattggctttaaaatgaattttctgcttcaaggccaatatctctacaaacgttctgtagaagtattgttagggcaggccaacttctttatgatgtcgcattatgtgctggttcttttctgaaggtcttcggaagcctttcttgcagtactcacaccggtgaggatagtctttcgtgtgaatggaaataacgtgccgtttaaagcctgaggcatctgtagtgctatactcacagtactcacactgatacactttcctgccactgtgtgtcttcatatgctttttaagctcactctgttgcctaaatccctttctacatctcttgcacctaaatggaagatcctttgtgtgaactgagagaatatggcgacttagaacaaatggatctgcaatcttaaagtcacaatgtctacactggtgcatttttttgcccttgtgggcagccacgtgtttcttgagttctgaaggcctgtgaaagcctttatcacacatgtcacacttatgggggtagtctttcgtgtgaactgaaattatgtgtcgtttcaaatcacttgagttcgaactcttgtggtcgcaatgcaaacactggtgtgttttgctttcttggtggataagagcatgttgctgcacctctttggtatccgagaaagtcagaagacaaatgtcacacttgaatggcatctctttactatgcttagttttgacatgcgttttcaagttagaagagtctgcagacctatattcgcagtactggcattggtacggcttctccccagtatggattctcatgtgctttttgagctctgacgggtgacgaaaacccttaccacactccacacaaatatgaggaaagttcttgctgtggactgccaagaggtggcgattcaataacccttgttcagctgtctcgtattcacagaatttacacttgtgcattttgttggctcctttttccttatgcaccattttgtgagtaaacaaagcccctgcatgagagaaatgcttcccacactcatcgcattcaatggccttctctgccttgctggtcagcttgtggctctccaggtggttgtgtaaacttatcttcttgttggtagtgtaatcacagtcagtacagcggtatttcttcttggcaaggtgttcgggatggtttttcatgtgccttttcaaaaaacctctcgacttaaacttcttcccacaaatcatgcaaggatagacagtcaaaggatgtccatcagggccaataattattgctgtttggtactgcctggaatcaggtcttctccttttctttggtttttgtttagccagtctgccgaggccagcagactcatctatgtgcaagagggcacttgcagtgccattccggttttcaattccatcagaattattaccataagctgctgcccatgcaatcggcatgaaggttttgatttcattgtcatccatttgctgctcgtgcacggcggcggctgccgctgctgctgcagcatcctcctctcctacgatcacttccatataaacttcgtcagcgatttcagcaacatttaaatcttcatcttctggctgagagtcattgacagtcatataaaccatcttttccctgggaacacgaatactgctgttctgatcaagcagttcaactccatgatcattctcaggctcactctccacaatgtctacagttccacctaagtcatcttctccagggtcagctttaaaaatgtacaccttgatgacctcagggcaagtgccatccactttacaaggatcaatttccgactctgtgtccatggtcattccagaagaaccatcgtgttctattttgccagcatcatccaaggaaatcataaggtagtcctcacagttgcctttgtcatcatcctgctggtccacagggatcccattggcatctatgactgcttcagaggcacagtctgctaccaatacttcttctgaaactacgtcggtagtcagaggatcagtgacaatttctgcttccactacactatcatgaaccacatgttcaacatgtccaacatgtccaacatgtccaacgtcagacacatgtatagaatcacccgtcaagacgtgttctggcatagacattgaggctgaagtaatgtcagaagctaaaacatcatctgggactgtgcaatgtgctaaagaaacttcttcagttacatctgagtccagcacttgctcaggaatgatgaccgtttcagacacatctgcttcttccatgatatctgggcactgaacatcttctataacaacgtcctcaataacatcttggattacaactgaatctgggtcatcaggaacaaagttatgcacagttatgtctgaatccacaacatctgaaacaaaaacagtttcttgtacttccacaacaatttgatcaccatccatgtgtgtaccatcagctcctgaagtcaagggttcgagaccagcctggccaacattgtgaaaccccgtctctactaaaaatataaaaattaaccaggcgtagtggtgcatgcctgtaatcc

SEQ ID NO: 18208 - RNA, 4451 nt, Homo sapiens
  source 1..4451: mol_type = other RNA
tgaagtaccagctactcgagaggctgaggcagataattgcttgaacccaggaagcagaggttgcagtgagctgcagaggttgcagtgatcacaccactgcagtccagcctgggcaacagagcaagactccgtcttaagaaaaaaaaacaacaaaaaaaaacaaacaaacaaaaaacctgtggaagacttagtgatgttccaaataaggcctcagactttccttatccacttaaaacacatctttaccttttaatcaaagccaacttgagtgttaagtttttaaagtttgctaactgtaactgagaaataacagatcagcctgaacttgccgagtgtgaagtcataattagcacccgttctctggtccacagagccatcacttcttttccatccccctcactaggtaagacagagttccctctcaggcttctcaaagagaactgtgggagtcatgtctggatactcatttgcttttcagaaaaacataaagacatggaggtgaaattgtatgaaaacattctacctagaaacatcttaacctctatgtttcaattaccaaagatatttaaaagaaaatatctttactctttaaaaatactagtgtccttattttccttctaattcttcacctgagtagtctctctgaagagcatgacttacaaaatgctctctcatgcatccctggatctttcatgttattgtaaatttaatacttttcattatagattttaaacaactactacttggggttgtgtgtataaatatgtaaaataagcaatacacacaggtacatgatatatatgtgtatatatataattcagggtacatttacatacataaagttgcaaaagatcctataagccatgagttacctctaggagattccaaaatgcagtcctcagtaagtgtcatttgtagcacacaaccattccaagatgaagccgcacagacagaataatcaaaatacaacatgagcaagcacagtttttcaataaggttttctaaaagtttgctacgctgacaaaagatgtaaataatccaaagaaagccaaaagaagtatatttgaaaagtaaacacgaacccagccactgctctttactcagcaaagccagggacgcaacagctcaaatggaaactttcactgtcaagtggtctgaaaatattaagcaagacaagtaaatgacttccatgttatgataattagacctgactgtaaaatctcccatttatattagtagatgtctctgacaattttattgtgagaaatgtatggggaaaaaaatgagtcaacatgaatactttcagagttaccaatataaagttaccttaagttaatggtcttagaagagtaccatcaaggtaagcaaggtaaatatttaaataaatataaaattctaagatataaaacttcggtatagaatcagggattactttattaaaagtaactagcatgttgccagttttccctatttattaaacaaactgaatagaattcagaacacactactgagcaaaatgtatatttaaaaaaaagtcaactagaagtaataattctatttgtacacagcataaatcaatatacagtattgtatgtgaatgagactgattggctttaaaatgaattttctgcttcaaggccaatatctctacaaacgttctgtagaagtattgttagggcaggccaacttctttatgatgtcgcattatgtgctggttcttttctgaaggtcttcggaagcctttcttgcagtactcacaccggtgaggatagtctttcgtgtgaatggaaataacgtgccgtttaaagcctgaggcatctgtagtgctatactcacagtactcacactgatacactttcctgccactgtgtgtcttcatatgctttttaagctcactctgttgcctaaatccctttctacatctcttgcacctaaatggaagatcctttgtgtgaactgagagaatatggcgacttagaacaaatggatctgcaatcttaaagtcacaatgtctacactggtgcatttttttgcccttgtgggcagccacgtgtttcttgagttctgaaggcctgtgaaagcctttatcacacatgtcacacttatgggggtagtctttcgtgtgaactgaaattatgtgtcgtttcaaatcacttgagttcgaactcttgtggtcgcaatgcaaacactggtgtgttttgctttcttggtggataagagcatgttgctgcacctctttggtatccgagaaagtcagaagacaaatgtcacacttgaatggcatctctttactatgcttagttttgacatgcgttttcaagttagaagagtctgcagacctatattcgcagtactggcattggtacggcttctccccagtatggattctcatgtgctttttgagctctgacgggtgacgaaaacccttaccacactccacacaaatatgaggaaagttcttgctgtggactgccaagaggtggcgattcaataacccttgttcagctgtctcgtattcacagaatttacacttgtgcattttgttggctcctttttccttatgcaccattttgtgagtaaacaaagcccctgcatgagagaaatgcttcccacactcatcgcattcaatggccttctctgccttgctggtcagcttgtggctctccaggtggttgtgtaaacttatcttcttgttggtagtgtaatcacagtcagtacagcggtatttcttcttggcaaggtgttcgggatggtttttcatgtgccttttcaaaaaacctctcgacttaaacttcttcccacaaatcatgcaaggatagacagtcaaaggatgtccatcagggccaataattattgctgtttggtactgcctggaatcaggtcttctccttttctttggtttttgtttagccagtctgccgaggccagcagactcatctatgtgcaagagggcacttgcagtgccattccggttttcaattccatcagaattattaccataagctgctgcccatgcaatcggcatgaaggttttgatttcattgtcatccatttgctgctcgtgcacggcggcggctgccgctgctgctgcagcatcctcctctcctacgatcacttccatataaacttcgtcagcgatttcagcaacatttaaatcttcatcttctggctgagagtcattgacagtcatataaaccatcttttccctgggaacacgaatactgctgttctgatcaagcagttcaactccatgatcattctcaggctcactctccacaatgtctacagttccacctaagtcatcttctccagggtcagctttaaaaatgtacaccttgatgacctcagggcaagtgccatccactttacaaggatcaatttccgactctgtgtccatggtcattccagaagaaccatcgtgttctattttgccagcatcatccaaggaaatcataaggtagtcctcacagttgcctttgtcatcatcctgctggtccacagggatcccattggcatctatgactgcttcagaggcacagtctgctaccaatacttcttctgaaactacgtcggtagtcagaggatcagtgacaatttctgcttccactacactatcatgaaccacatgttcaacatgtccaacatgtccaacatgtccaacgtcagacacatgtatagaatcacccgtcaagacgtgttctggcatagacattgaggctgaagtaatgtcagaagctaaaacatcatctgggactgtgcaatgtgctaaagaaacttcttcagttacatctgagtccagcacttgctcaggaatgatgaccgtttcagacacatctgcttcttccatgatatctgggcactgaacatcttctataacaacgtcctcaataacatcttggattacaactgaatctgggtcatcaggaacaaagttatgcacagttatgtctgaatccacaacatctgaaacaaaaacagtttcttgtacttccacaacaatttgatcaccatccatgtgtgtaccatcagctcctgtagccccagttactcgggaagctgagcagatcacttgagcctgggaggcggaggttgcagtggacccagatggcgccactgtgctccagcctgggtgacagaacgagaccctgtctgttgcatcaaaaaatgagtttggctcttgttgtaattcaagcccatcttcatccatggcctttaattctcatcagtcacagctccgcctctcgcgccggtcctggccgaggctccagctcgagttgtttgcaggccctcagacccccgcccgcagtaaatgtgttttcttcatccccgtggctggggaggaagataaatttagcaacccccgccgtcccctgccttcgcttaaaaaaaaaaaatctttgaaataaaatgaaaacgggcttgccagtctaaatgggtgtgcgggaaggggg

SEQ ID NO: 18209 - RNA, 4571 nt, Homo sapiens
  source 1..4571: mol_type = other RNA
tgaagtaccagctactcgagaggctgaggcagataattgcttgaacccaggaagcagaggttgcagtgagctgcagaggttgcagtgatcacaccactgcagtccagcctgggcaacagagcaagactccgtcttaagaaaaaaaaacaacaaaaaaaaacaaacaaacaaaaaacctgtggaagacttagtgatgttccaaataaggcctcagactttccttatccacttaaaacacatctttaccttttaatcaaagccaacttgagtgttaagtttttaaagtttgctaactgtaactgagaaataacagatcagcctgaacttgccgagtgtgaagtcataattagcacccgttctctggtccacagagccatcacttcttttccatccccctcactaggtaagacagagttccctctcaggcttctcaaagagaactgtgggagtcatgtctggatactcatttgcttttcagaaaaacataaagacatggaggtgaaattgtatgaaaacattctacctagaaacatcttaacctctatgtttcaattaccaaagatatttaaaagaaaatatctttactctttaaaaatactagtgtccttattttccttctaattcttcacctgagtagtctctctgaagagcatgacttacaaaatgctctctcatgcatccctggatctttcatgttattgtaaatttaatacttttcattatagattttaaacaactactacttggggttgtgtgtataaatatgtaaaataagcaatacacacaggtacatgatatatatgtgtatatatataattcagggtacatttacatacataaagttgcaaaagatcctataagccatgagttacctctaggagattccaaaatgcagtcctcagtaagtgtcatttgtagcacacaaccattccaagatgaagccgcacagacagaataatcaaaatacaacatgagcaagcacagtttttcaataaggttttctaaaagtttgctacgctgacaaaagatgtaaataatccaaagaaagccaaaagaagtatatttgaaaagtaaacacgaacccagccactgctctttactcagcaaagccagggacgcaacagctcaaatggaaactttcactgtcaagtggtctgaaaatattaagcaagacaagtaaatgacttccatgttatgataattagacctgactgtaaaatctcccatttatattagtagatgtctctgacaattttattgtgagaaatgtatggggaaaaaaatgagtcaacatgaatactttcagagttaccaatataaagttaccttaagttaatggtcttagaagagtaccatcaaggtaagcaaggtaaatatttaaataaatataaaattctaagatataaaacttcggtatagaatcagggattactttattaaaagtaactagcatgttgccagttttccctatttattaaacaaactgaatagaattcagaacacactactgagcaaaatgtatatttaaaaaaaagtcaactagaagtaataattctatttgtacacagcataaatcaatatacagtattgtatgtgaatgagactgattggctttaaaatgaattttctgcttcaaggccaatatctctacaaacgttctgtagaagtattgttagggcaggccaacttctttatgatgtcgcattatgtgctggttcttttctgaaggtcttcggaagcctttcttgcagtactcacaccggtgaggatagtctttcgtgtgaatggaaataacgtgccgtttaaagcctgaggcatctgtagtgctatactcacagtactcacactgatacactttcctgccactgtgtgtcttcatatgctttttaagctcactctgttgcctaaatccctttctacatctcttgcacctaaatggaagatcctttgtgtgaactgagagaatatggcgacttagaacaaatggatctgcaatcttaaagtcacaatgtctacactggtgcatttttttgcccttgtgggcagccacgtgtttcttgagttctgaaggcctgtgaaagcctttatcacacatgtcacacttatgggggtagtctttcgtgtgaactgaaattatgtgtcgtttcaaatcacttgagttcgaactcttgtggtcgcaatgcaaacactggtgtgttttgctttcttggtggataagagcatgttgctgcacctctttggtatccgagaaagtcagaagacaaatgtcacacttgaatggcatctctttactatgcttagttttgacatgcgttttcaagttagaagagtctgcagacctatattcgcagtactggcattggtacggcttctccccagtatggattctcatgtgctttttgagctctgacgggtgacgaaaacccttaccacactccacacaaatatgaggaaagttcttgctgtggactgccaagaggtggcgattcaataacccttgttcagctgtctcgtattcacagaatttacacttgtgcattttgttggctcctttttccttatgcaccattttgtgagtaaacaaagcccctgcatgagagaaatgcttcccacactcatcgcattcaatggccttctctgccttgctggtcagcttgtggctctccaggtggttgtgtaaacttatcttcttgttggtagtgtaatcacagtcagtacagcggtatttcttcttggcaaggtgttcgggatggtttttcatgtgccttttcaaaaaacctctcgacttaaacttcttcccacaaatcatgcaaggatagacagtcaaaggatgtccatcagggccaataattattgctgtttggtactgcctggaatcaggtcttctccttttctttggtttttgtttagccagtctgccgaggccagcagactcatctatgtgcaagagggcacttgcagtgccattccggttttcaattccatcagaattattaccataagctgctgcccatgcaatcggcatgaaggttttgatttcattgtcatccatttgctgctcgtgcacggcggcggctgccgctgctgctgcagcatcctcctctcctacgatcacttccatataaacttcgtcagcgatttcagcaacatttaaatcttcatcttctggctgagagtcattgacagtcatataaaccatcttttccctgggaacacgaatactgctgttctgatcaagcagttcaactccatgatcattctcaggctcactctccacaatgtctacagttccacctaagtcatcttctccagggtcagctttaaaaatgtacaccttgatgacctcagggcaagtgccatccactttacaaggatcaatttccgactctgtgtccatggtcattccagaagaaccatcgtgttctattttgccagcatcatccaaggaaatcataaggtagtcctcacagttgcctttgtcatcatcctgctggtccacagggatcccattggcatctatgactgcttcagaggcacagtctgctaccaatacttcttctgaaactacgtcggtagtcagaggatcagtgacaatttctgcttccactacactatcatgaaccacatgttcaacatgtccaacatgtccaacatgtccaacgtcagacacatgtatagaatcacccgtcaagacgtgttctggcatagacattgaggctgaagtaatgtcagaagctaaaacatcatctgggactgtgcaatgtgctaaagaaacttcttcagttacatctgagtccagcacttgctcaggaatgatgaccgtttcagacacatctgcttcttccatgatatctgggcactgaacatcttctataacaacgtcctcaataacatcttggattacaactgaatctgggtcatcaggaacaaagttatgcacagttatgtctgaatccacaacatctgaaacaaaaacagtttcttgtacttccacaacaatttgatcaccatccatgtgtgtaccatcagctcctgtagccccagttactcgggaagctgagcagatcacttgagcctgggaggcggaggttgcagtggacccagatggcgccactgtgctccagcctgggtgacagaacgagaccctgtctgttgcatcaaaaaatgagtttggctcttgttgtaattcaagcccatcttcatccatggcctttaattctcatcagtcacagctccggacggacgtgcgggcggccggcgacggtggcgggtgctgcaggccggcctttctctggagcactgggccgggctccggctggtggggcgggcggagggagggaggaggggccgagctcggagctgacaaaaagcggcccagctccccggcacgggcccgccgtcagcacgtcacgtcaccgcccgggagagagacccaggaaaatgcggaagggtagacaggccccctcctccgcccggtgggtcctcctggcaccccgtgtcggcgccgctcccgccccgcgaccggggagcccagtggcctcgctgcggcggggtctccggcggccggagtc

SEQ ID NO: 18210 - RNA, 4249 nt, Homo sapiens
  source 1..4249: mol_type = other RNA
tgaagtaccagctactcgagaggctgaggcagataattgcttgaacccaggaagcagaggttgcagtgagctgcagaggttgcagtgatcacaccactgcagtccagcctgggcaacagagcaagactccgtcttaagaaaaaaaaacaacaaaaaaaaacaaacaaacaaaaaacctgtggaagacttagtgatgttccaaataaggcctcagactttccttatccacttaaaacacatctttaccttttaatcaaagccaacttgagtgttaagtttttaaagtttgctaactgtaactgagaaataacagatcagcctgaacttgccgagtgtgaagtcataattagcacccgttctctggtccacagagccatcacttcttttccatccccctcactaggtaagacagagttccctctcaggcttctcaaagagaactgtgggagtcatgtctggatactcatttgcttttcagaaaaacataaagacatggaggtgaaattgtatgaaaacattctacctagaaacatcttaacctctatgtttcaattaccaaagatatttaaaagaaaatatctttactctttaaaaatactagtgtccttattttccttctaattcttcacctgagtagtctctctgaagagcatgacttacaaaatgctctctcatgcatccctggatctttcatgttattgtaaatttaatacttttcattatagattttaaacaactactacttggggttgtgtgtataaatatgtaaaataagcaatacacacaggtacatgatatatatgtgtatatatataattcagggtacatttacatacataaagttgcaaaagatcctataagccatgagttacctctaggagattccaaaatgcagtcctcagtaagtgtcatttgtagcacacaaccattccaagatgaagccgcacagacagaataatcaaaatacaacatgagcaagcacagtttttcaataaggttttctaaaagtttgctacgctgacaaaagatgtaaataatccaaagaaagccaaaagaagtatatttgaaaagtaaacacgaacccagccactgctctttactcagcaaagccagggacgcaacagctcaaatggaaactttcactgtcaagtggtctgaaaatattaagcaagacaagtaaatgacttccatgttatgataattagacctgactgtaaaatctcccatttatattagtagatgtctctgacaattttattgtgagaaatgtatggggaaaaaaatgagtcaacatgaatactttcagagttaccaatataaagttaccttaagttaatggtcttagaagagtaccatcaaggtaagcaaggtaaatatttaaataaatataaaattctaagatataaaacttcggtatagaatcagggattactttattaaaagtaactagcatgttgccagttttccctatttattaaacaaactgaatagaattcagaacacactactgagcaaaatgtatatttaaaaaaaagtcaactagaagtaataattctatttgtacacagcataaatcaatatacagtattgtatgtgaatgagactgattggctttaaaatgaattttctgcttcaaggccaatatctctacaaacgttctgtagaagtattgttagggcaggccaacttctttatgatgtcgcattatgtgctggttcttttctgaaggtcttcggaagcctttcttgcagtactcacaccggtgaggatagtctttcgtgtgaatggaaataacgtgccgtttaaagcctgaggcatctgtagtgctatactcacagtactcacactgatacactttcctgccactgtgtgtcttcatatgctttttaagctcactctgttgcctaaatccctttctacatctcttgcacctaaatggaagatcctttgtgtgaactgagagaatatggcgacttagaacaaatggatctgcaatcttaaagtcacaatgtctacactggtgcatttttttgcccttgtgggcagccacgtgtttcttgagttctgaaggcctgtgaaagcctttatcacacatgtcacacttatgggggtagtctttcgtgtgaactgaaattatgtgtcgtttcaaatcacttgagttcgaactcttgtggtcgcaatgcaaacactggtgtgttttgctttcttggtggataagagcatgttgctgcacctctttggtatccgagaaagtcagaagacaaatgtcacacttgaatggcatctctttactatgcttagttttgacatgcgttttcaagttagaagagtctgcagacctatattcgcagtactggcattggtacggcttctccccagtatggattctcatgtgctttttgagctctgacgggtgacgaaaacccttaccacactccacacaaatatgaggaaagttcttgctgtggactgccaagaggtggcgattcaataacccttgttcagctgtctcgtattcacagaatttacacttgtgcattttgttggctcctttttccttatgcaccattttgtgagtaaacaaagcccctgcatgagagaaatgcttcccacactcatcgcattcaatggccttctctgccttgctggtcagcttgtggctctccaggtggttgtgtaaacttatcttcttgttggtagtgtaatcacagtcagtacagcggtatttcttcttggcaaggtgttcgggatggtttttcatgtgccttttcaaaaaacctctcgacttaaacttcttcccacaaatcatgcaaggatagacagtcaaaggatgtccatcagggccaataattattgctgtttggtactgcctggaatcaggtcttctccttttctttggtttttgtttagccagtctgccgaggccagcagactcatctatgtgcaagagggcacttgcagtgccattccggttttcaattccatcagaattattaccataagctgctgcccatgcaatcggcatgaaggttttgatttcattgtcatccatttgctgctcgtgcacggcggcggctgccgctgctgctgcagcatcctcctctcctacgatcacttccatataaacttcgtcagcgatttcagcaacatttaaatcttcatcttctggctgagagtcattgacagtcatataaaccatcttttccctgggaacacgaatactgctgttctgatcaagcagttcaactccatgatcattctcaggctcactctccacaatgtctacagttccacctaagtcatcttctccagggtcagctttaaaaatgtacaccttgatgacctcagggcaagtgccatccactttacaaggatcaatttccgactctgtgtccatggtcattccagaagaaccatcgtgttctattttgccagcatcatccaaggaaatcataaggtagtcctcacagttgcctttgtcatcatcctgctggtccacagggatcccattggcatctatgactgcttcagaggcacagtctgctaccaatacttcttctgaaactacgtcggtagtcagaggatcagtgacaatttctgcttccactacactatcatgaaccacatgttcaacatgtccaacatgtccaacatgtccaacgtcagacacatgtatagaatcacccgtcaagacgtgttctggcatagacattgaggctgaagtaatgtcagaagctaaaacatcatctgggactgtgcaatgtgctaaagaaacttcttcagttacatctgagtccagcacttgctcaggaatgatgaccgtttcagacacatctgcttcttccatgatatctgggcactgaacatcttctataacaacgtcctcaataacatcttggattacaactgaatctgggtcatcaggaacaaagttatgcacagttatgtctgaatccacaacatctgaaacaaaaacagtttcttgtacttccacaacaatttgatcaccatccatgtgtgtaccatcagctcctgtagccccagttactcgggaagctgagcagatcacttgagcctgggaggcggaggttgcagtggacccagatggcgccactgtgctccagcctgggtgacagaacgagaccctgtctgttgcatcaaaaaatgagtttggctcttgttgtaattcaagcccatcttcatccatggcctttaattctcatcagtcacagctcctgtaatcccagca

SEQ ID NO: 18211 - RNA, 4715 nt, Homo sapiens
  source 1..4715: mol_type = other RNA
tgaagtaccagctactcgagaggctgaggcagataattgcttgaacccaggaagcagaggttgcagtgagctgcagaggttgcagtgatcacaccactgcagtccagcctgggcaacagagcaagactccgtcttaagaaaaaaaaacaacaaaaaaaaacaaacaaacaaaaaacctgtggaagacttagtgatgttccaaataaggcctcagactttccttatccacttaaaacacatctttaccttttaatcaaagccaacttgagtgttaagtttttaaagtttgctaactgtaactgagaaataacagatcagcctgaacttgccgagtgtgaagtcataattagcacccgttctctggtccacagagccatcacttcttttccatccccctcactaggtaagacagagttccctctcaggcttctcaaagagaactgtgggagtcatgtctggatactcatttgcttttcagaaaaacataaagacatggaggtgaaattgtatgaaaacattctacctagaaacatcttaacctctatgtttcaattaccaaagatatttaaaagaaaatatctttactctttaaaaatactagtgtccttattttccttctaattcttcacctgagtagtctctctgaagagcatgacttacaaaatgctctctcatgcatccctggatctttcatgttattgtaaatttaatacttttcattatagattttaaacaactactacttggggttgtgtgtataaatatgtaaaataagcaatacacacaggtacatgatatatatgtgtatatatataattcagggtacatttacatacataaagttgcaaaagatcctataagccatgagttacctctaggagattccaaaatgcagtcctcagtaagtgtcatttgtagcacacaaccattccaagatgaagccgcacagacagaataatcaaaatacaacatgagcaagcacagtttttcaataaggttttctaaaagtttgctacgctgacaaaagatgtaaataatccaaagaaagccaaaagaagtatatttgaaaagtaaacacgaacccagccactgctctttactcagcaaagccagggacgcaacagctcaaatggaaactttcactgtcaagtggtctgaaaatattaagcaagacaagtaaatgacttccatgttatgataattagacctgactgtaaaatctcccatttatattagtagatgtctctgacaattttattgtgagaaatgtatggggaaaaaaatgagtcaacatgaatactttcagagttaccaatataaagttaccttaagttaatggtcttagaagagtaccatcaaggtaagcaaggtaaatatttaaataaatataaaattctaagatataaaacttcggtatagaatcagggattactttattaaaagtaactagcatgttgccagttttccctatttattaaacaaactgaatagaattcagaacacactactgagcaaaatgtatatttaaaaaaaagtcaactagaagtaataattctatttgtacacagcataaatcaatatacagtattgtatgtgaatgagactgattggctttaaaatgaattttctgcttcaaggccaatatctctacaaacgttctgtagaagtattgttagggcaggccaacttctttatgatgtcgcattatgtgctggttcttttctgaaggtcttcggaagcctttcttgcagtactcacaccggtgaggatagtctttcgtgtgaatggaaataacgtgccgtttaaagcctgaggcatctgtagtgctatactcacagtactcacactgatacactttcctgccactgtgtgtcttcatatgctttttaagctcactctgttgcctaaatccctttctacatctcttgcacctaaatggaagatcctttgtgtgaactgagagaatatggcgacttagaacaaatggatctgcaatcttaaagtcacaatgtctacactggtgcatttttttgcccttgtgggcagccacgtgtttcttgagttctgaaggcctgtgaaagcctttatcacacatgtcacacttatgggggtagtctttcgtgtgaactgaaattatgtgtcgtttcaaatcacttgagttcgaactcttgtggtcgcaatgcaaacactggtgtgttttgctttcttggtggataagagcatgttgctgcacctctttggtatccgagaaagtcagaagacaaatgtcacacttgaatggcatctctttactatgcttagttttgacatgcgttttcaagttagaagagtctgcagacctatattcgcagtactggcattggtacggcttctccccagtatggattctcatgtgctttttgagctctgacgggtgacgaaaacccttaccacactccacacaaatatgaggaaagttcttgctgtggactgccaagaggtggcgattcaataacccttgttcagctgtctcgtattcacagaatttacacttgtgcattttgttggctcctttttccttatgcaccattttgtgagtaaacaaagcccctgcatgagagaaatgcttcccacactcatcgcattcaatggccttctctgccttgctggtcagcttgtggctctccaggtggttgtgtaaacttatcttcttgttggtagtgtaatcacagtcagtacagcggtatttcttcttggcaaggtgttcgggatggtttttcatgtgccttttcaaaaaacctctcgacttaaacttcttcccacaaatcatgcaaggatagacagtcaaaggatgtccatcagggccaataattattgctgtttggtactgcctggaatcaggtcttctccttttctttggtttttgtttagccagtctgccgaggccagcagactcatctatgtgcaagagggcacttgcagtgccattccggttttcaattccatcagaattattaccataagctgctgcccatgcaatcggcatgaaggttttgatttcattgtcatccatttgctgctcgtgcacggcggcggctgccgctgctgctgcagcatcctcctctcctacgatcacttccatataaacttcgtcagcgatttcagcaacatttaaatcttcatcttctggctgagagtcattgacagtcatataaaccatcttttccctgggaacacgaatactgctgttctgatcaagcagttcaactccatgatcattctcaggctcactctccacaatgtctacagttccacctaagtcatcttctccagggtcagctttaaaaatgtacaccttgatgacctcagggcaagtgccatccactttacaaggatcaatttccgactctgtgtccatggtcattccagaagaaccatcgtgttctattttgccagcatcatccaaggaaatcataaggtagtcctcacagttgcctttgtcatcatcctgctggtccacagggatcccattggcatctatgactgcttcagaggcacagtctgctaccaatacttcttctgaaactacgtcggtagtcagaggatcagtgacaatttctgcttccactacactatcatgaaccacatgttcaacatgtccaacatgtccaacatgtccaacgtcagacacatgtatagaatcacccgtcaagacgtgttctggcatagacattgaggctgaagtaatgtcagaagctaaaacatcatctgggactgtgcaatgtgctaaagaaacttcttcagttacatctgagtccagcacttgctcaggaatgatgaccgtttcagacacatctgcttcttccatgatatctgggcactgaacatcttctataacaacgtcctcaataacatcttggattacaactgaatctgggtcatcaggaacaaagttatgcacagttatgtctgaatccacaacatctgaaacaaaaacagtttcttgtacttccacaacaatttgatcaccatccatgtgtgtaccatcagctcctgtagccccagttactcgggaagctgagcagatcacttgagcctgggaggcggaggttgcagtggacccagatggcgccactgtgctccagcctgggtgacagaacgagaccctgtctgttgcatcaaaaaatgagtttggctcttgttgtaattcaagcccatcttcatccatggcctttaattctcatcagtcacagctcctgtaatcccagctactcgagaggctgaggcagaagaagaatcacttgaacacagaaggcagaggctgcagtgagccaaatttgcaccactgcactgcattccagcctggatgacagaggaagactgtctgtcttaatcacacaacttgactctaatcttaatcttgaacatccactgttgctgtactgcgcagcaaaacaattctatcttcttaatagttcttctatgtctttcccagcgtaaagcacagctcagggaacagacggcagtgacaggcgggcagtgggaggcgggagaacggcttgagcccaggagttcgagaccagcctggggcaatatagcaagaacctgtctcaaaataaaaaataagtaaataacaaggtgcagctcaggtgtgccatcactcttctagttgagggcacccccgctgcctaccccattgagtataagcccctccacctggcaagcaagcccttctg

SEQ ID NO: 18212 - RNA, 4682 nt, Homo sapiens
  source 1..4682: mol_type = other RNA
tgaagtaccagctactcgagaggctgaggcagataattgcttgaacccaggaagcagaggttgcagtgagctgcagaggttgcagtgatcacaccactgcagtccagcctgggcaacagagcaagactccgtcttaagaaaaaaaaacaacaaaaaaaaacaaacaaacaaaaaacctgtggaagacttagtgatgttccaaataaggcctcagactttccttatccacttaaaacacatctttaccttttaatcaaagccaacttgagtgttaagtttttaaagtttgctaactgtaactgagaaataacagatcagcctgaacttgccgagtgtgaagtcataattagcacccgttctctggtccacagagccatcacttcttttccatccccctcactaggtaagacagagttccctctcaggcttctcaaagagaactgtgggagtcatgtctggatactcatttgcttttcagaaaaacataaagacatggaggtgaaattgtatgaaaacattctacctagaaacatcttaacctctatgtttcaattaccaaagatatttaaaagaaaatatctttactctttaaaaatactagtgtccttattttccttctaattcttcacctgagtagtctctctgaagagcatgacttacaaaatgctctctcatgcatccctggatctttcatgttattgtaaatttaatacttttcattatagattttaaacaactactacttggggttgtgtgtataaatatgtaaaataagcaatacacacaggtacatgatatatatgtgtatatatataattcagggtacatttacatacataaagttgcaaaagatcctataagccatgagttacctctaggagattccaaaatgcagtcctcagtaagtgtcatttgtagcacacaaccattccaagatgaagccgcacagacagaataatcaaaatacaacatgagcaagcacagtttttcaataaggttttctaaaagtttgctacgctgacaaaagatgtaaataatccaaagaaagccaaaagaagtatatttgaaaagtaaacacgaacccagccactgctctttactcagcaaagccagggacgcaacagctcaaatggaaactttcactgtcaagtggtctgaaaatattaagcaagacaagtaaatgacttccatgttatgataattagacctgactgtaaaatctcccatttatattagtagatgtctctgacaattttattgtgagaaatgtatggggaaaaaaatgagtcaacatgaatactttcagagttaccaatataaagttaccttaagttaatggtcttagaagagtaccatcaaggtaagcaaggtaaatatttaaataaatataaaattctaagatataaaacttcggtatagaatcagggattactttattaaaagtaactagcatgttgccagttttccctatttattaaacaaactgaatagaattcagaacacactactgagcaaaatgtatatttaaaaaaaagtcaactagaagtaataattctatttgtacacagcataaatcaatatacagtattgtatgtgaatgagactgattggctttaaaatgaattttctgcttcaaggccaatatctctacaaacgttctgtagaagtattgttagggcaggccaacttctttatgatgtcgcattatgtgctggttcttttctgaaggtcttcggaagcctttcttgcagtactcacaccggtgaggatagtctttcgtgtgaatggaaataacgtgccgtttaaagcctgaggcatctgtagtgctatactcacagtactcacactgatacactttcctgccactgtgtgtcttcatatgctttttaagctcactctgttgcctaaatccctttctacatctcttgcacctaaatggaagatcctttgtgtgaactgagagaatatggcgacttagaacaaatggatctgcaatcttaaagtcacaatgtctacactggtgcatttttttgcccttgtgggcagccacgtgtttcttgagttctgaaggcctgtgaaagcctttatcacacatgtcacacttatgggggtagtctttcgtgtgaactgaaattatgtgtcgtttcaaatcacttgagttcgaactcttgtggtcgcaatgcaaacactggtgtgttttgctttcttggtggataagagcatgttgctgcacctctttggtatccgagaaagtcagaagacaaatgtcacacttgaatggcatctctttactatgcttagttttgacatgcgttttcaagttagaagagtctgcagacctatattcgcagtactggcattggtacggcttctccccagtatggattctcatgtgctttttgagctctgacgggtgacgaaaacccttaccacactccacacaaatatgaggaaagttcttgctgtggactgccaagaggtggcgattcaataacccttgttcagctgtctcgtattcacagaatttacacttgtgcattttgttggctcctttttccttatgcaccattttgtgagtaaacaaagcccctgcatgagagaaatgcttcccacactcatcgcattcaatggccttctctgccttgctggtcagcttgtggctctccaggtggttgtgtaaacttatcttcttgttggtagtgtaatcacagtcagtacagcggtatttcttcttggcaaggtgttcgggatggtttttcatgtgccttttcaaaaaacctctcgacttaaacttcttcccacaaatcatgcaaggatagacagtcaaaggatgtccatcagggccaataattattgctgtttggtactgcctggaatcaggtcttctccttttctttggtttttgtttagccagtctgccgaggccagcagactcatctatgtgcaagagggcacttgcagtgccattccggttttcaattccatcagaattattaccataagctgctgcccatgcaatcggcatgaaggttttgatttcattgtcatccatttgctgctcgtgcacggcggcggctgccgctgctgctgcagcatcctcctctcctacgatcacttccatataaacttcgtcagcgatttcagcaacatttaaatcttcatcttctggctgagagtcattgacagtcatataaaccatcttttccctgggaacacgaatactgctgttctgatcaagcagttcaactccatgatcattctcaggctcactctccacaatgtctacagttccacctaagtcatcttctccagggtcagctttaaaaatgtacaccttgatgacctcagggcaagtgccatccactttacaaggatcaatttccgactctgtgtccatggtcattccagaagaaccatcgtgttctattttgccagcatcatccaaggaaatcataaggtagtcctcacagttgcctttgtcatcatcctgctggtccacagggatcccattggcatctatgactgcttcagaggcacagtctgctaccaatacttcttctgaaactacgtcggtagtcagaggatcagtgacaatttctgcttccactacactatcatgaaccacatgttcaacatgtccaacatgtccaacatgtccaacgtcagacacatgtatagaatcacccgtcaagacgtgttctggcatagacattgaggctgaagtaatgtcagaagctaaaacatcatctgggactgtgcaatgtgctaaagaaacttcttcagttacatctgagtccagcacttgctcaggaatgatgaccgtttcagacacatctgcttcttccatgatatctgggcactgaacatcttctataacaacgtcctcaataacatcttggattacaactgaatctgggtcatcaggaacaaagttatgcacagttatgtctgaatccacaacatctgaaacaaaaacagtttcttgtacttccacaacaatttgatcaccatccatgtgtgtaccatcagctcctgtagccccagttactcgggaagctgagcagatcacttgagcctgggaggcggaggttgcagtggacccagatggcgccactgtgctccagcctgggtgacagaacgagaccctgtctgttgcatcaaaaaatgagtttggctcttgttgtaattcaagcccatcttcatccatggcctttaattctcatcagtcacagctcctgtcttaatcacacaacttgactctaatcttaatcttgaacatccactgttgctgtactgcgcagcaaaacaattctatcttcttaatagttcttctatgtctttcccagcggacggacgtgcgggcggccggcgacggtggcgggtgctgcaggccggcctttctctggagcactgggccgggctccggctggtggggcgggcggagggagggaggaggggccgagctcggagctgacaaaaagcggcccagctccccggcacgggcccgccgtcagcacgtcacgtcaccgcccgggagagagacccaggaaaatgcggaagggtagacaggccccctcctccgcccggtgggtcctcctggcaccccgtgtcggcgccgctcccgccccgcgaccggggagcccagtggcctcgctgcggcggggtctccggcggccggagtc

SEQ ID NO: 18213 - RNA, 4728 nt, Homo sapiens
  source 1..4728: mol_type = other RNA
tgaagtaccagctactcgagaggctgaggcagataattgcttgaacccaggaagcagaggttgcagtgagctgcagaggttgcagtgatcacaccactgcagtccagcctgggcaacagagcaagactccgtcttaagaaaaaaaaacaacaaaaaaaaacaaacaaacaaaaaacctgtggaagacttagtgatgttccaaataaggcctcagactttccttatccacttaaaacacatctttaccttttaatcaaagccaacttgagtgttaagtttttaaagtttgctaactgtaactgagaaataacagatcagcctgaacttgccgagtgtgaagtcataattagcacccgttctctggtccacagagccatcacttcttttccatccccctcactaggtaagacagagttccctctcaggcttctcaaagagaactgtgggagtcatgtctggatactcatttgcttttcagaaaaacataaagacatggaggtgaaattgtatgaaaacattctacctagaaacatcttaacctctatgtttcaattaccaaagatatttaaaagaaaatatctttactctttaaaaatactagtgtccttattttccttctaattcttcacctgagtagtctctctgaagagcatgacttacaaaatgctctctcatgcatccctggatctttcatgttattgtaaatttaatacttttcattatagattttaaacaactactacttggggttgtgtgtataaatatgtaaaataagcaatacacacaggtacatgatatatatgtgtatatatataattcagggtacatttacatacataaagttgcaaaagatcctataagccatgagttacctctaggagattccaaaatgcagtcctcagtaagtgtcatttgtagcacacaaccattccaagatgaagccgcacagacagaataatcaaaatacaacatgagcaagcacagtttttcaataaggttttctaaaagtttgctacgctgacaaaagatgtaaataatccaaagaaagccaaaagaagtatatttgaaaagtaaacacgaacccagccactgctctttactcagcaaagccagggacgcaacagctcaaatggaaactttcactgtcaagtggtctgaaaatattaagcaagacaagtaaatgacttccatgttatgataattagacctgactgtaaaatctcccatttatattagtagatgtctctgacaattttattgtgagaaatgtatggggaaaaaaatgagtcaacatgaatactttcagagttaccaatataaagttaccttaagttaatggtcttagaagagtaccatcaaggtaagcaaggtaaatatttaaataaatataaaattctaagatataaaacttcggtatagaatcagggattactttattaaaagtaactagcatgttgccagttttccctatttattaaacaaactgaatagaattcagaacacactactgagcaaaatgtatatttaaaaaaaagtcaactagaagtaataattctatttgtacacagcataaatcaatatacagtattgtatgtgaatgagactgattggctttaaaatgaattttctgcttcaaggccaatatctctacaaacgttctgtagaagtattgttagggcaggccaacttctttatgatgtcgcattatgtgctggttcttttctgaaggtcttcggaagcctttcttgcagtactcacaccggtgaggatagtctttcgtgtgaatggaaataacgtgccgtttaaagcctgaggcatctgtagtgctatactcacagtactcacactgatacactttcctgccactgtgtgtcttcatatgctttttaagctcactctgttgcctaaatccctttctacatctcttgcacctaaatggaagatcctttgtgtgaactgagagaatatggcgacttagaacaaatggatctgcaatcttaaagtcacaatgtctacactggtgcatttttttgcccttgtgggcagccacgtgtttcttgagttctgaaggcctgtgaaagcctttatcacacatgtcacacttatgggggtagtctttcgtgtgaactgaaattatgtgtcgtttcaaatcacttgagttcgaactcttgtggtcgcaatgcaaacactggtgtgttttgctttcttggtggataagagcatgttgctgcacctctttggtatccgagaaagtcagaagacaaatgtcacacttgaatggcatctctttactatgcttagttttgacatgcgttttcaagttagaagagtctgcagacctatattcgcagtactggcattggtacggcttctccccagtatggattctcatgtgctttttgagctctgacgggtgacgaaaacccttaccacactccacacaaatatgaggaaagttcttgctgtggactgccaagaggtggcgattcaataacccttgttcagctgtctcgtattcacagaatttacacttgtgcattttgttggctcctttttccttatgcaccattttgtgagtaaacaaagcccctgcatgagagaaatgcttcccacactcatcgcattcaatggccttctctgccttgctggtcagcttgtggctctccaggtggttgtgtaaacttatcttcttgttggtagtgtaatcacagtcagtacagcggtatttcttcttggcaaggtgttcgggatggtttttcatgtgccttttcaaaaaacctctcgacttaaacttcttcccacaaatcatgcaaggatagacagtcaaaggatgtccatcagggccaataattattgctgtttggtactgcctggaatcaggtcttctccttttctttggtttttgtttagccagtctgccgaggccagcagactcatctatgtgcaagagggcacttgcagtgccattccggttttcaattccatcagaattattaccataagctgctgcccatgcaatcggcatgaaggttttgatttcattgtcatccatttgctgctcgtgcacggcggcggctgccgctgctgctgcagcatcctcctctcctacgatcacttccatataaacttcgtcagcgatttcagcaacatttaaatcttcatcttctggctgagagtcattgacagtcatataaaccatcttttccctgggaacacgaatactgctgttctgatcaagcagttcaactccatgatcattctcaggctcactctccacaatgtctacagttccacctaagtcatcttctccagggtcagctttaaaaatgtacaccttgatgacctcagggcaagtgccatccactttacaaggatcaatttccgactctgtgtccatggtcattccagaagaaccatcgtgttctattttgccagcatcatccaaggaaatcataaggtagtcctcacagttgcctttgtcatcatcctgctggtccacagggatcccattggcatctatgactgcttcagaggcacagtctgctaccaatacttcttctgaaactacgtcggtagtcagaggatcagtgacaatttctgcttccactacactatcatgaaccacatgttcaacatgtccaacatgtccaacatgtccaacgtcagacacatgtatagaatcacccgtcaagacgtgttctggcatagacattgaggctgaagtaatgtcagaagctaaaacatcatctgggactgtgcaatgtgctaaagaaacttcttcagttacatctgagtccagcacttgctcaggaatgatgaccgtttcagacacatctgcttcttccatgatatctgggcactgaacatcttctataacaacgtcctcaataacatcttggattacaactgaatctgggtcatcaggaacaaagttatgcacagttatgtctgaatccacaacatctgaaacaaaaacagtttcttgtacttccacaacaatttgatcaccatccatgtgtgtaccatcagctcctgtagccccagttactcgggaagctgagcagatcacttgagcctgggaggcggaggttgcagtggacccagatggcgccactgtgctccagcctgggtgacagaacgagaccctgtctgttgcatcaaaaaatgagtttggctcttgttgtaattcaagcccatcttcatccatggcctttaattctcatcagtcacagctcctgtcttaatcacacaacttgactctaatcttaatcttgaacatccactgttgctgtactgcgcagcaaaacaattctatcttcttaatagttcttctatgtctttcccagcgtaaagcacagctcagggaacagacggcagtgacaggcgggcagtgggaggcgggagaacggcttgagcccaggagttcgagaccagcctggggcaatatagcaagaaccgcctctcgcgccggtcctggccgaggctccagctcgagttgtttgcaggccctcagacccccgcccgcagtaaatgtgttttcttcatccccgtggctggggaggaagataaatttagcaacccccgccgtcccctgccttcgcttaaaaaaaaaaaatctttgaaataaaatgaaaacgggcttgccagtctaaatgggtgtgcgggaaggggggtggagtggggggagaagggttatccctagagcacctaccaggccgtctacttttt

SEQ ID NO: 18214 - RNA, 4792 nt, Homo sapiens
  source 1..4792: mol_type = other RNA
tgaagtaccagctactcgagaggctgaggcagataattgcttgaacccaggaagcagaggttgcagtgagctgcagaggttgcagtgatcacaccactgcagtccagcctgggcaacagagcaagactccgtcttaagaaaaaaaaacaacaaaaaaaaacaaacaaacaaaaaacctgtggaagacttagtgatgttccaaataaggcctcagactttccttatccacttaaaacacatctttaccttttaatcaaagccaacttgagtgttaagtttttaaagtttgctaactgtaactgagaaataacagatcagcctgaacttgccgagtgtgaagtcataattagcacccgttctctggtccacagagccatcacttcttttccatccccctcactaggtaagacagagttccctctcaggcttctcaaagagaactgtgggagtcatgtctggatactcatttgcttttcagaaaaacataaagacatggaggtgaaattgtatgaaaacattctacctagaaacatcttaacctctatgtttcaattaccaaagatatttaaaagaaaatatctttactctttaaaaatactagtgtccttattttccttctaattcttcacctgagtagtctctctgaagagcatgacttacaaaatgctctctcatgcatccctggatctttcatgttattgtaaatttaatacttttcattatagattttaaacaactactacttggggttgtgtgtataaatatgtaaaataagcaatacacacaggtacatgatatatatgtgtatatatataattcagggtacatttacatacataaagttgcaaaagatcctataagccatgagttacctctaggagattccaaaatgcagtcctcagtaagtgtcatttgtagcacacaaccattccaagatgaagccgcacagacagaataatcaaaatacaacatgagcaagcacagtttttcaataaggttttctaaaagtttgctacgctgacaaaagatgtaaataatccaaagaaagccaaaagaagtatatttgaaaagtaaacacgaacccagccactgctctttactcagcaaagccagggacgcaacagctcaaatggaaactttcactgtcaagtggtctgaaaatattaagcaagacaagtaaatgacttccatgttatgataattagacctgactgtaaaatctcccatttatattagtagatgtctctgacaattttattgtgagaaatgtatggggaaaaaaatgagtcaacatgaatactttcagagttaccaatataaagttaccttaagttaatggtcttagaagagtaccatcaaggtaagcaaggtaaatatttaaataaatataaaattctaagatataaaacttcggtatagaatcagggattactttattaaaagtaactagcatgttgccagttttccctatttattaaacaaactgaatagaattcagaacacactactgagcaaaatgtatatttaaaaaaaagtcaactagaagtaataattctatttgtacacagcataaatcaatatacagtattgtatgtgaatgagactgattggctttaaaatgaattttctgcttcaaggccaatatctctacaaacgttctgtagaagtattgttagggcaggccaacttctttatgatgtcgcattatgtgctggttcttttctgaaggtcttcggaagcctttcttgcagtactcacaccggtgaggatagtctttcgtgtgaatggaaataacgtgccgtttaaagcctgaggcatctgtagtgctatactcacagtactcacactgatacactttcctgccactgtgtgtcttcatatgctttttaagctcactctgttgcctaaatccctttctacatctcttgcacctaaatggaagatcctttgtgtgaactgagagaatatggcgacttagaacaaatggatctgcaatcttaaagtcacaatgtctacactggtgcatttttttgcccttgtgggcagccacgtgtttcttgagttctgaaggcctgtgaaagcctttatcacacatgtcacacttatgggggtagtctttcgtgtgaactgaaattatgtgtcgtttcaaatcacttgagttcgaactcttgtggtcgcaatgcaaacactggtgtgttttgctttcttggtggataagagcatgttgctgcacctctttggtatccgagaaagtcagaagacaaatgtcacacttgaatggcatctctttactatgcttagttttgacatgcgttttcaagttagaagagtctgcagacctatattcgcagtactggcattggtacggcttctccccagtatggattctcatgtgctttttgagctctgacgggtgacgaaaacccttaccacactccacacaaatatgaggaaagttcttgctgtggactgccaagaggtggcgattcaataacccttgttcagctgtctcgtattcacagaatttacacttgtgcattttgttggctcctttttccttatgcaccattttgtgagtaaacaaagcccctgcatgagagaaatgcttcccacactcatcgcattcaatggccttctctgccttgctggtcagcttgtggctctccaggtggttgtgtaaacttatcttcttgttggtagtgtaatcacagtcagtacagcggtatttcttcttggcaaggtgttcgggatggtttttcatgtgccttttcaaaaaacctctcgacttaaacttcttcccacaaatcatgcaaggatagacagtcaaaggatgtccatcagggccaataattattgctgtttggtactgcctggaatcaggtcttctccttttctttggtttttgtttagccagtctgccgaggccagcagactcatctatgtgcaagagggcacttgcagtgccattccggttttcaattccatcagaattattaccataagctgctgcccatgcaatcggcatgaaggttttgatttcattgtcatccatttgctgctcgtgcacggcggcggctgccgctgctgctgcagcatcctcctctcctacgatcacttccatataaacttcgtcagcgatttcagcaacatttaaatcttcatcttctggctgagagtcattgacagtcatataaaccatcttttccctgggaacacgaatactgctgttctgatcaagcagttcaactccatgatcattctcaggctcactctccacaatgtctacagttccacctaagtcatcttctccagggtcagctttaaaaatgtacaccttgatgacctcagggcaagtgccatccactttacaaggatcaatttccgactctgtgtccatggtcattccagaagaaccatcgtgttctattttgccagcatcatccaaggaaatcataaggtagtcctcacagttgcctttgtcatcatcctgctggtccacagggatcccattggcatctatgactgcttcagaggcacagtctgctaccaatacttcttctgaaactacgtcggtagtcagaggatcagtgacaatttctgcttccactacactatcatgaaccacatgttcaacatgtccaacatgtccaacatgtccaacgtcagacacatgtatagaatcacccgtcaagacgtgttctggcatagacattgaggctgaagtaatgtcagaagctaaaacatcatctgggactgtgcaatgtgctaaagaaacttcttcagttacatctgagtccagcacttgctcaggaatgatgaccgtttcagacacatctgcttcttccatgatatctgggcactgaacatcttctataacaacgtcctcaataacatcttggattacaactgaatctgggtcatcaggaacaaagttatgcacagttatgtctgaatccacaacatctgaaacaaaaacagtttcttgtacttccacaacaatttgatcaccatccatgtgtgtaccatcagctcctgtagccccagttactcgggaagctgagcagatcacttgagcctgggaggcggaggttgcagtggacccagatggcgccactgtgctccagcctgggtgacagaacgagaccctgtctgttgcatcaaaaaatgagtttggctcttgttgtaattcaagcccatcttcatccatggcctttaattctcatcagtcacagctcctgtcttaatcacacaacttgactctaatcttaatcttgaacatccactgttgctgtactgcgcagcaaaacaattctatcttcttaatagttcttctatgtctttcccagcgtaaagcacagctcagggaacagacggcagtgacaggcgggcagtgggaggcgggagaacggcttgagcccaggagttcgagaccagcctggggcaatatagcaagaaccggacggacgtgcgggcggccggcgacggtggcgggtgctgcaggccggcctttctctggagcactgggccgggctccggctggtggggcgggcggagggagggaggaggggccgagctcggagctgacaaaaagcggcccagctccccggcacgggcccgccgtcagcacgtcacgtcaccgcccgggagagagacccaggaaaatgcggaagggtagacaggccccctcctccgcccggtgggtcctcctggcaccccgtgtcggcgccgctcccgccccgcgaccggggagcccagtggcctcgctgcggcggggtctccggcggccggagtc

SEQ ID NO: 18215 - RNA, 5277 nt, Homo sapiens
  source 1..5277: mol_type = other RNA
tgaagtaccagctactcgagaggctgaggcagataattgcttgaacccaggaagcagaggttgcagtgagctgcagaggttgcagtgatcacaccactgcagtccagcctgggcaacagagcaagactccgtcttaagaaaaaaaaacaacaaaaaaaaacaaacaaacaaaaaacctgtggaagacttagtgatgttccaaataaggcctcagactttccttatccacttaaaacacatctttaccttttaatcaaagccaacttgagtgttaagtttttaaagtttgctaactgtaactgagaaataacagatcagcctgaacttgccgagtgtgaagtcataattagcacccgttctctggtccacagagccatcacttcttttccatccccctcactaggtaagacagagttccctctcaggcttctcaaagagaactgtgggagtcatgtctggatactcatttgcttttcagaaaaacataaagacatggaggtgaaattgtatgaaaacattctacctagaaacatcttaacctctatgtttcaattaccaaagatatttaaaagaaaatatctttactctttaaaaatactagtgtccttattttccttctaattcttcacctgagtagtctctctgaagagcatgacttacaaaatgctctctcatgcatccctggatctttcatgttattgtaaatttaatacttttcattatagattttaaacaactactacttggggttgtgtgtataaatatgtaaaataagcaatacacacaggtacatgatatatatgtgtatatatataattcagggtacatttacatacataaagttgcaaaagatcctataagccatgagttacctctaggagattccaaaatgcagtcctcagtaagtgtcatttgtagcacacaaccattccaagatgaagccgcacagacagaataatcaaaatacaacatgagcaagcacagtttttcaataaggttttctaaaagtttgctacgctgacaaaagatgtaaataatccaaagaaagccaaaagaagtatatttgaaaagtaaacacgaacccagccactgctctttactcagcaaagccagggacgcaacagctcaaatggaaactttcactgtcaagtggtctgaaaatattaagcaagacaagtaaatgacttccatgttatgataattagacctgactgtaaaatctcccatttatattagtagatgtctctgacaattttattgtgagaaatgtatggggaaaaaaatgagtcaacatgaatactttcagagttaccaatataaagttaccttaagttaatggtcttagaagagtaccatcaaggtaagcaaggtaaatatttaaataaatataaaattctaagatataaaacttcggtatagaatcagggattactttattaaaagtaactagcatgttgccagttttccctatttattaaacaaactgaatagaattcagaacacactactgagcaaaatgtatatttaaaaaaaagtcaactagaagtaataattctatttgtacacagcataaatcaatatacagtattgtatgtgaatgagactgattggctttaaaatgaattttctgcttcaaggccaatatctctacaaacgttctgtagaagtattgttagggcaggccaacttctttatgatgtcgcattatgtgctggttcttttctgaaggtcttcggaagcctttcttgcagtactcacaccggtgaggatagtctttcgtgtgaatggaaataacgtgccgtttaaagcctgaggcatctgtagtgctatactcacagtactcacactgatacactttcctgccactgtgtgtcttcatatgctttttaagctcactctgttgcctaaatccctttctacatctcttgcacctaaatggaagatcctttgtgtgaactgagagaatatggcgacttagaacaaatggatctgcaatcttaaagtcacaatgtctacactggtgcatttttttgcccttgtgggcagccacgtgtttcttgagttctgaaggcctgtgaaagcctttatcacacatgtcacacttatgggggtagtctttcgtgtgaactgaaattatgtgtcgtttcaaatcacttgagttcgaactcttgtggtcgcaatgcaaacactggtgtgttttgctttcttggtggataagagcatgttgctgcacctctttggtatccgagaaagtcagaagacaaatgtcacacttgaatggcatctctttactatgcttagttttgacatgcgttttcaagttagaagagtctgcagacctatattcgcagtactggcattggtacggcttctccccagtatggattctcatgtgctttttgagctctgacgggtgacgaaaacccttaccacactccacacaaatatgaggaaagttcttgctgtggactgccaagaggtggcgattcaataacccttgttcagctgtctcgtattcacagaatttacacttgtgcattttgttggctcctttttccttatgcaccattttgtgagtaaacaaagcccctgcatgagagaaatgcttcccacactcatcgcattcaatggccttctctgccttgctggtcagcttgtggctctccaggtggttgtgtaaacttatcttcttgttggtagtgtaatcacagtcagtacagcggtatttcttcttggcaaggtgttcgggatggtttttcatgtgccttttcaaaaaacctctcgacttaaacttcttcccacaaatcatgcaaggatagacagtcaaaggatgtccatcagggccaataattattgctgtttggtactgcctggaatcaggtcttctccttttctttggtttttgtttagccagtctgccgaggccagcagactcatctatgtgcaagagggcacttgcagtgccattccggttttcaattccatcagaattattaccataagctgctgcccatgcaatcggcatgaaggttttgatttcattgtcatccatttgctgctcgtgcacggcggcggctgccgctgctgctgcagcatcctcctctcctacgatcacttccatataaacttcgtcagcgatttcagcaacatttaaatcttcatcttctggctgagagtcattgacagtcatataaaccatcttttccctgggaacacgaatactgctgttctgatcaagcagttcaactccatgatcattctcaggctcactctccacaatgtctacagttccacctaagtcatcttctccagggtcagctttaaaaatgtacaccttgatgacctcagggcaagtgccatccactttacaaggatcaatttccgactctgtgtccatggtcattccagaagaaccatcgtgttctattttgccagcatcatccaaggaaatcataaggtagtcctcacagttgcctttgtcatcatcctgctggtccacagggatcccattggcatctatgactgcttcagaggcacagtctgctaccaatacttcttctgaaactacgtcggtagtcagaggatcagtgacaatttctgcttccactacactatcatgaaccacatgttcaacatgtccaacatgtccaacatgtccaacgtcagacacatgtatagaatcacccgtcaagacgtgttctggcatagacattgaggctgaagtaatgtcagaagctaaaacatcatctgggactgtgcaatgtgctaaagaaacttcttcagttacatctgagtccagcacttgctcaggaatgatgaccgtttcagacacatctgcttcttccatgatatctgggcactgaacatcttctataacaacgtcctcaataacatcttggattacaactgaatctgggtcatcaggaacaaagttatgcacagttatgtctgaatccacaacatctgaaacaaaaacagtttcttgtacttccacaacaatttgatcaccatccatgtgtgtaccatcagctcctgtagccccagttactcgggaagctgagcagatcacttgagcctgggaggcggaggttgcagtggacccagatggcgccactgtgctccagcctgggtgacagaacgagaccctgtctgttgcatcaaaaaatgagtttggctcttgttgtaattcaagcccatcttcatccatggcctttaattctcatcagtcacagctcctgtcttaatcacacaacttgactctaatcttaatcttgaacatccactgttgctgtactgcgcagcaaaacaattctatcttcttaatagttcttctatgtctttcccagtgtttactgaagaagcttcacccttgaaacgtcctttctccacctccacctctacctaacaaagtcctacccatccctcggtaaccttctcaaaatgccacctattaatacttcaggaacccgtccctccctgatcctccaatggcaaccttgcttccctcggaaatcccagtaattagttgtacctctcactttactgcatttcaccttgccccacctacctctaaacatgagacttcttgcagccaccgtctgcattacaagaacctttttaatgtttcttagcatctagcacggtgcatcgctaacagtaggctccgagtttatcaagaaagttgcacagtgtgcaatcaaaaaagtacgttaggggatgaaactccgccttaaaacttcacaaatgaaaaatcgaaataccatgacaggcaaatgcacaataaatatgcaccacactaagttgtcctccaataagaaaataaaaaagtctgcccttattcctcgatttaaaaaaataccaccaacagatcactacttaaatcgtttttcaagaaagttgtttccacataaatgagtacgaatgattcaaaattttattcctccgctctcgtgttgtgcaatttttttccctataggacaaaagaatggcaaaaactttcccatcaatctttatttttcttcctttattcagatactcggggcggcaaagattgttggaaaaacaactgcatcgaaagcaccttagcagccacatatgatttgacttaagcaaaaataacatttcctggggtcccgtatgccctggtaagcccaggtgtccggaatgccacctgccccgactgccctcgggtggctacaggcgcgggggaaggcgcagggccaggggcgctgagggtgaaacggtcccggcgtccgggcggcggcggtggccgcctgc

SEQ ID NO: 18216 - RNA, 4378 nt, Homo sapiens
  source 1..4378: mol_type = other RNA
tgaagtaccagctactcgagaggctgaggcagataattgcttgaacccaggaagcagaggttgcagtgagctgcagaggttgcagtgatcacaccactgcagtccagcctgggcaacagagcaagactccgtcttaagaaaaaaaaacaacaaaaaaaaacaaacaaacaaaaaacctgtggaagacttagtgatgttccaaataaggcctcagactttccttatccacttaaaacacatctttaccttttaatcaaagccaacttgagtgttaagtttttaaagtttgctaactgtaactgagaaataacagatcagcctgaacttgccgagtgtgaagtcataattagcacccgttctctggtccacagagccatcacttcttttccatccccctcactaggtaagacagagttccctctcaggcttctcaaagagaactgtgggagtcatgtctggatactcatttgcttttcagaaaaacataaagacatggaggtgaaattgtatgaaaacattctacctagaaacatcttaacctctatgtttcaattaccaaagatatttaaaagaaaatatctttactctttaaaaatactagtgtccttattttccttctaattcttcacctgagtagtctctctgaagagcatgacttacaaaatgctctctcatgcatccctggatctttcatgttattgtaaatttaatacttttcattatagattttaaacaactactacttggggttgtgtgtataaatatgtaaaataagcaatacacacaggtacatgatatatatgtgtatatatataattcagggtacatttacatacataaagttgcaaaagatcctataagccatgagttacctctaggagattccaaaatgcagtcctcagtaagtgtcatttgtagcacacaaccattccaagatgaagccgcacagacagaataatcaaaatacaacatgagcaagcacagtttttcaataaggttttctaaaagtttgctacgctgacaaaagatgtaaataatccaaagaaagccaaaagaagtatatttgaaaagtaaacacgaacccagccactgctctttactcagcaaagccagggacgcaacagctcaaatggaaactttcactgtcaagtggtctgaaaatattaagcaagacaagtaaatgacttccatgttatgataattagacctgactgtaaaatctcccatttatattagtagatgtctctgacaattttattgtgagaaatgtatggggaaaaaaatgagtcaacatgaatactttcagagttaccaatataaagttaccttaagttaatggtcttagaagagtaccatcaaggtaagcaaggtaaatatttaaataaatataaaattctaagatataaaacttcggtatagaatcagggattactttattaaaagtaactagcatgttgccagttttccctatttattaaacaaactgaatagaattcagaacacactactgagcaaaatgtatatttaaaaaaaagtcaactagaagtaataattctatttgtacacagcataaatcaatatacagtattgtatgtgaatgagactgattggctttaaaatgaattttctgcttcaaggccaatatctctacaaacgttctgtagaagtattgttagggcaggccaacttctttatgatgtcgcattatgtgctggttcttttctgaaggtcttcggaagcctttcttgcagtactcacaccggtgaggatagtctttcgtgtgaatggaaataacgtgccgtttaaagcctgaggcatctgtagtgctatactcacagtactcacactgatacactttcctgccactgtgtgtcttcatatgctttttaagctcactctgttgcctaaatccctttctacatctcttgcacctaaatggaagatcctttgtgtgaactgagagaatatggcgacttagaacaaatggatctgcaatcttaaagtcacaatgtctacactggtgcatttttttgcccttgtgggcagccacgtgtttcttgagttctgaaggcctgtgaaagcctttatcacacatgtcacacttatgggggtagtctttcgtgtgaactgaaattatgtgtcgtttcaaatcacttgagttcgaactcttgtggtcgcaatgcaaacactggtgtgttttgctttcttggtggataagagcatgttgctgcacctctttggtatccgagaaagtcagaagacaaatgtcacacttgaatggcatctctttactatgcttagttttgacatgcgttttcaagttagaagagtctgcagacctatattcgcagtactggcattggtacggcttctccccagtatggattctcatgtgctttttgagctctgacgggtgacgaaaacccttaccacactccacacaaatatgaggaaagttcttgctgtggactgccaagaggtggcgattcaataacccttgttcagctgtctcgtattcacagaatttacacttgtgcattttgttggctcctttttccttatgcaccattttgtgagtaaacaaagcccctgcatgagagaaatgcttcccacactcatcgcattcaatggccttctctgccttgctggtcagcttgtggctctccaggtggttgtgtaaacttatcttcttgttggtagtgtaatcacagtcagtacagcggtatttcttcttggcaaggtgttcgggatggtttttcatgtgccttttcaaaaaacctctcgacttaaacttcttcccacaaatcatgcaaggatagacagtcaaaggatgtccatcagggccaataattattgctgtttggtactgcctggaatcaggtcttctccttttctttggtttttgtttagccagtctgccgaggccagcagactcatctatgtgcaagagggcacttgcagtgccattccggttttcaattccatcagaattattaccataagctgctgcccatgcaatcggcatgaaggttttgatttcattgtcatccatttgctgctcgtgcacggcggcggctgccgctgctgctgcagcatcctcctctcctacgatcacttccatataaacttcgtcagcgatttcagcaacatttaaatcttcatcttctggctgagagtcattgacagtcatataaaccatcttttccctgggaacacgaatactgctgttctgatcaagcagttcaactccatgatcattctcaggctcactctccacaatgtctacagttccacctaagtcatcttctccagggtcagctttaaaaatgtacaccttgatgacctcagggcaagtgccatccactttacaaggatcaatttccgactctgtgtccatggtcattccagaagaaccatcgtgttctattttgccagcatcatccaaggaaatcataaggtagtcctcacagttgcctttgtcatcatcctgctggtccacagggatcccattggcatctatgactgcttcagaggcacagtctgctaccaatacttcttctgaaactacgtcggtagtcagaggatcagtgacaatttctgcttccactacactatcatgaaccacatgttcaacatgtccaacatgtccaacatgtccaacgtcagacacatgtatagaatcacccgtcaagacgtgttctggcatagacattgaggctgaagtaatgtcagaagctaaaacatcatctgggactgtgcaatgtgctaaagaaacttcttcagttacatctgagtccagcacttgctcaggaatgatgaccgtttcagacacatctgcttcttccatgatatctgggcactgaacatcttctataacaacgtcctcaataacatcttggattacaactgaatctgggtcatcaggaacaaagttatgcacagttatgtctgaatccacaacatctgaaacaaaaacagtttcttgtacttccacaacaatttgatcaccatccatgtgtgtaccatcagctcctgttgcatcaaaaaatgagtttggctcttgttgtaattcaagcccatcttcatccatggcctttaattctcatcagtcacagctccgcctctcgcgccggtcctggccgaggctccagctcgagttgtttgcaggccctcagacccccgcccgcagtaaatgtgttttcttcatccccgtggctggggaggaagataaatttagcaacccccgccgtcccctgccttcgcttaaaaaaaaaaaatctttgaaataaaatgaaaacgggcttgccagtctaaatgggtgtgcgggaaggggggtggagtggggggagaagggttatccctagagcacctaccaggc

SEQ ID NO: 18217 - RNA, 4184 nt, Homo sapiens
  source 1..4184: mol_type = other RNA
tgaagtaccagctactcgagaggctgaggcagataattgcttgaacccaggaagcagaggttgcagtgagctgcagaggttgcagtgatcacaccactgcagtccagcctgggcaacagagcaagactccgtcttaagaaaaaaaaacaacaaaaaaaaacaaacaaacaaaaaacctgtggaagacttagtgatgttccaaataaggcctcagactttccttatccacttaaaacacatctttaccttttaatcaaagccaacttgagtgttaagtttttaaagtttgctaactgtaactgagaaataacagatcagcctgaacttgccgagtgtgaagtcataattagcacccgttctctggtccacagagccatcacttcttttccatccccctcactaggtaagacagagttccctctcaggcttctcaaagagaactgtgggagtcatgtctggatactcatttgcttttcagaaaaacataaagacatggaggtgaaattgtatgaaaacattctacctagaaacatcttaacctctatgtttcaattaccaaagatatttaaaagaaaatatctttactctttaaaaatactagtgtccttattttccttctaattcttcacctgagtagtctctctgaagagcatgacttacaaaatgctctctcatgcatccctggatctttcatgttattgtaaatttaatacttttcattatagattttaaacaactactacttggggttgtgtgtataaatatgtaaaataagcaatacacacaggtacatgatatatatgtgtatatatataattcagggtacatttacatacataaagttgcaaaagatcctataagccatgagttacctctaggagattccaaaatgcagtcctcagtaagtgtcatttgtagcacacaaccattccaagatgaagccgcacagacagaataatcaaaatacaacatgagcaagcacagtttttcaataaggttttctaaaagtttgctacgctgacaaaagatgtaaataatccaaagaaagccaaaagaagtatatttgaaaagtaaacacgaacccagccactgctctttactcagcaaagccagggacgcaacagctcaaatggaaactttcactgtcaagtggtctgaaaatattaagcaagacaagtaaatgacttccatgttatgataattagacctgactgtaaaatctcccatttatattagtagatgtctctgacaattttattgtgagaaatgtatggggaaaaaaatgagtcaacatgaatactttcagagttaccaatataaagttaccttaagttaatggtcttagaagagtaccatcaaggtaagcaaggtaaatatttaaataaatataaaattctaagatataaaacttcggtatagaatcagggattactttattaaaagtaactagcatgttgccagttttccctatttattaaacaaactgaatagaattcagaacacactactgagcaaaatgtatatttaaaaaaaagtcaactagaagtaataattctatttgtacacagcataaatcaatatacagtattgtatgtgaatgagactgattggctttaaaatgaattttctgcttcaaggccaatatctctacaaacgttctgtagaagtattgttagggcaggccaacttctttatgatgtcgcattatgtgctggttcttttctgaaggtcttcggaagcctttcttgcagtactcacaccggtgaggatagtctttcgtgtgaatggaaataacgtgccgtttaaagcctgaggcatctgtagtgctatactcacagtactcacactgatacactttcctgccactgtgtgtcttcatatgctttttaagctcactctgttgcctaaatccctttctacatctcttgcacctaaatggaagatcctttgtgtgaactgagagaatatggcgacttagaacaaatggatctgcaatcttaaagtcacaatgtctacactggtgcatttttttgcccttgtgggcagccacgtgtttcttgagttctgaaggcctgtgaaagcctttatcacacatgtcacacttatgggggtagtctttcgtgtgaactgaaattatgtgtcgtttcaaatcacttgagttcgaactcttgtggtcgcaatgcaaacactggtgtgttttgctttcttggtggataagagcatgttgctgcacctctttggtatccgagaaagtcagaagacaaatgtcacacttgaatggcatctctttactatgcttagttttgacatgcgttttcaagttagaagagtctgcagacctatattcgcagtactggcattggtacggcttctccccagtatggattctcatgtgctttttgagctctgacgggtgacgaaaacccttaccacactccacacaaatatgaggaaagttcttgctgtggactgccaagaggtggcgattcaataacccttgttcagctgtctcgtattcacagaatttacacttgtgcattttgttggctcctttttccttatgcaccattttgtgagtaaacaaagcccctgcatgagagaaatgcttcccacactcatcgcattcaatggccttctctgccttgctggtcagcttgtggctctccaggtggttgtgtaaacttatcttcttgttggtagtgtaatcacagtcagtacagcggtatttcttcttggcaaggtgttcgggatggtttttcatgtgccttttcaaaaaacctctcgacttaaacttcttcccacaaatcatgcaaggatagacagtcaaaggatgtccatcagggccaataattattgctgtttggtactgcctggaatcaggtcttctccttttctttggtttttgtttagccagtctgccgaggccagcagactcatctatgtgcaagagggcacttgcagtgccattccggttttcaattccatcagaattattaccataagctgctgcccatgcaatcggcatgaaggttttgatttcattgtcatccatttgctgctcgtgcacggcggcggctgccgctgctgctgcagcatcctcctctcctacgatcacttccatataaacttcgtcagcgatttcagcaacatttaaatcttcatcttctggctgagagtcattgacagtcatataaaccatcttttccctgggaacacgaatactgctgttctgatcaagcagttcaactccatgatcattctcaggctcactctccacaatgtctacagttccacctaagtcatcttctccagggtcagctttaaaaatgtacaccttgatgacctcagggcaagtgccatccactttacaaggatcaatttccgactctgtgtccatggtcattccagaagaaccatcgtgttctattttgccagcatcatccaaggaaatcataaggtagtcctcacagttgcctttgtcatcatcctgctggtccacagggatcccattggcatctatgactgcttcagaggcacagtctgctaccaatacttcttctgaaactacgtcggtagtcagaggatcagtgacaatttctgcttccactacactatcatgaaccacatgttcaacatgtccaacatgtccaacatgtccaacgtcagacacatgtatagaatcacccgtcaagacgtgttctggcatagacattgaggctgaagtaatgtcagaagctaaaacatcatctgggactgtgcaatgtgctaaagaaacttcttcagttacatctgagtccagcacttgctcaggaatgatgaccgtttcagacacatctgcttcttccatgatatctgggcactgaacatcttctataacaacgtcctcaataacatcttggattacaactgaatctgggtcatcaggaacaaagttatgcacagttatgtctgaatccacaacatctgaaacaaaaacagtttcttgtacttccacaacaatttgatcaccatccatgtgtgtaccatcagctcctgttgcatcaaaaaatgagtttggctcttgttgtaattcaagcccatcttcatccatggcctttaattctcatcagtcacagctccggacggacgtgcgggcggccggcgacggtggcgggtgctgcaggccggcctttctctggagcact

SEQ ID NO: 18218 - RNA, 4132 nt, Homo sapiens
  source 1..4132: mol_type = other RNA
tgaagtaccagctactcgagaggctgaggcagataattgcttgaacccaggaagcagaggttgcagtgagctgcagaggttgcagtgatcacaccactgcagtccagcctgggcaacagagcaagactccgtcttaagaaaaaaaaacaacaaaaaaaaacaaacaaacaaaaaacctgtggaagacttagtgatgttccaaataaggcctcagactttccttatccacttaaaacacatctttaccttttaatcaaagccaacttgagtgttaagtttttaaagtttgctaactgtaactgagaaataacagatcagcctgaacttgccgagtgtgaagtcataattagcacccgttctctggtccacagagccatcacttcttttccatccccctcactaggtaagacagagttccctctcaggcttctcaaagagaactgtgggagtcatgtctggatactcatttgcttttcagaaaaacataaagacatggaggtgaaattgtatgaaaacattctacctagaaacatcttaacctctatgtttcaattaccaaagatatttaaaagaaaatatctttactctttaaaaatactagtgtccttattttccttctaattcttcacctgagtagtctctctgaagagcatgacttacaaaatgctctctcatgcatccctggatctttcatgttattgtaaatttaatacttttcattatagattttaaacaactactacttggggttgtgtgtataaatatgtaaaataagcaatacacacaggtacatgatatatatgtgtatatatataattcagggtacatttacatacataaagttgcaaaagatcctataagccatgagttacctctaggagattccaaaatgcagtcctcagtaagtgtcatttgtagcacacaaccattccaagatgaagccgcacagacagaataatcaaaatacaacatgagcaagcacagtttttcaataaggttttctaaaagtttgctacgctgacaaaagatgtaaataatccaaagaaagccaaaagaagtatatttgaaaagtaaacacgaacccagccactgctctttactcagcaaagccagggacgcaacagctcaaatggaaactttcactgtcaagtggtctgaaaatattaagcaagacaagtaaatgacttccatgttatgataattagacctgactgtaaaatctcccatttatattagtagatgtctctgacaattttattgtgagaaatgtatggggaaaaaaatgagtcaacatgaatactttcagagttaccaatataaagttaccttaagttaatggtcttagaagagtaccatcaaggtaagcaaggtaaatatttaaataaatataaaattctaagatataaaacttcggtatagaatcagggattactttattaaaagtaactagcatgttgccagttttccctatttattaaacaaactgaatagaattcagaacacactactgagcaaaatgtatatttaaaaaaaagtcaactagaagtaataattctatttgtacacagcataaatcaatatacagtattgtatgtgaatgagactgattggctttaaaatgaattttctgcttcaaggccaatatctctacaaacgttctgtagaagtattgttagggcaggccaacttctttatgatgtcgcattatgtgctggttcttttctgaaggtcttcggaagcctttcttgcagtactcacaccggtgaggatagtctttcgtgtgaatggaaataacgtgccgtttaaagcctgaggcatctgtagtgctatactcacagtactcacactgatacactttcctgccactgtgtgtcttcatatgctttttaagctcactctgttgcctaaatccctttctacatctcttgcacctaaatggaagatcctttgtgtgaactgagagaatatggcgacttagaacaaatggatctgcaatcttaaagtcacaatgtctacactggtgcatttttttgcccttgtgggcagccacgtgtttcttgagttctgaaggcctgtgaaagcctttatcacacatgtcacacttatgggggtagtctttcgtgtgaactgaaattatgtgtcgtttcaaatcacttgagttcgaactcttgtggtcgcaatgcaaacactggtgtgttttgctttcttggtggataagagcatgttgctgcacctctttggtatccgagaaagtcagaagacaaatgtcacacttgaatggcatctctttactatgcttagttttgacatgcgttttcaagttagaagagtctgcagacctatattcgcagtactggcattggtacggcttctccccagtatggattctcatgtgctttttgagctctgacgggtgacgaaaacccttaccacactccacacaaatatgaggaaagttcttgctgtggactgccaagaggtggcgattcaataacccttgttcagctgtctcgtattcacagaatttacacttgtgcattttgttggctcctttttccttatgcaccattttgtgagtaaacaaagcccctgcatgagagaaatgcttcccacactcatcgcattcaatggccttctctgccttgctggtcagcttgtggctctccaggtggttgtgtaaacttatcttcttgttggtagtgtaatcacagtcagtacagcggtatttcttcttggcaaggtgttcgggatggtttttcatgtgccttttcaaaaaacctctcgacttaaacttcttcccacaaatcatgcaaggatagacagtcaaaggatgtccatcagggccaataattattgctgtttggtactgcctggaatcaggtcttctccttttctttggtttttgtttagccagtctgccgaggccagcagactcatctatgtgcaagagggcacttgcagtgccattccggttttcaattccatcagaattattaccataagctgctgcccatgcaatcggcatgaaggttttgatttcattgtcatccatttgctgctcgtgcacggcggcggctgccgctgctgctgcagcatcctcctctcctacgatcacttccatataaacttcgtcagcgatttcagcaacatttaaatcttcatcttctggctgagagtcattgacagtcatataaaccatcttttccctgggaacacgaatactgctgttctgatcaagcagttcaactccatgatcattctcaggctcactctccacaatgtctacagttccacctaagtcatcttctccagggtcagctttaaaaatgtacaccttgatgacctcagggcaagtgccatccactttacaaggatcaatttccgactctgtgtccatggtcattccagaagaaccatcgtgttctattttgccagcatcatccaaggaaatcataaggtagtcctcacagttgcctttgtcatcatcctgctggtccacagggatcccattggcatctatgactgcttcagaggcacagtctgctaccaatacttcttctgaaactacgtcggtagtcagaggatcagtgacaatttctgcttccactacactatcatgaaccacatgttcaacatgtccaacatgtccaacatgtccaacgtcagacacatgtatagaatcacccgtcaagacgtgttctggcatagacattgaggctgaagtaatgtcagaagctaaaacatcatctgggactgtgcaatgtgctaaagaaacttcttcagttacatctgagtccagcacttgctcaggaatgatgaccgtttcagacacatctgcttcttccatgatatctgggcactgaacatcttctataacaacgtcctcaataacatcttggattacaactgaatctgggtcatcaggaacaaagttatgcacagttatgtctgaatccacaacatctgaaacaaaaacagtttcttgtacttccacaacaatttgatcaccatccatgtgtgtaccatcagctcctgttgcatcaaaaaatgagtttggctcttgttgtaattcaagcccatcttcatccatggcctttaattctcatcagtcacagctcctgtaatcccagca

SEQ ID NO: 18219 - RNA, 4533 nt, Homo sapiens
  source 1..4533: mol_type = other RNA
tgaagtaccagctactcgagaggctgaggcagataattgcttgaacccaggaagcagaggttgcagtgagctgcagaggttgcagtgatcacaccactgcagtccagcctgggcaacagagcaagactccgtcttaagaaaaaaaaacaacaaaaaaaaacaaacaaacaaaaaacctgtggaagacttagtgatgttccaaataaggcctcagactttccttatccacttaaaacacatctttaccttttaatcaaagccaacttgagtgttaagtttttaaagtttgctaactgtaactgagaaataacagatcagcctgaacttgccgagtgtgaagtcataattagcacccgttctctggtccacagagccatcacttcttttccatccccctcactaggtaagacagagttccctctcaggcttctcaaagagaactgtgggagtcatgtctggatactcatttgcttttcagaaaaacataaagacatggaggtgaaattgtatgaaaacattctacctagaaacatcttaacctctatgtttcaattaccaaagatatttaaaagaaaatatctttactctttaaaaatactagtgtccttattttccttctaattcttcacctgagtagtctctctgaagagcatgacttacaaaatgctctctcatgcatccctggatctttcatgttattgtaaatttaatacttttcattatagattttaaacaactactacttggggttgtgtgtataaatatgtaaaataagcaatacacacaggtacatgatatatatgtgtatatatataattcagggtacatttacatacataaagttgcaaaagatcctataagccatgagttacctctaggagattccaaaatgcagtcctcagtaagtgtcatttgtagcacacaaccattccaagatgaagccgcacagacagaataatcaaaatacaacatgagcaagcacagtttttcaataaggttttctaaaagtttgctacgctgacaaaagatgtaaataatccaaagaaagccaaaagaagtatatttgaaaagtaaacacgaacccagccactgctctttactcagcaaagccagggacgcaacagctcaaatggaaactttcactgtcaagtggtctgaaaatattaagcaagacaagtaaatgacttccatgttatgataattagacctgactgtaaaatctcccatttatattagtagatgtctctgacaattttattgtgagaaatgtatggggaaaaaaatgagtcaacatgaatactttcagagttaccaatataaagttaccttaagttaatggtcttagaagagtaccatcaaggtaagcaaggtaaatatttaaataaatataaaattctaagatataaaacttcggtatagaatcagggattactttattaaaagtaactagcatgttgccagttttccctatttattaaacaaactgaatagaattcagaacacactactgagcaaaatgtatatttaaaaaaaagtcaactagaagtaataattctatttgtacacagcataaatcaatatacagtattgtatgtgaatgagactgattggctttaaaatgaattttctgcttcaaggccaatatctctacaaacgttctgtagaagtattgttagggcaggccaacttctttatgatgtcgcattatgtgctggttcttttctgaaggtcttcggaagcctttcttgcagtactcacaccggtgaggatagtctttcgtgtgaatggaaataacgtgccgtttaaagcctgaggcatctgtagtgctatactcacagtactcacactgatacactttcctgccactgtgtgtcttcatatgctttttaagctcactctgttgcctaaatccctttctacatctcttgcacctaaatggaagatcctttgtgtgaactgagagaatatggcgacttagaacaaatggatctgcaatcttaaagtcacaatgtctacactggtgcatttttttgcccttgtgggcagccacgtgtttcttgagttctgaaggcctgtgaaagcctttatcacacatgtcacacttatgggggtagtctttcgtgtgaactgaaattatgtgtcgtttcaaatcacttgagttcgaactcttgtggtcgcaatgcaaacactggtgtgttttgctttcttggtggataagagcatgttgctgcacctctttggtatccgagaaagtcagaagacaaatgtcacacttgaatggcatctctttactatgcttagttttgacatgcgttttcaagttagaagagtctgcagacctatattcgcagtactggcattggtacggcttctccccagtatggattctcatgtgctttttgagctctgacgggtgacgaaaacccttaccacactccacacaaatatgaggaaagttcttgctgtggactgccaagaggtggcgattcaataacccttgttcagctgtctcgtattcacagaatttacacttgtgcattttgttggctcctttttccttatgcaccattttgtgagtaaacaaagcccctgcatgagagaaatgcttcccacactcatcgcattcaatggccttctctgccttgctggtcagcttgtggctctccaggtggttgtgtaaacttatcttcttgttggtagtgtaatcacagtcagtacagcggtatttcttcttggcaaggtgttcgggatggtttttcatgtgccttttcaaaaaacctctcgacttaaacttcttcccacaaatcatgcaaggatagacagtcaaaggatgtccatcagggccaataattattgctgtttggtactgcctggaatcaggtcttctccttttctttggtttttgtttagccagtctgccgaggccagcagactcatctatgtgcaagagggcacttgcagtgccattccggttttcaattccatcagaattattaccataagctgctgcccatgcaatcggcatgaaggttttgatttcattgtcatccatttgctgctcgtgcacggcggcggctgccgctgctgctgcagcatcctcctctcctacgatcacttccatataaacttcgtcagcgatttcagcaacatttaaatcttcatcttctggctgagagtcattgacagtcatataaaccatcttttccctgggaacacgaatactgctgttctgatcaagcagttcaactccatgatcattctcaggctcactctccacaatgtctacagttccacctaagtcatcttctccagggtcagctttaaaaatgtacaccttgatgacctcagggcaagtgccatccactttacaaggatcaatttccgactctgtgtccatggtcattccagaagaaccatcgtgttctattttgccagcatcatccaaggaaatcataaggtagtcctcacagttgcctttgtcatcatcctgctggtccacagggatcccattggcatctatgactgcttcagaggcacagtctgctaccaatacttcttctgaaactacgtcggtagtcagaggatcagtgacaatttctgcttccactacactatcatgaaccacatgttcaacatgtccaacatgtccaacatgtccaacgtcagacacatgtatagaatcacccgtcaagacgtgttctggcatagacattgaggctgaagtaatgtcagaagctaaaacatcatctgggactgtgcaatgtgctaaagaaacttcttcagttacatctgagtccagcacttgctcaggaatgatgaccgtttcagacacatctgcttcttccatgatatctgggcactgaacatcttctataacaacgtcctcaataacatcttggattacaactgaatctgggtcatcaggaacaaagttatgcacagttatgtctgaatccacaacatctgaaacaaaaacagtttcttgtacttccacaacaatttgatcaccatccatgtgtgtaccatcagctcctgttgcatcaaaaaatgagtttggctcttgttgtaattcaagcccatcttcatccatggcctttaattctcatcagtcacagctcctgtaatcccagctactcgagaggctgaggcagaagaagaatcacttgaacacagaaggcagaggctgcagtgagccaaatttgcaccactgcactgcattccagcctggatgacagaggaagactgtctgtcttaatcacacaacttgactctaatcttaatcttgaacatccactgttgctgtactgcgcagcaaaacaattctatcttcttaatagttcttctatgtctttcccagcgtaaagcacagctcagggaacagacggcagtgacaggcgggcagtgggaggcgggagaacggcttgagcccaggagttcgagaccagcctggggcaatatagcaagaaccggacggacgtgcgggcggccggcgacggtggcgggtgctgcaggccggcctttctctggagcact

SEQ ID NO: 18220 - RNA, 4563 nt, Homo sapiens
  source 1..4563: mol_type = other RNA
tgaagtaccagctactcgagaggctgaggcagataattgcttgaacccaggaagcagaggttgcagtgagctgcagaggttgcagtgatcacaccactgcagtccagcctgggcaacagagcaagactccgtcttaagaaaaaaaaacaacaaaaaaaaacaaacaaacaaaaaacctgtggaagacttagtgatgttccaaataaggcctcagactttccttatccacttaaaacacatctttaccttttaatcaaagccaacttgagtgttaagtttttaaagtttgctaactgtaactgagaaataacagatcagcctgaacttgccgagtgtgaagtcataattagcacccgttctctggtccacagagccatcacttcttttccatccccctcactaggtaagacagagttccctctcaggcttctcaaagagaactgtgggagtcatgtctggatactcatttgcttttcagaaaaacataaagacatggaggtgaaattgtatgaaaacattctacctagaaacatcttaacctctatgtttcaattaccaaagatatttaaaagaaaatatctttactctttaaaaatactagtgtccttattttccttctaattcttcacctgagtagtctctctgaagagcatgacttacaaaatgctctctcatgcatccctggatctttcatgttattgtaaatttaatacttttcattatagattttaaacaactactacttggggttgtgtgtataaatatgtaaaataagcaatacacacaggtacatgatatatatgtgtatatatataattcagggtacatttacatacataaagttgcaaaagatcctataagccatgagttacctctaggagattccaaaatgcagtcctcagtaagtgtcatttgtagcacacaaccattccaagatgaagccgcacagacagaataatcaaaatacaacatgagcaagcacagtttttcaataaggttttctaaaagtttgctacgctgacaaaagatgtaaataatccaaagaaagccaaaagaagtatatttgaaaagtaaacacgaacccagccactgctctttactcagcaaagccagggacgcaacagctcaaatggaaactttcactgtcaagtggtctgaaaatattaagcaagacaagtaaatgacttccatgttatgataattagacctgactgtaaaatctcccatttatattagtagatgtctctgacaattttattgtgagaaatgtatggggaaaaaaatgagtcaacatgaatactttcagagttaccaatataaagttaccttaagttaatggtcttagaagagtaccatcaaggtaagcaaggtaaatatttaaataaatataaaattctaagatataaaacttcggtatagaatcagggattactttattaaaagtaactagcatgttgccagttttccctatttattaaacaaactgaatagaattcagaacacactactgagcaaaatgtatatttaaaaaaaagtcaactagaagtaataattctatttgtacacagcataaatcaatatacagtattgtatgtgaatgagactgattggctttaaaatgaattttctgcttcaaggccaatatctctacaaacgttctgtagaagtattgttagggcaggccaacttctttatgatgtcgcattatgtgctggttcttttctgaaggtcttcggaagcctttcttgcagtactcacaccggtgaggatagtctttcgtgtgaatggaaataacgtgccgtttaaagcctgaggcatctgtagtgctatactcacagtactcacactgatacactttcctgccactgtgtgtcttcatatgctttttaagctcactctgttgcctaaatccctttctacatctcttgcacctaaatggaagatcctttgtgtgaactgagagaatatggcgacttagaacaaatggatctgcaatcttaaagtcacaatgtctacactggtgcatttttttgcccttgtgggcagccacgtgtttcttgagttctgaaggcctgtgaaagcctttatcacacatgtcacacttatgggggtagtctttcgtgtgaactgaaattatgtgtcgtttcaaatcacttgagttcgaactcttgtggtcgcaatgcaaacactggtgtgttttgctttcttggtggataagagcatgttgctgcacctctttggtatccgagaaagtcagaagacaaatgtcacacttgaatggcatctctttactatgcttagttttgacatgcgttttcaagttagaagagtctgcagacctatattcgcagtactggcattggtacggcttctccccagtatggattctcatgtgctttttgagctctgacgggtgacgaaaacccttaccacactccacacaaatatgaggaaagttcttgctgtggactgccaagaggtggcgattcaataacccttgttcagctgtctcgtattcacagaatttacacttgtgcattttgttggctcctttttccttatgcaccattttgtgagtaaacaaagcccctgcatgagagaaatgcttcccacactcatcgcattcaatggccttctctgccttgctggtcagcttgtggctctccaggtggttgtgtaaacttatcttcttgttggtagtgtaatcacagtcagtacagcggtatttcttcttggcaaggtgttcgggatggtttttcatgtgccttttcaaaaaacctctcgacttaaacttcttcccacaaatcatgcaaggatagacagtcaaaggatgtccatcagggccaataattattgctgtttggtactgcctggaatcaggtcttctccttttctttggtttttgtttagccagtctgccgaggccagcagactcatctatgtgcaagagggcacttgcagtgccattccggttttcaattccatcagaattattaccataagctgctgcccatgcaatcggcatgaaggttttgatttcattgtcatccatttgctgctcgtgcacggcggcggctgccgctgctgctgcagcatcctcctctcctacgatcacttccatataaacttcgtcagcgatttcagcaacatttaaatcttcatcttctggctgagagtcattgacagtcatataaaccatcttttccctgggaacacgaatactgctgttctgatcaagcagttcaactccatgatcattctcaggctcactctccacaatgtctacagttccacctaagtcatcttctccagggtcagctttaaaaatgtacaccttgatgacctcagggcaagtgccatccactttacaaggatcaatttccgactctgtgtccatggtcattccagaagaaccatcgtgttctattttgccagcatcatccaaggaaatcataaggtagtcctcacagttgcctttgtcatcatcctgctggtccacagggatcccattggcatctatgactgcttcagaggcacagtctgctaccaatacttcttctgaaactacgtcggtagtcagaggatcagtgacaatttctgcttccactacactatcatgaaccacatgttcaacatgtccaacatgtccaacatgtccaacgtcagacacatgtatagaatcacccgtcaagacgtgttctggcatagacattgaggctgaagtaatgtcagaagctaaaacatcatctgggactgtgcaatgtgctaaagaaacttcttcagttacatctgagtccagcacttgctcaggaatgatgaccgtttcagacacatctgcttcttccatgatatctgggcactgaacatcttctataacaacgtcctcaataacatcttggattacaactgaatctgggtcatcaggaacaaagttatgcacagttatgtctgaatccacaacatctgaaacaaaaacagtttcttgtacttccacaacaatttgatcaccatccatgtgtgtaccatcagctcctgttgcatcaaaaaatgagtttggctcttgttgtaattcaagcccatcttcatccatggcctttaattctcatcagtcacagctcctgtcttaatcacacaacttgactctaatcttaatcttgaacatccactgttgctgtactgcgcagcaaaacaattctatcttcttaatagttcttctatgtctttcccagcggacggacgtgcgggcggccggcgacggtggcgggtgctgcaggccggcctttctctggagcactgggccgggctccggctggtggggcgggcggagggagggaggaggggccgagctcggagctgacaaaaagcggcccagctccccggcacgggcccgccgtcagcacgtcacgtcaccgcccgggagagagacccaggaaaatgcggaagggtagacaggccccctcctccgcccggtgggtcctcctggcaccccgtgtcggcgccgctcccgccccgcgaccggggagcccagtggcctcgctgcggcggggtctccggcggccggag

SEQ ID NO: 18221 - RNA, 4503 nt, Homo sapiens
  source 1..4503: mol_type = other RNA
tgaagtaccagctactcgagaggctgaggcagataattgcttgaacccaggaagcagaggttgcagtgagctgcagaggttgcagtgatcacaccactgcagtccagcctgggcaacagagcaagactccgtcttaagaaaaaaaaacaacaaaaaaaaacaaacaaacaaaaaacctgtggaagacttagtgatgttccaaataaggcctcagactttccttatccacttaaaacacatctttaccttttaatcaaagccaacttgagtgttaagtttttaaagtttgctaactgtaactgagaaataacagatcagcctgaacttgccgagtgtgaagtcataattagcacccgttctctggtccacagagccatcacttcttttccatccccctcactaggtaagacagagttccctctcaggcttctcaaagagaactgtgggagtcatgtctggatactcatttgcttttcagaaaaacataaagacatggaggtgaaattgtatgaaaacattctacctagaaacatcttaacctctatgtttcaattaccaaagatatttaaaagaaaatatctttactctttaaaaatactagtgtccttattttccttctaattcttcacctgagtagtctctctgaagagcatgacttacaaaatgctctctcatgcatccctggatctttcatgttattgtaaatttaatacttttcattatagattttaaacaactactacttggggttgtgtgtataaatatgtaaaataagcaatacacacaggtacatgatatatatgtgtatatatataattcagggtacatttacatacataaagttgcaaaagatcctataagccatgagttacctctaggagattccaaaatgcagtcctcagtaagtgtcatttgtagcacacaaccattccaagatgaagccgcacagacagaataatcaaaatacaacatgagcaagcacagtttttcaataaggttttctaaaagtttgctacgctgacaaaagatgtaaataatccaaagaaagccaaaagaagtatatttgaaaagtaaacacgaacccagccactgctctttactcagcaaagccagggacgcaacagctcaaatggaaactttcactgtcaagtggtctgaaaatattaagcaagacaagtaaatgacttccatgttatgataattagacctgactgtaaaatctcccatttatattagtagatgtctctgacaattttattgtgagaaatgtatggggaaaaaaatgagtcaacatgaatactttcagagttaccaatataaagttaccttaagttaatggtcttagaagagtaccatcaaggtaagcaaggtaaatatttaaataaatataaaattctaagatataaaacttcggtatagaatcagggattactttattaaaagtaactagcatgttgccagttttccctatttattaaacaaactgaatagaattcagaacacactactgagcaaaatgtatatttaaaaaaaagtcaactagaagtaataattctatttgtacacagcataaatcaatatacagtattgtatgtgaatgagactgattggctttaaaatgaattttctgcttcaaggccaatatctctacaaacgttctgtagaagtattgttagggcaggccaacttctttatgatgtcgcattatgtgctggttcttttctgaaggtcttcggaagcctttcttgcagtactcacaccggtgaggatagtctttcgtgtgaatggaaataacgtgccgtttaaagcctgaggcatctgtagtgctatactcacagtactcacactgatacactttcctgccactgtgtgtcttcatatgctttttaagctcactctgttgcctaaatccctttctacatctcttgcacctaaatggaagatcctttgtgtgaactgagagaatatggcgacttagaacaaatggatctgcaatcttaaagtcacaatgtctacactggtgcatttttttgcccttgtgggcagccacgtgtttcttgagttctgaaggcctgtgaaagcctttatcacacatgtcacacttatgggggtagtctttcgtgtgaactgaaattatgtgtcgtttcaaatcacttgagttcgaactcttgtggtcgcaatgcaaacactggtgtgttttgctttcttggtggataagagcatgttgctgcacctctttggtatccgagaaagtcagaagacaaatgtcacacttgaatggcatctctttactatgcttagttttgacatgcgttttcaagttagaagagtctgcagacctatattcgcagtactggcattggtacggcttctccccagtatggattctcatgtgctttttgagctctgacgggtgacgaaaacccttaccacactccacacaaatatgaggaaagttcttgctgtggactgccaagaggtggcgattcaataacccttgttcagctgtctcgtattcacagaatttacacttgtgcattttgttggctcctttttccttatgcaccattttgtgagtaaacaaagcccctgcatgagagaaatgcttcccacactcatcgcattcaatggccttctctgccttgctggtcagcttgtggctctccaggtggttgtgtaaacttatcttcttgttggtagtgtaatcacagtcagtacagcggtatttcttcttggcaaggtgttcgggatggtttttcatgtgccttttcaaaaaacctctcgacttaaacttcttcccacaaatcatgcaaggatagacagtcaaaggatgtccatcagggccaataattattgctgtttggtactgcctggaatcaggtcttctccttttctttggtttttgtttagccagtctgccgaggccagcagactcatctatgtgcaagagggcacttgcagtgccattccggttttcaattccatcagaattattaccataagctgctgcccatgcaatcggcatgaaggttttgatttcattgtcatccatttgctgctcgtgcacggcggcggctgccgctgctgctgcagcatcctcctctcctacgatcacttccatataaacttcgtcagcgatttcagcaacatttaaatcttcatcttctggctgagagtcattgacagtcatataaaccatcttttccctgggaacacgaatactgctgttctgatcaagcagttcaactccatgatcattctcaggctcactctccacaatgtctacagttccacctaagtcatcttctccagggtcagctttaaaaatgtacaccttgatgacctcagggcaagtgccatccactttacaaggatcaatttccgactctgtgtccatggtcattccagaagaaccatcgtgttctattttgccagcatcatccaaggaaatcataaggtagtcctcacagttgcctttgtcatcatcctgctggtccacagggatcccattggcatctatgactgcttcagaggcacagtctgctaccaatacttcttctgaaactacgtcggtagtcagaggatcagtgacaatttctgcttccactacactatcatgaaccacatgttcaacatgtccaacatgtccaacatgtccaacgtcagacacatgtatagaatcacccgtcaagacgtgttctggcatagacattgaggctgaagtaatgtcagaagctaaaacatcatctgggactgtgcaatgtgctaaagaaacttcttcagttacatctgagtccagcacttgctcaggaatgatgaccgtttcagacacatctgcttcttccatgatatctgggcactgaacatcttctataacaacgtcctcaataacatcttggattacaactgaatctgggtcatcaggaacaaagttatgcacagttatgtctgaatccacaacatctgaaacaaaaacagtttcttgtacttccacaacaatttgatcaccatccatgtgtgtaccatcagctcctgttgcatcaaaaaatgagtttggctcttgttgtaattcaagcccatcttcatccatggcctttaattctcatcagtcacagctcctgtcttaatcacacaacttgactctaatcttaatcttgaacatccactgttgctgtactgcgcagcaaaacaattctatcttcttaatagttcttctatgtctttcccagcgtaaagcacagctcagggaacagacggcagtgacaggcgggcagtgggaggcgggagaacggcttgagcccaggagttcgagaccagcctggggcaatatagcaagaacatagcgaaaatcggcccggccggcctgcggccttcacctcacgcctgcagccttcgcctcctcgccaggcctcaccccggcgcggtgccccaggtcggccgcggagccgacccggggcccctcgaccgcctccggcacaaccgggcgaccctcccccaaccccc

SEQ ID NO: 18222 - RNA, 4405 nt, Homo sapiens
  source 1..4405: mol_type = other RNA
tgaagtaccagctactcgagaggctgaggcagataattgcttgaacccaggaagcagaggttgcagtgagctgcagaggttgcagtgatcacaccactgcagtccagcctgggcaacagagcaagactccgtcttaagaaaaaaaaacaacaaaaaaaaacaaacaaacaaaaaacctgtggaagacttagtgatgttccaaataaggcctcagactttccttatccacttaaaacacatctttaccttttaatcaaagccaacttgagtgttaagtttttaaagtttgctaactgtaactgagaaataacagatcagcctgaacttgccgagtgtgaagtcataattagcacccgttctctggtccacagagccatcacttcttttccatccccctcactaggtaagacagagttccctctcaggcttctcaaagagaactgtgggagtcatgtctggatactcatttgcttttcagaaaaacataaagacatggaggtgaaattgtatgaaaacattctacctagaaacatcttaacctctatgtttcaattaccaaagatatttaaaagaaaatatctttactctttaaaaatactagtgtccttattttccttctaattcttcacctgagtagtctctctgaagagcatgacttacaaaatgctctctcatgcatccctggatctttcatgttattgtaaatttaatacttttcattatagattttaaacaactactacttggggttgtgtgtataaatatgtaaaataagcaatacacacaggtacatgatatatatgtgtatatatataattcagggtacatttacatacataaagttgcaaaagatcctataagccatgagttacctctaggagattccaaaatgcagtcctcagtaagtgtcatttgtagcacacaaccattccaagatgaagccgcacagacagaataatcaaaatacaacatgagcaagcacagtttttcaataaggttttctaaaagtttgctacgctgacaaaagatgtaaataatccaaagaaagccaaaagaagtatatttgaaaagtaaacacgaacccagccactgctctttactcagcaaagccagggacgcaacagctcaaatggaaactttcactgtcaagtggtctgaaaatattaagcaagacaagtaaatgacttccatgttatgataattagacctgactgtaaaatctcccatttatattagtagatgtctctgacaattttattgtgagaaatgtatggggaaaaaaatgagtcaacatgaatactttcagagttaccaatataaagttaccttaagttaatggtcttagaagagtaccatcaaggtaagcaaggtaaatatttaaataaatataaaattctaagatataaaacttcggtatagaatcagggattactttattaaaagtaactagcatgttgccagttttccctatttattaaacaaactgaatagaattcagaacacactactgagcaaaatgtatatttaaaaaaaagtcaactagaagtaataattctatttgtacacagcataaatcaatatacagtattgtatgtgaatgagactgattggctttaaaatgaattttctgcttcaaggccaatatctctacaaacgttctgtagaagtattgttagggcaggccaacttctttatgatgtcgcattatgtgctggttcttttctgaaggtcttcggaagcctttcttgcagtactcacaccggtgaggatagtctttcgtgtgaatggaaataacgtgccgtttaaagcctgaggcatctgtagtgctatactcacagtactcacactgatacactttcctgccactgtgtgtcttcatatgctttttaagctcactctgttgcctaaatccctttctacatctcttgcacctaaatggaagatcctttgtgtgaactgagagaatatggcgacttagaacaaatggatctgcaatcttaaagtcacaatgtctacactggtgcatttttttgcccttgtgggcagccacgtgtttcttgagttctgaaggcctgtgaaagcctttatcacacatgtcacacttatgggggtagtctttcgtgtgaactgaaattatgtgtcgtttcaaatcacttgagttcgaactcttgtggtcgcaatgcaaacactggtgtgttttgctttcttggtggataagagcatgttgctgcacctctttggtatccgagaaagtcagaagacaaatgtcacacttgaatggcatctctttactatgcttagttttgacatgcgttttcaagttagaagagtctgcagacctatattcgcagtactggcattggtacggcttctccccagtatggattctcatgtgctttttgagctctgacgggtgacgaaaacccttaccacactccacacaaatatgaggaaagttcttgctgtggactgccaagaggtggcgattcaataacccttgttcagctgtctcgtattcacagaatttacacttgtgcattttgttggctcctttttccttatgcaccattttgtgagtaaacaaagcccctgcatgagagaaatgcttcccacactcatcgcattcaatggccttctctgccttgctggtcagcttgtggctctccaggtggttgtgtaaacttatcttcttgttggtagtgtaatcacagtcagtacagcggtatttcttcttggcaaggtgttcgggatggtttttcatgtgccttttcaaaaaacctctcgacttaaacttcttcccacaaatcatgcaaggatagacagtcaaaggatgtccatcagggccaataattattgctgtttggtactgcctggaatcaggtcttctccttttctttggtttttgtttagccagtctgccgaggccagcagactcatctatgtgcaagagggcacttgcagtgccattccggttttcaattccatcagaattattaccataagctgctgcccatgcaatcggcatgaaggttttgatttcattgtcatccatttgctgctcgtgcacggcggcggctgccgctgctgctgcagcatcctcctctcctacgatcacttccatataaacttcgtcagcgatttcagcaacatttaaatcttcatcttctggctgagagtcattgacagtcatataaaccatcttttccctgggaacacgaatactgctgttctgatcaagcagttcaactccatgatcattctcaggctcactctccacaatgtctacagttccacctaagtcatcttctccagggtcagctttaaaaatgtacaccttgatgacctcagggcaagtgccatccactttacaaggatcaatttccgactctgtgtccatggtcattccagaagaaccatcgtgttctattttgccagcatcatccaaggaaatcataaggtagtcctcacagttgcctttgtcatcatcctgctggtccacagggatcccattggcatctatgactgcttcagaggcacagtctgctaccaatacttcttctgaaactacgtcggtagtcagaggatcagtgacaatttctgcttccactacactatcatgaaccacatgttcaacatgtccaacatgtccaacatgtccaacgtcagacacatgtatagaatcacccgtcaagacgtgttctggcatagacattgaggctgaagtaatgtcagaagctaaaacatcatctgggactgtgcaatgtgctaaagaaacttcttcagttacatctgagtccagcacttgctcaggaatgatgaccgtttcagacacatctgcttcttccatgatatctgggcactgaacatcttctataacaacgtcctcaataacatcttggattacaactgaatctgggtcatcaggaacaaagttatgcacagttatgtctgaatccacaacatctgaaacaaaaacagtttcttgtacttccacaacaatttgatcaccatccatgtgtgtaccatcagctcctgttgcatcaaaaaatgagtttggctcttgttgtaattcaagcccatcttcatccatggcctttaattctcatcagtcacagctcctgtcttaatcacacaacttgactctaatcttaatcttgaacatccactgttgctgtactgcgcagcaaaacaattctatcttcttaatagttcttctatgtctttcccagcgtaaagcacagctcagggaacagacggcagtgacaggcgggcagtgggaggcgggagaacggcttgagcccaggagttcgagaccagcctggggcaatatagcaagaaccggacggacgtgcgggcggccggcgacggtggcgggtgctgcaggccggcctttctctggagcact

SEQ ID NO: 18223 - RNA, 4462 nt, Homo sapiens
  source 1..4462: mol_type = other RNA
tgaagtaccagctactcgagaggctgaggcagataattgcttgaacccaggaagcagaggttgcagtgagctgcagaggttgcagtgatcacaccactgcagtccagcctgggcaacagagcaagactccgtcttaagaaaaaaaaacaacaaaaaaaaacaaacaaacaaaaaacctgtggaagacttagtgatgttccaaataaggcctcagactttccttatccacttaaaacacatctttaccttttaatcaaagccaacttgagtgttaagtttttaaagtttgctaactgtaactgagaaataacagatcagcctgaacttgccgagtgtgaagtcataattagcacccgttctctggtccacagagccatcacttcttttccatccccctcactaggtaagacagagttccctctcaggcttctcaaagagaactgtgggagtcatgtctggatactcatttgcttttcagaaaaacataaagacatggaggtgaaattgtatgaaaacattctacctagaaacatcttaacctctatgtttcaattaccaaagatatttaaaagaaaatatctttactctttaaaaatactagtgtccttattttccttctaattcttcacctgagtagtctctctgaagagcatgacttacaaaatgctctctcatgcatccctggatctttcatgttattgtaaatttaatacttttcattatagattttaaacaactactacttggggttgtgtgtataaatatgtaaaataagcaatacacacaggtacatgatatatatgtgtatatatataattcagggtacatttacatacataaagttgcaaaagatcctataagccatgagttacctctaggagattccaaaatgcagtcctcagtaagtgtcatttgtagcacacaaccattccaagatgaagccgcacagacagaataatcaaaatacaacatgagcaagcacagtttttcaataaggttttctaaaagtttgctacgctgacaaaagatgtaaataatccaaagaaagccaaaagaagtatatttgaaaagtaaacacgaacccagccactgctctttactcagcaaagccagggacgcaacagctcaaatggaaactttcactgtcaagtggtctgaaaatattaagcaagacaagtaaatgacttccatgttatgataattagacctgactgtaaaatctcccatttatattagtagatgtctctgacaattttattgtgagaaatgtatggggaaaaaaatgagtcaacatgaatactttcagagttaccaatataaagttaccttaagttaatggtcttagaagagtaccatcaaggtaagcaaggtaaatatttaaataaatataaaattctaagatataaaacttcggtatagaatcagggattactttattaaaagtaactagcatgttgccagttttccctatttattaaacaaactgaatagaattcagaacacactactgagcaaaatgtatatttaaaaaaaagtcaactagaagtaataattctatttgtacacagcataaatcaatatacagtattgtatgtgaatgagactgattggctttaaaatgaattttctgcttcaaggccaatatctctacaaacgttctgtagaagtattgttagggcaggccaacttctttatgatgtcgcattatgtgctggttcttttctgaaggtcttcggaagcctttcttgcagtactcacaccggtgaggatagtctttcgtgtgaatggaaataacgtgccgtttaaagcctgaggcatctgtagtgctatactcacagtactcacactgatacactttcctgccactgtgtgtcttcatatgctttttaagctcactctgttgcctaaatccctttctacatctcttgcacctaaatggaagatcctttgtgtgaactgagagaatatggcgacttagaacaaatggatctgcaatcttaaagtcacaatgtctacactggtgcatttttttgcccttgtgggcagccacgtgtttcttgagttctgaaggcctgtgaaagcctttatcacacatgtcacacttatgggggtagtctttcgtgtgaactgaaattatgtgtcgtttcaaatcacttgagttcgaactcttgtggtcgcaatgcaaacactggtgtgttttgctttcttggtggataagagcatgttgctgcacctctttggtatccgagaaagtcagaagacaaatgtcacacttgaatggcatctctttactatgcttagttttgacatgcgttttcaagttagaagagtctgcagacctatattcgcagtactggcattggtacggcttctccccagtatggattctcatgtgctttttgagctctgacgggtgacgaaaacccttaccacactccacacaaatatgaggaaagttcttgctgtggactgccaagaggtggcgattcaataacccttgttcagctgtctcgtattcacagaatttacacttgtgcattttgttggctcctttttccttatgcaccattttgtgagtaaacaaagcccctgcatgagagaaatgcttcccacactcatcgcattcaatggccttctctgccttgctggtcagcttgtggctctccaggtggttgtgtaaacttatcttcttgttggtagtgtaatcacagtcagtacagcggtatttcttcttggcaaggtgttcgggatggtttttcatgtgccttttcaaaaaacctctcgacttaaacttcttcccacaaatcatgcaaggatagacagtcaaaggatgtccatcagggccaataattattgctgtttggtactgcctggaatcaggtcttctccttttctttggtttttgtttagccagtctgccgaggccagcagactcatctatgtgcaagagggcacttgcagtgccattccggttttcaattccatcagaattattaccataagctgctgcccatgcaatcggcatgaaggttttgatttcattgtcatccatttgctgctcgtgcacggcggcggctgccgctgctgctgcagcatcctcctctcctacgatcacttccatataaacttcgtcagcgatttcagcaacatttaaatcttcatcttctggctgagagtcattgacagtcatataaaccatcttttccctgggaacacgaatactgctgttctgatcaagcagttcaactccatgatcattctcaggctcactctccacaatgtctacagttccacctaagtcatcttctccagggtcagctttaaaaatgtacaccttgatgacctcagggcaagtgccatccactttacaaggatcaatttccgactctgtgtccatggtcattccagaagaaccatcgtgttctattttgccagcatcatccaaggaaatcataaggtagtcctcacagttgcctttgtcatcatcctgctggtccacagggatcccattggcatctatgactgcttcagaggcacagtctgctaccaatacttcttctgaaactacgtcggtagtcagaggatcagtgacaatttctgcttccactacactatcatgaaccacatgttcaacatgtccaacatgtccaacatgtccaacgtcagacacatgtatagaatcacccgtcaagacgtgttctggcatagacattgaggctgaagtaatgtcagaagctaaaacatcatctgggactgtgcaatgtgctaaagaaacttcttcagttacatctgagtccagcacttgctcaggaatgatgaccgtttcagacacatctgcttcttccatgatatctgggcactgaacatcttctataacaacgtcctcaataacatcttggattacaactgaatctgggtcatcaggaacaaagttatgcacagttatgtctgaatccacaacatctgaaacaaaaacagtttcttgtacttccacaacaatttgatcaccatccatgtgtgtaccatcagctcctgttgcatcaaaaaatgagtttggctcttgttgtaattcaagcccatcttcatccatggcctttaattctcatcagtcacagctcctgtcttaatcacacaacttgactctaatcttaatcttgaacatccactgttgctgtactgcgcagcaaaacaattctatcttcttaatagttcttctatgtctttcccagcgtaaagcacagctcagggaacagacggcagtgacaggcgggcagtgggaggcgggagaacggcttgagcccaggagttcgagaccagcctggggcaatatagcaagaacctctaaacatgagacttcttgcagccaccgtctgcattacaagaacctttttaatgtttcttagcatctagcacggtgcatcgctaacagtaggctccgagtttatcaagaaagttgcacagt

SEQ ID NO: 18224 - RNA, 4604 nt, Homo sapiens
  source 1..4604: mol_type = other RNA
tgaagtaccagctactcgagaggctgaggcagataattgcttgaacccaggaagcagaggttgcagtgagctgcagaggttgcagtgatcacaccactgcagtccagcctgggcaacagagcaagactccgtcttaagaaaaaaaaacaacaaaaaaaaacaaacaaacaaaaaacctgtggaagacttagtgatgttccaaataaggcctcagactttccttatccacttaaaacacatctttaccttttaatcaaagccaacttgagtgttaagtttttaaagtttgctaactgtaactgagaaataacagatcagcctgaacttgccgagtgtgaagtcataattagcacccgttctctggtccacagagccatcacttcttttccatccccctcactaggtaagacagagttccctctcaggcttctcaaagagaactgtgggagtcatgtctggatactcatttgcttttcagaaaaacataaagacatggaggtgaaattgtatgaaaacattctacctagaaacatcttaacctctatgtttcaattaccaaagatatttaaaagaaaatatctttactctttaaaaatactagtgtccttattttccttctaattcttcacctgagtagtctctctgaagagcatgacttacaaaatgctctctcatgcatccctggatctttcatgttattgtaaatttaatacttttcattatagattttaaacaactactacttggggttgtgtgtataaatatgtaaaataagcaatacacacaggtacatgatatatatgtgtatatatataattcagggtacatttacatacataaagttgcaaaagatcctataagccatgagttacctctaggagattccaaaatgcagtcctcagtaagtgtcatttgtagcacacaaccattccaagatgaagccgcacagacagaataatcaaaatacaacatgagcaagcacagtttttcaataaggttttctaaaagtttgctacgctgacaaaagatgtaaataatccaaagaaagccaaaagaagtatatttgaaaagtaaacacgaacccagccactgctctttactcagcaaagccagggacgcaacagctcaaatggaaactttcactgtcaagtggtctgaaaatattaagcaagacaagtaaatgacttccatgttatgataattagacctgactgtaaaatctcccatttatattagtagatgtctctgacaattttattgtgagaaatgtatggggaaaaaaatgagtcaacatgaatactttcagagttaccaatataaagttaccttaagttaatggtcttagaagagtaccatcaaggtaagcaaggtaaatatttaaataaatataaaattctaagatataaaacttcggtatagaatcagggattactttattaaaagtaactagcatgttgccagttttccctatttattaaacaaactgaatagaattcagaacacactactgagcaaaatgtatatttaaaaaaaagtcaactagaagtaataattctatttgtacacagcataaatcaatatacagtattgtatgtgaatgagactgattggctttaaaatgaattttctgcttcaaggccaatatctctacaaacgttctgtagaagtattgttagggcaggccaacttctttatgatgtcgcattatgtgctggttcttttctgaaggtcttcggaagcctttcttgcagtactcacaccggtgaggatagtctttcgtgtgaatggaaataacgtgccgtttaaagcctgaggcatctgtagtgctatactcacagtactcacactgatacactttcctgccactgtgtgtcttcatatgctttttaagctcactctgttgcctaaatccctttctacatctcttgcacctaaatggaagatcctttgtgtgaactgagagaatatggcgacttagaacaaatggatctgcaatcttaaagtcacaatgtctacactggtgcatttttttgcccttgtgggcagccacgtgtttcttgagttctgaaggcctgtgaaagcctttatcacacatgtcacacttatgggggtagtctttcgtgtgaactgaaattatgtgtcgtttcaaatcacttgagttcgaactcttgtggtcgcaatgcaaacactggtgtgttttgctttcttggtggataagagcatgttgctgcacctctttggtatccgagaaagtcagaagacaaatgtcacacttgaatggcatctctttactatgcttagttttgacatgcgttttcaagttagaagagtctgcagacctatattcgcagtactggcattggtacggcttctccccagtatggattctcatgtgctttttgagctctgacgggtgacgaaaacccttaccacactccacacaaatatgaggaaagttcttgctgtggactgccaagaggtggcgattcaataacccttgttcagctgtctcgtattcacagaatttacacttgtgcattttgttggctcctttttccttatgcaccattttgtgagtaaacaaagcccctgcatgagagaaatgcttcccacactcatcgcattcaatggccttctctgccttgctggtcagcttgtggctctccaggtggttgtgtaaacttatcttcttgttggtagtgtaatcacagtcagtacagcggtatttcttcttggcaaggtgttcgggatggtttttcatgtgccttttcaaaaaacctctcgacttaaacttcttcccacaaatcatgcaaggatagacagtcaaaggatgtccatcagggccaataattattgctgtttggtactgcctggaatcaggtcttctccttttctttggtttttgtttagccagtctgccgaggccagcagactcatctatgtgcaagagggcacttgcagtgccattccggttttcaattccatcagaattattaccataagctgctgcccatgcaatcggcatgaaggttttgatttcattgtcatccatttgctgctcgtgcacggcggcggctgccgctgctgctgcagcatcctcctctcctacgatcacttccatataaacttcgtcagcgatttcagcaacatttaaatcttcatcttctggctgagagtcattgacagtcatataaaccatcttttccctgggaacacgaatactgctgttctgatcaagcagttcaactccatgatcattctcaggctcactctccacaatgtctacagttccacctaagtcatcttctccagggtcagctttaaaaatgtacaccttgatgacctcagggcaagtgccatccactttacaaggatcaatttccgactctgtgtccatggtcattccagaagaaccatcgtgttctattttgccagcatcatccaaggaaatcataaggtagtcctcacagttgcctttgtcatcatcctgctggtccacagggatcccattggcatctatgactgcttcagaggcacagtctgctaccaatacttcttctgaaactacgtcggtagtcagaggatcagtgacaatttctgcttccactacactatcatgaaccacatgttcaacatgtccaacatgtccaacatgtccaacgtcagacacatgtatagaatcacccgtcaagacgtgttctggcatagacattgaggctgaagtaatgtcagaagctaaaacatcatctgggactgtgcaatgtgctaaagaaacttcttcagttacatctgagtccagcacttgctcaggaatgatgaccgtttcagacacatctgcttcttccatgatatctgggcactgaacatcttctataacaacgtcctcaataacatcttggattacaactgaatctgggtcatcaggaacaaagttatgcacagttatgtctgaatccacaacatctgaaacaaaaacagtttcttgtacttccacaacaatttgatcaccatccatgtgtgtaccatcagctcctgttgcatcaaaaaatgagtttggctcttgttgtaattcaagcccatcttcatccatggcctttaattctcatcagtcacagctcctgtcttaatcacacaacttgactctaatcttaatcttgaacatccactgttgctgtactgcgcagcaaaacaattctatcttcttaatagttcttctatgtctttcccagtactctcattatttttcaactttgaaacttttcctagtccaatggaactactaagtaccgtaaagcacagctcagggaacagacggcagtgacaggcgggcagtgggaggcgggagaacggcttgagcccaggagttcgagaccagcctggggcaatatagcaagaaccgcctctcgcgccggtcctggccgaggctccagctcgagttgtttgcaggccctcagacccccgcccgcagtaaatgtgttttcttcatccccgtggctggggaggaagataaatttagcaacccccgccgtcccctgccttcgcttaaaaaaaaaaaatctttgaaataaaatgaaaacgggcttgccagtctaaatgggtgtgcg

SEQ ID NO: 18225 - RNA, 4632 nt, Homo sapiens
  source 1..4632: mol_type = other RNA
tgaagtaccagctactcgagaggctgaggcagataattgcttgaacccaggaagcagaggttgcagtgagctgcagaggttgcagtgatcacaccactgcagtccagcctgggcaacagagcaagactccgtcttaagaaaaaaaaacaacaaaaaaaaacaaacaaacaaaaaacctgtggaagacttagtgatgttccaaataaggcctcagactttccttatccacttaaaacacatctttaccttttaatcaaagccaacttgagtgttaagtttttaaagtttgctaactgtaactgagaaataacagatcagcctgaacttgccgagtgtgaagtcataattagcacccgttctctggtccacagagccatcacttcttttccatccccctcactaggtaagacagagttccctctcaggcttctcaaagagaactgtgggagtcatgtctggatactcatttgcttttcagaaaaacataaagacatggaggtgaaattgtatgaaaacattctacctagaaacatcttaacctctatgtttcaattaccaaagatatttaaaagaaaatatctttactctttaaaaatactagtgtccttattttccttctaattcttcacctgagtagtctctctgaagagcatgacttacaaaatgctctctcatgcatccctggatctttcatgttattgtaaatttaatacttttcattatagattttaaacaactactacttggggttgtgtgtataaatatgtaaaataagcaatacacacaggtacatgatatatatgtgtatatatataattcagggtacatttacatacataaagttgcaaaagatcctataagccatgagttacctctaggagattccaaaatgcagtcctcagtaagtgtcatttgtagcacacaaccattccaagatgaagccgcacagacagaataatcaaaatacaacatgagcaagcacagtttttcaataaggttttctaaaagtttgctacgctgacaaaagatgtaaataatccaaagaaagccaaaagaagtatatttgaaaagtaaacacgaacccagccactgctctttactcagcaaagccagggacgcaacagctcaaatggaaactttcactgtcaagtggtctgaaaatattaagcaagacaagtaaatgacttccatgttatgataattagacctgactgtaaaatctcccatttatattagtagatgtctctgacaattttattgtgagaaatgtatggggaaaaaaatgagtcaacatgaatactttcagagttaccaatataaagttaccttaagttaatggtcttagaagagtaccatcaaggtaagcaaggtaaatatttaaataaatataaaattctaagatataaaacttcggtatagaatcagggattactttattaaaagtaactagcatgttgccagttttccctatttattaaacaaactgaatagaattcagaacacactactgagcaaaatgtatatttaaaaaaaagtcaactagaagtaataattctatttgtacacagcataaatcaatatacagtattgtatgtgaatgagactgattggctttaaaatgaattttctgcttcaaggccaatatctctacaaacgttctgtagaagtattgttagggcaggccaacttctttatgatgtcgcattatgtgctggttcttttctgaaggtcttcggaagcctttcttgcagtactcacaccggtgaggatagtctttcgtgtgaatggaaataacgtgccgtttaaagcctgaggcatctgtagtgctatactcacagtactcacactgatacactttcctgccactgtgtgtcttcatatgctttttaagctcactctgttgcctaaatccctttctacatctcttgcacctaaatggaagatcctttgtgtgaactgagagaatatggcgacttagaacaaatggatctgcaatcttaaagtcacaatgtctacactggtgcatttttttgcccttgtgggcagccacgtgtttcttgagttctgaaggcctgtgaaagcctttatcacacatgtcacacttatgggggtagtctttcgtgtgaactgaaattatgtgtcgtttcaaatcacttgagttcgaactcttgtggtcgcaatgcaaacactggtgtgttttgctttcttggtggataagagcatgttgctgcacctctttggtatccgagaaagtcagaagacaaatgtcacacttgaatggcatctctttactatgcttagttttgacatgcgttttcaagttagaagagtctgcagacctatattcgcagtactggcattggtacggcttctccccagtatggattctcatgtgctttttgagctctgacgggtgacgaaaacccttaccacactccacacaaatatgaggaaagttcttgctgtggactgccaagaggtggcgattcaataacccttgttcagctgtctcgtattcacagaatttacacttgtgcattttgttggctcctttttccttatgcaccattttgtgagtaaacaaagcccctgcatgagagaaatgcttcccacactcatcgcattcaatggccttctctgccttgctggtcagcttgtggctctccaggtggttgtgtaaacttatcttcttgttggtagtgtaatcacagtcagtacagcggtatttcttcttggcaaggtgttcgggatggtttttcatgtgccttttcaaaaaacctctcgacttaaacttcttcccacaaatcatgcaaggatagacagtcaaaggatgtccatcagggccaataattattgctgtttggtactgcctggaatcaggtcttctccttttctttggtttttgtttagccagtctgccgaggccagcagactcatctatgtgcaagagggcacttgcagtgccattccggttttcaattccatcagaattattaccataagctgctgcccatgcaatcggcatgaaggttttgatttcattgtcatccatttgctgctcgtgcacggcggcggctgccgctgctgctgcagcatcctcctctcctacgatcacttccatataaacttcgtcagcgatttcagcaacatttaaatcttcatcttctggctgagagtcattgacagtcatataaaccatcttttccctgggaacacgaatactgctgttctgatcaagcagttcaactccatgatcattctcaggctcactctccacaatgtctacagttccacctaagtcatcttctccagggtcagctttaaaaatgtacaccttgatgacctcagggcaagtgccatccactttacaaggatcaatttccgactctgtgtccatggtcattccagaagaaccatcgtgttctattttgccagcatcatccaaggaaatcataaggtagtcctcacagttgcctttgtcatcatcctgctggtccacagggatcccattggcatctatgactgcttcagaggcacagtctgctaccaatacttcttctgaaactacgtcggtagtcagaggatcagtgacaatttctgcttccactacactatcatgaaccacatgttcaacatgtccaacatgtccaacatgtccaacgtcagacacatgtatagaatcacccgtcaagacgtgttctggcatagacattgaggctgaagtaatgtcagaagctaaaacatcatctgggactgtgcaatgtgctaaagaaacttcttcagttacatctgagtccagcacttgctcaggaatgatgaccgtttcagacacatctgcttcttccatgatatctgggcactgaacatcttctataacaacgtcctcaataacatcttggattacaactgaatctgggtcatcaggaacaaagttatgcacagttatgtctgaatccacaacatctgaaacaaaaacagtttcttgtacttccacaacaatttgatcaccatccatgtgtgtaccatcagctcctttttgctccacctccctctcctcaactcatatttgttcttctttccatctctcccatgtgtttcttttacttctattttttttcctttctcccttcacacgcttccctttttgttctggtgcaatataccaccaatatgctccatctatggctatagaaatttagaaatcatcctctgaatctaggacatacaaggatcaaaggataaattaaaagagggactaaagaccacagttgaggaggaaagacaactgggttgaggaggctctggagactgataggataaatacaagtgcagctgcgctggagtggtggaggttgagagtagttggagcaggagctgccccaacttcaccagggtacgttgcctccatctagcctcctcccgtccccctagacccgaactcccaaggcagttcctcggaacatagttcccctactctagtccattttgcagttaaggaatgaaggtagaggactgaatcagttgaagcccagtgagattaaatgacttaaccaagatcacacagtttgcacagtgtatggtgctcagaaaatattattctgaatgaatgtcacaaatggaaatagaatcaaa

SEQ ID NO: 18226 - RNA, 3981 nt, Homo sapiens
  source 1..3981: mol_type = other RNA
tgaagtaccagctactcgagaggctgaggcagataattgcttgaacccaggaagcagaggttgcagtgagctgcagaggttgcagtgatcacaccactgcagtccagcctgggcaacagagcaagactccgtcttaagaaaaaaaaacaacaaaaaaaaacaaacaaacaaaaaacctgtggaagacttagtgatgttccaaataaggcctcagactttccttatccacttaaaacacatctttaccttttaatcaaagccaacttgagtgttaagtttttaaagtttgctaactgtaactgagaaataacagatcagcctgaacttgccgagtgtgaagtcataattagcacccgttctctggtccacagagccatcacttcttttccatccccctcactaggtaagacagagttccctctcaggcttctcaaagagaactgtgggagtcatgtctggatactcatttgcttttcagaaaaacataaagacatggaggtgaaattgtatgaaaacattctacctagaaacatcttaacctctatgtttcaattaccaaagatatttaaaagaaaatatctttactctttaaaaatactagtgtccttattttccttctaattcttcacctgagtagtctctctgaagagcatgacttacaaaatgctctctcatgcatccctggatctttcatgttattgtaaatttaatacttttcattatagattttaaacaactactacttggggttgtgtgtataaatatgtaaaataagcaatacacacaggtacatgatatatatgtgtatatatataattcagggtacatttacatacataaagttgcaaaagatcctataagccatgagttacctctaggagattccaaaatgcagtcctcagtaagtgtcatttgtagcacacaaccattccaagatgaagccgcacagacagaataatcaaaatacaacatgagcaagcacagtttttcaataaggttttctaaaagtttgctacgctgacaaaagatgtaaataatccaaagaaagccaaaagaagtatatttgaaaagtaaacacgaacccagccactgctctttactcagcaaagccagggacgcaacagctcaaatggaaactttcactgtcaagtggtctgaaaatattaagcaagacaagtaaatgacttccatgttatgataattagacctgactgtaaaatctcccatttatattagtagatgtctctgacaattttattgtgagaaatgtatggggaaaaaaatgagtcaacatgaatactttcagagttaccaatataaagttaccttaagttaatggtcttagaagagtaccatcaaggtaagcaaggtaaatatttaaataaatataaaattctaagatataaaacttcggtatagaatcagggattactttattaaaagtaactagcatgttgccagttttccctatttattaaacaaactgaatagaattcagaacacactactgagcaaaatgtatatttaaaaaaaagtcaactagaagtaataattctatttgtacacagcataaatcaatatacagtattgtatgtgaatgagactgattggctttaaaatgaattttctgcttcaaggccaatatctctacaaacgttctgtagaagtattgttagggcaggccaacttctttatgatgtcgcattatgtgctggttcttttctgaaggtcttcggaagcctttcttgcagtactcacaccggtgaggatagtctttcgtgtgaatggaaataacgtgccgtttaaagcctgaggcatctgtagtgctatactcacagtactcacactgatacactttcctgccactgtgtgtcttcatatgctttttaagctcactctgttgcctaaatccctttctacatctcttgcacctaaatggaagatcctttgtgtgaactgagagaatatggcgacttagaacaaatggatctgcaatcttaaagtcacaatgtctacactggtgcatttttttgcccttgtgggcagccacgtgtttcttgagttctgaaggcctgtgaaagcctttatcacacatgtcacacttatgggggtagtctttcgtgtgaactgaaattatgtgtcgtttcaaatcacttgagttcgaactcttgtggtcgcaatgcaaacactggtgtgttttgctttcttggtggataagagcatgttgctgcacctctttggtatccgagaaagtcagaagacaaatgtcacacttgaatggcatctctttactatgcttagttttgacatgcgttttcaagttagaagagtctgcagacctatattcgcagtactggcattggtacggcttctccccagtatggattctcatgtgctttttgagctctgacgggtgacgaaaacccttaccacactccacacaaatatgaggaaagttcttgctgtggactgccaagaggtggcgattcaataacccttgttcagctgtctcgtattcacagaatttacacttgtgcattttgttggctcctttttccttatgcaccattttgtgagtaaacaaagcccctgcatgagagaaatgcttcccacactcatcgcattcaatggccttctctgccttgctggtcagcttgtggctctccaggtggttgtgtaaacttatcttcttgttggtagtgtaatcacagtcagtacagcggtatttcttcttggcaaggtgttcgggatggtttttcatgtgccttttcaaaaaacctctcgacttaaacttcttcccacaaatcatgcaaggatagacagtcaaaggatgtccatcagggccaataattattgctgtttggtactgcctggaatcaggtcttctccttttctttggtttttgtttagccagtctgccgaggccagcagactcatctatgtgcaagagggcacttgcagtgccattccggttttcaattccatcagaattattaccataagctgctgcccatgcaatcggcatgaaggttttgatttcattgtcatccatttgctgctcgtgcacggcggcggctgccgctgctgctgcagcatcctcctctcctacgatcacttccatataaacttcgtcagcgatttcagcaacatttaaatcttcatcttctggctgagagtcattgacagtcatataaaccatcttttccctgggaacacgaatactgctgttctgatcaagcagttcaactccatgatcattctcaggctcactctccacaatgtctacagttccacctaagtcatcttctccagggtcagctttaaaaatgtacaccttgatgacctcagggcaagtgccatccactttacaaggatcaatttccgactctgtgtccatggtcattccagaagaaccatcgtgttctattttgccagcatcatccaccgaattcattcagctaatgagtagcagagctggtatccaaatccaaggctgcctgactcagctgcaagctgagtttccatataccagatgttgcttctctaagataggcaaggagaggtatgttctctctctccctctctccttttctcttccctccccaagcccattacctcacaaagtaatcatatatctgttcaaagggcagggtgacatttttgtctaggtttcagcagataaacagtaaatattaaccacaaggccagtctgaagctccaattgcttgtaatgctttcaaaatagagaccttttcccaaccttgtttttggcaggggaagggagaaactaaaacatctttgccttatttgagtgctttattcttgttataaagctagccaacacctagattgaacattatactgaaaactcttaagtcattaattgtagtgttgatttctaaataaatttcagtttacagtaaagatacaattttagatggattaaaataaccacttttcgaattttatctgaaaaagctt

SEQ ID NO: 18227 - RNA, 3510 nt, Homo sapiens
  source 1..3510: mol_type = other RNA
tgaagtaccagctactcgagaggctgaggcagataattgcttgaacccaggaagcagaggttgcagtgagctgcagaggttgcagtgatcacaccactgcagtccagcctgggcaacagagcaagactccgtcttaagaaaaaaaaacaacaaaaaaaaacaaacaaacaaaaaacctgtggaagacttagtgatgttccaaataaggcctcagactttccttatccacttaaaacacatctttaccttttaatcaaagccaacttgagtgttaagtttttaaagtttgctaactgtaactgagaaataacagatcagcctgaacttgccgagtgtgaagtcataattagcacccgttctctggtccacagagccatcacttcttttccatccccctcactaggtaagacagagttccctctcaggcttctcaaagagaactgtgggagtcatgtctggatactcatttgcttttcagaaaaacataaagacatggaggtgaaattgtatgaaaacattctacctagaaacatcttaacctctatgtttcaattaccaaagatatttaaaagaaaatatctttactctttaaaaatactagtgtccttattttccttctaattcttcacctgagtagtctctctgaagagcatgacttacaaaatgctctctcatgcatccctggatctttcatgttattgtaaatttaatacttttcattatagattttaaacaactactacttggggttgtgtgtataaatatgtaaaataagcaatacacacaggtacatgatatatatgtgtatatatataattcagggtacatttacatacataaagttgcaaaagatcctataagccatgagttacctctaggagattccaaaatgcagtcctcagtaagtgtcatttgtagcacacaaccattccaagatgaagccgcacagacagaataatcaaaatacaacatgagcaagcacagtttttcaataaggttttctaaaagtttgctacgctgacaaaagatgtaaataatccaaagaaagccaaaagaagtatatttgaaaagtaaacacgaacccagccactgctctttactcagcaaagccagggacgcaacagctcaaatggaaactttcactgtcaagtggtctgaaaatattaagcaagacaagtaaatgacttccatgttatgataattagacctgactgtaaaatctcccatttatattagtagatgtctctgacaattttattgtgagaaatgtatggggaaaaaaatgagtcaacatgaatactttcagagttaccaatataaagttaccttaagttaatggtcttagaagagtaccatcaaggtaagcaaggtaaatatttaaataaatataaaattctaagatataaaacttcggtatagaatcagggattactttattaaaagtaactagcatgttgccagttttccctatttattaaacaaactgaatagaattcagaacacactactgagcaaaatgtatatttaaaaaaaagtcaactagaagtaataattctatttgtacacagcataaatcaatatacagtattgtatgtgaatgagactgattggctttaaaatgaattttctgcttcaaggccaatatctctacaaacgttctgtagaagtattgttagggcaggccaacttctttatgatgtcgcattatgtgctggttcttttctgaaggtcttcggaagcctttcttgcagtactcacaccggtgaggatagtctttcgtgtgaatggaaataacgtgccgtttaaagcctgaggcatctgtagtgctatactcacagtactcacactgatacactttcctgccactgtgtgtcttcatatgctttttaagctcactctgttgcctaaatccctttctacatctcttgcacctaaatggaagatcctttgtgtgaactgagagaatatggcgacttagaacaaatggatctgcaatcttaaagtcacaatgtctacactggtgcatttttttgcccttgtgggcagccacgtgtttcttgagttctgaaggcctgtgaaagcctttatcacacatgtcacacttatgggggtagtctttcgtgtgaactgaaattatgtgtcgtttcaaatcacttgagttcgaactcttgtggtcgcaatgcaaacactggtgtgttttgctttcttggtggataagagcatgttgctgcacctctttggtatccgagaaagtcagaagacaaatgtcacacttgaatggcatctctttactatgcttagttttgacatgcgttttcaagttagaagagtctgcagacctatattcgcagtactggcattggtacggcttctccccagtatggattctcatgtgctttttgagctctgacgggtgacgaaaacccttaccacactccacacaaatatgaggaaagttcttgctgtggactgccaagaggtggcgattcaataacccttgttcagctgtctcgtattcacagaatttacacttgtgcattttgttggctcctttttccttatgcaccattttgtgagtaaacaaagcccctgcatgagagaaatgcttcccacactcatcgcattcaatggccttctctgccttgctggtcagcttgtggctctccaggtggttgtgtaaacttatcttcttgttggtagtgtaatcacagtcagtacagcggtatttcttcttggcaaggtgttcgggatggtttttcatgtgccttttcaaaaaacctctcgacttaaacttcttcccacaaatcatgcaaggatagacagtcaaaggatgtccatcagggccaataattattgctgtttggtactgcctggaatcaggtcttctccttttctttggtttttgtttagccagtctgccgaggccagcagactcatctatgtgcaagagggcacttgcagtgccattccggttttcaattccatcagaattattaccataagctgctgcccatgcaatcggcatgaaggttttgatttcattgtcatccatttgctgctcgtgcacggcggcggctgccgctgctgctgcagcatcctcctctcctacgatcacttccatataaacttcgtcagcgatttcagcaacatttaaatcttcatcttctggctgagagtcattgacagtcatataaaccatcttttccctgggaacacgaatactgctgttctgatcaagcagttcaactccatgatcattctcaggctcactctccacaatgtctacagttccacctaagtcatcttctccagggtcagctttaaaaatgtacaccttgatgacctcagggcaagtgccatccactttacaaggatcaatttccgactctgtgtccatggtcattccagaagaaccatcgtgttctattttgccagcatcatccacggacggacgtgcgggcggccggcgacggtggcgggtgctgcaggccggcctttctctggagcact

SEQ ID NO: 18228 - RNA, 4243 nt, Homo sapiens
  source 1..4243: mol_type = other RNA
tgaagtaccagctactcgagaggctgaggcagataattgcttgaacccaggaagcagaggttgcagtgagctgcagaggttgcagtgatcacaccactgcagtccagcctgggcaacagagcaagactccgtcttaagaaaaaaaaacaacaaaaaaaaacaaacaaacaaaaaacctgtggaagacttagtgatgttccaaataaggcctcagactttccttatccacttaaaacacatctttaccttttaatcaaagccaacttgagtgttaagtttttaaagtttgctaactgtaactgagaaataacagatcagcctgaacttgccgagtgtgaagtcataattagcacccgttctctggtccacagagccatcacttcttttccatccccctcactaggtaagacagagttccctctcaggcttctcaaagagaactgtgggagtcatgtctggatactcatttgcttttcagaaaaacataaagacatggaggtgaaattgtatgaaaacattctacctagaaacatcttaacctctatgtttcaattaccaaagatatttaaaagaaaatatctttactctttaaaaatactagtgtccttattttccttctaattcttcacctgagtagtctctctgaagagcatgacttacaaaatgctctctcatgcatccctggatctttcatgttattgtaaatttaatacttttcattatagattttaaacaactactacttggggttgtgtgtataaatatgtaaaataagcaatacacacaggtacatgatatatatgtgtatatatataattcagggtacatttacatacataaagttgcaaaagatcctataagccatgagttacctctaggagattccaaaatgcagtcctcagtaagtgtcatttgtagcacacaaccattccaagatgaagccgcacagacagaataatcaaaatacaacatgagcaagcacagtttttcaataaggttttctaaaagtttgctacgctgacaaaagatgtaaataatccaaagaaagccaaaagaagtatatttgaaaagtaaacacgaacccagccactgctctttactcagcaaagccagggacgcaacagctcaaatggaaactttcactgtcaagtggtctgaaaatattaagcaagacaagtaaatgacttccatgttatgataattagacctgactgtaaaatctcccatttatattagtagatgtctctgacaattttattgtgagaaatgtatggggaaaaaaatgagtcaacatgaatactttcagagttaccaatataaagttaccttaagttaatggtcttagaagagtaccatcaaggtaagcaaggtaaatatttaaataaatataaaattctaagatataaaacttcggtatagaatcagggattactttattaaaagtaactagcatgttgccagttttccctatttattaaacaaactgaatagaattcagaacacactactgagcaaaatgtatatttaaaaaaaagtcaactagaagtaataattctatttgtacacagcataaatcaatatacagtattgtatgtgaatgagactgattggctttaaaatgaattttctgcttcaaggccaatatctctacaaacgttctgtagaagtattgttagggcaggccaacttctttatgatgtcgcattatgtgctggttcttttctgaaggtcttcggaagcctttcttgcagtactcacaccggtgaggatagtctttcgtgtgaatggaaataacgtgccgtttaaagcctgaggcatctgtagtgctatactcacagtactcacactgatacactttcctgccactgtgtgtcttcatatgctttttaagctcactctgttgcctaaatccctttctacatctcttgcacctaaatggaagatcctttgtgtgaactgagagaatatggcgacttagaacaaatggatctgcaatcttaaagtcacaatgtctacactggtgcatttttttgcccttgtgggcagccacgtgtttcttgagttctgaaggcctgtgaaagcctttatcacacatgtcacacttatgggggtagtctttcgtgtgaactgaaattatgtgtcgtttcaaatcacttgagttcgaactcttgtggtcgcaatgcaaacactggtgtgttttgctttcttggtggataagagcatgttgctgcacctctttggtatccgagaaagtcagaagacaaatgtcacacttgaatggcatctctttactatgcttagttttgacatgcgttttcaagttagaagagtctgcagacctatattcgcagtactggcattggtacggcttctccccagtatggattctcatgtgctttttgagctctgacgggtgacgaaaacccttaccacactccacacaaatatgaggaaagttcttgctgtggactgccaagaggtggcgattcaataacccttgttcagctgtctcgtattcacagaatttacacttgtgcattttgttggctcctttttccttatgcaccattttgtgagtaaacaaagcccctgcatgagagaaatgcttcccacactcatcgcattcaatggccttctctgccttgctggtcagcttgtggctctccaggtggttgtgtaaacttatcttcttgttggtagtgtaatcacagtcagtacagcggtatttcttcttggcaaggtgttcgggatggtttttcatgtgccttttcaaaaaacctctcgacttaaacttcttcccacaaatcatgcaaggatagacagtcaaaggatgtccatcagggccaataattattgtagagtttcctctgagagctcgcagagcacgctgcgccatggaactcgtgcgccctcacctgtttggtactgcctggaatcaggtcttctccttttctttggtttttgtttagccagtctgccgaggccagcagactcatctatgtgcaagagggcacttgcagtgccattccggttttcaattccatcagaattattaccataagctgctgcccatgcaatcggcatgaaggttttgatttcattgtcatccatttgctgctcgtgcacggcggcggctgccgctgctgctgcagcatcctcctctcctacgatcacttccatataaacttcgtcagcgatttcagcaacatttaaatcttcatcttctggctgagagtcattgacagtcatataaaccatcttttccctgggaacacgaatactgctgttctgatcaagcagttcaactccatgatcattctcaggctcactctccacaatgtctacagttccacctaagtcatcttctccagggtcagctttaaaaatgtacaccttgatgacctcagggcaagtgccatccactttacaaggatcaatttccgactctgtgtccatggtcattccagaagaaccatcgtgttctattttgccagcatcatccaaggaaatcataaggtagtcctcacagttgcctttgtcatcatcctgctggtccacagggatcccattggcatctatgactgcttcagaggcacagtctgctaccaatacttcttctgaaactacgtcggtagtcagaggatcagtgacaatttctgcttccactacactatcatgaaccacatgttcaacatgtccaacatgtccaacatgtccaacgtcagacacatgtatagaatcacccgtcaagacgtgttctggcatagacattgaggctgaagtaatgtcagaagctaaaacatcatctgggactgtgcaatgtgctaaagaaacttcttcagttacatctgagtccagcacttgctcaggaatgatgaccgtttcagacacatctgcttcttccatgatatctgggcactgaacatcttctataacaacgtcctcaataacatcttggattacaactgaatctgggtcatcaggaacaaagttatgcacagttatgtctgaatccacaacatctgaaacaaaaacagtttcttgtacttccacaacaatttgatcaccatccatgtgtgtaccatcagctcctgttgcatcaaaaaatgagtttggctcttgttgtaattcaagcccatcttcatccatggcctttaattctcatcagtcacagctccggacggacgtgcgggcggccggcgacggtggcgggtgctgcaggccggcctttctctggagcact

SEQ ID NO: 18229 - RNA, 2337 nt, Homo sapiens
  source 1..2337: mol_type = other RNA
tgaagtaccagctactcgagaggctgaggcaggagaactgcttgaacccgggtggcggaggttgcagtgagcctagatcgctccactgcactccagcctgggtgacagagcgagactctgtctcaaaaaaaaaaaaaagaagctgtgtataaatgtttgcacgaaatctgcagaatgtgccttctggcacattctggattcttgcttcctcatctgttaagtgaggttaatacctcttacttatagttgttgtaaagattaatataaagcatgacatctaccaaaatcagaacctacacaaagtgtgtgctcaataaatactatcttaagaggcagcctgctgtgtaaaatgaacatggactttaaagtcagatctgcactttaataccgggtctgctacttgagaatttcaattttctgctctgtagataggatagaacatctgctttgtaggtagttgtaagaagttttaaaattattactgtggaaaccaatgtctaagagcttcaatttctctaaaaaaggaaacagggtcacctgatgagggtggggtatgggattaaggacagcagtagaggtgtaaaataactgccatggtaattagagaaggaaatggaccaggaacccataaaggtgtgtgttggtgtgactgcgtgttggtgtgaggacttggctgaggttggaggccttgaatatttagtggcattcattacacaactgtttttctctagcagtttgaatgaaggaatggaaaagacagaataagtggaatgatacaaaaagatggccaatggtggcaagaaaatggggtgatggaatgatatgctatccaggctgctgaatacagaagtaaattacacaaagttggggggcgggggaggcaataatgagaaaagaatggagaggctggaattagaaatcacagaatgtactcaatgggaccaatgtggggcagatgatagaaagctggatttaggagtttctagacgagcagtgaaacattaacgtagcattaaagaagtcccgaagatttagttttatccctttttatcataaccattgccatctacttctcccttcagtttctcttcctcggatttggctgcattgcagaatatggtccccagctctctcccttcctgattgcccgtgaagacaaccacacagacctttgttcaaaggttttactgctcatcctgagaagactgtacatactaagaaagtaacaacctggggaaatggctgaagttccaaaagactccagacttcttacaggtttcatctctcttctgtggccactaacttcccaaggaggcagtgcccaaaagccctgtggttttttgatccgttgtacttcgatagctcctcctttccctagatccagcagaactctagacatgtaagacatagttcacaaaacaacagttatgaaccaacaaatacttggctcacggttatgagccactgaagtcagtcagacttaaggacaactagacagagctcccattttctgtcatctgggcaggaaccaatctcctgttgtataaaatgaccttctggtactttctggaatcttgcttcctcatctgttaagtgaggctaataccgcttactcatagttttgttgtgaagatgaactaagagcatgacatattacccgttttaaaattgtacacacagaccctgctttaaccagatgcctgcaaatgctcaggttttccttctacatatagaaaacaatttctcagctgccagggctgaagccagcagatatgcactaaacgacagaacaacggattgtgccaataaagtaggcaaagcttccttgcccagaatataaatcaaactgagtaaaaactgggtatattggctccaggaaaaggagcaaggacacccagctttcaggcaacctcgaattctctctgtttaggattcaccaaccccaaggtccaccgggtccttcaatctgagggtccatccaaggccttccttcctggggttgggtatggctagctgcctgatggagagaccccaggctgttcagcagcaacgcctggcacagccgaggcagcctcgtagtctgcgatgcggcgctgtaccagggcaggcatgagctgcacgtaagcggccatgaggcggtggttggaatggatcagcttcccagcacagctgtgcagacaggcctcctcctcagcgtccagagctcggtggtgcaagctgggcacacagcgctggaagcagagttctgtcatccgattgtagaccaacaggaagtcacgcaggtttcgcagttgctgttgctgctgctgctgccgctccatcacgccaccggcgcat

SEQ ID NO: 18230 - RNA, 644 nt, Homo sapiens
  source 1..644: mol_type = other RNA
tgaagtaccagctactcgagaggctgaggcaggagaatcacttgaacaagggaggcggaggttgtggtgagccaagatcctgccactgcactccagcctgggcaacagagggagactccataatgttaagtgcagatatagaatcaccagctcctccatacaggtggggtctcactcaagggacagtgactcctgagttgaaactccttctaaagcttccaactcggaataacaatgtcttctttctttccacattttgcgcaaacttcaagttcacaggcacatggcctgcacattatgtgataagaatccttcactgtcttttgtaaacatttaacacactttttaggttttgataatggtttgtatttgctgtattttacacgccactcaagaacttctttacagcgctgacatactccatcatgaagttttgcattaattttcttggtctgcacacttttatcgaacttgtcatttttgaagctaaacgtattctggtgcttctgaggtctggaacgagccacgttgcctttctgggagctcatcgccgaaatcaaagccacccctcgccgggagcaggcaaaaggatgaggggaaagaaaaccaacgaactactcccaggaattgacgcttctgtcaat

SEQ ID NO: 18231 - RNA, 557 nt, Homo sapiens
  source 1..557: mol_type = other RNA
tgaagtaccagctactcgagaggctgaggcaggagaatcacttgaacaagggaggcggaggttgtggtgagccaagatcctgccactgcactccagcctgggcaacagagggagactccatcactttttaggttttgataatggtttgtatttgctgtattttacacgccactcaagaacttctttacagcgctgacatactccatcatgaagttttgcattaattttctgcagttcaactcctgctgtgtggcccagttcctgacaggccatggaccgatgcgggggtcgggggctggggacccctgctccacagggagacaaactcaaacatcatgactagagtttgcagataaagacttggtctgcacacttttatcgaacttgtcatttttgaagctaaacgtattctggtgcttctgaggtctggaacgagccacgttgcctttctgggagctcatcgccgaaatcaaagccacccctcgccgggagcaggcaaaaggatgaggggaaagaaaaccaacgaactactcccaggaattgacgcttctgtcaat

SEQ ID NO: 18232 - RNA, 426 nt, Homo sapiens
  source 1..426: mol_type = other RNA
tgaagtaccagctactcgagaggctgaggcaggagaatcacttgaacaagggaggcggaggttgtggtgagccaagatcctgccactgcactccagcctgggcaacagagggagactccatcactttttaggttttgataatggtttgtatttgctgtattttacacgccactcaagaacttctttacagcgctgacatactccatcatgaagttttgcattaattttcttggtctgcacacttttatcgaacttgtcatttttgaagctaaacgtattctggtgcttctgaggtctggaacgagccacgttgcctttctgggagctcatcgccgaaatcaaagccacccctcgccgggagcaggcaaaaggatgaggggaaagaaaaccaacgaactactcccaggaattgacgcttctgtcaat

SEQ ID NO: 18233 - RNA, 540 nt, Homo sapiens
  source 1..540: mol_type = other RNA
tgaagtaccagctactcgagaggctgaggcaggagaatcacttgaacaagggaggcggaggttgtggtgagccaagatcctgccactgcactccagcctgggcaacagagggagactccatggaataacaatgtcttctttctttccacattttgcgcaaacttcaagttcacaggcacatggcctgcacattatgtgataagaatccttcactgtcttttgtaaacatttaacacactttttaggttttgataatggtttgtatttgctgtattttacacgccactcaagaacttctttacagcgctgacatactccatcatgaagttttgcattaattttcttggtctgcacacttttatcgaacttgtcatttttgaagctaaacgtattctggtgcttctgaggtctggaacgagccacgttgcctttctgggagctcatcgccgaaatcaaagccacccctcgccgggagcaggcaaaaggatgaggggaaagaaaaccaacgaactactcccaggaattgacgcttctgtcaat

SEQ ID NO: 18234 - RNA, 4261 nt, Homo sapiens
  source 1..4261: mol_type = other RNA
tgaagtaccagctactcgagaggctgaggcaggagaatcacttgaacccaggaggcagaggttgcagtgagctgagatcgtgccaccgcactccagcctggttgacagagcaagactctgtctcaaaaaaaaaaacaaaaaaactgaagtaggaagatttctgttctatatcaatcaggactttctttgtaaacgaggtgcgttccttttgttctgtggagacccaggagtaatatcaccagagtgagggtgatgaggttagtagggatgctcgcagtctgagaaatgaacggactgctttgcatcagtcccttccccttccctgattttaaaaatttaattttaaggagaaaatacttcagcatgagacttcagttcctgaggaaaataacactattgctccatccttagtattcacttaaacaaatgtttagctaaaattttattaaaaactttcagcccacccggacacggaagactttgcttttacagcagctaaggtatgttttcattaccccgtgagtgatgctaatgcattgcaaatagttattatgagtttatgtagtgcttggtgcctaaaataaatttcatttaaatatttaaaataactcctgaatataagcaatttattctgattactgataaaataacattcacattcaagcctacaaatctgagaaatcattattccatatgcacagaaggccacagtcagtagtctaatagtactgcttaccagtgtagtgtaaacttctttcagaatcagggaacaattctagatcagccatggtgagaaataagtgctcttctcttaggccagcgacacttccgatgggtcttgacatcccacctatgggctggtgtgtgaaactctcatctctacgtccctccccagttttaagagtcaccatgtcacataaaagctccagcatcagccaggcacggtggctcatgcctataatcccaacactttgggtggccaaggcaggtggatcacgaggtcaggagttcaagaccagcctggccaacatagcgaaaccttgtctctacttaaatatacaaaaattagccaggcgtggtggtgcatgcctgtaatcccagctactcgggaggctgagacagagaattgcttgaacctgggaggtggaggttgcagtaagccaagatcgtgccactgcactctagcctggatgacagagagattctgtctcaaaagaaagaaaaaaaaaaggctgggcgtggtggctcacacctgtaatcccagcactttgggagtctgaggcaggcggatcacgaggtcagaagatcgagaccatcctggctaacacggtgaaacctcgtctctactaaaaaatacaaaaaattagttgggcaaggtggtggcgcctgtagtcccagctactcgggaggctgaggcaggagaatggcgtgaacccaggaggcggagcttgcagtgagccaagatcgcaccactgcaccccagcctgggaagcggagcttgcggtgagccgagatggcgccactgcaccccagcctgggcgacagagtgagactccatctcaaaaaagaaaaaaaaaaaaaatgctgcagcagcctacacaaggccctgctgatcttccggggtgttatgtggcccatctatcagcaccctgttagtatgcttttcgataggtctaagactcacccactttattcaagcctactgtggcaggtgcctttgtcaaacttgagcctaaccatcccactggccagggtcctgctcatcactgtcctcctcagagtcagcagacaccctcttgattctctggagcgcagccttgatgctcctctcaaggtcactggtgcgtctgttgctggttggtttgctgctggggtttgggccaagatcagggtgaactttcttcagtttgaccccttgccttatggcagccagaatgtgctcattgattgaggcgtggggagggcgcaccgccggcacttccaccttccggagaggagctctgccatgccttaaggaggccaacacttcatccatagatcctggacatgaaaaactttccaaggagtcacgtggtcgctcagcaggtgattcgcacactagaggacgtggctggtcatctttcactggagcccggaagcctaagttctgatgagttgcagcttgagaggatgaggacagagcacggagaggagggggtgggggcggcggtggcggcggtggtggtggtggaggaggaggaggtggtggcagtgacaattcctcactggatttggaatgtgtttgatcaccaactggaacaaaaacctggacagggatatttccatgacagttttgacacttggggcttttcacattaccagcttccgataggggaacacctctagttttcctagaggacgggtgaattactgacaccgcgtgggaagctggcaagcacatctgctgggaaagatcacttggcaggtttggagccacaggttctgagccagaggtgtttcggacagattgagctaggcgtttatctttaaatgatctcaatcgttggagtgttttttgacgttcttggttgatccattcttttttcttttgctcctcttcttttatcttgtctcttttcatctgaatactgtgatgctgacgagagtatcttatgctttcttcagcctgttgcaatctgaaccgatgattttctttgcactgatcctttctactccggagagaggctcttttggcacagatcctgccccgtttagactccagctgctggcactgccttctgagttctttcacttccaaattcttatcatcctgcagccccaccacacagtcaatgactttaagttcctctggattttcacatggatcgtaatagacaacttcatcttgtttttcttttataagtcttttaagagagtccaactgtgtagtaagcagtatttcttcgttttttaatatctcaaatttaacttcatatagttctaattgaatttcataaaattgtatttctaattcatctacaacatttgtatttttttcttgttctggaagatcttccatctttccctgaatttcagctcttttgtgatttaaacacaactctttcgctctcatgagttgcagagtctctcgagctagcattagctgaagtttttccaacctgggaattgctgtggcccaggcagcctgaccaaatctcttcgcatcctgttccatttctttctgcattcctgctaatgcttttactgtctccttaaaataattcactgtgatatcctgaatagagacgacagcttcttcagcccgtctggtccattcttcagcttctttctccagggcaactacccttctaggacctaggtcatcctcatccaaagacttcaaaatatcaagcttacataaagttgcaacttctcgcatagccctaaatggctgcaataagtactggaagaacatggttgccacggtaaccaattcctggtatgcttcatcttcctcttggtaaacgttcattaatgctaccatggtgttggcttttccgtgtccttgaataacctggcgcagccgcgcgtccgcctcgacccaccgcgcgcgcaaggcccgctcccggaactcgcgcgggctttcgcagtcggccgcgccgccctcagccgggaagagtgcgtcgcgcactgtggcgccgccgcagccgtcggccgccgcgcccagatagcgttccagctgcccgcacagctcctgcagcgccgcctcgccgggacccgcgcgcgtcggccacagcagcgcccacagcccgagccccagaccccaggccccgccgccgcccacgtccagctccggcggcagccgcgggaagcagcgctccagaggcggccacagcgccgccaactgccggtgcgcgccgcggagccccgcggccgagagcaggccggcccagctggacggggagacggcggcctcaggcttgggctcgggctcgggccccaaccgggccccctcgcgcagccgccgctgctgcgcggtacggtcgtgacaagtcacagcgaacttgccctccgcgccgttccaggccaccaggaagcgcagccggtgcctctcgggctcggcgaagaggccctcccggaccggcacccagccctccaggctgtcaggctgctcgtcctccatggctgtcggcagcagcggccctagggctcggcgggcgcgggcctggcctcctcgcaccgcctgtcacgggacagtccgagccaaatcatttttcgctag

SEQ ID NO: 18235 - RNA, 3630 nt, Homo sapiens
  source 1..3630: mol_type = other RNA
tgaagtaccagctactcgagaggctgaggcaggagaatcacttgaacccgggaggcggaggttgcagtgagccaagatcacaccactgcactccagcctgggcaacagagcaagattcctcctcaaaacaaaacaaaacaaaactgggggcaagtgttaaatatatagttgaagaactaagaataaatgggggataaaaggaagaaagtacagtatgctataccagtatgttctgaaaatgttgacatagtataactattttaaaaattgggatgtcgggcgcagtggctcacacctgtaatcccagcactttgggaggccgaggcaggcggatcacctgaggtcgagagtttgaggccagcctgaccaatgtggagaaatcctgactctactaaaaatacaaaattagcagggcgtggtggcgcatgcctataatcccagctactcgggaagctgaggcaggagaattgcttgaatccaggaggcagaggttgcagtgagccgagatcgtgccattgcactccagcctgggcaacaagagcgcgagactccatctcaaaaaaaaaaaaaaattgggaaagaatgagaaaagcaaatgaaaactttttaattgtttcaattgccatattatttgtggttgtatttctattgttattctgagacagctgtaagtgtaagataaataaaagaaatgagtaattgtgggatgttctaattctatcgtgccctgtgttcttgaaaaccaggactttcagtacagaaggagaggtacagttgtaacagaaaggttagataaaaaccctgtaggccgggcacagtggctcacgcctataatcccagcactttggaaggctgaggtgggcggatcacaaggtaaggagtttgagaccagcctggctattatggtgaaaccctgtctctactaaaaatacaaaaattagctgggcatggtggctcatgcctgtaatcccagcattttgggaggccaaggctggtggatcacttgagttcaggagttcaagaccagcctgaccattatggtgaaacccctctactaaaaatacaaaaattagccgggcatggtggcgtgcacctgtagtcccagctacttgggaggctgaaacaggagaactgcttgaacccgggagatggaggttgcagtgagtcgagatcgtgccactgtactccagcctgggcaacagagtgcaactctgaaaaaaagagaaagaaaaggaaagagagagagagagagagagagaagaaggaggaaggaaagaaagacaccgtgatttacagtcttgccaaaggactgaacctaagtcttctcaaattcaatgtgcctgaacctgcactgtgtgctaatatcgagaggacagggcaatgtgctgaaccgtgccatgagtgtgcaatcagcaaaatacaaagtatgggaaactctataggtcctaggatcaggttcttcaccaggtaaattttaaggaactggaaagaaggaggaacttctagattaaaaaagagatgtaaaataaaatatacatttaataacaactttaaattgataatattaaaatatagatatatgcatttaggtgtggcagcagtaatcaaatgcaacaaagtgattaccatttaaatcagtctagcagttacttttgtggggttgtaattgtgacaggacacaaaaaggacacgtggggtgactggctgagtcctaaaagagtatttccttataataaggcattcagctataaattttgtgtctggttttcagtacttttatttcataatttttaaaatgttacaatcaaaaaagatatcaaagcccttagggttttctactaaaaagtctggatgtgaatacttatactgtaagtatcatctgatggtttttaagaaattgcttatattatagaaatatttctaaataagctataaatatttgaaaaatattgaattcttatgtatgcagttataaaaagtcaaagaattaagtatacttttctaacacaaaatttgttttgttacagtattatgtaagacaatttggttaaatggattttttttttttttttttttgagatggagtctagctctgttacccaggctggagtgtactggtgcgatctcagctcactgtaacctctgcctcccgggttcaagtgattcttctgcctcagcctcccaagtagctggtattacagatgcccgccaacacgtccagctaatttttgtatttttagtagagacggagtttcacagagaccagtgttggccaggctggtctcgaactcctgaccttgtgatccgcctgcttcagcctcccaaagtgctgggattacaagcgtaagccaccgcgtccggcctaaatggactttcttgacttccaaaattttcctttccaactcccatacaagattattaacgttaacctattagagattagaacaagagcattggagcagatttcttatttctttgaatgtctgcactttgtttcactctccatatttttttacacagaacaaagattagttatcgtgcctaaccatgatggtagttattgatatgtagcattatacacagagtattatctaatttgcaaaccgagatcctccacctacttgcctaccacctgtcttttccatgtaacaatgactgatgtagataattttttttgttgttagatgtgtaagaatctcaaggatgtaaaacagatttaaaccattaaaattaaagcagtttttaaatgcactataacaataaacatggacaaacacataactgtgttgtacatttttgcccatcaatcattgacaacttccctcccatttgttcaagcagcatcttaaatggtgcaattcagtggtcccttttcccttcgttttaataaaattatgtggtgttcgagtgattcacatattcaagaagtgaccggtctaagactcttcggataagagcttcctcaattatattaaaatctatgaaatcatcataaaacaaagtgtgactaacttgcagatgtcttattaaactgccactgaagctgcttggattctcatcgggtattaaacggcaaagtggacagaacacaggcctccgttccgatctgtgatgagtaatacaatgatccagcaagctgtcttcatacagttccctctgacaaaagggacatacacaccttgctgctgtctcctcaagttcttgtagtggtccatacttatctatgtacttctgacaagtccgaatatgtgccctcatttcactgaggcaaaccagggtgtcacactcagcgcagttcttatactctgatttcattcttttggctacatcagttgctggaactccttctgaaggaagatatgcccggcaataaggacaggtccacttgttgttctttagactggtagcaatacaggaacggcagaatacgtggccacagcgggtccggacaggctggtgtaacacctcaaggcacacggcgcagtcgaaggacgtgacgggcaactccgggtccctcctgcgctccagggcccgcgcggtggcagaggcgggcgccgatttgccgctgtcggtgctcagcacggagcccatcgctgtgcctctcgcccagacagctgcgaagcactcagt

SEQ ID NO: 18236 - RNA, 3028 nt, Homo sapiens
  source 1..3028: mol_type = other RNA
tgaagtaccagctactcgagaggctgaggcaggagaatcactttaagccaggaagcagaggttgcggtgagccgagatcgtgccattgcactccagcctgggcaacaagagtgaaactctgtctcaaacaaacaaacaaagatatccaattcagtcatgtatatctttctttgttttacatgctaatgacagtagtcttttactttcatggcaactcttctgcttactatatgataggaatggcctgggtaaaggatatgctttatagatctctggagttagctctttaatgcttccctcccctcttctgccctgcttttgagtggtgtgccttagcttgtgaaggattggttgaggatgacttaggttgagggggtctgggctgagaaggcttagactggggaggccagggctggcttggcttaggctgagtagatttgcatggagaaggtttagtttgggagggctgggactgacaggattttgtctgagaggatttaggttgagagggcacagaatggaagggtttaggctgggagtgtttgactgtggatgggttggactgatcggatttgaactgagagctcttgcacatgggatgggaccctatttggagagctggatttgaagccccaccttgtgtcttcatctggactccttgctgagaagcaggtcttagtttttgtgtggctgctgctggttgaaaggactgagggtgaggctttccaatatgggatgttcttatcagttttccagttgcttcagttaactctgttaccctggtgcaagcttgctgaggccatggcttccctactgctcttgctggctgtgaatccagggaataggagtgacctatcttggaggctactgccctagacctttcaagagttcccatcatttgtggtctctcagggcaggcctgtacatgctgacaaatgggtcttggcagtctcccaaatgttccattcgagtgacatccccgagcaactctggaaaatttcatgaatctttcacctgaataaaatatctggggatggaaggattgaataccaaaacttttacctcggccctgggcccctgcattctgaaaaggcaaaggatggaaccacttaggcctctgctctgacccaaaggggcggcccataacccaggaggctttcaaggaaacatggttaaagttacctccaattctggttggaaagagccaggagttctctagaacaggcctgaatactggggtaccatagagattctgaagattctggctgagctcacattgagtcccaggctcttgaattggcattagagcctggcttttagatgagctttttagctgactgtgtctttgctgaccctcaccttcagctgtcccagccatgttttctccagaggaaacttgaattctctgagtgttttcaaagtcttcatctacctgaatccccagctccctggccagggcggccatatcctccacagacacacatctgaggcaagaagagaacatcacttcctggagggcagcttgaaggccctccatgttcttccttctatccccagcatctcccctctcccaaaacagtagctgtgctggcttcaagttcagtatcctctgaaaaatttgagcctcttcactctccctggcttgggaactgagaacaaagtagcatctttcaatggcagcctctcctaaaaacattagcaagtcccattccttctcacctaaacagtcagtgaaaaaaaacacagctgaagaaacttccatcaaaaaaccaaactgagtccaaaagctttctagatttccacggagattagccagagcaacaggcttttggaaaaaggggttttcctttctatcatcgctatcaggaaaacaccatgttatctcaaccaggccatcagagatttgccggggaagcaccaaaagaggcaaatcttgatgaagaaagattttgtgtaatttcaactgggcagggctgagaagtgtgttgaggattctggacttagagaagctacagtatcctagacgcacaaaagagatgacaggcatcttcatgagagtcagaaacttttctgtatcctctgtaggcccccctgaaaactgtgttgactgcttcttcacaatgtctttcatggcccccagcattaagatgcttttgttgttttctgcatctggcagtagcaggggaagagcaaactggcactgatacatgtttgacatgacttggcgttgcaaagagctatctgaacacagcatggtggcacaaagcacgtcaaggggattaatggtttgtatgtctcgaatttccaaattctccactccagccagcaaatcctccttgctatcttcatccagaaccttgtgactgaggattgaatccctagccgtcacatctcgtgcttgaactttcatcaggaaattccaggctaagtctcctggactctcaggggtccacttacatcctcgatctaaggagaattgtttaacaaaatctggcagaacctttctgcttctatccatgttcaaacataacaggacatctttaaacaccttttttctttcatgccttaagccgcaaatggcagctgactgtggaaaagtactaaataaacacttgagaaaatgctgacaggtcgcctctccctttttctgtaccaaaattaacagcttccgacttttcttcaggagatctgtaacattctccagagtctcatactcttcctcagaaatcagcctccgagaagttaacgtgtctaagatagaatcaggatcatgttgaaggatttcaagcaacttttttctttctctttctatgatctctgagggagtactctcggtagccattgttcctgtttcctctaaaccaggaaatatattatgaaatcatcctaatgaataagtaaaagttaaaaaaagaatgacaaagaacaattctatttggctaagctttaacatgtcaatgatgcctagtgttggagagtgcagatacaagcacagtggggcaacccagctcggagcactctctgatcc

SEQ ID NO: 18237 - RNA, 3252 nt, Homo sapiens
  source 1..3252: mol_type = other RNA
tgaagtaccagctactcgagaggctgaggcaggagaatcactttaagccaggaagcagaggttgcggtgagccgagatcgtgccattgcactccagcctgggcaacaagagtgaaactctgtctcaaacaaacaaacaaagatatccaattcagtcatgtatatctttctttgttttacatgctaatgacagtagtcttttactttcatggcaactcttctgcttactatatgataggaatggcctgggtaaaggatatgctttatagatctctggagttagctctttaatgcttccctcccctcttctgccctgcttttgagtggtgtgccttagcttgtgaaggattggttgaggatgacttaggttgagggggtctgggctgagaaggcttagactggggaggccagggctggcttggcttaggctgagtagatttgcatggagaaggtttagtttgggagggctgggactgacaggattttgtctgagaggatttaggttgagagggcacagaatggaagggtttaggctgggagtgtttgactgtggatgggttggactgatcggatttgaactgagagctcttgcacatgggatgggaccctatttggagagctggatttgaagccccaccttgtgtcttcatctggactccttgctgagaagcaggtcttagtttttgtgtggctgctgctggttgaaaggactgagggtgaggctttccaatatgggatgttcttatcagttttccagttgcttcagttaactctgttaccctggtgcaagcttgctgaggccatggcttccctactgctcttgctggctgtgaatccagggaataggagtgacctatcttggaggctactgccctagacctttcaagagttcccatcatttgtggtctctcagggcaggcctgtacatgctgacaaatgggtcttggcagtctcccaaatgttccattcgagtgacatccccgagcaactctggaaaatttcatgaatctttcacctgaataaaatatctggggatggaaggattgaataccaaaacttttacctcggccctgggcccctgcattctgaaaaggcaaaggatggaaccacttaggcctctgctctgacccaaaggggcggcccataacccaggaggctttcaaggaaacatggttaaagttacctccaattctggttggaaagagccaggagttctctagaacaggcctgaatactggggtaccatagagattctgaagattctggctgagctcacattgagtcccaggctcttgaattggcattagagcctggcttttagatgagctttttagctgactgtgtctttgctgaccctcaccttcagctgtcccagccatgttttctccagaggaaacttgaattctctgagtgttttcaaagtcttcatctacctgaatccccagctccctggccagggcggccatatcctccacagacacacatctgaggcaagaagagaacatcacttcctggagggcagcttgaaggccctccatgttcttccttctatccccagcatctcccctctcccaaaacagtagctgtgctggcttcaagttcagtatcctctgaaaaatttgagcctcttcactctccctggcttgggaactgagaacaaagtagcatctttcaatggcagcctctcctaaaaacattagcaagtcccattccttctcacctaaacagtcagtgaaaaaaaacacagctgaagaaacttccatcaaaaaaccaaactgagtccaaaagctttctagatttccacggagattagccagagcaacaggcttttggaaaaaggggttttcctttctatcatcgctatcaggaaaacaccatgttatctcaaccaggccatcagagatttgccggggaagcaccaaaagaggcaaatcttgatgaagaaagattttgtgtaatttcaactgggcagggctgagaagtgtgttgaggattctggacttagagaagctacagtatcctagacgcacaaaagagatgacaggcatcttcatgagagtcagaaacttttctgtatcctctgtaggcccccctgaaaactgtgttgactgcttcttcacaatgtctttcatggcccccagcattaagatgcttttgttgttttctgcatctggcagtagcaggggaagagcaaactggcactgatacatgtttgacatgacttggcgttgcaaagagctatctgaacacagcatggtggcacaaagcacgtcaaggggattaatggtttgtatgtctcgaatttccaaattctccactccagccagcaaatcctccttgctatcttcatccagaaccttgtgactgaggattgaatccctagccgtcacatctcgtgcttgaactttcatcaggaaattccaggctaagtctcctggactctcaggggtccacttacatcctcgatctaaggagaattgtttaacaaaatctggcagaacctttctgcttctatccatgttcaaacataacaggacatctttaaacaccttttttctttctgtaatcccagctacctggggagctgaggcaggtgaatcgcttgaacccgggaggcggagggtacagtgagcaaggtcacaccattgcactccagcctgggcgacgagtgagactcttctatacttttctcctgttcctcctccaatgaaaggctggtttctgatccctcataacttggttcttcaccagagaactctgtggtttctgaattctcgaagtcctcttcaccatcatatccaacgtgctctgggtcatcataaacctcctcttccacagtggcttctgcatcttcaggggtgtcaacagatcctagatattcctcttttcctaagtataaagaatcatctagctcctcatatctctgtccatcttttatatatgtaatagttgctggaacttcacatccaactttctcaactgaatatgataatgtgacttctggtgtgtcatattccttctcattcttcctggcagacaaagctgtttccctataactagttttcttgtccctgaaaaactcagaggtttccaaatccaagtgttccttctcactgaagaacactgtgatctcaggggcttcaggctgttttattccaggagaaaaagcatcttctgaattactgcttgcccccatagattgaggaggtactgtattctcatgttttaaaacttcatgccttaagccgcaaat

SEQ ID NO: 18238 - RNA, 3416 nt, Homo sapiens
  source 1..3416: mol_type = other RNA
tgaagtaccagctactcgagaggctgaggcaggagaatcactttaagccaggaagcagaggttgcggtgagccgagatcgtgccattgcactccagcctgggcaacaagagtgaaactctgtctcaaacaaacaaacaaagatatccaattcagtcatgtatatctttctttgttttacatgctaatgacagtagtcttttactttcatggcaactcttctgcttactatatgataggaatggcctgggtaaaggatatgctttatagatctctggagttagctctttaatgcttccctcccctcttctgccctgcttttgagtggtgtgccttagcttgtgaaggattggttgaggatgacttaggttgagggggtctgggctgagaaggcttagactggggaggccagggctggcttggcttaggctgagtagatttgcatggagaaggtttagtttgggagggctgggactgacaggattttgtctgagaggatttaggttgagagggcacagaatggaagggtttaggctgggagtgtttgactgtggatgggttggactgatcggatttgaactgagagctcttgcacatgggatgggaccctatttggagagctggatttgaagccccaccttgtgtcttcatctggactccttgctgagaagcaggtcttagtttttgtgtggctgctgctggttgaaaggactgagggtgaggctttccaatatgggatgttcttatcagttttccagttgcttcagttaactctgttaccctggtgcaagcttgctgaggccatggcttccctactgctcttgctggctgtgaatccagggaataggagtgacctatcttggaggctactgccctagacctttcaagagttcccatcatttgtggtctctcagggcaggcctgtacatgctgacaaatgggtcttggcagtctcccaaatgttccattcgagtgacatccccgagcaactctggaaaatttcatgaatctttcacctgaataaaatatctggggatggaaggattgaataccaaaacttttacctcggccctgggcccctgcattctgaaaaggcaaaggatggaaccacttaggcctctgctctgacccaaaggggcggcccataacccaggaggctttcaaggaaacatggttaaagttacctccaattctggttggaaagagccaggagttctctagaacaggcctgaatactggggtaccatagagattctgaagattctggctgagctcacattgagtcccaggctcttgaattggcattagagcctggcttttagatgagctttttagctgactgtgtctttgctgaccctcaccttcagctgtcccagccatgttttctccagaggaaacttgaattctctgagtgttttcaaagtcttcatctacctgaatccccagctccctggccagggcggccatatcctccacagacacacatctgaggcaagaagagaacatcacttcctggagggcagcttgaaggccctccatgttcttccttctatccccagcatctcccctctcccaaaacagtagctgtgctggcttcaagttcagtatcctctgaaaaatttgagcctcttcactctccctggcttgggaactgagaacaaagtagcatctttcaatggcagcctctcctaaaaacattagcaagtcccattccttctcacctaaacagtcagtgaaaaaaaacacagctgaagaaacttccatcaaaaaaccaaactgagtccaaaagctttctagatttccacggagattagccagagcaacaggcttttggaaaaaggggttttcctttctatcatcgctatcaggaaaacaccatgttatctcaaccaggccatcagagatttgccggggaagcaccaaaagaggcaaatcttgatgaagaaagattttgtgtaatttcaactgggcagggctgagaagtgtgttgaggattctggacttagagaagctacagtatcctagacgcacaaaagagatgacaggcatcttcatgagagtcagaaacttttctgtatcctctgtaggcccccctgaaaactgtgttgactgcttcttcacaatgtctttcatggcccccagcattaagatgcttttgttgttttctgcatctggcagtagcaggggaagagcaaactggcactgatacatgtttgacatgacttggcgttgcaaagagctatctgaacacagcatggtggcacaaagcacgtcaaggggattaatggtttgtatgtctcgaatttccaaattctccactccagccagcaaatcctccttgctatcttcatccagaaccttgtgactgaggattgaatccctagccgtcacatctcgtgcttgaactttcatcaggaaattccaggctaagtctcctggactctcaggggtccacttacatcctcgatctaaggagaattgtttaacaaaatctggcagaacctttctgcttctatccatgttcaaacataacaggacatctttaaacaccttttttctttcttctatacttttctcctgttcctcctccaatgaaaggctggtttctgatccctcataacttggttcttcaccagagaactctgtggtttctgaattctcgaagtcctcttcaccatcatatccaacgtgctctgggtcatcataaacctcctcttccacagtggcttctgcatcttcaggggtgtcaacagatcctagatattcctcttttcctaagtataaagaatcatctagctcctcatatctctgtccatcttttatatatgtaatagttgctggaacttcacatccaactttctcaactgaatatgataatgtgacttctggtgtgtcatattccttctcattcttcctggcagacaaagctgtttccctataactagttttcttgtccctgaaaaactcagaggtttccaaatccaagtgttccttctcactgaagaacactgtgatctcaggggcttcaggctgttttattccaggagaaaaagcatcttctgaattactgcttgcccccatagattgaggaggtactgtattctcatgttttaaaacttcatgccttaagccgcaaatggcagctgactgtggaaaagtactaaataaacacttgagaaaatgctgacaggtcgcctctccctttttctgtaccaaaattaacagcttccgacttttcttcaggagatctgtaacattctccagagtctcatactcttcctcagaaatcagcctccgagaagttaacgtgtctaagatagaatcaggatcatgttgaaggatttcaagcaacttttttctttctctttctatgatctctgagggagtactctcggtagccattgttcctgtttcctct

SEQ ID NO: 18239 - RNA, 5428 nt, Homo sapiens
  source 1..5428: mol_type = other RNA
tgaagtaccagctactcgagaggctgaggcaggagaatcgcatgaacctgggaggcggagcttgcagtgagcggagagtgtgccactgcactccagcctgggcaacaaagcgagactctgtctcaaaaaaaaaaaaaaaaaaaaaacaaagattggattatgatattcagtatctatgtacacatcctatggtgggatggctatccaaaaaaacaagtaaaaagccaaaggtacagataaaatttcatttctgcggaaaagtaaagctcttactgaatggaacagggaagtgagaaactgcagccggcctggccaggcgcggtgccgcagaccctgtcacacagctgctcccagttacgcagcctctccctgtcacccgcagagagcagcatcggtggccgctcagaagccacgacctacaagtaacccttcagacacgttcaaagctcctcgccgagagcctatcaggcttttaagagttggtcattccatgtgaaaagctaattgtgatcttcgaatgtttttctagtccttggctctcattctgctatatattttacttcttgttaaaggcaaaacaaaacttaaatttcatgtcttagaaaaacatcgaccacacaatcaaataaataacattgataagagccttctggggcagcggcgcacggaggcgagtccacagcagtcactctcccggcccttctttggaagccctgctctgactgtgtctctgtgggtcgccgcgtgggccggcgtgaccccccgggggcacagggctggcagtggctggctccagcggcgtccacgaggacagagactcgtgcaccgtcagggcgtgctcctccatctggcgctgcaggctgtccatctcctgcttgagctgctggaggcagctgttcaggttcttgaggggctccttgctcacggcgggcggtggtctcagcagctcctccagcagcgaggcgggaactgggcagtccgggatcttgatgggcgtggcagggttggaagagctggcctcgcctttcggctcctttctcgtcttggccgcgccgcggcgtaggtccagcttgagctgctggttctgctggagcagggtcttcatgttgttcttcagctccgacacttttgcctggagcataaatttatccttctgggtcatggacaggtcttcctgggccatctccaactcagacttgacgttctgcagcagctgctgtagcccttccagttccttcctgccctgctgctccgtcaagtccagctgctgcttcaaggactggatttctctttctttctgatccacctcccatttgagattttccatctcttggtttcccacgggctgtttgctgagctgctcgtccagctgcttctgcaggagctggagctgtgcccgggcctcggccagctctgcttggaactgtgctatctcctgggaatgtttcccctcccgaatctgaaggtcgtcggcctcggcctgcagcttctgcaccaggtgttccttggcctgcagctccttcttcacctcactcagctccaaggaggccgccttgaagtggcggcggttatgcccggcttccaccttggcagcagccacctgctccttgaggctgttcaccttctccttctccttctctagtgaggcctgcagggcctggacaagatgcttcatctggcgatcctcctcttctttgcgctgcaaaactgcctgcacctgaaggttcaactggactaggtctgcctccctcttggccaaagctgtttctaggatgctgttgtgttcccgcagagctgcgttggactgaccgaggcccgtaagcttccctttctcgtgctctaattcaagagccaacttcttgtttgactcctcaaggcgttttatcttcttcctaaagcctctggattcttgaagctcgtcctccagctccagcaccttctcccgggactcctccagctcctggctggtcagcgctatgacctcctgcagttccttttccagcagcgtcttgctatgactgacagcctgcagctccgcctccagggcctggatcctttcatgtagagccaggctgctgtcactgctgccaccctgggctcggagctggcccagctccgcgtccgcagcctccttggccgcgagggcctcctgcaggcggcggctgaggatgcccacggcgttctcgtaggccttatgtttggtcttcatctccttctgggcgctggtcaagtctgagcccagccgcctcatcttctgcttctgttccgtgatggccttccgggcctcttgctgcaactcttcgatttgtttcttcagcgcctcattggcctctgtgaccgcgaccatctgctccttatcgaactgcaacgactgcaagtgtgtttccatctcgtctcgctccttctgcgccgactggagatgcccttcaaggtccgccatgtgctgacggacctgggccacctctctgtgcaggcgcgagagctccgcctcggcagtccgcttctccccgtgcacttgcatcagctcctgccgcagctccttcagctccgagtccagcctcttcctggtggctttcagctcactgatgagctggtctttggaggtggcgtcgcgccggtaggcctccaccatcaccttttgttggagaaactgttcctttattttttgcatttgctttttcagagcagcagtctcctgctgcaggtgttccacctggccggatttgatagctaattcttctcttaacttctctaaagtttccgacgtttcctcggtaccttcttccaagcgtcttgctcctctgtcaagctcctccttgccactcttggccgcctgcaaagccgcctccaagatgatcttctcgttctgcaggaggcagatcgtgtcctccctggaggcggcctcgccctgcagctcccccagcctggcctgcagctcatcgtagtgtgtctgcagggcatcgagggactgctccctgctctgcagagcctcctgagtcaaggtgagctgtttcatcaggtccaggtgctcctgctgcaaagcctcaagctgctggtctcgctggagtaaagtcaacttcacctgctccagctgctgctccagggatgccgccgagtccgccatcctctgcagccgctccctctcaccttcaaactcttccagcctcctctgaaggtcctcctccaccatcgtctttgcctcctgaatctgcatgaaggctgcttcctgatccaacatgtcagcctcaatgccctgcagctgtgccgcgatgcgccccttctccttcatggacctgtgctgagtttccgtcagctgctgggacagggacacattctcgagtttcaggtgctccaggagacctgcctgggtcatctgtccaacctggatgtgggccatctcaccctgcagcctgacgcgggcctcctgtgccagggcgagctgctgctggtaccactgccggacactctgcagggacgagatctccgcctgcgacgccttcagcttgctggtcagcgtcgtccgctccagctgcacctgctgaagctggctctgcaaggctgtcatctgctgtcgcaggtcgtgcactgtgttgtccttgctgagcatgctcctctgcatgtcctctaccttggccataagcctctggtactgctcctcggccacctgcaagtcgttgttggacgacgccaggctggcattttttgcctccagcatgttctgcaggtcagtcatggctcgctccaggtcccagcacgactgcttcagggtgtccacctccgagctcagcgaatcctgccgctgctggctgctgtggctgcactccacctgcgcctgcagcttcgtgctgagggcggccagctgggcctgcagctcagccttctctttaagtgcctgactcgcctccagtgacaaggcttccagctgtccttcgagtcgcattttctctttgagcacctgcagcatctcctcctgtgtttctgctgcagagctctccaaggacacgctgctgcagatgctgtctctccgactccgcacctccccgttgacctcctgcccctggtcttggtgctcagcggctgcggcctggaggacgtccttaatggaggggaactggcccagggtatccgcaggaatctcctggccgttgaccatatagggggtgtcctgcgtgcccactgtcttcgacagaatgccataggtccctcgggtggaggcgctgctgtacgatgagctgtcgctgtcatttccatccacctcagacacgctgtctccagccagggaggtgttctccagacggtcgtcagtgtcgggggacaggctgatctcagacacaacggacgccgcactgcttctgttctgcttcagggaacccttggtagaatcgggagccgggacatttcccccagaattccccgcatttgaatcttcagttctgtaatcggccagagaccggattttgcttgatttggaagtttttttctccctaggatgtgccggaagccccaggctgcccaccttaggcccccgagggacactggtgcgcaggaaggaatattcttttgtcatagccagggtactggcccttggtaagttttctgggtttaacatgagctcaggatcaagcgtgctaaaaagtctcgttttggttgcaggttgactggacctctcctgctggcgcttcaccctgtactgtttgagctgctcttccagccacttccgagcctgaagtcggacctgctcctccttctccaggggcaggggagaatctgtagagcacagttgcgtttcttgcataggaagactgagtctgagagactgcaaagcttcttttctaacactgccctcagcactagttccctgagacttccttaggttgtcatggaaaccagccacacctggagaggcatcagggcccactgggcttgtggtgggatcgagagacgacggagggtctgggaagggtggcgttggcccgttctgacagaggcctccctggccaggtccatccgggctttccccttccgtggatgctctgtttacctcggcacactggactttgtcctgctggtcaggtggcaccagtgggcccgggggcttcagtggggcctcggggagagacgaggggccactgtgggatctgtcctcctggaggccatcttgctcggccgacgcgccgtccatggtcaggacgacaccagctgagctgacgctgaggggctacaagtgaaccttggacaagcttggcttctgccatcagcaacagccaagagctcctgggaggggccctactgtgtctcccattttcaggagaagatctgatgactcacaaatgacttgatgtcaaaccagctaatatcatgatacccgtgacaacgcccggccccactcgctctggccacctggaatgaagacaagtcggccagcgac

SEQ ID NO: 18240 - RNA, 5468 nt, Homo sapiens
  source 1..5468: mol_type = other RNA
tgaagtaccagctactcgagaggctgaggcaggagaatcgcatgaacctgggaggcggagcttgcagtgagcggagagtgtgccactgcactccagcctgggcaacaaagcgagactctgtctcaaaaaaaaaaaaaaaaaaaaaacaaagattggattatgatattcagtatctatgtacacatcctatggtgggatggctatccaaaaaaacaagtaaaaagccaaaggtacagataaaatttcatttctgcggaaaagtaaagctcttactgaatggaacagggaagtgagaaactgcagccggcctggccaggcgcggtgccgcagaccctgtcacacagctgctcccagttacgcagcctctccctgtcacccgcagagagcagcatcggtggccgctcagaagccacgacctacaagtaacccttcagacacgttcaaagctcctcgccgagagcctatcaggcttttaagagttggtcattccatgtgaaaagctaattgtgatcttcgaatgtttttctagtccttggctctcattctgctatatattttacttcttgttaaaggcaaaacaaaacttaaatttcatgtcttagaaaaacatcgaccacacaatcaaataaataacattgataagagccttctggggcagcggcgcacggaggcgagtccacagcagtcactctcccggcccttctttggaagccctgctctgactgtgtctctgtgggtcgccgcgtgggccggcgtgaccccccgggggcacagggctggcagtggctggctccagcggcgtccacgaggacagagactcgtgcaccgtcagggcgtgctcctccatctggcgctgcaggctgtccatctcctgcttgagctgctggaggcagctgttcaggttcttgaggggctccttgctcacggcgggcggtggtctcagcagctcctccagcagcgaggcgggaactgggcagtccgggatcttgatgggcgtggcagggttggaagagctggcctcgcctttcggctcctttctcgtcttggccgcgccgcggcgtaggtccagcttgagctgctggttctgctggagcagggtcttcatgttgttcttcagctccgacacttttgcctggagcataaatttatccttctgggtcatggacaggtcttcctgggccatctccaactcagacttgacgttctgcagcagctgctgtagcccttccagttccttcctgccctgctgctccgtcaagtccagctgctgcttcaaggactggatttctctttctttctgatccacctcccatttgagattttccatctcttggtttcccacgggctgtttgctgagctgctcgtccagctgcttctgcaggagctggagctgtgcccgggcctcggccagctctgcttggaactgtgctatctcctgggaatgtttcccctcccgaatctgaaggtcgtcggcctcggcctgcagcttctgcaccaggtgttccttggcctgcagctccttcttcacctcactcagctccaaggaggccgccttgaagtggcggcggttatgcccggcttccaccttggcagcagccacctgctccttgaggctgttcaccttctccttctccttctctagtgaggcctgcagggcctggacaagatgcttcatctggcgatcctcctcttctttgcgctgcaaaactgcctgcacctgaaggttcaactggactaggtctgcctccctcttggccaaagctgtttctaggatgctgttgtgttcccgcagagctgcgttggactgaccgaggcccgtaagcttccctttctcgtgctctaattcaagagccaacttcttgtttgactcctcaaggcgttttatcttcttcctaaagcctctggattcttgaagctcgtcctccagctccagcaccttctcccgggactcctccagctcctggctggtcagcgctatgacctcctgcagttccttttccagcagcgtcttgctatgactgacagcctgcagctccgcctccagggcctggatcctttcatgtagagccaggctgctgtcactgctgccaccctgggctcggagctggcccagctccgcgtccgcagcctccttggccgcgagggcctcctgcaggcggcggctgaggatgcccacggcgttctcgtaggccttatgtttggtcttcatctccttctgggcgctggtcaagtctgagcccagccgcctcatcttctgcttctgttccgtgatggccttccgggcctcttgctgcaactcttcgatttgtttcttcagcgcctcattggcctctgtgaccgcgaccatctgctccttatcgaactgcaacgactgcaagtgtgtttccatctcgtctcgctccttctgcgccgactggagatgcccttcaaggtccgccatgtgctgacggacctgggccacctctctgtgcaggcgcgagagctccgcctcggcagtccgcttctccccgtgcacttgcatcagctcctgccgcagctccttcagctccgagtccagcctcttcctggtggctttcagctcactgatgagctggtctttggaggtggcgtcgcgccggtaggcctccaccatcaccttttgttggagaaactgttcctttattttttgcatttgctttttcagagcagcagtctcctgctgcaggtgttccacctggccggatttgatagctaattcttctcttaacttctctaaagtttccgacgtttcctcggtaccttcttccaagcgtcttgctcctctgtcaagctcctccttgccactcttggccgcctgcaaagccgcctccaagatgatcttctcgttctgcaggaggcagatcgtgtcctccctggaggcggcctcgccctgcagctcccccagcctggcctgcagctcatcgtagtgtgtctgcagggcatcgagggactgctccctgctctgcagagcctcctgagtcaaggtgagctgtttcatcaggtccaggtgctcctgctgcaaagcctcaagctgctggtctcgctggagtaaagtcaacttcacctgctccagctgctgctccagggatgccgccgagtccgccatcctctgcagccgctccctctcaccttcaaactcttccagcctcctctgaaggtcctcctccaccatcgtctttgcctcctgaatctgcatgaaggctgcttcctgatccaacatgtcagcctcaatgccctgcagctgtgccgcgatgcgccccttctccttcatggacctgtgctgagtttccgtcagctgctgggacagggacacattctcgagtttcaggtgctccaggagacctgcctgggtcatctgtccaacctggatgtgggccatctcaccctgcagcctgacgcgggcctcctgtgccagggcgagctgctgctggtaccactgccggacactctgcagggacgagatctccgcctgcgacgccttcagcttgctggtcagcgtcgtccgctccagctgcacctgctgaagctggctctgcaaggctgtcatctgctgtcgcaggtcgtgcactgtgttgtccttgctgagcatgctcctctgcatgtcctctaccttggccataagcctctggtactgctcctcggccacctgcaagtcgttgttggacgacgccaggctggcattttttgcctccagcatgttctgcaggtcagtcatggctcgctccaggtcccagcacgactgcttcagggtgtccacctccgagctcagcgaatcctgccgctgctggctgctgtggctgcactccacctgcgcctgcagcttcgtgctgagggcggccagctgggcctgcagctcagccttctctttaagtgcctgactcgcctccagtgacaaggcttccagctgtccttcgagtcgcattttctctttgagcacctgcagcatctcctcctgtgtttctgctgcagagctctccaaggacacgctgctgcagatgctgtctctccgactccgcacctccccgttgacctcctgcccctggtcttggtgctcagcggctgcggcctggaggacgtccttaatggaggggaactggcccagggtatccgcaggaatctcctggccgttgaccatatagggggtgtcctgcgtgcccactgtcttcgacagaatgccataggtccctcgggtggaggcgctgctgtacgatgagctgtcgctgtcatttccatccacctcagacacgctgtctccagccagggaggtgttctccagacggtcgtcagtgtcgggggacaggctgatctcagacacaacggacgccgcactgcttctgttctgcttcagggaacccttggtagaatcgggagccgggacatttcccccagaattccccgcatttgaatcttcagttctgtaatcggccagagaccggattttgcttgatttggaagtttttttctccctaggatgtgccggaagccccaggctgcccaccttaggcccccgagggacactggtgcgcaggaaggaatattcttttgtcatagccagggtactggcccttggtaagttttctgggtttaacatgagctcaggatcaagcgtgctaaaaagtctcgttttggttgcaggttgactggacctctcctgctggcgcttcaccctgtactgtttgagctgctcttccagccacttccgagcctgaagtcggacctgctcctccttctccaggggcaggggagaatctgtagagcacagttgcgtttcttgcataggaagactgagtctgagagactgcaaagcttcttttctaacactgccctcagcactagttccctgagacttccttaggttgtcatggaaaccagccacacctggagaggcatcagggcccactgggcttgtggtgggatcgagagacgacggagggtctgggaagggtggcgttggcccgttctgacagaggcctccctggccaggtccatccgggctttccccttccgtggatgctctgtttacctcggcacactggactttgtcctgctggtcaggtggcaccagtgggcccgggggcttcagtggggcctcggggagagacgaggggccactgtgggatctgtcctcctggaggccatcttgctcggccgacgcgccgtccatggtcaggacgacaccagctgagctgacgctgaggggctacaagtgaaccttggacaagcttggcttctgccatcagcaacagccaagagctcctgggaggggccctactgtgtctcccattttcaggagaagatctgatgactcacaaatgacttgatgtcaaaccagctaatatcatgataccctgctgctctggcagccccggaggccgcccggcccggatgctccggcggagacgtggccgtgagaggggcggggcgagcggtgcatcggcctcgggtccccg

SEQ ID NO: 18241 - RNA, 5478 nt, Homo sapiens
  source 1..5478: mol_type = other RNA
tgaagtaccagctactcgagaggctgaggcaggagaatcgcatgaacctgggaggcggagcttgcagtgagcggagagtgtgccactgcactccagcctgggcaacaaagcgagactctgtctcaaaaaaaaaaaaaaaaaaaaaacaaagattggattatgatattcagtatctatgtacacatcctatggtgggatggctatccaaaaaaacaagtaaaaagccaaaggtacagataaaatttcatttctgcggaaaagtaaagctcttactgaatggaacagggaagtgagaaactgcagccggcctggccaggcgcggtgccgcagaccctgtcacacagctgctcccagttacgcagcctctccctgtcacccgcagagagcagcatcggtggccgctcagaagccacgacctacaagtaacccttcagacacgttcaaagctcctcgccgagagcctatcaggcttttaagagttggtcattccatgtgaaaagctaattgtgatcttcgaatgtttttctagtccttggctctcattctgctatatattttacttcttgttaaaggcaaaacaaaacttaaatttcatgtcttagaaaaacatcgaccacacaatcaaataaataacattgataagagccttctggggcagcggcgcacggaggcgagtccacagcagtcactctcccggcccttctttggaagccctgctctgactgtgtctctgtgggtcgccgcgtgggccggcgtgaccccccgggggcacagggctggcagtggctggctccagcggcgtccacgaggacagagactcgtgcaccgtcagggcgtgctcctccatctggcgctgcaggctgtccatctcctgcttgagctgctggaggcagctgttcaggttcttgaggggctccttgctcacggcgggcggtggtctcagcagctcctccagcagcgaggcgggaactgggcagtccgggatcttgatgggcgtggcagggttggaagagctggcctcgcctttcggctcctttctcgtcttggccgcgccgcggcgtaggtccagcttgagctgctggttctgctggagcagggtcttcatgttgttcttcagctccgacacttttgcctggagcataaatttatccttctgggtcatggacaggtcttcctgggccatctccaactcagacttgacgttctgcagcagctgctgtagcccttccagttccttcctgccctgctgctccgtcaagtccagctgctgcttcaaggactggatttctctttctttctgatccacctcccatttgagattttccatctcttggtttcccacgggctgtttgctgagctgctcgtccagctgcttctgcaggagctggagctgtgcccgggcctcggccagctctgcttggaactgtgctatctcctgggaatgtttcccctcccgaatctgaaggtcgtcggcctcggcctgcagcttctgcaccaggtgttccttggcctgcagctccttcttcacctcactcagctccaaggaggccgccttgaagtggcggcggttatgcccggcttccaccttggcagcagccacctgctccttgaggctgttcaccttctccttctccttctctagtgaggcctgcagggcctggacaagatgcttcatctggcgatcctcctcttctttgcgctgcaaaactgcctgcacctgaaggttcaactggactaggtctgcctccctcttggccaaagctgtttctaggatgctgttgtgttcccgcagagctgcgttggactgaccgaggcccgtaagcttccctttctcgtgctctaattcaagagccaacttcttgtttgactcctcaaggcgttttatcttcttcctaaagcctctggattcttgaagctcgtcctccagctccagcaccttctcccgggactcctccagctcctggctggtcagcgctatgacctcctgcagttccttttccagcagcgtcttgctatgactgacagcctgcagctccgcctccagggcctggatcctttcatgtagagccaggctgctgtcactgctgccaccctgggctcggagctggcccagctccgcgtccgcagcctccttggccgcgagggcctcctgcaggcggcggctgaggatgcccacggcgttctcgtaggccttatgtttggtcttcatctccttctgggcgctggtcaagtctgagcccagccgcctcatcttctgcttctgttccgtgatggccttccgggcctcttgctgcaactcttcgatttgtttcttcagcgcctcattggcctctgtgaccgcgaccatctgctccttatcgaactgcaacgactgcaagtgtgtttccatctcgtctcgctccttctgcgccgactggagatgcccttcaaggtccgccatgtgctgacggacctgggccacctctctgtgcaggcgcgagagctccgcctcggcagtccgcttctccccgtgcacttgcatcagctcctgccgcagctccttcagctccgagtccagcctcttcctggtggctttcagctcactgatgagctggtctttggaggtggcgtcgcgccggtaggcctccaccatcaccttttgttggagaaactgttcctttattttttgcatttgctttttcagagcagcagtctcctgctgcaggtgttccacctggccggatttgatagctaattcttctcttaacttctctaaagtttccgacgtttcctcggtaccttcttccaagcgtcttgctcctctgtcaagctcctccttgccactcttggccgcctgcaaagccgcctccaagatgatcttctcgttctgcaggaggcagatcgtgtcctccctggaggcggcctcgccctgcagctcccccagcctggcctgcagctcatcgtagtgtgtctgcagggcatcgagggactgctccctgctctgcagagcctcctgagtcaaggtgagctgtttcatcaggtccaggtgctcctgctgcaaagcctcaagctgctggtctcgctggagtaaagtcaacttcacctgctccagctgctgctccagggatgccgccgagtccgccatcctctgcagccgctccctctcaccttcaaactcttccagcctcctctgaaggtcctcctccaccatcgtctttgcctcctgaatctgcatgaaggctgcttcctgatccaacatgtcagcctcaatgccctgcagctgtgccgcgatgcgccccttctccttcatggacctgtgctgagtttccgtcagctgctgggacagggacacattctcgagtttcaggtgctccaggagacctgcctgggtcatctgtccaacctggatgtgggccatctcaccctgcagcctgacgcgggcctcctgtgccagggcgagctgctgctggtaccactgccggacactctgcagggacgagatctccgcctgcgacgccttcagcttgctggtcagcgtcgtccgctccagctgcacctgctgaagctggctctgcaaggctgtcatctgctgtcgcaggtcgtgcactgtgttgtccttgctgagcatgctcctctgcatgtcctctaccttggccataagcctctggtactgctcctcggccacctgcaagtcgttgttggacgacgccaggctggcattttttgcctccagcatgttctgcaggtcagtcatggctcgctccaggtcccagcacgactgcttcagggtgtccacctccgagctcagcgaatcctgccgctgctggctgctgtggctgcactccacctgcgcctgcagcttcgtgctgagggcggccagctgggcctgcagctcagccttctctttaagtgcctgactcgcctccagtgacaaggcttccagctgtccttcgagtcgcattttctctttgagcacctgcagcatctcctcctgtgtttctgctgcagagctctccaaggacacgctgctgcagatgctgtctctccgactccgcacctccccgttgacctcctgcccctggtcttggtgctcagcggctgcggcctggaggacgtccttaatggaggggaactggcccagggtatccgcaggaatctcctggccgttgaccatatagggggtgtcctgcgtgcccactgtcttcgacagaatgccataggtccctcgggtggaggcgctgctgtacgatgagctgtcgctgtcatttccatccacctcagacacgctgtctccagccagggaggtgttctccagacggtcgtcagtgtcgggggacaggctgatctcagacacaacggacgccgcactgcttctgttctgcttcagggaacccttggtagaatcgggagccgggacatttcccccagaattccccgcatttgaatcttcagttctgtaatcggccagagaccggattttgcttgatttggaagtttttttctccctaggatgtgccggaagccccaggctgcccaccttaggcccccgagggacactggtgcgcaggaaggaatattcttttgtcatagccagggtactggcccttggtaagttttctgggtttaacatgagctcaggatcaagcgtgctaaaaagtctcgttttggttgcaggttgactggacctctcctgctggcgcttcaccctgtactgtttgagctgctcttccagccacttccgagcctgaagtcggacctgctcctccttctccaggggcaggggagaatctgtagagcacagttgcgtttcttgcataggaagactgagtctgagagactgcaaagcttcttttctaacactgccctcagcactagttccctgagacttccttaggttgtcatggaaaccagccacacctggagaggcatcagggcccactgggcttgtggtgggatcgagagacgacggagggtctgggaagggtggcgttggcccgttctgacagaggcctccctggccaggtccatccgggctttccccttccgtggatgctctgtttacctcggcacactggactttgtcctgctggtcaggtggcaccagtgggcccgggggcttcagtggggcctcggggagagacgaggggccactgtgggatctgtcctcctggaggccatcttgctcggccgacgcgccgtccatggtcaggacgacaccagctgagctgacgctgaggggctacaagtgaaccttggacaagcttggcttctgccatcagcaacagccaagagctcctgggaggggccctactgtgtctcccattttcaggagaagatctgatgactcacaaatgacttgatgtcaaaccagctaatatcatgatacctccgactgtgatgaggccgccttcagaaagtgaccttaagagtttgcggacctttccctagtagaaacgcaacttccggaactgcaggaccaactctttcaggaagctgaac

SEQ ID NO: 18242 - RNA, 6231 nt, Homo sapiens
  source 1..6231: mol_type = other RNA
tgaagtaccagctactcgagaggctgaggcaggagaatcgcatgaacctgggaggcggagcttgcagtgagcggagagtgtgccactgcactccagcctgggcaacaaagcgagactctgtctcaaaaaaaaaaaaaaaaaaaaaacaaagattggattatgatattcagtatctatgtacacatcctatggtgggatggctatccaaaaaaacaagtaaaaagccaaaggtacagataaaatttcatttctgcggaaaagtaaagctcttactgaatggaacagggaagtgagaaactgcagccggcctggccaggcgcggtgccgcagaccctgtcacacagctgctcccagttacgcagcctctccctgtcacccgcagagagcagcatcggtggccgctcagaagccacgacctacaagtaacccttcagacacgttcaaagctcctcgccgagagcctatcaggcttttaagagttggtcattccatgtgaaaagctaattgtgatcttcgaatgtttttctagtccttggctctcattctgctatatattttacttcttgttaaaggcaaaacaaaacttaaatttcatgtcttagaaaaacatcgaccacacaatcaaataaataacattgataagagccttctggggcagcggcgcacggaggcgagtccacagcagtcactctcccggcccttctttggaagccctgctctgactgtgtctctgtgggtcgccgcgtgggccggcgtgaccccccgggggcacagggctggcagtggctggctccagcggcgtccacgaggacagagactcgtgcaccgtcagggcgtgctcctccatctggcgctgcaggctgtccatctcctgcttgagctgctggaggcagctgttcaggttcttgaggggctccttgctcacggcgggcggtggtctcagcagctcctccagcagcgaggcgggaactgggcagtccgggatcttgatgggcgtggcagggttggaagagctggcctcgcctttcggctcctttctcgtcttggccgcgccgcggcgtaggtccagcttgagctgctggttctgctggagcagggtcttcatgttgttcttcagctccgacacttttgcctggagcataaatttatccttctgggtcatggacaggtcttcctgggccatctccaactcagacttgacgttctgcagcagctgctgtagcccttccagttccttcctgccctgctgctccgtcaagtccagctgctgcttcaaggactggatttctctttctttctgatccacctcccatttgagattttccatctcttggtttcccacgggctgtttgctgagctgctcgtccagctgcttctgcaggagctggagctgtgcccgggcctcggccagctctgcttggaactgtgctatctcctgggaatgtttcccctcccgaatctgaaggtcgtcggcctcggcctgcagcttctgcaccaggtgttccttggcctgcagctccttcttcacctcactcagctccaaggaggccgccttgaagtggcggcggttatgcccggcttccaccttggcagcagccacctgctccttgaggctgttcaccttctccttctccttctctagtgaggcctgcagggcctggacaagatgcttcatctggcgatcctcctcttctttgcgctgcaaaactgcctgcacctgaaggttcaactggactaggtctgcctccctcttggccaaagctgtttctaggatgctgttgtgttcccgcagagctgcgttggactgaccgaggcccgtaagcttccctttctcgtgctctaattcaagagccaacttcttgtttgactcctcaaggcgttttatcttcttcctaaagcctctggattcttgaagctcgtcctccagctccagcaccttctcccgggactcctccagctcctggctggtcagcgctatgacctcctgcagttccttttccagcagcgtcttgctatgactgacagcctgcagctccgcctccagggcctggatcctttcatgtagagccaggctgctgtcactgctgccaccctgggctcggagctggcccagctccgcgtccgcagcctccttggccgcgagggcctcctgcaggcggcggctgaggatgcccacggcgttctcgtaggccttatgtttggtcttcatctccttctgggcgctggtcaagtctgagcccagccgcctcatcttctgcttctgttccgtgatggccttccgggcctcttgctgcaactcttcgatttgtttcttcagcgcctcattggcctctgtgaccgcgaccatctgctccttatcgaactgcaacgactgcaagtgtgtttccatctcgtctcgctccttctgcgccgactggagatgcccttcaaggtccgccatgtgctgacggacctgggccacctctctgtgcaggcgcgagagctccgcctcggcagtccgcttctccccgtgcacttgcatcagctcctgccgcagctccttcagctccgagtccagcctcttcctggtggctttcagctcactgatgagctggtctttggaggtggcgtcgcgccggtaggcctccaccatcaccttttgttggagaaactgttcctttattttttgcatttgctttttcagagcagcagtctcctgctgcaggtgttccacctggccggatttgatagctaattcttctcttaacttctctaaagtttccgacgtttcctcggtaccttcttccaagcgtcttgctcctctgtcaagctcctccttgccactcttggccgcctgcaaagccgcctccaagatgatcttctcgttctgcaggaggcagatcgtgtcctccctggaggcggcctcgccctgcagctcccccagcctggcctgcagctcatcgtagtgtgtctgcagggcatcgagggactgctccctgctctgcagagcctcctgagtcaaggtgagctgtttcatcaggtccaggtgctcctgctgcaaagcctcaagctgctggtctcgctggagtaaagtcaacttcacctgctccagctgctgctccagggatgccgccgagtccgccatcctctgcagccgctccctctcaccttcaaactcttccagcctcctctgaaggtcctcctccaccatcgtctttgcctcctgaatctgcatgaaggctgcttcctgatccaacatgtcagcctcaatgccctgcagctgtgccgcgatgcgccccttctccttcatggacctgtgctgagtttccgtcagctgctgggacagggacacattctcgagtttcaggtgctccaggagacctgcctgggtcatctgtccaacctggatgtgggccatctcaccctgcagcctgacgcgggcctcctgtgccagggcgagctgctgctggtaccactgccggacactctgcagggacgagatctccgcctgcgacgccttcagcttgctggtcagcgtcgtccgctccagctgcacctgctgaagctggctctgcaaggctgtcatctgctgtcgcaggtcgtgcactgtgttgtccttgctgagcatgctcctctgcatgtcctctaccttggccataagcctctggtactgctcctcggccacctgcaagtcgttgttggacgacgccaggctggcattttttgcctccagcatgttctgcaggtcagtcatggctcgctccaggtcccagcacgactgcttcagggtgtccacctccgagctcagcgaatcctgccgctgctggctgctgtggctgcactccacctgcgcctgcagcttcgtgctgagggcggccagctgggcctgcagctcagccttctctttaagtgcctgactcgcctccagtgacaaggcttccagctgtccttcgagtcgcattttctctttgagcacctgcagcatctcctcctgtgtttctgctgcagagctctccaaggacacgctgctgcagatgctgtctctccgactccgcacctccccgttgacctcctgcccctggtcttggtgctcagcggctgcggcctggaggacgtccttaatggaggggaactggcccagggtatccgcaggaatctcctggccgttgaccatatagggggtgtcctgcgtgcccactgtcttcgacagaatgccataggtccctcgggtggaggcgctgctgtacgatgagctgtcgctgtcatttccatccacctcagacacgctgtctccagccagggaggtgttctccagacggtcgtcagtgtcgggggacaggctgatctcagacacaacggacgccgcactgcttctgttctgcttcagggaacccttggtagaatcgggagccgggacatttcccccagaattccccgcatttgaatcttcagttctgtaatcggccagagaccggattttgcttgatttggaagtttttttctccctaggatgtgccggaagccccaggctgcccaccttaggcccccgagggacactggtgcgcaggaaggaatattcttttgtcatagccagggtactggcccttggtaagttttctgggtttaacatgagctcaggatcaagcgtgctaaaaagtctcgttttggttgcaggttgactggacctctcctgctggcgcttcaccctgtactgtttgagctgctcttccagccacttccgagcctgaagtcggacctgctcctccttctccaggggcaggggagaatctgtagagcacagttgcgtttcttgcataggaagactgagtctgagagactgcaaagcttcttttctaacactgccctcagcactagttccctgagacttccttaggttgtcatggaaaccagccacacctggagaggcatcagggcccactgggcttgtggtgggatcgagagacgacggagggtctgggaagggtggcgttggcccgttctgacagaggcctccctggccaggtccatccgggctttccccttccgtggatgctctgtttacctcggcacactggactttgtcctgctggtcaggtggcaccagtgggcccgggggcttcagtggggcctcggggagagacgaggggccactgtgggatctgtcctcctggaggccatcttgctcggccgacgcgccgtccatggtcaggacgacaccagctgagctgacgctgaggggctacaagtgaaccttggacaagcttggcttctgccatcagcaacagccaagagctcctgggaggggccctactgtgtctcccattttcaggagaagatctgatgactcacaaatgacttgatgtcaaaccagctaatatcatgatacctgggaatggagaagacacccacaaaacaaggggaggagcatcagcaaaatgatggctgcttatcacaggcttgcccctttgacagatgaattacaaactggcacggaggactacacgcggtggaatgtggactcgactgcgccactgaatactggtaccctgtacatctggtcctcttgaaaatttcctagcaaaagaaaacttgcgttttgctttgtgatgtctttgcttctgccttgcgggggtggggtgattatatggaaccgaccgtgtgtgcctacgcgtgcagaccctcctggcccctcaggtaaaggaaccgacggtgtgtgcctgcgcgtgcagaccctcctggccccgcaggtaaagtgtctcgtctaccccctctgccatcactgtacctcacgtggcctccaccacagcacgtcatgtctgccattgcgtgtgtgcccattacatggcgagatccttgaagacagagactcattccccgtctgcctcccaccaccttgaacactcccaactcctaaagtgccaacacaggtttaatttgccgaattaaatcttcagttctgctgattctgctgagtacattcctctgctacaaagctaatggttccaaaacaaaatgattaagtatttgaatcctggagcatcaacactgccttttaaaatacagcaaagtctaaactagtccagctgaaacatctgtgagcttcagttccaatgagggagtccagggagttagaaactggaagagcaccttttttcagtggccgggaagatggcggacattcagactgagcgtgcctaccaaaagcagccgaccatctttcaaaacaagaagagggtcctgctgggagaaact
